European Patent Application EP 4 520 821 A1 - sequence listing, part 9

SEQ ID NO: 14452 - RNA, 2191 nt, Homo sapiens
  source 1..2191: mol_type = other RNA
gctgggattacaggcatgagccaccgcggccggcaggtctttcctacattttttatttccgtaaggagtctctgcagtgtgagttcttgtatgaaccatgaatttgagaccacgctgaaggctttgtcatattccttttagattcgcagtttctctccagggtgagaacaaatgtctactcaagatgaatgaagatgaaaggctttctgtagactttaccttcacagggttttttttcacatttctgtaagatacgagagttcagggaagatgttctcactcatgctaaccccttgagctcccttccaatatgtcctcctcacatgtttggtacagtcagaaaattaatgaaaaattttccaccttcctttcattcacagggcttctcatctttgtgagtcttaagatgttttttaagtcctgacgactttgcaaagtcttttccacatgtcttacatttatagggtttctctccagtgtggctccttatatgtgtatattttgaggactcccgaatgactttcccacattcttcacattcgtagggcttcttctgcacaacatgctttcttaaatgtttattaaggtgtaaggaatatctaaaggctttcccacatttcccacattcatacggtttctctccagtgtgaattttcatatgtctcataaggaatgactgataaaaaaaggctctcccacattcggggcatttatgggttttctctccagtgcaatgactcttgtgtgaaccggaatttggagcgttggcagaggttgccccagtttgacaatccttcttgtttgtctctgcggtatacaactgcatctgcatggcgtgaattgagttatttctggaggtgttctcgcactgagtaaaatcatacattttctctcgaccatgagtgttgtgtgccctaagggatccgtcttcacggaaagcttttccaaatggattccgctggtgcctgttggcccccgtatcaatttcatcacgtatatgatgcacagtgttctgactgccagtccatgtgcttgatttcagctctgtttttctcccacacggaacccactgaatgttccaccccaagactccatcgtcttcgttgttttcatgtgttttttgactatcgtttaagacaggattatacttgaaaatacttgagtcacgtgttaggatacattgtcttatggaatctccctgtgaaggcacaagcctgcaggtaggtttagagtggttcctcatttcatgatcttcacaaatgctaacaggagattcatctttctcaggggcaactgcaggtggcttcacattattcaccccctgcctgtgtggttcctctgttttggggcatctccagtcttctcttaatgtggagtgctgggaactgatgctcgtgagacacactctgttggcttcaggaaatgttcttttaggaagaatatccggctgaggggttgcgtctttggttttacatggagttgcccaatctatgaatgccaagttcctagaattttccagcatcacgtctctgtagagattcctctgagctgggtccagcagggtccactcctctttggtgaagttcacagccacgtctgcgaaggtcaccgagtcctgggacatatttgtcaccaacgtgacggccagtcctggcttccccgtgtttccttcaaggaggcaggtgaggcagagtcttccactagctccggcttccagatgtctctgtcggtggcgcagcccaaaagcgcgcgcagcccaggagcgtctcggagtccccaggcactcctgatccaagcaggaaaccccagccttgggtcctcgctgtcgcctccgcccgcgccaccgttcctaggctctccagctgggaagcgcgctctctgcgcagccaacgcgcctccttgcgggctccggagactccggccgcttgctggcttcctgcatttcccaaggaaagaaggcttttttttcccctcagtaccttgaaatgatttttttcttccttccttcctttcttttctttctttcttttttttttttgagacggagtctcgctctgtcgcccaggctggagtgcagtggcgcgatctcggttcactgcaacctccgcctcccgggttcatgccattctctcgcctcagcctccgagtagctgggactacaggcgcccgccaccaccctggctaagttttt

SEQ ID NO: 14453 - RNA, 4889 nt, Homo sapiens
  source 1..4889: mol_type = other RNA
gctgggattacaggcatgagccaccgcgtccagccttttatcatgatgaattttaaaagatatgctttaaaactgaaaattacaaaactttccttctgaaattaaggctgtattctttgcccttttaaactatggaggtgcctgttcctcctactatccatggtaaagatgcagacacaactttcctttaaaactgcttattgcactaaaagatagcaaaaacaagttgtcagttcttaaaataaacatgattatatttctataaaagatgctgccaatacaattctataattattaaagcactattctaataaatataaaagaaaaggaagctatacttccaaacacatacatatgtgtttatatacacacacatacatatatatatataaaaaatatatgaaaatcacattaaggtatgagaggcagcaagtaaactatcaaaaaacaaaacaaaaaaatccctcaacaaactcttctctctactcaatttcagaggtctcaaccctacagagctctaatcttttaaaatatttaccctttataaaacctttaaagaatttccatgtataacccatagaaacagaaggcttcagaatacacatcacttaccagagagaaagttacaacttctgacaggttttatatttatagcagctttaacaaactcactaaagaaaaagaatagtaggccgggtgcggtggctcatgcctgtaatcccagcactttgggaggtcgaggcgggtggatcacaaggtcaagagatcgagaccatcctggccaacacggtgaaaccccgtctctactaaaaatacaaaaattagctgggtgtggtggcacatgcctgtaaacccagctactcgggaggctgaggcaggagaattgcttgaacccgagaggcggaagttgcagtgagccgagatctcgccactgcactccagcctggtgacagagcgaggctctgtctcattaaaaaaaaaaaagaaagaaaagaaaaagaaaaaagaaaaagaatagttcaggttgctactgcttatatacaaattgcgcaaatggtaaatgtatgttctgagtgggaggggagagacgcactctcacagaaagttattttatgtatatatatgtgtgtgtctgtgtctgtgtatgtatgtatacatatatatataaaattttgtttcttaagacagcaatatcaagagttgagaactcagaattgtgtatgagataggagtcaggagtagggtatgcaaaataaaagtagaattctagtttgccatattttatattcaaacgaaccagatacatcaacatttgaatgtcactggtaggactgggaaaaaaatgtaggtgatgaaggcaagggaaatagagaaataaaggcggtagtgggggtagaataaaagggaaagaaaattccccaatggaatgaactctaaaatatataacagacacatatatatctattatcaatccagatctagatatatatgcatatgaagtatggatgtatatattttaaaaatacacagacaccttttacaagaatatatgaatgcacattaattttttgcacacataattctgaaaaatcactttgattattcatgaaggtgtgtattttttaaaccatcatttactttttctttacttttttttgcaaagatagttgtgctgccaagcaacttgaggtaaaggcattaaaagggttagactacaagaaatgaaaacaaaacaattgcgatacttcctataggagaccgcacaaaaagcagttggctggtttcatattgcataatgatgctgtgttccttgatgaagtaaacaatcttccttgtattaacataaggatcagaccttggcccccacacagtgttggtttctgtatggctggaggtgtccttactcaattgacttcactggaaacatacgttgtatgtcaattcatctttcagtacttcctctcagagaatatacttggactatttaagcgaagtacattgtgcgtaaggtatcttggtgaatctgtacagccttggcaagagcttgtggatctcgcccattgctttgtcctgaaacgtgacttccttcagcactgtcatgttctttgtccacaagatgatatctggctctaaatgctaccaggtgagcataatacgctggtgcaggtatagaaacagatcgtgtacagcgtacgtaagtgtggcagagctggtaagttagcagctgaagttcatctgcagtaaagcagttatcatcccataaaacatgatagtgtgaaggacgactggtaccctgtattccagcatggctacagaggtaaaaatcgaactcatatgggtgtgtaatgtctgtatcaactgttgttccagctgggatattgccacttcttccaaccctttctgtcctatcagcacaaaataatcgagtgtgatgtctcttctgaactacaatgtaggttattccaggttgatagtctttctccaaactgatgcaggcttctcgaattgctagtagttcataatataatacctgcctaaactgcccctctgaaacaccatcccgataaaagatgatacgagtaggcttgaaccgagttgacttataaaattgaataagaagttcccggaccatggaggccaagtcctggatgatctcctgtcggggtctctgaactcttactgtggcacagtatctgcttgggtgtgcatccatactacctacaacagcagcaatagaaggcttctttccatcaccagcaggtggatgagtgacatcggctcccaaaaagatcactggttgctggaacacagaaggtctttgatgaggtacaagaatattattgatccctccgagtttaacatttatctttaggcacaagtttgacagagtttgaggagatgtttttattacattcttgacttgaacacattgtgtagccatacccaaaagtgtgtctcctacacgtttcacttccgcatacactggtgtcttccccggcaggatgacgataataagctgtaggccagaatatgtgttcttgagatgccggaacatgggctctacgctgtctgccccctgtgcatatttgcagaagcatggctggccctggatgggcatccctgcatccttagaaatcttacgcagctggtctgtgaaacccttcaatatttcttctctgcactgcctctgtgtggcaaaacaagcgatagcccacattttgatttcaactcctgtgtggaattgtttccctcgcatgtcccatactccatggctcggtgttgctactgtccgattccgtcctccatactggagcataggtgctggaagtacgcgtccagttacatgagccatttcatcccgaactttaaattgaaactcctgaacaaatggatctgtttcataatttgcacttcttaccaatctgctaatttcctcttgtctatctggtgcagatcttgctgttgccttgatcatagtggaagtctgattgtctgttagcttcttgatacatcgttgccctgccacaatattacagacttctagtggcaggtaggtgtgtttctgttcctgcccgacttgcagacagggaaggtgcgggtacttcagctgaagagtatacttttctctgaaatactgcgctactgttctctccacagtttggccgttttctaactgtaaaggaaaggtttgatgactggcaggcctccttgttacattacaaacacggtatttccgtctcattgttccacaatgagtcacttcaaccttcaaaccttttatctctttggtgaattttacccgatgagaatcagtcagaggtcttggttgctcatcaatattatgaatatcaagaacttcacacatgaactgaattacaggttgtgctttgtagaaggcagtggcagaaacatcgatattaagcatcattttccacatggcaggccgaacagactgatggaatccaaaccacacttccctgccccctcccagagggtggtcatatccttctggagcggagaaaaatgaacgccccacaggtgtgtatttcatggagggcagatgtcgtagcaccacatcaacggcatggacagggttagtgctgattggcttgtctaattccagtggctcaggcaaggtccgtcctgtcagtacttcatgcagtaggtgccaactcacccgagagacaaatttgattgacaccttgaaaggtcgatcttttccaccttccccaggtaaagtaacgtctaaatctacccctgtagttgccacaggaagtggattggcggtgtaaagacttctttttccatcataaactggtctacggtctccaaatatagttactttaaaatgctgaaccattgagtcaaccacctccctgttcactctcctaggacacttgtctggtttaatatctacctcatagaggtagacatcaatctttgggatttcaacttgaaaacagttagccagcagtttaatgggtttgcccatggtgccatagccaggtcttctgggcaccatgagtaggggctgggccccagcgggtcctgcggagccgatttccattcatggagctggggggagtgcttcgagggagaacggagcccgccactggcggcaaggaggcggcccggggggcgacgcggcgcgacgcgacgggcactctcactcggccccgaggcgggggcggcgacggcttcccctgagcaaccgcactccgaaagctctgggccggaagagtcgcggacggaaaacggcacaggactaggcgagaggaaggggagatgtgaggcgcggacagaggggagtcccgtccggaagttgcatcgcccgcggccgccgacgctcccaccgctcctccacgactgcgggccgccgccgccgacct

SEQ ID NO: 14454 - RNA, 4631 nt, Homo sapiens
  source 1..4631: mol_type = other RNA
gctgggattacaggcatgagccaccgcgtccagccttttatcatgatgaattttaaaagatatgctttaaaactgaaaattacaaaactttccttctgaaattaaggctgtattctttgcccttttaaactatggaggtgcctgttcctcctactatccatggtaaagatgcagacacaactttcctttaaaactgcttattgcactaaaagatagcaaaaacaagttgtcagttcttaaaataaacatgattatatttctataaaagatgctgccaatacaattctataattattaaagcactattctaataaatataaaagaaaaggaagctatacttccaaacacatacatatgtgtttatatacacacacatacatatatatatataaaaaatatatgaaaatcacattaaggtatgagaggcagcaagtaaactatcaaaaaacaaaacaaaaaaatccctcaacaaactcttctctctactcaatttcagaggtctcaaccctacagagctctaatcttttaaaatatttaccctttataaaacctttaaagaatttccatgtataacccatagaaacagaaggcttcagaatacacatcacttaccagagagaaagttacaacttctgacaggttttatatttatagcagctttaacaaactcactaaagaaaaagaatagtaggccgggtgcggtggctcatgcctgtaatcccagcactttgggaggtcgaggcgggtggatcacaaggtcaagagatcgagaccatcctggccaacacggtgaaaccccgtctctactaaaaatacaaaaattagctgggtgtggtggcacatgcctgtaaacccagctactcgggaggctgaggcaggagaattgcttgaacccgagaggcggaagttgcagtgagccgagatctcgccactgcactccagcctggtgacagagcgaggctctgtctcattaaaaaaaaaaaagaaagaaaagaaaaagaaaaaagaaaaagaatagttcaggttgctactgcttatatacaaattgcgcaaatggtaaatgtatgttctgagtgggaggggagagacgcactctcacagaaagttattttatgtatatatatgtgtgtgtctgtgtctgtgtatgtatgtatacatatatatataaaattttgtttcttaagacagcaatatcaagagttgagaactcagaattgtgtatgagataggagtcaggagtagggtatgcaaaataaaagtagaattctagtttgccatattttatattcaaacgaaccagatacatcaacatttgaatgtcactggtaggactgggaaaaaaatgtaggtgatgaaggcaagggaaatagagaaataaaggcggtagtgggggtagaataaaagggaaagaaaattccccaatggaatgaactctaaaatatataacagacacatatatatctattatcaatccagatctagatatatatgcatatgaagtatggatgtatatattttaaaaatacacagacaccttttacaagaatatatgaatgcacattaattttttgcacacataattctgaaaaatcactttgattattcatgaaggtgtgtattttttaaaccatcatttactttttctttacttttttttgcaaagatagttgtgctgccaagcaacttgaggtaaaggcattaaaagggttagactacaagaaatgaaaacaaaacaattgcgatacttcctataggagaccgcacaaaaagcagttggctggtttcatattgcataatgatgctgtgttccttgatgaagtaaacaatcttccttgtattaacataaggatcagaccttggcccccacacagtgttggtttctgtatggctggaggtgtccttactcaattgacttcactggaaacatacgttgtatgtcaattcatctttcagtacttcctctcagagaatatacttggactatttaagcgaagtacattgtgcgtaaggtatcttggtgaatctgtacagccttggcaagagcttgtggatctcgcccattgctttgtcctgaaacgtgacttccttcagcactgtcatgttctttgtccacaagatgatatctggctctaaatgctaccaggtgagcataatacgctggtgcaggtatagaaacagatcgtgtacagcgtacgtaagtgtggcagagctggtaagttagcagctgaagttcatctgcagtaaagcagttatcatcccataaaacatgatagtgtgaaggacgactggtaccctgtattccagcatggctacagaggtaaaaatcgaactcatatgggtgtgtaatgtctgtatcaactgttgttccagctgggatattgccacttcttccaaccctttctgtcctatcagcacaaaataatcgagtgtgatgtctcttctgaactacaatgtaggttattccaggttgatagtctttctccaaactgatgcaggcttctcgaattgctagtagttcataatataatacctgcctaaactgcccctctgaaacaccatcccgataaaagatgatacgagtaggcttgaaccgagttgacttataaaattgaataagaagttcccggaccatggaggccaagtcctggatgatctcctgtcggggtctctgaactcttactgtggcacagtatctgcttgggtgtgcatccatactacctacaacagcagcaatagaaggcttctttccatcaccagcaggtggatgagtgacatcggctcccaaaaagatcactggttgctggaacacagaaggtctttgatgaggtacaagaatattattgatccctccgagtttaacatttatctttaggcacaagtttgacagagtttgaggagatgtttttattacattcttgacttgaacacattgtgtagccatacccaaaagtgtgtctcctacacgtttcacttccgcatacactggtgtcttccccggcaggatgacgataataagctgtaggccagaatatgtgttcttgagatgccggaacatgggctctacgctgtctgccccctgtgcatatttgcagaagcatggctggccctggatgggcatccctgcatccttagaaatcttacgcagctggtctgtgaaacccttcaatatttcttctctgcactgcctctgtgtggcaaaacaagcgatagcccacattttgatttcaactcctgtgtggaattgtttccctcgcatgtcccatactccatggctcggtgttgctactgtccgattccgtcctccatactggagcataggtgctggaagtacgcgtccagttacatgagccatttcatcccgaactttaaattgaaactcctgaacaaatggatctgtttcataatttgcacttcttaccaatctgctaatttcctcttgtctatctggtgcagatcttgctgttgccttgatcatagtggaagtctgattgtctgttagcttcttgatacatcgttgccctgccacaatattacagacttctagtggcaggtaggtgtgtttctgttcctgcccgacttgcagacagggaaggtgcgggtacttcagctgaagagtatacttttctctgaaatactgcgctactgttctctccacagtttggccgttttctaactgtaaaggaaaggtttgatgactggcaggcctccttgttacattacaaacacggtatttccgtctcattgttccacaatgagtcacttcaaccttcaaaccttttatctctttggtgaattttacccgatgagaatcagtcagaggtcttggttgctcatcaatattatgaatatcaagaacttcacacatgaactgaattacaggttgtgctttgtagaaggcagtggcagaaattcatggagggcagatgtcgtagcaccacatcaacggcatggacagggttagtgctgattggcttgtctaattccagtggctcaggcaaggtccgtcctgtcagtacttcatgcagtaggtgccaactcacccgagagacaaatttgattgacaccttgaaaggtcgatcttttccaccttccccaggtaaagtaacgtctaaatctacctgttcactctcctaggacacttgtctggtttaatatctacctcatagaggtagacatcaatctttgggatttcaacttgaaaacagttagccagcagtttaatgggtttgcccatggtgccatagccaggtcttctgggcaccatgagtaggggctgggccccagcgggtcctgcggagccgatttccattcatggagctggggggagtgcttcgagggagaacggagcccgccactggcggcaaggaggcggcccggggggcgacgcggcgcgacgcgacgggcactctcactcggccccgaggcgggggcggcgacggcttcccctgagcaaccgcactccgaaagctctgggccggaagagtcgcggacggaaaacggcacaggactaggcgagaggaaggggagatgtgaggcgcggacagaggggagtcccgtccggaagttgcatcgcccgcggccgccgacgctcccaccgctcctccacgactgcgggccgccgccgccgacct

SEQ ID NO: 14455 - RNA, 932 nt, Homo sapiens
  source 1..932: mol_type = other RNA
gctgggattacaggcatgagccaccgcgtccggccctcattttttattttcaattgaattagaattcaaatcaaagcataattctacttgattatagctcttgtgaaagattcttagggaaaagaataacatgaacgttaggatggcctttgtttgtagattggattttcatgaattattcccatggttaactgaaagttaaatgcatataaacaagagttggcaagggctgatgctgtacactctcaagaggctcccaagttttgttttgtttcttttttcatgagcacccagaatctttcctctcactggatccagattttattctcagggtatctaaccagatgatgcaacatctgtgctctcttttaagaacgtgagaaatgaagctttttcatttttccttgctttgacttctgggaaatctaatcaaaactgctcagactttccttttcttgtttgctttagaagacagcttgctggaagggttctgtggaggtctcccacctgtagtcccagctactcgagaggctgaggcagaatcgcttgaacccgagaggtgaggttgcagtgagccaaggtcatgccactgcactccagtctgagcaagagagcaagattccatcttatctcactaaatgcagaaactactgggagtgaggctgccataaatctcttctggagaattttactggccataaagaagacagagaagaccgcttgcacctcgcccgcggctccggaagcggctgcggccccgaccggaaagcccccagcatcgcccgaaggaatcgcggctggcctgcggctccggcccggcctcgggtaccacgcgcctagtgggaagccgcactgacgcctgcagcatctcgcgagatttcgggctcagcccaagtactgcgagttcaccaaagcggggggaaaaaaaaaaa

SEQ ID NO: 14456 - RNA, 1167 nt, Homo sapiens
  source 1..1167: mol_type = other RNA
gctgggattacaggcatgagccaccgcgtccggccctcattttttattttcaattgaattagaattcaaatcaaagcataattctacttgattatagctcttgtgaaagattcttagggaaaagaataacatgaacgttaggatggcctttgtttgtagattggattttcatgaattattcccatggttaactgaaagttaaatgcatataaacaagagttggcaagggctgatgctgtacactctcaagaggctcccaagttttgttttgtttcttttttcatgagcacccagaatctttcctctcactggatccagattttattctcagggtatctaaccagatgatgcaacatctgtgctctcttttaagaacgtgagaaatgaagctttttcatttttccttgctttgacttctgggaaatctaatcaaaactgctcagactttccttttcttgtttgctttagaagacagcttgctggaagggttctgtggaggtctcccacctgtagtcccagctactcgagaggctgaggcagaatcgcttgaacccgagaggtgaggttgcagtgagccaaggtcatgccactgcactccagtctgagcaagagagcaagattccatcttatctcactaaatgcagaaactactgggagtgaggctgccataaatctcttctggagaattttactggccataaagaagacagagaagaccgcttgcaccttggaacatcagcttttaaaataaaggtgtcatcagaagtgtgtagacacccactgcatcacaactggaactgatctctggttatgccaatctaggtctgcctggcagggtgagtctaccgctcgaaagctgcacagaggaaatcctccctcctccaggttcaggcccggagttacgagcggagattcgcggcggcgggtcagagcccagagcaaaccaggctggggaacgcacctcgcccgcggctccggaagcggctgcggccccgaccggaaagcccccagcatcgcccgaaggaatcgcggctggcctgcggctccggcccggcctcgggtaccacgcgcctagtgggaagccgcactgacgcctgcagcatctcgcgagatttcgggctcagcccaagtactgcgagttcaccaaagcggggggaaaaaaaaaaa

SEQ ID NO: 14457 - RNA, 3334 nt, Homo sapiens
  source 1..3334: mol_type = other RNA
gctgggattacaggcatgagccaccgctccaggccttttctaaatacctattctttatttctatacttaccatgtcatagacaggtaacagtttatgggctggcagtggcccaagggccatactctggggggcactgctttagagaaaggtggcaggatagcagaaaggaaggaggggggtgactgttttgttaatggaatggcacatacagcctccctgaagaggggacatttgaagaagatatcagtaagggatggtcaaggaagattcagccaagtctagctgaaggcaatgactggaaagaagaaaaccctttcccatttgtcacctctggaatctgactgctgagggaaggagtctcaccagatcctcaaggaccatagcgctgcacactgctgcattccccctccctgctgggaagcttcctgacctcttagccaagccagcacctccccgtcctaggacctgaggccaggccacctccaggaacccctgagcctcagtgtcttatctttaaaatggggacaataatacttggctattgcagagatgaaagaagaaaacccatttagggagcttggcatcacgcctggcccacaggaaatgtgaatagttatttatcgctggctttctctgtttctagctctgtttctgaactagagggagaggagacacagatgtcatgactccagtccttgggaagctgagggtctagtgggggagtggcactaactcattcccaaaaaacagagggcaattcgtactcagggagtggcagtaatggggtgtgacagatgaggaatgaccaggcatttacaaggtgctctcccacatatcccatcttcctgcagctctgggtgtagcaaggagaggcgggtgtgggctggtgctgggtttgggcgtctcctgagaaggtgagcctggaccctaggagaggagaagtcagaggcagatggagcaggggctgggaccaggggtgcttgtttcttggccacatatgggctaggtcaggaattctcaaccttggccgcacactggaattttctgggatgatgtccgggcctcatgcctcacccatattaaatcagaatctctagggaatggggctgaggcctgggtattcttctaaagctctgtgggtgaatctaatgtgcttcccagcattgcaaacttcaagggtgagagtaagaagggtcaactctctacttcccaccatcaagcccatcaggcccaccaagcctatcaggcccttcaggccctagcgggtaggttcacagggccctgcaaatgttgtctctctgtctttctgaagaacagacaggctcagagccctctgaatgtgtccctcctgccccaggaaaccttcatttccatctcaggttcatcctcttctcaaggttaaatccaaagtgatcggtccttatccacttctgggaaaccattcctagccgacttcacagggtggcggggccagcacacctccgcagctgtgcctctcccctcacctgcccagtgcaccttctgggctgtctccctcctctgttttctcagggtcctgtgtggcctcctggaggctgccatcttgactccctgggactcagtgagtgcttggtggctgccccgcccccctccgcgatctcttgctgggccacactgtgacccatggcactgccccctccctgatttctttctgggccacactgtgatccatggccgcgcaccaggagatgggcacagtttccacttggctgccaggactacagaggaattttccaggagattatccaccagcttctttgggctcatggtcaatatcaaattccaggattcattgttgatctggaaatggcattcatcttttgaagactgttttctgtgaccatgggcccatacttaatctgaggtgagtggtatctgtgtatctaggatggcttggtttttgtaatctgcactaggaaggtaccatctatcgtgctgttctggaagaagccatctgaggcagaggcatcaagcatgaggctgaggacaatgctgaagggctggagcagctcttacccaagctaggtgggcatcccggggggatattgggacttggcagtttgttctccacctggctcctgggctcctggccctgagaacgtcctccagcccagctgcaggaggggagtcctgagccagcttctcatcttcctttcctctgcagccacatcctcttatgtcctacttggaccctggtactctggtcattcattcaggcaacacagaaatatcaagcatttgatgcaagccaggcattgccaggtgctgaaaaaacaaaaataaataaaactccattttgaccctcttggctgtcagacactagcagggtgggtcatgggcaagcagtaagtgttacaacacggtaagtgttttggttgaagtagcaaacaatatagtggaggagacaatatatagtagcaaactatcgtggagaatcagaggtcagacagccactgattcaattctggttcccttaactagctagatgacttaagtcaagttacttaacttcttggagcctcagtttccccaccagtaaaatggggttcttaactcttcctcatagttttgttgtgatgactcggtgggctaataatcacagacttattaaagtgctggcagttgatgaagtcttttaagcaacatggtgatcacatcatctggtcagatttgctcacttttccataagccagtgattctcagacatcactgtgcattaaatcactgttgtatgctaatgaggtgattcagggtggatctctaggtagtttcaggactggggctggttctgggtctcggagaggttcagctggcgggccagctcagtgcgctcgcggcccaccacatactggcagcgctggaactccatctccaggcggtacagctgctcggcagtgaaggatgtacgtgtccgcttgggccggtccaggtccaggcccttaggcaggacaatttcccgaattgtccctttggcatctcgcaccagtatgcggcggcagtggtctgcctcgccgggcccgggctgcccgtcgctgtcggctccactctccctggagcctgcgggactggaggctgaggtcccggccacctccgttgggctgtggccaccgccatcagctcgcaagtcccccgctccgctgcggtctccgcagcgcccaccgccgccaccagactccgcccggcgcgcggggccccggtcgcgctcggcgcccccatcgcccatgctgaccgccactgccaacccctctacggcggagccagcctacgctggccgggagcgccgctccccgcccc

SEQ ID NO: 14458 - RNA, 2874 nt, Homo sapiens
  source 1..2874: mol_type = other RNA
gctgggattacaggcatgagccaccgctccaggccttttctaaatacctattctttatttctatacttaccatgtcatagacaggtaacagtttatgggctggcagtggcccaagggccatactctggggggcactgctttagagaaaggtggcaggatagcagaaaggaaggaggggggtgactgttttgttaatggaatggcacatacagcctccctgaagaggggacatttgaagaagatatcagtaagggatggtcaaggaagattcagccaagtctagctgaaggcaatgactggaaagaagaaaaccctttcccatttgtcacctctggaatctgactgctgagggaaggagtctcaccagatcctcaaggaccatagcgctgcacactgctgcattccccctccctgctgggaagcttcctgacctcttagccaagccagcacctccccgtcctaggacctgaggccaggccacctccaggaacccctgagcctcagtgtcttatctttaaaatggggacaataatacttggctattgcagagatgaaagaagaaaacccatttagggagcttggcatcacgcctggcccacaggaaatgtgaatagttatttatcgctggctttctctgtttctagctctgtttctgaactagagggagaggagacacagatgtcatgactccagtccttgggaagctgagggtctagtgggggagtggcactaactcattcccaaaaaacagagggcaattcgtactcagggagtggcagtaatggggtgtgacagatgaggaatgaccaggcatttacaaggtgctctcccacatatcccatcttcctgcagctctgggtgtagcaaggagaggcgggtgtgggctggtgctgggtttgggcgtctcctgagaaggtgagcctggaccctaggagaggagaagtcagaggcagatggagcaggggctgggaccaggggtgcttgtttcttggccacatatgggctaggtcaggaattctcaaccttggccgcacactggaattttctgggatgatgtccgggcctcatgcctcacccatattaaatcagaatctctagggaatggggctgaggcctgggtattcttctaaagctctgtgggtgaatctaatgtgcttcccagcattgcaaacttcaagggtgagagtaagaagggtcaactctctacttcccaccatcaagcccatcaggcccaccaagcctatcaggcccttcaggccctagcgggtaggttcacagggccctgcaaatgttgtctctctgtctttctgaagaacagacaggctcagagccctctgaatgtgtccctcctgccccaggaaaccttcatttccatctcaggttcatcctcttctcaaggttaaatccaaagtgatcggtccttatccacttctgggaaaccattcctagccgacttcacagggtggcggggccagcacacctccgcagctgtgcctctcccctcacctgcccagtgcaccttctgggctgtctccctcctctgttttctcagggtcctgtgtggcctcctggaggctgccatcttgactccctgggactcagtgagtgcttggtggctgccccgcccccctccgcgatctcttgctgggccacactgtgacccatggcactgccccctccctgatttctttctgggccacactgtgatccatggccgcgcaccaggagatgggcacagtttccacttggctgccaggactacagaggaattttccaggagattatccaccagcttctttgggctcatggtcaatatcaaattccaggattcattgttgatctggaaatggcattcatcttttgaagactgttttctgtgaccatgggcccatacttaatctgaggtgagtggtatctgtgtatctaggatggcttggtttttgtaatctgcactaggaaggtaccatctatcgtgctgttctggaagaagccatctgaggcagaggcatcaagcatgaggctgaggacaatgctgaagggctggagcagctcttacccaagctaggtgggcatcccggggggatattgggacttggcagtttgttctccacctggctcctgggctcctggccctgagaacgtcctccagcccagctgcaggaggggagtcctgagccagcttctcatcttcctttcctctgcagccacatcctcttatgtcctacttggaccctggtactctggtcattcattcaggcaacacagaaatatcaagcatttgatgcaagccaggcattgccaggtgtgttgtatgctaatgaggtgattcagggtggatctctaggtagtttcaggactggggctggttctgggtctcggagaggttcagctggcgggccagctcagtgcgctcgcggcccaccacatactggcagcgctggaactccatctccaggcggtacagctgctcggcagtgaaggatgtacgtgtccgcttgggccggtccaggtccaggcccttaggcaggacaatttcccgaattgtccctttggcatctcgcaccagtatgcggcggcagtggtctgcctcgccgggcccgggctgcccgtcgctgtcggctccactctccctggagcctgcgggactggaggctgaggtcccggccacctccgttgggctgtggccaccgccatcagctcgcaagtcccccgctccgctgcggtctccgcagcgcccaccgccgccaccagactccgcccggcgcgcggggccccggtcgcgctcggcgcccccatcgcccatgctgaccgccactgccaacccctctacggcggagccagcctacgctggccgggagcgccgctccccgcccc

SEQ ID NO: 14459 - RNA, 2208 nt, Homo sapiens
  source 1..2208: mol_type = other RNA
gctgggattacaggcatgagccaccgctcccggccaaaacttttctttttaaaataagtttagttttaaaaaagtgagttgacaggagcaaaactgctaagtaaataatgcaaaaggcagtggtgctcaaatatgggaaaataatatgcaggtgataccagagtcttgcctttgggaaatgcagacccaggtccttttgtctttagagctcaccggcaatgcgaggtgtttcaggtagaaggaacagcatcaatggggtgttggctagtgtttaacagctggctctctgaaaaagcaaaataaaacacacacacaccaaatctgatggtctgtttccatgatgtgagtacctccagctgggccgaactgacatcactgaacacagtggaaagtgatgactgcagttgtctctcctgggagcttcaacacagtacaggctgacaaaagtgggcagggggtaagggcaggtggtgggagtggcctctacgccagagaagggaatggagaggtcaggctggctagagagtggggttgagtcgtccatgcccttgaatgccaggatgagggctaaagagtcaaatggaatgggtgacttcatatgcagaagtttttacaagagaagagaactcagtttggccaagagaagtggggtcgtcatgttggtaatcacgtaacagtgatcgttcagtcatgcggaatgctttcaaggtgttggacactgttcattttttatttttagtttttgaggcagggtctcactctgtcgcccaggctggagtgcagtggtgcaatcttggctcactgcaacctctgtctcctgggttcaagcgattcttctgcctcagcctccctagtagctcggattacagttgtttgccaccacgcccggctaatttttgtatttttagtagaaatgaggtttcgccatgttggccagactggtctcgaactcctgacctcaaatgatccacctgcctcggcctcccaaagtgctgggattgcaggtgtgatccaccacacctggccgcttgcagggtgttggacactgtggatatcacctcattcattctcctaacaacccaagagaagaggaactgaggcaaagagaagttaagcaagttgcccaaggccatacggctagtaaacggcagaacgaggctcaaacccaggcactctggctctagagtgtgtgttcctaaccactgtgctctagcacctcggaaccttagtctcttcatctgcaaaatcagcactgaggtgacaaggccaacgagcagagggttggagttacccagaacaacaacaacaacaaaagtaatagtaacacatatttggtcaaggcttagattctggcgtcatggggatctgggttcaaatcctaattctgccttagccgattagggtccctatcctcttaaagccttggtttccttatctgtaaaatggggatatcatgaagctgttagatgttaaatgagaaaatgaatgagaaaattgcatgtactgtccataaagttgaaaagataataggggtgggaaggagaacagtccgagtttgaatgcaggtgggccctggggcattgtctggactgaaggacaagggtcagttgaattgccaaagagctctgagactggctgaagggacactcgtcttgtgctagctgctaagaccaaggggaagcctgtgcctcgcccgaattttagtcttgcaaacagctgctcacccagtaggagagaattgtgataaaactcatagccaccatttcttgaatatctactatgccccgggacacagcagactattttagagaatttgcgaaggaaacacagtgacatctgttggacaccttgcaaactaccagctcaggatagttaaatttgaatgttagatggagggaacttcctttccacaatgacatgattttgtaaagctgagtgtatggcagttgtcatgattaaaagcaagtgccatgcagaagttattgtgtaacaggaaatgagattagatagcgtccaatctaatctcaaggtttgagtagctgtggacagcccaacaggcacaggcctcccgttagtacatccatacgagaagttaagaatgagtgaaaatagtttttttttttttaatttatgtgcattatttttttcaagcagctaccttgttaggacatacttaatagttatcttggcctacctactgcacttact

SEQ ID NO: 14460 - RNA, 536 nt, Homo sapiens
  source 1..536: mol_type = other RNA
gctgggattacaggcatgagccaccgctccgggccccaccgggtactttttaaagcctttttcttacaaggaagtgcaggccggcctaggagaagtttccagagcccgactgcagtttagccaagcagagaatctttgtcagtccacactgtttaaggaaagaggagacattctcgtttccctccaacaatataagtccattttcttgttgggtggcctttcgttcattaagaaccagctggattttctgttgggactggatagaagaggacatttcgccgcatggtgctagcagttggacattcgaagaggagagactcttcagaagggcagacactcacgagatcatcaaccacggctccctcgctgggaggcagacacagagctggaggcggcggccacaaactaggtgggcagagaggcgtcagcatcgggacttgcgggaggcccctgtgacacagaaaccaccagaagaaaagggaacttcaggaagtaagcggtgccgccggtttcaatcctgttcttagtctttgcag

SEQ ID NO: 14461 - RNA, 1701 nt, Homo sapiens
  source 1..1701: mol_type = other RNA
gctgggattacaggcatgagccaccgctcctgccctatataaagtatcttcttgtatatcttgtctgatttaagccatactctttcacacttctccctcctccttcatttacctaggatgactatataatttatttttcacagcagggcacttttcagaatggaagtggacactactcatcatgatgccagaatgatgggtatcattcactactcataattcaggactaataataatgggtattatttgggttcatttcaggcaaactaggatgcagatgacagcttcttcctatcatttcccaccctgaccacccaaggctgaggtccaaaatcaaaaaagaagtcaataataaactcatatctgtttattctccccaaatcaggggacacaaaggcttttttttttttttctgatgagtgggtaatcctaaaataagcaggaaatgcctgtggctcagcctaactcaaggtgagacgaagctggagctgggagctcgaaagtgtcccccagctccctcctcactttgcctgtaactccacctctgcagaaggtaaagtagaattggtagctgtgtcactggtttgggttgagtcctcggtcagggccctctccagactggcgggaagggcgtggatcagcctctcccggaagtcctggcccatgaagacatagagcatggggttgaggcagctgttgaagaaggccagggcacttgtcacatccactgcaataccaatttctttgtacatgccttgcaataactcacggattctgactgtggctataagggccaccacctgatatggggaccagcagagaaaaaaggctgctgcgacaaaggagaggacccgtaagggacgactggacttaatcaagccttgcttgtggatcttggtggcaataagcccataactgacagcaacgatggacatgggtgcgctgaagccaatgatgaaccggatgatgcctctcaccgtcaacatggcaacggccacatttatcctctctttagggtcgttggtccagggcgaaaagttaaaagtgcaggctactgtccccgttttaccaggtactgtagtcacacgaatgataactggcaatgtgaggagcagagccatcacccagggcccaatgatcaccttcttggccaggctcacggtgcggtggttctgggtccagactggatgcaggacgcaaacacagcggtccagagcaatgagggcgatcaggaagacacttccgaacaagttgatgtccactatggtaaagacgaatttgcacaggaaccagccgaaaggccaatgtcctcccatggccttcctgaccatgaagaatggcaaagtggaggtgaaacagaagtcagccacggccaggttcaggtaactgatggtggtgactgtgtgtgtcatccggaatccagccacccagatcacaagcccgttgcccaggaccccgaggacaaaggtgactgcaaataccagataagtgatgatatccaggaagagatagccagcagatacagcaggtgtccctccagagatgttcgtggggagagaggaatttgtctccatcttgtctgctccacatgtggttttcaagcacttgaattgtggctagtccaactggagacaggctggactgttcaccagctgtggtcttgctctgggtagttctaggtctgggtctcctggggagagt

SEQ ID NO: 14462 - RNA, 1190 nt, Homo sapiens
  source 1..1190: mol_type = other RNA
gctgggattacaggcatgagccaccgctcctggcccttgtgcatattcttaattgcttccagctatagccaagctgattctggatgaacctcttccacattctgatggcttcagccttttcaacttgcgcctgtgtaacttcaatcattgtacccttcttcacatgggattcttctcttctgcttcatatcttctcctcctctgaattattccatctcaaaatctttagcttaattatatcttctttttttctgaggcacacagtgtcttgatccttctactttctaaatacatctctttgtatctttcatggctctctttttgcttcattctttccatttatttttctcattttttctatctttggtgtatagaccttgactttactgtaggttgcttttgagaaacgatgattttcatttttcatgaagagtaaatttttggaagcgagacagtgcggctcacccagtcatggcctctgttctaccagacttttagtttttcatttgtttgtagtgatcttctggatttttagaacgctggagtcattgctgacatcttggtccgtttctgctcccacatccacagcatgaatccttatgttctcagttggttaaaattgtgtgtaggtattggcggaagcttgtctgaccagctttgcctcttgaccaggacgctctgcattccttggctggtgaaagacaggatgatgaatcaggtatcccactggacttttggaagaggatcttaaagtctggatggatctaggtctttattaatgcattgcaattcttttgttattctttgatttcttgattgggccaaatttgactgacgtcagttcttcacatgggaagagcagcatggactgtaagcatcataaggaagatcttgagggatttacttttctcctgaatgagatcaagatgagttctcaggaactgagggccttatgaggtggaaagagagtgctgcatctttaaagactaatcagatgacaaaggagaccaaaaagagggtagcacacatttatatcaacacagctacacagttctgacagcactagagcacaaggaacaggagtcctccagaaaaaaaaagaagtgaaaacaggggaaattcaattactaatgggtcattcttgtgggaactccgaaccattataagaaagaaatggatgacacctctca

SEQ ID NO: 14463 - RNA, 7041 nt, Homo sapiens
  source 1..7041: mol_type = other RNA
gctgggattacaggcatgagccaccgctcctggccggaatgctttagagtgtaggaacacaaataacacactgtccagacacaaactggtataatgagccattggcttcatatgaaattcacttcgtcttacatttctcccttgttttaatatggaaaacaattaaatgacatttaaatagtggggtctcttgagctcttctttttcccagtgaagaaaaacactttcatttatgacctatttcaggcaacatggataacaacgttagaaaaatagcaaatgaccattatggttgggtttatttcaaatgtagttgagaggttaggctgtctttggagcctgcagctgtttttctgacaacatgaagttttctgagatatgttttcactgaatgctaaaagaaactggatatttattttgatacaaatcaacgtgcctttggggtgttatgtttctgccccaggaggattactatgggtgaaggagaagtactatgttgcccttgatccctaacaagcaccatcactctctgcagcttcctagtgtggtcccgatggacaatcgaatgcaaaggaacttgaactccatgattaagaaaggaaaaggaaaaaaaaatgtgaaaaaaaaatatcaaagttttaaaaaaagggtttgtctgccaagcaaacaaaagtcatggctttaacaaaagtcatggtatcatctacacatttttttttcctttgtgaagaactgtggctagactaaacaaaacagaacagtacagaactcagggattcaaaccaaggtaatatgtccttcttccctttctccagttggcattgccacattctacataagacaatgggggctgaagcctcatccttcatgctacctcaatcaagaagctttctttcttggacatgtgcacaagtttgtccttcttgtggtgtgagtattcactagggatgctccccctcctaaacttctcttgagttgagcccacaatccccacaaccattgggatgcattgcattgcatcagcagcaggtgttttcttgctgttgttaatcgttagaagtgtcatatttgcaccgtatgtctaggctagttccggctgatgggactgatgccacatgtgaatcatgagttgaatgtataaaaatttcagctttgccactgttgtcctttggatggatattatgcacagggaaaagtagatggagaggaaaacaaagagttgatcagctcctagttctggagttggttattagaaattataaaaaatggtggctctgctcagaagacatgggcatatgaaagcctggagtgcttaatgctcacattttcccttcaatgatagaaatggaagtaaacatttattaccatttggtcaagtgtagcttaacttgcattcatatttcattgttagtaatggaggtatgtggagatatacacagaccttgagacagctgttttttaatattgcatacaggctagcagttcattgaaaacagaggagagaagcctgaaggttagatcttagaagaaggcagttcttcatgcacagcttttgtcaatcctgatttggtttgaaaataaaaatcatggaataccaaaatcaaaggagagttgattaagggaaagggaaaaggggatcatcccaggaagggtgatgtcactggccaggaaaatgtcaggcgaggttccatgtcctcactcaagtccaaaggtgctggtttcctctactgctgttaacagcttttcatacaacatggagtacgagggatacggtggaagatccagtcggttgaagcatgtgtgtgccctggggagagaagtaattttcccccatttctctatgcagaagcgccgaagcccattgctcccacggagggctgcgaagccttcgtagggcacgctggatgttcccgtgacaaactgcagtaatctcagcctctgctcattattgaagcgctccaccgcagcccagaaccagcggatcacaagatgcccatcgtggtaacctccccggtactcagtgttattccgccagtcatttaggtcgatttccgcggtgccagctatcaccagctccagctccctggcatcaaacacggacaccagcctcgagtctacaacctcgtagaagccgcgcaccagcgcctcggtctgctgtaccacgccgcgctccacccgccacttcaccatgcgctcgatgtactccttcttgtttttctccgtcacctgtgtgttggctcctccagacttcaactccctttccgtgacctgtccaaaaacctcttcattaacagtgaaagtgaggtctaagatgtctgtgatgttgttgtccttcatccactgcaaactctggtggaattcctcatccaaatattccaggtcactcaaatcacagggcagtctcaggagtgccttgtagaagggcctcgtgaagaaagcgtcaagaaggtactgatggatcagagccagacccaggatgcgaccgctaaacctgaaccactcaagatggttttctacaaatgcggacatggggctgatctgcaccgtgtaagtatcatttgccgagtactcaaagagtccatagtaagggttgaagagctcctgagacagaaggaagaagaactcccgcgaggggccactgtagtccaggccctcctctccaacaaaggtgacgtagagcttgtttcgctggagctctttccgcgaataggccatcacctgattgaaggttccctccaacaaatgatcccggcgaataatgagcttaattttccccggaccctgaccaaatcctttggcttccagttttctgtagaaattgcggagcttggcctcaaagtctcttcggtagggggaaggggctcttgcactggctctctgtaaacctggggagttctgaggtgaagaacagggtgaacatcggggagagaagctatacccagggtggaaggcagcctgcagggggacgtaggacataatctcttcttcaaagagactcagcaaaatgaccagatccgcatcacaggacaacttctcaagcccgtgattaccctcagtccgaatgtaatggattttctccctgagtgtgtggtttcttgctaagcttggctgacgctcttgcagcatttcaaaaatgtttggctggcgaagaaatgccacaatcttgtcattatatgccagtggcaatgactcatgttgatgttggcttcgaatagcagctactaagctgtgtcctggcctggccagtaaagaggctcctctgtttctagaaacttctgaggcctctccagcgctgtaacttcggagcctctggaggtgctgtcggtgagttagatgattgggaagacgaccgttctgaagagggattcgggggtcaatgaaagtggtagctcgactgttgtggtccacgaaaaaagactttccctgctggtccgttttgatctcccagccccggggcagttccagccgagtgtctgcgaacatgttgatgaaattcaccaagtcccggttgtgctggtagcgttcaaaattgcgagcatcccgtcggactttcagaatcatgtgctttaagcaggtgctactggtgaagactcggtaggcactataattggcatgtagcacagtgaagaactcggggttggtgatgaacttgaccgctggggactgcagcagcaaggtgattttttgtgagttcactggagaaagtgacccttctctccttagatctaagctggactgggaagattcggcttctgagtcactccctccacctccgcctcctcctgctggggcttgctcgcagctttggctgccagaatcttcttcggacctctctgttgcaatggttcgctgaatgttttgataccgcctgttgagttgctccatctgctggatggaccccgatctccgcatgccatccggggtggctgctgccgtcggacgctgccaggtggttgtgcggttcacgtggtccacataaaagacccgcccgtggctgtcaattcgagcttcccagtcttctctccgattgcttggacctgccacgggggattccagaccttccgggcttctttccacgtgcccgctaggggcggccagctcgtcttgccacggcccagcgccgttcgtggactccgggtccagctcagggctctgcatggagtcgggtaccgactcgaacgcgctgttctcctcctcctcgtcgtcttgcgaggagaagaccgtgctctcggagatcttggcgctgtccacggaggagaagcgcgtgtggctggcgaacctgttgccgttgtagcaggaggggctgtagcacgaggcgctgtagcacgagctgctgtagcaggacgtgctgtagcacgaggagctgtagcacgaggggctgcagcaggacgcgtcacagccctcgcaactgtggtccccgccttgcctggggctggagtcgctctcgctcccggtgctggggtgcgtgtcgccatcctgggccgcgccattggccaggctggggaagtggcccccggagtggccagggtgcgccgtgcctggagtagccccctcgggctcttctctgtcctcttccagggcagacgggtcagcggccaccgtgtccacctcgctgagcccatccttctccgaggagtccttgagggtggactcctcctccgcgccgtcctcctcctctgccgcgctgccgccctgggcggagggcatgctgtgcagcagggtgtggatgcggatgtagtgtgtccgcggggtctcggggtccccgcaggctgacgcgatcaccgtctccagctcggacacaggcaaggagcagggcctgctttttctcttcaccgaggcccgcagctgcagcctgccctctccctgctccagggtagacacatctccctcctcctcctgctccttctcctcttcttcccttccagcccggctctgggtcgttgcttcctcctccaagggctcctccttggtgctggctggggcttcaccgtcttccagcagcagtgctgatgcctcctcacccaggtccagctgctcggccagctcttctgcactgggggcaggctggatgtccttttgcacctgggccaggagctccccagccccttcaggtcccacagagaccatgccctggtctcctgcctccgtgatgactgctgcttcctcagctggtctggaaagctctatgctttggttccctggaccatcggggacactgccctcacccagctgctctggcttccagctctcagaggactctggtgcctcagaccgaggttccccactgccgctttccatcaggttgttcatggggctgtcctgaatttgggctgactcaggctcggtactcagggaaatctcctcatcatctgctgggtggatggaggaagtgatctcaaatcggaattgcagctgtccactcacatgatctgttggaagcctgcggccaagtgtgtagctgaccaccctatcccctatggcgtgtctctccaggagtctttgaacgggcatcgacagctttcccaagaagcgcttgatgatggggcggctcttggcaaacttgtccttcacctcaatttccagcacgtcagtgggcaaggacacaaaactgaattgctcggcctgccagatggggttcacggtgttgcctatgatcttggatctcctctcctgtccatggtgagggagggcggggaagatgctgtgtttcccaggctgaatggaaatcttcagataagggtctgggttgaaaaacatccctttcttcaaccccatggcttggaaatctgagagagagaagctgatcagcctccgacttccttgtccttggacggtctcatcagcaccaatgcttttaaaaataggagctgccgagtttttgaccgtgacactgggggtggttgctcgcagggccccactcactccatggtagtatttgaagcagatcttagtttcaggttccacaaagtacgagctggcatcgatcttccagatgatctggccccgatgagaaccattgactccacggtttttatagtccagaaagttttcggacaagacctcatcaatgaggtacatgccaatccagtccccagcgtccacttcctcctttatgtcccagtggatgaccaggtcctgagagtgcccgatggaatagtaggagctgctgaccatgagcgtggagcggctgtccgaggtgaccaggtcagtgtcgctggtggagcggggaatggtgacgccatcgtgggggccgcccctgaggtccatgttgtggaactggtcggggttgtagctgtatcggagcggctccttgcaccggcgtcggctctgggagtttctagaaggagacgccatggcggccaggcctaaaaacctgttctggtacagattcgtaatagccacagccggagtgagtctgctgatgagaaacgcagatctggccacctgctttgagacgccttggaccacaacactgccggggtctttaacggttggccttttcgggtagggcatctgccctcctaaatcgcgtttaaatcccaggaaaagagagaagatgcctccctcaatttttgaactatgctgctcttgctgtatccgtttctgctgaacatagcattgatatcttttcaaagagaaggggggaaaacaaggggagaattgcaccactgcagattccaagagaagtaagcacaaaactacagcaacgtcaaataatatcttcttcggcaactaggaaaatccccacatgctctctggtgtcagcccaatgcagactgaggcgcgctgtgcccggaaccacaggaagccgggcatctctgcagcctgtgtccctgccagctccccctacgcgctgaaattcggcagggaagaagttatggtgcccagcctctgtgtgcaagacagagacaccgcgcatcatggctctgaaaatcagccaagtggccgggacgtcaaagcggcagagcaatcagaatgccctggagccggggatggaggggccacattgtttgagccctcggattttgctgcattgtcacc

SEQ ID NO: 14464 - RNA, 7038 nt, Homo sapiens
  source 1..7038: mol_type = other RNA
gctgggattacaggcatgagccaccgctcctggccggaatgctttagagtgtaggaacacaaataacacactgtccagacacaaactggtataatgagccattggcttcatatgaaattcacttcgtcttacatttctcccttgttttaatatggaaaacaattaaatgacatttaaatagtggggtctcttgagctcttctttttcccagtgaagaaaaacactttcatttatgacctatttcaggcaacatggataacaacgttagaaaaatagcaaatgaccattatggttgggtttatttcaaatgtagttgagaggttaggctgtctttggagcctgcagctgtttttctgacaacatgaagttttctgagatatgttttcactgaatgctaaaagaaactggatatttattttgatacaaatcaacgtgcctttggggtgttatgtttctgccccaggaggattactatgggtgaaggagaagtactatgttgcccttgatccctaacaagcaccatcactctctgcagcttcctagtgtggtcccgatggacaatcgaatgcaaaggaacttgaactccatgattaagaaaggaaaaggaaaaaaaaatgtgaaaaaaaaatatcaaagttttaaaaaaagggtttgtctgccaagcaaacaaaagtcatggctttaacaaaagtcatggtatcatctacacatttttttttcctttgtgaagaactgtggctagactaaacaaaacagaacagtacagaactcagggattcaaaccaaggtaatatgtccttcttccctttctccagttggcattgccacattctacataagacaatgggggctgaagcctcatccttcatgctacctcaatcaagaagctttctttcttggacatgtgcacaagtttgtccttcttgtggtgtgagtattcactagggatgctccccctcctaaacttctcttgagttgagcccacaatccccacaaccattgggatgcattgcattgcatcagcagcaggtgttttcttgctgttgttaatcgttagaagtgtcatatttgcaccgtatgtctaggctagttccggctgatgggactgatgccacatgtgaatcatgagttgaatgtataaaaatttcagctttgccactgttgtcctttggatggatattatgcacagggaaaagtagatggagaggaaaacaaagagttgatcagctcctagttctggagttggttattagaaattataaaaaatggtggctctgctcagaagacatgggcatatgaaagcctggagtgcttaatgctcacattttcccttcaatgatagaaatggaagtaaacatttattaccatttggtcaagtgtagcttaacttgcattcatatttcattgttagtaatggaggtatgtggagatatacacagaccttgagacagctgttttttaatattgcatacaggctagcagttcattgaaaacagaggagagaagcctgaaggttagatcttagaagaaggcagttcttcatgcacagcttttgtcaatcctgatttggtttgaaaataaaaatcatggaataccaaaatcaaaggagagttgattaagggaaagggaaaaggggatcatcccaggaagggtgatgtcactggccaggaaaatgtcaggcgaggttccatgtcctcactcaagtccaaaggtgctggtttcctctactgctgttaacagcttttcatacaacatggagtacgagggatacggtggaagatccagtcggttgaagcatgtgtgtgccctggggagagaagtaattttcccccatttctctatgcagaagcgccgaagcccattgctcccacggagggctgcgaagccttcgtagggcacgctggatgttcccgtgacaaactgcagtaatctcagcctctgctcattattgaagcgctccaccgcagcccagaaccagcggatcacaagatgcccatcgtggtaacctccccggtactcagtgttattccgccagtcatttaggtcgatttccgcggtgccagctatcaccagctccagctccctggcatcaaacacggacaccagcctcgagtctacaacctcgtagaagccgcgcaccagcgcctcggtctgctgtaccacgccgcgctccacccgccacttcaccatgcgctcgatgtactccttcttgtttttctccgtcacctgtgtgttggctcctccagacttcaactccctttccgtgacctgtccaaaaacctcttcattaacagtgaaagtgaggtctaagatgtctgtgatgttgttgtccttcatccactgcaaactctggtggaattcctcatccaaatattccaggtcactcaaatcacagggcagtctcaggagtgccttgtagaagggcctcgtgaagaaagcgtcaagaaggtactgatggatcagagccagacccaggatgcgaccgctaaacctgaaccactcaagatggttttctacaaatgcggacatggggctgatctgcaccgtgtaagtatcatttgccgagtactcaaagagtccatagtaagggttgaagagctcctgagacagaaggaagaagaactcccgcgaggggccactgtagtccaggccctcctctccaacaaaggtgacgtagagcttgtttcgctggagctctttccgcgaataggccatcacctgattgaaggttccctccaacaaatgatcccggcgaataatgagcttaattttccccggaccctgaccaaatcctttggcttccagttttctgtagaaattgcggagcttggcctcaaagtctcttcggtagggggaaggggctcttgcactggctctctgtaaacctggggagttctgaggtgaagaacagggtgaacatcggggagagaagctatacccagggtggaaggcagcctgcagggggacgtaggacataatctcttcttcaaagagactcagcaaaatgaccagatccgcatcacaggacaacttctcaagcccgtgattaccctcagtccgaatgtaatggattttctccctgagtgtgtggtttcttgctaagcttggctgacgctcttgcagcatttcaaaaatgtttggctggcgaagaaatgccacaatcttgtcattatatgccagtggcaatgactcatgttgatgttggcttcgaatagcagctactaagctgtgtcctggcctggccagtaaagaggctcctctgtttctagaaacttctgaggcctctccagcgctgtaacttcggagcctctggaggtgctgtcggtgagttagatgattgggaagacgaccgttctgaagagggattcgggggtcaatgaaagtggtagctcgactgttgtggtccacgaaaaaagactttccctgctggtccgttttgatctcccagccccggggcagttccagccgagtgtctgcgaacatgttgatgaaattcaccaagtcccggttgtgctggtagcgttcaaaattgcgagcatcccgtcggactttcagaatcatgtgctttaagcaggtgctactggtgaagactcggtaggcactataattggcatgtagcacagtgaagaactcggggttggtgatgaacttgaccgctggggactgcagcagcaaggtgattttttgtgagttcactggagaaagtgacccttctctccttagatctaagctggactgggaagattcggcttctgagtcactccctccacctccgcctcctcctgctggggcttgctcgcagctttggctgccagaatcttcttcggacctctctgttgcaatggttcgctgaatgttttgataccgcctgttgagttgctccatctgctggatggaccccgatctccgcatgccatccggggtggctgctgccgtcggacgctgccaggtggttgtgcggttcacgtggtccacataaaagacccgcccgtggctgtcaattcgagcttcccagtcttctctccgattgcttggacctgccacgggggattccagaccttccgggcttctttccacgtgcccgctaggggcggccagctcgtcttgccacggcccagcgccgttcgtggactccgggtccagctcagggctctgcatggagtcgggtaccgactcgaacgcgctgttctcctcctcctcgtcgtcttgcgaggagaagaccgtgctctcggagatcttggcgctgtccacggaggagaagcgcgtgtggctggcgaacctgttgccgttgtagcaggaggggctgtagcacgaggcgctgtagcacgagctgctgtagcaggacgtgctgtagcacgaggagctgtagcacgaggggctgcagcaggacgcgtcacagccctcgcaactgtggtccccgccttgcctggggctggagtcgctctcgctcccggtgctggggtgcgtgtcgccatcctgggccgcgccattggccaggctggggaagtggcccccggagtggccagggtgcgccgtgcctggagtagccccctcgggctcttctctgtcctcttccagggcagacgggtcagcggccaccgtgtccacctcgctgagcccatccttctccgaggagtccttgagggtggactcctcctccgcgccgtcctcctcctctgccgcgctgccgccctgggcggagggcatgctgtgcagcagggtgtggatgcggatgtagtgtgtccgcggggtctcggggtccccgcaggctgacgcgatcaccgtctccagctcggacacaggcaaggagcagggcctgctttttctcttcaccgaggcccgcagctgcagcctgccctctccctgctccagggtagacacatctccctcctcctcctgctccttctcctcttcttcccttccagcccggctctgggtcgttgcttcctcctccaagggctcctccttggtgctggctggggcttcaccgtcttccagcagcagtgctgatgcctcctcacccaggtccagctgctcggccagctcttctgcactgggggcaggctggatgtccttttgcacctgggccaggagctccccagccccttcaggtcccacagagaccatgccctggtctcctgcctccgtgatgactgctgcttcctcagctggtctggaaagctctatgctttggttccctggaccatcggggacactgccctcacccagctgctctggcttccagctctcagaggactctggtgcctcagaccgaggttccccactgccgctttccatcaggttgttcatggggctgtcctgaatttgggctgactcaggctcggtactcagggaaatctcctcatcatctgggtggatggaggaagtgatctcaaatcggaattgcagctgtccactcacatgatctgttggaagcctgcggccaagtgtgtagctgaccaccctatcccctatggcgtgtctctccaggagtctttgaacgggcatcgacagctttcccaagaagcgcttgatgatggggcggctcttggcaaacttgtccttcacctcaatttccagcacgtcagtgggcaaggacacaaaactgaattgctcggcctgccagatggggttcacggtgttgcctatgatcttggatctcctctcctgtccatggtgagggagggcggggaagatgctgtgtttcccaggctgaatggaaatcttcagataagggtctgggttgaaaaacatccctttcttcaaccccatggcttggaaatctgagagagagaagctgatcagcctccgacttccttgtccttggacggtctcatcagcaccaatgcttttaaaaataggagctgccgagtttttgaccgtgacactgggggtggttgctcgcagggccccactcactccatggtagtatttgaagcagatcttagtttcaggttccacaaagtacgagctggcatcgatcttccagatgatctggccccgatgagaaccattgactccacggtttttatagtccagaaagttttcggacaagacctcatcaatgaggtacatgccaatccagtccccagcgtccacttcctcctttatgtcccagtggatgaccaggtcctgagagtgcccgatggaatagtaggagctgctgaccatgagcgtggagcggctgtccgaggtgaccaggtcagtgtcgctggtggagcggggaatggtgacgccatcgtgggggccgcccctgaggtccatgttgtggaactggtcggggttgtagctgtatcggagcggctccttgcaccggcgtcggctctgggagtttctagaaggagacgccatggcggccaggcctaaaaacctgttctggtacagattcgtaatagccacagccggagtgagtctgctgatgagaaacgcagatctggccacctgctttgagacgccttggaccacaacactgccggggtctttaacggttggccttttcgggtagggcatctgccctcctaaatcgcgtttaaatcccaggaaaagagagaagatgcctccctcaatttttgaactatgctgctcttgctgtatccgtttctgctgaacatagcattgatatcttttcaaagagaaggggggaaaacaaggggagaattgcaccactgcagattccaagagaagtaagcacaaaactacagcaacgtcaaataatatcttcttcggcaactaggaaaatccccacatgctctctggtgtcagcccaatgcagactgaggcgcgctgtgcccggaaccacaggaagccgggcatctctgcagcctgtgtccctgccagctccccctacgcgctgaaattcggcagggaagaagttatggtgcccagcctctgtgtgcaagacagagacaccgcgcatcatggctctgaaaatcagccaagtggccgggacgtcaaagcggcagagcaatcagaatgccctggagccggggatggaggggccacattgtttgagccctcggattttgctgcattgtcacc

SEQ ID NO: 14465 - RNA, 7095 nt, Homo sapiens
  source 1..7095: mol_type = other RNA
gctgggattacaggcatgagccaccgctcctggccggaatgctttagagtgtaggaacacaaataacacactgtccagacacaaactggtataatgagccattggcttcatatgaaattcacttcgtcttacatttctcccttgttttaatatggaaaacaattaaatgacatttaaatagtggggtctcttgagctcttctttttcccagtgaagaaaaacactttcatttatgacctatttcaggcaacatggataacaacgttagaaaaatagcaaatgaccattatggttgggtttatttcaaatgtagttgagaggttaggctgtctttggagcctgcagctgtttttctgacaacatgaagttttctgagatatgttttcactgaatgctaaaagaaactggatatttattttgatacaaatcaacgtgcctttggggtgttatgtttctgccccaggaggattactatgggtgaaggagaagtactatgttgcccttgatccctaacaagcaccatcactctctgcagcttcctagtgtggtcccgatggacaatcgaatgcaaaggaacttgaactccatgattaagaaaggaaaaggaaaaaaaaatgtgaaaaaaaaatatcaaagttttaaaaaaagggtttgtctgccaagcaaacaaaagtcatggctttaacaaaagtcatggtatcatctacacatttttttttcctttgtgaagaactgtggctagactaaacaaaacagaacagtacagaactcagggattcaaaccaaggtaatatgtccttcttccctttctccagttggcattgccacattctacataagacaatgggggctgaagcctcatccttcatgctacctcaatcaagaagctttctttcttggacatgtgcacaagtttgtccttcttgtggtgtgagtattcactagggatgctccccctcctaaacttctcttgagttgagcccacaatccccacaaccattgggatgcattgcattgcatcagcagcaggtgttttcttgctgttgttaatcgttagaagtgtcatatttgcaccgtatgtctaggctagttccggctgatgggactgatgccacatgtgaatcatgagttgaatgtataaaaatttcagctttgccactgttgtcctttggatggatattatgcacagggaaaagtagatggagaggaaaacaaagagttgatcagctcctagttctggagttggttattagaaattataaaaaatggtggctctgctcagaagacatgggcatatgaaagcctggagtgcttaatgctcacattttcccttcaatgatagaaatggaagtaaacatttattaccatttggtcaagtgtagcttaacttgcattcatatttcattgttagtaatggaggtatgtggagatatacacagaccttgagacagctgttttttaatattgcatacaggctagcagttcattgaaaacagaggagagaagcctgaaggttagatcttagaagaaggcagttcttcatgcacagcttttgtcaatcctgatttggtttgaaaataaaaatcatggaataccaaaatcaaaggagagttgattaagggaaagggaaaaggggatcatcccaggaagggtgatgtcactggccaggaaaatgtcaggcgaggttccatgtcctcactcaagtccaaaggtgctggtttcctctactgctgttaacagcttttcatacaacatggagtacgagggatacggtggaagatccagtcggttgaagcatgtgtgtgccctggggagagaagtaattttcccccatttctctatgcagaagcgccgaagcccattgctcccacggagggctgcgaagccttcgtagggcacgctggatgttcccgtgacaaactgcagtaatctcagcctctgctcattattgaagcgctccaccgcagcccagaaccagcggatcacaagatgcccatcgtggtaacctccccggtactcagtgttattccgccagtcatttaggtcgatttccgcggtgccagctatcaccagctccagctccctggcatcaaacacggacaccagcctcgagtctacaacctcgtagaagccgcgcaccagcgcctcggtctgctgtaccacgccgcgctccacccgccacttcaccatgcgctcgatgtactccttcttgtttttctccgtcacctgtgtgttggctcctccagacttcaactccctttccgtgacctgtccaaaaacctcttcattaacagtgaaagtgaggtctaagatgtctgtgatgttgttgtccttcatccactgcaaactctggtggaattcctcatccaaatattccaggtcactcaaatcacagggcagtctcaggagtgccttgtagaagggcctcgtgaagaaagcgtcaagaaggtactgatggatcagagccagacccaggatgcgaccgctaaacctgaaccactcaagatggttttctacaaatgcggacatggggctgatctgcaccgtgtaagtatcatttgccgagtactcaaagagtccatagtaagggttgaagagctcctgagacagaaggaagaagaactcccgcgaggggccactgtagtccaggccctcctctccaacaaaggtgacgtagagcttgtttcgctggagctctttccgcgaataggccatcacctgattgaaggttccctccaacaaatgatcccggcgaataatgagcttaattttccccggaccctgaccaaatcctttggcttccagttttctgtagaaattgcggagcttggcctcaaagtctcttcggtagggggaaggggctcttgcactggctctctgtaaacctggggagttctgaggtgaagaacagggtgaacatcggggagagaagctatacccagggtggaaggcagcctgcagggggacgtaggacataatctcttcttcaaagagactcagcaaaatgaccagatccgcatcacaggacaacttctcaagcccgtgattaccctcagtccgaatgtaatggattttctccctgagtgtgtggtttcttgctaagcttggctgacgctcttgcagcatttcaaaaatgtttggctggcgaagaaatgccacaatcttgtcattatatgccagtggcaatgactcatgttgatgttggcttcgaatagcagctactaagctgtgtcctggcctggccagtaaagaggctcctctgtttctagaaacttctgaggcctctccagcgctgtaacttcggagcctctggaggtgctgtcggtgagttagatgattgggaagacgaccgttctgaagagggattcgggggtcaatgaaagtggtagctcgactgttgtggtccacgaaaaaagactttccctgctggtccgttttgatctcccagccccggggcagttccagccgagtgtctgcgaacatgttgatgaaattcaccaagtcccggttgtgctggtagcgttcaaaattgcgagcatcccgtcggactttcagaatcatgtgctttaagcaggtgctactggtgaagactcggtaggcactataattggcatgtagcacagtgaagaactcggggttggtgatgaacttgaccgctggggactgcagcagcaaggtgattttttgtgagttcactggagaaagtgacccttctctccttagatctaagctggactgggaagattcggcttctgagtcactccctccacctccgcctcctcctgctggggcttgctcgcagctttggctgccagaatcttcttcggacctctctgttgcaatggttcgctgaatgttttgataccgcctgttgagttgctccatctgctggatggaccccgatctccgcatgccatccggggtggctgctgccgtcggacgctgccaggtggttgtgcggttcacgtggtccacataaaagacccgcccgtggctgtcaattcgagcttcccagtcttctctccgattgcttggacctgccacgggggattccagaccttccgggcttctttccacgtgcccgctaggggcggccagctcgtcttgccacggcccagcgccgttcgtggactccgggtccagctcagggctctgcatggagtcgggtaccgactcgaacgcgctgttctcctcctcctcgtcgtcttgcgaggagaagaccgtgctctcggagatcttggcgctgtccacggaggagaagcgcgtgtggctggcgaacctgttgccgttgtagcaggaggggctgtagcacgaggcgctgtagcacgagctgctgtagcaggacgtgctgtagcacgaggagctgtagcacgaggggctgcagcaggacgcgtcacagccctcgcaactgtggtccccgccttgcctggggctggagtcgctctcgctcccggtgctggggtgcgtgtcgccatcctgggccgcgccattggccaggctggggaagtggcccccggagtggccagggtgcgccgtgcctggagtagccccctcgggctcttctctgtcctcttccagggcagacgggtcagcggccaccgtgtccacctcgctgagcccatccttctccgaggagtccttgagggtggactcctcctccgcgccgtcctcctcctctgccgcgctgccgccctgggcggagggcatgctgtgcagcagggtgtggatgcggatgtagtgtgtccgcggggtctcggggtccccgcaggctgacgcgatcaccgtctccagctcggacacaggcaaggagcagggcctgctttttctcttcaccgaggcccgcagctgcagcctgccctctccctgctccagggtagacacatctccctcctcctcctgctccttctcctcttcttcccttccagcccggctctgggtcgttgcttcctcctccaagggctcctccttggtgctggctggggcttcaccgtcttccagcagcagtgctgatgcctcctcacccaggtccagctgctcggccagctcttctgcactgggggcaggctggatgtccttttgcacctgggccaggagctccccagccccttcaggtcccacagagaccatgccctggtctcctgcctccgtgatgactgctgcttcctcagctggtctggaaagctctatgctttggttccctggaccatcggggacactgccctcacccagctgctctggcttccagctctcagaggactctggtgcctcagaccgaggttccccactgccgctttccatcaggttgttcatggggctgtcctgaatttgggctgactcaggctcggtactcagggaaatctcctcatcatctgggtggatggaggaagtgatctcaaatcggaattgcagctgtccactcacatgatctgttggaagcctgcggccaagtgtgtagctgaccaccctatcccctatggcgtgtctctccaggagtctttgaacgggcatcgacagctttcccaagaagcgcttgatgatggggcggctcttggcaaacttgtccttcacctcaatttccagcacgtcagtgggcaaggacacaaaactgaattgctcggcctgccagatggggttcacggtgttgcctatgatcttggatctcctctcctgtccatggtgagggagggcggggaagatgctgtgtttcccaggctgaatggaaatcttcagataagggtctgggttgaaaaacatccctttcttcaaccccatggcttggaaatctgagagagagaagctgatcagcctccgacttccttgtccttggacggtctcatcagcaccaatgcttttaaaaataggagctgccgagtttttgaccgtgacactgggggtggttgctcgcagggccccactcactccatggtagtatttgaagcagatcttagtttcaggttccacaaagtacgagctggcatcgatcttccagatgatctggccccgatgagaaccattgactccacggtttttatagtccagaaagttttcggacaagacctcatcaatgaggtacatgccaatccagtccccagcgtccacttcctcctttatgtcccagtggatgaccaggtcctgagagtgcccgatggaatagtaggagctgctgaccatgagcgtggagcggctgtccgaggtgaccaggtcagtgtcgctggtggagcggggaatggtgacgccatcgtgggggccgcccctgaggtccatgttgtggaactggtcggggttgtagctgtatcggagcggctccttgcaccggcgtcggctctgggagtttctagaaggagacgccatggcggccaggcctaaaaacctgttctggtacagattcttcacactacacaggtgcagcagcataatgacccaccacgtgtacgcgcatcaattccgtaatagccacagccggagtgagtctgctgatgagaaacgcagatctggccacctgctttgagacgccttggaccacaacactgccggggtctttaacggttggccttttcgggtagggcatctgccctcctaaatcgcgtttaaatcccaggaaaagagagaagatgcctccctcaatttttgaactatgctgctcttgctgtatccgtttctgctgaacatagcattgatatcttttcaaagagaaggggggaaaacaaggggagaattgcaccactgcagattccaagagaagtaagcacaaaactacagcaacgtcaaataatatcttcttcggcaactaggaaaatccccacatgctctctggtgtcagcccaatgcagactgaggcgcgctgtgcccggaaccacaggaagccgggcatctctgcagcctgtgtccctgccagctccccctacgcgctgaaattcggcagggaagaagttatggtgcccagcctctgtgtgcaagacagagacaccgcgcatcatggctctgaaaatcagccaagtggccgggacgtcaaagcggcagagcaatcagaatgccctggagccggggatggaggggccacattgtttgagccctcggattttgctgcattgtcac

SEQ ID NO: 14466 - RNA, 6736 nt, Homo sapiens
  source 1..6736: mol_type = other RNA
gctgggattacaggcatgagccaccgctcctggccggaatgctttagagtgtaggaacacaaataacacactgtccagacacaaactggtataatgagccattggcttcatatgaaattcacttcgtcttacatttctcccttgttttaatatggaaaacaattaaatgacatttaaatagtggggtctcttgagctcttctttttcccagtgaagaaaaacactttcatttatgacctatttcaggcaacatggataacaacgttagaaaaatagcaaatgaccattatggttgggtttatttcaaatgtagttgagaggttaggctgtctttggagcctgcagctgtttttctgacaacatgaagttttctgagatatgttttcactgaatgctaaaagaaactggatatttattttgatacaaatcaacgtgcctttggggtgttatgtttctgccccaggaggattactatgggtgaaggagaagtactatgttgcccttgatccctaacaagcaccatcactctctgcagcttcctagtgtggtcccgatggacaatcgaatgcaaaggaacttgaactccatgattaagaaaggaaaaggaaaaaaaaatgtgaaaaaaaaatatcaaagttttaaaaaaagggtttgtctgccaagcaaacaaaagtcatggctttaacaaaagtcatggtatcatctacacatttttttttcctttgtgaagaactgtggctagactaaacaaaacagaacagtacagaactcagggattcaaaccaaggtaatatgtccttcttccctttctccagttggcattgccacattctacataagacaatgggggctgaagcctcatccttcatgctacctcaatcaagaagctttctttcttggacatgtgcacaagtttgtccttcttgtggtgtgagtattcactagggatgctccccctcctaaacttctcttgagttgagcccacaatccccacaaccattgggatgcattgcattgcatcagcagcaggtgttttcttgctgttgttaatcgttagaagtgtcatatttgcaccgtatgtctaggctagttccggctgatgggactgatgccacatgtgaatcatgagttgaatgtataaaaatttcagctttgccactgttgtcctttggatggatattatgcacagggaaaagtagatggagaggaaaacaaagagttgatcagctcctagttctggagttggttattagaaattataaaaaatggtggctctgctcagaagacatgggcatatgaaagcctggagtgcttaatgctcacattttcccttcaatgatagaaatggaagtaaacatttattaccatttggtcaagtgtagcttaacttgcattcatatttcattgttagtaatggaggtatgtggagatatacacagaccttgagacagctgttttttaatattgcatacaggctagcagttcattgaaaacagaggagagaagcctgaaggttagatcttagaagaaggcagttcttcatgcacagcttttgtcaatcctgatttggtttgaaaataaaaatcatggaataccaaaatcaaaggagagttgattaagggaaagggaaaaggggatcatcccaggaagggtgatgtcactggccaggaaaatgtcaggcgaggttccatgtcctcactcaagtccaaaggtgctggtttcctctactgctgttaacagcttttcatacaacatggagtacgagggatacggtggaagatccagtcggttgaagcatgtgtgtgccctggggagagaagtaattttcccccatttctctatgcagaagcgccgaagcccattgctcccacggagggctgcgaagccttcgtagggcacgctggatgttcccgtgacaaactgcagtaatctcagcctctgctcattattgaagcgctccaccgcagcccagaaccagcggatcacaagatgcccatcgtggtaacctccccggtactcagtgttattccgccagtcatttaggtcgatttccgcggtgccagctatcaccagctccagctccctggcatcaaacacggacaccagcctcgagtctacaacctcgtagaagccgcgcaccagcgcctcggtctgctgtaccacgccgcgctccacccgccacttcaccatgcgctcgatgtactccttcttgtttttctccgtcacctgtgtgttggctcctccagacttcaactccctttccgtgacctgtccaaaaacctcttcattaacagtgaaagtgaggtctaagatgtctgtgatgttgttgtccttcatccactgcaaactctggtggaattcctcatccaaatattccaggtcactcaaatcacagggcagtctcaggagtgccttgtagaagggcctcgtgaagaaagcgtcaagaaggtactgatggatcagagccagacccaggatgcgaccgctaaacctgaaccactcaagatggttttctacaaatgcggacatggggctgatctgcaccgtgtaagtatcatttgccgagtactcaaagagtccatagtaagggttgaagagctcctgagacagaaggaagaagaactcccgcgaggggccactgtagtccaggccctcctctccaacaaaggtgacgtagagcttgtttcgctggagctctttccgcgaataggccatcacctgattgaaggttccctccaacaaatgatcccggcgaataatgagcttaattttccccggaccctgaccaaatcctttggcttccagttttctgtagaaattgcggagcttggcctcaaagtctcttcggtagggggaaggggctcttgcactggctctctgtaaacctggggagttctgaggtgaagaacagggtgaacatcggggagagaagctatacccagggtggaaggcagcctgcagggggacgtaggacataatctcttcttcaaagagactcagcaaaatgaccagatccgcatcacaggacaacttctcaagcccgtgattaccctcagtccgaatgtaatggattttctccctgagtgtgtggtttcttgctaagcttggctgacgctcttgcagcatttcaaaaatgtttggctggcgaagaaatgccacaatcttgtcattatatgccagtggcaatgactcatgttgatgttggcttcgaatagcagctactaagctgtgtcctggcctggccagtaaagaggctcctctgtttctagaaacttctgaggcctctccagcgctgtaacttcggagcctctggaggtgctgtcggtgagttagatgattgggaagacgaccgttctgaagagggattcgggggtcaatgaaagtggtagctcgactgttgtggtccacgaaaaaagactttccctgctggtccgttttgatctcccagccccggggcagttccagccgagtgtctgcgaacatgttgatgaaattcaccaagtcccggttgtgctggtagcgttcaaaattgcgagcatcccgtcggactttcagaatcatgtgctttaagcaggtgctactggtgaagactcggtaggcactataattggcatgtagcacagtgaagaactcggggttggtgatgaacttgaccgctggggactgcagcagcaaggtgattttttgtgagttcactggagaaagtgacccttctctccttagatctaagctggactgggaagattcggcttctgagtcactccctccacctccgcctcctcctgctggggcttgctcgcagctttggctgccagaatcttcttcggacctctctgttgcaatggttcgctgaatgttttgataccgcctgttgagttgctccatctgctggatggaccccgatctccgcatgccatccggggtggctgctgccgtcggacgctgccaggtggttgtgcggttcacgtggtccacataaaagacccgcccgtggctgtcaattcgagcttcccagtcttctctccgattgcttggacctgccacgggggattccagaccttccgggcttctttccacgtgcccgctaggggcggccagctcgtcttgccacggcccagcgccgttcgtggactccgggtccagctcagggctctgcatggagtcgggtaccgactcgaacgcgctgttctcctcctcctcgtcgtcttgcgaggagaagaccgtgctctcggagatcttggcgctgtccacggaggagaagcgcgtgtggctggcgaacctgttgccgttgtagcaggaggggctgtagcacgaggcgctgtagcacgagctgctgtagcaggacgtgctgtagcacgaggagctgtagcacgaggggctgcagcaggacgcgtcacagccctcgcaactgtggtccccgccttgcctggggctggagtcgctctcgctcccggtgctggggtgcgtgtcgccatcctgggccgcgccattggccaggctggggaagtggcccccggagtggccagggtgcgccgtgcctggagtagccccctcgggctcttctctgtcctcttccagggcagacgggtcagcggccaccgtgtccacctcgctgagcccatccttctccgaggagtccttgagggtggactcctcctccgcgccgtcctcctcctctgccgcgctgccgccctgggcggagggcatgctgtgcagcagggtgtggatgcggatgtagtgtgtccgcggggtctcggggtccccgcaggctgacgcgatcaccgtctccagctcggacacaggcaaggagcagggcctgctttttctcttcaccgaggcccgcagctgcagcctgccctctccctgctccagggtagacacatctccctcctcctcctgctccttctcctcttcttcccttccagcccggctctgggtcgttgcttcctcctccaagggctcctccttggtgctggctggggcttcaccgtcttccagcagcagtgctgatgcctcctcacccaggtccagctgctcggccagctcttctgcactgggggcaggctggatgtccttttgcacctgggccaggagctccccagccccttcaggtcccacagagaccatgccctggtctcctgcctccgtgatgactgctgcttcctcagctggtctggaaagctctatgctttggttccctggaccatcggggacactgccctcacccagctgctctggcttccagctctcagaggactctggtgcctcagaccgaggttccccactgccgctttccatcaggttgttcatggggctgtcctgaatttgggctgactcaggctcggtactcagggaaatctcctcatcatctgggtggatggaggaagtgatctcaaatcggaattgcagctgtccactcacatgatctgttggaagcctgcggccaagtgtgtagctgaccaccctatcccctatggcgtgtctctccaggagtctttgaacgggcatcgacagctttcccaagaagcgcttgatgatggggcggctcttggcaaacttgtccttcacctcaatttccagcacgtcagtgggcaaggacacaaaactgaattgctcggcctgccagatggggttcacggtgttgcctatgatcttggatctcctctcctgtccatggtgagggagggcggggaagatgctgtgtttcccaggctgaatggaaatcttcagataagggtctgggttgaaaaacatccctttcttcaaccccatggcttggaaatctgagagagagaagctgatcagcctccgacttccttgtccttggacggtctcatcagcaccaatgcttttaaaaataggagctgccgagtttttgaccgtgacactgggggtggttgctcgcagggccccactcactccatggtagtatttgaagcagatcttagtttcaggttccacaaagtacgagctggcatcgatcttccagatgatctggccccgatgagaaccattgactccacggtttttatagtccagaaagttttcggacaagacctcatcaatgaggtacatgccaatccagtccccagcgtccacttcctcctttatgtcccagtggatgaccaggtcctgagagtgcccgatggaatagtaggagctgctgaccatgagcgtggagcggctgtccgaggtgaccaggtcagtgtcgctggtggagcggggaatggtgacgccatcgtgggggccgcccctgaggtccatgttgtggaactggtcggggttgtagctgtatcggagcggctccttgcaccggcgtcggctctgggagtttctagaaggagacgccatggcggccaggcctaaaaacctgttctggtacagattcttcacactacacaggtgcagcagcataatgacccaccacgtgtacgcgcatcaattccttggcagccctggcctgggcacagatcatgctcctgtcagcgcgcagattagagctggggggcgcacgtgccccgcatagtgcaccgggcgcctgggactggctggggaggggaccctggcgaccgcccgctctcgctgcgctctggctgccgggtgccccgagagagcggaggccacggccactgtcacggcggaggggcgcgcgcggctcggcgagtgtgtgcgcgaggagggggccggttcggtcagagtcgcacggtgttccggctccaacaacagcgcctgatgc

SEQ ID NO: 14467 - RNA, 6696 nt, Homo sapiens
  source 1..6696: mol_type = other RNA
gctgggattacaggcatgagccaccgctcctggccggaatgctttagagtgtaggaacacaaataacacactgtccagacacaaactggtataatgagccattggcttcatatgaaattcacttcgtcttacatttctcccttgttttaatatggaaaacaattaaatgacatttaaatagtggggtctcttgagctcttctttttcccagtgaagaaaaacactttcatttatgacctatttcaggcaacatggataacaacgttagaaaaatagcaaatgaccattatggttgggtttatttcaaatgtagttgagaggttaggctgtctttggagcctgcagctgtttttctgacaacatgaagttttctgagatatgttttcactgaatgctaaaagaaactggatatttattttgatacaaatcaacgtgcctttggggtgttatgtttctgccccaggaggattactatgggtgaaggagaagtactatgttgcccttgatccctaacaagcaccatcactctctgcagcttcctagtgtggtcccgatggacaatcgaatgcaaaggaacttgaactccatgattaagaaaggaaaaggaaaaaaaaatgtgaaaaaaaaatatcaaagttttaaaaaaagggtttgtctgccaagcaaacaaaagtcatggctttaacaaaagtcatggtatcatctacacatttttttttcctttgtgaagaactgtggctagactaaacaaaacagaacagtacagaactcagggattcaaaccaaggtaatatgtccttcttccctttctccagttggcattgccacattctacataagacaatgggggctgaagcctcatccttcatgctacctcaatcaagaagctttctttcttggacatgtgcacaagtttgtccttcttgtggtgtgagtattcactagggatgctccccctcctaaacttctcttgagttgagcccacaatccccacaaccattgggatgcattgcattgcatcagcagcaggtgttttcttgctgttgttaatcgttagaagtgtcatatttgcaccgtatgtctaggctagttccggctgatgggactgatgccacatgtgaatcatgagttgaatgtataaaaatttcagctttgccactgttgtcctttggatggatattatgcacagggaaaagtagatggagaggaaaacaaagagttgatcagctcctagttctggagttggttattagaaattataaaaaatggtggctctgctcagaagacatgggcatatgaaagcctggagtgcttaatgctcacattttcccttcaatgatagaaatggaagtaaacatttattaccatttggtcaagtgtagcttaacttgcattcatatttcattgttagtaatggaggtatgtggagatatacacagaccttgagacagctgttttttaatattgcatacaggctagcagttcattgaaaacagaggagagaagcctgaaggttagatcttagaagaaggcagttcttcatgcacagcttttgtcaatcctgatttggtttgaaaataaaaatcatggaataccaaaatcaaaggagagttgattaagggaaagggaaaaggggatcatcccaggaagggtgatgtcactggccaggaaaatgtcaggcgaggttccatgtcctcactcaagtccaaaggtgctggtttcctctactgctgttaacagcttttcatacaacatggagtacgagggatacggtggaagatccagtcggttgaagcatgtgtgtgccctggggagagaagtaattttcccccatttctctatgcagaagcgccgaagcccattgctcccacggagggctgcgaagccttcgtagggcacgctggatgttcccgtgacaaactgcagtaatctcagcctctgctcattattgaagcgctccaccgcagcccagaaccagcggatcacaagatgcccatcgtggtaacctccccggtactcagtgttattccgccagtcatttaggtcgatttccgcggtgccagctatcaccagctccagctccctggcatcaaacacggacaccagcctcgagtctacaacctcgtagaagccgcgcaccagcgcctcggtctgctgtaccacgccgcgctccacccgccacttcaccatgcgctcgatgtactccttcttgtttttctccgtcacctgtgtgttggctcctccagacttcaactccctttccgtgacctgtccaaaaacctcttcattaacagtgaaagtgaggtctaagatgtctgtgatgttgttgtccttcatccactgcaaactctggtggaattcctcatccaaatattccaggtcactcaaatcacagggcagtctcaggagtgccttgtagaagggcctcgtgaagaaagcgtcaagaaggtactgatggatcagagccagacccaggatgcgaccgctaaacctgaaccactcaagatggttttctacaaatgcggacatggggctgatctgcaccgtgtaagtatcatttgccgagtactcaaagagtccatagtaagggttgaagagctcctgagacagaaggaagaagaactcccgcgaggggccactgtagtccaggccctcctctccaacaaaggtgacgtagagcttgtttcgctggagctctttccgcgaataggccatcacctgattgaaggttccctccaacaaatgatcccggcgaataatgagcttaattttccccggaccctgaccaaatcctttggcttccagttttctgtagaaattgcggagcttggcctcaaagtctcttcggtagggggaaggggctcttgcactggctctctgtaaacctggggagttctgaggtgaagaacagggtgaacatcggggagagaagctatacccagggtggaaggcagcctgcagggggacgtaggacataatctcttcttcaaagagactcagcaaaatgaccagatccgcatcacaggacaacttctcaagcccgtgattaccctcagtccgaatgtaatggattttctccctgagtgtgtggtttcttgctaagcttggctgacgctcttgcagcatttcaaaaatgtttggctggcgaagaaatgccacaatcttgtcattatatgccagtggcaatgactcatgttgatgttggcttcgaatagcagctactaagctgtgtcctggcctggccagtaaagaggctcctctgtttctagaaacttctgaggcctctccagcgctgtaacttcggagcctctggaggtgctgtcggtgagttagatgattgggaagacgaccgttctgaagagggattcgggggtcaatgaaagtggtagctcgactgttgtggtccacgaaaaaagactttccctgctggtccgttttgatctcccagccccggggcagttccagccgagtgtctgcgaacatgttgatgaaattcaccaagtcccggttgtgctggtagcgttcaaaattgcgagcatcccgtcggactttcagaatcatgtgctttaagcaggtgctactggtgaagactcggtaggcactataattggcatgtagcacagtgaagaactcggggttggtgatgaacttgaccgctggggactgcagcagcaaggtgattttttgtgagttcactggagaaagtgacccttctctccttagatctaagctggactgggaagattcggcttctgagtcactccctccacctccgcctcctcctgctggggcttgctcgcagctttggctgccagaatcttcttcggacctctctgttgcaatggttcgctgaatgttttgataccgcctgttgagttgctccatctgctggatggaccccgatctccgcatgccatccggggtggctgctgccgtcggacgctgccaggtggttgtgcggttcacgtggtccacataaaagacccgcccgtggctgtcaattcgagcttcccagtcttctctccgattgcttggacctgccacgggggattccagaccttccgggcttctttccacgtgcccgctaggggcggccagctcgtcttgccacggcccagcgccgttcgtggactccgggtccagctcagggctctgcatggagtcgggtaccgactcgaacgcgctgttctcctcctcctcgtcgtcttgcgaggagaagaccgtgctctcggagatcttggcgctgtccacggaggagaagcgcgtgtggctggcgaacctgttgccgttgtagcaggaggggctgtagcacgaggcgctgtagcacgagctgctgtagcaggacgtgctgtagcacgaggagctgtagcacgaggggctgcagcaggacgcgtcacagccctcgcaactgtggtccccgccttgcctggggctggagtcgctctcgctcccggtgctggggtgcgtgtcgccatcctgggccgcgccattggccaggctggggaagtggcccccggagtggccagggtgcgccgtgcctggagtagccccctcgggctcttctctgtcctcttccagggcagacgggtcagcggccaccgtgtccacctcgctgagcccatccttctccgaggagtccttgagggtggactcctcctccgcgccgtcctcctcctctgccgcgctgccgccctgggcggagggcatgctgtgcagcagggtgtggatgcggatgtagtgtgtccgcggggtctcggggtccccgcaggctgacgcgatcaccgtctccagctcggacacaggcaaggagcagggcctgctttttctcttcaccgaggcccgcagctgcagcctgccctctccctgctccagggtagacacatctccctcctcctcctgctccttctcctcttcttcccttccagcccggctctgggtcgttgcttcctcctccaagggctcctccttggtgctggctggggcttcaccgtcttccagcagcagtgctgatgcctcctcacccaggtccagctgctcggccagctcttctgcactgggggcaggctggatgtccttttgcacctgggccaggagctccccagccccttcaggtcccacagagaccatgccctggtctcctgcctccgtgatgactgctgcttcctcagctggtctggaaagctctatgctttggttccctggaccatcggggacactgccctcacccagctgctctggcttccagctctcagaggactctggtgcctcagaccgaggttccccactgccgctttccatcaggttgttcatggggctgtcctgaatttgggctgactcaggctcggtactcagggaaatctcctcatcatctgggtggatggaggaagtgatctcaaatcggaattgcagctgtccactcacatgatctgttggaagcctgcggccaagtgtgtagctgaccaccctatcccctatggcgtgtctctccaggagtctttgaacgggcatcgacagctttcccaagaagcgcttgatgatggggcggctcttggcaaacttgtccttcacctcaatttccagcacgtcagtgggcaaggacacaaaactgaattgctcggcctgccagatggggttcacggtgttgcctatgatcttggatctcctctcctgtccatggtgagggagggcggggaagatgctgtgtttcccaggctgaatggaaatcttcagataagggtctgggttgaaaaacatccctttcttcaaccccatggcttggaaatctgagagagagaagctgatcagcctccgacttccttgtccttggacggtctcatcagcaccaatgcttttaaaaataggagctgccgagtttttgaccgtgacactgggggtggttgctcgcagggccccactcactccatggtagtatttgaagcagatcttagtttcaggttccacaaagtacgagctggcatcgatcttccagatgatctggccccgatgagaaccattgactccacggtttttatagtccagaaagttttcggacaagacctcatcaatgaggtacatgccaatccagtccccagcgtccacttcctcctttatgtcccagtggatgaccaggtcctgagagtgcccgatggaatagtaggagctgctgaccatgagcgtggagcggctgtccgaggtgaccaggtcagtgtcgctggtggagcggggaatggtgacgccatcgtgggggccgcccctgaggtccatgttgtggaactggtcggggttgtagctgtatcggagcggctccttgcaccggcgtcggctctgggagtttctagaaggagacgccatggcggccaggcctaaaaacctgttctggtacagattcttggcagccctggcctgggcacagatcatgctcctgtcagcgcgcagattagagctggggggcgcacgtgccccgcatagtgcaccgggcgcctgggactggctggggaggggaccctggcgaccgcccgctctcgctgcgctctggctgccgggtgccccgagagagcggaggccacggccactgtcacggcggaggggcgcgcgcggctcggcgagtgtgtgcgcgaggagggggccggttcggtcagagtcgcacggtgttccggctccaacaacagcgcctgatgcgcggtaacgcagcacact

SEQ ID NO: 14468 - RNA, 6153 nt, Homo sapiens
  source 1..6153: mol_type = other RNA
gctgggattacaggcatgagccaccgctcctggccggaatgctttagagtgtaggaacacaaataacacactgtccagacacaaactggtataatgagccattggcttcatatgaaattcacttcgtcttacatttctcccttgttttaatatggaaaacaattaaatgacatttaaatagtggggtctcttgagctcttctttttcccagtgaagaaaaacactttcatttatgacctatttcaggcaacatggataacaacgttagaaaaatagcaaatgaccattatggttgggtttatttcaaatgtagttgagaggttaggctgtctttggagcctgcagctgtttttctgacaacatgaagttttctgagatatgttttcactgaatgctaaaagaaactggatatttattttgatacaaatcaacgtgcctttggggtgttatgtttctgccccaggaggattactatgggtgaaggagaagtactatgttgcccttgatccctaacaagcaccatcactctctgcagcttcctagtgtggtcccgatggacaatcgaatgcaaaggaacttgaactccatgattaagaaaggaaaaggaaaaaaaaatgtgaaaaaaaaatatcaaagttttaaaaaaagggtttgtctgccaagcaaacaaaagtcatggctttaacaaaagtcatggtatcatctacacatttttttttcctttgtgaagaactgtggctagactaaacaaaacagaacagtacagaactcagggattcaaaccaaggtaatatgtccttcttccctttctccagttggcattgccacattctacataagacaatgggggctgaagcctcatccttcatgctacctcaatcaagaagctttctttcttggacatgtgcacaagtttgtccttcttgtggtgtgagtattcactagggatgctccccctcctaaacttctcttgagttgagcccacaatccccacaaccattgggatgcattgcattgcatcagcagcaggtgttttcttgctgttgttaatcgttagaagtgtcatatttgcaccgtatgtctaggctagttccggctgatgggactgatgccacatgtgaatcatgagttgaatgtataaaaatttcagctttgccactgttgtcctttggatggatattatgcacagggaaaagtagatggagaggaaaacaaagagttgatcagctcctagttctggagttggttattagaaattataaaaaatggtggctctgctcagaagacatgggcatatgaaagcctggagtgcttaatgctcacattttcccttcaatgatagaaatggaagtaaacatttattaccatttggtcaagtgtagcttaacttgcattcatatttcattgttagtaatggaggtatgtggagatatacacagaccttgagacagctgttttttaatattgcatacaggctagcagttcattgaaaacagaggagagaagcctgaaggttagatcttagaagaaggcagttcttcatgcacagcttttgtcaatcctgatttggtttgaaaataaaaatcatggaataccaaaatcaaaggagagttgattaagggaaagggaaaaggggatcatcccaggaagggtgatgtcactggccaggaaaatgtcaggcgaggttccatgtcctcactcaagtccaaaggtgctggtttcctctactgctgttaacagcttttcatacaacatggagtacgagggatacggtggaagatccagtcggttgaagcatgtgtgtgccctggggagagaagtaattttcccccatttctctatgcagaagcgccgaagcccattgctcccacggagggctgcgaagccttcgtagggcacgctggatgttcccgtgacaaactgcagtaatctcagcctctgctcattattgaagcgctccaccgcagcccagaaccagcggatcacaagatgcccatcgtggtaacctccccggtactcagtgttattccgccagtcatttaggtcgatttccgcggtgccagctatcaccagctccagctccctggcatcaaacacggacaccagcctcgagtctacaacctcgtagaagccgcgcaccagcgcctcggtctgctgtaccacgccgcgctccacccgccacttcaccatgcgctcgatgtactccttcttgtttttctccgtcacctgtgtgttggctcctccagacttcaactccctttccgtgacctgtccaaaaacctcttcattaacagtgaaagtgaggtctaagatgtctgtgatgttgttgtccttcatccactgcaaactctggtggaattcctcatccaaatattccaggtcactcaaatcacagggcagtctcaggagtgccttgtagaagggcctcgtgaagaaagcgtcaagaaggtactgatggatcagagccagacccaggatgcgaccgctaaacctgaaccactcaagatggttttctacaaatgcggacatggggctgatctgcaccgtgtaagtatcatttgccgagtactcaaagagtccatagtaagggttgaagagctcctgagacagaaggaagaagaactcccgcgaggggccactgtagtccaggccctcctctccaacaaaggtgacgtagagcttgtttcgctggagctctttccgcgaataggccatcacctgattgaaggttccctccaacaaatgatcccggcgaataatgagcttaattttccccggaccctgaccaaatcctttggcttccagttttctgtagaaattgcggagcttggcctcaaagtctcttcggtagggggaaggggctcttgcactggctctctgtaaacctggggagttctgaggtgaagaacagggtgaacatcggggagagaagctatacccagggtggaaggcagcctgcagggggacgtaggacataatctcttcttcaaagagactcagcaaaatgaccagatccgcatcacaggacaacttctcaagcccgtgattaccctcagtccgaatgtaatggattttctccctgagtgtgtggtttcttgctaagcttggctgacgctcttgcagcatttcaaaaatgtttggctggcgaagaaatgccacaatcttgtcattatatgccagtggcaatgactcatgttgatgttggcttcgaatagcagctactaagctgtgtcctggcctggccagtaaagaggctcctctgtttctagaaacttctgaggcctctccagcgctgtaacttcggagcctctggaggtgctgtcggtgagttagatgattgggaagacgaccgttctgaagagggattcgggggtcaatgaaagtggtagctcgactgttgtggtccacgaaaaaagactttccctgctggtccgttttgatctcccagccccggggcagttccagccgagtgtctgcgaacatgttgatgaaattcaccaagtcccggttgtgctggtagcgttcaaaattgcgagcatcccgtcggactttcagaatcatgtgctttaagcaggtgctactggtgaagactcggtaggcactataattggcatgtagcacagtgaagaactcggggttggtgatgaacttgaccgctggggactgcagcagcaaggtgattttttgtgagttcactggagaaagtgacccttctctccttagatctaagctggactgggaagattcggcttctgagtcactccctccacctccgcctcctcctgctggggcttgctcgcagctttggctgccagaatcttcttcggacctctctgttgcaatggttcgctgaatgttttgataccgcctgttgagttgctccatctgctggatggaccccgatctccgcatgccatccggggtggctgctgccgtcggacgctgccaggtggttgtgcggttcacgtggtccacataaaagacccgcccgtggctgtcaattcgagcttcccagtttggtggaagaggctcatcgattgttgggtagtgatgatgttcaggcctcagggaaggaagctggcttactggctgggaattatggagtataggacattcaccttctctccgattgcttggacctgccacgggggattccagaccttccgggcttctttccacgtgcccgctaggggcggccagctcgtcttgccacggcccagcgccgttcgtggactccgggtccagctcagggctctgcatggagtcgggtaccgactcgaacgcgctgttctcctcctcctcgtcgtcttgcgaggagaagaccgtgctctcggagatcttggcgctgtccacggaggagaagcgcgtgtggctggcgaacctgttgccgttgtagcaggaggggctgtagcacgaggcgctgtagcacgagctgctgtagcaggacgtgctgtagcacgaggagctgtagcacgaggggctgcagcaggacgcgtcacagccctcgcaactgtggtccccgccttgcctggggctggagtcgctctcgctcccggtgctggggtgcgtgtcgccatcctgggccgcgccattggccaggctggggaagtggcccccggagtggccagggtgcgccgtgcctggagtagccccctcgggctcttctctgtcctcttccagggcagacgggtcagcggccaccgtgtccacctcgctgagcccatccttctccgaggagtccttgagggtggactcctcctccgcgccgtcctcctcctctgccgcgctgccgccctgggcggagggcatgctgtgcagcagggtgtggatgcggatgtagtgtgtccgcggggtctcggggtccccgcaggctgacgcgatcaccgtctccagctcggacacaggcaaggagcagggcctgctttttctcttcaccgaggcccgcagctgcagcctgccctctccctgctccagggtagacacatctccctcctcctcctgctccttctcctcttcttcccttccagcccggctctgggtcgttgcttcctcctccaagggctcctccttggtgctggctggggcttcaccgtcttccagcagcagtgctgatgcctcctcacccaggtccagctgctcggccagctcttctgcactgggggcaggctggatgtccttttgcacctgggccaggagctccccagccccttcaggtcccacagagaccatgccctggtctcctgcctccgtgatgactgctgcttcctcagctggtctggaaagctctatgctttggttccctggaccatcggggacactgccctcacccagctgctctggcttccagctctcagaggactctggtgcctcagaccgaggttccccactgccgctttccatcaggttgttcatggggctgtcctgaatttgggctgactcaggctcggtactcagggaaatctcctcatcatctgctgggtggatggaggaagtgatctcaaatcggaattgcagctgtccactcacatgatctgttggaagcctgcggccaagtgtgtagctgaccaccctatcccctatggcgtgtctctccaggagtctttgaacgggcatcgacagctttcccaagaagcgcttgatgatggggcggctcttggcaaacttgtccttcacctcaatttccagcacgtcagtgggcaaggacacaaaactgaattgctcggcctgccagatggggttcacggtgttgcctatgatcttggatctcctctcctgtccatggtgagggagggcggggaagatgctgtgtttcccaggctgaatggaaatcttcagataagggtctgggttgaaaaacatccctttcttcaaccccatggcttggaaatctgagagagagaagctgatcagcctccgacttccttgtccttggacggtctcatcagcaccaatgcttttaaaaataggagctgccgagtttttgaccgtgacactgggggtggttgctcgcagggccccactcactccatggtagtatttgaagcagatcttagtttcagccatcaatgataacctctttgcatcacaatttgtttccttcaaagttctatagatgtagctggcagtggtagcacgcatctgtagttcccagct

SEQ ID NO: 14469 - RNA, 6815 nt, Homo sapiens
  source 1..6815: mol_type = other RNA
gctgggattacaggcatgagccaccgctcctggccggaatgctttagagtgtaggaacacaaataacacactgtccagacacaaactggtataatgagccattggcttcatatgaaattcacttcgtcttacatttctcccttgttttaatatggaaaacaattaaatgacatttaaatagtggggtctcttgagctcttctttttcccagtgaagaaaaacactttcatttatgacctatttcaggcaacatggataacaacgttagaaaaatagcaaatgaccattatggttgggtttatttcaaatgtagttgagaggttaggctgtctttggagcctgcagctgtttttctgacaacatgaagttttctgagatatgttttcactgaatgctaaaagaaactggatatttattttgatacaaatcaacgtgcctttggggtgttatgtttctgccccaggaggattactatgggtgaaggagaagtactatgttgcccttgatccctaacaagcaccatcactctctgcagcttcctagtgtggtcccgatggacaatcgaatgcaaaggaacttgaactccatgattaagaaaggaaaaggaaaaaaaaatgtgaaaaaaaaatatcaaagttttaaaaaaagggtttgtctgccaagcaaacaaaagtcatggctttaacaaaagtcatggtatcatctacacatttttttttcctttgtgaagaactgtggctagactaaacaaaacagaacagtacagaactcagggattcaaaccaaggtaatatgtccttcttccctttctccagttggcattgccacattctacataagacaatgggggctgaagcctcatccttcatgctacctcaatcaagaagctttctttcttggacatgtgcacaagtttgtccttcttgtggtgtgagtattcactagggatgctccccctcctaaacttctcttgagttgagcccacaatccccacaaccattgggatgcattgcattgcatcagcagcaggtgttttcttgctgttgttaatcgttagaagtgtcatatttgcaccgtatgtctaggctagttccggctgatgggactgatgccacatgtgaatcatgagttgaatgtataaaaatttcagctttgccactgttgtcctttggatggatattatgcacagggaaaagtagatggagaggaaaacaaagagttgatcagctcctagttctggagttggttattagaaattataaaaaatggtggctctgctcagaagacatgggcatatgaaagcctggagtgcttaatgctcacattttcccttcaatgatagaaatggaagtaaacatttattaccatttggtcaagtgtagcttaacttgcattcatatttcattgttagtaatggaggtatgtggagatatacacagaccttgagacagctgttttttaatattgcatacaggctagcagttcattgaaaacagaggagagaagcctgaaggttagatcttagaagaaggcagttcttcatgcacagcttttgtcaatcctgatttggtttgaaaataaaaatcatggaataccaaaatcaaaggagagttgattaagggaaagggaaaaggggatcatcccaggaagggtgatgtcactggccaggaaaatgtcaggcgaggttccatgtcctcactcaagtccaaaggtgctggtttcctctactgctgttaacagcttttcatacaacatggagtacgagggatacggtggaagatccagtcggttgaagcatgtgtgtgccctggggagagaagtaattttcccccatttctctatgcagaagcgccgaagcccattgctcccacggagggctgcgaagccttcgtagggcacgctggatgttcccgtgacaaactgcagtaatctcagcctctgctcattattgaagcgctccaccgcagcccagaaccagcggatcacaagatgcccatcgtggtaacctccccggtactcagtgttattccgccagtcatttaggtcgatttccgcggtgccagctatcaccagctccagctccctggcatcaaacacggacaccagcctcgagtctacaacctcgtagaagccgcgcaccagcgcctcggtctgctgtaccacgccgcgctccacccgccacttcaccatgcgctcgatgtactccttcttgtttttctccgtcacctgtgtgttggctcctccagacttcaactccctttccgtgacctgtccaaaaacctcttcattaacagtgaaagtgaggtctaagatgtctgtgatgttgttgtccttcatccactgcaaactctggtggaattcctcatccaaatattccaggtcactcaaatcacagggcagtctcaggagtgccttgtagaagggcctcgtgaagaaagcgtcaagaaggtactgatggatcagagccagacccaggatgcgaccgctaaacctgaaccactcaagatggttttctacaaatgcggacatggggctgatctgcaccgtgtaagtatcatttgccgagtactcaaagagtccatagtaagggttgaagagctcctgagacagaaggaagaagaactcccgcgaggggccactgtagtccaggccctcctctccaacaaaggtgacgtagagcttgtttcgctggagctctttccgcgaataggccatcacctgattgaaggttccctccaacaaatgatcccggcgaataatgagcttaattttccccggaccctgaccaaatcctttggcttccagttttctgtagaaattgcggagcttggcctcaaagtctcttcggtagggggaaggggctcttgcactggctctctgtaaacctggggagttctgaggtgaagaacagggtgaacatcggggagagaagctatacccagggtggaaggcagcctgcagggggacgtaggacataatctcttcttcaaagagactcagcaaaatgaccagatccgcatcacaggacaacttctcaagcccgtgattaccctcagtccgaatgtaatggattttctccctgagtgtgtggtttcttgctaagcttggctgacgctcttgcagcatttcaaaaatgtttggctggcgaagaaatgccacaatcttgtcattatatgccagtggcaatgactcatgttgatgttggcttcgaatagcagctactaagctgtgtcctggcctggccagtaaagaggctcctctgtttctagaaacttctgaggcctctccagcgctgtaacttcggagcctctggaggtgctgtcggtgagttagatgattgggaagacgaccgttctgaagagggattcgggggtcaatgaaagtggtagctcgactgttgtggtccacgaaaaaagactttccctgctggtccgttttgatctcccagccccggggcagttccagccgagtgtctgcgaacatgttgatgaaattcaccaagtcccggttgtgctggtagcgttcaaaattgcgagcatcccgtcggactttcagaatcatgtgctttaagcaggtgctactggtgaagactcggtaggcactataattggcatgtagcacagtgaagaactcggggttggtgatgaacttgaccgctggggactgcagcagcaaggtgattttttgtgagttcactggagaaagtgacccttctctccttagatctaagctggactgggaagattcggcttctgagtcactccctccacctccgcctcctcctgctggggcttgctcgcagctttggctgccagaatcttcttcggacctctctgttgcaatggttcgctgaatgttttgataccgcctgttgagttgctccatctgctggatggaccccgatctccgcatgccatccggggtggctgctgccgtcggacgctgccaggtggttgtgcggttcacgtggtccacataaaagacccgcccgtggctgtcaattcgagcttcccagtttggtggaagaggctcatcgattgttgggtagtgatgatgttcaggcctcagggaaggaagctggcttactggctgggaattatggagtataggacattcaccttctctccgattgcttggacctgccacgggggattccagaccttccgggcttctttccacgtgcccgctaggggcggccagctcgtcttgccacggcccagcgccgttcgtggactccgggtccagctcagggctctgcatggagtcgggtaccgactcgaacgcgctgttctcctcctcctcgtcgtcttgcgaggagaagaccgtgctctcggagatcttggcgctgtccacggaggagaagcgcgtgtggctggcgaacctgttgccgttgtagcaggaggggctgtagcacgaggcgctgtagcacgagctgctgtagcaggacgtgctgtagcacgaggagctgtagcacgaggggctgcagcaggacgcgtcacagccctcgcaactgtggtccccgccttgcctggggctggagtcgctctcgctcccggtgctggggtgcgtgtcgccatcctgggccgcgccattggccaggctggggaagtggcccccggagtggccagggtgcgccgtgcctggagtagccccctcgggctcttctctgtcctcttccagggcagacgggtcagcggccaccgtgtccacctcgctgagcccatccttctccgaggagtccttgagggtggactcctcctccgcgccgtcctcctcctctgccgcgctgccgccctgggcggagggcatgctgtgcagcagggtgtggatgcggatgtagtgtgtccgcggggtctcggggtccccgcaggctgacgcgatcaccgtctccagctcggacacaggcaaggagcagggcctgctttttctcttcaccgaggcccgcagctgcagcctgccctctccctgctccagggtagacacatctccctcctcctcctgctccttctcctcttcttcccttccagcccggctctgggtcgttgcttcctcctccaagggctcctccttggtgctggctggggcttcaccgtcttccagcagcagtgctgatgcctcctcacccaggtccagctgctcggccagctcttctgcactgggggcaggctggatgtccttttgcacctgggccaggagctccccagccccttcaggtcccacagagaccatgccctggtctcctgcctccgtgatgactgctgcttcctcagctggtctggaaagctctatgctttggttccctggaccatcggggacactgccctcacccagctgctctggcttccagctctcagaggactctggtgcctcagaccgaggttccccactgccgctttccatcaggttgttcatggggctgtcctgaatttgggctgactcaggctcggtactcagggaaatctcctcatcatctgctgggtggatggaggaagtgatctcaaatcggaattgcagctgtccactcacatgatctgttggaagcctgcggccaagtgtgtagctgaccaccctatcccctatggcgtgtctctccaggagtctttgaacgggcatcgacagctttcccaagaagcgcttgatgatggggcggctcttggcaaacttgtccttcacctcaatttccagcacgtcagtgggcaaggacacaaaactgaattgctcggcctgccagatggggttcacggtgttgcctatgatcttggatctcctctcctgtccatggtgagggagggcggggaagatgctgtgtttcccaggctgaatggaaatcttcagataagggtctgggttgaaaaacatccctttcttcaaccccatggcttggaaatctgagagagagaagctgatcagcctccgacttccttgtccttggacggtctcatcagcaccaatgcttttaaaaataggagctgccgagtttttgaccgtgacactgggggtggttgctcgcagggccccactcactccatggtagtatttgaagcagatcttagtttcaggttccacaaagtacgagctggcatcgatcttccagatgatctggccccgatgagaaccattgactccacggtttttatagtccagaaagttttcggacaagacctcatcaatgaggtacatgccaatccagtccccagcgtccacttcctcctttatgtcccagtggatgaccaggtcctgagagtgcccgatggaatagtaggagctgctgaccatgagcgtggagcggctgtccgaggtgaccaggtcagtgtcgctggtggagcggggaatggtgacgccatcgtgggggccgcccctgaggtccatgttgtggaactggtcggggttgtagctgtatcggagcggctccttgcaccggcgtcggctctgggagtttctagaaggagacgccatggcggccaggcctaaaaacctgttctggtacagattcgtaatagccacagccggagtgagtctgctgatgagaaacgcagatctggccacctgctttgagacgccttggaccacaacactgccggggtctttaacggttggccttttcgggtagggcatctgccctcctaaatcgcgtttaaatcccaggaaaagagagaagatgcctccctcaatttttgaactatgctgctcttgctgtatccgtttctgctgaacatagcattgatatcttggcagccctggcctgggcacagatcatgctcctgtcagcgcgcagattagagctggggggcgcacgtgccccgcatagtgcaccg

SEQ ID NO: 14470 - RNA, 7143 nt, Homo sapiens
  source 1..7143: mol_type = other RNA
gctgggattacaggcatgagccaccgctcctggccggaatgctttagagtgtaggaacacaaataacacactgtccagacacaaactggtataatgagccattggcttcatatgaaattcacttcgtcttacatttctcccttgttttaatatggaaaacaattaaatgacatttaaatagtggggtctcttgagctcttctttttcccagtgaagaaaaacactttcatttatgacctatttcaggcaacatggataacaacgttagaaaaatagcaaatgaccattatggttgggtttatttcaaatgtagttgagaggttaggctgtctttggagcctgcagctgtttttctgacaacatgaagttttctgagatatgttttcactgaatgctaaaagaaactggatatttattttgatacaaatcaacgtgcctttggggtgttatgtttctgccccaggaggattactatgggtgaaggagaagtactatgttgcccttgatccctaacaagcaccatcactctctgcagcttcctagtgtggtcccgatggacaatcgaatgcaaaggaacttgaactccatgattaagaaaggaaaaggaaaaaaaaatgtgaaaaaaaaatatcaaagttttaaaaaaagggtttgtctgccaagcaaacaaaagtcatggctttaacaaaagtcatggtatcatctacacatttttttttcctttgtgaagaactgtggctagactaaacaaaacagaacagtacagaactcagggattcaaaccaaggtaatatgtccttcttccctttctccagttggcattgccacattctacataagacaatgggggctgaagcctcatccttcatgctacctcaatcaagaagctttctttcttggacatgtgcacaagtttgtccttcttgtggtgtgagtattcactagggatgctccccctcctaaacttctcttgagttgagcccacaatccccacaaccattgggatgcattgcattgcatcagcagcaggtgttttcttgctgttgttaatcgttagaagtgtcatatttgcaccgtatgtctaggctagttccggctgatgggactgatgccacatgtgaatcatgagttgaatgtataaaaatttcagctttgccactgttgtcctttggatggatattatgcacagggaaaagtagatggagaggaaaacaaagagttgatcagctcctagttctggagttggttattagaaattataaaaaatggtggctctgctcagaagacatgggcatatgaaagcctggagtgcttaatgctcacattttcccttcaatgatagaaatggaagtaaacatttattaccatttggtcaagtgtagcttaacttgcattcatatttcattgttagtaatggaggtatgtggagatatacacagaccttgagacagctgttttttaatattgcatacaggctagcagttcattgaaaacagaggagagaagcctgaaggttagatcttagaagaaggcagttcttcatgcacagcttttgtcaatcctgatttggtttgaaaataaaaatcatggaataccaaaatcaaaggagagttgattaagggaaagggaaaaggggatcatcccaggaagggtgatgtcactggccaggaaaatgtcaggcgaggttccatgtcctcactcaagtccaaaggtgctggtttcctctactgctgttaacagcttttcatacaacatggagtacgagggatacggtggaagatccagtcggttgaagcatgtgtgtgccctggggagagaagtaattttcccccatttctctatgcagaagcgccgaagcccattgctcccacggagggctgcgaagccttcgtagggcacgctggatgttcccgtgacaaactgcagtaatctcagcctctgctcattattgaagcgctccaccgcagcccagaaccagcggatcacaagatgcccatcgtggtaacctccccggtactcagtgttattccgccagtcatttaggtcgatttccgcggtgccagctatcaccagctccagctccctggcatcaaacacggacaccagcctcgagtctacaacctcgtagaagccgcgcaccagcgcctcggtctgctgtaccacgccgcgctccacccgccacttcaccatgcgctcgatgtactccttcttgtttttctccgtcacctgtgtgttggctcctccagacttcaactccctttccgtgacctgtccaaaaacctcttcattaacagtgaaagtgaggtctaagatgtctgtgatgttgttgtccttcatccactgcaaactctggtggaattcctcatccaaatattccaggtcactcaaatcacagggcagtctcaggagtgccttgtagaagggcctcgtgaagaaagcgtcaagaaggtactgatggatcagagccagacccaggatgcgaccgctaaacctgaaccactcaagatggttttctacaaatgcggacatggggctgatctgcaccgtgtaagtatcatttgccgagtactcaaagagtccatagtaagggttgaagagctcctgagacagaaggaagaagaactcccgcgaggggccactgtagtccaggccctcctctccaacaaaggtgacgtagagcttgtttcgctggagctctttccgcgaataggccatcacctgattgaaggttccctccaacaaatgatcccggcgaataatgagcttaattttccccggaccctgaccaaatcctttggcttccagttttctgtagaaattgcggagcttggcctcaaagtctcttcggtagggggaaggggctcttgcactggctctctgtaaacctggggagttctgaggtgaagaacagggtgaacatcggggagagaagctatacccagggtggaaggcagcctgcagggggacgtaggacataatctcttcttcaaagagactcagcaaaatgaccagatccgcatcacaggacaacttctcaagcccgtgattaccctcagtccgaatgtaatggattttctccctgagtgtgtggtttcttgctaagcttggctgacgctcttgcagcatttcaaaaatgtttggctggcgaagaaatgccacaatcttgtcattatatgccagtggcaatgactcatgttgatgttggcttcgaatagcagctactaagctgtgtcctggcctggccagtaaagaggctcctctgtttctagaaacttctgaggcctctccagcgctgtaacttcggagcctctggaggtgctgtcggtgagttagatgattgggaagacgaccgttctgaagagggattcgggggtcaatgaaagtggtagctcgactgttgtggtccacgaaaaaagactttccctgctggtccgttttgatctcccagccccggggcagttccagccgagtgtctgcgaacatgttgatgaaattcaccaagtcccggttgtgctggtagcgttcaaaattgcgagcatcccgtcggactttcagaatcatgtgctttaagcaggtgctactggtgaagactcggtaggcactataattggcatgtagcacagtgaagaactcggggttggtgatgaacttgaccgctggggactgcagcagcaaggtgattttttgtgagttcactggagaaagtgacccttctctccttagatctaagctggactgggaagattcggcttctgagtcactccctccacctccgcctcctcctgctggggcttgctcgcagctttggctgccagaatcttcttcggacctctctgttgcaatggttcgctgaatgttttgataccgcctgttgagttgctccatctgctggatggaccccgatctccgcatgccatccggggtggctgctgccgtcggacgctgccaggtggttgtgcggttcacgtggtccacataaaagacccgcccgtggctgtcaattcgagcttcccagtttggtggaagaggctcatcgattgttgggtagtgatgatgttcaggcctcagggaaggaagctggcttactggctgggaattatggagtataggacattcaccttctctccgattgcttggacctgccacgggggattccagaccttccgggcttctttccacgtgcccgctaggggcggccagctcgtcttgccacggcccagcgccgttcgtggactccgggtccagctcagggctctgcatggagtcgggtaccgactcgaacgcgctgttctcctcctcctcgtcgtcttgcgaggagaagaccgtgctctcggagatcttggcgctgtccacggaggagaagcgcgtgtggctggcgaacctgttgccgttgtagcaggaggggctgtagcacgaggcgctgtagcacgagctgctgtagcaggacgtgctgtagcacgaggagctgtagcacgaggggctgcagcaggacgcgtcacagccctcgcaactgtggtccccgccttgcctggggctggagtcgctctcgctcccggtgctggggtgcgtgtcgccatcctgggccgcgccattggccaggctggggaagtggcccccggagtggccagggtgcgccgtgcctggagtagccccctcgggctcttctctgtcctcttccagggcagacgggtcagcggccaccgtgtccacctcgctgagcccatccttctccgaggagtccttgagggtggactcctcctccgcgccgtcctcctcctctgccgcgctgccgccctgggcggagggcatgctgtgcagcagggtgtggatgcggatgtagtgtgtccgcggggtctcggggtccccgcaggctgacgcgatcaccgtctccagctcggacacaggcaaggagcagggcctgctttttctcttcaccgaggcccgcagctgcagcctgccctctccctgctccagggtagacacatctccctcctcctcctgctccttctcctcttcttcccttccagcccggctctgggtcgttgcttcctcctccaagggctcctccttggtgctggctggggcttcaccgtcttccagcagcagtgctgatgcctcctcacccaggtccagctgctcggccagctcttctgcactgggggcaggctggatgtccttttgcacctgggccaggagctccccagccccttcaggtcccacagagaccatgccctggtctcctgcctccgtgatgactgctgcttcctcagctggtctggaaagctctatgctttggttccctggaccatcggggacactgccctcacccagctgctctggcttccagctctcagaggactctggtgcctcagaccgaggttccccactgccgctttccatcaggttgttcatggggctgtcctgaatttgggctgactcaggctcggtactcagggaaatctcctcatcatctgctgggtggatggaggaagtgatctcaaatcggaattgcagctgtccactcacatgatctgttggaagcctgcggccaagtgtgtagctgaccaccctatcccctatggcgtgtctctccaggagtctttgaacgggcatcgacagctttcccaagaagcgcttgatgatggggcggctcttggcaaacttgtccttcacctcaatttccagcacgtcagtgggcaaggacacaaaactgaattgctcggcctgccagatggggttcacggtgttgcctatgatcttggatctcctctcctgtccatggtgagggagggcggggaagatgctgtgtttcccaggctgaatggaaatcttcagataagggtctgggttgaaaaacatccctttcttcaaccccatggcttggaaatctgagagagagaagctgatcagcctccgacttccttgtccttggacggtctcatcagcaccaatgcttttaaaaataggagctgccgagtttttgaccgtgacactgggggtggttgctcgcagggccccactcactccatggtagtatttgaagcagatcttagtttcaggttccacaaagtacgagctggcatcgatcttccagatgatctggccccgatgagaaccattgactccacggtttttatagtccagaaagttttcggacaagacctcatcaatgaggtacatgccaatccagtccccagcgtccacttcctcctttatgtcccagtggatgaccaggtcctgagagtgcccgatggaatagtaggagctgctgaccatgagcgtggagcggctgtccgaggtgaccaggtcagtgtcgctggtggagcggggaatggtgacgccatcgtgggggccgcccctgaggtccatgttgtggaactggtcggggttgtagctgtatcggagcggctccttgcaccggcgtcggctctgggagtttctagaaggagacgccatggcggccaggcctaaaaacctgttctggtacagattcgtaatagccacagccggagtgagtctgctgatgagaaacgcagatctggccacctgctttgagacgccttggaccacaacactgccggggtctttaacggttggccttttcgggtagggcatctgccctcctaaatcgcgtttaaatcccaggaaaagagagaagatgcctccctcaatttttgaactatgctgctcttgctgtatccgtttctgctgaacatagcattgatatcttttcaaagagaaggggggaaaacaaggggagaattgcaccactgcagattccaagagaagtaagcacaaaactacagcaacgtcaaataatatcttcttcggcaactaggaaaatccccacatgctctctggtgtcagcccaatgcagactgaggcgcgctgtgcccggaaccacaggaagccgggcatctctgcagcctgtgtccctgccagctccccctacgcgctgaaattcggcagggaagaagttatggtgcccagcctctgtgtgcaagacagagacaccgcgcatcatggctctgaaaatcagccaagtggccgggacgtcaaagcggcagagcaatcagaatgccctggagccggggatggaggggccacattgtttgagccctcggattttgctgcattgtcacc

SEQ ID NO: 14471 - RNA, 7076 nt, Homo sapiens
  source 1..7076: mol_type = other RNA
gctgggattacaggcatgagccaccgctcctggccggaatgctttagagtgtaggaacacaaataacacactgtccagacacaaactggtataatgagccattggcttcatatgaaattcacttcgtcttacatttctcccttgttttaatatggaaaacaattaaatgacatttaaatagtggggtctcttgagctcttctttttcccagtgaagaaaaacactttcatttatgacctatttcaggcaacatggataacaacgttagaaaaatagcaaatgaccattatggttgggtttatttcaaatgtagttgagaggttaggctgtctttggagcctgcagctgtttttctgacaacatgaagttttctgagatatgttttcactgaatgctaaaagaaactggatatttattttgatacaaatcaacgtgcctttggggtgttatgtttctgccccaggaggattactatgggtgaaggagaagtactatgttgcccttgatccctaacaagcaccatcactctctgcagcttcctagtgtggtcccgatggacaatcgaatgcaaaggaacttgaactccatgattaagaaaggaaaaggaaaaaaaaatgtgaaaaaaaaatatcaaagttttaaaaaaagggtttgtctgccaagcaaacaaaagtcatggctttaacaaaagtcatggtatcatctacacatttttttttcctttgtgaagaactgtggctagactaaacaaaacagaacagtacagaactcagggattcaaaccaaggtaatatgtccttcttccctttctccagttggcattgccacattctacataagacaatgggggctgaagcctcatccttcatgctacctcaatcaagaagctttctttcttggacatgtgcacaagtttgtccttcttgtggtgtgagtattcactagggatgctccccctcctaaacttctcttgagttgagcccacaatccccacaaccattgggatgcattgcattgcatcagcagcaggtgttttcttgctgttgttaatcgttagaagtgtcatatttgcaccgtatgtctaggctagttccggctgatgggactgatgccacatgtgaatcatgagttgaatgtataaaaatttcagctttgccactgttgtcctttggatggatattatgcacagggaaaagtagatggagaggaaaacaaagagttgatcagctcctagttctggagttggttattagaaattataaaaaatggtggctctgctcagaagacatgggcatatgaaagcctggagtgcttaatgctcacattttcccttcaatgatagaaatggaagtaaacatttattaccatttggtcaagtgtagcttaacttgcattcatatttcattgttagtaatggaggtatgtggagatatacacagaccttgagacagctgttttttaatattgcatacaggctagcagttcattgaaaacagaggagagaagcctgaaggttagatcttagaagaaggcagttcttcatgcacagcttttgtcaatcctgatttggtttgaaaataaaaatcatggaataccaaaatcaaaggagagttgattaagggaaagggaaaaggggatcatcccaggaagggtgatgtcactggccaggaaaatgtcaggcgaggttccatgtcctcactcaagtccaaaggtgctggtttcctctactgctgttaacagcttttcatacaacatggagtacgagggatacggtggaagatccagtcggttgaagcatgtgtgtgccctggggagagaagtaattttcccccatttctctatgcagaagcgccgaagcccattgctcccacggagggctgcgaagccttcgtagggcacgctggatgttcccgtgacaaactgcagtaatctcagcctctgctcattattgaagcgctccaccgcagcccagaaccagcggatcacaagatgcccatcgtggtaacctccccggtactcagtgttattccgccagtcatttaggtcgatttccgcggtgccagctatcaccagctccagctccctggcatcaaacacggacaccagcctcgagtctacaacctcgtagaagccgcgcaccagcgcctcggtctgctgtaccacgccgcgctccacccgccacttcaccatgcgctcgatgtactccttcttgtttttctccgtcacctgtgtgttggctcctccagacttcaactccctttccgtgacctgtccaaaaacctcttcattaacagtgaaagtgaggtctaagatgtctgtgatgttgttgtccttcatccactgcaaactctggtggaattcctcatccaaatattccaggtcactcaaatcacagggcagtctcaggagtgccttgtagaagggcctcgtgaagaaagcgtcaagaaggtactgatggatcagagccagacccaggatgcgaccgctaaacctgaaccactcaagatggttttctacaaatgcggacatggggctgatctgcaccgtgtaagtatcatttgccgagtactcaaagagtccatagtaagggttgaagagctcctgagacagaaggaagaagaactcccgcgaggggccactgtagtccaggccctcctctccaacaaaggtgacgtagagcttgtttcgctggagctctttccgcgaataggccatcacctgattgaaggttccctccaacaaatgatcccggcgaataatgagcttaattttccccggaccctgaccaaatcctttggcttccagttttctgtagaaattgcggagcttggcctcaaagtctcttcggtagggggaaggggctcttgcactggctctctgtaaacctggggagttctgaggtgaagaacagggtgaacatcggggagagaagctatacccagggtggaaggcagcctgcagggggacgtaggacataatctcttcttcaaagagactcagcaaaatgaccagatccgcatcacaggacaacttctcaagcccgtgattaccctcagtccgaatgtaatggattttctccctgagtgtgtggtttcttgctaagcttggctgacgctcttgcagcatttcaaaaatgtttggctggcgaagaaatgccacaatcttgtcattatatgccagtggcaatgactcatgttgatgttggcttcgaatagcagctactaagctgtgtcctggcctggccagtaaagaggctcctctgtttctagaaacttctgaggcctctccagcgctgtaacttcggagcctctggaggtgctgtcggtgagttagatgattgggaagacgaccgttctgaagagggattcgggggtcaatgaaagtggtagctcgactgttgtggtccacgaaaaaagactttccctgctggtccgttttgatctcccagccccggggcagttccagccgagtgtctgcgaacatgttgatgaaattcaccaagtcccggttgtgctggtagcgttcaaaattgcgagcatcccgtcggactttcagaatcatgtgctttaagcaggtgctactggtgaagactcggtaggcactataattggcatgtagcacagtgaagaactcggggttggtgatgaacttgaccgctggggactgcagcagcaaggtgattttttgtgagttcactggagaaagtgacccttctctccttagatctaagctggactgggaagattcggcttctgagtcactccctccacctccgcctcctcctgctggggcttgctcgcagctttggctgccagaatcttcttcggacctctctgttgcaatggttcgctgaatgttttgataccgcctgttgagttgctccatctgctggatggaccccgatctccgcatgccatccggggtggctgctgccgtcggacgctgccaggtggttgtgcggttcacgtggtccacataaaagacccgcccgtggctgtcaattcgagcttcccagtttggtggaagaggctcatcgattgttgggtagtgatgatgttcaggcctcagggaaggaagctggcttactggctgggaattatggagtataggacattcaccttctctccgattgcttggacctgccacgggggattccagaccttccgggcttctttccacgtgcccgctaggggcggccagctcgtcttgccacggcccagcgccgttcgtggactccgggtccagctcagggctctgcatggagtcgggtaccgactcgaacgcgctgttctcctcctcctcgtcgtcttgcgaggagaagaccgtgctctcggagatcttggcgctgtccacggaggagaagcgcgtgtggctggcgaacctgttgccgttgtagcaggaggggctgtagcacgaggcgctgtagcacgagctgctgtagcaggacgtgctgtagcacgaggagctgtagcacgaggggctgcagcaggacgcgtcacagccctcgcaactgtggtccccgccttgcctggggctggagtcgctctcgctcccggtgctggggtgcgtgtcgccatcctgggccgcgccattggccaggctggggaagtggcccccggagtggccagggtgcgccgtgcctggagtagccccctcgggctcttctctgtcctcttccagggcagacgggtcagcggccaccgtgtccacctcgctgagcccatccttctccgaggagtccttgagggtggactcctcctccgcgccgtcctcctcctctgccgcgctgccgccctgggcggagggcatgctgtgcagcagggtgtggatgcggatgtagtgtgtccgcggggtctcggggtccccgcaggctgacgcgatcaccgtctccagctcggacacaggcaaggagcagggcctgctttttctcttcaccgaggcccgcagctgcagcctgccctctccctgctccagggtagacacatctccctcctcctcctgctccttctcctcttcttcccttccagcccggctctgggtcgttgcttcctcctccaagggctcctccttggtgctggctggggcttcaccgtcttccagcagcagtgctgatgcctcctcacccaggtccagctgctcggccagctcttctgcactgggggcaggctggatgtccttttgcacctgggccaggagctccccagccccttcaggtcccacagagaccatgccctggtctcctgcctccgtgatgactgctgcttcctcagctggtctggaaagctctatgctttggttccctggaccatcggggacactgccctcacccagctgctctggcttccagctctcagaggactctggtgcctcagaccgaggttccccactgccgctttccatcaggttgttcatggggctgtcctgaatttgggctgactcaggctcggtactcagggaaatctcctcatcatctgctgggtggatggaggaagtgatctcaaatcggaattgcagctgtccactcacatgatctgttggaagcctgcggccaagtgtgtagctgaccaccctatcccctatggcgtgtctctccaggagtctttgaacgggcatcgacagctttcccaagaagcgcttgatgatggggcggctcttggcaaacttgtccttcacctcaatttccagcacgtcagtgggcaaggacacaaaactgaattgctcggcctgccagatggggttcacggtgttgcctatgatcttggatctcctctcctgtccatggtgagggagggcggggaagatgctgtgtttcccaggctgaatggaaatcttcagataagggtctgggttgaaaaacatccctttcttcaaccccatggcttggaaatctgagagagagaagctgatcagcctccgacttccttgtccttggacggtctcatcagcaccaatgcttttaaaaataggagctgccgagtttttgaccgtgacactgggggtggttgctcgcagggccccactcactccatggtagtatttgaagcagatcttagtttcaggttccacaaagtacgagctggcatcgatcttccagatgatctggccccgatgagaaccattgactccacggtttttatagtccagaaagttttcggacaagacctcatcaatgaggtacatgccaatccagtccccagcgtccacttcctcctttatgtcccagtggatgaccaggtcctgagagtgcccgatggaatagtaggagctgctgaccatgagcgtggagcggctgtccgaggtgaccaggtcagtgtcgctggtggagcggggaatggtgacgccatcgtgggggccgcccctgaggtccatgttgtggaactggtcggggttgtagctgtatcggagcggctccttgcaccggcgtcggctctgggagtttctagaaggagacgccatggcggccaggcctaaaaacctgttctggtacagattcttcacactacacaggtgcagcagcataatgacccaccacgtgtacgcgcatcaattccgtaatagccacagccggagtgagtctgctgatgagaaacgcagatctggccacctgctttgagacgccttggaccacaacactgccggggtctttaacggttggccttttcgggtagggcatctgccctcctaaatcgcgtttaaatcccaggaaaagagagaagatgcctccctcaatttttgaactatgctgctcttgctgtatccgtttctgctgaacatagcattgatatcttggcagccctggcctgggcacagatcatgctcctgtcagcgcgcagattagagctggggggcgcacgtgccccgcatagtgcaccgggcgcctgggactggctggggaggggaccctggcgaccgcccgctctcgctgcgctctggctgccgggtgccccgagagagcggaggccacggccactgtcacggcggaggggcgcgcgcggctcggcgagtgtgtgcgcgaggagggggccggttcggtcagagtcgcacggtgttccggctccaacaacagcgcctgatgc

SEQ ID NO: 14472 - RNA, 6695 nt, Homo sapiens
  source 1..6695: mol_type = other RNA
gctgggattacaggcatgagccaccgctcctggccggaatgctttagagtgtaggaacacaaataacacactgtccagacacaaactggtataatgagccattggcttcatatgaaattcacttcgtcttacatttctcccttgttttaatatggaaaacaattaaatgacatttaaatagtggggtctcttgagctcttctttttcccagtgaagaaaaacactttcatttatgacctatttcaggcaacatggataacaacgttagaaaaatagcaaatgaccattatggttgggtttatttcaaatgtagttgagaggttaggctgtctttggagcctgcagctgtttttctgacaacatgaagttttctgagatatgttttcactgaatgctaaaagaaactggatatttattttgatacaaatcaacgtgcctttggggtgttatgtttctgccccaggaggattactatgggtgaaggagaagtactatgttgcccttgatccctaacaagcaccatcactctctgcagcttcctagtgtggtcccgatggacaatcgaatgcaaaggaacttgaactccatgattaagaaaggaaaaggaaaaaaaaatgtgaaaaaaaaatatcaaagttttaaaaaaagggtttgtctgccaagcaaacaaaagtcatggctttaacaaaagtcatggtatcatctacacatttttttttcctttgtgaagaactgtggctagactaaacaaaacagaacagtacagaactcagggattcaaaccaaggtaatatgtccttcttccctttctccagttggcattgccacattctacataagacaatgggggctgaagcctcatccttcatgctacctcaatcaagaagctttctttcttggacatgtgcacaagtttgtccttcttgtggtgtgagtattcactagggatgctccccctcctaaacttctcttgagttgagcccacaatccccacaaccattgggatgcattgcattgcatcagcagcaggtgttttcttgctgttgttaatcgttagaagtgtcatatttgcaccgtatgtctaggctagttccggctgatgggactgatgccacatgtgaatcatgagttgaatgtataaaaatttcagctttgccactgttgtcctttggatggatattatgcacagggaaaagtagatggagaggaaaacaaagagttgatcagctcctagttctggagttggttattagaaattataaaaaatggtggctctgctcagaagacatgggcatatgaaagcctggagtgcttaatgctcacattttcccttcaatgatagaaatggaagtaaacatttattaccatttggtcaagtgtagcttaacttgcattcatatttcattgttagtaatggaggtatgtggagatatacacagaccttgagacagctgttttttaatattgcatacaggctagcagttcattgaaaacagaggagagaagcctgaaggttagatcttagaagaaggcagttcttcatgcacagcttttgtcaatcctgatttggtttgaaaataaaaatcatggaataccaaaatcaaaggagagttgattaagggaaagggaaaaggggatcatcccaggaagggtgatgtcactggccaggaaaatgtcaggcgaggttccatgtcctcactcaagtccaaaggtgctggtttcctctactgctgttaacagcttttcatacaacatggagtacgagggatacggtggaagatccagtcggttgaagcatgtgtgtgccctggggagagaagtaattttcccccatttctctatgcagaagcgccgaagcccattgctcccacggagggctgcgaagccttcgtagggcacgctggatgttcccgtgacaaactgcagtaatctcagcctctgctcattattgaagcgctccaccgcagcccagaaccagcggatcacaagatgcccatcgtggtaacctccccggtactcagtgttattccgccagtcatttaggtcgatttccgcggtgccagctatcaccagctccagctccctggcatcaaacacggacaccagcctcgagtctacaacctcgtagaagccgcgcaccagcgcctcggtctgctgtaccacgccgcgctccacccgccacttcaccatgcgctcgatgtactccttcttgtttttctccgtcacctgtgtgttggctcctccagacttcaactccctttccgtgacctgtccaaaaacctcttcattaacagtgaaagtgaggtctaagatgtctgtgatgttgttgtccttcatccactgcaaactctggtggaattcctcatccaaatattccaggtcactcaaatcacagggcagtctcaggagtgccttgtagaagggcctcgtgaagaaagcgtcaagaaggtactgatggatcagagccagacccaggatgcgaccgctaaacctgaaccactcaagatggttttctacaaatgcggacatggggctgatctgcaccgtgtaagtatcatttgccgagtactcaaagagtccatagtaagggttgaagagctcctgagacagaaggaagaagaactcccgcgaggggccactgtagtccaggccctcctctccaacaaaggtgacgtagagcttgtttcgctggagctctttccgcgaataggccatcacctgattgaaggttccctccaacaaatgatcccggcgaataatgagcttaattttccccggaccctgaccaaatcctttggcttccagttttctgtagaaattgcggagcttggcctcaaagtctcttcggtagggggaaggggctcttgcactggctctctgtaaacctggggagttctgaggtgaagaacagggtgaacatcggggagagaagctatacccagggtggaaggcagcctgcagggggacgtaggacataatctcttcttcaaagagactcagcaaaatgaccagatccgcatcacaggacaacttctcaagcccgtgattaccctcagtccgaatgtaatggattttctccctgagtgtgtggtttcttgctaagcttggctgacgctcttgcagcatttcaaaaatgtttggctggcgaagaaatgccacaatcttgtcattatatgccagtggcaatgactcatgttgatgttggcttcgaatagcagctactaagctgtgtcctggcctggccagtaaagaggctcctctgtttctagaaacttctgaggcctctccagcgctgtaacttcggagcctctggaggtgctgtcggtgagttagatgattgggaagacgaccgttctgaagagggattcgggggtcaatgaaagtggtagctcgactgttgtggtccacgaaaaaagactttccctgctggtccgttttgatctcccagccccggggcagttccagccgagtgtctgcgaacatgttgatgaaattcaccaagtcccggttgtgctggtagcgttcaaaattgcgagcatcccgtcggactttcagaatcatgtgctttaagcaggtgctactggtgaagactcggtaggcactataattggcatgtagcacagtgaagaactcggggttggtgatgaacttgaccgctggggactgcagcagcaaggtgattttttgtgagttcactggagaaagtgacccttctctccttagatctaagctggactgggaagattcggcttctgagtcactccctccacctccgcctcctcctgctggggcttgctcgcagctttggctgccagaatcttcttcggacctctctgttgcaatggttcgctgaatgttttgataccgcctgttgagttgctccatctgctggatggaccccgatctccgcatgccatccggggtggctgctgccgtcggacgctgccaggtggttgtgcggttcacgtggtccacataaaagacccgcccgtggctgtcaattcgagcttcccagtttggtggaagaggctcatcgattgttgggtagtgatgatgttcaggcctcagggaaggaagctggcttactggctgggaattatggagtataggacattcaccttctctccgattgcttggacctgccacgggggattccagaccttccgggcttctttccacgtgcccgctaggggcggccagctcgtcttgccacggcccagcgccgttcgtggactccgggtccagctcagggctctgcatggagtcgggtaccgactcgaacgcgctgttctcctcctcctcgtcgtcttgcgaggagaagaccgtgctctcggagatcttggcgctgtccacggaggagaagcgcgtgtggctggcgaacctgttgccgttgtagcaggaggggctgtagcacgaggcgctgtagcacgagctgctgtagcaggacgtgctgtagcacgaggagctgtagcacgaggggctgcagcaggacgcgtcacagccctcgcaactgtggtccccgccttgcctggggctggagtcgctctcgctcccggtgctggggtgcgtgtcgccatcctgggccgcgccattggccaggctggggaagtggcccccggagtggccagggtgcgccgtgcctggagtagccccctcgggctcttctctgtcctcttccagggcagacgggtcagcggccaccgtgtccacctcgctgagcccatccttctccgaggagtccttgagggtggactcctcctccgcgccgtcctcctcctctgccgcgctgccgccctgggcggagggcatgctgtgcagcagggtgtggatgcggatgtagtgtgtccgcggggtctcggggtccccgcaggctgacgcgatcaccgtctccagctcggacacaggcaaggagcagggcctgctttttctcttcaccgaggcccgcagctgcagcctgccctctccctgctccagggtagacacatctccctcctcctcctgctccttctcctcttcttcccttccagcccggctctgggtcgttgcttcctcctccaagggctcctccttggtgctggctggggcttcaccgtcttccagcagcagtgctgatgcctcctcacccaggtccagctgctcggccagctcttctgcactgggggcaggctggatgtccttttgcacctgggccaggagctccccagccccttcaggtcccacagagaccatgccctggtctcctgcctccgtgatgactgctgcttcctcagctggtctggaaagctctatgctttggttccctggaccatcggggacactgccctcacccagctgctctggcttccagctctcagaggactctggtgcctcagaccgaggttccccactgccgctttccatcaggttgttcatggggctgtcctgaatttgggctgactcaggctcggtactcagggaaatctcctcatcatctgctgggtggatggaggaagtgatctcaaatcggaattgcagctgtccactcacatgatctgttggaagcctgcggccaagtgtgtagctgaccaccctatcccctatggcgtgtctctccaggagtctttgaacgggcatcgacagctttcccaagaagcgcttgatgatggggcggctcttggcaaacttgtccttcacctcaatttccagcacgtcagtgggcaaggacacaaaactgaattgctcggcctgccagatggggttcacggtgttgcctatgatcttggatctcctctcctgtccatggtgagggagggcggggaagatgctgtgtttcccaggctgaatggaaatcttcagataagggtctgggttgaaaaacatccctttcttcaaccccatggcttggaaatctgagagagagaagctgatcagcctccgacttccttgtccttggacggtctcatcagcaccaatgcttttaaaaataggagctgccgagtttttgaccgtgacactgggggtggttgctcgcagggccccactcactccatggtagtatttgaagcagatcttagtttcaggttccacaaagtacgagctggcatcgatcttccagatgatctggccccgatgagaaccattgactccacggtttttatagtccagaaagttttcggacaagacctcatcaatgaggtacatgccaatccagtccccagcgtccacttcctcctttatgtcccagtggatgaccaggtcctgagagtgcccgatggaatagtaggagctgctgaccatgagcgtggagcggctgtccgaggtgaccaggtcagtgtcgctggtggagcggggaatggtgacgccatcgtgggggccgcccctgaggtccatgttgtggaactggtcggggttgtagctgtatcggagcggctccttgcaccggcgtcggctctgggagtttctagaaggagacgccatggcggccaggcctaaaaacctgttctggtacagattcttcacactacacaggtgcagcagcataatgacccaccacgtgtacgcgcatcaattccttgcacctgcctcttctgtcccactttgctcttcctggccagggtcctgggacgctgactgggaggaggcattcatgggccccctcacccgctgcctcccagctgggttcagccaatgtggaacacacagaagactggagggag

SEQ ID NO: 14473 - RNA, 6866 nt, Homo sapiens
  source 1..6866: mol_type = other RNA
gctgggattacaggcatgagccaccgctcctggccggaatgctttagagtgtaggaacacaaataacacactgtccagacacaaactggtataatgagccattggcttcatatgaaattcacttcgtcttacatttctcccttgttttaatatggaaaacaattaaatgacatttaaatagtggggtctcttgagctcttctttttcccagtgaagaaaaacactttcatttatgacctatttcaggcaacatggataacaacgttagaaaaatagcaaatgaccattatggttgggtttatttcaaatgtagttgagaggttaggctgtctttggagcctgcagctgtttttctgacaacatgaagttttctgagatatgttttcactgaatgctaaaagaaactggatatttattttgatacaaatcaacgtgcctttggggtgttatgtttctgccccaggaggattactatgggtgaaggagaagtactatgttgcccttgatccctaacaagcaccatcactctctgcagcttcctagtgtggtcccgatggacaatcgaatgcaaaggaacttgaactccatgattaagaaaggaaaaggaaaaaaaaatgtgaaaaaaaaatatcaaagttttaaaaaaagggtttgtctgccaagcaaacaaaagtcatggctttaacaaaagtcatggtatcatctacacatttttttttcctttgtgaagaactgtggctagactaaacaaaacagaacagtacagaactcagggattcaaaccaaggtaatatgtccttcttccctttctccagttggcattgccacattctacataagacaatgggggctgaagcctcatccttcatgctacctcaatcaagaagctttctttcttggacatgtgcacaagtttgtccttcttgtggtgtgagtattcactagggatgctccccctcctaaacttctcttgagttgagcccacaatccccacaaccattgggatgcattgcattgcatcagcagcaggtgttttcttgctgttgttaatcgttagaagtgtcatatttgcaccgtatgtctaggctagttccggctgatgggactgatgccacatgtgaatcatgagttgaatgtataaaaatttcagctttgccactgttgtcctttggatggatattatgcacagggaaaagtagatggagaggaaaacaaagagttgatcagctcctagttctggagttggttattagaaattataaaaaatggtggctctgctcagaagacatgggcatatgaaagcctggagtgcttaatgctcacattttcccttcaatgatagaaatggaagtaaacatttattaccatttggtcaagtgtagcttaacttgcattcatatttcattgttagtaatggaggtatgtggagatatacacagaccttgagacagctgttttttaatattgcatacaggctagcagttcattgaaaacagaggagagaagcctgaaggttagatcttagaagaaggcagttcttcatgcacagcttttgtcaatcctgatttggtttgaaaataaaaatcatggaataccaaaatcaaaggagagttgattaagggaaagggaaaaggggatcatcccaggaagggtgatgtcactggccaggaaaatgtcaggcgaggttccatgtcctcactcaagtccaaaggtgctggtttcctctactgctgttaacagcttttcatacaacatggagtacgagggatacggtggaagatccagtcggttgaagcatgtgtgtgccctggggagagaagtaattttcccccatttctctatgcagaagcgccgaagcccattgctcccacggagggctgcgaagccttcgtagggcacgctggatgttcccgtgacaaactgcagtaatctcagcctctgctcattattgaagcgctccaccgcagcccagaaccagcggatcacaagatgcccatcgtggtaacctccccggtactcagtgttattccgccagtcatttaggtcgatttccgcggtgccagctatcaccagctccagctccctggcatcaaacacggacaccagcctcgagtctacaacctcgtagaagccgcgcaccagcgcctcggtctgctgtaccacgccgcgctccacccgccacttcaccatgcgctcgatgtactccttcttgtttttctccgtcacctgtgtgttggctcctccagacttcaactccctttccgtgacctgtccaaaaacctcttcattaacagtgaaagtgaggtctaagatgtctgtgatgttgttgtccttcatccactgcaaactctggtggaattcctcatccaaatattccaggtcactcaaatcacagggcagtctcaggagtgccttgtagaagggcctcgtgaagaaagcgtcaagaaggtactgatggatcagagccagacccaggatgcgaccgctaaacctgaaccactcaagatggttttctacaaatgcggacatggggctgatctgcaccgtgtaagtatcatttgccgagtactcaaagagtccatagtaagggttgaagagctcctgagacagaaggaagaagaactcccgcgaggggccactgtagtccaggccctcctctccaacaaaggtgacgtagagcttgtttcgctggagctctttccgcgaataggccatcacctgattgaaggttccctccaacaaatgatcccggcgaataatgagcttaattttccccggaccctgaccaaatcctttggcttccagttttctgtagaaattgcggagcttggcctcaaagtctcttcggtagggggaaggggctcttgcactggctctctgtaaacctggggagttctgaggtgaagaacagggtgaacatcggggagagaagctatacccagggtggaaggcagcctgcagggggacgtaggacataatctcttcttcaaagagactcagcaaaatgaccagatccgcatcacaggacaacttctcaagcccgtgattaccctcagtccgaatgtaatggattttctccctgagtgtgtggtttcttgctaagcttggctgacgctcttgcagcatttcaaaaatgtttggctggcgaagaaatgccacaatcttgtcattatatgccagtggcaatgactcatgttgatgttggcttcgaatagcagctactaagctgtgtcctggcctggccagtaaagaggctcctctgtttctagaaacttctgaggcctctccagcgctgtaacttcggagcctctggaggtgctgtcggtgagttagatgattgggaagacgaccgttctgaagagggattcgggggtcaatgaaagtggtagctcgactgttgtggtccacgaaaaaagactttccctgctggtccgttttgatctcccagccccggggcagttccagccgagtgtctgcgaacatgttgatgaaattcaccaagtcccggttgtgctggtagcgttcaaaattgcgagcatcccgtcggactttcagaatcatgtgctttaagcaggtgctactggtgaagactcggtaggcactataattggcatgtagcacagtgaagaactcggggttggtgatgaacttgaccgctggggactgcagcagcaaggtgattttttgtgagttcactggagaaagtgacccttctctccttagatctaagctggactgggaagattcggcttctgagtcactccctccacctccgcctcctcctgctggggcttgctcgcagctttggctgccagaatcttcttcggacctctctgttgcaatggttcgctgaatgttttgataccgcctgttgagttgctccatctgctggatggaccccgatctccgcatgccatccggggtggctgctgccgtcggacgctgccaggtggttgtgcggttcacgtggtccacataaaagacccgcccgtggctgtcaattcgagcttcccagtttggtggaagaggctcatcgattgttgggtagtgatgatgttcaggcctcagggaaggaagctggcttactggctgggaattatggagtataggacattcaccttctctccgattgcttggacctgccacgggggattccagaccttccgggcttctttccacgtgcccgctaggggcggccagctcgtcttgccacggcccagcgccgttcgtggactccgggtccagctcagggctctgcatggagtcgggtaccgactcgaacgcgctgttctcctcctcctcgtcgtcttgcgaggagaagaccgtgctctcggagatcttggcgctgtccacggaggagaagcgcgtgtggctggcgaacctgttgccgttgtagcaggaggggctgtagcacgaggcgctgtagcacgagctgctgtagcaggacgtgctgtagcacgaggagctgtagcacgaggggctgcagcaggacgcgtcacagccctcgcaactgtggtccccgccttgcctggggctggagtcgctctcgctcccggtgctggggtgcgtgtcgccatcctgggccgcgccattggccaggctggggaagtggcccccggagtggccagggtgcgccgtgcctggagtagccccctcgggctcttctctgtcctcttccagggcagacgggtcagcggccaccgtgtccacctcgctgagcccatccttctccgaggagtccttgagggtggactcctcctccgcgccgtcctcctcctctgccgcgctgccgccctgggcggagggcatgctgtgcagcagggtgtggatgcggatgtagtgtgtccgcggggtctcggggtccccgcaggctgacgcgatcaccgtctccagctcggacacaggcaaggagcagggcctgctttttctcttcaccgaggcccgcagctgcagcctgccctctccctgctccagggtagacacatctccctcctcctcctgctccttctcctcttcttcccttccagcccggctctgggtcgttgcttcctcctccaagggctcctccttggtgctggctggggcttcaccgtcttccagcagcagtgctgatgcctcctcacccaggtccagctgctcggccagctcttctgcactgggggcaggctggatgtccttttgcacctgggccaggagctccccagccccttcaggtcccacagagaccatgccctggtctcctgcctccgtgatgactgctgcttcctcagctggtctggaaagctctatgctttggttccctggaccatcggggacactgccctcacccagctgctctggcttccagctctcagaggactctggtgcctcagaccgaggttccccactgccgctttccatcaggttgttcatggggctgtcctgaatttgggctgactcaggctcggtactcagggaaatctcctcatcatctgctgggtggatggaggaagtgatctcaaatcggaattgcagctgtccactcacatgatctgttggaagcctgcggccaagtgtgtagctgaccaccctatcccctatggcgtgtctctccaggagtctttgaacgggcatcgacagctttcccaagaagcgcttgatgatggggcggctcttggcaaacttgtccttcacctcaatttccagcacgtcagtgggcaaggacacaaaactgaattgctcggcctgccagatggggttcacggtgttgcctatgatcttggatctcctctcctgtccatggtgagggagggcggggaagatgctgtgtttcccaggctgaatggaaatcttcagataagggtctgggttgaaaaacatccctttcttcaaccccatggcttggaaatctgagagagagaagctgatcagcctccgacttccttgtccttggacggtctcatcagcaccaatgcttttaaaaataggagctgccgagtttttgaccgtgacactgggggtggttgctcgcagggccccactcactccatggtagtatttgaagcagatcttagtttcaggttccacaaagtacgagctggcatcgatcttccagatgatctggccccgatgagaaccattgactccacggtttttatagtccagaaagttttcggacaagacctcatcaatgaggtacatgccaatccagtccccagcgtccacttcctcctttatgtcccagtggatgaccaggtcctgagagtgcccgatggaatagtaggagctgctgaccatgagcgtggagcggctgtccgaggtgaccaggtcagtgtcgctggtggagcggggaatggtgacgccatcgtgggggccgcccctgaggtccatgttgtggaactggtcggggttgtagctgtatcggagcggctccttgcaccggcgtcggctctgggagtttctagaaggagacgccatggcggccaggcctaaaaacctgttctggtacagattcttcacactacacaggtgcagcagcataatgacccaccacgtgtacgcgcatcaattccttggcagccctggcctgggcacagatcatgctcctgtcagcgcgcagattagagctggggggcgcacgtgccccgcatagtgcaccgggcgcctgggactggctggggaggggaccctggcgaccgcccgctctcgctgcgctctggctgccgggtgccccgagagagcggaggccacggccactgtcacggcggaggggcgcgcgcggctcggcgagtgtgtgcgcgaggagggggccggttcggtcagagtcgcacggtgttccggctccaacaacagcgcctgatgcgcggtaacgcagcacacttcatcgc

SEQ ID NO: 14474 - RNA, 6636 nt, Homo sapiens
  source 1..6636: mol_type = other RNA
gctgggattacaggcatgagccaccgctcctggccggaatgctttagagtgtaggaacacaaataacacactgtccagacacaaactggtataatgagccattggcttcatatgaaattcacttcgtcttacatttctcccttgttttaatatggaaaacaattaaatgacatttaaatagtggggtctcttgagctcttctttttcccagtgaagaaaaacactttcatttatgacctatttcaggcaacatggataacaacgttagaaaaatagcaaatgaccattatggttgggtttatttcaaatgtagttgagaggttaggctgtctttggagcctgcagctgtttttctgacaacatgaagttttctgagatatgttttcactgaatgctaaaagaaactggatatttattttgatacaaatcaacgtgcctttggggtgttatgtttctgccccaggaggattactatgggtgaaggagaagtactatgttgcccttgatccctaacaagcaccatcactctctgcagcttcctagtgtggtcccgatggacaatcgaatgcaaaggaacttgaactccatgattaagaaaggaaaaggaaaaaaaaatgtgaaaaaaaaatatcaaagttttaaaaaaagggtttgtctgccaagcaaacaaaagtcatggctttaacaaaagtcatggtatcatctacacatttttttttcctttgtgaagaactgtggctagactaaacaaaacagaacagtacagaactcagggattcaaaccaaggtaatatgtccttcttccctttctccagttggcattgccacattctacataagacaatgggggctgaagcctcatccttcatgctacctcaatcaagaagctttctttcttggacatgtgcacaagtttgtccttcttgtggtgtgagtattcactagggatgctccccctcctaaacttctcttgagttgagcccacaatccccacaaccattgggatgcattgcattgcatcagcagcaggtgttttcttgctgttgttaatcgttagaagtgtcatatttgcaccgtatgtctaggctagttccggctgatgggactgatgccacatgtgaatcatgagttgaatgtataaaaatttcagctttgccactgttgtcctttggatggatattatgcacagggaaaagtagatggagaggaaaacaaagagttgatcagctcctagttctggagttggttattagaaattataaaaaatggtggctctgctcagaagacatgggcatatgaaagcctggagtgcttaatgctcacattttcccttcaatgatagaaatggaagtaaacatttattaccatttggtcaagtgtagcttaacttgcattcatatttcattgttagtaatggaggtatgtggagatatacacagaccttgagacagctgttttttaatattgcatacaggctagcagttcattgaaaacagaggagagaagcctgaaggttagatcttagaagaaggcagttcttcatgcacagcttttgtcaatcctgatttggtttgaaaataaaaatcatggaataccaaaatcaaaggagagttgattaagggaaagggaaaaggggatcatcccaggaagggtgatgtcactggccaggaaaatgtcaggcgaggttccatgtcctcactcaagtccaaaggtgctggtttcctctactgctgttaacagcttttcatacaacatggagtacgagggatacggtggaagatccagtcggttgaagcatgtgtgtgccctggggagagaagtaattttcccccatttctctatgcagaagcgccgaagcccattgctcccacggagggctgcgaagccttcgtagggcacgctggatgttcccgtgacaaactgcagtaatctcagcctctgctcattattgaagcgctccaccgcagcccagaaccagcggatcacaagatgcccatcgtggtaacctccccggtactcagtgttattccgccagtcatttaggtcgatttccgcggtgccagctatcaccagctccagctccctggcatcaaacacggacaccagcctcgagtctacaacctcgtagaagccgcgcaccagcgcctcggtctgctgtaccacgccgcgctccacccgccacttcaccatgcgctcgatgtactccttcttgtttttctccgtcacctgtgtgttggctcctccagacttcaactccctttccgtgacctgtccaaaaacctcttcattaacagtgaaagtgaggtctaagatgtctgtgatgttgttgtccttcatccactgcaaactctggtggaattcctcatccaaatattccaggtcactcaaatcacagggcagtctcaggagtgccttgtagaagggcctcgtgaagaaagcgtcaagaaggtactgatggatcagagccagacccaggatgcgaccgctaaacctgaaccactcaagatggttttctacaaatgcggacatggggctgatctgcaccgtgtaagtatcatttgccgagtactcaaagagtccatagtaagggttgaagagctcctgagacagaaggaagaagaactcccgcgaggggccactgtagtccaggccctcctctccaacaaaggtgacgtagagcttgtttcgctggagctctttccgcgaataggccatcacctgattgaaggttccctccaacaaatgatcccggcgaataatgagcttaattttccccggaccctgaccaaatcctttggcttccagttttctgtagaaattgcggagcttggcctcaaagtctcttcggtagggggaaggggctcttgcactggctctctgtaaacctggggagttctgaggtgaagaacagggtgaacatcggggagagaagctatacccagggtggaaggcagcctgcagggggacgtaggacataatctcttcttcaaagagactcagcaaaatgaccagatccgcatcacaggacaacttctcaagcccgtgattaccctcagtccgaatgtaatggattttctccctgagtgtgtggtttcttgctaagcttggctgacgctcttgcagcatttcaaaaatgtttggctggcgaagaaatgccacaatcttgtcattatatgccagtggcaatgactcatgttgatgttggcttcgaatagcagctactaagctgtgtcctggcctggccagtaaagaggctcctctgtttctagaaacttctgaggcctctccagcgctgtaacttcggagcctctggaggtgctgtcggtgagttagatgattgggaagacgaccgttctgaagagggattcgggggtcaatgaaagtggtagctcgactgttgtggtccacgaaaaaagactttccctgctggtccgttttgatctcccagccccggggcagttccagccgagtgtctgcgaacatgttgatgaaattcaccaagtcccggttgtgctggtagcgttcaaaattgcgagcatcccgtcggactttcagaatcatgtgctttaagcaggtgctactggtgaagactcggtaggcactataattggcatgtagcacagtgaagaactcggggttggtgatgaacttgaccgctggggactgcagcagcaaggtgattttttgtgagttcactggagaaagtgacccttctctccttagatctaagctggactgggaagattcggcttctgagtcactccctccacctccgcctcctcctgctggggcttgctcgcagctttggctgccagaatcttcttcggacctctctgttgcaatggttcgctgaatgttttgataccgcctgttgagttgctccatctgctggatggaccccgatctccgcatgccatccggggtggctgctgccgtcggacgctgccaggtggttgtgcggttcacgtggtccacataaaagacccgcccgtggctgtcaattcgagcttcccagtttggtggaagaggctcatcgattgttgggtagtgatgatgttcaggcctcagggaaggaagctggcttactggctgggaattatggagtataggacattcaccttctctccgattgcttggacctgccacgggggattccagaccttccgggcttctttccacgtgcccgctaggggcggccagctcgtcttgccacggcccagcgccgttcgtggactccgggtccagctcagggctctgcatggagtcgggtaccgactcgaacgcgctgttctcctcctcctcgtcgtcttgcgaggagaagaccgtgctctcggagatcttggcgctgtccacggaggagaagcgcgtgtggctggcgaacctgttgccgttgtagcaggaggggctgtagcacgaggcgctgtagcacgagctgctgtagcaggacgtgctgtagcacgaggagctgtagcacgaggggctgcagcaggacgcgtcacagccctcgcaactgtggtccccgccttgcctggggctggagtcgctctcgctcccggtgctggggtgcgtgtcgccatcctgggccgcgccattggccaggctggggaagtggcccccggagtggccagggtgcgccgtgcctggagtagccccctcgggctcttctctgtcctcttccagggcagacgggtcagcggccaccgtgtccacctcgctgagcccatccttctccgaggagtccttgagggtggactcctcctccgcgccgtcctcctcctctgccgcgctgccgccctgggcggagggcatgctgtgcagcagggtgtggatgcggatgtagtgtgtccgcggggtctcggggtccccgcaggctgacgcgatcaccgtctccagctcggacacaggcaaggagcagggcctgctttttctcttcaccgaggcccgcagctgcagcctgccctctccctgctccagggtagacacatctccctcctcctcctgctccttctcctcttcttcccttccagcccggctctgggtcgttgcttcctcctccaagggctcctccttggtgctggctggggcttcaccgtcttccagcagcagtgctgatgcctcctcacccaggtccagctgctcggccagctcttctgcactgggggcaggctggatgtccttttgcacctgggccaggagctccccagccccttcaggtcccacagagaccatgccctggtctcctgcctccgtgatgactgctgcttcctcagctggtctggaaagctctatgctttggttccctggaccatcggggacactgccctcacccagctgctctggcttccagctctcagaggactctggtgcctcagaccgaggttccccactgccgctttccatcaggttgttcatggggctgtcctgaatttgggctgactcaggctcggtactcagggaaatctcctcatcatctgctgggtggatggaggaagtgatctcaaatcggaattgcagctgtccactcacatgatctgttggaagcctgcggccaagtgtgtagctgaccaccctatcccctatggcgtgtctctccaggagtctttgaacgggcatcgacagctttcccaagaagcgcttgatgatggggcggctcttggcaaacttgtccttcacctcaatttccagcacgtcagtgggcaaggacacaaaactgaattgctcggcctgccagatggggttcacggtgttgcctatgatcttggatctcctctcctgtccatggtgagggagggcggggaagatgctgtgtttcccaggctgaatggaaatcttcagataagggtctgggttgaaaaacatccctttcttcaaccccatggcttggaaatctgagagagagaagctgatcagcctccgacttccttgtccttggacggtctcatcagcaccaatgcttttaaaaataggagctgccgagtttttgaccgtgacactgggggtggttgctcgcagggccccactcactccatggtagtatttgaagcagatcttagtttcaggttccacaaagtacgagctggcatcgatcttccagatgatctggccccgatgagaaccattgactccacggtttttatagtccagaaagttttcggacaagacctcatcaatgaggtacatgccaatccagtccccagcgtccacttcctcctttatgtcccagtggatgaccaggtcctgagagtgcccgatggaatagtaggagctgctgaccatgagcgtggagcggctgtccgaggtgaccaggtcagtgtcgctggtggagcggggaatggtgacgccatcgtgggggccgcccctgaggtccatgttgtggaactggtcggggttgtagctgtatcggagcggctccttgcaccggcgtcggctctgggagtttctagaaggagacgccatggcggccaggcctaaaaacctgttctggtacagattcttgcacctgcctcttctgtcccactttgctcttcctggccagggtcctgggacgctgactgggaggaggcattcatgggccccctcacccgctgcctcccagctgggttcagccaatgtggaacacacagaagactggaggga

SEQ ID NO: 14475 - RNA, 6801 nt, Homo sapiens
  source 1..6801: mol_type = other RNA
gctgggattacaggcatgagccaccgctcctggccggaatgctttagagtgtaggaacacaaataacacactgtccagacacaaactggtataatgagccattggcttcatatgaaattcacttcgtcttacatttctcccttgttttaatatggaaaacaattaaatgacatttaaatagtggggtctcttgagctcttctttttcccagtgaagaaaaacactttcatttatgacctatttcaggcaacatggataacaacgttagaaaaatagcaaatgaccattatggttgggtttatttcaaatgtagttgagaggttaggctgtctttggagcctgcagctgtttttctgacaacatgaagttttctgagatatgttttcactgaatgctaaaagaaactggatatttattttgatacaaatcaacgtgcctttggggtgttatgtttctgccccaggaggattactatgggtgaaggagaagtactatgttgcccttgatccctaacaagcaccatcactctctgcagcttcctagtgtggtcccgatggacaatcgaatgcaaaggaacttgaactccatgattaagaaaggaaaaggaaaaaaaaatgtgaaaaaaaaatatcaaagttttaaaaaaagggtttgtctgccaagcaaacaaaagtcatggctttaacaaaagtcatggtatcatctacacatttttttttcctttgtgaagaactgtggctagactaaacaaaacagaacagtacagaactcagggattcaaaccaaggtaatatgtccttcttccctttctccagttggcattgccacattctacataagacaatgggggctgaagcctcatccttcatgctacctcaatcaagaagctttctttcttggacatgtgcacaagtttgtccttcttgtggtgtgagtattcactagggatgctccccctcctaaacttctcttgagttgagcccacaatccccacaaccattgggatgcattgcattgcatcagcagcaggtgttttcttgctgttgttaatcgttagaagtgtcatatttgcaccgtatgtctaggctagttccggctgatgggactgatgccacatgtgaatcatgagttgaatgtataaaaatttcagctttgccactgttgtcctttggatggatattatgcacagggaaaagtagatggagaggaaaacaaagagttgatcagctcctagttctggagttggttattagaaattataaaaaatggtggctctgctcagaagacatgggcatatgaaagcctggagtgcttaatgctcacattttcccttcaatgatagaaatggaagtaaacatttattaccatttggtcaagtgtagcttaacttgcattcatatttcattgttagtaatggaggtatgtggagatatacacagaccttgagacagctgttttttaatattgcatacaggctagcagttcattgaaaacagaggagagaagcctgaaggttagatcttagaagaaggcagttcttcatgcacagcttttgtcaatcctgatttggtttgaaaataaaaatcatggaataccaaaatcaaaggagagttgattaagggaaagggaaaaggggatcatcccaggaagggtgatgtcactggccaggaaaatgtcaggcgaggttccatgtcctcactcaagtccaaaggtgctggtttcctctactgctgttaacagcttttcatacaacatggagtacgagggatacggtggaagatccagtcggttgaagcatgtgtgtgccctggggagagaagtaattttcccccatttctctatgcagaagcgccgaagcccattgctcccacggagggctgcgaagccttcgtagggcacgctggatgttcccgtgacaaactgcagtaatctcagcctctgctcattattgaagcgctccaccgcagcccagaaccagcggatcacaagatgcccatcgtggtaacctccccggtactcagtgttattccgccagtcatttaggtcgatttccgcggtgccagctatcaccagctccagctccctggcatcaaacacggacaccagcctcgagtctacaacctcgtagaagccgcgcaccagcgcctcggtctgctgtaccacgccgcgctccacccgccacttcaccatgcgctcgatgtactccttcttgtttttctccgtcacctgtgtgttggctcctccagacttcaactccctttccgtgacctgtccaaaaacctcttcattaacagtgaaagtgaggtctaagatgtctgtgatgttgttgtccttcatccactgcaaactctggtggaattcctcatccaaatattccaggtcactcaaatcacagggcagtctcaggagtgccttgtagaagggcctcgtgaagaaagcgtcaagaaggtactgatggatcagagccagacccaggatgcgaccgctaaacctgaaccactcaagatggttttctacaaatgcggacatggggctgatctgcaccgtgtaagtatcatttgccgagtactcaaagagtccatagtaagggttgaagagctcctgagacagaaggaagaagaactcccgcgaggggccactgtagtccaggccctcctctccaacaaaggtgacgtagagcttgtttcgctggagctctttccgcgaataggccatcacctgattgaaggttccctccaacaaatgatcccggcgaataatgagcttaattttccccggaccctgaccaaatcctttggcttccagttttctgtagaaattgcggagcttggcctcaaagtctcttcggtagggggaaggggctcttgcactggctctctgtaaacctggggagttctgaggtgaagaacagggtgaacatcggggagagaagctatacccagggtggaaggcagcctgcagggggacgtaggacataatctcttcttcaaagagactcagcaaaatgaccagatccgcatcacaggacaacttctcaagcccgtgattaccctcagtccgaatgtaatggattttctccctgagtgtgtggtttcttgctaagcttggctgacgctcttgcagcatttcaaaaatgtttggctggcgaagaaatgccacaatcttgtcattatatgccagtggcaatgactcatgttgatgttggcttcgaatagcagctactaagctgtgtcctggcctggccagtaaagaggctcctctgtttctagaaacttctgaggcctctccagcgctgtaacttcggagcctctggaggtgctgtcggtgagttagatgattgggaagacgaccgttctgaagagggattcgggggtcaatgaaagtggtagctcgactgttgtggtccacgaaaaaagactttccctgctggtccgttttgatctcccagccccggggcagttccagccgagtgtctgcgaacatgttgatgaaattcaccaagtcccggttgtgctggtagcgttcaaaattgcgagcatcccgtcggactttcagaatcatgtgctttaagcaggtgctactggtgaagactcggtaggcactataattggcatgtagcacagtgaagaactcggggttggtgatgaacttgaccgctggggactgcagcagcaaggtgattttttgtgagttcactggagaaagtgacccttctctccttagatctaagctggactgggaagattcggcttctgagtcactccctccacctccgcctcctcctgctggggcttgctcgcagctttggctgccagaatcttcttcggacctctctgttgcaatggttcgctgaatgttttgataccgcctgttgagttgctccatctgctggatggaccccgatctccgcatgccatccggggtggctgctgccgtcggacgctgccaggtggttgtgcggttcacgtggtccacataaaagacccgcccgtggctgtcaattcgagcttcccagtttggtggaagaggctcatcgattgttgggtagtgatgatgttcaggcctcagggaaggaagctggcttactggctgggaattatggagtataggacattcaccttctctccgattgcttggacctgccacgggggattccagaccttccgggcttctttccacgtgcccgctaggggcggccagctcgtcttgccacggcccagcgccgttcgtggactccgggtccagctcagggctctgcatggagtcgggtaccgactcgaacgcgctgttctcctcctcctcgtcgtcttgcgaggagaagaccgtgctctcggagatcttggcgctgtccacggaggagaagcgcgtgtggctggcgaacctgttgccgttgtagcaggaggggctgtagcacgaggcgctgtagcacgagctgctgtagcaggacgtgctgtagcacgaggagctgtagcacgaggggctgcagcaggacgcgtcacagccctcgcaactgtggtccccgccttgcctggggctggagtcgctctcgctcccggtgctggggtgcgtgtcgccatcctgggccgcgccattggccaggctggggaagtggcccccggagtggccagggtgcgccgtgcctggagtagccccctcgggctcttctctgtcctcttccagggcagacgggtcagcggccaccgtgtccacctcgctgagcccatccttctccgaggagtccttgagggtggactcctcctccgcgccgtcctcctcctctgccgcgctgccgccctgggcggagggcatgctgtgcagcagggtgtggatgcggatgtagtgtgtccgcggggtctcggggtccccgcaggctgacgcgatcaccgtctccagctcggacacaggcaaggagcagggcctgctttttctcttcaccgaggcccgcagctgcagcctgccctctccctgctccagggtagacacatctccctcctcctcctgctccttctcctcttcttcccttccagcccggctctgggtcgttgcttcctcctccaagggctcctccttggtgctggctggggcttcaccgtcttccagcagcagtgctgatgcctcctcacccaggtccagctgctcggccagctcttctgcactgggggcaggctggatgtccttttgcacctgggccaggagctccccagccccttcaggtcccacagagaccatgccctggtctcctgcctccgtgatgactgctgcttcctcagctggtctggaaagctctatgctttggttccctggaccatcggggacactgccctcacccagctgctctggcttccagctctcagaggactctggtgcctcagaccgaggttccccactgccgctttccatcaggttgttcatggggctgtcctgaatttgggctgactcaggctcggtactcagggaaatctcctcatcatctgctgggtggatggaggaagtgatctcaaatcggaattgcagctgtccactcacatgatctgttggaagcctgcggccaagtgtgtagctgaccaccctatcccctatggcgtgtctctccaggagtctttgaacgggcatcgacagctttcccaagaagcgcttgatgatggggcggctcttggcaaacttgtccttcacctcaatttccagcacgtcagtgggcaaggacacaaaactgaattgctcggcctgccagatggggttcacggtgttgcctatgatcttggatctcctctcctgtccatggtgagggagggcggggaagatgctgtgtttcccaggctgaatggaaatcttcagataagggtctgggttgaaaaacatccctttcttcaaccccatggcttggaaatctgagagagagaagctgatcagcctccgacttccttgtccttggacggtctcatcagcaccaatgcttttaaaaataggagctgccgagtttttgaccgtgacactgggggtggttgctcgcagggccccactcactccatggtagtatttgaagcagatcttagtttcaggttccacaaagtacgagctggcatcgatcttccagatgatctggccccgatgagaaccattgactccacggtttttatagtccagaaagttttcggacaagacctcatcaatgaggtacatgccaatccagtccccagcgtccacttcctcctttatgtcccagtggatgaccaggtcctgagagtgcccgatggaatagtaggagctgctgaccatgagcgtggagcggctgtccgaggtgaccaggtcagtgtcgctggtggagcggggaatggtgacgccatcgtgggggccgcccctgaggtccatgttgtggaactggtcggggttgtagctgtatcggagcggctccttgcaccggcgtcggctctgggagtttctagaaggagacgccatggcggccaggcctaaaaacctgttctggtacagattcttggcagccctggcctgggcacagatcatgctcctgtcagcgcgcagattagagctggggggcgcacgtgccccgcatagtgcaccgggcgcctgggactggctggggaggggaccctggcgaccgcccgctctcgctgcgctctggctgccgggtgccccgagagagcggaggccacggccactgtcacggcggaggggcgcgcgcggctcggcgagtgtgtgcgcgaggagggggccggttcggtcagagtcgcacggtgttccggctccaacaacagcgcctgatgcgcggtaacgcagcacact

SEQ ID NO: 14476 - RNA, 7116 nt, Homo sapiens
  source 1..7116: mol_type = other RNA
gctgggattacaggcatgagccaccgctcctggccggaatgctttagagtgtaggaacacaaataacacactgtccagacacaaactggtataatgagccattggcttcatatgaaattcacttcgtcttacatttctcccttgttttaatatggaaaacaattaaatgacatttaaatagtggggtctcttgagctcttctttttcccagtgaagaaaaacactttcatttatgacctatttcaggcaacatggataacaacgttagaaaaatagcaaatgaccattatggttgggtttatttcaaatgtagttgagaggttaggctgtctttggagcctgcagctgtttttctgacaacatgaagttttctgagatatgttttcactgaatgctaaaagaaactggatatttattttgatacaaatcaacgtgcctttggggtgttatgtttctgccccaggaggattactatgggtgaaggagaagtactatgttgcccttgatccctaacaagcaccatcactctctgcagcttcctagtgtggtcccgatggacaatcgaatgcaaaggaacttgaactccatgattaagaaaggaaaaggaaaaaaaaatgtgaaaaaaaaatatcaaagttttaaaaaaagggtttgtctgccaagcaaacaaaagtcatggctttaacaaaagtcatggtatcatctacacatttttttttcctttgtgaagaactgtggctagactaaacaaaacagaacagtacagaactcagggattcaaaccaaggtaatatgtccttcttccctttctccagttggcattgccacattctacataagacaatgggggctgaagcctcatccttcatgctacctcaatcaagaagctttctttcttggacatgtgcacaagtttgtccttcttgtggtgtgagtattcactagggatgctccccctcctaaacttctcttgagttgagcccacaatccccacaaccattgggatgcattgcattgcatcagcagcaggtgttttcttgctgttgttaatcgttagaagtgtcatatttgcaccgtatgtctaggctagttccggctgatgggactgatgccacatgtgaatcatgagttgaatgtataaaaatttcagctttgccactgttgtcctttggatggatattatgcacagggaaaagtagatggagaggaaaacaaagagttgatcagctcctagttctggagttggttattagaaattataaaaaatggtggctctgctcagaagacatgggcatatgaaagcctggagtgcttaatgctcacattttcccttcaatgatagaaatggaagtaaacatttattaccatttggtcaagtgtagcttaacttgcattcatatttcattgttagtaatggaggtatgtggagatatacacagaccttgagacagctgttttttaatattgcatacaggctagcagttcattgaaaacagaggagagaagcctgaaggttagatcttagaagaaggcagttcttcatgcacagcttttgtcaatcctgatttggtttgaaaataaaaatcatggaataccaaaatcaaaggagagttgattaagggaaagggaaaaggggatcatcccaggaagggtgatgtcactggccaggaaaatgtcaggcgaggttccatgtcctcactcaagtccaaaggtgctggtttcctctactgctgttaacagcttttcatacaacatggagtacgagggatacggtggaagatccagtcggttgaagcatgtgtgtgccctggggagagaagtaattttcccccatttctctatgcagaagcgccgaagcccattgctcccacggagggctgcgaagccttcgtagggcacgctggatgttcccgtgacaaactgcagtaatctcagcctctgctcattattgaagcgctccaccgcagcccagaaccagcggatcacaagatgcccatcgtggtaacctccccggtactcagtgttattccgccagtcatttaggtcgatttccgcggtgccagctatcaccagctccagctccctggcatcaaacacggacaccagcctcgagtctacaacctcgtagaagccgcgcaccagcgcctcggtctgctgtaccacgccgcgctccacccgccacttcaccatgcgctcgatgtactccttcttgtttttctccgtcacctgtgtgttggctcctccagacttcaactccctttccgtgacctgtccaaaaacctcttcattaacagtgaaagtgaggtctaagatgtctgtgatgttgttgtccttcatccactgcaaactctggtggaattcctcatccaaatattccaggtcactcaaatcacagggcagtctcaggagtgccttgtagaagggcctcgtgaagaaagcgtcaagaaggtactgatggatcagagccagacccaggatgcgaccgctaaacctgaaccactcaagatggttttctacaaatgcggacatggggctgatctgcaccgtgtaagtatcatttgccgagtactcaaagagtccatagtaagggttgaagagctcctgagacagaaggaagaagaactcccgcgaggggccactgtagtccaggccctcctctccaacaaaggtgacgtagagcttgtttcgctggagctctttccgcgaataggccatcacctgattgaaggttccctccaacaaatgatcccggcgaataatgagcttaattttccccggaccctgaccaaatcctttggcttccagttttctgtagaaattgcggagcttggcctcaaagtctcttcggtagggggaaggggctcttgcactggctctctgtaaacctggggagttctgaggtgaagaacagggtgaacatcggggagagaagctatacccagggtggaaggcagcctgcagggggacgtaggacataatctcttcttcaaagagactcagcaaaatgaccagatccgcatcacaggacaacttctcaagcccgtgattaccctcagtccgaatgtaatggattttctccctgagtgtgtggtttcttgctaagcttggctgacgctcttgcagcatttcaaaaatgtttggctggcgaagaaatgccacaatcttgtcattatatgccagtggcaatgactcatgttgatgttggcttcgaatagcagctactaagctgtgtcctggcctggccagtaaagaggctcctctgtttctagaaacttctgaggcctctccagcgctgtaacttcggagcctctggaggtgctgtcggtgagttagatgattgggaagacgaccgttctgaagagggattcgggggtcaatgaaagtggtagctcgactgttgtggtccacgaaaaaagactttccctgctggtccgttttgatctcccagccccggggcagttccagccgagtgtctgcgaacatgttgatgaaattcaccaagtcccggttgtgctggtagcgttcaaaattgcgagcatcccgtcggactttcagaatcatgtgctttaagcaggtgctactggtgaagactcggtaggcactataattggcatgtagcacagtgaagaactcggggttggtgatgaacttgaccgctggggactgcagcagcaaggtgattttttgtgagttcactggagaaagtgacccttctctccttagatctaagctggactgggaagattcggcttctgagtcactccctccacctccgcctcctcctgctggggcttgctcgcagctttggctgccagaatcttcttcggacctctctgttgcaatggttcgctgaatgttttgataccgcctgttgagttgctccatctgctggatggaccccgatctccgcatgccatccggggtggctgctgccgtcggacgctgccaggtggttgtgcggttcacgtggtccacataaaagacccgcccgtggctgtcaattcgagcttcccagtttggtggaagaggctcatcgattgttgggtagtgatgatgttcaggcctcagggaaggaagctggcttactggctgggaattatggagtataggacattcaccttctctccgattgcttggacctgccacgggggattccagaccttccgggcttctttccacgtgcccgctaggggcggccagctcgtcttgccacggcccagcgccgttcgtggactccgggtccagctcagggctctgcatggagtcgggtaccgactcgaacgcgctgttctcctcctcctcgtcgtcttgcgaggagaagaccgtgctctcggagatcttggcgctgtccacggaggagaagcgcgtgtggctggcgaacctgttgccgttgtagcaggaggggctgtagcacgaggcgctgtagcacgagctgctgtagcaggacgtgctgtagcacgaggagctgtagcacgaggggctgcagcaggacgcgtcacagccctcgcaactgtggtccccgccttgcctggggctggagtcgctctcgctcccggtgctggggtgcgtgtcgccatcctgggccgcgccattggccaggctggggaagtggcccccggagtggccagggtgcgccgtgcctggagtagccccctcgggctcttctctgtcctcttccagggcagacgggtcagcggccaccgtgtccacctcgctgagcccatccttctccgaggagtccttgagggtggactcctcctccgcgccgtcctcctcctctgccgcgctgccgccctgggcggagggcatgctgtgcagcagggtgtggatgcggatgtagtgtgtccgcggggtctcggggtccccgcaggctgacgcgatcaccgtctccagctcggacacaggcaaggagcagggcctgctttttctcttcaccgaggcccgcagctgcagcctgccctctccctgctccagggtagacacatctccctcctcctcctgctccttctcctcttcttcccttccagcccggctctgggtcgttgcttcctcctccaagggctcctccttggtgctggctggggcttcaccgtcttccagcagcagtgctgatgcctcctcacccaggtccagctgctcggccagctcttctgcactgggggcaggctggatgtccttttgcacctgggccaggagctccccagccccttcaggtcccacagagaccatgccctggtctcctgcctccgtgatgactgctgcttcctcagctggtctggaaagctctatgctttggttccctggaccatcggggacactgccctcacccagctgctctggcttccagctctcagaggactctggtgcctcagaccgaggttccccactgccgctttccatcaggttgttcatggggctgtcctgaatttgggctgactcaggctcggtactcagggaaatctcctcatcatctgctgggtggatggaggaagtgatctcaaatcggaattgcagctgtccactcacatgatctgttggaagcctgcggccaagtgtgtagctgaccaccctatcccctatggcgtgtctctccaggagtctttgaacgggcatcgacagctttcccaagaagcgcttgatgatggggcggctcttggcaaacttgtccttcacctcaatttccagcacgtcagtgggcaaggacacaaaactgaattgctcggcctgccagatggggttcacggtgttgcctatgatcttggatctcctctcctgtccatggtgagggagggcggggaagatgctgtgtttcccaggctgaatggaaatcttcagataagggtctgggttgaaaaacatccctttcttcaaccccatggcttggaaatctgagagagagaagctgatcagcctccgacttccttgtccttggacggtctcatcagcaccaatgcttttaaaaataggagctgccgagtttttgaccgtgacactgggggtggttgctcgcagggccccactcactccatggtagtatttgaagcagatcttagtttcaggttccacaaagtacgagctggcatcgatcttccagatgatctggccccgatgagaaccattgactccacggtttttatagtccagaaagttttcggacaagacctcatcaatgaggtacatgccaatccagtccccagcgtccacttcctcctttatgtcccagtggatgaccaggtcctgagagtgcccgatggaatagtaggagctgctgaccatgagcgtggagcggctgtccgaggtgaccaggtcagtgtcgctggtggagcggggaatggtgacgccatcgtgggggccgcccctgaggtccatgttgtggaactggtcggggttgtagctgtatcggagcggctccttgcaccggcgtcggctctgggagtttctagaaggagacgccatggcggccaggcctaaaaacctgttctggtacagattcttggtttgttttggtagagtttttgccagcccctgagatggtctcaattatccttaccacctgatgttcacagcattatgaagtgcccttccacactgaaccagagcttgtcagtgtgaccagtagaattcagcaggagtaacaatgtgtgacttctcaggctaagtcataaaggcactgcagcttctacctcagtctcctggctcccttgtttgtggagaggcagctgccatgctttgaggatgcacatgcagtcctgtggagagcccgagttgctagctgatacctccatctgacagtttccctagtttgccagccacactagtgagacacattggaagtgggtcctcctgccctagtcaacccatcagatgacagcagccccagctgacatctgacttacaaccttctaagagatccgaagtctaaacctgccagccaagctgctgctgaatgactgaccggcagaaaccacgagagactattaaatgattgctgttttgagtcactaaattttagggctgatttgttatggtttattattaagcaacagataacacacagaatttcaaaagaatgtaagtgaaaaaaatccaacaattattgagcacttactatattct

SEQ ID NO: 14477 - RNA, 6835 nt, Homo sapiens
  source 1..6835: mol_type = other RNA
gctgggattacaggcatgagccaccgctcctggccggaatgctttagagtgtaggaacacaaataacacactgtccagacacaaactggtataatgagccattggcttcatatgaaattcacttcgtcttacatttctcccttgttttaatatggaaaacaattaaatgacatttaaatagtggggtctcttgagctcttctttttcccagtgaagaaaaacactttcatttatgacctatttcaggcaacatggataacaacgttagaaaaatagcaaatgaccattatggttgggtttatttcaaatgtagttgagaggttaggctgtctttggagcctgcagctgtttttctgacaacatgaagttttctgagatatgttttcactgaatgctaaaagaaactggatatttattttgatacaaatcaacgtgcctttggggtgttatgtttctgccccaggaggattactatgggtgaaggagaagtactatgttgcccttgatccctaacaagcaccatcactctctgcagcttcctagtgtggtcccgatggacaatcgaatgcaaaggaacttgaactccatgattaagaaaggaaaaggaaaaaaaaatgtgaaaaaaaaatatcaaagttttaaaaaaagggtttgtctgccaagcaaacaaaagtcatggctttaacaaaagtcatggtatcatctacacatttttttttcctttgtgaagaactgtggctagactaaacaaaacagaacagtacagaactcagggattcaaaccaaggtaatatgtccttcttccctttctccagttggcattgccacattctacataagacaatgggggctgaagcctcatccttcatgctacctcaatcaagaagctttctttcttggacatgtgcacaagtttgtccttcttgtggtgtgagtattcactagggatgctccccctcctaaacttctcttgagttgagcccacaatccccacaaccattgggatgcattgcattgcatcagcagcaggtgttttcttgctgttgttaatcgttagaagtgtcatatttgcaccgtatgtctaggctagttccggctgatgggactgatgccacatgtgaatcatgagttgaatgtataaaaatttcagctttgccactgttgtcctttggatggatattatgcacagggaaaagtagatggagaggaaaacaaagagttgatcagctcctagttctggagttggttattagaaattataaaaaatggtggctctgctcagaagacatgggcatatgaaagcctggagtgcttaatgctcacattttcccttcaatgatagaaatggaagtaaacatttattaccatttggtcaagtgtagcttaacttgcattcatatttcattgttagtaatggaggtatgtggagatatacacagaccttgagacagctgttttttaatattgcatacaggctagcagttcattgaaaacagaggagagaagcctgaaggttagatcttagaagaaggcagttcttcatgcacagcttttgtcaatcctgatttggtttgaaaataaaaatcatggaataccaaaatcaaaggagagttgattaagggaaagggaaaaggggatcatcccaggaagggtgatgtcactggccaggaaaatgtcaggcgaggttccatgtcctcactcaagtccaaaggtgctggtttcctctactgctgttaacagcttttcatacaacatggagtacgagggatacggtggaagatccagtcggttgaagcatgtgtgtgccctggggagagaagtaattttcccccatttctctatgcagaagcgccgaagcccattgctcccacggagggctgcgaagccttcgtagggcacgctggatgttcccgtgacaaactgcagtaatctcagcctctgctcattattgaagcgctccaccgcagcccagaaccagcggatcacaagatgcccatcgtggtaacctccccggtactcagtgttattccgccagtcatttaggtcgatttccgcggtgccagctatcaccagctccagctccctggcatcaaacacggacaccagcctcgagtctacaacctcgtagaagccgcgcaccagcgcctcggtctgctgtaccacgccgcgctccacccgccacttcaccatgcgctcgatgtactccttcttgtttttctccgtcacctgtgtgttggctcctccagacttcaactccctttccgtgacctgtccaaaaacctcttcattaacagtgaaagtgaggtctaagatgtctgtgatgttgttgtccttcatccactgcaaactctggtggaattcctcatccaaatattccaggtcactcaaatcacagggcagtctcaggagtgccttgtagaagggcctcgtgaagaaagcgtcaagaaggtactgatggatcagagccagacccaggatgcgaccgctaaacctgaaccactcaagatggttttctacaaatgcggacatggggctgatctgcaccgtgtaagtatcatttgccgagtactcaaagagtccatagtaagggttgaagagctcctgagacagaaggaagaagaactcccgcgaggggccactgtagtccaggccctcctctccaacaaaggtgacgtagagcttgtttcgctggagctctttccgcgaataggccatcacctgattgaaggttccctccaacaaatgatcccggcgaataatgagcttaattttccccggaccctgaccaaatcctttggcttccagttttctgtagaaattgcggagcttggcctcaaagtctcttcggtagggggaaggggctcttgcactggctctctgtaaacctggggagttctgaggtgaagaacagggtgaacatcggggagagaagctatacccagggtggaaggcagcctgcagggggacgtaggacataatctcttcttcaaagagactcagcaaaatgaccagatccgcatcacaggacaacttctcaagcccgtgattaccctcagtccgaatgtaatggattttctccctgagtgtgtggtttcttgctaagcttggctgacgctcttgcagcatttcaaaaatgtttggctggcgaagaaatgccacaatcttgtcattatatgccagtggcaatgactcatgttgatgttggcttcgaatagcagctactaagctgtgtcctggcctggccagtaaagaggctcctctgtttctagaaacttctgaggcctctccagcgctgtaacttcggagcctctggaggtgctgtcggtgagttagatgattgggaagacgaccgttctgaagagggattcgggggtcaatgaaagtggtagctcgactgttgtggtccacgaaaaaagactttccctgctggtccgttttgatctcccagccccggggcagttccagccgagtgtctgcgaacatgttgatgaaattcaccaagtcccggttgtgctggtagcgttcaaaattgcgagcatcccgtcggactttcagaatcatgtgctttaagcaggtgctactggtgaagactcggtaggcactataattggcatgtagcacagtgaagaactcggggttggtgatgaacttgaccgctggggactgcagcagcaaggtgattttttgtgagttcactggagaaagtgacccttctctccttagatctaagctggactgggaagattcggcttctgagtcactccctccacctccgcctcctcctgctggggcttgctcgcagctttggctgccagaatcttcttcggacctctctgttgcaatggttcgctgaatgttttgataccgcctgttgagttgctccatctgctggatggaccccgatctccgcatgccatccggggtggctgctgccgtcggacgctgccaggtggttgtgcggttcacgtggtccacataaaagacccgcccgtggctgtcaattcgagcttcccagtttggtggaagaggctcatcgattgttgggtagtgatgatgttcaggcctcagggaaggaagctggcttactggctgggaattatggagtataggacattcaccttctctccgattgcttggacctgccacgggggattccagaccttccgggcttctttccacgtgcccgctaggggcggccagctcgtcttgccacggcccagcgccgttcgtggactccgggtccagctcagggctctgcatggagtcgggtaccgactcgaacgcgctgttctcctcctcctcgtcgtcttgcgaggagaagaccgtgctctcggagatcttggcgctgtccacggaggagaagcgcgtgtggctggcgaacctgttgccgttgtagcaggaggggctgtagcacgaggcgctgtagcacgagctgctgtagcaggacgtgctgtagcacgaggagctgtagcacgaggggctgcagcaggacgcgtcacagccctcgcaactgtggtccccgccttgcctggggctggagtcgctctcgctcccggtgctggggtgcgtgtcgccatcctgggccgcgccattggccaggctggggaagtggcccccggagtggccagggtgcgccgtgcctggagtagccccctcgggctcttctctgtcctcttccagggcagacgggtcagcggccaccgtgtccacctcgctgagcccatccttctccgaggagtccttgagggtggactcctcctccgcgccgtcctcctcctctgccgcgctgccgccctgggcggagggcatgctgtgcagcagggtgtggatgcggatgtagtgtgtccgcggggtctcggggtccccgcaggctgacgcgatcaccgtctccagctcggacacaggcaaggagcagggcctgctttttctcttcaccgaggcccgcagctgcagcctgccctctccctgctccagggtagacacatctccctcctcctcctgctccttctcctcttcttcccttccagcccggctctgggtcgttgcttcctcctccaagggctcctccttggtgctggctggggcttcaccgtcttccagcagcagtgctgatgcctcctcacccaggtccagctgctcggccagctcttctgcactgggggcaggctggatgtccttttgcacctgggccaggagctccccagccccttcaggtcccacagagaccatgccctggtctcctgcctccgtgatgactgctgcttcctcagctggtctggaaagctctatgctttggttccctggaccatcggggacactgccctcacccagctgctctggcttccagctctcagaggactctggtgcctcagaccgaggttccccactgccgctttccatcaggttgttcatggggctgtcctgaatttgggctgactcaggctcggtactcagggaaatctcctcatcatctgctgggtggatggaggaagtgatctcaaatcggaattgcagctgtccactcacatgatctgttggaagcctgcggccaagtgtgtagctgaccaccctatcccctatggcgtgtctctccaggagtctttgaacgggcatcgacagctttcccaagaagcgcttgatgatggggcggctcttggcaaacttgtccttcacctcaatttccagcacgtcagtgggcaaggacacaaaactgaattgctcggcctgccagatggggttcacggtgttgcctatgatcttggatctcctctcctgtccatggtgagggagggcggggaagatgctgtgtttcccaggctgaatggaaatcttcagataagggtctgggttgaaaaacatccctttcttcaaccccatggcttggaaatctgagagagagaagctgatcagcctccgacttccttgtccttggacggtctcatcagcaccaatgcttttaaaaataggagctgccgagtttttgaccgtgacactgggggtggttgctcgcagggccccactcactccatggtagtatttgaagcagatcttagtttcaggttccacaaagtacgagctggcatcgatcttccagatgatctggccccgatgagaaccattgactccacggtttttatagtccagaaagttttcggacaagacctcatcaatgaggtacatgccaatccagtccccagcgtccacttcctcctttatgtcccagtggatgaccaggtcctgagagtgcccgatggaatagtaggagctgctgaccatgagcgtggagcggctgtccgaggtgaccaggtcagtgtcgctggtggagcggggaatggtgacgccatcgtgggggccgcccctgaggtccatgttgtggaactggtcggggttgtagctgtatcggagcggctccttgcaccggcgtcggctctgggagtttctagaaggagacgccatggcggccaggcctaaaaacctgttctggtacagatttttgaaagaacaggacagactacgtattcaaaacaagagcgccttcttaaagtgcaggctcagaagttgttcaatggccaggaccttcatttgtgctggcagctctggtcctgctgggcatggttaagggcgaggctcgcagcccgcacggcgtggtccttcaggggtgctgcgtcaggctgacgctccggaacagttactgggacaggctgtgagcgactcaccaggacagttttatttctgtgctgagcttgctgcttcctgctgggaaaatgttagtggcggagtcacacccaggtaccgggccgcagccaaggctccgcagatgacccgagttctgatg

SEQ ID NO: 14478 - RNA, 6378 nt, Homo sapiens
  source 1..6378: mol_type = other RNA
gctgggattacaggcatgagccaccgctcctggccggaatgctttagagtgtaggaacacaaataacacactgtccagacacaaactggtataatgagccattggcttcatatgaaattcacttcgtcttacatttctcccttgttttaatatggaaaacaattaaatgacatttaaatagtggggtctcttgagctcttctttttcccagtgaagaaaaacactttcatttatgacctatttcaggcaacatggataacaacgttagaaaaatagcaaatgaccattatggttgggtttatttcaaatgtagttgagaggttaggctgtctttggagcctgcagctgtttttctgacaacatgaagttttctgagatatgttttcactgaatgctaaaagaaactggatatttattttgatacaaatcaacgtgcctttggggtgttatgtttctgccccaggaggattactatgggtgaaggagaagtactatgttgcccttgatccctaacaagcaccatcactctctgcagcttcctagtgtggtcccgatggacaatcgaatgcaaaggaacttgaactccatgattaagaaaggaaaaggaaaaaaaaatgtgaaaaaaaaatatcaaagttttaaaaaaagggtttgtctgccaagcaaacaaaagtcatggctttaacaaaagtcatggtatcatctacacatttttttttcctttgtgaagaactgtggctagactaaacaaaacagaacagtacagaactcagggattcaaaccaaggtaatatgtccttcttccctttctccagttggcattgccacattctacataagacaatgggggctgaagcctcatccttcatgctacctcaatcaagaagctttctttcttggacatgtgcacaagtttgtccttcttgtggtgtgagtattcactagggatgctccccctcctaaacttctcttgagttgagcccacaatccccacaaccattgggatgcattgcattgcatcagcagcaggtgttttcttgctgttgttaatcgttagaagtgtcatatttgcaccgtatgtctaggctagttccggctgatgggactgatgccacatgtgaatcatgagttgaatgtataaaaatttcagctttgccactgttgtcctttggatggatattatgcacagggaaaagtagatggagaggaaaacaaagagttgatcagctcctagttctggagttggttattagaaattataaaaaatggtggctctgctcagaagacatgggcatatgaaagcctggagtgcttaatgctcacattttcccttcaatgatagaaatggaagtaaacatttattaccatttggtcaagtgtagcttaacttgcattcatatttcattgttagtaatggaggtatgtggagatatacacagaccttgagacagctgttttttaatattgcatacaggctagcagttcattgaaaacagaggagagaagcctgaaggttagatcttagaagaaggcagttcttcatgcacagcttttgtcaatcctgatttggtttgaaaataaaaatcatggaataccaaaatcaaaggagagttgattaagggaaagggaaaaggggatcatcccaggaagggtgatgtcactggccaggaaaatgtcaggcgaggttccatgtcctcactcaagtccaaaggtgctggtttcctctactgctgttaacagcttttcatacaacatggagtacgagggatacggtggaagatccagtcggttgaagcatgtgtgtgccctggggagagaagtaattttcccccatttctctatgcagaagcgccgaagcccattgctcccacggagggctgcgaagccttcgtagggcacgctggatgttcccgtgacaaactgcagtaatctcagcctctgctcattattgaagcgctccaccgcagcccagaaccagcggatcacaagatgcccatcgtggtaacctccccggtactcagtgttattccgccagtcatttaggtcgatttccgcggtgccagctatcaccagctccagctccctggcatcaaacacggacaccagcctcgagtctacaacctcgtagaagccgcgcaccagcgcctcggtctgctgtaccacgccgcgctccacccgccacttcaccatgcgctcgatgtactccttcttgtttttctccgtcacctgtgtgttggctcctccagacttcaactccctttccgtgacctgtccaaaaacctcttcattaacagtgaaagtgaggtctaagatgtctgtgatgttgttgtccttcatccactgcaaactctggtggaattcctcatccaaatattccaggtcactcaaatcacagggcagtctcaggagtgccttgtagaagggcctcgtgaagaaagcgtcaagaaggtactgatggatcagagccagacccaggatgcgaccgctaaacctgaaccactcaagatggttttctacaaatgcggacatggggctgatctgcaccgtgtaagtatcatttgccgagtactcaaagagtccatagtaagggttgaagagctcctgagacagaaggaagaagaactcccgcgaggggccactgtagtccaggccctcctctccaacaaaggtgacgtagagcttgtttcgctggagctctttccgcgaataggccatcacctgattgaaggttccctccaacaaatgatcccggcgaataatgagcttaattttccccggaccctgaccaaatcctttggcttccagttttctgtagaaattgcggagcttggcctcaaagtctcttcggtagggggaaggggctcttgcactggctctctgtaaacctggggagttctgaggtgaagaacagggtgaacatcggggagagaagctatacccagggtggaaggcagcctgcagggggacgtaggacataatctcttcttcaaagagactcagcaaaatgaccagatccgcatcacaggacaacttctcaagcccgtgattaccctcagtccgaatgtaatggattttctccctgagtgtgtggtttcttgctaagcttggctgacgctcttgcagcatttcaaaaatgtttggctggcgaagaaatgccacaatcttgtcattatatgccagtggcaatgactcatgttgatgttggcttcgaatagcagctactaagctgtgtcctggcctggccagtaaagaggctcctctgtttctagaaacttctgaggcctctccagcgctgtaacttcggagcctctggaggtgctgtcggtgagttagatgattgggaagacgaccgttctgaagagggattcgggggtcaatgaaagtggtagctcgactgttgtggtccacgaaaaaagactttccctgctggtccgttttgatctcccagccccggggcagttccagccgagtgtctgcgaacatgttgatgaaattcaccaagtcccggttgtgctggtagcgttcaaaattgcgagcatcccgtcggactttcagaatcatgtgctttaagcaggtgctactggtgaagactcggtaggcactataattggcatgtagcacagtgaagaactcggggttggtgatgaacttgaccgctggggactgcagcagcaaggtgattttttgtgagttcactggagaaagtgacccttctctccttagatctaagctggactgggaagattcggcttctgagtcactccctccacctccgcctcctcctgctggggcttgctcgcagctttggctgccagaatcttcttcggacctctctgttgcaatggttcgctgaatgttttgataccgcctgttgagttgctccatctgctggatggaccccgatctccgcatgccatccggggtggctgctgccgtcggacgctgccaggtggttgtgcggttcacgtggtccacataaaagacccgcccgtggctgtcaattcgagcttcccagtttggtggaagaggctcatcgattgttgggtagtgatgatgttcaggcctcagggaaggaagctggcttactggctgggaattatggagtataggacattcaccttctctccgattgcttggacctgccacgggggattccagaccttccgggcttctttccacgtgcccgctaggggcggccagctcgtcttgccacggcccagcgccgttcgtggactccgggtccagctcagggctctgcatggagtcgggtaccgactcgaacgcgctgttctcctcctcctcgtcgtcttgcgaggagaagaccgtgctctcggagatcttggcgctgtccacggaggagaagcgcgtgtggctggcgaacctgttgccgttgtagcaggaggggctgtagcacgaggcgctgtagcacgagctgctgtagcaggacgtgctgtagcacgaggagctgtagcacgaggggctgcagcaggacgcgtcacagccctcgcaactgtggtccccgccttgcctggggctggagtcgctctcgctcccggtgctggggtgcgtgtcgccatcctgggccgcgccattggccaggctggggaagtggcccccggagtggccagggtgcgccgtgcctggagtagccccctcgggctcttctctgtcctcttccagggcagacgggtcagcggccaccgtgtccacctcgctgagcccatccttctccgaggagtccttgagggtggactcctcctccgcgccgtcctcctcctctgccgcgctgccgccctgggcggagggcatgctgtgcagcagggtgtggatgcggatgtagtgtgtccgcggggtctcggggtccccgcaggctgacgcgatcaccgtctccagctcggacacaggcaaggagcagggcctgctttttctcttcaccgaggcccgcagctgcagcctgccctctccctgctccagggtagacacatctccctcctcctcctgctccttctcctcttcttcccttccagcccggctctgggtcgttgcttcctcctccaagggctcctccttggtgctggctggggcttcaccgtcttccagcagcagtgctgatgcctcctcacccaggtccagctgctcggccagctcttctgcactgggggcaggctggatgtccttttgcacctgggccaggagctccccagccccttcaggtcccacagagaccatgccctggtctcctgcctccgtgatgactgctgcttcctcagctggtctggaaagctctatgctttggttccctggaccatcggggacactgccctcacccagctgctctggcttccagctctcagaggactctggtgcctcagaccgaggttccccactgccgctttccatcaggttgttcatggggctgtcctgaatttgggctgactcaggctcggtactcagggaaatctcctcatcatctgctgggtggatggaggaagtgatctcaaatcggaattgcagctgtccactcacatgatctgttggaagcctgcggccaagtgtgtagctgaccaccctatcccctatggcgtgtctctccaggagtctttgaacgggcatcgacagctttcccaagaagcgcttgatgatggggcggctcttggcaaacttgtccttcacctcaatttccagcacgtcagtgggcaaggacacaaaactgaattgctcggcctgccagatggggttcacggtgttgcctatgatcttggatctcctctcctgtccatggtgagggagggcggggaagatgctgtgtttcccaggctgaatggaaatcttcagataagggtctgggttgaaaaacatccctttcttcaaccccatggcttggaaatctgagagagagaagctgatcagcctccgacttccttgtccttggacggtctcatcagcaccaatgcttttaaaaatctccttggaaatgcagtcatctttgtgttctgccagagcagccatttctcataaaagagagttgcagtgaagaatgcaggcagggaaattatccatagctctgggggaggcataagaaagtccccaggatcagacttccctttgatccaagggctgcttgataattccgacttcccattggcagagagcacacagataagggcctttacaccctggcaacatgcctggggacttcattaacttaagggcttctgccatctttgctgtaagtaacataggaaaaactcacaaagagaaaaaaaatgttatttctgtgcattcatatgcaaggatttgattctaattttttggactctttcaggaaacagcccaccggagaaaacccctgatctaaaagcaccagtcctgtcttaa

SEQ ID NO: 14479 - RNA, 7140 nt, Homo sapiens
  source 1..7140: mol_type = other RNA
gctgggattacaggcatgagccaccgctcctggccggaatgctttagagtgtaggaacacaaataacacactgtccagacacaaactggtataatgagccattggcttcatatgaaattcacttcgtcttacatttctcccttgttttaatatggaaaacaattaaatgacatttaaatagtggggtctcttgagctcttctttttcccagtgaagaaaaacactttcatttatgacctatttcaggcaacatggataacaacgttagaaaaatagcaaatgaccattatggttgggtttatttcaaatgtagttgagaggttaggctgtctttggagcctgcagctgtttttctgacaacatgaagttttctgagatatgttttcactgaatgctaaaagaaactggatatttattttgatacaaatcaacgtgcctttggggtgttatgtttctgccccaggaggattactatgggtgaaggagaagtactatgttgcccttgatccctaacaagcaccatcactctctgcagcttcctagtgtggtcccgatggacaatcgaatgcaaaggaacttgaactccatgattaagaaaggaaaaggaaaaaaaaatgtgaaaaaaaaatatcaaagttttaaaaaaagggtttgtctgccaagcaaacaaaagtcatggctttaacaaaagtcatggtatcatctacacatttttttttcctttgtgaagaactgtggctagactaaacaaaacagaacagtacagaactcagggattcaaaccaaggtaatatgtccttcttccctttctccagttggcattgccacattctacataagacaatgggggctgaagcctcatccttcatgctacctcaatcaagaagctttctttcttggacatgtgcacaagtttgtccttcttgtggtgtgagtattcactagggatgctccccctcctaaacttctcttgagttgagcccacaatccccacaaccattgggatgcattgcattgcatcagcagcaggtgttttcttgctgttgttaatcgttagaagtgtcatatttgcaccgtatgtctaggctagttccggctgatgggactgatgccacatgtgaatcatgagttgaatgtataaaaatttcagctttgccactgttgtcctttggatggatattatgcacagggaaaagtagatggagaggaaaacaaagagttgatcagctcctagttctggagttggttattagaaattataaaaaatggtggctctgctcagaagacatgggcatatgaaagcctggagtgcttaatgctcacattttcccttcaatgatagaaatggaagtaaacatttattaccatttggtcaagtgtagcttaacttgcattcatatttcattgttagtaatggaggtatgtggagatatacacagaccttgagacagctgttttttaatattgcatacaggctagcagttcattgaaaacagaggagagaagcctgaaggttagatcttagaagaaggcagttcttcatgcacagcttttgtcaatcctgatttggtttgaaaataaaaatcatggaataccaaaatcaaaggagagttgattaagggaaagggaaaaggggatcatcccaggaagggtgatgtcactggccaggaaaatgtcaggcgaggttccatgtcctcactcaagtccaaaggtgctggtttcctctactgctgttaacagcttttcatacaacatggagtacgagggatacggtggaagatccagtcggttgaagcatgtgtgtgccctggggagagaagtaattttcccccatttctctatgcagaagcgccgaagcccattgctcccacggagggctgcgaagccttcgtagggcacgctggatgttcccgtgacaaactgcagtaatctcagcctctgctcattattgaagcgctccaccgcagcccagaaccagcggatcacaagatgcccatcgtggtaacctccccggtactcagtgttattccgccagtcatttaggtcgatttccgcggtgccagctatcaccagctccagctccctggcatcaaacacggacaccagcctcgagtctacaacctcgtagaagccgcgcaccagcgcctcggtctgctgtaccacgccgcgctccacccgccacttcaccatgcgctcgatgtactccttcttgtttttctccgtcacctgtgtgttggctcctccagacttcaactccctttccgtgacctgtccaaaaacctcttcattaacagtgaaagtgaggtctaagatgtctgtgatgttgttgtccttcatccactgcaaactctggtggaattcctcatccaaatattccaggtcactcaaatcacagggcagtctcaggagtgccttgtagaagggcctcgtgaagaaagcgtcaagaaggtactgatggatcagagccagacccaggatgcgaccgctaaacctgaaccactcaagatggttttctacaaatgcggacatggggctgatctgcaccgtgtaagtatcatttgccgagtactcaaagagtccatagtaagggttgaagagctcctgagacagaaggaagaagaactcccgcgaggggccactgtagtccaggccctcctctccaacaaaggtgacgtagagcttgtttcgctggagctctttccgcgaataggccatcacctgattgaaggttccctccaacaaatgatcccggcgaataatgagcttaattttccccggaccctgaccaaatcctttggcttccagttttctgtagaaattgcggagcttggcctcaaagtctcttcggtagggggaaggggctcttgcactggctctctgtaaacctggggagttctgaggtgaagaacagggtgaacatcggggagagaagctatacccagggtggaaggcagcctgcagggggacgtaggacataatctcttcttcaaagagactcagcaaaatgaccagatccgcatcacaggacaacttctcaagcccgtgattaccctcagtccgaatgtaatggattttctccctgagtgtgtggtttcttgctaagcttggctgacgctcttgcagcatttcaaaaatgtttggctggcgaagaaatgccacaatcttgtcattatatgccagtggcaatgactcatgttgatgttggcttcgaatagcagctactaagctgtgtcctggcctggccagtaaagaggctcctctgtttctagaaacttctgaggcctctccagcgctgtaacttcggagcctctggaggtgctgtcggtgagttagatgattgggaagacgaccgttctgaagagggattcgggggtcaatgaaagtggtagctcgactgttgtggtccacgaaaaaagactttccctgctggtccgttttgatctcccagccccggggcagttccagccgagtgtctgcgaacatgttgatgaaattcaccaagtcccggttgtgctggtagcgttcaaaattgcgagcatcccgtcggactttcagaatcatgtgctttaagcaggtgctactggtgaagactcggtaggcactataattggcatgtagcacagtgaagaactcggggttggtgatgaacttgaccgctggggactgcagcagcaaggtgattttttgtgagttcactggagaaagtgacccttctctccttagatctaagctggactgggaagattcggcttctgagtcactccctccacctccgcctcctcctgctggggcttgctcgcagctttggctgccagaatcttcttcggacctctctgttgcaatggttcgctgaatgttttgataccgcctgttgagttgctccatctgctggatggaccccgatctccgcatgccatccggggtggctgctgccgtcggacgctgccaggtggttgtgcggttcacgtggtccacataaaagacccgcccgtggctgtcaattcgagcttcccagtttggtggaagaggctcatcgattgttgggtagtgatgatgttcaggcctcagggaaggaagctggcttactggctgggaattatggagtataggacattcaccttctctccgattgcttggacctgccacgggggattccagaccttccgggcttctttccacgtgcccgctaggggcggccagctcgtcttgccacggcccagcgccgttcgtggactccgggtccagctcagggctctgcatggagtcgggtaccgactcgaacgcgctgttctcctcctcctcgtcgtcttgcgaggagaagaccgtgctctcggagatcttggcgctgtccacggaggagaagcgcgtgtggctggcgaacctgttgccgttgtagcaggaggggctgtagcacgaggcgctgtagcacgagctgctgtagcaggacgtgctgtagcacgaggagctgtagcacgaggggctgcagcaggacgcgtcacagccctcgcaactgtggtccccgccttgcctggggctggagtcgctctcgctcccggtgctggggtgcgtgtcgccatcctgggccgcgccattggccaggctggggaagtggcccccggagtggccagggtgcgccgtgcctggagtagccccctcgggctcttctctgtcctcttccagggcagacgggtcagcggccaccgtgtccacctcgctgagcccatccttctccgaggagtccttgagggtggactcctcctccgcgccgtcctcctcctctgccgcgctgccgccctgggcggagggcatgctgtgcagcagggtgtggatgcggatgtagtgtgtccgcggggtctcggggtccccgcaggctgacgcgatcaccgtctccagctcggacacaggcaaggagcagggcctgctttttctcttcaccgaggcccgcagctgcagcctgccctctccctgctccagggtagacacatctccctcctcctcctgctccttctcctcttcttcccttccagcccggctctgggtcgttgcttcctcctccaagggctcctccttggtgctggctggggcttcaccgtcttccagcagcagtgctgatgcctcctcacccaggtccagctgctcggccagctcttctgcactgggggcaggctggatgtccttttgcacctgggccaggagctccccagccccttcaggtcccacagagaccatgccctggtctcctgcctccgtgatgactgctgcttcctcagctggtctggaaagctctatgctttggttccctggaccatcggggacactgccctcacccagctgctctggcttccagctctcagaggactctggtgcctcagaccgaggttccccactgccgctttccatcaggttgttcatggggctgtcctgaatttgggctgactcaggctcggtactcagggaaatctcctcatcatctgggtggatggaggaagtgatctcaaatcggaattgcagctgtccactcacatgatctgttggaagcctgcggccaagtgtgtagctgaccaccctatcccctatggcgtgtctctccaggagtctttgaacgggcatcgacagctttcccaagaagcgcttgatgatggggcggctcttggcaaacttgtccttcacctcaatttccagcacgtcagtgggcaaggacacaaaactgaattgctcggcctgccagatggggttcacggtgttgcctatgatcttggatctcctctcctgtccatggtgagggagggcggggaagatgctgtgtttcccaggctgaatggaaatcttcagataagggtctgggttgaaaaacatccctttcttcaaccccatggcttggaaatctgagagagagaagctgatcagcctccgacttccttgtccttggacggtctcatcagcaccaatgcttttaaaaataggagctgccgagtttttgaccgtgacactgggggtggttgctcgcagggccccactcactccatggtagtatttgaagcagatcttagtttcaggttccacaaagtacgagctggcatcgatcttccagatgatctggccccgatgagaaccattgactccacggtttttatagtccagaaagttttcggacaagacctcatcaatgaggtacatgccaatccagtccccagcgtccacttcctcctttatgtcccagtggatgaccaggtcctgagagtgcccgatggaatagtaggagctgctgaccatgagcgtggagcggctgtccgaggtgaccaggtcagtgtcgctggtggagcggggaatggtgacgccatcgtgggggccgcccctgaggtccatgttgtggaactggtcggggttgtagctgtatcggagcggctccttgcaccggcgtcggctctgggagtttctagaaggagacgccatggcggccaggcctaaaaacctgttctggtacagattcgtaatagccacagccggagtgagtctgctgatgagaaacgcagatctggccacctgctttgagacgccttggaccacaacactgccggggtctttaacggttggccttttcgggtagggcatctgccctcctaaatcgcgtttaaatcccaggaaaagagagaagatgcctccctcaatttttgaactatgctgctcttgctgtatccgtttctgctgaacatagcattgatatcttttcaaagagaaggggggaaaacaaggggagaattgcaccactgcagattccaagagaagtaagcacaaaactacagcaacgtcaaataatatcttcttcggcaactaggaaaatccccacatgctctctggtgtcagcccaatgcagactgaggcgcgctgtgcccggaaccacaggaagccgggcatctctgcagcctgtgtccctgccagctccccctacgcgctgaaattcggcagggaagaagttatggtgcccagcctctgtgtgcaagacagagacaccgcgcatcatggctctgaaaatcagccaagtggccgggacgtcaaagcggcagagcaatcagaatgccctggagccggggatggaggggccacattgtttgagccctcggattttgctgcattgtcacc

SEQ ID NO: 14480 - RNA, 7073 nt, Homo sapiens
  source 1..7073: mol_type = other RNA
gctgggattacaggcatgagccaccgctcctggccggaatgctttagagtgtaggaacacaaataacacactgtccagacacaaactggtataatgagccattggcttcatatgaaattcacttcgtcttacatttctcccttgttttaatatggaaaacaattaaatgacatttaaatagtggggtctcttgagctcttctttttcccagtgaagaaaaacactttcatttatgacctatttcaggcaacatggataacaacgttagaaaaatagcaaatgaccattatggttgggtttatttcaaatgtagttgagaggttaggctgtctttggagcctgcagctgtttttctgacaacatgaagttttctgagatatgttttcactgaatgctaaaagaaactggatatttattttgatacaaatcaacgtgcctttggggtgttatgtttctgccccaggaggattactatgggtgaaggagaagtactatgttgcccttgatccctaacaagcaccatcactctctgcagcttcctagtgtggtcccgatggacaatcgaatgcaaaggaacttgaactccatgattaagaaaggaaaaggaaaaaaaaatgtgaaaaaaaaatatcaaagttttaaaaaaagggtttgtctgccaagcaaacaaaagtcatggctttaacaaaagtcatggtatcatctacacatttttttttcctttgtgaagaactgtggctagactaaacaaaacagaacagtacagaactcagggattcaaaccaaggtaatatgtccttcttccctttctccagttggcattgccacattctacataagacaatgggggctgaagcctcatccttcatgctacctcaatcaagaagctttctttcttggacatgtgcacaagtttgtccttcttgtggtgtgagtattcactagggatgctccccctcctaaacttctcttgagttgagcccacaatccccacaaccattgggatgcattgcattgcatcagcagcaggtgttttcttgctgttgttaatcgttagaagtgtcatatttgcaccgtatgtctaggctagttccggctgatgggactgatgccacatgtgaatcatgagttgaatgtataaaaatttcagctttgccactgttgtcctttggatggatattatgcacagggaaaagtagatggagaggaaaacaaagagttgatcagctcctagttctggagttggttattagaaattataaaaaatggtggctctgctcagaagacatgggcatatgaaagcctggagtgcttaatgctcacattttcccttcaatgatagaaatggaagtaaacatttattaccatttggtcaagtgtagcttaacttgcattcatatttcattgttagtaatggaggtatgtggagatatacacagaccttgagacagctgttttttaatattgcatacaggctagcagttcattgaaaacagaggagagaagcctgaaggttagatcttagaagaaggcagttcttcatgcacagcttttgtcaatcctgatttggtttgaaaataaaaatcatggaataccaaaatcaaaggagagttgattaagggaaagggaaaaggggatcatcccaggaagggtgatgtcactggccaggaaaatgtcaggcgaggttccatgtcctcactcaagtccaaaggtgctggtttcctctactgctgttaacagcttttcatacaacatggagtacgagggatacggtggaagatccagtcggttgaagcatgtgtgtgccctggggagagaagtaattttcccccatttctctatgcagaagcgccgaagcccattgctcccacggagggctgcgaagccttcgtagggcacgctggatgttcccgtgacaaactgcagtaatctcagcctctgctcattattgaagcgctccaccgcagcccagaaccagcggatcacaagatgcccatcgtggtaacctccccggtactcagtgttattccgccagtcatttaggtcgatttccgcggtgccagctatcaccagctccagctccctggcatcaaacacggacaccagcctcgagtctacaacctcgtagaagccgcgcaccagcgcctcggtctgctgtaccacgccgcgctccacccgccacttcaccatgcgctcgatgtactccttcttgtttttctccgtcacctgtgtgttggctcctccagacttcaactccctttccgtgacctgtccaaaaacctcttcattaacagtgaaagtgaggtctaagatgtctgtgatgttgttgtccttcatccactgcaaactctggtggaattcctcatccaaatattccaggtcactcaaatcacagggcagtctcaggagtgccttgtagaagggcctcgtgaagaaagcgtcaagaaggtactgatggatcagagccagacccaggatgcgaccgctaaacctgaaccactcaagatggttttctacaaatgcggacatggggctgatctgcaccgtgtaagtatcatttgccgagtactcaaagagtccatagtaagggttgaagagctcctgagacagaaggaagaagaactcccgcgaggggccactgtagtccaggccctcctctccaacaaaggtgacgtagagcttgtttcgctggagctctttccgcgaataggccatcacctgattgaaggttccctccaacaaatgatcccggcgaataatgagcttaattttccccggaccctgaccaaatcctttggcttccagttttctgtagaaattgcggagcttggcctcaaagtctcttcggtagggggaaggggctcttgcactggctctctgtaaacctggggagttctgaggtgaagaacagggtgaacatcggggagagaagctatacccagggtggaaggcagcctgcagggggacgtaggacataatctcttcttcaaagagactcagcaaaatgaccagatccgcatcacaggacaacttctcaagcccgtgattaccctcagtccgaatgtaatggattttctccctgagtgtgtggtttcttgctaagcttggctgacgctcttgcagcatttcaaaaatgtttggctggcgaagaaatgccacaatcttgtcattatatgccagtggcaatgactcatgttgatgttggcttcgaatagcagctactaagctgtgtcctggcctggccagtaaagaggctcctctgtttctagaaacttctgaggcctctccagcgctgtaacttcggagcctctggaggtgctgtcggtgagttagatgattgggaagacgaccgttctgaagagggattcgggggtcaatgaaagtggtagctcgactgttgtggtccacgaaaaaagactttccctgctggtccgttttgatctcccagccccggggcagttccagccgagtgtctgcgaacatgttgatgaaattcaccaagtcccggttgtgctggtagcgttcaaaattgcgagcatcccgtcggactttcagaatcatgtgctttaagcaggtgctactggtgaagactcggtaggcactataattggcatgtagcacagtgaagaactcggggttggtgatgaacttgaccgctggggactgcagcagcaaggtgattttttgtgagttcactggagaaagtgacccttctctccttagatctaagctggactgggaagattcggcttctgagtcactccctccacctccgcctcctcctgctggggcttgctcgcagctttggctgccagaatcttcttcggacctctctgttgcaatggttcgctgaatgttttgataccgcctgttgagttgctccatctgctggatggaccccgatctccgcatgccatccggggtggctgctgccgtcggacgctgccaggtggttgtgcggttcacgtggtccacataaaagacccgcccgtggctgtcaattcgagcttcccagtttggtggaagaggctcatcgattgttgggtagtgatgatgttcaggcctcagggaaggaagctggcttactggctgggaattatggagtataggacattcaccttctctccgattgcttggacctgccacgggggattccagaccttccgggcttctttccacgtgcccgctaggggcggccagctcgtcttgccacggcccagcgccgttcgtggactccgggtccagctcagggctctgcatggagtcgggtaccgactcgaacgcgctgttctcctcctcctcgtcgtcttgcgaggagaagaccgtgctctcggagatcttggcgctgtccacggaggagaagcgcgtgtggctggcgaacctgttgccgttgtagcaggaggggctgtagcacgaggcgctgtagcacgagctgctgtagcaggacgtgctgtagcacgaggagctgtagcacgaggggctgcagcaggacgcgtcacagccctcgcaactgtggtccccgccttgcctggggctggagtcgctctcgctcccggtgctggggtgcgtgtcgccatcctgggccgcgccattggccaggctggggaagtggcccccggagtggccagggtgcgccgtgcctggagtagccccctcgggctcttctctgtcctcttccagggcagacgggtcagcggccaccgtgtccacctcgctgagcccatccttctccgaggagtccttgagggtggactcctcctccgcgccgtcctcctcctctgccgcgctgccgccctgggcggagggcatgctgtgcagcagggtgtggatgcggatgtagtgtgtccgcggggtctcggggtccccgcaggctgacgcgatcaccgtctccagctcggacacaggcaaggagcagggcctgctttttctcttcaccgaggcccgcagctgcagcctgccctctccctgctccagggtagacacatctccctcctcctcctgctccttctcctcttcttcccttccagcccggctctgggtcgttgcttcctcctccaagggctcctccttggtgctggctggggcttcaccgtcttccagcagcagtgctgatgcctcctcacccaggtccagctgctcggccagctcttctgcactgggggcaggctggatgtccttttgcacctgggccaggagctccccagccccttcaggtcccacagagaccatgccctggtctcctgcctccgtgatgactgctgcttcctcagctggtctggaaagctctatgctttggttccctggaccatcggggacactgccctcacccagctgctctggcttccagctctcagaggactctggtgcctcagaccgaggttccccactgccgctttccatcaggttgttcatggggctgtcctgaatttgggctgactcaggctcggtactcagggaaatctcctcatcatctgggtggatggaggaagtgatctcaaatcggaattgcagctgtccactcacatgatctgttggaagcctgcggccaagtgtgtagctgaccaccctatcccctatggcgtgtctctccaggagtctttgaacgggcatcgacagctttcccaagaagcgcttgatgatggggcggctcttggcaaacttgtccttcacctcaatttccagcacgtcagtgggcaaggacacaaaactgaattgctcggcctgccagatggggttcacggtgttgcctatgatcttggatctcctctcctgtccatggtgagggagggcggggaagatgctgtgtttcccaggctgaatggaaatcttcagataagggtctgggttgaaaaacatccctttcttcaaccccatggcttggaaatctgagagagagaagctgatcagcctccgacttccttgtccttggacggtctcatcagcaccaatgcttttaaaaataggagctgccgagtttttgaccgtgacactgggggtggttgctcgcagggccccactcactccatggtagtatttgaagcagatcttagtttcaggttccacaaagtacgagctggcatcgatcttccagatgatctggccccgatgagaaccattgactccacggtttttatagtccagaaagttttcggacaagacctcatcaatgaggtacatgccaatccagtccccagcgtccacttcctcctttatgtcccagtggatgaccaggtcctgagagtgcccgatggaatagtaggagctgctgaccatgagcgtggagcggctgtccgaggtgaccaggtcagtgtcgctggtggagcggggaatggtgacgccatcgtgggggccgcccctgaggtccatgttgtggaactggtcggggttgtagctgtatcggagcggctccttgcaccggcgtcggctctgggagtttctagaaggagacgccatggcggccaggcctaaaaacctgttctggtacagattcttcacactacacaggtgcagcagcataatgacccaccacgtgtacgcgcatcaattccgtaatagccacagccggagtgagtctgctgatgagaaacgcagatctggccacctgctttgagacgccttggaccacaacactgccggggtctttaacggttggccttttcgggtagggcatctgccctcctaaatcgcgtttaaatcccaggaaaagagagaagatgcctccctcaatttttgaactatgctgctcttgctgtatccgtttctgctgaacatagcattgatatcttggcagccctggcctgggcacagatcatgctcctgtcagcgcgcagattagagctggggggcgcacgtgccccgcatagtgcaccgggcgcctgggactggctggggaggggaccctggcgaccgcccgctctcgctgcgctctggctgccgggtgccccgagagagcggaggccacggccactgtcacggcggaggggcgcgcgcggctcggcgagtgtgtgcgcgaggagggggccggttcggtcagagtcgcacggtgttccggctccaacaacagcgcctgatgc

SEQ ID NO: 14481 - RNA, 6905 nt, Homo sapiens
  source 1..6905: mol_type = other RNA
gctgggattacaggcatgagccaccgctcctggccggaatgctttagagtgtaggaacacaaataacacactgtccagacacaaactggtataatgagccattggcttcatatgaaattcacttcgtcttacatttctcccttgttttaatatggaaaacaattaaatgacatttaaatagtggggtctcttgagctcttctttttcccagtgaagaaaaacactttcatttatgacctatttcaggcaacatggataacaacgttagaaaaatagcaaatgaccattatggttgggtttatttcaaatgtagttgagaggttaggctgtctttggagcctgcagctgtttttctgacaacatgaagttttctgagatatgttttcactgaatgctaaaagaaactggatatttattttgatacaaatcaacgtgcctttggggtgttatgtttctgccccaggaggattactatgggtgaaggagaagtactatgttgcccttgatccctaacaagcaccatcactctctgcagcttcctagtgtggtcccgatggacaatcgaatgcaaaggaacttgaactccatgattaagaaaggaaaaggaaaaaaaaatgtgaaaaaaaaatatcaaagttttaaaaaaagggtttgtctgccaagcaaacaaaagtcatggctttaacaaaagtcatggtatcatctacacatttttttttcctttgtgaagaactgtggctagactaaacaaaacagaacagtacagaactcagggattcaaaccaaggtaatatgtccttcttccctttctccagttggcattgccacattctacataagacaatgggggctgaagcctcatccttcatgctacctcaatcaagaagctttctttcttggacatgtgcacaagtttgtccttcttgtggtgtgagtattcactagggatgctccccctcctaaacttctcttgagttgagcccacaatccccacaaccattgggatgcattgcattgcatcagcagcaggtgttttcttgctgttgttaatcgttagaagtgtcatatttgcaccgtatgtctaggctagttccggctgatgggactgatgccacatgtgaatcatgagttgaatgtataaaaatttcagctttgccactgttgtcctttggatggatattatgcacagggaaaagtagatggagaggaaaacaaagagttgatcagctcctagttctggagttggttattagaaattataaaaaatggtggctctgctcagaagacatgggcatatgaaagcctggagtgcttaatgctcacattttcccttcaatgatagaaatggaagtaaacatttattaccatttggtcaagtgtagcttaacttgcattcatatttcattgttagtaatggaggtatgtggagatatacacagaccttgagacagctgttttttaatattgcatacaggctagcagttcattgaaaacagaggagagaagcctgaaggttagatcttagaagaaggcagttcttcatgcacagcttttgtcaatcctgatttggtttgaaaataaaaatcatggaataccaaaatcaaaggagagttgattaagggaaagggaaaaggggatcatcccaggaagggtgatgtcactggccaggaaaatgtcaggcgaggttccatgtcctcactcaagtccaaaggtgctggtttcctctactgctgttaacagcttttcatacaacatggagtacgagggatacggtggaagatccagtcggttgaagcatgtgtgtgccctggggagagaagtaattttcccccatttctctatgcagaagcgccgaagcccattgctcccacggagggctgcgaagccttcgtagggcacgctggatgttcccgtgacaaactgcagtaatctcagcctctgctcattattgaagcgctccaccgcagcccagaaccagcggatcacaagatgcccatcgtggtaacctccccggtactcagtgttattccgccagtcatttaggtcgatttccgcggtgccagctatcaccagctccagctccctggcatcaaacacggacaccagcctcgagtctacaacctcgtagaagccgcgcaccagcgcctcggtctgctgtaccacgccgcgctccacccgccacttcaccatgcgctcgatgtactccttcttgtttttctccgtcacctgtgtgttggctcctccagacttcaactccctttccgtgacctgtccaaaaacctcttcattaacagtgaaagtgaggtctaagatgtctgtgatgttgttgtccttcatccactgcaaactctggtggaattcctcatccaaatattccaggtcactcaaatcacagggcagtctcaggagtgccttgtagaagggcctcgtgaagaaagcgtcaagaaggtactgatggatcagagccagacccaggatgcgaccgctaaacctgaaccactcaagatggttttctacaaatgcggacatggggctgatctgcaccgtgtaagtatcatttgccgagtactcaaagagtccatagtaagggttgaagagctcctgagacagaaggaagaagaactcccgcgaggggccactgtagtccaggccctcctctccaacaaaggtgacgtagagcttgtttcgctggagctctttccgcgaataggccatcacctgattgaaggttccctccaacaaatgatcccggcgaataatgagcttaattttccccggaccctgaccaaatcctttggcttccagttttctgtagaaattgcggagcttggcctcaaagtctcttcggtagggggaaggggctcttgcactggctctctgtaaacctggggagttctgaggtgaagaacagggtgaacatcggggagagaagctatacccagggtggaaggcagcctgcagggggacgtaggacataatctcttcttcaaagagactcagcaaaatgaccagatccgcatcacaggacaacttctcaagcccgtgattaccctcagtccgaatgtaatggattttctccctgagtgtgtggtttcttgctaagcttggctgacgctcttgcagcatttcaaaaatgtttggctggcgaagaaatgccacaatcttgtcattatatgccagtggcaatgactcatgttgatgttggcttcgaatagcagctactaagctgtgtcctggcctggccagtaaagaggctcctctgtttctagaaacttctgaggcctctccagcgctgtaacttcggagcctctggaggtgctgtcggtgagttagatgattgggaagacgaccgttctgaagagggattcgggggtcaatgaaagtggtagctcgactgttgtggtccacgaaaaaagactttccctgctggtccgttttgatctcccagccccggggcagttccagccgagtgtctgcgaacatgttgatgaaattcaccaagtcccggttgtgctggtagcgttcaaaattgcgagcatcccgtcggactttcagaatcatgtgctttaagcaggtgctactggtgaagactcggtaggcactataattggcatgtagcacagtgaagaactcggggttggtgatgaacttgaccgctggggactgcagcagcaaggtgattttttgtgagttcactggagaaagtgacccttctctccttagatctaagctggactgggaagattcggcttctgagtcactccctccacctccgcctcctcctgctggggcttgctcgcagctttggctgccagaatcttcttcggacctctctgttgcaatggttcgctgaatgttttgataccgcctgttgagttgctccatctgctggatggaccccgatctccgcatgccatccggggtggctgctgccgtcggacgctgccaggtggttgtgcggttcacgtggtccacataaaagacccgcccgtggctgtcaattcgagcttcccagtttggtggaagaggctcatcgattgttgggtagtgatgatgttcaggcctcagggaaggaagctggcttactggctgggaattatggagtataggacattcaccttctctccgattgcttggacctgccacgggggattccagaccttccgggcttctttccacgtgcccgctaggggcggccagctcgtcttgccacggcccagcgccgttcgtggactccgggtccagctcagggctctgcatggagtcgggtaccgactcgaacgcgctgttctcctcctcctcgtcgtcttgcgaggagaagaccgtgctctcggagatcttggcgctgtccacggaggagaagcgcgtgtggctggcgaacctgttgccgttgtagcaggaggggctgtagcacgaggcgctgtagcacgagctgctgtagcaggacgtgctgtagcacgaggagctgtagcacgaggggctgcagcaggacgcgtcacagccctcgcaactgtggtccccgccttgcctggggctggagtcgctctcgctcccggtgctggggtgcgtgtcgccatcctgggccgcgccattggccaggctggggaagtggcccccggagtggccagggtgcgccgtgcctggagtagccccctcgggctcttctctgtcctcttccagggcagacgggtcagcggccaccgtgtccacctcgctgagcccatccttctccgaggagtccttgagggtggactcctcctccgcgccgtcctcctcctctgccgcgctgccgccctgggcggagggcatgctgtgcagcagggtgtggatgcggatgtagtgtgtccgcggggtctcggggtccccgcaggctgacgcgatcaccgtctccagctcggacacaggcaaggagcagggcctgctttttctcttcaccgaggcccgcagctgcagcctgccctctccctgctccagggtagacacatctccctcctcctcctgctccttctcctcttcttcccttccagcccggctctgggtcgttgcttcctcctccaagggctcctccttggtgctggctggggcttcaccgtcttccagcagcagtgctgatgcctcctcacccaggtccagctgctcggccagctcttctgcactgggggcaggctggatgtccttttgcacctgggccaggagctccccagccccttcaggtcccacagagaccatgccctggtctcctgcctccgtgatgactgctgcttcctcagctggtctggaaagctctatgctttggttccctggaccatcggggacactgccctcacccagctgctctggcttccagctctcagaggactctggtgcctcagaccgaggttccccactgccgctttccatcaggttgttcatggggctgtcctgaatttgggctgactcaggctcggtactcagggaaatctcctcatcatctgggtggatggaggaagtgatctcaaatcggaattgcagctgtccactcacatgatctgttggaagcctgcggccaagtgtgtagctgaccaccctatcccctatggcgtgtctctccaggagtctttgaacgggcatcgacagctttcccaagaagcgcttgatgatggggcggctcttggcaaacttgtccttcacctcaatttccagcacgtcagtgggcaaggacacaaaactgaattgctcggcctgccagatggggttcacggtgttgcctatgatcttggatctcctctcctgtccatggtgagggagggcggggaagatgctgtgtttcccaggctgaatggaaatcttcagataagggtctgggttgaaaaacatccctttcttcaaccccatggcttggaaatctgagagagagaagctgatcagcctccgacttccttgtccttggacggtctcatcagcaccaatgcttttaaaaataggagctgccgagtttttgaccgtgacactgggggtggttgctcgcagggccccactcactccatggtagtatttgaagcagatcttagtttcaggttccacaaagtacgagctggcatcgatcttccagatgatctggccccgatgagaaccattgactccacggtttttatagtccagaaagttttcggacaagacctcatcaatgaggtacatgccaatccagtccccagcgtccacttcctcctttatgtcccagtggatgaccaggtcctgagagtgcccgatggaatagtaggagctgctgaccatgagcgtggagcggctgtccgaggtgaccaggtcagtgtcgctggtggagcggggaatggtgacgccatcgtgggggccgcccctgaggtccatgttgtggaactggtcggggttgtagctgtatcggagcggctccttgcaccggcgtcggctctgggagtttctagaaggagacgccatggcggccaggcctaaaaacctgttctggtacagattcttcacactacacaggtgcagcagcataatgacccaccacgtgtacgcgcatcaattccttggcagccctggcctgggcacagatcatgctcctgtcagcgcgcagattagagctggggggcgcacgtgccccgcatagtgcaccgggcgcctgggactggctggggaggggaccctggcgaccgcccgctctcgctgcgctctggctgccgggtgccccgagagagcggaggccacggccactgtcacggcggaggggcgcgcgcggctcggcgagtgtgtgcgcgaggagggggccggttcggtcagagtcgcacggtgttccggctccaacaacagcgcctgatgcgcggtaacgcagcacacttcatcgctttatcctcccgcttgcatcccctccctccctgcctgctcct

SEQ ID NO: 14482 - RNA, 6798 nt, Homo sapiens
  source 1..6798: mol_type = other RNA
gctgggattacaggcatgagccaccgctcctggccggaatgctttagagtgtaggaacacaaataacacactgtccagacacaaactggtataatgagccattggcttcatatgaaattcacttcgtcttacatttctcccttgttttaatatggaaaacaattaaatgacatttaaatagtggggtctcttgagctcttctttttcccagtgaagaaaaacactttcatttatgacctatttcaggcaacatggataacaacgttagaaaaatagcaaatgaccattatggttgggtttatttcaaatgtagttgagaggttaggctgtctttggagcctgcagctgtttttctgacaacatgaagttttctgagatatgttttcactgaatgctaaaagaaactggatatttattttgatacaaatcaacgtgcctttggggtgttatgtttctgccccaggaggattactatgggtgaaggagaagtactatgttgcccttgatccctaacaagcaccatcactctctgcagcttcctagtgtggtcccgatggacaatcgaatgcaaaggaacttgaactccatgattaagaaaggaaaaggaaaaaaaaatgtgaaaaaaaaatatcaaagttttaaaaaaagggtttgtctgccaagcaaacaaaagtcatggctttaacaaaagtcatggtatcatctacacatttttttttcctttgtgaagaactgtggctagactaaacaaaacagaacagtacagaactcagggattcaaaccaaggtaatatgtccttcttccctttctccagttggcattgccacattctacataagacaatgggggctgaagcctcatccttcatgctacctcaatcaagaagctttctttcttggacatgtgcacaagtttgtccttcttgtggtgtgagtattcactagggatgctccccctcctaaacttctcttgagttgagcccacaatccccacaaccattgggatgcattgcattgcatcagcagcaggtgttttcttgctgttgttaatcgttagaagtgtcatatttgcaccgtatgtctaggctagttccggctgatgggactgatgccacatgtgaatcatgagttgaatgtataaaaatttcagctttgccactgttgtcctttggatggatattatgcacagggaaaagtagatggagaggaaaacaaagagttgatcagctcctagttctggagttggttattagaaattataaaaaatggtggctctgctcagaagacatgggcatatgaaagcctggagtgcttaatgctcacattttcccttcaatgatagaaatggaagtaaacatttattaccatttggtcaagtgtagcttaacttgcattcatatttcattgttagtaatggaggtatgtggagatatacacagaccttgagacagctgttttttaatattgcatacaggctagcagttcattgaaaacagaggagagaagcctgaaggttagatcttagaagaaggcagttcttcatgcacagcttttgtcaatcctgatttggtttgaaaataaaaatcatggaataccaaaatcaaaggagagttgattaagggaaagggaaaaggggatcatcccaggaagggtgatgtcactggccaggaaaatgtcaggcgaggttccatgtcctcactcaagtccaaaggtgctggtttcctctactgctgttaacagcttttcatacaacatggagtacgagggatacggtggaagatccagtcggttgaagcatgtgtgtgccctggggagagaagtaattttcccccatttctctatgcagaagcgccgaagcccattgctcccacggagggctgcgaagccttcgtagggcacgctggatgttcccgtgacaaactgcagtaatctcagcctctgctcattattgaagcgctccaccgcagcccagaaccagcggatcacaagatgcccatcgtggtaacctccccggtactcagtgttattccgccagtcatttaggtcgatttccgcggtgccagctatcaccagctccagctccctggcatcaaacacggacaccagcctcgagtctacaacctcgtagaagccgcgcaccagcgcctcggtctgctgtaccacgccgcgctccacccgccacttcaccatgcgctcgatgtactccttcttgtttttctccgtcacctgtgtgttggctcctccagacttcaactccctttccgtgacctgtccaaaaacctcttcattaacagtgaaagtgaggtctaagatgtctgtgatgttgttgtccttcatccactgcaaactctggtggaattcctcatccaaatattccaggtcactcaaatcacagggcagtctcaggagtgccttgtagaagggcctcgtgaagaaagcgtcaagaaggtactgatggatcagagccagacccaggatgcgaccgctaaacctgaaccactcaagatggttttctacaaatgcggacatggggctgatctgcaccgtgtaagtatcatttgccgagtactcaaagagtccatagtaagggttgaagagctcctgagacagaaggaagaagaactcccgcgaggggccactgtagtccaggccctcctctccaacaaaggtgacgtagagcttgtttcgctggagctctttccgcgaataggccatcacctgattgaaggttccctccaacaaatgatcccggcgaataatgagcttaattttccccggaccctgaccaaatcctttggcttccagttttctgtagaaattgcggagcttggcctcaaagtctcttcggtagggggaaggggctcttgcactggctctctgtaaacctggggagttctgaggtgaagaacagggtgaacatcggggagagaagctatacccagggtggaaggcagcctgcagggggacgtaggacataatctcttcttcaaagagactcagcaaaatgaccagatccgcatcacaggacaacttctcaagcccgtgattaccctcagtccgaatgtaatggattttctccctgagtgtgtggtttcttgctaagcttggctgacgctcttgcagcatttcaaaaatgtttggctggcgaagaaatgccacaatcttgtcattatatgccagtggcaatgactcatgttgatgttggcttcgaatagcagctactaagctgtgtcctggcctggccagtaaagaggctcctctgtttctagaaacttctgaggcctctccagcgctgtaacttcggagcctctggaggtgctgtcggtgagttagatgattgggaagacgaccgttctgaagagggattcgggggtcaatgaaagtggtagctcgactgttgtggtccacgaaaaaagactttccctgctggtccgttttgatctcccagccccggggcagttccagccgagtgtctgcgaacatgttgatgaaattcaccaagtcccggttgtgctggtagcgttcaaaattgcgagcatcccgtcggactttcagaatcatgtgctttaagcaggtgctactggtgaagactcggtaggcactataattggcatgtagcacagtgaagaactcggggttggtgatgaacttgaccgctggggactgcagcagcaaggtgattttttgtgagttcactggagaaagtgacccttctctccttagatctaagctggactgggaagattcggcttctgagtcactccctccacctccgcctcctcctgctggggcttgctcgcagctttggctgccagaatcttcttcggacctctctgttgcaatggttcgctgaatgttttgataccgcctgttgagttgctccatctgctggatggaccccgatctccgcatgccatccggggtggctgctgccgtcggacgctgccaggtggttgtgcggttcacgtggtccacataaaagacccgcccgtggctgtcaattcgagcttcccagtttggtggaagaggctcatcgattgttgggtagtgatgatgttcaggcctcagggaaggaagctggcttactggctgggaattatggagtataggacattcaccttctctccgattgcttggacctgccacgggggattccagaccttccgggcttctttccacgtgcccgctaggggcggccagctcgtcttgccacggcccagcgccgttcgtggactccgggtccagctcagggctctgcatggagtcgggtaccgactcgaacgcgctgttctcctcctcctcgtcgtcttgcgaggagaagaccgtgctctcggagatcttggcgctgtccacggaggagaagcgcgtgtggctggcgaacctgttgccgttgtagcaggaggggctgtagcacgaggcgctgtagcacgagctgctgtagcaggacgtgctgtagcacgaggagctgtagcacgaggggctgcagcaggacgcgtcacagccctcgcaactgtggtccccgccttgcctggggctggagtcgctctcgctcccggtgctggggtgcgtgtcgccatcctgggccgcgccattggccaggctggggaagtggcccccggagtggccagggtgcgccgtgcctggagtagccccctcgggctcttctctgtcctcttccagggcagacgggtcagcggccaccgtgtccacctcgctgagcccatccttctccgaggagtccttgagggtggactcctcctccgcgccgtcctcctcctctgccgcgctgccgccctgggcggagggcatgctgtgcagcagggtgtggatgcggatgtagtgtgtccgcggggtctcggggtccccgcaggctgacgcgatcaccgtctccagctcggacacaggcaaggagcagggcctgctttttctcttcaccgaggcccgcagctgcagcctgccctctccctgctccagggtagacacatctccctcctcctcctgctccttctcctcttcttcccttccagcccggctctgggtcgttgcttcctcctccaagggctcctccttggtgctggctggggcttcaccgtcttccagcagcagtgctgatgcctcctcacccaggtccagctgctcggccagctcttctgcactgggggcaggctggatgtccttttgcacctgggccaggagctccccagccccttcaggtcccacagagaccatgccctggtctcctgcctccgtgatgactgctgcttcctcagctggtctggaaagctctatgctttggttccctggaccatcggggacactgccctcacccagctgctctggcttccagctctcagaggactctggtgcctcagaccgaggttccccactgccgctttccatcaggttgttcatggggctgtcctgaatttgggctgactcaggctcggtactcagggaaatctcctcatcatctgggtggatggaggaagtgatctcaaatcggaattgcagctgtccactcacatgatctgttggaagcctgcggccaagtgtgtagctgaccaccctatcccctatggcgtgtctctccaggagtctttgaacgggcatcgacagctttcccaagaagcgcttgatgatggggcggctcttggcaaacttgtccttcacctcaatttccagcacgtcagtgggcaaggacacaaaactgaattgctcggcctgccagatggggttcacggtgttgcctatgatcttggatctcctctcctgtccatggtgagggagggcggggaagatgctgtgtttcccaggctgaatggaaatcttcagataagggtctgggttgaaaaacatccctttcttcaaccccatggcttggaaatctgagagagagaagctgatcagcctccgacttccttgtccttggacggtctcatcagcaccaatgcttttaaaaataggagctgccgagtttttgaccgtgacactgggggtggttgctcgcagggccccactcactccatggtagtatttgaagcagatcttagtttcaggttccacaaagtacgagctggcatcgatcttccagatgatctggccccgatgagaaccattgactccacggtttttatagtccagaaagttttcggacaagacctcatcaatgaggtacatgccaatccagtccccagcgtccacttcctcctttatgtcccagtggatgaccaggtcctgagagtgcccgatggaatagtaggagctgctgaccatgagcgtggagcggctgtccgaggtgaccaggtcagtgtcgctggtggagcggggaatggtgacgccatcgtgggggccgcccctgaggtccatgttgtggaactggtcggggttgtagctgtatcggagcggctccttgcaccggcgtcggctctgggagtttctagaaggagacgccatggcggccaggcctaaaaacctgttctggtacagattcttggcagccctggcctgggcacagatcatgctcctgtcagcgcgcagattagagctggggggcgcacgtgccccgcatagtgcaccgggcgcctgggactggctggggaggggaccctggcgaccgcccgctctcgctgcgctctggctgccgggtgccccgagagagcggaggccacggccactgtcacggcggaggggcgcgcgcggctcggcgagtgtgtgcgcgaggagggggccggttcggtcagagtcgcacggtgttccggctccaacaacagcgcctgatgcgcggtaacgcagcacact

SEQ ID NO: 14483 - RNA, 1719 nt, Homo sapiens
  source 1..1719: mol_type = other RNA
gctgggattacaggcatgagccaccgctctcggctgtgttctgccttttataatattccccttcataaagaatctcactactttgccttcacctgggaaaataaacaatacacctggactgttatgccccaacgatttactaaggccctacatatttctcatgaacctatatgatggacttaaaattcccagaagactccactgtaatccaatatgtaaatgacctctttctatgcactttcatttatgacaactccctttaggacactgaatactttaaggcaatggcaagaaaagaccacaaagtttctagacgaaaagtttaattattctgtgtgttcaatatctgggtcatggtatttcagctgcaggtaaaattatcttcacaggcggagcttctactattcatcattttcctcttccttgtctggatccatctttcctttgataaattcttgcttccagaactgcaatgcctgttccaaagttaaaccaatgcccttcagaaataggccatactgcattcggcctccatgacgaagatggtgattttcccgcaaggctttatgtaactgacgcatgcaaggtgggaaggatttggtagaaagcaaatcaatctgatctaaagaaatcttcccaacatttccctgggtactgtaatcttggccagtgtaggaatgactgaggtgattgagcagaggctgaagtctttcatcagactgcacagcaggcaaggacctggctgttaatactgaagctgactttgccacctcttctctatgtgagtaaagactgttccatccacagcctgtgtgagtcgtgtatctcttcaggaatccaacaattgcaaccatgtggtgggctgacatcctgggactgctgctcctgacagtaggtgttgttatgctccttgctgtcctccacacagtgggactcctccctgccaaagccttggacagtttggctctaaattcattcaggatgattgccacaatgtccttaagtggtacgtaagcaaagccatcttccaaatagactttccttcctcgaaacaaatccagagcatcagcaaaagggatcttataaatggactcgaaccccaacttaagtccacttaaacttggtgatgaggcaacaatctcctgttctcgaagagtcttctcttcatcacttatagcctcaaactgcaattggctatcctttaagaaatcctgaattttatccttgggtaaaatactaaatctaaatcgaaggagatccatttcttgttgaatgaaccagcgtctaagttcttcagactggcaataagcaagccgcaaaataaaatgagaaatatgatctcttcttcgtggttcatattcatcttctaagttttctctgtaggaaaacttgagcttccgaagctcactctccaacttactctggtattgttcagttcctttcacatagctcactccaagattttcaactgattttaacaatttaactctatcaatagccaagttttcaaattctattaaagatatgttttcagaaggtggctgcaagtaaaactgaaggcaatgagggtaggaagcattcctctggtcacctgccaacctcagcttcctccactttcttccagaaaactccatcttggtcacctgcaagaattcaaactcgggaaaacacaaacggtggcagccactgttcccgggtggcgggagagttcatatgaaa

SEQ ID NO: 14484 - RNA, 9652 nt, Homo sapiens
  source 1..9652: mol_type = other RNA
gctgggattacaggcatgagccaccgctcttggccgtcacttttttttttttaatgctgccaagttgaagtggacattgtcactttaaaaaaaattattttaaccattctgattggagtatagtgatgtcttgttggggttttatttgcgtctccgtcatggctaatgatgttgcatattttttgtgtgcttatctgccatctgtacatcaccttcagggaaaaacgtcttcagtgaaaaatgtcactttattttgtccattttctaattggattgttttttaatgatgagttttgagagttctttatatattctaaatacgagccgtttgtcagatatgttttgcaaatattttctccctctctgtaacttgtctcttcatcctcttaatagggtccttcccagagcaaaaatttaatgatgataaagtccaatttagcatctcagtgttaacatccattgattatttcagtttgtttgtgatatgacaaacaatttttaattgaaaccaggacattttcatgttagctcatgagagagtcatatttaaacctcctgctttaactcgtgtttcatggtaccactctggcaggggaaaagggcaggggacagcctcattattgccaggtggaagtggaagtccaggttgcccactcaacctcctccgacgccgcaggggtgcttgctgtcaccgctgggtggaggtgggagttccggatccccatgtggtcccctctgacatgcagtggggctggcctcatcatccctgggagtctatgaagtctgactcactatttctgacaccaccccagcaggaaggagagggacacctcgatactgcccagtgggggtgcaagtcaggttcctgctgtctccagtgacaccatggggcgtgggtaggagccttctcaccagttggcggggacgaaagtcacagctccccactggccttctctgacactactctggtagggggttggagcccctctgatagcccagcaggggtgggatctgagctcccacttggtcttggctgggatggatgggggtggggatgtgttctgtggtgtttggctggggtacagcagtgacagtcgaaaagttttttgttttgctagatcttttcctatcattttccttcttctctatcctatctttttctcttttcttagtccgtttcctgtagagagcagctttttattgggatttttttttttttttgcctgtgtccattagcatttcctagtgccaagtatgggacacatgaggcaaaaagaaaacaagctcctcgctgtgtcgttcctcaggttctgggcaccctagcaggtctgccttcttccctccacctctccgagtcttcttacgttcattttatacagaatgtcttgggtttttagttgtatttagcaggagaaatatagataagaacatctattgcattttccagaagcagaagtttaggtctatattttcaacaagacattttgatggccttacatctagttcacctcctcattttatagagcagaaactgaggctgcagtgagataatgtatcttatccacgatccaatagtaagtttggatccaatagtaagttggaagcacagcccaggctgaaagcacatctcctaaacccaggtgcaatgctgcttccgcgacatcatggcggctcccactttgcctgtatgtctcacctctcctgctacaatgcaaggccctgtgcggacaccagcctactcctccccatactcacatgctgccatctcctccagaatagcttatttccctaagcagattccagcttccctgagtgcagagaccaggccatgtggctcagaatgtatacagcaagcacccaatgcatggctgctgatggttctccctataggagctagttgtcagcattgtttagtaagtgtggcatcctgttcctccaagtgagctggagccagaaggcactttgaggatgaggacagatggcattttctgaaagacagacatacacgctggtgagcacagaggttgtgccatgtttgtttctgggaggaatgttaaggggaatcacagcgcacacttctagtgctcctgggcatgtgacccaggcccgaaggaccactgtgtcatgtcccagacatcttctcactgcagcttcagcatctgttctctccactctaccctccatgcaaacagccaccatggctatgttcctcaccatcccagtgcccagtgcccaacctggagtacagcagccctcagtgatgactggctgattggagccgatcaataggtgaaagaacaaataaataaacaaaggaatgacccaaccacagcaaaggcaattcctcatgcaggaaagaggatatttagcttaaaaagacttgccgtgctcggctgctgaggaaagtaagtaggcaaaagacacaagcaaaagagttaaataaaaaccgtcagctggagcaatgagaagggggcttgcggctgaatcaaagaaagaacttttttattaatggagctgcctaacaatatgctgagatgccttctgaagcagtgagctccctgctgctggaaatgctccctgctactggaaatcaacctttgctaacatggtggggacttggatcaggtgacctctgagcttcctgccatctgagagcccatgatgtttcagaattcactggaggccttaaactccagtgcatgggagtttgttggggctcagaaaacaatatcccaaaatgaaggcctcagcagcagcctcagaagcaaaagtctttctctgactttctgccctcctgcctgtcagtctcactctcccctgaagctagccatagaagttagactccctcttccccaccacgagaaaccacagcctctttctcccaaagccagccatgaaacctaaagatagagctctaattctccctctgcctttctttttaaaaactggccataaataaattatctgatctgctttgtttgattataggtcatgacacccccattccagagagggtcctgccccaactcagaaggaaggaatgctgcacagacaggccagggagagtctagacagacaggccttgctgtgtttccccattttgtctattagcattagatcatgcccttttggtccaatcccatttctacaactgtccatactttgttgaacttaaccataaaaatagataattttccctgtatctttgggtcttcattctgcagcctcccatgtatacatgttaaataaatgtgtatgccttttctcttattaatctgccttttacaagttgatttttcagcaaatcttcagagagctaagcgttaccctaggcccccacaagtttaatccttgagttccatcaaggatttgaggtggtgaagaagaagagggaaagaaaagttcagccccagcctccgggaagctgctactagagatagggcatgtgacagtcattccagccagtcaccaaataattctggttcccctcattccaggcacagagtagcgttgtacttcttaatgtgcttatggttggatgaggccacatgacccgttctgggtaacaagctcagagcggaagtgacaagtgttgtatctaggctggagcactgaactgccaatgcatgatcctccagagctcctttttctctgtcatggcaactggttaaaacggaactgccccaccaagctgtgccctggttgtttaatgttactaagatttggattgtttggttgttggttgtttaatgttaatgttactgagatttgggcttgtttgttactgcagcattatctaggctatcctgactgatacaggggaacagactttgcctgtatggaacaccagagaaagatacaagaaaaaagttcaaggcacacaacaggggctgggttggacagaggttccaacatctgagcccacacacagacccctctgcattcaccattctcagccccccacttgagtaacacccaatatgatcctcctctagctgtgctgcctcctaactattactctaacatcccaacactgtgccctactcaacctttgctaacatcatgtcttctctcttcatcttcttctctcttcccttccatctagtcaaacatcctacccattcccaaaggcataggtcaggcctcatgtcctgcaagacacctccctacccacagagaccaactgaaccactctttggaatcaccacagttcttgtggccaggatgacatctctttggggatcttacgtgtatgttgtcatcttgttctgtgtaaactagtttttaccctacaaactggcagtgatccagaagctcccactcagacgcatctgctgggctcacagcagggactcaataaatacgaactaaacagagagcagcactatgaacatatacctggtatttcttacgtatccaaggaagtgctaaaaaatgtaggcacttttactaagatatcatttgcactaattattttttaaattagcacagaaccaaatcctataattactgaagggtagcaagttgacttgcagaaaactccttccatctttttctggggccagaggtaattagtgtatttgagggtctcctccacctaccatctgttatcccctgggtcggagtcaatgttggtgcccatatagctggcctgaaggttggcaaaggtatcaggggatggggaacagtagagaaattaggaagacccagacctgctgtggcagtgatttggatccagttgggtgtttcacggagttacagaatgcaaacagagatttctggagagactctaaggagtctgtgtagttgtttttctgaataggtgcttggagccagtgtcactcctgggtcaacatctggttctcctggagcttgggacaaggctctttgactctctttatgcttctgtttgctacagggcgtcaggatgaaacaagagagtgcccttcacttattccagggaatgttgggatcataggccctcagtcaaaactcaaagtcatcatttgtgacacacccccatctttcccagggcttcaggtgaacctgcctgataggcagtcgtgctcatcaggttcctagcaaagatttcatcaccttgcttaacagccaacacggtgggccaacaagtccttccgtcaagggaagtccttcccaagtctaatcagaggctgtgctgttgtggtgcatattaatttcctgttcttggcacacctgtgcagatggaaaacagctgctcactcctgaccccatacaacctttcccatgcatttggtttctttcctgaattctaaatcccatgccaacaccttgaaaagctttctgaatgtactgctgctgcagtctctcatttcaacaatccctatacatttcccccattacaataaaaagctggaaacgtctgacgtcctaactaaatgactaggtgatgggtgagtcttttgggaagaggatgccaggatgtcaggcaatcccaaatacagctgaatcccagttgccggcagctggtcagcctcttctgaactatctgtagccctttttatgctctacactctctgggctctcttcctcctctctcgtgggacccaatctcttctaggttgcccccactttctgcctctgaaagggttcagaaaaagcaaggttttctttttgacattagctaaaataacaaacaggatgaggctggaagcctgctggggatgaatcaatcatcccagtgtatgactaatctgcaaatggggccacatctgggccctgggccctggtgcagggcatggtctgtgacccaccacccagaggttgcttggcagaatgcaggacctctgcatcttcctgccaactctaccttcctggacatgtgcagccaacgtgggcagtcaagaggagcaccagagcagccagccaccgcatctccatgtagcctcagtttctccctgaaactaattgtccccacgggtgaaaatgggttagcagtgttctcccatcatcctgatggccccagaaagctcatcaaagttggtgtggcaggaggaaaagggcccactagggaatgactgcacagactgagcctgggccaactcagtgcagtctcaggcatcactattgagtgcctactgagtacaaggccctaggccagaagtggttgaggaagtagagcccgccctgactcccgtcttagggttgaccagctggctgaggcacaggcaggtgtgcgcggaacagcttggcaacagcatgagtcagtgtgagggtgtctgcctgggcgcgtgagtgcagcaaggagccagccggggtgctcatgggtggtgtccccgagagctggtcctgtgctcttgcctctggtgggccaggctgaagggagccttgaaggatgaagggaacagcagcatcccatcagagtggcactcagcaaaggcacccttcagtgggcagctgcctgggtcctcctccatcagagagcccctgcatgacaggggtgacaaggacactgccacaggccagctacatggggctttccttggggtgccgtcactcaaaggaagccgcccagctttgatccctccagtagggggcaacaggagatggctgcttcgtgggcagaaatcagagtttcctgggaaggaaacccaggtgggtgtccccacgggcagatgcatggacgtgggtatgagccaccatgggccacgtggccaagggcaacactctagagagggtagagcagtgagaagcaaggatccggcccccacactgttgggctaccacaccagccccaaacgcccatccaggctggtggcaagagaaaaataaagattcctcttgtttatgccaccctgttgtttgtacctaataaattcagtctctgatgtctaaaaataaagcctgtcatcactgaaccaaggtgctgccaaccacaggagacctcgtgtaaattcaggcccacagatgctcctgcctccccctgcagcacccaggtctgaaccttggccatccatccaggaggtgcaactccccctcacctcctctgtgcacctgcccaggtttctgaactccaggctgccccctgggccccatctcatgccgtgcagggtgcatttttttacacctgtgtcttgtccttcccacttagcagtgacgcccttgaaggcaggtccctggcttcaagcccaccgggagctcagcaccaggtccctgcaaacactcctggttgacaaacctctaagaaatcgctcctgaaagaccctctccaaccttcagaggtttccgtggctgtaagcaatttcatacagcacaggtggtgcatcccacgccagactcaggcaaacccagcattctgactgagccttcccttccgtcccagccggctctccaggcatgggcgtcgcagactctgcacccaagaccaacacggcaccaggcacacatgtctgtggcagggggtgtccctcagtggcccagcccctcttccacttctcggaagtagacatctctccctcttccctctgagatgatcagtcggccaccgcaggtcaggggtgatgggaatgccagtgcccctaaggcctgtaggaggtccctcccacaaaaccttgcctctgggcatgtcaggtgattaggtggggttctatgcagagaccctgtcctccaccctccttgggctcctcccctgtaatgaagctacgtctcagttccacctgtcaagaaaggatttaatatgagcttttcacaacttcacttttaagttgagttatatttcgttttgtcaaacactgcgtaccccgagtcaactgctcagctgcttcttgaaggtgagattggggtgagctgctccttgcggtgttagggtgcctggagcagggacaagcccatacctaaccccactccacaagcccccagccctgctccatgggcccatattatctggcgaacccctacatgacctcctgcaggtggggaaggcagacccgagaggacagctgggtgcgggaggtgaggcagatgaggggagaaagggggtagaacacttcctgaacccctggagaccctatcaggagtgatgtggagaaggggaccagaggggaaagacagcagacaagcccccagaaagatggtaaagaggagaggaaaaaggactcttcattggaacattccagaaccagacacctgctgaccaaacagcagagagctctcagtgacaaacctcttatttcccatccaagagcttcaagcacttcctgaaagcctctctctggtgcttgagtccccaaatccaagttcaccattgctgctgaagagtgaggggaatctccttttaggagaccccagaataactggcaggagctagagacagtgcccctgaggagcagggcctagaccaaaagctagggggtcagggagcataacatggggtcccaggcagggaggcagcagagacagaggcaccccctagaaggccacctcctgcagttgggcaaggtagcagtgccgtatggggaggagggcagacaagtggcacctccgtgggactcagtttcctcatctgcaaatggcacggagatgttagaaggaccctcagaggccgtcgaggctccttctgggttttatgtgaggaagctgagacccaagaaggaagagtttgccaccaagtttgcggcagaacaaaaacgagactccaggtctcccatcaccccccacccccggggctcttattatggcctccttcttaagaaacaagacgtacaagcacattttgtcacgtgaaagaaccatcctgggcagccgtccctccacaccatggggcagccacgccctacagcctaagaaagatctagaaccaaggccactgaccagcttctctcgggacagaatagaggagttgggtgaatctgccaggagaccgaagctgaacatgattaagtggactgaagctgaacatgagcaagcaggcccagggcaacccatgactgcagcggctctgaaaccaggcatggcccctcgcaggagcctgcaggggctccctccgctttccagacaggcatagtcggaggctggactcgggatggggacacatgtttttttcagcctctaatcccacaggctccgcaagcagcagggagaaaggtggcaggctctggcggggtcccaggactgttggttggctggggggatggacaggtctctgacagctcccccacaggctgcccctcccaggccttctgcagatctggagcagaagtgatatccaaagcacccaccagcatcaaaatgccgagtcccattgtttgtggggctgcaatgtcggtacctgaaccctcagtgcagtcatttgagagccgtgtaatattccactgtaaggatggatcccaaggcacctctccattcccctcagtgaacatctgggctgcttccagatatgtgttaatatatagaacgcagctactaaaaagaaatctcatcaatcgatgagtttgggggagtgggagcttccctgtgggcagggagttagggagggctttccagggaacagatgccccctcccctctcccacctctctgcactctccatgtcaccactcctcaggagccactgtgggccggcccaggaacccaggcagacaagacataggacacccccagacagagcgcagagctgg

SEQ ID NO: 14485 - RNA, 846 nt, Homo sapiens
  source 1..846: mol_type = other RNA
gctgggattacaggcatgagccaccgggccaagccagcatttcttgtttgatagactaagcgtaaatttctcaaggatcagctggttcttctagtttgtatgagcaaagatatgctgctctgtctggatcaagatctcttgctgtctccgcgctcagccccatgggctctcgcctgcagacacatgcagctgcgagatttcaggaggctccacaggctctgcagggcctcgggcagcccctccccagtgagggcactgcagccccggagctcccagcagtggtcctggaatctctctagactcagcctgtttctgatcttaagcagcggaagtgcatcaggtgcctcctgcttgttggccagcaccaagaaggggacgccagccatgttggggtcgttcaggacttctgtgagctcagccgccgactcgggtaagcgggcttcatctgtgctgtccagcacgtacacgaggatatctgtgccttccagatagtccttccagctggctctgagcggggcctgccccccaacgtcccagagagtcagtgacacgtgcccaggagctttcagaggctccacgttgaaaccaacagtgggcagggtctccaccagctggtggcccttcagcttgtaaaggagcgtggtcttgcccgccgagtccaggcccatcatcaccacctgggcttccgccttgtgacctctggaattcacagaacccatggtggccactgctgaatcctctgtgttactattagactgcagctgtgagatcctgcgtggctctcctcccctatggagctgctttctgctggccaggcatgacccaagagcgagatgggaaggaagc

SEQ ID NO: 14486 - RNA, 963 nt, Homo sapiens
  source 1..963: mol_type = other RNA
gctgggattacaggcatgagccaccgggccaagccagcatttcttgtttgatagactaagcgtaaatttctcaaggatcagctggttcttctagtttgtatgagcaaagatatgctgctctgtctggatcaagatctcttgctgtctccgcgctcagccccatgggctctcgcctgcagacacatgcagctgcgagatttcaggaggctccacaggctctgcagggcctcgggcagcccctccccagtgagggcactgcagccccggagctcccagcagtggtcctggaatctctctagactcagcctgtttctgatcttaagcagcggaagtgcatcaggtgcctcctgcttgttggccagcaccaagaaggggacgccagccatgttggggtcgttcaggacttctgtgagctcagccgccgactcgggtaagcgggcttcatctgtgctgtccagcacgtacacgaggatatctgtgccttccagatagtccttccagctggctctgagcggggcctgccccccaacgtcccagagagtcagtgacacgtgcccaggagctttcagaggctccacgttgaaaccaacagtgggcagggtctccaccagctggtggcccttcagcttgtaaaggagcgtggtcttgcccgccgagtccaggcccatcatcaccacctgggcttccgccttgtgacctctggaattcacagaacccatggtggccactgctgaatcctgtctctgggtcagataagagtggtccctgagcagagaagatcaggggcctcctggaagacattcctctgtgttactattagactgcagctgtgagatcctgcgtggctctcctcccctatggagctgctttctgctggccaggcatgacccaagagcgagatgggaaggaagcagagcagccgttgctgcttctcctttttgtgcttccttttcccaggtggct

SEQ ID NO: 14487 - RNA, 4804 nt, Homo sapiens
  source 1..4804: mol_type = other RNA
gctgggattacaggcatgagccaccgggcccagccagaaaattataaacacgcacaaactctcaagtggcctaattccctctcatcaaaccaatcacaatacaaataaaagagaataacttatattagtttttgtacaaacaaaaaagactgataaattgtgaatgatgcatgatttttaattacaagtaaactgggcatatgcttctgcattatttaaagctaaagggtgatcagtggaaattttcttctgttagtactttaatactttttatatttatcggctcactacaacctatgcctcccaggttcaagcgattctcctgtctcagccacctgagtagctgagactacaggacgcactaccatgtccggttaattttgtatttttaatagagacggggtttcactgtgttggccatgctggtcttgaactcctgacctcaaccgatccacctgccttggcctcccaaagtgctgggattacaagcatgagccaccgcgcccagccttcttataattgttattatttaaatctcttttgctctctccttcaagagagacctcatctcattcagttgcatccatttatttattcatcttctgcctcctgagctcgagagatcctcctgcatgagtcttccaagtagctgggactacaggctcacaccaccatgcttggctaatttttgtaggttttggagagacaggctcttgccatgttgcctaggctggtctcaaactcctgggctcagatgatccacctgccttcgcctcccaaagcacttggattatagacataagcgatcatgcccagccccaagtacttttatacaaaatgcaaacactattcttctatcataaaagtgataccacagcttctgtaaagttttgcaccaggtagtacttataattaacttgggtacagttttttgtttgtttgtttgttttgagacagattctcgctctgtcgcctaggctggagtgcagtggcctgatctctgctcactgcaagctccgcctcccgggttcatgcaattctcctgcctcagcctccagagcagctgggactacaggcgcccgccaccatgcccagctaattttttgtatttttagtagagatggcgtttcaccatgttagccaggatggtctcgatctcctgacctcgtgatctgcccgcctcggcctcccaaagtgctgggattacaggcgtaagccactgtgcccggcctacgttttgatgttaaaatgtatcttcttattacgaaaccatttttccattgtattaactacttttacaacaaagcaaataacaagttattttacaaaccatttagaaatttctgtactatggtcccaataatgtaaaatatattaatgccttttacattcaggtaaattatccacttggaaactacatatttatgacttacagaaacttacataaacaaattatacaaattatatgctcaatttttaggtatatagtcttaaattaagcttaaatatacattctcaggataaattaacagttcagggcttcacaacttgaaatctgtggaacatgacattggagatgacagaactctggtggaattcttaggtggaatttactgaaactttttttttttgagacggagtctcactctgtcacccaggctggagtgcagtggcacaatctcagctcactgcaatctctgcctcccgggttcatgccattcgtctgcctcagcctcccgagtagctgggactacaggcgcccaccaccacgcctggctaattttttgtatttttagtagagatggggttttaccatgttagccaggatggtctcgatctcctgaccttgtgatccaaccgccttggcctcccaaagtgaaacttttctttaaaatagagatgggatcttgctgtattgcccaggctggtctcaaactccttgccttaagcaatcctcccacctcagcctcccaaagtgctgggattacaagcgtgaaccactacgtccaagtgaaacttcttgagatagttacataatttttaaatctgctggtgtagaagttaataaagtgtagaactgaataaatattaaatattagatcaagtttctcatgtttaccttaaagtataaatatttatcttaaagcactgattttcacaaaataacatcagtgtgaaattggaaaagaaaccaagtattttatttcatgtatctgggaaatgaggtgctttagtcaactgaatctgcccaaaactaaaaagcattcattaaaaattataaaaatagaagacatcaataaaatacattctacacagaatacgccaatcatacactactctgtttttgataataaaaaatgtacttactgagccaggtgcggtggctcatgcctataatcccagcaccttgggaggccaatgagagtggatcagttgaggccaggagttggagactgtctcacgtgtccgtgtgaagaggccaccaaacaggctttgtatgagcaacatggctgtttatttcacctgagtgcaggcgggctgagtccaaaaaaggagtcagcaaagggtggtggattatcattagttcttacaggtttggggataggtggtggagtttggagcaatgttttgcgggcaggggtggatctcacaaagtacattctcaagggtggggagaattaaaaagaaccttcttaagggtgggaggattacaaagtacattgatcagttagggtggggcagtaacatatcacaatggtgcaatgtcatcagttaaggctattttcacttctgtggatcttcagtaacttcaggccatctggatgtatatgtgcaggtcactgggatatgatggcttagcttgagctcagaggacggacagagaccagcctagccaacatggcaaaacgccctctctactaaaaatacaaaaatgagccaggcatggtggcacctgcctgtaatcccagctactccgaaggatgaggcagtaggatcgtttgaacccaggagacagaggttgcagtgagccgaaatcatgccactgcactccagcctgggtgacagagcgagtctctgtctcaaaaaaaaaaaaaaaaaaaagtcggttgtggtggctcacgcctgtaatcccagcactttgggaggccgaggtgggtggattatgcggtcaggagatcaagaccatcctggccaacacggtgaaacttcatctctactaaaaatacaaaaaattagctaggcatcgtggcaggtgcctgtagtcccagctacttgggaggctgacgcagaatggcgtgaacccgggaggcggagcttgcagtgagccgagatctcacaactgcattccagcctgggcgacagagcgagactctgtgtcaaaaacaaaagcaaatgaacaaaaatacaaaaatcagctgggcctggtgtcacgtgcctgtaatcccagctactcaggagcctgaggcaggagaattgcttgaacccagaggatggaggctgcagtgagccgcgatcgtgccactgcgctccagccggggagacagcaagactccaccacaaaaaaaaaaaaaaaaaaaaaggtatttactaaaataacaaattgtgtatgttttggagaaagaaatctggttattaaatcttcatttcgattgagttctatgtaaattaaaattcactctaagaactattttttggtataaaacttcatctgcccaaaagtgttcaggagataacctgagattttagaatagaaatgtgaacaatcaaaaccaagtttcctgaaacttgtgttaaaatattagaaatattaataattctaaaatgccattttgccactattattcatattaaccaaaatattagagaagtaatatttcagactagaacaggaaaaaagtctgaatacaattcaaaaataatcattgataattttttaaaaagtgggtctataaatagtagtaattcctcaaaatgaagtgcataattggcacatcaaatattttgtctgcaggcaattctgtgcattttaggtaaaaaatgtggtccctttaagagagtccttgacttctcatttcttcgggtacccttctgtggcactggtcccctttgtatataaaatggtgaaagctgacttgaatgtgccgtcaccactctgctgggaaaaacagatgaaggtggcccagagaaaaccacagactccagcgtaagctgttctccattgaacaggaacaaggctgaagttggtcagctgtacaaagggccagtacatcagtccactcagataggtattccagaatttctgtttcaggtccaaaaatatgtcatcctttccttggagaatgctcataccgacatagaaggccgagaccgcgatgggcgcaccgaccacctggtcgcacagcaacttggccagcagggcgtgcggcgctcggcccgggagcgcgcgctccagcaggcgcagccacacgtagttgaagttggcgtggaaggtcaccaccaacgtggccacgcgccgcgtctggcgccagttggcctcgcggccctgcagccgctgttgcagcgcgtccccggccgagacgagcgagccgtaaagcagcacgttggtgggccacgggtggcgccgggccgcgcgcgacaacgccggccaccagcccgccatgtccgcgctgtgggcgcccgcgatcaggagcccgcgtggtcggcgtcttcctgcaccgggtccgggcctccccagcctccagcagctactgcactgcagcagccggcacctgcatctgccccctccagaagctccggagcgatt

SEQ ID NO: 14488 - RNA, 4733 nt, Homo sapiens
  source 1..4733: mol_type = other RNA
gctgggattacaggcatgagccaccgggcccagccagaaaattataaacacgcacaaactctcaagtggcctaattccctctcatcaaaccaatcacaatacaaataaaagagaataacttatattagtttttgtacaaacaaaaaagactgataaattgtgaatgatgcatgatttttaattacaagtaaactgggcatatgcttctgcattatttaaagctaaagggtgatcagtggaaattttcttctgttagtactttaatactttttatatttatcggctcactacaacctatgcctcccaggttcaagcgattctcctgtctcagccacctgagtagctgagactacaggacgcactaccatgtccggttaattttgtatttttaatagagacggggtttcactgtgttggccatgctggtcttgaactcctgacctcaaccgatccacctgccttggcctcccaaagtgctgggattacaagcatgagccaccgcgcccagccttcttataattgttattatttaaatctcttttgctctctccttcaagagagacctcatctcattcagttgcatccatttatttattcatcttctgcctcctgagctcgagagatcctcctgcatgagtcttccaagtagctgggactacaggctcacaccaccatgcttggctaatttttgtaggttttggagagacaggctcttgccatgttgcctaggctggtctcaaactcctgggctcagatgatccacctgccttcgcctcccaaagcacttggattatagacataagcgatcatgcccagccccaagtacttttatacaaaatgcaaacactattcttctatcataaaagtgataccacagcttctgtaaagttttgcaccaggtagtacttataattaacttgggtacagttttttgtttgtttgtttgttttgagacagattctcgctctgtcgcctaggctggagtgcagtggcctgatctctgctcactgcaagctccgcctcccgggttcatgcaattctcctgcctcagcctccagagcagctgggactacaggcgcccgccaccatgcccagctaattttttgtatttttagtagagatggcgtttcaccatgttagccaggatggtctcgatctcctgacctcgtgatctgcccgcctcggcctcccaaagtgctgggattacaggcgtaagccactgtgcccggcctacgttttgatgttaaaatgtatcttcttattacgaaaccatttttccattgtattaactacttttacaacaaagcaaataacaagttattttacaaaccatttagaaatttctgtactatggtcccaataatgtaaaatatattaatgccttttacattcaggtaaattatccacttggaaactacatatttatgacttacagaaacttacataaacaaattatacaaattatatgctcaatttttaggtatatagtcttaaattaagcttaaatatacattctcaggataaattaacagttcagggcttcacaacttgaaatctgtggaacatgacattggagatgacagaactctggtggaattcttaggtggaatttactgaaactttttttttttgagacggagtctcactctgtcacccaggctggagtgcagtggcacaatctcagctcactgcaatctctgcctcccgggttcatgccattcgtctgcctcagcctcccgagtagctgggactacaggcgcccaccaccacgcctggctaattttttgtatttttagtagagatggggttttaccatgttagccaggatggtctcgatctcctgaccttgtgatccaaccgccttggcctcccaaagtgaaacttttctttaaaatagagatgggatcttgctgtattgcccaggctggtctcaaactccttgccttaagcaatcctcccacctcagcctcccaaagtgctgggattacaagcgtgaaccactacgtccaagtgaaacttcttgagatagttacataatttttaaatctgctggtgtagaagttaataaagtgtagaactgaataaatattaaatattagatcaagtttctcatgtttaccttaaagtataaatatttatcttaaagcactgattttcacaaaataacatcagtgtgaaattggaaaagaaaccaagtattttatttcatgtatctgggaaatgaggtgctttagtcaactgaatctgcccaaaactaaaaagcattcattaaaaattataaaaatagaagacatcaataaaatacattctacacagaatacgccaatcatacactactctgtttttgataataaaaaatgtacttactgagccaggtgcggtggctcatgcctataatcccagcaccttgggaggccaatgagagtggatcagttgaggccaggagttggagactgtctcacgtgtccgtgtgaagaggccaccaaacaggctttgtatgagcaacatggctgtttatttcacctgagtgcaggcgggctgagtccaaaaaaggagtcagcaaagggtggtggattatcattagttcttacaggtttggggataggtggtggagtttggagcaatgttttgcgggcaggggtggatctcacaaagtacattctcaagggtggggagaattaaaaagaaccttcttaagggtgggaggattacaaagtacattgatcagttagggtggggcagtaacatatcacaatggtgcaatgtcatcagttaaggctattttcacttctgtggatcttcagtaacttcaggccatctggatgtatatgtgcaggtcactgggatatgatggcttagcttgagctcagaggacggacagagaccagcctagccaacatggcaaaacgccctctctactaaaaatacaaaaatgagccaggcatggtggcacctgcctgtaatcccagctactccgaaggatgaggcagtaggatcgtttgaacccaggagacagaggttgcagtgagccgaaatcatgccactgcactccagcctgggtgacagagcgagtctctgtctcaaaaaaaaaaaaaaaaaaaagtcggttgtggtggctcacgcctgtaatcccagcactttgggaggccgaggtgggtggattatgcggtcaggagatcaagaccatcctggccaacacggtgaaacttcatctctactaaaaatacaaaaaattagctaggcatcgtggcaggtgcctgtagtcccagctacttgggaggctgacgcagaatggcgtgaacccgggaggcggagcttgcagtgagccgagatctcacaactgcattccagcctgggcgacagagcgagactctgtgtcaaaaacaaaagcaaatgaacaaaaatacaaaaatcagctgggcctggtgtcacgtgcctgtaatcccagctactcaggagcctgaggcaggagaattgcttgaacccagaggatggaggctgcagtgagccgcgatcgtgccactgcgctccagccggggagacagcaagactccaccacaaaaaaaaaaaaaaaaaaaaaggtatttactaaaataacaaattgtgtatgttttggagaaagaaatctggttattaaatcttcatttcgattgagttctatgtaaattaaaattcactctaagaactattttttggtataaaacttcatctgcccaaaagtgttcaggagataacctgagattttagaatagaaatgtgaacaatcaaaaccaagtttcctgaaacttgtgttaaaatattagaaatattaataattctaaaatgccattttgccactattattcatattaaccaaaatattagagaagtaatatttcagactagaacaggaaaaaagtctgaatacaattcaaaaataatcattgataattttttaaaaagtgggtctataaatagtagtaattcctcaaaatgaagtgcataattggcacatcaaatattttgtctgcaggcaattctgtgcattttaggtaaaaaatgtggtccctttaagagagtccttgacttctcatttcttcgggtacccttctgtggcactggtcccctttgtatataaaatggtgaaagctgacttgaatgtgccgtcaccactctgctgggaaaaacagatgaaggtggcccagagaaaaccacagactccagcgtaagctgttctccattgaacaggaacaaggctgaagttggtcagctgtacaaagggccagtacatcagtccactcgacatagaaggccgagaccgcgatgggcgcaccgaccacctggtcgcacagcaacttggccagcagggcgtgcggcgctcggcccgggagcgcgcgctccagcaggcgcagccacacgtagttgaagttggcgtggaaggtcaccaccaacgtggccacgcgccgcgtctggcgccagttggcctcgcggccctgcagccgctgttgcagcgcgtccccggccgagacgagcgagccgtaaagcagcacgttggtgggccacgggtggcgccgggccgcgcgcgacaacgccggccaccagcccgccatgtccgcgctgtgggcgcccgcgatcaggagcccgcgtggtcggcgtcttcctgcaccgggtccgggcctccccagcctccagcagctactgcactgcagcagccggcacctgcatctgccccctccagaagctccggagcgatt

SEQ ID NO: 14489 - RNA, 3120 nt, Homo sapiens
  source 1..3120: mol_type = other RNA
gctgggattacaggcatgagccaccgggcccagccagaaattttttttaaaataattcattttaaactggctataatttcatggataatttgatctttaaaagaacatcatggaaaattttaaatacacaaaagtagaatagcaaaaacaaaacaaataaaaaccatgtatccaagacttaggttaccatcattttgccaaacttgttattcatcctcatttttcttttgtatgaacaaaaggacattccagatatatcatctcctgtgtatagacttcagaaattatctctaacaaatacacttttacataaccacaatgctattatcacacataacaaagtttcttaatattatctaatattgtcaatattccattctcccaattattgttaagtatctcttcttttacatgtttgttcaactcatgatctaagtaaaaaccactgtttcattgcatttgactgatgtctcaagtctgtcaatacctaggagttccaccttatttcttaaaatgccattttattggttgggaaaccaggtgattcctcttgtagaattacccttattttagatttaattgctcctttttgtgtcatgtaatttactcttccattccttgaattttctctaaactgggagttggctcttgaggcttaaattcaggttcaatatttttggcaagatgtgtatatcttactgtagcacattaggaggcacgtaatttttactctcttgctttttgtgaagttgagatgatgagtgggttcagacgttgtcagtctcatctattcactataaagttcacaaccttcactgaatggtgtcaacctgtacagagaatcatgcctagatccattatttcattatgtgttacacaatagtttttctaatataattttctattattctttctgcattcattagcctggaattttctaataaagaagaactttacctccttaacttctggttgccctgaaatacagttcctacaggaaatgcagactaaatgactttcctttcatttacacattttcagaatgaagtggttccctagcaaccttcgtgtgtatatacacagatggaagaatatggagataataataggtaagatcaaaagcttttccacattcagtcctgtaataaagttcttttctaggatgaatttcctaaagtttaacatggtttcaaaggtgatgaaaggcttctatatgttcattaacatattctttcctttaaataaaacttcctatgcttagttgtgagcatgaagcaaaagggattcccacgttcaaaaacctttcctctagaatgtacttcctatgctcaacataaaattcgcaaaggaagagttctaataattattaagttacattatgaattcgctgatggtaagtaagatgtgaatgttgtctaaatgcctttttacattccttacatttgtatggtttctcaccagaatgaattctctgatgttgaatcagtgatgaatgaagtctaaaggcctttccacattccttacagtcatagggcttttcaccagtatgaatactttgatgttgggtaagttgtgaaagcagtctaaaagtcttctcacattccttacacttaaagggtttctcaccaaaatgaatactctgatgttgagtaagctgtgagaacagcctaaatgccttcccacattccttacattcataaggtttctctccaatgtgaataccctgatgtgaaataagttctgagtaacgacgaaagaacttctgacattccttacattcatagggcttttcaccagtatgtattctctgatggagagttagatgatagccacgactgaaagtcttcccacattccttacaatcataaggcttctcaccagtgtgaattctctgatggagagtaagttgctgccgcactctaaaggcctttccacactccttacattcatagggtttttctccagtatgaagtttgtgatgtagtcgaaggcctgtactacacagaaaggcctgaccacattccttacactcatagcacttctcagcaatgttcagtctctgatgtcgagtaaggtgtgcatactgcctaaaggccttcccacattctttacattcatagggtttctcacccgtgtgaatcctttgatggagattaagttgtcctctaactctaaaggctttcccacattctttacattcatacggcttctcaccaatatgaattctctgatgtactcgaaggtctgagccacatgtgaagatctttccacattttttacattcatagagtttgtcagaagtatgaattctctgatgtcgactgaggtgggcacactgtctaaaggcttttccacattctttacattcatagggtttctcaccagtatgaattctttgatggaaagtaagttgttgtcgtactctaaaagccttcccacattccccacattcgtagggtttctctctgttatgacttttctgatacagaggaagagatgtgagttttctgtaagtaggcattttttcagaggtggtttttgtcacttgcctgaaacacacctcatgaggactttcttgttcttcaagtccacagcttttaattctttccattaccttccactgagataagttcatttcataaatatcctttccttgaaataactttttagtgtcatatctggattccaaatctagagtccatcttcttttctcatccctcacaaccatccagggctctttcccttgttccaatagggtgatcacatctggcttagaaatagaacatcccagtgacaccaagttgctatagttctctaatatcacatctctgtacaaattcctctgatatgagttcaggcattcccattcttcctgagaaaagtctacagccacatctctgaacatcaccaaatcacgagccatgattttagaactgctagaactggtcaattttcctcaaggttcatgtacttcagaagcagggtccacagacaccagagagggaaccggcttttagaagagcagcagcgattcgtttctccttctcaagcgccttctctggaaactggcagggccgactcagaggatagcccagccctgggagtcagcggcgccagaat

SEQ ID NO: 14490 - RNA, 3214 nt, Homo sapiens
  source 1..3214: mol_type = other RNA
gctgggattacaggcatgagccaccgggcccagccagaaattttttttaaaataattcattttaaactggctataatttcatggataatttgatctttaaaagaacatcatggaaaattttaaatacacaaaagtagaatagcaaaaacaaaacaaataaaaaccatgtatccaagacttaggttaccatcattttgccaaacttgttattcatcctcatttttcttttgtatgaacaaaaggacattccagatatatcatctcctgtgtatagacttcagaaattatctctaacaaatacacttttacataaccacaatgctattatcacacataacaaagtttcttaatattatctaatattgtcaatattccattctcccaattattgttaagtatctcttcttttacatgtttgttcaactcatgatctaagtaaaaaccactgtttcattgcatttgactgatgtctcaagtctgtcaatacctaggagttccaccttatttcttaaaatgccattttattggttgggaaaccaggtgattcctcttgtagaattacccttattttagatttaattgctcctttttgtgtcatgtaatttactcttccattccttgaattttctctaaactgggagttggctcttgaggcttaaattcaggttcaatatttttggcaagatgtgtatatcttactgtagcacattaggaggcacgtaatttttactctcttgctttttgtgaagttgagatgatgagtgggttcagacgttgtcagtctcatctattcactataaagttcacaaccttcactgaatggtgtcaacctgtacagagaatcatgcctagatccattatttcattatgtgttacacaatagtttttctaatataattttctattattctttctgcattcattagcctggaattttctaataaagaagaactttacctccttaacttctggttgccctgaaatacagttcctacaggaaatgcagactaaatgactttcctttcatttacacattttcagaatgaagtggttccctagcaaccttcgtgtgtatatacacagatggaagaatatggagataataataggtaagatcaaaagcttttccacattcagtcctgtaataaagttcttttctaggatgaatttcctaaagtttaacatggtttcaaaggtgatgaaaggcttctatatgttcattaacatattctttcctttaaataaaacttcctatgcttagttgtgagcatgaagcaaaagggattcccacgttcaaaaacctttcctctagaatgtacttcctatgctcaacataaaattcgcaaaggaagagttctaataattattaagttacattatgaattcgctgatggtaagtaagatgtgaatgttgtctaaatgcctttttacattccttacatttgtatggtttctcaccagaatgaattctctgatgttgaatcagtgatgaatgaagtctaaaggcctttccacattccttacagtcatagggcttttcaccagtatgaatactttgatgttgggtaagttgtgaaagcagtctaaaagtcttctcacattccttacacttaaagggtttctcaccaaaatgaatactctgatgttgagtaagctgtgagaacagcctaaatgccttcccacattccttacattcataaggtttctctccaatgtgaataccctgatgtgaaataagttctgagtaacgacgaaagaacttctgacattccttacattcatagggcttttcaccagtatgtattctctgatggagagttagatgatagccacgactgaaagtcttcccacattccttacaatcataaggcttctcaccagtgtgaattctctgatggagagtaagttgctgccgcactctaaaggcctttccacactccttacattcatagggtttttctccagtatgaagtttgtgatgtagtcgaaggcctgtactacacagaaaggcctgaccacattccttacactcatagcacttctcagcaatgttcagtctctgatgtcgagtaaggtgtgcatactgcctaaaggccttcccacattctttacattcatagggtttctcacccgtgtgaatcctttgatggagattaagttgtcctctaactctaaaggctttcccacattctttacattcatacggcttctcaccaatatgaattctctgatgtactcgaaggtctgagccacatgtgaagatctttccacattttttacattcatagagtttgtcagaagtatgaattctctgatgtcgactgaggtgggcacactgtctaaaggcttttccacattctttacattcatagggtttctcaccagtatgaattctttgatggaaagtaagttgttgtcgtactctaaaagccttcccacattccccacattcgtagggtttctctctgttatgacttttctgatacagaggaagagatgtgagttttctgtaagtaggcattttttcagaggtggtttttgtcacttgcctgaaacacacctcatgaggactttcttgttcttcaagtccacagcttttaattctttccattaccttccactgagataagttcatttcataaatatcctttccttgaaataactttttagtgtcatatctggattccaaatctagagtccatcttcttttctcatccctcacaaccatccagggctctttcccttgttccaatagggtgatcacatctggcttagaaatagaacatcccagtgacaccaagttgctatagttctctaatatcacatctctgtacaaattcctctgatatgagttcaggcattcccattcttcctgagaaaagtctacagccacatctctgaacatcaccaaatcacgagccatgattttagaactgctagaactggtcaattttcctcaaggttcatgtacttcagaagcagggtccacagacaccagagagggaaccggcttttagaagagcagcagcgattcgtttctccttctcaagcgccttctctggaaactggcagggctggggaagcaggcagagttcaggacaccccaggcttttcttgactcgattggaacccaccctccacgcttccctggccccaactaaccgccacccgactcagaggatagcccagccctgggagtcagcggcgccagaat

SEQ ID NO: 14491 - RNA, 3496 nt, Homo sapiens
  source 1..3496: mol_type = other RNA
gctgggattacaggcatgagccaccgggcccagccagaaattttttttaaaataattcattttaaactggctataatttcatggataatttgatctttaaaagaacatcatggaaaattttaaatacacaaaagtagaatagcaaaaacaaaacaaataaaaaccatgtatccaagacttaggttaccatcattttgccaaacttgttattcatcctcatttttcttttgtatgaacaaaaggacattccagatatatcatctcctgtgtatagacttcagaaattatctctaacaaatacacttttacataaccacaatgctattatcacacataacaaagtttcttaatattatctaatattgtcaatattccattctcccaattattgttaagtatctcttcttttacatgtttgttcaactcatgatctaagtaaaaaccactgtttcattgcatttgactgatgtctcaagtctgtcaatacctaggagttccaccttatttcttaaaatgccattttattggttgggaaaccaggtgattcctcttgtagaattacccttattttagatttaattgctcctttttgtgtcatgtaatttactcttccattccttgaattttctctaaactgggagttggctcttgaggcttaaattcaggttcaatatttttggcaagatgtgtatatcttactgtagcacattaggaggcacgtaatttttactctcttgctttttgtgaagttgagatgatgagtgggttcagacgttgtcagtctcatctattcactataaagttcacaaccttcactgaatggtgtcaacctgtacagagaatcatgcctagatccattatttcattatgtgttacacaatagtttttctaatataattttctattattctttctgcattcattagcctggaattttctaataaagaagaactttacctccttaacttctggttgccctgaaatacagttcctacaggaaatgcagactaaatgactttcctttcatttacacattttcagaatgaagtggttccctagcaaccttcgtgtgtatatacacagatggaagaatatggagataataataggtaagatcaaaagcttttccacattcagtcctgtaataaagttcttttctaggatgaatttcctaaagtttaacatggtttcaaaggtgatgaaaggcttctatatgttcattaacatattctttcctttaaataaaacttcctatgcttagttgtgagcatgaagcaaaagggattcccacgttcaaaaacctttcctctagaatgtacttcctatgctcaacataaaattcgcaaaggaagagttctaataattattaagttacattatgaattcgctgatggtaagtaagatgtgaatgttgtctaaatgcctttttacattccttacatttgtatggtttctcaccagaatgaattctctgatgttgaatcagtgatgaatgaagtctaaaggcctttccacattccttacagtcatagggcttttcaccagtatgaatactttgatgttgggtaagttgtgaaagcagtctaaaagtcttctcacattccttacacttaaagggtttctcaccaaaatgaatactctgatgttgagtaagctgtgagaacagcctaaatgccttcccacattccttacattcataaggtttctctccaatgtgaataccctgatgtgaaataagttctgagtaacgacgaaagaacttctgacattccttacattcatagggcttttcaccagtatgtattctctgatggagagttagatgatagccacgactgaaagtcttcccacattccttacaatcataaggcttctcaccagtgtgaattctctgatggagagtaagttgctgccgcactctaaaggcctttccacactccttacattcatagggtttttctccagtatgaagtttgtgatgtagtcgaaggcctgtactacacagaaaggcctgaccacattccttacactcatagcacttctcagcaatgttcagtctctgatgtcgagtaaggtgtgcatactgcctaaaggccttcccacattctttacattcatagggtttctcacccgtgtgaatcctttgatggagattaagttgtcctctaactctaaaggctttcccacattctttacattcatacggcttctcaccaatatgaattctctgatgtactcgaaggtctgagccacatgtgaagatctttccacattttttacattcatagagtttgtcagaagtatgaattctctgatgtcgactgaggtgggcacactgtctaaaggcttttccacattctttacattcatagggtttctcaccagtatgaattctttgatggaaagtaagttgttgtcgtactctaaaagccttcccacattccccacattcgtagggtttctctctgttatgacttttctgatacagaggaagagatgtgagttttctgtaagtaggcattttttcagaggtggtttttgtcacttgcctgaaacacacctcatgaggactttcttgttcttcaagtccacagcttttaattctttccattaccttccactgagataagttcatttcataaatatcctttccttgaaataactttttagtgtcatatctggattccaaatctagagtccatcttcttttctcatccctcacaaccatccagggctctttcccttgttccaatagggtgatcacatctggcttagaaatagaacatcctgccagtgacaccaagttgctatagttctctaatatcacatctctgtacaaattcctctgatatgagttcaggcattcccattcttcctgagaaaagtctacagccacatctctgaacatcaccaaatcacgagccatgattttagaactgctagaactggtcaattttcctcaaggttcatgtacttcagaagcagggtccacagacaccagagagggaaccggcttttagaagagcagcagcgattcgtttctccttctcaagcgccttctctggaaactggcagggcccaaatctaggtcccagcgttttgcaggggaccttcatcctggggcgttcacctctgacttccctcttgggccttttcgctacggccgagcctaagtggctgaagcgcggacgaggatgcgcggggcctcggtctccaactgcaccacaggccgcacccacgaacctggtccggcacagttactaccgcccgggcctccaggcctcagggctgcagaagctcagtcccgggaaaaaaagcacaccggcctgaggctccacaggaaccttttctccaccttggcccggcctgcaaaacctggcccactccgcgctcttttccctcagaaaagcagcggccacagtggcgcccggctcccagccccagcctcacccgactcagaggatagcccagccctgggagtcagcggcgccagaat

SEQ ID NO: 14492 - RNA, 3590 nt, Homo sapiens
  source 1..3590: mol_type = other RNA
gctgggattacaggcatgagccaccgggcccagccagaaattttttttaaaataattcattttaaactggctataatttcatggataatttgatctttaaaagaacatcatggaaaattttaaatacacaaaagtagaatagcaaaaacaaaacaaataaaaaccatgtatccaagacttaggttaccatcattttgccaaacttgttattcatcctcatttttcttttgtatgaacaaaaggacattccagatatatcatctcctgtgtatagacttcagaaattatctctaacaaatacacttttacataaccacaatgctattatcacacataacaaagtttcttaatattatctaatattgtcaatattccattctcccaattattgttaagtatctcttcttttacatgtttgttcaactcatgatctaagtaaaaaccactgtttcattgcatttgactgatgtctcaagtctgtcaatacctaggagttccaccttatttcttaaaatgccattttattggttgggaaaccaggtgattcctcttgtagaattacccttattttagatttaattgctcctttttgtgtcatgtaatttactcttccattccttgaattttctctaaactgggagttggctcttgaggcttaaattcaggttcaatatttttggcaagatgtgtatatcttactgtagcacattaggaggcacgtaatttttactctcttgctttttgtgaagttgagatgatgagtgggttcagacgttgtcagtctcatctattcactataaagttcacaaccttcactgaatggtgtcaacctgtacagagaatcatgcctagatccattatttcattatgtgttacacaatagtttttctaatataattttctattattctttctgcattcattagcctggaattttctaataaagaagaactttacctccttaacttctggttgccctgaaatacagttcctacaggaaatgcagactaaatgactttcctttcatttacacattttcagaatgaagtggttccctagcaaccttcgtgtgtatatacacagatggaagaatatggagataataataggtaagatcaaaagcttttccacattcagtcctgtaataaagttcttttctaggatgaatttcctaaagtttaacatggtttcaaaggtgatgaaaggcttctatatgttcattaacatattctttcctttaaataaaacttcctatgcttagttgtgagcatgaagcaaaagggattcccacgttcaaaaacctttcctctagaatgtacttcctatgctcaacataaaattcgcaaaggaagagttctaataattattaagttacattatgaattcgctgatggtaagtaagatgtgaatgttgtctaaatgcctttttacattccttacatttgtatggtttctcaccagaatgaattctctgatgttgaatcagtgatgaatgaagtctaaaggcctttccacattccttacagtcatagggcttttcaccagtatgaatactttgatgttgggtaagttgtgaaagcagtctaaaagtcttctcacattccttacacttaaagggtttctcaccaaaatgaatactctgatgttgagtaagctgtgagaacagcctaaatgccttcccacattccttacattcataaggtttctctccaatgtgaataccctgatgtgaaataagttctgagtaacgacgaaagaacttctgacattccttacattcatagggcttttcaccagtatgtattctctgatggagagttagatgatagccacgactgaaagtcttcccacattccttacaatcataaggcttctcaccagtgtgaattctctgatggagagtaagttgctgccgcactctaaaggcctttccacactccttacattcatagggtttttctccagtatgaagtttgtgatgtagtcgaaggcctgtactacacagaaaggcctgaccacattccttacactcatagcacttctcagcaatgttcagtctctgatgtcgagtaaggtgtgcatactgcctaaaggccttcccacattctttacattcatagggtttctcacccgtgtgaatcctttgatggagattaagttgtcctctaactctaaaggctttcccacattctttacattcatacggcttctcaccaatatgaattctctgatgtactcgaaggtctgagccacatgtgaagatctttccacattttttacattcatagagtttgtcagaagtatgaattctctgatgtcgactgaggtgggcacactgtctaaaggcttttccacattctttacattcatagggtttctcaccagtatgaattctttgatggaaagtaagttgttgtcgtactctaaaagccttcccacattccccacattcgtagggtttctctctgttatgacttttctgatacagaggaagagatgtgagttttctgtaagtaggcattttttcagaggtggtttttgtcacttgcctgaaacacacctcatgaggactttcttgttcttcaagtccacagcttttaattctttccattaccttccactgagataagttcatttcataaatatcctttccttgaaataactttttagtgtcatatctggattccaaatctagagtccatcttcttttctcatccctcacaaccatccagggctctttcccttgttccaatagggtgatcacatctggcttagaaatagaacatcctgccagtgacaccaagttgctatagttctctaatatcacatctctgtacaaattcctctgatatgagttcaggcattcccattcttcctgagaaaagtctacagccacatctctgaacatcaccaaatcacgagccatgattttagaactgctagaactggtcaattttcctcaaggttcatgtacttcagaagcagggtccacagacaccagagagggaaccggcttttagaagagcagcagcgattcgtttctccttctcaagcgccttctctggaaactggcagggctggggaagcaggcagagttcaggacaccccaggcttttcttgactcgattggaacccaccctccacgcttccctggccccaactaaccgccaccccaaatctaggtcccagcgttttgcaggggaccttcatcctggggcgttcacctctgacttccctcttgggccttttcgctacggccgagcctaagtggctgaagcgcggacgaggatgcgcggggcctcggtctccaactgcaccacaggccgcacccacgaacctggtccggcacagttactaccgcccgggcctccaggcctcagggctgcagaagctcagtcccgggaaaaaaagcacaccggcctgaggctccacaggaaccttttctccaccttggcccggcctgcaaaacctggcccactccgcgctcttttccctcagaaaagcagcggccacagtggcgcccggctcccagccccagcctcacccgactcagaggatagcccagccctgggagtcagcggcgccagaat

SEQ ID NO: 14493 - RNA, 3217 nt, Homo sapiens
  source 1..3217: mol_type = other RNA
gctgggattacaggcatgagccaccgggcccagccagaaattttttttaaaataattcattttaaactggctataatttcatggataatttgatctttaaaagaacatcatggaaaattttaaatacacaaaagtagaatagcaaaaacaaaacaaataaaaaccatgtatccaagacttaggttaccatcattttgccaaacttgttattcatcctcatttttcttttgtatgaacaaaaggacattccagatatatcatctcctgtgtatagacttcagaaattatctctaacaaatacacttttacataaccacaatgctattatcacacataacaaagtttcttaatattatctaatattgtcaatattccattctcccaattattgttaagtatctcttcttttacatgtttgttcaactcatgatctaagtaaaaaccactgtttcattgcatttgactgatgtctcaagtctgtcaatacctaggagttccaccttatttcttaaaatgccattttattggttgggaaaccaggtgattcctcttgtagaattacccttattttagatttaattgctcctttttgtgtcatgtaatttactcttccattccttgaattttctctaaactgggagttggctcttgaggcttaaattcaggttcaatatttttggcaagatgtgtatatcttactgtagcacattaggaggcacgtaatttttactctcttgctttttgtgaagttgagatgatgagtgggttcagacgttgtcagtctcatctattcactataaagttcacaaccttcactgaatggtgtcaacctgtacagagaatcatgcctagatccattatttcattatgtgttacacaatagtttttctaatataattttctattattctttctgcattcattagcctggaattttctaataaagaagaactttacctccttaacttctggttgccctgaaatacagttcctacaggaaatgcagactaaatgactttcctttcatttacacattttcagaatgaagtggttccctagcaaccttcgtgtgtatatacacagatggaagaatatggagataataataggtaagatcaaaagcttttccacattcagtcctgtaataaagttcttttctaggatgaatttcctaaagtttaacatggtttcaaaggtgatgaaaggcttctatatgttcattaacatattctttcctttaaataaaacttcctatgcttagttgtgagcatgaagcaaaagggattcccacgttcaaaaacctttcctctagaatgtacttcctatgctcaacataaaattcgcaaaggaagagttctaataattattaagttacattatgaattcgctgatggtaagtaagatgtgaatgttgtctaaatgcctttttacattccttacatttgtatggtttctcaccagaatgaattctctgatgttgaatcagtgatgaatgaagtctaaaggcctttccacattccttacagtcatagggcttttcaccagtatgaatactttgatgttgggtaagttgtgaaagcagtctaaaagtcttctcacattccttacacttaaagggtttctcaccaaaatgaatactctgatgttgagtaagctgtgagaacagcctaaatgccttcccacattccttacattcataaggtttctctccaatgtgaataccctgatgtgaaataagttctgagtaacgacgaaagaacttctgacattccttacattcatagggcttttcaccagtatgtattctctgatggagagttagatgatagccacgactgaaagtcttcccacattccttacaatcataaggcttctcaccagtgtgaattctctgatggagagtaagttgctgccgcactctaaaggcctttccacactccttacattcatagggtttttctccagtatgaagtttgtgatgtagtcgaaggcctgtactacacagaaaggcctgaccacattccttacactcatagcacttctcagcaatgttcagtctctgatgtcgagtaaggtgtgcatactgcctaaaggccttcccacattctttacattcatagggtttctcacccgtgtgaatcctttgatggagattaagttgtcctctaactctaaaggctttcccacattctttacattcatacggcttctcaccaatatgaattctctgatgtactcgaaggtctgagccacatgtgaagatctttccacattttttacattcatagagtttgtcagaagtatgaattctctgatgtcgactgaggtgggcacactgtctaaaggcttttccacattctttacattcatagggtttctcaccagtatgaattctttgatggaaagtaagttgttgtcgtactctaaaagccttcccacattccccacattcgtagggtttctctctgttatgacttttctgatacagaggaagagatgtgagttttctgtaagtaggcattttttcagaggtggtttttgtcacttgcctgaaacacacctcatgaggactttcttgttcttcaagtccacagcttttaattctttccattaccttccactgagataagttcatttcataaatatcctttccttgaaataactttttagtgtcatatctggattccaaatctagagtccatcttcttttctcatccctcacaaccatccagggctctttcccttgttccaatagggtgatcacatctggcttagaaatagaacatcctgccagtgacaccaagttgctatagttctctaatatcacatctctgtacaaattcctctgatatgagttcaggcattcccattcttcctgagaaaagtctacagccacatctctgaacatcaccaaatcacgagccatgattttagaactgctagaactggtcaattttcctcaaggttcatgtacttcagaagcagggtccacagacaccagagagggaaccggcttttagaagagcagcagcgattcgtttctccttctcaagcgccttctctggaaactggcagggctggggaagcaggcagagttcaggacaccccaggcttttcttgactcgattggaacccaccctccacgcttccctggccccaactaaccgccacccgactcagaggatagcccagccctgggagtcagcggcgccagaat

SEQ ID NO: 14494 - RNA, 3537 nt, Homo sapiens
  source 1..3537: mol_type = other RNA
gctgggattacaggcatgagccaccgggcccagccagaaattttttttaaaataattcattttaaactggctataatttcatggataatttgatctttaaaagaacatcatggaaaattttaaatacacaaaagtagaatagcaaaaacaaaacaaataaaaaccatgtatccaagacttaggttaccatcattttgccaaacttgttattcatcctcatttttcttttgtatgaacaaaaggacattccagatatatcatctcctgtgtatagacttcagaaattatctctaacaaatacacttttacataaccacaatgctattatcacacataacaaagtttcttaatattatctaatattgtcaatattccattctcccaattattgttaagtatctcttcttttacatgtttgttcaactcatgatctaagtaaaaaccactgtttcattgcatttgactgatgtctcaagtctgtcaatacctaggagttccaccttatttcttaaaatgccattttattggttgggaaaccaggtgattcctcttgtagaattacccttattttagatttaattgctcctttttgtgtcatgtaatttactcttccattccttgaattttctctaaactgggagttggctcttgaggcttaaattcaggttcaatatttttggcaagatgtgtatatcttactgtagcacattaggaggcacgtaatttttactctcttgctttttgtgaagttgagatgatgagtgggttcagacgttgtcagtctcatctattcactataaagttcacaaccttcactgaatggtgtcaacctgtacagagaatcatgcctagatccattatttcattatgtgttacacaatagtttttctaatataattttctattattctttctgcattcattagcctggaattttctaataaagaagaactttacctccttaacttctggttgccctgaaatacagttcctacaggaaatgcagactaaatgactttcctttcatttacacattttcagaatgaagtggttccctagcaaccttcgtgtgtatatacacagatggaagaatatggagataataataggtaagatcaaaagcttttccacattcagtcctgtaataaagttcttttctaggatgaatttcctaaagtttaacatggtttcaaaggtgatgaaaggcttctatatgttcattaacatattctttcctttaaataaaacttcctatgcttagttgtgagcatgaagcaaaagggattcccacgttcaaaaacctttcctctagaatgtacttcctatgctcaacataaaattcgcaaaggaagagttctaataattattaagttacattatgaattcgctgatggtaagtaagatgtgaatgttgtctaaatgcctttttacattccttacatttgtatggtttctcaccagaatgaattctctgatgttgaatcagtgatgaatgaagtctaaaggcctttccacattccttacagtcatagggcttttcaccagtatgaatactttgatgttgggtaagttgtgaaagcagtctaaaagtcttctcacattccttacacttaaagggtttctcaccaaaatgaatactctgatgttgagtaagctgtgagaacagcctaaatgccttcccacattccttacattcataaggtttctctccaatgtgaataccctgatgtgaaataagttctgagtaacgacgaaagaacttctgacattccttacattcatagggcttttcaccagtatgtattctctgatggagagttagatgatagccacgactgaaagtcttcccacattccttacaatcataaggcttctcaccagtgtgaattctctgatggagagtaagttgctgccgcactctaaaggcctttccacactccttacattcatagggtttttctccagtatgaagtttgtgatgtagtcgaaggcctgtactacacagaaaggcctgaccacattccttacactcatagcacttctcagcaatgttcagtctctgatgtcgagtaaggtgtgcatactgcctaaaggccttcccacattctttacattcatagggtttctcacccgtgtgaatcctttgatggagattaagttgtcctctaactctaaaggctttcccacattctttacattcatacggcttctcaccaatatgaattctctgatgtactcgaaggtctgagccacatgtgaagatctttccacattttttacattcatagagtttgtcagaagtatgaattctctgatgtcgactgaggtgggcacactgtctaaaggcttttccacattctttacattcatagggtttctcaccagtatgaattctttgatggaaagtaagttgttgtcgtactctaaaagccttcccacattccccacattcgtagggtttctctctgttatgacttttctgatacagaggaagagatgtgagttttctgtaagtaggcattttttcagaggtggtttttgtcacttgcctgaaacacacctcatgaggactttcttgttcttcaagtccacagcttttaattctttccattaccttccactgagataagttcatttcataaatatcctttccttgaaataactttttagtgtcatatctggattccaaatctagagtccatcttcttttctcatccctcacaaccatccagggctctttcccttgttccaatagggtgatcacatctggcttagaaatagaacatcctgccagtgacaccaagttgctatagttctctaatatcacatctctgtacaaattcctctgatatgagttcaggcattcccattcttcctgagaaaagtctacagccacatctctgaacatcaccaaatcacgagccatgattttagaactgctagaactggtcaattttcctcaaggttcatgtacttcagaagcagggtccacagacaccagagagggaaccggcttttagaagagcagcagcgattcgtttctccttctcaagcgccttctctggaaactggcagggctggggaagcaggcagagttcaggacaccccaggcttttcttgactcgattggaacccaccctccacgcttccctggccccaactaaccgccacctctgacttccctcttgggccttttcgctacggccgagcctaagtggctgaagcgcggacgaggatgcgcggggcctcggtctccaactgcaccacaggccgcacccacgaacctggtccggcacagttactaccgcccgggcctccaggcctcagggctgcagaagctcagtcccgggaaaaaaagcacaccggcctgaggctccacaggaaccttttctccaccttggcccggcctgcaaaacctggcccactccgcgctcttttccctcagaaaagcagcggccacagtggcgcccggctcccagccccagcctcacccgactcagaggatagcccagccctgggagtcagcggcgccagaat

SEQ ID NO: 14495 - RNA, 3313 nt, Homo sapiens
  source 1..3313: mol_type = other RNA
gctgggattacaggcatgagccaccgggcccagccagaaattttttttaaaataattcattttaaactggctataatttcatggataatttgatctttaaaagaacatcatggaaaattttaaatacacaaaagtagaatagcaaaaacaaaacaaataaaaaccatgtatccaagacttaggttaccatcattttgccaaacttgttattcatcctcatttttcttttgtatgaacaaaaggacattccagatatatcatctcctgtgtatagacttcagaaattatctctaacaaatacacttttacataaccacaatgctattatcacacataacaaagtttcttaatattatctaatattgtcaatattccattctcccaattattgttaagtatctcttcttttacatgtttgttcaactcatgatctaagtaaaaaccactgtttcattgcatttgactgatgtctcaagtctgtcaatacctaggagttccaccttatttcttaaaatgccattttattggttgggaaaccaggtgattcctcttgtagaattacccttattttagatttaattgctcctttttgtgtcatgtaatttactcttccattccttgaattttctctaaactgggagttggctcttgaggcttaaattcaggttcaatatttttggcaagatgtgtatatcttactgtagcacattaggaggcacgtaatttttactctcttgctttttgtgaagttgagatgatgagtgggttcagacgttgtcagtctcatctattcactataaagttcacaaccttcactgaatggtgtcaacctgtacagagaatcatgcctagatccattatttcattatgtgttacacaatagtttttctaatataattttctattattctttctgcattcattagcctggaattttctaataaagaagaactttacctccttaacttctggttgccctgaaatacagttcctacaggaaatgcagactaaatgactttcctttcatttacacattttcagaatgaagtggttccctagcaaccttcgtgtgtatatacacagatggaagaatatggagataataataggtaagatcaaaagcttttccacattcagtcctgtaataaagttcttttctaggatgaatttcctaaagtttaacatggtttcaaaggtgatgaaaggcttctatatgttcattaacatattctttcctttaaataaaacttcctatgcttagttgtgagcatgaagcaaaagggattcccacgttcaaaaacctttcctctagaatgtacttcctatgctcaacataaaattcgcaaaggaagagttctaataattattaagttacattatgaattcgctgatggtaagtaagatgtgaatgttgtctaaatgcctttttacattccttacatttgtatggtttctcaccagaatgaattctctgatgttgaatcagtgatgaatgaagtctaaaggcctttccacattccttacagtcatagggcttttcaccagtatgaatactttgatgttgggtaagttgtgaaagcagtctaaaagtcttctcacattccttacacttaaagggtttctcaccaaaatgaatactctgatgttgagtaagctgtgagaacagcctaaatgccttcccacattccttacattcataaggtttctctccaatgtgaataccctgatgtgaaataagttctgagtaacgacgaaagaacttctgacattccttacattcatagggcttttcaccagtatgtattctctgatggagagttagatgatagccacgactgaaagtcttcccacattccttacaatcataaggcttctcaccagtgtgaattctctgatggagagtaagttgctgccgcactctaaaggcctttccacactccttacattcatagggtttttctccagtatgaagtttgtgatgtagtcgaaggcctgtactacacagaaaggcctgaccacattccttacactcatagcacttctcagcaatgttcagtctctgatgtcgagtaaggtgtgcatactgcctaaaggccttcccacattctttacattcatagggtttctcacccgtgtgaatcctttgatggagattaagttgtcctctaactctaaaggctttcccacattctttacattcatacggcttctcaccaatatgaattctctgatgtactcgaaggtctgagccacatgtgaagatctttccacattttttacattcatagagtttgtcagaagtatgaattctctgatgtcgactgaggtgggcacactgtctaaaggcttttccacattctttacattcatagggtttctcaccagtatgaattctttgatggaaagtaagttgttgtcgtactctaaaagccttcccacattccccacattcgtagggtttctctctgttatgacttttctgatacagaggaagagatgtgagttttctgtaagtaggcattttttcagaggtggtttttgtcacttgcctgaaacacacctcatgaggactttcttgttcttcaagtccacagcttttaattctttccattaccttccactgagataagttcatttcataaatatcctttccttgaaataactttttagtgtcatatctggattccaaatctagagtccatcttcttttctcatccctcacaaccatccagggctctttcccttgttccaatagggtgatcacatctggcttagaaatagaacatcctgccagtgacaccaagttgctatagttctctaatatcacatctctgtacaaattcctctgatatgagttcaggcattcccattcttcctgagaaaagtctacagccacatctctgaacatcaccaaatcacgagccatgattttagaactgctagaactggtcaattttcctcaaggttcatgtacttcagaagcagggtccacagacaccagagagggaaccggcttttagaagagcagcagcgattcgtttctccttctcaagcgccttctctggaaactggcagggctggggaagcaggcagagttcaggacaccccaggcttttcttgactcgattggaacccaccctccacgcttccctggccccaactaaccgccacctggaccgagtgcctggccgctggcggagtagtgtttccgtgcacggggctgctgcgtgcgcgtgtgccgttctctagcgggggattaggatggtgccgcagagaaggctgcgcggtggtgcctgactctgacgctggctgt

SEQ ID NO: 14496 - RNA, 1300 nt, Homo sapiens
  source 1..1300: mol_type = other RNA
gctgggattacaggcatgagccaccgggcccagcctacttcttgaattaaaaaacaaaaaacaaacaaaaaacccaggcagataatgaaatcctgcatacactcaagtctgcatgaagcataaggccaaactggaaagtgggcatttgaacaaccctcttcctgctcccttcccctaactaagatgggcttctgggcctatcaaccattctttggtaaagagcagcaattccccataggctctttaacaacagcattggtgtttgaggttgcatctttaaaacatctatttcaggatttggaagcttctggaaccataactttaacccagccttccataacagtctttttactttctattacagaacatgacactgcaataatagcaatgaaccgcttcagctttttcacttctgcagaagctaaaacaacttctccaatatataaaggggctggaaagctaatttcctgggaaagaaatacacagcctggccctggcattttagttcctaggagagctgagataagtccgttgatcaaaactccatgtacaattgtatttccaaacttggtgtgttttgcaaagtcttcattcaaatgcaaaggattgacatcccctgttaattctgagaaggtagccacatcagtctgtgtgaaggccctcctaagttcagcgcggtctccaactttgatgtgcatatgctgaaagtgctgcagggtcagcactggcaggttcagacagactgtcctccgaagcccaccccaccaaaggtgatggctggaaattagtgggaacatcttcagcaccctcaaatttcatcaagagcttttagcctgcttcagtcttcaaacatgcaggcaccaaaaaataaatatgagagtggatgaacgtttccaaaatggaagactattcattcaatccaatactagttccctactattaccagataatgcaagaagaaatggagaaacctgaatcacccggaaagcacattttttgcctttataggatcctaacagggtcaaagagctccacaatttgacaagaccactgctacatattctcaagatggctgacaaggtcttctcttcataggttaggatgtccaaaggtaaggcggcatcaacccactcttcgtcggactagcctgacgcctgaccagactcctattcgccgcaaggacccgccaaggcttggggctccccggcagcagccacagctgggcccgagaaactcctggtgtctttacgtttggcttctcctcgtcccgccccacgaagcgtgacgcccaggcggatat

SEQ ID NO: 14497 - RNA, 1483 nt, Homo sapiens
  source 1..1483: mol_type = other RNA
gctgggattacaggcatgagccaccgggcccagcctacttcttgaattaaaaaacaaaaaacaaacaaaaaacccaggcagataatgaaatcctgcatacactcaagtctgcatgaagcataaggccaaactggaaagtgggcatttgaacaaccctcttcctgctcccttcccctaactaagatgggcttctgggcctatcaaccattctttggtaaagagcagcaattccccataggctctttaacaacagcattggtgtttgaggttgcatctttaaaacatctatttcaggatttggaagcttctggaaccataactttaacccagccttccataacagtctttttactttctattacagaacatgacactgcaataatagcaatgaaccgcttcagctttttcacttctgcagaagctaaaacaacttctccaatatataaaggggctggaaagctaatttcctgggaaagaaatacacagcctggccctggcattttagttcctaggagagctgagataagtccgttgatcaaaactccatgtacaattgtatttccaaacttggtgtgttttgcaaagtcttcattcaaatgcaaaggattgacatcccctgttaattctgagaaggtagccacatcagtctgtgtgaaggccctcctaagttcagcgcggtctccaactttgatgtgcatatgctgaaagtgctgcagggtcagcactggcaggttcagacagactgtcctccgaagcccaccccaccaaaggtgatggctggaaattagtgggaacatcttcagcaccctcaaatttcatcaagagcttttagcctgcttcagtcttcaaacatgcaggcaccaaaaaataaatatgagagtggatgaacgtttccaaaatggaagactattcattcaatccaatactagttccctactattaccagataatgcaagaagaaatggagaaacctgaatcacccggaaagcacattttttgcctttataggatcctaacagggtcaaagagctccacaatttgacaagaccactgctacatattctcaagatggctgacaaggtcttctcttcataggttaggatgtccaaaggtaaggcggcatcaacctccccaaacaggtccttcacagccgaaataagcagctgtttgaactgtgcagcattcagtccaactccacaatcttgaaattctaggcagactttcatgtagtggtactcggaagggtttttgtaaactactctttcatatgtggcagcaggggcaggcatcttttccagtgctgatcacacccactcttcgtcggactagcctgacgcctgaccagactcctattcgccgcaaggacccgccaaggcttggggctccccggcagcagccacagctgggcccgagaaactcctggtgtctttacgtttggcttctcctcgtcccgccccacgaagcgtgacgcccaggcggatat

SEQ ID NO: 14498 - RNA, 1442 nt, Homo sapiens
  source 1..1442: mol_type = other RNA
gctgggattacaggcatgagccaccgggcccagcctacttcttgaattaaaaaacaaaaaacaaacaaaaaacccaggcagataatgaaatcctgcatacactcaagtctgcatgaagcataaggccaaactggaaagtgggcatttgaacaaccctcttcctgctcccttcccctaactaagatgggcttctgggcctatcaaccattctttggtaaagagcagcaattccccataggctctttaacaacagcattggtgtttgaggttgcatctttaaaacatctatttcaggatttggaagcttctggaaccataactttaacccagccttccataacagtctttttactttctattacagaacatgacactgcaataatagcaatgaaccgcttcagctttttcacttctgcagaagctaaaacaacttctccaatatataaaggggctggaaagctaatttcctgggaaagaaatacacagcctggccctggcattttagttcctaggagagctgagataagtccgttgatcaaaactccatgtacaattgtatttccaaacttggtgtgttttgcaaagtcttcattcaaatgcaaaggattgacatcccctgttaattctgagaaggtagccacatcagtctgtgtgaaggccctcctaagttcagcgcggtctccaactttgatgtgcatatgctgaaagtgctgcagggtcagcactggcaggttcagacagactgtcctccgaagcccaccccaccaaaggtgatggctggaaattagtgggaacatcttcagcaccctcaaatttcatcaagagcttttagcctgcttcagtcttcaaacatgcaggcaccaaaaaataaatatgagagtggatgaacgtttccaaaatggaagactattcattcaatccaatactagttccctactattaccagataatgcaagaagaaatggagaaacctgaatcacccggaaagcacattttttgcctttataggatcctaacagggtcaaagagctccacaatttgacaagaccactgctacatattctcaagatggctgacaaggtcttctcttcataggttaggatgtccaaaggtaaggcggcatcaacctccccaaacaggtccttcacagccgaaataagcagctgtttgaactgtgcagcattcagtccaactccacaatcttgaaattctaggcagactttcatgtagtggtactcggaagggtttttgtaaactactctttcatatgtggcagcaggggcaggcatcttttccagtgctgatcacacctcgcgccgggcgcatggagagcgctcaggacacggtcccgaagtctcgcccgggcctctcggccacgttctgcggccgagaccctacgcggcgccgtacagaggccctcagcgcccggggtcggagaggac

SEQ ID NO: 14499 - RNA, 1385 nt, Homo sapiens
  source 1..1385: mol_type = other RNA
gctgggattacaggcatgagccaccgggcccagcctacttcttgaattaaaaaacaaaaaacaaacaaaaaacccaggcagataatgaaatcctgcatacactcaagtctgcatgaagcataaggccaaactggaaagtgggcatttgaacaaccctcttcctgctcccttcccctaactaagatgggcttctgggcctatcaaccattctttggtaaagagcagcaattccccataggctctttaacaacagcattggtgtttgaggttgcatctttaaaacatctatttcaggatttggaagcttctggaaccataactttaacccagccttccataacagtctttttactttctattacagaacatgacactgcaataatagcaatgaaccgcttcagctttttcacttctgcagaagctaaaacaacttctccaatatataaaggggctggaaagctaatttcctgggaaagaaatacacagcctggccctggcattttagttcctaggagagctgagataagtccgttgatcaaaactccatgtacaattgtatttccaaacttggtgtgttttgcaaagtcttcattcaaatgcaaaggattgacatcccctgttaattctgagaaggtagccacatcagtctgtgtgaaggccctcctaagttcagcgcggtctccaactttgatgtgcatatgctgaaagtgctgcagggtcagcactggcaggttcagacagactgtcctccgaagcccaccccaccaaaggtgatggctggaaattagtgggaacatcttcagcaccctcaaatttcatcaagagcttttagcctgcttcagtcttcaaacatgcaggcaccaaaaaataaatatgagagtggatgaacgtttccaaaatggaagactattcattcaatccaatactagttccctactattaccagataatgcaagaagaaatggagaaacctgaatcacccggaaagcacattttttgcctttataggatcctaacagggtcaaagagctccacaatttgacaagaccactgctacatattctcaagatggctgacaaggtcttctcttcataggttaggatgtccaaaggtaaggcggcatcaacctccccaaacaggtccttcacagccgaaataagcagctgtttgaactgtgcagcattcagtccaactccacaatcttgaaattctccactcttcgtcggactagcctgacgcctgaccagactcctattcgccgcaaggacccgccaaggcttggggctccccggcagcagccacagctgggcccgagaaactcctggtgtctttacgtttggcttctcctcgtcccgccccacgaagcgtgacgcccaggcggatat

SEQ ID NO: 14500 - RNA, 1344 nt, Homo sapiens
  source 1..1344: mol_type = other RNA
gctgggattacaggcatgagccaccgggcccagcctacttcttgaattaaaaaacaaaaaacaaacaaaaaacccaggcagataatgaaatcctgcatacactcaagtctgcatgaagcataaggccaaactggaaagtgggcatttgaacaaccctcttcctgctcccttcccctaactaagatgggcttctgggcctatcaaccattctttggtaaagagcagcaattccccataggctctttaacaacagcattggtgtttgaggttgcatctttaaaacatctatttcaggatttggaagcttctggaaccataactttaacccagccttccataacagtctttttactttctattacagaacatgacactgcaataatagcaatgaaccgcttcagctttttcacttctgcagaagctaaaacaacttctccaatatataaaggggctggaaagctaatttcctgggaaagaaatacacagcctggccctggcattttagttcctaggagagctgagataagtccgttgatcaaaactccatgtacaattgtatttccaaacttggtgtgttttgcaaagtcttcattcaaatgcaaaggattgacatcccctgttaattctgagaaggtagccacatcagtctgtgtgaaggccctcctaagttcagcgcggtctccaactttgatgtgcatatgctgaaagtgctgcagggtcagcactggcaggttcagacagactgtcctccgaagcccaccccaccaaaggtgatggctggaaattagtgggaacatcttcagcaccctcaaatttcatcaagagcttttagcctgcttcagtcttcaaacatgcaggcaccaaaaaataaatatgagagtggatgaacgtttccaaaatggaagactattcattcaatccaatactagttccctactattaccagataatgcaagaagaaatggagaaacctgaatcacccggaaagcacattttttgcctttataggatcctaacagggtcaaagagctccacaatttgacaagaccactgctacatattctcaagatggctgacaaggtcttctcttcataggttaggatgtccaaaggtaaggcggcatcaacctccccaaacaggtccttcacagccgaaataagcagctgtttgaactgtgcagcattcagtccaactccacaatcttgaaattctctcgcgccgggcgcatggagagcgctcaggacacggtcccgaagtctcgcccgggcctctcggccacgttctgcggccgagaccctacgcggcgccgtacagaggccctcagcgcccggggtcggagaggac

SEQ ID NO: 14501 - RNA, 1483 nt, Homo sapiens
  source 1..1483: mol_type = other RNA
gctgggattacaggcatgagccaccgggcccagcctacttcttgaattaaaaaacaaaaaacaaacaaaaaacccaggcagataatgaaatcctgcatacactcaagtctgcatgaagcataaggccaaactggaaagtgggcatttgaacaaccctcttcctgctcccttcccctaactaagatgggcttctgggcctatcaaccattctttggtaaagagcagcaattccccataggctctttaacaacagcattggtgtttgaggttgcatctttaaaacatctatttcaggatttggaagcttctggaaccataactttaacccagccttccataacagtctttttactttctattacagaacatgacactgcaataatagcaatgaaccgcttcagctttttcacttctgcagaagctaaaacaacttctccaatatataaaggggctggaaagctaatttcctgggaaagaaatacacagcctggccctggcattttagttcctaggagagctgagataagtccgttgatcaaaactccatgtacaattgtatttccaaacttggtgtgttttgcaaagtcttcattcaaatgcaaaggattgacatcccctgttaattctgagaaggtagccacatcagtctgtgtgaaggccctcctaagttcagcgcggtctccaactttgatgtgcatatgctgaaagtgctgcagggtcagcactggcaggttcagacagactgtcctccgaagcccaccccaccaaaggtgatggctggaaattagtgggaacatcttcagcaccctcaaatttcatcaagagcttttagcctgcttcagtcttcaaacatgcaggcaccaaaaaataaatatgagagtggatgaacgtttccaaaatggaagactattcattcaatccaatactagttccctactattaccagataatgcaagaagaaatggagaaacctgaatcacccggaaagcacattttttgcctttataggatcctaacagggtcaaagagctccacaatttgacaagaccactgctacatattctcaagatggctgacaaggtcttctcttcataggttaggatgtccaaaggtaaggcggcatcaacctgtaatcccagctacttgcgaggctgaggcaggagaatcgcttgaacctgggaggcggagggtgcggtgagccaagatcgtgccattgcactccagcctccccaaacaggtccttcacagccgaaataagcagctgtttgaactgtgcagcattcagtccaactccacaatcttgaaattctccactcttcgtcggactagcctgacgcctgaccagactcctattcgccgcaaggacccgccaaggcttggggctccccggcagcagccacagctgggcccgagaaactcctggtgtctttacgtttggcttctcctcgtcccgccccacgaagcgtgacgcccaggcggatat

SEQ ID NO: 14502 - RNA, 1730 nt, Homo sapiens
  source 1..1730: mol_type = other RNA
gctgggattacaggcatgagccaccgggctcagccatattaagccagtctcaaataagctggagacttaagtttatagaccctataatgacaactttgttccacctctgagataaagacaatactaaacccatctccagtgcttctttccccatgcataaggaatgatgctgtcatattttttcaaaaaattttttggctgcttaatagaaaagctgaatgagcttgatttcagtagaagacccactgattatgggtatatttattgggacatattttaatagaagataattcatgtaggatatcttcaatgcattataatatgattttcactgtatctcttcacatgttattccataacattctaattggatggagaaagactggaatagttcaaaaaggtgtagcttttaagatctgaataaagttaatagtgagtcttttaaaatacatttaaacaactggaagtataatcacaacaagggactatgaaggaagaataaatattgcaaacgacgctttatagtcaatgcaaatacagtactttgaattacccaaaatgtataatgcacaagaactctaagtcatgtagtttacttgctgaccatctggctacagttcagtttcttctgcaaaagctgtacctagtaaccttccaaaattgtttttaaataaagttcttaaattgtagcaataaacaaaaggacaaagtacacttaaagaatactgcagtttatcaaaagacataagaaatttcaactcatacttggagagttataaaaatcaatgttttggctaagttataaacatgtttataatgcaattatttgcataactctagtaatgctaatggcggctataagattaggtttctaaaaaaccactaaaaacataaaaatacttagcctcattatttccctgtagaacgtattgatttacacctaaatttcagtatttactatatcatcattgctgattttaagtcacattcaaaggataaggcaaaaccacctacgaattggcatatttgtttatttctcagtttgtgaaaatgtccttaatttgttgatgtagcaaacaaatttcaactttgattgctatgcaaaaaaacaagataatctgctttgcaatgaactttatatagttcaactgcatacaggcaacatgctatatatgaaaaagttactaactgaactacaggtattaaatactgaaaagagttaacagtttattataatttattttatttaacaatctaagaagttcgcagccatcagcagttccagtgcaatttcaggtgcaattgggaattcaggaatctcggtggagctgttagtgtagcgaaccttgtacgtaaaatacatgcatactttcgatagcacatgtgaaggtatctctctaaaattgacctcattggtttcgttctcagcaaactgacctgggccactcaacatggcttttatcgtgcctgatgttaatgcatgttctctttttacaataaattcatggccatcagatgatatcaatttgacatacatggcatcaggtccttcacagccaccataggttttctcctctccatccattttgttcttatgaaattctactttgcttccccaggaactttagtagtttccacagctgtttccttgccattgtatctccagaatgaataaatccacatgtaaactgcgagcggcgccaggaaaggtcccgccgccctcttctccc

SEQ ID NO: 14503 - RNA, 1869 nt, Homo sapiens
  source 1..1869: mol_type = other RNA
gctgggattacaggcatgagccaccgggctcagccatattaagccagtctcaaataagctggagacttaagtttatagaccctataatgacaactttgttccacctctgagataaagacaatactaaacccatctccagtgcttctttccccatgcataaggaatgatgctgtcatattttttcaaaaaattttttggctgcttaatagaaaagctgaatgagcttgatttcagtagaagacccactgattatgggtatatttattgggacatattttaatagaagataattcatgtaggatatcttcaatgcattataatatgattttcactgtatctcttcacatgttattccataacattctaattggatggagaaagactggaatagttcaaaaaggtgtagcttttaagatctgaataaagttaatagtgagtcttttaaaatacatttaaacaactggaagtataatcacaacaagggactatgaaggaagaataaatattgcaaacgacgctttatagtcaatgcaaatacagtactttgaattacccaaaatgtataatgcacaagaactctaagtcatgtagtttacttgctgaccatctggctacagttcagtttcttctgcaaaagctgtacctagtaaccttccaaaattgtttttaaataaagttcttaaattgtagcaataaacaaaaggacaaagtacacttaaagaatactgcagtttatcaaaagacataagaaatttcaactcatacttggagagttataaaaatcaatgttttggctaagttataaacatgtttataatgcaattatttgcataactctagtaatgctaatggcggctataagattaggtttctaaaaaaccactaaaaacataaaaatacttagcctcattatttccctgtagaacgtattgatttacacctaaatttcagtatttactatatcatcattgctgattttaagtcacattcaaaggataaggcaaaaccacctacgaattggcatatttgtttatttctcagtttgtgaaaatgtccttaatttgttgatgtagcaaacaaatttcaactttgattgctatgcaaaaaaacaagataatctgctttgcaatgaactttatatagttcaactgcatacaggcaacatgctatatatgaaaaagttactaactgaactacaggtattaaatactgaaaagagttaacagtttattataatttattttatttaacaatctaagaagttcgcagccatcagcagttccagtgcaatttcaggtgcaattgggaattcaggaatctcggtggagctgttagtgtagcgaaccttgtacgtaaaatacatgcatactttcgatagcacatgtgaaggtatctctctaaaattgacctcattggtttcgttctcagcaaactgacctgggccactcaacatggcttttatcgtgcctgatgttaatgcatgttctctttttacaataaattcatggccatcagatgatatcaatttgacatacatggcatcaggtccttcacagccaccataggttttctcctctccatccattttgttcttatgaaattctactttgcttccccaggaactttagtagtttccctcactgtaggcaaagatttctcagcagccaggtgcagtggctcacacctgcaatcgcaacactttgggagggagatcacttgaggtcaggaatttgagaccagccgggcactccagcctgggccacacagcaagactcacagctgtttccttgccattgtatctccagaatgaataaatccacatgtaaactgcgagcggcgccaggaaaggtcccgccgccctcttctccc

SEQ ID NO: 14504 - RNA, 1817 nt, Homo sapiens
  source 1..1817: mol_type = other RNA
gctgggattacaggcatgagccaccgggctcagccatattaagccagtctcaaataagctggagacttaagtttatagaccctataatgacaactttgttccacctctgagataaagacaatactaaacccatctccagtgcttctttccccatgcataaggaatgatgctgtcatattttttcaaaaaattttttggctgcttaatagaaaagctgaatgagcttgatttcagtagaagacccactgattatgggtatatttattgggacatattttaatagaagataattcatgtaggatatcttcaatgcattataatatgattttcactgtatctcttcacatgttattccataacattctaattggatggagaaagactggaatagttcaaaaaggtgtagcttttaagatctgaataaagttaatagtgagtcttttaaaatacatttaaacaactggaagtataatcacaacaagggactatgaaggaagaataaatattgcaaacgacgctttatagtcaatgcaaatacagtactttgaattacccaaaatgtataatgcacaagaactctaagtcatgtagtttacttgctgaccatctggctacagttcagtttcttctgcaaaagctgtacctagtaaccttccaaaattgtttttaaataaagttcttaaattgtagcaataaacaaaaggacaaagtacacttaaagaatactgcagtttatcaaaagacataagaaatttcaactcatacttggagagttataaaaatcaatgttttggctaagttataaacatgtttataatgcaattatttgcataactctagtaatgctaatggcggctataagattaggtttctaaaaaaccactaaaaacataaaaatacttagcctcattatttccctgtagaacgtattgatttacacctaaatttcagtatttactatatcatcattgctgattttaagtcacattcaaaggataaggcaaaaccacctacgaattggcatatttgtttatttctcagtttgtgaaaatgtccttaatttgttgatgtagcaaacaaatttcaactttgattgctatgcaaaaaaacaagataatctgctttgcaatgaactttatatagttcaactgcatacaggcaacatgctatatatgaaaaagttactaactgaactacaggtattaaatactgaaaagagttaacagtttattataatttattttatttaacaatctaagaagttcgcagccatcagcagttccagtgcaatttcaggtgcaattgggaattcaggaatctcggtggagctgttagtgtagcgaaccttgtacgtaaaatacatgcatactttcgatagcacatgtgaaggtatctctctaaaattgacctcattggtttcgttctcagcaaactgacctgggccactcaacatggcttttatcgtgcctgatgttaatgcatgttctctttttacaataaattcatggccatcagatgatatcaatttgacatacatggcatcaggtccttcacagccaccataggttttctcctctccatccattttgttcttatgaaattctactttgcttccccaggaactttagtagtttccctcactgtaggcaaagatttctcagcagccaggtgcagtggctcacacctgcaatcgcaacactttgggagggagatcacttgaggtcaggaatttgagaccagccgggcactccagcctgggccacacagcaagactctggtgaggcgaggacgcagagtgtgtcgctcacttccgtctg

SEQ ID NO: 14505 - RNA, 1893 nt, Homo sapiens
  source 1..1893: mol_type = other RNA
gctgggattacaggcatgagccaccgggctcagccatattaagccagtctcaaataagctggagacttaagtttatagaccctataatgacaactttgttccacctctgagataaagacaatactaaacccatctccagtgcttctttccccatgcataaggaatgatgctgtcatattttttcaaaaaattttttggctgcttaatagaaaagctgaatgagcttgatttcagtagaagacccactgattatgggtatatttattgggacatattttaatagaagataattcatgtaggatatcttcaatgcattataatatgattttcactgtatctcttcacatgttattccataacattctaattggatggagaaagactggaatagttcaaaaaggtgtagcttttaagatctgaataaagttaatagtgagtcttttaaaatacatttaaacaactggaagtataatcacaacaagggactatgaaggaagaataaatattgcaaacgacgctttatagtcaatgcaaatacagtactttgaattacccaaaatgtataatgcacaagaactctaagtcatgtagtttacttgctgaccatctggctacagttcagtttcttctgcaaaagctgtacctagtaaccttccaaaattgtttttaaataaagttcttaaattgtagcaataaacaaaaggacaaagtacacttaaagaatactgcagtttatcaaaagacataagaaatttcaactcatacttggagagttataaaaatcaatgttttggctaagttataaacatgtttataatgcaattatttgcataactctagtaatgctaatggcggctataagattaggtttctaaaaaaccactaaaaacataaaaatacttagcctcattatttccctgtagaacgtattgatttacacctaaatttcagtatttactatatcatcattgctgattttaagtcacattcaaaggataaggcaaaaccacctacgaattggcatatttgtttatttctcagtttgtgaaaatgtccttaatttgttgatgtagcaaacaaatttcaactttgattgctatgcaaaaaaacaagataatctgctttgcaatgaactttatatagttcaactgcatacaggcaacatgctatatatgaaaaagttactaactgaactacaggtattaaatactgaaaagagttaacagtttattataatttattttatttaacaatctaagaagttcgcagccatcagcagttccagtgcaatttcaggtgcaattgggaattcaggaatctcggtggagctgttagtgtagcgaaccttgtacgtaaaatacatgcatactttcgatagcacatgtgaaggtatctctctaaaattgacctcattggtttcgttctcagcaaactgacctgggccactcaacatggcttttatcgtgcctgatgttaatgcatgttctctttttacaataaattcatggccatcagatgatatcaatttgacatacatggcatcaggtccttcacagccaccataggttttctcctctccatccattttgttcttatgaaattctactttgcttccccaggaactttagtagtttccctcactgtaggcaaagatttctcagcagccaggtgcagtggctcacacctgcaatcgcaacactttgggagggagatcacttgaggtcaggaatttgagaccagccgggcactccagcctgggccacacagcaagactctgttcgtcagtcccgcagccaccgcagccgggtccccgcgtactgccacagcccctatcccagggccgcccccccacccccagctgcctgctccggtgggttccggggcagtcgaaag

SEQ ID NO: 14506 - RNA, 1889 nt, Homo sapiens
  source 1..1889: mol_type = other RNA
gctgggattacaggcatgagccaccgggctcagccatattaagccagtctcaaataagctggagacttaagtttatagaccctataatgacaactttgttccacctctgagataaagacaatactaaacccatctccagtgcttctttccccatgcataaggaatgatgctgtcatattttttcaaaaaattttttggctgcttaatagaaaagctgaatgagcttgatttcagtagaagacccactgattatgggtatatttattgggacatattttaatagaagataattcatgtaggatatcttcaatgcattataatatgattttcactgtatctcttcacatgttattccataacattctaattggatggagaaagactggaatagttcaaaaaggtgtagcttttaagatctgaataaagttaatagtgagtcttttaaaatacatttaaacaactggaagtataatcacaacaagggactatgaaggaagaataaatattgcaaacgacgctttatagtcaatgcaaatacagtactttgaattacccaaaatgtataatgcacaagaactctaagtcatgtagtttacttgctgaccatctggctacagttcagtttcttctgcaaaagctgtacctagtaaccttccaaaattgtttttaaataaagttcttaaattgtagcaataaacaaaaggacaaagtacacttaaagaatactgcagtttatcaaaagacataagaaatttcaactcatacttggagagttataaaaatcaatgttttggctaagttataaacatgtttataatgcaattatttgcataactctagtaatgctaatggcggctataagattaggtttctaaaaaaccactaaaaacataaaaatacttagcctcattatttccctgtagaacgtattgatttacacctaaatttcagtatttactatatcatcattgctgattttaagtcacattcaaaggataaggcaaaaccacctacgaattggcatatttgtttatttctcagtttgtgaaaatgtccttaatttgttgatgtagcaaacaaatttcaactttgattgctatgcaaaaaaacaagataatctgctttgcaatgaactttatatagttcaactgcatacaggcaacatgctatatatgaaaaagttactaactgaactacaggtattaaatactgaaaagagttaacagtttattataatttattttatttaacaatctaagaagttcgcagccatcagcagttccagtgcaatttcaggtgcaattgggaattcaggaatctcggtggagctgttagtgtagcgaaccttgtacgtaaaatacatgcatactttcgatagcacatgtgaaggtatctctctaaaattgacctcattggtttcgttctcagcaaactgacctgggccactcaacatggcttttatcgtgcctgatgttaatgcatgttctctttttacaataaattcatggccatcagatgatatcaatttgacatacatggcatcaggtccttcacagccaccataggttttctcctctccatccattttgttcttatgaaattctactttgcttccccaggaactttagtagtttccctcactgtaggcaaagatttctcagcagccaggtgcagtggctcacacctgcaatcgcaacactttgggagggagatcacttgaggtcaggaatttgagaccagccgggcactccagcctgggccacacagcaagacttcgtcagtcccgcagccaccgcagccgggtccccgcgtactgccacagcccctatcccagggccgcccccccacccccagctgcctgctccggtgggttccggggcagtcgaaag

SEQ ID NO: 14507 - RNA, 1678 nt, Homo sapiens
  source 1..1678: mol_type = other RNA
gctgggattacaggcatgagccaccgggctcagccatattaagccagtctcaaataagctggagacttaagtttatagaccctataatgacaactttgttccacctctgagataaagacaatactaaacccatctccagtgcttctttccccatgcataaggaatgatgctgtcatattttttcaaaaaattttttggctgcttaatagaaaagctgaatgagcttgatttcagtagaagacccactgattatgggtatatttattgggacatattttaatagaagataattcatgtaggatatcttcaatgcattataatatgattttcactgtatctcttcacatgttattccataacattctaattggatggagaaagactggaatagttcaaaaaggtgtagcttttaagatctgaataaagttaatagtgagtcttttaaaatacatttaaacaactggaagtataatcacaacaagggactatgaaggaagaataaatattgcaaacgacgctttatagtcaatgcaaatacagtactttgaattacccaaaatgtataatgcacaagaactctaagtcatgtagtttacttgctgaccatctggctacagttcagtttcttctgcaaaagctgtacctagtaaccttccaaaattgtttttaaataaagttcttaaattgtagcaataaacaaaaggacaaagtacacttaaagaatactgcagtttatcaaaagacataagaaatttcaactcatacttggagagttataaaaatcaatgttttggctaagttataaacatgtttataatgcaattatttgcataactctagtaatgctaatggcggctataagattaggtttctaaaaaaccactaaaaacataaaaatacttagcctcattatttccctgtagaacgtattgatttacacctaaatttcagtatttactatatcatcattgctgattttaagtcacattcaaaggataaggcaaaaccacctacgaattggcatatttgtttatttctcagtttgtgaaaatgtccttaatttgttgatgtagcaaacaaatttcaactttgattgctatgcaaaaaaacaagataatctgctttgcaatgaactttatatagttcaactgcatacaggcaacatgctatatatgaaaaagttactaactgaactacaggtattaaatactgaaaagagttaacagtttattataatttattttatttaacaatctaagaagttcgcagccatcagcagttccagtgcaatttcaggtgcaattgggaattcaggaatctcggtggagctgttagtgtagcgaaccttgtacgtaaaatacatgcatactttcgatagcacatgtgaaggtatctctctaaaattgacctcattggtttcgttctcagcaaactgacctgggccactcaacatggcttttatcgtgcctgatgttaatgcatgttctctttttacaataaattcatggccatcagatgatatcaatttgacatacatggcatcaggtccttcacagccaccataggttttctcctctccatccattttgttcttatgaaattctactttgcttccccaggaactttagtagtttcctggtgaggcgaggacgcagagtgtgtcgctcacttccgtctg

SEQ ID NO: 14508 - RNA, 1750 nt, Homo sapiens
  source 1..1750: mol_type = other RNA
gctgggattacaggcatgagccaccgggctcagccatattaagccagtctcaaataagctggagacttaagtttatagaccctataatgacaactttgttccacctctgagataaagacaatactaaacccatctccagtgcttctttccccatgcataaggaatgatgctgtcatattttttcaaaaaattttttggctgcttaatagaaaagctgaatgagcttgatttcagtagaagacccactgattatgggtatatttattgggacatattttaatagaagataattcatgtaggatatcttcaatgcattataatatgattttcactgtatctcttcacatgttattccataacattctaattggatggagaaagactggaatagttcaaaaaggtgtagcttttaagatctgaataaagttaatagtgagtcttttaaaatacatttaaacaactggaagtataatcacaacaagggactatgaaggaagaataaatattgcaaacgacgctttatagtcaatgcaaatacagtactttgaattacccaaaatgtataatgcacaagaactctaagtcatgtagtttacttgctgaccatctggctacagttcagtttcttctgcaaaagctgtacctagtaaccttccaaaattgtttttaaataaagttcttaaattgtagcaataaacaaaaggacaaagtacacttaaagaatactgcagtttatcaaaagacataagaaatttcaactcatacttggagagttataaaaatcaatgttttggctaagttataaacatgtttataatgcaattatttgcataactctagtaatgctaatggcggctataagattaggtttctaaaaaaccactaaaaacataaaaatacttagcctcattatttccctgtagaacgtattgatttacacctaaatttcagtatttactatatcatcattgctgattttaagtcacattcaaaggataaggcaaaaccacctacgaattggcatatttgtttatttctcagtttgtgaaaatgtccttaatttgttgatgtagcaaacaaatttcaactttgattgctatgcaaaaaaacaagataatctgctttgcaatgaactttatatagttcaactgcatacaggcaacatgctatatatgaaaaagttactaactgaactacaggtattaaatactgaaaagagttaacagtttattataatttattttatttaacaatctaagaagttcgcagccatcagcagttccagtgcaatttcaggtgcaattgggaattcaggaatctcggtggagctgttagtgtagcgaaccttgtacgtaaaatacatgcatactttcgatagcacatgtgaaggtatctctctaaaattgacctcattggtttcgttctcagcaaactgacctgggccactcaacatggcttttatcgtgcctgatgttaatgcatgttctctttttacaataaattcatggccatcagatgatatcaatttgacatacatggcatcaggtccttcacagccaccataggttttctcctctccatccattttgttcttatgaaattctactttgcttccccaggaactttagtagtttctcgtcagtcccgcagccaccgcagccgggtccccgcgtactgccacagcccctatcccagggccgcccccccacccccagctgcctgctccggtgggttccggggcagtcgaaag

SEQ ID NO: 14509 - RNA, 1624 nt, Homo sapiens
  source 1..1624: mol_type = other RNA
gctgggattacaggcatgagccaccgggctcagccatattaagccagtctcaaataagctggagacttaagtttatagaccctataatgacaactttgttccacctctgagataaagacaatactaaacccatctccagtgcttctttccccatgcataaggaatgatgctgtcatattttttcaaaaaattttttggctgcttaatagaaaagctgaatgagcttgatttcagtagaagacccactgattatgggtatatttattgggacatattttaatagaagataattcatgtaggatatcttcaatgcattataatatgattttcactgtatctcttcacatgttattccataacattctaattggatggagaaagactggaatagttcaaaaaggtgtagcttttaagatctgaataaagttaatagtgagtcttttaaaatacatttaaacaactggaagtataatcacaacaagggactatgaaggaagaataaatattgcaaacgacgctttatagtcaatgcaaatacagtactttgaattacccaaaatgtataatgcacaagaactctaagtcatgtagtttacttgctgaccatctggctacagttcagtttcttctgcaaaagctgtacctagtaaccttccaaaattgtttttaaataaagttcttaaattgtagcaataaacaaaaggacaaagtacacttaaagaatactgcagtttatcaaaagacataagaaatttcaactcatacttggagagttataaaaatcaatgttttggctaagttataaacatgtttataatgcaattatttgcataactctagtaatgctaatggcggctataagattaggtttctaaaaaaccactaaaaacataaaaatacttagcctcattatttccctgtagaacgtattgatttacacctaaatttcagtatttactatatcatcattgctgattttaagtcacattcaaaggataaggcaaaaccacctacgaattggcatatttgtttatttctcagtttgtgaaaatgtccttaatttgttgatgtagcaaacaaatttcaactttgattgctatgcaaaaaaacaagataatctgctttgcaatgaactttatatagttcaactgcatacaggcaacatgctatatatgaaaaagttactaactgaactacaggtattaaatactgaaaagagttaacagtttattataatttattttatttaacaatctaagaagttcgcagccatcagcagttccagtgcaatttcaggtgcaattgggaattcaggaatctcggtggagctgttagtgtagcgaaccttgtacgtaaaatacatgcatactttcgatagcacatgtgaaggtatctctctaaaattgacctcattggtttcgttctcagcaaactgacctgggccactcaacatggcttttatcgtgcctgatgttaatgcatgttctctttttacaataaattcatggccatcagatgatatcaatttgacatacatggcatcaggtccttcacagccaccataggttttctcctctccatctggtgaggcgaggacgcagagtgtgtcgctcacttccgtctg

SEQ ID NO: 14510 - RNA, 1696 nt, Homo sapiens
  source 1..1696: mol_type = other RNA
gctgggattacaggcatgagccaccgggctcagccatattaagccagtctcaaataagctggagacttaagtttatagaccctataatgacaactttgttccacctctgagataaagacaatactaaacccatctccagtgcttctttccccatgcataaggaatgatgctgtcatattttttcaaaaaattttttggctgcttaatagaaaagctgaatgagcttgatttcagtagaagacccactgattatgggtatatttattgggacatattttaatagaagataattcatgtaggatatcttcaatgcattataatatgattttcactgtatctcttcacatgttattccataacattctaattggatggagaaagactggaatagttcaaaaaggtgtagcttttaagatctgaataaagttaatagtgagtcttttaaaatacatttaaacaactggaagtataatcacaacaagggactatgaaggaagaataaatattgcaaacgacgctttatagtcaatgcaaatacagtactttgaattacccaaaatgtataatgcacaagaactctaagtcatgtagtttacttgctgaccatctggctacagttcagtttcttctgcaaaagctgtacctagtaaccttccaaaattgtttttaaataaagttcttaaattgtagcaataaacaaaaggacaaagtacacttaaagaatactgcagtttatcaaaagacataagaaatttcaactcatacttggagagttataaaaatcaatgttttggctaagttataaacatgtttataatgcaattatttgcataactctagtaatgctaatggcggctataagattaggtttctaaaaaaccactaaaaacataaaaatacttagcctcattatttccctgtagaacgtattgatttacacctaaatttcagtatttactatatcatcattgctgattttaagtcacattcaaaggataaggcaaaaccacctacgaattggcatatttgtttatttctcagtttgtgaaaatgtccttaatttgttgatgtagcaaacaaatttcaactttgattgctatgcaaaaaaacaagataatctgctttgcaatgaactttatatagttcaactgcatacaggcaacatgctatatatgaaaaagttactaactgaactacaggtattaaatactgaaaagagttaacagtttattataatttattttatttaacaatctaagaagttcgcagccatcagcagttccagtgcaatttcaggtgcaattgggaattcaggaatctcggtggagctgttagtgtagcgaaccttgtacgtaaaatacatgcatactttcgatagcacatgtgaaggtatctctctaaaattgacctcattggtttcgttctcagcaaactgacctgggccactcaacatggcttttatcgtgcctgatgttaatgcatgttctctttttacaataaattcatggccatcagatgatatcaatttgacatacatggcatcaggtccttcacagccaccataggttttctcctctccattcgtcagtcccgcagccaccgcagccgggtccccgcgtactgccacagcccctatcccagggccgcccccccacccccagctgcctgctccggtgggttccggggcagtcgaaag

SEQ ID NO: 14511 - RNA, 3498 nt, Homo sapiens
  source 1..3498: mol_type = other RNA
gctgggattacaggcatgagccaccgggctcagcctgatgtctcttcttataaaggcactaatcccatcacgagggctccaccctcatgacctcatctaatcctaattgcctcccaaatgcctcatttccaagtaacatcacattgatggtgaggattttaacataattagttttgggagggacataaacattcagtccataacaactcatattacaccacttattgcataccagtattgttacatgaaaataccaatgtttactcatataaatatagatgatttatttccaaataaaacaatactgatttctcctggctctgaaatcctcattcttcactatatcttggttcttttactgatagcttgtctcagccaagttagacgttcacaccatgaagatcatatatcctcatatccgtggagatggtaaagtaaggtttctactgttacacaccattatgagtgacaactttatctacctaaagactcacttttctttattctcacccacaagtttgtcagctgaaagtggcaccctgttttgccgagaagttccttatatttgataattctagatctgagaaacagactcaaattcttttttctgtgaccttaaatcaggctcagagccctataatggacttcacaattctattttgttgtatgtgaccaataaattatctttaaaactatgctggaagtaaaatatcggtaattttttttttttttgacacagagtcttgctctgttgcccagactggagtgcagtggtgcaatctctgctcggtgcaacccccacctcctgggttcaagcgattctcctgcctcagcctctccagtagctgagattacaggtgcgcaccaccacgcccagctaattttgtattttttagtagagacagggtttcaccgtggtctcaaactcttgacctcgtgatccgcctgtctcagcctcccaaagtgctggggttacaggtgtaagccactgcgcccagccagtaattcttatcaaatgaaaaatgatcttcattcacaatgactgaccaaacttctgagtttccttcagttaatttcaaatcctgaggtcaaaatcaccaatgacttttgctctttggctttcaaagtgggacatatcatcaaatggtcccatatacacaaaatttacattatagacaaatacatatttgccatatgtttgatagcctcattcgttgattttatagatttaaaacaaccttaggctttttcttcagaatgtgtattctgatgtcgaatcagggatgaactccgactatatgccttcccacatttactacattcatagggtttctctgaagaatgacttctctgatgtcgaataaggtctgagccactgctaaatgccttcccacattcattacattcatagggtttctctccagtatgacttctttcatgtagaataagagatgtgcgctgactaaaggccttaccacatgttttgcatgtatatggcttctctccagtgtgaattctttcatgttgggcgaggtgtgcactctggctgaaggccttcccacactgatcacattcatagggtctatcttcagtatgaattctcttatgtcgtgtgagagatattcggtggctgaaggcttttccacattcctcacactggtagggtttttctccagtatgaattctttgatgttcaataagaaatgattggcggccgaaaactttactacatttattgcatttgaaaggtttctcttcagaatgaatattctgatgtattttaaggtttgcagttccagaaaacatcttcccacattccttacactcaaatagtttctttttctttgtatgaactttctgatgttgaataagggatgaatgccgattgcagaccttctcacatttattgcatctgtatagtttttctccattatgaattcttagatgcagaataagggttgaaagccgcctgaagaacttgtcacatttatcacatttgtacggtttctctgaagtgtgaattctctggtgaagcatcaggggtgaaatcctattaaataatttcccacattttctgcatttaaaaggattctctaaatggtgacttctttgctgtagactctgacttaaggccttcgcattttcagggattttctctccagcatgaattcttttatgtacaacaaagactgatttctttttgaagcctctcccacatttattatatttatgtgttttctttccattgtgaattttcttatgaagtaaaagggatgacatctgattgaaggcttttccgcactttctgcactggcagacattcccaacaacatgaattttctgatgtatattgaaagactgacattgactcaaggccttcccacagtcaagaatttcctttccatcatgaattctcatatgtagaataagggttgttctttgattgaagctttccccacatttattgcattcatggcttttctttccactgtgaattctctgatgaagtaggatggatgagatctgtctgaaagcttttctacaattactgcattcaaaaggcttctctcctgtatgaatgttctgatgaagtttaagagagaagcttcgactaaaggttttaccacagtcattacattttaaaggtttcttccctgaatgccctttcttaggttttactaggactgaatttttgttgcagccactctttcgtgtaggagctttttgttgtgcagaaactagtttctggcagatgctttgcccagatttgttgcattgatttggaggtaacttcttggtctcacatttagaccccgagtcaggagcccggcgtcttcttactggctctaccatccagggtgctttccctttctccaataaggtgatcacatttggtctccgaaaggaaagaccaagcgagaccaggttccggtaattctccaacatgacatcttcatacaaatccttctgaatggggctcagccattcccactcctcctgggagaagtagatggctaagtccccaaatgttataggtgccttggatttggatttcccccgtgcagaaggcatcctttcctccccctttagggtccacactgagagatgggcagagagctggtaaggcagggcacatcaaggcagggctgtaaacctggctcgtcttccgagtccctgatgatagatgagaaagggctttgaaaggcacaaagctatgtcctcctgaggtgaggacggctggaacctcggtcttcccgggctcagaccccggcggcgaccaccgagacagccgagcagggactcagcgcctgcgcactcccctccgggaccccgggaccgcgcgctgcaccccccttcacacacgcaccacgcatgcgggcgcgtggccccgcccccaaacaaggccacgcggcgtgcgctcacccgcctctcggggacagtaccaccagccccggcctgaggccccgacccctcagcgccacacgcacaagcgcgttc

SEQ ID NO: 14512 - RNA, 3840 nt, Homo sapiens
  source 1..3840: mol_type = other RNA
gctgggattacaggcatgagccaccgggctcagcctgatgtctcttcttataaaggcactaatcccatcacgagggctccaccctcatgacctcatctaatcctaattgcctcccaaatgcctcatttccaagtaacatcacattgatggtgaggattttaacataattagttttgggagggacataaacattcagtccataacaactcatattacaccacttattgcataccagtattgttacatgaaaataccaatgtttactcatataaatatagatgatttatttccaaataaaacaatactgatttctcctggctctgaaatcctcattcttcactatatcttggttcttttactgatagcttgtctcagccaagttagacgttcacaccatgaagatcatatatcctcatatccgtggagatggtaaagtaaggtttctactgttacacaccattatgagtgacaactttatctacctaaagactcacttttctttattctcacccacaagtttgtcagctgaaagtggcaccctgttttgccgagaagttccttatatttgataattctagatctgagaaacagactcaaattcttttttctgtgaccttaaatcaggctcagagccctataatggacttcacaattctattttgttgtatgtgaccaataaattatctttaaaactatgctggaagtaaaatatcggtaattttttttttttttgacacagagtcttgctctgttgcccagactggagtgcagtggtgcaatctctgctcggtgcaacccccacctcctgggttcaagcgattctcctgcctcagcctctccagtagctgagattacaggtgcgcaccaccacgcccagctaattttgtattttttagtagagacagggtttcaccgtggtctcaaactcttgacctcgtgatccgcctgtctcagcctcccaaagtgctggggttacaggtgtaagccactgcgcccagccagtaattcttatcaaatgaaaaatgatcttcattcacaatgactgaccaaacttctgagtttccttcagttaatttcaaatcctgaggtcaaaatcaccaatgacttttgctctttggctttcaaagtgggacatatcatcaaatggtcccatatacacaaaatttacattatagacaaatacatatttgccatatgtttgatagcctcattcgttgattttatagatttaaaacaaccttaggctttttcttcagaatgtgtattctgatgtcgaatcagggatgaactccgactatatgccttcccacatttactacattcatagggtttctctgaagaatgacttctctgatgtcgaataaggtctgagccactgctaaatgccttcccacattcattacattcatagggtttctctccagtatgacttctttcatgtagaataagagatgtgcgctgactaaaggccttaccacatgttttgcatgtatatggcttctctccagtgtgaattctttcatgttgggcgaggtgtgcactctggctgaaggccttcccacactgatcacattcatagggtctatcttcagtatgaattctcttatgtcgtgtgagagatattcggtggctgaaggcttttccacattcctcacactggtagggtttttctccagtatgaattctttgatgttcaataagaaatgattggcggccgaaaactttactacatttattgcatttgaaaggtttctcttcagaatgaatattctgatgtattttaaggtttgcagttccagaaaacatcttcccacattccttacactcaaatagtttctttttctttgtatgaactttctgatgttgaataagggatgaatgccgattgcagaccttctcacatttattgcatctgtatagtttttctccattatgaattcttagatgcagaataagggttgaaagccgcctgaagaacttgtcacatttatcacatttgtacggtttctctgaagtgtgaattctctggtgaagcatcaggggtgaaatcctattaaataatttcccacattttctgcatttaaaaggattctctaaatggtgacttctttgctgtagactctgacttaaggccttcgcattttcagggattttctctccagcatgaattcttttatgtacaacaaagactgatttctttttgaagcctctcccacatttattatatttatgtgttttctttccattgtgaattttcttatgaagtaaaagggatgacatctgattgaaggcttttccgcactttctgcactggcagacattcccaacaacatgaattttctgatgtatattgaaagactgacattgactcaaggccttcccacagtcaagaatttcctttccatcatgaattctcatatgtagaataagggttgttctttgattgaagctttccccacatttattgcattcatggcttttctttccactgtgaattctctgatgaagtaggatggatgagatctgtctgaaagcttttctacaattactgcattcaaaaggcttctctcctgtatgaatgttctgatgaagtttaagagagaagcttcgactaaaggttttaccacagtcattacattttaaaggtttcttccctgaatgccctttcttaggttttactaggactgaatttttgttgcagccactctttcgtgtaggagctttttgttgtgcagaaactagtttctggcagatgctttgcccagatttgttgcattgatttggaggtaacttcttggtctcacatttagaccccgagtcaggagcccggcgtcttcttactggctctaccatccagggtgctttccctttctccaataaggtgatcacatttggtctccgaaaggaaagaccaagcgagaccaggttccggtaattctccaacatgacatcttcatacaaatccttctgaatggggctcagccattcccactcctcctgggagaagtagatggctaagtccccaaatgttataggtgccttggatttggatttcccccgtgcagaaggcatcctttcctccccctttagggtccacactgagagatgggcagagagctggtaaggcagggcagataagcagatcagttggctttccccttccaattacttaggtaaaatgacttgttccaggaagttgtaatgcattcatcccgcagttttcacaggtgtgtgcactcagccacgcaccccaaatttgagaagatgattcttgtctgatatggtctggctgtgtccccactcaaatctcatcttgaattatagctcccataatttccacgtgttgtgggagggacccggtgggagataactgaatcatgggggcggtttcccccatgctgttctcatggcagtgagtaagtctcatgtgatctgatggttctgtacagggactctcattctccctgtggccatgtaagacgtgtctttcaccttccatcacgattgtgaggcctccccagccacgtagaactgtgagtctgggtatgtctttatcagcagcacgaaaacagactcatacattgtccataaaataattttcttcaaggaactcggcacacatcaaggcagggctgtaaacctggctcgtcttccgagtccctgatgatagatgagaaagggctttgaaaggcacaaagctatgtcctcctgaggtgaggacggctggaacctcggtcttcccgggctcagaccccggcggcgaccaccgagacagccgagcagggactcagcgcctgcgcactcccctccgggaccccgggaccgcgcgctgcacccccc

SEQ ID NO: 14513 - RNA, 5621 nt, Homo sapiens
  source 1..5621: mol_type = other RNA
gctgggattacaggcatgagccaccgggctcagcctgatgtctcttcttataaaggcactaatcccatcacgagggctccaccctcatgacctcatctaatcctaattgcctcccaaatgcctcatttccaagtaacatcacattgatggtgaggattttaacataattagttttgggagggacataaacattcagtccataacaactcatattacaccacttattgcataccagtattgttacatgaaaataccaatgtttactcatataaatatagatgatttatttccaaataaaacaatactgatttctcctggctctgaaatcctcattcttcactatatcttggttcttttactgatagcttgtctcagccaagttagacgttcacaccatgaagatcatatatcctcatatccgtggagatggtaaagtaaggtttctactgttacacaccattatgagtgacaactttatctacctaaagactcacttttctttattctcacccacaagtttgtcagctgaaagtggcaccctgttttgccgagaagttccttatatttgataattctagatctgagaaacagactcaaattcttttttctgtgaccttaaatcaggctcagagccctataatggacttcacaattctattttgttgtatgtgaccaataaattatctttaaaactatgctggaagtaaaatatcggtaattttttttttttttgacacagagtcttgctctgttgcccagactggagtgcagtggtgcaatctctgctcggtgcaacccccacctcctgggttcaagcgattctcctgcctcagcctctccagtagctgagattacaggtgcgcaccaccacgcccagctaattttgtattttttagtagagacagggtttcaccgtggtctcaaactcttgacctcgtgatccgcctgtctcagcctcccaaagtgctggggttacaggtgtaagccactgcgcccagccagtaattcttatcaaatgaaaaatgatcttcattcacaatgactgaccaaacttctgagtttccttcagttaatttcaaatcctgaggtcaaaatcaccaatgacttttgctctttggctttcaaagtgggacatatcatcaaatggtcccatatacacaaaatttacattatagacaaatacatatttgccatatgtttgatagcctcattcgttgattttatagatttaaaacaaccttaggctttttcttcagaatgtgtattctgatgtcgaatcagggatgaactccgactatatgccttcccacatttactacattcatagggtttctctgaagaatgacttctctgatgtcgaataaggtctgagccactgctaaatgccttcccacattcattacattcatagggtttctctccagtatgacttctttcatgtagaataagagatgtgcgctgactaaaggccttaccacatgttttgcatgtatatggcttctctccagtgtgaattctttcatgttgggcgaggtgtgcactctggctgaaggccttcccacactgatcacattcatagggtctatcttcagtatgaattctcttatgtcgtgtgagagatattcggtggctgaaggcttttccacattcctcacactggtagggtttttctccagtatgaattctttgatgttcaataagaaatgattggcggccgaaaactttactacatttattgcatttgaaaggtttctcttcagaatgaatattctgatgtattttaaggtttgcagttccagaaaacatcttcccacattccttacactcaaatagtttctttttctttgtatgaactttctgatgttgaataagggatgaatgccgattgcagaccttctcacatttattgcatctgtatagtttttctccattatgaattcttagatgcagaataagggttgaaagccgcctgaagaacttgtcacatttatcacatttgtacggtttctctgaagtgtgaattctctggtgaagcatcaggggtgaaatcctattaaataatttcccacattttctgcatttaaaaggattctctaaatggtgacttctttgctgtagactctgacttaaggccttcgcattttcagggattttctctccagcatgaattcttttatgtacaacaaagactgatttctttttgaagcctctcccacatttattatatttatgtgttttctttccattgtgaattttcttatgaagtaaaagggatgacatctgattgaaggcttttccgcactttctgcactggcagacattcccaacaacatgaattttctgatgtatattgaaagactgacattgactcaaggccttcccacagtcaagaatttcctttccatcatgaattctcatatgtagaataagggttgttctttgattgaagctttccccacatttattgcattcatggcttttctttccactgtgaattctctgatgaagtaggatggatgagatctgtctgaaagcttttctacaattactgcattcaaaaggcttctctcctgtatgaatgttctgatgaagtttaagagagaagcttcgactaaaggttttaccacagtcattacattttaaaggtttcttccctgaatgccctttcttaggttttactaggactgaatttttgttgcagccactctttcgtgtaggagctttttgttgtgcagaaactagtttctggcagatgctttgcccagatttgttgcattgatttggaggtaacttcttggtctcacatttagaccccgagtcaggagcccggcgtcttcttactggctctaccatccagggtgctttccctttctccaataaggtgatcacatttggtctccgaaaggaaagaccaagcgagaccaggttccggtaattctccaacatgacatcttcatacaaatccttctgaatggggctcagccattcccactcctcctgggagaagtagatggctaagtccccaaatgttataggtgccttggatttggatttcccccgtgcagaaggcatcctttcctccccctttagggtccacactgagagatgggcagagagctggtaaggcagggcagataagcagatcagttggctttccccttccaattacttaggtaaaatgacttgttccaggaagttgtaatgcattcatcccgcagttttcacaggtgtgtgcactcagccacgcaccccaaatttgagaagatgattcttgtctgatatggtctggctgtgtccccactcaaatctcatcttgaattatagctcccataatttccacgtgttgtgggagggacccggtgggagataactgaatcatgggggcggtttcccccatgctgttctcatggcagtgagtaagtctcatgtgatctgatggttctgtacagggactctcattctccctgtggccatgtaagacgtgtctttcaccttccatcacgattgtgaggcctccccagccacgtagaactgtgagtctgggtatgtctttatcagcagcacgaaaacagactcatacattgtccataaaataattttcttcaaggaactcggcactacacatcaaggcagggctgtaaacctggctcgtcttccgagtccctgatgatagatgagaaagggctttgaaaggcacaaagctatgtcctcctgaggtgaggacggctggaacccgggctgcaggccgtttcttctcatctcagaacactatccttttatcatctctccgtgccccgccttccccagctcccttactcttctccctgtcatcatgccttcggtctgtccatgcgcttgcatcacggtcctctcaatcagagtgattttgcccctgcaggggacatctgacagtgtctggagacatttttttttcgcttgtcacaacccagagggaggcgcggtgtgctactggcctggtaaatagagcccagggttgctgcacaacatcctataatacatagaatagcagcccctcccacctcccaacaaaaaactatctggccccaaatgtcacagtgccaaggctgtgaaacactggtctggacagaaacatttccagacccatgtgttatatggaaacatcccttagtccctgacacttcaaagttctgttcttgaccccatgggctccctagggacatctccatcaggaagatcctttgttcctgaccccacctcctctaccctaatgctgccctcccaggaccctgcctacacaattctgaacctaagccctgatctagacgtccaagttattttacctctggacctgcaacccttactctggggctcatccttttgcatttctacctatggattttattctccaggtgtgggacgcctgcggttattatgctaataataaaacgatgatcattgatgtggcacttccttgtgccaagttctacttatgctcaccataaacctgaggttggttctgttattactactgttttacaagtgaaccgaggagtggtggacttaagtaagctctctcagtcacacagccagccagtggtgaaaccaggagtcaacaccagacagcggggcgccacagtccatgctcttatttttccaagctaccttggtaggaaggggacacaaccatacttagcgtcagtggagggctctgtcctccactcaaatgtacacatgcagaaaactgacgacgcaggtggttggcgggggcagcgcaccactgctcaactggagatggtcagatgccctggtatgtggacaaagatagcccagtccgaagctcagagatgcaaagtcctccagtattcaccactacctctgcctctgtatagggtcaaagaaaaacgaccaccagcaccataaccaacacctaaacacggtgattagtatgtgacaagctctgtgcagggtgtttcagctacgtcatcccatttaatcttcccaataacacccaggcaggtgctattaatatgctattttaccaaggaggaaagtcatgcacaattaaacagttccacagatttccagggcagcccatcacatcttagagctgctaagaattcttcccctgtgggcctccatttccatggttacagtgagatatacaccagaaaggcacagtcacacactcataaccgcaaagccactgacgctaagtggcagacagacgcccaggcaagtcacacagtaacccaaggctacaataaacgcccacatcagcctgacactgacacacgcacacactccagaaacacaaatcttcacagtcagcgtcacacacccactcccggcttcccaatggctccattgtttccttcgcgtgggtcacgcagcgatacacatccgcggtcccgacatagctccctcacacacaggcacacacggctcgcctcacacgcggcgccaacttcacacttgggcgcacaagccccgagaaccacagcagcgaagggcgcaaaccccacgccgtggcgggccgagaacccacgcaggcgcgagcccaccgcccacgcaagcacccgcgcagacgcccacgccatcgtggatgcgcaaacccacgcgcgccttggcaggaacgtcca

SEQ ID NO: 14514 - RNA, 3807 nt, Homo sapiens
  source 1..3807: mol_type = other RNA
gctgggattacaggcatgagccaccgggctcagcctgatgtctcttcttataaaggcactaatcccatcacgagggctccaccctcatgacctcatctaatcctaattgcctcccaaatgcctcatttccaagtaacatcacattgatggtgaggattttaacataattagttttgggagggacataaacattcagtccataacaactcatattacaccacttattgcataccagtattgttacatgaaaataccaatgtttactcatataaatatagatgatttatttccaaataaaacaatactgatttctcctggctctgaaatcctcattcttcactatatcttggttcttttactgatagcttgtctcagccaagttagacgttcacaccatgaagatcatatatcctcatatccgtggagatggtaaagtaaggtttctactgttacacaccattatgagtgacaactttatctacctaaagactcacttttctttattctcacccacaagtttgtcagctgaaagtggcaccctgttttgccgagaagttccttatatttgataattctagatctgagaaacagactcaaattcttttttctgtgaccttaaatcaggctcagagccctataatggacttcacaattctattttgttgtatgtgaccaataaattatctttaaaactatgctggaagtaaaatatcggtaattttttttttttttgacacagagtcttgctctgttgcccagactggagtgcagtggtgcaatctctgctcggtgcaacccccacctcctgggttcaagcgattctcctgcctcagcctctccagtagctgagattacaggtgcgcaccaccacgcccagctaattttgtattttttagtagagacagggtttcaccgtggtctcaaactcttgacctcgtgatccgcctgtctcagcctcccaaagtgctggggttacaggtgtaagccactgcgcccagccagtaattcttatcaaatgaaaaatgatcttcattcacaatgactgaccaaacttctgagtttccttcagttaatttcaaatcctgaggtcaaaatcaccaatgacttttgctctttggctttcaaagtgggacatatcatcaaatggtcccatatacacaaaatttacattatagacaaatacatatttgccatatgtttgatagcctcattcgttgattttatagatttaaaacaaccttaggctttttcttcagaatgtgtattctgatgtcgaatcagggatgaactccgactatatgccttcccacatttactacattcatagggtttctctgaagaatgacttctctgatgtcgaataaggtctgagccactgctaaatgccttcccacattcattacattcatagggtttctctccagtatgacttctttcatgtagaataagagatgtgcgctgactaaaggccttaccacatgttttgcatgtatatggcttctctccagtgtgaattctttcatgttgggcgaggtgtgcactctggctgaaggccttcccacactgatcacattcatagggtctatcttcagtatgaattctcttatgtcgtgtgagagatattcggtggctgaaggcttttccacattcctcacactggtagggtttttctccagtatgaattctttgatgttcaataagaaatgattggcggccgaaaactttactacatttattgcatttgaaaggtttctcttcagaatgaatattctgatgtattttaaggtttgcagttccagaaaacatcttcccacattccttacactcaaatagtttctttttctttgtatgaactttctgatgttgaataagggatgaatgccgattgcagaccttctcacatttattgcatctgtatagtttttctccattatgaattcttagatgcagaataagggttgaaagccgcctgaagaacttgtcacatttatcacatttgtacggtttctctgaagtgtgaattctctggtgaagcatcaggggtgaaatcctattaaataatttcccacattttctgcatttaaaaggattctctaaatggtgacttctttgctgtagactctgacttaaggccttcgcattttcagggattttctctccagcatgaattcttttatgtacaacaaagactgatttctttttgaagcctctcccacatttattatatttatgtgttttctttccattgtgaattttcttatgaagtaaaagggatgacatctgattgaaggcttttccgcactttctgcactggcagacattcccaacaacatgaattttctgatgtatattgaaagactgacattgactcaaggccttcccacagtcaagaatttcctttccatcatgaattctcatatgtagaataagggttgttctttgattgaagctttccccacatttattgcattcatggcttttctttccactgtgaattctctgatgaagtaggatggatgagatctgtctgaaagcttttctacaattactgcattcaaaaggcttctctcctgtatgaatgttctgatgaagtttaagagagaagcttcgactaaaggttttaccacagtcattacattttaaaggtttcttccctgaatgccctttcttaggttttactaggactgaatttttgttgcagccactctttcgtgtaggagctttttgttgtgcagaaactagtttctggcagatgctttgcccagatttgttgcattgatttggaggtaacttcttggtctcacatttagaccccgagtcaggagcccggcgtcttcttactggctctaccatccagggtgctttccctttctccaataaggtgatcacatttggtctccgaaaggaaagaccaagcgagaccaggttccggtaattctccaacatgacatcttcatacaaatccttctgaatggggctcagccattcccactcctcctgggagaagtagatggctaagtccccaaatgttataggtgccttggatttggatttcccccgtgcagaaggcatcctttcctccccctttagggtccacactgagagatgggcagagagctggtaaggcagggcagataagcagatcagttggctttccccttccaattacttaggtaaaatgacttgttccaggaagttgtaatgcattcatcccgcagttttcacaggtgtgtgcactcagccacgcaccccaaatttgagaagatgattcttgtctgatatggtctggctgtgtccccactcaaatctcatcttgaattatagctcccataatttccacgtgttgtgggagggacccggtgggagataactgaatcatgggggcggtttcccccatgctgttctcatggcagtgagtaagtctcatgtgatctgatggttctgtacagggactctcattctccctgtggccatgtaagacgtgtctttcaccttccatcacgattgtgaggcctccccagccacgtagaactgtgagtctgggtatgtctttatcagcagcacgaaaacagactcatacattgtccataaaataattttcttcaaggaactcggcactacacatcaaggcagggctgtaaacctggctcgtcttccgagtccctgatgatagatgagaaagggctttgaaaggcacaaagctatgtcctcctgaggtgaggacggctggaacctcggtcttcccgggctcagaccccggcggcgaccaccgagacagccgagcagggactcagcgcctgcgcactc

SEQ ID NO: 14515 - RNA, 3761 nt, Homo sapiens
  source 1..3761: mol_type = other RNA
gctgggattacaggcatgagccaccgggctcagcctgatgtctcttcttataaaggcactaatcccatcacgagggctccaccctcatgacctcatctaatcctaattgcctcccaaatgcctcatttccaagtaacatcacattgatggtgaggattttaacataattagttttgggagggacataaacattcagtccataacaactcatattacaccacttattgcataccagtattgttacatgaaaataccaatgtttactcatataaatatagatgatttatttccaaataaaacaatactgatttctcctggctctgaaatcctcattcttcactatatcttggttcttttactgatagcttgtctcagccaagttagacgttcacaccatgaagatcatatatcctcatatccgtggagatggtaaagtaaggtttctactgttacacaccattatgagtgacaactttatctacctaaagactcacttttctttattctcacccacaagtttgtcagctgaaagtggcaccctgttttgccgagaagttccttatatttgataattctagatctgagaaacagactcaaattcttttttctgtgaccttaaatcaggctcagagccctataatggacttcacaattctattttgttgtatgtgaccaataaattatctttaaaactatgctggaagtaaaatatcggtaattttttttttttttgacacagagtcttgctctgttgcccagactggagtgcagtggtgcaatctctgctcggtgcaacccccacctcctgggttcaagcgattctcctgcctcagcctctccagtagctgagattacaggtgcgcaccaccacgcccagctaattttgtattttttagtagagacagggtttcaccgtggtctcaaactcttgacctcgtgatccgcctgtctcagcctcccaaagtgctggggttacaggtgtaagccactgcgcccagccagtaattcttatcaaatgaaaaatgatcttcattcacaatgactgaccaaacttctgagtttccttcagttaatttcaaatcctgaggtcaaaatcaccaatgacttttgctctttggctttcaaagtgggacatatcatcaaatggtcccatatacacaaaatttacattatagacaaatacatatttgccatatgtttgatagcctcattcgttgattttatagatttaaaacaaccttaggctttttcttcagaatgtgtattctgatgtcgaatcagggatgaactccgactatatgccttcccacatttactacattcatagggtttctctgaagaatgacttctctgatgtcgaataaggtctgagccactgctaaatgccttcccacattcattacattcatagggtttctctccagtatgacttctttcatgtagaataagagatgtgcgctgactaaaggccttaccacatgttttgcatgtatatggcttctctccagtgtgaattctttcatgttgggcgaggtgtgcactctggctgaaggccttcccacactgatcacattcatagggtctatcttcagtatgaattctcttatgtcgtgtgagagatattcggtggctgaaggcttttccacattcctcacactggtagggtttttctccagtatgaattctttgatgttcaataagaaatgattggcggccgaaaactttactacatttattgcatttgaaaggtttctcttcagaatgaatattctgatgtattttaaggtttgcagttccagaaaacatcttcccacattccttacactcaaatagtttctttttctttgtatgaactttctgatgttgaataagggatgaatgccgattgcagaccttctcacatttattgcatctgtatagtttttctccattatgaattcttagatgcagaataagggttgaaagccgcctgaagaacttgtcacatttatcacatttgtacggtttctctgaagtgtgaattctctggtgaagcatcaggggtgaaatcctattaaataatttcccacattttctgcatttaaaaggattctctaaatggtgacttctttgctgtagactctgacttaaggccttcgcattttcagggattttctctccagcatgaattcttttatgtacaacaaagactgatttctttttgaagcctctcccacatttattatatttatgtgttttctttccattgtgaattttcttatgaagtaaaagggatgacatctgattgaaggcttttccgcactttctgcactggcagacattcccaacaacatgaattttctgatgtatattgaaagactgacattgactcaaggccttcccacagtcaagaatttcctttccatcatgaattctcatatgtagaataagggttgttctttgattgaagctttccccacatttattgcattcatggcttttctttccactgtgaattctctgatgaagtaggatggatgagatctgtctgaaagcttttctacaattactgcattcaaaaggcttctctcctgtatgaatgttctgatgaagtttaagagagaagcttcgactaaaggttttaccacagtcattacattttaaaggtttcttccctgaatgccctttcttaggttttactaggactgaatttttgttgcagccactctttcgtgtaggagctttttgttgtgcagaaactagtttctggcagatgctttgcccagatttgttgcattgatttggaggtaacttcttggtctcacatttagaccccgagtcaggagcccggcgtcttcttactggctctaccatccagggtgctttccctttctccaataaggtgatcacatttggtctccgaaaggaaagaccaagcgagaccaggttccggtaattctccaacatgacatcttcatacaaatccttctgaatggggctcagccattcccactcctcctgggagaagtagatggctaagtccccaaatgttataggtgccttggatttggatttcccccgtgcagaaggcatcctttcctccccctttagggtccacactgagagatgggcagagagctggtaaggcagggcagataagcagatcagttggctttccccttccaattacttaggtaaaatgacttgttccaggaagttgtaatgcattcatcccgcagttttcacaggtgtgtgcactcagccacgcaccccaaatttgagaagatgattcttgtctgatatggtctggctgtgtccccactcaaatctcatcttgaattatagctcccataatttccacgtgttgtgggagggacccggtgggagataactgaatcatgggggcggtttcccccatgctgttctcatggcagtgagtaagtctcatgtgatctgatggttctgtacagggactctcattctccctgtggccatgtaagacgtgtctttcaccttccatcacgattgtgaggcctccccagccacgtagaactgtgagtctgggtatgtctttatcagcagcacgaaaacagactcatacattgtccataaaataattttcttcaaggaactcggcactacacatcaaggcagggctgtaaacctggctcgtcttccgagtccctgatgatagatgagaaagggctttgaaaggcacaaagctatgtcctcctgaggtgaggacggctggaacctgcacgttttgcgaagaggcccacagt

SEQ ID NO: 14516 - RNA, 3711 nt, Homo sapiens
  source 1..3711: mol_type = other RNA
gctgggattacaggcatgagccaccgggctcagcctgatgtctcttcttataaaggcactaatcccatcacgagggctccaccctcatgacctcatctaatcctaattgcctcccaaatgcctcatttccaagtaacatcacattgatggtgaggattttaacataattagttttgggagggacataaacattcagtccataacaactcatattacaccacttattgcataccagtattgttacatgaaaataccaatgtttactcatataaatatagatgatttatttccaaataaaacaatactgatttctcctggctctgaaatcctcattcttcactatatcttggttcttttactgatagcttgtctcagccaagttagacgttcacaccatgaagatcatatatcctcatatccgtggagatggtaaagtaaggtttctactgttacacaccattatgagtgacaactttatctacctaaagactcacttttctttattctcacccacaagtttgtcagctgaaagtggcaccctgttttgccgagaagttccttatatttgataattctagatctgagaaacagactcaaattcttttttctgtgaccttaaatcaggctcagagccctataatggacttcacaattctattttgttgtatgtgaccaataaattatctttaaaactatgctggaagtaaaatatcggtaattttttttttttttgacacagagtcttgctctgttgcccagactggagtgcagtggtgcaatctctgctcggtgcaacccccacctcctgggttcaagcgattctcctgcctcagcctctccagtagctgagattacaggtgcgcaccaccacgcccagctaattttgtattttttagtagagacagggtttcaccgtggtctcaaactcttgacctcgtgatccgcctgtctcagcctcccaaagtgctggggttacaggtgtaagccactgcgcccagccagtaattcttatcaaatgaaaaatgatcttcattcacaatgactgaccaaacttctgagtttccttcagttaatttcaaatcctgaggtcaaaatcaccaatgacttttgctctttggctttcaaagtgggacatatcatcaaatggtcccatatacacaaaatttacattatagacaaatacatatttgccatatgtttgatagcctcattcgttgattttatagatttaaaacaaccttaggctttttcttcagaatgtgtattctgatgtcgaatcagggatgaactccgactatatgccttcccacatttactacattcatagggtttctctgaagaatgacttctctgatgtcgaataaggtctgagccactgctaaatgccttcccacattcattacattcatagggtttctctccagtatgacttctttcatgtagaataagagatgtgcgctgactaaaggccttaccacatgttttgcatgtatatggcttctctccagtgtgaattctttcatgttgggcgaggtgtgcactctggctgaaggccttcccacactgatcacattcatagggtctatcttcagtatgaattctcttatgtcgtgtgagagatattcggtggctgaaggcttttccacattcctcacactggtagggtttttctccagtatgaattctttgatgttcaataagaaatgattggcggccgaaaactttactacatttattgcatttgaaaggtttctcttcagaatgaatattctgatgtattttaaggtttgcagttccagaaaacatcttcccacattccttacactcaaatagtttctttttctttgtatgaactttctgatgttgaataagggatgaatgccgattgcagaccttctcacatttattgcatctgtatagtttttctccattatgaattcttagatgcagaataagggttgaaagccgcctgaagaacttgtcacatttatcacatttgtacggtttctctgaagtgtgaattctctggtgaagcatcaggggtgaaatcctattaaataatttcccacattttctgcatttaaaaggattctctaaatggtgacttctttgctgtagactctgacttaaggccttcgcattttcagggattttctctccagcatgaattcttttatgtacaacaaagactgatttctttttgaagcctctcccacatttattatatttatgtgttttctttccattgtgaattttcttatgaagtaaaagggatgacatctgattgaaggcttttccgcactttctgcactggcagacattcccaacaacatgaattttctgatgtatattgaaagactgacattgactcaaggccttcccacagtcaagaatttcctttccatcatgaattctcatatgtagaataagggttgttctttgattgaagctttccccacatttattgcattcatggcttttctttccactgtgaattctctgatgaagtaggatggatgagatctgtctgaaagcttttctacaattactgcattcaaaaggcttctctcctgtatgaatgttctgatgaagtttaagagagaagcttcgactaaaggttttaccacagtcattacattttaaaggtttcttccctgaatgccctttcttaggttttactaggactgaatttttgttgcagccactctttcgtgtaggagctttttgttgtgcagaaactagtttctggcagatgctttgcccagatttgttgcattgatttggaggtaacttcttggtctcacatttagaccccgagtcaggagcccggcgtcttcttactggctctaccatccagggtgctttccctttctccaataaggtgatcacatttggtctccgaaaggaaagaccaagcgagaccaggttccggtaattctccaacatgacatcttcatacaaatccttctgaatggggctcagccattcccactcctcctgggagaagtagatggctaagtccccaaatgttataggtgccttggatttggatttcccccgtgcagaaggcatcctttcctccccctttagggtccacactgagagatgggcagagagctggtaaggcagggcagataagcagatcagttggctttccccttccaattacttaggtaaaatgacttgttccaggaagttgtaatgcattcatcccgcagttttcacaggtgtgtgcactcagccacgcaccccaaatttgagaagatgattcttgtctgatatggtctggctgtgtccccactcaaatctcatcttgaattatagctcccataatttccacgtgttgtgggagggacccggtgggagataactgaatcatgggggcggtttcccccatgctgttctcatggcagtgagtaagtctcatgtgatctgatggttctgtacagggactctcattctccctgtggccatgtaagacgtgtctttcaccttccatcacgattgtgaggcctccccagccacgtagaactgtgagtctgggtatgtctttatcagcagcacgaaaacagactcatacattgtccataaaataattttcttcaaggaactcggcactactcggtcttcccgggctcagaccccggcggcgaccaccgagacagccgagcagggactcagcgcctgcgcactcccctccgggaccccggg

SEQ ID NO: 14517 - RNA, 3740 nt, Homo sapiens
  source 1..3740: mol_type = other RNA
gctgggattacaggcatgagccaccgggctcagcctgatgtctcttcttataaaggcactaatcccatcacgagggctccaccctcatgacctcatctaatcctaattgcctcccaaatgcctcatttccaagtaacatcacattgatggtgaggattttaacataattagttttgggagggacataaacattcagtccataacaactcatattacaccacttattgcataccagtattgttacatgaaaataccaatgtttactcatataaatatagatgatttatttccaaataaaacaatactgatttctcctggctctgaaatcctcattcttcactatatcttggttcttttactgatagcttgtctcagccaagttagacgttcacaccatgaagatcatatatcctcatatccgtggagatggtaaagtaaggtttctactgttacacaccattatgagtgacaactttatctacctaaagactcacttttctttattctcacccacaagtttgtcagctgaaagtggcaccctgttttgccgagaagttccttatatttgataattctagatctgagaaacagactcaaattcttttttctgtgaccttaaatcaggctcagagccctataatggacttcacaattctattttgttgtatgtgaccaataaattatctttaaaactatgctggaagtaaaatatcggtaattttttttttttttgacacagagtcttgctctgttgcccagactggagtgcagtggtgcaatctctgctcggtgcaacccccacctcctgggttcaagcgattctcctgcctcagcctctccagtagctgagattacaggtgcgcaccaccacgcccagctaattttgtattttttagtagagacagggtttcaccgtggtctcaaactcttgacctcgtgatccgcctgtctcagcctcccaaagtgctggggttacaggtgtaagccactgcgcccagccagtaattcttatcaaatgaaaaatgatcttcattcacaatgactgaccaaacttctgagtttccttcagttaatttcaaatcctgaggtcaaaatcaccaatgacttttgctctttggctttcaaagtgggacatatcatcaaatggtcccatatacacaaaatttacattatagacaaatacatatttgccatatgtttgatagcctcattcgttgattttatagatttaaaacaaccttaggctttttcttcagaatgtgtattctgatgtcgaatcagggatgaactccgactatatgccttcccacatttactacattcatagggtttctctgaagaatgacttctctgatgtcgaataaggtctgagccactgctaaatgccttcccacattcattacattcatagggtttctctccagtatgacttctttcatgtagaataagagatgtgcgctgactaaaggccttaccacatgttttgcatgtatatggcttctctccagtgtgaattctttcatgttgggcgaggtgtgcactctggctgaaggccttcccacactgatcacattcatagggtctatcttcagtatgaattctcttatgtcgtgtgagagatattcggtggctgaaggcttttccacattcctcacactggtagggtttttctccagtatgaattctttgatgttcaataagaaatgattggcggccgaaaactttactacatttattgcatttgaaaggtttctcttcagaatgaatattctgatgtattttaaggtttgcagttccagaaaacatcttcccacattccttacactcaaatagtttctttttctttgtatgaactttctgatgttgaataagggatgaatgccgattgcagaccttctcacatttattgcatctgtatagtttttctccattatgaattcttagatgcagaataagggttgaaagccgcctgaagaacttgtcacatttatcacatttgtacggtttctctgaagtgtgaattctctggtgaagcatcaggggtgaaatcctattaaataatttcccacattttctgcatttaaaaggattctctaaatggtgacttctttgctgtagactctgacttaaggccttcgcattttcagggattttctctccagcatgaattcttttatgtacaacaaagactgatttctttttgaagcctctcccacatttattatatttatgtgttttctttccattgtgaattttcttatgaagtaaaagggatgacatctgattgaaggcttttccgcactttctgcactggcagacattcccaacaacatgaattttctgatgtatattgaaagactgacattgactcaaggccttcccacagtcaagaatttcctttccatcatgaattctcatatgtagaataagggttgttctttgattgaagctttccccacatttattgcattcatggcttttctttccactgtgaattctctgatgaagtaggatggatgagatctgtctgaaagcttttctacaattactgcattcaaaaggcttctctcctgtatgaatgttctgatgaagtttaagagagaagcttcgactaaaggttttaccacagtcattacattttaaaggtttcttccctgaatgccctttcttaggttttactaggactgaatttttgttgcagccactctttcgtgtaggagctttttgttgtgcagaaactagtttctggcagatgctttgcccagatttgttgcattgatttggaggtaacttcttggtctcacatttagaccccgagtcaggagcccggcgtcttcttactggctctaccatccagggtgctttccctttctccaataaggtgatcacatttggtctccgaaaggaaagaccaagcgagaccaggttccggtaattctccaacatgacatcttcatacaaatccttctgaatggggctcagccattcccactcctcctgggagaagtagatggctaagtccccaaatgttataggtgccttggatttggatttcccccgtgcagaaggcatcctttcctccccctttagggtccacactgagagatgggcagagagctggtaaggcagggcagataagcagatcagttggctttccccttccaattacttaggtaaaatgacttgttccaggaagttgtaatgcattcatcccgcagttttcacaggtgtgtgcactcagccacgcaccccaaatttgagaagatgattcttgtctgatatggtctggctgtgtccccactcaaatctcatcttgaattatagctcccataatttccacgtgttgtgggagggacccggtgggagataactgaatcatgggggcggtttcccccatgctgttctcatggcagtgagtaagtctcatgtgatctgatggttctgtacagggactctcattctccctgtggccatgtaagacgtgtctttcaccttccatcacgattgtgaggcctccccagccacgtagaactgtgagtctgggtatgtctttatcagcagcacgaaaacagactcatacattgtccataaaataattttcttcaaggaactcggcactactctccggcctcccccttccggctcctccacctcttccacctctgagacagtaagaccagctcctcctcttcctcctcagcctactcaacttgaaggccatgacgatgaaaaccactcta

SEQ ID NO: 14518 - RNA, 3689 nt, Homo sapiens
  source 1..3689: mol_type = other RNA
gctgggattacaggcatgagccaccgggctcagcctgatgtctcttcttataaaggcactaatcccatcacgagggctccaccctcatgacctcatctaatcctaattgcctcccaaatgcctcatttccaagtaacatcacattgatggtgaggattttaacataattagttttgggagggacataaacattcagtccataacaactcatattacaccacttattgcataccagtattgttacatgaaaataccaatgtttactcatataaatatagatgatttatttccaaataaaacaatactgatttctcctggctctgaaatcctcattcttcactatatcttggttcttttactgatagcttgtctcagccaagttagacgttcacaccatgaagatcatatatcctcatatccgtggagatggtaaagtaaggtttctactgttacacaccattatgagtgacaactttatctacctaaagactcacttttctttattctcacccacaagtttgtcagctgaaagtggcaccctgttttgccgagaagttccttatatttgataattctagatctgagaaacagactcaaattcttttttctgtgaccttaaatcaggctcagagccctataatggacttcacaattctattttgttgtatgtgaccaataaattatctttaaaactatgctggaagtaaaatatcggtaattttttttttttttgacacagagtcttgctctgttgcccagactggagtgcagtggtgcaatctctgctcggtgcaacccccacctcctgggttcaagcgattctcctgcctcagcctctccagtagctgagattacaggtgcgcaccaccacgcccagctaattttgtattttttagtagagacagggtttcaccgtggtctcaaactcttgacctcgtgatccgcctgtctcagcctcccaaagtgctggggttacaggtgtaagccactgcgcccagccagtaattcttatcaaatgaaaaatgatcttcattcacaatgactgaccaaacttctgagtttccttcagttaatttcaaatcctgaggtcaaaatcaccaatgacttttgctctttggctttcaaagtgggacatatcatcaaatggtcccatatacacaaaatttacattatagacaaatacatatttgccatatgtttgatagcctcattcgttgattttatagatttaaaacaaccttaggctttttcttcagaatgtgtattctgatgtcgaatcagggatgaactccgactatatgccttcccacatttactacattcatagggtttctctgaagaatgacttctctgatgtcgaataaggtctgagccactgctaaatgccttcccacattcattacattcatagggtttctctccagtatgacttctttcatgtagaataagagatgtgcgctgactaaaggccttaccacatgttttgcatgtatatggcttctctccagtgtgaattctttcatgttgggcgaggtgtgcactctggctgaaggccttcccacactgatcacattcatagggtctatcttcagtatgaattctcttatgtcgtgtgagagatattcggtggctgaaggcttttccacattcctcacactggtagggtttttctccagtatgaattctttgatgttcaataagaaatgattggcggccgaaaactttactacatttattgcatttgaaaggtttctcttcagaatgaatattctgatgtattttaaggtttgcagttccagaaaacatcttcccacattccttacactcaaatagtttctttttctttgtatgaactttctgatgttgaataagggatgaatgccgattgcagaccttctcacatttattgcatctgtatagtttttctccattatgaattcttagatgcagaataagggttgaaagccgcctgaagaacttgtcacatttatcacatttgtacggtttctctgaagtgtgaattctctggtgaagcatcaggggtgaaatcctattaaataatttcccacattttctgcatttaaaaggattctctaaatggtgacttctttgctgtagactctgacttaaggccttcgcattttcagggattttctctccagcatgaattcttttatgtacaacaaagactgatttctttttgaagcctctcccacatttattatatttatgtgttttctttccattgtgaattttcttatgaagtaaaagggatgacatctgattgaaggcttttccgcactttctgcactggcagacattcccaacaacatgaattttctgatgtatattgaaagactgacattgactcaaggccttcccacagtcaagaatttcctttccatcatgaattctcatatgtagaataagggttgttctttgattgaagctttccccacatttattgcattcatggcttttctttccactgtgaattctctgatgaagtaggatggatgagatctgtctgaaagcttttctacaattactgcattcaaaaggcttctctcctgtatgaatgttctgatgaagtttaagagagaagcttcgactaaaggttttaccacagtcattacattttaaaggtttcttccctgaatgccctttcttaggttttactaggactgaatttttgttgcagccactctttcgtgtaggagctttttgttgtgcagaaactagtttctggcagatgctttgcccagatttgttgcattgatttggaggtaacttcttggtctcacatttagaccccgagtcaggagcccggcgtcttcttactggctctaccatccagggtgctttccctttctccaataaggtgatcacatttggtctccgaaaggaaagaccaagcgagaccaggttccggtaattctccaacatgacatcttcatacaaatccttctgaatggggctcagccattcccactcctcctgggagaagtagatggctaagtccccaaatgttataggtgccttggatttggatttcccccgtgcagaaggcatcctttcctccccctttagggtccacactgagagatgggcagagagctggtaaggcagggcagataagcagatcagttggctttccccttccaattacttaggtaaaatgacttgttccaggaagttgtaatgcattcatcccgcagttttcacaggtgtgtgcactcagccacgcaccccaaatttgagaagatgattcttgtctgatatggtctggctgtgtccccactcaaatctcatcttgaattatagctcccataatttccacgtgttgtgggagggacccggtgggagataactgaatcatgggggcggtttcccccatgctgttctcatggcagtgagtaagtctcatgtgatctgatggttctgtacagggactctcattctccctgtggccatgtaagacgtgtctttcaccttccatcacgattgtgaggcctccccagccacgtagaactgtgagtctgggtatgtctttatcagcagcacgaaaacagactcatacattgtccataaaataattttcttcaaggaactcggcactcggtcttcccgggctcagaccccggcggcgaccaccgagacagccgagcagggactcagcgcctgcgcac

SEQ ID NO: 14519 - RNA, 3737 nt, Homo sapiens
  source 1..3737: mol_type = other RNA
gctgggattacaggcatgagccaccgggctcagcctgatgtctcttcttataaaggcactaatcccatcacgagggctccaccctcatgacctcatctaatcctaattgcctcccaaatgcctcatttccaagtaacatcacattgatggtgaggattttaacataattagttttgggagggacataaacattcagtccataacaactcatattacaccacttattgcataccagtattgttacatgaaaataccaatgtttactcatataaatatagatgatttatttccaaataaaacaatactgatttctcctggctctgaaatcctcattcttcactatatcttggttcttttactgatagcttgtctcagccaagttagacgttcacaccatgaagatcatatatcctcatatccgtggagatggtaaagtaaggtttctactgttacacaccattatgagtgacaactttatctacctaaagactcacttttctttattctcacccacaagtttgtcagctgaaagtggcaccctgttttgccgagaagttccttatatttgataattctagatctgagaaacagactcaaattcttttttctgtgaccttaaatcaggctcagagccctataatggacttcacaattctattttgttgtatgtgaccaataaattatctttaaaactatgctggaagtaaaatatcggtaattttttttttttttgacacagagtcttgctctgttgcccagactggagtgcagtggtgcaatctctgctcggtgcaacccccacctcctgggttcaagcgattctcctgcctcagcctctccagtagctgagattacaggtgcgcaccaccacgcccagctaattttgtattttttagtagagacagggtttcaccgtggtctcaaactcttgacctcgtgatccgcctgtctcagcctcccaaagtgctggggttacaggtgtaagccactgcgcccagccagtaattcttatcaaatgaaaaatgatcttcattcacaatgactgaccaaacttctgagtttccttcagttaatttcaaatcctgaggtcaaaatcaccaatgacttttgctctttggctttcaaagtgggacatatcatcaaatggtcccatatacacaaaatttacattatagacaaatacatatttgccatatgtttgatagcctcattcgttgattttatagatttaaaacaaccttaggctttttcttcagaatgtgtattctgatgtcgaatcagggatgaactccgactatatgccttcccacatttactacattcatagggtttctctgaagaatgacttctctgatgtcgaataaggtctgagccactgctaaatgccttcccacattcattacattcatagggtttctctccagtatgacttctttcatgtagaataagagatgtgcgctgactaaaggccttaccacatgttttgcatgtatatggcttctctccagtgtgaattctttcatgttgggcgaggtgtgcactctggctgaaggccttcccacactgatcacattcatagggtctatcttcagtatgaattctcttatgtcgtgtgagagatattcggtggctgaaggcttttccacattcctcacactggtagggtttttctccagtatgaattctttgatgttcaataagaaatgattggcggccgaaaactttactacatttattgcatttgaaaggtttctcttcagaatgaatattctgatgtattttaaggtttgcagttccagaaaacatcttcccacattccttacactcaaatagtttctttttctttgtatgaactttctgatgttgaataagggatgaatgccgattgcagaccttctcacatttattgcatctgtatagtttttctccattatgaattcttagatgcagaataagggttgaaagccgcctgaagaacttgtcacatttatcacatttgtacggtttctctgaagtgtgaattctctggtgaagcatcaggggtgaaatcctattaaataatttcccacattttctgcatttaaaaggattctctaaatggtgacttctttgctgtagactctgacttaaggccttcgcattttcagggattttctctccagcatgaattcttttatgtacaacaaagactgatttctttttgaagcctctcccacatttattatatttatgtgttttctttccattgtgaattttcttatgaagtaaaagggatgacatctgattgaaggcttttccgcactttctgcactggcagacattcccaacaacatgaattttctgatgtatattgaaagactgacattgactcaaggccttcccacagtcaagaatttcctttccatcatgaattctcatatgtagaataagggttgttctttgattgaagctttccccacatttattgcattcatggcttttctttccactgtgaattctctgatgaagtaggatggatgagatctgtctgaaagcttttctacaattactgcattcaaaaggcttctctcctgtatgaatgttctgatgaagtttaagagagaagcttcgactaaaggttttaccacagtcattacattttaaaggtttcttccctgaatgccctttcttaggttttactaggactgaatttttgttgcagccactctttcgtgtaggagctttttgttgtgcagaaactagtttctggcagatgctttgcccagatttgttgcattgatttggaggtaacttcttggtctcacatttagaccccgagtcaggagcccggcgtcttcttactggctctaccatccagggtgctttccctttctccaataaggtgatcacatttggtctccgaaaggaaagaccaagcgagaccaggttccggtaattctccaacatgacatcttcatacaaatccttctgaatggggctcagccattcccactcctcctgggagaagtagatggctaagtccccaaatgttataggtgccttggatttggatttcccccgtgcagaaggcatcctttcctccccctttagggtccacactgagagatgggcagagagctggtaaggcagggcagataagcagatcagttggctttccccttccaattacttaggtaaaatgacttgttccaggaagttgtaatgcattcatcccgcagttttcacaggtgtgtgcactcagccacgcaccccaaatttgagaagatgattcttgtctgatatggtctggctgtgtccccactcaaatctcatcttgaattatagctcccataatttccacgtgttgtgggagggacccggtgggagataactgaatcatgggggcggtttcccccatgctgttctcatggcagtgagtaagtctcatgtgatctgatggttctgtacagggactctcattctccctgtggccatgtaagacgtgtctttcaccttccatcacgattgtgaggcctccccagccacgtagaactgtgagtctgggtatgtctttatcagcagcacgaaaacagactcatacattgtccataaaataattttcttcaaggaactcggcactctccggcctcccccttccggctcctccacctcttccacctctgagacagtaagaccagctcctcctcttcctcctcagcctactcaacttgaaggccatgacgatgaaaaccactcta

SEQ ID NO: 14520 - RNA, 3217 nt, Homo sapiens
  source 1..3217: mol_type = other RNA
gctgggattacaggcatgagccaccgggctcagcctgatgtctcttcttataaaggcactaatcccatcacgagggctccaccctcatgacctcatctaatcctaattgcctcccaaatgcctcatttccaagtaacatcacattgatggtgaggattttaacataattagttttgggagggacataaacattcagtccataacaactcatattacaccacttattgcataccagtattgttacatgaaaataccaatgtttactcatataaatatagatgatttatttccaaataaaacaatactgatttctcctggctctgaaatcctcattcttcactatatcttggttcttttactgatagcttgtctcagccaagttagacgttcacaccatgaagatcatatatcctcatatccgtggagatggtaaagtaaggtttctactgttacacaccattatgagtgacaactttatctacctaaagactcacttttctttattctcacccacaagtttgtcagctgaaagtggcaccctgttttgccgagaagttccttatatttgataattctagatctgagaaacagactcaaattcttttttctgtgaccttaaatcaggctcagagccctataatggacttcacaattctattttgttgtatgtgaccaataaattatctttaaaactatgctggaagtaaaatatcggtaattttttttttttttgacacagagtcttgctctgttgcccagactggagtgcagtggtgcaatctctgctcggtgcaacccccacctcctgggttcaagcgattctcctgcctcagcctctccagtagctgagattacaggtgcgcaccaccacgcccagctaattttgtattttttagtagagacagggtttcaccgtggtctcaaactcttgacctcgtgatccgcctgtctcagcctcccaaagtgctggggttacaggtgtaagccactgcgcccagccagtaattcttatcaaatgaaaaatgatcttcattcacaatgactgaccaaacttctgagtttccttcagttaatttcaaatcctgaggtcaaaatcaccaatgacttttgctctttggctttcaaagtgggacatatcatcaaatggtcccatatacacaaaatttacattatagacaaatacatatttgccatatgtttgatagcctcattcgttgattttatagatttaaaacaaccttaggctttttcttcagaatgtgtattctgatgtcgaatcagggatgaactccgactatatgccttcccacatttactacattcatagggtttctctgaagaatgacttctctgatgtcgaataaggtctgagccactgctaaatgccttcccacattcattacattcatagggtttctctccagtatgacttctttcatgtagaataagagatgtgcgctgactaaaggccttaccacatgttttgcatgtatatggcttctctccagtgtgaattctttcatgttgggcgaggtgtgcactctggctgaaggccttcccacactgatcacattcatagggtctatcttcagtatgaattctcttatgtcgtgtgagagatattcggtggctgaaggcttttccacattcctcacactggtagggtttttctccagtatgaattctttgatgttcaataagaaatgattggcggccgaaaactttactacatttattgcatttgaaaggtttctcttcagaatgaatattctgatgtattttaaggtttgcagttccagaaaacatcttcccacattccttacactcaaatagtttctttttctttgtatgaactttctgatgttgaataagggatgaatgccgattgcagaccttctcacatttattgcatctgtatagtttttctccattatgaattcttagatgcagaataagggttgaaagccgcctgaagaacttgtcacatttatcacatttgtacggtttctctgaagtgtgaattctctggtgaagcatcaggggtgaaatcctattaaataatttcccacattttctgcatttaaaaggattctctaaatggtgacttctttgctgtagactctgacttaaggccttcgcattttcagggattttctctccagcatgaattcttttatgtacaacaaagactgatttctttttgaagcctctcccacatttattatatttatgtgttttctttccattgtgaattttcttatgaagtaaaagggatgacatctgattgaaggcttttccgcactttctgcactggcagacattcccaacaacatgaattttctgatgtatattgaaagactgacattgactcaaggccttcccacagtcaagaatttcctttccatcatgaattctcatatgtagaataagggttgttctttgattgaagctttccccacatttattgcattcatggcttttctttccactgtgaattctctgatgaagtaggatggatgagatctgtctgaaagcttttctacaattactgcattcaaaaggcttctctcctgtatgaatgttctgatgaagtttaagagagaagcttcgactaaaggttttaccacagtcattacattttaaaggtttcttccctgaatgccctttcttaggttttactaggactgaatttttgttgcagccactctttcgtgtaggagctttttgttgtgcagaaactagtttctggcagatgctttgcccagatttgttgcattgatttggaggtaacttcttggtctcacatttagaccccgagtcaggagcccggcgtcttcttactggctctaccatccagggtgctttccctttctccaataaggtgatcacatttggtctccgaaaggaaagaccaagcgagaccaggttccggtaattctccaacatgacatcttcatacaaatccttctgaatggggctcagccattcccactcctcctgggagaagtagatggctaagtccccaaatgttataggtgccttggatttggatttcccccgtgcagaaggcatcctttcctccccctttagggtccacactgagagatgggcagagagctggtaaggcagggccgcctctcggggacagtaccaccagccccggcctgaggccccgacccctcagcgccacacgcacaagcgcgttcgcacgattggt

SEQ ID NO: 14521 - RNA, 3386 nt, Homo sapiens
  source 1..3386: mol_type = other RNA
gctgggattacaggcatgagccaccgggctcagcctgatgtctcttcttataaaggcactaatcccatcacgagggctccaccctcatgacctcatctaatcctaattgcctcccaaatgcctcatttccaagtaacatcacattgatggtgaggattttaacataattagttttgggagggacataaacattcagtccataacaactcatattacaccacttattgcataccagtattgttacatgaaaataccaatgtttactcatataaatatagatgatttatttccaaataaaacaatactgatttctcctggctctgaaatcctcattcttcactatatcttggttcttttactgatagcttgtctcagccaagttagacgttcacaccatgaagatcatatatcctcatatccgtggagatggtaaagtaaggtttctactgttacacaccattatgagtgacaactttatctacctaaagactcacttttctttattctcacccacaagtttgtcagctgaaagtggcaccctgttttgccgagaagttccttatatttgataattctagatctgagaaacagactcaaattcttttttctgtgaccttaaatcaggctcagagccctataatggacttcacaattctattttgttgtatgtgaccaataaattatctttaaaactatgctggaagtaaaatatcggtaattttttttttttttgacacagagtcttgctctgttgcccagactggagtgcagtggtgcaatctctgctcggtgcaacccccacctcctgggttcaagcgattctcctgcctcagcctctccagtagctgagattacaggtgcgcaccaccacgcccagctaattttgtattttttagtagagacagggtttcaccgtggtctcaaactcttgacctcgtgatccgcctgtctcagcctcccaaagtgctggggttacaggtgtaagccactgcgcccagccagtaattcttatcaaatgaaaaatgatcttcattcacaatgactgaccaaacttctgagtttccttcagttaatttcaaatcctgaggtcaaaatcaccaatgacttttgctctttggctttcaaagtgggacatatcatcaaatggtcccatatacacaaaatttacattatagacaaatacatatttgccatatgtttgatagcctcattcgttgattttatagatttaaaacaaccttaggctttttcttcagaatgtgtattctgatgtcgaatcagggatgaactccgactatatgccttcccacatttactacattcatagggtttctctgaagaatgacttctctgatgtcgaataaggtctgagccactgctaaatgccttcccacattcattacattcatagggtttctctccagtatgacttctttcatgtagaataagagatgtgcgctgactaaaggccttaccacatgttttgcatgtatatggcttctctccagtgtgaattctttcatgttgggcgaggtgtgcactctggctgaaggccttcccacactgatcacattcatagggtctatcttcagtatgaattctcttatgtcgtgtgagagatattcggtggctgaaggcttttccacattcctcacactggtagggtttttctccagtatgaattctttgatgttcaataagaaatgattggcggccgaaaactttactacatttattgcatttgaaaggtttctcttcagaatgaatattctgatgtattttaaggtttgcagttccagaaaacatcttcccacattccttacactcaaatagtttctttttctttgtatgaactttctgatgttgaataagggatgaatgccgattgcagaccttctcacatttattgcatctgtatagtttttctccattatgaattcttagatgcagaataagggttgaaagccgcctgaagaacttgtcacatttatcacatttgtacggtttctctgaagtgtgaattctctggtgaagcatcaggggtgaaatcctattaaataatttcccacattttctgcatttaaaaggattctctaaatggtgacttctttgctgtagactctgacttaaggccttcgcattttcagggattttctctccagcatgaattcttttatgtacaacaaagactgatttctttttgaagcctctcccacatttattatatttatgtgttttctttccattgtgaattttcttatgaagtaaaagggatgacatctgattgaaggcttttccgcactttctgcactggcagacattcccaacaacatgaattttctgatgtatattgaaagactgacattgactcaaggccttcccacagtcaagaatttcctttccatcatgaattctcatatgtagaataagggttgttctttgattgaagctttccccacatttattgcattcatggcttttctttccactgtgaattctctgatgaagtaggatggatgagatctgtctgaaagcttttctacaattactgcattcaaaaggcttctctcctgtatgaatgttctgatgaagtttaagagagaagcttcgactaaaggttttaccacagtcattacattttaaaggtttcttccctgaatgccctttcttaggttttactaggactgaatttttgttgcagccactctttcgtgtaggagctttttgttgtgcagaaactagtttctggcagatgctttgcccagatttgttgcattgatttggaggtaacttcttggtctcacatttagaccccgagtcaggagcccggcgtcttcttactggctctaccatccagggtgctttccctttctccaataaggtgatcacatttggtctccgaaaggaaagaccaagcgagaccaggttccggtaattctccaacatgacatcttcatacaaatccttctgaatggggctcagccattcccactcctcctgggagaagtagatggctaagtccccaaatgttataggtgccttggatttggatttcccccgtgcagaaggcatcctttcctccccctttagggtccacactgagagatgggcagagagctggtaaggcagggcggtctcctaggggactggcgcctggccctgcttttcatcctctcaggagatcacgtgtggacactgaggcccttcctcgagctctttaaccaaacccaacctccccaattcgccgccttccccgctcccacaaccacacgttcccgtgtgagggcttattgcctccagccagccagcgtccttcgcccccacattcacgaggtttggagccggcctcacccgcggaggcggacaccgcccacccgcgcgtgcgc

SEQ ID NO: 14522 - RNA, 3205 nt, Homo sapiens
  source 1..3205: mol_type = other RNA
gctgggattacaggcatgagccaccgggctcagcctgatgtctcttcttataaaggcactaatcccatcacgagggctccaccctcatgacctcatctaatcctaattgcctcccaaatgcctcatttccaagtaacatcacattgatggtgaggattttaacataattagttttgggagggacataaacattcagtccataacaactcatattacaccacttattgcataccagtattgttacatgaaaataccaatgtttactcatataaatatagatgatttatttccaaataaaacaatactgatttctcctggctctgaaatcctcattcttcactatatcttggttcttttactgatagcttgtctcagccaagttagacgttcacaccatgaagatcatatatcctcatatccgtggagatggtaaagtaaggtttctactgttacacaccattatgagtgacaactttatctacctaaagactcacttttctttattctcacccacaagtttgtcagctgaaagtggcaccctgttttgccgagaagttccttatatttgataattctagatctgagaaacagactcaaattcttttttctgtgaccttaaatcaggctcagagccctataatggacttcacaattctattttgttgtatgtgaccaataaattatctttaaaactatgctggaagtaaaatatcggtaattttttttttttttgacacagagtcttgctctgttgcccagactggagtgcagtggtgcaatctctgctcggtgcaacccccacctcctgggttcaagcgattctcctgcctcagcctctccagtagctgagattacaggtgcgcaccaccacgcccagctaattttgtattttttagtagagacagggtttcaccgtggtctcaaactcttgacctcgtgatccgcctgtctcagcctcccaaagtgctggggttacaggtgtaagccactgcgcccagccagtaattcttatcaaatgaaaaatgatcttcattcacaatgactgaccaaacttctgagtttccttcagttaatttcaaatcctgaggtcaaaatcaccaatgacttttgctctttggctttcaaagtgggacatatcatcaaatggtcccatatacacaaaatttacattatagacaaatacatatttgccatatgtttgatagcctcattcgttgattttatagatttaaaacaaccttaggctttttcttcagaatgtgtattctgatgtcgaatcagggatgaactccgactatatgccttcccacatttactacattcatagggtttctctgaagaatgacttctctgatgtcgaataaggtctgagccactgctaaatgccttcccacattcattacattcatagggtttctctccagtatgacttctttcatgtagaataagagatgtgcgctgactaaaggccttaccacatgttttgcatgtatatggcttctctccagtgtgaattctttcatgttgggcgaggtgtgcactctggctgaaggccttcccacactgatcacattcatagggtctatcttcagtatgaattctcttatgtcgtgtgagagatattcggtggctgaaggcttttccacattcctcacactggtagggtttttctccagtatgaattctttgatgttcaataagaaatgattggcggccgaaaactttactacatttattgcatttgaaaggtttctcttcagaatgaatattctgatgtattttaaggtttgcagttccagaaaacatcttcccacattccttacactcaaatagtttctttttctttgtatgaactttctgatgttgaataagggatgaatgccgattgcagaccttctcacatttattgcatctgtatagtttttctccattatgaattcttagatgcagaataagggttgaaagccgcctgaagaacttgtcacatttatcacatttgtacggtttctctgaagtgtgaattctctggtgaagcatcaggggtgaaatcctattaaataatttcccacattttctgcatttaaaaggattctctaaatggtgacttctttgctgtagactctgacttaaggccttcgcattttcagggattttctctccagcatgaattcttttatgtacaacaaagactgatttctttttgaagcctctcccacatttattatatttatgtgttttctttccattgtgaattttcttatgaagtaaaagggatgacatctgattgaaggcttttccgcactttctgcactggcagacattcccaacaacatgaattttctgatgtatattgaaagactgacattgactcaaggccttcccacagtcaagaatttcctttccatcatgaattctcatatgtagaataagggttgttctttgattgaagctttccccacatttattgcattcatggcttttctttccactgtgaattctctgatgaagtaggatggatgagatctgtctgaaagcttttctacaattactgcattcaaaaggcttctctcctgtatgaatgttctgatgaagtttaagagagaagcttcgactaaaggttttaccacagtcattacattttaaaggtttcttccctgaatgccctttcttaggttttactaggactgaatttttgttgcagccactctttcgtgtaggagctttttgttgtgcagaaactagtttctggcagatgctttgcccagatttgttgcattgatttggaggtaacttcttggtctcacatttagaccccgagtcaggagcccggcgtcttcttactggctctaccatccagggtgctttccctttctccaataaggtgatcacatttggtctccgaaaggaaagaccaagcgagaccaggttccggtaattctccaacatgacatcttcatacaaatccttctgaatggggctcagccattcccactcctcctgggagaagtagatggctaagtccccaaatgttataggtgccttggatttggatttcccccgtgcagaaggcatcctttcctccccctttagggtccacactgagagatgggcagagagctggtaaggcagggctcggtcttcccgggctcagaccccggcggcgaccaccgagacagccgagcagggactcagcgcctgcgcactc

SEQ ID NO: 14523 - RNA, 3164 nt, Homo sapiens
  source 1..3164: mol_type = other RNA
gctgggattacaggcatgagccaccgggctcagcctgatgtctcttcttataaaggcactaatcccatcacgagggctccaccctcatgacctcatctaatcctaattgcctcccaaatgcctcatttccaagtaacatcacattgatggtgaggattttaacataattagttttgggagggacataaacattcagtccataacaactcatattacaccacttattgcataccagtattgttacatgaaaataccaatgtttactcatataaatatagatgatttatttccaaataaaacaatactgatttctcctggctctgaaatcctcattcttcactatatcttggttcttttactgatagcttgtctcagccaagttagacgttcacaccatgaagatcatatatcctcatatccgtggagatggtaaagtaaggtttctactgttacacaccattatgagtgacaactttatctacctaaagactcacttttctttattctcacccacaagtttgtcagctgaaagtggcaccctgttttgccgagaagttccttatatttgataattctagatctgagaaacagactcaaattcttttttctgtgaccttaaatcaggctcagagccctataatggacttcacaattctattttgttgtatgtgaccaataaattatctttaaaactatgctggaagtaaaatatcggtaattttttttttttttgacacagagtcttgctctgttgcccagactggagtgcagtggtgcaatctctgctcggtgcaacccccacctcctgggttcaagcgattctcctgcctcagcctctccagtagctgagattacaggtgcgcaccaccacgcccagctaattttgtattttttagtagagacagggtttcaccgtggtctcaaactcttgacctcgtgatccgcctgtctcagcctcccaaagtgctggggttacaggtgtaagccactgcgcccagccagtaattcttatcaaatgaaaaatgatcttcattcacaatgactgaccaaacttctgagtttccttcagttaatttcaaatcctgaggtcaaaatcaccaatgacttttgctctttggctttcaaagtgggacatatcatcaaatggtcccatatacacaaaatttacattatagacaaatacatatttgccatatgtttgatagcctcattcgttgattttatagatttaaaacaaccttaggctttttcttcagaatgtgtattctgatgtcgaatcagggatgaactccgactatatgccttcccacatttactacattcatagggtttctctgaagaatgacttctctgatgtcgaataaggtctgagccactgctaaatgccttcccacattcattacattcatagggtttctctccagtatgacttctttcatgtagaataagagatgtgcgctgactaaaggccttaccacatgttttgcatgtatatggcttctctccagtgtgaattctttcatgttgggcgaggtgtgcactctggctgaaggccttcccacactgatcacattcatagggtctatcttcagtatgaattctcttatgtcgtgtgagagatattcggtggctgaaggcttttccacattcctcacactggtagggtttttctccagtatgaattctttgatgttcaataagaaatgattggcggccgaaaactttactacatttattgcatttgaaaggtttctcttcagaatgaatattctgatgtattttaaggtttgcagttccagaaaacatcttcccacattccttacactcaaatagtttctttttctttgtatgaactttctgatgttgaataagggatgaatgccgattgcagaccttctcacatttattgcatctgtatagtttttctccattatgaattcttagatgcagaataagggttgaaagccgcctgaagaacttgtcacatttatcacatttgtacggtttctctgaagtgtgaattctctggtgaagcatcaggggtgaaatcctattaaataatttcccacattttctgcatttaaaaggattctctaaatggtgacttctttgctgtagactctgacttaaggccttcgcattttcagggattttctctccagcatgaattcttttatgtacaacaaagactgatttctttttgaagcctctcccacatttattatatttatgtgttttctttccattgtgaattttcttatgaagtaaaagggatgacatctgattgaaggcttttccgcactttctgcactggcagacattcccaacaacatgaattttctgatgtatattgaaagactgacattgactcaaggccttcccacagtcaagaatttcctttccatcatgaattctcatatgtagaataagggttgttctttgattgaagctttccccacatttattgcattcatggcttttctttccactgtgaattctctgatgaagtaggatggatgagatctgtctgaaagcttttctacaattactgcattcaaaaggcttctctcctgtatgaatgttctgatgaagtttaagagagaagcttcgactaaaggttttaccacagtcattacattttaaaggtttcttccctgaatgccctttcttaggttttactaggactgaatttttgttgcagccactctttcgtgtaggagctttttgttgtgcagaaactagtttctggcagatgctttgcccagatttgttgcattgatttggaggtaacttcttggtctcacatttagaccccgagtcaggagcccggcgtcttcttactggctctaccatccagggtgctttccctttctccaataaggtgatcacatttggtctccgaaaggaaagaccaagcgagaccaggttccggtaattctccaacatgacatcttcatacaaatccttctgaatggggctcagccattcccactcctcctgggagaagtagatggctaagtccccaaatgttataggtgccttggatttggatttcccccgtgcagaaggcatcctttcctccccctttagggtccacactgagagatgggcagagagctggtaaggcagggctgcacgttttgcgaagaggcccacagtccttt

SEQ ID NO: 14524 - RNA, 3174 nt, Homo sapiens
  source 1..3174: mol_type = other RNA
gctgggattacaggcatgagccaccgggctcagcctgatgtctcttcttataaaggcactaatcccatcacgagggctccaccctcatgacctcatctaatcctaattgcctcccaaatgcctcatttccaagtaacatcacattgatggtgaggattttaacataattagttttgggagggacataaacattcagtccataacaactcatattacaccacttattgcataccagtattgttacatgaaaataccaatgtttactcatataaatatagatgatttatttccaaataaaacaatactgatttctcctggctctgaaatcctcattcttcactatatcttggttcttttactgatagcttgtctcagccaagttagacgttcacaccatgaagatcatatatcctcatatccgtggagatggtaaagtaaggtttctactgttacacaccattatgagtgacaactttatctacctaaagactcacttttctttattctcacccacaagtttgtcagctgaaagtggcaccctgttttgccgagaagttccttatatttgataattctagatctgagaaacagactcaaattcttttttctgtgaccttaaatcaggctcagagccctataatggacttcacaattctattttgttgtatgtgaccaataaattatctttaaaactatgctggaagtaaaatatcggtaattttttttttttttgacacagagtcttgctctgttgcccagactggagtgcagtggtgcaatctctgctcggtgcaacccccacctcctgggttcaagcgattctcctgcctcagcctctccagtagctgagattacaggtgcgcaccaccacgcccagctaattttgtattttttagtagagacagggtttcaccgtggtctcaaactcttgacctcgtgatccgcctgtctcagcctcccaaagtgctggggttacaggtgtaagccactgcgcccagccagtaattcttatcaaatgaaaaatgatcttcattcacaatgactgaccaaacttctgagtttccttcagttaatttcaaatcctgaggtcaaaatcaccaatgacttttgctctttggctttcaaagtgggacatatcatcaaatggtcccatatacacaaaatttacattatagacaaatacatatttgccatatgtttgatagcctcattcgttgattttatagatttaaaacaaccttaggctttttcttcagaatgtgtattctgatgtcgaatcagggatgaactccgactatatgccttcccacatttactacattcatagggtttctctgaagaatgacttctctgatgtcgaataaggtctgagccactgctaaatgccttcccacattcattacattcatagggtttctctccagtatgacttctttcatgtagaataagagatgtgcgctgactaaaggccttaccacatgttttgcatgtatatggcttctctccagtgtgaattctttcatgttgggcgaggtgtgcactctggctgaaggccttcccacactgatcacattcatagggtctatcttcagtatgaattctcttatgtcgtgtgagagatattcggtggctgaaggcttttccacattcctcacactggtagggtttttctccagtatgaattctttgatgttcaataagaaatgattggcggccgaaaactttactacatttattgcatttgaaaggtttctcttcagaatgaatattctgatgtattttaaggtttgcagttccagaaaacatcttcccacattccttacactcaaatagtttctttttctttgtatgaactttctgatgttgaataagggatgaatgccgattgcagaccttctcacatttattgcatctgtatagtttttctccattatgaattcttagatgcagaataagggttgaaagccgcctgaagaacttgtcacatttatcacatttgtacggtttctctgaagtgtgaattctctggtgaagcatcaggggtgaaatcctattaaataatttcccacattttctgcatttaaaaggattctctaaatggtgacttctttgctgtagactctgacttaaggccttcgcattttcagggattttctctccagcatgaattcttttatgtacaacaaagactgatttctttttgaagcctctcccacatttattatatttatgtgttttctttccattgtgaattttcttatgaagtaaaagggatgacatctgattgaaggcttttccgcactttctgcactggcagacattcccaacaacatgaattttctgatgtatattgaaagactgacattgactcaaggccttcccacagtcaagaatttcctttccatcatgaattctcatatgtagaataagggttgttctttgattgaagctttccccacatttattgcattcatggcttttctttccactgtgaattctctgatgaagtaggatggatgagatctgtctgaaagcttttctacaattactgcattcaaaaggcttctctcctgtatgaatgttctgatgaagtttaagagagaagcttcgactaaaggttttaccacagtcattacattttaaaggtttcttccctgaatgccctttcttaggttttactaggactgaatttttgttgcagccactctttcgtgtaggagctttttgttgtgcagaaactagtttctggcagatgctttgcccagatttgttgcattgatttggaggtaacttcttggtctcacatttagaccccgagtcaggagcccggcgtcttcttactggctctaccatccagggtgctttccctttctccaataaggtgatcacatttggtctccgaaaggaaagaccaagcgagaccaggttccggtaattctccaacatgacatcttcatacaaatccttctgaatggggctcagccattcccactcctcctgggagaagtagatggctaagtccccaaatgttataggtgccttggatttggatttcccccgtgcagaaggcatcctttcctccccctttagggtccacactgagagatgggcagagagctggtaaggcagggtaggtagctttgcagaaatccggggaagatgttggtggcatga

SEQ ID NO: 14525 - RNA, 3306 nt, Homo sapiens
  source 1..3306: mol_type = other RNA
gctgggattacaggcatgagccaccgggctcagcctgatgtctcttcttataaaggcactaatcccatcacgagggctccaccctcatgacctcatctaatcctaattgcctcccaaatgcctcatttccaagtaacatcacattgatggtgaggattttaacataattagttttgggagggacataaacattcagtccataacaactcatattacaccacttattgcataccagtattgttacatgaaaataccaatgtttactcatataaatatagatgatttatttccaaataaaacaatactgatttctcctggctctgaaatcctcattcttcactatatcttggttcttttactgatagcttgtctcagccaagttagacgttcacaccatgaagatcatatatcctcatatccgtggagatggtaaagtaaggtttctactgttacacaccattatgagtgacaactttatctacctaaagactcacttttctttattctcacccacaagtttgtcagctgaaagtggcaccctgttttgccgagaagttccttatatttgataattctagatctgagaaacagactcaaattcttttttctgtgaccttaaatcaggctcagagccctataatggacttcacaattctattttgttgtatgtgaccaataaattatctttaaaactatgctggaagtaaaatatcggtaattttttttttttttgacacagagtcttgctctgttgcccagactggagtgcagtggtgcaatctctgctcggtgcaacccccacctcctgggttcaagcgattctcctgcctcagcctctccagtagctgagattacaggtgcgcaccaccacgcccagctaattttgtattttttagtagagacagggtttcaccgtggtctcaaactcttgacctcgtgatccgcctgtctcagcctcccaaagtgctggggttacaggtgtaagccactgcgcccagccagtaattcttatcaaatgaaaaatgatcttcattcacaatgactgaccaaacttctgagtttccttcagttaatttcaaatcctgaggtcaaaatcaccaatgacttttgctctttggctttcaaagtgggacatatcatcaaatggtcccatatacacaaaatttacattatagacaaatacatatttgccatatgtttgatagcctcattcgttgattttatagatttaaaacaaccttaggctttttcttcagaatgtgtattctgatgtcgaatcagggatgaactccgactatatgccttcccacatttactacattcatagggtttctctgaagaatgacttctctgatgtcgaataaggtctgagccactgctaaatgccttcccacattcattacattcatagggtttctctccagtatgacttctttcatgtagaataagagatgtgcgctgactaaaggccttaccacatgttttgcatgtatatggcttctctccagtgtgaattctttcatgttgggcgaggtgtgcactctggctgaaggccttcccacactgatcacattcatagggtctatcttcagtatgaattctcttatgtcgtgtgagagatattcggtggctgaaggcttttccacattcctcacactggtagggtttttctccagtatgaattctttgatgttcaataagaaatgattggcggccgaaaactttactacatttattgcatttgaaaggtttctcttcagaatgaatattctgatgtattttaaggtttgcagttccagaaaacatcttcccacattccttacactcaaatagtttctttttctttgtatgaactttctgatgttgaataagggatgaatgccgattgcagaccttctcacatttattgcatctgtatagtttttctccattatgaattcttagatgcagaataagggttgaaagccgcctgaagaacttgtcacatttatcacatttgtacggtttctctgaagtgtgaattctctggtgaagcatcaggggtgaaatcctattaaataatttcccacattttctgcatttaaaaggattctctaaatggtgacttctttgctgtagactctgacttaaggccttcgcattttcagggattttctctccagcatgaattcttttatgtacaacaaagactgatttctttttgaagcctctcccacatttattatatttatgtgttttctttccattgtgaattttcttatgaagtaaaagggatgacatctgattgaaggcttttccgcactttctgcactggcagacattcccaacaacatgaattttctgatgtatattgaaagactgacattgactcaaggccttcccacagtcaagaatttcctttccatcatgaattctcatatgtagaataagggttgttctttgattgaagctttccccacatttattgcattcatggcttttctttccactgtgaattctctgatgaagtaggatggatgagatctgtctgaaagcttttctacaattactgcattcaaaaggcttctctcctgtatgaatgttctgatgaagtttaagagagaagcttcgactaaaggttttaccacagtcattacattttaaaggtttcttccctgaatgccctttcttaggttttactaggactgaatttttgttgcagccactctttcgtgtaggagctttttgttgtgcagaaactagtttctggcagatgctttgcccagatttgttgcattgatttggaggtaacttcttggtctcacatttagaccccgagtctgtaatcccagccgctcgggaggctgaggcacgagaattgcttgaacccaggaggcggaggttgcagtgagccgagatcatgccatcattgtagtccagccaggagcccggcgtcttcttactggctctaccatccagggtgctttccctttctccaataaggtgatcacatttggtctccgaaaggaaagaccaagcgagaccaggttccggtaattctccaacatgacatcttcatacaaatccttctgaatggggctcagccattcccactcctcctgggagaagtagatggctaagtccccaaatgttataggtgccttggatttggatttcccccgtgcagaaggcatcctttcctccccctttagggtccacactgagagatgggcagagagctggtaaggcagggctcggtcttcccgggctcagaccccggcggcgaccaccgagacagccgagcagggactcagcgcctgcgcactc

SEQ ID NO: 14526 - RNA, 6549 nt, Homo sapiens
  source 1..6549: mol_type = other RNA
gctgggattacaggcatgagccaccgtacccagccaatttttctgtctttacttaatggttacttttgctgaacatcaaaaagtgggtaatttttgcaaaaatatctaaagacttcagcagttttcccaagagcctctcttcaacatttgatattaaaacgcttctttttggaagctcccatctcatcatcatccttgtttatttacctctgattcagctgctaaccggtctaactctgctccatgctcttttatcaatagttgaagtgtattttagcagttctgtgacacctctcttacctccttcacagaatcctgaatgtttgtcaagatcatcaattaaagttcgaggacagtttgcacattgactctcaggcatcacaagactgatccacaaaactgtagatgaggcagtgagagagactctggtgctaagcagggggaggcctgatggtacccattttataagtgatacatttgctaatgttttcatatcaaggattttttttcccatataaccttgcaaagttaaacagtcaaatgttaggttaaagagaaaagaagcttcttgtttgtggaatcaagcaagcaaatacttgattgctcccacctcctcctttcttcacttctaccacccactcctcaccatctcattcagcagcctgaacagctgggtgtcttgtcttgtgctgctcctctccatgagaaaaagcacaggaaaaagtatgtatggcttgatgtgttttcctttccagaagtgattcctaatttaagaagaggttgagtaaaaagacaaatttcaacctaacagaactactcttctaatggtgaaattctagggatgcccgtaaagcatcttctaagtgctccttaaacaactccatgaaggcagccaacgatcccatctccatctccatcagtcactggagctgtgaggcacaaagagaggggatggctgctggtggctctccagttgctcatctcagtgcatacaatgctgtctccagagaaacaaccagtatgtgtggcagggagcaggctagtcaaggccagtggtgctgttcaccaaccctcctccatcctgattcctgaaaattctgtcctccgttatcctggactgaaattgatggtgcaggacagagagggagaattgctggcgaaatgccatcgggcaggcaacaggggaaggggttggagcatcttagccagggtatcaccttagccagggaggggcatagtgagttccccctgagcacacaggggagaggctgatatgaagaagatggagctaggtcagcagaggggacagcggggatgtctggaagagttcttccggttgcttctattccccttgtgtaaaggggagccagccatcatttgctgagagtgaggaagggaaagatgtggaaagtctgggaaagaaaaggtatggcacggttatccaggaactcagcttccagaggctctcctgagtctctaatgcttgagctggacgtagatggataaatggagtttgctagattaaaaaaaggtagagcagtctgtgcaaagggaatagcatagcaagggggacagggtgaccagcggtgtacttcactgaaaaaagaataggggcaggcccggcgcagtggctcactcctgtaatcccagctacttgggaggctgaggcaggagaattgcttgaacctgggaggtggaggttgcagtgagccgaaatcacgccaccgcactccagctggggcaacagagcaagactctgtctcaaaaaaaaaaaaaaaaaaaaaaaaggaaaagaaaagaaaagaaaaaagaaacggtggggaaatgaatgggttacaagcacctgcaggacattgggtcaaaaagtccattagatgattggacacacaggactggagcccagcaaagggttctggtcagcaaatgtctatttgaggttcattaataagcaggtgattatggatcaggatccagggagatttctcagaaagaggagagcagaggcccagccactgaattatggaaaatgtgtccatttaagggaggagcagtagaagagggaggaaagaagtgagaagattccaatcaggaagataggattcaaaaagagagctggagaaaaatgtagcaaactagaatccaagaaaagagataatttcaggaagactgtgggtattaaatgccacaaaaggcataggtagaaaacagcccatcagatttgacactgtggaagttactcaccttcctatctggaccaatctctctatgatggtcaggctgcaagacaaatggcaggatgttgaggggtgaattgtggcaagagtcaggacagtgagtgtggaagagcctttccagaaggtggtttggaaggaagggagggaggggagatagaaactggaaagggctgtggggcaaggaatggcttctggttaggtggaagcaatttgagtctatttatatgtacaaaggaaacagcccagagaggggtgcagtggattcgaccaacacagcaaataagctggggctacagcagtgagcaaagctacgtccctgccctcaaggagcttatagtctagcgtgaagagacagagaacgagcaaataagcaaatcgatatatggcatgatgagtgctgaggagaaaccccagtgggcaggggagggaacagaagaggctgcatgcaatatgggggtggcaggaagagcccctgctgtggtgacctctgccacacaattttgttcctaacacttgtcaaacaaacttgtgtgcagcctggtgttgtagttatgcggtgtctctttctcctatgacatagacagcggcttccgcttccccgtctttgccttgtccacatcatggtgttctgcagagaaggctgtgcatgaatctttgtagtaggaatgctacaaacccttcccgttcagttaggacaggcattatccaaacaatctcctccccatccccaaggaattctcggaagtggcacctagtaacctacaatgacttaggcaaattgtctgaatgcctaaaggatacaaatgatttagtattctctacatatttgcaaatttacttaaatcttcttgttatagttttaaccttacagttcactttgggaatgggtttgggggaagacagaaagaaattagtctttataaccctgccaaactctgaatcctacctcctacctcttggtaaggcatcattttaaaaggttagaataatttttatattcattatcacattcgatttccccactttatctgcagaaaaacaataaataggggcttcctattagttcaccatattttccttaggtagaaattccttgtatctgatagtctttagggtcctctttgagactaagatccccttagagatgagacgaggttggccccctttccctaccccagaggccagcacacagcacacacaggagaggacaggaaacagaggggagttgctctgatctccatattctgttctttcccagggaaaatgctctgttttcaaccaaaaacaagatcattctaaatgtcattgctccacaccccatctgggctcctgaaagcaaagctgccttgtttctgaatcagatgttgtcacccactgaaaagcctcctgcatccaagcttggctggcagtggggtccttgctcgaggggacagactcctctcccccagcgaagctgccccacatcatttcttttgagaaaggaagaggatggggaaggacaagcagcaacagagaacaattacatcactgcctctctgaccttttaaagagcaaatggttaaaataaatactatcgggctcatttctatggacttgaacattttacaacctgtagaatcatgtgacatattgcccttttgtggaactcctagaagggacagaaggaaataaacatagctatgcgacgggcttcacagctaaaacccaggacgtgcagtgtctggagggcaactcatggcaggcaagaggcagagccccccctggagtgctgagtaaagattctgaggaagtcatgcaaggatctgtcatgagcaaaaatatcagagtcctccaggatgtgaccacattttcattagcccttgccactgagcctccttccaggtgtgatgaaaaaaaaaaaaaaagcctcaggaggagaggaggcagacaggtgcagagacccgcacttggctgcaggtgagaactctggctacaaataacccacctcttcatgggggaggaaggtcccagtcacccccaggaagtcataaattcaactccattcgtaaaaatgtttatgcaatcaaaggatttcaaaacacagactttcatttcatctagtattcccacagagggaaggggagccatgagaaactcctctactggtggccaaatgtatttcttcacaacctgaaatgatgcactagcacatggcttgttagatcataacatccgcgatgtttttcaatagaggtgtaatgccatgaaatgctttcatgctgcaagcaaaaagaagaccttcgtaaatttacattcaacatgtaaaaacacataataacttctgtacatgatagagctgtgtgtgtgtgtgtgtgtgtgtgtgtgtgtgtgtgctttacaaaacaaaaatttatatcttgtctaccattgaagggagtgaggagagactgatatttgttgaacatccacaatgtgccaggtgctttacaagcctcatcttctcatttcatcttcacagcagaccaaggaggtatagactattgccgcaaccattttatgagtgagaaaatgaggctctgagaggtttaacaacttgcctgaggtcacacaggaagcgacccttgttcttcctgctacatcaagctgcctcctcaagttccaacaaatagttttgttaccttgtcccgtacacatctgtaaatcttcctgcaaaagtcatttttatggttcatggtaagatgctgccaaaagagctgaaagaaatagagtctttgtcaagtacagaaatgacaggtcatttccagaagatacagtacaagagttcaatttcatcattaattagtatctcatgcatatgggatgagatgttcttctgtatcacatttaggagatacttaagtcatattccaagcacaaactaaaaatgacctgtgttccaccatttttatccacaacttccctcacagttcttagacgacagtctcaactgtgaccgtattacaattgtctttctggcgccgaggttgcatttcatctttgaaagccctggtcagaacaacttttaaggactccttgaatctcttcttcttactgcttcccacaaagaagtaaatgaaagggttggcgctactgttgattgtggagaagagcagggaaatgtggtgtaggttcccaaaggtcgaccaatactcatagtacagcaggtaaaggagtctcatgggcatagcgaagatgaggaatataatgatggtgaccatgatgactatgtaaagcttggaggaatgggaagcccacgtgttcttccggatcttcacgaccaagatggtgctggacaccagcatgaggggcgtgaagaccaggaagctcaggatggctataaagatgatgactgctcggcagtcattccgagagtgactctcttcttctctgtcgatgcacatgacatactccatggtggtcaccaagcaagaaagagcccacagaagggcacagaccaatgccgactggtacttggggcgatggcatcggtaccagatggggtaaaggactgacaggcacctctccacactaatggccgtcagcagatagaggcccgtgttgtagccaaacagaaaagtcactgataatgtgacaattgtgtagtaatggccagaagaaagctcataatctaaagcatagtcgatagacaagatgaaaatacagaagagcagtgagatgtctgcgatagacaggtgggtgatgtagacagtgaagggatttcttctcatccggaagcacaggaaccagaggagaatcccattctcaacaaaccccactggggagatgctcataatgacccagtgcacgatggggatttgccgatgtgcattcccgactgaggcgttcctgccagttgagatgttcgtgggttcctcaacaacaaatgatgtcacgtttgacccatccatgaggaggcctcaggttggaactcttcaggtaattttctggcagtgacagcctggggtggagggatagctcatcctgacagccctcagtggcccctggagtggtcagttacactgcaatggaaacctcagttgggaacagattgcaaagacagccaaggaggtgacagcaccacgactggtcagcattactggcagcatcacagagcatcttccctcctctctttcttctcacgaaagagatgttggtgtcatttgctcaggaagggtcagacgtggccaacaggttggctgccccttcacatctggggcatcaatgcccagccagcctgcagggtctccggtcccaacatctcgaaggatggctgcagcctctcatctctgaaggaatc

SEQ ID NO: 14527 - RNA, 6392 nt, Homo sapiens
  source 1..6392: mol_type = other RNA
gctgggattacaggcatgagccaccgtacccagccaatttttctgtctttacttaatggttacttttgctgaacatcaaaaagtgggtaatttttgcaaaaatatctaaagacttcagcagttttcccaagagcctctcttcaacatttgatattaaaacgcttctttttggaagctcccatctcatcatcatccttgtttatttacctctgattcagctgctaaccggtctaactctgctccatgctcttttatcaatagttgaagtgtattttagcagttctgtgacacctctcttacctccttcacagaatcctgaatgtttgtcaagatcatcaattaaagttcgaggacagtttgcacattgactctcaggcatcacaagactgatccacaaaactgtagatgaggcagtgagagagactctggtgctaagcagggggaggcctgatggtacccattttataagtgatacatttgctaatgttttcatatcaaggattttttttcccatataaccttgcaaagttaaacagtcaaatgttaggttaaagagaaaagaagcttcttgtttgtggaatcaagcaagcaaatacttgattgctcccacctcctcctttcttcacttctaccacccactcctcaccatctcattcagcagcctgaacagctgggtgtcttgtcttgtgctgctcctctccatgagaaaaagcacaggaaaaagtatgtatggcttgatgtgttttcctttccagaagtgattcctaatttaagaagaggttgagtaaaaagacaaatttcaacctaacagaactactcttctaatggtgaaattctagggatgcccgtaaagcatcttctaagtgctccttaaacaactccatgaaggcagccaacgatcccatctccatctccatcagtcactggagctgtgaggcacaaagagaggggatggctgctggtggctctccagttgctcatctcagtgcatacaatgctgtctccagagaaacaaccagtatgtgtggcagggagcaggctagtcaaggccagtggtgctgttcaccaaccctcctccatcctgattcctgaaaattctgtcctccgttatcctggactgaaattgatggtgcaggacagagagggagaattgctggcgaaatgccatcgggcaggcaacaggggaaggggttggagcatcttagccagggtatcaccttagccagggaggggcatagtgagttccccctgagcacacaggggagaggctgatatgaagaagatggagctaggtcagcagaggggacagcggggatgtctggaagagttcttccggttgcttctattccccttgtgtaaaggggagccagccatcatttgctgagagtgaggaagggaaagatgtggaaagtctgggaaagaaaaggtatggcacggttatccaggaactcagcttccagaggctctcctgagtctctaatgcttgagctggacgtagatggataaatggagtttgctagattaaaaaaaggtagagcagtctgtgcaaagggaatagcatagcaagggggacagggtgaccagcggtgtacttcactgaaaaaagaataggggcaggcccggcgcagtggctcactcctgtaatcccagctacttgggaggctgaggcaggagaattgcttgaacctgggaggtggaggttgcagtgagccgaaatcacgccaccgcactccagctggggcaacagagcaagactctgtctcaaaaaaaaaaaaaaaaaaaaaaaaggaaaagaaaagaaaagaaaaaagaaacggtggggaaatgaatgggttacaagcacctgcaggacattgggtcaaaaagtccattagatgattggacacacaggactggagcccagcaaagggttctggtcagcaaatgtctatttgaggttcattaataagcaggtgattatggatcaggatccagggagatttctcagaaagaggagagcagaggcccagccactgaattatggaaaatgtgtccatttaagggaggagcagtagaagagggaggaaagaagtgagaagattccaatcaggaagataggattcaaaaagagagctggagaaaaatgtagcaaactagaatccaagaaaagagataatttcaggaagactgtgggtattaaatgccacaaaaggcataggtagaaaacagcccatcagatttgacactgtggaagttactcaccttcctatctggaccaatctctctatgatggtcaggctgcaagacaaatggcaggatgttgaggggtgaattgtggcaagagtcaggacagtgagtgtggaagagcctttccagaaggtggtttggaaggaagggagggaggggagatagaaactggaaagggctgtggggcaaggaatggcttctggttaggtggaagcaatttgagtctatttatatgtacaaaggaaacagcccagagaggggtgcagtggattcgaccaacacagcaaataagctggggctacagcagtgagcaaagctacgtccctgccctcaaggagcttatagtctagcgtgaagagacagagaacgagcaaataagcaaatcgatatatggcatgatgagtgctgaggagaaaccccagtgggcaggggagggaacagaagaggctgcatgcaatatgggggtggcaggaagagcccctgctgtggtgacctctgccacacaattttgttcctaacacttgtcaaacaaacttgtgtgcagcctggtgttgtagttatgcggtgtctctttctcctatgacatagacagcggcttccgcttccccgtctttgccttgtccacatcatggtgttctgcagagaaggctgtgcatgaatctttgtagtaggaatgctacaaacccttcccgttcagttaggacaggcattatccaaacaatctcctccccatccccaaggaattctcggaagtggcacctagtaacctacaatgacttaggcaaattgtctgaatgcctaaaggatacaaatgatttagtattctctacatatttgcaaatttacttaaatcttcttgttatagttttaaccttacagttcactttgggaatgggtttgggggaagacagaaagaaattagtctttataaccctgccaaactctgaatcctacctcctacctcttggtaaggcatcattttaaaaggttagaataatttttatattcattatcacattcgatttccccactttatctgcagaaaaacaataaataggggcttcctattagttcaccatattttccttaggtagaaattccttgtatctgatagtctttagggtcctctttgagactaagatccccttagagatgagacgaggttggccccctttccctaccccagaggccagcacacagcacacacaggagaggacaggaaacagaggggagttgctctgatctccatattctgttctttcccagggaaaatgctctgttttcaaccaaaaacaagatcattctaaatgtcattgctccacaccccatctgggctcctgaaagcaaagctgccttgtttctgaatcagatgttgtcacccactgaaaagcctcctgcatccaagcttggctggcagtggggtccttgctcgaggggacagactcctctcccccagcgaagctgccccacatcatttcttttgagaaaggaagaggatggggaaggacaagcagcaacagagaacaattacatcactgcctctctgaccttttaaagagcaaatggttaaaataaatactatcgggctcatttctatggacttgaacattttacaacctgtagaatcatgtgacatattgcccttttgtggaactcctagaagggacagaaggaaataaacatagctatgcgacgggcttcacagctaaaacccaggacgtgcagtgtctggagggcaactcatggcaggcaagaggcagagccccccctggagtgctgagtaaagattctgaggaagtcatgcaaggatctgtcatgagcaaaaatatcagagtcctccaggatgtgaccacattttcattagcccttgccactgagcctccttccaggtgtgatgaaaaaaaaaaaaaaagcctcaggaggagaggaggcagacaggtgcagagacccgcacttggctgcaggtgagaactctggctacaaataacccacctcttcatgggggaggaaggtcccagtcacccccaggaagtcataaattcaactccattcgtaaaaatgtttatgcaatcaaaggatttcaaaacacagactttcatttcatctagtattcccacagagggaaggggagccatgagaaactcctctactggtggccaaatgtatttcttcacaacctgaaatgatgcactagcacatggcttgttagatcataacatccgcgatgtttttcaatagaggtgtaatgccatgaaatgctttcatgctgcaagcaaaaagaagaccttcgtaaatttacattcaacatgtaaaaacacataataacttctgtacatgatagagctgtgtgtgtgtgtgtgtgtgtgtgtgtgtgtgtgtgctttacaaaacaaaaatttatatcttgtctaccattgaagggagtgaggagagactgatatttgttgaacatccacaatgtgccaggtgctttacaagcctcatcttctcatttcatcttcacagcagaccaaggaggtatagactattgccgcaaccattttatgagtgagaaaatgaggctctgagaggtttaacaacttgcctgaggtcacacaggaagcgacccttgttcttcctgctacatcaagctgcctcctcaagttccaacaaatagttttgttaccttgtcccgtacacatctgtaaatcttcctgcaaaagtcatttttatggttcatggtaagatgctgccaaaagagctgaaagaaatagagtctttgtcaagtacagaaatgacaggtcatttccagaagatacagtacaagagttcaatttcatcattaattagtatctcatgcatatgggatgagatgttcttctgtatcacatttaggagatacttaagtcatattccaagcacaaactaaaaatgacctgtgttccaccatttttatccacaacttccctcacagttcttagacgacagtctcaactgtgaccgtattacaattgtctttctggcgccgaggttgcatttcatctttgaaagccctggtcagaacaacttttaaggactccttgaatctcttcttcttactgcttcccacaaagaagtaaatgaaagggttggcgctactgttgattgtggagaagagcagggaaatgtggtgtaggttcccaaaggtcgaccaatactcatagtacagcaggtaaaggagtctcatgggcatagcgaagatgaggaatataatgatggtgaccatgatgactatgtaaagcttggaggaatgggaagcccacgtgttcttccggatcttcacgaccaagatggtgctggacaccagcatgaggggcgtgaagaccaggaagctcaggatggctataaagatgatgactgctcggcagtcattccgagagtgactctcttcttctctgtcgatgcacatgacatactccatggtggtcaccaagcaagaaagagcccacagaagggcacagaccaatgccgactggtacttggggcgatggcatcggtaccagatggggtaaaggactgacaggcacctctccacactaatggccgtcagcagatagaggcccgtgttgtagccaaacagaaaagtcactgataatgtgacaattgtgtagtaatggccagaagaaagctcataatctaaagcatagtcgatagacaagatgaaaatacagaagagcagtgagatgtctgcgatagacaggtgggtgatgtagacagtgaagggatttcttctcatccggaagcacaggaaccagaggagaatcccattctcaacaaaccccactggggagatgctcataatgacccagtgcacgatggggatttgccgatgtgcattcccgactgaggcgttcctgccagttgagatgttcgtgggttcctcaacaacaaatgatgtcacgtttgacccatccatgaggaggcctcaggttggaactcttcaggtaatttttctggttgtcaaggacagctaagcaatgaaaaactgggacgcagactcactggtgtcatttgctcaggaagggtcagacgtggccaacaggttggctgccccttcacatctggggcatcaatgcccagccagcctgcagggtctccggtcccaacatctcgaaggatggctgcagcctctcatctctgaaggaatc

SEQ ID NO: 14528 - RNA, 1802 nt, Homo sapiens
  source 1..1802: mol_type = other RNA
gctgggattacaggcatgagccaccgtacccagccagcaaatctgtttttaaaaggtatgggggaggagggctgtggacagaggaagcacttagaaatgcagtctccactccggtccctggggcaaatggccgactctggacattagtttcctactccttgtctcttttcactctgcttcctggaagcgacatccagttacaccttgctgctgaccatttggcaggccactgggaactacgttgaacatgctttgcagagaggtgcttcctggggacaccctctgaactgcagtgtgaagatgggtttcagcaggttttgctgacatcggaatcagtaacttggatgagtgcactccttggctcttccactgacttgctgtgtcatgcagtaagtcccctgatctgctcggtgccaaatggtaattggagtaaaatgagcctgccttgggatactctttgccgtgggttttatttttttgagacaaccttatagtaactaacatttgtacagccttttacacacgtgccttatctcagctgatcctgtgaggcagatatgatccctagtgacagatgtggggactgcggagcagagagttgggcagctttcccagaacaatccagccggcacggtgcagccaggccccaagcccaggccttccactcttctgactccaaattctgtgctcattcctctccacagggctcccttgtgatgagactttcttcctatcctacttccaaaatgctgatgttactgagctctgagttactatataactcttatcctcttcggccttttgcccagtggtggtcagtcccttcccacttcagttctgcagcatctgggtcctgatttcacgcacaactcccaggtgggggcctggcacagagcaggttctccgcgttgaactctcaagcttccgggtggttctgcacagctccccttgcctttctttctctaccaccatttcttctcctctcctctcccctagaagggcagagatccgtttgtcaaggctaagtttggggtgcggtgggaagggcaggaggtagagctggccaaccttccaatccccggccctcctgcccgaccccaccaaccccgtcctgcctcatggaacttaggtttgaaacacagggacgaaccggaggatggcctgccagccgcagggcaggccacagcggagccctggggcgctccccggtgctggggtgtggggaggtggcagctgtgtgccccatcccgggaacaggctgcacgggcccgcgtgcagagagcccaccccgggaccaggctgcacgggcccgcagacagcatcacagcctgggctggcagccttttccaagggctgctcttgacttccgcctccctctcccgtcacttcatcaacactctaggaaccatggtgagcccacgcttcttcattcattcccgcccactcacagcacaagcccacgtcacaggaggcatgactcgcctcagaggctgattagctttccaggcagcatccagctcacgcaggcgctgagtcagtgccgccgaagcctggccaggagggaggtgactcaagcccgaaactgtgggtctcctcccctccagccctgccaagcagccagcggccgggagaagccaccaggggccaggccctgggctaatgctctgggtgctaagccctcctaagtccccacaccccacctgtaaggcacgtatgtggtgccagctgccccgcagtctctctccccatttcccgggtgaagacccaacaacccccgggcttccagccgggctccacagcat

SEQ ID NO: 14529 - RNA, 7133 nt, Homo sapiens
  source 1..7133: mol_type = other RNA
gctgggattacaggcatgagccaccgtacccggcctctaccaaaaatgtaaaaattagccgggcatggtggtgcatgcctgtagtcccagctacttgggaggctgaggtgggaggaccacttgagcccaggaggtcgaggctgcagtgagctatgatcacaccactgcactccagcctggatgacagaaagaaactctgtcaaaaaaaaaaaagaacaaattatttccaaaggggaaaaaattacacattctccaattaatctctctgctggtgaaatggtatcccaataggagagcctcacctatccctgggtcctggcagagtaagaacatgtttctaaaatctcatgatgctaagaaacggctcatgtccacgtgaacagtgccctgcatcctcaggtcacgtggcttctctcttcactgatggaactccttcaaccctagtttatcaaacaccaacatattaatgcagttgtgtgcgagtctagatcctgtatgtgaaacgctagaaatccaacccaaatcagctgaagcgagtgcaaattcctggaggcgcacagctgagaagagcaggtggagccggcttcaggtgctcaccccggcccggcccccgatctggtggcccttcctccctcagcagttggtctcagttccgggacggcttttctaggtggccacagcactgtaacgtccatcccctccacctgccagaacctcttcccagaggctcacagctaagagcactgggtctcaggggtccaggtcaggaaatcagccccgtcccgtatcaaccatgggacacaatggctcaggtgcatctgcccttgggcctgggtagggaggcctgactcagccctcctagggtaagggagagggcggaagagacgggctctctgaccaggaggaggaatgcacacaggcaaaacacaacagatgtgtgcaaacagtcactccaacactcgggagaaacgtttaaagacttttaggttaattacgtccatgcaagccaagctttcccttttgatattcttaggtttggtaggatagaagaggatgtgtggcttataaataagtgagcaaaaattacccctggataatgggcatgggagcgccccagcctggtgatggcatccttgggggctgggtggtatctgcagcctgtgtgatatttgggagtctgttattcttcagggtggggctgccaatgagaacagagcgtccccagctctctgccaagagtctcagccgctcccctgggctgcctccatacaggcgggtgagcacacatggaggggagcaccaccaggaacccaggcttcctttcagagactctagggagaagactctggggacgttggtgtggccccaacattctgccgcagggaaacacctgtcaccatgccgaaccaacacattcaggaaaggtccccccaccaaggtacaaccaaggcagttcacatccagggacaggtgccccgggcagctcagctcaggagggtccctctggggagacctggtctgcaccaggaagcagaccacgtgttcacaaaatgcacacgccacccactttgcttggacccacacaaggaccatgtccacagcttccagctcagatggctgctcccatccgtgtcactgtccctcacagggacgagggcttagccaccctgcgttcactctccacccctacggcagccctgccagcctctcacctgagtgcaggagacagggcggggagagagaggtgcggccatccaggccccgatgaatgcagctggcctcatcggagggtttgcaggaacaaacttggaacacaactcctacaccctctggaagaaggaaacaagaaaaatatcccgatgtgtgtgtgagagagagtgtgtgtgtgtgtgtgtgtgtgcgcgcgtgtgtgtgtgtgttctgattcctaagtggcagagctaggttaaagccccaccttcaccaaaccacccacctcagggcacagacgtgctcagacctcaccgggaagataaactgaaatcctaacccttgccctccatcaagacatagggccaaaaccaaacctgaaatttttccaatagtccaaataaatggcaaaagcactacagcaaactccactaaatatccactgggggttgtaagtatcagcgaatgaagaagcatgagatgctttaagaggaaagagggagggaggcatcacccacacaacctgcaagtcacacctgtgtcaaattcctggggcagatggaaaatacacagcatcagacgctgggaggcgagtccaggagcagccaggccgcccagcccaagcattgcccaactgtaaacgggcgaggtgccctcccactgattcgaggcgcagccatcacacaagagacagggctttgtgacaccaccccgcacccaaccaagtcattctcatgactgtgctcaaagtgtggacacagctggaggatgggggccaacagggtaaaagagttttaagtttatggttaaattttccagttgtacgatgccaattttcataaaatgtataatttgctgtgtttcagtggaaaaagaaaaaaccagagccaaaggtctctacgcagtgtggtgctgcgcatcaggcaaacagcgaagaatcaaagtgggttctccccgctcacacctccctctcttcccggagacgcctcccctcggcccagcaggcccttttctgccactcccatccggagtcatccccacgggcggtggccccgaccatggcccgggaatctgagcaggtgcgtggatgtgggtggtgtcttctgcaggaacccctccacatccctgcaaacaccccaggtgctcaggaaaaccgaacctcagaggaaccataccaagaactgggaatgcagaaatggaggggacgcgggcccccctcagtgagtgaaccgcccagtgggttctgacattcgtctgaacatcctataaacaaacgcatcccggggaggtgctccagcaaaggcagacacaaagggccatgcccagaatacggaaaacaagccctcagcagattcactgacaccctgttcacagcagcattcaattcacattcgcaggaaggcagaagcaactcagtgtccaccaactgatgaacagataaacaaaccatgcctcttccacacaatgggacattattccgcctcagaaaggaagttagttctgacacctgccacgacaccgatgaacctagaggacattgcatgaggtgaagtacttcagtcccaaaaggaccaatactgtgtgactccatttctgagggagctcgggtagtagaaatcagagagtggaagctgctgccttctaccaatggggagcgagtgctgaatggggacagagtttcagtttgggaagatgagaaagctctggagatgatggtggtggtggcacgacaatacgaatgtgcttaatgccacacaacagtgcacttaacaatggttaagatggtacgtttaaaattaaacatttttatcataataaaaaacttggaggggccaggtgtgatggctcatgcctgtaatcccagcactttgggagggtgatgcaggagggtcacttgagcccaggagtttgagagcagcctgggcaacacagtgagacctcatctctgctgaaaataaaaaactagctgggcaggctggcgctcacctgtaaccccagctacttgggagtctgagatgggaagatcacttgagcccaggaggttgaagctgcagtgagctgtgattgcaccagtgtattccagcccggatgacagagcgagaccctgtctccaaaaacaaaacaaaacaaaaataaaagaaagcgaagcttcagaaaggaaggcaggaggtgtctaacacaggggacacctgaggctagcaggcactgggggccaagacccacacaagcccacctgagcctgggaaacacagggacaccacacacagaggacaccagggtatgtcccaactgagcgtggccagcaaccagggactgggcagtggtgacaaataccacacacgaggaagacaggtcaagcagggtgcccgacaccacgaaatgattgcaaccatctctccaactacagcttagaagcagaaatagcaaaggagtttcagccagatgtttccagagcctcctctgacacttttatcaagacagggcccatcaaacctgagggttcaaggtcagtcgtgtccttgagggtgaaggcactggagctaaaccaaccagaaagccacagagacagtcacacggagcctcttcttggtgacactgggtactgtcatccagcacggtctagagataaacgccaaaccactccactcctgccaactgtaaacctcaacagccatagtttactttctatttaatctatctatctacctatcttctatctgtctatttagaaacagagtctcactttgctgcccaggctggagtgcagtggcacgatcataggtcactgcagccttgaactcctgggctccagcgatcctcctgcctcagcctcccgagtagctgggattacaggtgtgcaccatcatgtccggctgattttcttattttttgtagacacagggtctcgctatgtggtccaaactgatcttgaactcctgggctcaagtgatcctccctcctcagcctcctgagtagctgggtttacagatgtgcaccaccacgtcctttttattttttgtagagatgaggtccttgctatgttgcccaagctggtcttgaactcctgggctcaagtgatcttcccccctcagcctcccaaagtgccaggattgcaggcatgagccaccgtgcccagccttaatagccataatgtattaatatttatttatttattttgagatggaatctcactctgtcacccaggctagagtgcaatgtcgcgatctcagctcactgcagcctctgcctcctgggttcaagcaatctttccatctcagaactcctgagtagctgggactacaggtgcacaccaccacacccgactcatttttttttttttttttttttttttttttttttttttagtagagacagggtttcaccatgttggccaggtctcaaattcctgacctcaagcgatccttctgtctgggcctcccaaagttctgggattacctgcctgagtcacccgcccggccttaacagccataatttaaactagacagtatgggaacagctggagttagaaatcctagaaatcctgcttctgtaactgaccggtttacctctgacttgacttcaaacaggaagccctgaagattgaccttttcaagtacaacacttaaacaaagaactttccctctggaaggatttgtcggctacccttccaaaaacagacaggtgcggcctgacttcaagtgcaggccccgccctcctccggtgagtggccctagccctggaggcagctccatcagcctcagcatcccctcccggcgcccgcacgctcagaaaaaccacaggagcgggcgagcgggcgagcgggcgggcgggtgggcgggcggaggggagaggggatattttactccagcattcccttccacatttcgtattaaatacctgaaatatattaatcttaaaaaacaatatcgatacagtactcaatggatagaggcagtggagtgaacaagaagcccagattgcaaaatcgtaggtcataaaaaaactggagtgcgcgtgcgtcaggttccaggcacgcgagaaaaagcaacgcgaaagctttcagtctcggaggaggttttcgggcttggggtagccgaagagaacaaagtcggcctcgtagagtttatacagctgctgcctccaggccagggggatcttggcgaaccagtcctcctcccagctgctggcggtcctgttccggtagctcggggggaagcggagctgccggtccacctggagtagctgcagcagctgcgcggcgtcctcgtccagagtctccagcttccccacgaagtcgtagtcgatctggcacgggtggcagaggcggtacacctgccgccagtgctcgttgaagggcgccagcttctccgtgtgcgggtccagcaggtactggatgaagttggcgaaggacaccttgaggccagcgcggaaggcctcgcgcgccgaggcgggcaggctggtgtggttggcgtacagccgcagcatgggcacggcgaacttgcggtagaactcctcgttctccagctcgaacttgctgcggaaggcggagatcaggcgcacgaaggggtcgcgcacgaagaggaacttggtgtacttcttgagcttgaccttcatgaggtggcgggagagcttcccgtagcggcgccagaacttgttgaaggtcaggtgcgcgctggcgttgtgcacgtgctcgcgcgggatgcgcagcgggtcgcggtagggcgcaccgcggtgcagcaggcttccgctcagcacgatcatcacgcgcttccagttggtgcaggccaccttgggcacgtagcagtagatggccccgtgccggtcgtccacgatcaggtggctcagctccgagttggggatgtcgtcgaatgcgcgctccttggtggggaaggccaggctggagttggcgcagaagccccgcagcacgctcctccgctccgcctgctgccggccctggtctgggctgcgccgggcgtcgcgcggggaccagtcgtagcctctcacgctctcctccatgctccccggcgcaggcggctgctccgtctcctttctgggaaggtcgctctgcttcacgccagcactgagaaacttgtccagaaactcgtcgacatcggagtcggccgtgagctccctgtccctgtccggcccgggcgtgggcagcggcggccccgtgtgcggcctagagaaggacgtgtgcaagtagaagtgcgcggcgcctgcgctgtcccagtacacgatgatcagcaggatcatgaacaccgaccccagcaccagccacagccggaacagccgggccttggtcatcctgccccgggcgggctgggccctctccgggcctctcacttcagcttcctgcagagccggggcatcctgctgggaacctcgcgaccctcacctcgcgcccctcacctcgcgcccgcagccgccgccgccgccccgcgact

SEQ ID NO: 14530 - RNA, 7119 nt, Homo sapiens
  source 1..7119: mol_type = other RNA
gctgggattacaggcatgagccaccgtacccggcctctaccaaaaatgtaaaaattagccgggcatggtggtgcatgcctgtagtcccagctacttgggaggctgaggtgggaggaccacttgagcccaggaggtcgaggctgcagtgagctatgatcacaccactgcactccagcctggatgacagaaagaaactctgtcaaaaaaaaaaaagaacaaattatttccaaaggggaaaaaattacacattctccaattaatctctctgctggtgaaatggtatcccaataggagagcctcacctatccctgggtcctggcagagtaagaacatgtttctaaaatctcatgatgctaagaaacggctcatgtccacgtgaacagtgccctgcatcctcaggtcacgtggcttctctcttcactgatggaactccttcaaccctagtttatcaaacaccaacatattaatgcagttgtgtgcgagtctagatcctgtatgtgaaacgctagaaatccaacccaaatcagctgaagcgagtgcaaattcctggaggcgcacagctgagaagagcaggtggagccggcttcaggtgctcaccccggcccggcccccgatctggtggcccttcctccctcagcagttggtctcagttccgggacggcttttctaggtggccacagcactgtaacgtccatcccctccacctgccagaacctcttcccagaggctcacagctaagagcactgggtctcaggggtccaggtcaggaaatcagccccgtcccgtatcaaccatgggacacaatggctcaggtgcatctgcccttgggcctgggtagggaggcctgactcagccctcctagggtaagggagagggcggaagagacgggctctctgaccaggaggaggaatgcacacaggcaaaacacaacagatgtgtgcaaacagtcactccaacactcgggagaaacgtttaaagacttttaggttaattacgtccatgcaagccaagctttcccttttgatattcttaggtttggtaggatagaagaggatgtgtggcttataaataagtgagcaaaaattacccctggataatgggcatgggagcgccccagcctggtgatggcatccttgggggctgggtggtatctgcagcctgtgtgatatttgggagtctgttattcttcagggtggggctgccaatgagaacagagcgtccccagctctctgccaagagtctcagccgctcccctgggctgcctccatacaggcgggtgagcacacatggaggggagcaccaccaggaacccaggcttcctttcagagactctagggagaagactctggggacgttggtgtggccccaacattctgccgcagggaaacacctgtcaccatgccgaaccaacacattcaggaaaggtccccccaccaaggtacaaccaaggcagttcacatccagggacaggtgccccgggcagctcagctcaggagggtccctctggggagacctggtctgcaccaggaagcagaccacgtgttcacaaaatgcacacgccacccactttgcttggacccacacaaggaccatgtccacagcttccagctcagatggctgctcccatccgtgtcactgtccctcacagggacgagggcttagccaccctgcgttcactctccacccctacggcagccctgccagcctctcacctgagtgcaggagacagggcggggagagagaggtgcggccatccaggccccgatgaatgcagctggcctcatcggagggtttgcaggaacaaacttggaacacaactcctacaccctctggaagaaggaaacaagaaaaatatcccgatgtgtgtgtgagagagagtgtgtgtgtgtgtgtgtgtgtgcgcgcgtgtgtgtgtgtgttctgattcctaagtggcagagctaggttaaagccccaccttcaccaaaccacccacctcagggcacagacgtgctcagacctcaccgggaagataaactgaaatcctaacccttgccctccatcaagacatagggccaaaaccaaacctgaaatttttccaatagtccaaataaatggcaaaagcactacagcaaactccactaaatatccactgggggttgtaagtatcagcgaatgaagaagcatgagatgctttaagaggaaagagggagggaggcatcacccacacaacctgcaagtcacacctgtgtcaaattcctggggcagatggaaaatacacagcatcagacgctgggaggcgagtccaggagcagccaggccgcccagcccaagcattgcccaactgtaaacgggcgaggtgccctcccactgattcgaggcgcagccatcacacaagagacagggctttgtgacaccaccccgcacccaaccaagtcattctcatgactgtgctcaaagtgtggacacagctggaggatgggggccaacagggtaaaagagttttaagtttatggttaaattttccagttgtacgatgccaattttcataaaatgtataatttgctgtgtttcagtggaaaaagaaaaaaccagagccaaaggtctctacgcagtgtggtgctgcgcatcaggcaaacagcgaagaatcaaagtgggttctccccgctcacacctccctctcttcccggagacgcctcccctcggcccagcaggcccttttctgccactcccatccggagtcatccccacgggcggtggccccgaccatggcccgggaatctgagcaggtgcgtggatgtgggtggtgtcttctgcaggaacccctccacatccctgcaaacaccccaggtgctcaggaaaaccgaacctcagaggaaccataccaagaactgggaatgcagaaatggaggggacgcgggcccccctcagtgagtgaaccgcccagtgggttctgacattcgtctgaacatcctataaacaaacgcatcccggggaggtgctccagcaaaggcagacacaaagggccatgcccagaatacggaaaacaagccctcagcagattcactgacaccctgttcacagcagcattcaattcacattcgcaggaaggcagaagcaactcagtgtccaccaactgatgaacagataaacaaaccatgcctcttccacacaatgggacattattccgcctcagaaaggaagttagttctgacacctgccacgacaccgatgaacctagaggacattgcatgaggtgaagtacttcagtcccaaaaggaccaatactgtgtgactccatttctgagggagctcgggtagtagaaatcagagagtggaagctgctgccttctaccaatggggagcgagtgctgaatggggacagagtttcagtttgggaagatgagaaagctctggagatgatggtggtggtggcacgacaatacgaatgtgcttaatgccacacaacagtgcacttaacaatggttaagatggtacgtttaaaattaaacatttttatcataataaaaaacttggaggggccaggtgtgatggctcatgcctgtaatcccagcactttgggagggtgatgcaggagggtcacttgagcccaggagtttgagagcagcctgggcaacacagtgagacctcatctctgctgaaaataaaaaactagctgggcaggctggcgctcacctgtaaccccagctacttgggagtctgagatgggaagatcacttgagcccaggaggttgaagctgcagtgagctgtgattgcaccagtgtattccagcccggatgacagagcgagaccctgtctccaaaaacaaaacaaaacaaaaataaaagaaagcgaagcttcagaaaggaaggcaggaggtgtctaacacaggggacacctgaggctagcaggcactgggggccaagacccacacaagcccacctgagcctgggaaacacagggacaccacacacagaggacaccagggtatgtcccaactgagcgtggccagcaaccagggactgggcagtggtgacaaataccacacacgaggaagacaggtcaagcagggtgcccgacaccacgaaatgattgcaaccatctctccaactacagcttagaagcagaaatagcaaaggagtttcagccagatgtttccagagcctcctctgacacttttatcaagacagggcccatcaaacctgagggttcaaggtcagtcgtgtccttgagggtgaaggcactggagctaaaccaaccagaaagccacagagacagtcacacggagcctcttcttggtgacactgggtactgtcatccagcacggtctagagataaacgccaaaccactccactcctgccaactgtaaacctcaacagccatagtttactttctatttaatctatctatctacctatcttctatctgtctatttagaaacagagtctcactttgctgcccaggctggagtgcagtggcacgatcataggtcactgcagccttgaactcctgggctccagcgatcctcctgcctcagcctcccgagtagctgggattacaggtgtgcaccatcatgtccggctgattttcttattttttgtagacacagggtctcgctatgtggtccaaactgatcttgaactcctgggctcaagtgatcctccctcctcagcctcctgagtagctgggtttacagatgtgcaccaccacgtcctttttattttttgtagagatgaggtccttgctatgttgcccaagctggtcttgaactcctgggctcaagtgatcttcccccctcagcctcccaaagtgccaggattgcaggcatgagccaccgtgcccagccttaatagccataatgtattaatatttatttatttattttgagatggaatctcactctgtcacccaggctagagtgcaatgtcgcgatctcagctcactgcagcctctgcctcctgggttcaagcaatctttccatctcagaactcctgagtagctgggactacaggtgcacaccaccacacccgactcatttttttttttttttttttttttttttttttttttttagtagagacagggtttcaccatgttggccaggtctcaaattcctgacctcaagcgatccttctgtctgggcctcccaaagttctgggattacctgcctgagtcacccgcccggccttaacagccataatttaaactagacagtatgggaacagctggagttagaaatcctagaaatcctgcttctgtaactgaccggtttacctctgacttgacttcaaacaggaagccctgaagattgaccttttcaagtacaacacttaaacaaagaactttccctctggaaggatttgtcggctacccttccaaaaacagacaggtgcggcctgacttcaagtgcaggccccgccctcctccggtgagtggccctagccctggaggcagctccatcagcctcagcatcccctcccggcgcccgcacgctcagaaaaaccacaggagcgggcgagcgggcgagcgggcgggcgggtgggcgggcggaggggagaggggatattttactccagcattcccttccacatttcgtattaaatacctgaaatatattaatcttaaaaaacaatatcgatacagtactcaatggatagaggcagtggagtgaacaagaagcccagattgcaaaatcgtaggtcataaaaaaactggagtgcgcgtgcgtcaggttccaggcacgcgagaaaaagcaacgcgaaagctttcagtctcggaggaggttttcgggcttggggtagccgaagagaacaaagtcggcctcgtagagtttatacagctgctgcctccaggccagggggatcttggcgaaccagtcctcctcccagctgctggcggtcctgttccggtagctcggggggaagcggagctgccggtccacctggagtagctgcagcagctgcgcggcgtcctcgtccagagtctccagcttccccacgaagtcgtagtcgatctggcacgggtggcagaggcggtacacctgccgccagtgctcgttgaagggcgccagcttctccgtgtgcgggtccagcaggtactggatgaagttggcgaaggacaccttgaggccagcgcggaaggcctcgcgcgccgaggcgggcaggctggtgtggttggcgtacagccgcagcatgggcacggcgaacttgcggtagaactcctcgttctccagctcgaacttgctgcggaaggcggagatcaggcgcacgaaggggtcgcgcacgaagaggaacttggtgtacttcttgagcttgaccttcatgaggtggcgggagagcttcccgtagcggcgccagaacttgttgaaggtcaggtgcgcgctggcgttgtgcacgtgctcgcgcgggatgcgcagcgggtcgcggtagggcgcaccgcggtgcagcaggcttccgctcagcacgatcatcacgcgcttccagttggtgcaggccaccttgggcacgtagcagtagatggccccgtgccggtcgtccacgatcaggtggctcagctccgagttggggatgtcgtcgaatgcgcgctccttggtggggaaggccaggctggagttggcgcagaagccccgcagcacgctcctccgctccgcctgctgccggccctggtctgggctgcgccgggcgtcgcgcggggaccagtcgtagcctctcacgctctcctccatgctccccggcgcaggcggctgctccgtctcctttctgggaaggtcgctctgcttcacgccagcactgagaaacttgtccagaaactcgtcgacatcggagtcggccgtgagctccctgtccctgtccggcccgggcgtgggcagcggcggccccgtgtgcggcctagagaaggacgtgtgcaagtagaagtgcgcggcgcctgcgctgtcccagtacacgatgatcagcaggatcatgaacaccgaccccagcaccagccacagccggaacagccgggccttggtcatcctgccccgggcgggctgggccctctccgggcctctcacttcagcttcctgcagagccggggcatcctgctgggaacctcgcgcccctcacctcgcgcccgcagccgccgccgccgccccgcgact

SEQ ID NO: 14531 - RNA, 7105 nt, Homo sapiens
  source 1..7105: mol_type = other RNA
gctgggattacaggcatgagccaccgtacccggcctctaccaaaaatgtaaaaattagccgggcatggtggtgcatgcctgtagtcccagctacttgggaggctgaggtgggaggaccacttgagcccaggaggtcgaggctgcagtgagctatgatcacaccactgcactccagcctggatgacagaaagaaactctgtcaaaaaaaaaaaagaacaaattatttccaaaggggaaaaaattacacattctccaattaatctctctgctggtgaaatggtatcccaataggagagcctcacctatccctgggtcctggcagagtaagaacatgtttctaaaatctcatgatgctaagaaacggctcatgtccacgtgaacagtgccctgcatcctcaggtcacgtggcttctctcttcactgatggaactccttcaaccctagtttatcaaacaccaacatattaatgcagttgtgtgcgagtctagatcctgtatgtgaaacgctagaaatccaacccaaatcagctgaagcgagtgcaaattcctggaggcgcacagctgagaagagcaggtggagccggcttcaggtgctcaccccggcccggcccccgatctggtggcccttcctccctcagcagttggtctcagttccgggacggcttttctaggtggccacagcactgtaacgtccatcccctccacctgccagaacctcttcccagaggctcacagctaagagcactgggtctcaggggtccaggtcaggaaatcagccccgtcccgtatcaaccatgggacacaatggctcaggtgcatctgcccttgggcctgggtagggaggcctgactcagccctcctagggtaagggagagggcggaagagacgggctctctgaccaggaggaggaatgcacacaggcaaaacacaacagatgtgtgcaaacagtcactccaacactcgggagaaacgtttaaagacttttaggttaattacgtccatgcaagccaagctttcccttttgatattcttaggtttggtaggatagaagaggatgtgtggcttataaataagtgagcaaaaattacccctggataatgggcatgggagcgccccagcctggtgatggcatccttgggggctgggtggtatctgcagcctgtgtgatatttgggagtctgttattcttcagggtggggctgccaatgagaacagagcgtccccagctctctgccaagagtctcagccgctcccctgggctgcctccatacaggcgggtgagcacacatggaggggagcaccaccaggaacccaggcttcctttcagagactctagggagaagactctggggacgttggtgtggccccaacattctgccgcagggaaacacctgtcaccatgccgaaccaacacattcaggaaaggtccccccaccaaggtacaaccaaggcagttcacatccagggacaggtgccccgggcagctcagctcaggagggtccctctggggagacctggtctgcaccaggaagcagaccacgtgttcacaaaatgcacacgccacccactttgcttggacccacacaaggaccatgtccacagcttccagctcagatggctgctcccatccgtgtcactgtccctcacagggacgagggcttagccaccctgcgttcactctccacccctacggcagccctgccagcctctcacctgagtgcaggagacagggcggggagagagaggtgcggccatccaggccccgatgaatgcagctggcctcatcggagggtttgcaggaacaaacttggaacacaactcctacaccctctggaagaaggaaacaagaaaaatatcccgatgtgtgtgtgagagagagtgtgtgtgtgtgtgtgtgtgtgcgcgcgtgtgtgtgtgtgttctgattcctaagtggcagagctaggttaaagccccaccttcaccaaaccacccacctcagggcacagacgtgctcagacctcaccgggaagataaactgaaatcctaacccttgccctccatcaagacatagggccaaaaccaaacctgaaatttttccaatagtccaaataaatggcaaaagcactacagcaaactccactaaatatccactgggggttgtaagtatcagcgaatgaagaagcatgagatgctttaagaggaaagagggagggaggcatcacccacacaacctgcaagtcacacctgtgtcaaattcctggggcagatggaaaatacacagcatcagacgctgggaggcgagtccaggagcagccaggccgcccagcccaagcattgcccaactgtaaacgggcgaggtgccctcccactgattcgaggcgcagccatcacacaagagacagggctttgtgacaccaccccgcacccaaccaagtcattctcatgactgtgctcaaagtgtggacacagctggaggatgggggccaacagggtaaaagagttttaagtttatggttaaattttccagttgtacgatgccaattttcataaaatgtataatttgctgtgtttcagtggaaaaagaaaaaaccagagccaaaggtctctacgcagtgtggtgctgcgcatcaggcaaacagcgaagaatcaaagtgggttctccccgctcacacctccctctcttcccggagacgcctcccctcggcccagcaggcccttttctgccactcccatccggagtcatccccacgggcggtggccccgaccatggcccgggaatctgagcaggtgcgtggatgtgggtggtgtcttctgcaggaacccctccacatccctgcaaacaccccaggtgctcaggaaaaccgaacctcagaggaaccataccaagaactgggaatgcagaaatggaggggacgcgggcccccctcagtgagtgaaccgcccagtgggttctgacattcgtctgaacatcctataaacaaacgcatcccggggaggtgctccagcaaaggcagacacaaagggccatgcccagaatacggaaaacaagccctcagcagattcactgacaccctgttcacagcagcattcaattcacattcgcaggaaggcagaagcaactcagtgtccaccaactgatgaacagataaacaaaccatgcctcttccacacaatgggacattattccgcctcagaaaggaagttagttctgacacctgccacgacaccgatgaacctagaggacattgcatgaggtgaagtacttcagtcccaaaaggaccaatactgtgtgactccatttctgagggagctcgggtagtagaaatcagagagtggaagctgctgccttctaccaatggggagcgagtgctgaatggggacagagtttcagtttgggaagatgagaaagctctggagatgatggtggtggtggcacgacaatacgaatgtgcttaatgccacacaacagtgcacttaacaatggttaagatggtacgtttaaaattaaacatttttatcataataaaaaacttggaggggccaggtgtgatggctcatgcctgtaatcccagcactttgggagggtgatgcaggagggtcacttgagcccaggagtttgagagcagcctgggcaacacagtgagacctcatctctgctgaaaataaaaaactagctgggcaggctggcgctcacctgtaaccccagctacttgggagtctgagatgggaagatcacttgagcccaggaggttgaagctgcagtgagctgtgattgcaccagtgtattccagcccggatgacagagcgagaccctgtctccaaaaacaaaacaaaacaaaaataaaagaaagcgaagcttcagaaaggaaggcaggaggtgtctaacacaggggacacctgaggctagcaggcactgggggccaagacccacacaagcccacctgagcctgggaaacacagggacaccacacacagaggacaccagggtatgtcccaactgagcgtggccagcaaccagggactgggcagtggtgacaaataccacacacgaggaagacaggtcaagcagggtgcccgacaccacgaaatgattgcaaccatctctccaactacagcttagaagcagaaatagcaaaggagtttcagccagatgtttccagagcctcctctgacacttttatcaagacagggcccatcaaacctgagggttcaaggtcagtcgtgtccttgagggtgaaggcactggagctaaaccaaccagaaagccacagagacagtcacacggagcctcttcttggtgacactgggtactgtcatccagcacggtctagagataaacgccaaaccactccactcctgccaactgtaaacctcaacagccatagtttactttctatttaatctatctatctacctatcttctatctgtctatttagaaacagagtctcactttgctgcccaggctggagtgcagtggcacgatcataggtcactgcagccttgaactcctgggctccagcgatcctcctgcctcagcctcccgagtagctgggattacaggtgtgcaccatcatgtccggctgattttcttattttttgtagacacagggtctcgctatgtggtccaaactgatcttgaactcctgggctcaagtgatcctccctcctcagcctcctgagtagctgggtttacagatgtgcaccaccacgtcctttttattttttgtagagatgaggtccttgctatgttgcccaagctggtcttgaactcctgggctcaagtgatcttcccccctcagcctcccaaagtgccaggattgcaggcatgagccaccgtgcccagccttaatagccataatgtattaatatttatttatttattttgagatggaatctcactctgtcacccaggctagagtgcaatgtcgcgatctcagctcactgcagcctctgcctcctgggttcaagcaatctttccatctcagaactcctgagtagctgggactacaggtgcacaccaccacacccgactcatttttttttttttttttttttttttttttttttttttagtagagacagggtttcaccatgttggccaggtctcaaattcctgacctcaagcgatccttctgtctgggcctcccaaagttctgggattacctgcctgagtcacccgcccggccttaacagccataatttaaactagacagtatgggaacagctggagttagaaatcctagaaatcctgcttctgtaactgaccggtttacctctgacttgacttcaaacaggaagccctgaagattgaccttttcaagtacaacacttaaacaaagaactttccctctggaaggatttgtcggctacccttccaaaaacagacaggtgcggcctgacttcaagtgcaggccccgccctcctccggtgagtggccctagccctggaggcagctccatcagcctcagcatcccctcccggcgcccgcacgctcagaaaaaccacaggagcgggcgagcgggcgagcgggcgggcgggtgggcgggcggaggggagaggggatattttactccagcattcccttccacatttcgtattaaatacctgaaatatattaatcttaaaaaacaatatcgatacagtactcaatggatagaggcagtggagtgaacaagaagcccagattgcaaaatcgtaggtcataaaaaaactggagtgcgcgtgcgtcaggttccaggcacgcgagaaaaagcaacgcgaaagctttcagtctcggaggaggttttcgggcttggggtagccgaagagaacaaagtcggcctcgtagagtttatacagctgctgcctccaggccagggggatcttggcgaaccagtcctcctcccagctgctggcggtcctgttccggtagctcggggggaagcggagctgccggtccacctggagtagctgcagcagctgcgcggcgtcctcgtccagagtctccagcttccccacgaagtcgtagtcgatctggcacgggtggcagaggcggtacacctgccgccagtgctcgttgaagggcgccagcttctccgtgtgcgggtccagcaggtactggatgaagttggcgaaggacaccttgaggccagcgcggaaggcctcgcgcgccgaggcgggcaggctggtgtggttggcgtacagccgcagcatgggcacggcgaacttgcggtagaactcctcgttctccagctcgaacttgctgcggaaggcggagatcaggcgcacgaaggggtcgcgcacgaagaggaacttggtgtacttcttgagcttgaccttcatgaggtggcgggagagcttcccgtagcggcgccagaacttgttgaaggtcaggtgcgcgctggcgttgtgcacgtgctcgcgcgggatgcgcagcgggtcgcggtagggcgcaccgcggtgcagcaggcttccgctcagcacgatcatcacgcgcttccagttggtgcaggccaccttgggcacgtagcagtagatggccccgtgccggtcgtccacgatcaggtggctcagctccgagttggggatgtcgtcgaatgcgcgctccttggtggggaaggccaggctggagttggcgcagaagccccgcagcacgctcctccgctccgcctgctgccggccctggtctgggctgcgccgggcgtcgcgcggggaccagtcgtagcctctcacgctctcctccatgctccccggcgcaggcggctgctccgtctcctttctgggaaggtcgctctgcttcacgccagcactgagaaacttgtccagaaactcgtcgacatcggagtcggccgtgagctccctgtccctgtccggcccgggcgtgggcagcggcggccccgtgtgcggcctagagaaggacgtgtgcaagtagaagtgcgcggcgcctgcgctgtcccagtacacgatgatcagcaggatcatgaacaccgaccccagcaccagccacagccggaacagccgggccttggtcatcctgccccgggcgggctgggccctctccgggcctctcacttcagcttcctgcagagccggggcatcctgctgggaacctcgcgcccgcagccgccgccgccgccccgcgact

SEQ ID NO: 14532 - RNA, 1038 nt, Homo sapiens
  source 1..1038: mol_type = other RNA
gctgggattacaggcatgagccaccgtacctagccctattgctatttttattagcattacattaagtttataggctaacttaagaggacatggcatttttatgataatgagtttttgcagtcaagaacgcaggccagttttttttaaatggggtaaatgattgtccaagcgcctccaggcaggctcacgtgcacactctggagtcagtgaagaaggtgaacagctgacaggagcagcctcccagtcagagaagccctgcacactgttgcaaacagacagcttgcatctggagtcttctgtgatccgaggaggaagcgtggctgagtccttcccagaagagggtctggagccatagagatcagctcccaggcagcaggatggagggtgtagactggacatgaagaggcagctggaatgtatcgggcactcagctccagctcaccacgatccaggcactcaagttcccaagacaatagtttccttctcgagctagctggcttattttatccggaccaggatataacagctctaaacaggctttgccaggaagagacgtcatggacttcaaccagggcacctgaccaggaagaaatcactgcaggatgatctgaaagagttttcataaattattttacgtaaggtagattctgaccttgatggggacagccaaggttctggaccctcagctgggaaagatgggactaagtctacaactgctgaggttgtagaacaggcttcttgttgggaggaaccctcttgtggacatgggccgtcgaggtggagtgagagaacaccgtgccacctggacgctgaaacaccattgagtcacctctgtttgaaatgcttgttccctggtgccgtaaagaaatagcacttgaacataaatttaatttactcagcaaggacatttttatactttctgtgaaagggtacactcaccaggagttttgccacgagagtacaccaaacaaaggagacagggtcatttataacctgacgcgtccaccctactgctgtgtccagtttccattggctgga

SEQ ID NO: 14533 - RNA, 907 nt, Homo sapiens
  source 1..907: mol_type = other RNA
gctgggattacaggcatgagccaccgtacctagccctattgctatttttattagcattacattaagtttataggctaacttaagaggacatggcatttttatgataatgagtttttgcagtcaagaacgcaggccagttttttttaaatggggtaaatgattgtccaagcgcctccaggcaggctcacgtgcacactctggagtcagtgaagaaggtgaacagctgacaggagcagcctcccagtcagagaagccctgcacactgttgcaaacagacagcttgcatctggagtcttctgtgatccgaggaggaagcgtggctgagtccttcccagaagagggtctggagctgtgagttggggacaattgtcagattctagcagtgaaagtggttcatgtgcaggtgcaacctgccccgcagtcacgggacacagccacatggagccgagccacgctctcagagaaggagccagggaagaaacaccctaactgcactcctcccttcttctggcccccagcagccataggccctgggcccccggtgagatacccatagagatcagctcccaggcagcaggatggagggtgtagactggacatgaagaggcagctggaatgtatcgggcactcagctccagctcaccacgatccaggcactcaagttcccaagacaatagtttccttctcgagctagctggcttattttatccggaccaggatataacagctctaaacaggctttgccaggaagagacgtcatggacttcaaccagggcacctgaccaggaagaaatcactgcaggatgatcaggagttttgccacgagagtacaccaaacaaaggagacagggtcatttataacctgacgcgtccaccctactgctgtgtccagtttccattggctgga

SEQ ID NO: 14534 - RNA, 2065 nt, Homo sapiens
  source 1..2065: mol_type = other RNA
gctgggattacaggcatgagccaccgtacctggccctattttttgttttttttttggagacagagtctcgctctgttgcccaggctggggtgcggttgtgcaatctcggctcactgcaacctctgcctccctggttcacgtgattctcctgcctcagctgagtagctggattgcaggtgtgcaccacactgcctggctaatttttgtatttttaggagagatggcatttcaccatgttggccaggccagtttcaaactcctggcctcaagtggtctgcccgccttggcctcccaaagtgctgggattacaggtgacttctggttattttaaaaaatctgagatgcaggggaaaaaaaatatttcaccaaccctattttttagttaggtctttacaataattatactatatatgagcattttggagatattctagctataagacctgtaaagtcagaatcttgtgctttaaaaaatagctttttcacttaaaggttcctctaaacccaagaaaatagtttaaaaataatgactttttatattttaagttcaattaacttcataatttttaatgagtcaacaatattaagtaaaatacacctgtttatactaagattttccagcaaatcttatataactgaaaattatgaagtataatgttttaaaatattttcttaaaaacaaacaaaatttcaaaccatggaaacaactggctccaaaagtttatctccagggacatccatccatgtcatttcaatggcaccagggtcacctggagagcaaggtgttagcagatcatctacaagatggttaggatcagctcgggaaggtccgcgaacctttttaaaatgagtagctgactgtactttcctaacaggctgcataagggcatcacgtacaatgatacttatatctgcccctgaataaccatctgttttcctcccaagttcccgaaagtctgcttccgtgagactgttctgagtggtccctaggtgcagtttaaacattgctgctcgggcatggggttccggcaagggaatataaattcgtttctcaaatcttcgcctaatggcagaatccagaacccagggtatatttgtagctcccagaaccaaaattccatcattgtctacaccaaccccttgcatttgcactaggaactccgtcttaattctacgtgcggcttcactttcattttcacttcttgaaccacagagagaatcaatttcatcaatgaagataatggagggcttgttctctctggcaagttggaataaattcttaaccagtttttcactttcacctagccacttagaaacaagatcagaggaagatattgaaaaaaatgttgagttgttggcttctgttgctacagctttggctaagtaggactttcctgttccaggcggcccaaataataggattcccctccaaggtgttctcttgcctgtaaaaagatgaggaaatttaataggcagtatcacagcctctttcagtgcttctttggctccttcaagtccagcaacgtcactccatttcacatttggtcgttctataacaatggcaccccttctcatctgctggactcggctgtccttctttcactggcttctgtgcttttttctctttatttttcaggtactcctttagtttttctgctctatcaagatattctgtacactttgccctgatactttgcttggctttatcaccctgtgcttcatatttaacgacatgaagaaaatactgcacagcatgctgatagagctgaagggcttcttcgtagttcccagccttgtcttcttgcgctgctttgctagccagatctatcgctttctggaggttgggcgaagtggatgacatggcggagttcccaggcggttcccaagggaacgaggggcgaggagagccaacagcagcaacgtcgaagcgcgcacggggtaacagccctcaaactggggaggccggtggttctcggaccgcgaagggcagcctcccttccggaacttgttttagacaacactctctccaccagagctccgaccctccccaccaaacttccgcaat

SEQ ID NO: 14535 - RNA, 1698 nt, Homo sapiens
  source 1..1698: mol_type = other RNA
gctgggattacaggcatgagccaccgtatccggccccaagttttatatatgaagtgacttagtgactatatattgcttaggtatctgatcttaccaaataaagttttacctgaatagctgacttcagcgatgaagaatccaacaccacattaagataataccacaggagacaaatttataagcatttctggaaccctaactggggctactgtgtgtgaaatacagtaaactgaactgacaatctgatcatcacaagaacaaatcctaatagtcttcacaaagaatatgaattcaatctctatcccacatcttttgctcaattttatatgctagcatttgtagatgttttcagggcaaaacaacctccctcacccaccttataaaacataccaaaatgattactatagtcatgtctatgatagggttaaatttgactcacttctttgaaattacagaaacgtatacacaaatatgtaattaaagagcaaatgtgtgatagtgagaaacagactacgcagggctgaatataaggaagataacatgagcctacaatgtgagaaacttacatactatctcatttaattcttacaataatcctgtaatagtatatattattattcatttcttctagctgagcaaacaaaggctcagagaaaataaaaattaaacccaaagtcacctagctaataagtggcattcctagaaatctagcccagagttgacaactcactctaaagaccatgatcagttgagaaagttttataacaccatggaatgagaaaaataaagacgacctacatttttcataaagatgcatttattcaatttataggattctcctataagatggtatcctttccacttctttgcatgagaaagtcctttactttataaagtaatgataaaagtatatcatggtactttttattcaagtcttatgtggcaagagtaaaagatggcaactgtaaattagtttccacttctgttgttgaacctttactcttacatgatgtcccaaagcctcataatcacaatgctatttcatattttcaaaagaccagattttacccaaaaaagaaaaatgtttgattaaatatttaagaaatgattaccttcctacatgaatgacaaatatttttaaaactgctatgtgtagctgcctttataggcaaaattataagggaggtctccccattccctccaccaccatctttccaccagttgcccagttttaacaatttggcttctttctccctccagcacactgcatctgccctcccaccagcacatttcaacactcaacctcagtggatatgctcattatcttgactgtggctgtagtttcacagatatatatgtatatcaacatttattgaatgttatactttaaatatgtgcagtttaatgtatatcagaaaaaaaccttaatacagatgctaaaaaaaaacctcctaaggtaataacgtatttgattcttttgatgtacattattattttcaccacctgaaggtatttacacctgttttcatggccaccagcaaaagatgcatggaagaatttttttccccccatacatgagacttaaagaaatttcttttctcatcctcctcagtatcatatttaagttttctcaactgaatgtttcttttttaatctggcttatttctttctttgattactagaaagatacattttaaa

SEQ ID NO: 14536 - RNA, 1817 nt, Homo sapiens
  source 1..1817: mol_type = other RNA
gctgggattacaggcatgagccaccgtgccaggcctcaaggctacgtttgttacacagctgtcttgactaaactagatggcctggctagacctagaagcctgtatgttgtataacttctcaatagaatgagacaacatactttaaaaaaaaacgtactgagattttaaagtcttaggatacctaaacctttttctctgaggaaataatttcgatttgataaatggcagctacaagaggaaaaacaaaaatgagactaatgtgagcaaaaaactactgaaactcaaaattacatggacctcaattctcatgttccaattcaaaaaagagcagaacagtgcatagcatagtacaagacagtccaaacgtgtgtctgtgtcactggaatcacctggagagctttggaatactagatctttggatatagcgggtgcagggtgggccagaatgtcaatattgaacatcaagaagttggagtgcctgacacattattaaaagacccagttggccctagcaaatgatggtggaagaggtgatgttacaaatctctatttaaaaacatctcccaaattaattctgatgctcacatttggaaaccataggtgtagggggaagaatacagcttttgtgatccaatggcaactttactacttaaaactgcaagacctcgaacaattactatacttctatgaacgttagttcattccccggtagacagatcataaaatcactatttctgggctgatataatagaaattatacaaagcatcaggcacagttcctggcatacagcaggtattcaatatataataggtctcattaaatggtctaaaacatccactatgtatatttataaacacaaggacacacctactggcaccacggtgttatttttctacactagaaattaactatttactttccatgtatgtggacttctagagagatcagagctttatagacctttcccctcctcttttcaataataatgtaaaagttaaacccctcccccatctctaatagatactaccaacagatacttacatggatgcttttaataatgcagttttgctttttagaagagtttcagactgttttaaagcgtatttaacttttcagattagagttctaagaaactgttttaattcactgccatttgaagtaatatgaaagccaacaaaaaaagtttcaaaaaactggaacccatcaccttcccgtaatctgacaactagtaaatgtctcctcagggttgttttagagtaaaactaagaaacgaagcgtagggtacccacagagaaccatgctaccggaaggcagacagacaatgtcctggactcttttttttagttttgtaacctggttggactctactttcaataactgaagaattaaggaaaaggctcaatgccctgcccccacgccgggccagagaagacaaagacgtccactctcagaccgcaggagagaaaatggcaggagcgcctcacctccaatttcgactgggaggagtgggggtgcggggtcagggagggaacccatcagccgcgaggctcgacccccagcccccttcttccatcacaaacaagtggttaggaggaagaagctggccccagcccttcccgctccgagccggcggcctcgtcttttgggtctgggggcgtggggaaggagaaggccgcgcgaccccagtcccatctccagaattcagcaccctgctctcggctcccgctagccccgggcctcgcggcgccctggtcatcgagatgtcctcggagggcgccgcccgcgccgcgagaaagatggcgcccgccgagcaact

SEQ ID NO: 14537 - RNA, 4912 nt, Homo sapiens
  source 1..4912: mol_type = other RNA
gctgggattacaggcatgagccaccgtgccaggcctcatttgtctttttagaaaagttatacgcatatataagccaatacagatatttttgtcctttttatacaaatgctgagttgctgcgttcattattattttggtgcttgacttttttccacttgatagtagagctcttagagttctgtgtcactaaagatcttcctcattttttagcagttaattttgttataggtgaatatgtgaaggaatcataatgcattttttaatccactttgggtctcactctgtcgctcaggctggagtgcagtggcacaatctcaactcactgcaacctctgcctcctgggtttaagtgactcttatgcttcagccaccgagtggctgggattacaggcatggaccacacccggctaattttgttgtttttagtacatacagggtttcatcatgttgcccaggcttgcctccaattcctggcctcatgtgatctgaccgcctcagcctcccaaagtgttgggattacaggcgtgagccactgcacctggcctcctttccaatttctgacctctgatttttcttgtttgtctaattgtgatgcctaatgcctccagaataataagttaaaaaagaaggataatagactgggtgtgaggtggctgaagcctgtaatcccaacactttgggagaccgagacgggcggatcacctgagaccaggagtttgaaaccagcctgaccaacatggtgaaaccccgtctctactaaatatacaaaaatcagccgggcatggtggtgcacgcctgtaatcccagctactcgggaggctgaggcaggagaattgcttgaacccgggaggcggaggttgcagtgagctgacattgcgtcattgcactccagcctgggtgacagagcaagattctatcaaaaaaaaaaaaaaaaaaaaaaaaagaagaagaagaaaaagaatagcggccattccttccttgcctttaatgtaagtaggaatgttattagttttctccactaagtgagtgcattgattcttgggctggatcttagtccagtgaagaatttcgggatttggagaggagtatacttgagaaacatattagtccattatcacattgctataaagaaacacctgagactagatagtttgtaagaaaaggggtttaattagctcacaggctatataggaagcgtggcaacatctgcttctagggagtcctcggggaatttttactcatggcagaaggcaaagtgggagcaggcatcttcacgtggccaaagcaggagaaagagagagtggggaggtgctacacacttttaaactaccagatctcacgataactcactgtcatgagaccagcactgaggggacggtgccaaaccattcatgaaggcttcacacccatgatccagtcgcctcccagccggccccacctctaacattggggattacacttcaacgtgagatttggtggggacacagatccaaaccatatcaaaatccaattaaaaatttttttgtttgttttagacacagggtcttgctatattggccaagatggtctcatacccctaccctcaaattaacctctcacttcagcctcccaaaatgctgggattacaggtgtgagccacagcttccagccttaatataaatcttgactcagcattctttattctcactgtcagactgctcaatgcatcccttattgaagtttcttgaagtttcgaaaaacaggtatgttcagataattttcagcagaattcatcaaaaaatgttaacaactctttaaaatttttacacattttatttagcacaattgctaccatttaaaaatcaggtgttttggccaggcatggtggctcacgcctgtaatctcagctctttgggaggccgaggcagacagatcacctgaagtcaggagtttgagaccagcctggccaacattgtgaaaccccatctccactaaaaatacaaaaattagccaggcgtggtggtgtgcacccatagtcccagctacttgggaggctgaggtaggagaatggcttgaactcaggaggtgaagtttgcagtgagccaagatcacgccattgcattccagcctgggtgagagagcgagactgtctcaaaaaccaaaacaaaacaaaatcaggtgttttattccactccccccatcagtgttttcttatttctaatacttctagaaacctcctttaagttttcctattttagacagacaccacacaggtgctcttttttgggaggagggggatgagagtcttactctgttgcccaggctggagtgcaatggtgcaatcatagctcactgtagcctctgactcctgtgctcaacccatcctcccaccatggcctcccaagtagctgagactacaggcacacaccacgctgcccagctaattttttaattttttagtagagtcaggtgtcactgtgttgcccaggctggtcttgaacctctggcctcaagcaaaactcccaccttggcctcccaaattgctcggattacaggagtgagccactgcacctggcccatagatgcattaacacctgtctatggtggtggagagaaggctcactgcctctcccaggccactgggaaatgaccttgtgtattctgcaaatacacaagaggatctgaagctattcttgagggagactttcaacagcaaaactcagagcacaaaatggaaaataatcataaaaaaattaaataataatactatcaaatcataacgtgaataatgctgttattagagttgaagagaagcccttagaaatgggacaaacattgtaattctcttagagaactgtaacttaaacagaaatacacttaatagaagaggaaagaaaatggttcatgtgacacaaaggtcccatgtgttgacttctttggtaagatcaaataagtatttaagcctagcaatagggtcagtccagttagtatttctcctcacaaatggtgaatatcaactccaggatggctggagttttctcatggtttggttccacgccatctgcatgtctttacaagtgataaaaaccagaattttccagctgctactagtcacagggggtccccaatatgggttgtttaattatgatgacgggtcctgtcaattgcatccagtaaaattggtcacatagagaactcatctaaaactgaggttttgttgtggttttgaaaggtccattggaatccagatttgcaaagcatgtcaagttatggcaaaacatatgccacccatctcaaaatctttccttattattgcataactttgaaagccactgttgcgtttgttgcgatgaggttagagttttgttgacatgatgatattactctcttcctctgggtgagacacatctggattctcacttggagcagggctctgtacatccttctgggatttggttgagtaggtaatatacatgcttctcattaggaaaattccagcaattactgcaaaatagctcccataaactaaaaactgaatgctgactggcaagttgagccctctctgatctactacaatcacagtcatgatggtctgaatcaccaaggcaataaaggtgttgattccaaataccaaggcatagcgttccacattcagattaactgcaatctgaaatactgctatggttataagaagcatatagctggacttgaatatcaaatagccagcatagcacgcccagatattggctgtgtaatgcatgagaaataaagaaccggcattgacaactgagaagaccaccagagccagctctcccagaaggtcccagttgactttcacataacccactgcaaaggcagccacagcccctccaaaggttgcaatagcttctacggccccattatagatggaagaatcttgggatggcgccttgtaatcccacaggatttgaacatagttcaaaacctggttaaaacctgctgtggcgaaagcccaccatagagaccagtagaaaagacgttttgaggagtagcactccttcaaatcttggaaccactgcacaaaaacgtccacagtcacattgcttggtttcaggctgttcagctggcccttattcagcttccctgaagtgctgagtatttctgatgtgggtttctgctcttcacagcctggtgcttcaccttcgtgagtttcctctaatactggattcacgcttgatgacttctttatttctctgctgggttttgcatgaaaaaacatgcttttcttgggcattggtaggaaaagtgagaaaaggaaagccacggagacagaggccaaggatatgacgttgaggtaaaagtacgacatgttcgccagggataccaagagttgagccagcaccgaccctgctgtgtaggcggccagcgtgacgctcctgcagtagccgctcactctctggtagtgctcggggctgaccacgctgtatatgtaggcgtagtaggccacctcggcggcggtgaccatcccatagaagaactctacaacctgcatggtcttcactccttggccaaacaacagcagcagccaggtaatgatgaaactgataccttgcaagatgatgactggcttgtagcggacataatcggtgaggacaaacacaggcagcagcagcaccaggtaggagtatgtccaaacggggaagatctcatttgttatctctgcactggtcaggtttttatctggtccagataaatatgggataaggaatggttctgagggtctcatcatggagaaaaaaccaaataagcagaggatcacagtggggtaaatccaggaactgcttagtgaagttctgtaacaatccatggctacagaagggagtgtctgttcaccaaatcgctcacttgccgcacgaccacgcacccgcggctgtcggatggatccaggcgctctt

SEQ ID NO: 14538 - RNA, 5168 nt, Homo sapiens
  source 1..5168: mol_type = other RNA
gctgggattacaggcatgagccaccgtgccaggcctcatttgtctttttagaaaagttatacgcatatataagccaatacagatatttttgtcctttttatacaaatgctgagttgctgcgttcattattattttggtgcttgacttttttccacttgatagtagagctcttagagttctgtgtcactaaagatcttcctcattttttagcagttaattttgttataggtgaatatgtgaaggaatcataatgcattttttaatccactttgggtctcactctgtcgctcaggctggagtgcagtggcacaatctcaactcactgcaacctctgcctcctgggtttaagtgactcttatgcttcagccaccgagtggctgggattacaggcatggaccacacccggctaattttgttgtttttagtacatacagggtttcatcatgttgcccaggcttgcctccaattcctggcctcatgtgatctgaccgcctcagcctcccaaagtgttgggattacaggcgtgagccactgcacctggcctcctttccaatttctgacctctgatttttcttgtttgtctaattgtgatgcctaatgcctccagaataataagttaaaaaagaaggataatagactgggtgtgaggtggctgaagcctgtaatcccaacactttgggagaccgagacgggcggatcacctgagaccaggagtttgaaaccagcctgaccaacatggtgaaaccccgtctctactaaatatacaaaaatcagccgggcatggtggtgcacgcctgtaatcccagctactcgggaggctgaggcaggagaattgcttgaacccgggaggcggaggttgcagtgagctgacattgcgtcattgcactccagcctgggtgacagagcaagattctatcaaaaaaaaaaaaaaaaaaaaaaaaagaagaagaagaaaaagaatagcggccattccttccttgcctttaatgtaagtaggaatgttattagttttctccactaagtgagtgcattgattcttgggctggatcttagtccagtgaagaatttcgggatttggagaggagtatacttgagaaacatattagtccattatcacattgctataaagaaacacctgagactagatagtttgtaagaaaaggggtttaattagctcacaggctatataggaagcgtggcaacatctgcttctagggagtcctcggggaatttttactcatggcagaaggcaaagtgggagcaggcatcttcacgtggccaaagcaggagaaagagagagtggggaggtgctacacacttttaaactaccagatctcacgataactcactgtcatgagaccagcactgaggggacggtgccaaaccattcatgaaggcttcacacccatgatccagtcgcctcccagccggccccacctctaacattggggattacacttcaacgtgagatttggtggggacacagatccaaaccatatcaaaatccaattaaaaatttttttgtttgttttagacacagggtcttgctatattggccaagatggtctcatacccctaccctcaaattaacctctcacttcagcctcccaaaatgctgggattacaggtgtgagccacagcttccagccttaatataaatcttgactcagcattctttattctcactgtcagactgctcaatgcatcccttattgaagtttcttgaagtttcgaaaaacaggtatgttcagataattttcagcagaattcatcaaaaaatgttaacaactctttaaaatttttacacattttatttagcacaattgctaccatttaaaaatcaggtgttttggccaggcatggtggctcacgcctgtaatctcagctctttgggaggccgaggcagacagatcacctgaagtcaggagtttgagaccagcctggccaacattgtgaaaccccatctccactaaaaatacaaaaattagccaggcgtggtggtgtgcacccatagtcccagctacttgggaggctgaggtaggagaatggcttgaactcaggaggtgaagtttgcagtgagccaagatcacgccattgcattccagcctgggtgagagagcgagactgtctcaaaaaccaaaacaaaacaaaatcaggtgttttattccactccccccatcagtgttttcttatttctaatacttctagaaacctcctttaagttttcctattttagacagacaccacacaggtgctcttttttgggaggagggggatgagagtcttactctgttgcccaggctggagtgcaatggtgcaatcatagctcactgtagcctctgactcctgtgctcaacccatcctcccaccatggcctcccaagtagctgagactacaggcacacaccacgctgcccagctaattttttaattttttagtagagtcaggtgtcactgtgttgcccaggctggtcttgaacctctggcctcaagcaaaactcccaccttggcctcccaaattgctcggattacaggagtgagccactgcacctggcccatagatgcattaacacctgtctatggtggtggagagaaggctcactgcctctcccaggccactgggaaatgaccttgtgtattctgcaaatacacaagaggatctgaagctattcttgagggagactttcaacagcaaaactcagagcacaaaatggaaaataatcataaaaaaattaaataataatactatcaaatcataacgtgaataatgctgttattagagttgaagagaagcccttagaaatgggacaaacattgtaattctcttagagaactgtaacttaaacagaaatacacttaatagaagaggaaagaaaatggttcatgtgacacaaaggtcccatgtgttgacttctttggtaagatcaaataagtatttaagcctagcaatagggtcagtccagttagtatttctcctcacaaatggtgaatatcaactccaggatggctggagttttctcatggtttggttccacgccatctgcatgtctttacaagtgataaaaaccagaattttccagctgctactagtcacagggggtccccaatatgggttgtttaattatgatgacgggtcctgtcaattgcatccagtaaaattggtcacatagagaactcatctaaaactgaggttttgttgtggttttgaaaggtccattggaatccagatttgcaaagcatgtcaagttatggcaaaacatatgccacccatctcaaaatctttccttattattgcataactttgaaagccactgttgcgtttgttgcgatgaggttagagttttgttgacatgatgatattactctcttcctctgggtgagacacatctggattctcacttggagcagggctctgtacatccttctgggatttggttgagtaggtaatatacatgcttctcattaggaaaattccagcaattactgcaaaatagctcccataaactaaaaactgaatgctgactggcaagttgagccctctctgatctactacaatcacagtcatgatggtctgaatcaccaaggcaataaaggtgttgattccaaataccaaggcatagcgttccacattcagattaactgcaatctgaaatactgctatggttataagaagcatatagctggacttgaatatcaaatagccagcatagcacgcccagatattggctgtgtaatgcatgagaaataaagaaccggcattgacaactgagaagaccaccagagccagctctcccagaaggtcccagttgactttcacataacccactgcaaaggcagccacagcccctccaaaggttgcaatagcttctacggccccattatagatggaagaatcttgggatggcgccttgtaatcccacaggatttgaacatagttcaaaacctggttaaaacctgctgtggcgaaagcccaccatagagaccagtagaaaagacgttttgaggagtagcactccttcaaatcttggaaccactgcacaaaaacgtccacagtcacattgcttggtttcaggctgttcagctggcccttattcagcttccctgaagtgctgagtatttctgatgtgggtttctgctcttcacagcctggtgcttcaccttcgtgagtttcctctaatactggattcacgcttgatgacttctttatttctctgctgggttttgcatgaaaaaacatgcttttcttgggcattggtaggaaaagtgagaaaaggaaagccacggagacagaggccaaggatatgacgttgaggtaaaagtacgacatgttcgccagggataccaagagttgagccagcaccgaccctgctgtgtaggcggccagcgtgacgctcctgcagtagccgctcactctctggtagtgctcggggctgaccacgctgtatatgtaggcgtagtaggccacctcggcggcggtgaccatcccatagaagaactctacaacctgcatggtcttcactccttggccaaacaacagcagcagccaggtaatgatgaaactgataccttgcaagatgatgactggcttgtagcggacataatcggtgaggacaaacacaggcagcagcagcaccaggtaggagtatgtccaaacggggaagatctcatttgttatctctgcactggtcaggtttttatctggtccagataaatatgggataaggaatggttctgagggtctcatcatggagaaaaaaccaaataagcagaggatcacagtggggtaaatccaggaactgcttagtgaagttctgtaacaatccatggctgtgaaagccagatgtttacctttccccttcattttctgtgtgttccaaatcacaagatagtccttttaaaagttactcctgtagcagtcatcttcacccattattataagctctatcactttttaaaaaggtacaagaacactgtgtaaacggtagattaaaaattttaaaaggctgggtgtagtggctcatgcttgtaatcccagcgctttgggaggctgaggcaggtggatcacctgaggtcaggagttcaagactagcctggccaacagagtgaaaccccatctctactaataacgcaaaaattagtcggttgcggtggtgggtgcctgtaatccca

SEQ ID NO: 14539 - RNA, 5002 nt, Homo sapiens
  source 1..5002: mol_type = other RNA
gctgggattacaggcatgagccaccgtgccaggcctcatttgtctttttagaaaagttatacgcatatataagccaatacagatatttttgtcctttttatacaaatgctgagttgctgcgttcattattattttggtgcttgacttttttccacttgatagtagagctcttagagttctgtgtcactaaagatcttcctcattttttagcagttaattttgttataggtgaatatgtgaaggaatcataatgcattttttaatccactttgggtctcactctgtcgctcaggctggagtgcagtggcacaatctcaactcactgcaacctctgcctcctgggtttaagtgactcttatgcttcagccaccgagtggctgggattacaggcatggaccacacccggctaattttgttgtttttagtacatacagggtttcatcatgttgcccaggcttgcctccaattcctggcctcatgtgatctgaccgcctcagcctcccaaagtgttgggattacaggcgtgagccactgcacctggcctcctttccaatttctgacctctgatttttcttgtttgtctaattgtgatgcctaatgcctccagaataataagttaaaaaagaaggataatagactgggtgtgaggtggctgaagcctgtaatcccaacactttgggagaccgagacgggcggatcacctgagaccaggagtttgaaaccagcctgaccaacatggtgaaaccccgtctctactaaatatacaaaaatcagccgggcatggtggtgcacgcctgtaatcccagctactcgggaggctgaggcaggagaattgcttgaacccgggaggcggaggttgcagtgagctgacattgcgtcattgcactccagcctgggtgacagagcaagattctatcaaaaaaaaaaaaaaaaaaaaaaaaagaagaagaagaaaaagaatagcggccattccttccttgcctttaatgtaagtaggaatgttattagttttctccactaagtgagtgcattgattcttgggctggatcttagtccagtgaagaatttcgggatttggagaggagtatacttgagaaacatattagtccattatcacattgctataaagaaacacctgagactagatagtttgtaagaaaaggggtttaattagctcacaggctatataggaagcgtggcaacatctgcttctagggagtcctcggggaatttttactcatggcagaaggcaaagtgggagcaggcatcttcacgtggccaaagcaggagaaagagagagtggggaggtgctacacacttttaaactaccagatctcacgataactcactgtcatgagaccagcactgaggggacggtgccaaaccattcatgaaggcttcacacccatgatccagtcgcctcccagccggccccacctctaacattggggattacacttcaacgtgagatttggtggggacacagatccaaaccatatcaaaatccaattaaaaatttttttgtttgttttagacacagggtcttgctatattggccaagatggtctcatacccctaccctcaaattaacctctcacttcagcctcccaaaatgctgggattacaggtgtgagccacagcttccagccttaatataaatcttgactcagcattctttattctcactgtcagactgctcaatgcatcccttattgaagtttcttgaagtttcgaaaaacaggtatgttcagataattttcagcagaattcatcaaaaaatgttaacaactctttaaaatttttacacattttatttagcacaattgctaccatttaaaaatcaggtgttttggccaggcatggtggctcacgcctgtaatctcagctctttgggaggccgaggcagacagatcacctgaagtcaggagtttgagaccagcctggccaacattgtgaaaccccatctccactaaaaatacaaaaattagccaggcgtggtggtgtgcacccatagtcccagctacttgggaggctgaggtaggagaatggcttgaactcaggaggtgaagtttgcagtgagccaagatcacgccattgcattccagcctgggtgagagagcgagactgtctcaaaaaccaaaacaaaacaaaatcaggtgttttattccactccccccatcagtgttttcttatttctaatacttctagaaacctcctttaagttttcctattttagacagacaccacacaggtgctcttttttgggaggagggggatgagagtcttactctgttgcccaggctggagtgcaatggtgcaatcatagctcactgtagcctctgactcctgtgctcaacccatcctcccaccatggcctcccaagtagctgagactacaggcacacaccacgctgcccagctaattttttaattttttagtagagtcaggtgtcactgtgttgcccaggctggtcttgaacctctggcctcaagcaaaactcccaccttggcctcccaaattgctcggattacaggagtgagccactgcacctggcccatagatgcattaacacctgtctatggtggtggagagaaggctcactgcctctcccaggccactgggaaatgaccttgtgtattctgcaaatacacaagaggatctgaagctattcttgagggagactttcaacagcaaaactcagagcacaaaatggaaaataatcataaaaaaattaaataataatactatcaaatcataacgtgaataatgctgttattagagttgaagagaagcccttagaaatgggacaaacattgtaattctcttagagaactgtaacttaaacagaaatacacttaatagaagaggaaagaaaatggttcatgtgacacaaaggtcccatgtgttgacttctttggtaagatcaaataagtatttaagcctagcaatagggtcagtccagttagtatttctcctcacaaatggtgaatatcaactccaggatggctggagttttctcatggtttggttccacgccatctgcatgtctttacaagtgataaaaaccagaattttccagctgctactagtcacagggggtccccaatatgggttgtttaattatgatgacgggtcctgtcaattgcatccagtaaaattggtcacatagagaactcatctaaaactgaggttttgttgtggttttgaaaggtccattggaatccagatttgcaaagcatgtcaagttatggcaaaacatatgccacccatctcaaaatctttccttattattgcataactttgaaagccactgttgcgtttgttgcgatgaggttagagttttgttgacatgatgatattactctcttcctctgggtgagacacatctggattctcacttggagcagggctctgtacatccttctgggatttggttgagtaggtaatatacatgcttctcattaggaaaattccagcaattactgcaaaatagctcccataaactaaaaactgaatgctgactggcaagttgagccctctctgatctactacaatcacagtcatgatggtctgaatcaccaaggcaataaaggtgttgattccaaataccaaggcatagcgttccacattcagattaactgcaatctgaaatactgctatggttataagaagcatatagctggacttgaatatcaaatagccagcatagcacgcccagatattggctgtgtaatgcatgagaaataaagaaccggcattgacaactgagaagaccaccagagccagctctcccagaaggtcccagttgactttcacataacccactgcaaaggcagccacagcccctccaaaggttgcaatagcttctacggccccattatagatggaagaatcttgggatggcgccttgtaatcccacaggatttgaacatagttcaaaacctggttaaaacctgctgtggcgaaagcccaccatagagaccagtagaaaagacgttttgaggagtagcactccttcaaatcttggaaccactgcacaaaaacgtccacagtcacattgcttggtttcaggctgttcagctggcccttattcagcttccctgaagtgctgagtatttctgatgtgggtttctgctcttcacagcctggtgcttcaccttcgtgagtttcctctaatactggattcacgcttgatgacttctttatttctctgctgggttttgcatgaaaaaacatgcttttcttgggcattggtaggaaaagtgagaaaaggaaagccacggagacagaggccaaggatatgacgttgaggtaaaagtacgacatgttcgccagggataccaagagttgagccagcaccgaccctgctgtgtaggcggccagcgtgacgctcctgcagtagccgctcactctctggtagtgctcggggctgaccacgctgtatatgtaggcgtagtaggccacctcggcggcggtgaccatcccatagaagaactctacaacctgcatggtcttcactccttggccaaacaacagcagcagccaggtaatgatgaaactgataccttgcaagatgatgactggcttgtagcggacataatcggtgaggacaaacacaggcagcagcagcaccaggtaggagtatgtccaaacggggaagatctcatttgttatctctgcactggtcaggtttttatctggtccagataaatatgggataaggaatggttctgagggtctcatcatggagaaaaaaccaaataagcagaggatcacagtggggtaaatccaggaactgcttagtgaagttctgtaacaatccatggctgtttttttctgtgcccccagtttctttctttctagaaccaagctggcttcctgccttcaggtccaacttctgctccttcctgctgcccgccactatgaaaatccctttccataccctggagtctcttgtcctcctccttcagacagagctgccaagagcaatagctttatacgc

SEQ ID NO: 14540 - RNA, 5108 nt, Homo sapiens
  source 1..5108: mol_type = other RNA
gctgggattacaggcatgagccaccgtgccaggcctcatttgtctttttagaaaagttatacgcatatataagccaatacagatatttttgtcctttttatacaaatgctgagttgctgcgttcattattattttggtgcttgacttttttccacttgatagtagagctcttagagttctgtgtcactaaagatcttcctcattttttagcagttaattttgttataggtgaatatgtgaaggaatcataatgcattttttaatccactttgggtctcactctgtcgctcaggctggagtgcagtggcacaatctcaactcactgcaacctctgcctcctgggtttaagtgactcttatgcttcagccaccgagtggctgggattacaggcatggaccacacccggctaattttgttgtttttagtacatacagggtttcatcatgttgcccaggcttgcctccaattcctggcctcatgtgatctgaccgcctcagcctcccaaagtgttgggattacaggcgtgagccactgcacctggcctcctttccaatttctgacctctgatttttcttgtttgtctaattgtgatgcctaatgcctccagaataataagttaaaaaagaaggataatagactgggtgtgaggtggctgaagcctgtaatcccaacactttgggagaccgagacgggcggatcacctgagaccaggagtttgaaaccagcctgaccaacatggtgaaaccccgtctctactaaatatacaaaaatcagccgggcatggtggtgcacgcctgtaatcccagctactcgggaggctgaggcaggagaattgcttgaacccgggaggcggaggttgcagtgagctgacattgcgtcattgcactccagcctgggtgacagagcaagattctatcaaaaaaaaaaaaaaaaaaaaaaaaagaagaagaagaaaaagaatagcggccattccttccttgcctttaatgtaagtaggaatgttattagttttctccactaagtgagtgcattgattcttgggctggatcttagtccagtgaagaatttcgggatttggagaggagtatacttgagaaacatattagtccattatcacattgctataaagaaacacctgagactagatagtttgtaagaaaaggggtttaattagctcacaggctatataggaagcgtggcaacatctgcttctagggagtcctcggggaatttttactcatggcagaaggcaaagtgggagcaggcatcttcacgtggccaaagcaggagaaagagagagtggggaggtgctacacacttttaaactaccagatctcacgataactcactgtcatgagaccagcactgaggggacggtgccaaaccattcatgaaggcttcacacccatgatccagtcgcctcccagccggccccacctctaacattggggattacacttcaacgtgagatttggtggggacacagatccaaaccatatcaaaatccaattaaaaatttttttgtttgttttagacacagggtcttgctatattggccaagatggtctcatacccctaccctcaaattaacctctcacttcagcctcccaaaatgctgggattacaggtgtgagccacagcttccagccttaatataaatcttgactcagcattctttattctcactgtcagactgctcaatgcatcccttattgaagtttcttgaagtttcgaaaaacaggtatgttcagataattttcagcagaattcatcaaaaaatgttaacaactctttaaaatttttacacattttatttagcacaattgctaccatttaaaaatcaggtgttttggccaggcatggtggctcacgcctgtaatctcagctctttgggaggccgaggcagacagatcacctgaagtcaggagtttgagaccagcctggccaacattgtgaaaccccatctccactaaaaatacaaaaattagccaggcgtggtggtgtgcacccatagtcccagctacttgggaggctgaggtaggagaatggcttgaactcaggaggtgaagtttgcagtgagccaagatcacgccattgcattccagcctgggtgagagagcgagactgtctcaaaaaccaaaacaaaacaaaatcaggtgttttattccactccccccatcagtgttttcttatttctaatacttctagaaacctcctttaagttttcctattttagacagacaccacacaggtgctcttttttgggaggagggggatgagagtcttactctgttgcccaggctggagtgcaatggtgcaatcatagctcactgtagcctctgactcctgtgctcaacccatcctcccaccatggcctcccaagtagctgagactacaggcacacaccacgctgcccagctaattttttaattttttagtagagtcaggtgtcactgtgttgcccaggctggtcttgaacctctggcctcaagcaaaactcccaccttggcctcccaaattgctcggattacaggagtgagccactgcacctggcccatagatgcattaacacctgtctatggtggtggagagaaggctcactgcctctcccaggccactgggaaatgaccttgtgtattctgcaaatacacaagaggatctgaagctattcttgagggagactttcaacagcaaaactcagagcacaaaatggaaaataatcataaaaaaattaaataataatactatcaaatcataacgtgaataatgctgttattagagttgaagagaagcccttagaaatgggacaaacattgtaattctcttagagaactgtaacttaaacagaaatacacttaatagaagaggaaagaaaatggttcatgtgacacaaaggtcccatgtgttgacttctttggtaagatcaaataagtatttaagcctagcaatagggtcagtccagttagtatttctcctcacaaatggtgaatatcaactccaggatggctggagttttctcatggtttggttccacgccatctgcatgtctttacaagtgataaaaaccagaattttccagctgctactagtcacagggggtccccaatatgggttgtttaattatgatgacgggtcctgtcaattgcatccagtaaaattggtcacatagagaactcatctaaaactgaggttttgttgtggttttgaaaggtccattggaatccagatttgcaaagcatgtcaagttatggcaaaacatatgccacccatctcaaaatctttccttattattgcataactttgaaagccactgttgcgtttgttgcgatgaggttagagttttgttgacatgatgatattactctcttcctctgggtgagacacatctggattctcacttggagcagggctctgtacatccttctgggatttggttgagtaggtaatatacatgcttctcattaggaaaattccagcaattactgcaaaatagctcccataaactaaaaactgaatgctgactggcaagttgagccctctctgatctactacaatcacagtcatgatggtctgaatcaccaaggcaataaaggtgttgattccaaataccaaggcatagcgttccacattcagattaactgcaatctgaaatactgctatggttataagaagcatatagctggacttgaatatcaaatagccagcatagcacgcccagatattggctgtgtaatgcatgagaaataaagaaccggcattgacaactgagaagaccaccagagccagctctcccagaaggtcccagttgactttcacataacccactgcaaaggcagccacagcccctccaaaggttgcaatagcttctacggccccattatagatggaagaatcttgggatggcgccttgtaatcccacaggatttgaacatagttcaaaacctggttaaaacctgctgtggcgaaagcccaccatagagaccagtagaaaagacgttttgaggagtagcactccttcaaatcttggaaccactgcacaaaaacgtccacagtcacattgcttggtttcaggctgttcagctggcccttattcagcttccctgaagtgctgagtatttctgatgtgggtttctgctcttcacagcctggtgcttcaccttcgtgagtttcctctaatactggattcacgcttgatgacttctttatttctctgctgggttttgcatgaaaaaacatgcttttcttgggcattggtaggaaaagtgagaaaaggaaagccacggagacagaggccaaggatatgacgttgaggtaaaagtacgacatgttcgccagggataccaagagttgagccagcaccgaccctgctgtgtaggcggccagcgtgacgctcctgcagtagccgctcactctctggtagtgctcggggctgaccacgctgtatatgtaggcgtagtaggccacctcggcggcggtgaccatcccatagaagaactctacaacctgcatggtcttcactccttggccaaacaacagcagcagccaggtaatgatgaaactgataccttgcaagatgatgactggcttgtagcggacataatcggtgaggacaaacacaggcagcagcagcaccaggtaggagtatgtccaaacggggaagatctcatttgttatcttgacacctggatcactgaggttgctggagaaagcaggaggccacagagcaaagaccacacaactgagctgctccttggagggaaggtctgttaactggtccacagtggctcgagaagcagaacccagtggattcattgagttgcttctgaccctgcatctgtcctttgttgtcttaattgtggcatgcttcaacctctgcactggtcaggtttttatctggtccagataaatatgggataaggaatggttctgagggtctcatcatggagaaaaaaccaaataagcagaggatcacagtggggtaaatccaggaactgcttagtgaagttctgtaacaatccatggctacagaagggagtgtctgttcaccaaatcgctcacttgccgcacgaccacgcacccgcggctgtcggatggatccaggcgctctt

SEQ ID NO: 14541 - RNA, 5487 nt, Homo sapiens
  source 1..5487: mol_type = other RNA
gctgggattacaggcatgagccaccgtgccaggcctcatttgtctttttagaaaagttatacgcatatataagccaatacagatatttttgtcctttttatacaaatgctgagttgctgcgttcattattattttggtgcttgacttttttccacttgatagtagagctcttagagttctgtgtcactaaagatcttcctcattttttagcagttaattttgttataggtgaatatgtgaaggaatcataatgcattttttaatccactttgggtctcactctgtcgctcaggctggagtgcagtggcacaatctcaactcactgcaacctctgcctcctgggtttaagtgactcttatgcttcagccaccgagtggctgggattacaggcatggaccacacccggctaattttgttgtttttagtacatacagggtttcatcatgttgcccaggcttgcctccaattcctggcctcatgtgatctgaccgcctcagcctcccaaagtgttgggattacaggcgtgagccactgcacctggcctcctttccaatttctgacctctgatttttcttgtttgtctaattgtgatgcctaatgcctccagaataataagttaaaaaagaaggataatagactgggtgtgaggtggctgaagcctgtaatcccaacactttgggagaccgagacgggcggatcacctgagaccaggagtttgaaaccagcctgaccaacatggtgaaaccccgtctctactaaatatacaaaaatcagccgggcatggtggtgcacgcctgtaatcccagctactcgggaggctgaggcaggagaattgcttgaacccgggaggcggaggttgcagtgagctgacattgcgtcattgcactccagcctgggtgacagagcaagattctatcaaaaaaaaaaaaaaaaaaaaaaaaagaagaagaagaaaaagaatagcggccattccttccttgcctttaatgtaagtaggaatgttattagttttctccactaagtgagtgcattgattcttgggctggatcttagtccagtgaagaatttcgggatttggagaggagtatacttgagaaacatattagtccattatcacattgctataaagaaacacctgagactagatagtttgtaagaaaaggggtttaattagctcacaggctatataggaagcgtggcaacatctgcttctagggagtcctcggggaatttttactcatggcagaaggcaaagtgggagcaggcatcttcacgtggccaaagcaggagaaagagagagtggggaggtgctacacacttttaaactaccagatctcacgataactcactgtcatgagaccagcactgaggggacggtgccaaaccattcatgaaggcttcacacccatgatccagtcgcctcccagccggccccacctctaacattggggattacacttcaacgtgagatttggtggggacacagatccaaaccatatcaaaatccaattaaaaatttttttgtttgttttagacacagggtcttgctatattggccaagatggtctcatacccctaccctcaaattaacctctcacttcagcctcccaaaatgctgggattacaggtgtgagccacagcttccagccttaatataaatcttgactcagcattctttattctcactgtcagactgctcaatgcatcccttattgaagtttcttgaagtttcgaaaaacaggtatgttcagataattttcagcagaattcatcaaaaaatgttaacaactctttaaaatttttacacattttatttagcacaattgctaccatttaaaaatcaggtgttttggccaggcatggtggctcacgcctgtaatctcagctctttgggaggccgaggcagacagatcacctgaagtcaggagtttgagaccagcctggccaacattgtgaaaccccatctccactaaaaatacaaaaattagccaggcgtggtggtgtgcacccatagtcccagctacttgggaggctgaggtaggagaatggcttgaactcaggaggtgaagtttgcagtgagccaagatcacgccattgcattccagcctgggtgagagagcgagactgtctcaaaaaccaaaacaaaacaaaatcaggtgttttattccactccccccatcagtgttttcttatttctaatacttctagaaacctcctttaagttttcctattttagacagacaccacacaggtgctcttttttgggaggagggggatgagagtcttactctgttgcccaggctggagtgcaatggtgcaatcatagctcactgtagcctctgactcctgtgctcaacccatcctcccaccatggcctcccaagtagctgagactacaggcacacaccacgctgcccagctaattttttaattttttagtagagtcaggtgtcactgtgttgcccaggctggtcttgaacctctggcctcaagcaaaactcccaccttggcctcccaaattgctcggattacaggagtgagccactgcacctggcccatagatgcattaacacctgtctatggtggtggagagaaggctcactgcctctcccaggccactgggaaatgaccttgtgtattctgcaaatacacaagaggatctgaagctattcttgagggagactttcaacagcaaaactcagagcacaaaatggaaaataatcataaaaaaattaaataataatactatcaaatcataacgtgaataatgctgttattagagttgaagagaagcccttagaaatgggacaaacattgtaattctcttagagaactgtaacttaaacagaaatacacttaatagaagaggaaagaaaatggttcatgtgacacaaaggtcccatgtgttgacttctttggtaagatcaaataagtatttaagcctagcaatagggtcagtccagttagtatttctcctcacaaatggtgaatatcaactccaggatggctggagttttctcatggtttggttccacgccatctgcatgtctttacaagtgataaaaaccagaattttccagctgctactagtcacagggggtccccaatatgggttgtttaattatgatgacgggtcctgtcaattgcatccagtaaaattggtcacatagagaactcatctaaaactgaggttttgttgtggttttgaaaggtccattggaatccagatttgcaaagcatgtcaagttatggcaaaacatatgccacccatctcaaaatctttccttattattgcataactttgaaagccactgttgcgtttgttgcgatgaggttagagttttgttgacatgatgatattactctcttcctctgggtgagacacatctggattctcacttggagcagggctctgtacatccttctgggatttggttgagtaggtaatatacatgcttctcattaggaaaattccagcaattactgcaaaatagctcccataaactaaaaactgaatgctgactggcaagttgagccctctctgatctactacaatcacagtcatgatggtctgaatcaccaaggcaataaaggtgttgattccaaataccaaggcatagcgttccacattcagattaactgcaatctgaaatactgctatggttataagaagcatatagctggacttgaatatcaaatagccagcatagcacgcccagatattggctgtgtaatgcatgagaaataaagaaccggcattgacaactgagaagaccaccagagccagctctcccagaaggtcccagttgactttcacataacccactgcaaaggcagccacagcccctccaaaggttgcaatagcttctacggccccattatagatggaagaatcttgggatggcgccttgtaatcccacaggatttgaacatagttcaaaacctggttaaaacctgctgtggcgaaagcccaccatagagaccagtagaaaagacgttttgaggagtagcactccttcaaatcttggaaccactgcacaaaaacgtccacagtcacattgcttggtttcaggctgttcagctggcccttattcagcttccctgaagtgctgagtatttctgatgtgggtttctgctcttcacagcctggtgcttcaccttcgtgagtttcctctaatactggattcacgcttgatgacttctttatttctctgctgggttttgcatgaaaaaacatgcttttcttgggcattggtaggaaaagtgagaaaaggaaagccacggagacagaggccaaggatatgacgttgaggtaaaagtacgacatgttcgccagggataccaagagttgagccagcaccgaccctgctgtgtaggcggccagcgtgacgctcctgcagtagccgctcactctctggtagtgctcggggctgaccacgctgtatatgtaggcgtagtaggccacctcggcggcggtgaccatcccatagaagaactctacaacctgcatggtcttcactccttggccaaacaacagcagcagccaggtaatgatgaaactgataccttgcaagatgatgactggcttgtagcggacataatcggtgaggacaaacacaggcagcagcagcaccaggtaggagtatgtccaaacggggaagatctcatttgttatcttgacacctggatcactgaggttgctggagaaagcaggaggccacagagcaaagaccacacaactgagctgctccttggagggaaggtctgttaactggtccacagtggctcgagaagcagaacccagtggattcattgagttgcttctgaccctgcatctgtcctttgttgtcttaattgtggcatgcttcaacctctgcactggtcaggtttttatctggtccagataaatatgggataaggaatggttctgagggtctcatcatggagaaaaaaccaaataagcagaggatcacagtggggtaaatccaggaactgcttagtgaagttctgtaacaatccatggctgtgaaagccagatgtttacctttccccttcattttctgtgtgttccaaatcacaagatagtccttttaaaagttactcctgtagcagtcatcttcacccattattataagctctatcactttttaaaaaggtacaagaacactgtgtaaacggtagattaaaaattttaaaaggctgggtgtagtggctcatgcttgtaatcccagcgctttgggaggctgaggcaggtggatcacctgaggtcaggagttcaagactagcctggccaacagagtgaaaccccatctctactaataacgcaaaaattagtcggttgcggtggtgggtgcctgtaatcccagctacttgggtggctgaggcaggagaatcacttgaacccgggagatggaggttgcagtgagtggagatcatgccactgcaccccaacctgggcaacagagaacgactgtgttaataacaacaa

SEQ ID NO: 14542 - RNA, 593 nt, Homo sapiens
  source 1..593: mol_type = other RNA
gctgggattacaggcatgagccaccgtgccaggcctgcttcatataacttctcattcagaattttattcaaaaatcaatttatccctgtggctacatgtataatttcagtcactccactccaacactgtcaccttctgtagcatatcttttctgaataaaatttatgcagtctgctccatgaggacacaatttttttctgttttgttcatcctgtatagtctcatcaacgggaatagtgtatggtcttctgaaatgctgaaagggtagttacacttcagaggctctctagattgttgatacaatcttgcttatttataacaagtccaaatagaatcctctctgcacatttccccacaactgaatgacttttacaatatattattttccatgttgggtcatctgtgtgtctatattgctgtcaatcattccattctctacatccatgtgtacacattttttagtccctacttaggagtgagaatatgtgatatttgactttctttgcttggcttgtttcatttaagatatgacctccagttccatccacctcttaatcttgtgcctaaaactctttccaggggtttagaatcct

SEQ ID NO: 14543 - RNA, 1053 nt, Homo sapiens
  source 1..1053: mol_type = other RNA
gctgggattacaggcatgagccaccgtgccaggctccattctcctctttggattgtcagttgaaatactacctcttcagagggaacttttccagctacccttgcaaagttgagtccccaagttcatttctgacatggcatcccatttatcctcctcaaggcatttactgcaatatggaattattttccttattgtctactgttaaaattttctgtctataatgtaatttattacatgaaaatgtatgcttatcaaagcagatattttgtatagatcactgctaaatcctcagcacctggcaccatgctggcactcagtagctgctcaatatatactttttaaataaatgaatgattgctatgaccatggcaaacatctgaatctggatacaacaacaaaaaataacaacaaaatctgtgctggcatgaaattggtgcttggtgaatgctggggaaaaatcccctgccattggaagccacttggcagtgtttatggatggagctgtgtcttccttcacctgggaactggcatttctgaaggtgtgattgtactcatccttaacatacgcttggggggaatgatctaggcatagggtttttcttaagctaagaaatgagtctatttcacaaaagaactaaaaacagaactctgattcatgaatttgccaatggcttgtccttctcaggggaacctccctgggcacagtgaaacccttcttggggcacgacctcatgcttgatgtgaaggtcatcacagaacatcagctctgcctgaagggtggccggcagcccagtcaggcttaacccgaggggtactcaaacggaggttcttgacaccttatcagggtgtgtacgcttctgcagaacgaaggttccttcccatgctttgccaggattggttttgaagaattactgacctagttgacagtctcgtgaataaaaatggcaatgatgaaaacaaacccttcagaaaggagagttctctttagatatgttcagggggatccttccatggctggaggtcaccttgactgggggcttggcttctccaaac

SEQ ID NO: 14544 - RNA, 3055 nt, Homo sapiens
  source 1..3055: mol_type = other RNA
gctgggattacaggcatgagccaccgtgcccagcaattttttgctactttttgtttgtttttgttttgtttctgagacagagtcttgctctgttgcccaggctggagtgcaatgatgcgatcttggctcactgcaacctccgcttcccgggttcaagcgattctcctgcctcagcctcctgagtagctgggattacaggcaagtgccaccacaccaggctaatttttctatttttagtagagacggggtttcaccatgttgatgaggctggtctcaagctcctgacctcatgatctgcctgcctcggcctcccaaagtgctgggattacaggtgtgagtcaccatgctcggccttttgctactgttaatctgccttatattggtttaatgtgtaagccagccaaagaacttagaagcatagcaggaggggccgggcgcagcggctcatgcctataatcctagcattttgggaggccaaggcgggcagatcacgaggtcaggagttagtagaccagcctgattaacatggtaaaaccccgtctctattaaaaatacaaaaattagcaaagcatggtggcacatgcctgtaattccagctacttaagaggctgaggcaggagaatcgcttgaacctgtgaggcggaggttgcagtgtactgagatggcgccactgcactccagcctgggcgacagagcaataatccgtctccaaaaaaaacgggtagcgggaagccatttttcactcccttcgagtttctggtgcccaacgtggggcatctttcactttttactctaggactgcttcagcagcaggctcctgacatgcctgaccaaacactggccacagataagatttcctaccacattagccccccagatctctgcctgtagagtccagcggaagcaagataggtaagggtctctttgtctttttcccttttctaagtttggattagcaggagaaaatgtgtgcgaactagttcttgtataataactctggtttttttgtttggttatttttttttttggtggtgaggggaggtattattgttttctgattcctcccctcccagagatggtcattattttcccatgtctgtgtcttttgtgttgtgtcatacagaagagaatcatagggcaagaacacaggcctcaaagactggtgagttcacagttctctgcaaaccaatgtctgttcagactaattttgctgtgggtccccaagacaaaaaccagatgaggtgctccttgggtcttgttttatgtcctcagagcttggcttttccatcagtgagaacactctggcctctgccagctgagggtgcaagtgtcagcctgtgtcagccagccagtcaaataggctggaagcccacgatgcagtgacaagcggcattctctttgtccactcgtgccagctctcaggagagtttggtcccaataactgtcccagtccgtagggctttgttgtctcaaccttcaattggacaatgctaggaaagtccaatcccagtagtgcttgcccggtgtcacagattagcgggtcagtgagtgtcatgagacaccatttacacaaacactatccttaatgcctgtggcaacaaaggtctttgctttctttttttcttttttgagacggagtctcgccctgtcgcccaggctggagtgcagtggcttaatctcgcctcactgcaacctccgcctcctgggttcaaatgattctcctgcctcagcctcccaagtagctgggattacaggtgcctgctaccacgcccagctaatttttgtatttttagtagagacagggttttaccatgttggccaggctggtcttgaactcctcacctcgtgatccgcctgcctcagcctcccaaagtgctgggatgacaggcgtgagccaccgtgcccggcctaaacagctgtcttattggtactcttggtgctggtgacctggctgtcctgggcctcgggcacaagggcagctgcgcccagtctcttgatgatgctgactttagacaaggactccggcttcctctcaagcccagaccgtgaggaaagcgccaggcgccgcagtgtcggggcagcagccgttgtcgctgagcttgtggccttggctttgacagtcagtgctggctggggactggccttggctgggccccgtcctagcttcttcaggaccccggcatactgcaagacagagctgctgctgtcattgtcgctgtcccaagccagatcctcgtccgtttctggggtggcccccaggcggctgaagactcctgtgggtttactccctgtcgtggtgtctgccttggtctcggcgccgaggcggtcaaacacagacgtcctatggagaccttttgcagcctgctgctgctccaggatcttgcgggtgcggggtgtggtgcctttgggcatgttgatgacgtacttcccctccatctcagcagtgacccggcgccgcttggcaggaacagccaggctctcctcctcccggcgggccagggctgcagtggccttggcactctttgctgccatcttgttggacacagtgaccgagatcttggaggtgctggtgtccgggcgcctggggggtgtgctgggtggagagtcatggttcaggctgttggtgatcattcgggaggcagcactggtgccacggcgaatttcgcctgcaagggggctagggctgcagggtactgactcagtggcagctttgcacatgtcctgacggtgcaccactttggcatgcttgagaatggcgatgatgtcacccaccacggtcacgcccagctcattcattatctccttattgagatccagcagcatgctcttctgaatcctattatccacaaacatcacggcataattgacggcaggtcctggaggaatgccggcttccttaaagaactggatccactcggaagtggccatagtcacggagaccatcgtctccctggccctgacactgctccctggagccgccggaagctgaactgactcgtccgcggccgctctaccccaacaggccgccaccagcgagagtgcggccataaccatc

SEQ ID NO: 14545 - RNA, 890 nt, Homo sapiens
  source 1..890: mol_type = other RNA
gctgggattacaggcatgagccaccgtgcccagccaaaccattcttaacaagaaacaacactaaatcttcctttttcttcttgtctcacaggctgttctcaaggaaaaaagaaaaaagaaatttaaggaaaaaaataatgccaaaaggaaaatctacagattcaaaaacctttgggtttctaagttctttttaaagaactgctaggaaattttcttctataaattctggaaaagaaaaacaaaatgctgatgattaccttataatgaattcttctaatgaatttaaaatcttaaagatgaattcaagaaaaacaaaataatttcattattcccttgtatctaacaaaaacctaataatttaacaaagaacacttagtgtattacagactgagtatatcccttatccaaaatgcctgggaccagaagtattttggaatttttggacttccaaatatttgcaatattactagttgagtatctctaattcaaaaatctgaagtgctccaatgaacatttcctttcagtgtcgtgtcagggctcaaagttttgaattttggagcatttcagatttcagattttcagattagggatactcaacccatacatggattattaaacttacacagcagggtcttgataagttcacatccaaaaccaatgtttacaaaaatctgcaggttaggaaatcaacattttcttccttatttaggaagtatctgtcatgatgtctttgaataattttcaatgagtttatttcagtgtgatgatcaatgagatggcaaggaactcatgtcctttttactgatttcctcatttttataaaatgagcgttttcattcttaaatggccttcaatgtcccattctaagtaatactttaatacatcaaatt

SEQ ID NO: 14546 - RNA, 5695 nt, Homo sapiens
  source 1..5695: mol_type = other RNA
gctgggattacaggcatgagccaccgtgcccagccaactgtggttgtttttaaaggacaaagttggtctctttcagaggcacatgctgggaatgggctggggtggcagtgggtgggggggtgcagacaaaattaaatggtggtaatcactgaagcttgctgatgggtacatcaattagttaactattctactttttgaataagtttccaaattttcacaataaaaaggaaaaaaagaaaactcaagttttctttcggttaaatacccacatcaatgttctcatgaaatagtgcacagagtcagtgactttaaggccccttatgagggggacattagcatcctcatgttgaagattgaaaggaaatacctccaagtattatttcttggtagtggaacaacagtgattgaaaattttcttccttcaacttttctgtatgccaaactttctttactgaggatatagtataattacggaagaagagccaacaaactttcaaatacattggaaaagtatatagaaaataattacccctataaggtctaaaggtgttattaaggaatatgtggctaaagaggctattacttgaatcttgttaatgaatagaaataaccgtccattttgttacacagtaatataacccctaactggtaagtaaaaagcacaaactaggccgggcgcagtggctcacgcgtgtaatcccagcactttgggaggccaaggcgggcggatcacctgaggttgagagttcgagaccagcctgaccaacatggagaaacccgtctctactaaaaatacaaaaatttagctgggtgtgctggtgggcgcctgtaatcccagctactcgggagactcaggctggagaatcgcttgaacctgggaggcggaggttgcagtgagccaagattatgccattattgcattccagcctgcgtgagaagagcgagactccatctcaaaaagaaacaaataacaacaacaaaataaaaaccaaaaaaaagtacaaactaattgggtaacaaatgctcgcatgggtgactgctcttttaaaggtagctcatatacacatacacaaagatttaaatggtactaaacagaaaaccaaaaaaggtttgggagattatggatgatttgaaaatattaatgtcaatttcttttaaacataaatttaagaacaataaaagctattttaaaggatcttatgcagacgcatttacaatttaaaatcattagcctcccaactcgcatattttactggtagtcagtaaatctcacctcttacacttaagatatcagctgcttcatgaacagccagacacatgaatacattcatgcctactgcattgataggattcttatacttttcaaataaacaagtggcatttcttaaaatattaattctattgaagagtctagtgaaaacactgtaacccacccaggtaaagatttgcaagggatatttcactgaaacacagccttgaggccgggcgtggtggctcacacctgtaatcccagcactttgggaggccgaggcggcggatcacctgaggtcgggagtttgagaccagtctgaccaacatagagaaacccagtctctactaaaaatacaaaattagccgggtgtggtggcacatgcttgtaatcccagctacttgggaggctgaggcaggagaattgcttgaacctgggaggtggaggttgcagtgagctgagattgcgccattgcactccagcctgggcaacaagagtgaaactctgtctcaaaaaagaaaagaaaaaaaaaacagccttgcttttgatttcccaagatttgcagctgaaaaacgttgccccactggcatacggaacctccgttttggttggattcacacagtcaccataagcgcacgatagcagcagaacaaacaggaacctacctagaaattgggacccgagttttgcgccttaattctccgagactgtccccttgtgcataaacaggaacatctggaagacgtcacctctaaggtccccttccccacttctaacattctgacttcaagcctttaaacttgacactagaatgaagaacaaataaaagttttctccaaaagctgctgttccctttttggatcatttcacaagccttaacctgcaacagctgagaacgaagactgaatcttatctaagagcaaacttgctgcaaagggatccacacaaatgttttgtggcttaaaacagataatctttttaaagatttggcctttgagatacttaatatctcttttgttaaatgagaatagtcttttagtaagttcctttcttgaccagattcctaggaaagtcattctaaaccaactgcttccgagctggtttctataaactaaatcttgcagttgtttattaaggaacaggctattgtattagcttgctaggactgccttaccaggtttggtggctaaaacaacagacatttatttcctcacagttctggagcttggaaggcaaaaatcaaggagtcagcagggtttgtttttttttttttttctcacaacttctctcttggcttgtaagatggctgttttctctctggcttctcatggtcgtctcactgtgtctcctattctttttgagacggagtcttgctctgtcgcccaggctggagtacgatggcgcaatcttgcctcactgccacctctgcctcctgggttcaagcgattctcctgcctcagcctccggagtaactgagattacaggcacccgctaccatgcccggctaatttttgtatttttaggagagagacgacgtttcaccatgttggccaggctggtctcgaactcctgaccttaggtgatctgcacgcctcggcctcccaaagtgctgggattacaggcataagccactgtgcccagctaatctattattttaagaacaccagtcatatagaattagggccaacctagcagcctcattttaatttaactatctctctaaagaccctatctccaattacagtcacattctgaagtactgagattagggcttcaatgtataaattttgggggacattattcaacctataactagcatagttttttttcacatacttttactttgatatatttaggtttaagtattgagaatttaaaaaccaaaagacctctatcatgtgcgtgtagaaacatatcatgtaaaaagaatctgttgtctatctaggcattatatttgttgcatcttaggatttactgaaaaacttttggagaactttgcccctagggcagcagcttctggcagaaaaaggccaaacccaggattctagggcagttaaatttagaaacaaaagccaagattcattctatcactcaataatcattttcttcaatggctgacacaccaaaagaagggtcaaatttatttatttttaaattcattttaatttctgtatctctacatagatatatctagagggtctcactctgttgcccaggctggaatgcagtggtgtgattatagctcactgaagccttgaattcctgggctcaagtgatactccatttcagtctcctgagtagccaggactacaggcatgtgccaccatgccaaaaaaatcttctgtagagatgggggcggggggggggggtctcactatgttgcccaggcttgtcttgaatacctaacctctagcaatcctcaggccctggcctcccaaagttttgggattataggcattagccattgtgccaggcaagttatttccccaaaaaacactttcttaagggatggtcccagtccgccagcatccgagtcacctggggtatctgtcatggaagcaggtctctgcatcatactgcagattcagtgaattcagctctgggtctggggaactgcacttcagcaagcgtcccacccacctgcccgctggagcctgtgggtctctttcctgagaactgtgtgcagccatctatgtacccactcatcacccatgaaaaagatcacgcttgtctgaacagcaaaactgagtatgtttactttacacaaagtacaatccagtatatgcagaaaggtactcagcatcacactcgtgatcaatatcctcttatttccatttggtatgtcactgaaaacctggcacaccacttagctaaaaatcacataaaagaacccctagagaaatcaaactgatgttttttttcccccaaacaatagatttcctcttcattagtcaaatctgatagtgatattcattaataaggaaaactaaagttttcaagcatcaactctgaatggcagagaccctaatctgactgttattagccaccaagaactcagaagagcaaagaactcaagaagaggcaagcaagagcactatggaaattatattcttttctgtgaaattcagtcccacagctatttgagcaagggcccaagacgatggagaggcggcaaagctgctgggagggcctgttcgcaggcaggaatgcactggctgtgcctcgccccgccatgtccttccacaggtgggctcttcactggcttcacttcagcttgatcctctggtctccccacagcttcctgggagactttgggttgtaatctttacagttccaagaatcaattttggttgaacgcaagggtaacatccccatccaaaacagaaatgttctcatggtatgaaggccattctgtagagtgcacgtatatatgtttatatttatataggctcctatgcgagacagtttccttcctcttagcaagagaatactgcatccagcaacactgctttggctagctcttttttctgtatggcctcatgtgtgtggcaattgaagcagctatttctcccttcctcttgttctggccaaaataatctagaaactcaccatctggtccaatcaagtacattattattgtgtgatccactatgtagtcttcatcttcgtccttggggccagggctgtaatacactctgtatgctctggccacttgatcgacctcttctctcgtgccagtcaagccaaccagtttgggagaaaattctttcacataatttgcgatggcttcttttgtgtccctctctgggtcaatgctgatgaaaagtggagttagatctggcagagttgtaatgctatctatttcatccacgacttgaatcatcttttctagttcttctggacagacatcagggcaatgagtgaagccaaaataaatcaataaccactgacccaagtagtccttgtcagttttacgctccccagtatgagttgtgagggaaaacggtcccccaagtaaaggcttgccgatgtgtcgctgccgttccttctctaacttctctgccttttctttcttgacgtgcttcattccagccagtaaagctcctccaatagcaaatgtgattgctaaagacttccaggaaacaggcccgggcttcgaggggcgcgtggagtctccggggcccttctgcgaccacgggggtggcggcctcgcagtgctgaggggccgggttcccaggcaatagccagggcgccccgaggcacgccacgcctccgcttgccgcgcgcagaactgcctcagcaagactctcgcagtcccctcggctgggccccaaaactcgagtccgcgaggcaagaagcgccaaagttggccacccagaggccgcataactcgtccgggtactaggaccagcatcgccatgagcctcggagaccgggtctcctttg

SEQ ID NO: 14547 - RNA, 5402 nt, Homo sapiens
  source 1..5402: mol_type = other RNA
gctgggattacaggcatgagccaccgtgcccagccaagggaatattgtgtaatttaactgtactggtgattatgcaagtattttgttagagctcatagggttgcaacactttaaattggtgcattttactgtatataaattatggcaaaagaagttgatttaataacaaggaaagctgtttctctctaagatctcttctagctcctggaaaccttgacaaatatgcagaattaccttctcctcattatgaaaattcttcgctttttcacactgccttaaattctcccaataaaatgaaattcatctatgctaactcatcttcttttagagcaggggtctttaaccttttgtgtgggcctgttgccagcctgggaaacctatggactcctccaaatagcacatttcaaagaaggaggtaaaatagataagatttctaaggaagccagtaatattaaaatatagttaccaaaatatttttaaatacttgcatttgcaatatagtaatatatgtactttgttagcacattaaatgacaagatctagtggcagcctaaacattaccatcattccaaaatatgagctgaaacaatatttcaaatgcctgcaacaattgtaaagtgatatcaagatgcatgtgctttctgttggtgacaaagtcacaagccacctgacatccctataatctattcctcacttgcaattgaaagtaatacttatttatttatttatttatttatttattgagacagagttttgttcttgttgccaaggctggagcaatggcgtgatcttggctcactgcaacctctgcctcctgggttcaagcgattctcctacctcagccccccaggtaactgggattacagacacccaccaccacactcggttaattttgtatttttagtagagacagggtttctccatgttggtcaggctggtctcaaactcctgacctcaggtcatctacctgcctaggcctcccaaagcactgggattacaggcatgagccaccgcgcctggccaatactaaattttaattagaagttagtgagaatgaagacctaattttccatccgacttcatagattgaattctgtctatggaacccagtttgagaacccctagtttaacaagtgatttacacctagtgtgaaatttttaatcagatttatttcagttaactctgagactaccccctcacacacaggaaggtgaaaagaaggcttggagcaccagctagggaggacagggaggacaggaaggcctctgagggtgggcagagctggagaatggacgcaaaatcaagatgggaaggagccgcctcaagatttcatgggtgtggtggtgggggacctggtttagcttctctcctgttctagacagctctacagagacagagctcaagggagcgttttctacaggttccccgtccggaatgcccagctcctatgggccctaactgaggcactagaggaaggatggacgagcagagccaggagtgggcacgcctttgtgcccagccttctaggtctcctgggttgggcaggacacagagcaaaaccccttccccaactcacacagctccagtcagctgctggctgttggcagggcaaggcccaccccccagagcccaccccccacaagctgtcctctgagacctcactgccacaagggtgaactcccacccagggttctgggctttgcttcagggtgctttgctctctgcccagaaaaacatcccccagaaaaggaaagacaaaggggtggttacctgctgacctccccacaggtttaccctgaaccgaggcccagagaggggaagggacctggccgaggtctccaggaggtcggggatgtgctggtgccctgccagccctgggcttctgccctctcctcccctcagaccagctcccaggggaatgtgaagaaaggagggccacaggcaccagtgaggccaccctggggacaaacaggtggttagaggcagctcagacctcagacattatccagggcacttttataaacaggaaaaatgtggccgggcaaagagtagaggctcctgctaacaccaccagctggtaggtggtgaaaccgcacattagcccttggatacgtgattccccagcctgaccatgtattagaatcacctggattgctcactcaaaacatgtctgctggcatcaggcctgacgctacagaatcagcagctctgtagaggggcctagcatctgcaccatcaatgagcagcccagatagctccagtgtgcagccaggtttggggcccatggcactgagccattcccaagtatagcctaggaagagatcctgagctgtgggcagagggagggaagagctcggggagagcatctggttcaagacacttgattcacttctttttgttggttacatctaaaactaaggatgggtggctggggcgggagccagaatttagtcttagctgagctgggggccaagtggagtgtgccctgaggcttgggacaggagcatgtgggtgggacttcccatccctgacccccacccttatcctgcccttcagtggctatgagagatggcaaccaggtcacagggctggactttgtcgtctcaagccccaaggagtaaagctgggcagggctttggcctggatcaatggccttaggactcagcccacacgtaagtggggtgagtgcagcgcaggacagcgtctgtgttctccagaatctgtcttcactctgactcaatcaccaggggattctgcaccccggtcttagtagaaatgcacctctgagtttcagtttagctccctgcccatcacgtcaccacagtggtccatggaatctgatgcgtcccgcagctcagcccttccaccttgcccagtgtgccctcctcaccgacagctcccgctcccagccccctgcctctccacttctagggctgcaatctgcttctgtctcctccttggatcacacacttggacccagctccctgttttgctctgggctctgctttctcttgtggagttggtgtcaccaaggtctcaggtgagaaactccttcctgccgtgtgactgtctgcggagaagtggggcaccctgtgggggatgggataaaaggggtgtccatgcactccaagctgtggccccttgggttatagatcagtttttatccaaagacccttgtgatgagtccaggcttgagtttagtccctattccaagacatgagtttgcatttcttctttcattggaagatgacatttcaaaaactttccttggctttcaaaaagcttagcattagatgatagaaatcagctcatgggccccttgcttttaggtgatgtttattctgtttcatccttgaatatcaatttgtcgtgcatccaaactcgctatgtcaaaccttttgaatgaatgcagggtatacgtcttaaattaactccataaaacttgagtagctagcatagaaatttaaggagtatgtgagcaggacgttatttcccccagttcacctggccttcttgcactcagtgctttcagcagctgtagggcgttttgtgtgaagttattgacatgaagggatgggagtgaaatcagttatcagataacaaacaagtgctctcatgtctgatgggtagaagagggggcagtcacttcctcaacacgtgagatgacactgactttgcagtgagctctccccaggaaagaggaggagccctgggcaggcgggatggggaaggaccctgcgggaaccatggaggaagtttggagctccctgctggagcatgcagcctgcagggctgcagacagaaaacctcgttccgccctggtttggaggtttgctggctgtgtgaaccttgacaatgtacctctcctctctgaatgtcagttttctcaactgtataaaggaaacagtaatagctactttggttgtttgtgagggtcaaacgcaacacacatacagaagccctataaaatgcaaatacttttatcctcagttctgtgcagaggccactgggtttacttatgtattgattctctctgtcctctctcccacccctatcctcctccccacatgccctcaccttcttggttttgccctcccagaagtaggggagtacagttattcggttagagcagttacactcttgggggtttgcttcagccaagaagacagtgagccgtggggatcgtaattaatggaggcagactgattagaaatgagccactggatcggggtgtttgctgattcatcttggaaacactaggtcctgagtcccaatcggcttctaccacattggtcattgttctacttctgcactgttctgtgcagaagcacctgtgtttactcataaacttacatattgattctgtctcttctcctacccccatcctcctcctcatatcctaagtgctcagcatggtgctaggtacacagcaggcactaaataaatgtttctttaattaaattcccattgatagctacactgtgtgaatggtactttcatgatagatttttctgtcaccccttgagtttctgcagacattaggattcacagagaatgctgtgttccaagtcaaaatattcattatgacacatgctgtttgcaatttccacaatccaagtcattacccataatgtgcttggggaggaaaacaaacctctcttggaaatgctgccgtgtaggggttggggtcagagctctgcctccaaactccgtgacctttcctggagcacttctctgttgaccgtgaccaggaggcattccaggcttgggagcaccagccagaggacccccagccagatgagatccagtcacacatctcaggcaaggtcagacagcccagggaccccaggaatgcagcccaccagatgtgtgctaaggacagcatgcttatttggaacgctgggtaacctgtcatgcattgcagaaacatggagatccccctgtttgacattttctcctgttaatcccattttttaaaaatagctgtgcggtgtagaagtttcctcctggtctcattaggtgtctccttataattgcaggttttaaagcaagctcaaggcagagcctttcagagaaattaaacttcaggtgttgtctaggaccaggggcagccaattatcccattacagaaaccatgtacttggaatactgattgtgcttcagaataatccaattccattcactgtgggctgggggatgcgcctggcaatagaatttcaatagcgaagagtctcagtttatcctcatgaagctttcagtcttcttcctggggttagttcccttcttcttgaaatatattcactagaagttcctcagtggggatattttggtggtaacagggtcaggactagagtgaggcacagttccatatggctggggaggcctcacaatcatggtggaa

SEQ ID NO: 14548 - RNA, 1012 nt, Homo sapiens
  source 1..1012: mol_type = other RNA
gctgggattacaggcatgagccaccgtgcccagccagagagacaagagtggttacttctaaaatgacaagatgatgtaaccctggctcagggagtagatcaagttctaaatctcaggaataaaaaactgatactcattatccaattcatatagtcttgtattatatacatattaacagtctatgcaatgaaaaataaagaaatttcataaaactatttcaaaactcagaacataaaaatgtaaagaaacaaaacatttaatgtacaatctactccatttggcaatgtgtactgagagataaaaaacctatctacaaacagaatataacaaaaggaaaatgtgacttaagaagtgatctcaggtccatagctcttcggttcttccaaatttgtagatcagagtgctaaaaaatataagtgcattttgaaaaaacacagctagtcccggataaacatcagtattttgggtaacatatgcaccaaaaagaatccacatggaagcaataagtgacccaaacatcaacatgaaaccaatgaaaagccaaactcgagcacctgttcttcctaaacagccgctttcatagctatcacctctcacctgagcattggatacagcatttatcatgaagaaagccaatgtggaaaatacaccacatgtgtgaaaggcatggttcaactgttctggcttaggatacaccacagctgcatcaatcattatccaccagcctgtaaaaaacaatatacctgcgacaacagatgccacagcatttcttctctcactccagtcaatacattcacattctggccaacgaaaattatctaggaagcctgccatttttacttcttaagcataaatttttcattaaatgctgtatcccagcttcctcaaacgcccacgccgacttcaggcgcgcgcgcaggaaggagactgctgcgccacaaccctgccggcgtcccgcggctccacctcagccccgggagcccggagctgggagcagacgcgaggatagagc

SEQ ID NO: 14549 - RNA, 1042 nt, Homo sapiens
  source 1..1042: mol_type = other RNA
gctgggattacaggcatgagccaccgtgcccagccagagagacaagagtggttacttctaaaatgacaagatgatgtaaccctggctcagggagtagatcaagttctaaatctcaggaataaaaaactgatactcattatccaattcatatagtcttgtattatatacatattaacagtctatgcaatgaaaaataaagaaatttcataaaactatttcaaaactcagaacataaaaatgtaaagaaacaaaacatttaatgtacaatctactccatttggcaatgtgtactgagagataaaaaacctatctacaaacagaatataacaaaaggaaaatgtgacttaagaagtgatctcaggtccatagctcttcggttcttccaaatttgtagatcagagtgctaaaaaatataagtgcattttgaaaaaacacagctagtcccggataaacatcagtattttgggtaacatatgcaccaaaaagaatccacatggaagcaataagtgacccaaacatcaacatgaaaccaatgaaaagccaaactcgagcacctgttcttcctaaacagccgctttcatagctatcacctctcacctgagcattggatacagcatttatcatgaagaaagccaatgtggaaaatacaccacatgtgtgaaaggcatggttcaactgttctggcttaggatacaccacagctgcatcaatcattatccaccagcctgtaaaaaacaatatacctgcgacaacagatgccacagcatttcttctctcactccagtcaatacattcacattctggccaacgaaaattatctaggaagcctgccatttttacttcttaagcataaatttttcattaaatgctgtatcccagcttcctcaaacgcccacgccgacttcaggcgcgcgcgcaggaaggagactgctgcgccacaaccctgccggcgtcccgcggctccacctcagccccgggagcccggagctgggagcagacgcgaggatagagcgccggtgaggcggggcgaggcgccgtgtgc

SEQ ID NO: 14550 - RNA, 2179 nt, Homo sapiens
  source 1..2179: mol_type = other RNA
gctgggattacaggcatgagccaccgtgcccagccagccatgttcttaataaatagtctgatagatgccaaacatcttaatataaaaagagaatacgttgggaaagcataaaaatctacatttaatgcaataaaaatagatcatatttcaccaagaagcaaacagtttaaagtgacagaatatctcctctcatttacatgggtcttatatgtttttttttcccaaaatattttcatctaaaacaaccctgcctacatacaattgattaaaaagctgatgaaaagactacccaagatcacagagctagttagggatggggccaaaagaagcagctaagtcttctgaggtttaatttgttgacattttcataactccatgatttagtaaattattaagaataagtcttctatttttaagaaaaacaacttcataaatatacacaaatacatgtgtaattagcatgtagttggtgcacagacaagctacagaacttgaaaaaggcacatgcccagaatttggaaataaagttaaaaataatcaaattctgtataacaagatgcaaaaatataaacattaattagattagattagctaaaagaaaagttagaagtgtgttgttgtttagactagtgcctctctaaataggaagcctgatatttaaaatataactaatcaaaataaaccaaattatcaaaaaatgttttgctagtcatcatacatgcagatattctgatactgaacaaggagttttaggttgataacccattttcaatgtttatgtagaactgtttaagtgagctgagactgcgccattgcactccagcctgggcaacagtgcgagactctgtctcgaaaaaaaaaaaaaagagagagagggagagagagatatacctgattgtttttgtggcttgtgtttttttgttgttgttcattggaatggagctgggatgcttttctaggctttactgtttcagagaaacatcctataaatctattcaatcttcaatcccctttacctcgttctaaactctgaaagcaatctttcaattactagtttggctccccatgccctttaattcccaaacgggctatcttgggtatctgacatgaatattccaggttatgacaagaaatacttatacaaaaaacctgaagacctataatgcaaactaataaactaaaattatccagtttattaaatttatttaaatacaaatcatcttaagctgcaatttactgcttgttttatatcacttactaaactgaaaattctataaatgtaatatgtatatacagcaagctattgcaagcactcgacatacgtttttgaataaatgaacgaagtgaatgaatgagcgaatttagaagatcaagttcttgagacagcaataatattgactcagaaaacccagttatttcatcagtgataaacctctgcaatgataataatgctgatgcttacttgatgtgttccctcatagtttacaagtacttccacatatcaatgcatgagatccttgtaagcaatcctcatttccaccaactgccttggttaaaatcactgcagaagacacaggcggaggcatgcaacctactgtctgcaaaccttttaaaagccattcgttgatgggtgtgattgataaaagctgaagaaaaagccatattgttgctgggaagaatgcaagagtaaagatctgaataaaaagatgcagttttagatgcaccaaagcactggtcagctcctctgttttcaatgatagtccactgttaaagaatattgttgcaacagcaatgtaggatacagttatttctggcttcagtggtcccccattcacccctatggacggctccagtttagctccagcgatcgccagcactattccgaccatgaaccagtctttcctcattctctccagcagcctcatatttgttagggtgggtgggttttgtttatttgtttggctttttttcttttcaagctccgatcacctaatccttggagcgtctccacactttccttggtccctccagacatgcagcagagcaagtcaaattgccgattgtaaagtaaagacctgggggttgctccggcggctttgaggagggttgggagtagtagtagccagtgacaggaaagtctcactgagcgccgccatcactaccacgcgcctcagaatac

SEQ ID NO: 14551 - RNA, 4933 nt, Homo sapiens
  source 1..4933: mol_type = other RNA
gctgggattacaggcatgagccaccgtgcccagccctgctaaagcttcatctacacgtccagtattacccaactctgttactgaaacacaagctaacatcattcaacataggccacaatatcatattatttttcccaatatctttttcactgagtccacttaggtttaatcagcacttaactacccatgctaatggcgggtaagtagcagcttgcataacccaagtgatcagatactctgaaatcaatggggtgcattactttttattccctcccagcacccagcagatttgtcttcatcattaaatatggaatggagactaaaatttttgaattaaaatgatgttaacctttaaattagcatgttgattctctcttttagataaaagagaaccagagagcaagttatctttgaaacagatacttcaaaaagtagagaatagctttccctatggtagaaacctaactgtgtatttggatggaattatagcatcagatttaaaggcctgtcttttagccttagaatggtcatcctgctgatgaagacccacagatgcctgggtctgcgtttcattttcaggttacaggtggctgctttggactctggcctccctacaggcagtttctctggttgcagggtcatgggtactatagaattagtctttgttttttttttttgagatgaagtttcgctcttgttgcccaggctggagtgcaatggcacgatctcagctcaccgcaatctccacctcctgggttcaagccattctcctgtctcagcctcccaagtagctgggattacaggcgcccgccaccatgcctgggtaattttttgtatttttagtagagacagggtttcaccatgttggccaggctggtcttgaactcttgacctcaggcaatccacccacctcagcctcccaaagtgtgggattacaggcataagccaccacgcccggcctgtagaattagtcttctctgccttgaaattatttctaccaattcttggtcccttggaatcatttccctaaaactcagcatttattcaaggaccctggaacatcttatgttataataattgtaaagttaggtctaaagcattttcttccaaatctttgcttgtttttgtttaaaaaaaaaaatcacacttcgctaaacatggctgctaggaagccctgagctgaacttacagttgaccttacttttactaatggtgtgggattttcctgcatgcaatttctgccacaactttttctgtagtcttgttttataactatacctctttttatttttgtatggatttatctatccaaaatcttattgaacatatttttctgagccacaggaagtacttttgggagtgaggtggtgtgaatttatacagaacaaaagcagcacattaagaaggacacccacaggtggagcacttagtcactcccaccggccaacagcgcttgcttagggagccggatgaggaaagctcatttaaaaatatggtaacatctatgtgtgagatgctgagtgatgctctcagatgaaacccaaagatgatgacatccttgcagacacccaggtgtgtatttcttcatactctagaaaatgatcagtcaatgaaatggatattgtctcttttcttatcgcttgtaaatgtcagtttggggaacgaaaaaaatgccactttatggtgtgaagtgcctgtctacaatagtccttgcagagcggctcagtgagtccatggcattaaagatatgacagttactatgtatacagtcagtgaggaaggcagcacagcagtatctccgagaggtggggccccaccaacactcacaccacaccccctgcacgctgcatattcattggcaggtgagggtgcttttgttttgtgaacaatgtcttctggtctttagtacgcattgtggttttccttttttttttttttttttttttttttttttttttttgagactgagttttgctcttgttgctcaggctagagtgcagtggcacaatctcagcttactgcaacctccacctcccaagttcaagtgattctcctgcctcagcctcccgagcagctaggattacaggcacgtgacaccacgcccgactaatttacatatttttagtagtgatggggtttcaccatgttggccaggctggtctcgaactcctgacctcgggtgatccacccacctcggcctcccaaagtgctgggattacaggtgtaagccaccacgcccggccatgcattgtggttttcttaatgcccagctttgtatgaagtcctctaaagtcccctttgaggagtcgtcgaattacatttccattttctttcattaggaagctatgtctggcctgaaaaataaaaacaattttatggtttctcataaaggtgtaattttgcttcactcttattcacttattttcacgatggagagaatgaaattgtttccccacaggaatcatagtccattttttgcctttcatgttagtgatttttccccctcatagctccctaagaaaaactaaagcaatttgaaaagaaaaaaatgcaatcttataacaaagttggctttgtcttgataaatacaatgatggatgaccacaaccacttaagtccttttgggcaaatgaataattctctgactatatctgagaagtggaaacacatgaatttacattctggttcttcaaatatcttctccctttcccttcttacattgacctcacttgcctgaaattaatgaagcaaatccccaagggcagaggctagaaggtttgtgaggcttgaagcttatacgaggttcctctttaagaaaaacaatacaaacatatcttactttcacaattttttacaaaaacatatgaccacatgaacatactgcccaagtccctcctgggccttggcaaggcccgtgcaagagagatccctgaagcttgaactttattggcttcacggtaagtccatttctgcgggcagtgtgttgtggcaaatgtccatctacactatgcatactcgaatttgctacttgtgtatgtaaacacaggaacgtaggtaatgcctatacagagaataaataggaatatacaagtatacatataaaaacacaagattacatattgagttttcaatacacaaacacacagatacttatttttttctatttttgttgtttctaaagatcatatccaggcatgatccctcttctccagactttgaattgtctacctgcatttcagtgttcgctttaagggggaggtaatcaatttagcacattatcattcaatcagacaagctgactcaaacaccgttctctgaattggactcatgctgagcaatcctctattctagaagccaggtgtgaggggtgggaggcaggaagccagtgtgggtagggagcccattgccagtagacagagcatggcttggttctttcccaccccccaagcagttcagatactggtttggaggtctccattgaggagggtcctctgggtctccgtggtctcattcagccgggatttgtcctgcttactgtcactccgctccccatcatctgtgccgctcaccttgaccaagcagaggacattctggaagctcttcttgaagttgtcagacaagaaggcatataggatagggttggcacagctgttagcataggtgaggaccaccacaaagtcaaacatgcctttaagggctggggtggggctgatggccatggagacggaagaaacgttgaatatgtagaagggaagccagcagaagatgaagacagccaccacgatggacaccattcgggtgaccttcttctcagacttcttcctcttagaggagcccactcggattccagaggacttcaccttgatgataatgaacaggtagcaaagacagatgatggtgaggggtaccaggaaccccagaatgaaagtgtagatgatgaaccctgtgtaccaagccccagattcacctggccagttgatggtgcagctgcttctcccccactggttgctccggagcccagcatatatcatgatgggcaagatgaccagcagagagactccccacacagccatggtgatcatcttggccgtccggggtctcctccacttggccgacttgatggggtggaccacagccaggtatcggtcgatgctcatgactgtcaggcagaagatgctggtgaactgattgatgccatccacagtcatgaccacccggcaaatggccttgccaaagggccagtggaccagagccacctgcatagccaagaaaggcagacccagcatgaagagctcatctgcgatggccaggttgaggatgtaaatgttggtgatggtcttcatcttggcatagcggaggatgacataaatgacaagtgtgttgccacacaacccaatgatgcagaccacaaaatagatgaatgtgaggactgcattgcttgtcaggtcatagtacggctctgtctggtttgaggtgttggttgacaccacagagccattgaggtcaaatggaatggatagccatgtgtggcttccattgagtggctcatccgccatgtccatggctgcttttcagtcttaggctagttccagccagcccagagatcttattctcaccttaatggaccctggaggccaaggatccagtgtgacatctttgcttttccgctgcaatccgctagctccggtctccgacacccagcggctgtccccgagccagctgggcgccggggcgcgcagcagcttggctagcgcctggcgccggacgtttggggttcctggctcctcgaccctcttgtgccggctcccgctagcccctcgcacgtagagagctcccctcgcccgcagacccccggcgccaagcctcagactggggctctgggcgctggtggtcttgcgagcgcgcgcgcatgggtggctgcgccgctgggact

SEQ ID NO: 14552 - RNA, 2983 nt, Homo sapiens
  source 1..2983: mol_type = other RNA
gctgggattacaggcatgagccaccgtgcccagcccttaaatctcatttttaagaaaccctcacctattctgtagtcagctaagcttttaattacattaattttaagcacttgagaataaaatgactgcatttatcatccaagtgtcaaacaattaaaaacctaaaaatggtaactatatataagctgaggtaatatgggcttgataaagcccatgaggtaaatatgaacactaaacttggttttaattctaacagactatatctaaacctgtaagcagtatactcctaacagtaccctcataaattctgaatataattcttgtttgctgcagtcaatatttggcagtttaaattagcacagacgttgaggccttgctgagttattaggctatgtaaaagaggttaaaaatatgatcattctttattgttaattggtaatattttctcatacattaggtaaatgtcaagctttgggtctctggagtataactttttgtaacattagccattatttggtaacagaatttaaggatgatggaatgatggaaggtattacatatttctaaaacttaattaagctctaggtcagataacaatggagtaaagtgatacctgcatttttttccccagtgtaatcttaatttactattgtatttttcacttaaaattttgtagggaaaaaaagttttcaagggaacactaagattaaattgactaggttcaaatatgcttccttatgagattcaaaatttactgtgtgaaattaaagtttaagagacctaaaaaaatgtactcccaataaagaatcaatactgcttcacatgttttattttggtgtacattcttctagaaccaggttcatttttccagttttgtagaaaaatagatgttccagccaccttttacttaactgtctagtcttttaagaccaatcagtatgttccctggaaagatgaataagtctcatgactaattttttaaaaattctttaagacaaagaaataactttctttttttactcccaaagcacagtatctcaacagcagcagccaacatggggttttagcagcttaactttaccccctaaataaagctttgtataaaccagtgattttactacaaaaaacactgtccttgaaagaaaggagtggcagtcagacatcaatgcaaaacttggaatgattagataataaacatggcacttacaaaaggtagcttattagaatattccacttaagaagaggttacttttctgtccctccttgccccctcgaaaaacaaaaaaaaaagaaaaaacatttcctttaaaaattccccttaaatgtaggtttataaaatgtcagaaatgccttgtacccaaaacaagtgcttaaaaaaaaaaaaaaaaaaaacttgtgctaacaactcttacaattcagatatatatttttataacatctaagactgcaagagttcttatattcagtagctctctggtttaagacgacctccatctccttcgcttacaaaacgctttctgccccttgaaggacaaagatctctgagttgtttggaaattattccagcctgaaaacattcttctacaaaccgctccagcacagagtatgaatgtgggacatccagattaatgtccggaatttcattgtaaattctctcataacctcttttcatttggtctacagtaatggtagaagacttccaaagggactttaataaatccaaaatcatcttaaatgtactttctccagttgactctaaaaccattataatagcttcatatacaagctcatggtgaaaatgaggtacttccagttccttaaggcaatgttcagcttcagatatgtctccagagagtaaatattctttcagcagcatatcaatctctttaacaaggtgattgacagattgctgcccacctccagagccccacacactatctttacgctttccacctttagacatactcagaagcacggtagccttatccagagcagctctagcctgcacacaatctacagttcctttgtaactatcaatataggtattacataaaattccatctccaacagctctagcaataaactggcccaccaactgtggtgctctaggagtatccagtgctaattcaggtagatctttcaacaatttatcaaatgatttttccacatcagttgtgctcattactgtcccacaaaggtcagaaagaagcttagatgtcatctctctatgactagccttcccctccaatgctaaggatactgccaacactggtactccacttttcatttcaccaagatttaaatctcttaacatttccgcaacttcattagtatctccatgctcaaaatattcctgtatgattggtgttaaagtcttctcaaatgccctttcatccaaaggcaaaactacagtttcataaacacagttctcctggtcatcatcatagttaggatctttcacatccacctcctccacatcatacacctgtccaggtgtaccccagacacctttgcctcctgcaccacctttctttggtagtccccttcctttcccagatctggatcgcctatccagcaaccttccctttggactggttggcacagttaatccacttctaagggcgtcactcccactgtcgctgaccgaatcgcctctgccagagtcccgggatgagtttttccttagtcgcctttttgccttggcattaattctagcttcgttaatggaggatgctgaaatccaatttccatttatttcattctttatttcctcagtcccagcattttctgcagggtttacattcagtatctgctcattttctacatccattttcccttaatttcgcttgcactgattaaacaaattacctaatggaaatcttccttcagaatccctcgggcccccgccgctgctcgcccaggttcctggtcagccggccccgaccccgctcttctgtctctgccgccgcctcggagagtctct

SEQ ID NO: 14553 - RNA, 3109 nt, Homo sapiens
  source 1..3109: mol_type = other RNA
gctgggattacaggcatgagccaccgtgcccagcccttaaatctcatttttaagaaaccctcacctattctgtagtcagctaagcttttaattacattaattttaagcacttgagaataaaatgactgcatttatcatccaagtgtcaaacaattaaaaacctaaaaatggtaactatatataagctgaggtaatatgggcttgataaagcccatgaggtaaatatgaacactaaacttggttttaattctaacagactatatctaaacctgtaagcagtatactcctaacagtaccctcataaattctgaatataattcttgtttgctgcagtcaatatttggcagtttaaattagcacagacgttgaggccttgctgagttattaggctatgtaaaagaggttaaaaatatgatcattctttattgttaattggtaatattttctcatacattaggtaaatgtcaagctttgggtctctggagtataactttttgtaacattagccattatttggtaacagaatttaaggatgatggaatgatggaaggtattacatatttctaaaacttaattaagctctaggtcagataacaatggagtaaagtgatacctgcatttttttccccagtgtaatcttaatttactattgtatttttcacttaaaattttgtagggaaaaaaagttttcaagggaacactaagattaaattgactaggttcaaatatgcttccttatgagattcaaaatttactgtgtgaaattaaagtttaagagacctaaaaaaatgtactcccaataaagaatcaatactgcttcacatgttttattttggtgtacattcttctagaaccaggttcatttttccagttttgtagaaaaatagatgttccagccaccttttacttaactgtctagtcttttaagaccaatcagtatgttccctggaaagatgaataagtctcatgactaattttttaaaaattctttaagacaaagaaataactttctttttttactcccaaagcacagtatctcaacagcagcagccaacatggggttttagcagcttaactttaccccctaaataaagctttgtataaaccagtgattttactacaaaaaacactgtccttgaaagaaaggagtggcagtcagacatcaatgcaaaacttggaatgattagataataaacatggcacttacaaaaggtagcttattagaatattccacttaagaagaggttacttttctgtccctccttgccccctcgaaaaacaaaaaaaaaagaaaaaacatttcctttaaaaattccccttaaatgtaggtttataaaatgtcagaaatgccttgtacccaaaacaagtgcttaaaaaaaaaaaaaaaaaaaacttgtgctaacaactcttacaattcagatatatatttttataacatctaagactgcaagagttcttatattcagtagctctctggtttaagacgacctccatctccttcgcttacaaaacgctttctgccccttgaaggacaaagatctctgagttgtttggaaattattccagcctgaaaacattcttctacaaaccgctccagcacagagtatgaatgtgggacatccagattaatgtccggaatttcattgtaaattctctcataacctcttttcatttggtctacagtaatggtagaagacttccaaagggactttaataaatccaaaatcatcttaaatgtactttctccagttgactctaaaaccattataatagcttcatatacaagctcatggtgaaaatgaggtacttccagttccttaaggcaatgttcagcttcagatatgtctccagagagtaaatattctttcagcagcatatcaatctctttaacaaggtgattgacagattgctgcccacctccagagccccacacactatctttacgctttccacctttagacatactcagaagcacggtagccttatccagagcagctctagcctgcacacaatctacagttcctttgtaactatcaatataggtattacataaaattccatctccaacagctctagcaataaactggcccaccaactgtggtgctctaggagtatccagtgctaattcaggtagatctttcaacaatttatcaaatgatttttccacatcagttgtgctcattactgtcccacaaaggtcagaaagaagcttagatgtcatctctctatgactagccttcccctccaatgctaaggatactgccaacactggtactccacttttcatttcaccaagatttaaatctcttaacatttccgcaacttcattagtatctccatgctcaaaatattcctgtatgattggtgttaaagtcttctcaaatgccctttcatccaaaggcaaaactacagtttcataaacacagttctcctggtcatcatcatagttaggatctttcacatccacctcctccacatcatacacctgtccaggtgtaccccagacacctttgcctcctgcaccacctttctttggtagtccccttcctttcccagatctggatcgcctatccagcaaccttccctttggactggttggcacagttaatccacttctaagggcgtcactcccactgtcgctgaccgaatcgcctctgccagagtcccgggatgagtttttccttagtcgcctttttgccttggcattaattctagcttcgttaatggaggatgctgaaatccaatttccatttatttcattctttatttcctcagtcccagcattttcttcatcaccggaaaagagagagtcacttaagttatcaggatatttggtcatctattccacaaaactgttcatttttatgataataacatgctattgaagcaccatggagaattagggaaaataccctgcagggtttacattcagtatctgctcattttctacatccattttcccttaatttcgcttgcactgattaaacaaattacctaatggaaatcttccttcagaatccctcgggcccccgccgctgctcgcccaggttcctggtcagccggccccgaccccgctcttctgtctctgccgccgcctcggagagtctct

SEQ ID NO: 14554 - RNA, 3025 nt, Homo sapiens
  source 1..3025: mol_type = other RNA
gctgggattacaggcatgagccaccgtgcccagcccttaaatctcatttttaagaaaccctcacctattctgtagtcagctaagcttttaattacattaattttaagcacttgagaataaaatgactgcatttatcatccaagtgtcaaacaattaaaaacctaaaaatggtaactatatataagctgaggtaatatgggcttgataaagcccatgaggtaaatatgaacactaaacttggttttaattctaacagactatatctaaacctgtaagcagtatactcctaacagtaccctcataaattctgaatataattcttgtttgctgcagtcaatatttggcagtttaaattagcacagacgttgaggccttgctgagttattaggctatgtaaaagaggttaaaaatatgatcattctttattgttaattggtaatattttctcatacattaggtaaatgtcaagctttgggtctctggagtataactttttgtaacattagccattatttggtaacagaatttaaggatgatggaatgatggaaggtattacatatttctaaaacttaattaagctctaggtcagataacaatggagtaaagtgatacctgcatttttttccccagtgtaatcttaatttactattgtatttttcacttaaaattttgtagggaaaaaaagttttcaagggaacactaagattaaattgactaggttcaaatatgcttccttatgagattcaaaatttactgtgtgaaattaaagtttaagagacctaaaaaaatgtactcccaataaagaatcaatactgcttcacatgttttattttggtgtacattcttctagaaccaggttcatttttccagttttgtagaaaaatagatgttccagccaccttttacttaactgtctagtcttttaagaccaatcagtatgttccctggaaagatgaataagtctcatgactaattttttaaaaattctttaagacaaagaaataactttctttttttactcccaaagcacagtatctcaacagcagcagccaacatggggttttagcagcttaactttaccccctaaataaagctttgtataaaccagtgattttactacaaaaaacactgtccttgaaagaaaggagtggcagtcagacatcaatgcaaaacttggaatgattagataataaacatggcacttacaaaaggtagcttattagaatattccacttaagaagaggttacttttctgtccctccttgccccctcgaaaaacaaaaaaaaaagaaaaaacatttcctttaaaaattccccttaaatgtaggtttataaaatgtcagaaatgccttgtacccaaaacaagtgcttaaaaaaaaaaaaaaaaaaaacttgtgctaacaactcttacaattcagatatatatttttataacatctaagactgcaagagttcttatattcagtagctctctggtttaagacgacctccatctccttcgcttacaaaacgctttctgccccttgaaggacaaagatctctgagttgtttggaaattattccagcctgaaaacattcttctacaaaccgctccagcacagagtatgaatgtgggacatccagattaatgtccggaatttcattgtaaattctctcataacctcttttcatttggtctacagtaatggtagaagacttccaaagggactttaataaatccaaaatcatcttaaatgtactttctccagttgactctaaaaccattataatagcttcatatacaagctcatggtgaaaatgaggtacttccagttccttaaggcaatgttcagcttcagatatgtctccagagagtaaatattctttcagcagcatatcaatctctttaacaaggtgattgacagattgctgcccacctccagagccccacacactatctttacgctttccacctttagacatactcagaagcacggtagccttatccagagcagctctagcctgcacacaatctacagttcctttgtaactatcaatataggtattacataaaattccatctccaacagctctagcaataaactggcccaccaactgtggtgctctaggagtatccagtgctaattcaggtagatctttcaacaatttatcaaatgatttttccacatcagttgtgctcattactgtcccacaaaggtcagaaagaagcttagatgtcatctctctatgactagccttcccctccaatgctaaggatactgccaacactggtactccacttttcatttcaccaagatttaaatctcttaacatttccgcaacttcattagtatctccatgctcaaaatattcctgtatgattggtgttaaagtcttctcaaatgccctttcatccaaaggcaaaactacagtttcataaacacagttctcctggtcatcatcatagttaggatctttcacatccacctcctccacatcatacacctgtccaggtgtaccccagacacctttgcctcctgcaccacctttctttggtagtccccttcctttcccagatctggatcgcctatccagcaaccttccctttggactggttggcacagttaatccacttctaagggcgtcactcccactgtcgctgaccgaatcgcctctgccagagtcccgggatgagtttttccttagtcgcctttttgccttggcattaattctagcttcgttaatggaggatgctgaaatccaatttccatttatttcattctttatttcctcagtcccagcattttcttcatcaccggaaaagagagagtcacttaagttatcaggatctgcagggtttacattcagtatctgctcattttctacatccattttcccttaatttcgcttgcactgattaaacaaattacctaatggaaatcttccttcagaatccctcgggcccccgccgctgctcgcccaggttcctggtcagccggccccgaccccgctcttctgtctctgccgccgcctcggagagtctct

SEQ ID NO: 14555 - RNA, 9844 nt, Homo sapiens
  source 1..9844: mol_type = other RNA
gctgggattacaggcatgagccaccgtgcccagcccttaattgctgtctgaaccttttttttttttttcaacctgacctgaggcatcaattcaggcacagtataactctgaccagtaagcggaagctaacccaaatgctttccagggctgaggggacatcatgagagttgtggtcatgtacagaagcacagtcccaggggcacaggtggtacccctgtaaacaaagaatttgcaatattagggcacctcaagcaggacatccattaggctgtacaggtgaacagacctcctaccaggggaactcctgcccaagtgtttccagtcccatctgaaaagttcccagagtccttggcttccaagggactgcctgaaggcagtgagtcccaaacagttttgcttgttcaggatacaagttgatccatctcatgagcatggatgacatttgtgggagatcttcatggaaagcatagaagctagacccactctgttgtcagtctgaactcaaagcactcacagcacatggaaaggcagcactgggaattttccttcagcaagaggaggcttccagggatcaagcctccccaggtgccaggctttaattattttctccaatattacaaaaacagtcgtgccctgttcagcaatcataacattgcattttttcaaccatctcttactctcagctaggcctttcctctggaagggttgtatgtaagaggcacaaaagcatttttgtagataaacttttttttttttttttttgagatatggtctggctctgttgcccaggctagagtgcggtggcacgattttggctcactgcaacctccgcctcctgggctcaagccatcctcctacctcagcctcctaagtagctggaaccaaaggcacatgccatcatgtccagctaatttttgcattttttgtagacacaggatttcaccatgttgccaggctggtcttgaactcctgaactcaagcaatctgcccacctcggcctcccaaagtgctgggatcatatgcatccatcactgcgcctggccaacatttttttttttaactatcatcctagagttcaagtagataaacgtttttatgcaacttaaccagaaagacattcagaaattggtaattatgtgtggagggttgaattatgtccccacaaaaattcatgctgaagccctaaccatctacctgtacctcaaaatgtgagtatatttgaagataggccctgaagaggtaactaagttaaaatgggattgttaggatgggccctaatccaacctgagtggtatccttattaaaagagaagattaggacacagacacccagacagagggaccatacaaggacacagtaagaaggcagccatctgcaagccaagcagagaggcctcagaagaatctaaagctgtcgacaccttgtcctggactttcagcctccagaactgcaggaaaataagtttctattgtgtaagtcactcagtttgtggtactttgttatggtatccttagcaaactaataaaggatgaaaccctgaatttttaaaaatttcaaaatgtgtttacataatcttctaccccttttgtcctgattattcaatgagcagactagaaaagcctaatacctttctggggacagctacgttttaataatccacctaccttactaagctgtgtgtgctgggagaaaagtgagggaagtagagtcaggctgtcagtccactgttgcaagctgcaactaatcccaaaagctgaatgcaacaagtcaacagcagtgagagaagccccagagaaggtttgagtctggtctgtcaaaagcaggaggagaggtcatagtccttgcgatgtgcccttccccagcttggagcgtttggcaaatattagaagttaggaatgcaattagcctctgtattagagacaaagagcctatcagcagcttgatcttagatggtcccattagagaataagcccttttcagccaggttccaggacgttttcatagtttagcgctccacggagggggtccttaatctccaacggccccaacgtctgagtcctggtcattgagcctgtgcctgctttcagttcagcatagctcgtgttgaggctaaaacagctcaaggcagacagtagcaggtttcagcttagagtcagggccaggcaattaggatctgagaatttgagattctcaacaagcagctgcttttcttcagcagcagtgaaggcatgctgcatggccagacagctgtggtccaagtgacatgcaaggctgcctttttatcttgttggtcttagagtccaattgacccactcaaaaaaaatgcatattagactagacaatcatcagcctctaaggggagacatttgattttgacaagggttcattagcaatttaactgtattttcattttccaaacagattgcttctctttacatgttgtctccctctttcccgaggctccagtaagcacgaatcacagcaaaaataatcagttacagcctgttctggttccaatatccgaagaatttaaattccaacctatccactagtggcaaaaaactagaaagctgtatcccactaacacctttcatattttatttttgagtagctttatttgattagggtgatccctctagcatttatgaaattaacaagcataaaactttttttttaagagatgagtagctgggactacaggcgcacgccactgcgtccagctaaggtatgttttttaagcaatgaaatcaaccagtaaaaacaagttcaaatatttttcattcacacactcaaggcctgctgagcatccactgcatgtgttttacttgttccattagaaaggtttattaaaaaatggcggggcacagtggctcatgactgtaatcccagcacttagggaggccaagatcgcttgagcccaggagttcaagactagtctgggcaacatggtaaaaccctgtctctatttaaaaaataaacaaatacaagcaagtttttttttaaaaaatgatatattaaagaaaatcctcctaattctcttatgtcttttcatagctgtttccatgttctcatattcccatccttgtcaacatggaatttttgttgttgttgttgtggtttttttttttttttttgagacggagtctcgctctgtcgcccaggctggagtgcagtggcacaattacagctcactgcaagctccgccccctgggttcgcgccattctcctgcctcagcctcccaagtagctgggaatacaggcacccgccaccatgcctggctaatttttttgtatttttagtagagatggggtttcactgtgttagccaggatggtcttgatctcctgacctcgtgatctgcccacctcggcctcccgaagtgatgggattacaggcttgagccactgcgcctggccaaacatggaatttgttttatacagttgcaattatggtccattaatacaatctatttgtatgttatcagtaacagtaatactaacagtgaacccttattaagcatttactatgtgccaggcacaaggctaagagttttacagagatgatctcatttaccttgggttacttacccaaccaaggtttatagccagcaggtggcaaagcttgaattccaacccaactctgctgactcccaactacacccacctgcacacttgcctcttgggccttgtttgtctggcaagtcctaaatcccagactcatttgttcacttgcttgcttcctccctccctccctaccaaaacacagtatgatctgtcggttaaactcaatagactaaaaactccgggttcaaatgctagctcctccatcactagctgtatgaccttgggaaagtacttaatctctctgtgcctcaatttccatgtttataaaatgggataaagtgcccattatagtgcccatttcctaggattctatccaggagatgatgtgcctatttcctaaggttcttataatgagattctgcaaggacagcactccaaatagtacaggcacatggttttgacagttgtttctgttattattgaaataaaaagaacctatacctgttcccaggaagctcagagtctctcacaggccttttcagttcctggggctctcatatttcctcattctcccagactcctctgaccctactcttcctcaggttcttactgctcctgtgggaaatcagaaagagcagccagcagacaacaccaactgagatgaatgcagctgaaatggcacaggtcagtatggccaagaaacaccatgggctaatgttcagacccatggtatgaaagccagagtgggtgtgaatttcactcccatgtctcttatcttggatggttttcatctgcatgacccatttgcccaatgcccaatggatgtgaagatacagaaaagtccaggtactgttttcagggaagtaagatgtcctgtgccaactcttctcacttcagggtccaagtcagagtgcacaaggaaagcaggtggggctggcccaccagcaaaagcttcaggagagcaagggattggctgactgggctgcaagggtagtgttcaaagccagctgccttggaggccaagatagtggaggagctgcataaaacatggattttgcagccaagtaagagctggccttgattccagctcagccatttattagatgtgtggcattgggcaaatttacttaacctctctgaatatcagtttcctctgctgtaaaacaggctgtgaaactctcacttttttgacagttgggaggattaaatgtttgcaccccatagatacaaaacaaggaagggtgatttctccatctcttgtttgtggcggactgattataaagggcaagatgttttaaattttattttaaattttaaaaatatgtaagaatgctatgccttatactctaaggggttttgctcaaggtgtatcacttcctaataaaagtgcctaataaactgccgtttattgagtgctcaccctgagccagtacttatgctttacatgtataaatgcatttcaatcatcataataccctatccaacttccccattttatggatgagaaacctgaggttccacgaagtaagataacttgctcaaagtcacaaggctagccaatggcaggctgggatttgatcagcctgactctagcactcacactcctcaccactatgatggctctcaaaatgggcccctcagaccctctctgtattttgactctttggctttctcactcactaagctgtgagatccctatgagaaagaactggctccatcttagtctccactgtatccccaggacctaggaagtgcttggcacctagtagtggcttggaaagcacttgttaaatgaataaatgagtgatggtgtctctcttctctgtgcagcatatggtgaggggcccaccttcttacccctaaatggaagcaagcacatattctactaaaagcacaagcccattgctggggggctctagaagtgtttcagttatcatgtacttatgggaactgtagaagttggcgagacattttgctgagaccagttctgaaaaaaccaggccttcggacacgctgtcccaacactgccagtatcatttcaggggacttgcagctccatggaagctaacccccaggagaccagccagctggatttgactacctatagtcaccatccaggttgtcagatgccaattttttttcaggagaaccgctgaggctagccagaatatggctgggcagcaccctctaggctctcactggatagaacaggatacagagaaaggcctccctagccaccaagacctcttccttatagctgagaaacttccaaggatatgttaactatgaacaatgtttgtctgattaatttcaagtctgccagatgtatcagtgactaagaaaggaactgtggcctcagatcctgagtgaaatggttcatgcagaagtgactaatacagaagccaccaccccaaccccaaataaccacaagggctctgtgcagccatgtaaaacagaatcagtcaacaggaggctcacaagacaatcattcacctttgttccctgcagcaggtatcctgcaatctgagacttatcttgagctggggtaaggtctgaggcatgctggcagggtgtgtgagggttgggggtgagggtggtcacatccaggcaatcattctattaaggatgtgctagatgacccacagactcaggcctgactcctcaggagctcacagttagtaggggttcagacaagaacacaggtacataactaaaactctattgataagggcgcctcggtaaggtgctatgggaaccataaggatgcagttccatggcccagtcagctcatctggggaaaaataataaaacaaaaaggaagcagttccagacagaagaccatctccaaatggttctttattgaacacccactttggctaggcaatatcctccccctgccctctaatccaggctcaggtacccccagtggagtatcctcagaaggcaactcccaagaccaggagtaatgagagattgggcagagggtaagggacagcagggagacggaggaaaatgaagacaccagggaaagaggagaggcctgaactggacagctgatgctttgtcctgcccagcacccattcgtcccttcttcaggtaatatcatctgccaccacaaccaccagcaccaactctcagtctctgtgggtacatgccaggcctgtccatttggtgtattccatcttcctggccacaatgatgacttgaggctggataccttcctcgtctggaccaatgagaaccaaatccagcagttctgtcagcaaaggggagctctttttatcaataactggtgctgtggggccacactgtgaagcccaagaataaagccaactcaaatgaaagcagagctgagagccaaagagacagatccctgtttggagtcctgggatgcagcctgaagcccaatctagcccatccttttcagctacgtgagccattaaattccctctgccccaagtgaactggaaagagtcccaaccaaggtccttcccatctggttgttcttctggaagtattttgaggacaaggagattttcatctccagggttataaaagtaattgtgtggtgacaggctgttcctaggtccctggggtgagagccaccatggagacagagtccagctcgcctttcctaggatacacactcacgactgtcaacacatcttcgaatacatcagcacataattataaactcctattgtttgtagtagctattgtttttgtcttcccatcaccttgttttggatgaagaaaaggtcatgacccagactggattaatcatgtggccaaacatgcatggccacagtgactgatccaagaggacatggaactcacaacaaaccattgagaactttgggagtttccaaattcgaactggaagggaagaaacctttcattcagagcccccaagctaggaggatgcaggtctggagctatcagctgtcatggctccaaatgcacggcgaaggctcatgtgcagcaggaggaaaggaagccaacaaagaggcctggttgagtctgcttgttgtctcccaatggccattcttcccccactcctttttactagcagaatctccttcctcagagttttggctgcccaagtagaaactaaatttacagcctcctttgttgctaactgtggccacatggcaagacagtaggaacctgggtgcctgatgacatcatggaccagccccttgcctggcctggaccagctgactatcactgcactgttatgggagagagaaataaacttccatcttgtcgaagctatgtattttggtggttttatgtataaacattttaaaaataacaaactagaaaggagttctagatggaactagtggcaatgattacatacagctgttttgttttgcaaaccccacaactggatattaagtcaggatagctcctgctaaattctaacctcaaggctgaactgttctgccctattcacttacagatcagagcattaggcaaggacaaccttcttagcccctcacttctgaatcttccttctaagctaagaggtcagagcagaacgaggaaatgttgtgctatttggccagaaggagatggtaagaacagccctagtaacttcatttactcctgaggctctgtgcccacaaactgattctaagagcccttcctgtatatatgcgaattagctctaagtacagacattttggtgtgaattgtggagtttatggcaaatacagggtaggctgaatggttctaggccaggaagcaagagttcacaaatgcggtgtcttcaatgaaataaggtaagtaccttgaagcaaggagtaaccacctgactaatgcatccacatgagagactcaaatctaacacttggcaaaattacaatctgggatactgaggtccccacttttagtgaaagccaaaggccctaggtcaaaatgctaaaaagtcttttactaactatcctaggacagctaaggtcattttgggaagaagagagaaacactattcacccctcccttcaagttttaatagacaacaggaatctgggctctgaaaagtcacaaacacctttcccaagatgatgagcaactgcaacaactggccaaatgtgttagcagcagaaaagctgggcattacctgtgtgagaggcgctcagcatgggcagtgaatggccgtgagcagcgcaccagctacatagcctccacaccggaagggtgctgctgctctgcaggtccgtttcaggcgggatccagccatccacaggaccaaggggctggagtgttgggaacagatgattctgtgttccacagataatggtacaaagtgactgttcatagataaggtgtaagcacagcatttgaagacagctcctccagatggtctgtctgttagtgaattcttaagcacttagagccttgaagattgagaaattctaaagaaattttttaaaaggaggagggtggtagatgtcaaagacacaaaagctctttgtaggtgctgactggctcactttgtccccaggttcatcttagagctcaagcagattcaagacatgaggcagagatgctagacttgcgtcaggggcaaaaacttctggtagtagctcttggtgacgtcaatcatcagctcctgagtgcactccgggagctcccctgagaagagtcctgggcagcctgagaagacagtgaatggtggaaccacagtttctggaggtaatactgtgttgtcaagaattttgcagcagtctttcaacacacatcggcgcccaatcacacagttcttcccaacatgaacataggaaccaatctgtgctgcgttgaccacacaatcttcctcaataaagacatggtctccaatatgtaaaggaaagaatgcaacacctttgctgaacttcttgaatggtggccttatgacactacgacttttcacaacacaatgacgtccaactcttacatttgccagatcccctcggataatacagtcattcatcacaatggtctgcagtaatcccagctactcgggaggctgaggcaggagaatcgcttgaacctgggaggcggaggttgcagtgagccgagatcgcgccattgcactccagccttgccattgagaacgatgttctggcttccacacaacactgactggcgactgactttgttcccagatgccgtctcgatgtactcagacttgttgtagagcagctcgcccaactccatggccgccgcctccttccctcagccccggatcctgtcagagtcagtcggtcagtctttcagagattccggctacttcc

SEQ ID NO: 14556 - RNA, 9743 nt, Homo sapiens
  source 1..9743: mol_type = other RNA
gctgggattacaggcatgagccaccgtgcccagcccttaattgctgtctgaaccttttttttttttttcaacctgacctgaggcatcaattcaggcacagtataactctgaccagtaagcggaagctaacccaaatgctttccagggctgaggggacatcatgagagttgtggtcatgtacagaagcacagtcccaggggcacaggtggtacccctgtaaacaaagaatttgcaatattagggcacctcaagcaggacatccattaggctgtacaggtgaacagacctcctaccaggggaactcctgcccaagtgtttccagtcccatctgaaaagttcccagagtccttggcttccaagggactgcctgaaggcagtgagtcccaaacagttttgcttgttcaggatacaagttgatccatctcatgagcatggatgacatttgtgggagatcttcatggaaagcatagaagctagacccactctgttgtcagtctgaactcaaagcactcacagcacatggaaaggcagcactgggaattttccttcagcaagaggaggcttccagggatcaagcctccccaggtgccaggctttaattattttctccaatattacaaaaacagtcgtgccctgttcagcaatcataacattgcattttttcaaccatctcttactctcagctaggcctttcctctggaagggttgtatgtaagaggcacaaaagcatttttgtagataaacttttttttttttttttttgagatatggtctggctctgttgcccaggctagagtgcggtggcacgattttggctcactgcaacctccgcctcctgggctcaagccatcctcctacctcagcctcctaagtagctggaaccaaaggcacatgccatcatgtccagctaatttttgcattttttgtagacacaggatttcaccatgttgccaggctggtcttgaactcctgaactcaagcaatctgcccacctcggcctcccaaagtgctgggatcatatgcatccatcactgcgcctggccaacatttttttttttaactatcatcctagagttcaagtagataaacgtttttatgcaacttaaccagaaagacattcagaaattggtaattatgtgtggagggttgaattatgtccccacaaaaattcatgctgaagccctaaccatctacctgtacctcaaaatgtgagtatatttgaagataggccctgaagaggtaactaagttaaaatgggattgttaggatgggccctaatccaacctgagtggtatccttattaaaagagaagattaggacacagacacccagacagagggaccatacaaggacacagtaagaaggcagccatctgcaagccaagcagagaggcctcagaagaatctaaagctgtcgacaccttgtcctggactttcagcctccagaactgcaggaaaataagtttctattgtgtaagtcactcagtttgtggtactttgttatggtatccttagcaaactaataaaggatgaaaccctgaatttttaaaaatttcaaaatgtgtttacataatcttctaccccttttgtcctgattattcaatgagcagactagaaaagcctaatacctttctggggacagctacgttttaataatccacctaccttactaagctgtgtgtgctgggagaaaagtgagggaagtagagtcaggctgtcagtccactgttgcaagctgcaactaatcccaaaagctgaatgcaacaagtcaacagcagtgagagaagccccagagaaggtttgagtctggtctgtcaaaagcaggaggagaggtcatagtccttgcgatgtgcccttccccagcttggagcgtttggcaaatattagaagttaggaatgcaattagcctctgtattagagacaaagagcctatcagcagcttgatcttagatggtcccattagagaataagcccttttcagccaggttccaggacgttttcatagtttagcgctccacggagggggtccttaatctccaacggccccaacgtctgagtcctggtcattgagcctgtgcctgctttcagttcagcatagctcgtgttgaggctaaaacagctcaaggcagacagtagcaggtttcagcttagagtcagggccaggcaattaggatctgagaatttgagattctcaacaagcagctgcttttcttcagcagcagtgaaggcatgctgcatggccagacagctgtggtccaagtgacatgcaaggctgcctttttatcttgttggtcttagagtccaattgacccactcaaaaaaaatgcatattagactagacaatcatcagcctctaaggggagacatttgattttgacaagggttcattagcaatttaactgtattttcattttccaaacagattgcttctctttacatgttgtctccctctttcccgaggctccagtaagcacgaatcacagcaaaaataatcagttacagcctgttctggttccaatatccgaagaatttaaattccaacctatccactagtggcaaaaaactagaaagctgtatcccactaacacctttcatattttatttttgagtagctttatttgattagggtgatccctctagcatttatgaaattaacaagcataaaactttttttttaagagatgagtagctgggactacaggcgcacgccactgcgtccagctaaggtatgttttttaagcaatgaaatcaaccagtaaaaacaagttcaaatatttttcattcacacactcaaggcctgctgagcatccactgcatgtgttttacttgttccattagaaaggtttattaaaaaatggcggggcacagtggctcatgactgtaatcccagcacttagggaggccaagatcgcttgagcccaggagttcaagactagtctgggcaacatggtaaaaccctgtctctatttaaaaaataaacaaatacaagcaagtttttttttaaaaaatgatatattaaagaaaatcctcctaattctcttatgtcttttcatagctgtttccatgttctcatattcccatccttgtcaacatggaatttttgttgttgttgttgtggtttttttttttttttttgagacggagtctcgctctgtcgcccaggctggagtgcagtggcacaattacagctcactgcaagctccgccccctgggttcgcgccattctcctgcctcagcctcccaagtagctgggaatacaggcacccgccaccatgcctggctaatttttttgtatttttagtagagatggggtttcactgtgttagccaggatggtcttgatctcctgacctcgtgatctgcccacctcggcctcccgaagtgatgggattacaggcttgagccactgcgcctggccaaacatggaatttgttttatacagttgcaattatggtccattaatacaatctatttgtatgttatcagtaacagtaatactaacagtgaacccttattaagcatttactatgtgccaggcacaaggctaagagttttacagagatgatctcatttaccttgggttacttacccaaccaaggtttatagccagcaggtggcaaagcttgaattccaacccaactctgctgactcccaactacacccacctgcacacttgcctcttgggccttgtttgtctggcaagtcctaaatcccagactcatttgttcacttgcttgcttcctccctccctccctaccaaaacacagtatgatctgtcggttaaactcaatagactaaaaactccgggttcaaatgctagctcctccatcactagctgtatgaccttgggaaagtacttaatctctctgtgcctcaatttccatgtttataaaatgggataaagtgcccattatagtgcccatttcctaggattctatccaggagatgatgtgcctatttcctaaggttcttataatgagattctgcaaggacagcactccaaatagtacaggcacatggttttgacagttgtttctgttattattgaaataaaaagaacctatacctgttcccaggaagctcagagtctctcacaggccttttcagttcctggggctctcatatttcctcattctcccagactcctctgaccctactcttcctcaggttcttactgctcctgtgggaaatcagaaagagcagccagcagacaacaccaactgagatgaatgcagctgaaatggcacaggtcagtatggccaagaaacaccatgggctaatgttcagacccatggtatgaaagccagagtgggtgtgaatttcactcccatgtctcttatcttggatggttttcatctgcatgacccatttgcccaatgcccaatggatgtgaagatacagaaaagtccaggtactgttttcagggaagtaagatgtcctgtgccaactcttctcacttcagggtccaagtcagagtgcacaaggaaagcaggtggggctggcccaccagcaaaagcttcaggagagcaagggattggctgactgggctgcaagggtagtgttcaaagccagctgccttggaggccaagatagtggaggagctgcataaaacatggattttgcagccaagtaagagctggccttgattccagctcagccatttattagatgtgtggcattgggcaaatttacttaacctctctgaatatcagtttcctctgctgtaaaacaggctgtgaaactctcacttttttgacagttgggaggattaaatgtttgcaccccatagatacaaaacaaggaagggtgatttctccatctcttgtttgtggcggactgattataaagggcaagatgttttaaattttattttaaattttaaaaatatgtaagaatgctatgccttatactctaaggggttttgctcaaggtgtatcacttcctaataaaagtgcctaataaactgccgtttattgagtgctcaccctgagccagtacttatgctttacatgtataaatgcatttcaatcatcataataccctatccaacttccccattttatggatgagaaacctgaggttccacgaagtaagataacttgctcaaagtcacaaggctagccaatggcaggctgggatttgatcagcctgactctagcactcacactcctcaccactatgatggctctcaaaatgggcccctcagaccctctctgtattttgactctttggctttctcactcactaagctgtgagatccctatgagaaagaactggctccatcttagtctccactgtatccccaggacctaggaagtgcttggcacctagtagtggcttggaaagcacttgttaaatgaataaatgagtgatggtgtctctcttctctgtgcagcatatggtgaggggcccaccttcttacccctaaatggaagcaagcacatattctactaaaagcacaagcccattgctggggggctctagaagtgtttcagttatcatgtacttatgggaactgtagaagttggcgagacattttgctgagaccagttctgaaaaaaccaggccttcggacacgctgtcccaacactgccagtatcatttcaggggacttgcagctccatggaagctaacccccaggagaccagccagctggatttgactacctatagtcaccatccaggttgtcagatgccaattttttttcaggagaaccgctgaggctagccagaatatggctgggcagcaccctctaggctctcactggatagaacaggatacagagaaaggcctccctagccaccaagacctcttccttatagctgagaaacttccaaggatatgttaactatgaacaatgtttgtctgattaatttcaagtctgccagatgtatcagtgactaagaaaggaactgtggcctcagatcctgagtgaaatggttcatgcagaagtgactaatacagaagccaccaccccaaccccaaataaccacaagggctctgtgcagccatgtaaaacagaatcagtcaacaggaggctcacaagacaatcattcacctttgttccctgcagcaggtatcctgcaatctgagacttatcttgagctggggtaaggtctgaggcatgctggcagggtgtgtgagggttgggggtgagggtggtcacatccaggcaatcattctattaaggatgtgctagatgacccacagactcaggcctgactcctcaggagctcacagttagtaggggttcagacaagaacacaggtacataactaaaactctattgataagggcgcctcggtaaggtgctatgggaaccataaggatgcagttccatggcccagtcagctcatctggggaaaaataataaaacaaaaaggaagcagttccagacagaagaccatctccaaatggttctttattgaacacccactttggctaggcaatatcctccccctgccctctaatccaggctcaggtacccccagtggagtatcctcagaaggcaactcccaagaccaggagtaatgagagattgggcagagggtaagggacagcagggagacggaggaaaatgaagacaccagggaaagaggagaggcctgaactggacagctgatgctttgtcctgcccagcacccattcgtcccttcttcaggtaatatcatctgccaccacaaccaccagcaccaactctcagtctctgtgggtacatgccaggcctgtccatttggtgtattccatcttcctggccacaatgatgacttgaggctggataccttcctcgtctggaccaatgagaaccaaatccagcagttctgtcagcaaaggggagctctttttatcaataactggtgctgtggggccacactgtgaagcccaagaataaagccaactcaaatgaaagcagagctgagagccaaagagacagatccctgtttggagtcctgggatgcagcctgaagcccaatctagcccatccttttcagctacgtgagccattaaattccctctgccccaagtgaactggaaagagtcccaaccaaggtccttcccatctggttgttcttctggaagtattttgaggacaaggagattttcatctccagggttataaaagtaattgtgtggtgacaggctgttcctaggtccctggggtgagagccaccatggagacagagtccagctcgcctttcctaggatacacactcacgactgtcaacacatcttcgaatacatcagcacataattataaactcctattgtttgtagtagctattgtttttgtcttcccatcaccttgttttggatgaagaaaaggtcatgacccagactggattaatcatgtggccaaacatgcatggccacagtgactgatccaagaggacatggaactcacaacaaaccattgagaactttgggagtttccaaattcgaactggaagggaagaaacctttcattcagagcccccaagctaggaggatgcaggtctggagctatcagctgtcatggctccaaatgcacggcgaaggctcatgtgcagcaggaggaaaggaagccaacaaagaggcctggttgagtctgcttgttgtctcccaatggccattcttcccccactcctttttactagcagaatctccttcctcagagttttggctgcccaagtagaaactaaatttacagcctcctttgttgctaactgtggccacatggcaagacagtaggaacctgggtgcctgatgacatcatggaccagccccttgcctggcctggaccagctgactatcactgcactgttatgggagagagaaataaacttccatcttgtcgaagctatgtattttggtggttttatgtataaacattttaaaaataacaaactagaaaggagttctagatggaactagtggcaatgattacatacagctgttttgttttgcaaaccccacaactggatattaagtcaggatagctcctgctaaattctaacctcaaggctgaactgttctgccctattcacttacagatcagagcattaggcaaggacaaccttcttagcccctcacttctgaatcttccttctaagctaagaggtcagagcagaacgaggaaatgttgtgctatttggccagaaggagatggtaagaacagccctagtaacttcatttactcctgaggctctgtgcccacaaactgattctaagagcccttcctgtatatatgcgaattagctctaagtacagacattttggtgtgaattgtggagtttatggcaaatacagggtaggctgaatggttctaggccaggaagcaagagttcacaaatgcggtgtcttcaatgaaataaggtaagtaccttgaagcaaggagtaaccacctgactaatgcatccacatgagagactcaaatctaacacttggcaaaattacaatctgggatactgaggtccccacttttagtgaaagccaaaggccctaggtcaaaatgctaaaaagtcttttactaactatcctaggacagctaaggtcattttgggaagaagagagaaacactattcacccctcccttcaagttttaatagacaacaggaatctgggctctgaaaagtcacaaacacctttcccaagatgatgagcaactgcaacaactggccaaatgtgttagcagcagaaaagctgggcattacctgtgtgagaggcgctcagcatgggcagtgaatggccgtgagcagcgcaccagctacatagcctccacaccggaagggtgctgctgctctgcaggtccgtttcaggcgggatccagccatccacaggaccaaggggctggagtgttgggaacagatgattctgtgttccacagataatggtacaaagtgactgttcatagataaggtgtaagcacagcatttgaagacagctcctccagatggtctgtctgttagtgaattcttaagcacttagagccttgaagattgagaaattctaaagaaattttttaaaaggaggagggtggtagatgtcaaagacacaaaagctctttgtaggtgctgactggctcactttgtccccaggttcatcttagagctcaagcagattcaagacatgaggcagagatgctagacttgcgtcaggggcaaaaacttctggtagtagctcttggtgacgtcaatcatcagctcctgagtgcactccgggagctcccctgagaagagtcctgggcagcctgagaagacagtgaatggtggaaccacagtttctggaggtaatactgtgttgtcaagaattttgcagcagtctttcaacacacatcggcgcccaatcacacagttcttcccaacatgaacataggaaccaatctgtgctgcgttgaccacacaatcttcctcaataaagacatggtctccaatatgtaaaggaaagaatgcaacacctttgctgaacttcttgaatggtggccttatgacactacgacttttcacaacacaatgacgtccaactcttacatttgccagatcccctcggataatacagtcattcatcacaatggtcttgccattgagaacgatgttctggcttccacacaacactgactggcgactgactttgttcccagatgccgtctcgatgtactcagacttgttgtagagcagctcgcccaactccatggccgccgcctccttccctcagccccggatcctgtcagagtcagtcggtcagtctttcagagattccggctacttcc

SEQ ID NO: 14557 - RNA, 12039 nt, Homo sapiens
  source 1..12039: mol_type = other RNA
gctgggattacaggcatgagccaccgtgcccagcctacaggtgaattttttaattagcttcaaattgaccgacattaaatgttagacacaagaacgggctacactccatgccacatgaaatgcaattgagttgacgtgcaggtctgtcagaggcaggaaacaaactatatatgaccttgaaggaagagttgcatttgagcagcgagagcagagggggaggatggagcaataagttggaagtacgcaagtgagcaaaggaattgagaatcaggggaaatggagaggagtctttctggaatgtgatgaattgaaaggcaatagcttctgataggatctaaaatgtgggttaggaccagatcacagagtttacctggaggactgtgagtttggcagaggcaagggaagccattggagatttagcaggggaatggcagagtctaaattcatttgagaaggagtcccctggcagcagtaaatagggcaagtggttaggaatggggagaatcttgctggcactcatgggaaacatggtggcctcagcatgctggctgcggggcaggaagggcagatccggaggaagctttatagaggaactcagctgcactgtgccatgccgaaggctactggctgcagagggctgcaagcactcgaaatgtgactgggtcaaattctgaagcactgacaatgcaaaatacacagagatttccaagaaaggagaacgtaagacatctcattagtaaagctttatattggttacatgttgaaataaaattttcgatctatcgggttaaataaattttatcctttttccttttatttccagagtcttgctctgttaatgcaggctggagtgctcctttttcttgttaaagtggttcctggcacacttgtaatcccagcactttgggaggccaaggcatgctttgagcccaggagttccaggccagactgggccacatagggtgaccccatcactacacaaaacttaaaaatcagctcggcgtggtggcgccacacctatggtcccagctacttgggagactcaggcagcaagatcacttgagcctggttggttgaagctgcagtgagccatgattacattactacactccagcctgggtgacagagcgagaccctgtctcaaaaaataaaatggctcctggaaagtttaaaattgtagatatgtggctctcagttatattgctgttggacagccctgatgtagacggctttagctaactattaccagctgtggaaaaaggcaggaggtgggtccctgaggtgagagtaatagcagttataggatacagaggcaaaaggtagagtgtgaggtgctgattggtgggtctagggatgggccatggttttggtggcaagatggacgctagaaatgtaggtttgtagttgtccacttagagaggggctttggactctgaggaagagggtgaagagagaggaagtccctggaacttaaattgagcctgtatttgagatggaggaaatccagagaaagaggccagtgatggcagaggagactcagatctgagtggtgtacaagccagaagaaagtacatttcaggaagaaaaagcctcagcatgcaaacagaaaaatagggttctttttcagttgtgatgtgcacgctgccttcttaaacggatgagattggacttcccttgggctgccttggagacctagtgctgtcattgtggattctggctgcgtgccgctgcctgaccccggaagggtgggctgtttcctccacctcaaggggtcctgactgctgggcttttgtgagcggcacattcttcctgccatcagtgtgtcaacctccagagctctgctgactccagttaatgtgctgcttctgacatgctgccaactggaagtcagtatttgggaaagagagaataaactatgtctaagaatgaaaagatagagattctcttgtggaaccctcaggggactcagtgacatgatgttgctactctggacccttctttgtgtcctctgtaccagggaggactccagataggtcatacatgctcatgaagacgttgctctgctggtctcacatggtcggaaggacttgagtgaagtggtcagcaaggaaacttaggtagacatggaaaatgggctgcctgtgggaagctcgcaggtcttttggagggaggtggcatttaatttgttaacaggattcatgcataatggtttagctgaaaccttcttcaagttcccttaaagccttggtcatctctgttgtttttctcccaaagaaatctctgccagtacatttttctttatgacatgcttattcatgtgaagaagtatgagtggttttctaatctgctttttctttgtagaaccaccaccacctaaaatccccaaaattgagaccactcatccaccgttgcctccagcccacccacctccaggtaagcatctgctgaagcagcttggccagctgtgcacatcgcctctgaatgttggacgcagcaggtcctgggaacttagaaaagggagactggggcccagattgacaatgtcagccacaggcaggaatctttgcaaaattgttcttgggctgggcacaatggcttgtgtttttgatcccagcactttgggaggcggaggcaggagaatcacctgaccccaggagttcgaggtcagcctgggcaacaaagtgagaccctgtctaaaaaattagccaggtgtggtagcacacacctgtagtcccaactacttaggagtctgagatgggaagatcatttgagccctgggcagtcaaggctgcagtgagctatgattgcaccaccgtactccagcctgggtgagagggagaccgtgtctcaaagttctgattttgaccaggtattttgagaatgttgtaaattgttaagtatatctgaatattttccgacctctcacatccagaaatgctaaactacacattgtattagaatcagttttaggaaagaaagccaaaccccgccttctgagatagaggcagggttactgtggctactaggctccggccgcccctacacctgcttcctattggcagtgtgtcgtcttagtgcattctgaagaataagcaattgtacagagagtaaatgaaagagtgaaaagttctcaacaagtagtacatggtaagctggaaagcctctctgataccgctggcaatagaggagaaaagctgtaaagtagatggcattctttacctgtggcaccatttcagaaggtgatgcgctagagaaggccagagtgacctgtgcttgctctccaaaaggtggtcgatactccggaggcttccaagcctctgtcagcagctcctccagcctgctacactcactgttggtcggtgcacgtggctcacactggggctgacagcactgtgtgcccgtaacagatgtgccacagattacatttctgttcctactcaatcatgatagtgtttgtgctttgggagaacagaggcgtcattttccactttggggccaaatcccaaaacccccaattcaatatgaaccttacttaaatgcctgtggttgctcatgaagcatttatggagcacctcctcgccaagtgcagttcccctggtccgagcctggggctgtgccttcactgaggagatgggtggtttatctggggagcctggggcagccacaggggtgctgctacctccagggcactgagtagctgctgtggaggcctcagagctctgctccctcccccattacagatagccaggagtaggcctgggacttgagtgggacctgggtgccagatacactgccaggaggccatggctgaagagagcagggcctgggaggcgcagtaaagctgggccgtgaggaagggagggaagtacgcttcctgggaggccctaggccatgggaagaggcattcaggtcagcagtgatgtttagggagcagtttggtggcagtgtgtgggacttggtcaggagcaagtgtacagagagggaatggggtgcccaggagagacccccacttgctgttccagctcagtcacacagcacaagggcaggcacactggtgacttgaagattcaggctacagggtcgagtgttggaaaagttgatttctgcaaggtggaggagcaggcctgtgggcccaggtggctgtggagtgacacacaggaggcattgaagggtgtcagcacttttctgcacctcttttttagtcagctcctagaaccacagggcatctggccctgacctggagccaaagccagttatctaaggccaggcacatatgaccttcctacccggtaggctggcggggtgctgatgtggcacaccagtggcacacctgttaccgacctgatgaaatcctgctcatgctcgctttggcaagatcaaacgggttgtgtgccaatggccacgtctacccaaccaggatgtcgtgctgtgccttgcctaacccaagtgcctggggaaccagaagcatcttcgtggctttgtcctctctatgttctctggaaccagaaatgttgctcctgtggtctgtctcctgggctgccttgggaaaggacactcattctgtgtgtttggctacctgtggtggggtgttgcgatgtcattttccagtggtctgacggtgacccgggatcacaggccaaaacatgttaaataaggctttggcagaagggggcgtgagggctcatgggttgggaggcgctgtgggaggggcctgaggctggttctgagcacgagtatcttgggcgtgctcaacacctagtgctgcctgtccctgctgcacacgcagcacgcacacacacgcagcacgcacagacatgcagcacgcacgcagcacgcacacgcacacacatgcacacactcctctcaaggaggctgctatctgagagcacacagtggggtttgatgtagcctctcttgagtagaatagaacctgaattgctgcttcgatgggtacaccgggaatgtcagagacttgtacagaattgttttaagtgccatcacattcatttgactaactctgaggttttctgcaaaatgccactgctgcagacaggagttcagtgtggccctgacccctggggtcagtttctgaaggcagaaaaacagaggagcccccacacgttttgcactaggaagagggggctggggccagggcacaagggggcttcgggtgctgccgagactgcctgtaggtggtgtggtcagggctgagggagggaaaaccccaggtcgtcgcagacagggtggagggccttcttgacagatggtggggagacatctggtggcatcaggacatggggcatgggcccatgcgttgggccacagaggaggcgggcagctgctccctgctcctctgtaaagatggccctgaagggccaggaggcactgaaaaagcaaccattgctggcggaggccgggcactgatgcgtctctctcctgcagaccggaagcctcccctcgctgctgccttaggtgaggctgagccgccgggccctgtggatgccactgacctccccaaagtccagattccccctccggcccacccggcccctgtgcaccagccaccgccgctgccacaccggcccccgcccccacccccctccagctacatgaccgggatgtccaccaccagctcctacatgtctggagagggctaccagagcctgcagtccatgatgaagaccgagggaccctcctacggtgccctgccccccgcctacggcccacctgcacacctgccctaccacccccatgtctacccgcccaacccgcccccgccacctgtgcctcctcccccagcctccttccccccacctgccatcccaccccctactcctggctaccccccacccccacccacctacaaccccaacttcccacccccacccccacgcctcccgcctacccacgcagtcccccctcatcctcctccagggttgggcctgccgccagccagctacccacctcctgccgtcccccctggaggacagcctcctgtgcccccgcccattcccccacccggcatgcctccagttggggggctggggcgggcagcctggatgagataacgtgagccttttttccctctttgtttttttaacaagattttctaatcgacttgcagagtagttgaagtgggtaagcagcagggtaccttgtataatgcacgacagttgcagtatgggaagaatggaccgggcccctgggataaaatcagagtggtcctcacacctagaggacggggacaaccagctttcagagtagcctcatcagtgcccttgcagtctgactgtgtacacttggttcagctaatgtctgagagtcctgcactgggttactttatactagtgaggacgttaaccagccatattggctcaataaatagcttcggtaaggagttaatttccttctagaaatcagtgcctatttttcctggaaactcaattttaaatagtccaattccatctgaagccaagctgttgtcattttcattcggtgacattctctcccatgacacccagaaggggcagaagaaccacatttttcatttatagatgtttgcatcctttgtattaaaattattttgaaggggttgcctcattggatggctttttttttttcctccagggagaaggggagaaatgtacttggaaattaatgtatgtttacatctctttgcaaattcctgtacatagagatatattttttaagtgtgaatgtaacaacatactgtgaattccatcttggttacaaatgagactccttcagtcagttatccaaataaaagcagttctgaaactatccctttctttgttatgggtggaaggtggggctccaggccttcgcagtctgtggcttataaaatgtgcagaggccctccttccagaccctggggacgcgggagaggcctggctgcagctcacagcagccacagccaaccccactgcctcccaaggcactctgggtggatccgcacagctgcctgccaagccagcctgcccccatcctgtgcctgccttggtttcctttggaggacctggttgagttccaaaccagtttgaaactttgaagccttgctgcgtagaacgcacacaggaacccgggggcttggatttgaaaccctttccacttctggcctgtgatgagacagaggcagctggaggagcagcggcctcactgtccaccttgaggggccacggctctgtctgtggaaggggccccgactgagcccccatctgcggtgcttgaggggccttggccctgtctctgcctgctgaccctgccacccacgacagaaacaagcactgagcacccagccaggaggctcacaaagaggcctttatttatctagctcaaagtagacactatcacaatcttgtttgttactccttttactaaaatagttcaaatcaatgtttttaccacactatcaaaaagttctatttcttcttgtctccccacgtcagagtggttgaatagaaggtagaaacaggccgggagtccacgggctcccagctctaaacggcgccagggcaggaaggggtggctccaggtctcactgtggcaccttctacagaaaatagacgtagctgccgggcccggggacagaaaccagacgttccagtccatctccaaaaagcagcacaaatactttgccccacagtatgaaaaatatacacctctaccgctctgcagtcatgcatttagttttaagaaaaaaaaaaaatcagtagtatgtatcttgtttcctcaagtttcaagaaaaaaaaaatgaaaggtcacttttttctctttaaacactgatgtgtagctagtaacttggataaaaaggtgccaccctacaaaatgtgctcagcatgttctgaggccaggatgggcttggccacctgggctggggcgaaaggagacctccatctgtcacagtggaaactgaagccgagtgccagtgccgcgtccggcttcaagatcaagagtcagagcctttgaaatggaaagggggcatctgaaagggcacccccactgggggctttcagagctaaggctccagaaggaagggggtcgccctgctagtgacggagctgggagtcaccctgagctacagcatgcccagatttcccctgtgggaagccccatctgaccttctacagcccacggctctgcaactgccacctgtactcaggtacatggcgtcgctgctgctggcttttaaaatcagctattagtttgagatgtgacagtcgccgacagggttctgtcctagaaagccatcccagtgccgtgttggctcaggggtcaccagctttgtgctgcctccgtaacagcaggagggttctcaaagcaatgttccactgatccctggatgccactgcagcattaaagacagggtcagtccccttgaggggaaaggtggcttcaaggctgttctctgggcctgtttgcaggagatccgcaggtaccaggagcccgtacttattgcttatttcagtggtggccacgccaacctgacccaaacatgatgcacacgggctcccagacttggctgccactcaaaatggacccacagcccttgggctactctgcggttctttggactgcaagacccagaggggcctctgctcagctgcccactcgggcaagaatcactgggtaccatgagcagcaggtgttcacccaacttcacgtgtacacccctagtgaccgggagcgcaccacctgaccgggcgacactccttcccaaagagcctcctggcaacacccacggcaggagcgccacaccatcccatcaccagcacccacttacccccctggggctaagatggggggcgtgagcctttcccctgagagcaaacgggcagcaagaactgctcagaatagagccgccagctagggagagggacagggcggccatctccctcctcttgcctgcatccccagccctgggcctgcatgagacctgctgggtaggaagacagcctctctgggctcttcaggtggggctgagcagcccctggaagagcacaggagtctgacgaggacctggtgaggtcctggacccaagagctagggctgcttacagtggcatgagcggatgtggggaagcggcctgtccccgtgctgcagctgtgggatcaaaatccctgtcatgtgccacacatcaccccctctaggccttactttcctcacacacacagttttctattgcactttacagtttatacatggtcatttacactgaagatctcacttgatgccagaatcctgtgaggagggccttatgctgcccattttactactgaggacacgggctcagagtggggaggcaactctccacccgcagcgactgcaaggcagcagaactcagctccacccggcccgccctcagccgtcggctgttggctcacgccccctcagtgaggacccctgccctgtggcgctggatgacctggagccataagcatggccgaaaaggaacctcagagacctgtttccaccaagagcccagacaggctgagtgaactgctaaaggtcacaccacaaactaaaggcagaacctggccagacacgctccttcccaaaaagaacagaactctcatctgcagcctacacagctctgtccacagggacccaagatgcagccaggccctgggggaggtcacagccaaccagagccccagctgtggcccagtgctgcccatcaggaaaatcacatgtggctcagcccagaaactctccccaggcccttcctgttactggcctgtcatgtaaaccacgaaaagggacgtgcctcaggcatggggcaggaggagcccaagaagggcatagcctggacagggtggcagggggacattgcagagactgggggggagggggatgacctccaaaagcaaggagcagcgggcatcgggtggctgagcacagatccccaggtgtgagggcaccctgacctccaaggctgagggtcacaggaagggcccagggcagcctccagccagccacagatgtggtgagtggccttgtccacatgccggggacccagtgcttggggggcctggggccaggccacggcatttgggcaagaagtggtgccacctgcgtcaagacccaggtagtggtggtctctgtccagtgtgggtggcagccggggagtagagggtttgatgagtggcccctccatcccaggcaggacagaggagcctggacagttcccaggctggatctcagaagcagcctgcagcctcttgctcatggagcccagggcccagagggggaatgaggcgtccgggccgctctgctgcaggaacagtcgcagcgtctcgtcttcccaggttgctggtgtatgaggcgggagatggcggcttgggccagtgcatcggacccatggcagctgggccagggcgggcagcgtcctatgtacagttcaccacagaggaagaagacaggggctgggctggaggtcctgcccgtgtctggggcctgaaactccccctggggacccccagcagggccagtccacgtccacagaagagtggccctacaaaggccccttgaactggttcccagacaggtgctgccgtatggagggcttggagctggctgcatctcccagctttctccagaccacgttgcacatctcgcgaacgatggccttctccttctcactcaggtcctcctcacagctgtcctggagctgccggtccagattctcgtgtacctccaggaccttcatggcatgcacgacagcctcgggcttctgtcctgcagggctgtagccagcagaggggggcgagggcagctcaggtgcggggcaggccgggccgttctgcagggagtcctggtaggagggcggcagggacgcaagctgggactccgagtggtagggcgagaagcctttccgcagcgtgcggaactctccggagcctgcctgctgtgcgaggagcttgtcaccctccagcagcctcactttgctctccagttgcctgatgtaggtggatgagggatcgtgcaggccgttggggatgctgcggtggtgcggcggcgccgacaagtcgtccagggaccgacgtgtggctcctgccttgccgtcgggggccttgtgcggcccggggggcagcagcgggggtgggacgtggtggtggtggtcggggctgccgccgctgcccgcgctggacgtactgctgccgtcgcccacgtcgcgggcccccgcgccgggcgcgccacccgacagcggcccgctcaggctggcctggctgtcgatggagctgcgggagccggcgccgcccccgccgccgccgccaccgcttgcggcccccgtcgccgccagtgccgcgcgctcctcgtccagcagcagcaccagctccttgagctccaggttctcgcgcagcagggcctcctggcgcgcctcgagctcgcgcagcttctgctgcgagcgggccacctcgtgccacacggcgccggccgcgtggcgcccgaagcgctgccactcgcgcgccagcttgcgccccttctgccggtcgtcgtcgaggaagcagcagagctcgcgcagctcctggttgtcgtcctgcagccgctggttcacgtccttgaggccgcggatctccagcaggtgctgctgcagccgccggttcacgtcgcgcatcaggccgccgtgctccagcatgaggcccaccttctcgccctcggcgcgccgcagccgccgcgccagctcctccttgctccagcgcagcagctcctcgtccggcacctggctcagctcctccgacgccgccgccgccgtcgccgcgggcttagccatggcggggccgtcaccgcggcatcgccctcgccctcgcccggccggcgcttccccgcgccggggctccgctgggccggtccgcgcgcgggcggggggcggccgggggcgcgtgcggcccgccccgcgccgcctggcgcgtcctctcgccgcgcccgccggggccgcccgggagcccgcgcgcctcggggttgacgagcggaggcggctgctgcgtcggcggccgcggtgccgggcgctctcagggttct

SEQ ID NO: 14558 - RNA, 1686 nt, Homo sapiens
  source 1..1686: mol_type = other RNA
gctgggattacaggcatgagccaccgtgcccagcctcagcctctgttttctaaagtgtaagatactggtaatattgccccatgaactttaaagggtagtggttaaggtatgagggaacataaagtatttggtaaagtataaggcggtaggaaataaattactaaaattattatccttgcaacctagctgacgtgaaaaggggttgtctccataaaggatgcgggccttcaggggcagcattattctgcaggtctcctgcttcctgatggcacaaggactccacatcacccagtcctaccttaaatccaatcggacaccagtccacaaactggttggtgtgcttgctcttgatggtggcgacagccgcactgacatctttcaggaccacatcccctctgtacaacatgcagcaggccatgtacttgccatggtgagggtcacacttgaccatctgattggctggctcgaagcgggcactggcgatcttggccacggacagctgctcatggtaggccttcttggctgagatgaccagggcgtaggtggccagggggaggtggatgtgggggtatggcaccaagttggtttggaattctgtcaagtacacattcagggccccatcgaatcacagggaggccgtgatggaggacacgatctgcccagacgactgaggttggtgtacatgggacactcgatgtccaggttgtgctgacatgtcataggtggctttgctgtcgactatgaaggcacagtcagaatgttccagggtcgtgtaggtggtcaggatggagttgtagggctccgtcatggccatggagacctggggggctgggcaaatggcaaactccagcttggacttcttcccgtagtccaccgagagccgcttcatgagcagagacacgaacccagagccagtgccgcccccaaagctgtggaagatgaggaagccctgcagtcccatgcacagatctgcctgcttggtcattcagctggttgtagctcaggtccagggacttcaggtctgtgtgggccagcaggagttcggcaaggtgctgggccgcctgctcctccaggccattccctgacagctgcatcttccgcatggcctggttcactgtgagggcggcacagagggcctgggctcctgccactcccagctggttctccaacaggtccacatctgtggattgggaaaacccagctctgattgcatttcagggcgggacagcctttggtgcactgtctggcgggattttccattttaacctccttctagaagcgccttctcatggtaaagttcctgatgccgccaggagcgccgaggagagggcagggggctggagacgccccgcagagggctacgtgccctgctggacagaggtctcctgcctcctcggcggcgccagcccacctcccacaacccctgcgggagaagcccccaaggggaggagacgggcctggcccctgccccgagcaccttccgtctctaggtcggagtctgaatcggccttgggaccctgcttggcttcggggacccctgcaagacgtccacaggccgccgtcgcctcttcctcctgctttttatcctccccagacctctggcaggaaccgctcatcgttacgcccctttcgcagcctcagaccctgaggcggagaccgcttggcgcctcacttagagcgcgaccc

SEQ ID NO: 14559 - RNA, 1670 nt, Homo sapiens
  source 1..1670: mol_type = other RNA
gctgggattacaggcatgagccaccgtgcccagcctcctgaccttgttttaactaagcctctcactccctctgatcccatctgtgttctgtctgtttggatatcttgccacttttctctggacatgcttcagtttctccacattcatctgaagtttggggatcaagacaaaataaaatactctaatgagaatctgattgatttaaaatatattcaccctccaactgttatctgttacattttttaactttttattttcttattacttcatagtggcagtatgttgttgactcagtcaccatatcagtaatagtgactctatctctccaatgtccttggacttagcaaaatttactcgttctccatttatgcgtggtcccatggccatgaatggccttgactgggttcctgttaagtctccttatgctagtctcttttcagtcttgaaagtcttagccctgcctctgaagaattaatgtggatcctttcacagctttcacctaggtcatgaggtttaaattgttggagaggcccactgtgatatgattgtaagagtcaccatgccatttttacaaccttgagttataagtttcttgtaggtgcttcactagcctcatgatatgccttgccagaagtagcgcctgagatggagatttgggtgcaggtgatttattgacgatgtgttcttcaggaaaaatactttctattcacatttttagatggcaggatggtggctggcaaagtgttgatggcaaagcaagaaattgttgaatgtgtagcctcagcagctatgatatcgccgggaaaacttcctggagaaacacattcccaacggatagctgaagaagctttgggaggtctggacaacttaattcctcgaaatgaaggttcctgagggagtccctgtgatttttcttctgagatgccctcttttgttgctgtttcactgttctcacaatcacttttaggggaaaggcatggtttccaggatttcagctgtgtctttaagggctggaggtggatgtctgttgactcttgggatgctctgagacatgttaaatccttccatggcactgctggtccctgtggactagctgggacctgctgccctgggtcatcaaactccctctctaaatcctccaacagggtcacagcttcctcgccgctttctggattatgttgctgaacccagatctgcagctcctcaggcagaatgctcaggaactgctccagtaccagcagttctaagatctgctcctttgtgtgcaactctggcattagccactgatagcaaagttcctggagtcggctcagagcctcccggggcccaggtgtctcctggtagcaaaattttctgaattgctgacgaaacaattcttggcaggattgagtactcccattctgcttaaatttctcatcccaggaaaagttatcttctactttcactagtattagttcttgttccggaggatcctgaggtatcagggttgaaatcactccagattccacagccattcttggctgaaacagcttagcaaaaagctcagtacaactggttctgtgcttgcgaaggagtgtgagtaatctcttctttccgcgaagcccaggagcggccaggaaatgagccacccaccccgagctgcaagccacaaagaccggaagtgcgcgtac

SEQ ID NO: 14560 - RNA, 4429 nt, Homo sapiens
  source 1..4429: mol_type = other RNA
gctgggattacaggcatgagccaccgtgcccagcctgaaaaaaatcttttactagaaacagttccaatgttaacttttcccacatggaaagcaaaacaaaacaaaacaaaacaaacaaacaaatgcaacaaaacaacctcccactattattgtgcataaaaacacattaaatgactctaaaacaaaataaacttttttttttttggtagagacagggtcttgctatgttgcccaggctagtctcaaactcctgggctcaagcagttcttgcctcagcctcccaaattgctgggattacaggcatgagccaccatgactggcctaaaacaaaataaattcttaatggcatttgtggaatgtgtttaagagccaaaactgtgaaaatgtaagctttatctttcttttttcctagattatttaaagaggattgtagccacacttcagatgaatgtttacaagccaaataatgatttaagagtgtgctcaataaaaaggccataggtttaagaattaaatggaataatataaattactaggtcaacaagaatatttcatgtatagtacactgtctaaggaatgcagagaaattttacaagaaacccaagactaaatacttcattaagaacactggttactaagtaaatagatggctcatgtaggaaaaagctaatatatgtagatgtaatgtcaactaagtgcatgtgacagaaatgaagaactaggaataagaatccagattttctggccaggcacggtggctcacatctgtaatcctagcactttgggaggccatagtgggtggatcacctgaggtcaggagtttgagaccagcctggcctacatggcgaaaccccatctctactaaagatacaaaaattagctgggcgtggtggtgggcacttataatcccagctactcaggaggctgaggaaggagaatcgctcgaacctgggggtggatgttgcagtgagccaaggtcgcgccacttcactccagcttgggcgaaagagcaaaactccatctcaaaacaacaaccaaaaagaatccagatttttaggtgtctaatactagacattctgtatccaagtttcagccatttcatccaataaagccttctaaagccttttttttttgagacagggtctcactctgtcactcaagctggagtgcagtggcgtgatcttggcttactgcaacctgtctcccaggctcaagcgattctcctgcctcagcctcccgagtagctaagactacaggccgtgtcaccaaacccggctaattttttgtaggcacggggtttcaccgtcttggccaggctggtctcaacctcctgacctcaagtgatccacctgccccagcctcccaaagtgctgggattacaggcatgagtcactgcgcccagctcccaaagccaattttcaattatttgtgagccatagattcagtgactacatcaatatctcttgccagggattggcctaacagctcagagaacagattgttaggatatatgggcaagccttctaagttcaagaggcaagagcagaaaatggaatgctatagggatttagctccatcttaagccattctggccctttctgctctactttaccagctatagagttaggaaggcttccagtaggccacagcaagaggaaaaacctttattctgtggggctcatttatccaggatttaacttacctgtgtcatgttaccgatctattaacacaagtaatttagagttggttatattatttcaagaaattgagcacaaagccaggatgtacaaggaggaattcaaacaatcaatattggattatataatgaaaagatgcccttacaatgtttatgatctagaatgtaatcataataaaggggggaaaataccttatgagtatcacaattgtatcagagactattaaacagtacaatgatacagagaatttattcaattcatacaagtaatttaccagatctaaacagtgaatagactgacctaaggggaaaaaaatccttacattgatagcaaaatatcttctagcccccataaataatctgcaatcatttgctaggaaaaaaacttcataaccatatgggtcatgcagacatttttatttatttatttattttgagacagagtctcgctctgtcgccctgattggagtgcagtggcacgatctcagcttactgcaacctccgtctcccaggttcaagcaatttcctgcctcagcttccccagtagctgggattataggcacacaccaccatgcctggctaatttttgcatttttagtagagataaggtttcaccatgttggtcaggctggtctcgaactcctgacctcaggtgattcgcctgcctcggcctcccaaagtgctgggattacaggcgtgagccaccgtgcccagcccatgcagacatttttaagtgctattggtattcactttatttcaaactgagcaaaacaatacaaccttttacttttttatacattttaaaatttctctcatattaacattccttcctaccccaatccatcccatcaccaaacaggaatgagataaggagtgaaaaaaagatgtatgtttctcattttccttcttttcccttgaagtaaaccagtaatttattaaaatattttataggtcagaggataacaaaagactcaatgtagtaaataagtaaataggcattcaaatatcagtaacctaacaggccctaatacagctttaagattttcttctttttttttttttgagagggagtctcgctctattgcttaggctggaatgcagtggtgcgatcttggttcactgcaacctccacctcccgggttcaagcaattctcctgctttggcctcctgagtagctgggattacaggcacatgcaccaaccctggctaatttttctgtatttttagtagagacagggtttcaccatgttggccaggctggtctcgaactcctgacctcaagtgatccacccacctcagcctcccaaagtgctgggattacaggtgtgagccactgcactggcctaagattttcattttaacagggaactgttagaacagaaaagaagcttcccaagaggcactcattttaaaaataaattatagcttaaattattactatgtggattatatcagcaaaggcagaaagaattaatgttttcctcctttcatgaaccttgtaaggctagtgttgagtggcttacaaatgtcatataatggactgtaaatcatctgccatattgatcaatcatgtttatttaaggttttcttaacattagagatttttaatgggagtataaaattagtaaacaaccatttcattttttctctcttcctattctagccacataagccagtttaatccatgacacagatttcagctgtaatttgcaaaacaatccaagagctaccacagtccccaaaactacagaaaactgccatccacaaataaactaccaaggtaaatgtaaatacagcgtggttctaattttctttcacacaatcccagacaaccccaaataactttataaataccttatgaaaaaaagcaatttaaaaacctatcaaatctatttaaaatatataaatgcagacctctcaaatttccttcaatcaggccagaaattatcacaaaaattataatcacagttacaaacagaatgagtggaatgtttgtaagtttaggacaaccaaaaaagccccatgtaactttttaaaaatataatcattcactcaaatatactgtaaataggaatggcagtaacacaggaagcaaaaataaacttgcaagtgaaatttctagaagctcatgaaaacaataccatcccatattgcagatacaaaaggaaaaacagttctaatggggttaagagtactctggtcatcttcgttcgtttggtcgtgcaaggtgttaactattttcacttcccatatcacaaagttagtccacaggaggagctggtggatcttgtccattatgaggactggttggctttccaggtaggctggatcctcttagattaggaggtctcagtaagaacaagatcaatgcaataaccatccaggctaccaagatcattgtaacactgatgccattatcaccagagggtcccggtaattcctgaagacactctgtgtctgtgcagtaggactgggactgccgtaacagattgatcagtcttctcattgcatgttcatgagagcaaacacattcacagggatcaaatccaccttctgccatgattacccagcttgattttacttgactgtttaaataaacagaaatttacttctcacggttctggaggctaggaagtccaagatcaaggcactggtagattcagtgtctgctgaggacccactctctggttggtagatggtgccttctcactgtgtcctactatggtggaagag

SEQ ID NO: 14561 - RNA, 4418 nt, Homo sapiens
  source 1..4418: mol_type = other RNA
gctgggattacaggcatgagccaccgtgcccagcctgaaaaaaatcttttactagaaacagttccaatgttaacttttcccacatggaaagcaaaacaaaacaaaacaaaacaaacaaacaaatgcaacaaaacaacctcccactattattgtgcataaaaacacattaaatgactctaaaacaaaataaacttttttttttttggtagagacagggtcttgctatgttgcccaggctagtctcaaactcctgggctcaagcagttcttgcctcagcctcccaaattgctgggattacaggcatgagccaccatgactggcctaaaacaaaataaattcttaatggcatttgtggaatgtgtttaagagccaaaactgtgaaaatgtaagctttatctttcttttttcctagattatttaaagaggattgtagccacacttcagatgaatgtttacaagccaaataatgatttaagagtgtgctcaataaaaaggccataggtttaagaattaaatggaataatataaattactaggtcaacaagaatatttcatgtatagtacactgtctaaggaatgcagagaaattttacaagaaacccaagactaaatacttcattaagaacactggttactaagtaaatagatggctcatgtaggaaaaagctaatatatgtagatgtaatgtcaactaagtgcatgtgacagaaatgaagaactaggaataagaatccagattttctggccaggcacggtggctcacatctgtaatcctagcactttgggaggccatagtgggtggatcacctgaggtcaggagtttgagaccagcctggcctacatggcgaaaccccatctctactaaagatacaaaaattagctgggcgtggtggtgggcacttataatcccagctactcaggaggctgaggaaggagaatcgctcgaacctgggggtggatgttgcagtgagccaaggtcgcgccacttcactccagcttgggcgaaagagcaaaactccatctcaaaacaacaaccaaaaagaatccagatttttaggtgtctaatactagacattctgtatccaagtttcagccatttcatccaataaagccttctaaagccttttttttttgagacagggtctcactctgtcactcaagctggagtgcagtggcgtgatcttggcttactgcaacctgtctcccaggctcaagcgattctcctgcctcagcctcccgagtagctaagactacaggccgtgtcaccaaacccggctaattttttgtaggcacggggtttcaccgtcttggccaggctggtctcaacctcctgacctcaagtgatccacctgccccagcctcccaaagtgctgggattacaggcatgagtcactgcgcccagctcccaaagccaattttcaattatttgtgagccatagattcagtgactacatcaatatctcttgccagggattggcctaacagctcagagaacagattgttaggatatatgggcaagccttctaagttcaagaggcaagagcagaaaatggaatgctatagggatttagctccatcttaagccattctggccctttctgctctactttaccagctatagagttaggaaggcttccagtaggccacagcaagaggaaaaacctttattctgtggggctcatttatccaggatttaacttacctgtgtcatgttaccgatctattaacacaagtaatttagagttggttatattatttcaagaaattgagcacaaagccaggatgtacaaggaggaattcaaacaatcaatattggattatataatgaaaagatgcccttacaatgtttatgatctagaatgtaatcataataaaggggggaaaataccttatgagtatcacaattgtatcagagactattaaacagtacaatgatacagagaatttattcaattcatacaagtaatttaccagatctaaacagtgaatagactgacctaaggggaaaaaaatccttacattgatagcaaaatatcttctagcccccataaataatctgcaatcatttgctaggaaaaaaacttcataaccatatgggtcatgcagacatttttatttatttatttattttgagacagagtctcgctctgtcgccctgattggagtgcagtggcacgatctcagcttactgcaacctccgtctcccaggttcaagcaatttcctgcctcagcttccccagtagctgggattataggcacacaccaccatgcctggctaatttttgcatttttagtagagataaggtttcaccatgttggtcaggctggtctcgaactcctgacctcaggtgattcgcctgcctcggcctcccaaagtgctgggattacaggcgtgagccaccgtgcccagcccatgcagacatttttaagtgctattggtattcactttatttcaaactgagcaaaacaatacaaccttttacttttttatacattttaaaatttctctcatattaacattccttcctaccccaatccatcccatcaccaaacaggaatgagataaggagtgaaaaaaagatgtatgtttctcattttccttcttttcccttgaagtaaaccagtaatttattaaaatattttataggtcagaggataacaaaagactcaatgtagtaaataagtaaataggcattcaaatatcagtaacctaacaggccctaatacagctttaagattttcttctttttttttttttgagagggagtctcgctctattgcttaggctggaatgcagtggtgcgatcttggttcactgcaacctccacctcccgggttcaagcaattctcctgctttggcctcctgagtagctgggattacaggcacatgcaccaaccctggctaatttttctgtatttttagtagagacagggtttcaccatgttggccaggctggtctcgaactcctgacctcaagtgatccacccacctcagcctcccaaagtgctgggattacaggtgtgagccactgcactggcctaagattttcattttaacagggaactgttagaacagaaaagaagcttcccaagaggcactcattttaaaaataaattatagcttaaattattactatgtggattatatcagcaaaggcagaaagaattaatgttttcctcctttcatgaaccttgtaaggctagtgttgagtggcttacaaatgtcatataatggactgtaaatcatctgccatattgatcaatcatgtttatttaaggttttcttaacattagagatttttaatgggagtataaaattagtaaacaaccatttcattttttctctcttcctattctagccacataagccagtttaatccatgacacagatttcagctgtaatttgcaaaacaatccaagagctaccacagtccccaaaactacagaaaactgccatccacaaataaactaccaaggtaaatgtaaatacagcgtggttctaattttctttcacacaatcccagacaaccccaaataactttataaataccttatgaaaaaaagcaatttaaaaacctatcaaatctatttaaaatatataaatgcagacctctcaaatttccttcaatcaggccagaaattatcacaaaaattataatcacagttacaaacagaatgagtggaatgtttgtaagtttaggacaaccaaaaaagccccatgtaactttttaaaaatataatcattcactcaaatatactgtaaataggaatggcagtaacacaggaagcaaaaataaacttgcaagtgaaatttctagaagctcatgaaaacaataccatcccatattgcagatacaaaaggaaaaacagttctaatggggttaagagtactctggtcatcttcgttcgtttggtcgtgcaaggtgttaactattttcacttcccatatcacaaagttagtccacaggaggagctggtggatcttgtccattatgaggactggttggctttccaggtaggctggatcctcttagattaggaggtctcagtaagaacaagatcaatgcaataaccatccaggctaccaagatcattgtaacactgatgccattatcaccagagggtcccggtaattcctgaagacactctgtgtctgtgcagtaggactgggactgccgtaacagattgatcagtcttctcattgcatgttcatgagagcaaacacattcacagggatcaaatccaccttctgccatgattacccagcttgattttacttgactgtttaaatccgcccagacaacaaccgatggggcggggaggatgggggccgggaccgaggctcggcagaaagaccgcctggagcttccagaaggctgcggctgctccggacgctgctgccactgccgtttctggcc

SEQ ID NO: 14562 - RNA, 4563 nt, Homo sapiens
  source 1..4563: mol_type = other RNA
gctgggattacaggcatgagccaccgtgcccagcctgaaaaaaatcttttactagaaacagttccaatgttaacttttcccacatggaaagcaaaacaaaacaaaacaaaacaaacaaacaaatgcaacaaaacaacctcccactattattgtgcataaaaacacattaaatgactctaaaacaaaataaacttttttttttttggtagagacagggtcttgctatgttgcccaggctagtctcaaactcctgggctcaagcagttcttgcctcagcctcccaaattgctgggattacaggcatgagccaccatgactggcctaaaacaaaataaattcttaatggcatttgtggaatgtgtttaagagccaaaactgtgaaaatgtaagctttatctttcttttttcctagattatttaaagaggattgtagccacacttcagatgaatgtttacaagccaaataatgatttaagagtgtgctcaataaaaaggccataggtttaagaattaaatggaataatataaattactaggtcaacaagaatatttcatgtatagtacactgtctaaggaatgcagagaaattttacaagaaacccaagactaaatacttcattaagaacactggttactaagtaaatagatggctcatgtaggaaaaagctaatatatgtagatgtaatgtcaactaagtgcatgtgacagaaatgaagaactaggaataagaatccagattttctggccaggcacggtggctcacatctgtaatcctagcactttgggaggccatagtgggtggatcacctgaggtcaggagtttgagaccagcctggcctacatggcgaaaccccatctctactaaagatacaaaaattagctgggcgtggtggtgggcacttataatcccagctactcaggaggctgaggaaggagaatcgctcgaacctgggggtggatgttgcagtgagccaaggtcgcgccacttcactccagcttgggcgaaagagcaaaactccatctcaaaacaacaaccaaaaagaatccagatttttaggtgtctaatactagacattctgtatccaagtttcagccatttcatccaataaagccttctaaagccttttttttttgagacagggtctcactctgtcactcaagctggagtgcagtggcgtgatcttggcttactgcaacctgtctcccaggctcaagcgattctcctgcctcagcctcccgagtagctaagactacaggccgtgtcaccaaacccggctaattttttgtaggcacggggtttcaccgtcttggccaggctggtctcaacctcctgacctcaagtgatccacctgccccagcctcccaaagtgctgggattacaggcatgagtcactgcgcccagctcccaaagccaattttcaattatttgtgagccatagattcagtgactacatcaatatctcttgccagggattggcctaacagctcagagaacagattgttaggatatatgggcaagccttctaagttcaagaggcaagagcagaaaatggaatgctatagggatttagctccatcttaagccattctggccctttctgctctactttaccagctatagagttaggaaggcttccagtaggccacagcaagaggaaaaacctttattctgtggggctcatttatccaggatttaacttacctgtgtcatgttaccgatctattaacacaagtaatttagagttggttatattatttcaagaaattgagcacaaagccaggatgtacaaggaggaattcaaacaatcaatattggattatataatgaaaagatgcccttacaatgtttatgatctagaatgtaatcataataaaggggggaaaataccttatgagtatcacaattgtatcagagactattaaacagtacaatgatacagagaatttattcaattcatacaagtaatttaccagatctaaacagtgaatagactgacctaaggggaaaaaaatccttacattgatagcaaaatatcttctagcccccataaataatctgcaatcatttgctaggaaaaaaacttcataaccatatgggtcatgcagacatttttatttatttatttattttgagacagagtctcgctctgtcgccctgattggagtgcagtggcacgatctcagcttactgcaacctccgtctcccaggttcaagcaatttcctgcctcagcttccccagtagctgggattataggcacacaccaccatgcctggctaatttttgcatttttagtagagataaggtttcaccatgttggtcaggctggtctcgaactcctgacctcaggtgattcgcctgcctcggcctcccaaagtgctgggattacaggcgtgagccaccgtgcccagcccatgcagacatttttaagtgctattggtattcactttatttcaaactgagcaaaacaatacaaccttttacttttttatacattttaaaatttctctcatattaacattccttcctaccccaatccatcccatcaccaaacaggaatgagataaggagtgaaaaaaagatgtatgtttctcattttccttcttttcccttgaagtaaaccagtaatttattaaaatattttataggtcagaggataacaaaagactcaatgtagtaaataagtaaataggcattcaaatatcagtaacctaacaggccctaatacagctttaagattttcttctttttttttttttgagagggagtctcgctctattgcttaggctggaatgcagtggtgcgatcttggttcactgcaacctccacctcccgggttcaagcaattctcctgctttggcctcctgagtagctgggattacaggcacatgcaccaaccctggctaatttttctgtatttttagtagagacagggtttcaccatgttggccaggctggtctcgaactcctgacctcaagtgatccacccacctcagcctcccaaagtgctgggattacaggtgtgagccactgcactggcctaagattttcattttaacagggaactgttagaacagaaaagaagcttcccaagaggcactcattttaaaaataaattatagcttaaattattactatgtggattatatcagcaaaggcagaaagaattaatgttttcctcctttcatgaaccttgtaaggctagtgttgagtggcttacaaatgtcatataatggactgtaaatcatctgccatattgatcaatcatgtttatttaaggttttcttaacattagagatttttaatgggagtataaaattagtaaacaaccatttcattttttctctcttcctattctagccacataagccagtttaatccatgacacagatttcagctgtaatttgcaaaacaatccaagagctaccacagtccccaaaactacagaaaactgccatccacaaataaactaccaaggtaaatgtaaatacagcgtggttctaattttctttcacacaatcccagacaaccccaaataactttataaataccttatgaaaaaaagcaatttaaaaacctatcaaatctatttaaaatatataaatgcagacctctcaaatttccttcaatcaggccagaaattatcacaaaaattataatcacagttacaaacagaatgagtggaatgtttgtaagtttaggacaaccaaaaaagccccatgtaactttttaaaaatataatcattcactcaaatatactgtaaataggaatggcagtaacacaggaagcaaaaataaacttgcaagtgaaatttctagaagctcatgaaaacaataccatcccatattgcagatacaaaaggaaaaacagttctaatggggttaagagtactctggtcatcttcgttcgtttggtcgtgcaaggtgttaactattttcacttcccatatcacaaagttagtccacaggaggagctggtggatcttgtccattatgaggactggttggctttccaggtaggctggatcctcttagattaggaggtctcagtaagaacaagatcaatgcaataaccatccaggctaccaagatcattgtaacactgatgccattatcaccagagggtcccggtaattcctgaagacactctgtgtctgtgcagtaggactgggactgccgtaacagattgatcagtcttctcattgcatgttcatgagagcaaacacattcacagggatcaaatccaccttctgccatgattacccagcttgattttacttgactgtttaaatctgagctaaggggagaaggggaggtgagaattggaaagggagatggagatgcggcctgagctggagaggctcactttccagaaggtaagcaacaccatatgcaaactctacttcacagttttgtctgaggccactctgtcaacacccgcccagacaacaaccgatggggcggggaggatgggggccgggaccgaggctcggcagaaagaccgcctggagcttccagaaggctgcggctgctccggacgctgctgccactgccgtttctggcc

SEQ ID NO: 14563 - RNA, 3685 nt, Homo sapiens
  source 1..3685: mol_type = other RNA
gctgggattacaggcatgagccaccgtgcccagcctggattcttctttttagattcatttgttggagctacaaatgaaatcatcaaaagagagagggatgctaatagaagagtctacagtgatttaccaattttgctagtagataaggtttcacaccctaaaaactacaaatatagataaccactacaaagttcttcgtaacatagaacaatctaaaaaccacaactcaatctttagagctgagaataaatcatgtgaaacctgtaacattttatttgttaaaaatgaacagcttcagaatagatctaaatgtaacttttccaaaaaacaccaaaaagtacagtgtaaagcacctcctcgttaaatacaaactttcatttggtgatgcacggcaccaatgttttgcatataccttgatgcaaagaaaagtttaagttgcatcctgtttttaaaaaaaaccgaaacttaagaactgaacaaggattacaaccacattccaataaagaaaattttccttcaacaaagcatattgttttgtttatatacaatatgtgaccaccaagagttttaatttagttgtaccaaaggcaaaacattatacttaaaattaaattacagatgcatgaagaataaaagtttaatgtatcaaagataatttgttatttaatgcactcaatgtcagtatttggggcaatttttaaagttttcccaaaaaatggcatgaatagctctatacaataataggtaagaacaggaaaatgaaaacacctttataccatattttcacaaaccattctaaagacagcaaacttgagctcagctgcttttccttgctttaaaataagctaccagtaattctaaatcagactaaaatgtactgttcctagaccaaatacaggcattcatccttgcaaaaatgttttgcaatgagttcttggcctatatgaaaagcatcaaatagctaaggagagactagaatttatttccaaattctgtgactgacttccaataatcccttatcagtacgagtaccaggaaaatatcagatattaaagatcagatttaattctttggtataagcatgaaactgttactgatagctttccatggcgagcataaaccatgaagcaactcaagaagcatgagagacaacaatgaaatctagtatacaatgcagggcaggccaagaacgatgtctgctttacaggaaaagtcaacactaacaatctactcctgagaaactaacacctatttagatgtttttaacataatggcaaactaaaatgtcaagcttcaaaatgaccaaacttgtaacgtacagctggaagattttgctgcatttggcattatactgtaatttacagtatacaacatctggggactcagtactatcttagcacagactaacttctcccactccgtcagaggtggcaggtggcgggtcggtggggagggccttttctccccataaatgcctgaactttaatttataccatataagaaatcagtgaaaggtaaacaacaaggttaatgtaactctattataaattttgcattttttttctctgtgacatatacaagtatatttttgtttttggagctataaattatttaatttagcaatcttcaaagctcataaatttcaacttttcaaataagaaattttaacttcaaataagaagtctaggactttatggctattaattttactatcaaaatatccaagggactccattcaatgtaatagttataattcttctaaatatcatttgaataattctttgtggacgctagactcaagactatgctacatccaaacagtacatctataaccagggttttgaagtgtttcatctcaactacctgtccttcaacttgctacttacttcctctcatgccttcatttattaaacacaaactgtcattttttaaaactggaccttctcctccaaggccctatcagataactttgtgaatatgcatttacagtctctaaacaccaacattttaaactaagactaatacctagggccacatttcctgttaaaagctcagcactaaagctgtgtaattccaggggactttacaccgtctgaaagaggaagcacgttctggatgtccccctaagtcttcaaacccacagctggaaattctaatacattgttctgtgtctctaatgaagaaaaggcaacggcactgactacatcaacactattaaagggcaagtgacagcaaccaagggacctactcatgtttatgaagaccaggatttaccatgacaaagtctaaaacacgggcaaaggtgatgagatcctgaatactgctatcataaaaataatcaatttctatctttctgtcttccttctgctgcatgaggaaccaaagaagtcaaacagatgattgttctgtctgagccaaccatgaaatctttaagaacagacaggtataatccctattattctttcagggcattattttatacgtttttttttttaaaaaaaaaaaccttcaaaaataaaaataagagttatttagccttgtgaatattttgaagtaaagtttcttgaatttccgtgatgaactcttcaagcaattcaacttctcagagtcatcactcaaaagttcctttgacatgggacctatcccacggtgacaaagcggcttccccctttgttgtatgtgagagtggctctttgttccttcaggatcccaaaccgctcattcaacgtcatccctgtctgttttccgacactgtttatgtcaaactgcaggggaacacctttaggaactttcttgacgtcactttgctcccgctttgttaaaaatgaaggtacagcagtacgagttaatcgtggtttctgagttactgggcattgcactgctccaggattgtcaatagatacagtcaaaatccctccatttgtggtggaagtccgccattgacgagttctctttgctactacatcgtctagcagttgttctgtattcaactgggcctgcaccttcaggcctcttctgaaaagaaaagttgcctgacgagtatctttctgatgatttaatttatttccactcctggtaaaattagctggaatgttattttttctgcttagctggctaggtctcttgagaactgctactggtttcctctgcccttcattttgtctcagaaggtttgccttcctttttaacactggaaaatattgttctatattcttgtcacttagaggtggacgattcataggactaattccttttcgaattccagtcgttttcctagctgcaaggccagtgataactccattaggacgtctctttccaggcattactcttcctctacgattcagactagtcttaccaaaaccagaattctgttggattccccatcgcactctcatcctgaattgctgggcaccactttgctggaggagtcttctatttagtcttggaaaattctgcttcttcccttcctttcgattcaacttgatgatatcatccaaagacatatctattttgtcgaggttttcattgctgcgggccttcggcggcggcgaagaagtcgccgtggctcccaccaaccgggtaccaaaccggttcatggctggagacgtcgcgccgagagcgggcgcggacaaggccggagtcgcaggcctgccacctcccactcgcgcacgcagcccgccgcacc

SEQ ID NO: 14564 - RNA, 4069 nt, Homo sapiens
  source 1..4069: mol_type = other RNA
gctgggattacaggcatgagccaccgtgcccagcctggattcttctttttagattcatttgttggagctacaaatgaaatcatcaaaagagagagggatgctaatagaagagtctacagtgatttaccaattttgctagtagataaggtttcacaccctaaaaactacaaatatagataaccactacaaagttcttcgtaacatagaacaatctaaaaaccacaactcaatctttagagctgagaataaatcatgtgaaacctgtaacattttatttgttaaaaatgaacagcttcagaatagatctaaatgtaacttttccaaaaaacaccaaaaagtacagtgtaaagcacctcctcgttaaatacaaactttcatttggtgatgcacggcaccaatgttttgcatataccttgatgcaaagaaaagtttaagttgcatcctgtttttaaaaaaaaccgaaacttaagaactgaacaaggattacaaccacattccaataaagaaaattttccttcaacaaagcatattgttttgtttatatacaatatgtgaccaccaagagttttaatttagttgtaccaaaggcaaaacattatacttaaaattaaattacagatgcatgaagaataaaagtttaatgtatcaaagataatttgttatttaatgcactcaatgtcagtatttggggcaatttttaaagttttcccaaaaaatggcatgaatagctctatacaataataggtaagaacaggaaaatgaaaacacctttataccatattttcacaaaccattctaaagacagcaaacttgagctcagctgcttttccttgctttaaaataagctaccagtaattctaaatcagactaaaatgtactgttcctagaccaaatacaggcattcatccttgcaaaaatgttttgcaatgagttcttggcctatatgaaaagcatcaaatagctaaggagagactagaatttatttccaaattctgtgactgacttccaataatcccttatcagtacgagtaccaggaaaatatcagatattaaagatcagatttaattctttggtataagcatgaaactgttactgatagctttccatggcgagcataaaccatgaagcaactcaagaagcatgagagacaacaatgaaatctagtatacaatgcagggcaggccaagaacgatgtctgctttacaggaaaagtcaacactaacaatctactcctgagaaactaacacctatttagatgtttttaacataatggcaaactaaaatgtcaagcttcaaaatgaccaaacttgtaacgtacagctggaagattttgctgcatttggcattatactgtaatttacagtatacaacatctggggactcagtactatcttagcacagactaacttctcccactccgtcagaggtggcaggtggcgggtcggtggggagggccttttctccccataaatgcctgaactttaatttataccatataagaaatcagtgaaaggtaaacaacaaggttaatgtaactctattataaattttgcattttttttctctgtgacatatacaagtatatttttgtttttggagctataaattatttaatttagcaatcttcaaagctcataaatttcaacttttcaaataagaaattttaacttcaaataagaagtctaggactttatggctattaattttactatcaaaatatccaagggactccattcaatgtaatagttataattcttctaaatatcatttgaataattctttgtggacgctagactcaagactatgctacatccaaacagtacatctataaccagggttttgaagtgtttcatctcaactacctgtccttcaacttgctacttacttcctctcatgccttcatttattaaacacaaactgtcattttttaaaactggaccttctcctccaaggccctatcagataactttgtgaatatgcatttacagtctctaaacaccaacattttaaactaagactaatacctagggccacatttcctgttaaaagctcagcactaaagctgtgtaattccaggggactttacaccgtctgaaagaggaagcacgttctggatgtccccctaagtcttcaaacccacagctggaaattctaatacattgttctgtgtctctaatgaagaaaaggcaacggcactgactacatcaacactattaaagggcaagtgacagcaaccaagggacctactcatgtttatgaagaccaggatttaccatgacaaagtctaaaacacgggcaaaggtgatgagatcctgaatactgctatcataaaaataatcaatttctatctttctgtcttccttctgctgcatgaggaaccaaagaagtcaaacagatgattgttctgtctgagccaaccatgaaatctttaagaacagacaggtataatccctattattctttcagggcattattttatacgtttttttttttaaaaaaaaaaaccttcaaaaataaaaataagagttatttagccttgtgaatattttgaagtaaagtttcttgaatttccgtgatgaactcttcaagcaattcaacttctcagagtcatcactcaaaagttcctttgacatgggacctatcccacggtgacaaagcggcttccccctttgttgtatgtgagagtggctctttgttccttcaggatcccaaaccgctcattcaacgtcatccctgtctgttttccgacactgtttatgtcaaactgcaggggaacacctttaggaactttcttgacgtcactttgctcccgctttgttaaaaatgaaggtacagcagtacgagttaatcgtggtttctgagttactgggcattgcactgctccaggattgtcaatagatacagtcaaaatccctccatttgtggtggaagtccgccattgacgagttctctttgctactacatcgtctagcagttgttctgtattcaactgggcctgcaccttcaggcctcttctgaaaagaaaagttgcctgacgagtatctttctgatgatttaatttatttccactcctggtaaaattagctggaatgttattttttctgcttagctggctaggtctcttgagaactgctactggtttcctctgcccttcattttgtctcagaaggtttgccttcctttttaacactggaaaatattgttctatattcttgtcacttagaggtggacgattcataggactaattccttttcgaattccagtcgttttcctagctgcaaggccagtgataactccattaggacgtctctttccaggcattactcttcctctacgattcagactagtcttaccaaaaccagaattctgttggattccccatcgcactctcatcctgaattgctgggcaccactttgctggaggagtcttctatttagtcttggaaaattctgcttcttcccttcctttcgattcaacttgatgatatcatctggcttctcagcgagccacagcaatcatctctccttcaaagatgtttgctttctcccccattagctagctctgaggcctggagagggagactgtgcttttctaggcagcgctcaatacacaaccacatcccacaggcggccgagcgctgcttcctttctgacagacgctccggggccgcggccggaggtggccccgagagtcgcgcccggcagccatggccggcgccggcctggaacgcccggcgaccagggaaagctccggaagcgctggtttaaccgaccgcagccccggccgggctctccaagacctttcttcagagagaacggctcggtcggaccattcccctcgctccccgataacgcccaccgcgaacgcgctccggggaaaccggcagatctttcctcacaaagagccggcgagcggcgagccgtagcccctccggggagaagagacgccccccgcgaccctgcgaaccttcgggcccgcagcgcccctgcccccgcctccacagcccctcctccgactgccgcggccgaggggacgcccgggtccctcgcggtccagccgggcacct

SEQ ID NO: 14565 - RNA, 3776 nt, Homo sapiens
  source 1..3776: mol_type = other RNA
gctgggattacaggcatgagccaccgtgcccagcctggattcttctttttagattcatttgttggagctacaaatgaaatcatcaaaagagagagggatgctaatagaagagtctacagtgatttaccaattttgctagtagataaggtttcacaccctaaaaactacaaatatagataaccactacaaagttcttcgtaacatagaacaatctaaaaaccacaactcaatctttagagctgagaataaatcatgtgaaacctgtaacattttatttgttaaaaatgaacagcttcagaatagatctaaatgtaacttttccaaaaaacaccaaaaagtacagtgtaaagcacctcctcgttaaatacaaactttcatttggtgatgcacggcaccaatgttttgcatataccttgatgcaaagaaaagtttaagttgcatcctgtttttaaaaaaaaccgaaacttaagaactgaacaaggattacaaccacattccaataaagaaaattttccttcaacaaagcatattgttttgtttatatacaatatgtgaccaccaagagttttaatttagttgtaccaaaggcaaaacattatacttaaaattaaattacagatgcatgaagaataaaagtttaatgtatcaaagataatttgttatttaatgcactcaatgtcagtatttggggcaatttttaaagttttcccaaaaaatggcatgaatagctctatacaataataggtaagaacaggaaaatgaaaacacctttataccatattttcacaaaccattctaaagacagcaaacttgagctcagctgcttttccttgctttaaaataagctaccagtaattctaaatcagactaaaatgtactgttcctagaccaaatacaggcattcatccttgcaaaaatgttttgcaatgagttcttggcctatatgaaaagcatcaaatagctaaggagagactagaatttatttccaaattctgtgactgacttccaataatcccttatcagtacgagtaccaggaaaatatcagatattaaagatcagatttaattctttggtataagcatgaaactgttactgatagctttccatggcgagcataaaccatgaagcaactcaagaagcatgagagacaacaatgaaatctagtatacaatgcagggcaggccaagaacgatgtctgctttacaggaaaagtcaacactaacaatctactcctgagaaactaacacctatttagatgtttttaacataatggcaaactaaaatgtcaagcttcaaaatgaccaaacttgtaacgtacagctggaagattttgctgcatttggcattatactgtaatttacagtatacaacatctggggactcagtactatcttagcacagactaacttctcccactccgtcagaggtggcaggtggcgggtcggtggggagggccttttctccccataaatgcctgaactttaatttataccatataagaaatcagtgaaaggtaaacaacaaggttaatgtaactctattataaattttgcattttttttctctgtgacatatacaagtatatttttgtttttggagctataaattatttaatttagcaatcttcaaagctcataaatttcaacttttcaaataagaaattttaacttcaaataagaagtctaggactttatggctattaattttactatcaaaatatccaagggactccattcaatgtaatagttataattcttctaaatatcatttgaataattctttgtggacgctagactcaagactatgctacatccaaacagtacatctataaccagggttttgaagtgtttcatctcaactacctgtccttcaacttgctacttacttcctctcatgccttcatttattaaacacaaactgtcattttttaaaactggaccttctcctccaaggccctatcagataactttgtgaatatgcatttacagtctctaaacaccaacattttaaactaagactaatacctagggccacatttcctgttaaaagctcagcactaaagctgtgtaattccaggggactttacaccgtctgaaagaggaagcacgttctggatgtccccctaagtcttcaaacccacagctggaaattctaatacattgttctgtgtctctaatgaagaaaaggcaacggcactgactacatcaacactattaaagggcaagtgacagcaaccaagggacctactcatgtttatgaagaccaggatttaccatgacaaagtctaaaacacgggcaaaggtgatgagatcctgaatactgctatcataaaaataatcaatttctatctttctgtcttccttctgctgcatgaggaaccaaagaagtcaaacagatgattgttctgtctgagccaaccatgaaatctttaagaacagacaggtataatccctattattctttcagggcattattttatacgtttttttttttaaaaaaaaaaaccttcaaaaataaaaataagagttatttagccttgtgaatattttgaagtaaagtttcttgaatttccgtgatgaactcttcaagcaattcaacttctcagagtcatcactcaaaagttcctttgacatgggacctatcccacggtgacaaagcggcttccccctttgttgtatgtgagagtggctctttgttccttcaggatcccaaaccgctcattcaacgtcatccctgtctgttttccgacactgtttatgtcaaactgcaggggaacacctttaggaactttcttgacgtcactttgctcccgctttgttaaaaatgaaggtacagcagtacgagttaatcgtggtttctgagttactgggcattgcactgctccaggattgtcaatagatacagtcaaaatccctccatttgtggtggaagtccgccattgacgagttctctttgctactacatcgtctagcagttgttctgtattcaactgggcctgcaccttcaggcctcttctgaaaagaaaagttgcctgacgagtatctttctgatgatttaatttatttccactcctggtaaaattagctggaatgttattttttctgcttagctggctaggtctcttgagaactgctactggtttcctctgcccttcattttgtctcagaaggtttgccttcctttttaacactggaaaatattgttctatattcttgtcacttagaggtggacgattcataggactaattccttttcgaattccagtcgttttcctagctgcaaggccagtgataactccattaggacgtctctttccaggcattactcttcctctacgattcagactagtcttaccaaaaccagaattctgttggattccccatcgcactctcatcctgaattgctgggcaccactttgctggaggagtcttctatttagtcttggaaaattctgcttcttcccttcctttcgattcaacttgatgatatcatttcccataatcacagaaggctccattttttaaagatgacccccttccggccaggcatggtgactcacacctataatcccagcactttgggaggctgaggtgggcggatcatttgaggtcaggagttcgggactggcctgaccaacatggtgaaatcccgtctctactctgaatcttatgccttcagtgatataatcctccgtgtccttcgagtccctcctgctgcagacaggtcccctatacttcggtacacacgagcctttcgcgcccaccgcaacgcagcc

SEQ ID NO: 14566 - RNA, 639 nt, Homo sapiens
  source 1..639: mol_type = other RNA
gctgggattacaggcatgagccaccgtgcccagcctgttaactcaactttttataggatatgataaaagacctaattctaaattcaccaaatttatgcttctctatcaatgaaaacttatggccacagaacacattttttttttttttttttttggaaagcactgtctccttggctctagtctaaaggaacgtaagcaatatgaaggaccctagaggccaaggaaattgaagagaagtcagaggaagggatataaaatggaatgtattaatggattttagcccctttaagcttgtacttttgtgagagggttcaatggagagctttaatgcagatgagacttgaagcttctgaagaagatctaagtcttgatgaggttattcaaactcaaatcttgaatgcataatgatgataggccatggtcttcaaaaacgtggtacttgatgctctcccagagtgctaggatttgaatgccacaatacatattgactcatgtttttgtccattaatggtccgtgggtttctttaaatgaagtccattttagagtccatagatttcagtgttctgcaaaactgtcggggatcctaggctcccagcgcatcccagacgctccgccccacccatggcgtcaccctccac

SEQ ID NO: 14567 - RNA, 4273 nt, Homo sapiens
  source 1..4273: mol_type = other RNA
gctgggattacaggcatgagccaccgtgcccagccttcagcttgagttttaaggtaagtcttaaacttaaagcacggcggtataattaacagttgtgttgatactcttcagtagcattcacagccaggtccagggagttagcaccctttagtctcaccttattcagaggatgaacaaaaatatcttagatcatctctaggtaaggtagtactttcttgggaaacagggtattgtgtaacattctgtgcaaattcctgtcagttgaagctgattattagttgaatgggaatagaatgccacattctgcattcaattagtataatattggccaatttgtttctatagggttttcatctccaacttttatgctaattaatacacttctatgcctgtcaaatattagtaaataaatgggtttaatttcctaagggctattcagtaacatactcagtggaaggacatgttcctacttataaatgtacatctaagagaaggtaaaatatatcaatttaagaagaggccgtcagacatctctacctttttaaccaactctaggttttcaagaatgttttacatacaggtttataattgacaattatttgctagagtggtttttcccttttaaagtctcagtgtgtatggaactaagatgattaatatggcaaactcataagccattttaattttgatcatgcccttaagcattatgataaagcataccacagcagcatcaggcacttgaaatactgcattttatgtgtagctactgttgaagagctaatctttaaagaatttaatggctattttccagtgactataaagtctcagaaattctgaagcagaaaagtcacattaataataggactttagtttccattgttactgtgctttcctccttccaggttcattcatggcccaacagaactttaaaagtgcttttctgtagaatctgcagttaccagcaataactgatcatcttgctgcaaaaagctatagaattgatgctttgaatggttgatccatagttttttttttttttaatcaaagtacttatgtgtcaatgccaaagcaacgaagaattcccctttttccttcactattgacagcttcagtttctgtacttactgtgtcatcctatccgttcccttccctgagcctggactgctcttccaagggagactaggagtgaagggaggagtcctcccaaagttaccctttaagcttgataattagctccatagccatgctaaagcatgactgtagatccccaagtccctgacacattttcttctaagaaactggttagccaagaaagtaaagacgtaagccctgaagatggcaaaaggtgtcataatctcccaaagtcatctgtatagatgcttcatttaaccctttttcttttgcagacaaagggttaaaaatctcttctttctacctatatctttaaagagggattgacaagcccaaatttccttttatgaaaagacccaaggtttctggccaacaattcacttttttcagtctcttaggtcctcttgcatgcctgagaatattgagtattcggaatctcctaccagcccttggtaaatgaccctaccaggtggaatagtttgagctttatctgctcttttttaatgggatagaggggaaggcaacacgtcttattttatcaaaaattgcaaagctacacgctctttgtggagaagcaccaaaaggaaaaccttagtttggaaggattcattgtaaataaaaatagtaactcagccctccattcagggaggagaaaggcattttaaagctagtatattgaaggtttcccccttgacttcagtgttgaatggctcttgcaaggacttcttgaaggttttttttctcactagccagtgtttggccgacaggttgcacctctgcctgagaagatgccaggttaaaccccttcacatgggtgctccattgccgccatgggctttttgtcagggataagggtgcagccagccagcatgtccagagaggccaagatagagtcatacaggcgatctgcgtggctctccagctcaccagactgctttgcgatcctcccaaggacatcctctaaaaccggtaaagctgcagagaagacttgagacttgtaagattggacctggctgcagtcccgtggtcagtaacatctgcaacattatacagccagcagatcagctcttccagctgacagcaaaatgtcttcacacattgcaccagtgattcttttccctgttctcctcctttcctgggaagctgcccttcaacatctgggtctgagaatggccaccggtccaacctagctggcaaggaggggcgtgttttcagcagtccagaggagaccccgagggcctggctgctccccagactgccttcccctgcggagtcgtgggcacggacgaaggagcgcaggaaacagggattctggccctcaggatccccagatccttggagggcagctccagggggaagctggctttggctggagcttgaagggaaggaagctggcccatcactgtctgacacttccaaggggctctgccctttgatatccccagtgggcagggtaaccaaggtagaaatggatcctagatacgaaaccaggctagaaacctgtgtcagccgagcggggagggcaagatactcgtcatcactttccacttcctcttctgatttccacctagactctgtgcaggtagggcgccgggcactctggctggtcctcttctccctctctggcctgggcgagggccaccctctgtcccgtgtccttagctggggagagcccatatcaaggtgcttgcctatagtcagccggtccttcgcacccctcagggctggctctctgcgctcccaacgagcatccctactgcctggggctctgggggtagatgcaagttggctccaagatgccaagcccatgccaccctgtttctggggtactctggagggccactgcttaaggcttggctctctgggcccagaaaatggcagggcagtggcctctgctggtgggcagttgggggagacattagtaggtgatttgagggtgcttgctggagagacagagaagctatccaggtctaccccggagtcctgcaggacagggtcagctggcacacggctatcaaggtgctttgggagctgaggcccgggcctcagtgggtaagtatagtcaagcagatcttcatactctttatttgggttccagagaggggagtggcggtcgggtgatggaggcagggaatctggcagcacacaggcccagtactcagcctggaaggagaggcgtctcctgcctagcccagaagcatcacccccagagaacacaggctgtggtgaccactggggccgaggtcctagccccaccacagaggaaggttcctgggggacgaccggctccagggaggaggagaccttggccagagaaccaccacgaggctccgccctctcctggtgaccctggagactgctgcctgtggaggaagcagagatgctgcagctggaaggctgagctgcggaacctgggctcagcacggacttccactgtgacaggcaagagagacctgagctgtgaggctgctggctgaggtccagtgcctggggcaaatctgctagggatggatcatcttcggtatcagcatcatgtcctgagcaaatagttgttgttctgggaaggctcagagtctgagggaactcctcggaggaagaaagcttggtcttctccacctggctttccccggagagcagaaggtctccagaccccatggtggcaggaggcaggccactgagtgcaggctcagacctctcagctacgggctctctgttggcatcactggcctgtggctggtgggctctagaggggccgccagggtcagtcccaatccagcaagtaggggcaggtatcccttctgccccccatacaggggagatgagccctccctcagcttccaggcgtgggggctgctccccactcatgggccctgggatgtccagctcccgctccctgcagctccctctcccataggactgggcctttgtgtcttcagatgcttccgcttctgccttttcttcacccagggccattgagactccctacctaggtcagggttctgctgaagacttcagcttccgcaccgcgaacgcttcgcacgtccggagcggtctcagcagccccatgcgctggccccgagctggcggaccctgactgcaactgcggccctccaaccgcagcccaaaacgcgcagggcaggac

SEQ ID NO: 14568 - RNA, 4263 nt, Homo sapiens
  source 1..4263: mol_type = other RNA
gctgggattacaggcatgagccaccgtgcccagccttcagcttgagttttaaggtaagtcttaaacttaaagcacggcggtataattaacagttgtgttgatactcttcagtagcattcacagccaggtccagggagttagcaccctttagtctcaccttattcagaggatgaacaaaaatatcttagatcatctctaggtaaggtagtactttcttgggaaacagggtattgtgtaacattctgtgcaaattcctgtcagttgaagctgattattagttgaatgggaatagaatgccacattctgcattcaattagtataatattggccaatttgtttctatagggttttcatctccaacttttatgctaattaatacacttctatgcctgtcaaatattagtaaataaatgggtttaatttcctaagggctattcagtaacatactcagtggaaggacatgttcctacttataaatgtacatctaagagaaggtaaaatatatcaatttaagaagaggccgtcagacatctctacctttttaaccaactctaggttttcaagaatgttttacatacaggtttataattgacaattatttgctagagtggtttttcccttttaaagtctcagtgtgtatggaactaagatgattaatatggcaaactcataagccattttaattttgatcatgcccttaagcattatgataaagcataccacagcagcatcaggcacttgaaatactgcattttatgtgtagctactgttgaagagctaatctttaaagaatttaatggctattttccagtgactataaagtctcagaaattctgaagcagaaaagtcacattaataataggactttagtttccattgttactgtgctttcctccttccaggttcattcatggcccaacagaactttaaaagtgcttttctgtagaatctgcagttaccagcaataactgatcatcttgctgcaaaaagctatagaattgatgctttgaatggttgatccatagttttttttttttttaatcaaagtacttatgtgtcaatgccaaagcaacgaagaattcccctttttccttcactattgacagcttcagtttctgtacttactgtgtcatcctatccgttcccttccctgagcctggactgctcttccaagggagactaggagtgaagggaggagtcctcccaaagttaccctttaagcttgataattagctccatagccatgctaaagcatgactgtagatccccaagtccctgacacattttcttctaagaaactggttagccaagaaagtaaagacgtaagccctgaagatggcaaaaggtgtcataatctcccaaagtcatctgtatagatgcttcatttaaccctttttcttttgcagacaaagggttaaaaatctcttctttctacctatatctttaaagagggattgacaagcccaaatttccttttatgaaaagacccaaggtttctggccaacaattcacttttttcagtctcttaggtcctcttgcatgcctgagaatattgagtattcggaatctcctaccagcccttggtaaatgaccctaccaggtggaatagtttgagctttatctgctcttttttaatgggatagaggggaaggcaacacgtcttattttatcaaaaattgcaaagctacacgctctttgtggagaagcaccaaaaggaaaaccttagtttggaaggattcattgtaaataaaaatagtaactcagccctccattcagggaggagaaaggcattttaaagctagtatattgaaggtttcccccttgacttcagtgttgaatggctcttgcaaggacttcttgaaggttttttttctcactagccagtgtttggccgacaggttgcacctctgcctgagaagatgccaggttaaaccccttcacatgggtgctccattgccgccatgggctttttgtcagggataagggtgcagccagccagcatgtccagagaggccaagatagagtcatacaggcgatctgcgtggctctccagctcaccagactgctttgcgatcctcccaaggacatcctctaaaaccggtaaagctgcagagaagacttgagacttgtaagattggacctggctgcagtcccgtggtcagtaacatctgcaacattatacagccagcagatcagctcttccagctgacagcaaaatgtcttcacacattgcaccagtgattcttttccctgttctcctcctttcctgggaagctgcccttcaacatctgggtctgagaatggccaccggtccaacctagctggcaaggaggggcgtgttttcagcagtccagaggagaccccgagggcctggctgctccccagactgccttcccctgcggagtcgtgggcacggacgaaggagcgcaggaaacagggattctggccctcaggatccccagatccttggagggcagctccagggggaagctggctttggctggagcttgaagggaaggaagctggcccatcactgtctgacacttccaaggggctctgccctttgatatccccagtgggcagggtaaccaaggtagaaatggatcctagatacgaaaccaggctagaaacctgtgtcagccgagcggggagggcaagatactcgtcatcactttccacttcctcttctgatttccacctagactctgtgcaggtagggcgccgggcactctggctggtcctcttctccctctctggcctgggcgagggccaccctctgtcccgtgtccttagctggggagagcccatatcaaggtgcttgcctatagtcagccggtccttcgcacccctcagggctggctctctgcgctcccaacgagcatccctactgcctggggctctgggggtagatgcaagttggctccaagatgccaagcccatgccaccctgtttctggggtactctggagggccactgcttaaggcttggctctctgggcccagaaaatggcagggcagtggcctctgctggtgggcagttgggggagacattagtaggtgatttgagggtgcttgctggagagacagagaagctatccaggtctaccccggagtcctgcaggacagggtcagctggcacacggctatcaaggtgctttgggagctgaggcccgggcctcagtgggtaagtatagtcaagcagatcttcatactctttatttgggttccagagaggggagtggcggtcgggtgatggaggcagggaatctggcagcacacaggcccagtactcagcctggaaggagaggcgtctcctgcctagcccagaagcatcacccccagagaacacaggctgtggtgaccactggggccgaggtcctagccccaccacagaggaaggttcctgggggacgaccggctccagggaggaggagaccttggccagagaaccaccacgaggctccgccctctcctggtgaccctggagactgctgcctgtggaggaagcagagatgctgcagctggaaggctgagctgcggaacctgggctcagcacggacttccactgtgacaggcaagagagacctgagctgtgaggctgctggctgaggtccagtgcctggggcaaatctgctagggatggatcatcttcggtatcagcatcatgtcctgagcaaatagttgttgttctgggaaggctcagagtctgagggaactcctcggaggaagaaagcttggtcttctccacctggctttccccggagagcagaaggtctccagaccccatggtggcaggaggcaggccactgagtgcaggctcagacctctcagctacgggctctctgttggcatcactggcctgtggctggtgggctctagaggggccgccagggtcagtcccaatccagcaagtaggggcaggtatcccttctgccccccatacaggggagatgagccctccctcagcttccaggcgtgggggctgctccccactcatgggccctgggatgtccagctcccgctccctgcagctccctctcccataggactgggcctttgtgtcttcagatgcttccgcttctgccttttcttcacccagggccattgagactccctacctaggtcagggttctgctgaagacttcagcttcctaccgcaccgcgaacgcttcgcacgtccggagcggtctcagcagccccatgcgctggccccgagctggcggaccctgactgcaactgcggccctccaaccgcagcccaaaac

SEQ ID NO: 14569 - RNA, 3949 nt, Homo sapiens
  source 1..3949: mol_type = other RNA
gctgggattacaggcatgagccaccgtgcccagccttcagcttgagttttaaggtaagtcttaaacttaaagcacggcggtataattaacagttgtgttgatactcttcagtagcattcacagccaggtccagggagttagcaccctttagtctcaccttattcagaggatgaacaaaaatatcttagatcatctctaggtaaggtagtactttcttgggaaacagggtattgtgtaacattctgtgcaaattcctgtcagttgaagctgattattagttgaatgggaatagaatgccacattctgcattcaattagtataatattggccaatttgtttctatagggttttcatctccaacttttatgctaattaatacacttctatgcctgtcaaatattagtaaataaatgggtttaatttcctaagggctattcagtaacatactcagtggaaggacatgttcctacttataaatgtacatctaagagaaggtaaaatatatcaatttaagaagaggccgtcagacatctctacctttttaaccaactctaggttttcaagaatgttttacatacaggtttataattgacaattatttgctagagtggtttttcccttttaaagtctcagtgtgtatggaactaagatgattaatatggcaaactcataagccattttaattttgatcatgcccttaagcattatgataaagcataccacagcagcatcaggcacttgaaatactgcattttatgtgtagctactgttgaagagctaatctttaaagaatttaatggctattttccagtgactataaagtctcagaaattctgaagcagaaaagtcacattaataataggactttagtttccattgttactgtgctttcctccttccaggttcattcatggcccaacagaactttaaaagtgcttttctgtagaatctgcagttaccagcaataactgatcatcttgctgcaaaaagctatagaattgatgctttgaatggttgatccatagttttttttttttttaatcaaagtacttatgtgtcaatgccaaagcaacgaagaattcccctttttccttcactattgacagcttcagtttctgtacttactgtgtcatcctatccgttcccttccctgagcctggactgctcttccaagggagactaggagtgaagggaggagtcctcccaaagttaccctttaagcttgataattagctccatagccatgctaaagcatgactgtagatccccaagtccctgacacattttcttctaagaaactggttagccaagaaagtaaagacgtaagccctgaagatggcaaaaggtgtcataatctcccaaagtcatctgtatagatgcttcatttaaccctttttcttttgcagacaaagggttaaaaatctcttctttctacctatatctttaaagagggattgacaagcccaaatttccttttatgaaaagacccaaggtttctggccaacaattcacttttttcagtctcttaggtcctcttgcatgcctgagaatattgagtattcggaatctcctaccagcccttggtaaatgaccctaccaggtggaatagtttgagctttatctgctcttttttaatgggatagaggggaaggcaacacgtcttattttatcaaaaattgcaaagctacacgctctttgtggagaagcaccaaaaggaaaaccttagtttggaaggattcattgtaaataaaaatagtaactcagccctccattcagggaggagaaaggcattttaaagctagtatattgaaggtttcccccttgacttcagtgttgaatggctcttgcaaggacttcttgaaggttttttttctcactagccagtgtttggccgacaggttgcacctctgcctgagaagatgccaggttaaaccccttcacatgggtgctccattgccgccatgggctttttgtcagggataagggtgcagccagccagcatgtccagagaggccaagatagagtcatacaggcgatctgcgtggctctccagctcaccagactgctttgcgatcctcccaaggacatcctctaaaactggggtgttctccaacaggcactgaagaagaatctcccccttctgtaagacactctccgtcagagactgatgttcatctatatctttcttaaattgccggtaaagctgcagagaagacttgagacttgtaagattggacctggctgcagtcccgtggtcagtaacatctgcaacattatacagccagcagatcagctcttccagctgacagcaaaatgtctgtgtcagccgagcggggagggcaagatactcgtcatcactttccacttcctcttctgatttccacctagactctgtgcaggtagggcgccgggcactctggctggtcctcttctccctctctggcctgggcgagggccaccctctgtcccgtgtccttagctggggagagcccatatcaaggtgcttgcctatagtcagccggtccttcgcacccctcagggctggctctctgcgctcccaacgagcatccctactgcctggggctctgggggtagatgcaagttggctccaagatgccaagcccatgccaccctgtttctggggtactctggagggccactgcttaaggcttggctctctgggcccagaaaatggcagggcagtggcctctgctggtgggcagttgggggagacattagtaggtgatttgagggtgcttgctggagagacagagaagctatccaggtctaccccggagtcctgcaggacagggtcagctggcacacggctatcaaggtgctttgggagctgaggcccgggcctcagtgggtaagtatagtcaagcagatcttcatactctttatttgggttccagagaggggagtggcggtcgggtgatggaggcagggaatctggcagcacacaggcccagtactcagcctggaaggagaggcgtctcctgcctagcccagaagcatcacccccagagaacacaggctgtggtgaccactggggccgaggtcctagccccaccacagaggaaggttcctgggggacgaccggctccagggaggaggagaccttggccagagaaccaccacgaggctccgccctctcctggtgaccctggagactgctgcctgtggaggaagcagagatgctgcagctggaaggctgagctgcggaacctgggctcagcacggacttccactgtgacaggcaagagagacctgagctgtgaggctgctggctgaggtccagtgcctggggcaaatctgctagggatggatcatcttcggtatcagcatcatgtcctgagcaaatagttgttgttctgggaaggctcagagtctgagggaactcctcggaggaagaaagcttggtcttctccacctggctttccccggagagcagaaggtctccagaccccatggtggcaggaggcaggccactgagtgcaggctcagacctctcagctacgggctctctgttggcatcactggcctgtggctggtgggctctagaggggccgccagggtcagtcccaatccagcaagtaggggcaggtatcccttctgccccccatacaggggagatgagccctccctcagcttccaggcgtgggggctgctccccactcatgggccctgggatgtccagctcccgctccctgcagctccctctcccataggactgggcctttgtgtcttcagatgcttccgcttctgccttttcttcacccagggccattgagactccctacctaggtcagggttctgctgaagacttcagcttcctaccgcaccgcgaacgcttcgcacgtccggagcggtctcagcagccccatgcgctggccccgagctggcggaccctgactgcaactgcggccctccaaccgcagcccaaaac

SEQ ID NO: 14570 - RNA, 4356 nt, Homo sapiens
  source 1..4356: mol_type = other RNA
gctgggattacaggcatgagccaccgtgcccagccttcagcttgagttttaaggtaagtcttaaacttaaagcacggcggtataattaacagttgtgttgatactcttcagtagcattcacagccaggtccagggagttagcaccctttagtctcaccttattcagaggatgaacaaaaatatcttagatcatctctaggtaaggtagtactttcttgggaaacagggtattgtgtaacattctgtgcaaattcctgtcagttgaagctgattattagttgaatgggaatagaatgccacattctgcattcaattagtataatattggccaatttgtttctatagggttttcatctccaacttttatgctaattaatacacttctatgcctgtcaaatattagtaaataaatgggtttaatttcctaagggctattcagtaacatactcagtggaaggacatgttcctacttataaatgtacatctaagagaaggtaaaatatatcaatttaagaagaggccgtcagacatctctacctttttaaccaactctaggttttcaagaatgttttacatacaggtttataattgacaattatttgctagagtggtttttcccttttaaagtctcagtgtgtatggaactaagatgattaatatggcaaactcataagccattttaattttgatcatgcccttaagcattatgataaagcataccacagcagcatcaggcacttgaaatactgcattttatgtgtagctactgttgaagagctaatctttaaagaatttaatggctattttccagtgactataaagtctcagaaattctgaagcagaaaagtcacattaataataggactttagtttccattgttactgtgctttcctccttccaggttcattcatggcccaacagaactttaaaagtgcttttctgtagaatctgcagttaccagcaataactgatcatcttgctgcaaaaagctatagaattgatgctttgaatggttgatccatagttttttttttttttaatcaaagtacttatgtgtcaatgccaaagcaacgaagaattcccctttttccttcactattgacagcttcagtttctgtacttactgtgtcatcctatccgttcccttccctgagcctggactgctcttccaagggagactaggagtgaagggaggagtcctcccaaagttaccctttaagcttgataattagctccatagccatgctaaagcatgactgtagatccccaagtccctgacacattttcttctaagaaactggttagccaagaaagtaaagacgtaagccctgaagatggcaaaaggtgtcataatctcccaaagtcatctgtatagatgcttcatttaaccctttttcttttgcagacaaagggttaaaaatctcttctttctacctatatctttaaagagggattgacaagcccaaatttccttttatgaaaagacccaaggtttctggccaacaattcacttttttcagtctcttaggtcctcttgcatgcctgagaatattgagtattcggaatctcctaccagcccttggtaaatgaccctaccaggtggaatagtttgagctttatctgctcttttttaatgggatagaggggaaggcaacacgtcttattttatcaaaaattgcaaagctacacgctctttgtggagaagcaccaaaaggaaaaccttagtttggaaggattcattgtaaataaaaatagtaactcagccctccattcagggaggagaaaggcattttaaagctagtatattgaaggtttcccccttgacttcagtgttgaatggctcttgcaaggacttcttgaaggttttttttctcactagccagtgtttggccgacaggttgcacctctgcctgagaagatgccaggttaaaccccttcacatgggtgctccattgccgccatgggctttttgtcagggataagggtgcagccagccagcatgtccagagaggccaagatagagtcatacaggcgatctgcgtggctctccagctcaccagactgctttgcgatcctcccaaggacatcctctaaaactggggtgttctccaacaggcactgaagaagaatctcccccttctgtaagacactctccgtcagagactgatgttcatctatatctttcttaaattgccggtaaagctgcagagaagacttgagacttgtaagattggacctggctgcagtcccgtggtcagtaacatctgcaacattatacagccagcagatcagctcttccagctgacagcaaaatgtcttcacacattgcaccagtgattcttttccctgttctcctcctttcctgggaagctgcccttcaacatctgggtctgagaatggccaccggtccaacctagctggcaaggaggggcgtgttttcagcagtccagaggagaccccgagggcctggctgctccccagactgccttcccctgcggagtcgtgggcacggacgaaggagcgcaggaaacagggattctggccctcaggatccccagatccttggagggcagctccagggggaagctggctttggctggagcttgaagggaaggaagctggcccatcactgtctgacacttccaaggggctctgccctttgatatccccagtgggcagggtaaccaaggtagaaatggatcctagatacgaaaccaggctagaaacctgtgtcagccgagcggggagggcaagatactcgtcatcactttccacttcctcttctgatttccacctagactctgtgcaggtagggcgccgggcactctggctggtcctcttctccctctctggcctgggcgagggccaccctctgtcccgtgtccttagctggggagagcccatatcaaggtgcttgcctatagtcagccggtccttcgcacccctcagggctggctctctgcgctcccaacgagcatccctactgcctggggctctgggggtagatgcaagttggctccaagatgccaagcccatgccaccctgtttctggggtactctggagggccactgcttaaggcttggctctctgggcccagaaaatggcagggcagtggcctctgctggtgggcagttgggggagacattagtaggtgatttgagggtgcttgctggagagacagagaagctatccaggtctaccccggagtcctgcaggacagggtcagctggcacacggctatcaaggtgctttgggagctgaggcccgggcctcagtgggtaagtatagtcaagcagatcttcatactctttatttgggttccagagaggggagtggcggtcgggtgatggaggcagggaatctggcagcacacaggcccagtactcagcctggaaggagaggcgtctcctgcctagcccagaagcatcacccccagagaacacaggctgtggtgaccactggggccgaggtcctagccccaccacagaggaaggttcctgggggacgaccggctccagggaggaggagaccttggccagagaaccaccacgaggctccgccctctcctggtgaccctggagactgctgcctgtggaggaagcagagatgctgcagctggaaggctgagctgcggaacctgggctcagcacggacttccactgtgacaggcaagagagacctgagctgtgaggctgctggctgaggtccagtgcctggggcaaatctgctagggatggatcatcttcggtatcagcatcatgtcctgagcaaatagttgttgttctgggaaggctcagagtctgagggaactcctcggaggaagaaagcttggtcttctccacctggctttccccggagagcagaaggtctccagaccccatggtggcaggaggcaggccactgagtgcaggctcagacctctcagctacgggctctctgttggcatcactggcctgtggctggtgggctctagaggggccgccagggtcagtcccaatccagcaagtaggggcaggtatcccttctgccccccatacaggggagatgagccctccctcagcttccaggcgtgggggctgctccccactcatgggccctgggatgtccagctcccgctccctgcagctccctctcccataggactgggcctttgtgtcttcagatgcttccgcttctgccttttcttcacccagggccattgagactccctacctaggtcagggttctgctgaagacttcagcttccgcaccgcgaacgcttcgcacgtccggagcggtctcagcagccccatgcgctggccccgagctggcggaccctgactgcaactgcggccctccaaccgcagcccaaaac

SEQ ID NO: 14571 - RNA, 4360 nt, Homo sapiens
  source 1..4360: mol_type = other RNA
gctgggattacaggcatgagccaccgtgcccagccttcagcttgagttttaaggtaagtcttaaacttaaagcacggcggtataattaacagttgtgttgatactcttcagtagcattcacagccaggtccagggagttagcaccctttagtctcaccttattcagaggatgaacaaaaatatcttagatcatctctaggtaaggtagtactttcttgggaaacagggtattgtgtaacattctgtgcaaattcctgtcagttgaagctgattattagttgaatgggaatagaatgccacattctgcattcaattagtataatattggccaatttgtttctatagggttttcatctccaacttttatgctaattaatacacttctatgcctgtcaaatattagtaaataaatgggtttaatttcctaagggctattcagtaacatactcagtggaaggacatgttcctacttataaatgtacatctaagagaaggtaaaatatatcaatttaagaagaggccgtcagacatctctacctttttaaccaactctaggttttcaagaatgttttacatacaggtttataattgacaattatttgctagagtggtttttcccttttaaagtctcagtgtgtatggaactaagatgattaatatggcaaactcataagccattttaattttgatcatgcccttaagcattatgataaagcataccacagcagcatcaggcacttgaaatactgcattttatgtgtagctactgttgaagagctaatctttaaagaatttaatggctattttccagtgactataaagtctcagaaattctgaagcagaaaagtcacattaataataggactttagtttccattgttactgtgctttcctccttccaggttcattcatggcccaacagaactttaaaagtgcttttctgtagaatctgcagttaccagcaataactgatcatcttgctgcaaaaagctatagaattgatgctttgaatggttgatccatagttttttttttttttaatcaaagtacttatgtgtcaatgccaaagcaacgaagaattcccctttttccttcactattgacagcttcagtttctgtacttactgtgtcatcctatccgttcccttccctgagcctggactgctcttccaagggagactaggagtgaagggaggagtcctcccaaagttaccctttaagcttgataattagctccatagccatgctaaagcatgactgtagatccccaagtccctgacacattttcttctaagaaactggttagccaagaaagtaaagacgtaagccctgaagatggcaaaaggtgtcataatctcccaaagtcatctgtatagatgcttcatttaaccctttttcttttgcagacaaagggttaaaaatctcttctttctacctatatctttaaagagggattgacaagcccaaatttccttttatgaaaagacccaaggtttctggccaacaattcacttttttcagtctcttaggtcctcttgcatgcctgagaatattgagtattcggaatctcctaccagcccttggtaaatgaccctaccaggtggaatagtttgagctttatctgctcttttttaatgggatagaggggaaggcaacacgtcttattttatcaaaaattgcaaagctacacgctctttgtggagaagcaccaaaaggaaaaccttagtttggaaggattcattgtaaataaaaatagtaactcagccctccattcagggaggagaaaggcattttaaagctagtatattgaaggtttcccccttgacttcagtgttgaatggctcttgcaaggacttcttgaaggttttttttctcactagccagtgtttggccgacaggttgcacctctgcctgagaagatgccaggttaaaccccttcacatgggtgctccattgccgccatgggctttttgtcagggataagggtgcagccagccagcatgtccagagaggccaagatagagtcatacaggcgatctgcgtggctctccagctcaccagactgctttgcgatcctcccaaggacatcctctaaaactggggtgttctccaacaggcactgaagaagaatctcccccttctgtaagacactctccgtcagagactgatgttcatctatatctttcttaaattgccggtaaagctgcagagaagacttgagacttgtaagattggacctggctgcagtcccgtggtcagtaacatctgcaacattatacagccagcagatcagctcttccagctgacagcaaaatgtcttcacacattgcaccagtgattcttttccctgttctcctcctttcctgggaagctgcccttcaacatctgggtctgagaatggccaccggtccaacctagctggcaaggaggggcgtgttttcagcagtccagaggagaccccgagggcctggctgctccccagactgccttcccctgcggagtcgtgggcacggacgaaggagcgcaggaaacagggattctggccctcaggatccccagatccttggagggcagctccagggggaagctggctttggctggagcttgaagggaaggaagctggcccatcactgtctgacacttccaaggggctctgccctttgatatccccagtgggcagggtaaccaaggtagaaatggatcctagatacgaaaccaggctagaaacctgtgtcagccgagcggggagggcaagatactcgtcatcactttccacttcctcttctgatttccacctagactctgtgcaggtagggcgccgggcactctggctggtcctcttctccctctctggcctgggcgagggccaccctctgtcccgtgtccttagctggggagagcccatatcaaggtgcttgcctatagtcagccggtccttcgcacccctcagggctggctctctgcgctcccaacgagcatccctactgcctggggctctgggggtagatgcaagttggctccaagatgccaagcccatgccaccctgtttctggggtactctggagggccactgcttaaggcttggctctctgggcccagaaaatggcagggcagtggcctctgctggtgggcagttgggggagacattagtaggtgatttgagggtgcttgctggagagacagagaagctatccaggtctaccccggagtcctgcaggacagggtcagctggcacacggctatcaaggtgctttgggagctgaggcccgggcctcagtgggtaagtatagtcaagcagatcttcatactctttatttgggttccagagaggggagtggcggtcgggtgatggaggcagggaatctggcagcacacaggcccagtactcagcctggaaggagaggcgtctcctgcctagcccagaagcatcacccccagagaacacaggctgtggtgaccactggggccgaggtcctagccccaccacagaggaaggttcctgggggacgaccggctccagggaggaggagaccttggccagagaaccaccacgaggctccgccctctcctggtgaccctggagactgctgcctgtggaggaagcagagatgctgcagctggaaggctgagctgcggaacctgggctcagcacggacttccactgtgacaggcaagagagacctgagctgtgaggctgctggctgaggtccagtgcctggggcaaatctgctagggatggatcatcttcggtatcagcatcatgtcctgagcaaatagttgttgttctgggaaggctcagagtctgagggaactcctcggaggaagaaagcttggtcttctccacctggctttccccggagagcagaaggtctccagaccccatggtggcaggaggcaggccactgagtgcaggctcagacctctcagctacgggctctctgttggcatcactggcctgtggctggtgggctctagaggggccgccagggtcagtcccaatccagcaagtaggggcaggtatcccttctgccccccatacaggggagatgagccctccctcagcttccaggcgtgggggctgctccccactcatgggccctgggatgtccagctcccgctccctgcagctccctctcccataggactgggcctttgtgtcttcagatgcttccgcttctgccttttcttcacccagggccattgagactccctacctaggtcagggttctgctgaagacttcagcttcctaccgcaccgcgaacgcttcgcacgtccggagcggtctcagcagccccatgcgctggccccgagctggcggaccctgactgcaactgcggccctccaaccgcagcccaaaac

SEQ ID NO: 14572 - RNA, 4052 nt, Homo sapiens
  source 1..4052: mol_type = other RNA
gctgggattacaggcatgagccaccgtgcccagccttcagcttgagttttaaggtaagtcttaaacttaaagcacggcggtataattaacagttgtgttgatactcttcagtagcattcacagccaggtccagggagttagcaccctttagtctcaccttattcagaggatgaacaaaaatatcttagatcatctctaggtaaggtagtactttcttgggaaacagggtattgtgtaacattctgtgcaaattcctgtcagttgaagctgattattagttgaatgggaatagaatgccacattctgcattcaattagtataatattggccaatttgtttctatagggttttcatctccaacttttatgctaattaatacacttctatgcctgtcaaatattagtaaataaatgggtttaatttcctaagggctattcagtaacatactcagtggaaggacatgttcctacttataaatgtacatctaagagaaggtaaaatatatcaatttaagaagaggccgtcagacatctctacctttttaaccaactctaggttttcaagaatgttttacatacaggtttataattgacaattatttgctagagtggtttttcccttttaaagtctcagtgtgtatggaactaagatgattaatatggcaaactcataagccattttaattttgatcatgcccttaagcattatgataaagcataccacagcagcatcaggcacttgaaatactgcattttatgtgtagctactgttgaagagctaatctttaaagaatttaatggctattttccagtgactataaagtctcagaaattctgaagcagaaaagtcacattaataataggactttagtttccattgttactgtgctttcctccttccaggttcattcatggcccaacagaactttaaaagtgcttttctgtagaatctgcagttaccagcaataactgatcatcttgctgcaaaaagctatagaattgatgctttgaatggttgatccatagttttttttttttttaatcaaagtacttatgtgtcaatgccaaagcaacgaagaattcccctttttccttcactattgacagcttcagtttctgtacttactgtgtcatcctatccgttcccttccctgagcctggactgctcttccaagggagactaggagtgaagggaggagtcctcccaaagttaccctttaagcttgataattagctccatagccatgctaaagcatgactgtagatccccaagtccctgacacattttcttctaagaaactggttagccaagaaagtaaagacgtaagccctgaagatggcaaaaggtgtcataatctcccaaagtcatctgtatagatgcttcatttaaccctttttcttttgcagacaaagggttaaaaatctcttctttctacctatatctttaaagagggattgacaagcccaaatttccttttatgaaaagacccaaggtttctggccaacaattcacttttttcagtctcttaggtcctcttgcatgcctgagaatattgagtattcggaatctcctaccagcccttggtaaatgaccctaccaggtggaatagtttgagctttatctgctcttttttaatgggatagaggggaaggcaacacgtcttattttatcaaaaattgcaaagctacacgctctttgtggagaagcaccaaaaggaaaaccttagtttggaaggattcattgtaaataaaaatagtaactcagccctccattcagggaggagaaaggcattttaaagctagtatattgaaggtttcccccttgacttcagtgttgaatggctcttgcaaggacttcttgaaggttttttttctcactagccagtgtttggccgacaggttgcacctctgcctgagaagatgccaggttaaaccccttcacatgggtgctccattgccgccatgggctttttgtcagggataagggtgcagccagccagcatgtccagagaggccaagatagagtcatacaggcgatctgcgtggctctccagctcaccagactgctttgcgatcctcccaaggacatcctctaaaactggggtgttctccaacaggcactgaagaagaatctcccccttctgtaagacactctccgtcagagactgatgttcatctatatctttcttaaattgccggtaaagctgcagagaagacttgagacttgtaagattggacctggctgcagtcccgtggtcagtaacatctgcaacattatacagccagcagatcagctcttccagctgacagcaaaatgtcttcacacattgcaccagtgattcttttccctgttctcctcctttcctgggaagctgcccttcaacatctgggtctgagaatggccaccggtccaacctgtgtcagccgagcggggagggcaagatactcgtcatcactttccacttcctcttctgatttccacctagactctgtgcaggtagggcgccgggcactctggctggtcctcttctccctctctggcctgggcgagggccaccctctgtcccgtgtccttagctggggagagcccatatcaaggtgcttgcctatagtcagccggtccttcgcacccctcagggctggctctctgcgctcccaacgagcatccctactgcctggggctctgggggtagatgcaagttggctccaagatgccaagcccatgccaccctgtttctggggtactctggagggccactgcttaaggcttggctctctgggcccagaaaatggcagggcagtggcctctgctggtgggcagttgggggagacattagtaggtgatttgagggtgcttgctggagagacagagaagctatccaggtctaccccggagtcctgcaggacagggtcagctggcacacggctatcaaggtgctttgggagctgaggcccgggcctcagtgggtaagtatagtcaagcagatcttcatactctttatttgggttccagagaggggagtggcggtcgggtgatggaggcagggaatctggcagcacacaggcccagtactcagcctggaaggagaggcgtctcctgcctagcccagaagcatcacccccagagaacacaggctgtggtgaccactggggccgaggtcctagccccaccacagaggaaggttcctgggggacgaccggctccagggaggaggagaccttggccagagaaccaccacgaggctccgccctctcctggtgaccctggagactgctgcctgtggaggaagcagagatgctgcagctggaaggctgagctgcggaacctgggctcagcacggacttccactgtgacaggcaagagagacctgagctgtgaggctgctggctgaggtccagtgcctggggcaaatctgctagggatggatcatcttcggtatcagcatcatgtcctgagcaaatagttgttgttctgggaaggctcagagtctgagggaactcctcggaggaagaaagcttggtcttctccacctggctttccccggagagcagaaggtctccagaccccatggtggcaggaggcaggccactgagtgcaggctcagacctctcagctacgggctctctgttggcatcactggcctgtggctggtgggctctagaggggccgccagggtcagtcccaatccagcaagtaggggcaggtatcccttctgccccccatacaggggagatgagccctccctcagcttccaggcgtgggggctgctccccactcatgggccctgggatgtccagctcccgctccctgcagctccctctcccataggactgggcctttgtgtcttcagatgcttccgcttctgccttttcttcacccagggccattgagactccctacctaggtcagggttctgctgaagacttcagcttcctaccgcaccgcgaacgcttcgcacgtccggagcggtctcagcagccccatgcgctggccccgagctggcggaccctgactgcaactgcggccctccaaccgcagcccaaaacgcgcag

SEQ ID NO: 14573 - RNA, 4207 nt, Homo sapiens
  source 1..4207: mol_type = other RNA
gctgggattacaggcatgagccaccgtgcccagccttccttcatctacttattttcctgtgatgcctccatgttttagagtatgtgtctgaggggcaggaatatgtattagatatatctagggcagtcccaccagctttacattcttgagacctcatccatcagttcttgttttgcagacatatacttctattgactacaatgagaagtgtgtctcttaaaaaggtaagtctggccgcgcgtggtggctcacgcctgtaatcccagcactttgggaggcagaggcaggtggatcacgaggtcaggagatcgagaccatcctggctaacatagtgaaaccccgtctctactaaaaatacaaaaattagctgggttcgtgggggtgcgtgcctgtagtcccagctactcaggaggctgaggcaggagaatcgcttaaacctgggaggcggaggctgcagtgagcccagatcatgccactgcactccagcctgggcgacagagtgagattctgtctccaaaaaaaaaaaaaattagccaggtgtggcagtgcacgcctgtagtcccagctactggggaggctgaggcaggagaattgcttgaactggggaggcagaggctgcagtgagcccagattgtgccactgcactccagcctcagtgacagagcgagaccctgtctcaaaaaaaaaaaaaaaaaacaagtgaacaaaggtctctggttttcctaggcagaggaccctgcggccttccgcagtgtttgtgtccctgggtacttgagattagggagtggtgatgactcttaaggagcatgctgccttcaagcatctgtttaacaaagcacatcttgcaccgcccttaatccattgtttatctgctgaccttccctccactattgtcctgtgaccctgccaaatccccctctgcaagaaacacccaagaatgatcaattaaaaaaaaaaaaaaaaagttaagagcaaaaaaaaaaaaaaaaaagtcctggttgggtgtggtggcgtgtgcctgtaatcctagcactttgggaggccaatcccttgggcccaggagtttgagaccagcctgggcaatataaggagaccctatctctaaaaaaatgaaaaaaaaaataaataaataagttcaagttcaggtccctagtacctgtgaatgtcaccttacttggaaagagtattcgctgatctaattaaggtaaggatctcgagatgagatcatcctcattagagtgggccctaaatccagtgacatggatttggtgtccagtgatgtctttacaagagacaggaaagaatacacacaggtattcctgtgtatttcaagtcaagttgtatatggtagtccttgcttaataagggaaaagttcgggtctgtgtatttattcttagggctgccataaaaaattatggccttctcaggggagaaggccacatgaagatagaagcagagactggacttacactgtcacaagccaaggactgccaaggattgccgatggccactagagaaaggagaaaggcatggaatggattctcccccagagcctccagaaagaacctaccttactaacactttaatttcagactttgggcctccagaactgtgagactcaatttctgttaagtcacccatgtggtggtaattttttttttttttttttgagacagagtcttgctttgtcacccaggccggagtgcagtggcatggtctcggctcactgcaacctctgcctcctgggttcaagtgattctcctgcctcagcctcctggttagctgggattacaggcacacagctccaagcctggctaatttctatattttcagtagagacagggtttcatcatgttggccaggctagtcttgaactcctgatctcaagtgacccgcccaccttggcctaccaaagtgctgggattacgggcatgagcgctgcgcccggccaggttgtggtaattttttatggcagccctaagaataaatacacagacctgaacttttgtctttttgagcaaggactgccatgtacaacttgacctgagagtgcagccttcaatcttttcctctggggcctctggcaacagttctcagatgactatgctcagagagacacctgtgactgtccacccagcagccatctgttcaccagcagaggagaccggaagtcccttgtgaggtgctgggttctgaagcttcaggagtgggatccatgtcatcgtccatatcagatctgtctgctccaatctcagccctttcttcctgcctgatccaaaggctattttctagctgttcttcagcaatttctagctcttcttccgtttgtaaagtagccacagtttcccggggcaagtttgaggaatatagcccaaatttggctttatagccaaacattgcctcaaatggactttgctgcaaggaaacgtcgaaagcctgattcctcaccatctgcatgaatcggaggcctttggcccagtgacatgagtggttactctgcatccaggtacttatcatgttctttacatcacggcttgctccttccagggagccctggctttggccagggtggtacttaccagatacaatctttaggtctggccacaactcattgagctcatgaacaacctggtttgtgaactcaacgccactgtcagagtctaacacactgggtgtaccaagaattgtgaaaatatctaacaagacactgaccacctcatgggcctgtttggttcttaatggccgtaaaataataaacttggttgagtgatcctggtagtataaaatgaacttgaactcaccatcggcactggactgcatgtcaagtatttcaacttggcatgtggagtctatgtccttaaaagtcatgggctttggtgcaaggcctctcttgggtactgggttcttctggtggcactgtttacacagagtcagatataagacaataacttctttggtgacattcccatattttccttgcagctccttgagcatgcgtgtccgcccaccatgtccaatactgagatgtgtatcatgaagaatatcaaacaactcttccttatgtacataataccgtattcgatcacgttctccatgagtagcctctatcagtttctctgtgccctgtacagagatcacatcatattttgctgcacggcgataatcacgtgatgacttcttccctttttctttagcttctttaacttcctttattgtttgaaagtacttttctttggaaaataccttgctgttgtaacttttgctttctactaactttgttacactcataagaaacttttctctcatgttacttatctccatttccatttcacttgcatttgaaaccccaggtggatcatttccagctctctgaggcatcatggagagctgtaagaaggatcctgtgagtcttcgccttggctgtttccgactcggaatgtcctcgcattgatcctcccaatcacagccagctgaaaccagcctccttcctgacgtattcagtaactttagctgattgccatctctccttcatctcaacaacctgtaccacactcactggagcacttcgctttgcatctttagtcgaccagttcagatatatacaacctataaggtagggacggaggcttctacctgcctgtaccccctttggagggcccacgaatacagagctgagcacaaaagatgtttaaaggacattttgtcaaaaatgtcgcttacaggtaggtcgttattagcaaggtagagcagcggtacggccgagtctacgcttgggaattcatttgctgactcttatcatttactgactaaagcaaagttactgaggcctcagtttcctcatctacaacccggggagatgaccagtacccatcacaatcgattgctatgaagattcaatgataatgcagataaggcacttaatacagtgtcccctcaccgtccacaccacacgggcacgcccgcttattcctgaggaccgggctgggatgtcgcctcctttgtgtagccttcctaccctgacttcgcagactgctcccaccgcctggatccatgcccgtccacccgccagctcagggctgaacggctgaggcgggcgcgcggtggagaaaagagctgcagactgaggaaggtcaggaaggagaaagggacacaccagacgcggcgtctgaatccccctccacccagaggcccccgagcagcaactcc

SEQ ID NO: 14574 - RNA, 4696 nt, Homo sapiens
  source 1..4696: mol_type = other RNA
gctgggattacaggcatgagccaccgtgcccagctgacaccattttttgaagcagaaaattttttctcacaatatttttactcacctcaaagaaacaatgcttgtacattcttaccagttctaataaaatttcctttccaatcttaggtacaaaaacttaaactcattcaattccaatatgaaatattataaacagaaatatggtttttctaacaagttttgaaccaatgtggggttcgaaaaatgtggggatatacagaataaaaacactttagataaataatctgaatttaattaggatacaatatacccctaggaaaaaaggtaaattaaagttataaagctattcattttactaatacttacacaagtattaataattccaatactaaatatcggagagctgctacatattaaccaaagttaaatacatacagtgattactaccatataaaatacatgcatatttacaaagatcaaaagaggatgtggaataattataatcctgtttttaattataatcctgttttctagcaagcttattatcagcataataacaaagaaatacaaactttccccctacattttgtcttactatagaaacggaattcctacccacattctgtatttactttaactcctttctcaaactcttcaattccatccctttgaattccatatcttcataatttggtcaaagatctgccatccttttgtctcctcaaacaaccaagagaactttacgacaaaggttttgctccagtagttaaacattagtgaatcccacaaacataattattacaaagtaagttttttatataacacatgaagaaaatgtattttcttcagcaaaaatcaacagtaacttaggaccattttctggatgttttaattcctagaccaagaaccaatatccttaaaaccatcttttcctggttgtggcaaatgactaaatattttataacccactctgcctcctatgtgtcctatttggtgcacatttactattcatatgagtcatactgcaatttactttgtttttaaaattaagaatttaagaacctctcaaaacaagtggcaagccctgggtaacccaggtttgctgtaggtgctgagtcaggactcccggcttcatattacaggcactcatcactggaaaggcgacagcctttgtttctccccgccctgccaactccttgctggcaggaacatactggaagacttttttgtgctgttatagaagcagcacaacacaggagttgcccctcccccaaatggatttttgacactcaatcatactttgagatttagaaataccctctctggatgcataaagcaactaatcagatggtactgtgtgcttcatgttggtgcactcaggccattagcattttaaagattcaccccagagaaaaggaatgtaatccaatgatcggaggtagagaagtatcatttgcattctactcctattagtatcaagatgctttccttgtatcaacagccaagtgaggaaatttggtgtatatctacagccagcactgtctcttctcacatcacagctacttcctaactagcaggttcatcaaatgattgtctgtattagctcaacagacacgtgtgtgaatgtcaaatacacgtctatttatagtgtcaaagcattgcctggagtgaactcactgctacttaaacaaaatgctcactgcggataagggcaatccctgctctcagatgtggaagacagaacaaggaaggccatggagctgtgggacatgacctccatagtcacacagagacctccacagccacatgggacgtgacctccatagtcacacaaagacctccacagccacgtggacgagacctccatagtcacacacgacctccacagccacatgggaccatgggacgtgaccaccatagtcacccaaagacctccacagccacacagacgagacctccatagtcacacagagaccgccacagccacatggacgagacctccatagtcacacacgcgacctccacagccacacggacgagacctccatagtcacacagcgacctccacagccacatgggacgcgacctccatagtcacacagcgacctccacagccacacagacgagacctccatagtcacacagcgacctctacagccacacgggacgcgacctccatagccacacagcgacctccacagccacatgggacgcgacctccatagtcacacagagaccttcagagccacatggatgaaacctccatagtcacacagagatctccacagccacacgggacgtgacctccacagtcacgcagagacctccacggccacatgggacgtgacctccatagtcacaaagagacctccacagccacatggacgagacctccatagtcacacaacaacctccatagtcacatagcgacctccataggcacacagtaacctccatggtcacacagcgacctccacagccacatgggacgtgacctccatagtcacacagcgacctccacggccacatgcgacgtgacctccatggtcacagagacctccacagccacatggatgagacctccatagtcacacagcgacctccatagtcacatagcgacctccatagtcacacagcaacctccacagtcacacagcgacctccacagccacacgggatgtgacctccatactcccacacagacctccatagccacacggacgagagagacctccatagtcacacagcgacctccacagccacacggaacgcgacttccatggtcacacagtgacctccacagccacacgggacgcgacctccacagtcacacagcaacctccacagtcacatagacaagacgtccacagccacaaaggacgagacctccatagtcacacagcaacctccacagccacacagacaagatgtccacagccacatgggacgtgacctccacagtcacacagcgacctccacagccacacgggacgagacctccatagtcacatagctacctccagagtcatatagcgaccttcacagccacacaggatgagacctgtgtggctgtggaggtcccattcctacgctgggcctgcagcttgggtgtgagggaaggatgccacctaatacaaaggactaacctctctctttcactgaccattatcacctggtatcaacatgtcatgaagacaactactccgtgactcaagaaagacagcctggctttcctcagaacttgcatgtcagccgggtgcaatggctcacgcctggaatcccagcacttcgggaggccaaggcaggaggactgtttgagtccaggagttcccaaggagcctggacaacatagggaggccacacctctctctctctttttttttaaagggcctgagaggtttgtttttgtgcaacaaaaaacaaaaaaaccagttctaaatcaaaacacagcctttctctgaaacctttctagaaatgcagtcttcagttttctgttgtctcatttagcaacaagcaggactaaaacatagagacacaagacacagaagatgcactttcttcaggagttagttattacagaccgaaattcaggtcgttcaatggaaaagatccatgccttcacaacattctcctctacacactacaggaggaaaatgataaaaacaaagtaacaaacagaaacaacaggccagctgaggcccaaaaagtgtaagtgacaggactcctaaggtgtttagacgtagagggagagtgagcaaaaccaaaaaccaaacacgaaaccaaacctttcaaacttgggtgagaattggtcctttcacataagattctttggcaaagtatacaccaccccacctatacaaaaactgagactttattttgaaacaccaagtcaaatgtattgcctgcttgatcagacatcagtaatttcacatttgcttttcttagatttctatcccatttgcttccaatagatctgaggcagctcatgcttcagactctgtgagaggccagaagcccacctgtgcgtggagagatgatcacaagtaagtgaatcaactgattccacatatcccctggtggggcagcacctccagagatgcccctggaatttgcgatgtctcattccaaggaggaaccagtgactgtcattttggggtaagcactcctagttctcagggtttcaagacagacacctaaggcacctacaaacattgttcataatatctagtgattgttttataagacatatcactgtgtacaaggtgttgcaaagtaattccgcctttttaagtaaaaataatgaggcagcagatatcagacagccaaatctccaggaaaagagtagtaagaagctttagctgtaaggtatcatattttattaaaccaaagacctctgagagttcaggtgggactcgtttctagtcaagacacagtacaagaactgtattaactttctgcctgaaataaccacaaaatcaggcaaaatatacgaagcaacagttttcgaagcactgagtactgggctatgaaagacagtgaatctcagaaagatgggagacaaacaggccccaactgctcagcttcctgtgtgaagagcttccaggttgtggtgtgggggccctgagtagctgggactacaggcatgcaacaccccactaggctaatttttaaattttttgtagagatggggtttcac

SEQ ID NO: 14575 - RNA, 4420 nt, Homo sapiens
  source 1..4420: mol_type = other RNA
gctgggattacaggcatgagccaccgtgcccagctgataatatacttttaaaacatggacataccaatagtccttgagatatgtaagatcatcttatacgcatacaattaagagatactcttgatatttgcctgcagtttaaaagactaacaataaaaatggtaataataatagtgaaaataataaaaatagtaacattttattatatgtctactctatgactgatgctatccaaacattacctgtagtctcacaagaacactattaagcagaaattaatattagctccattcgacagaggaagaaactgagaaatagcttgcccaagattagctataacttgaaagagcaagaattcaaatttaggttgttctgactgcaaattattttcataccatttctaagtaatgctcactacttcagcatattttatcttaatttttaaatatattatttaattatggctgttaattgaaggcttatttcacagagaataggataaggatttacagcgaaaatatagaggctattttggagggaaaaaaattaccttgagtttcatgtccttgatattgctggccaaaattagccacatacctcagactatagtggaggcagacagttcaattaaccaaatatggggaaaaatagcattgattaagtagaaatcttaagaagtggttaattacatttcctggataactgaagacattttgtgtttcagcccatcttaatgaaaatctaaatatatcaggccctttgcagagaacagatcacagcgcctttctctgtgtccttgaagtttatttaatcaagtttttcagaacacatatattgacttcttcagcgtctccactataattgtgatatttagtaatgattcctgattccacaggagagattgtttcctaaatgtttataatcattttatggtatgacatcacaacacttgaaaacctgtatctcactcatgcatctctaacaattggaaattcatataatttcaatttcattcttctgaacctcacccatgtcttgttctgaacttgtctctgtcttatcctaaacttcatttaagtcattttggggtaacagacatagagttgtaaatgatttcctggaggggagactgagcacagctaatccccagggagatgcccaaaacttctaaacccttgtagttaatttacacattagattcttggcattcatatattttctctttctactgttgtagttgtggttatttttaatttttctcagcttatatttagagtatattagttcctgtggtttcaagccaaatgtataatctcaacaatcaataagtgtagatatggtgacattaatatcagtgcccaaatcccagttattctgagcctactctgctgtgttccctctgccctgccttcagcaggatagtgatgtttcctatgggcttaggagaaagttcacttattttctactttaggtactcttcaaggcttcttctcacagcccctgcttcattgggcatagctatgcttacctgctgattacccaagcccacagagtcattgagctacactttagtaagcagtagactattgagggggaaaggacttatccataattcagactttatcagatggacttcagaggagagtcgcttgagcccggtgtctctcaggttttgcctgagcaccatttctgcattttctattttgcttaggagttcaaatctgattcattcacagggcggaaagaacatacgccatctcatccattgtcttcctcttcccccagatgcttcgaaggaaaataaagaaaaccaacaaagacaataagctgctccttcttcatttagcccatctcactgttgacttctccagagaagacgctgtaacagagtttgaagaacaagatctttcttggaaatcaacaccacttcctgtaggtagttaacaatgccgttctccttgcagaagatctacaaacttttgcagaatgagcaagtgaaggagtagcagtggcatctttcatattcattcagaatcccaaccagaacaggtgttacagcagcctccctccatctttctccatcctctctcccatctgctgacagcacgcatgtctcttccaaagtcacttccccacttaaattgtaagtctaatcagaaactgatgtggctgcaaaacgaatatccctgctttccaacttttgaccttgctgcagtcgatgcagacatgagaatttgctggaactcagactttcaagacccactgggctctccaacgtgtcatgttctccaatattcattagctggcagtgcacatatttgtcatgggctgcttgctgcttcactttcgtgtttggaccaaattcatactgctggtttatgtcacaggtaaaaccagcacacaagtttcctgactctcgtatttggcccatttcatcttagcgcttgtctgcacacctgttagcaggaggctctgtgatttgctctatattctaatcagagccccataacaactcttttcttttgtctcagctcctcagacactatgtggatcttctttctttttcaattctcttttctcccataatggagacatgatcacacatatctggtccttctctccttctggacacatagaaggactatccattctggtcccttctagttaggaagggccatgttgctaattctggtcaatgagctgtcaggagaagcacatgtcatttgaggatataaagcatttccctgctgatgcagcagtctccaatacccacttcaactctccaggtcacatgtttccttcttcctctattggagtttcatgttgagaaagtggagccacaaaaccaaagccacctggatagctgagctatgaccctcttattatgttgtttcaacagactcttaaagacagcacaatggtcggttgatagctgcactaaatctctttcattttctccccgtattaatttcgcctcctgaatttttttctctctcttcatgagtcaaattttatgggtcttccctagagaagggcttgctcaaacataccacatggtttttagtgacaatcagtcttgtgtcttcatccattttttttgccatttgctagatgcatgcctttaagcatataacttcactcccagacttcttcttttcttttttctttcggctttttgtttaattttcctggtgctcatgggctgggttgtcatctgtgtaggaaaaaggtggtacttgtcagccaggtatccagctcaggctgttgaccagggtagcagcaaagaccagattgatcaggatgttctctccatgtgtctcaggcttatccctgagtcgcgacttgtttcccagagaggaaagagacatgagcagaatctgcaaggcttcttatgagacagcttcagaagttacagaaagtcccttctgacaaattctgttggtcaaataagtaggacagccatcccagattccaagggagacaattagattccacctgttaattctattaatgtccctgttataaggctacagtcgaagagagaactatataatttaatgatatctcctgtacttctcttctttttcttaattcctgacaccaataacacacacaaaattaaatgcatttttaaaagtacattcaaagacatcctttcacacacatatatatttcattctcaaatgtatccccatttggatgataaattacatgattgcctaactttcgaacataaaaagtacactcctctgcaaaacataccattcacaaacaaacacacaaacacagaaacacactgaattccccttctccttgcaaatacacacagataaccaaccactctaaaatgcacacacaaacacacatacactcataataacacagagatgccctcaatttctaaatgcacactttcaaatccttgcctaaatcatcctccccagacaaatagcacacacccattcacatattaatactaacagactctcatacccacaaacatgcaagagagaaatctaggaaaaccagacacacacaaaaagaaaaaatatatagagagacatgtagactaatgcactctcttcagtattccctgcacatatgacacctctaaggaggctgttgatacgtcctggacacacaaaaatgcccgtgttcaaatgaactcctccacacccacatactacagacaaatccaagcatatcctttttttaattgtggtagaatcaagcatctactttcaaatacaaaatcacacatagactataataaataaaacatattcaggcataattatacacacacacacacacacacacacacaacttctggccttaagttctcttcttccaccaacactgtctctcatttcgtcttaaagcccagccttcactcagaagatcatctttatggaaatct

SEQ ID NO: 14576 - RNA, 2276 nt, Homo sapiens
  source 1..2276: mol_type = other RNA
gctgggattacaggcatgagccaccgtgccccgcctattcttcttttaaaccaaaaaaactttcaggtgagtcaaaaccaaaaccaataagctttttatgacttaaccatggatgaaagagacaccttcaaaatcaggtgcaaaggaggcagcccccccagcccggaaccaccccacagacagtagagaagggcccttgtcagcgcaggagtgaggggcgctttccagcactgacccagcgacaaaggtgaaggtgggaaaagccccttgtggacgtggacggtgaaactgagctggcgcctcgggcagtgatgcttgggctggcagagaccagggagagagttctcactggtcataaggccaagctctcaagacacaagacaaacaggaaagaaacacctgcccctgggaggaaagaacccttgagcaccaaaaccaaatttacatgagcgtcccgagccacgcgaatgactttctcccaccaagctgaactgggaagagcaggaacaaggcgtgtttgcctcccaccctcagccgggcactgcagacagacagccagagagcgggctgtggtcagagtcccctctgacctctgctggcttcgtgtcagtctcccggatctcatctgcaggctccagagcaggctgcgtgtcagcagctgagacccaaggcacacacgatggagtaaggagaggagcacacgcgtgtattggacgcagacactccacatttgtgaacctttcctgcacccatcacctcagtaaaccccagggaagcgcgtgggccttgatcccaggtccaggccctctgcccaggcccctcctcagcagggcccggccatgcccgctccacagcagctcaggtcgggttctcgtagctggtgaagctggagagcctctcccgcagggccttgaagcagggtctctgctcggggtccctgcaccagcatgtcagcatcagcttgtgcacgctgggcgggcactccagagggcagggcatgcggtagccggcgtccaccctcaggaaggcctcatggttggacatgcctgggtagggcacctgacccctgctgaacatctcatgcaggagaatcccaaaggaccagacgtcggatttggtggagtaatggcctcgggagagcgcttcaggggccgtccacttgtaggggatattgtggtcatgggagaggtagacgtcctccttgataagcctggctaacccgaagtccccaactttgcagagggtgttttccccgacgaggatgttcctggcggccaggtcccggtggatgtaattctgcgactccaggtaacacatgccctcagccacctgccaggcgatgtccagcagctccgaaacgggcaggactttctcatcagagtcgcggagcagctccagcaggctgcccttggccatgagctccgtgatgatgtacacggggtcccccacggacaccacggcgtacagcgccaggatgtgtttgtgccgcagcttcttcatggcctggatctccgactgcagcatctgctggtgcaggaggttgtctcgagaaatcaccttaatggccacctggacccggtctttccagagcccctcgaagacctccccaaagtagccggaccccagcttcctgcagagcgtgaactcctccctcggcctctcccagtcatcccaatggggcaggggctcaggctcgtgcttccggcagggcgcggccagccgcaggccgtgggacaggctctgggccctgtggtagttcacaagctcgggcaggctgaggaaggacaccgcctcgttcaggtgcagccggcccccggcacgccgccagatcttgtagtgccgcacagcctgcgtgtcccgcaccgacaggacgtagtcggcactcggcttctcgctgaccctgatcaggaaggcgcccgtggcgttgccctcggcctgcagccgacgcacagcttccgagcgggagatgcagccaaagaaccacggttccgactccaccgtctccctctcggccaggtagttgtggggcacatagccctgggccacggccccacccgcctcgtccagcagcgtggcccaccaccactgctcctccttcctggccacgtggaagacgtcccccgcgcggaagctcagctcctcgtccgtccgggacttgaagtcccagaggcccacatacttggggcccaggtgagcctggtcccgggacaccatggcgggcgggcgcagcggcaggaccaggctgtggcccagctggagcacccagagctgggcgt

SEQ ID NO: 14577 - RNA, 2154 nt, Homo sapiens
  source 1..2154: mol_type = other RNA
gctgggattacaggcatgagccaccgtgccccgcctattcttcttttaaaccaaaaaaactttcaggtgagtcaaaaccaaaaccaataagctttttatgacttaaccatggatgaaagagacaccttcaaaatcaggtgcaaaggaggcagcccccccagcccggaaccaccccacagacagtagagaagggcccttgtcagcgcaggagtgaggggcgctttccagcactgacccagcgacaaaggtgaaggtgggaaaagccccttgtggacgtggacggtgaaactgagctggcgcctcgggcagtgatgcttgggctggcagagaccagggagagagttctcactggtcataaggccaagctctcaagacacaagacaaacaggaaagaaacacctgcccctgggaggaaagaacccttgagcaccaaaaccaaatttacatgagcgtcccgagccacgcgaatgactttctcccaccaagctgaactgggaagagcaggaacaaggcgtgtttgcctcccaccctcagccgggcactgcagacagacagccagagagcgggctgtggtcagagtcccctctgacctctgctggcttcgtgtcagtctcccggatctcatctgcaggctccagagcaggctgcgtgtcagcagctgagacccaaggcacacacgatggagtaaggagaggagcacacgcgtgtattggacgcagacactccacatttgtgaacctttcctgcacccatcacctcagtaaaccccagggaagcgcgtgggccttgatcccaggtccaggccctctgcccaggcccctcctcagcagggcccggccatgcccgctccacagcagctcaggtcgggttctcgtagctggtgaagctggagagcctctcccgcagggccttgaagcagggtctctgctcggggtccctgcaccagcatgtcagcatcagcttgtgcacgctgggcgggcactccagagggcagggcatgcggtagccggcgtccaccctcaggaaggcctcatggttggacatgcctgggtagggcacctgacccctgctgaacatctcatgcaggagaatcccaaaggaccagacgtcggatttggtggagtaatggcctcgggagagcgcttcaggggccgtccacttgtaggggatattgtggtcatgggagaggtagacgtcctccttgataagcctggctaacccgaagtccccaactttgcagagggtgttttccccgacgaggatgttcctggcggccaggtcccggtggatgtaattctgcgactccaggtaacacatgccctcagccacctgccaggcgatgtccagcagctccgaaacgggcaggactttctcatcagagtcgcggagcagctccagcaggctgcccttggccatgagctccgtgatgatgtacacggggtcccccacggacaccacggcgtacagcgccaggatgtgtttgtgccgcagcttcttcatggcctggatctccgactgcagcatctgctggtgcaggaggttgtctcgagaaatcaccttaatggccacctggacccggtctttccagagcccctcgaagacctccccaaagtagccggaccccagcttcctgcagagcgtgaactcctccctcggcctctcccagtcatcccaatggggcaggggctcaggctcgtgcttccggcagggcgcggccagccgcaggccgtgggacaggctctgggccctgtggtagttcacaagctcgggcaggctgaggaaggacaccgcctcgttcaggtgcagccggcccccggcacgccgccagatcttgtagtgccgcacagcctgcgtgtcccgcaggttccgactccaccgtctccctctcggccaggtagttgtggggcacatagccctgggccacggccccacccgcctcgtccagcagcgtggcccaccaccactgctcctccttcctggccacgtggaagacgtcccccgcgcggaagctcagctcctcgtccgtccgggacttgaagtcccagaggcccacatacttggggcccaggtgagcctggtcccgggacaccatggcgggcgggcgcagcggcaggaccaggctgtggcccagctggagcacccagagctgggcgt

SEQ ID NO: 14578 - RNA, 2761 nt, Homo sapiens
  source 1..2761: mol_type = other RNA
gctgggattacaggcatgagccaccgtgcccgaccgagttctttttttaatgaaaagaatttgacattcctgcagtagatataaggcagcagaaacaggaactgtgcaggcatgtgtaacaagaatgcagatgccatttatttggtccataagtatagtcgttatttgagttttacaaaacatcgaatataaataacctgaaactgtaacaatacacaaaaattggcttcttacacagacataccaggcggtacaaactgaaaacttgagtaaattaacattgttttacattaatatacatagtgccatctaacatttaaaaacaagtttcaatgcatagcactcgatacttctttgaatctgtttcaatcagttaagagtatgaaaatggttagatctaggctaaaaataattcttcttctagccaaaaataaaggcataatatttataaccaggtatcaactttactaaaccacaatattttgaaactattaatgatacctacgggtatttacattaaaaaggcaacatgcattgtgttgttttatctcatgactggttatgcacacactttgttcaaagggtttttaaaactatattcctactttcaatacagcatactgcaatgtgtctaacagttctagcaaaatgaatgctttcaaagggagcagaatcattttcaagtcactgctgtcaattttttccctttggaacaaaggacataacaatctggttctgcccagataaactaaatagtaagagggttctgtttagaggcatttctgttcaatctaatgctatgacatcatcaagctcttccttctgttctatacgtgacctctttgcactgagattctctttctcatctaatttcctcttgcggcttctctcttcttcactgacgtcggcattatttgaagaatcttcttcatctgaatcaactatgagaacgtcatcttgctcttgagctgtggaggtggagggctgagctccatcatcactgccattggttatgcttttggcagcatcttcagcttgtttgggccccactttttccggggcatcaccaacaacttcaaattcaacgtcctttcctaggtcttcactatgaaggatgttgatcaataaagtatagtcctggaggaagtcatctgcttgaagccggctgccatttctaattccaaattctgacaacttcttgtgattattagcttccgtctctccctcttcggaagatattaggattgttcctttcccatcttcaatttggacatctggtgctaccatagcaaatttttctttcactatcttgtcttgtaaggtgagaacagtcactttatggacattcagccgcacagtcacctctggcttgctggcacatacataacaattggggttgggaggatccagtgcacaaggcacaagaagcttctttcttgggtttggttgtttattcaaaaaaattgttctgcactggtctatttttcctgataaaatcttcaatccttccaatactatcaacccagcaattactgcattagtagtagcaatagcaggaataatgttccctgccattgatttgatatcaaatctactcttcatattcatactgaaaatatgcatcctgaggtttgcagcagaggtgacaaaatccattgcagatgggtcatccttatcccatatgagctcagctccatcccccttttctgctaaatgaactctcaaagtctcgatgctctttgaaaaaagacgtgcatagctctttacatctagaacctgctggtctttcaggcctaactggggttcattctgttgatctgatgcattcgtttcttctccttgactttgtacttcagcccagtccaacggaactggaggtttccttttccgccatagtttgtccattgtcaacagatacctgatgtcatctttaaaaagcttggtaaaaagtttaactggatcatatccagttgatttagcccattccttagtagaaatacgtttaatgtcaccatcttcattagatgctctagctctggcttcggcttccgttggttcccaggcagcttcagggtcagctctgtcaggagatacttcttgatcagcatcttcttccccaaacaactggttgaacaagtactttgcccaaacgatgcaatgtataggttctgaaggtgtgttacgaattgtacagccaggaaaggttctctgggtcggcttaggatgacactcataacactcggtcacaccctttttgatagtagttacttgtccaagatacccagctgttccactttcaataagaggaacatcagctgccaggcacattctattaacatggtttcgggcagctctgttatctaaagcattcataaccagtataaactgtcggaaaaattccacattatagtcagggttcatgatgctgtcatggtaggcaacgatattagctttcgggtaaaactgcagtacactttccttggcaacctgtgcctttgatcttccaacatgtttcttttgaaacaaaaactgtctgttgaggttgcttacatcaatagtatccagatcaatcaggtcgatgtgggagaaaccggtgagcacgagattcttgaggagctcgcagccgatgccgcccgcccccaccaccagcacccggcccccggccaccgcctcagccagctcccggggcagcccccgcgacagtgccatggcgggacaaccacgagccgcggcggaggcggaggcgggagaaccgagccgc

SEQ ID NO: 14579 - RNA, 1523 nt, Homo sapiens
  source 1..1523: mol_type = other RNA
gctgggattacaggcatgagccaccgtgcccgacctctaactattcattatggaaatttcccatatgcataaaaagcagggagagaattacaccatgaacccccatgcactcatcatcccactgcaagaacttgtcaatatttctccaatctcattccagtttccacttttcttttccttcttgctattttaggatattttaaagcaaattccagacacttcatttcacccacatccataacacaccagggtgcattcttgatgtaaggattttgttttgttttataacctccattacattgccacagttaatagatttaacatgaagaaactaagattcttgcaggtggagaaaagatctaattaccaccttaaagtctcccttattagcgcttctcagatctgaacgtgtatgcaaatcacctgagcatcttgttaaaatgcagattctggcccaggaggtccttccgggtgagccctgagagtcttcaattccaaaagctcctaggtgatgcaatgctgagggtccatgaatcacacaagaggaagagtcggccaaacacccacaacaactgggtgcaaagtcctgactgttcctgactgcagggccttcagtgaacggggaagctggggagcatttgggaaagaagggaggtttttcgtatcagctccaggccttgtagaaacatgagcaagagcagtttagggaaacgggtgtcttcaggttctgttttctccatctagaaaagggctgccttcgtggaatgctggtcccagggagaagcctcatttcgcgagggtccgcggcttcattcttgaagtcagtgagaccaagaacccaccagttccggacacgctatgctccacttcggggctcccctgccctgcgtcaactgcactctggcctgggtggcagagagagagaccctatctgatctagcatttgctcctgatgactcagtgcagaaaagctctgtaactcagtttccccagctgttcccattggttttccttgtctcctgcaggcagagagctgatcaaaacagcaaaagcaaagcagtgcccctggcccagttctgaagccaaccttccttaatcacccagacccatccctggttaggacttgctgtggattcttaggtgactccatctcaggatacagggactttttttttctttgtcagatcttgcgctcatttggttctggtgtggaacaacagtttttctcaccgttacatctcccttgtcaggcacatggtaggcgcttaataagtatttttgatgaacgaatggcttgtttggtgacagtccaaaggctgggggacagagggaaagctccctcgtttcgggccccagacgggtggcgctgatggagaggaggttaggataaggcctccaggaccgaagcgcgcacccgtaaggcctctgctaaaaagaccttcctgaaggcggaggaactgcgagagtgcctacgttagcccaagacctgacccgtcgatcccagggaccctcaccctaactgg

SEQ ID NO: 14580 - RNA, 5071 nt, Homo sapiens
  source 1..5071: mol_type = other RNA
gctgggattacaggcatgagccaccgtgcccgattgtttttgttttatgaaattttattctaatctcacatcttctaggcattctgctgggtttacactggcagattctggagactccgttccatcttcaggtagtcataggggtaacctctcacatggccatgactataacctttactattttgaaaatattctagcatttgttcccagaacaactctgtgggagtagatactgttagtcccatatgagcaatctaaggctcagcatcagtgacttacccaacaccacccagctaataagacgccgagccccaaattgaatccagacccgctggctcccactccagtgctctttctactgttgtgaaacccagacccctcaactatcacccttattactaagcactcatttgtgttgatgcagttgttcttgttatttgttcttgttatcctgcaccttcatgttcttgtcaattgtatttgtagccacgtgcttactatgtttccttcctgtgattgggaacttccagaggtgagggatggaattttcctttctctgttggtccctcagaacccaggataggggtctgccaaccaaaggaacggaccctgaggataaaggcaggcaccatggttgtggatctttgccaccttcaagtgcatatggagagtggatgtggacagaaatttgataacagtaagtaacagcagctgctatttgttgagcacttactagatgctgagtgttatgctagttctttatttacattatttaatcctcacaacaaacttctaagggaggtattattattggcaaatgagaaatctaatgctcagagacatggagttaggatgcaaccacatctgtctgactccaaaaggatcacataaatagtagaattcaatttaaaaaatatgtaccgggcgtggtggctcacacctgtaatcccagcactttgggaggccgaggcaggtcgattacctgaggtcaggagttcaagagcagcctggccaacatggtgaaaccctgtctctactaaaaatacaaaaattagttgggcgtggccaggcacggtggctcacgcctgtaatcccagcactttgggagatgaaggcgagtggatcacctaaggtcaggagttcgagaccagcctggccaacatggtgaaaccccgtctctactaaaaatacaaaaattagccgggcgtggtggtaggtgcctataatctcagctactcgggaggctgaggcaggagaattgctggaacccaggtggcgaaggttgcagtgagctgaaatcattccagccctggtgacaatagcgagactctgtctccaaacaaaacaaaacaaaaattagccgggcgtggtggcaggagcctgtaatcccagctactcaggaggctgaggcatgagaatcacttgaacccgggaggcggaggatgcagtgagccgagattgtgccattgcactccagcctgggcgacagagcgagattctgtctcaaaaaaaaaaaagaaagaaagaaagaaaaaaaaaaaaagataatccctcactccctgaaggcccaccctacccttgacttttcttttcccaaaaaataaaattcaggaagaggaaagcagaacaggttgtacctcatacataagcacacacacattttcacacacacacacacgcatacacacaccacttatacctatcaccaccaccctggatttcctagccccagggtgagggctatgaggggtcaggggtcaggttccccaggaccctagtccttgtccccttccctggtgctaaataaaagtgaataaatactaaataaatacaactggggcccaggccctccctgccttccccctccctcctgtgacccgcagggcagagggggcagtttagatggagggctgtctgtcagccccttccatccactaacccatcactgcctcccagggcaggaaaccagggcagggccagcctgcgcattagggcagagaggaggggcaggtctcacgcccacagcccctccccactgagtcttagcatgaggcagcaacagaagctctctctttctcccagctaagtccgaggccccggtgcccagaaagggcagccgggatagtgaggttatttcctgcccgcccaggggcgccgccgaaggatctccagaatctgtgctcttcggtgcagccagtcctggggagtggggcgtggcgttgaaggggtcggccggggcacgaagaagctgtatcggaggcgtgtgtcctgggggttgccagccactaggacttgcagtgtcaaaggctgggccagtggcccatggcctgacagtgtctctgaggctgcagtggccccgctgtagcgcaagctgactgccccaggcagtaccacatctgtgggggagggcatcagcgtgtattcaccattgagggcataggagccatctggcagcttcagggccaagtagatgctccggtggccagggtttccctgctgccggacaagaatgtgggtggcccccgcggggatagtgaccacattgttgtatccgtacctgaatttcctgaaggagcctgactgcttgctgcaaccagaaccgtcccctccgcacaccatgcacttgtcaaacttcttcttggagccaatgatgcgatcacagccagcatggatgcatcggccctggacacagaccgaggagctgtccggggaacagggggtcccatctaccacccgtggctccagcacatagtagtagcccagtgcctgggcctggcaggtgagtttgcactggtcctggggggccacgcctgtgtagcgaggaacccagtccatgggccctgggaagctcttgaagaggtcggtgcggtggttgtaggcagcacactgctcctcgcggaaggtcagggctgagccagttgggcagtcctcagtgttgcaggagcggaagcgggtacggcggccctcacagtacttgccaccattccgggggacaggcctcgtgcagtctcgggaggagaactggacaccacccccacaggtccgagagcagtcaccccatggtccccaaggaccccagccaccagcctgtggaatattgaagtcctggagctggtccatgtggaggcagcgaccacccatgcaggcctgtgcgggcccgcagggtgtgccatcggcccagggcgagtgtttggtctggcacatggcatggccattgaggtggccagagcaccagagggcagcacagggcggcggcagctgtggacaatggcgtgagtcgggcccgaaggtcagctggcactggcggtcagcatcatagtccttgccagggaaagtcacaggcagatgcaatggagcctctggtttgtctaagagacagtgcccatagccattgtccaggaagtcagtgatgaagcgggcactgcagggggaccagggctcctcaggatccacatgagccatcacaggggccatgacatggcgagaggtgctcaaaggcccattcaaactgatgcatggcttggagttgtcatggagcatgttgaagacatgacccagttcatgagcagcagtgaaggctgactggagcccatcatcctccacaatggcacagctccgagccgggtcacagacggtgcccacatcagccatacccagcgtgtcgcaagtggagactccacacaggtcctgacgggtaaacagaatggctgtgtcaaagtggtcagggtccgagtcctcaggggtgttgaggccccgctgccaggcacagaagctgcgcagggtctgggcagcactgggccccacttggggcccctcctcgcctgaccccaggatcactagccgagtcaccaccaagctgacaggattgcggatgcttgggtgcttgaaggccttggctgctgctgccatcactgttagcaggtagcgctttagccccgcaccgtggaatgcggccatcttgtcatctgccaccaccagtgtctccacaaatctactcagtgaagcaaagcgcttggctcttcggggtctggggctggggcttccaagaggagccttgacgttgcacatgggaccttgaccgctggcaggactcttccggcgtaggatgtgagccccaggtcccccagcagagttaggggtgcctccctccaggggctggaggtggagttcagccccccgatattgtaacacgcctaacagggctcccccatcccagtgcagagatgccaccgactccggatctccattgatggtgccagtcaggtaggtgccaggctctgctccacccagcagctcaggcgcctggcccaggtactgcactgtcagcccctcgacctgcacaccggagtcctgctccagctctagtagcagcgtctccccaaaggcctgcaagcggcacaacagcctggcaggggcgcccgagccaggcaggacgctgccgttgagcttctctggaaacacgatctcctcctcccgggggagggggctggccagccgggctgagggcaggagagaggccagcagtagcagaagcagccacaccagccaggagagcggcacaatggggagcaggaggcagggttgggctccccacagccagcgccctgccaagcccctcccgggatgcgagcctgtctgggacatggcactggtactgcagctgggagggactgaggccgtctagggcaccaagtcctccacaccctagctttggaaagctcctctctgtagcctgggggcttggactcctgccaaggtcagaggcaaagttttcagaagggctgaggaccgttaaaggaaatggagaaaacttagtccttgggcttgggagaggtgcccaggggtctggcttctccaaactctcctcctgagccctcctttcctggatctttgtctctccctgcctgtgtcttctgcagcttctctggcctctccctctgtaggactctgtctgggccgcttctgtgcctgccctgtctctgccttcttccgctgtgcctttgtctctgtctctttcctcctctgtctctctcgtgcatatgtgtctgtgggtctccctgtgggttctccc

SEQ ID NO: 14581 - RNA, 93 nt, Homo sapiens
  source 1..93: mol_type = other RNA
gctgggattacaggcatgagccaccgtgcccgcagtcttgggttttcgtaggttcaggatcggcgtatggcgggccagggaggtcttagaaaa

SEQ ID NO: 14582 - RNA, 3549 nt, Homo sapiens
  source 1..3549: mol_type = other RNA
gctgggattacaggcatgagccaccgtgcccggcagtattttttttttaatcatctctttatattatgattcttttagtattataaaatcccccaggaagaaacataaatgctacaagtgcataacagaatgttttgtcatcacatccttgtccttgcctcctcttcatccatttggacatattatgtgttaggtgtagggcaaggccttggaaacacagaggctttttatctgtgtctttgatgagagtatcctgcagttgcagaatcaaaaggcatttacatagatacattatcacctgtgtctatgtaaatatgtaccttttcactttaaatgcccacccaaaaatatattacatcctaactattctgattgtaagaagaaaccattccagaaataaacttgcctacattctcttcacagtgcaacactgcttaaaagtggcacggaaattgcccatggcaaccctaaaaacaaaataaacacaactgtgcttctatgcaactcaacaggcaccggaaaagagagatgtacagtggtagcttcatatatggaattacatgggacagtggagcaaggaggaagcctggcaggtgagctcttagaggcctggcacactgagggtatctttctttttttttttggagacagagtcttgctccgttgcccaggctggagtgcagtggtgtgatctcggctcactgccacctctgccttatagattcaagtgattctcctgccttagcctcccaagtagctgggactataggcacatgccaccatgcccagctaattatttgtattttagtagagacagggtttcaccgtgttgcccaggctggtcttgaactcctgagctcagggaatccgcctgcctcagcctcccaaagtgctaggattacaggcgtgagccactgtgcccgggctgaaggtacctttatctgaggctgtaatgattaaagccaaaggtcaaatgtcacagtcaaggtcaagggagagcagaggtcaaacctgaggtgcaggacaaaagccacttgtcaaagttcaggtcactgaagtaagcattagggctcaggtgcagagtcaaacggggtcagagaagtaggaccgaggaatgtgtgactggcagccccagggcaagtagctccacatggcagggcagtaggtgaggcctcaggggttggggatagtaaggaacattaaggggatgttcattctcaccatgggcttttattgattcccagtgcatatgtatgaagacaacctatgtaggaaggcaagtcatgcccagctaccatgagccagcacaggaaaggcagaaatgagaattgagccctctcctgacaccaaatatactgttattattattattattattattattattattattattattttgagatagagtctcactctgtcgccaggctggagtgcagtggcgtgatctcggctcactgcaatctctgcctcccgggttcaagcaattcccctgtctcagcctcccaagtagctgggactacaggcacgcaacaccatgcccagctaattttttgtattttagtagagacagggtttcaccatattggccaggatggtcttaatctcctgacctcgtgatccgcccgccttggctgctcaaagtgatgggattacaggcgtgagccactgcacctggccatactgttatttttacattaaaatagtgcagctgggtccaggtctctgtagttccactggaggtgatgatatgtctgataattatttctcttaatttcccacaaaagacaaaaagggtgagactacctccatagatccaaccgggcagattaccaagattccaagctcccaggcagggttgctgtgaacagcaggggactttggctttctctcaggccagaaaatgtataaaaataatcagtccattcccaggccattgtagaaacctgccggctactctcatggagtgatccaatcctacctgtagggtcacagtcatggtgcccatgatattcaaagcgcttgtacaataaatgttcccatgaaagatgaatgagaaaggccattttatgaagtactgaggttcccttcacatggtgttcaagtggaggctggaggctcaagtccaaggcattgcagaagacagttcctgctctggttgaaaagattccttcctgctctgagaatctccaactagttgcaaatcatcattgacaaatagaatgtagggaagcgttgtgtcatgagacaagctgtatttaaagtcaactctgataaaacagtccatcaaaagagactgaaagctgacagtctttttggagccaaagaacaaagaacattttgtggctcctctgttgctgccataaatgctcaatcccattactctcatgtatgttgtgggtgtcgtcaggaccttcaagcactaggcttgactctatgggggacagaggataacatggctcctagaggaaggagaactggaaaagagggatctgcaatcatcgatctggtgttggaaggtagatggctccattttgctctcggggccttcttctccagactagaacaccaactccagccagcacaatgacaaggacaatggacccagagacagctttcatcacaagagggatagtttctgattcctgggggacctgaagaaccatgtggacaccgcagtgctccacatgacaggagtaaaggttgctgctctgaggatcaagctcaattgatgcccacgcctgataggttccatccccactgggaagaatgtctccataatcaatttcttggacaatttcttccccgtttttcatccatgtcatgtaaatttctggggggtaaaagccatgagctttgcagaagagagctgtaacccctggaaaagtttctttgcgatttactctgaccagtgggggctctgttctttgtagggtgtctttcccatactccaggaatctctttagccaggcaatacattcttcttccagccaattcttttgatacagcaactcatgctgattggcctcccatgcctgcttgatggtgtgagccacattatctacagccagccaggagagggtgtctttattgaagatcaggaaatcctgcccgtcatatgcatactgcagaaatcctgtggtgcttccatcctccagcagctcacagccaatcattctctggtaagtgtgagaccctgagtgattgtagtgcctctgtaggcgcttcagttccaccttgaacatctgctgccagcccctcagcagctgagtgtacctctcccagtgatcaggcgcgaggttctctgccatccatggggcccgtggctccttctgccgagtgacactgtcatatgtggtgatagggtgcgagtccacgtacccaaccgaaataaattcagggaccccatggatgggatccgaaacgcccaggcgaaaatatctcagagagtgcgtccgggaatcgctgtgcttcaccattaacacaatgatgagaggtaacaggaacgccatcagttcccccatagtccttctctttccgggttctttt

SEQ ID NO: 14583 - RNA, 3723 nt, Homo sapiens
  source 1..3723: mol_type = other RNA
gctgggattacaggcatgagccaccgtgcccggcagtattttttttttaatcatctctttatattatgattcttttagtattataaaatcccccaggaagaaacataaatgctacaagtgcataacagaatgttttgtcatcacatccttgtccttgcctcctcttcatccatttggacatattatgtgttaggtgtagggcaaggccttggaaacacagaggctttttatctgtgtctttgatgagagtatcctgcagttgcagaatcaaaaggcatttacatagatacattatcacctgtgtctatgtaaatatgtaccttttcactttaaatgcccacccaaaaatatattacatcctaactattctgattgtaagaagaaaccattccagaaataaacttgcctacattctcttcacagtgcaacactgcttaaaagtggcacggaaattgcccatggcaaccctaaaaacaaaataaacacaactgtgcttctatgcaactcaacaggcaccggaaaagagagatgtacagtggtagcttcatatatggaattacatgggacagtggagcaaggaggaagcctggcaggtgagctcttagaggcctggcacactgagggtatctttctttttttttttggagacagagtcttgctccgttgcccaggctggagtgcagtggtgtgatctcggctcactgccacctctgccttatagattcaagtgattctcctgccttagcctcccaagtagctgggactataggcacatgccaccatgcccagctaattatttgtattttagtagagacagggtttcaccgtgttgcccaggctggtcttgaactcctgagctcagggaatccgcctgcctcagcctcccaaagtgctaggattacaggcgtgagccactgtgcccgggctgaaggtacctttatctgaggctgtaatgattaaagccaaaggtcaaatgtcacagtcaaggtcaagggagagcagaggtcaaacctgaggtgcaggacaaaagccacttgtcaaagttcaggtcactgaagtaagcattagggctcaggtgcagagtcaaacggggtcagagaagtaggaccgaggaatgtgtgactggcagccccagggcaagtagctccacatggcagggcagtaggtgaggcctcaggggttggggatagtaaggaacattaaggggatgttcattctcaccatgggcttttattgattcccagtgcatatgtatgaagacaacctatgtaggaaggcaagtcatgcccagctaccatgagccagcacaggaaaggcagaaatgagaattgagccctctcctgacaccaaatatactgttattattattattattattattattattattattattattttgagatagagtctcactctgtcgccaggctggagtgcagtggcgtgatctcggctcactgcaatctctgcctcccgggttcaagcaattcccctgtctcagcctcccaagtagctgggactacaggcacgcaacaccatgcccagctaattttttgtattttagtagagacagggtttcaccatattggccaggatggtcttaatctcctgacctcgtgatccgcccgccttggctgctcaaagtgatgggattacaggcgtgagccactgcacctggccatactgttatttttacattaaaatagtgcagctgggtccaggtctctgtagttccactggaggtgatgatatgtctgataattatttctcttaatttcccacaaaagacaaaaagggtgagactacctccatagatccaaccgggcagattaccaagattccaagctcccaggcagggttgctgtgaacagcaggggactttggctttctctcaggccagaaaatgtataaaaataatcagtccattcccaggccattgtagaaacctgccggctactctcatggagtgatccaatcctacctgtagggtcacagtcatggtgcccatgatattcaaagcgcttgtacaataaatgttcccatgaaagatgaatgagaaaggccattttatgaagtactgaggttcccttcacatggtgttcaagtggaggctggaggctcaagtccaaggcattgcagaagacagttcctgctctggttgaaaagattccttcctgctctgagaatctccaactagttgcaaatcatcattgacaaatagaatgtagggaagcgttgtgtcatgagacaagctgtatttaaagtcaactctgataaaacagtccatcaaaagagactgaaagctgacagtctttttggagccaaagaacaaagaacattttgtggctcctctgttgctgccataaatgctcaatcccattactctcatgtatgttgtgggtgtcgtcaggaccttcaagcactaggcttgactctatgggggacagaggataacatggctcctagaggaaggagaactggaaaagagggatctgcaatcatcgatctggtgttggaaggtagatggctccattttgctctcggggccttcttctccagactagaacaccaactccagccagcacaatgacaaggacaatggacccagagacagctttcatcacaagagggatagtttctgattcctgggggacctgaagaaccatgtggacaccgcagtgctccacatgacaggagtaaaggttgctgctctgaggatcaagctcaattgatgcccacgcctgataggttccatccccactgggaagaatgtctccataatcaatttcttggacaatttcttccccgtttttcatccatgtcatgtaaatttctggggggtaaaagccatgagctttgcagaagagagctgtaacccctggaaaagtttctttgcgatttactctgaccagtgggggctctgttctttgtagggtgtctttcccatactccaggaatctctttagccaggcaatacattcttcttccagccaattcttttgatacagcaactcatgctgattggcctcccatgcctgcttgatggtgtgagccacattatctacagccagccaggagagggtgtctttattgaagatcaggaaatcctgcccgtcatatgcatactgcagaaatcctgtggtgcttccatcctccagcagctcacagccaatcattctctggtaagtgtgagaccctgagtgattgtagtgcctctgtaggcgcttcagttccaccttgaacatctgctgccagcccctcagcagctgagtgtacctctcccagtgatcaggcgcgaggttctctgccatccatggggcccgtggctccttctgccgagtgacactgtcatatgtggtgatagggtgcgagtccacgtacccaaccgaaataaattcagggaccccatggatgggatccgaaacgcccaggcgaaaatatctcagagagtgcgtccgggaatcgctgtgcttcaccattaacacaatgatgagaggtaacaggaacgccatcagttcccccatagtccttctctttccgggttcttttaaccaaaaactgacaggtcccttctgagaacctcttggtgacacacaaggccttctcccaataagaacaggggaagatatgcagtgtcatcagttgtgaataaaagaaggcaagagaaaggcctacagaagattctgaggggcagccactcagcttgctcaatcagcaatcccc

SEQ ID NO: 14584 - RNA, 3457 nt, Homo sapiens
  source 1..3457: mol_type = other RNA
gctgggattacaggcatgagccaccgtgcccggcagtattttttttttaatcatctctttatattatgattcttttagtattataaaatcccccaggaagaaacataaatgctacaagtgcataacagaatgttttgtcatcacatccttgtccttgcctcctcttcatccatttggacatattatgtgttaggtgtagggcaaggccttggaaacacagaggctttttatctgtgtctttgatgagagtatcctgcagttgcagaatcaaaaggcatttacatagatacattatcacctgtgtctatgtaaatatgtaccttttcactttaaatgcccacccaaaaatatattacatcctaactattctgattgtaagaagaaaccattccagaaataaacttgcctacattctcttcacagtgcaacactgcttaaaagtggcacggaaattgcccatggcaaccctaaaaacaaaataaacacaactgtgcttctatgcaactcaacaggcaccggaaaagagagatgtacagtggtagcttcatatatggaattacatgggacagtggagcaaggaggaagcctggcaggtgagctcttagaggcctggcacactgagggtatctttctttttttttttggagacagagtcttgctccgttgcccaggctggagtgcagtggtgtgatctcggctcactgccacctctgccttatagattcaagtgattctcctgccttagcctcccaagtagctgggactataggcacatgccaccatgcccagctaattatttgtattttagtagagacagggtttcaccgtgttgcccaggctggtcttgaactcctgagctcagggaatccgcctgcctcagcctcccaaagtgctaggattacaggcgtgagccactgtgcccgggctgaaggtacctttatctgaggctgtaatgattaaagccaaaggtcaaatgtcacagtcaaggtcaagggagagcagaggtcaaacctgaggtgcaggacaaaagccacttgtcaaagttcaggtcactgaagtaagcattagggctcaggtgcagagtcaaacggggtcagagaagtaggaccgaggaatgtgtgactggcagccccagggcaagtagctccacatggcagggcagtaggtgaggcctcaggggttggggatagtaaggaacattaaggggatgttcattctcaccatgggcttttattgattcccagtgcatatgtatgaagacaacctatgtaggaaggcaagtcatgcccagctaccatgagccagcacaggaaaggcagaaatgagaattgagccctctcctgacaccaaatatactgttattattattattattattattattattattattattattttgagatagagtctcactctgtcgccaggctggagtgcagtggcgtgatctcggctcactgcaatctctgcctcccgggttcaagcaattcccctgtctcagcctcccaagtagctgggactacaggcacgcaacaccatgcccagctaattttttgtattttagtagagacagggtttcaccatattggccaggatggtcttaatctcctgacctcgtgatccgcccgccttggctgctcaaagtgatgggattacaggcgtgagccactgcacctggccatactgttatttttacattaaaatagtgcagctgggtccaggtctctgtagttccactggaggtgatgatatgtctgataattatttctcttaatttcccacaaaagacaaaaagggtgagactacctccatagatccaaccgggcagattaccaagattccaagctcccaggcagggttgctgtgaacagcaggggactttggctttctctcaggccagaaaatgtataaaaataatcagtccattcccaggccattgtagaaacctgccggctactctcatggagtgatccaatcctacctgtagggtcacagtcatggtgcccatgatattcaaagcgcttgtacaataaatgttcccatgaaagatgaatgagaaaggccattttatgaagtactgaggttcccttcacatggtgttcaagtggaggctggaggctcaagtccaaggcattgcagaagacagttcctgctctggttgaaaagattccttcctgctctgagaatctccaactagttgcaaatcatcattgacaaatagaatgtagggaagcgttgtgtcatgagacaagctgtatttaaagtcaactctgataaaacagtccatcaaaagagactgaaagctgacagtctttttggagccaaagaacaaagaacattttgtggctcctctgttgctgccataaatgctcaatcccattactctcatgtatgttgtgggtgtcgtcaggaccttcaagcactaggcttgactctatgggggacagaggataacatggctcctagaggaaggagaactggaaaagagggatctgcaatcatcgatctggtgttggaaggtagatggctccattttgctctcggggccttcttctccagactagaacaccaactccagccagcacaatgacaaggacaatggacccagagacagctttcatcacaagagggatagtttctgattcctgggggacctgaagaaccatgtggacaccgcagtgctccacatgacaggagtaaaggttgctgctctgaggatcaagctcaattgatgcccacgcctgataggttccatccccactgggaagaatgtctccataatcaatttcttggacaatttcttccccgtttttcatccatgtcatgtaaatttctggggggtaaaagccatgagctttgcagaagagagctgtaacccctggaaaagtttctttgcgatttactctgaccagtgggggctctgttctttgtagggtgtctttcccatactccaggaatctctttagccaggcaatacattcttcttccagccaattcttttgatacagcaactcatgctgattggcctcccatgcctgcttgatggtgtgagccacattatctacagccagccaggagagggtgtctttattgaagatcaggaaatcctgcccgtcatatgcatactgcagaaatcctgtggtgcttccatcctccagcagctcacagccaatcattctctggtaagtgtgagaccgggaatcgctgtgcttcaccattaacacaatgatgagaggtaacaggaacgccatcagttcccccatagtccttctctttccgggttcttttaaccaaaaactgacaggtcccttctgagaacctcttggtgacacacaaggccttctcccaataagaacaggggaagatatgcagtgtcatcagttgtgaataaaagaaggcaagagaaaggcctacagaagattctgaggggcagccactcagcttgctcaatcagcaa

SEQ ID NO: 14585 - RNA, 3588 nt, Homo sapiens
  source 1..3588: mol_type = other RNA
gctgggattacaggcatgagccaccgtgcccggcagtattttttttttaatcatctctttatattatgattcttttagtattataaaatcccccaggaagaaacataaatgctacaagtgcataacagaatgttttgtcatcacatccttgtccttgcctcctcttcatccatttggacatattatgtgttaggtgtagggcaaggccttggaaacacagaggctttttatctgtgtctttgatgagagtatcctgcagttgcagaatcaaaaggcatttacatagatacattatcacctgtgtctatgtaaatatgtaccttttcactttaaatgcccacccaaaaatatattacatcctaactattctgattgtaagaagaaaccattccagaaataaacttgcctacattctcttcacagtgcaacactgcttaaaagtggcacggaaattgcccatggcaaccctaaaaacaaaataaacacaactgtgcttctatgcaactcaacaggcaccggaaaagagagatgtacagtggtagcttcatatatggaattacatgggacagtggagcaaggaggaagcctggcaggtgagctcttagaggcctggcacactgagggtatctttctttttttttttggagacagagtcttgctccgttgcccaggctggagtgcagtggtgtgatctcggctcactgccacctctgccttatagattcaagtgattctcctgccttagcctcccaagtagctgggactataggcacatgccaccatgcccagctaattatttgtattttagtagagacagggtttcaccgtgttgcccaggctggtcttgaactcctgagctcagggaatccgcctgcctcagcctcccaaagtgctaggattacaggcgtgagccactgtgcccgggctgaaggtacctttatctgaggctgtaatgattaaagccaaaggtcaaatgtcacagtcaaggtcaagggagagcagaggtcaaacctgaggtgcaggacaaaagccacttgtcaaagttcaggtcactgaagtaagcattagggctcaggtgcagagtcaaacggggtcagagaagtaggaccgaggaatgtgtgactggcagccccagggcaagtagctccacatggcagggcagtaggtgaggcctcaggggttggggatagtaaggaacattaaggggatgttcattctcaccatgggcttttattgattcccagtgcatatgtatgaagacaacctatgtaggaaggcaagtcatgcccagctaccatgagccagcacaggaaaggcagaaatgagaattgagccctctcctgacaccaaatatactgttattattattattattattattattattattattattattttgagatagagtctcactctgtcgccaggctggagtgcagtggcgtgatctcggctcactgcaatctctgcctcccgggttcaagcaattcccctgtctcagcctcccaagtagctgggactacaggcacgcaacaccatgcccagctaattttttgtattttagtagagacagggtttcaccatattggccaggatggtcttaatctcctgacctcgtgatccgcccgccttggctgctcaaagtgatgggattacaggcgtgagccactgcacctggccatactgttatttttacattaaaatagtgcagctgggtccaggtctctgtagttccactggaggtgatgatatgtctgataattatttctcttaatttcccacaaaagacaaaaagggtgagactacctccatagatccaaccgggcagattaccaagattccaagctcccaggcagggttgctgtgaacagcaggggactttggctttctctcaggccagaaaatgtataaaaataatcagtccattcccaggccattgtagaaacctgccggctactctcatggagtgatccaatcctacctgtagggtcacagtcatggtgcccatgatattcaaagcgcttgtacaataaatgttcccatgaaagatgaatgagaaaggccattttatgaagtactgaggttcccttcacatggtgttcaagtggaggctggaggctcaagtccaaggcattgcagaagacagttcctgctctggttgaaaagattccttcctgctctgagaatctccaactagttgcaaatcatcattgacaaatagaatgtagggaagcgttgtgtcatgagacaagctgtatttaaagtcaactctgataaaacagtccatcaaaagagactgaaagctgacagtctttttggagccaaagaacaaagaacattttgtggctcctctgttgctgccataaatgctcaatcccattactctcatgtatgttgtgggtgtcgtcaggaccttcaagcactaggcttgactctatgggggacagaggataacatggctcctagaggaaggagaactggaaaagagggatctgcaatcatcgatctggtgttggaaggtagatggctccattttgctctcggggccttcttctccagactagaacaccaactccagccagcacaatgacaaggacaatggacccagagacagctttcatcacaagagggatagtttctgattcctgggggacctgaagaaccatgtggacaccgcagtgctccacatgacaggagtaaaggttgctgctctgaggatcaagctcaattgatgcccacgcctgataggttccatccccactgggaagaatgtctccataatcaatttcttggacaatttcttccccgtttttcatccatgtcatgtaaatttctggggggtaaaagccatgagctttgcagaagagagctgtaacccctggaaaagtttctttgcgatttactctgaccagtgggggctctgttctttgtagggtgtctttcccatactccaggaatctctttagccaggcaatacattcttcttccagccaattcttttgatacagcaactcatgctgattggcctcccatgcctgcttgatggtgtgagccacattatctgagtgattgtagtgcctctgtaggcgcttcagttccaccttgaacatctgctgccagcccctcagcagctgagtgtacctctcccagtgatcaggcgcgaggttctctgccatccatggggcccgtggctccttctgccgagtgacactgtcatatgtggtgatagggtgcgagtccacgtacccaaccgaaataaattcagggaccccatggatgggatccgaaacgcccaggcgaaaatatctcagagagtgcgtccgggaatcgctgtgcttcaccattaacacaatgatgagaggtaacaggaacgccatcagttcccccatagtccttctctttccgggttcttttaaccaaaaactgacaggtcccttctgagaacctcttggtgacacacaaggccttctcccaataagaacaggggaagatatgcagtgtcatcagttgtgaataaaagaaggcaagagaaaggcctacagaagattctgaggggcagccactcagcttgctcaatcagcaatcccc

SEQ ID NO: 14586 - RNA, 3462 nt, Homo sapiens
  source 1..3462: mol_type = other RNA
gctgggattacaggcatgagccaccgtgcccggcagtattttttttttaatcatctctttatattatgattcttttagtattataaaatcccccaggaagaaacataaatgctacaagtgcataacagaatgttttgtcatcacatccttgtccttgcctcctcttcatccatttggacatattatgtgttaggtgtagggcaaggccttggaaacacagaggctttttatctgtgtctttgatgagagtatcctgcagttgcagaatcaaaaggcatttacatagatacattatcacctgtgtctatgtaaatatgtaccttttcactttaaatgcccacccaaaaatatattacatcctaactattctgattgtaagaagaaaccattccagaaataaacttgcctacattctcttcacagtgcaacactgcttaaaagtggcacggaaattgcccatggcaaccctaaaaacaaaataaacacaactgtgcttctatgcaactcaacaggcaccggaaaagagagatgtacagtggtagcttcatatatggaattacatgggacagtggagcaaggaggaagcctggcaggtgagctcttagaggcctggcacactgagggtatctttctttttttttttggagacagagtcttgctccgttgcccaggctggagtgcagtggtgtgatctcggctcactgccacctctgccttatagattcaagtgattctcctgccttagcctcccaagtagctgggactataggcacatgccaccatgcccagctaattatttgtattttagtagagacagggtttcaccgtgttgcccaggctggtcttgaactcctgagctcagggaatccgcctgcctcagcctcccaaagtgctaggattacaggcgtgagccactgtgcccgggctgaaggtacctttatctgaggctgtaatgattaaagccaaaggtcaaatgtcacagtcaaggtcaagggagagcagaggtcaaacctgaggtgcaggacaaaagccacttgtcaaagttcaggtcactgaagtaagcattagggctcaggtgcagagtcaaacggggtcagagaagtaggaccgaggaatgtgtgactggcagccccagggcaagtagctccacatggcagggcagtaggtgaggcctcaggggttggggatagtaaggaacattaaggggatgttcattctcaccatgggcttttattgattcccagtgcatatgtatgaagacaacctatgtaggaaggcaagtcatgcccagctaccatgagccagcacaggaaaggcagaaatgagaattgagccctctcctgacaccaaatatactgttattattattattattattattattattattattattattttgagatagagtctcactctgtcgccaggctggagtgcagtggcgtgatctcggctcactgcaatctctgcctcccgggttcaagcaattcccctgtctcagcctcccaagtagctgggactacaggcacgcaacaccatgcccagctaattttttgtattttagtagagacagggtttcaccatattggccaggatggtcttaatctcctgacctcgtgatccgcccgccttggctgctcaaagtgatgggattacaggcgtgagccactgcacctggccatactgttatttttacattaaaatagtgcagctgggtccaggtctctgtagttccactggaggtgatgatatgtctgataattatttctcttaatttcccacaaaagacaaaaagggtgagactacctccatagatccaaccgggcagattaccaagattccaagctcccaggcagggttgctgtgaacagcaggggactttggctttctctcaggccagaaaatgtataaaaataatcagtccattcccaggccattgtagaaacctgccggctactctcatggagtgatccaatcctacctgtagggtcacagtcatggtgcccatgatattcaaagcgcttgtacaataaatgttcccatgaaagatgaatgagaaaggccattttatgaagtactgaggttcccttcacatggtgttcaagtggaggctggaggctcaagtccaaggcattgcagaagacagttcctgctctggttgaaaagattccttcctgctctgagaatctccaactagttgcaaatcatcattgacaaatagaatgtagggaagcgttgtgtcatgagacaagctgtatttaaagtcaactctgataaaacagtccatcaaaagagactgaaagctgacagtctttttggagccaaagaacaaagaacattttgtggctcctctgttgctgccataaatgctcaatcccattactctcatgtatgttgtgggtgtcgtcaggaccttcaagcactaggcttgactctatgggggacagaggataacatggctcctagaggaaggagaactggaaaagagggatctgcaatcatcgatctggtgttggaaggtagatggctccattttgctctcggggccttcttctccagactagaacaccaactccagccagcacaatgacaaggacaatggacccagagacagctttcatcacaagagggatagtttctgattcctgggggacctgaagaaccatgtggacaccgcagtgctccacatgacaggagtaaaggttgctgctctgaggatcaagctcaattgatgcccacgcctgataggttccatccccactgggaagaatgtctccataatcaatttcttggacaatttcttccccgtttttcatccatgtcatgtaaatttctgttctttgtagggtgtctttcccatactccaggaatctctttagccaggcaatacattcttcttccagccaattcttttgatacagcaactcatgctgattggcctcccatgcctgcttgatggtgtgagccacattatctacagccagccaggagagggtgtctttattgaagatcaggaaatcctgcccgtcatatgcatactgcagaaatcctgtggtgcttccatcctccagcagctcacagccaatcattctctggtaagtgtgagaccctgagtgattgtagtgcctctgtaggcgcttcagttccaccttgaacatctgctgccagcccctcagcagctgagtgtacctctcccagtgatcaggcgcgaggttctctgccatccatggggcccgtggctccttctgccgagtgacactgtcatatgtggtgatagggtgcgagtccacgtacccaaccgaaataaattcagggaccccatggatgggatccgaaacgcccaggcgaaaatatctcagagagtgcgtccgggaatcgctgtgcttcaccattaacacaatgatgagaggtaacaggaacgccatcagttcccccatagtccttctctttccgggttctttt

SEQ ID NO: 14587 - RNA, 3563 nt, Homo sapiens
  source 1..3563: mol_type = other RNA
gctgggattacaggcatgagccaccgtgcccggcagtattttttttttaatcatctctttatattatgattcttttagtattataaaatcccccaggaagaaacataaatgctacaagtgcataacagaatgttttgtcatcacatccttgtccttgcctcctcttcatccatttggacatattatgtgttaggtgtagggcaaggccttggaaacacagaggctttttatctgtgtctttgatgagagtatcctgcagttgcagaatcaaaaggcatttacatagatacattatcacctgtgtctatgtaaatatgtaccttttcactttaaatgcccacccaaaaatatattacatcctaactattctgattgtaagaagaaaccattccagaaataaacttgcctacattctcttcacagtgcaacactgcttaaaagtggcacggaaattgcccatggcaaccctaaaaacaaaataaacacaactgtgcttctatgcaactcaacaggcaccggaaaagagagatgtacagtggtagcttcatatatggaattacatgggacagtggagcaaggaggaagcctggcaggtgagctcttagaggcctggcacactgagggtatctttctttttttttttggagacagagtcttgctccgttgcccaggctggagtgcagtggtgtgatctcggctcactgccacctctgccttatagattcaagtgattctcctgccttagcctcccaagtagctgggactataggcacatgccaccatgcccagctaattatttgtattttagtagagacagggtttcaccgtgttgcccaggctggtcttgaactcctgagctcagggaatccgcctgcctcagcctcccaaagtgctaggattacaggcgtgagccactgtgcccgggctgaaggtacctttatctgaggctgtaatgattaaagccaaaggtcaaatgtcacagtcaaggtcaagggagagcagaggtcaaacctgaggtgcaggacaaaagccacttgtcaaagttcaggtcactgaagtaagcattagggctcaggtgcagagtcaaacggggtcagagaagtaggaccgaggaatgtgtgactggcagccccagggcaagtagctccacatggcagggcagtaggtgaggcctcaggggttggggatagtaaggaacattaaggggatgttcattctcaccatgggcttttattgattcccagtgcatatgtatgaagacaacctatgtaggaaggcaagtcatgcccagctaccatgagccagcacaggaaaggcagaaatgagaattgagccctctcctgacaccaaatatactgttattattattattattattattattattattattattattttgagatagagtctcactctgtcgccaggctggagtgcagtggcgtgatctcggctcactgcaatctctgcctcccgggttcaagcaattcccctgtctcagcctcccaagtagctgggactacaggcacgcaacaccatgcccagctaattttttgtattttagtagagacagggtttcaccatattggccaggatggtcttaatctcctgacctcgtgatccgcccgccttggctgctcaaagtgatgggattacaggcgtgagccactgcacctggccatactgttatttttacattaaaatagtgcagctgggtccaggtctctgtagttccactggaggtgatgatatgtctgataattatttctcttaatttcccacaaaagacaaaaagggtgagactacctccatagatccaaccgggcagattaccaagattccaagctcccaggcagggttgctgtgaacagcaggggactttggctttctctcaggccagaaaatgtataaaaataatcagtccattcccaggccattgtagaaacctgccggctactctcatggagtgatccaatcctacctgtagggtcacagtcatggtgcccatgatattcaaagcgcttgtacaataaatgttcccatgaaagatgaatgagaaaggccattttatgaagtactgaggttcccttcacatggtgttcaagtggaggctggaggctcaagtccaaggcattgcagaagacagttcctgctctggttgaaaagattccttcctgctctgagaatctccaactagttgcaaatcatcattgacaaatagaatgtagggaagcgttgtgtcatgagacaagctgtatttaaagtcaactctgataaaacagtccatcaaaagagactgaaagctgacagtctttttggagccaaagaacaaagaacattttgtggctcctctgttgctgccataaatgctcaatcccattactctcatgtatgttgtgggtgtcgtcaggaccttcaagcactaggcttgactctatgggggacagaggataacatggctcctagaggaaggagaactggaaaagagggatctgcaatcatcgatctggtgttggaaggtagatggctccattttgctctcggggccttcttctccagactagaacaccaactccagccagcacaatgacaaggacaatggacccagagacagctttcatcacaagagggatagtttctgattctgttctttgtagggtgtctttcccatactccaggaatctctttagccaggcaatacattcttcttccagccaattcttttgatacagcaactcatgctgattggcctcccatgcctgcttgatggtgtgagccacattatctacagccagccaggagagggtgtctttattgaagatcaggaaatcctgcccgtcatatgcatactgcagaaatcctgtggtgcttccatcctccagcagctcacagccaatcattctctggtaagtgtgagaccctgagtgattgtagtgcctctgtaggcgcttcagttccaccttgaacatctgctgccagcccctcagcagctgagtgtacctctcccagtgatcaggcgcgaggttctctgccatccatggggcccgtggctccttctgccgagtgacactgtcatatgtggtgatagggtgcgagtccacgtacccaaccgaaataaattcagggaccccatggatgggatccgaaacgcccaggcgaaaatatctcagagagtgcgtcccttggttatgtcgagatgaaacatacaaatcacatatggcaatgcatgagaaatctcatgccagcccccagtctgattacacccacccatatcgccaattcacagtttcacacagggggaatcgctgtgcttcaccattaacacaatgatgagaggtaacaggaacgccatcagttcccccatagtccttctctttccgggttcttttaaccaaaaactgacaggtcccttctgagaacctcttggtgacacacaaggccttctcccaataagaacaggggaagatatgcagtgtcatcagttgtgaataaaagaaggcaagagaaaggcctacagaagattctgaggggcagccactcagcttgctcaatcagcaatcccc

SEQ ID NO: 14588 - RNA, 3273 nt, Homo sapiens
  source 1..3273: mol_type = other RNA
gctgggattacaggcatgagccaccgtgcccggcagtattttttttttaatcatctctttatattatgattcttttagtattataaaatcccccaggaagaaacataaatgctacaagtgcataacagaatgttttgtcatcacatccttgtccttgcctcctcttcatccatttggacatattatgtgttaggtgtagggcaaggccttggaaacacagaggctttttatctgtgtctttgatgagagtatcctgcagttgcagaatcaaaaggcatttacatagatacattatcacctgtgtctatgtaaatatgtaccttttcactttaaatgcccacccaaaaatatattacatcctaactattctgattgtaagaagaaaccattccagaaataaacttgcctacattctcttcacagtgcaacactgcttaaaagtggcacggaaattgcccatggcaaccctaaaaacaaaataaacacaactgtgcttctatgcaactcaacaggcaccggaaaagagagatgtacagtggtagcttcatatatggaattacatgggacagtggagcaaggaggaagcctggcaggtgagctcttagaggcctggcacactgagggtatctttctttttttttttggagacagagtcttgctccgttgcccaggctggagtgcagtggtgtgatctcggctcactgccacctctgccttatagattcaagtgattctcctgccttagcctcccaagtagctgggactataggcacatgccaccatgcccagctaattatttgtattttagtagagacagggtttcaccgtgttgcccaggctggtcttgaactcctgagctcagggaatccgcctgcctcagcctcccaaagtgctaggattacaggcgtgagccactgtgcccgggctgaaggtacctttatctgaggctgtaatgattaaagccaaaggtcaaatgtcacagtcaaggtcaagggagagcagaggtcaaacctgaggtgcaggacaaaagccacttgtcaaagttcaggtcactgaagtaagcattagggctcaggtgcagagtcaaacggggtcagagaagtaggaccgaggaatgtgtgactggcagccccagggcaagtagctccacatggcagggcagtaggtgaggcctcaggggttggggatagtaaggaacattaaggggatgttcattctcaccatgggcttttattgattcccagtgcatatgtatgaagacaacctatgtaggaaggcaagtcatgcccagctaccatgagccagcacaggaaaggcagaaatgagaattgagccctctcctgacaccaaatatactgttattattattattattattattattattattattattattttgagatagagtctcactctgtcgccaggctggagtgcagtggcgtgatctcggctcactgcaatctctgcctcccgggttcaagcaattcccctgtctcagcctcccaagtagctgggactacaggcacgcaacaccatgcccagctaattttttgtattttagtagagacagggtttcaccatattggccaggatggtcttaatctcctgacctcgtgatccgcccgccttggctgctcaaagtgatgggattacaggcgtgagccactgcacctggccatactgttatttttacattaaaatagtgcagctgggtccaggtctctgtagttccactggaggtgatgatatgtctgataattatttctcttaatttcccacaaaagacaaaaagggtgagactacctccatagatccaaccgggcagattaccaagattccaagctcccaggcagggttgctgtgaacagcaggggactttggctttctctcaggccagaaaatgtataaaaataatcagtccattcccaggccattgtagaaacctgccggctactctcatggagtgatccaatcctacctgtagggtcacagtcatggtgcccatgatattcaaagcgcttgtacaataaatgttcccatgaaagatgaatgagaaaggccattttatgaagtactgaggttcccttcacatggtgttcaagtggaggctggaggctcaagtccaaggcattgcagaagacagttcctgctctggttgaaaagattccttcctgctctgagaatctccaactagttgcaaatcatcattgacaaatagaatgtagggaagcgttgtgtcatgagacaagctgtatttaaagtcaactctgataaaacagtccatcaaaagagactgaaagctgacagtctttttggagccaaagaacaaagaacattttgtggctcctctgttgctgccataaatgctcaatcccattactctcatgtatgttgtgggtgtcgtcaggaccttcaagcactaggcttgactctatgggggacagaggataacatggctcctagaggaaggagaactggaaaagagggatctgcaatcatcgatctggtgttggaaggtagatggctccattttgctctcggggccttcttctccagactagaacaccaactccagccagcacaatgacaaggacaatggacccagagacagctttcatcacaagagggatagtttctgattctgttctttgtagggtgtctttcccatactccaggaatctctttagccaggcaatacattcttcttccagccaattcttttgatacagcaactcatgctgattggcctcccatgcctgcttgatggtgtgagccacattatctacagccagccaggagagggtgtctttattgaagatcaggaaatcctgcccgtcatatgcatactgcagaaatcctgtggtgcttccatcctccagcagctcacagccaatcattctctggtaagtgtgagaccctgagtgattgtagtgcctctgtaggcgcttcagttccaccttgaacatctgctgccagcccctcagcagctgagtgtacctctcccagtgatcaggcgcgaggttctctgccatccatggggcccgtggctccttctgccgagtgacactgtcatatgtggtgatagggtgcgagtccacgtacccaaccgaaataaattcagggaccccatggatgggatccgaaacgcccaggcgaaaatatctcagagagtgcgtccgggaatcgctgtgcttcaccattaacacaatgatgagaggtaacaggaacgccatcagttcccccatagtccttctctttccgggttctttt

SEQ ID NO: 14589 - RNA, 3447 nt, Homo sapiens
  source 1..3447: mol_type = other RNA
gctgggattacaggcatgagccaccgtgcccggcagtattttttttttaatcatctctttatattatgattcttttagtattataaaatcccccaggaagaaacataaatgctacaagtgcataacagaatgttttgtcatcacatccttgtccttgcctcctcttcatccatttggacatattatgtgttaggtgtagggcaaggccttggaaacacagaggctttttatctgtgtctttgatgagagtatcctgcagttgcagaatcaaaaggcatttacatagatacattatcacctgtgtctatgtaaatatgtaccttttcactttaaatgcccacccaaaaatatattacatcctaactattctgattgtaagaagaaaccattccagaaataaacttgcctacattctcttcacagtgcaacactgcttaaaagtggcacggaaattgcccatggcaaccctaaaaacaaaataaacacaactgtgcttctatgcaactcaacaggcaccggaaaagagagatgtacagtggtagcttcatatatggaattacatgggacagtggagcaaggaggaagcctggcaggtgagctcttagaggcctggcacactgagggtatctttctttttttttttggagacagagtcttgctccgttgcccaggctggagtgcagtggtgtgatctcggctcactgccacctctgccttatagattcaagtgattctcctgccttagcctcccaagtagctgggactataggcacatgccaccatgcccagctaattatttgtattttagtagagacagggtttcaccgtgttgcccaggctggtcttgaactcctgagctcagggaatccgcctgcctcagcctcccaaagtgctaggattacaggcgtgagccactgtgcccgggctgaaggtacctttatctgaggctgtaatgattaaagccaaaggtcaaatgtcacagtcaaggtcaagggagagcagaggtcaaacctgaggtgcaggacaaaagccacttgtcaaagttcaggtcactgaagtaagcattagggctcaggtgcagagtcaaacggggtcagagaagtaggaccgaggaatgtgtgactggcagccccagggcaagtagctccacatggcagggcagtaggtgaggcctcaggggttggggatagtaaggaacattaaggggatgttcattctcaccatgggcttttattgattcccagtgcatatgtatgaagacaacctatgtaggaaggcaagtcatgcccagctaccatgagccagcacaggaaaggcagaaatgagaattgagccctctcctgacaccaaatatactgttattattattattattattattattattattattattattttgagatagagtctcactctgtcgccaggctggagtgcagtggcgtgatctcggctcactgcaatctctgcctcccgggttcaagcaattcccctgtctcagcctcccaagtagctgggactacaggcacgcaacaccatgcccagctaattttttgtattttagtagagacagggtttcaccatattggccaggatggtcttaatctcctgacctcgtgatccgcccgccttggctgctcaaagtgatgggattacaggcgtgagccactgcacctggccatactgttatttttacattaaaatagtgcagctgggtccaggtctctgtagttccactggaggtgatgatatgtctgataattatttctcttaatttcccacaaaagacaaaaagggtgagactacctccatagatccaaccgggcagattaccaagattccaagctcccaggcagggttgctgtgaacagcaggggactttggctttctctcaggccagaaaatgtataaaaataatcagtccattcccaggccattgtagaaacctgccggctactctcatggagtgatccaatcctacctgtagggtcacagtcatggtgcccatgatattcaaagcgcttgtacaataaatgttcccatgaaagatgaatgagaaaggccattttatgaagtactgaggttcccttcacatggtgttcaagtggaggctggaggctcaagtccaaggcattgcagaagacagttcctgctctggttgaaaagattccttcctgctctgagaatctccaactagttgcaaatcatcattgacaaatagaatgtagggaagcgttgtgtcatgagacaagctgtatttaaagtcaactctgataaaacagtccatcaaaagagactgaaagctgacagtctttttggagccaaagaacaaagaacattttgtggctcctctgttgctgccataaatgctcaatcccattactctcatgtatgttgtgggtgtcgtcaggaccttcaagcactaggcttgactctatgggggacagaggataacatggctcctagaggaaggagaactggaaaagagggatctgcaatcatcgatctggtgttggaaggtagatggctccattttgctctcggggccttcttctccagactagaacaccaactccagccagcacaatgacaaggacaatggacccagagacagctttcatcacaagagggatagtttctgattctgttctttgtagggtgtctttcccatactccaggaatctctttagccaggcaatacattcttcttccagccaattcttttgatacagcaactcatgctgattggcctcccatgcctgcttgatggtgtgagccacattatctacagccagccaggagagggtgtctttattgaagatcaggaaatcctgcccgtcatatgcatactgcagaaatcctgtggtgcttccatcctccagcagctcacagccaatcattctctggtaagtgtgagaccctgagtgattgtagtgcctctgtaggcgcttcagttccaccttgaacatctgctgccagcccctcagcagctgagtgtacctctcccagtgatcaggcgcgaggttctctgccatccatggggcccgtggctccttctgccgagtgacactgtcatatgtggtgatagggtgcgagtccacgtacccaaccgaaataaattcagggaccccatggatgggatccgaaacgcccaggcgaaaatatctcagagagtgcgtccgggaatcgctgtgcttcaccattaacacaatgatgagaggtaacaggaacgccatcagttcccccatagtccttctctttccgggttcttttaaccaaaaactgacaggtcccttctgagaacctcttggtgacacacaaggccttctcccaataagaacaggggaagatatgcagtgtcatcagttgtgaataaaagaaggcaagagaaaggcctacagaagattctgaggggcagccactcagcttgctcaatcagcaatcccc

SEQ ID NO: 14590 - RNA, 3342 nt, Homo sapiens
  source 1..3342: mol_type = other RNA
gctgggattacaggcatgagccaccgtgcccggcagtattttttttttaatcatctctttatattatgattcttttagtattataaaatcccccaggaagaaacataaatgctacaagtgcataacagaatgttttgtcatcacatccttgtccttgcctcctcttcatccatttggacatattatgtgttaggtgtagggcaaggccttggaaacacagaggctttttatctgtgtctttgatgagagtatcctgcagttgcagaatcaaaaggcatttacatagatacattatcacctgtgtctatgtaaatatgtaccttttcactttaaatgcccacccaaaaatatattacatcctaactattctgattgtaagaagaaaccattccagaaataaacttgcctacattctcttcacagtgcaacactgcttaaaagtggcacggaaattgcccatggcaaccctaaaaacaaaataaacacaactgtgcttctatgcaactcaacaggcaccggaaaagagagatgtacagtggtagcttcatatatggaattacatgggacagtggagcaaggaggaagcctggcaggtgagctcttagaggcctggcacactgagggtatctttctttttttttttggagacagagtcttgctccgttgcccaggctggagtgcagtggtgtgatctcggctcactgccacctctgccttatagattcaagtgattctcctgccttagcctcccaagtagctgggactataggcacatgccaccatgcccagctaattatttgtattttagtagagacagggtttcaccgtgttgcccaggctggtcttgaactcctgagctcagggaatccgcctgcctcagcctcccaaagtgctaggattacaggcgtgagccactgtgcccgggctgaaggtacctttatctgaggctgtaatgattaaagccaaaggtcaaatgtcacagtcaaggtcaagggagagcagaggtcaaacctgaggtgcaggacaaaagccacttgtcaaagttcaggtcactgaagtaagcattagggctcaggtgcagagtcaaacggggtcagagaagtaggaccgaggaatgtgtgactggcagccccagggcaagtagctccacatggcagggcagtaggtgaggcctcaggggttggggatagtaaggaacattaaggggatgttcattctcaccatgggcttttattgattcccagtgcatatgtatgaagacaacctatgtaggaaggcaagtcatgcccagctaccatgagccagcacaggaaaggcagaaatgagaattgagccctctcctgacaccaaatatactgttattattattattattattattattattattattattattttgagatagagtctcactctgtcgccaggctggagtgcagtggcgtgatctcggctcactgcaatctctgcctcccgggttcaagcaattcccctgtctcagcctcccaagtagctgggactacaggcacgcaacaccatgcccagctaattttttgtattttagtagagacagggtttcaccatattggccaggatggtcttaatctcctgacctcgtgatccgcccgccttggctgctcaaagtgatgggattacaggcgtgagccactgcacctggccatactgttatttttacattaaaatagtgcagctgggtccaggtctctgtagttccactggaggtgatgatatgtctgataattatttctcttaatttcccacaaaagacaaaaagggtgagactacctccatagatccaaccgggcagattaccaagattccaagctcccaggcagggttgctgtgaacagcaggggactttggctttctctcaggccagaaaatgtataaaaataatcagtccattcccaggccattgtagaaacctgccggctactctcatggagtgatccaatcctacctgtagggtcacagtcatggtgcccatgatattcaaagcgcttgtacaataaatgttcccatgaaagatgaatgagaaaggccattttatgaagtactgaggttcccttcacatggtgttcaagtggaggctggaggctcaagtccaaggcattgcagaagacagttcctgctctggttgaaaagattccttcctgctctgagaatctccaactagttgcaaatcatcattgacaaatagaatgtagggaagcgttgtgtcatgagacaagctgtatttaaagtcaactctgataaaacagtccatcaaaagagactgaaagctgacagtctttttggagccaaagaacaaagaacattttgtggctcctctgttgctgccataaatgctcaatcccattactctcatgtatgttgtgggtgtcgtcaggaccttcaagcactaggcttgactctatgggggacagaggataacatggctcctagaggaaggagaactggaaaagagggatctgcaatcatcgatctggtgttggaaggtagatggctccattttgctctgttctttgtagggtgtctttcccatactccaggaatctctttagccaggcaatacattcttcttccagccaattcttttgatacagcaactcatgctgattggcctcccatgcctgcttgatggtgtgagccacattatctacagccagccaggagagggtgtctttattgaagatcaggaaatcctgcccgtcatatgcatactgcagaaatcctgtggtgcttccatcctccagcagctcacagccaatcattctctggtaagtgtgagaccctgagtgattgtagtgcctctgtaggcgcttcagttccaccttgaacatctgctgccagcccctcagcagctgagtgtacctctcccagtgatcaggcgcgaggttctctgccatccatggggcccgtggctccttctgccgagtgacactgtcatatgtggtgatagggtgcgagtccacgtacccaaccgaaataaattcagggaccccatggatgggatccgaaacgcccaggcgaaaatatctcagagagtgcgtccgggaatcgctgtgcttcaccattaacacaatgatgagaggtaacaggaacgccatcagttcccccatagtccttctctttccgggttcttttaaccaaaaactgacaggtcccttctgagaacctcttggtgacacacaaggccttctcccaataagaacaggggaagatatgcagtgtcatcagttgtgaataaaagaaggcaagagaaaggcctacagaagattctgaggggcagccactcagcttgctcaatcagcaatcccc

SEQ ID NO: 14591 - RNA, 1066 nt, Homo sapiens
  source 1..1066: mol_type = other RNA
gctgggattacaggcatgagccaccgtgcccggccaagaaattcctttctgatgcacgcttaaccatttgagcagggaagaggcgattccttgtccctacgcattttgcacttccttctcatcatacacaagagaatgcagtttttgtaatataagaagggggttgttcttttagcttcacctgtttcaggtgcttctttagtaactgccatcatgtcaaaaatattaagtcttttccctgtgaatatatttttcctttttttaagatcatccgtcttctcctggccaggataattgtcatagccttcatcaaactgaatccgaagctctggtcttgaacgaactctagctgtagcagatctggcaactttcatatctgatattatgttactgaaactaattttaggtcgctttgcatctctctgtgcccttgactcttcctcatgctgctggagctggctcagcagctctgacttggttgtttgcttatcaaaagggagagaatctgccacagcagatgcagctgccaccaactcaggactcaggggctcaattctcttctttggagcatattctgtagctcttcgaagcctgccaagtgtagcttccaaacttttaagtggtcttcttttggggggctttgttgttcgtacatttactgtgcttaattcaactttcatgcccttaataatgcctaacaagtcttttttcgtattttccttttcactgtcttggctctctgaagtctccttggaagtctcctcagttcgaacagactgcttatctttcttgctacagatcacactgttagtgccaaaatatctttggatgttattttttgtccgggccaacagcgctgaactgcggtacctgactgttccgtgccgaacagtgagtagcataatcgcagccgctgatgtctccgggcttccagaggacaaagggtggcgggaaagggggcgaagaggtaggaacgtcgagactctaggaaacatcgccgagacacgaaatgaaccaagaacacaactgaaatggtgcgtcccgctgccaaacacgtccccgccct

SEQ ID NO: 14592 - RNA, 7932 nt, Homo sapiens
  source 1..7932: mol_type = other RNA
gctgggattacaggcatgagccaccgtgcccggccactttctttctttctttttttttttttttaaaaaaacaaaacaactttgggttttatttaaaatgcccgtggaggtggttagcgccccattcttctgctgtagttatttcaccccgggagggtgtgggccttagccatgtggccgtgatggtcgtatctgaagtgtgaatacttccccgcgctatcttctaacctgcgctgtctcagcttagtgtgaacgtacggaccgttctcaaatcctggtgaagtcactggcagttttttcctgcacacagagtagctgtgctgtttttgagctgagggcagtgtcatgctgggctgcatctggcacatggagaggacgggccagtcgagcaggtggcctcctggccgctcacagactctgcgcccgccagactgtgagaggggttcaggcacgacacttccggagctgtcatctggaggagattctcatcattttttccaccacttaaaataaaaccactcaatgccttctccagtgtactctctggtctatttaaaaatagcagcgcaagtcccaccacttcttatttataaagggaacagccagtgaacatatttttacctcccgtgtctgtcatcatgttcttgccactcattgcctccaattccaaataggtaaagagtgagggccgtgccgctgtgcctggagtggcaggggcagccacacagacctgggggtccctgagctcccccagctccagggaggacgccccaggcatgagcaggggccgccaacaggacaaagaggccactctgtcagcctctgctggacccctgagctcccctctcatgggcctctccgtttgggtggctccgagaggccaactccagccccaactgcaggctcccaggactgcaggggcagggactctggaggtccgtgtgcttcgtgagagaggggaccctgtcctcctagcaggggtccagcggcaccacagcaagacttctgtggccaagtacacgccatgctcagctctgcccccacccgcacccccggaccatcctgtgtgcagctgggctgccccgggacccacacgcgcgaggggcacccggtgctcaggagcctccacacacagcagctcgcacttagaacccacacgccaagcagaaacccctcgaagcgggctgggagcacggacccctgatttatagaggaggccccgggggccctgtcgggggagctgtggggaccggccccccagagctcagcacagcccggccctccttccagacaccagcactcgcatgtcccagcaggtgagggtgggtcaaacctgctggatctgaagttaattgttcgactggaaggaaacctgtgcgctccccggagcatgacgccacgccgcctccttggcgctgcagagccaaagccactggcgtctgccgggatggaccttccctggaaggagagacctcagccccgcgtgggtaggacgcgcctgctgaacgccctctcagggccgacactggaaaacaccttcctctaaaggaacatccgagtcagaaaacaggtgctcgcagcaggcaccaaagcgcctttgcgaacgcttagggctgtttcaggaaaccgctcagtagcaaaggcagaagatgccaagacaccttcaaaaagcaggaattaactttccacagggagggcaccaccaaaaacaagggtgcggggctgtagggcgacaggctgcatcggttcacgctgaaaatccagctgctccggggccactcaggcagccgtgtggcctcacgggtccgggtttcagaggccaccgagtggcctgggacgatggatcgcgacacggaggtgcatggctccatcatggggaagaatgtgctttaaaataggtgcatggaggaagagcctaaaaaatagtccagagtagcaacaaaaaccatctcgaggcaatgtgaccacaggtggctttgatttccttcttgtgcctctagacagcattcaaatattccagcctgaacatgcattacctcagtacctgaacagggccggagtcgtgggccgtctcgggccagggcaggaaacacttctatgctgttcgggaggacggaggacagacagcgaggctctcaggtcaccggcaccagtggcaccacccacagggactgcagggaagggcgggcaggctcccgttcgttctcccagcacccagtttccagacgaagcctccctgggatcctggcttcccacggctctgcactgtccctttctcagaacttaacgtgggcatttcctgaggcctcttcctccggatgagctggtttcggcctgggatcccagcgtccccacaccctctggtgaccaccacatggcccagcagccacacagcacccggcacccacctgggcgtctgaggctggaggaagctctgccctttctttcgagtcatgggggtggggcggtgtgcatcactttgggcccatggatggtgggtgccatgcggccacgtcagagcagggcatggtggggtgtgggcagggagcagtgggaggtggccctgtgagagctggggaggtgtcccaaagtgccagcatcctgcagatcgaaggggacgcacacaccgtgccactgcgggaggtgtgagctccacgctgcaggctgtgtgagagaggggtgagccggcgcccccgagtgaagacacaaagaatcccgagggcctggtgaggccacaggcccgcacctcccacccccatggcctcgtggctctgtggggtgacaggaacccgacccacatgtagctcaatcctcccaaggtcagcttgtgaagaagggaaagaaaattatggaaacaggcgtctctgtaggggatgctccaagacgcatttggaggcaggaaaatgcctgaagtccctcaatgggcggatgtcacagtgctgggcgagccacggtgtgtactcggggcctcactttgggagctcagacgtgtcgctggccctgacgctcattggtctgaaggacaaatcgaaggccctctggtcacggaagctctgggctttgtacttggccaggtgcctggacctcccgcgacgctcgggctccgatgcctccatcctgtcctgcagggccctctcagccccagggtggtctggggacccctcctgggccggggcctggggagtcccgcagcccccagcctcaggcttgggctcagttgggctctttcccagccccaggggagaggtggcaatgctcttgcccctgagggggcggcttcctgggggtgggtacccggcgctgggctcccccaggccactgccccctgactgtccaccatccctgggggctgggcttctggaccccccactcctgccagcagcatccactccctcagctatgccactaatgggctgctcccaggcccgaggcgccatcccacttgtcaaggcctgttcccgaccctgttcccaagcccgttcctgagcccctttctgggtctgcctctgagtctctatctgggtctgctcccagccctgatcccgagcccgatcccgagcccattcctgagcccctttctgggcctgaccctgagcctctatgtgggtctgctcccgaccctgttcctgagcccgttcctgagcccctttctgggcctgttcccgagcccgttcctgagcccctttctgggcctgttcccgagcccgttcctgagcccctttctgggcctgttcccgagcccgctcctgagcccctttctgggcctgttcccgagcccgttcctgagcccctttctgggcctgttcccgagcccgttcctgagcccctttctgggcctgttcccgagcccgttcctgagcccccttctgggcctgaccctgagcctctatctgggtctgctcctgagcctgttcctgggcccgttcctgagcccctttctgggcctgaccctgaacccgttcctgagcccctttctgggtctgttcctgagcccatttctgggcctttatctgggtctgccactgggcctgtccctgagcctcttcctgggcccatttctgaacctctccttgaacctgtttctgggcctgtccctgaatctgcccctgagcccatttctgggcctgtccctgaacctgtccctgggccccaccctgagctggttcctgtgcctgcccctgggcctctatctgggtctgccactgggcctgttcttgagcgtgtccctgagcctgtccctgggcccaattctgaaactgtttctgggcctgtccctgactgtgtccctgggtcccaccctgagcctgttcctgtgcctgcccctgggcctctatctgggtctgccactgggcctgttcttgagcgtgtccctgaacctgtccccggtcccattcctgaacctgtttctgggcctgtccttgggctgccgggcttcccggcccctcgggctcccctggaggcacagctgggttcctggcagccctggtgccctctccccacgccgtgctccgcccccgctcctcccagggtccctgcagatgctgctgaccttggtcactgcgctggcaggcgcccccaaccccaatggccatccctttgtccccggccagatcctgtgcccaccatgtctgaggctcttttgctgggttcagcacaaccttcgagcccgacggcgccaccctcttccccgcatccccgggctggggggtctcctcctgtgcctggtgactctgttgcctccccaggtccgcctgtgtcaggggacgctcctgggattcacctgcctgcgtcctaggctcggggacactggcccggagctttgcctgtgtgtcaccagcagtagggggcaggtgtgcctgtagatggggagggccccgctggtgggtgccacctacccaccccatgtccacctccgcgggaggcactgcgggaagcagatggtcaggctccgccccacggggaaacctgacgccctccctgccctttgcctgtgggttctcaggaggcgacggcgggaggccagggccatagctgggggactctgccacgctccttgcctgtggcctaggatgatcagaagcaggaattccagactctgtgctgaaacccaaaaggtttccttccacagccacatcctttctgcctcctacagctgctgtatgtctgctggctgctgatgtgtttgaaatgtataatcgggccgcctctgggtgccgggcgagggccgcagcatcctccgggtggcgggcgagggtcgcaatgtcctctgggtgctggacgagggccacgcctctcaggaggctcctccctgctgctccactcttgggctccaaggatcccccaggggccaggaggccgtggctgtgagggtctcgagggagagcctctcctctggggtggctttcggacaaggctctgcttccccactggcccagcgtctctggctctcccgctgtgcggtctccagggctctgggtgctgcctggcgctggtgcaggcgtggcgcggctcgcaacgctccctgcagctgccatcgccccacaggctttcatacctggtttgggtggttcatttaatgaggacagtgggttctcgcgaacatcatggctggtgatttcctcggcagccttcaggggctgagaagactctattagcagcggccttctgcattcctccagcgcaccgggcactgtcatgcccatcggggtgacaccctcaggccccgtacgccccttggatgatgccgccagtgacgtgggggctcctgttgggtttctcccagtcggggacggcacttgctggctgctggaggcatggctggtgtttcccctcagaaggttttgtgaggctgcaggatcatttgttgcggagcccttcttctgcattgatatttcattagattccggcaacggatgcttcacatctctgagctcagaggtcctctctcctgaaatatcgtcaggattcctgggaccgtgtgaattctcaaagctgcctttgttttccttcccgccagcaggatctgtctggagtctctgtgtcagaagtgtctctgggacactgtggtcggcgcccacagcccctcttgctgctgccagacgcggagctgcccgtggcccctgcggcgaagaggcgctgagtcccgcctgcatccctgaaagcttgctcagttccactggggctcggtgaccccttctgttctcagtcacggtgggaaattctgtgtgggcattttcaaccacattctctcctccacaaatacaaggtttgttttcaccacttgacatattttgcagcctggtgggaggggctggcatttcatggacaactggaatttggacagttatccgtggaggctccgtggcaggctgtgttctccgagcagcctggaccgatggagcgttcaggggtgggatgtgctccggcaccttctgttctgggaaatacttctgggtggcaaagagggggtctctccctgggtctgggaagcctgctccttccctttcatcctctgaactgcaaacagtcatggtgatttcagggccctcccctgcacactcgcctgggggcccaggaggccacgtgagcctggctcccctcacctcctggacgcctcctgcggtgctctctgcggtggggtctgcagtcccatcacctccggctgatccggtgccccaagggctggccggtcccagtggggatgatgcaggcacaaggccaggaaggactccacctgtgcagggagcacaagagaaggccagcgaggggacagcgtggccgtccctctgagccatcacctggggtgtcacgggcttcgagggccttggctgtctttggggctcctcctccaggggcccctttcccactgctttgttcccactgggccccgtctccctggcactagggggcacgctggcttctcctctgggtggacgccttgcctccgagtggctgattttggtgcagtgggacagccagctcctggggccacagacgacggtggcgatgctgagggccggcaggggctcagccgtgcaggccagaaagcgggcagggggcatcttgacgcaggtgctggccatggtggccgtgtgcagcacgcgcacctccggccggtgcatcctcttcctctgcaggttcctcttcttccgctcctgcgtgtgcagcctcagcgcactggcctcggagcacaggcagctgttctgctcgaacttctcccgcagcttggacagcaccgagctcttgcccatgatcttcggcaagaggcccctggcggctttgggccgctccacagggggcttctcgcgtgcttctttctccttcgcctccttctcctcggcggccaagaatatcttcaggatgtttttcacggtgctcttcccggccgggtggccccagcggggcttctcgctgaggcagggctttggggccggctccttggtcttctccaggagcttgttgatggtggcacccacgaggcccccacccggcccctgcttgtccttggagatcagccggcccacctccctggtcctcttgaggtagcgctcccggccagtgcccaggaacttggcctgcaggagctggaagcgcgtgggccgctgggtggcctcctgggtctggggctggtggctgggcctgctccccccggcctctgtccccgggggccggtctgcgcggcccgtgacgtagagcagcaggctgctgaggatggagtgggcggccgggtcacaggccagcttgcccatcttcttcttcagggtttgggcgtccacagacatgacgtcactgcaggtcttgctgctcttccggctgccttccgccgggcgtctctggacacgtcccctctgctatgacttggcggcccgtggagggctgcgctcccttcaccccaggaggctgaacttctcagagcctgtcacacgttttgtc

SEQ ID NO: 14593 - RNA, 8051 nt, Homo sapiens
  source 1..8051: mol_type = other RNA
gctgggattacaggcatgagccaccgtgcccggccactttctttctttctttttttttttttttaaaaaaacaaaacaactttgggttttatttaaaatgcccgtggaggtggttagcgccccattcttctgctgtagttatttcaccccgggagggtgtgggccttagccatgtggccgtgatggtcgtatctgaagtgtgaatacttccccgcgctatcttctaacctgcgctgtctcagcttagtgtgaacgtacggaccgttctcaaatcctggtgaagtcactggcagttttttcctgcacacagagtagctgtgctgtttttgagctgagggcagtgtcatgctgggctgcatctggcacatggagaggacgggccagtcgagcaggtggcctcctggccgctcacagactctgcgcccgccagactgtgagaggggttcaggcacgacacttccggagctgtcatctggaggagattctcatcattttttccaccacttaaaataaaaccactcaatgccttctccagtgtactctctggtctatttaaaaatagcagcgcaagtcccaccacttcttatttataaagggaacagccagtgaacatatttttacctcccgtgtctgtcatcatgttcttgccactcattgcctccaattccaaataggtaaagagtgagggccgtgccgctgtgcctggagtggcaggggcagccacacagacctgggggtccctgagctcccccagctccagggaggacgccccaggcatgagcaggggccgccaacaggacaaagaggccactctgtcagcctctgctggacccctgagctcccctctcatgggcctctccgtttgggtggctccgagaggccaactccagccccaactgcaggctcccaggactgcaggggcagggactctggaggtccgtgtgcttcgtgagagaggggaccctgtcctcctagcaggggtccagcggcaccacagcaagacttctgtggccaagtacacgccatgctcagctctgcccccacccgcacccccggaccatcctgtgtgcagctgggctgccccgggacccacacgcgcgaggggcacccggtgctcaggagcctccacacacagcagctcgcacttagaacccacacgccaagcagaaacccctcgaagcgggctgggagcacggacccctgatttatagaggaggccccgggggccctgtcgggggagctgtggggaccggccccccagagctcagcacagcccggccctccttccagacaccagcactcgcatgtcccagcaggtgagggtgggtcaaacctgctggatctgaagttaattgttcgactggaaggaaacctgtgcgctccccggagcatgacgccacgccgcctccttggcgctgcagagccaaagccactggcgtctgccgggatggaccttccctggaaggagagacctcagccccgcgtgggtaggacgcgcctgctgaacgccctctcagggccgacactggaaaacaccttcctctaaaggaacatccgagtcagaaaacaggtgctcgcagcaggcaccaaagcgcctttgcgaacgcttagggctgtttcaggaaaccgctcagtagcaaaggcagaagatgccaagacaccttcaaaaagcaggaattaactttccacagggagggcaccaccaaaaacaagggtgcggggctgtagggcgacaggctgcatcggttcacgctgaaaatccagctgctccggggccactcaggcagccgtgtggcctcacgggtccgggtttcagaggccaccgagtggcctgggacgatggatcgcgacacggaggtgcatggctccatcatggggaagaatgtgctttaaaataggtgcatggaggaagagcctaaaaaatagtccagagtagcaacaaaaaccatctcgaggcaatgtgaccacaggtggctttgatttccttcttgtgcctctagacagcattcaaatattccagcctgaacatgcattacctcagtacctgaacagggccggagtcgtgggccgtctcgggccagggcaggaaacacttctatgctgttcgggaggacggaggacagacagcgaggctctcaggtcaccggcaccagtggcaccacccacagggactgcagggaagggcgggcaggctcccgttcgttctcccagcacccagtttccagacgaagcctccctgggatcctggcttcccacggctctgcactgtccctttctcagaacttaacgtgggcatttcctgaggcctcttcctccggatgagctggtttcggcctgggatcccagcgtccccacaccctctggtgaccaccacatggcccagcagccacacagcacccggcacccacctgggcgtctgaggctggaggaagctctgccctttctttcgagtcatgggggtggggcggtgtgcatcactttgggcccatggatggtgggtgccatgcggccacgtcagagcagggcatggtggggtgtgggcagggagcagtgggaggtggccctgtgagagctggggaggtgtcccaaagtgccagcatcctgcagatcgaaggggacgcacacaccgtgccactgcgggaggtgtgagctccacgctgcaggctgtgtgagagaggggtgagccggcgcccccgagtgaagacacaaagaatcccgagggcctggtgaggccacaggcccgcacctcccacccccatggcctcgtggctctgtggggtgacaggaacccgacccacatgtagctcaatcctcccaaggtcagcttgtgaagaagggaaagaaaattatggaaacaggcgtctctgtaggggatgctccaagacgcatttggaggcaggaaaatgcctgaagtccctcaatgggcggatgtcacagtgctgggcgagccacggtgtgtactcggggcctcactttgggagctcagacgtgtcgctggccctgacgctcattggtctgaaggacaaatcgaaggccctctggtcacggaagctctgggctttgtacttggccaggtgcctggacctcccgcgacgctcgggctccgatgcctccatcctgtcctgcagggccctctcagccccagggtggtctggggacccctcctgggccggggcctggggagtcccgcagcccccagcctcaggcttgggctcagttgggctctttcccagccccaggggagaggtggcaatgctcttgcccctgagggggcggcttcctgggggtgggtacccggcgctgggctcccccaggccactgccccctgactgtccaccatccctgggggctgggcttctggaccccccactcctgccagcagcatccactccctcagctatgccactaatgggctgctcccaggcccgaggcgccatcccacttgtcaaggcctgttcccgaccctgttcccaagcccgttcctgagcccctttctgggtctgcctctgagtctctatctgggtctgctcccagccctgatcccgagcccgatcccgagcccattcctgagcccctttctgggcctgaccctgagcctctatgtgggtctgctcccgaccctgttcctgagcccgttcctgagcccctttctgggcctgttcccgagcccgttcctgagcccctttctgggcctgttcccgagcccgttcctgagcccctttctgggcctgttcccgagcccgctcctgagcccctttctgggcctgttcccgagcccgttcctgagcccctttctgggcctgttcccgagcccgttcctgagcccctttctgggcctgttcccgagcccgttcctgagcccccttctgggcctgaccctgagcctctatctgggtctgctcctgagcctgttcctgggcccgttcctgagcccctttctgggcctgaccctgaacccgttcctgagcccctttctgggtctgttcctgagcccatttctgggcctttatctgggtctgccactgggcctgtccctgagcctcttcctgggcccatttctgaacctctccttgaacctgtttctgggcctgtccctgaatctgcccctgagcccatttctgggcctgtccctgaacctgtccctgggccccaccctgagctggttcctgtgcctgcccctgggcctctatctgggtctgccactgggcctgttcttgagcgtgtccctgagcctgtccctgggcccaattctgaaactgtttctgggcctgtccctgactgtgtccctgggtcccaccctgagcctgttcctgtgcctgcccctgggcctctatctgggtctgccactgggcctgttcttgagcgtgtccctgaacctgtccccggtcccattcctgaacctgtttctgggcctgtccttgggctgccgggcttcccggcccctcgggctcccctggaggcacagctgggttcctggcagccctggtgccctctccccacgccgtgctccgcccccgctcctcccagggtccctgcagatgctgctgaccttggtcactgcgctggcaggcgcccccaaccccaatggccatccctttgtccccggccagatcctgtgcccaccatgtctgaggctcttttgctgggttcagcacaaccttcgagcccgacggcgccaccctcttccccgcatccccgggctggggggtctcctcctgtgcctggtgactctgttgcctccccaggtccgcctgtgtcaggggacgctcctgggattcacctgcctgcgtcctaggctcggggacactggcccggagctttgcctgtgtgtcaccagcagtagggggcaggtgtgcctgtagatggggagggccccgctggtgggtgccacctacccaccccatgtccacctccgcgggaggcactgcgggaagcagatggtcaggctccgccccacggggaaacctgacgccctccctgccctttgcctgtgggttctcaggaggcgacggcgggaggccagggccatagctgggggactctgccacgctccttgcctgtggcctaggatgatcagaagcaggaattccagactctgtgctgaaacccaaaaggtttccttccacagccacatcctttctgcctcctacagctgctgtatgtctgctggctgctgatgtgtttgaaatgtataatcgggccgcctctgggtgccgggcgagggccgcagcatcctccgggtggcgggcgagggtcgcaatgtcctctgggtgctggacgagggccacgcctctcaggaggctcctccctgctgctccactcttgggctccaaggatcccccaggggccaggaggccgtggctgtgagggtctcgagggagagcctctcctctggggtggctttcggacaaggctctgcttccccactggcccagcgtctctggctctcccgctgtgcggtctccagggctctgggtgctgcctggcgctggtgcaggcgtggcgcggctcgcaacgctccctgcagctgccatcgccccacaggctttcatacctggtttgggtggttcatttaatgaggacagtgggttctcgcgaacatcatggctggtgatttcctcggcagccttcaggggctgagaagactctattagcagcggccttctgcattcctccagcgcaccgggcactgtcatgcccatcggggtgacaccctcaggccccgtacgccccttggatgatgccgccagtgacgtgggggctcctgttgggtttctcccagtcggggacggcacttgctggctgctggaggcatggctggtgtttcccctcagaaggttttgtgaggctgcaggatcatttgttgcggagcccttcttctgcattgatatttcattagattccggcaacggatgcttcacatctctgagctcagaggtcctctctcctgaaatatcgtcaggattcctgggaccgtgtgaattctcaaagctgcctttgttttccttcccgccagcaggatctgtctggagtctctgtgtcagaagtgtctctgggacactgtggtcggcgcccacagcccctcttgctgctgccagacgcggagctgcccgtggcccctgcggcgaagaggcgctgagtcccgcctgcatccctgaaagcttgctcagttccactggggctcggtgaccccttctgttctcagtcacggtgggaaattctgtgtgggcattttcaaccacattctctcctccacaaatacaaggtttgttttcaccacttgacatattttgcagcctggtgggaggggctggcatttcatggacaactggaatttggacagttatccgtggaggctccgtggcaggctgtgttctccgagcagcctggaccgatggagcgttcaggggtgggatgtgctccggcaccttctgttctgggaaatacttctgggtggcaaagagggggtctctccctgggtctgggaagcctgctccttccctttcatcctctgaactgcaaacagtcatggtgatttcagggccctcccctgcacactcgcctgggggcccaggaggccacgtgagcctggctcccctcacctcctggacgcctcctgcggtgctctctgcggtggggtctgcagtcccatcacctccggctgatccggtgccccaagggctggccggtcccagtggggatgatgcaggcacaaggccaggaaggactccacctgtgcagggagcacaagagaaggccagcgaggggacagcgtggccgtccctctgagccatcacctggggtgtcacgggcttcgagggccttggctgtctttggggctcctcctccaggggcccctttcccactgctttgttcccactgggccccgtctccctggcactagggggcacgctggcttctcctctgggtggacgccttgcctccgagtggctgattttggtgcagtgggacagccagctcctggggccacagacgacggtggcgatgctgagggccggcaggggctcagccgtgcaggccagaaagcgggcagggggcatcttgacgcaggtgctggccatggtggccgtgtgcagcacgcgcacctccggccggtgcatcctcttcctctgcaggttcctcttcttccgctcctgcgtgtgcagcctcagcgcactggcctcggagcacaggcagctgttctgctcgaacttctcccgcagcttggacagcaccgagctcttgcccatgatcttcggcaagaggcccctggcggctttgggccgctccacagggggcttctcgcgtgcttctttctccttcgcctccttctcctcggcggccaagaatatcttcaggatgtttttcacggtgctcttcccggccgggtggccccagcggggcttctcgctgaggcagggctttggggccggctccttggtcttctccaggagcttgttgatggtggcacccacgaggcccccacccggcccctgcttgtccttggagatcagccggcccacctccctggtcctcttgaggtagcgctcccggccagtgcccaggaacttggcctgcaggagctggaagcgcgtgggccgctgggtggcctcctgggtctggggctggtggctgggcctgctccccccggcctctgtccccgggggccggtctgcgcggcccgtgacgtagagcagcaggctgctgaggatggagtgggcggccgggtcacaggccagcttgcccatcttcttcttcagggtttgggcgtccacagacatgacgtcactgcaggtcttgctgctcttccggcttaattgggtttcttttcctgaaaggtaattctcagttaatttccccacacccacgggtgctgggaccacactccatggacgtgtgtgacgtgaggcccttcgcccccgtgtgcctgtctctctggttcttctgacttaaagcaccagtagcagcacagttagtccagttattcggaagctcagcacggagccacattgctgcagcatagaaggccacggattcctccatcagcatgg

SEQ ID NO: 14594 - RNA, 8606 nt, Homo sapiens
  source 1..8606: mol_type = other RNA
gctgggattacaggcatgagccaccgtgcccggccactttctttctttctttttttttttttttaaaaaaacaaaacaactttgggttttatttaaaatgcccgtggaggtggttagcgccccattcttctgctgtagttatttcaccccgggagggtgtgggccttagccatgtggccgtgatggtcgtatctgaagtgtgaatacttccccgcgctatcttctaacctgcgctgtctcagcttagtgtgaacgtacggaccgttctcaaatcctggtgaagtcactggcagttttttcctgcacacagagtagctgtgctgtttttgagctgagggcagtgtcatgctgggctgcatctggcacatggagaggacgggccagtcgagcaggtggcctcctggccgctcacagactctgcgcccgccagactgtgagaggggttcaggcacgacacttccggagctgtcatctggaggagattctcatcattttttccaccacttaaaataaaaccactcaatgccttctccagtgtactctctggtctatttaaaaatagcagcgcaagtcccaccacttcttatttataaagggaacagccagtgaacatatttttacctcccgtgtctgtcatcatgttcttgccactcattgcctccaattccaaataggtaaagagtgagggccgtgccgctgtgcctggagtggcaggggcagccacacagacctgggggtccctgagctcccccagctccagggaggacgccccaggcatgagcaggggccgccaacaggacaaagaggccactctgtcagcctctgctggacccctgagctcccctctcatgggcctctccgtttgggtggctccgagaggccaactccagccccaactgcaggctcccaggactgcaggggcagggactctggaggtccgtgtgcttcgtgagagaggggaccctgtcctcctagcaggggtccagcggcaccacagcaagacttctgtggccaagtacacgccatgctcagctctgcccccacccgcacccccggaccatcctgtgtgcagctgggctgccccgggacccacacgcgcgaggggcacccggtgctcaggagcctccacacacagcagctcgcacttagaacccacacgccaagcagaaacccctcgaagcgggctgggagcacggacccctgatttatagaggaggccccgggggccctgtcgggggagctgtggggaccggccccccagagctcagcacagcccggccctccttccagacaccagcactcgcatgtcccagcaggtgagggtgggtcaaacctgctggatctgaagttaattgttcgactggaaggaaacctgtgcgctccccggagcatgacgccacgccgcctccttggcgctgcagagccaaagccactggcgtctgccgggatggaccttccctggaaggagagacctcagccccgcgtgggtaggacgcgcctgctgaacgccctctcagggccgacactggaaaacaccttcctctaaaggaacatccgagtcagaaaacaggtgctcgcagcaggcaccaaagcgcctttgcgaacgcttagggctgtttcaggaaaccgctcagtagcaaaggcagaagatgccaagacaccttcaaaaagcaggaattaactttccacagggagggcaccaccaaaaacaagggtgcggggctgtagggcgacaggctgcatcggttcacgctgaaaatccagctgctccggggccactcaggcagccgtgtggcctcacgggtccgggtttcagaggccaccgagtggcctgggacgatggatcgcgacacggaggtgcatggctccatcatggggaagaatgtgctttaaaataggtgcatggaggaagagcctaaaaaatagtccagagtagcaacaaaaaccatctcgaggcaatgtgaccacaggtggctttgatttccttcttgtgcctctagacagcattcaaatattccagcctgaacatgcattacctcagtacctgaacagggccggagtcgtgggccgtctcgggccagggcaggaaacacttctatgctgttcgggaggacggaggacagacagcgaggctctcaggtcaccggcaccagtggcaccacccacagggactgcagggaagggcgggcaggctcccgttcgttctcccagcacccagtttccagacgaagcctccctgggatcctggcttcccacggctctgcactgtccctttctcagaacttaacgtgggcatttcctgaggcctcttcctccggatgagctggtttcggcctgggatcccagcgtccccacaccctctggtgaccaccacatggcccagcagccacacagcacccggcacccacctgggcgtctgaggctggaggaagctctgccctttctttcgagtcatgggggtggggcggtgtgcatcactttgggcccatggatggtgggtgccatgcggccacgtcagagcagggcatggtggggtgtgggcagggagcagtgggaggtggccctgtgagagctggggaggtgtcccaaagtgccagcatcctgcagatcgaaggggacgcacacaccgtgccactgcgggaggtgtgagctccacgctgcaggctgtgtgagagaggggtgagccggcgcccccgagtgaagacacaaagaatcccgagggcctggtgaggccacaggcccgcacctcccacccccatggcctcgtggctctgtggggtgacaggaacccgacccacatgtagctcaatcctcccaaggtcagcttgtgaagaagggaaagaaaattatggaaacaggcgtctctgtaggggatgctccaagacgcatttggaggcaggaaaatgcctgaagtccctcaatgggcggatgtcacagtgctgggcgagccacggtgtgtactcggggcctcactttgggagctcagacgtgtcgctggccctgacgctcattggtctgaaggacaaatcgaaggccctctggtcacggaagctctgggctttgtacttggccaggtgcctggacctcccgcgacgctcgggctccgatgcctccatcctgtcctgcagggccctctcagccccagggtggtctggggacccctcctgggccggggcctggggagtcccgcagcccccagcctcaggcttgggctcagttgggctctttcccagccccaggggagaggtggcaatgctcttgcccctgagggggcggcttcctgggggtgggtacccggcgctgggctcccccaggccactgccccctgactgtccaccatccctgggggctgggcttctggaccccccactcctgccagcagcatccactccctcagctatgccactaatgggctgctcccaggcccgaggcgccatcccacttgtcaaggcctgttcccgaccctgttcccaagcccgttcctgagcccctttctgggtctgcctctgagtctctatctgggtctgctcccagccctgatcccgagcccgatcccgagcccattcctgagcccctttctgggcctgaccctgagcctctatgtgggtctgctcccgaccctgttcctgagcccgttcctgagcccctttctgggcctgttcccgagcccgttcctgagcccctttctgggcctgttcccgagcccgttcctgagcccctttctgggcctgttcccgagcccgctcctgagcccctttctgggcctgttcccgagcccgttcctgagcccctttctgggcctgttcccgagcccgttcctgagcccctttctgggcctgttcccgagcccgttcctgagcccccttctgggcctgaccctgagcctctatctgggtctgctcctgagcctgttcctgggcccgttcctgagcccctttctgggcctgaccctgaacccgttcctgagcccctttctgggtctgttcctgagcccatttctgggcctttatctgggtctgccactgggcctgtccctgagcctcttcctgggcccatttctgaacctctccttgaacctgtttctgggcctgtccctgaatctgcccctgagcccatttctgggcctgtccctgaacctgtccctgggccccaccctgagctggttcctgtgcctgcccctgggcctctatctgggtctgccactgggcctgttcttgagcgtgtccctgagcctgtccctgggcccaattctgaaactgtttctgggcctgtccctgactgtgtccctgggtcccaccctgagcctgttcctgtgcctgcccctgggcctctatctgggtctgccactgggcctgttcttgagcgtgtccctgaacctgtccccggtcccattcctgaacctgtttctgggcctgtccttgggctgccgggcttcccggcccctcgggctcccctggaggcacagctgggttcctggcagccctggtgccctctccccacgccgtgctccgcccccgctcctcccagggtccctgcagatgctgctgaccttggtcactgcgctggcaggcgcccccaaccccaatggccatccctttgtccccggccagatcctgtgcccaccatgtctgaggctcttttgctgggttcagcacaaccttcgagcccgacggcgccaccctcttccccgcatccccgggctggggggtctcctcctgtgcctggtgactctgttgcctccccaggtccgcctgtgtcaggggacgctcctgggattcacctgcctgcgtcctaggctcggggacactggcccggagctttgcctgtgtgtcaccagcagtagggggcaggtgtgcctgtagatggggagggccccgctggtgggtgccacctacccaccccatgtccacctccgcgggaggcactgcgggaagcagatggtcaggctccgccccacggggaaacctgacgccctccctgccctttgcctgtgggttctcaggaggcgacggcgggaggccagggccatagctgggggactctgccacgctccttgcctgtggcctaggatgatcagaagcaggaattccagactctgtgctgaaacccaaaaggtttccttccacagccacatcctttctgcctcctacagctgctgtatgtctgctggctgctgatgtgtttgaaatgtataatcgggccgcctctgggtgccgggcgagggccgcagcatcctccgggtggcgggcgagggtcgcaatgtcctctgggtgctggacgagggccacgcctctcaggaggctcctccctgctgctccactcttgggctccaaggatcccccaggggccaggaggccgtggctgtgagggtctcgagggagagcctctcctctggggtggctttcggacaaggctctgcttccccactggcccagcgtctctggctctcccgctgtgcggtctccagggctctgggtgctgcctggcgctggtgcaggcgtggcgcggctcgcaacgctccctgcagctgccatcgccccacaggctttcatacctggtttgggtggttcatttaatgaggacagtgggttctcgcgaacatcatggctggtgatttcctcggcagccttcaggggctgagaagactctattagcagcggccttctgcattcctccagcgcaccgggcactgtcatgcccatcggggtgacaccctcaggccccgtacgccccttggatgatgccgccagtgacgtgggggctcctgttgggtttctcccagtcggggacggcacttgctggctgctggaggcatggctggtgtttcccctcagaaggttttgtgaggctgcaggatcatttgttgcggagcccttcttctgcattgatatttcattagattccggcaacggatgcttcacatctctgagctcagaggtcctctctcctgaaatatcgtcaggattcctgggaccgtgtgaattctcaaagctgcctttgttttccttcccgccagcaggatctgtctggagtctctgtgtcagaagtgtctctgggacactgtggtcggcgcccacagcccctcttgctgctgccagacgcggagctgcccgtggcccctgcggcgaagaggcgctgagtcccgcctgcatccctgaaagcttgctcagttccactggggctcggtgaccccttctgttctcagtcacggtgggaaattctgtgtgggcattttcaaccacattctctcctccacaaatacaaggtttgttttcaccacttgacatattttgcagcctggtgggaggggctggcatttcatggacaactggaatttggacagttatccgtggaggctccgtggcaggctgtgttctccgagcagcctggaccgatggagcgttcaggggtgggatgtgctccggcaccttctgttctgggaaatacttctgggtggcaaagagggggtctctccctgggtctgggaagcctgctccttccctttcatcctctgaactgcaaacagtcatggtgatttcagggccctcccctgcacactcgcctgggggcccaggaggccacgtgagcctggctcccctcacctcctggacgcctcctgcggtgctctctgcggtggggtctgcagtcccatcacctccggctgatccggtgccccaagggctggccggtcccagtggggatgatgcaggcacaaggccaggaaggactccacctgtgcagggagcacaagagaaggccagcgaggggacagcgtggccgtccctctgagccatcacctggggtgtcacgggcttcgagggccttggctgtctttggggctcctcctccaggggcccctttcccactgctttgttcccactgggccccgtctccctggcactagggggcacgctggcttctcctctgggtggacgccttgcctccgagtggctgattttggtgcagtgggacagccagctcctggggccacagacgacggtggcgatgctgagggccggcaggggctcagccgtgcaggccagaaagcgggcagggggcatcttgacgcaggtgctggccatggtggccgtgtgcagcacgcgcacctccggccggtgcatcctcttcctctgcaggttcctcttcttccgctcctgcgtgtgcagcctcagcgcactggcctcggagcacaggcagctgttctgctcgaacttctcccgcagcttggacagcaccgagctcttgcccatgatcttcggcaagaggcccctggcggctttgggccgctccacagggggcttctcgcgtgcttctttctccttcgcctccttctcctcggcggccaagaatatcttcaggatgtttttcacggtgctcttcccggccgggtggccccagcggggcttctcgctgaggcagggctttggggccggctccttggtcttctccaggagcttgttgatggtggcacccacgaggcccccacccggcccctgcttgtccttggagatcagccggcccacctccctggtcctcttgaggtagcgctcccggccagtgcccaggaacttggcctgcaggagctggaagcgcgtgggccgctgggtggcctcctgggtctggggctggtggctgggcctgctccccccggcctctgtccccgggggccggtctgcgcggcccgtgacgtagagcagcaggctgctgaggatggagtgggcggccgggtcacaggccagcttgcccatcttcttcttcagggtttgggcgtccacagacatgacgtcactgcaggtcttgctgctcttccggcttgctgctgagtgaacgcgtcctcatgcgctggagccagtgctgccccttgggccgtcagccccacccctcaaagcctcctgaaaaggcccccggtcagagctgcgctggcggagtctgggctgccctgtgtgaccgctgcccgcccagcagtgcggggcgagaccgggcctccctcagcgtcccctcagcacttggacaagctgcagaacccacagggaatggaatgtcttcctcccaggggccaatataaacagcagggtgcccggctttcctaatttagttgttggtggctctggccagccagagaggtcgtttgaaaatacaatgagactagaggccatcacagcgcaggagacacacccgggcccaccatgatatggacagcagcccctgttggcaggttctttgctggggactttctggccagcagggcctggaggtcactgttctgcccagtcagtggctgtgctgggctcacccgagcctggccctgcggcagggaacaccctcagccgcagtttcctcctctgagagaagggcagggccggtttcacgtggcagctgggcctgcaactgtctggctgttccaggagcctgctcagaacacggaccagcctcagccatgtcacacacatccctgtgccagcctccacatgtttctgacagggacacttggatgccctcggccaacagcgcttagaaaacatgtcctgggcctccatcaacaccagaggcctgcactgccatttcctgcccctctgcggatgagcctggagccgcccccccttcct

SEQ ID NO: 14595 - RNA, 4521 nt, Homo sapiens
  source 1..4521: mol_type = other RNA
gctgggattacaggcatgagccaccgtgcccggccagaggtagatttcttaactagcatatcagccttcagcatgtctctaagcttaaaatataatcaaagctaaagctgacatttatgtaaagtttataatgtatgcagtcaccagtttagagtcatagtatagatgtggaattatacttttggtttgtggaggtaatgaggaaaaaaaaaaacggttcccagatgaagcataacaaattaaatctcagtagtgtgtgtatataagccatgcatacaaggagttcaaactaccacttgcacagtggtatgtggctcttttccatctcgtactctatggtctcatggccacgtcgcggtgtctgttcacttccatgaagaggagaggttcttgtccaccaacacctgtgaaccgtaagaccagtgagtgcctttaaacttgtatttcaagttgtacccctcccccacttaccccatgtctcatcagagccatactttctagcctgaggtagatcattacgtaaaatccatccgatgtcacaggccatcagtggtcttggggagggggtctcatttttgtctgggaagtagtgtactttccaagtagcaatttatatttaggccttaaattgtgtaaaatgacataatggaaaacaccttgggataggataagcatttcaacagaaacagaacaccttctgtaaacaacattgtacaattagactattgttctgtacttaaaaaggaaaaaagcaactttctggccgggggcagggtggtgcatagaaaaccaccacatttcaaaaggtgtattaaaaaaaagccctcgctcagctcaaattagagaaagaaatgacaagaattcagaactgtcaggctgcttcacttccttttttgtttgtttgtttaatttttttttaacctgtaatttaggaaaaaaataaattactccagcaagtgttcgtgctacctcaaggtattctataggtaatgtggaagctaggtactgcccaggacctcctggctttgtctgccgaagctggccatccaatcccttgctctgggagggagggggatgagtttgatgtctgtaagagaaccccaccctgtagggaggagagaaacaataacacacatggaagaattaggttctgagcaatgaggggactgagagtaagtgtagttgatatttaggagaatttcctccatttttctggacaatgggttcttggtcctggagggataaggaaatacttggagaggagaaaaaaccacagagaactttccagctatggagtgagagctaggtcaggcctggagacctggaatgggtcataaagaggggattgcccatgaaagttgggggtacacagtagagactctcctgactagaagagaagtgtgttggtggtaccagttgggtttttagagaatgaggacatatcctggagggctttggaagccagactctgagatatttcagtgatgatggaaacaacatatcccaagaagtcttccatagataacttccaggtcctccttttgcctttgtcctttattcttaggagaggaaaaaagaaagtgggataggtatattaagtccagtgagcctttattttttaaacagaataaatgtgtttatttctcattttacagtattggccccaagtctcagagcattcagctctcttctttatgagcatagagaactctggacttgtctccttatggggtttagaatttttagggtcttactgaagacagagatgtcatacctagattgttttagccttaccccttagagctttgttgcactatcggtcacaaactgcttatttcttatttatttcaccagtagcacagttaaaattaagagtgtgtccatcacaggtgtacagagatgtgcctgtactccatcaatagaaacatgacaccatctgttggcaatgtagaagatgacaccatgaagatgtgtcattgagggagagtcaggtgttaaatccgcgattacaaagaggtctgacttttggggtgctgctagctgataaagaatgctcattaagcaagttgctctctacaaattactctcactgcatttcataggcaccttttcaaacagataaaatgtttgggtgtataaatctcagaatggtaggaaaagaacagaccagaaattgtggccctgtgttgaaggtgatggtaaataaaatagttcttgtcatatactatgtggcataagttagggaaggacgaacgcatttctcgaagagatgtgaggggtaggggtggttgagagggtgagagaacaccttggttcttgctgcagtgatccagaaatccaattcctgagtaaaatgcagtcttcttaaacctcttgcgttcacccctgattttcgtactcatgaggcccatatgtgcattaaaaaaataaaacaaaaacgatgacccagtgtagcagaaaaactagcccatctctttgacagaggattttcggttaatttatgcaggcctctttgcacttcagcattttttccactggttgctaagcaactgtttgagttactgcgcatgccttttttatgataactgtcattatgattactttttaattatacaactgggactgtggattaaaacagcatgttgtcactcatgctttgccactgccttctagtattctcacaagctcctagaatcaccttctgaaatttttatggcagtgatttatgattaatttttgatatttctggcttcacaaaggaagtagagatggcatcctaaggggagtgagacttttgtgaaaaatgactgtatcacacaccacaagctgttattgatctgagtagaccaaatcagatattaggatcttgaacctaaattgtgaatctctttgtgcctttaaccacatctgcttccaacagtaagtgatgttaaaagctcatatgctttgtagcctgtgtttgaaaattacaaaaatgctaagcatttgttgctatagaacctgctttcaaataaacttaccatgaatttgggggagggtacagcactaatcccagaaatgtgaagcatccacacttaagcttgtgaaacatgttcttctttcacccaaattgctctacacacacacaatggcagttaggcaagatgaaggggttcctctggcaagtaataataaaggtatgtgtggtttacagtatgtaaaatacccttctgccagttttttttcataagtagtactgtgtagtcttaagtgaacaatctctgtgttagagtgccaggatttgaagctcctcccttctgctaattatgtaacccccctttccttttcctggaagtggttttgttgtaggacagccacaggtggacggctggaccttaccaagctttgaagggcgaggaccgggcgaaggcaaaacctgggaaggctctggctgccgccagaggaccgggcggagcaaccacagtcactgtggttatcatgtccagcctcctgggacctccacttagcttggctgtcaccctgacccccgcccgcacctccccagctgctgatctcggggaggcagccctccctgaggtgctgagggcaggaccctggcgagcagaagtgaagggtttaagagccatctccctactagaatggtgccctgatgtttaatggcaaattacccagcaagcacctatttttaaaactttcaccccttttccttgggaaccccccactgttatggaaaatttaagcctttaaagaaaacacgtgtgagtgtgtgtatgtgtgtgtgtgcgcgcgcatgagcatgagagagagagagagagaaagagatagctgtcgaggtaagttgagagatggaggggaggggaaggatttcagcatcatgacgtagtataggaggaagctttgttcctggaggattgattttgtgagggagggcagaaccagacaacaaggaacatttagataatacgtctgtactccgtaaaggtgagggtctacaacagtcatctaaggcagtgacagacatgggtctgcacactgaaaccgcagggtgtcaacaaggcacagaaaagaatgcaatgtagggcgcagtcctttggctgggctaggcgtgaagcattcctgagaaaggtctacactatgaagccagctcactgtagacttgggactcactgatcagccttggctctctgtggagactcaggtgtttgctaaatgaacataagatactgcagagaaggctgctagtctccaaagctcatggaaagcgtttcttcctgaccaactgcaaaagagtggatgtatactgtgctaacctttgtgaggaaaaggaaaaatgggagaaatacatgtacctgcatatctttcaaaaaaatagaaatataggaggaataaaccagtaaagaatgaagtgagatgaagcaggtcacctaacaagaaggtgggaaacagggtggaaggaatatgagagggagaaacacttctatggtatagctctttgtattatttttgatttttggaagttta

SEQ ID NO: 14596 - RNA, 4567 nt, Homo sapiens
  source 1..4567: mol_type = other RNA
gctgggattacaggcatgagccaccgtgcccggccagaggtagatttcttaactagcatatcagccttcagcatgtctctaagcttaaaatataatcaaagctaaagctgacatttatgtaaagtttataatgtatgcagtcaccagtttagagtcatagtatagatgtggaattatacttttggtttgtggaggtaatgaggaaaaaaaaaaacggttcccagatgaagcataacaaattaaatctcagtagtgtgtgtatataagccatgcatacaaggagttcaaactaccacttgcacagtggtatgtggctcttttccatctcgtactctatggtctcatggccacgtcgcggtgtctgttcacttccatgaagaggagaggttcttgtccaccaacacctgtgaaccgtaagaccagtgagtgcctttaaacttgtatttcaagttgtacccctcccccacttaccccatgtctcatcagagccatactttctagcctgaggtagatcattacgtaaaatccatccgatgtcacaggccatcagtggtcttggggagggggtctcatttttgtctgggaagtagtgtactttccaagtagcaatttatatttaggccttaaattgtgtaaaatgacataatggaaaacaccttgggataggataagcatttcaacagaaacagaacaccttctgtaaacaacattgtacaattagactattgttctgtacttaaaaaggaaaaaagcaactttctggccgggggcagggtggtgcatagaaaaccaccacatttcaaaaggtgtattaaaaaaaagccctcgctcagctcaaattagagaaagaaatgacaagaattcagaactgtcaggctgcttcacttccttttttgtttgtttgtttaatttttttttaacctgtaatttaggaaaaaaataaattactccagcaagtgttcgtgctacctcaaggtattctataggtaatgtggaagctaggtactgcccaggacctcctggctttgtctgccgaagctggccatccaatcccttgctctgggagggagggggatgagtttgatgtctgtaagagaaccccaccctgtagggaggagagaaacaataacacacatggaagaattaggttctgagcaatgaggggactgagagtaagtgtagttgatatttaggagaatttcctccatttttctggacaatgggttcttggtcctggagggataaggaaatacttggagaggagaaaaaaccacagagaactttccagctatggagtgagagctaggtcaggcctggagacctggaatgggtcataaagaggggattgcccatgaaagttgggggtacacagtagagactctcctgactagaagagaagtgtgttggtggtaccagttgggtttttagagaatgaggacatatcctggagggctttggaagccagactctgagatatttcagtgatgatggaaacaacatatcccaagaagtcttccatagataacttccaggtcctccttttgcctttgtcctttattcttaggagaggaaaaaagaaagtgggataggtatattaagtccagtgagcctttattttttaaacagaataaatgtgtttatttctcattttacagtattggccccaagtctcagagcattcagctctcttctttatgagcatagagaactctggacttgtctccttatggggtttagaatttttagggtcttactgaagacagagatgtcatacctagattgttttagccttaccccttagagctttgttgcactatcggtcacaaactgcttatttcttatttatttcaccagtagcacagttaaaattaagagtgtgtccatcacaggtgtacagagatgtgcctgtactccatcaatagaaacatgacaccatctgttggcaatgtagaagatgacaccatgaagatgtgtcattgagggagagtcaggtgttaaatccgcgattacaaagaggtctgacttttggggtgctgctagctgataaagaatgctcattaagcaagttgctctctacaaattactctcactgcatttcataggcaccttttcaaacagataaaatgtttgggtgtataaatctcagaatggtaggaaaagaacagaccagaaattgtggccctgtgttgaaggtgatggtaaataaaatagttcttgtcatatactatgtggcataagttagggaaggacgaacgcatttctcgaagagatgtgaggggtaggggtggttgagagggtgagagaacaccttggttcttgctgcagtgatccagaaatccaattcctgagtaaaatgcagtcttcttaaacctcttgcgttcacccctgattttcgtactcatgaggcccatatgtgcattaaaaaaataaaacaaaaacgatgacccagtgtagcagaaaaactagcccatctctttgacagaggattttcggttaatttatgcaggcctctttgcacttcagcattttttccactggttgctaagcaactgtttgagttactgcgcatgccttttttatgataactgtcattatgattactttttaattatacaactgggactgtggattaaaacagcatgttgtcactcatgctttgccactgccttctagtattctcacaagctcctagaatcaccttctgaaatttttatggcagtgatttatgattaatttttgatatttctggcttcacaaaggaagtagagatggcatcctaaggggagtgagacttttgtgaaaaatgactgtatcacacaccacaagctgttattgatctgagtagaccaaatcagatattaggatcttgaacctaaattgtgaatctctttgtgcctttaaccacatctgcttccaacagtaagtgatgttaaaagctcatatgctttgtagcctgtgtttgaaaattacaaaaatgctaagcatttgttgctatagaacctgctttcaaataaacttaccatgaatttgggggagggtacagcactaatcccagaaatgtgaagcatccacacttaagcttgtgaaacatgttcttctttcacccaaattgctctacacacacacaatggcagttaggcaagatgaaggggttcctctggcaagtaataataaaggtatgtgtggtttacagtatgtaaaatacccttctgccagttttttttcataagtagtactgtgtagtcttaagtgaacaatctctgtgttagagtgccaggatttgaagctcctcccttctgctaattatgtaacccggttgtcatccggtttgtagcctgacttcttcggcctgtcacgtacccctttccttttcctggaagtggttttgttgtaggacagccacaggtggacggctggaccttaccaagctttgaagggcgaggaccgggcgaaggcaaaacctgggaaggctctggctgccgccagaggaccgggcggagcaaccacagtcactgtggttatcatgtccagcctcctgggacctccacttagcttggctgtcaccctgacccccgcccgcacctccccagctgctgatctcggggaggcagccctccctgaggtgctgagggcaggaccctggcgagcagaagtgaagggtttaagagccatctccctactagaatggtgccctgatgtttaatggcaaattacccagcaagcacctatttttaaaactttcaccccttttccttgggaaccccccactgttatggaaaatttaagcctttaaagaaaacacgtgtgagtgtgtgtatgtgtgtgtgtgcgcgcgcatgagcatgagagagagagagagagaaagagatagctgtcgaggtaagttgagagatggaggggaggggaaggatttcagcatcatgacgtagtataggaggaagctttgttcctggaggattgattttgtgagggagggcagaaccagacaacaaggaacatttagataatacgtctgtactccgtaaaggtgagggtctacaacagtcatctaaggcagtgacagacatgggtctgcacactgaaaccgcagggtgtcaacaaggcacagaaaagaatgcaatgtagggcgcagtcctttggctgggctaggcgtgaagcattcctgagaaaggtctacactatgaagccagctcactgtagacttgggactcactgatcagccttggctctctgtggagactcaggtgtttgctaaatgaacataagatactgcagagaaggctgctagtctccaaagctcatggaaagcgtttcttcctgaccaactgcaaaagagtggatgtatactgtgctaacctttgtgaggaaaaggaaaaatgggagaaatacatgtacctgcatatctttcaaaaaaatagaaatataggaggaataaaccagtaaagaatgaagtgagatgaagcaggtcacctaacaagaaggtgggaaacagggtggaaggaatatgagagggagaaacacttctatggtatagctctttgtattatttttgatttttggaagttta

SEQ ID NO: 14597 - RNA, 8159 nt, Homo sapiens
  source 1..8159: mol_type = other RNA
gctgggattacaggcatgagccaccgtgcccggccagtctctatttctttttaatgtactgaaaaaaatagtatcaaaactaagcacactgtaaagttacagtagaactttgaaatagatgtctactcatacaaaaggctaaatttattttgtagttttcttgtaagagaattaacatccaaccttgaaggttgaattttgttacctggctaatctggagtatttcatgaattatgaattagaattgctacttacaaagcttttttttttgtttttgagatggagtcttgctctgtggaccaggctggagtgcagtggtgcaatagcggcccactgcaatctccgcttcccaggttcaaacgattctcctgtctcagcctcccgagtagcagggattacaggcccacgtcaccacgcctggctaatttttgtatttttagaggcggggtttcaccacgttggccaggctggtcttgaactactgacctcaagtgattcgtcaccttggcctcccaaagtgctgagattacaggcgtgagccacagcgcacagtccaaagctctttaagtgtaacattgaagagctaaagtgtaactttctttaatgaactgaaaaaattagtacaatctttacacaaagaatagttaagaaaatataaccagcacagaatgttagctgtagttagctactgcagttcaaagatcagcagggtagtaactacagaaagttacatccttggagttcaaataatggtccaaaataggttgtcttgaaaaatgggatgatgaaaagacaattcaatacatcctgatctcacctctctaaattttaagagagactatttgagccaactttttaaaaacaagaatgtgatagcaccttgacttgagacccccattagaattatagtgtatagtagtgacatatcctatagtagtgacatatcctaaaagctatggataatgaggatggcatgacttaaattactcacaatttcgttcaggttgaaaatcaatttgatgtttagcaaaataatctctctaaaggggtgaataatgcaaaccaatgaaggtcatagacacctatgtatagagatagatactgccatcattcaagcactgttcttggaagaattcagctaaattagtaattatggcacttctggatttctgaaaaaatttaatctctggattactctggaaacacaggtataatttcaaattagcttttcattactttgcaaacttagtttttcattaagttgaacacttaaaaacttgtaccgtaagtttacttctgtttaaaaggaatgagtatgggagttttatgccctattttggactcagtccaaatctcagtctcaatgattagtgtctgtcttgtctgtaaagacaagacatattttactaaaaacaaacaaacaaacaaaaaacaaaaccacaatgtgaaatcttaatgatattaaaatatttaagaaaagagactctcacttgaaatacactgtgaatcttgcctactattgcctttaaaaaaacattagcacttaaataaatatattcattaattaagaaaaatgttcacaataaaaatacattctacccattcacctgataacaaacatacacatattctactatagtttgaagcaaatcagagtttaaacatttttcttccaggtacctctgaaatgtattagttttatagcaacatggtccccttttagtaaaaataaaccaaaataggtaaatttatataaattatatttacaaaatattagtatattctcatgaatataggcttttctcatttttttgcttaatagaaagtatagtgtttcaaaacgaaagtaaaatgcatagcccaaaccaaatcaaaaacatatgcaaaaacattttatttataatagatcaacatttttgacatgaaaggtagccactttcaatttctcaggaatgcctagaacccaacagttttcagaaagactacttagttcacaattatttcactgtaggtaaatgaaataatttcagaatgaactttttaaatggctttgcctatggcaaattgttttataaacttgaatgtatggtaagctagctttcccaggaaatgaatgtaatccaactatgttccaaatgtattaaaccagtttatacaacaaatatgagaatcacttatgtgcatcaactgtgctaaaacaagaattctttttatcaaaatattcatttttcaaaaaggcctcacattaacccctcaaaccaagcacccccttcctatgtccagcactcttttctacttcgagttgcatgactgtagagacaactgtcaaattccagtggaactgtacactgacttaagactctatgtaatatacatcaaacacaggaggtcactgactttaagggacgaggtgataactaactagttataattcagccaatgtcttttttagtttagagggaaaaaagtagcccccaagtgtccttaacttttcagtacttctctgtaacacacagaatgaaaaggtactctctaaaattaaaatcattagaaaatatcttaaataaagtgttttacataaataagtgttaaatttcagattcaaactatattttcttctgtatctcaatttgggaaaaatctcacaattattaactcttctcagttacatttatttttgagcatttaaatctactatacaccagtttgtaaaattcaccttggttacctctccccatgcctatgtgctgtctttcctcaggtaagtccattatatgcatctaagtgctggggaggtttaaatagcacttaaagaatattcatgagagttctgaaatgaaggtttcgtctttagctattgactgtaggatttgtaattcaaatcatcacagcatcctaaagaaatactgtgtgaatggaatgcacacaattcctacagaacacacaaactgatgtccaaaaggcacagagtaatgctggtggctctttctagtcagttaagaaacaataaaaagtctgcattattctttcataatttaaatacttaagtaatctccactttattattttataacaatgacttcaaatttacattattttaagtaccattgtaatagcttagtgtataatacagatatttgcgaatatcccatccaaaaattaaaaaaaacttcttcactatatatatatttatataaaaattattctgaaagacaagaacatagacaagggacttggtacagaccatcaactcaattttctatcaccacagttgtaactccaaaatcaacaaatatacagcagtaattaaaagcagtgcaaatatctttggaggttaggataaaattataatgcaagaacataaaactgaggaaacaaaaaaggcaagtacttcaagtacaaggaaccagtcggcttgaggtccatcttagtgtttactgggggcttctttcctgcttctacttctttctctgaaatacattggccaacatggcacctgatgttgtcaactggcccattttgttcaaaaacttggtctttgtatcttcactcactaagcttgcagcaattgacattgagccttgaggctcttggacggtcttgttttcaactttttgttcacattcttttatcatggaacttaaaataacctcatgctctggagagagatgttccatgtcagtccgtaaacatctgagaccaggtaaaaagtgattaaccattaaatcctctgaaatgaaacaacaggaaagtgcactgtaggcttcaaaaagatgcgtagcaatgtccagtcttttagaatccacaatctgtaagttgttcaccaaggctaacttatgcaaatgtggtataacaaactcatctcggaacctgggttctgcgttagggccaactctaccaaatgtttttatgatctctgtatgcaaagaatgttggtcttgatactgaggatcttccaggaaagaagccaactgcattttcactctttccagcaactctctttgaattactgtttccataatagtgccaaaggctggaattgtggcaatcctgacagagaattcaggatcactggacaaggtaacaagggccggagcaacccgcttgtcaactaacgcttcactcatgcctcgaagagtcagatttcagggtcactggagagagtaatgagagcaggaacaaccctctgagctaccagagtttcattcacccccttcaccaacagctcaaacattctagcagcagtacacctcacgagtgctgaagtatggacaacaccataccacaaaacagttaatagtaactcatggtaggctgggtttgcacccaattccacaaaagaagccttcaggctatcaagaggagcatgagataatgaaagcagcgtcattacatcttctaagaatccaactaacagttttcggtcttcttcctgaatataacacgtaaggactcctgttgcataaatggggactgtagctttagtgaggaccccatttcctgctgaggaatcaatgttttcttcagatagtcttaaaatctcctggaactgaggttttaccttagtgtttgtaaaaattttgccaaatgtccggcaaaggcgccagaaaaatctggagaattcatggacacaggcagttgaagtaacattaattttgccaactatttctataagttgtggcaacaattgattgacaacccacagtaaactctcccagcctgttgtaccctcttgttctagctggtagtcataaagttgcagcagcactgccaattgctcacgacttccgataatagtggacacatcttgaagaggcgacataggccgaggaaacctagtcacttctatctgtggcacttcaccatgaagcttggctttgctggagaaaggtgcattctgtagcactaatgcaaagagagatgggatcaaggactgcaaggcagaaagatacatgtggagtttgtgttcatccagtccatgttctccttccctgagaagtttttcaatcttgttcagtagtgtaagtataagatgagactgtaaatttccaagttctgtagtccacgcagcgtaagctggtaaaaatacttgatgtgtagcactaactactctttctgagggatcacccaaggctgacagcaacaattcaaaaccctgatgatatttgtctggatcatcaatgtatcccataatgataccaaggcttttgataacagcttctcttaccaaatctgccttatcttccattaacatttgttgcaacattgaaagaaccaaggagctacggatttctttaggaaggtaaggtgccagtgctccacaggattctgccacaagcagtcgtctttctgggtatttgtgattaatctgttcccaacactgtggtaaaagttcagcttctacacgtgttggtccaacatgacgcgcaaatgccacacaacctgtcagtatcatttgcctttgctcatcatctggcctcttgatcaaattgaaaagtatgtggagaagctgatctcgctctttaggctcaggatgtagacatgctgtacacaatatgagggggatcaactcctatctgtgagcctttgttggtctgtagatagtgtacaacctctgatttaacttttcagttgaaacttttcagcttgttcctgttttgcagaagtgaaaggctgagcatcaaattcatgcggaactgcaagggaccctgaacagacaatagtgatgtgcagttagaggactcatatatcccaatttcaaaacttactacaaacaacagttatcaaaacagtgtggtagtggcatatggctagacatacagaccaatggaacagaactgaaagtccagaaataaacccgaagaatctaggcccaactgatttttgacaaaagtagcaagactattcaaaagaggaatttttttatcttgaacaaatgtttctggataactggatagccatatgaaaagaataaagttagacgctgttttactccatatataaaaattaactcaaaatgaatcgttgacctaaatatatataacaaatgttttcttctaattgtttcatagctttagctcttatatatattcatatacatatagatatatatatcttctataacattgattgacttggcaatggtttcttaaaattgatacttagagcacaaacaacacaacaaaaaaatagataaatcagatttcataaaaatggaaaacatttgcccatcaaaggatatggtcaagagtgtaaaaagaaaacctgacagaggtgtaaaaccattctctctctctttgccaatagcacattgggaacaatgtgtggcaggcagcgtcccagcattaacataacgcttttttcactgtctgcaatacgagacacctcgtatcctaaacgactatctgctgacattcgacaaaaagagagtagtgcttgatggaatgcaggagacaatttcctattaggtttatcaaaatgaactgtctttttacttgatagagaagaaggtggcattccttctctttctctcctggggaatgaatttggggaattctctttaggaatagtggaatcagcttcatctgatattgaaagatggatgtctgtgttttttcccttgtctgaactatttacatctggatgctgtccactgtcctcagagtctttgtggggcaactgatccaaaggaggctgaacagagtcacaaactgctgggatggcaaagtgttcatttttgaggaagtccatttcacttttaagtcttctgatttgctccatcaatgaccatttctcactatttaacaaactaattttatcttctaatttctgtactaacatggagttctctgcaggctggggagtttcaagagttggaggaaggttgcttataattggtgtaagggcctctaattcatcttcttctactccactggccacatctacaagatcttttccagttacttgatgatttccaaaatcccggtagagttgcaataagtctggaggttttggaatgtttaatcctacatcatcccataattcaaaatcctgatcatcgttttcatctgaaaaggttattgatgtaagcttatagttattcttcaataaaaattcattgactaagaagtttagagctctcttttcaagaggtttgattggctcctgaatttcaggacttgatttgtaattttttcgttcctgtaaaggaacttcatgttctgcggcctttgtcaggttggctcggagggcctgaatggtctccttggctttccgtagttcaaactccaggactgccactttttcatctgtttccctgttaccatcatctgaatatcttgcaaagtctaaagaatcaagggtactaatgctcccagctcgattgagctgtcccccgcccgacgctgtactcggttcccgacctccagcgcccccaacgccggctgctccagggacccctggcgcccccatccccggcggggttccactttgcctctcgaagttgcctggattggagaagtagtcgcgcagccgaggcagctcccggccactctctaacagctcggtatgcagctccagggcggtcagcaagtattgatcgcgcaacagctgagcagcgatcgcatcaattgataatcgggccggggtctccccggtgccccccagggccactgcagccgccgacgcctccccagggagccctggccgcgcactgcttcctaaggccacgggatcctgtggcgacagcgagcccgcagagccaggatctaggccacttccggcgcccagccgaagtactgcccgccgttcctctgttgcagctacctcgtcatcgtcctcatccgaatcactgagaaatggattcacgccgccaccactgccactacctccaggcgccatcgccgccatcttatcctgtcaggagtgtgggcgcctccctgactggttccgacgggccgcagcccgaatcctctaggcctcaggggacacagcgcacctccacagccccggcctgaccacgtcctgcctcccgacttagagacaaggagtacgctccaaggcaggagatccggatgcagctgcacctgatgcctcagcctctgctgcaccagcagcccggctctgcaggcgtcttcctggtctccagtctcgcgagaact

SEQ ID NO: 14598 - RNA, 7443 nt, Homo sapiens
  source 1..7443: mol_type = other RNA
gctgggattacaggcatgagccaccgtgcccggccagtctctatttctttttaatgtactgaaaaaaatagtatcaaaactaagcacactgtaaagttacagtagaactttgaaatagatgtctactcatacaaaaggctaaatttattttgtagttttcttgtaagagaattaacatccaaccttgaaggttgaattttgttacctggctaatctggagtatttcatgaattatgaattagaattgctacttacaaagcttttttttttgtttttgagatggagtcttgctctgtggaccaggctggagtgcagtggtgcaatagcggcccactgcaatctccgcttcccaggttcaaacgattctcctgtctcagcctcccgagtagcagggattacaggcccacgtcaccacgcctggctaatttttgtatttttagaggcggggtttcaccacgttggccaggctggtcttgaactactgacctcaagtgattcgtcaccttggcctcccaaagtgctgagattacaggcgtgagccacagcgcacagtccaaagctctttaagtgtaacattgaagagctaaagtgtaactttctttaatgaactgaaaaaattagtacaatctttacacaaagaatagttaagaaaatataaccagcacagaatgttagctgtagttagctactgcagttcaaagatcagcagggtagtaactacagaaagttacatccttggagttcaaataatggtccaaaataggttgtcttgaaaaatgggatgatgaaaagacaattcaatacatcctgatctcacctctctaaattttaagagagactatttgagccaactttttaaaaacaagaatgtgatagcaccttgacttgagacccccattagaattatagtgtatagtagtgacatatcctatagtagtgacatatcctaaaagctatggataatgaggatggcatgacttaaattactcacaatttcgttcaggttgaaaatcaatttgatgtttagcaaaataatctctctaaaggggtgaataatgcaaaccaatgaaggtcatagacacctatgtatagagatagatactgccatcattcaagcactgttcttggaagaattcagctaaattagtaattatggcacttctggatttctgaaaaaatttaatctctggattactctggaaacacaggtataatttcaaattagcttttcattactttgcaaacttagtttttcattaagttgaacacttaaaaacttgtaccgtaagtttacttctgtttaaaaggaatgagtatgggagttttatgccctattttggactcagtccaaatctcagtctcaatgattagtgtctgtcttgtctgtaaagacaagacatattttactaaaaacaaacaaacaaacaaaaaacaaaaccacaatgtgaaatcttaatgatattaaaatatttaagaaaagagactctcacttgaaatacactgtgaatcttgcctactattgcctttaaaaaaacattagcacttaaataaatatattcattaattaagaaaaatgttcacaataaaaatacattctacccattcacctgataacaaacatacacatattctactatagtttgaagcaaatcagagtttaaacatttttcttccaggtacctctgaaatgtattagttttatagcaacatggtccccttttagtaaaaataaaccaaaataggtaaatttatataaattatatttacaaaatattagtatattctcatgaatataggcttttctcatttttttgcttaatagaaagtatagtgtttcaaaacgaaagtaaaatgcatagcccaaaccaaatcaaaaacatatgcaaaaacattttatttataatagatcaacatttttgacatgaaaggtagccactttcaatttctcaggaatgcctagaacccaacagttttcagaaagactacttagttcacaattatttcactgtaggtaaatgaaataatttcagaatgaactttttaaatggctttgcctatggcaaattgttttataaacttgaatgtatggtaagctagctttcccaggaaatgaatgtaatccaactatgttccaaatgtattaaaccagtttatacaacaaatatgagaatcacttatgtgcatcaactgtgctaaaacaagaattctttttatcaaaatattcatttttcaaaaaggcctcacattaacccctcaaaccaagcacccccttcctatgtccagcactcttttctacttcgagttgcatgactgtagagacaactgtcaaattccagtggaactgtacactgacttaagactctatgtaatatacatcaaacacaggaggtcactgactttaagggacgaggtgataactaactagttataattcagccaatgtcttttttagtttagagggaaaaaagtagcccccaagtgtccttaacttttcagtacttctctgtaacacacagaatgaaaaggtactctctaaaattaaaatcattagaaaatatcttaaataaagtgttttacataaataagtgttaaatttcagattcaaactatattttcttctgtatctcaatttgggaaaaatctcacaattattaactcttctcagttacatttatttttgagcatttaaatctactatacaccagtttgtaaaattcaccttggttacctctccccatgcctatgtgctgtctttcctcaggtaagtccattatatgcatctaagtgctggggaggtttaaatagcacttaaagaatattcatgagagttctgaaatgaaggtttcgtctttagctattgactgtaggatttgtaattcaaatcatcacagcatcctaaagaaatactgtgtgaatggaatgcacacaattcctacagaacacacaaactgatgtccaaaaggcacagagtaatgctggtggctctttctagtcagttaagaaacaataaaaagtctgcattattctttcataatttaaatacttaagtaatctccactttattattttataacaatgacttcaaatttacattattttaagtaccattgtaatagcttagtgtataatacagatatttgcgaatatcccatccaaaaattaaaaaaaacttcttcactatatatatatttatataaaaattattctgaaagacaagaacatagacaagggacttggtacagaccatcaactcaattttctatcaccacagttgtaactccaaaatcaacaaatatacagcagtaattaaaagcagtgcaaatatctttggaggttaggataaaattataatgcaagaacataaaactgaggaaacaaaaaaggcaagtacttcaagtacaaggaaccagtcggcttgaggtccatcttagtgtttactgggggcttctttcctgcttctacttctttctctgaaatacattggccaacatggcacctgatgttgtcaactggcccattttgttcaaaaacttggtctttgtatcttcactcactaagcttgcagcaattgacattgagccttgaggctcttggacggtcttgttttcaactttttgttcacattcttttatcatggaacttaaaataacctcatgctctggagagagatgttccatgtcagtccgtaaacatctgagaccaggtaaaaagtgattaaccattaaatcctctgaaatgaaacaacaggaaagtgcactgtaggcttcaaaaagatgcgtagcaatgtccagtcttttagaatccacaatctgtaagttgttcaccaaggctaacttatgcaaatgtggtataacaaactcatctcggaacctgggttctgcgttagggccaactctaccaaatgtttttatgatctctgtatgcaaagaatgttggtcttgatactgaggatcttccaggaaagaagccaactgcattttcactctttccagcaactctctttgaattactgtttccataatagtgccaaaggctggaattgtggcaatcctgacagagaattcaggatcactggacaaggtaacaagggccggagcaacccgcttgtcaactaacgcttcactcatgcctcgaagagtcagatttcagggtcactggagagagtaatgagagcaggaacaaccctctgagctaccagagtttcattcacccccttcaccaacagctcaaacattctagcagcagtacacctcacgagtgctgaagtatggacaacaccataccacaaaacagttaatagtaactcatggtaggctgggtttgcacccaattccacaaaagaagccttcaggctatcaagaggagcatgagataatgaaagcagcgtcattacatcttctaagaatccaactaacagttttcggtcttcttcctgaatataacacgtaaggactcctgttgcataaatggggactgtagctttagtgaggaccccatttcctgctgaggaatcaatgttttcttcagatagtcttaaaatctcctggaactgaggttttaccttagtgtttgtaaaaattttgccaaatgtccggcaaaggcgccagaaaaatctggagaattcatggacacaggcagttgaagtaacattaattttgccaactatttctataagttgtggcaacaattgattgacaacccacagtaaactctcccagcctgttgtaccctcttgttctagctggtagtcataaagttgcagcagcactgccaattgctcacgacttccgataatagtggacacatcttgaagaggcgacataggccgaggaaacctagtcacttctatctgtggcacttcaccatgaagcttggctttgctggagaaaggtgcattctgtagcactaatgcaaagagagatgggatcaaggactgcaaggcagaaagatacatgtggagtttgtgttcatccagtccatgttctccttccctgagaagtttttcaatcttgttcagtagtgtaagtataagatgagactgtaaatttccaagttctgtagtccacgcagcgtaagctggtaaaaatacttgatgtgtagcactaactactctttctgagggatcacccaaggctgacagcaacaattcaaaaccctgatgatatttgtctggatcatcaatgtatcccataatgataccaaggcttttgataacagcttctcttaccaaatctgccttatcttccattaacatttgttgcaacattgaaagaaccaaggagctacggatttctttaggaaggtaaggtgccagtgctccacaggattctgccacaagcagtcgtctttctgggtatttgtgattaatctgttcccaacactgtggtaaaagttcagcttctacacgtgttggtccaacatgacgcgcaaatgccacacaacctgtcagtatcatttgcctttgctcatcatctggcctcttgatcaaattgaaaagtatgtggagaagctgatctcgctctttaggctcaggatgtagacatgctgtacacaatatgagggggatcaactcctctctctttgccaatagcacattgggaacaatgtgtggcaggcagcgtcccagcattaacataacgcttttttcactgtctgcaatacgagacacctcgtatcctaaacgactatctgctgacattcgacaaaaagagagtagtgcttgatggaatgcaggagacaatttcctattaggtttatcaaaatgaactgtctttttacttgatagagaagaaggtggcattccttctctttctctcctggggaatgaatttggggaattctctttaggaatagtggaatcagcttcatctgatattgaaagatggatgtctgtgttttttcccttgtctgaactatttacatctggatgctgtccactgtcctcagagtctttgtggggcaactgatccaaaggaggctgaacagagtcacaaactgctgggatggcaaagtgttcatttttgaggaagtccatttcacttttaagtcttctgatttgctccatcaatgaccatttctcactatttaacaaactaattttatcttctaatttctgtactaacatggagttctctgcaggctggggagtttcaagagttggaggaaggttgcttataattggtgtaagggcctctaattcatcttcttctactccactggccacatctacaagatcttttccagttacttgatgatttccaaaatcccggtagagttgcaataagtctggaggttttggaatgtttaatcctacatcatcccataattcaaaatcctgatcatcgttttcatctgaaaaggttattgatgtaagcttatagttattcttcaataaaaattcattgactaagaagtttagagctctcttttcaagaggtttgattggctcctgaatttcaggacttgatttgtaattttttcgttcctgtaaaggaacttcatgttctgcggcctttgtcaggttggctcggagggcctgaatggtctccttggctttccgtagttcaaactccaggactgccactttttcatctgtttccctgttaccatcatctgaatatcttgcaaagtctaaagaatcaagggtactaatgctcccagctcgattgagctgtcccccgcccgacgctgtactcggttcccgacctccagcgcccccaacgccggctgctccagggacccctggcgcccccatccccggcggggttccactttgcctctcgaagttgcctggattggagaagtagtcgcgcagccgaggcagctcccggccactctctaacagctcggtatgcagctccagggcggtcagcaagtattgatcgcgcaacagctgagcagcgatcgcatcaattgataatcgggccggggtctccccggtgccccccagggccactgcagccgccgacgcctccccagggagccctggccgcgcactgcttcctaaggccacgggatcctgtggcgacagcgagcccgcagagccaggatctaggccacttccggcgcccagccgaagtactgcccgccgttcctctgttgcagctacctcgtcatcgtcctcatccgaatcactgagaaatggattcacgccgccaccactgccactacctccaggcgccatcgccgccatcttatcctgtcaggagtgtgggcgcctccctgactggttccgacgggccgcagcccgaatcctctaggcctcaggggacacagcgcacctccacagccccggcctgaccacgtcctgcctcccgacttagagacaaggagtacgctccaaggcaggagatccggatgcagctgcacctgatgcctcagcctctgctgcaccagcagcccggctctgcaggcgtcttcctggtctccagtctcgcgagaact

SEQ ID NO: 14599 - RNA, 7565 nt, Homo sapiens
  source 1..7565: mol_type = other RNA
gctgggattacaggcatgagccaccgtgcccggccagtctctatttctttttaatgtactgaaaaaaatagtatcaaaactaagcacactgtaaagttacagtagaactttgaaatagatgtctactcatacaaaaggctaaatttattttgtagttttcttgtaagagaattaacatccaaccttgaaggttgaattttgttacctggctaatctggagtatttcatgaattatgaattagaattgctacttacaaagcttttttttttgtttttgagatggagtcttgctctgtggaccaggctggagtgcagtggtgcaatagcggcccactgcaatctccgcttcccaggttcaaacgattctcctgtctcagcctcccgagtagcagggattacaggcccacgtcaccacgcctggctaatttttgtatttttagaggcggggtttcaccacgttggccaggctggtcttgaactactgacctcaagtgattcgtcaccttggcctcccaaagtgctgagattacaggcgtgagccacagcgcacagtccaaagctctttaagtgtaacattgaagagctaaagtgtaactttctttaatgaactgaaaaaattagtacaatctttacacaaagaatagttaagaaaatataaccagcacagaatgttagctgtagttagctactgcagttcaaagatcagcagggtagtaactacagaaagttacatccttggagttcaaataatggtccaaaataggttgtcttgaaaaatgggatgatgaaaagacaattcaatacatcctgatctcacctctctaaattttaagagagactatttgagccaactttttaaaaacaagaatgtgatagcaccttgacttgagacccccattagaattatagtgtatagtagtgacatatcctatagtagtgacatatcctaaaagctatggataatgaggatggcatgacttaaattactcacaatttcgttcaggttgaaaatcaatttgatgtttagcaaaataatctctctaaaggggtgaataatgcaaaccaatgaaggtcatagacacctatgtatagagatagatactgccatcattcaagcactgttcttggaagaattcagctaaattagtaattatggcacttctggatttctgaaaaaatttaatctctggattactctggaaacacaggtataatttcaaattagcttttcattactttgcaaacttagtttttcattaagttgaacacttaaaaacttgtaccgtaagtttacttctgtttaaaaggaatgagtatgggagttttatgccctattttggactcagtccaaatctcagtctcaatgattagtgtctgtcttgtctgtaaagacaagacatattttactaaaaacaaacaaacaaacaaaaaacaaaaccacaatgtgaaatcttaatgatattaaaatatttaagaaaagagactctcacttgaaatacactgtgaatcttgcctactattgcctttaaaaaaacattagcacttaaataaatatattcattaattaagaaaaatgttcacaataaaaatacattctacccattcacctgataacaaacatacacatattctactatagtttgaagcaaatcagagtttaaacatttttcttccaggtacctctgaaatgtattagttttatagcaacatggtccccttttagtaaaaataaaccaaaataggtaaatttatataaattatatttacaaaatattagtatattctcatgaatataggcttttctcatttttttgcttaatagaaagtatagtgtttcaaaacgaaagtaaaatgcatagcccaaaccaaatcaaaaacatatgcaaaaacattttatttataatagatcaacatttttgacatgaaaggtagccactttcaatttctcaggaatgcctagaacccaacagttttcagaaagactacttagttcacaattatttcactgtaggtaaatgaaataatttcagaatgaactttttaaatggctttgcctatggcaaattgttttataaacttgaatgtatggtaagctagctttcccaggaaatgaatgtaatccaactatgttccaaatgtattaaaccagtttatacaacaaatatgagaatcacttatgtgcatcaactgtgctaaaacaagaattctttttatcaaaatattcatttttcaaaaaggcctcacattaacccctcaaaccaagcacccccttcctatgtccagcactcttttctacttcgagttgcatgactgtagagacaactgtcaaattccagtggaactgtacactgacttaagactctatgtaatatacatcaaacacaggaggtcactgactttaagggacgaggtgataactaactagttataattcagccaatgtcttttttagtttagagggaaaaaagtagcccccaagtgtccttaacttttcagtacttctctgtaacacacagaatgaaaaggtactctctaaaattaaaatcattagaaaatatcttaaataaagtgttttacataaataagtgttaaatttcagattcaaactatattttcttctgtatctcaatttgggaaaaatctcacaattattaactcttctcagttacatttatttttgagcatttaaatctactatacaccagtttgtaaaattcaccttggttacctctccccatgcctatgtgctgtctttcctcaggtaagtccattatatgcatctaagtgctggggaggtttaaatagcacttaaagaatattcatgagagttctgaaatgaaggtttcgtctttagctattgactgtaggatttgtaattcaaatcatcacagcatcctaaagaaatactgtgtgaatggaatgcacacaattcctacagaacacacaaactgatgtccaaaaggcacagagtaatgctggtggctctttctagtcagttaagaaacaataaaaagtctgcattattctttcataatttaaatacttaagtaatctccactttattattttataacaatgacttcaaatttacattattttaagtaccattgtaatagcttagtgtataatacagatatttgcgaatatcccatccaaaaattaaaaaaaacttcttcactatatatatatttatataaaaattattctgaaagacaagaacatagacaagggacttggtacagaccatcaactcaattttctatcaccacagttgtaactccaaaatcaacaaatatacagcagtaattaaaagcagtgcaaatatctttggaggttaggataaaattataatgcaagaacataaaactgaggaaacaaaaaaggcaagtacttcaagtacaaggaaccagtcggcttgaggtccatcttagtgtttactgggggcttctttcctgcttctacttctttctctgaaatacattggccaacatggcacctgatgttgtcaactggcccattttgttcaaaaacttggtctttgtatcttcactcactaagcttgcagcaattgacattgagccttgaggctcttggacggtcttgttttcaactttttgttcacattcttttatcatggaacttaaaataacctcatgctctggagagagatgttccatgtcagtccgtaaacatctgagaccaggtaaaaagtgattaaccattaaatcctctgaaatgaaacaacaggaaagtgcactgtaggcttcaaaaagatgcgtagcaatgtccagtcttttagaatccacaatctgtaagttgttcaccaaggctaacttatgcaaatgtggtataacaaactcatctcggaacctgggttctgcgttagggccaactctaccaaatgtttttatgatctctgtatgcaaagaatgttggtcttgatactgaggatcttccaggaaagaagccaactgcattttcactctttccagcaactctctttgaattactgtttccataatagtgccaaaggctggaattgtggcaatcctgacagagaattcaggatcactggacaaggtaacaagggccggagcaacccgcttgtcaactaacgcttcactcatgcctcgaagagtcagatttcagggtcactggagagagtaatgagagcaggaacaaccctctgagctaccagagtttcattcacccccttcaccaacagctcaaacattctagcagcagtacacctcacgagtgctgaagtatggacaacaccataccacaaaacagttaatagtaactcatggtaggctgggtttgcacccaattccacaaaagaagccttcaggctatcaagaggagcatgagataatgaaagcagcgtcattacatcttctaagaatccaactaacagttttcggtcttcttcctgaatataacacgtaaggactcctgttgcataaatggggactgtagctttagtgaggaccccatttcctgctgaggaatcaatgttttcttcagatagtcttaaaatctcctggaactgaggttttaccttagtgtttgtaaaaattttgccaaatgtccggcaaaggcgccagaaaaatctggagaattcatggacacaggcagttgaagtaacattaattttgccaactatttctataagttgtggcaacaattgattgacaacccacagtaaactctcccagcctgttgtaccctcttgttctagctggtagtcataaagttgcagcagcactgccaattgctcacgacttccgataatagtggacacatcttgaagaggcgacataggccgaggaaacctagtcacttctatctgtggcacttcaccatgaagcttggctttgctggagaaaggtgcattctgtagcactaatgcaaagagagatgggatcaaggactgcaaggcagaaagatacatgtggagtttgtgttcatccagtccatgttctccttccctgagaagtttttcaatcttgttcagtagtgtaagtataagatgagactgtaaatttccaagttctgtagtccacgcagcgtaagctggtaaaaatacttgatgtgtagcactaactactctttctgagggatcacccaaggctgacagcaacaattcaaaaccctgatgatatttgtctggatcatcaatgtatcccataatgataccaaggcttttgataacagcttctcttaccaaatctgccttatcttccattaacatttgttgcaacattgaaagaaccaaggagctacggatttctttaggaaggtaaggtgccagtgctccacaggattctgccacaagcagtcgtctttctgggtatttgtgattaattgggttttgttcccatatgtcttcttcatagaatataaatctttctttgactggaaaaggagtatatttgttctcatattcccatatgaaaaggtgacataattcattaatgtattggatgcctgttcccaacactgtggtaaaagttcagcttctacacgtgttggtccaacatgacgcgcaaatgccacacaacctgtcagtatcatttgcctttgctcatcatctggcctcttgatcaaattgaaaagtatgtggagaagctgatctcgctctttaggctcaggatgtagacatgctgtacacaatatgagggggatcaactcctctctctttgccaatagcacattgggaacaatgtgtggcaggcagcgtcccagcattaacataacgcttttttcactgtctgcaatacgagacacctcgtatcctaaacgactatctgctgacattcgacaaaaagagagtagtgcttgatggaatgcaggagacaatttcctattaggtttatcaaaatgaactgtctttttacttgatagagaagaaggtggcattccttctctttctctcctggggaatgaatttggggaattctctttaggaatagtggaatcagcttcatctgatattgaaagatggatgtctgtgttttttcccttgtctgaactatttacatctggatgctgtccactgtcctcagagtctttgtggggcaactgatccaaaggaggctgaacagagtcacaaactgctgggatggcaaagtgttcatttttgaggaagtccatttcacttttaagtcttctgatttgctccatcaatgaccatttctcactatttaacaaactaattttatcttctaatttctgtactaacatggagttctctgcaggctggggagtttcaagagttggaggaaggttgcttataattggtgtaagggcctctaattcatcttcttctactccactggccacatctacaagatcttttccagttacttgatgatttccaaaatcccggtagagttgcaataagtctggaggttttggaatgtttaatcctacatcatcccataattcaaaatcctgatcatcgttttcatctgaaaaggttattgatgtaagcttatagttattcttcaataaaaattcattgactaagaagtttagagctctcttttcaagaggtttgattggctcctgaatttcaggacttgatttgtaattttttcgttcctgtaaaggaacttcatgttctgcggcctttgtcaggttggctcggagggcctgaatggtctccttggctttccgtagttcaaactccaggactgccactttttcatctgtttccctgttaccatcatctgaatatcttgcaaagtctaaagaatcaagggtactaatgctcccagctcgattgagctgtcccccgcccgacgctgtactcggttcccgacctccagcgcccccaacgccggctgctccagggacccctggcgcccccatccccggcggggttccactttgcctctcgaagttgcctggattggagaagtagtcgcgcagccgaggcagctcccggccactctctaacagctcggtatgcagctccagggcggtcagcaagtattgatcgcgcaacagctgagcagcgatcgcatcaattgataatcgggccggggtctccccggtgccccccagggccactgcagccgccgacgcctccccagggagccctggccgcgcactgcttcctaaggccacgggatcctgtggcgacagcgagcccgcagagccaggatctaggccacttccggcgcccagccgaagtactgcccgccgttcctctgttgcagctacctcgtcatcgtcctcatccgaatcactgagaaatggattcacgccgccaccactgccactacctccaggcgccatcgccgccatcttatcctgtcaggagtgtgggcgcctccctgactggttccgacgggccgcagcccgaatcctctaggcctcaggggacacagcgcacctccacagccccggcctgaccacgtcctgcctcccgacttagagacaaggagtacgctccaaggcaggagatccggatgcagctgcacctgatgcctcagcctctgctgcaccagcagcccggctctgcaggcgtcttcctggtctccagtctcgcgagaact

SEQ ID NO: 14600 - RNA, 7360 nt, Homo sapiens
  source 1..7360: mol_type = other RNA
gctgggattacaggcatgagccaccgtgcccggccagtctctatttctttttaatgtactgaaaaaaatagtatcaaaactaagcacactgtaaagttacagtagaactttgaaatagatgtctactcatacaaaaggctaaatttattttgtagttttcttgtaagagaattaacatccaaccttgaaggttgaattttgttacctggctaatctggagtatttcatgaattatgaattagaattgctacttacaaagcttttttttttgtttttgagatggagtcttgctctgtggaccaggctggagtgcagtggtgcaatagcggcccactgcaatctccgcttcccaggttcaaacgattctcctgtctcagcctcccgagtagcagggattacaggcccacgtcaccacgcctggctaatttttgtatttttagaggcggggtttcaccacgttggccaggctggtcttgaactactgacctcaagtgattcgtcaccttggcctcccaaagtgctgagattacaggcgtgagccacagcgcacagtccaaagctctttaagtgtaacattgaagagctaaagtgtaactttctttaatgaactgaaaaaattagtacaatctttacacaaagaatagttaagaaaatataaccagcacagaatgttagctgtagttagctactgcagttcaaagatcagcagggtagtaactacagaaagttacatccttggagttcaaataatggtccaaaataggttgtcttgaaaaatgggatgatgaaaagacaattcaatacatcctgatctcacctctctaaattttaagagagactatttgagccaactttttaaaaacaagaatgtgatagcaccttgacttgagacccccattagaattatagtgtatagtagtgacatatcctatagtagtgacatatcctaaaagctatggataatgaggatggcatgacttaaattactcacaatttcgttcaggttgaaaatcaatttgatgtttagcaaaataatctctctaaaggggtgaataatgcaaaccaatgaaggtcatagacacctatgtatagagatagatactgccatcattcaagcactgttcttggaagaattcagctaaattagtaattatggcacttctggatttctgaaaaaatttaatctctggattactctggaaacacaggtataatttcaaattagcttttcattactttgcaaacttagtttttcattaagttgaacacttaaaaacttgtaccgtaagtttacttctgtttaaaaggaatgagtatgggagttttatgccctattttggactcagtccaaatctcagtctcaatgattagtgtctgtcttgtctgtaaagacaagacatattttactaaaaacaaacaaacaaacaaaaaacaaaaccacaatgtgaaatcttaatgatattaaaatatttaagaaaagagactctcacttgaaatacactgtgaatcttgcctactattgcctttaaaaaaacattagcacttaaataaatatattcattaattaagaaaaatgttcacaataaaaatacattctacccattcacctgataacaaacatacacatattctactatagtttgaagcaaatcagagtttaaacatttttcttccaggtacctctgaaatgtattagttttatagcaacatggtccccttttagtaaaaataaaccaaaataggtaaatttatataaattatatttacaaaatattagtatattctcatgaatataggcttttctcatttttttgcttaatagaaagtatagtgtttcaaaacgaaagtaaaatgcatagcccaaaccaaatcaaaaacatatgcaaaaacattttatttataatagatcaacatttttgacatgaaaggtagccactttcaatttctcaggaatgcctagaacccaacagttttcagaaagactacttagttcacaattatttcactgtaggtaaatgaaataatttcagaatgaactttttaaatggctttgcctatggcaaattgttttataaacttgaatgtatggtaagctagctttcccaggaaatgaatgtaatccaactatgttccaaatgtattaaaccagtttatacaacaaatatgagaatcacttatgtgcatcaactgtgctaaaacaagaattctttttatcaaaatattcatttttcaaaaaggcctcacattaacccctcaaaccaagcacccccttcctatgtccagcactcttttctacttcgagttgcatgactgtagagacaactgtcaaattccagtggaactgtacactgacttaagactctatgtaatatacatcaaacacaggaggtcactgactttaagggacgaggtgataactaactagttataattcagccaatgtcttttttagtttagagggaaaaaagtagcccccaagtgtccttaacttttcagtacttctctgtaacacacagaatgaaaaggtactctctaaaattaaaatcattagaaaatatcttaaataaagtgttttacataaataagtgttaaatttcagattcaaactatattttcttctgtatctcaatttgggaaaaatctcacaattattaactcttctcagttacatttatttttgagcatttaaatctactatacaccagtttgtaaaattcaccttggttacctctccccatgcctatgtgctgtctttcctcaggtaagtccattatatgcatctaagtgctggggaggtttaaatagcacttaaagaatattcatgagagttctgaaatgaaggtttcgtctttagctattgactgtaggatttgtaattcaaatcatcacagcatcctaaagaaatactgtgtgaatggaatgcacacaattcctacagaacacacaaactgatgtccaaaaggcacagagtaatgctggtggctctttctagtcagttaagaaacaataaaaagtctgcattattctttcataatttaaatacttaagtaatctccactttattattttataacaatgacttcaaatttacattattttaagtaccattgtaatagcttagtgtataatacagatatttgcgaatatcccatccaaaaattaaaaaaaacttcttcactatatatatatttatataaaaattattctgaaagacaagaacatagacaagggacttggtacagaccatcaactcaattttctatcaccacagttgtaactccaaaatcaacaaatatacagcagtaattaaaagcagtgcaaatatctttggaggttaggataaaattataatgcaagaacataaaactgaggaaacaaaaaaggcaagtacttcaagtacaaggaaccagtcggcttgaggtccatcttagtgtttactgggggcttctttcctgcttctacttctttctctgaaatacattggccaacatggcacctgatgttgtcaactggcccattttgttcaaaaacttggtctttgtatcttcactcactaagcttgcagcaattgacattgagccttgaggctcttggacggtcttgttttcaactttttgttcacattcttttatcatggaacttaaaataacctcatgctctggagagagatgttccatgtcagtccgtaaacatctgagaccaggtaaaaagtgattaaccattaaatcctctgaaatgaaacaacaggaaagtgcactgtaggcttcaaaaagatgcgtagcaatgtccagtcttttagaatccacaatctgtaagttgttcaccaaggctaacttatgcaaatgtggtataacaaactcatctcggaacctgggttctgcgttagggccaactctaccaaatgtttttatgatctctgtatgcaaagaatgttggtcttgatactgaggatcttccaggaaagaagccaactgcattttcactctttccagcaactctctttgaattactgtttccataatagtgccaaaggctggaattgtggcaatcctgacagagaattcaggatcactggacaaggtaacaagggccggagcaacccgcttgtcaactaacgcttcactcatgcctcgaagagtcagctcaaacattctagcagcagtacacctcacgagtgctgaagtatggacaacaccataccacaaaacagttaatagtaactcatggtaggctgggtttgcacccaattccacaaaagaagccttcaggctatcaagaggagcatgagataatgaaagcagcgtcattacatcttctaagaatccaactaacagttttcggtcttcttcctgaatataacacgtaaggactcctgttgcataaatggggactgtagctttagtgaggaccccatttcctgctgaggaatcaatgttttcttcagatagtcttaaaatctcctggaactgaggttttaccttagtgtttgtaaaaattttgccaaatgtccggcaaaggcgccagaaaaatctggagaattcatggacacaggcagttgaagtaacattaattttgccaactatttctataagttgtggcaacaattgattgacaacccacagtaaactctcccagcctgttgtaccctcttgttctagctggtagtcataaagttgcagcagcactgccaattgctcacgacttccgataatagtggacacatcttgaagaggcgacataggccgaggaaacctagtcacttctatctgtggcacttcaccatgaagcttggctttgctggagaaaggtgcattctgtagcactaatgcaaagagagatgggatcaaggactgcaaggcagaaagatacatgtggagtttgtgttcatccagtccatgttctccttccctgagaagtttttcaatcttgttcagtagtgtaagtataagatgagactgtaaatttccaagttctgtagtccacgcagcgtaagctggtaaaaatacttgatgtgtagcactaactactctttctgagggatcacccaaggctgacagcaacaattcaaaaccctgatgatatttgtctggatcatcaatgtatcccataatgataccaaggcttttgataacagcttctcttaccaaatctgccttatcttccattaacatttgttgcaacattgaaagaaccaaggagctacggatttctttaggaaggtaaggtgccagtgctccacaggattctgccacaagcagtcgtctttctgggtatttgtgattaatctgttcccaacactgtggtaaaagttcagcttctacacgtgttggtccaacatgacgcgcaaatgccacacaacctgtcagtatcatttgcctttgctcatcatctggcctcttgatcaaattgaaaagtatgtggagaagctgatctcgctctttaggctcaggatgtagacatgctgtacacaatatgagggggatcaactcctctctctttgccaatagcacattgggaacaatgtgtggcaggcagcgtcccagcattaacataacgcttttttcactgtctgcaatacgagacacctcgtatcctaaacgactatctgctgacattcgacaaaaagagagtagtgcttgatggaatgcaggagacaatttcctattaggtttatcaaaatgaactgtctttttacttgatagagaagaaggtggcattccttctctttctctcctggggaatgaatttggggaattctctttaggaatagtggaatcagcttcatctgatattgaaagatggatgtctgtgttttttcccttgtctgaactatttacatctggatgctgtccactgtcctcagagtctttgtggggcaactgatccaaaggaggctgaacagagtcacaaactgctgggatggcaaagtgttcatttttgaggaagtccatttcacttttaagtcttctgatttgctccatcaatgaccatttctcactatttaacaaactaattttatcttctaatttctgtactaacatggagttctctgcaggctggggagtttcaagagttggaggaaggttgcttataattggtgtaagggcctctaattcatcttcttctactccactggccacatctacaagatcttttccagttacttgatgatttccaaaatcccggtagagttgcaataagtctggaggttttggaatgtttaatcctacatcatcccataattcaaaatcctgatcatcgttttcatctgaaaaggttattgatgtaagcttatagttattcttcaataaaaattcattgactaagaagtttagagctctcttttcaagaggtttgattggctcctgaatttcaggacttgatttgtaattttttcgttcctgtaaaggaacttcatgttctgcggcctttgtcaggttggctcggagggcctgaatggtctccttggctttccgtagttcaaactccaggactgccactttttcatctgtttccctgttaccatcatctgaatatcttgcaaagtctaaagaatcaagggtactaatgctcccagctcgattgagctgtcccccgcccgacgctgtactcggttcccgacctccagcgcccccaacgccggctgctccagggacccctggcgcccccatccccggcggggttccactttgcctctcgaagttgcctggattggagaagtagtcgcgcagccgaggcagctcccggccactctctaacagctcggtatgcagctccagggcggtcagcaagtattgatcgcgcaacagctgagcagcgatcgcatcaattgataatcgggccggggtctccccggtgccccccagggccactgcagccgccgacgcctccccagggagccctggccgcgcactgcttcctaaggccacgggatcctgtggcgacagcgagcccgcagagccaggatctaggccacttccggcgcccagccgaagtactgcccgccgttcctctgttgcagctacctcgtcatcgtcctcatccgaatcactgagaaatggattcacgccgccaccactgccactacctccaggcgccatcgccgccatcttatcctgtcaggagtgtgggcgcctccctgactggttccgacgggccgcagcccgaatcctctaggcctcaggggacacagcgcacctccacagccccggcctgaccacgtcctgcctcccgacttagagacaaggagtacgctccaaggcaggagatccggatgcagctgcacctgatgcctcagcctctgctgcaccagcagcccggctctgcaggcgtcttcctggtctccagtctcgcgagaact

SEQ ID NO: 14601 - RNA, 7534 nt, Homo sapiens
  source 1..7534: mol_type = other RNA
gctgggattacaggcatgagccaccgtgcccggccagtctctatttctttttaatgtactgaaaaaaatagtatcaaaactaagcacactgtaaagttacagtagaactttgaaatagatgtctactcatacaaaaggctaaatttattttgtagttttcttgtaagagaattaacatccaaccttgaaggttgaattttgttacctggctaatctggagtatttcatgaattatgaattagaattgctacttacaaagcttttttttttgtttttgagatggagtcttgctctgtggaccaggctggagtgcagtggtgcaatagcggcccactgcaatctccgcttcccaggttcaaacgattctcctgtctcagcctcccgagtagcagggattacaggcccacgtcaccacgcctggctaatttttgtatttttagaggcggggtttcaccacgttggccaggctggtcttgaactactgacctcaagtgattcgtcaccttggcctcccaaagtgctgagattacaggcgtgagccacagcgcacagtccaaagctctttaagtgtaacattgaagagctaaagtgtaactttctttaatgaactgaaaaaattagtacaatctttacacaaagaatagttaagaaaatataaccagcacagaatgttagctgtagttagctactgcagttcaaagatcagcagggtagtaactacagaaagttacatccttggagttcaaataatggtccaaaataggttgtcttgaaaaatgggatgatgaaaagacaattcaatacatcctgatctcacctctctaaattttaagagagactatttgagccaactttttaaaaacaagaatgtgatagcaccttgacttgagacccccattagaattatagtgtatagtagtgacatatcctatagtagtgacatatcctaaaagctatggataatgaggatggcatgacttaaattactcacaatttcgttcaggttgaaaatcaatttgatgtttagcaaaataatctctctaaaggggtgaataatgcaaaccaatgaaggtcatagacacctatgtatagagatagatactgccatcattcaagcactgttcttggaagaattcagctaaattagtaattatggcacttctggatttctgaaaaaatttaatctctggattactctggaaacacaggtataatttcaaattagcttttcattactttgcaaacttagtttttcattaagttgaacacttaaaaacttgtaccgtaagtttacttctgtttaaaaggaatgagtatgggagttttatgccctattttggactcagtccaaatctcagtctcaatgattagtgtctgtcttgtctgtaaagacaagacatattttactaaaaacaaacaaacaaacaaaaaacaaaaccacaatgtgaaatcttaatgatattaaaatatttaagaaaagagactctcacttgaaatacactgtgaatcttgcctactattgcctttaaaaaaacattagcacttaaataaatatattcattaattaagaaaaatgttcacaataaaaatacattctacccattcacctgataacaaacatacacatattctactatagtttgaagcaaatcagagtttaaacatttttcttccaggtacctctgaaatgtattagttttatagcaacatggtccccttttagtaaaaataaaccaaaataggtaaatttatataaattatatttacaaaatattagtatattctcatgaatataggcttttctcatttttttgcttaatagaaagtatagtgtttcaaaacgaaagtaaaatgcatagcccaaaccaaatcaaaaacatatgcaaaaacattttatttataatagatcaacatttttgacatgaaaggtagccactttcaatttctcaggaatgcctagaacccaacagttttcagaaagactacttagttcacaattatttcactgtaggtaaatgaaataatttcagaatgaactttttaaatggctttgcctatggcaaattgttttataaacttgaatgtatggtaagctagctttcccaggaaatgaatgtaatccaactatgttccaaatgtattaaaccagtttatacaacaaatatgagaatcacttatgtgcatcaactgtgctaaaacaagaattctttttatcaaaatattcatttttcaaaaaggcctcacattaacccctcaaaccaagcacccccttcctatgtccagcactcttttctacttcgagttgcatgactgtagagacaactgtcaaattccagtggaactgtacactgacttaagactctatgtaatatacatcaaacacaggaggtcactgactttaagggacgaggtgataactaactagttataattcagccaatgtcttttttagtttagagggaaaaaagtagcccccaagtgtccttaacttttcagtacttctctgtaacacacagaatgaaaaggtactctctaaaattaaaatcattagaaaatatcttaaataaagtgttttacataaataagtgttaaatttcagattcaaactatattttcttctgtatctcaatttgggaaaaatctcacaattattaactcttctcagttacatttatttttgagcatttaaatctactatacaccagtttgtaaaattcaccttggttacctctccccatgcctatgtgctgtctttcctcaggtaagtccattatatgcatctaagtgctggggaggtttaaatagcacttaaagaatattcatgagagttctgaaatgaaggtttcgtctttagctattgactgtaggatttgtaattcaaatcatcacagcatcctaaagaaatactgtgtgaatggaatgcacacaattcctacagaacacacaaactgatgtccaaaaggcacagagtaatgctggtggctctttctagtcagttaagaaacaataaaaagtctgcattattctttcataatttaaatacttaagtaatctccactttattattttataacaatgacttcaaatttacattattttaagtaccattgtaatagcttagtgtataatacagatatttgcgaatatcccatccaaaaattaaaaaaaacttcttcactatatatatatttatataaaaattattctgaaagacaagaacatagacaagggacttggtacagaccatcaactcaattttctatcaccacagttgtaactccaaaatcaacaaatatacagcagtaattaaaagcagtgcaaatatctttggaggttaggataaaattataatgcaagaacataaaactgaggaaacaaaaaaggcaagtacttcaagtacaaggaaccagtcggcttgaggtccatcttagtgtttactgggggcttctttcctgcttctacttctttctctgaaatacattggccaacatggcacctgatgttgtcaactggcccattttgttcaaaaacttggtctttgtatcttcactcactaagcttgcagcaattgacattgagccttgaggctcttggacggtcttgttttcaactttttgttcacattcttttatcatggaacttaaaataacctcatgctctggagagagatgttccatgtcagtccgtaaacatctgagaccaggtaaaaagtgattaaccattaaatcctctgaaatgaaacaacaggaaagtgcactgtaggcttcaaaaagatgcgtagcaatgtccagtcttttagaatccacaatctgtaagttgttcaccaaggctaacttatgcaaatgtggtataacaaactcatctcggaacctgggttctgcgttagggccaactctaccaaatgtttttatgatctctgtatgcaaagaatgttggtcttgatactgaggatcttccaggaaagaagccaactgcattttcactctttccagcaactctctttgaattactgtttccataatagtgccaaaggctggaattgtggcaatcctgacagagatttcagggtcactggagagagtaatgagagcaggaacaaccctctgagctaccagagtttcattcacccccttcaccaacagcctattaggttcctggtatatgtatgcctcattttcttctcatttctcattttcttttctttctggtcttacctcaaacattctagcagcagtacacctcacgagtgctgaagtatggacaacaccataccacaaaacagttaatagtaactcatggtaggctgggtttgcacccaattccacaaaagaagccttcaggctatcaagaggagcatgagataatgaaagcagcgtcattacatcttctaagaatccaactaacagttttcggtcttcttccttcaggctatgtgtataatgtgtatatgaaacacattttgtgtttagacttgggtcccattcccaagatatctcattatgtatatgcaaatactcctttatctgaatataacacgtaaggactcctgttgcataaatggggactgtagctttagtgaggaccccatttcctgctgaggaatcaatgttttcttcagatagtcttaaaatctcctggaactgaggttttaccttagtgtttgtaaaaattttgccaaatgtccggcaaaggcgccagaaaaatctggagaattcatggacacaggcagttgaagtaacattaattttgccaactatttctataagttgtggcaacaattgattgacaacccacagtaaactctcccagcctgttgtaccctcttgttctagctggtagtcataaagttgcagcagcactgccaattgctcacgacttccgataatagtggacacatcttgaagaggcgacataggccgaggaaacctagtcacttctatctgtggcacttcaccatgaagcttggctttgctggagaaaggtgcattctgtagcactaatgcaaagagagatgggatcaaggactgcaaggcagaaagatacatgtggagtttgtgttcatccagtccatgttctccttccctgagaagtttttcaatcttgttcagtagtgtaagtataagatgagactgtaaatttccaagttctgtagtccacgcagcgtaagctggtaaaaatacttgatgtgtagcactaactactctttctgagggatcacccaaggctgacagcaacaattcaaaaccctgatgatatttgtctggatcatcaatgtatcccataatgataccaaggcttttgataacagcttctcttaccaaatctgccttatcttccattaacatttgttgcaacattgaaagaaccaaggagctacggatttctttaggaaggtaaggtgccagtgctccacaggattctgccacaagcagtcgtctttctgggtatttgtgattaatctgttcccaacactgtggtaaaagttcagcttctacacgtgttggtccaacatgacgcgcaaatgccacacaacctgtcagtatcatttgcctttgctcatcatctggcctcttgatcaaattgaaaagtatgtggagaagctgatctcgctctttaggctcaggatgtagacatgctgtacacaatatgagggggatcaactcctctctctttgccaatagcacattgggaacaatgtgtggcaggcagcgtcccagcattaacataacgcttttttcactgtctgcaatacgagacacctcgtatcctaaacgactatctgctgacattcgacaaaaagagagtagtgcttgatggaatgcaggagacaatttcctattaggtttatcaaaatgaactgtctttttacttgatagagaagaaggtggcattccttctctttctctcctggggaatgaatttggggaattctctttaggaatagtggaatcagcttcatctgatattgaaagatggatgtctgtgttttttcccttgtctgaactatttacatctggatgctgtccactgtcctcagagtctttgtggggcaactgatccaaaggaggctgaacagagtcacaaactgctgggatggcaaagtgttcatttttgaggaagtccatttcacttttaagtcttctgatttgctccatcaatgaccatttctcactatttaacaaactaattttatcttctaatttctgtactaacatggagttctctgcaggctggggagtttcaagagttggaggaaggttgcttataattggtgtaagggcctctaattcatcttcttctactccactggccacatctacaagatcttttccagttacttgatgatttccaaaatcccggtagagttgcaataagtctggaggttttggaatgtttaatcctacatcatcccataattcaaaatcctgatcatcgttttcatctgaaaaggttattgatgtaagcttatagttattcttcaataaaaattcattgactaagaagtttagagctctcttttcaagaggtttgattggctcctgaatttcaggacttgatttgtaattttttcgttcctgtaaaggaacttcatgttctgcggcctttgtcaggttggctcggagggcctgaatggtctccttggctttccgtagttcaaactccaggactgccactttttcatctgtttccctgttaccatcatctgaatatcttgcaaagtctaaagaatcaagggtactaatgctcccagctcgattgagctgtcccccgcccgacgctgtactcggttcccgacctccagcgcccccaacgccggctgctccagggacccctggcgcccccatccccggcggggttccactttgcctctcgaagttgcctggattggagaagtagtcgcgcagccgaggcagctcccggccactctctaacagctcggtatgcagctccagggcggtcagcaagtattgatcgcgcaacagctgagcagcgatcgcatcaattgataatcgggccggggtctccccggtgccccccagggccactgcagccgccgacgcctccccagggagccctggccgcgcactgcttcctaaggccacgggatcctgtggcgacagcgagcccgcagagccaggatctaggccacttccggcgcccagccgaagtactgcccgccgttcctctgttgcagctacctcgtcatcgtcctcatccgaatcactgagaaatggattcacgccgccaccactgccactacctccaggcgccatcgccgccatcttatcctgtcaggagtgtgggcgcctccctgactggttccgacgggccgcagcccgaatcctctaggcctcaggggacacagcgcacctccacagccccggcctgaccacgtcctgcctcccgacttagagacaaggagtacgctccaaggcaggagatccggatgcagctgcacctgatgcctcagcctctgctgcaccagcagcccggctctgcaggcgtcttcctggtctccagtctcgcgagaact

SEQ ID NO: 14602 - RNA, 7348 nt, Homo sapiens
  source 1..7348: mol_type = other RNA
gctgggattacaggcatgagccaccgtgcccggccagtctctatttctttttaatgtactgaaaaaaatagtatcaaaactaagcacactgtaaagttacagtagaactttgaaatagatgtctactcatacaaaaggctaaatttattttgtagttttcttgtaagagaattaacatccaaccttgaaggttgaattttgttacctggctaatctggagtatttcatgaattatgaattagaattgctacttacaaagcttttttttttgtttttgagatggagtcttgctctgtggaccaggctggagtgcagtggtgcaatagcggcccactgcaatctccgcttcccaggttcaaacgattctcctgtctcagcctcccgagtagcagggattacaggcccacgtcaccacgcctggctaatttttgtatttttagaggcggggtttcaccacgttggccaggctggtcttgaactactgacctcaagtgattcgtcaccttggcctcccaaagtgctgagattacaggcgtgagccacagcgcacagtccaaagctctttaagtgtaacattgaagagctaaagtgtaactttctttaatgaactgaaaaaattagtacaatctttacacaaagaatagttaagaaaatataaccagcacagaatgttagctgtagttagctactgcagttcaaagatcagcagggtagtaactacagaaagttacatccttggagttcaaataatggtccaaaataggttgtcttgaaaaatgggatgatgaaaagacaattcaatacatcctgatctcacctctctaaattttaagagagactatttgagccaactttttaaaaacaagaatgtgatagcaccttgacttgagacccccattagaattatagtgtatagtagtgacatatcctatagtagtgacatatcctaaaagctatggataatgaggatggcatgacttaaattactcacaatttcgttcaggttgaaaatcaatttgatgtttagcaaaataatctctctaaaggggtgaataatgcaaaccaatgaaggtcatagacacctatgtatagagatagatactgccatcattcaagcactgttcttggaagaattcagctaaattagtaattatggcacttctggatttctgaaaaaatttaatctctggattactctggaaacacaggtataatttcaaattagcttttcattactttgcaaacttagtttttcattaagttgaacacttaaaaacttgtaccgtaagtttacttctgtttaaaaggaatgagtatgggagttttatgccctattttggactcagtccaaatctcagtctcaatgattagtgtctgtcttgtctgtaaagacaagacatattttactaaaaacaaacaaacaaacaaaaaacaaaaccacaatgtgaaatcttaatgatattaaaatatttaagaaaagagactctcacttgaaatacactgtgaatcttgcctactattgcctttaaaaaaacattagcacttaaataaatatattcattaattaagaaaaatgttcacaataaaaatacattctacccattcacctgataacaaacatacacatattctactatagtttgaagcaaatcagagtttaaacatttttcttccaggtacctctgaaatgtattagttttatagcaacatggtccccttttagtaaaaataaaccaaaataggtaaatttatataaattatatttacaaaatattagtatattctcatgaatataggcttttctcatttttttgcttaatagaaagtatagtgtttcaaaacgaaagtaaaatgcatagcccaaaccaaatcaaaaacatatgcaaaaacattttatttataatagatcaacatttttgacatgaaaggtagccactttcaatttctcaggaatgcctagaacccaacagttttcagaaagactacttagttcacaattatttcactgtaggtaaatgaaataatttcagaatgaactttttaaatggctttgcctatggcaaattgttttataaacttgaatgtatggtaagctagctttcccaggaaatgaatgtaatccaactatgttccaaatgtattaaaccagtttatacaacaaatatgagaatcacttatgtgcatcaactgtgctaaaacaagaattctttttatcaaaatattcatttttcaaaaaggcctcacattaacccctcaaaccaagcacccccttcctatgtccagcactcttttctacttcgagttgcatgactgtagagacaactgtcaaattccagtggaactgtacactgacttaagactctatgtaatatacatcaaacacaggaggtcactgactttaagggacgaggtgataactaactagttataattcagccaatgtcttttttagtttagagggaaaaaagtagcccccaagtgtccttaacttttcagtacttctctgtaacacacagaatgaaaaggtactctctaaaattaaaatcattagaaaatatcttaaataaagtgttttacataaataagtgttaaatttcagattcaaactatattttcttctgtatctcaatttgggaaaaatctcacaattattaactcttctcagttacatttatttttgagcatttaaatctactatacaccagtttgtaaaattcaccttggttacctctccccatgcctatgtgctgtctttcctcaggtaagtccattatatgcatctaagtgctggggaggtttaaatagcacttaaagaatattcatgagagttctgaaatgaaggtttcgtctttagctattgactgtaggatttgtaattcaaatcatcacagcatcctaaagaaatactgtgtgaatggaatgcacacaattcctacagaacacacaaactgatgtccaaaaggcacagagtaatgctggtggctctttctagtcagttaagaaacaataaaaagtctgcattattctttcataatttaaatacttaagtaatctccactttattattttataacaatgacttcaaatttacattattttaagtaccattgtaatagcttagtgtataatacagatatttgcgaatatcccatccaaaaattaaaaaaaacttcttcactatatatatatttatataaaaattattctgaaagacaagaacatagacaagggacttggtacagaccatcaactcaattttctatcaccacagttgtaactccaaaatcaacaaatatacagcagtaattaaaagcagtgcaaatatctttggaggttaggataaaattataatgcaagaacataaaactgaggaaacaaaaaaggcaagtacttcaagtacaaggaaccagtcggcttgaggtccatcttagtgtttactgggggcttctttcctgcttctacttctttctctgaaatacattggccaacatggcacctgatgttgtcaactggcccattttgttcaaaaacttggtctttgtatcttcactcactaagcttgcagcaattgacattgagccttgaggctcttggacggtcttgttttcaactttttgttcacattcttttatcatggaacttaaaataacctcatgctctggagagagatgttccatgtcagtccgtaaacatctgagaccaggtaaaaagtgattaaccattaaatcctctgaaatgaaacaacaggaaagtgcactgtaggcttcaaaaagatgcgtagcaatgtccagtcttttagaatccacaatctgtaagttgttcaccaaggctaacttatgcaaatgtggtataacaaactcatctcggaacctgggttctgcgttagggccaactctaccaaatgtttttatgatctctgtatgcaaagaatgttggtcttgatactgaggatcttccaggaaagaagccaactgcattttcactctttccagcaactctctttgaattactgtttccataatagtgccaaaggctggaattgtggcaatcctgacagagatttcagggtcactggagagagtaatgagagcaggaacaaccctctgagctaccagagtttcattcacccccttcaccaacagctcaaacattctagcagcagtacacctcacgagtgctgaagtatggacaacaccataccacaaaacagttaatagtaactcatggtaggctgggtttgcacccaattccacaaaagaagccttcaggctatcaagaggagcatgagataatgaaagcagcgtcattacatcttctaagaatccaactaacagttttcggtcttcttcctgaatataacacgtaaggactcctgttgcataaatggggactgtagctttagtgaggaccccatttccaatgttttcttcagatagtcttaaaatctcctggaactgaggttttaccttagtgtttgtaaaaattttgccaaatgtccggcaaaggcgccagaaaaatctggagaattcatggacacaggcagttgaagtaacattaattttgccaactatttctataagttgtggcaacaattgattgacaacccacagtaaactctcccagcctgttgtaccctcttgttctagctggtagtcataaagttgcagcagcactgccaattgctcacgacttccgataatagtggacacatcttgaagaggcgacataggccgaggaaacctagtcacttctatctgtggcacttcaccatgaagcttggctttgctggagaaaggtgcattctgtagcactaatgcaaagagagatgggatcaaggactgcaaggcagaaagatacatgtggagtttgtgttcatccagtccatgttctccttccctgagaagtttttcaatcttgttcagtagtgtaagtataagatgagactgtaaatttccaagttctgtagtccacgcagcgtaagctggtaaaaatacttgatgtgtagcactaactactctttctgagggatcacccaaggctgacagcaacaattcaaaaccctgatgatatttgtctggatcatcaatgtatcccataatgataccaaggcttttgataacagcttctcttaccaaatctgccttatcttccattaacatttgttgcaacattgaaagaaccaaggagctacggatttctttaggaaggtaaggtgccagtgctccacaggattctgccacaagcagtcgtctttctgggtatttgtgattaatctgttcccaacactgtggtaaaagttcagcttctacacgtgttggtccaacatgacgcgcaaatgccacacaacctgtcagtatcatttgcctttgctcatcatctggcctcttgatcaaattgaaaagtatgtggagaagctgatctcgctctttaggctcaggatgtagacatgctgtacacaatatgagggggatcaactcctctctctttgccaatagcacattgggaacaatgtgtggcaggcagcgtcccagcattaacataacgcttttttcactgtctgcaatacgagacacctcgtatcctaaacgactatctgctgacattcgacaaaaagagagtagtgcttgatggaatgcaggagacaatttcctattaggtttatcaaaatgaactgtctttttacttgatagagaagaaggtggcattccttctctttctctcctggggaatgaatttggggaattctctttaggaatagtggaatcagcttcatctgatattgaaagatggatgtctgtgttttttcccttgtctgaactatttacatctggatgctgtccactgtcctcagagtctttgtggggcaactgatccaaaggaggctgaacagagtcacaaactgctgggatggcaaagtgttcatttttgaggaagtccatttcacttttaagtcttctgatttgctccatcaatgaccatttctcactatttaacaaactaattttatcttctaatttctgtactaacatggagttctctgcaggctggggagtttcaagagttggaggaaggttgcttataattggtgtaagggcctctaattcatcttcttctactccactggccacatctacaagatcttttccagttacttgatgatttccaaaatcccggtagagttgcaataagtctggaggttttggaatgtttaatcctacatcatcccataattcaaaatcctgatcatcgttttcatctgaaaaggttattgatgtaagcttatagttattcttcaataaaaattcattgactaagaagtttagagctctcttttcaagaggtttgattggctcctgaatttcaggacttgatttgtaattttttcgttcctgtaaaggaacttcatgttctgcggcctttgtcaggttggctcggagggcctgaatggtctccttggctttccgtagttcaaactccaggactgccactttttcatctgtttccctgttaccatcatctgaatatcttgcaaagtctaaagaatcaagggtactaatgctcccagctcgattgagctgtcccccgcccgacgctgtactcggttcccgacctccagcgcccccaacgccggctgctccagggacccctggcgcccccatccccggcggggttccactttgcctctcgaagttgcctggattggagaagtagtcgcgcagccgaggcagctcccggccactctctaacagctcggtatgcagctccagggcggtcagcaagtattgatcgcgcaacagctgagcagcgatcgcatcaattgataatcgggccggggtctccccggtgccccccagggccactgcagccgccgacgcctccccagggagccctggccgcgcactgcttcctaaggccacgggatcctgtggcgacagcgagcccgcagagccaggatctaggccacttccggcgcccagccgaagtactgcccgccgttcctctgttgcagctacctcgtcatcgtcctcatccgaatcactgagaaatggattcacgccgccaccactgccactacctccaggcgccatcgccgccatcttatcctgtcaggagtgtgggcgcctccctgactggttccgacgggccgcagcccgaatcctctaggcctcaggggacacagcgcacctccacagccccggcctgaccacgtcctgcctcccgacttagagacaaggagtacgctccaaggcaggagatccggatgcagctgcacctgatgcctcagcctctgctgcaccagcagcccggctctgcaggcgtcttcctggtctccagtctcgcgagaact

SEQ ID NO: 14603 - RNA, 7360 nt, Homo sapiens
  source 1..7360: mol_type = other RNA
gctgggattacaggcatgagccaccgtgcccggccagtctctatttctttttaatgtactgaaaaaaatagtatcaaaactaagcacactgtaaagttacagtagaactttgaaatagatgtctactcatacaaaaggctaaatttattttgtagttttcttgtaagagaattaacatccaaccttgaaggttgaattttgttacctggctaatctggagtatttcatgaattatgaattagaattgctacttacaaagcttttttttttgtttttgagatggagtcttgctctgtggaccaggctggagtgcagtggtgcaatagcggcccactgcaatctccgcttcccaggttcaaacgattctcctgtctcagcctcccgagtagcagggattacaggcccacgtcaccacgcctggctaatttttgtatttttagaggcggggtttcaccacgttggccaggctggtcttgaactactgacctcaagtgattcgtcaccttggcctcccaaagtgctgagattacaggcgtgagccacagcgcacagtccaaagctctttaagtgtaacattgaagagctaaagtgtaactttctttaatgaactgaaaaaattagtacaatctttacacaaagaatagttaagaaaatataaccagcacagaatgttagctgtagttagctactgcagttcaaagatcagcagggtagtaactacagaaagttacatccttggagttcaaataatggtccaaaataggttgtcttgaaaaatgggatgatgaaaagacaattcaatacatcctgatctcacctctctaaattttaagagagactatttgagccaactttttaaaaacaagaatgtgatagcaccttgacttgagacccccattagaattatagtgtatagtagtgacatatcctatagtagtgacatatcctaaaagctatggataatgaggatggcatgacttaaattactcacaatttcgttcaggttgaaaatcaatttgatgtttagcaaaataatctctctaaaggggtgaataatgcaaaccaatgaaggtcatagacacctatgtatagagatagatactgccatcattcaagcactgttcttggaagaattcagctaaattagtaattatggcacttctggatttctgaaaaaatttaatctctggattactctggaaacacaggtataatttcaaattagcttttcattactttgcaaacttagtttttcattaagttgaacacttaaaaacttgtaccgtaagtttacttctgtttaaaaggaatgagtatgggagttttatgccctattttggactcagtccaaatctcagtctcaatgattagtgtctgtcttgtctgtaaagacaagacatattttactaaaaacaaacaaacaaacaaaaaacaaaaccacaatgtgaaatcttaatgatattaaaatatttaagaaaagagactctcacttgaaatacactgtgaatcttgcctactattgcctttaaaaaaacattagcacttaaataaatatattcattaattaagaaaaatgttcacaataaaaatacattctacccattcacctgataacaaacatacacatattctactatagtttgaagcaaatcagagtttaaacatttttcttccaggtacctctgaaatgtattagttttatagcaacatggtccccttttagtaaaaataaaccaaaataggtaaatttatataaattatatttacaaaatattagtatattctcatgaatataggcttttctcatttttttgcttaatagaaagtatagtgtttcaaaacgaaagtaaaatgcatagcccaaaccaaatcaaaaacatatgcaaaaacattttatttataatagatcaacatttttgacatgaaaggtagccactttcaatttctcaggaatgcctagaacccaacagttttcagaaagactacttagttcacaattatttcactgtaggtaaatgaaataatttcagaatgaactttttaaatggctttgcctatggcaaattgttttataaacttgaatgtatggtaagctagctttcccaggaaatgaatgtaatccaactatgttccaaatgtattaaaccagtttatacaacaaatatgagaatcacttatgtgcatcaactgtgctaaaacaagaattctttttatcaaaatattcatttttcaaaaaggcctcacattaacccctcaaaccaagcacccccttcctatgtccagcactcttttctacttcgagttgcatgactgtagagacaactgtcaaattccagtggaactgtacactgacttaagactctatgtaatatacatcaaacacaggaggtcactgactttaagggacgaggtgataactaactagttataattcagccaatgtcttttttagtttagagggaaaaaagtagcccccaagtgtccttaacttttcagtacttctctgtaacacacagaatgaaaaggtactctctaaaattaaaatcattagaaaatatcttaaataaagtgttttacataaataagtgttaaatttcagattcaaactatattttcttctgtatctcaatttgggaaaaatctcacaattattaactcttctcagttacatttatttttgagcatttaaatctactatacaccagtttgtaaaattcaccttggttacctctccccatgcctatgtgctgtctttcctcaggtaagtccattatatgcatctaagtgctggggaggtttaaatagcacttaaagaatattcatgagagttctgaaatgaaggtttcgtctttagctattgactgtaggatttgtaattcaaatcatcacagcatcctaaagaaatactgtgtgaatggaatgcacacaattcctacagaacacacaaactgatgtccaaaaggcacagagtaatgctggtggctctttctagtcagttaagaaacaataaaaagtctgcattattctttcataatttaaatacttaagtaatctccactttattattttataacaatgacttcaaatttacattattttaagtaccattgtaatagcttagtgtataatacagatatttgcgaatatcccatccaaaaattaaaaaaaacttcttcactatatatatatttatataaaaattattctgaaagacaagaacatagacaagggacttggtacagaccatcaactcaattttctatcaccacagttgtaactccaaaatcaacaaatatacagcagtaattaaaagcagtgcaaatatctttggaggttaggataaaattataatgcaagaacataaaactgaggaaacaaaaaaggcaagtacttcaagtacaaggaaccagtcggcttgaggtccatcttagtgtttactgggggcttctttcctgcttctacttctttctctgaaatacattggccaacatggcacctgatgttgtcaactggcccattttgttcaaaaacttggtctttgtatcttcactcactaagcttgcagcaattgacattgagccttgaggctcttggacggtcttgttttcaactttttgttcacattcttttatcatggaacttaaaataacctcatgctctggagagagatgttccatgtcagtccgtaaacatctgagaccaggtaaaaagtgattaaccattaaatcctctgaaatgaaacaacaggaaagtgcactgtaggcttcaaaaagatgcgtagcaatgtccagtcttttagaatccacaatctgtaagttgttcaccaaggctaacttatgcaaatgtggtataacaaactcatctcggaacctgggttctgcgttagggccaactctaccaaatgtttttatgatctctgtatgcaaagaatgttggtcttgatactgaggatcttccaggaaagaagccaactgcattttcactctttccagcaactctctttgaattactgtttccataatagtgccaaaggctggaattgtggcaatcctgacagagatttcagggtcactggagagagtaatgagagcaggaacaaccctctgagctaccagagtttcattcacccccttcaccaacagctcaaacattctagcagcagtacacctcacgagtgctgaagtatggacaacaccataccacaaaacagttaatagtaactcatggtaggctgggtttgcacccaattccacaaaagaagccttcaggctatcaagaggagcatgagataatgaaagcagcgtcattacatcttctaagaatccaactaacagttttcggtcttcttcctgaatataacacgtaaggactcctgttgcataaatggggactgtagctttagtgaggaccccatttcctgctgaggaatcaatgttttcttcagatagtcttaaaatctcctggaactgaggttttaccttagtgtttgtaaaaattttgccaaatgtccggcaaaggcgccagaaaaatctggagaattcatggacacaggcagttgaagtaacattaattttgccaactatttctataagttgtggcaacaattgattgacaacccacagtaaactctcccagcctgttgtaccctcttgttctagctggtagtcataaagttgcagcagcactgccaattgctcacgacttccgataatagtggacacatcttgaagaggcgacataggccgaggaaacctagtcacttctatctgtggcacttcaccatgaagcttggctttgctggagaaaggtgcattctgtagcactaatgcaaagagagatgggatcaaggactgcaaggcagaaagatacatgtggagtttgtgttcatccagtccatgttctccttccctgagaagtttttcaatcttgttcagtagtgtaagtataagatgagactgtaaatttccaagttctgtagtccacgcagcgtaagctggtaaaaatacttgatgtgtagcactaactactctttctgagggatcacccaaggctgacagcaacaattcaaaaccctgatgatatttgtctggatcatcaatgtatcccataatgataccaaggcttttgataacagcttctcttaccaaatctgccttatcttccattaacatttgttgcaacattgaaagaaccaaggagctacggatttctttaggaaggtaaggtgccagtgctccacaggattctgccacaagcagtcgtctttctgggtatttgtgattaatctgttcccaacactgtggtaaaagttcagcttctacacgtgttggtccaacatgacgcgcaaatgccacacaacctgtcagtatcatttgcctttgctcatcatctggcctcttgatcaaattgaaaagtatgtggagaagctgatctcgctctttaggctcaggatgtagacatgctgtacacaatatgagggggatcaactcctctctctttgccaatagcacattgggaacaatgtgtggcaggcagcgtcccagcattaacataacgcttttttcactgtctgcaatacgagacacctcgtatcctaaacgactatctgctgacattcgacaaaaagagagtagtgcttgatggaatgcaggagacaatttcctattaggtttatcaaaatgaactgtctttttacttgatagagaagaaggtggcattccttctctttctctcctggggaatgaatttggggaattctctttaggaatagtggaatcagcttcatctgatattgaaagatggatgtctgtgttttttcccttgtctgaactatttacatctggatgctgtccactgtcctcagagtctttgtggggcaactgatccaaaggaggctgaacagagtcacaaactgctgggatggcaaagtgttcatttttgaggaagtccatttcacttttaagtcttctgatttgctccatcaatgaccatttctcactatttaacaaactaattttatcttctaatttctgtactaacatggagttctctgcaggctggggagtttcaagagttggaggaaggttgcttataattggtgtaagggcctctaattcatcttcttctactccactggccacatctacaagatcttttccagttacttgatgatttccaaaatcccggtagagttgcaataagtctggaggttttggaatgtttaatcctacatcatcccataattcaaaatcctgatcatcgttttcatctgaaaaggttattgatgtaagcttatagttattcttcaataaaaattcattgactaagaagtttagagctctcttttcaagaggtttgattggctcctgaatttcaggacttgatttgtaattttttcgttcctgtaaaggaacttcatgttctgcggcctttgtcaggttggctcggagggcctgaatggtctccttggctttccgtagttcaaactccaggactgccactttttcatctgtttccctgttaccatcatctgaatatcttgcaaagtctaaagaatcaagggtactaatgctcccagctcgattgagctgtcccccgcccgacgctgtactcggttcccgacctccagcgcccccaacgccggctgctccagggacccctggcgcccccatccccggcggggttccactttgcctctcgaagttgcctggattggagaagtagtcgcgcagccgaggcagctcccggccactctctaacagctcggtatgcagctccagggcggtcagcaagtattgatcgcgcaacagctgagcagcgatcgcatcaattgataatcgggccggggtctccccggtgccccccagggccactgcagccgccgacgcctccccagggagccctggccgcgcactgcttcctaaggccacgggatcctgtggcgacagcgagcccgcagagccaggatctaggccacttccggcgcccagccgaagtactgcccgccgttcctctgttgcagctacctcgtcatcgtcctcatccgaatcactgagaaatggattcacgccgccaccactgccactacctccaggcgccatcgccgccatcttatcctgtcaggagtgtgggcgcctccctgactggttccgacgggccgcagcccgaatcctctaggcctcaggggacacagcgcacctccacagccccggcctgaccacgtcctgcctcccgacttagagacaaggagtacgctccaaggcaggagatccggatgcagctgcacctgatgcctcagcctctgctgcaccagcagcccggctctgcaggcgtcttcctggtctccagtctcgcgagaact

SEQ ID NO: 14604 - RNA, 7384 nt, Homo sapiens
  source 1..7384: mol_type = other RNA
gctgggattacaggcatgagccaccgtgcccggccagtctctatttctttttaatgtactgaaaaaaatagtatcaaaactaagcacactgtaaagttacagtagaactttgaaatagatgtctactcatacaaaaggctaaatttattttgtagttttcttgtaagagaattaacatccaaccttgaaggttgaattttgttacctggctaatctggagtatttcatgaattatgaattagaattgctacttacaaagcttttttttttgtttttgagatggagtcttgctctgtggaccaggctggagtgcagtggtgcaatagcggcccactgcaatctccgcttcccaggttcaaacgattctcctgtctcagcctcccgagtagcagggattacaggcccacgtcaccacgcctggctaatttttgtatttttagaggcggggtttcaccacgttggccaggctggtcttgaactactgacctcaagtgattcgtcaccttggcctcccaaagtgctgagattacaggcgtgagccacagcgcacagtccaaagctctttaagtgtaacattgaagagctaaagtgtaactttctttaatgaactgaaaaaattagtacaatctttacacaaagaatagttaagaaaatataaccagcacagaatgttagctgtagttagctactgcagttcaaagatcagcagggtagtaactacagaaagttacatccttggagttcaaataatggtccaaaataggttgtcttgaaaaatgggatgatgaaaagacaattcaatacatcctgatctcacctctctaaattttaagagagactatttgagccaactttttaaaaacaagaatgtgatagcaccttgacttgagacccccattagaattatagtgtatagtagtgacatatcctatagtagtgacatatcctaaaagctatggataatgaggatggcatgacttaaattactcacaatttcgttcaggttgaaaatcaatttgatgtttagcaaaataatctctctaaaggggtgaataatgcaaaccaatgaaggtcatagacacctatgtatagagatagatactgccatcattcaagcactgttcttggaagaattcagctaaattagtaattatggcacttctggatttctgaaaaaatttaatctctggattactctggaaacacaggtataatttcaaattagcttttcattactttgcaaacttagtttttcattaagttgaacacttaaaaacttgtaccgtaagtttacttctgtttaaaaggaatgagtatgggagttttatgccctattttggactcagtccaaatctcagtctcaatgattagtgtctgtcttgtctgtaaagacaagacatattttactaaaaacaaacaaacaaacaaaaaacaaaaccacaatgtgaaatcttaatgatattaaaatatttaagaaaagagactctcacttgaaatacactgtgaatcttgcctactattgcctttaaaaaaacattagcacttaaataaatatattcattaattaagaaaaatgttcacaataaaaatacattctacccattcacctgataacaaacatacacatattctactatagtttgaagcaaatcagagtttaaacatttttcttccaggtacctctgaaatgtattagttttatagcaacatggtccccttttagtaaaaataaaccaaaataggtaaatttatataaattatatttacaaaatattagtatattctcatgaatataggcttttctcatttttttgcttaatagaaagtatagtgtttcaaaacgaaagtaaaatgcatagcccaaaccaaatcaaaaacatatgcaaaaacattttatttataatagatcaacatttttgacatgaaaggtagccactttcaatttctcaggaatgcctagaacccaacagttttcagaaagactacttagttcacaattatttcactgtaggtaaatgaaataatttcagaatgaactttttaaatggctttgcctatggcaaattgttttataaacttgaatgtatggtaagctagctttcccaggaaatgaatgtaatccaactatgttccaaatgtattaaaccagtttatacaacaaatatgagaatcacttatgtgcatcaactgtgctaaaacaagaattctttttatcaaaatattcatttttcaaaaaggcctcacattaacccctcaaaccaagcacccccttcctatgtccagcactcttttctacttcgagttgcatgactgtagagacaactgtcaaattccagtggaactgtacactgacttaagactctatgtaatatacatcaaacacaggaggtcactgactttaagggacgaggtgataactaactagttataattcagccaatgtcttttttagtttagagggaaaaaagtagcccccaagtgtccttaacttttcagtacttctctgtaacacacagaatgaaaaggtactctctaaaattaaaatcattagaaaatatcttaaataaagtgttttacataaataagtgttaaatttcagattcaaactatattttcttctgtatctcaatttgggaaaaatctcacaattattaactcttctcagttacatttatttttgagcatttaaatctactatacaccagtttgtaaaattcaccttggttacctctccccatgcctatgtgctgtctttcctcaggtaagtccattatatgcatctaagtgctggggaggtttaaatagcacttaaagaatattcatgagagttctgaaatgaaggtttcgtctttagctattgactgtaggatttgtaattcaaatcatcacagcatcctaaagaaatactgtgtgaatggaatgcacacaattcctacagaacacacaaactgatgtccaaaaggcacagagtaatgctggtggctctttctagtcagttaagaaacaataaaaagtctgcattattctttcataatttaaatacttaagtaatctccactttattattttataacaatgacttcaaatttacattattttaagtaccattgtaatagcttagtgtataatacagatatttgcgaatatcccatccaaaaattaaaaaaaacttcttcactatatatatatttatataaaaattattctgaaagacaagaacatagacaagggacttggtacagaccatcaactcaattttctatcaccacagttgtaactccaaaatcaacaaatatacagcagtaattaaaagcagtgcaaatatctttggaggttaggataaaattataatgcaagaacataaaactgaggaaacaaaaaaggcaagtacttcaagtacaaggaaccagtcggcttgaggtccatcttagtgtttactgggggcttctttcctgcttctacttctttctctgaaatacattggccaacatggcacctgatgttgtcaactggcccattttgttcaaaaacttggtctttgtatcttcactcactaagcttgcagcaattgacattgagccttgaggctcttggacggtcttgttttcaactttttgttcacattcttttatcatggaacttaaaataacctcatgctctggagagagatgttccatgtcagtccgtaaacatctgagaccaggtaaaaagtgattaaccattaaatcctctgaaatgaaacaacaggaaagtgcactgtaggcttcaaaaagatgcgtagcaatgtccagtcttttagaatccacaatctgtaagttgttcaccaaggctaacttatgcaaatgtggtataacaaactcatctcggaacctgggttctgcgttagggccaactctaccaaatgtttttatgatctctgtatgcaaagaatgttggtcttgatactgaggatcttccaggaaagaagccaactgcattttcactctttccagcaactctctttgaattactgtttccataatagtgccaaaggctggaattgtggcaatcctgacagagatttcagggtcactggagagagtaatgagagcaggaacaaccctctgagctaccagagtttcattcacccccttcaccaacagctcaaacattctagcagcagtacacctcacgagtgctgaagtatggacaacaccataccacaaaacagttaatagtaactcatggtaggctgggtttgcacccaattccacaaaagaagccttcaggctatcaagaggagcatgagataatgaaagcagcgtcattacatcttctaagaatccaactaacagttttcggtcttcttcctgaatataacacgtaaggactcctgttgcataaatggggactgtagctttagtgaggaccccatttcctgctgaggaatcaatgttttcttcagatagtcttaaaatctcctggaactgaggttttaccttagtgtttgtaaaaattttgccaaatgtccggcaaaggcgccagaaaaatctggagaattcatggacacaggcagttgaagtaacattaattttgccaactatttctataagttgtggcaacaattgattgacaacccacagtaaactctcccagcctgttgtaccctcttgttctagctggtagtcataaagttgcagcagcactgccaattgctcacgacttccgataatagtggacacatcttgaagaggcgacataggccgaggaaacctagtcacttctatctgtggcacttcaccatgaagcttggctttgctggagaaaggtgcattctgtagcactaatgcaaagagagatgggatcaaggactgcaaggcagaaagatacatgtggagtttgtgttcatccagtccatgttctccttccctgagaagtttttcaatcttgttcagtagtgtaagtataagatgagactgtaaatttccaagttctgtagtccacgcagcgtaagctggtaaaaatacttgatgtgtagcactaactactctttctgagggatcacccaaggctgacagcaacaattcaaaaccctgatgatatttgtctggatcatcaatgtatcccataatgataccaaggcttttgataacagcttctcttaccaaatctgccttatcttccattaacatttgttgcaacattgaaagaaccaaggagctacggatttctttaggaaggtaaggtgccagtgctccacaggattctgccacaagcagtcgtctttctgggtatttgtgattaatctgttcccaacactgtggtaaaagttcagcttctacacgtgttggtccaacatgacgcgcaaatgccacacaacctgtcagtatcatttgcctttgctcatcatctggcctcttgatcaaattgaaaagtatgtggagaagctgatctcgctctttaggctcaggatgtagacatgctgtacacaatatgagggggatcaactcctgacagaggtgtaaaaccattctctctctctttgccaatagcacattgggaacaatgtgtggcaggcagcgtcccagcattaacataacgcttttttcactgtctgcaatacgagacacctcgtatcctaaacgactatctgctgacattcgacaaaaagagagtagtgcttgatggaatgcaggagacaatttcctattaggtttatcaaaatgaactgtctttttacttgatagagaagaaggtggcattccttctctttctctcctggggaatgaatttggggaattctctttaggaatagtggaatcagcttcatctgatattgaaagatggatgtctgtgttttttcccttgtctgaactatttacatctggatgctgtccactgtcctcagagtctttgtggggcaactgatccaaaggaggctgaacagagtcacaaactgctgggatggcaaagtgttcatttttgaggaagtccatttcacttttaagtcttctgatttgctccatcaatgaccatttctcactatttaacaaactaattttatcttctaatttctgtactaacatggagttctctgcaggctggggagtttcaagagttggaggaaggttgcttataattggtgtaagggcctctaattcatcttcttctactccactggccacatctacaagatcttttccagttacttgatgatttccaaaatcccggtagagttgcaataagtctggaggttttggaatgtttaatcctacatcatcccataattcaaaatcctgatcatcgttttcatctgaaaaggttattgatgtaagcttatagttattcttcaataaaaattcattgactaagaagtttagagctctcttttcaagaggtttgattggctcctgaatttcaggacttgatttgtaattttttcgttcctgtaaaggaacttcatgttctgcggcctttgtcaggttggctcggagggcctgaatggtctccttggctttccgtagttcaaactccaggactgccactttttcatctgtttccctgttaccatcatctgaatatcttgcaaagtctaaagaatcaagggtactaatgctcccagctcgattgagctgtcccccgcccgacgctgtactcggttcccgacctccagcgcccccaacgccggctgctccagggacccctggcgcccccatccccggcggggttccactttgcctctcgaagttgcctggattggagaagtagtcgcgcagccgaggcagctcccggccactctctaacagctcggtatgcagctccagggcggtcagcaagtattgatcgcgcaacagctgagcagcgatcgcatcaattgataatcgggccggggtctccccggtgccccccagggccactgcagccgccgacgcctccccagggagccctggccgcgcactgcttcctaaggccacgggatcctgtggcgacagcgagcccgcagagccaggatctaggccacttccggcgcccagccgaagtactgcccgccgttcctctgttgcagctacctcgtcatcgtcctcatccgaatcactgagaaatggattcacgccgccaccactgccactacctccaggcgccatcgccgccatcttatcctgtcaggagtgtgggcgcctccctgactggttccgacgggccgcagcccgaatcctctaggcctcaggggacacagcgcacctccacagccccggcctgaccacgtcctgcctcccgacttagagacaaggagtacgctccaaggcaggagatccggatgcagctgcacctgatgcctcagcctctgctgcaccagcagcccggctctgcaggcgtcttcctggtctccagtctcgcgagaact

SEQ ID NO: 14605 - RNA, 7996 nt, Homo sapiens
  source 1..7996: mol_type = other RNA
gctgggattacaggcatgagccaccgtgcccggccagtctctatttctttttaatgtactgaaaaaaatagtatcaaaactaagcacactgtaaagttacagtagaactttgaaatagatgtctactcatacaaaaggctaaatttattttgtagttttcttgtaagagaattaacatccaaccttgaaggttgaattttgttacctggctaatctggagtatttcatgaattatgaattagaattgctacttacaaagcttttttttttgtttttgagatggagtcttgctctgtggaccaggctggagtgcagtggtgcaatagcggcccactgcaatctccgcttcccaggttcaaacgattctcctgtctcagcctcccgagtagcagggattacaggcccacgtcaccacgcctggctaatttttgtatttttagaggcggggtttcaccacgttggccaggctggtcttgaactactgacctcaagtgattcgtcaccttggcctcccaaagtgctgagattacaggcgtgagccacagcgcacagtccaaagctctttaagtgtaacattgaagagctaaagtgtaactttctttaatgaactgaaaaaattagtacaatctttacacaaagaatagttaagaaaatataaccagcacagaatgttagctgtagttagctactgcagttcaaagatcagcagggtagtaactacagaaagttacatccttggagttcaaataatggtccaaaataggttgtcttgaaaaatgggatgatgaaaagacaattcaatacatcctgatctcacctctctaaattttaagagagactatttgagccaactttttaaaaacaagaatgtgatagcaccttgacttgagacccccattagaattatagtgtatagtagtgacatatcctatagtagtgacatatcctaaaagctatggataatgaggatggcatgacttaaattactcacaatttcgttcaggttgaaaatcaatttgatgtttagcaaaataatctctctaaaggggtgaataatgcaaaccaatgaaggtcatagacacctatgtatagagatagatactgccatcattcaagcactgttcttggaagaattcagctaaattagtaattatggcacttctggatttctgaaaaaatttaatctctggattactctggaaacacaggtataatttcaaattagcttttcattactttgcaaacttagtttttcattaagttgaacacttaaaaacttgtaccgtaagtttacttctgtttaaaaggaatgagtatgggagttttatgccctattttggactcagtccaaatctcagtctcaatgattagtgtctgtcttgtctgtaaagacaagacatattttactaaaaacaaacaaacaaacaaaaaacaaaaccacaatgtgaaatcttaatgatattaaaatatttaagaaaagagactctcacttgaaatacactgtgaatcttgcctactattgcctttaaaaaaacattagcacttaaataaatatattcattaattaagaaaaatgttcacaataaaaatacattctacccattcacctgataacaaacatacacatattctactatagtttgaagcaaatcagagtttaaacatttttcttccaggtacctctgaaatgtattagttttatagcaacatggtccccttttagtaaaaataaaccaaaataggtaaatttatataaattatatttacaaaatattagtatattctcatgaatataggcttttctcatttttttgcttaatagaaagtatagtgtttcaaaacgaaagtaaaatgcatagcccaaaccaaatcaaaaacatatgcaaaaacattttatttataatagatcaacatttttgacatgaaaggtagccactttcaatttctcaggaatgcctagaacccaacagttttcagaaagactacttagttcacaattatttcactgtaggtaaatgaaataatttcagaatgaactttttaaatggctttgcctatggcaaattgttttataaacttgaatgtatggtaagctagctttcccaggaaatgaatgtaatccaactatgttccaaatgtattaaaccagtttatacaacaaatatgagaatcacttatgtgcatcaactgtgctaaaacaagaattctttttatcaaaatattcatttttcaaaaaggcctcacattaacccctcaaaccaagcacccccttcctatgtccagcactcttttctacttcgagttgcatgactgtagagacaactgtcaaattccagtggaactgtacactgacttaagactctatgtaatatacatcaaacacaggaggtcactgactttaagggacgaggtgataactaactagttataattcagccaatgtcttttttagtttagagggaaaaaagtagcccccaagtgtccttaacttttcagtacttctctgtaacacacagaatgaaaaggtactctctaaaattaaaatcattagaaaatatcttaaataaagtgttttacataaataagtgttaaatttcagattcaaactatattttcttctgtatctcaatttgggaaaaatctcacaattattaactcttctcagttacatttatttttgagcatttaaatctactatacaccagtttgtaaaattcaccttggttacctctccccatgcctatgtgctgtctttcctcaggtaagtccattatatgcatctaagtgctggggaggtttaaatagcacttaaagaatattcatgagagttctgaaatgaaggtttcgtctttagctattgactgtaggatttgtaattcaaatcatcacagcatcctaaagaaatactgtgtgaatggaatgcacacaattcctacagaacacacaaactgatgtccaaaaggcacagagtaatgctggtggctctttctagtcagttaagaaacaataaaaagtctgcattattctttcataatttaaatacttaagtaatctccactttattattttataacaatgacttcaaatttacattattttaagtaccattgtaatagcttagtgtataatacagatatttgcgaatatcccatccaaaaattaaaaaaaacttcttcactatatatatatttatataaaaattattctgaaagacaagaacatagacaagggacttggtacagaccatcaactcaattttctatcaccacagttgtaactccaaaatcaacaaatatacagcagtaattaaaagcagtgcaaatatctttggaggttaggataaaattataatgcaagaacataaaactgaggaaacaaaaaaggcaagtacttcaagtacaaggaaccagtcggcttgaggtccatcttagtgtttactgggggcttctttcctgcttctacttctttctctgaaatacattggccaacatggcacctgatgttgtcaactggcccattttgttcaaaaacttggtctttgtatcttcactcactaagcttgcagcaattgacattgagccttgaggctcttggacggtcttgttttcaactttttgttcacattcttttatcatggaacttaaaataacctcatgctctggagagagatgttccatgtcagtccgtaaacatctgagaccaggtaaaaagtgattaaccattaaatcctctgaaatgaaacaacaggaaagtgcactgtaggcttcaaaaagatgcgtagcaatgtccagtcttttagaatccacaatctgtaagttgttcaccaaggctaacttatgcaaatgtggtataacaaactcatctcggaacctgggttctgcgttagggccaactctaccaaatgtttttatgatctctgtatgcaaagaatgttggtcttgatactgaggatcttccaggaaagaagccaactgcattttcactctttccagcaactctctttgaattactgtttccataatagtgccaaaggctggaattgtggcaatcctgacagagatttcagggtcactggagagagtaatgagagcaggaacaaccctctgagctaccagagtttcattcacccccttcaccaacagctcaaacattctagcagcagtacacctcacgagtgctgaagtatggacaacaccataccacaaaacagttaatagtaactcatggtaggctgggtttgcacccaattccacaaaagaagccttcaggctatcaagaggagcatgagataatgaaagcagcgtcattacatcttctaagaatccaactaacagttttcggtcttcttcctgaatataacacgtaaggactcctgttgcataaatggggactgtagctttagtgaggaccccatttcctgctgaggaatcaatgttttcttcagatagtcttaaaatctcctggaactgaggttttaccttagtgtttgtaaaaattttgccaaatgtccggcaaaggcgccagaaaaatctggagaattcatggacacaggcagttgaagtaacattaattttgccaactatttctataagttgtggcaacaattgattgacaacccacagtaaactctcccagcctgttgtaccctcttgttctagctggtagtcataaagttgcagcagcactgccaattgctcacgacttccgataatagtggacacatcttgaagaggcgacataggccgaggaaacctagtcacttctatctgtggcacttcaccatgaagcttggctttgctggagaaaggtgcattctgtagcactaatgcaaagagagatgggatcaaggactgcaaggcagaaagatacatgtggagtttgtgttcatccagtccatgttctccttccctgagaagtttttcaatcttgttcagtagtgtaagtataagatgagactgtaaatttccaagttctgtagtccacgcagcgtaagctggtaaaaatacttgatgtgtagcactaactactctttctgagggatcacccaaggctgacagcaacaattcaaaaccctgatgatatttgtctggatcatcaatgtatcccataatgataccaaggcttttgataacagcttctcttaccaaatctgccttatcttccattaacatttgttgcaacattgaaagaaccaaggagctacggatttctttaggaaggtaaggtgccagtgctccacaggattctgccacaagcagtcgtctttctgggtatttgtgattaatctgttcccaacactgtggtaaaagttcagcttctacacgtgttggtccaacatgacgcgcaaatgccacacaacctgtcagtatcatttgcctttgctcatcatctggcctcttgatcaaattgaaaagtatgtggagaagctgatctcgctctttaggctcaggatgtagacatgctgtacacaatatgagggggatcaactcctgttttgcagaagtgaaaggctgagcatcaaattcatgcggaactgcaagggaccctgaacagacaatagtgatgtgcagttagaggactcatatatcccaatttcaaaacttactacaaacaacagttatcaaaacagtgtggtagtggcatatggctagacatacagaccaatggaacagaactgaaagtccagaaataaacccgaagaatctaggcccaactgatttttgacaaaagtagcaagactattcaaaagaggaatttttttatcttgaacaaatgtttctggataactggatagccatatgaaaagaataaagttagacgctgttttactccatatataaaaattaactcaaaatgaatcgttgacctaaatatatataacaaatgttttcttctaattgtttcatagctttagctcttatatatattcatatacatatagatatatatatcttctataacattgattgacttggcaatggtttcttaaaattgatacttagagcacaaacaacacaacaaaaaaatagataaatcagatttcataaaaatggaaaacatttgcccatcaaaggatatggtcaagagtgtaaaaagaaaacctgacagaggtgtaaaaccattctctctctctttgccaatagcacattgggaacaatgtgtggcaggcagcgtcccagcattaacataacgcttttttcactgtctgcaatacgagacacctcgtatcctaaacgactatctgctgacattcgacaaaaagagagtagtgcttgatggaatgcaggagacaatttcctattaggtttatcaaaatgaactgtctttttacttgatagagaagaaggtggcattccttctctttctctcctggggaatgaatttggggaattctctttaggaatagtggaatcagcttcatctgatattgaaagatggatgtctgtgttttttcccttgtctgaactatttacatctggatgctgtccactgtcctcagagtctttgtggggcaactgatccaaaggaggctgaacagagtcacaaactgctgggatggcaaagtgttcatttttgaggaagtccatttcacttttaagtcttctgatttgctccatcaatgaccatttctcactatttaacaaactaattttatcttctaatttctgtactaacatggagttctctgcaggctggggagtttcaagagttggaggaaggttgcttataattggtgtaagggcctctaattcatcttcttctactccactggccacatctacaagatcttttccagttacttgatgatttccaaaatcccggtagagttgcaataagtctggaggttttggaatgtttaatcctacatcatcccataattcaaaatcctgatcatcgttttcatctgaaaaggttattgatgtaagcttatagttattcttcaataaaaattcattgactaagaagtttagagctctcttttcaagaggtttgattggctcctgaatttcaggacttgatttgtaattttttcgttcctgtaaaggaacttcatgttctgcggcctttgtcaggttggctcggagggcctgaatggtctccttggctttccgtagttcaaactccaggactgccactttttcatctgtttccctgttaccatcatctgaatatcttgcaaagtctaaagaatcaagggtactaatgctcccagctcgattgagctgtcccccgcccgacgctgtactcggttcccgacctccagcgcccccaacgccggctgctccagggacccctggcgcccccatccccggcggggttccactttgcctctcgaagttgcctggattggagaagtagtcgcgcagccgaggcagctcccggccactctctaacagctcggtatgcagctccagggcggtcagcaagtattgatcgcgcaacagctgagcagcgatcgcatcaattgataatcgggccggggtctccccggtgccccccagggccactgcagccgccgacgcctccccagggagccctggccgcgcactgcttcctaaggccacgggatcctgtggcgacagcgagcccgcagagccaggatctaggccacttccggcgcccagccgaagtactgcccgccgttcctctgttgcagctacctcgtcatcgtcctcatccgaatcactgagaaatggattcacgccgccaccactgccactacctccaggcgccatcgccgccatcttatcctgtcaggagtgtgggcgcctccctgactggttccgacgggccgcagcccgaatcctctaggcctcaggggacacagcgcacctccacagccccggcctgaccacgtcctgcctcccgacttagagacaaggagtacgctccaaggcaggagatccggatgcagctgcacctgatgcctcagcctctgctgcaccagcagcccggctctgcaggcgtcttcctggtctccagtctcgcgagaact

SEQ ID NO: 14606 - RNA, 7482 nt, Homo sapiens
  source 1..7482: mol_type = other RNA
gctgggattacaggcatgagccaccgtgcccggccagtctctatttctttttaatgtactgaaaaaaatagtatcaaaactaagcacactgtaaagttacagtagaactttgaaatagatgtctactcatacaaaaggctaaatttattttgtagttttcttgtaagagaattaacatccaaccttgaaggttgaattttgttacctggctaatctggagtatttcatgaattatgaattagaattgctacttacaaagcttttttttttgtttttgagatggagtcttgctctgtggaccaggctggagtgcagtggtgcaatagcggcccactgcaatctccgcttcccaggttcaaacgattctcctgtctcagcctcccgagtagcagggattacaggcccacgtcaccacgcctggctaatttttgtatttttagaggcggggtttcaccacgttggccaggctggtcttgaactactgacctcaagtgattcgtcaccttggcctcccaaagtgctgagattacaggcgtgagccacagcgcacagtccaaagctctttaagtgtaacattgaagagctaaagtgtaactttctttaatgaactgaaaaaattagtacaatctttacacaaagaatagttaagaaaatataaccagcacagaatgttagctgtagttagctactgcagttcaaagatcagcagggtagtaactacagaaagttacatccttggagttcaaataatggtccaaaataggttgtcttgaaaaatgggatgatgaaaagacaattcaatacatcctgatctcacctctctaaattttaagagagactatttgagccaactttttaaaaacaagaatgtgatagcaccttgacttgagacccccattagaattatagtgtatagtagtgacatatcctatagtagtgacatatcctaaaagctatggataatgaggatggcatgacttaaattactcacaatttcgttcaggttgaaaatcaatttgatgtttagcaaaataatctctctaaaggggtgaataatgcaaaccaatgaaggtcatagacacctatgtatagagatagatactgccatcattcaagcactgttcttggaagaattcagctaaattagtaattatggcacttctggatttctgaaaaaatttaatctctggattactctggaaacacaggtataatttcaaattagcttttcattactttgcaaacttagtttttcattaagttgaacacttaaaaacttgtaccgtaagtttacttctgtttaaaaggaatgagtatgggagttttatgccctattttggactcagtccaaatctcagtctcaatgattagtgtctgtcttgtctgtaaagacaagacatattttactaaaaacaaacaaacaaacaaaaaacaaaaccacaatgtgaaatcttaatgatattaaaatatttaagaaaagagactctcacttgaaatacactgtgaatcttgcctactattgcctttaaaaaaacattagcacttaaataaatatattcattaattaagaaaaatgttcacaataaaaatacattctacccattcacctgataacaaacatacacatattctactatagtttgaagcaaatcagagtttaaacatttttcttccaggtacctctgaaatgtattagttttatagcaacatggtccccttttagtaaaaataaaccaaaataggtaaatttatataaattatatttacaaaatattagtatattctcatgaatataggcttttctcatttttttgcttaatagaaagtatagtgtttcaaaacgaaagtaaaatgcatagcccaaaccaaatcaaaaacatatgcaaaaacattttatttataatagatcaacatttttgacatgaaaggtagccactttcaatttctcaggaatgcctagaacccaacagttttcagaaagactacttagttcacaattatttcactgtaggtaaatgaaataatttcagaatgaactttttaaatggctttgcctatggcaaattgttttataaacttgaatgtatggtaagctagctttcccaggaaatgaatgtaatccaactatgttccaaatgtattaaaccagtttatacaacaaatatgagaatcacttatgtgcatcaactgtgctaaaacaagaattctttttatcaaaatattcatttttcaaaaaggcctcacattaacccctcaaaccaagcacccccttcctatgtccagcactcttttctacttcgagttgcatgactgtagagacaactgtcaaattccagtggaactgtacactgacttaagactctatgtaatatacatcaaacacaggaggtcactgactttaagggacgaggtgataactaactagttataattcagccaatgtcttttttagtttagagggaaaaaagtagcccccaagtgtccttaacttttcagtacttctctgtaacacacagaatgaaaaggtactctctaaaattaaaatcattagaaaatatcttaaataaagtgttttacataaataagtgttaaatttcagattcaaactatattttcttctgtatctcaatttgggaaaaatctcacaattattaactcttctcagttacatttatttttgagcatttaaatctactatacaccagtttgtaaaattcaccttggttacctctccccatgcctatgtgctgtctttcctcaggtaagtccattatatgcatctaagtgctggggaggtttaaatagcacttaaagaatattcatgagagttctgaaatgaaggtttcgtctttagctattgactgtaggatttgtaattcaaatcatcacagcatcctaaagaaatactgtgtgaatggaatgcacacaattcctacagaacacacaaactgatgtccaaaaggcacagagtaatgctggtggctctttctagtcagttaagaaacaataaaaagtctgcattattctttcataatttaaatacttaagtaatctccactttattattttataacaatgacttcaaatttacattattttaagtaccattgtaatagcttagtgtataatacagatatttgcgaatatcccatccaaaaattaaaaaaaacttcttcactatatatatatttatataaaaattattctgaaagacaagaacatagacaagggacttggtacagaccatcaactcaattttctatcaccacagttgtaactccaaaatcaacaaatatacagcagtaattaaaagcagtgcaaatatctttggaggttaggataaaattataatgcaagaacataaaactgaggaaacaaaaaaggcaagtacttcaagtacaaggaaccagtcggcttgaggtccatcttagtgtttactgggggcttctttcctgcttctacttctttctctgaaatacattggccaacatggcacctgatgttgtcaactggcccattttgttcaaaaacttggtctttgtatcttcactcactaagcttgcagcaattgacattgagccttgaggctcttggacggtcttgttttcaactttttgttcacattcttttatcatggaacttaaaataacctcatgctctggagagagatgttccatgtcagtccgtaaacatctgagaccaggtaaaaagtgattaaccattaaatcctctgaaatgaaacaacaggaaagtgcactgtaggcttcaaaaagatgcgtagcaatgtccagtcttttagaatccacaatctgtaagttgttcaccaaggctaacttatgcaaatgtggtataacaaactcatctcggaacctgggttctgcgttagggccaactctaccaaatgtttttatgatctctgtatgcaaagaatgttggtcttgatactgaggatcttccaggaaagaagccaactgcattttcactctttccagcaactctctttgaattactgtttccataatagtgccaaaggctggaattgtggcaatcctgacagagatttcagggtcactggagagagtaatgagagcaggaacaaccctctgagctaccagagtttcattcacccccttcaccaacagctcaaacattctagcagcagtacacctcacgagtgctgaagtatggacaacaccataccacaaaacagttaatagtaactcatggtaggctgggtttgcacccaattccacaaaagaagccttcaggctatcaagaggagcatgagataatgaaagcagcgtcattacatcttctaagaatccaactaacagttttcggtcttcttcctgaatataacacgtaaggactcctgttgcataaatggggactgtagctttagtgaggaccccatttcctgctgaggaatcaatgttttcttcagatagtcttaaaatctcctggaactgaggttttaccttagtgtttgtaaaaattttgccaaatgtccggcaaaggcgccagaaaaatctggagaattcatggacacaggcagttgaagtaacattaattttgccaactatttctataagttgtggcaacaattgattgacaacccacagtaaactctcccagcctgttgtaccctcttgttctagctggtagtcataaagttgcagcagcactgccaattgctcacgacttccgataatagtggacacatcttgaagaggcgacataggccgaggaaacctagtcacttctatctgtggcacttcaccatgaagcttggctttgctggagaaaggtgcattctgtagcactaatgcaaagagagatgggatcaaggactgcaaggcagaaagatacatgtggagtttgtgttcatccagtccatgttctccttccctgagaagtttttcaatcttgttcagtagtgtaagtataagatgagactgtaaatttccaagttctgtagtccacgcagcgtaagctggtaaaaatacttgatgtgtagcactaactactctttctgagggatcacccaaggctgacagcaacaattcaaaaccctgatgatatttgtctggatcatcaatgtatcccataatgataccaaggcttttgataacagcttctcttaccaaatctgccttatcttccattaacatttgttgcaacattgaaagaaccaaggagctacggatttctttaggaaggtaaggtgccagtgctccacaggattctgccacaagcagtcgtctttctgggtatttgtgattaattgggttttgttcccatatgtcttcttcatagaatataaatctttctttgactggaaaaggagtatatttgttctcatattcccatatgaaaaggtgacataattcattaatgtattggatgcctgttcccaacactgtggtaaaagttcagcttctacacgtgttggtccaacatgacgcgcaaatgccacacaacctgtcagtatcatttgcctttgctcatcatctggcctcttgatcaaattgaaaagtatgtggagaagctgatctcgctctttaggctcaggatgtagacatgctgtacacaatatgagggggatcaactcctctctctttgccaatagcacattgggaacaatgtgtggcaggcagcgtcccagcattaacataacgcttttttcactgtctgcaatacgagacacctcgtatcctaaacgactatctgctgacattcgacaaaaagagagtagtgcttgatggaatgcaggagacaatttcctattaggtttatcaaaatgaactgtctttttacttgatagagaagaaggtggcattccttctctttctctcctggggaatgaatttggggaattctctttaggaatagtggaatcagcttcatctgatattgaaagatggatgtctgtgttttttcccttgtctgaactatttacatctggatgctgtccactgtcctcagagtctttgtggggcaactgatccaaaggaggctgaacagagtcacaaactgctgggatggcaaagtgttcatttttgaggaagtccatttcacttttaagtcttctgatttgctccatcaatgaccatttctcactatttaacaaactaattttatcttctaatttctgtactaacatggagttctctgcaggctggggagtttcaagagttggaggaaggttgcttataattggtgtaagggcctctaattcatcttcttctactccactggccacatctacaagatcttttccagttacttgatgatttccaaaatcccggtagagttgcaataagtctggaggttttggaatgtttaatcctacatcatcccataattcaaaatcctgatcatcgttttcatctgaaaaggttattgatgtaagcttatagttattcttcaataaaaattcattgactaagaagtttagagctctcttttcaagaggtttgattggctcctgaatttcaggacttgatttgtaattttttcgttcctgtaaaggaacttcatgttctgcggcctttgtcaggttggctcggagggcctgaatggtctccttggctttccgtagttcaaactccaggactgccactttttcatctgtttccctgttaccatcatctgaatatcttgcaaagtctaaagaatcaagggtactaatgctcccagctcgattgagctgtcccccgcccgacgctgtactcggttcccgacctccagcgcccccaacgccggctgctccagggacccctggcgcccccatccccggcggggttccactttgcctctcgaagttgcctggattggagaagtagtcgcgcagccgaggcagctcccggccactctctaacagctcggtatgcagctccagggcggtcagcaagtattgatcgcgcaacagctgagcagcgatcgcatcaattgataatcgggccggggtctccccggtgccccccagggccactgcagccgccgacgcctccccagggagccctggccgcgcactgcttcctaaggccacgggatcctgtggcgacagcgagcccgcagagccaggatctaggccacttccggcgcccagccgaagtactgcccgccgttcctctgttgcagctacctcgtcatcgtcctcatccgaatcactgagaaatggattcacgccgccaccactgccactacctccaggcgccatcgccgccatcttatcctgtcaggagtgtgggcgcctccctgactggttccgacgggccgcagcccgaatcctctaggcctcaggggacacagcgcacctccacagccccggcctgaccacgtcctgcctcccgacttagagacaaggagtacgctccaaggcaggagatccggatgcagctgcacctgatgcctcagcctctgctgcaccagcagcccggctctgcaggcgtcttcctggtctccagtctcgcgagaact

SEQ ID NO: 14607 - RNA, 8118 nt, Homo sapiens
  source 1..8118: mol_type = other RNA
gctgggattacaggcatgagccaccgtgcccggccagtctctatttctttttaatgtactgaaaaaaatagtatcaaaactaagcacactgtaaagttacagtagaactttgaaatagatgtctactcatacaaaaggctaaatttattttgtagttttcttgtaagagaattaacatccaaccttgaaggttgaattttgttacctggctaatctggagtatttcatgaattatgaattagaattgctacttacaaagcttttttttttgtttttgagatggagtcttgctctgtggaccaggctggagtgcagtggtgcaatagcggcccactgcaatctccgcttcccaggttcaaacgattctcctgtctcagcctcccgagtagcagggattacaggcccacgtcaccacgcctggctaatttttgtatttttagaggcggggtttcaccacgttggccaggctggtcttgaactactgacctcaagtgattcgtcaccttggcctcccaaagtgctgagattacaggcgtgagccacagcgcacagtccaaagctctttaagtgtaacattgaagagctaaagtgtaactttctttaatgaactgaaaaaattagtacaatctttacacaaagaatagttaagaaaatataaccagcacagaatgttagctgtagttagctactgcagttcaaagatcagcagggtagtaactacagaaagttacatccttggagttcaaataatggtccaaaataggttgtcttgaaaaatgggatgatgaaaagacaattcaatacatcctgatctcacctctctaaattttaagagagactatttgagccaactttttaaaaacaagaatgtgatagcaccttgacttgagacccccattagaattatagtgtatagtagtgacatatcctatagtagtgacatatcctaaaagctatggataatgaggatggcatgacttaaattactcacaatttcgttcaggttgaaaatcaatttgatgtttagcaaaataatctctctaaaggggtgaataatgcaaaccaatgaaggtcatagacacctatgtatagagatagatactgccatcattcaagcactgttcttggaagaattcagctaaattagtaattatggcacttctggatttctgaaaaaatttaatctctggattactctggaaacacaggtataatttcaaattagcttttcattactttgcaaacttagtttttcattaagttgaacacttaaaaacttgtaccgtaagtttacttctgtttaaaaggaatgagtatgggagttttatgccctattttggactcagtccaaatctcagtctcaatgattagtgtctgtcttgtctgtaaagacaagacatattttactaaaaacaaacaaacaaacaaaaaacaaaaccacaatgtgaaatcttaatgatattaaaatatttaagaaaagagactctcacttgaaatacactgtgaatcttgcctactattgcctttaaaaaaacattagcacttaaataaatatattcattaattaagaaaaatgttcacaataaaaatacattctacccattcacctgataacaaacatacacatattctactatagtttgaagcaaatcagagtttaaacatttttcttccaggtacctctgaaatgtattagttttatagcaacatggtccccttttagtaaaaataaaccaaaataggtaaatttatataaattatatttacaaaatattagtatattctcatgaatataggcttttctcatttttttgcttaatagaaagtatagtgtttcaaaacgaaagtaaaatgcatagcccaaaccaaatcaaaaacatatgcaaaaacattttatttataatagatcaacatttttgacatgaaaggtagccactttcaatttctcaggaatgcctagaacccaacagttttcagaaagactacttagttcacaattatttcactgtaggtaaatgaaataatttcagaatgaactttttaaatggctttgcctatggcaaattgttttataaacttgaatgtatggtaagctagctttcccaggaaatgaatgtaatccaactatgttccaaatgtattaaaccagtttatacaacaaatatgagaatcacttatgtgcatcaactgtgctaaaacaagaattctttttatcaaaatattcatttttcaaaaaggcctcacattaacccctcaaaccaagcacccccttcctatgtccagcactcttttctacttcgagttgcatgactgtagagacaactgtcaaattccagtggaactgtacactgacttaagactctatgtaatatacatcaaacacaggaggtcactgactttaagggacgaggtgataactaactagttataattcagccaatgtcttttttagtttagagggaaaaaagtagcccccaagtgtccttaacttttcagtacttctctgtaacacacagaatgaaaaggtactctctaaaattaaaatcattagaaaatatcttaaataaagtgttttacataaataagtgttaaatttcagattcaaactatattttcttctgtatctcaatttgggaaaaatctcacaattattaactcttctcagttacatttatttttgagcatttaaatctactatacaccagtttgtaaaattcaccttggttacctctccccatgcctatgtgctgtctttcctcaggtaagtccattatatgcatctaagtgctggggaggtttaaatagcacttaaagaatattcatgagagttctgaaatgaaggtttcgtctttagctattgactgtaggatttgtaattcaaatcatcacagcatcctaaagaaatactgtgtgaatggaatgcacacaattcctacagaacacacaaactgatgtccaaaaggcacagagtaatgctggtggctctttctagtcagttaagaaacaataaaaagtctgcattattctttcataatttaaatacttaagtaatctccactttattattttataacaatgacttcaaatttacattattttaagtaccattgtaatagcttagtgtataatacagatatttgcgaatatcccatccaaaaattaaaaaaaacttcttcactatatatatatttatataaaaattattctgaaagacaagaacatagacaagggacttggtacagaccatcaactcaattttctatcaccacagttgtaactccaaaatcaacaaatatacagcagtaattaaaagcagtgcaaatatctttggaggttaggataaaattataatgcaagaacataaaactgaggaaacaaaaaaggcaagtacttcaagtacaaggaaccagtcggcttgaggtccatcttagtgtttactgggggcttctttcctgcttctacttctttctctgaaatacattggccaacatggcacctgatgttgtcaactggcccattttgttcaaaaacttggtctttgtatcttcactcactaagcttgcagcaattgacattgagccttgaggctcttggacggtcttgttttcaactttttgttcacattcttttatcatggaacttaaaataacctcatgctctggagagagatgttccatgtcagtccgtaaacatctgagaccaggtaaaaagtgattaaccattaaatcctctgaaatgaaacaacaggaaagtgcactgtaggcttcaaaaagatgcgtagcaatgtccagtcttttagaatccacaatctgtaagttgttcaccaaggctaacttatgcaaatgtggtataacaaactcatctcggaacctgggttctgcgttagggccaactctaccaaatgtttttatgatctctgtatgcaaagaatgttggtcttgatactgaggatcttccaggaaagaagccaactgcattttcactctttccagcaactctctttgaattactgtttccataatagtgccaaaggctggaattgtggcaatcctgacagagatttcagggtcactggagagagtaatgagagcaggaacaaccctctgagctaccagagtttcattcacccccttcaccaacagctcaaacattctagcagcagtacacctcacgagtgctgaagtatggacaacaccataccacaaaacagttaatagtaactcatggtaggctgggtttgcacccaattccacaaaagaagccttcaggctatcaagaggagcatgagataatgaaagcagcgtcattacatcttctaagaatccaactaacagttttcggtcttcttcctgaatataacacgtaaggactcctgttgcataaatggggactgtagctttagtgaggaccccatttcctgctgaggaatcaatgttttcttcagatagtcttaaaatctcctggaactgaggttttaccttagtgtttgtaaaaattttgccaaatgtccggcaaaggcgccagaaaaatctggagaattcatggacacaggcagttgaagtaacattaattttgccaactatttctataagttgtggcaacaattgattgacaacccacagtaaactctcccagcctgttgtaccctcttgttctagctggtagtcataaagttgcagcagcactgccaattgctcacgacttccgataatagtggacacatcttgaagaggcgacataggccgaggaaacctagtcacttctatctgtggcacttcaccatgaagcttggctttgctggagaaaggtgcattctgtagcactaatgcaaagagagatgggatcaaggactgcaaggcagaaagatacatgtggagtttgtgttcatccagtccatgttctccttccctgagaagtttttcaatcttgttcagtagtgtaagtataagatgagactgtaaatttccaagttctgtagtccacgcagcgtaagctggtaaaaatacttgatgtgtagcactaactactctttctgagggatcacccaaggctgacagcaacaattcaaaaccctgatgatatttgtctggatcatcaatgtatcccataatgataccaaggcttttgataacagcttctcttaccaaatctgccttatcttccattaacatttgttgcaacattgaaagaaccaaggagctacggatttctttaggaaggtaaggtgccagtgctccacaggattctgccacaagcagtcgtctttctgggtatttgtgattaattgggttttgttcccatatgtcttcttcatagaatataaatctttctttgactggaaaaggagtatatttgttctcatattcccatatgaaaaggtgacataattcattaatgtattggatgcctgttcccaacactgtggtaaaagttcagcttctacacgtgttggtccaacatgacgcgcaaatgccacacaacctgtcagtatcatttgcctttgctcatcatctggcctcttgatcaaattgaaaagtatgtggagaagctgatctcgctctttaggctcaggatgtagacatgctgtacacaatatgagggggatcaactcctgttttgcagaagtgaaaggctgagcatcaaattcatgcggaactgcaagggaccctgaacagacaatagtgatgtgcagttagaggactcatatatcccaatttcaaaacttactacaaacaacagttatcaaaacagtgtggtagtggcatatggctagacatacagaccaatggaacagaactgaaagtccagaaataaacccgaagaatctaggcccaactgatttttgacaaaagtagcaagactattcaaaagaggaatttttttatcttgaacaaatgtttctggataactggatagccatatgaaaagaataaagttagacgctgttttactccatatataaaaattaactcaaaatgaatcgttgacctaaatatatataacaaatgttttcttctaattgtttcatagctttagctcttatatatattcatatacatatagatatatatatcttctataacattgattgacttggcaatggtttcttaaaattgatacttagagcacaaacaacacaacaaaaaaatagataaatcagatttcataaaaatggaaaacatttgcccatcaaaggatatggtcaagagtgtaaaaagaaaacctgacagaggtgtaaaaccattctctctctctttgccaatagcacattgggaacaatgtgtggcaggcagcgtcccagcattaacataacgcttttttcactgtctgcaatacgagacacctcgtatcctaaacgactatctgctgacattcgacaaaaagagagtagtgcttgatggaatgcaggagacaatttcctattaggtttatcaaaatgaactgtctttttacttgatagagaagaaggtggcattccttctctttctctcctggggaatgaatttggggaattctctttaggaatagtggaatcagcttcatctgatattgaaagatggatgtctgtgttttttcccttgtctgaactatttacatctggatgctgtccactgtcctcagagtctttgtggggcaactgatccaaaggaggctgaacagagtcacaaactgctgggatggcaaagtgttcatttttgaggaagtccatttcacttttaagtcttctgatttgctccatcaatgaccatttctcactatttaacaaactaattttatcttctaatttctgtactaacatggagttctctgcaggctggggagtttcaagagttggaggaaggttgcttataattggtgtaagggcctctaattcatcttcttctactccactggccacatctacaagatcttttccagttacttgatgatttccaaaatcccggtagagttgcaataagtctggaggttttggaatgtttaatcctacatcatcccataattcaaaatcctgatcatcgttttcatctgaaaaggttattgatgtaagcttatagttattcttcaataaaaattcattgactaagaagtttagagctctcttttcaagaggtttgattggctcctgaatttcaggacttgatttgtaattttttcgttcctgtaaaggaacttcatgttctgcggcctttgtcaggttggctcggagggcctgaatggtctccttggctttccgtagttcaaactccaggactgccactttttcatctgtttccctgttaccatcatctgaatatcttgcaaagtctaaagaatcaagggtactaatgctcccagctcgattgagctgtcccccgcccgacgctgtactcggttcccgacctccagcgcccccaacgccggctgctccagggacccctggcgcccccatccccggcggggttccactttgcctctcgaagttgcctggattggagaagtagtcgcgcagccgaggcagctcccggccactctctaacagctcggtatgcagctccagggcggtcagcaagtattgatcgcgcaacagctgagcagcgatcgcatcaattgataatcgggccggggtctccccggtgccccccagggccactgcagccgccgacgcctccccagggagccctggccgcgcactgcttcctaaggccacgggatcctgtggcgacagcgagcccgcagagccaggatctaggccacttccggcgcccagccgaagtactgcccgccgttcctctgttgcagctacctcgtcatcgtcctcatccgaatcactgagaaatggattcacgccgccaccactgccactacctccaggcgccatcgccgccatcttatcctgtcaggagtgtgggcgcctccctgactggttccgacgggccgcagcccgaatcctctaggcctcaggggacacagcgcacctccacagccccggcctgaccacgtcctgcctcccgacttagagacaaggagtacgctccaaggcaggagatccggatgcagctgcacctgatgcctcagcctctgctgcaccagcagcccggctctgcaggcgtcttcctggtctccagtctcgcgagaact

SEQ ID NO: 14608 - RNA, 7462 nt, Homo sapiens
  source 1..7462: mol_type = other RNA
gctgggattacaggcatgagccaccgtgcccggccagtctctatttctttttaatgtactgaaaaaaatagtatcaaaactaagcacactgtaaagttacagtagaactttgaaatagatgtctactcatacaaaaggctaaatttattttgtagttttcttgtaagagaattaacatccaaccttgaaggttgaattttgttacctggctaatctggagtatttcatgaattatgaattagaattgctacttacaaagcttttttttttgtttttgagatggagtcttgctctgtggaccaggctggagtgcagtggtgcaatagcggcccactgcaatctccgcttcccaggttcaaacgattctcctgtctcagcctcccgagtagcagggattacaggcccacgtcaccacgcctggctaatttttgtatttttagaggcggggtttcaccacgttggccaggctggtcttgaactactgacctcaagtgattcgtcaccttggcctcccaaagtgctgagattacaggcgtgagccacagcgcacagtccaaagctctttaagtgtaacattgaagagctaaagtgtaactttctttaatgaactgaaaaaattagtacaatctttacacaaagaatagttaagaaaatataaccagcacagaatgttagctgtagttagctactgcagttcaaagatcagcagggtagtaactacagaaagttacatccttggagttcaaataatggtccaaaataggttgtcttgaaaaatgggatgatgaaaagacaattcaatacatcctgatctcacctctctaaattttaagagagactatttgagccaactttttaaaaacaagaatgtgatagcaccttgacttgagacccccattagaattatagtgtatagtagtgacatatcctatagtagtgacatatcctaaaagctatggataatgaggatggcatgacttaaattactcacaatttcgttcaggttgaaaatcaatttgatgtttagcaaaataatctctctaaaggggtgaataatgcaaaccaatgaaggtcatagacacctatgtatagagatagatactgccatcattcaagcactgttcttggaagaattcagctaaattagtaattatggcacttctggatttctgaaaaaatttaatctctggattactctggaaacacaggtataatttcaaattagcttttcattactttgcaaacttagtttttcattaagttgaacacttaaaaacttgtaccgtaagtttacttctgtttaaaaggaatgagtatgggagttttatgccctattttggactcagtccaaatctcagtctcaatgattagtgtctgtcttgtctgtaaagacaagacatattttactaaaaacaaacaaacaaacaaaaaacaaaaccacaatgtgaaatcttaatgatattaaaatatttaagaaaagagactctcacttgaaatacactgtgaatcttgcctactattgcctttaaaaaaacattagcacttaaataaatatattcattaattaagaaaaatgttcacaataaaaatacattctacccattcacctgataacaaacatacacatattctactatagtttgaagcaaatcagagtttaaacatttttcttccaggtacctctgaaatgtattagttttatagcaacatggtccccttttagtaaaaataaaccaaaataggtaaatttatataaattatatttacaaaatattagtatattctcatgaatataggcttttctcatttttttgcttaatagaaagtatagtgtttcaaaacgaaagtaaaatgcatagcccaaaccaaatcaaaaacatatgcaaaaacattttatttataatagatcaacatttttgacatgaaaggtagccactttcaatttctcaggaatgcctagaacccaacagttttcagaaagactacttagttcacaattatttcactgtaggtaaatgaaataatttcagaatgaactttttaaatggctttgcctatggcaaattgttttataaacttgaatgtatggtaagctagctttcccaggaaatgaatgtaatccaactatgttccaaatgtattaaaccagtttatacaacaaatatgagaatcacttatgtgcatcaactgtgctaaaacaagaattctttttatcaaaatattcatttttcaaaaaggcctcacattaacccctcaaaccaagcacccccttcctatgtccagcactcttttctacttcgagttgcatgactgtagagacaactgtcaaattccagtggaactgtacactgacttaagactctatgtaatatacatcaaacacaggaggtcactgactttaagggacgaggtgataactaactagttataattcagccaatgtcttttttagtttagagggaaaaaagtagcccccaagtgtccttaacttttcagtacttctctgtaacacacagaatgaaaaggtactctctaaaattaaaatcattagaaaatatcttaaataaagtgttttacataaataagtgttaaatttcagattcaaactatattttcttctgtatctcaatttgggaaaaatctcacaattattaactcttctcagttacatttatttttgagcatttaaatctactatacaccagtttgtaaaattcaccttggttacctctccccatgcctatgtgctgtctttcctcaggtaagtccattatatgcatctaagtgctggggaggtttaaatagcacttaaagaatattcatgagagttctgaaatgaaggtttcgtctttagctattgactgtaggatttgtaattcaaatcatcacagcatcctaaagaaatactgtgtgaatggaatgcacacaattcctacagaacacacaaactgatgtccaaaaggcacagagtaatgctggtggctctttctagtcagttaagaaacaataaaaagtctgcattattctttcataatttaaatacttaagtaatctccactttattattttataacaatgacttcaaatttacattattttaagtaccattgtaatagcttagtgtataatacagatatttgcgaatatcccatccaaaaattaaaaaaaacttcttcactatatatatatttatataaaaattattctgaaagacaagaacatagacaagggacttggtacagaccatcaactcaattttctatcaccacagttgtaactccaaaatcaacaaatatacagcagtaattaaaagcagtgcaaatatctttggaggttaggataaaattataatgcaagaacataaaactgaggaaacaaaaaaggcaagtacttcaagtacaaggaaccagtcggcttgaggtccatcttagtgtttactgggggcttctttcctgcttctacttctttctctgaaatacattggccaacatggcacctgatgttgtcaactggcccattttgttcaaaaacttggtctttgtatcttcactcactaagcttgcagcaattgacattgagccttgaggctcttggacggtcttgttttcaactttttgttcacattcttttatcatggaacttaaaataacctcatgctctggagagagatgttccatgtcagtccgtaaacatctgagaccaggtaaaaagtgattaaccattaaatcctctgaaatgaaacaacaggaaagtgcactgtaggcttcaaaaagatgcgtagcaatgtccagtcttttagaatccacaatctgtaagttgttcaccaaggctaacttatgcaaatgtggtataacaaactcatctcggaacctgggttctgcgttagggccaactctaccaaatgtttttatgatctctgtatgcaaagaatgttggtcttgatactgaggatcttccaggaaagaagccaactgcattttcactctttccagcaactctctttgaattactgtttccataatagtgccaaaggctggaattgtggcaatcctgacagagatttcagggtcactggagagagtaatgagagcaggaacaaccctctgagctaccagagtttcattcacccccttcaccaacagctcaaacattctagcagcagtacacctcacgagtgctgaagtatggacaacaccataccacaaaacagttaatagtaactcatggtaggctgggtttgcacccaattccacaaaagaagccttcaggctatcaagaggagcatgagataatgaaagcagcgtcattacatcttctaagaatccaactaacagttttcggtcttcttccttcaggctatgtgtataatgtgtatatgaaacacattttgtgtttagacttgggtcccattcccaagatatctcattatgtatatgcaaatactcctttatctgaatataacacgtaaggactcctgttgcataaatggggactgtagctttagtgaggaccccatttcctgctgaggaatcaatgttttcttcagatagtcttaaaatctcctggaactgaggttttaccttagtgtttgtaaaaattttgccaaatgtccggcaaaggcgccagaaaaatctggagaattcatggacacaggcagttgaagtaacattaattttgccaactatttctataagttgtggcaacaattgattgacaacccacagtaaactctcccagcctgttgtaccctcttgttctagctggtagtcataaagttgcagcagcactgccaattgctcacgacttccgataatagtggacacatcttgaagaggcgacataggccgaggaaacctagtcacttctatctgtggcacttcaccatgaagcttggctttgctggagaaaggtgcattctgtagcactaatgcaaagagagatgggatcaaggactgcaaggcagaaagatacatgtggagtttgtgttcatccagtccatgttctccttccctgagaagtttttcaatcttgttcagtagtgtaagtataagatgagactgtaaatttccaagttctgtagtccacgcagcgtaagctggtaaaaatacttgatgtgtagcactaactactctttctgagggatcacccaaggctgacagcaacaattcaaaaccctgatgatatttgtctggatcatcaatgtatcccataatgataccaaggcttttgataacagcttctcttaccaaatctgccttatcttccattaacatttgttgcaacattgaaagaaccaaggagctacggatttctttaggaaggtaaggtgccagtgctccacaggattctgccacaagcagtcgtctttctgggtatttgtgattaatctgttcccaacactgtggtaaaagttcagcttctacacgtgttggtccaacatgacgcgcaaatgccacacaacctgtcagtatcatttgcctttgctcatcatctggcctcttgatcaaattgaaaagtatgtggagaagctgatctcgctctttaggctcaggatgtagacatgctgtacacaatatgagggggatcaactcctctctctttgccaatagcacattgggaacaatgtgtggcaggcagcgtcccagcattaacataacgcttttttcactgtctgcaatacgagacacctcgtatcctaaacgactatctgctgacattcgacaaaaagagagtagtgcttgatggaatgcaggagacaatttcctattaggtttatcaaaatgaactgtctttttacttgatagagaagaaggtggcattccttctctttctctcctggggaatgaatttggggaattctctttaggaatagtggaatcagcttcatctgatattgaaagatggatgtctgtgttttttcccttgtctgaactatttacatctggatgctgtccactgtcctcagagtctttgtggggcaactgatccaaaggaggctgaacagagtcacaaactgctgggatggcaaagtgttcatttttgaggaagtccatttcacttttaagtcttctgatttgctccatcaatgaccatttctcactatttaacaaactaattttatcttctaatttctgtactaacatggagttctctgcaggctggggagtttcaagagttggaggaaggttgcttataattggtgtaagggcctctaattcatcttcttctactccactggccacatctacaagatcttttccagttacttgatgatttccaaaatcccggtagagttgcaataagtctggaggttttggaatgtttaatcctacatcatcccataattcaaaatcctgatcatcgttttcatctgaaaaggttattgatgtaagcttatagttattcttcaataaaaattcattgactaagaagtttagagctctcttttcaagaggtttgattggctcctgaatttcaggacttgatttgtaattttttcgttcctgtaaaggaacttcatgttctgcggcctttgtcaggttggctcggagggcctgaatggtctccttggctttccgtagttcaaactccaggactgccactttttcatctgtttccctgttaccatcatctgaatatcttgcaaagtctaaagaatcaagggtactaatgctcccagctcgattgagctgtcccccgcccgacgctgtactcggttcccgacctccagcgcccccaacgccggctgctccagggacccctggcgcccccatccccggcggggttccactttgcctctcgaagttgcctggattggagaagtagtcgcgcagccgaggcagctcccggccactctctaacagctcggtatgcagctccagggcggtcagcaagtattgatcgcgcaacagctgagcagcgatcgcatcaattgataatcgggccggggtctccccggtgccccccagggccactgcagccgccgacgcctccccagggagccctggccgcgcactgcttcctaaggccacgggatcctgtggcgacagcgagcccgcagagccaggatctaggccacttccggcgcccagccgaagtactgcccgccgttcctctgttgcagctacctcgtcatcgtcctcatccgaatcactgagaaatggattcacgccgccaccactgccactacctccaggcgccatcgccgccatcttatcctgtcaggagtgtgggcgcctccctgactggttccgacgggccgcagcccgaatcctctaggcctcaggggacacagcgcacctccacagccccggcctgaccacgtcctgcctcccgacttagagacaaggagtacgctccaaggcaggagatccggatgcagctgcacctgatgcctcagcctctgctgcaccagcagcccggctctgcaggcgtcttcctggtctccagtctcgcgagaact

SEQ ID NO: 14609 - RNA, 9491 nt, Homo sapiens
  source 1..9491: mol_type = other RNA
gctgggattacaggcatgagccaccgtgcccggccagtctctatttctttttaatgtactgaaaaaaatagtatcaaaactaagcacactgtaaagttacagtagaactttgaaatagatgtctactcatacaaaaggctaaatttattttgtagttttcttgtaagagaattaacatccaaccttgaaggttgaattttgttacctggctaatctggagtatttcatgaattatgaattagaattgctacttacaaagcttttttttttgtttttgagatggagtcttgctctgtggaccaggctggagtgcagtggtgcaatagcggcccactgcaatctccgcttcccaggttcaaacgattctcctgtctcagcctcccgagtagcagggattacaggcccacgtcaccacgcctggctaatttttgtatttttagaggcggggtttcaccacgttggccaggctggtcttgaactactgacctcaagtgattcgtcaccttggcctcccaaagtgctgagattacaggcgtgagccacagcgcacagtccaaagctctttaagtgtaacattgaagagctaaagtgtaactttctttaatgaactgaaaaaattagtacaatctttacacaaagaatagttaagaaaatataaccagcacagaatgttagctgtagttagctactgcagttcaaagatcagcagggtagtaactacagaaagttacatccttggagttcaaataatggtccaaaataggttgtcttgaaaaatgggatgatgaaaagacaattcaatacatcctgatctcacctctctaaattttaagagagactatttgagccaactttttaaaaacaagaatgtgatagcaccttgacttgagacccccattagaattatagtgtatagtagtgacatatcctatagtagtgacatatcctaaaagctatggataatgaggatggcatgacttaaattactcacaatttcgttcaggttgaaaatcaatttgatgtttagcaaaataatctctctaaaggggtgaataatgcaaaccaatgaaggtcatagacacctatgtatagagatagatactgccatcattcaagcactgttcttggaagaattcagctaaattagtaattatggcacttctggatttctgaaaaaatttaatctctggattactctggaaacacaggtataatttcaaattagcttttcattactttgcaaacttagtttttcattaagttgaacacttaaaaacttgtaccgtaagtttacttctgtttaaaaggaatgagtatgggagttttatgccctattttggactcagtccaaatctcagtctcaatgattagtgtctgtcttgtctgtaaagacaagacatattttactaaaaacaaacaaacaaacaaaaaacaaaaccacaatgtgaaatcttaatgatattaaaatatttaagaaaagagactctcacttgaaatacactgtgaatcttgcctactattgcctttaaaaaaacattagcacttaaataaatatattcattaattaagaaaaatgttcacaataaaaatacattctacccattcacctgataacaaacatacacatattctactatagtttgaagcaaatcagagtttaaacatttttcttccaggtacctctgaaatgtattagttttatagcaacatggtccccttttagtaaaaataaaccaaaataggtaaatttatataaattatatttacaaaatattagtatattctcatgaatataggcttttctcatttttttgcttaatagaaagtatagtgtttcaaaacgaaagtaaaatgcatagcccaaaccaaatcaaaaacatatgcaaaaacattttatttataatagatcaacatttttgacatgaaaggtagccactttcaatttctcaggaatgcctagaacccaacagttttcagaaagactacttagttcacaattatttcactgtaggtaaatgaaataatttcagaatgaactttttaaatggctttgcctatggcaaattgttttataaacttgaatgtatggtaagctagctttcccaggaaatgaatgtaatccaactatgttccaaatgtattaaaccagtttatacaacaaatatgagaatcacttatgtgcatcaactgtgctaaaacaagaattctttttatcaaaatattcatttttcaaaaaggcctcacattaacccctcaaaccaagcacccccttcctatgtccagcactcttttctacttcgagttgcatgactgtagagacaactgtcaaattccagtggaactgtacactgacttaagactctatgtaatatacatcaaacacaggaggtcactgactttaagggacgaggtgataactaactagttataattcagccaatgtcttttttagtttagagggaaaaaagtagcccccaagtgtccttaacttttcagtacttctctgtaacacacagaatgaaaaggtactctctaaaattaaaatcattagaaaatatcttaaataaagtgttttacataaataagtgttaaatttcagattcaaactatattttcttctgtatctcaatttgggaaaaatctcacaattattaactcttctcagttacatttatttttgagcatttaaatctactatacaccagtttgtaaaattcaccttggttacctctccccatgcctatgtgctgtctttcctcaggtaagtccattatatgcatctaagtgctggggaggtttaaatagcacttaaagaatattcatgagagttctgaaatgaaggtttcgtctttagctattgactgtaggatttgtaattcaaatcatcacagcatcctaaagaaatactgtgtgaatggaatgcacacaattcctacagaacacacaaactgatgtccaaaaggcacagagtaatgctggtggctctttctagtcagttaagaaacaataaaaagtctgcattattctttcataatttaaatacttaagtaatctccactttattattttataacaatgacttcaaatttacattattttaagtaccattgtaatagcttagtgtataatacagatatttgcgaatatcccatccaaaaattaaaaaaaacttcttcactatatatatatttatataaaaattattctgaaagacaagaacatagacaagggacttggtacagaccatcaactcaattttctatcaccacagttgtaactccaaaatcaacaaatatacagcagtaattaaaagcagtgcaaatatctttggaggttaggataaaattataatgcaagaacataaaactgaggaaacaaaaaaggcaagtacttcaagtacaaggaaccagtcggcttgaggtccatcttagtgtttactgggggcttctttcctgcttctacttctttctctgaaatacattggccaacatggcacctgatgttgtcaactggcccattttgttcaaaaacttggtctttgtatcttcactcactaagcttgcagcaattgacattgagccttgaggctcttggacggtcttgttttcaactttttgttcacattcttttatcatggaacttaaaataacctcatgctctggagagagatgttccatgtcagtccgtaaacatctgagaccaggtaaaaagtgattaaccattaaatcctctgaaatgaaacaacaggaaagtgcactgtaggcttcaaaaagatgcgtagcaatgtccagtcttttagaatccacaatctgtaagttgttcaccaaggctaacttatgcaaatgtggtataacaactgaaaacagaaaaaaaagggttaaatttttacccaaaacatgcatacaaaaccctgacacactttaacaataatttatcactttaatttatgaaatttcattttaattctgaatgacttcaaaagattacccatatcttatacttgctttttcttaactagggaagaaagtagtttttcaaaataaaaagtgatctggcatttgggggaaacaaattttagtactgtcactattacctaattatgaggatgtatatagattatttggcctcactgtaattcagtttcccagtttgaaaaatgaagcccaaataattataaacaacatacctcttgtattatttatacttgcagttaagtttctccataaaaataaaatattaccattgctatgaaatcaaaagagtatattctttttcaacaacctattatttcactccttcagaatactattatcagctttagtttctcaaattcttagcaaagaccaatgtcaaacagcactggcggctgagttttcaagttattcaatgagtttaataccctcaaagagtaacataaaatttcaacctactgctaaataaaagcaatggtccaagaaacaaaaaccaattcagtagcaatgagcacctctagagcctaagattgtgttttctgggtaccatttcccactaaaaccagggctctttgaagaaatggcttcagggtcagtgattgttaaattgttaatcacaagaccaatcacacaacccctttctagtctctgcttggttgaggatcacaaaacgccacccataagcatcaactgctgaccaactgtagtgacccctttcttgtttgcactgagtttgtgtatataaagtcataatcttctactggaaaaactcctgcatcctaaataagctggggcaataatcacaactttcatgcttagcttagtaaaaccccacaaaaactcagaataacaatgatcatttttaggggaccttttgacttgtcaaaattaataacagtatatttatgaggagctctagaacaaattaggaaacaaaaactccaaacattcagttgaaagcttcattaattggcacgctgaggcctcaacaaaatagtgactctaagtctctctcaaagactcactagttcatttctgcccaaacattcagaaacttatcattctttcactttatctattcatatatggttcctttatttcatcttctcctgagtctctgacctttttacaaggtttttctcagaaatgcaacaatcacactgcataatatccccttaaaattgcttgactagaagaaatctatagaagttcatttaaactgtagtctcaaggaagttaaagcctctaattaaggatcttcctaattctcaggaagacagacagaactttactatagaattcagatttcactacacacatattgtcctggggtaccacatatgtattaattaattcacttaacagttaacccctcagatgtagacagatggttaaaagcagtaggagatgaaggaccaggagatgatttaataataacccagatggatatcattctttcttttttattaagagatggggtcttgctctgttgcttgggctggaatgcaatgactattcacaggtgcaatcatagtgcaccacagcctcaaacacttggactcaagtgatcttcctgccttggcctcccgagttgatggactacagatacgtgccaccatgcctagctaatttttaaacatcttttgtagggacttatcttgctgtgttgctcaggctggtgttgaactcctggcctcaagtgatcctcccacctcagcttctgagtaggtgggactatagacacgtggcaccatgcctgacttagacaggctaattctaaaactgacactcatctcggaacctgggttctgcgttagggccaactctaccaaatgtttttatgatctctgtatgcaaagaatgttggtcttgatactgaggatcttccaggaaagaagccaactgcattttcactctttccagcaactctctttgaattactgtttccataatagtgccaaaggctggaattgtggcaatcctgacagagaattcaggatcactggacaaggtaacaagggccggagcaacccgcttgtcaactaacgcttcactcatgcctcgaagagtcagatttcagggtcactggagagagtaatgagagcaggaacaaccctctgagctaccagagtttcattcacccccttcaccaacagctcaaacattctagcagcagtacacctcacgagtgctgaagtatggacaacaccataccacaaaacagttaatagtaactcatggtaggctgggtttgcacccaattccacaaaagaagccttcaggctatcaagaggagcatgagataatgaaagcagcgtcattacatcttctaagaatccaactaacagttttcggtcttcttcctgaatataacacgtaaggactcctgttgcataaatggggactgtagctttagtgaggaccccatttcctgctgaggaatcaatgttttcttcagatagtcttaaaatctcctggaactgaggttttaccttagtgtttgtaaaaattttgccaaatgtccggcaaaggcgccagaaaaatctggagaattcatggacacaggcagttgaagtaacattaattttgccaactatttctataagttgtggcaacaattgattgacaacccacagtaaactctcccagcctgttgtaccctcttgttctagctggtagtcataaagttgcagcagcactgccaattgctcacgacttccgataatagtggacacatcttgaagaggcgacataggccgaggaaacctagtcacttctatctgtggcacttcaccatgaagcttggctttgctggagaaaggtgcattctgtagcactaatgcaaagagagatgggatcaaggactgcaaggcagaaagatacatgtggagtttgtgttcatccagtccatgttctccttccctgagaagtttttcaatcttgttcagtagtgtaagtataagatgagactgtaaatttccaagttctgtagtccacgcagcgtaagctggtaaaaatacttgatgtgtagcactaactactctttctgagggatcacccaaggctgacagcaacaattcaaaaccctgatgatatttgtctggatcatcaatgtatcccataatgataccaaggcttttgataacagcttctcttaccaaatctgccttatcttccattaacatttgttgcaacattgaaagaaccaaggagctacggatttctttaggaaggtaaggtgccagtgctccacaggattctgccacaagcagtcgtctttctgggtatttgtgattaattgggttttgttcccatatgtcttcttcatagaatataaatctttctttgactggaaaaggagtatatttgttctcatattcccatatgaaaaggtgacataattcattaatgtattggatgcctgttcccaacactgtggtaaaagttcagcttctacacgtgttggtccaacatgacgcgcaaatgccacacaacctgtcagtatcatttgcctttgctcatcatctggcctcttgatcaaattgaaaagtatgtggagaagctgatctcgctctttaggctcaggatgtagacatgctgtacacaatatgagggggatcaactcctgacagaggtgtaaaaccattctctctctctttgccaatagcacattgggaacaatgtgtggcaggcagcgtcccagcattaacataacgcttttttcactgtctgcaatacgagacacctcgtatcctaaacgactatctgctgacattcgacaaaaagagagtagtgcttgatggaatgcaggagacaatttcctattaggtttatcaaaatgaactgtctttttacttgatagagaagaaggtggcattccttctctttctctcctggggaatgaatttggggaattctctttaggaatagtggaatcagcttcatctgatattgaaagatggatgtctgtgttttttcccttgtctgaactatttacatctggatgctgtccactgtcctcagagtctttgtggggcaactgatccaaaggaggctgaacagagtcacaaactgctgggatggcaaagtgttcatttttgaggaagtccatttcacttttaagtcttctgatttgctccatcaatgaccatttctcactatttaacaaactaattttatcttctaatttctgtactaacatggagttctctgcaggctggggagtttcaagagttggaggaaggttgcttataattggtgtaagggcctctaattcatcttcttctactccactggccacatctacaagatcttttccagttacttgatgatttccaaaatcccggtagagttgcaataagtctggaggttttggaatgtttaatcctacatcatcccataattcaaaatcctgatcatcgttttcatctgaaaaggttattgatgtaagcttatagttattcttcaataaaaattcattgactaagaagtttagagctctcttttcaagaggtttgattggctcctgaatttcaggacttgatttgtaattttttcgttcctgtaaaggaacttcatgttctgcggcctttgtcaggttggctcggagggcctgaatggtctccttggctttccgtagttcaaactccaggactgccactttttcatctgtttccctgttaccatcatctgaatatcttgcaaagtctaaagaatcaagggtactaatgctcccagctcgattgagctgtcccccgcccgacgctgtactcggttcccgacctccagcgcccccaacgccggctgctccagggacccctggcgcccccatccccggcggggttccactttgcctctcgaagttgcctggattggagaagtagtcgcgcagccgaggcagctcccggccactctctaacagctcggtatgcagctccagggcggtcagcaagtattgatcgcgcaacagctgagcagcgatcgcatcaattgataatcgggccggggtctccccggtgccccccagggccactgcagccgccgacgcctccccagggagccctggccgcgcactgcttcctaaggccacgggatcctgtggcgacagcgagcccgcagagccaggatctaggccacttccggcgcccagccgaagtactgcccgccgttcctctgttgcagctacctcgtcatcgtcctcatccgaatcactgagaaatggattcacgccgccaccactgccactacctccaggcgccatcgccgccatcttatcctgtcaggagtgtgggcgcctccctgactggttccgacgggccgcagcccgaatcctctaggcctcaggggacacagcgcacctccacagccccggcctgaccacgtcctgcctcccgacttagagacaaggagtacgctccaaggcaggagatccggatgcagctgcacctgatgcctcagcctctgctgcaccagcagcccggctctgcaggcgtcttcctggtctccagtctcgcgagaact

SEQ ID NO: 14610 - RNA, 9262 nt, Homo sapiens
  source 1..9262: mol_type = other RNA
gctgggattacaggcatgagccaccgtgcccggccagtctctatttctttttaatgtactgaaaaaaatagtatcaaaactaagcacactgtaaagttacagtagaactttgaaatagatgtctactcatacaaaaggctaaatttattttgtagttttcttgtaagagaattaacatccaaccttgaaggttgaattttgttacctggctaatctggagtatttcatgaattatgaattagaattgctacttacaaagcttttttttttgtttttgagatggagtcttgctctgtggaccaggctggagtgcagtggtgcaatagcggcccactgcaatctccgcttcccaggttcaaacgattctcctgtctcagcctcccgagtagcagggattacaggcccacgtcaccacgcctggctaatttttgtatttttagaggcggggtttcaccacgttggccaggctggtcttgaactactgacctcaagtgattcgtcaccttggcctcccaaagtgctgagattacaggcgtgagccacagcgcacagtccaaagctctttaagtgtaacattgaagagctaaagtgtaactttctttaatgaactgaaaaaattagtacaatctttacacaaagaatagttaagaaaatataaccagcacagaatgttagctgtagttagctactgcagttcaaagatcagcagggtagtaactacagaaagttacatccttggagttcaaataatggtccaaaataggttgtcttgaaaaatgggatgatgaaaagacaattcaatacatcctgatctcacctctctaaattttaagagagactatttgagccaactttttaaaaacaagaatgtgatagcaccttgacttgagacccccattagaattatagtgtatagtagtgacatatcctatagtagtgacatatcctaaaagctatggataatgaggatggcatgacttaaattactcacaatttcgttcaggttgaaaatcaatttgatgtttagcaaaataatctctctaaaggggtgaataatgcaaaccaatgaaggtcatagacacctatgtatagagatagatactgccatcattcaagcactgttcttggaagaattcagctaaattagtaattatggcacttctggatttctgaaaaaatttaatctctggattactctggaaacacaggtataatttcaaattagcttttcattactttgcaaacttagtttttcattaagttgaacacttaaaaacttgtaccgtaagtttacttctgtttaaaaggaatgagtatgggagttttatgccctattttggactcagtccaaatctcagtctcaatgattagtgtctgtcttgtctgtaaagacaagacatattttactaaaaacaaacaaacaaacaaaaaacaaaaccacaatgtgaaatcttaatgatattaaaatatttaagaaaagagactctcacttgaaatacactgtgaatcttgcctactattgcctttaaaaaaacattagcacttaaataaatatattcattaattaagaaaaatgttcacaataaaaatacattctacccattcacctgataacaaacatacacatattctactatagtttgaagcaaatcagagtttaaacatttttcttccaggtacctctgaaatgtattagttttatagcaacatggtccccttttagtaaaaataaaccaaaataggtaaatttatataaattatatttacaaaatattagtatattctcatgaatataggcttttctcatttttttgcttaatagaaagtatagtgtttcaaaacgaaagtaaaatgcatagcccaaaccaaatcaaaaacatatgcaaaaacattttatttataatagatcaacatttttgacatgaaaggtagccactttcaatttctcaggaatgcctagaacccaacagttttcagaaagactacttagttcacaattatttcactgtaggtaaatgaaataatttcagaatgaactttttaaatggctttgcctatggcaaattgttttataaacttgaatgtatggtaagctagctttcccaggaaatgaatgtaatccaactatgttccaaatgtattaaaccagtttatacaacaaatatgagaatcacttatgtgcatcaactgtgctaaaacaagaattctttttatcaaaatattcatttttcaaaaaggcctcacattaacccctcaaaccaagcacccccttcctatgtccagcactcttttctacttcgagttgcatgactgtagagacaactgtcaaattccagtggaactgtacactgacttaagactctatgtaatatacatcaaacacaggaggtcactgactttaagggacgaggtgataactaactagttataattcagccaatgtcttttttagtttagagggaaaaaagtagcccccaagtgtccttaacttttcagtacttctctgtaacacacagaatgaaaaggtactctctaaaattaaaatcattagaaaatatcttaaataaagtgttttacataaataagtgttaaatttcagattcaaactatattttcttctgtatctcaatttgggaaaaatctcacaattattaactcttctcagttacatttatttttgagcatttaaatctactatacaccagtttgtaaaattcaccttggttacctctccccatgcctatgtgctgtctttcctcaggtaagtccattatatgcatctaagtgctggggaggtttaaatagcacttaaagaatattcatgagagttctgaaatgaaggtttcgtctttagctattgactgtaggatttgtaattcaaatcatcacagcatcctaaagaaatactgtgtgaatggaatgcacacaattcctacagaacacacaaactgatgtccaaaaggcacagagtaatgctggtggctctttctagtcagttaagaaacaataaaaagtctgcattattctttcataatttaaatacttaagtaatctccactttattattttataacaatgacttcaaatttacattattttaagtaccattgtaatagcttagtgtataatacagatatttgcgaatatcccatccaaaaattaaaaaaaacttcttcactatatatatatttatataaaaattattctgaaagacaagaacatagacaagggacttggtacagaccatcaactcaattttctatcaccacagttgtaactccaaaatcaacaaatatacagcagtaattaaaagcagtgcaaatatctttggaggttaggataaaattataatgcaagaacataaaactgaggaaacaaaaaaggcaagtacttcaagtacaaggaaccagtcggcttgaggtccatcttagtgtttactgggggcttctttcctgcttctacttctttctctgaaatacattggccaacatggcacctgatgttgtcaactggcccattttgttcaaaaacttggtctttgtatcttcactcactaagcttgcagcaattgacattgagccttgaggctcttggacggtcttgttttcaactttttgttcacattcttttatcatggaacttaaaataacctcatgctctggagagagatgttccatgtcagtccgtaaacatctgagaccaggtaaaaagtgattaaccattaaatcctctgaaatgaaacaacaggaaagtgcactgtaggcttcaaaaagatgcgtagcaatgtccagtcttttagaatccacaatctgtaagttgttcaccaaggctaacttatgcaaatgtggtataacaactgaaaacagaaaaaaaagggttaaatttttacccaaaacatgcatacaaaaccctgacacactttaacaataatttatcactttaatttatgaaatttcattttaattctgaatgacttcaaaagattacccatatcttatacttgctttttcttaactagggaagaaagtagtttttcaaaataaaaagtgatctggcatttgggggaaacaaattttagtactgtcactattacctaattatgaggatgtatatagattatttggcctcactgtaattcagtttcccagtttgaaaaatgaagcccaaataattataaacaacatacctcttgtattatttatacttgcagttaagtttctccataaaaataaaatattaccattgctatgaaatcaaaagagtatattctttttcaacaacctattatttcactccttcagaatactattatcagctttagtttctcaaattcttagcaaagaccaatgtcaaacagcactggcggctgagttttcaagttattcaatgagtttaataccctcaaagagtaacataaaatttcaacctactgctaaataaaagcaatggtccaagaaacaaaaaccaattcagtagcaatgagcacctctagagcctaagattgtgttttctgggtaccatttcccactaaaaccagggctctttgaagaaatggcttcagggtcagtgattgttaaattgttaatcacaagaccaatcacacaacccctttctagtctctgcttggttgaggatcacaaaacgccacccataagcatcaactgctgaccaactgtagtgacccctttcttgtttgcactgagtttgtgtatataaagtcataatcttctactggaaaaactcctgcatcctaaataagctggggcaataatcacaactttcatgcttagcttagtaaaaccccacaaaaactcagaataacaatgatcatttttaggggaccttttgacttgtcaaaattaataacagtatatttatgaggagctctagaacaaattaggaaacaaaaactccaaacattcagttgaaagcttcattaattggcacgctgaggcctcaacaaaatagtgactctaagtctctctcaaagactcactagttcatttctgcccaaacattcagaaacttatcattctttcactttatctattcatatatggttcctttatttcatcttctcctgagtctctgacctttttacaaggtttttctcagaaatgcaacaatcacactgcataatatccccttaaaattgcttgactagaagaaatctatagaagttcatttaaactgtagtctcaaggaagttaaagcctctaattaaggatcttcctaattctcaggaagacagacagaactttactatagaattcagatttcactacacacatattgtcctggggtaccacatatgtattaattaattcacttaacagttaacccctcagatgtagacagatggttaaaagcagtaggagatgaaggaccaggagatgatttaataataacccagatggatatcattctttcttttttattaagagatggggtcttgctctgttgcttgggctggaatgcaatgactattcacaggtgcaatcatagtgcaccacagcctcaaacacttggactcaagtgatcttcctgccttggcctcccgagttgatggactacagatacgtgccaccatgcctagctaatttttaaacatcttttgtagggacttatcttgctgtgttgctcaggctggtgttgaactcctggcctcaagtgatcctcccacctcagcttctgagtaggtgggactatagacacgtggcaccatgcctgacttagacaggctaattctaaaactgacactcatctcggaacctgggttctgcgttagggccaactctaccaaatgtttttatgatctctgtatgcaaagaatgttggtcttgatactgaggatcttccaggaaagaagccaactgcattttcactctttccagcaactctctttgaattactgtttccataatagtgccaaaggctggaattgtggcaatcctgacagagatttcagggtcactggagagagtaatgagagcaggaacaaccctctgagctaccagagtttcattcacccccttcaccaacagctcaaacattctagcagcagtacacctcacgagtgctgaagtatggacaacaccataccacaaaacagttaatagtaactcatggtaggctgggtttgcacccaattccacaaaagaagccttcaggctatcaagaggagcatgagataatgaaagcagcgtcattacatcttctaagaatccaactaacagttttcggtcttcttcctgaatataacacgtaaggactcctgttgcataaatggggactgtagctttagtgaggaccccatttcctgctgaggaatcaatgttttcttcagatagtcttaaaatctcctggaactgaggttttaccttagtgtttgtaaaaattttgccaaatgtccggcaaaggcgccagaaaaatctggagaattcatggacacaggcagttgaagtaacattaattttgccaactatttctataagttgtggcaacaattgattgacaacccacagtaaactctcccagcctgttgtaccctcttgttctagctggtagtcataaagttgcagcagcactgccaattgctcacgacttccgataatagtggacacatcttgaagaggcgacataggccgaggaaacctagtcacttctatctgtggcacttcaccatgaagcttggctttgctggagaaaggtgcattctgtagcactaatgcaaagagagatgggatcaaggactgcaaggcagaaagatacatgtggagtttgtgttcatccagtccatgttctccttccctgagaagtttttcaatcttgttcagtagtgtaagtataagatgagactgtaaatttccaagttctgtagtccacgcagcgtaagctggtaaaaatacttgatgtgtagcactaactactctttctgagggatcacccaaggctgacagcaacaattcaaaaccctgatgatatttgtctggatcatcaatgtatcccataatgataccaaggcttttgataacagcttctcttaccaaatctgccttatcttccattaacatttgttgcaacattgaaagaaccaaggagctacggatttctttaggaaggtaaggtgccagtgctccacaggattctgccacaagcagtcgtctttctgggtatttgtgattaatctgttcccaacactgtggtaaaagttcagcttctacacgtgttggtccaacatgacgcgcaaatgccacacaacctgtcagtatcatttgcctttgctcatcatctggcctcttgatcaaattgaaaagtatgtggagaagctgatctcgctctttaggctcaggatgtagacatgctgtacacaatatgagggggatcaactcctctctctttgccaatagcacattgggaacaatgtgtggcaggcagcgtcccagcattaacataacgcttttttcactgtctgcaatacgagacacctcgtatcctaaacgactatctgctgacattcgacaaaaagagagtagtgcttgatggaatgcaggagacaatttcctattaggtttatcaaaatgaactgtctttttacttgatagagaagaaggtggcattccttctctttctctcctggggaatgaatttggggaattctctttaggaatagtggaatcagcttcatctgatattgaaagatggatgtctgtgttttttcccttgtctgaactatttacatctggatgctgtccactgtcctcagagtctttgtggggcaactgatccaaaggaggctgaacagagtcacaaactgctgggatggcaaagtgttcatttttgaggaagtccatttcacttttaagtcttctgatttgctccatcaatgaccatttctcactatttaacaaactaattttatcttctaatttctgtactaacatggagttctctgcaggctggggagtttcaagagttggaggaaggttgcttataattggtgtaagggcctctaattcatcttcttctactccactggccacatctacaagatcttttccagttacttgatgatttccaaaatcccggtagagttgcaataagtctggaggttttggaatgtttaatcctacatcatcccataattcaaaatcctgatcatcgttttcatctgaaaaggttattgatgtaagcttatagttattcttcaataaaaattcattgactaagaagtttagagctctcttttcaagaggtttgattggctcctgaatttcaggacttgatttgtaattttttcgttcctgtaaaggaacttcatgttctgcggcctttgtcaggttggctcggagggcctgaatggtctccttggctttccgtagttcaaactccaggactgccactttttcatctgtttccctgttaccatcatctgaatatcttgcaaagtctaaagaatcaagggtactaatgctcccagctcgattgagctgtcccccgcccgacgctgtactcggttcccgacctccagcgcccccaacgccggctgctccagggacccctggcgcccccatccccggcggggttccactttgcctctcgaagttgcctggattggagaagtagtcgcgcagccgaggcagctcccggccactctctaacagctcggtatgcagctccagggcggtcagcaagtattgatcgcgcaacagctgagcagcgatcgcatcaattgataatcgggccggggtctccccggtgccccccagggccactgcagccgccgacgcctccccagggagccctggccgcgcactgcttcctaaggccacgggatcctgtggcgacagcgagcccgcagagccaggatctaggccacttccggcgcccagccgaagtactgcccgccgttcctctgttgcagctacctcgtcatcgtcctcatccgaatcactgagaaatggattcacgccgccaccactgccactacctccaggcgccatcgccgccatcttatcctgtcaggagtgtgggcgcctccctgactggttccgacgggccgcagcccgaatcctctaggcctcaggggacacagcgcacctccacagccccggcctgaccacgtcctgcctcccgacttagagacaaggagtacgctccaaggcaggagatccggatgcagctgcacctgatgcctcagcctctgctgcaccagcagcccggctctgcaggcgtcttcctggtctccagtctcgcgagaact

SEQ ID NO: 14611 - RNA, 9286 nt, Homo sapiens
  source 1..9286: mol_type = other RNA
gctgggattacaggcatgagccaccgtgcccggccagtctctatttctttttaatgtactgaaaaaaatagtatcaaaactaagcacactgtaaagttacagtagaactttgaaatagatgtctactcatacaaaaggctaaatttattttgtagttttcttgtaagagaattaacatccaaccttgaaggttgaattttgttacctggctaatctggagtatttcatgaattatgaattagaattgctacttacaaagcttttttttttgtttttgagatggagtcttgctctgtggaccaggctggagtgcagtggtgcaatagcggcccactgcaatctccgcttcccaggttcaaacgattctcctgtctcagcctcccgagtagcagggattacaggcccacgtcaccacgcctggctaatttttgtatttttagaggcggggtttcaccacgttggccaggctggtcttgaactactgacctcaagtgattcgtcaccttggcctcccaaagtgctgagattacaggcgtgagccacagcgcacagtccaaagctctttaagtgtaacattgaagagctaaagtgtaactttctttaatgaactgaaaaaattagtacaatctttacacaaagaatagttaagaaaatataaccagcacagaatgttagctgtagttagctactgcagttcaaagatcagcagggtagtaactacagaaagttacatccttggagttcaaataatggtccaaaataggttgtcttgaaaaatgggatgatgaaaagacaattcaatacatcctgatctcacctctctaaattttaagagagactatttgagccaactttttaaaaacaagaatgtgatagcaccttgacttgagacccccattagaattatagtgtatagtagtgacatatcctatagtagtgacatatcctaaaagctatggataatgaggatggcatgacttaaattactcacaatttcgttcaggttgaaaatcaatttgatgtttagcaaaataatctctctaaaggggtgaataatgcaaaccaatgaaggtcatagacacctatgtatagagatagatactgccatcattcaagcactgttcttggaagaattcagctaaattagtaattatggcacttctggatttctgaaaaaatttaatctctggattactctggaaacacaggtataatttcaaattagcttttcattactttgcaaacttagtttttcattaagttgaacacttaaaaacttgtaccgtaagtttacttctgtttaaaaggaatgagtatgggagttttatgccctattttggactcagtccaaatctcagtctcaatgattagtgtctgtcttgtctgtaaagacaagacatattttactaaaaacaaacaaacaaacaaaaaacaaaaccacaatgtgaaatcttaatgatattaaaatatttaagaaaagagactctcacttgaaatacactgtgaatcttgcctactattgcctttaaaaaaacattagcacttaaataaatatattcattaattaagaaaaatgttcacaataaaaatacattctacccattcacctgataacaaacatacacatattctactatagtttgaagcaaatcagagtttaaacatttttcttccaggtacctctgaaatgtattagttttatagcaacatggtccccttttagtaaaaataaaccaaaataggtaaatttatataaattatatttacaaaatattagtatattctcatgaatataggcttttctcatttttttgcttaatagaaagtatagtgtttcaaaacgaaagtaaaatgcatagcccaaaccaaatcaaaaacatatgcaaaaacattttatttataatagatcaacatttttgacatgaaaggtagccactttcaatttctcaggaatgcctagaacccaacagttttcagaaagactacttagttcacaattatttcactgtaggtaaatgaaataatttcagaatgaactttttaaatggctttgcctatggcaaattgttttataaacttgaatgtatggtaagctagctttcccaggaaatgaatgtaatccaactatgttccaaatgtattaaaccagtttatacaacaaatatgagaatcacttatgtgcatcaactgtgctaaaacaagaattctttttatcaaaatattcatttttcaaaaaggcctcacattaacccctcaaaccaagcacccccttcctatgtccagcactcttttctacttcgagttgcatgactgtagagacaactgtcaaattccagtggaactgtacactgacttaagactctatgtaatatacatcaaacacaggaggtcactgactttaagggacgaggtgataactaactagttataattcagccaatgtcttttttagtttagagggaaaaaagtagcccccaagtgtccttaacttttcagtacttctctgtaacacacagaatgaaaaggtactctctaaaattaaaatcattagaaaatatcttaaataaagtgttttacataaataagtgttaaatttcagattcaaactatattttcttctgtatctcaatttgggaaaaatctcacaattattaactcttctcagttacatttatttttgagcatttaaatctactatacaccagtttgtaaaattcaccttggttacctctccccatgcctatgtgctgtctttcctcaggtaagtccattatatgcatctaagtgctggggaggtttaaatagcacttaaagaatattcatgagagttctgaaatgaaggtttcgtctttagctattgactgtaggatttgtaattcaaatcatcacagcatcctaaagaaatactgtgtgaatggaatgcacacaattcctacagaacacacaaactgatgtccaaaaggcacagagtaatgctggtggctctttctagtcagttaagaaacaataaaaagtctgcattattctttcataatttaaatacttaagtaatctccactttattattttataacaatgacttcaaatttacattattttaagtaccattgtaatagcttagtgtataatacagatatttgcgaatatcccatccaaaaattaaaaaaaacttcttcactatatatatatttatataaaaattattctgaaagacaagaacatagacaagggacttggtacagaccatcaactcaattttctatcaccacagttgtaactccaaaatcaacaaatatacagcagtaattaaaagcagtgcaaatatctttggaggttaggataaaattataatgcaagaacataaaactgaggaaacaaaaaaggcaagtacttcaagtacaaggaaccagtcggcttgaggtccatcttagtgtttactgggggcttctttcctgcttctacttctttctctgaaatacattggccaacatggcacctgatgttgtcaactggcccattttgttcaaaaacttggtctttgtatcttcactcactaagcttgcagcaattgacattgagccttgaggctcttggacggtcttgttttcaactttttgttcacattcttttatcatggaacttaaaataacctcatgctctggagagagatgttccatgtcagtccgtaaacatctgagaccaggtaaaaagtgattaaccattaaatcctctgaaatgaaacaacaggaaagtgcactgtaggcttcaaaaagatgcgtagcaatgtccagtcttttagaatccacaatctgtaagttgttcaccaaggctaacttatgcaaatgtggtataacaactgaaaacagaaaaaaaagggttaaatttttacccaaaacatgcatacaaaaccctgacacactttaacaataatttatcactttaatttatgaaatttcattttaattctgaatgacttcaaaagattacccatatcttatacttgctttttcttaactagggaagaaagtagtttttcaaaataaaaagtgatctggcatttgggggaaacaaattttagtactgtcactattacctaattatgaggatgtatatagattatttggcctcactgtaattcagtttcccagtttgaaaaatgaagcccaaataattataaacaacatacctcttgtattatttatacttgcagttaagtttctccataaaaataaaatattaccattgctatgaaatcaaaagagtatattctttttcaacaacctattatttcactccttcagaatactattatcagctttagtttctcaaattcttagcaaagaccaatgtcaaacagcactggcggctgagttttcaagttattcaatgagtttaataccctcaaagagtaacataaaatttcaacctactgctaaataaaagcaatggtccaagaaacaaaaaccaattcagtagcaatgagcacctctagagcctaagattgtgttttctgggtaccatttcccactaaaaccagggctctttgaagaaatggcttcagggtcagtgattgttaaattgttaatcacaagaccaatcacacaacccctttctagtctctgcttggttgaggatcacaaaacgccacccataagcatcaactgctgaccaactgtagtgacccctttcttgtttgcactgagtttgtgtatataaagtcataatcttctactggaaaaactcctgcatcctaaataagctggggcaataatcacaactttcatgcttagcttagtaaaaccccacaaaaactcagaataacaatgatcatttttaggggaccttttgacttgtcaaaattaataacagtatatttatgaggagctctagaacaaattaggaaacaaaaactccaaacattcagttgaaagcttcattaattggcacgctgaggcctcaacaaaatagtgactctaagtctctctcaaagactcactagttcatttctgcccaaacattcagaaacttatcattctttcactttatctattcatatatggttcctttatttcatcttctcctgagtctctgacctttttacaaggtttttctcagaaatgcaacaatcacactgcataatatccccttaaaattgcttgactagaagaaatctatagaagttcatttaaactgtagtctcaaggaagttaaagcctctaattaaggatcttcctaattctcaggaagacagacagaactttactatagaattcagatttcactacacacatattgtcctggggtaccacatatgtattaattaattcacttaacagttaacccctcagatgtagacagatggttaaaagcagtaggagatgaaggaccaggagatgatttaataataacccagatggatatcattctttcttttttattaagagatggggtcttgctctgttgcttgggctggaatgcaatgactattcacaggtgcaatcatagtgcaccacagcctcaaacacttggactcaagtgatcttcctgccttggcctcccgagttgatggactacagatacgtgccaccatgcctagctaatttttaaacatcttttgtagggacttatcttgctgtgttgctcaggctggtgttgaactcctggcctcaagtgatcctcccacctcagcttctgagtaggtgggactatagacacgtggcaccatgcctgacttagacaggctaattctaaaactgacactcatctcggaacctgggttctgcgttagggccaactctaccaaatgtttttatgatctctgtatgcaaagaatgttggtcttgatactgaggatcttccaggaaagaagccaactgcattttcactctttccagcaactctctttgaattactgtttccataatagtgccaaaggctggaattgtggcaatcctgacagagatttcagggtcactggagagagtaatgagagcaggaacaaccctctgagctaccagagtttcattcacccccttcaccaacagctcaaacattctagcagcagtacacctcacgagtgctgaagtatggacaacaccataccacaaaacagttaatagtaactcatggtaggctgggtttgcacccaattccacaaaagaagccttcaggctatcaagaggagcatgagataatgaaagcagcgtcattacatcttctaagaatccaactaacagttttcggtcttcttcctgaatataacacgtaaggactcctgttgcataaatggggactgtagctttagtgaggaccccatttcctgctgaggaatcaatgttttcttcagatagtcttaaaatctcctggaactgaggttttaccttagtgtttgtaaaaattttgccaaatgtccggcaaaggcgccagaaaaatctggagaattcatggacacaggcagttgaagtaacattaattttgccaactatttctataagttgtggcaacaattgattgacaacccacagtaaactctcccagcctgttgtaccctcttgttctagctggtagtcataaagttgcagcagcactgccaattgctcacgacttccgataatagtggacacatcttgaagaggcgacataggccgaggaaacctagtcacttctatctgtggcacttcaccatgaagcttggctttgctggagaaaggtgcattctgtagcactaatgcaaagagagatgggatcaaggactgcaaggcagaaagatacatgtggagtttgtgttcatccagtccatgttctccttccctgagaagtttttcaatcttgttcagtagtgtaagtataagatgagactgtaaatttccaagttctgtagtccacgcagcgtaagctggtaaaaatacttgatgtgtagcactaactactctttctgagggatcacccaaggctgacagcaacaattcaaaaccctgatgatatttgtctggatcatcaatgtatcccataatgataccaaggcttttgataacagcttctcttaccaaatctgccttatcttccattaacatttgttgcaacattgaaagaaccaaggagctacggatttctttaggaaggtaaggtgccagtgctccacaggattctgccacaagcagtcgtctttctgggtatttgtgattaatctgttcccaacactgtggtaaaagttcagcttctacacgtgttggtccaacatgacgcgcaaatgccacacaacctgtcagtatcatttgcctttgctcatcatctggcctcttgatcaaattgaaaagtatgtggagaagctgatctcgctctttaggctcaggatgtagacatgctgtacacaatatgagggggatcaactcctgacagaggtgtaaaaccattctctctctctttgccaatagcacattgggaacaatgtgtggcaggcagcgtcccagcattaacataacgcttttttcactgtctgcaatacgagacacctcgtatcctaaacgactatctgctgacattcgacaaaaagagagtagtgcttgatggaatgcaggagacaatttcctattaggtttatcaaaatgaactgtctttttacttgatagagaagaaggtggcattccttctctttctctcctggggaatgaatttggggaattctctttaggaatagtggaatcagcttcatctgatattgaaagatggatgtctgtgttttttcccttgtctgaactatttacatctggatgctgtccactgtcctcagagtctttgtggggcaactgatccaaaggaggctgaacagagtcacaaactgctgggatggcaaagtgttcatttttgaggaagtccatttcacttttaagtcttctgatttgctccatcaatgaccatttctcactatttaacaaactaattttatcttctaatttctgtactaacatggagttctctgcaggctggggagtttcaagagttggaggaaggttgcttataattggtgtaagggcctctaattcatcttcttctactccactggccacatctacaagatcttttccagttacttgatgatttccaaaatcccggtagagttgcaataagtctggaggttttggaatgtttaatcctacatcatcccataattcaaaatcctgatcatcgttttcatctgaaaaggttattgatgtaagcttatagttattcttcaataaaaattcattgactaagaagtttagagctctcttttcaagaggtttgattggctcctgaatttcaggacttgatttgtaattttttcgttcctgtaaaggaacttcatgttctgcggcctttgtcaggttggctcggagggcctgaatggtctccttggctttccgtagttcaaactccaggactgccactttttcatctgtttccctgttaccatcatctgaatatcttgcaaagtctaaagaatcaagggtactaatgctcccagctcgattgagctgtcccccgcccgacgctgtactcggttcccgacctccagcgcccccaacgccggctgctccagggacccctggcgcccccatccccggcggggttccactttgcctctcgaagttgcctggattggagaagtagtcgcgcagccgaggcagctcccggccactctctaacagctcggtatgcagctccagggcggtcagcaagtattgatcgcgcaacagctgagcagcgatcgcatcaattgataatcgggccggggtctccccggtgccccccagggccactgcagccgccgacgcctccccagggagccctggccgcgcactgcttcctaaggccacgggatcctgtggcgacagcgagcccgcagagccaggatctaggccacttccggcgcccagccgaagtactgcccgccgttcctctgttgcagctacctcgtcatcgtcctcatccgaatcactgagaaatggattcacgccgccaccactgccactacctccaggcgccatcgccgccatcttatcctgtcaggagtgtgggcgcctccctgactggttccgacgggccgcagcccgaatcctctaggcctcaggggacacagcgcacctccacagccccggcctgaccacgtcctgcctcccgacttagagacaaggagtacgctccaaggcaggagatccggatgcagctgcacctgatgcctcagcctctgctgcaccagcagcccggctctgcaggcgtcttcctggtctccagtctcgcgagaact

SEQ ID NO: 14612 - RNA, 7289 nt, Homo sapiens
  source 1..7289: mol_type = other RNA
gctgggattacaggcatgagccaccgtgcccggccagtctctatttctttttaatgtactgaaaaaaatagtatcaaaactaagcacactgtaaagttacagtagaactttgaaatagatgtctactcatacaaaaggctaaatttattttgtagttttcttgtaagagaattaacatccaaccttgaaggttgaattttgttacctggctaatctggagtatttcatgaattatgaattagaattgctacttacaaagcttttttttttgtttttgagatggagtcttgctctgtggaccaggctggagtgcagtggtgcaatagcggcccactgcaatctccgcttcccaggttcaaacgattctcctgtctcagcctcccgagtagcagggattacaggcccacgtcaccacgcctggctaatttttgtatttttagaggcggggtttcaccacgttggccaggctggtcttgaactactgacctcaagtgattcgtcaccttggcctcccaaagtgctgagattacaggcgtgagccacagcgcacagtccaaagctctttaagtgtaacattgaagagctaaagtgtaactttctttaatgaactgaaaaaattagtacaatctttacacaaagaatagttaagaaaatataaccagcacagaatgttagctgtagttagctactgcagttcaaagatcagcagggtagtaactacagaaagttacatccttggagttcaaataatggtccaaaataggttgtcttgaaaaatgggatgatgaaaagacaattcaatacatcctgatctcacctctctaaattttaagagagactatttgagccaactttttaaaaacaagaatgtgatagcaccttgacttgagacccccattagaattatagtgtatagtagtgacatatcctatagtagtgacatatcctaaaagctatggataatgaggatggcatgacttaaattactcacaatttcgttcaggttgaaaatcaatttgatgtttagcaaaataatctctctaaaggggtgaataatgcaaaccaatgaaggtcatagacacctatgtatagagatagatactgccatcattcaagcactgttcttggaagaattcagctaaattagtaattatggcacttctggatttctgaaaaaatttaatctctggattactctggaaacacaggtataatttcaaattagcttttcattactttgcaaacttagtttttcattaagttgaacacttaaaaacttgtaccgtaagtttacttctgtttaaaaggaatgagtatgggagttttatgccctattttggactcagtccaaatctcagtctcaatgattagtgtctgtcttgtctgtaaagacaagacatattttactaaaaacaaacaaacaaacaaaaaacaaaaccacaatgtgaaatcttaatgatattaaaatatttaagaaaagagactctcacttgaaatacactgtgaatcttgcctactattgcctttaaaaaaacattagcacttaaataaatatattcattaattaagaaaaatgttcacaataaaaatacattctacccattcacctgataacaaacatacacatattctactatagtttgaagcaaatcagagtttaaacatttttcttccaggtacctctgaaatgtattagttttatagcaacatggtccccttttagtaaaaataaaccaaaataggtaaatttatataaattatatttacaaaatattagtatattctcatgaatataggcttttctcatttttttgcttaatagaaagtatagtgtttcaaaacgaaagtaaaatgcatagcccaaaccaaatcaaaaacatatgcaaaaacattttatttataatagatcaacatttttgacatgaaaggtagccactttcaatttctcaggaatgcctagaacccaacagttttcagaaagactacttagttcacaattatttcactgtaggtaaatgaaataatttcagaatgaactttttaaatggctttgcctatggcaaattgttttataaacttgaatgtatggtaagctagctttcccaggaaatgaatgtaatccaactatgttccaaatgtattaaaccagtttatacaacaaatatgagaatcacttatgtgcatcaactgtgctaaaacaagaattctttttatcaaaatattcatttttcaaaaaggcctcacattaacccctcaaaccaagcacccccttcctatgtccagcactcttttctacttcgagttgcatgactgtagagacaactgtcaaattccagtggaactgtacactgacttaagactctatgtaatatacatcaaacacaggaggtcactgactttaagggacgaggtgataactaactagttataattcagccaatgtcttttttagtttagagggaaaaaagtagcccccaagtgtccttaacttttcagtacttctctgtaacacacagaatgaaaaggtactctctaaaattaaaatcattagaaaatatcttaaataaagtgttttacataaataagtgttaaatttcagattcaaactatattttcttctgtatctcaatttgggaaaaatctcacaattattaactcttctcagttacatttatttttgagcatttaaatctactatacaccagtttgtaaaattcaccttggttacctctccccatgcctatgtgctgtctttcctcaggtaagtccattatatgcatctaagtgctggggaggtttaaatagcacttaaagaatattcatgagagttctgaaatgaaggtttcgtctttagctattgactgtaggatttgtaattcaaatcatcacagcatcctaaagaaatactgtgtgaatggaatgcacacaattcctacagaacacacaaactgatgtccaaaaggcacagagtaatgctggtggctctttctagtcagttaagaaacaataaaaagtctgcattattctttcataatttaaatacttaagtaatctccactttattattttataacaatgacttcaaatttacattattttaagtaccattgtaatagcttagtgtataatacagatatttgcgaatatcccatccaaaaattaaaaaaaacttcttcactatatatatatttatataaaaattattctgaaagacaagaacatagacaagggacttggtacagaccatcaactcaattttctatcaccacagttgtaactccaaaatcaacaaatatacagcagtaattaaaagcagtgcaaatatctttggaggttaggataaaattataatgcaagaacataaaactgaggaaacaaaaaaggcaagtacttcaagtacaaggaaccagtcggcttgaggtccatcttagtgtttactgggggcttctttcctgcttctacttctttctctgaaatacattggccaacatggcacctgatgttgtcaactggcccattttgttcaaaaacttggtctttgtatcttcactcactaagcttgcagcaattgacattgagctcatgctctggagagagatgttccatgtcagtccgtaaacatctgagaccaggtaaaaagtgattaaccattaaatcctctgaaatgaaacaacaggaaagtgcactgtaggcttcaaaaagatgcgtagcaatgtccagtcttttagaatccacaatctgtaagttgttcaccaaggctaacttatgcaaatgtggtataacaaactcatctcggaacctgggttctgcgttagggccaactctaccaaatgtttttatgatctctgtatgcaaagaatgttggtcttgatactgaggatcttccaggaaagaagccaactgcattttcactctttccagcaactctctttgaattactgtttccataatagtgccaaaggctggaattgtggcaatcctgacagagatttcagggtcactggagagagtaatgagagcaggaacaaccctctgagctaccagagtttcattcacccccttcaccaacagctcaaacattctagcagcagtacacctcacgagtgctgaagtatggacaacaccataccacaaaacagttaatagtaactcatggtaggctgggtttgcacccaattccacaaaagaagccttcaggctatcaagaggagcatgagataatgaaagcagcgtcattacatcttctaagaatccaactaacagttttcggtcttcttcctgaatataacacgtaaggactcctgttgcataaatggggactgtagctttagtgaggaccccatttcctgctgaggaatcaatgttttcttcagatagtcttaaaatctcctggaactgaggttttaccttagtgtttgtaaaaattttgccaaatgtccggcaaaggcgccagaaaaatctggagaattcatggacacaggcagttgaagtaacattaattttgccaactatttctataagttgtggcaacaattgattgacaacccacagtaaactctcccagcctgttgtaccctcttgttctagctggtagtcataaagttgcagcagcactgccaattgctcacgacttccgataatagtggacacatcttgaagaggcgacataggccgaggaaacctagtcacttctatctgtggcacttcaccatgaagcttggctttgctggagaaaggtgcattctgtagcactaatgcaaagagagatgggatcaaggactgcaaggcagaaagatacatgtggagtttgtgttcatccagtccatgttctccttccctgagaagtttttcaatcttgttcagtagtgtaagtataagatgagactgtaaatttccaagttctgtagtccacgcagcgtaagctggtaaaaatacttgatgtgtagcactaactactctttctgagggatcacccaaggctgacagcaacaattcaaaaccctgatgatatttgtctggatcatcaatgtatcccataatgataccaaggcttttgataacagcttctcttaccaaatctgccttatcttccattaacatttgttgcaacattgaaagaaccaaggagctacggatttctttaggaaggtaaggtgccagtgctccacaggattctgccacaagcagtcgtctttctgggtatttgtgattaatctgttcccaacactgtggtaaaagttcagcttctacacgtgttggtccaacatgacgcgcaaatgccacacaacctgtcagtatcatttgcctttgctcatcatctggcctcttgatcaaattgaaaagtatgtggagaagctgatctcgctctttaggctcaggatgtagacatgctgtacacaatatgagggggatcaactcctctctctttgccaatagcacattgggaacaatgtgtggcaggcagcgtcccagcattaacataacgcttttttcactgtctgcaatacgagacacctcgtatcctaaacgactatctgctgacattcgacaaaaagagagtagtgcttgatggaatgcaggagacaatttcctattaggtttatcaaaatgaactgtctttttacttgatagagaagaaggtggcattccttctctttctctcctggggaatgaatttggggaattctctttaggaatagtggaatcagcttcatctgatattgaaagatggatgtctgtgttttttcccttgtctgaactatttacatctggatgctgtccactgtcctcagagtctttgtggggcaactgatccaaaggaggctgaacagagtcacaaactgctgggatggcaaagtgttcatttttgaggaagtccatttcacttttaagtcttctgatttgctccatcaatgaccatttctcactatttaacaaactaattttatcttctaatttctgtactaacatggagttctctgcaggctggggagtttcaagagttggaggaaggttgcttataattggtgtaagggcctctaattcatcttcttctactccactggccacatctacaagatcttttccagttacttgatgatttccaaaatcccggtagagttgcaataagtctggaggttttggaatgtttaatcctacatcatcccataattcaaaatcctgatcatcgttttcatctgaaaaggttattgatgtaagcttatagttattcttcaataaaaattcattgactaagaagtttagagctctcttttcaagaggtttgattggctcctgaatttcaggacttgatttgtaattttttcgttcctgtaaaggaacttcatgttctgcggcctttgtcaggttggctcggagggcctgaatggtctccttggctttccgtagttcaaactccaggactgccactttttcatctgtttccctgttaccatcatctgaatatcttgcaaagtctaaagaatcaagggtactaatgctcccagctcgattgagctgtcccccgcccgacgctgtactcggttcccgacctccagcgcccccaacgccggctgctccagggacccctggcgcccccatccccggcggggttccactttgcctctcgaagttgcctggattggagaagtagtcgcgcagccgaggcagctcccggccactctctaacagctcggtatgcagctccagggcggtcagcaagtattgatcgcgcaacagctgagcagcgatcgcatcaattgataatcgggccggggtctccccggtgccccccagggccactgcagccgccgacgcctccccagggagccctggccgcgcactgcttcctaaggccacgggatcctgtggcgacagcgagcccgcagagccaggatctaggccacttccggcgcccagccgaagtactgcccgccgttcctctgttgcagctacctcgtcatcgtcctcatccgaatcactgagaaatggattcacgccgccaccactgccactacctccaggcgccatcgccgccatcttatcctgtcaggagtgtgggcgcctccctgactggttccgacgggccgcagcccgaatcctctaggcctcaggggacacagcgcacctccacagccccggcctgaccacgtcctgcctcccgacttagagacaaggagtacgctccaaggcaggagatccggatgcagctgcacctgatgcctcagcctctgctgcaccagcagcccggctctgcaggcgtcttcctggtctccagtctcgcgagaact

SEQ ID NO: 14613 - RNA, 6039 nt, Homo sapiens
  source 1..6039: mol_type = other RNA
gctgggattacaggcatgagccaccgtgcccggccagttaaacacaccttatcctacactgcttttagtgattttccatacttattaattttaggactaaaaaaaattttaaaaaccaatatgagtggaaatttcaatatatcttggcatgacttggcaaaataactttaatgaattgagttctgagctcataaataattgaagcaccaaacttctttcatccattaggcagtacttagccgtacagaaaacagtaactatgcttattttgattgcattactgaaaatataatattgaaacatttgttcctaaattttaaaaagtcttaagatctgatacccatagaaggaacatcatgtgctaaggatgtgatttgcttcactaagagaccatatggttacctgcttataagcaccgtgagtaacaggagtaacgaaatgaggctgcaaggctcaaagggaattcaggaagttgtctaattccatggttttcaacattgtgcacctgagttctgcagaggtgtctggggaaaggtttgtgggggactttaaccacagcagctctgattttagagtttatcccttaaatttgagcatctttaggaaacaattcatttgaagagtttctcgggttaaattattttaaactgcaggtctagtccattttgtttctcccagacactaggcatgactgcagtggtgctttctttttgtaatgcttcatcctatacccagacactcttgagggtaatggagttagaagggcattcagaagctgataaatggcattcctgcaagagcaaactttggtctaaccaagtcttgatattaaaaaaaaaatccttggcataaataaagcttatttaaacagattatacccctatgtaacatttgcccacatgtaaaaaccaaagaattcaattttctcaatcatcaatagacagtttcactctagaaaataactggtctctaacgtcttagatatatatgctataactggagtcattatttacaacttacaaacatgtcttaaatgttcttctatgatgttaaaatgatacaacagattctttgtctagtttggtgaacttgatcattttgtggggatagtttgatgctcgttataaacaattatgagaaagcattatttctgaaaaggcaattacaagtgctggtggcactgtgttcagtgaatgttggatattcatgctgatgtatgtaaagtttgcatgcagaagataatagcataaaaggacatttagatcatagactaaagtgcattagagtacacacatgcaagcactacttcatttataggaaaaaagttcaaatcagccatttttcctactggctccaacaactaaaaaatcaggttttaatttcaaaaggtgtcagtattaattgggtaagactagagaatgacaagcgtttccttcctcattcagatacactttaattgttaagaatcctgatttaggccgggcgtgctggctcacgcctgtaatcccagcactttgggaggctgaggcgggcagatcacgaggtcaggagttcgagaccagcctggccaacatagcgaaaccctgtctctactaaaaatacaaaaattagccaggcatggtggcacatgcctgtagtcccggctactcaggaggctgaggcaggagaatcgcttgaacccgggaggcagaggttgtggtgagcgagatcacgccactgcactccagcttggacaacagagcgagagtccatctcaaaaaaaccagaatcctgatttaggaacagccatgttgggagaacagagaactcaatgcacatcatccagtcttgaagcaactgcaaatgtgccatcaggggaatcttgaaaaagtctcaattaagtaccatgaaacaagtggttattcatctatttttaaattttttaaaagaaagtaaccaatttagcctagaaattggtatcaaggacaataattaatgaaagaacaagagaaaatagtaacataaaaaggataattttgaggtatgtcatggcatttaaaaatacagtaaaattggctgggcgcagtggctcacgcctgtaatcccagcactttgggaggccgaggggggcggatcacgagatcaggagattgagaccatcctggctaacacggtgaaaccccatctctattaaaaatacaaaaaattagctgggagtggtggtgggcgcctgtaagtcccagctactcgggaggctgaggcaggagaatggcgagaacccgggaggtggagcttgcagtgagctgagattgcaccactgcactccagcctgggcgacagagcgagactccgtctcgaaaaaaaaacaaaaacaaaaaagaaaacagtaaaatagatggagcctctccatatacagtgaaattctatcaagcttcactgtgataacttgcagaagagacctttatgaagctcagttctttacttcggatatttagattttacctttagaactgaaacaatgcttctctaatttagctgtaattttggaatgtttcataatttatgcaggggagaagttttttttttttttttttttgagacggagtttcgctcttgttgcccaggctggagtgcaatggcgcaacctcagcccaccgcagcctctgcctcctgggttcaagctatcctcctgcctcagccttctgagtagctgggattacaggcatgcaccaccacgcccggctaattttgtatttttagtagagacggggtttctccatgttggtcaggctggtctcaaactcccgacctcggtgatccacctgcctcagcctcccaaagtgctgggattacaggcgtgagccactgggcccagcccaaaggggagaagtttaaactttgtatactaggagaaaagtttgttttgaaaatattatataaacaagagaagcaaaaatgttcaacatatttaagtgaataatttgttcaaatagttttatactttaaatttacatataaataacgtgacataaaaacataccaataggtactgtagggacattacttagcattatttgaaaatctctagatcaagatattgtatgttgttgaaaatgattcaattcctcctttcatactttctaattctgattggcttatttttataatgactgccaactggtgaggtttgacttctattctttgccatttcaggagacatacagggagagaaggctgaaagaggattgtttaaaatcagatcctgtccaatcatcagttttctctctcagactttctgaccttaatttcctcatttgtaaatcggagatagtatccacctcactgagaaaatacatgagagagtactttataaataatatagcactacataaacgttagaaatcactcacatatggtaagaacctcctagtttgttttccttttttttttgagacggagtttcgctcttgttgcccaggctggagtgcaatggtgtgatctcggctcactgcaacttctgccttccaggttcaatcgattctcctgcctcagcctcccgagtagctgggattataggcacccgccaccatgcccggctaattttgtattttttagtagagacgaggtttcaccatgttggccaggctggtttcaaactcctgaccttgtgatccgcctgcctcggcctcccaaagtattgggattataggcatgagccacagcgcccagcctgcttttctttagagagatggacaaccatattgacagattgtcttcacaaactaccttgacttttaggcaacattagtttcctgctttaagaaaatatctgtatataatctttggccagcctctacttttttttttttttaacaatactgagagtaatttttaagctaatgataaaaatttcaaatatgaatgatttcaaacactttagtcttcttccataatccttaaacgttcaggatatcagagtaatgacaggttgtttcagatctcaaattaatagaaagactaatttgtttagtaaggtgggttgccagatccttaaatgtgctcttaactggttccctgtgaaattaaacattggtagttatgtgtttttgaaacaccttgaaattgtcttacataaagtttggttgtggtgaatttatttaaagtattttctttgaaaaaagtttgctaagtagatcctccaatattaaaagaaaaaggtatctctggaataaagtaagaggattgtaatgaaagtaagaggataattgttcatccatcaagccaactcaagctagttctttctttccagtgcagcaacacattttagggcaacaaagttcagaatggatacaatggcctgttcagaaagcatgcaagttatatcagatcatttctttaaagtcagtgtgataaatttgttaactagactccgaccatagaaagagagagatacaggaagtcaatgtaaattgcagacatgccagctctgttggttcacattacagctacctaatgttgggcttaatttctttttcttcttcttcttcactatcatcaacctgttggatgaccagatcagcagacccatcttctacaatctccacataggatctattctcatcttcactcaagtgccatctggaatccttatctccatctgatggggacataagatgttgttcagcttccaagtcaatggggaggctgtctatgccaaattctgcaagacactcattacacagtctgtagcgcctggttccctcctgtaccacttgccctgttagatctgtcacatgacgtttacattttctgcagatgagtttacatgcctggtgaattgttcgaaaatggctacttagatggtctagcctgctaaatctttttccacaagcttgacatggatagggcctttctcctgtatgacaacgaaggtggcgctttaggtctgccttccgcttcaccacatgtgtgcagtacgggcacttgaatcgcatccgaggcagatcatctggaaagcttttggatgtgacatcagatccttgaccgtactgatagccaacaggagtagagtccatttcagcatcaatctgtgcttgttcttcagactgggaaacatggctggaagaatcagatgttcgtacttctcgtttgcttgacttataatgagtaacttcagaaggctgtgacaatctcaaatgtttggtctttttaatggactctttccttggttcatgcttggccaagggttgttgagtattcttctgggaggctggatgataattatacttattccaagattttccacttattatacctgttccttgctctgggcttaggtgagaacgtggagaactgcttccttcttgccagccaccactataaaaagaggaacgttctacaccattagaattggcatctttatctgagagactgaaatagcgatctttttctttctcactaatgtctaaggaagatttaataaaagtcttacatacacttatgacatcagtcatctgaaggaagctagcagccgacatcacttctatgacattctgaccagtaagagacagtttgccagaatatacgaagtccaagataactgtaaaagtgtcaggggagaaagcctgaaatgtagctgtggttggctgactcgtctcctttgaattctgagaaagaagcattttaaagtagccgctactagcgaataatacatttcgatgtgctttgaagaccttcccttcaactagaatactgcagtcacaaaatacatcttgcctgcgctgctcgttcagttgctgcaggaggtgagactgatgagaggagatctccattctggaaatttatgaatgctgctcttgaatggagtaaaaaagggaagattctaagtcaaacagtctgtgtttggaggattgtccgcgggccgcggcgcaccggccggtcgcgcgcgcgggccgagggaagattcctggttctcggctggggaaggaccccctttcgaggccgttcctttgcgccctaaaacaagtagccccaacgtgagagaaacaaaaggtatttgct

SEQ ID NO: 14614 - RNA, 5858 nt, Homo sapiens
  source 1..5858: mol_type = other RNA
gctgggattacaggcatgagccaccgtgcccggccagttaaacacaccttatcctacactgcttttagtgattttccatacttattaattttaggactaaaaaaaattttaaaaaccaatatgagtggaaatttcaatatatcttggcatgacttggcaaaataactttaatgaattgagttctgagctcataaataattgaagcaccaaacttctttcatccattaggcagtacttagccgtacagaaaacagtaactatgcttattttgattgcattactgaaaatataatattgaaacatttgttcctaaattttaaaaagtcttaagatctgatacccatagaaggaacatcatgtgctaaggatgtgatttgcttcactaagagaccatatggttacctgcttataagcaccgtgagtaacaggagtaacgaaatgaggctgcaaggctcaaagggaattcaggaagttgtctaattccatggttttcaacattgtgcacctgagttctgcagaggtgtctggggaaaggtttgtgggggactttaaccacagcagctctgattttagagtttatcccttaaatttgagcatctttaggaaacaattcatttgaagagtttctcgggttaaattattttaaactgcaggtctagtccattttgtttctcccagacactaggcatgactgcagtggtgctttctttttgtaatgcttcatcctatacccagacactcttgagggtaatggagttagaagggcattcagaagctgataaatggcattcctgcaagagcaaactttggtctaaccaagtcttgatattaaaaaaaaaatccttggcataaataaagcttatttaaacagattatacccctatgtaacatttgcccacatgtaaaaaccaaagaattcaattttctcaatcatcaatagacagtttcactctagaaaataactggtctctaacgtcttagatatatatgctataactggagtcattatttacaacttacaaacatgtcttaaatgttcttctatgatgttaaaatgatacaacagattctttgtctagtttggtgaacttgatcattttgtggggatagtttgatgctcgttataaacaattatgagaaagcattatttctgaaaaggcaattacaagtgctggtggcactgtgttcagtgaatgttggatattcatgctgatgtatgtaaagtttgcatgcagaagataatagcataaaaggacatttagatcatagactaaagtgcattagagtacacacatgcaagcactacttcatttataggaaaaaagttcaaatcagccatttttcctactggctccaacaactaaaaaatcaggttttaatttcaaaaggtgtcagtattaattgggtaagactagagaatgacaagcgtttccttcctcattcagatacactttaattgttaagaatcctgatttaggccgggcgtgctggctcacgcctgtaatcccagcactttgggaggctgaggcgggcagatcacgaggtcaggagttcgagaccagcctggccaacatagcgaaaccctgtctctactaaaaatacaaaaattagccaggcatggtggcacatgcctgtagtcccggctactcaggaggctgaggcaggagaatcgcttgaacccgggaggcagaggttgtggtgagcgagatcacgccactgcactccagcttggacaacagagcgagagtccatctcaaaaaaaccagaatcctgatttaggaacagccatgttgggagaacagagaactcaatgcacatcatccagtcttgaagcaactgcaaatgtgccatcaggggaatcttgaaaaagtctcaattaagtaccatgaaacaagtggttattcatctatttttaaattttttaaaagaaagtaaccaatttagcctagaaattggtatcaaggacaataattaatgaaagaacaagagaaaatagtaacataaaaaggataattttgaggtatgtcatggcatttaaaaatacagtaaaattggctgggcgcagtggctcacgcctgtaatcccagcactttgggaggccgaggggggcggatcacgagatcaggagattgagaccatcctggctaacacggtgaaaccccatctctattaaaaatacaaaaaattagctgggagtggtggtgggcgcctgtaagtcccagctactcgggaggctgaggcaggagaatggcgagaacccgggaggtggagcttgcagtgagctgagattgcaccactgcactccagcctgggcgacagagcgagactccgtctcgaaaaaaaaacaaaaacaaaaaagaaaacagtaaaatagatggagcctctccatatacagtgaaattctatcaagcttcactgtgataacttgcagaagagacctttatgaagctcagttctttacttcggatatttagattttacctttagaactgaaacaatgcttctctaatttagctgtaattttggaatgtttcataatttatgcaggggagaagttttttttttttttttttttgagacggagtttcgctcttgttgcccaggctggagtgcaatggcgcaacctcagcccaccgcagcctctgcctcctgggttcaagctatcctcctgcctcagccttctgagtagctgggattacaggcatgcaccaccacgcccggctaattttgtatttttagtagagacggggtttctccatgttggtcaggctggtctcaaactcccgacctcggtgatccacctgcctcagcctcccaaagtgctgggattacaggcgtgagccactgggcccagcccaaaggggagaagtttaaactttgtatactaggagaaaagtttgttttgaaaatattatataaacaagagaagcaaaaatgttcaacatatttaagtgaataatttgttcaaatagttttatactttaaatttacatataaataacgtgacataaaaacataccaataggtactgtagggacattacttagcattatttgaaaatctctagatcaagatattgtatgttgttgaaaatgattcaattcctcctttcatactttctaattctgattggcttatttttataatgactgccaactggtgaggtttgacttctattctttgccatttcaggagacatacagggagagaaggctgaaagaggattgtttaaaatcagatcctgtccaatcatcagttttctctctcagactttctgaccttaatttcctcatttgtaaatcggagatagtatccacctcactgagaaaatacatgagagagtactttataaataatatagcactacataaacgttagaaatcactcacatatggtaagaacctcctagtttgttttccttttttttttgagacggagtttcgctcttgttgcccaggctggagtgcaatggtgtgatctcggctcactgcaacttctgccttccaggttcaatcgattctcctgcctcagcctcccgagtagctgggattataggcacccgccaccatgcccggctaattttgtattttttagtagagacgaggtttcaccatgttggccaggctggtttcaaactcctgaccttgtgatccgcctgcctcggcctcccaaagtattgggattataggcatgagccacagcgcccagcctgcttttctttagagagatggacaaccatattgacagattgtcttcacaaactaccttgacttttaggcaacattagtttcctgctttaagaaaatatctgtatataatctttggccagcctctacttttttttttttttaacaatactgagagtaatttttaagctaatgataaaaatttcaaatatgaatgatttcaaacactttagtcttcttccataatccttaaacgttcaggatatcagagtaatgacaggttgtttcagatctcaaattaatagaaagactaatttgtttagtaaggtgggttgccagatccttaaatgtgctcttaactggttccctgtgaaattaaacattggtagttatgtgtttttgaaacaccttgaaattgtcttacataaagtttggttgtggtgaatttatttaaagtattttctttgaaaaaagtttgctaagtagatcctccaatattaaaagaaaaaggtatctctggaataaagtaagaggattgtaatgaaagtaagaggataattgttcatccatcaagccaactcaagctagttctttctttccagtgcagcaacacattttagggcaacaaagttcagaatggatacaatggcctgttcagaaagcatgcaagttatatcagatcatttctttaaagtcagtgtgataaatttgttaactagactccgaccatagaaagagagagatacaggaagtcaatgtaaattgcagacatgccagctctgttggttcacattacagctacctaatgttgggcttaatttctttttcttcttcttcttcactatcatcaacctgttggatgaccagatcagcagacccatcttctacaatctccacataggatctattctcatcttcactcaagtgccatctggaatccttatctccattgttcgaaaatggctacttagatggtctagcctgctaaatctttttccacaagcttgacatggatagggcctttctcctgtatgacaacgaaggtggcgctttaggtctgccttccgcttcaccacatgtgtgcagtacgggcacttgaatcgcatccgaggcagatcatctggaaagcttttggatgtgacatcagatccttgaccgtactgatagccaacaggagtagagtccatttcagcatcaatctgtgcttgttcttcagactgggaaacatggctggaagaatcagatgttcgtacttctcgtttgcttgacttataatgagtaacttcagaaggctgtgacaatctcaaatgtttggtctttttaatggactctttccttggttcatgcttggccaagggttgttgagtattcttctgggaggctggatgataattatacttattccaagattttccacttattatacctgttccttgctctgggcttaggtgagaacgtggagaactgcttccttcttgccagccaccactataaaaagaggaacgttctacaccattagaattggcatctttatctgagagactgaaatagcgatctttttctttctcactaatgtctaaggaagatttaataaaagtcttacatacacttatgacatcagtcatctgaaggaagctagcagccgacatcacttctatgacattctgaccagtaagagacagtttgccagaatatacgaagtccaagataactgtaaaagtgtcaggggagaaagcctgaaatgtagctgtggttggctgactcgtctcctttgaattctgagaaagaagcattttaaagtagccgctactagcgaataatacatttcgatgtgctttgaagaccttcccttcaactagaatactgcagtcacaaaatacatcttgcctgcgctgctcgttcagttgctgcaggaggtgagactgatgagaggagatctccattctggaaatttatgaatgctgctcttgaatggagtaaaaaagggaagattctaagtcaaacagtctgtgtttggaggattgtccgcgggccgcggcgcaccggccggtcgcgcgcgcgggccgagggaagattcctggttctcggctggggaaggaccccctttcgaggccgttcctttgcgccctaaaacaagtagccccaacgtgagagaaacaaaaggtatttgct

SEQ ID NO: 14615 - RNA, 5034 nt, Homo sapiens
  source 1..5034: mol_type = other RNA
gctgggattacaggcatgagccaccgtgcccggccagttaaacacaccttatcctacactgcttttagtgattttccatacttattaattttaggactaaaaaaaattttaaaaaccaatatgagtggaaatttcaatatatcttggcatgacttggcaaaataactttaatgaattgagttctgagctcataaataattgaagcaccaaacttctttcatccattaggcagtacttagccgtacagaaaacagtaactatgcttattttgattgcattactgaaaatataatattgaaacatttgttcctaaattttaaaaagtcttaagatctgatacccatagaaggaacatcatgtgctaaggatgtgatttgcttcactaagagaccatatggttacctgcttataagcaccgtgagtaacaggagtaacgaaatgaggctgcaaggctcaaagggaattcaggaagttgtctaattccatggttttcaacattgtgcacctgagttctgcagaggtgtctggggaaaggtttgtgggggactttaaccacagcagctctgattttagagtttatcccttaaatttgagcatctttaggaaacaattcatttgaagagtttctcgggttaaattattttaaactgcaggtctagtccattttgtttctcccagacactaggcatgactgcagtggtgctttctttttgtaatgcttcatcctatacccagacactcttgagggtaatggagttagaagggcattcagaagctgataaatggcattcctgcaagagcaaactttggtctaaccaagtcttgatattaaaaaaaaaatccttggcataaataaagcttatttaaacagattatacccctatgtaacatttgcccacatgtaaaaaccaaagaattcaattttctcaatcatcaatagacagtttcactctagaaaataactggtctctaacgtcttagatatatatgctataactggagtcattatttacaacttacaaacatgtcttaaatgttcttctatgatgttaaaatgatacaacagattctttgtctagtttggtgaacttgatcattttgtggggatagtttgatgctcgttataaacaattatgagaaagcattatttctgaaaaggcaattacaagtgctggtggcactgtgttcagtgaatgttggatattcatgctgatgtatgtaaagtttgcatgcagaagataatagcataaaaggacatttagatcatagactaaagtgcattagagtacacacatgcaagcactacttcatttataggaaaaaagttcaaatcagccatttttcctactggctccaacaactaaaaaatcaggttttaatttcaaaaggtgtcagtattaattgggtaagactagagaatgacaagcgtttccttcctcattcagatacactttaattgttaagaatcctgatttaggccgggcgtgctggctcacgcctgtaatcccagcactttgggaggctgaggcgggcagatcacgaggtcaggagttcgagaccagcctggccaacatagcgaaaccctgtctctactaaaaatacaaaaattagccaggcatggtggcacatgcctgtagtcccggctactcaggaggctgaggcaggagaatcgcttgaacccgggaggcagaggttgtggtgagcgagatcacgccactgcactccagcttggacaacagagcgagagtccatctcaaaaaaaccagaatcctgatttaggaacagccatgttgggagaacagagaactcaatgcacatcatccagtcttgaagcaactgcaaatgtgccatcaggggaatcttgaaaaagtctcaattaagtaccatgaaacaagtggttattcatctatttttaaattttttaaaagaaagtaaccaatttagcctagaaattggtatcaaggacaataattaatgaaagaacaagagaaaatagtaacataaaaaggataattttgaggtatgtcatggcatttaaaaatacagtaaaattggctgggcgcagtggctcacgcctgtaatcccagcactttgggaggccgaggggggcggatcacgagatcaggagattgagaccatcctggctaacacggtgaaaccccatctctattaaaaatacaaaaaattagctgggagtggtggtgggcgcctgtaagtcccagctactcgggaggctgaggcaggagaatggcgagaacccgggaggtggagcttgcagtgagctgagattgcaccactgcactccagcctgggcgacagagcgagactccgtctcgaaaaaaaaacaaaaacaaaaaagaaaacagtaaaatagatggagcctctccatatacagtgaaattctatcaagcttcactgtgataacttgcagaagagacctttatgaagctcagttctttacttcggatatttagattttacctttagaactgaaacaatgcttctctaatttagctgtaattttggaatgtttcataatttatgcaggggagaagttttttttttttttttttttgagacggagtttcgctcttgttgcccaggctggagtgcaatggcgcaacctcagcccaccgcagcctctgcctcctgggttcaagctatcctcctgcctcagccttctgagtagctgggattacaggcatgcaccaccacgcccggctaattttgtatttttagtagagacggggtttctccatgttggtcaggctggtctcaaactcccgacctcggtgatccacctgcctcagcctcccaaagtgctgggattacaggcgtgagccactgggcccagcccaaaggggagaagtttaaactttgtatactaggagaaaagtttgttttgaaaatattatataaacaagagaagcaaaaatgttcaacatatttaagtgaataatttgttcaaatagttttatactttaaatttacatataaataacgtgacataaaaacataccaataggtactgtagggacattacttagcattatttgaaaatctctagatcaagatattgtatgttgttgaaaatgattcaattcctcctttcatactttctaattctgattggcttatttttataatgactgccaactggtgaggtttgacttctattctttgccatttcaggagacatacagggagagaaggctgaaagaggattgtttaaaatcagatcctgtccaatcatcagttttctctctcagactttctgaccttaatttcctcatttgtaaatcggagatagtatccacctcactgagaaaatacatgagagagtactttataaataatatagcactacataaacgttagaaatcactcacatatggtaagaacctcctagtttgttttccttttttttttgagacggagtttcgctcttgttgcccaggctggagtgcaatggtgtgatctcggctcactgcaacttctgccttccaggttcaatcgattctcctgcctcagcctcccgagtagctgggattataggcacccgccaccatgcccggctaattttgtattttttagtagagacgaggtttcaccatgttggccaggctggtttcaaactcctgaccttgtgatccgcctgcctcggcctcccaaagtattgggattataggcatgagccacagcgcccagcctgcttttctttagagagatggacaaccatattgacagattgtcttcacaaactaccttgacttttaggcaacattagtttcctgctttaagaaaatatctgtatataatctttggccagcctctacttttttttttttttaacaatactgagagtaatttttaagctaatgataaaaatttcaaatatgaatgatttcaaacactttagtcttcttccataatccttaaacgttcaggatatcagagtaatgacaggttgtttcagatctcaaattaatagaaagactaatttgtttagtaaggtgggttgccagatccttaaatgtgctcttaactggttccctgtgaaattaaacattggtagttatgtgtttttgaaacaccttgaaattgtcttacataaagtttggttgtggtgaatttatttaaagtattttctttgaaaaaagtttgctaagtagatcctccaatattaaaagaaaaaggtatctctggaataaagtaagaggattgtaatgaaagtaagaggataattgttcatccatcaagccaactcaagctagttctttctttccagtgcagcaacacattttagggcaacaaagttcagaatggatacaatggcctgttcagaaagcatgcaagttatatcagatcatttctttaaagtcagtgtgataaatttgttaactagactccgaccatagaaagagagagatacaggaagtcaatgtaaattgcagacatgccagctctgttggttcacattacagctacctaatgttgggcttaatttctttttcttcttcttcttcactatcatcaacctgttggatgaccagatcagcagacccatcttctacaatctccacataggatctattctcatcttcactcaagtgccatctggaatccttatctccattgttcgaaaatggctacttagatggtctagcctgctaaatctttttccacaagcttgacatggatagggcctttctcctgtatgacaacgaaggtggcgctttaggtctgccttccgcttcaccacatgtgtgcagtacgggcacttgaatcgcatccgaggcagatcatctggaaatttatgaatgctgctcttgaatggagtaaaaaagggaagattctaagtcaaacagtctgtgtttggaggattgtccgcgggccgcggcgcaccggccggtcgcgcgcgcgggccgagggaagattcctggttctcggctggggaaggaccccctttcgaggccgttcctttgcgccctaaaacaagtagccccaacgtgagagaaacaaaaggtatttgct

SEQ ID NO: 14616 - RNA, 112 nt, Homo sapiens
  source 1..112: mol_type = other RNA
gctgggattacaggcatgagccaccgtgcccggcccaacagtctcttattatttttaaagagtttgctagcaaaacttcagttttctttactttaaattttggttacaaaac

SEQ ID NO: 14617 - RNA, 6871 nt, Homo sapiens
  source 1..6871: mol_type = other RNA
gctgggattacaggcatgagccaccgtgcccggcccactttaccttccatatttaaactccagtttatctctctcctcttcttgtaggacaattctgccttaattctatgactaacctaatcttccaaactaatgttttgcctgattatttctttgatgaccccaagacccaaataaactgttagtctccatcctttaaatccaatccatatacctttgcccacttatactcagaggcacacacaaacccacacacagatgagcttaaaccttagaattcaaaggcatgagtggcttttgaatttttttttcccagaggtatgtgcatgtgttgagagaagaggatagaaaagaaaagggtgaaatgagagaagtagggaaattaattatcattttattctctctcacttaagcagtgaaaacaagtcaacaaacctgccacatatgtgtgcattataaagccttgaagaaagtgtttttctttgtgtgatggggttataggaaaattcttattttcctctttgtattaattattattttccaaattttctacaaaaactatttattctacaatttaaaagaatgcaatttctttccatgttaagatatcaactattttttttctaattcttttaccaccttttgtatttctaaaacaaagaacaactgaaaagcaatgagaagtactttattgaaggacacagaccatgactgtaaaggcattttgaaaaacaaatgagaaagaaagtccaaaaatgtttcttaagtggtagctccactggaatcagtgtgcagctttctaaggtaatgaagtaaatagtaacattgattttggatgtaaatatttgaattgattactttgcttgtcttggttttaatctttttctctccccctaaagaacttccacacatgatgccactatgggggtgtgtacccacactgactaaaagtacttatacttaaagaatgttttgctattcccaatccaatatacaatcccattagaaggtaggttaatagatagccccagttcaaaaaagaactgctattaccctccatttttcctctctctgaatcagagattctcttgacaactatcaacagcccaaccataagatacgaatggagatggtaatcatgccacaaaaaaagcccagcagccccatgggggtgcctggaatggtgagattcccatgttcccttccagggcatttttcaatctagaaacattctatttcagcaatctctcctttcagacccttttccatctgagcacctatccagacattaaaattcgtatcttcctttaagaaatctccgtcacaaagccatcatcacccttggctccagcatagataagtcttacatgtgtgatcagaagtaccctggagggagataggaggtgggggagaaactaaaagggcataaacagaaagtgttcctcaacattttcccccattttcacctgattcagaaacaccttgagttcattaccaaatccagaaattatttaacacagatgtacttaaggagttcttgcctttttgtctgtttctcaagttgcccttcatcaccctgaagtcatgaccaggttttttagcagaaaaagtcaacacctgcagcaggcttggccaaggactgagctcatctcctagtcactggctccaggttcaggtgctgcttcctcccacgcttctgcatgtccttggtttacaaagcagatcctactcacagggagctcagggaagaacagttccttcatattcagctcttccaaagacagtctttggataggcggctgtagccaatatagcacagtattcaaaccatcctctcccaaattcacattgttctgcatcccaccactaatagattgtggtgttcccaagggctatgtttttaattaactcaatatttattgatttctattgtatggcaatcattatacttttttgtctttgtaataccaggtcttggtcataagaagcatataataagtgtttgtttttcaataaatgaatatttcctcacctagaaagtgagctctaagaggtcaggaacttgtgcctgacacctcctgggtgcttaaaaattcttcgttaaaattaattaattagttaactcgtgagtaaataaaataatcaacccataccaaaaaactttgtagctgacagtagcaataagtaatacatctgtacaatgaaaatattttgacttttggaattagacccagatccaaattctaggtttatctatatgtccccatatatagaaggaaatcgtatttatctgattgaatcatgaggatttaatgagttattaaacataaaatgcttggcatatttaatggatataaagtgcctggcttttctaatgagtcaaagatgctagtttctcacctttatctcctgtttctgaatctcagttcgtcatccttaaaatgacaataataatggctacttcatcatgatgttgtgaagattaaattgctgtggaaagttcctgaaacagtgctcagcaaaaatcatctctatttttcttacatttcccctaatttcattatgtagctaatgtgtgaagctggaagaaagaagtggattagccattcttaagagtcttgggacatgtgtttcttaatcttcaagactccctggtcttcaacccttcaacagctccctggaagaagaggttgtaaccaagactggttgtgtcctgaaattgatgcctctctttttctccagtctagaaatccctgagatttaatacaaggattctcagaataaaactacattccccagcccctcttgctgttagctgtggtcatgtgactgagttccagctgacggattatgaacagtagtgatgaatgcacatctaagtcctgcctttataggggaggaatgtgtgtctttctctttcccacttcctgtatctgaaacgcagacacagtggctaatcatcttagacaatgtggacaagggcactgacctctggaaagcagacaacaagataatagtagcttagtccttcctgctgctataaccagggtctcaggaatttgacaggaattggtgcaggaatgtctcagtctattactaagtattagtaatactcaatattattgccactattaccccagactatgtcattcataaacaataaaaatgtatttctcatggttctggaggcagggaagtccaataccaaggtgcaaacaggtccagtatctggtgaaggccctctatttgcttcatgggtgacatcttcatcctgtgtcctcatgtggtgaaagagttaagggaagctcattccagtctcttttataaaagcactaatcctattcatgaggatggagccctcaagacttaatcatttccaaaagtcctgaccacttaatactatcacctggtgtattgggttctaacatataaattttgggggtataccaacattcagatcatagaagtaacctaactccccgaaccatggagaaatcatgtgagcccctgaatgcttatgttcagctatctgagagagaaagaaatgtttctcttgcttaaactacagatacttgagtctttgctgtttcagatgaaactaaatctgatctaatacagaggcattaggagatcttcgaatatccaggcattgttaatgacaaatccttaccttaggcactttttaagcctcccccatagggatcccagccaccaggcaaggctaatctgcttggtcggcactgcctgctcaccctcttactggcccgcctacccagagatttaaagttcccacctaggcaaccaaccagaatccaatctagccttgaaagccccttccagagccaatcttgtcaatgaagctttccctgctgaatgatagctctctgggatctctcccttgtctgagctccatagcagctgactagaccatctgttgtttggttccaaccccattctgttttctagcccatgggttttcatccctatgcccttcctctttatattaacaaattcattaagaataagatccatgttttaggcgtttttatcagatgtttgtatctttatctgattttggaagtcatttctaaccatgaagcatcatactctgtactctagaagtaaagtggactttagagattggtttctacatcttcctaaattgtgatgtcttcaaaggcaaaaaaaaactgtgtcacaatgagctctgtgtccacagtaactgattcatgcatgtacctcagtcaatgcttacagattgatagatagatgaatcttagcaggcccccgtcatctagaataatgtcttgtccttaatgcctacatgcctctataaactaattacttaatgtgggtgttgccaaggaaagaaactgtgaaaggaaaataaattttgggtaccccaaatcactaagctaaagggaaaagtcaagctgggaattgctctagactaacctgcctcccattctattcagtcacccctctgctcactgagacaaatgcatatctgattttctcctttggagaggcaaatcagaaactcaaaggaacacaaccattggtctcttacctacctatgacatcccgcctttgcttcaagttgtcccgcctttcccagaatgaaccaatgttcatcttacatatgttgattgatgtctcatgtctccctgggttatctgccaaagttctcacaaaaccaaaatcaaaggtcagccaggtggagttcttatctgaagcttctgaggaagaatctcccttgcagctcattctggtagcagagtccagttccttgtggtcgtaagattaaggtccctgttttcttgctggctgccagttggggttttctctcagttcccgcaggctacccttaggtcttttccatggggccacctccacctttaagtctcatacttcccctttttctaccagctggagaaagctctgctcttaaaggattcatgtcattaggccaggaccacacagatagtctccccttcttatagtcaatctcccaatataacatcacctgctcaccaaggagcactcacaggggagaagattttacaaggcatggatcactggggtcaccttagaatctaccagcacaccacctctgcccaatttcagtcacttaatcacttcacatgggcatttgccacaatctaacaagtgtgtttttccctgtcctgtctcatccatatttaatcagaggtcacaacactatacctttgcatatgcccgtctctcttcctggaatgctttccttgatgcttatcctccaacaaaatcccctttaaacttaatcctccttaagactcaaaggttacaccctctgagggtcttctcagcacccagccacccatcagagttaaataatcccttccctctgttttttatgagacaatccatctcatcacaccagaatctaatccagactattatcgtcttaaacaccagactgtgaggtctctgacatcagagtttgtgtttcattcatctttggtttcccagggcctcccacggatattggcacatagtaagtgctcggaaagtgtttgtcaaatttgaattgacctgaactttctatcctctgttctgcggattcatgattggaagagcagcacagatttgaagtctagtttggggcataaagtaaaatatctgcaatttttacctcccagcatggattatttggtgttctgattattgaaccctaataagccattatgaaaccacaacacccccactttccatccatgcaatcaacatgggatttccttactaccccatccaagtatagactcacctatgactcaggctttgctaataagaggcaccgtgattgattccaagatggacacctgatgcaattcagctgatgacatgcctttcatcctcttacaccctttgggaaagcagttttctctttccgtcggacttgtggagctggtaaaataaagacttgaagcaactagtggctttctctgccaccctctaaaggaaacctcataatgaaccaacacagaaaaaataatagaactaagagatgacaacagagaaacactgagtcctgaagacatcatgagccactggactgagccacgcctaaagcttgtcatcttttgaattggccagtaaatgaaatctcttcttacttacatttccactgacacactttcccgtttattaattagcgttgggtttctgttacttgcaaccaaaaccaaaaccctgctcaatcctttttactttgtgttggaatgcaaagaccaaggatttggggactgatactcagggtgttggaactttgctgtaagctgctcacagatcattaaagatcccagctgttcctggtccataacaacccctttcaactgggtctccttccaggaacagctgcaaaagctccagaaaggaagggaggagacacatttagcatgataacaaatcagtagggagtggccagtttacccagaaaggctgtgatgcagttatatccacccagcaactctccccaccctctaggagagagacaaattcgtgctgcctctgtgtgaaaactcttcatatctaaaggaatgaaatcaagaatcacaacccacccctgctccctggagaggaacctggacaaggttcttgctttttccatcatcattcacaaaaaggcctgtcagtggttacaagaagattattatcttgcatatacatacatataacatatactcacaccaaattaacaacatggaagaaggagctgtcatctatctcatgcagggcactgtgcaaagagttcaacatatgtttgcaggctgggcgtggtggctcatacctgtaatcccagcactttgtgaggccgaggctggtggatcac

SEQ ID NO: 14618 - RNA, 2426 nt, Homo sapiens
  source 1..2426: mol_type = other RNA
gctgggattacaggcatgagccaccgtgcccggcccagaatgttctttcatttttacactagataagttgttacctactggggagtgtgcatcagaatcaagtgcattactttttagtatattataatggtaatgcataatatacataatgttttgctacttgctttttgcttattatatccttggacatcttcccatgtcaataatataaattatgtcatttgtaaaatggaaatatgatagttataaaaactaacttaatacttataaataaggtagaacaatgtctaccttacataacataataattgcttaactaagattagctattgttttgtcattggaaaactgttccataatttgaataatctattgatgggcatgtagactgctttcagttttcccctactacaaataatatggaattgaccaactttatatgtaggcttgatatgtataatgttactaggatacgttttcagcagtggaaatactggattatagagaatatacctgtacccatcatatatttcagccaaagcccatccttctatacctgctttgtgaccctcgggtgggaatcagtaaactgccttttccagactggcttgccaactggcttttgatttctccaaggaagatattgccaaatcaagctcaaaaatggctgtatcaatttgtattcccaccaacaatatatgaaaaggcttctttcccaaactgtggagttaaaaaaaaaaagtgtaggaccccattccaagcctactgagaactgggtgggacctggacacaatgtattttccaaaagcactataaatgatcccaatgcacagccaggtaagaaccattgttctagatatttgattctcaaagtgtggtccccagatgggcagtgtcagccctgggagtctgttagaaatgcatcatctcagaagctatattttaacaggagccccaggagattcaaatgcacattgaagtttgagaaacactgctctagaaaggatacagcaacaggcctagattttgtggggcctaaagcttacataatctggggagtcctttttactgaaaaatatacaaaattacaaacaaagatggagtacaaatttaatatttacttacaatgaagtaataaatcctgattaaatacaaaattttaaaagccgaaaagtaccataaacatcacaaaattctggaggaaaaaaggaaaaaacgcatttattcatgagctgcctaatgcacgtctatatttttgtaaatttttagctatttctttgcatgataaaaaaaatttctatgatctttctatagagagatgagaattaattcagtcagctagaaatttgtgttttattcttggtaatctagaagagcttttttttttcaactttcaactcattataatatcatgtaaaattttttagaatttggtccagttaggataagttccatccaatgtctttcatgggagctgtaagagtcatggcatttcatggttctcatccagtggctaattttaaatgcccttggaatcaaggacagtcagacatccttgtgcagagcattactttcatgtttcttctcctcttctgttctgtgccccagagtgtcccaattcacataaatttctttacctcttctgttattgttttacctacattttctttgctcttgtgattctgagtttttgtttgttttttatttgttttttgtctttatgagtgtgaccatcagagtttttatcttctcttatgaaaaaagagagttctcaacattttgaagtctctgctagttcctaaaagttccttcttttcgttagatcttcagtttccagtaggttccagccttcccttcacatttgagttttacagtatgatcaaccacttgttatgtcataactctgagctttcactgctagcaatcacaaggttgtgtattctcttttcattctttatctgcggtgaatatagtagacgagatgacctccagtggccaggtatctcaaacatatgcctctgcagtggttgcattctcccgcgctgtttgttcacactgagcccagcatgggggaagcttcaggatgcaacaataaataagggaagggagccatctccagttgagtcagataaatcctcttcttcccattattttttcttttcccttctgctgccagatctttggtcatttcacagctcgttagcattctctctctgtagtctcagcactttgggaggccaaggcgggaggatcacttgagctcagaagttcaagaccagcctggacaacaaagcaagactctgcctcttttcaagcgtccggcggcagcggccgggcgcgggtccgcagaaaagccgaggcgtttcgggtcccaagctgttccgccgccggccccggcctggcaggcgcgcggagccggaacgcgc

SEQ ID NO: 14619 - RNA, 2652 nt, Homo sapiens
  source 1..2652: mol_type = other RNA
gctgggattacaggcatgagccaccgtgcccggccctgactttcaagagaaaaacctgactcttcccacagctgacttgattggcagcataggcaaagacttgaagcgagtttggagcgctgactgcctgccctgcactggctgggtttatcgccatctgtgaggtgctaccttcatccccctgtacagacaaggaccccaggctcaataggctgaggcactggcccagggacctccatgccacccttattgtgaggaggacacatttgtgactctgaagcagaaaaggccctttgtcctgccaaaccatgggcaggattcaggggtctacaatgtgactgctcgggtggcctgaccgctgagcctatgaggctggggttgggaggaggacactagcctggtgcctactcacagggagcactcaacaaacagcagcaggaggaagaggagaggatggggcagcagcagcaggagggaaggttcgagcctccgcagtggaggggaggctctgcgggcgtctctcagctggcgaaggctcctgagagcagggatcaggtctgcagccccagggccagctcagtaggggagcaaggtgtgtgaacacatcgatgagggccgtgccttgtgccatccttcttccccttcacaggcagctgggcatgttggggccagaggggagggcctgttagtttcctgtggcagccatgtaacaacttatggctgactcagtggcttaagcaacgcacatttattaccttacagtcaagggggtcagatgtctgaggtggggtcccagaactaaaatccaggtgttggcagggctggttcctcctggaactccaggggaaaaatccatcccttgccttttctggcctctggcggcacttgcactccttggctcctcgtcccttcttccgtctttaaagccagcagcgtccccttgttctgtctctgaccacggctgggaaggagtctctgcttttgggcacacgtggctaatccaggctaccctctcactgcagatcttcaactcaatcacacacctacaaagtccctttggtctgggaggtaacactttcccaggctccagggattagggcttggacatcttggggactttattctgcccaggaaaggtggtatcagggagtctgagcatctgaacctccccaggggactgaaggaatgccttcagtgtcctcttcctcctcctcagcagctgtgaatccagaatagaggccatctacaaggtcacacctggagggatctggggaaactgaggtcacagaggtcttgcccaggaccccaggccaggccctgtgtttcttccacagatggccccttccccaccaccctgtagtgcactgcccagggggtggaagtgttttagcctggagggacaccagcttgaggactctgtagagctctgggcctagggggagggcgggcaatgtcatctatggggtggcttccccacaccaggggcagctttacggaggttaccttttcatccccccaagtcctgtggcaagtgaagatctgtttcctcatctcatagggtaaggaagctgaggccctcaaaggggcagtggcttgtccgtggagaagagtctgctccttccgacaagcctgtggctggtggtgaagcaggtgtgaatggtctgtcccatgagcaggagggtgggtgtgcggcgatgtcggcgtggtctccgcagagctctgtgcacaggcctgtgcatctgctgacaggcagctgagaaggcttgcagtcacatcgctgatggtaaagctgtagcaacaggctcagagaggtgtgttagctttcccagagacacacagctctctggaagagtgccatcctctgagctccatcgcctggtgctttgcatcccttgccccaagggcacacgtagaagcagagttccttggggttggatctgtggggtggtttgtgagggggactgtgtcatccactgtggaaaagacttagctgcctctctgtaaaacatttttgcctgacgtgagttctctcccttgaccgggggccagcacagtacatagtagggtggttaagagccctgggtttgggctgagcgcggtagctcatacctgtaattccagcacattgggaggccgaggcaggaagattgcatgagcccaggagtttgagaccaaccctcgctggaaagttcgccctgcccgggctgggctcccaggcagcctggcaccgtgccaggctcgccgccgagctcgggcagcagggtggggcaaacgcggagcacggaggacggggccgggcgacctgggcaccagcaggacccgaggccaggagccaggggcccagaaggtgagggcaccccgggtgggcgcagggtgggcgctctgtgggcaacgggccctgcggccgggcccaggagcaggcctcgttgcggggttggggggggaggttggagcggaggctggcagaggaggcaggcacaaaggagggcagtgccaggcagctgtggccgacgcaggcatcgctgcccgcctgcccctagccggcctccccgccgaggggaggacgcgtgtgcaggggcccgggcaggagcggcagacaccgagccgcggccacagggccagccgcacagtcggaggaagggccggagcgag

SEQ ID NO: 14620 - RNA, 3697 nt, Homo sapiens
  source 1..3697: mol_type = other RNA
gctgggattacaggcatgagccaccgtgcccggccctggctgttttcctatgctctgtggaggccagccagctagaaatgattagaatggaggaagagggaatgagaaggctggtggcgagtggtctagcgttcttgtggtgcagcggaaggagccctggctcagcattgaagaacgagcctcagtcttggctccagccatctgctagctatgggactacagacaagcccctttacctgtgtctcagttttcgtatctgtaaaataggcacagtggtttctgtcctgtctttctcacaggattactgtacagataaagtaagataaaggacacctgtcaaggagatatctgtaaacagttctacagacttcaggtaataatagcaagggaggatctcttagacctctgatctgtctgttagaatatactttttttttttttttttttcctgagatggagtttcgctcttgttgctcaggctggggtgcaatggtgctgtcttggctcactgcaacctctgcctcctgggttcgagtgattctcctgcctcagcctcccaagtagctgggactgcaggtgcgtgccatcatgcccagctaatttttgtacttttagtagagatggagtttcaccatgtagtccaggctggtttcaaacttctgacctcaggtgatccacctgccttggcctcccaaagtgctaggattacaggtgtgagccactgtgcccagccagaatatatcatttcactggactctgcaggtgctttggatgatcaaggaataggacatggctgtagaagtacttttcttcttcttttttgtttttttttgagacagagtcttacctgttgcccaggctggagtgcagtgacacaatcaaggctcactgtagcttcaacctccggggaacaagcaatcctcccacctcagccttctgagtagctgcgactacaggcataagccaccatacccagctttttttttttgccggggggagggtgggcgtagagatgggatcctcactatgttgctcaggccggtcttgaactcctgggctcaagccattctcccacattgtcttcccaaagtgctaggatttcaggcatgagccactgtgcccagcctgaagtacttttcttgaactcagcattgctgccctgaaccctcccccagctgccttccctactttgggagcctctatttctagaacaggaaaacgctaggctaaatatatgtcctaatggtctcttccatcggtgtgaaggaaagaaaatgggcccaatgttgttgcaaggattaggaaggtcctgccttgccacccagtgggtttagaaatccatctttacggcctccagagaagctggtgatcaggttcccagacatcagcaatcctgtttcctgaggagcttgtgggggctctctctggggatgatctgggtcctagacaaagagccacaactgatgggggtcactgggattgcagggggccatggctggctttttgtcctgggatgtcaggcaggtaccagatcctgagttcctgatgagctgatcctgggccaattcccattcctcgtccttggggacctggctattcttgccagtgaagtgacagctcccaaggcccagagcacccttgctgacatgtagacacagctgctttgcgatgttgtggcgaaggtccctctgagttgtgtactcaaagtactggttgccgccaaggccgtggcaggagtacatgatgaggggcttccccccgcggttgttctcacccacatccaggcattggttggtgccgaggttcttgatggcaccatagaaggtgggcgtcaggtcaggaacaaacatctctgggtagacattgtgcaggtaccaggaaaagttgtgacagtgcagttgttccctcagctgcagtcgttccgaaatgtcaccgaaggatttctcttgggccatctttgctgcctgcagatttctcctatagaaaatcttcttgtagctgtccatccagacctctgccaggcgcacttgattgcgagcaatgacactagtgcccttggggaaggtgtgggggctcttggtccggaacacatggcctacgacagagcaggggatgatctccagctggcccccacactgccacacccggaaggacatttccacgttctcccctccccagatctccatctgattatcataggtaccgatgtgctcaaagtaggacttggagatggagaagaggccaccagcaaacgtcggggatttgatggggtaggtttcatccttgcgcctctgcttctcatgtggaggaagtgtttcccagccgaaggtcaggctccagtcaaagttgcctcggctatggactctgcccctctggacgggcttggcgaactcaaaagtattaaggtcgatggtgacgatgtctgggctcaccaccactgtcttgtcctcagcgattcgagccaggaggggctccagccagccgtggaagcactcacagtgggcatccaggaacgtgagcacctccgcctgtgccacgctggcccccagcagccgggcggtgatcagccccttccgctcctcctgccgcaccaccctcaccacctgcagctgcttcacgtactgctccagcttctcctttaggtgctcctctgtgctggcatcatccaccagtatgatctccttgagcaagatggcaggggtggtgtgtaggacgctgtacactgttcgcagcagtgtggaccaggcttcgttgtggaacacaatgatcacgctggtggtggccagtggggggcagcgccggaacttctggtccacacactcaggtggtcgggtgtctggccccagggacctctgcagggagatccggtcgctggcaaaggcattgaaacagtgcttcttatagccttcttccttttcctgggtctccaggggggtccacttgctcttctgaaatgcttttccatctgccccaggggcattggggtcctgtggtggccgttcccagaagggcttcagttcagctggggtatagaacccagggaggcaggactggtttatggagaacagagtctgctgggcttctggagccctgatttggagcttgggcattgaatctctaaggttgttcatggcctccagcatgaggtccaggacgtgatccttccggctcaccagggacttcagccacggcttctctgtggcctcctctctgctgctcacatccctatgcaggaggaagaggaagagcacaaaggcgcagcccaccatggccaggcgcaggggcatgtggcgtctgcggaggagcctcatcctccagaaccaaggggcaccccagctgcgtcagctctgagtcctgagcccaaccctggagatagcttgatacgttgtggtggccacaagctggggcctcagccccctccaggaaggcctcctgactgattcactcagaatcacctaggttactccaactctttcatcctggcactgcctcgtggtccctcacagcagggcctgtttttgcttcttttattttcccctctgcagacgtctgggtctgcgatgattggccctggatgcaagtaaaagctgtttctcctttttgtcagcctgggaatctgaacaacgagggaggagctacaggccaccgcgaccagcagagagcgaaggcaggagggaccagcctggcccagcccctt

SEQ ID NO: 14621 - RNA, 3785 nt, Homo sapiens
  source 1..3785: mol_type = other RNA
gctgggattacaggcatgagccaccgtgcccggccctggctgttttcctatgctctgtggaggccagccagctagaaatgattagaatggaggaagagggaatgagaaggctggtggcgagtggtctagcgttcttgtggtgcagcggaaggagccctggctcagcattgaagaacgagcctcagtcttggctccagccatctgctagctatgggactacagacaagcccctttacctgtgtctcagttttcgtatctgtaaaataggcacagtggtttctgtcctgtctttctcacaggattactgtacagataaagtaagataaaggacacctgtcaaggagatatctgtaaacagttctacagacttcaggtaataatagcaagggaggatctcttagacctctgatctgtctgttagaatatactttttttttttttttttttcctgagatggagtttcgctcttgttgctcaggctggggtgcaatggtgctgtcttggctcactgcaacctctgcctcctgggttcgagtgattctcctgcctcagcctcccaagtagctgggactgcaggtgcgtgccatcatgcccagctaatttttgtacttttagtagagatggagtttcaccatgtagtccaggctggtttcaaacttctgacctcaggtgatccacctgccttggcctcccaaagtgctaggattacaggtgtgagccactgtgcccagccagaatatatcatttcactggactctgcaggtgctttggatgatcaaggaataggacatggctgtagaagtacttttcttcttcttttttgtttttttttgagacagagtcttacctgttgcccaggctggagtgcagtgacacaatcaaggctcactgtagcttcaacctccggggaacaagcaatcctcccacctcagccttctgagtagctgcgactacaggcataagccaccatacccagctttttttttttgccggggggagggtgggcgtagagatgggatcctcactatgttgctcaggccggtcttgaactcctgggctcaagccattctcccacattgtcttcccaaagtgctaggatttcaggcatgagccactgtgcccagcctgaagtacttttcttgaactcagcattgctgccctgaaccctcccccagctgccttccctactttgggagcctctatttctagaacaggaaaacgctaggctaaatatatgtcctaatggtctcttccatcggtgtgaaggaaagaaaatgggcccaatgttgttgcaaggattaggaaggtcctgccttgccacccagtgggtttagaaatccatctttacggcctccagagaagctggtgatcaggttcccagacatcagcaatcctgtttcctgaggagcttgtgggggctctctctggggatgatctgggtcctagacaaagagccacaactgatgggggtcactgggattgcagggggccatggctggctttttgtcctgggatgtcaggcaggtaccagatcctgagttcctgatgagctgatcctgggccaattcccattcctcgtccttggggacctggctattcttgccagtgaagtgacagctcccaaggcccagagcacccttgctgacatgtagacacagctgctttgcgatgttgtggcgaaggtccctctgagttgtgtactcaaagtactggttgccgccaaggccgtggcaggagtacatgatgaggggcttccccccgcggttgttctcacccacatccaggcattggttggtgccgaggttcttgatggcaccatagaaggtgggcgtcaggtcaggaacaaacatctctgggtagacattgtgcaggtaccaggaaaagttgtgacagtgcagttgttccctcagctgcagtcgttccgaaatgtcaccgaaggatttctcttgggccatctttgctgcctgcagatttctcctatagaaaatcttcttgtagctgtccatccagacctctgccaggcgcacttgattgcgagcaatgacactagtgcccttggggaaggtgtgggggctcttggtccggaacacatggcctacgacagagcaggggatgatctccagctggcccccacactgccacacccggaaggacatttccacgttctcccctccccagatctccatctgattatcataggtaccgatgtgctcaaagtaggacttggagatggagaagaggccaccagcaaacgtcggggatttgatggggtaggtttcatccttgcgcctctgcttctcatgtggaggaagtgtttcccagccgaaggtcaggctccagtcaaagttgcctcggctatggactctgcccctctggacgggcttggcgaactcaaaagtattaaggtcgatggtgacgatgtctgggctcaccaccactgtcttgtcctcagcgattcgagccaggaggggctccagccagccgtggaagcactcacagtgggcatccaggaacgtgagcacctccgcctgtgccacgctggcccccagcagccgggcggtgatcagccccttccgctcctcctgccgcaccaccctcaccacctgcagctgcttcacgtactgctccagcttctcctttaggtgctcctctgtgctggcatcatccaccagtatgatctccttgagcaagatggcaggggtggtgtgtaggacgctgtacactgttcgcagcagtgtggaccaggcttcgttgtggaacacaatgatcacgctggtggtggccagtggggggcagcgccggaacttctggtccacacactcaggtggtcgggtgtctggccccagggacctctgcagggagatccggtcgctggcaaaggcattgaaacagtgcttcttatagccttcttccttttcctgggtctccaggggggtccacttgctcttctgaaatgcttttccatctgccccaggggcattggggtcctgtggtggccgttcccagaagggcttcagttcagctggggtatagaacccagggaggcaggactggtttatggagaacagagtctgctgggcttctggagccctgatttggagcttgggcattgaatctctaaggttgttcatggcctccagcatgaggtccaggacgtgatccttccggctcaccagggacttcagccacggcttctctgtggcctcctctctgctgctcacatccctatgcaggaggaagaggaagagcacaaaggcgcagcccaccatggccaggcgcaggggcatgtggcgtctgcggaggagcctcatcctccagaaccaaggggcaccccagctgcgtcagctctgagtcctgagcccaaccctggagatagcttgatacgttgtggtggccacaagctggggcctcagccccctccaggaaggcctcctgactgattcactcagaatcacctaggttactccaactctttcatcctggcactgcctcgtggtccctcacagcagggcctgtttttgcttcttttattttcccctctgcagacgtctgggtctgcgatgattggccctggatgcaagtaaaagctgtttctcctttttgtcagcctgggaatctgaacaactccaccagcgaggcttctccttgctgtccccttctgctcaggcgcaacgtggcagggcaggaggaaacctctctgcaagagttgccgtaccagagcacatggggtggcccgatctgtcgcgccgaggcaaagccgcagccgcgccgcggggtggctcccg

SEQ ID NO: 14622 - RNA, 3677 nt, Homo sapiens
  source 1..3677: mol_type = other RNA
gctgggattacaggcatgagccaccgtgcccggccctggctgttttcctatgctctgtggaggccagccagctagaaatgattagaatggaggaagagggaatgagaaggctggtggcgagtggtctagcgttcttgtggtgcagcggaaggagccctggctcagcattgaagaacgagcctcagtcttggctccagccatctgctagctatgggactacagacaagcccctttacctgtgtctcagttttcgtatctgtaaaataggcacagtggtttctgtcctgtctttctcacaggattactgtacagataaagtaagataaaggacacctgtcaaggagatatctgtaaacagttctacagacttcaggtaataatagcaagggaggatctcttagacctctgatctgtctgttagaatatactttttttttttttttttttcctgagatggagtttcgctcttgttgctcaggctggggtgcaatggtgctgtcttggctcactgcaacctctgcctcctgggttcgagtgattctcctgcctcagcctcccaagtagctgggactgcaggtgcgtgccatcatgcccagctaatttttgtacttttagtagagatggagtttcaccatgtagtccaggctggtttcaaacttctgacctcaggtgatccacctgccttggcctcccaaagtgctaggattacaggtgtgagccactgtgcccagccagaatatatcatttcactggactctgcaggtgctttggatgatcaaggaataggacatggctgtagaagtacttttcttcttcttttttgtttttttttgagacagagtcttacctgttgcccaggctggagtgcagtgacacaatcaaggctcactgtagcttcaacctccggggaacaagcaatcctcccacctcagccttctgagtagctgcgactacaggcataagccaccatacccagctttttttttttgccggggggagggtgggcgtagagatgggatcctcactatgttgctcaggccggtcttgaactcctgggctcaagccattctcccacattgtcttcccaaagtgctaggatttcaggcatgagccactgtgcccagcctgaagtacttttcttgaactcagcattgctgccctgaaccctcccccagctgccttccctactttgggagcctctatttctagaacaggaaaacgctaggctaaatatatgtcctaatggtctcttccatcggtgtgaaggaaagaaaatgggcccaatgttgttgcaaggattaggaaggtcctgccttgccacccagtgggtttagaaatccatctttacggcctccagagaagctggtgatcaggttcccagacatcagcaatcctgtttcctgaggagcttgtgggggctctctctggggatgatctgggtcctagacaaagagccacaactgatgggggtcactgggattgcagggggccatggctggctttttgtcctgggatgtcaggcaggtaccagatcctgagttcctgatgagctgatcctgggccaattcccattcctcgtccttggggacctggctattcttgccagtgaagtgacagctcccaaggcccagagcacccttgctgacatgtagacacagctgctttgcgatgttgtggcgaaggtccctctgagttgtgtactcaaagtactggttgccgccaaggccgtggcaggagtacatgatgaggggcttccccccgcggttgttctcacccacatccaggcattggttggtgccgaggttcttgatggcaccatagaaggtgggcgtcaggtcaggaacaaacatctctgggtagacattgtgcaggtaccaggaaaagttgtgacagtgcagttgttccctcagctgcagtcgttccgaaatgtcaccgaaggatttctcttgggccatctttgctgcctgcagatttctcctatagaaaatcttcttgtagctgtccatccagacctctgccaggcgcacttgattgcgagcaatgacactagtgcccttggggaaggtgtgggggctcttggtccggaacacatggcctacgacagagcaggggatgatctccagctggcccccacactgccacacccggaaggacatttccacgttctcccctccccagatctccatctgattatcataggtaccgatgtgctcaaagtaggacttggagatggagaagaggccaccagcaaacgtcggggatttgatggggtaggtttcatccttgcgcctctgcttctcatgtggaggaagtgtttcccagccgaaggtcaggctccagtcaaagttgcctcggctatggactctgcccctctggacgggcttggcgaactcaaaagtattaaggtcgatggtgacgatgtctgggctcaccaccactgtcttgtcctcagcgattcgagccaggaggggctccagccagccgtggaagcactcacagtgggcatccaggaacgtgagcacctccgcctgtgccacgctggcccccagcagccgggcggtgatcagccccttccgctcctcctgccgcaccaccctcaccacctgcagctgcttcacgtactgctccagcttctcctttaggtgctcctctgtgctggcatcatccaccagtatgatctccttgagcaagatggcaggggtggtgtgtaggacgctgtacactgttcgcagcagtgtggaccaggcttcgttgtggaacacaatgatcacgctggtggtggccagtggggggcagcgccggaacttctggtccacacactcaggtggtcgggtgtctggccccagggacctctgcagggagatccggtcgctggcaaaggcattgaaacagtgcttcttatagccttcttccttttcctgggtctccaggggggtccacttgctcttctgaaatgcttttccatctgccccaggggcattggggtcctgtggtggccgttcccagaagggcttcagttcagctggggtatagaacccagggaggcaggactggtttatggagaacagagtctgctgggcttctggagccctgatttggagcttgggcattgaatctctaaggttgttcatggcctccagcatgaggtccaggacgtgatccttccggctcaccagggacttcagccacggcttctctgtggcctcctctctgctgctcacatccctatgcaggaggaagaggaagagcacaaaggcgcagcccaccatggccaggcgcaggggcatgtggcgtctgcggaggagcctcatcctccagaaccaaggggcaccccagctgcgtcagctctgagtcctgagcccaaccctggagatagcttgatacgttgtggtggccacaagctggggcctcagccccctccaggaaggcctcctgactgattcactcagaatcacctaggttactccaactctttcatcctggcactgcctcgtggtccctcacagcagggcctgtttttgcttcttttattttcccctctgcagacgtctgggtctgcgatgattggccctggatgcaagtaaaagctgtttctcctttttgtcagcctgggaatctgaacaactgtcgcgccgaggcaaagccgcagccgcgccgcggggtggctcccgggtttc

SEQ ID NO: 14623 - RNA, 3891 nt, Homo sapiens
  source 1..3891: mol_type = other RNA
gctgggattacaggcatgagccaccgtgcccggccctggctgttttcctatgctctgtggaggccagccagctagaaatgattagaatggaggaagagggaatgagaaggctggtggcgagtggtctagcgttcttgtggtgcagcggaaggagccctggctcagcattgaagaacgagcctcagtcttggctccagccatctgctagctatgggactacagacaagcccctttacctgtgtctcagttttcgtatctgtaaaataggcacagtggtttctgtcctgtctttctcacaggattactgtacagataaagtaagataaaggacacctgtcaaggagatatctgtaaacagttctacagacttcaggtaataatagcaagggaggatctcttagacctctgatctgtctgttagaatatactttttttttttttttttttcctgagatggagtttcgctcttgttgctcaggctggggtgcaatggtgctgtcttggctcactgcaacctctgcctcctgggttcgagtgattctcctgcctcagcctcccaagtagctgggactgcaggtgcgtgccatcatgcccagctaatttttgtacttttagtagagatggagtttcaccatgtagtccaggctggtttcaaacttctgacctcaggtgatccacctgccttggcctcccaaagtgctaggattacaggtgtgagccactgtgcccagccagaatatatcatttcactggactctgcaggtgctttggatgatcaaggaataggacatggctgtagaagtacttttcttcttcttttttgtttttttttgagacagagtcttacctgttgcccaggctggagtgcagtgacacaatcaaggctcactgtagcttcaacctccggggaacaagcaatcctcccacctcagccttctgagtagctgcgactacaggcataagccaccatacccagctttttttttttgccggggggagggtgggcgtagagatgggatcctcactatgttgctcaggccggtcttgaactcctgggctcaagccattctcccacattgtcttcccaaagtgctaggatttcaggcatgagccactgtgcccagcctgaagtacttttcttgaactcagcattgctgccctgaaccctcccccagctgccttccctactttgggagcctctatttctagaacaggaaaacgctaggctaaatatatgtcctaatggtctcttccatcggtgtgaaggaaagaaaatgggcccaatgttgttgcaaggattaggaaggtcctgccttgccacccagtgggtttagaaatccatctttacggcctccagagaagctggtgatcaggttcccagacatcagcaatcctgtttcctgaggagcttgtgggggctctctctggggatgatctgggtcctagacaaagagccacaactgatgggggtcactgggattgcagggggccatggctggctttttgtcctgggatgtcaggcaggtaccagatcctgagttcctgatgagctgatcctgggccaattcccattcctcgtccttggggacctggctattcttgccagtgaagtgacagctcccaaggcccagagcacccttgctgacatgtagacacagctgctttgcgatgttgtggcgaaggtccctctgagttgtgtactcaaagtactggttgccgccaaggccgtggcaggagtacatgatgaggggcttccccccgcggttgttctcacccacatccaggcattggttggtgccgaggttcttgatggcaccatagaaggtgggcgtcaggtcaggaacaaacatctctgggtagacattgtgcaggtaccaggaaaagttgtgacagtgcagttgttccctcagctgcagtcgttccgaaatgtcaccgaaggatttctcttgggccatctttgctgcctgcagatttctcctatagaaaatcttcttgtagctgtccatccagacctctgccaggcgcacttgattgcgagcaatgacactagtgcccttggggaaggtgtgggggctcttggtccggaacacatggcctacgacagagcaggggatgatctccagctggcccccacactgccacacccggaaggacatttccacgttctcccctccccagatctccatctgattatcataggtaccgatgtgctcaaagtaggacttggagatggagaagaggccaccagcaaacgtcggggatttgatggggtaggtttcatccttgcgcctctgcttctcatgtggaggaagtgtttcccagccgaaggtcaggctccagtcaaagttgcctcggctatggactctgcccctctggacgggcttggcgaactcaaaagtattaaggtcgatggtgacgatgtctgggctcaccaccactgtcttgtcctcagcgattcgagccaggaggggctccagccagccgtggaagcactcacagtgggcatccaggaacgtgagcacctccgcctgtgccacgctggcccccagcagccgggcggtgatcagccccttccgctcctcctgccgcaccaccctcaccacctgcagctgcttcacgtactgctccagcttctcctttaggtgctcctctgtgctggcatcatccaccagtatgatctccttgagcaagatggcaggggtggtgtgtaggacgctgtacactgttcgcagcagtgtggaccaggcttcgttgtggaacacaatgatcacgctggtggtggccagtggggggcagcgccggaacttctggtccacacactcaggtggtcgggtgtctggccccagggacctctgcagggagatccggtcgctggcaaaggcattgaaacagtgcttcttatagccttcttccttttcctgggtctccaggggggtccacttgctcttctgaaatgcttttccatctgccccaggggcattggggtcctgtggtggccgttcccagaagggcttcagttcagctggggtatagaacccagggaggcaggactggtttatggagaacagagtctgctgggcttctggagccctgatttggagcttgggcattgaatctctaaggttgttcatggcctccagcatgaggtccaggacgtgatccttccggctcaccagggacttcagccacggcttctctgtggcctcctctctgctgctcacatccctatgcaggaggaagaggaagagcacaaaggcgcagcccaccatggccaggcgcaggggcatgtggcgtctgcggaggagcctcatcctccagaaccaaggggcaccccagctgcgtcagctctgagtcctgagcccaaccctggagatagcttgatacgttgtggtggccacaagctggggcctcagccccctccaggaaggcctcctgactgattcactcagaatcacctaggttactccaactctttcatcctggcactgcctcgtggtccctcacagcagggcctgtttttgcttcttttattttccctgtcgcgccgaggcaaagccgcagccgcgccgcggggtggctcccgggtttccccaccggacggccgggagggtgggaccggggcgggacctcccccagctgcactaacgcgcccgccccgcccctccctggccaggtgcagcgggtcccgccgtgtcctcagcctgctgcgggcccgggaactcccggcggaccggcagaggggcgccccggcttctctgcgtctcagcccgccccgggggtgcggtctttgcggccaggctttcagcgcggaaaaagattggagggtcctagtcaccccaaagaggacaggcattagcagagccgcgggcggcgggtgcatggaaccggaat

SEQ ID NO: 14624 - RNA, 3622 nt, Homo sapiens
  source 1..3622: mol_type = other RNA
gctgggattacaggcatgagccaccgtgcccggccctggctgttttcctatgctctgtggaggccagccagctagaaatgattagaatggaggaagagggaatgagaaggctggtggcgagtggtctagcgttcttgtggtgcagcggaaggagccctggctcagcattgaagaacgagcctcagtcttggctccagccatctgctagctatgggactacagacaagcccctttacctgtgtctcagttttcgtatctgtaaaataggcacagtggtttctgtcctgtctttctcacaggattactgtacagataaagtaagataaaggacacctgtcaaggagatatctgtaaacagttctacagacttcaggtaataatagcaagggaggatctcttagacctctgatctgtctgttagaatatactttttttttttttttttttcctgagatggagtttcgctcttgttgctcaggctggggtgcaatggtgctgtcttggctcactgcaacctctgcctcctgggttcgagtgattctcctgcctcagcctcccaagtagctgggactgcaggtgcgtgccatcatgcccagctaatttttgtacttttagtagagatggagtttcaccatgtagtccaggctggtttcaaacttctgacctcaggtgatccacctgccttggcctcccaaagtgctaggattacaggtgtgagccactgtgcccagccagaatatatcatttcactggactctgcaggtgctttggatgatcaaggaataggacatggctgtagaagtacttttcttcttcttttttgtttttttttgagacagagtcttacctgttgcccaggctggagtgcagtgacacaatcaaggctcactgtagcttcaacctccggggaacaagcaatcctcccacctcagccttctgagtagctgcgactacaggcataagccaccatacccagctttttttttttgccggggggagggtgggcgtagagatgggatcctcactatgttgctcaggccggtcttgaactcctgggctcaagccattctcccacattgtcttcccaaagtgctaggatttcaggcatgagccactgtgcccagcctgaagtacttttcttgaactcagcattgctgccctgaaccctcccccagctgccttccctactttgggagcctctatttctagaacaggaaaacgctaggctaaatatatgtcctaatggtctcttccatcggtgtgaaggaaagaaaatgggcccaatgttgttgcaaggattaggaaggtcctgccttgccacccagtgggtttagaaatccatctttacggcctccagagaagctggtgatcaggttcccagacatcagcaatcctgtttcctgaggagcttgtgggggctctctctggggatgatctgggtcctagacaaagagccacaactgatgggggtcactgggattgcagggggccatggctggctttttgtcctgggatgtcaggcaggtaccagatcctgagttcctgatgagctgatcctgggccaattcccattcctcgtccttggggacctggctattcttgccagtgaagtgacagctcccaaggcccagagcacccttgctgacatgtagacacagctgctttgcgatgttgtggcgaaggtccctctgagttgtgtactcaaagtactggttgccgccaaggccgtggcaggagtacatgatgaggggcttccccccgcggttgttctcacccacatccaggcattggttggtgccgaggttcttgatggcaccatagaaggtgggcgtcaggtcaggaacaaacatctctgggtagacattgtgcaggtaccaggaaaagttgtgacagtgcagttgttccctcagctgcagtcgttccgaaatgtcaccgaaggatttctcttgggccatctttgctgcctgcagatttctcctatagaaaatcttcttgtagctgtccatccagacctctgccaggcgcacttgattgcgagcaatgacactagtgcccttggggaaggtgtgggggctcttggtccggaacacatggcctacgacagagcaggggatgatctccagctggcccccacactgccacacccggaaggacatttccacgttctcccctccccagatctccatctgattatcataggtaccgatgtgctcaaagtaggacttggagatggagaagaggccaccagcaaacgtcggggatttgatggggtaggtttcatccttgcgcctctgcttctcatgtggaggaagtgtttcccagccgaaggtcaggctccagtcaaagttgcctcggctatggactctgcccctctggacgggcttggcgaactcaaaagtattaaggtcgatggtgacgatgtctgggctcaccaccactgtcttgtcctcagcgattcgagccaggaggggctccagccagccgtggaagcactcacagtgggcatccaggaacgtgagcacctccgcctgtgccacgctggcccccagcagccgggcggtgatcagccccttccgctcctcctgccgcaccaccctcaccacctgcagctgcttcacgtactgctccagcttctcctttaggtgctcctctgtgctggcatcatccaccagtatgatctccttgagcaagatggcaggggtggtgtgtaggacgctgtacactgttcgcagcagtgtggaccaggcttcgttgtggaacacaatgatcacgctggtggtggccagtggggggcagcgccggaacttctggtccacacactcaggtggtcgggtgtctggccccagggacctctgcagggagatccggtcgctggcaaaggcattgaaacagtgcttcttatagccttcttccttttcctgggtctccaggggggtccacttgctcttctgaaatgcttttccatctgccccaggggcattggggtcctgtggtggccgttcccagaagggcttcagttcagctggggtatagaacccagggaggcaggactggtttatggagaacagagtctgctgggcttctggagccctgatttggagcttgggcattgaatctctaaggttgttcatggcctccagcatgaggtccaggacgtgatccttccggctcaccagggacttcagccacggcttctctgtggcctcctctctgctgctcacatccctatgcaggaggaagaggaagagcacaaaggcgcagcccaccatggccaggcgcaggggcatgtggcgtctgcggaggagcctcatcctccagaaccaaggggcaccccagctgcgtcagctctgagtcctgagcccaaccctggagatagcttgatacgttgtggtggccacaagctggggcctcagccctctgcagacgtctgggtctgcgatgattggccctggatgcaagtaaaagctgtttctcctttttgtcagcctgggaatctgaacaaccctccaagttccagaggtctgggctcctcattcatctcgtaagcgccaaggtggaggggggtcctaccgagggaggagctacaggccaccgcgaccagcagagagcgaaggcaggaggg

SEQ ID NO: 14625 - RNA, 3568 nt, Homo sapiens
  source 1..3568: mol_type = other RNA
gctgggattacaggcatgagccaccgtgcccggccctggctgttttcctatgctctgtggaggccagccagctagaaatgattagaatggaggaagagggaatgagaaggctggtggcgagtggtctagcgttcttgtggtgcagcggaaggagccctggctcagcattgaagaacgagcctcagtcttggctccagccatctgctagctatgggactacagacaagcccctttacctgtgtctcagttttcgtatctgtaaaataggcacagtggtttctgtcctgtctttctcacaggattactgtacagataaagtaagataaaggacacctgtcaaggagatatctgtaaacagttctacagacttcaggtaataatagcaagggaggatctcttagacctctgatctgtctgttagaatatactttttttttttttttttttcctgagatggagtttcgctcttgttgctcaggctggggtgcaatggtgctgtcttggctcactgcaacctctgcctcctgggttcgagtgattctcctgcctcagcctcccaagtagctgggactgcaggtgcgtgccatcatgcccagctaatttttgtacttttagtagagatggagtttcaccatgtagtccaggctggtttcaaacttctgacctcaggtgatccacctgccttggcctcccaaagtgctaggattacaggtgtgagccactgtgcccagccagaatatatcatttcactggactctgcaggtgctttggatgatcaaggaataggacatggctgtagaagtacttttcttcttcttttttgtttttttttgagacagagtcttacctgttgcccaggctggagtgcagtgacacaatcaaggctcactgtagcttcaacctccggggaacaagcaatcctcccacctcagccttctgagtagctgcgactacaggcataagccaccatacccagctttttttttttgccggggggagggtgggcgtagagatgggatcctcactatgttgctcaggccggtcttgaactcctgggctcaagccattctcccacattgtcttcccaaagtgctaggatttcaggcatgagccactgtgcccagcctgaagtacttttcttgaactcagcattgctgccctgaaccctcccccagctgccttccctactttgggagcctctatttctagaacaggaaaacgctaggctaaatatatgtcctaatggtctcttccatcggtgtgaaggaaagaaaatgggcccaatgttgttgcaaggattaggaaggtcctgccttgccacccagtgggtttagaaatccatctttacggcctccagagaagctggtgatcaggttcccagacatcagcaatcctgtttcctgaggagcttgtgggggctctctctggggatgatctgggtcctagacaaagagccacaactgatgggggtcactgggattgcagggggccatggctggctttttgtcctgggatgtcaggcaggtaccagatcctgagttcctgatgagctgatcctgggccaattcccattcctcgtccttggggacctggctattcttgccagtgaagtgacagctcccaaggcccagagcacccttgctgacatgtagacacagctgctttgcgatgttgtggcgaaggtccctctgagttgtgtactcaaagtactggttgccgccaaggccgtggcaggagtacatgatgaggggcttccccccgcggttgttctcacccacatccaggcattggttggtgccgaggttcttgatggcaccatagaaggtgggcgtcaggtcaggaacaaacatctctgggtagacattgtgcaggtaccaggaaaagttgtgacagtgcagttgttccctcagctgcagtcgttccgaaatgtcaccgaaggatttctcttgggccatctttgctgcctgcagatttctcctatagaaaatcttcttgtagctgtccatccagacctctgccaggcgcacttgattgcgagcaatgacactagtgcccttggggaaggtgtgggggctcttggtccggaacacatggcctacgacagagcaggggatgatctccagctggcccccacactgccacacccggaaggacatttccacgttctcccctccccagatctccatctgattatcataggtaccgatgtgctcaaagtaggacttggagatggagaagaggccaccagcaaacgtcggggatttgatggggtaggtttcatccttgcgcctctgcttctcatgtggaggaagtgtttcccagccgaaggtcaggctccagtcaaagttgcctcggctatggactctgcccctctggacgggcttggcgaactcaaaagtattaaggtcgatggtgacgatgtctgggctcaccaccactgtcttgtcctcagcgattcgagccaggaggggctccagccagccgtggaagcactcacagtgggcatccaggaacgtgagcacctccgcctgtgccacgctggcccccagcagccgggcggtgatcagccccttccgctcctcctgccgcaccaccctcaccacctgcagctgcttcacgtactgctccagcttctcctttaggtgctcctctgtgctggcatcatccaccagtatgatctccttgagcaagatggcaggggtggtgtgtaggacgctgtacactgttcgcagcagtgtggaccaggcttcgttgtggaacacaatgatcacgctggtggtggccagtggggggcagcgccggaacttctggtccacacactcaggtggtcgggtgtctggccccagggacctctgcagggagatccggtcgctggcaaaggcattgaaacagtgcttcttatagccttcttccttttcctgggtctccaggggggtccacttgctcttctgaaatgcttttccatctgccccaggggcattggggtcctgtggtggccgttcccagaagggcttcagttcagctggggtatagaacccagggaggcaggactggtttatggagaacagagtctgctgggcttctggagccctgatttggagcttgggcattgaatctctaaggttgttcatggcctccagcatgaggtccaggacgtgatccttccggctcaccagggacttcagccacggcttctctgtggcctcctctctgctgctcacatccctatgcaggaggaagaggaagagcacaaaggcgcagcccaccatggccaggcgcaggggcatgtggcgtctgcggaggagcctcatcctccagaaccaaggggcaccccagctgcgtcagctctgagtcctgagcccaaccctggagatagcttgatacgttgtggtggccacaagctggggcctcagccctctgcagacgtctgggtctgcgatgattggccctggatgcaagtaaaagctgtttctcctttttgtcagcctgggaatctgaacaactgtcgcgccgaggcaaagccgcagccgcgccgcggggtggctcccgggtttccccaccggacggc

SEQ ID NO: 14626 - RNA, 3932 nt, Homo sapiens
  source 1..3932: mol_type = other RNA
gctgggattacaggcatgagccaccgtgcccggccctggctgttttcctatgctctgtggaggccagccagctagaaatgattagaatggaggaagagggaatgagaaggctggtggcgagtggtctagcgttcttgtggtgcagcggaaggagccctggctcagcattgaagaacgagcctcagtcttggctccagccatctgctagctatgggactacagacaagcccctttacctgtgtctcagttttcgtatctgtaaaataggcacagtggtttctgtcctgtctttctcacaggattactgtacagataaagtaagataaaggacacctgtcaaggagatatctgtaaacagttctacagacttcaggtaataatagcaagggaggatctcttagacctctgatctgtctgttagaatatactttttttttttttttttttcctgagatggagtttcgctcttgttgctcaggctggggtgcaatggtgctgtcttggctcactgcaacctctgcctcctgggttcgagtgattctcctgcctcagcctcccaagtagctgggactgcaggtgcgtgccatcatgcccagctaatttttgtacttttagtagagatggagtttcaccatgtagtccaggctggtttcaaacttctgacctcaggtgatccacctgccttggcctcccaaagtgctaggattacaggtgtgagccactgtgcccagccagaatatatcatttcactggactctgcaggtgctttggatgatcaaggaataggacatggctgtagaagtacttttcttcttcttttttgtttttttttgagacagagtcttacctgttgcccaggctggagtgcagtgacacaatcaaggctcactgtagcttcaacctccggggaacaagcaatcctcccacctcagccttctgagtagctgcgactacaggcataagccaccatacccagctttttttttttgccggggggagggtgggcgtagagatgggatcctcactatgttgctcaggccggtcttgaactcctgggctcaagccattctcccacattgtcttcccaaagtgctaggatttcaggcatgagccactgtgcccagcctgaagtacttttcttgaactcagcattgctgccctgaaccctcccccagctgccttccctactttgggagcctctatttctagaacaggaaaacgctaggctaaatatatgtcctaatggtctcttccatcggtgtgaaggaaagaaaatgggcccaatgttgttgcaaggattaggaaggtcctgccttgccacccagtgggtttagaaatccatctttacggcctccagagaagctggtgatcaggttcccagacatcagcaatcctgtttcctgaggagcttgtgggggctctctctggggatgatctgggtcctagacaaagagccacaactgatgggggtcactgggattgcagggggccatggctggctttttgtcctgggatgtcaggcaggtaccagatcctgagttcctgatgagctgatcctgggccaattcccattcctcgtccttggggacctggctattcttgccagtgaagtgacagctcccaaggcccagagcacccttgctgacatgtagacacagctgctttgcgatgttgtggcgaaggtccctctgagttgtgtactcaaagtactggttgccgccaaggccgtggcaggagtacatgatgaggggcttccccccgcggttgttctcacccacatccaggcattggttggtgccgaggttcttgatggcaccatagaaggtgggcgtcaggtcaggaacaaacatctctgggtagacattgtgcaggtaccaggaaaagttgtgacagtgcagttgttccctcagctgcagtcgttccgaaatgtcaccgaaggatttctcttgggccatctttgctgcctgcagatttctcctatagaaaatcttcttgtagctgtccatccagacctctgccaggcgcacttgattgcgagcaatgacactagtgcccttggggaaggtgtgggggctcttggtccggaacacatggcctacgacagagcaggggatgatctccagctggcccccacactgccacacccggaaggacatttccacgttctcccctccccagatctccatctgattatcataggtaccgatgtgctcaaagtaggacttggagatggagaagaggccaccagcaaacgtcggggatttgatggggtaggtttcatccttgcgcctctgcttctcatgtggaggaagtgtttcccagccgaaggtcaggctccagtcaaagttgcctcggctatggactctgcccctctggacgggcttggcgaactcaaaagtattaaggtcgatggtgacgatgtctgggctcaccaccactgtcttgtcctcagcgattcgagccaggaggggctccagccagccgtggaagcactcacagtgggcatccaggaacgtgagcacctccgcctgtgccacgctggcccccagcagccgggcggtgatcagccccttccgctcctcctgccgcaccaccctcaccacctgcagctgcttcacgtactgctccagcttctcctttaggtgctcctctgtgctggcatcatccaccagtatgatctccttgagcaagatggcaggggtggtgtgtaggacgctgtacactgttcgcagcagtgtggaccaggcttcgttgtggaacacaatgatcacgctggtggtggccagtggggggcagcgccggaacttctggtccacacactcaggtggtcgggtgtctggccccagggacctctgcagggagatccggtcgctggcaaaggcattgaaacagtgcttcttatagccttcttccttttcctgggtctccaggggggtccacttgctcttctgaaatgcttttccatctgccccaggggcattggggtcctgtggtggccgttcccagaagggcttcagttcagctggggtatagaacccagggaggcaggactggtttatggagaacagagtctgctgggcttctggagccctgatttggagcttgggcattgaatctctaaggttgttcatggcctccagcatgaggtccaggacgtgatccttccggctcaccagggacttcagccacggcttctctgtggcctcctctctgctgctcacatccctatgcaggaggaagaggaagagcacaaaggcgcagcccaccatggccaggcgcaggggcatgtggcgtctgcggaggagcctcatcctccagaaccaaggggcaccccagctgcgtcagctctgagtcctgagcccaaccctggagatagcttgatacgttgtggtggccacaagctggggcctcagccctgtgagaagcagaatcaaagaggtacccttgagtgctgaaggagccggcatgcaggaaactcagcaaatgggggagggcaacatctgtgaagaaatctcacgggggcagaaatgggccgaacactaactggcgagtaggagtcagcgaggcgaggtgagcacatttcaggcagaaggcacagtacctgcaatggtcccctccaggaaggcctcctgactgattcactcagaatcacctaggttactccaactctttcatcctggcactgcctcgtggtccctcacagcagggcctgtttttgcttcttttattttcccctctgcagacgtctgggtctgcgatgattggccctggatgcaagtaaaagctgtttctcctttttgtcagcctgggaatctgaacaactccaccagcgaggcttctccttgctgtccccttctgctcaggcgcaacgtggcagggcaggaggaaacctctctgcaagagttgccgtaccagagcacatggggtggccc

SEQ ID NO: 14627 - RNA, 3887 nt, Homo sapiens
  source 1..3887: mol_type = other RNA
gctgggattacaggcatgagccaccgtgcccggccctggctgttttcctatgctctgtggaggccagccagctagaaatgattagaatggaggaagagggaatgagaaggctggtggcgagtggtctagcgttcttgtggtgcagcggaaggagccctggctcagcattgaagaacgagcctcagtcttggctccagccatctgctagctatgggactacagacaagcccctttacctgtgtctcagttttcgtatctgtaaaataggcacagtggtttctgtcctgtctttctcacaggattactgtacagataaagtaagataaaggacacctgtcaaggagatatctgtaaacagttctacagacttcaggtaataatagcaagggaggatctcttagacctctgatctgtctgttagaatatactttttttttttttttttttcctgagatggagtttcgctcttgttgctcaggctggggtgcaatggtgctgtcttggctcactgcaacctctgcctcctgggttcgagtgattctcctgcctcagcctcccaagtagctgggactgcaggtgcgtgccatcatgcccagctaatttttgtacttttagtagagatggagtttcaccatgtagtccaggctggtttcaaacttctgacctcaggtgatccacctgccttggcctcccaaagtgctaggattacaggtgtgagccactgtgcccagccagaatatatcatttcactggactctgcaggtgctttggatgatcaaggaataggacatggctgtagaagtacttttcttcttcttttttgtttttttttgagacagagtcttacctgttgcccaggctggagtgcagtgacacaatcaaggctcactgtagcttcaacctccggggaacaagcaatcctcccacctcagccttctgagtagctgcgactacaggcataagccaccatacccagctttttttttttgccggggggagggtgggcgtagagatgggatcctcactatgttgctcaggccggtcttgaactcctgggctcaagccattctcccacattgtcttcccaaagtgctaggatttcaggcatgagccactgtgcccagcctgaagtacttttcttgaactcagcattgctgccctgaaccctcccccagctgccttccctactttgggagcctctatttctagaacaggaaaacgctaggctaaatatatgtcctaatggtctcttccatcggtgtgaaggaaagaaaatgggcccaatgttgttgcaaggattaggaaggtcctgccttgccacccagtgggtttagaaatccatctttacggcctccagagaagctggtgatcaggttcccagacatcagcaatcctgtttcctgaggagcttgtgggggctctctctggggatgatctgggtcctagacaaagagccacaactgatgggggtcactgggattgcagggggccatggctggctttttgtcctgggatgtcaggcaggtaccagatcctgagttcctgatgagctgatcctgggccaattcccattcctcgtccttggggacctggctattcttgccagtgaagtgacagctcccaaggcccagagcacccttgctgacatgtagacacagctgctttgcgatgttgtggcgaaggtccctctgagttgtgtactcaaagtactggttgccgccaaggccgtggcaggagtacatgatgaggggcttccccccgcggttgttctcacccacatccaggcattggttggtgccgaggttcttgatggcaccatagaaggtgggcgtcaggtcaggaacaaacatctctgggtagacattgtgcaggtaccaggaaaagttgtgacagtgcagttgttccctcagctgcagtcgttccgaaatgtcaccgaaggatttctcttgggccatctttgctgcctgcagatttctcctatagaaaatcttcttgtagctgtccatccagacctctgccaggcgcacttgattgcgagcaatgacactagtgcccttggggaaggtgtgggggctcttggtccggaacacatggcctacgacagagcaggggatgatctccagctggcccccacactgccacacccggaaggacatttccacgttctcccctccccagatctccatctgattatcataggtaccgatgtgctcaaagtaggacttggagatggagaagaggccaccagcaaacgtcggggatttgatggggtaggtttcatccttgcgcctctgcttctcatgtggaggaagtgtttcccagccgaaggtcaggctccagtcaaagttgcctcggctatggactctgcccctctggacgggcttggcgaactcaaaagtattaaggtcgatggtgacgatgtctgggctcaccaccactgtcttgtcctcagcgattcgagccaggaggggctccagccagccgtggaagcactcacagtgggcatccaggaacgtgagcacctccgcctgtgccacgctggcccccagcagccgggcggtgatcagccccttccgctcctcctgccgcaccaccctcaccacctgcagctgcttcacgtactgctccagcttctcctttaggtgctcctctgtgctggcatcatccaccagtatgatctccttgagcaagatggcaggggtggtgtgtaggacgctgtacactgttcgcagcagtgtggaccaggcttcgttgtggaacacaatgatcacgctggtggtggccagtggggggcagcgccggaacttctggtccacacactcaggtggtcgggtgtctggccccagggacctctgcagggagatccggtcgctggcaaaggcattgaaacagtgcttcttatagccttcttccttttcctgggtctccaggggggtccacttgctcttctgaaatgcttttccatctgccccaggggcattggggtcctgtggtggccgttcccagaagggcttcagttcagctggggtatagaacccagggaggcaggactggtttatggagaacagagtctgctgggcttctggagccctgatttggagcttgggcattgaatctctaaggttgttcatggcctccagcatgaggtccaggacgtgatccttccggctcaccagggacttcagccacggcttctctgtggcctcctctctgctgctcacatccctatgcaggaggaagaggaagagcacaaaggcgcagcccaccatggccaggcgcaggggcatgtggcgtctgcggaggagcctcatcctccagaaccaaggggcaccccagctgcgtcagctctgagtcctgagcccaaccctggagatagcttgatacgttgtggtggccacaagctggggcctcagccctgtgagaagcagaatcaaagaggtacccttgagtgctgaaggagccggcatgcaggaaactcagcaaatgggggagggcaacatctgtgaagaaatctcacgggggcagaaatgggccgaacactaactggcgagtaggagtcagcgaggcgaggtgagcacatttcaggcagaaggcacagtacctgcaatggtcccctccaggaaggcctcctgactgattcactcagaatcacctaggttactccaactctttcatcctggcactgcctcgtggtccctcacagcagggcctgtttttgcttcttttattttcccctctgcagacgtctgggtctgcgatgattggccctggatgcaagtaaaagctgtttctcctttttgtcagcctgggaatctgaacaactgtcgcgccgaggcaaagccgcagccgcgccgcggggtggctcccgggtttccccaccggacggc

SEQ ID NO: 14628 - RNA, 3758 nt, Homo sapiens
  source 1..3758: mol_type = other RNA
gctgggattacaggcatgagccaccgtgcccggccctggctgttttcctatgctctgtggaggccagccagctagaaatgattagaatggaggaagagggaatgagaaggctggtggcgagtggtctagcgttcttgtggtgcagcggaaggagccctggctcagcattgaagaacgagcctcagtcttggctccagccatctgctagctatgggactacagacaagcccctttacctgtgtctcagttttcgtatctgtaaaataggcacagtggtttctgtcctgtctttctcacaggattactgtacagataaagtaagataaaggacacctgtcaaggagatatctgtaaacagttctacagacttcaggtaataatagcaagggaggatctcttagacctctgatctgtctgttagaatatactttttttttttttttttttcctgagatggagtttcgctcttgttgctcaggctggggtgcaatggtgctgtcttggctcactgcaacctctgcctcctgggttcgagtgattctcctgcctcagcctcccaagtagctgggactgcaggtgcgtgccatcatgcccagctaatttttgtacttttagtagagatggagtttcaccatgtagtccaggctggtttcaaacttctgacctcaggtgatccacctgccttggcctcccaaagtgctaggattacaggtgtgagccactgtgcccagccagaatatatcatttcactggactctgcaggtgctttggatgatcaaggaataggacatggctgtagaagtacttttcttcttcttttttgtttttttttgagacagagtcttacctgttgcccaggctggagtgcagtgacacaatcaaggctcactgtagcttcaacctccggggaacaagcaatcctcccacctcagccttctgagtagctgcgactacaggcataagccaccatacccagctttttttttttgccggggggagggtgggcgtagagatgggatcctcactatgttgctcaggccggtcttgaactcctgggctcaagccattctcccacattgtcttcccaaagtgctaggatttcaggcatgagccactgtgcccagcctgaagtacttttcttgaactcagcattgctgccctgaaccctcccccagctgccttccctactttgggagcctctatttctagaacaggaaaacgctaggctaaatatatgtcctaatggtctcttccatcggtgtgaaggaaagaaaatgggcccaatgttgttgcaaggattaggaaggtcctgccttgccacccagtgggtttagaaatccatctttacggcctccagagaagctggtgatcaggttcccagacatcagcaatcctgtttcctgaggagcttgtgggggctctctctggggatgatctgggtcctagacaaagagccacaactgatgggggtcactgggattgcagggggccatggctggctttttgtcctgggatgtcaggcaggtaccagatcctgagttcctgatgagctgatcctgggccaattcccattcctcgtccttggggacctggctattcttgccagtgaagtgacagctcccaaggcccagagcacccttgctgacatgtagacacagctgctttgcgatgttgtggcgaaggtccctctgagttgtgtactcaaagtactggttgccgccaaggccgtggcaggagtacatgatgaggggcttccccccgcggttgttctcacccacatccaggcattggttggtgccgaggttcttgatggcaccatagaaggtgggcgtcaggtcaggaacaaacatctctgggtagacattgtgcaggtaccaggaaaagttgtgacagtgcagttgttccctcagctgcagtcgttccgaaatgtcaccgaaggatttctcttgggccatctttgctgcctgcagatttctcctatagaaaatcttcttgtagctgtccatccagacctctgccaggcgcacttgattgcgagcaatgacactagtgcccttggggaaggtgtgggggctcttggtccggaacacatggcctacgacagagcaggggatgatctccagctggcccccacactgccacacccggaaggacatttccacgttctcccctccccagatctccatctgattatcataggtaccgatgtgctcaaagtaggacttggagatggagaagaggccaccagcaaacgtcggggatttgatggggtaggtttcatccttgcgcctctgcttctcatgtggaggaagtgtttcccagccgaaggtcaggctccagtcaaagttgcctcggctatggactctgcccctctggacgggcttggcgaactcaaaagtattaaggtcgatggtgacgatgtctgggctcaccaccactgtcttgtcctcagcgattcgagccaggaggggctccagccagccgtggaagcactcacagtgggcatccaggaacgtgagcacctccgcctgtgccacgctggcccccagcagccgggcggtgatcagccccttccgctcctcctgccgcaccaccctcaccacctgcagctgcttcacgtactgctccagcttctcctttaggtgctcctctgtgctggcatcatccaccagtatgatctccttgagcaagatggcaggggtggtgtgtaggacgctgtacactgttcgcagcagtgtggaccaggcttcgttgtggaacacaatgatcacgctggtggtggccagtggggggcagcgccggaacttctggtccacacactcaggtggtcgggtgtctggccccagggacctctgcagggagatccggtcgctggcaaaggcattgaaacagtgcttcttatagccttcttccttttcctgggtctccaggggggtccacttgctcttctgaaatgcttttccatctgccccaggggcattggggtcctgtggtggccgttcccagaagggcttcagttcagctggggtatagaacccagggaggcaggactggtttatggagaacagagtctgctgggcttctggagccctgatttggagcttgggcattgaatctctaaggttgttcatggcctccagcatgaggtccaggacgtgatccttccggctcaccagggacttcagccacggcttctctgtggcctcctctctgctgctcacatccctatgcaggaggaagaggaagagcacaaaggcgcagcccaccatggccaggcgcaggggcatgtggcgtctgcggaggagcctcatcctccagaaccaaggggcaccccagctgcgtcagctctgagtcctgagcccaaccctggagatagcttgatacgttgtggtggccacaagctggggcctcagccctgtgagaagcagaatcaaagaggtacccttgagtgctgaaggagccggcatgcaggaaactcagcaaatgggggagggcaacatctgtgaagaaatctcacgggggcagaaatgggccgaacactaactggcgagtaggagtcagcgaggcgaggtgagcacatttcaggcagaaggcacagtacctgcaatggtcccctccaggaaggcctcctgactgattcactcagaatcacctaggttactccaactctttcatcctggcactgcctcgtggtccctcacagcagggcctgtttttgcttcttttattttcccgagggaggagctacaggccaccgc

SEQ ID NO: 14629 - RNA, 3845 nt, Homo sapiens
  source 1..3845: mol_type = other RNA
gctgggattacaggcatgagccaccgtgcccggccctggctgttttcctatgctctgtggaggccagccagctagaaatgattagaatggaggaagagggaatgagaaggctggtggcgagtggtctagcgttcttgtggtgcagcggaaggagccctggctcagcattgaagaacgagcctcagtcttggctccagccatctgctagctatgggactacagacaagcccctttacctgtgtctcagttttcgtatctgtaaaataggcacagtggtttctgtcctgtctttctcacaggattactgtacagataaagtaagataaaggacacctgtcaaggagatatctgtaaacagttctacagacttcaggtaataatagcaagggaggatctcttagacctctgatctgtctgttagaatatactttttttttttttttttttcctgagatggagtttcgctcttgttgctcaggctggggtgcaatggtgctgtcttggctcactgcaacctctgcctcctgggttcgagtgattctcctgcctcagcctcccaagtagctgggactgcaggtgcgtgccatcatgcccagctaatttttgtacttttagtagagatggagtttcaccatgtagtccaggctggtttcaaacttctgacctcaggtgatccacctgccttggcctcccaaagtgctaggattacaggtgtgagccactgtgcccagccagaatatatcatttcactggactctgcaggtgctttggatgatcaaggaataggacatggctgtagaagtacttttcttcttcttttttgtttttttttgagacagagtcttacctgttgcccaggctggagtgcagtgacacaatcaaggctcactgtagcttcaacctccggggaacaagcaatcctcccacctcagccttctgagtagctgcgactacaggcataagccaccatacccagctttttttttttgccggggggagggtgggcgtagagatgggatcctcactatgttgctcaggccggtcttgaactcctgggctcaagccattctcccacattgtcttcccaaagtgctaggatttcaggcatgagccactgtgcccagcctgaagtacttttcttgaactcagcattgctgccctgaaccctcccccagctgccttccctactttgggagcctctatttctagaacaggaaaacgctaggctaaatatatgtcctaatggtctcttccatcggtgtgaaggaaagaaaatgggcccaatgttgttgcaaggattaggaaggtcctgccttgccacccagtgggtttagaaatccatctttacggcctccagagaagctggtgatcaggttcccagacatcagcaatcctgtttcctgaggagcttgtgggggctctctctggggatgatctgggtcctagacaaagagccacaactgatgggggtcactgggattgcagggggccatggctggctttttgtcctgggatgtcaggcaggtaccagatcctgagttcctgatgagctgatcctgggccaattcccattcctcgtccttggggacctggctattcttgccagtgaagtgacagctcccaaggcccagagcacccttgctgacatgtagacacagctgctttgcgatgttgtggcgaaggtccctctgagttgtgtactcaaagtactggttgccgccaaggccgtggcaggagtacatgatgaggggcttccccccgcggttgttctcacccacatccaggcattggttggtgccgaggttcttgatggcaccatagaaggtgggcgtcaggtcaggaacaaacatctctgggtagacattgtgcaggtaccaggaaaagttgtgacagtgcagttgttccctcagctgcagtcgttccgaaatgtcaccgaaggatttctcttgggccatctttgctgcctgcagatttctcctatagaaaatcttcttgtagctgtccatccagacctctgccaggcgcacttgattgcgagcaatgacactagtgcccttggggaaggtgtgggggctcttggtccggaacacatggcctacgacagagcaggggatgatctccagctggcccccacactgccacacccggaaggacatttccacgttctcccctccccagatctccatctgattatcataggtaccgatgtgctcaaagtaggacttggagatggagaagaggccaccagcaaacgtcggggatttgatggggtaggtttcatccttgcgcctctgcttctcatgtggaggaagtgtttcccagccgaaggtcaggctccagtcaaagttgcctcggctatggactctgcccctctggacgggcttggcgaactcaaaagtattaaggtcgatggtgacgatgtctgggctcaccaccactgtcttgtcctcagcgattcgagccaggaggggctccagccagccgtggaagcactcacagtgggcatccaggaacgtgagcacctccgcctgtgccacgctggcccccagcagccgggcggtgatcagccccttccgctcctcctgccgcaccaccctcaccacctgcagctgcttcacgtactgctccagcttctcctttaggtgctcctctgtgctggcatcatccaccagtatgatctccttgagcaagatggcaggggtggtgtgtaggacgctgtacactgttcgcagcagtgtggaccaggcttcgttgtggaacacaatgatcacgctggtggtggccagtggggggcagcgccggaacttctggtccacacactcaggtggtcgggtgtctggccccagggacctctgcagggagatccggtcgctggcaaaggcattgaaacagtgcttcttatagccttcttccttttcctgggtctccaggggggtccacttgctcttctgaaatgcttttccatctgccccaggggcattggggtcctgtggtggccgttcccagaagggcttcagttcagctggggtatagaacccagggaggcaggactggtttatggagaacagagtctgctgggcttctggagccctgatttggagcttgggcattgaatctctaaggttgttcatggcctccagcatgaggtccaggacgtgatccttccggctcaccagggacttcagccacggcttctctgtggcctcctctctgctgctcacatccctatgcaggaggaagaggaagagcacaaaggcgcagcccaccatggccaggcgcaggggcatgtggcgtctgcggaggagcctcatcctccagaaccaaggggcaccccagctgcgtcagctctgagtcctgagcccaaccctggagatagcttgatacgttgtggtggccacaagctggggcctcagccctgtgagaagcagaatcaaagaggtacccttgagtgctgaaggagccggcatgcaggaaactcagcaaatgggggagggcaacatctgtgaagaaatctcacgggggcagaaatgggccgaacactaactggcgagtaggagtcagcgaggcgaggtgagcacatttcaggcagaaggcacagtacctgcaatggtcccctccaggaaggcctcctgactgattcactcagaatcacctaggttactccaactctttcatcctggcactgcctcgtggtccctcacagcagggcctgtttttgcttcttttattttccctccaccagcgaggcttctccttgctgtccccttctgctcaggcgcaacgtggcagggcaggaggaaacctctctgcaagagttgccgtaccagagcacatggggtggcccg

SEQ ID NO: 14630 - RNA, 3814 nt, Homo sapiens
  source 1..3814: mol_type = other RNA
gctgggattacaggcatgagccaccgtgcccggccctggctgttttcctatgctctgtggaggccagccagctagaaatgattagaatggaggaagagggaatgagaaggctggtggcgagtggtctagcgttcttgtggtgcagcggaaggagccctggctcagcattgaagaacgagcctcagtcttggctccagccatctgctagctatgggactacagacaagcccctttacctgtgtctcagttttcgtatctgtaaaataggcacagtggtttctgtcctgtctttctcacaggattactgtacagataaagtaagataaaggacacctgtcaaggagatatctgtaaacagttctacagacttcaggtaataatagcaagggaggatctcttagacctctgatctgtctgttagaatatactttttttttttttttttttcctgagatggagtttcgctcttgttgctcaggctggggtgcaatggtgctgtcttggctcactgcaacctctgcctcctgggttcgagtgattctcctgcctcagcctcccaagtagctgggactgcaggtgcgtgccatcatgcccagctaatttttgtacttttagtagagatggagtttcaccatgtagtccaggctggtttcaaacttctgacctcaggtgatccacctgccttggcctcccaaagtgctaggattacaggtgtgagccactgtgcccagccagaatatatcatttcactggactctgcaggtgctttggatgatcaaggaataggacatggctgtagaagtacttttcttcttcttttttgtttttttttgagacagagtcttacctgttgcccaggctggagtgcagtgacacaatcaaggctcactgtagcttcaacctccggggaacaagcaatcctcccacctcagccttctgagtagctgcgactacaggcataagccaccatacccagctttttttttttgccggggggagggtgggcgtagagatgggatcctcactatgttgctcaggccggtcttgaactcctgggctcaagccattctcccacattgtcttcccaaagtgctaggatttcaggcatgagccactgtgcccagcctgaagtacttttcttgaactcagcattgctgccctgaaccctcccccagctgccttccctactttgggagcctctatttctagaacaggaaaacgctaggctaaatatatgtcctaatggtctcttccatcggtgtgaaggaaagaaaatgggcccaatgttgttgcaaggattaggaaggtcctgccttgccacccagtgggtttagaaatccatctttacggcctccagagaagctggtgatcaggttcccagacatcagcaatcctgtttcctgaggagcttgtgggggctctctctggggatgatctgggtcctagacaaagagccacaactgatgggggtcactgggattgcagggggccatggctggctttttgtcctgggatgtcaggcaggtaccagatcctgagttcctgatgagctgatcctgggccaattcccattcctcgtccttggggacctggctattcttgccagtgaagtgacagctcccaaggcccagagcacccttgctgacatgtagacacagctgctttgcgatgttgtggcgaaggtccctctgagttgtgtactcaaagtactggttgccgccaaggccgtggcaggagtacatgatgaggggcttccccccgcggttgttctcacccacatccaggcattggttggtgccgaggttcttgatggcaccatagaaggtgggcgtcaggtcaggaacaaacatctctgggtagacattgtgcaggtaccaggaaaagttgtgacagtgcagttgttccctcagctgcagtcgttccgaaatgtcaccgaaggatttctcttgggccatctttgctgcctgcagatttctcctatagaaaatcttcttgtagctgtccatccagacctctgccaggcgcacttgattgcgagcaatgacactagtgcccttggggaaggtgtgggggctcttggtccggaacacatggcctacgacagagcaggggatgatctccagctggcccccacactgccacacccggaaggacatttccacgttctcccctccccagatctccatctgattatcataggtaccgatgtgctcaaagtaggacttggagatggagaagaggccaccagcaaacgtcggggatttgatggggtaggtttcatccttgcgcctctgcttctcatgtggaggaagtgtttcccagccgaaggtcaggctccagtcaaagttgcctcggctatggactctgcccctctggacgggcttggcgaactcaaaagtattaaggtcgatggtgacgatgtctgggctcaccaccactgtcttgtcctcagcgattcgagccaggaggggctccagccagccgtggaagcactcacagtgggcatccaggaacgtgagcacctccgcctgtgccacgctggcccccagcagccgggcggtgatcagccccttccgctcctcctgccgcaccaccctcaccacctgcagctgcttcacgtactgctccagcttctcctttaggtgctcctctgtgctggcatcatccaccagtatgatctccttgagcaagatggcaggggtggtgtgtaggacgctgtacactgttcgcagcagtgtggaccaggcttcgttgtggaacacaatgatcacgctggtggtggccagtggggggcagcgccggaacttctggtccacacactcaggtggtcgggtgtctggccccagggacctctgcagggagatccggtcgctggcaaaggcattgaaacagtgcttcttatagccttcttccttttcctgggtctccaggggggtccacttgctcttctgaaatgcttttccatctgccccaggggcattggggtcctgtggtggccgttcccagaagggcttcagttcagctggggtatagaacccagggaggcaggactggtttatggagaacagagtctgctgggcttctggagccctgatttggagcttgggcattgaatctctaaggttgttcatggcctccagcatgaggtccaggacgtgatccttccggctcaccagggacttcagccacggcttctctgtggcctcctctctgctgctcacatccctatgcaggaggaagaggaagagcacaaaggcgcagcccaccatggccaggcgcaggggcatgtggcgtctgcggaggagcctcatcctccagaaccaaggggcaccccagctgcgtcagctctgagtcctgagcccaaccctggagatagcttgatacgttgtggtggccacaagctggggcctcagccctgtgagaagcagaatcaaagaggtacccttgagtgctgaaggagccggcatgcaggaaactcagcaaatgggggagggcaacatctgtgaagaaatctcacgggggcagaaatgggccgaacactaactggcgagtaggagtcagcgaggcgaggtgagcacatttcaggcagaaggcacagtacctgcaatggtcccctccaggaaggcctcctgactgattcactcagaatcacctaggttactccaactctttcatcctggcactgcctcgtggtccctcacagcagggcctgtttttgcttcttttattttccctgtcgcgccgaggcaaagccgcagccgcgccgcggggtggctcccgggtttccccaccggacggccgggagggtgggacc

SEQ ID NO: 14631 - RNA, 3859 nt, Homo sapiens
  source 1..3859: mol_type = other RNA
gctgggattacaggcatgagccaccgtgcccggccctggctgttttcctatgctctgtggaggccagccagctagaaatgattagaatggaggaagagggaatgagaaggctggtggcgagtggtctagcgttcttgtggtgcagcggaaggagccctggctcagcattgaagaacgagcctcagtcttggctccagccatctgctagctatgggactacagacaagcccctttacctgtgtctcagttttcgtatctgtaaaataggcacagtggtttctgtcctgtctttctcacaggattactgtacagataaagtaagataaaggacacctgtcaaggagatatctgtaaacagttctacagacttcaggtaataatagcaagggaggatctcttagacctctgatctgtctgttagaatatactttttttttttttttttttcctgagatggagtttcgctcttgttgctcaggctggggtgcaatggtgctgtcttggctcactgcaacctctgcctcctgggttcgagtgattctcctgcctcagcctcccaagtagctgggactgcaggtgcgtgccatcatgcccagctaatttttgtacttttagtagagatggagtttcaccatgtagtccaggctggtttcaaacttctgacctcaggtgatccacctgccttggcctcccaaagtgctaggattacaggtgtgagccactgtgcccagccagaatatatcatttcactggactctgcaggtgctttggatgatcaaggaataggacatggctgtagaagtacttttcttcttcttttttgtttttttttgagacagagtcttacctgttgcccaggctggagtgcagtgacacaatcaaggctcactgtagcttcaacctccggggaacaagcaatcctcccacctcagccttctgagtagctgcgactacaggcataagccaccatacccagctttttttttttgccggggggagggtgggcgtagagatgggatcctcactatgttgctcaggccggtcttgaactcctgggctcaagccattctcccacattgtcttcccaaagtgctaggatttcaggcatgagccactgtgcccagcctgaagtacttttcttgaactcagcattgctgccctgaaccctcccccagctgccttccctactttgggagcctctatttctagaacaggaaaacgctaggctaaatatatgtcctaatggtctcttccatcggtgtgaaggaaagaaaatgggcccaatgttgttgcaaggattaggaaggtcctgccttgccacccagtgggtttagaaatccatctttacggcctccagagaagctggtgatcaggttcccagacatcagcaatcctgtttcctgaggagcttgtgggggctctctctggggatgatctgggtcctagacaaagagccacaactgatgggggtcactgggattgcagggggccatggctggctttttgtcctgggatgtcaggcaggtaccagatcctgagttcctgatgagctgatcctgggccaattcccattcctcgtccttggggacctggctattcttgccagtgaagtgacagctcccaaggcccagagcacccttgctgacatgtagacacagctgctttgcgatgttgtggcgaaggtccctctgagttgtgtactcaaagtactggttgccgccaaggccgtggcaggagtacatgatgaggggcttccccccgcggttgttctcacccacatccaggcattggttggtgccgaggttcttgatggcaccatagaaggtgggcgtcaggtcaggaacaaacatctctgggtagacattgtgcaggtaccaggaaaagttgtgacagtgcagttgttccctcagctgcagtcgttccgaaatgtcaccgaaggatttctcttgggccatctttgctgcctgcagatttctcctatagaaaatcttcttgtagctgtccatccagacctctgccaggcgcacttgattgcgagcaatgacactagtgcccttggggaaggtgtgggggctcttggtccggaacacatggcctacgacagagcaggggatgatctccagctggcccccacactgccacacccggaaggacatttccacgttctcccctccccagatctccatctgattatcataggtaccgatgtgctcaaagtaggacttggagatggagaagaggccaccagcaaacgtcggggatttgatggggtaggtttcatccttgcgcctctgcttctcatgtggaggaagtgtttcccagccgaaggtcaggctccagtcaaagttgcctcggctatggactctgcccctctggacgggcttggcgaactcaaaagtattaaggtcgatggtgacgatgtctgggctcaccaccactgtcttgtcctcagcgattcgagccaggaggggctccagccagccgtggaagcactcacagtgggcatccaggaacgtgagcacctccgcctgtgccacgctggcccccagcagccgggcggtgatcagccccttccgctcctcctgccgcaccaccctcaccacctgcagctgcttcacgtactgctccagcttctcctttaggtgctcctctgtgctggcatcatccaccagtatgatctccttgagcaagatggcaggggtggtgtgtaggacgctgtacactgttcgcagcagtgtggaccaggcttcgttgtggaacacaatgatcacgctggtggtggccagtggggggcagcgccggaacttctggtccacacactcaggtggtcgggtgtctggccccagggacctctgcagggagatccggtcgctggcaaaggcattgaaacagtgcttcttatagccttcttccttttcctgggtctccaggggggtccacttgctcttctgaaatgcttttccatctgccccaggggcattggggtcctgtggtggccgttcccagaagggcttcagttcagctggggtatagaacccagggaggcaggactggtttatggagaacagagtctgctgggcttctggagccctgatttggagcttgggcattgaatctctaaggttgttcatggcctccagcatgaggtccaggacgtgatccttccggctcaccagggacttcagccacggcttctctgtggcctcctctctgctgctcacatccctatgcaggaggaagaggaagagcacaaaggcgcagcccaccatggccaggcgcaggggcatgtggcgtctgcggaggagcctcatcctccagaaccaaggggcaccccagctgcgtcagctctgagtcctgagcccaaccctggagatagcttgatacgttgtggtggccacaagctggggcctcagcccttgagtgctgaaggagccggcatgcaggaaactcagcaaatgggggagggcaacatctgtgaagaaatctcacgggggcagaaatgggccgaacactaactggcgagtaggagtcagcgaggcgaggtgagcacatttcaggcagaaggcacagtacctgcaatggtcccctccaggaaggcctcctgactgattcactcagaatcacctaggttactccaactctttcatcctggcactgcctcgtggtccctcacagcagggcctgtttttgcttcttttattttcccctctgcagacgtctgggtctgcgatgattggccctggatgcaagtaaaagctgtttctcctttttgtcagcctgggaatctgaacaactgtcgcgccgaggcaaagccgcagccgcgccgcggggtggctcccgggtttccccaccggacggc

SEQ ID NO: 14632 - RNA, 3466 nt, Homo sapiens
  source 1..3466: mol_type = other RNA
gctgggattacaggcatgagccaccgtgcccggccctggctgttttcctatgctctgtggaggccagccagctagaaatgattagaatggaggaagagggaatgagaaggctggtggcgagtggtctagcgttcttgtggtgcagcggaaggagccctggctcagcattgaagaacgagcctcagtcttggctccagccatctgctagctatgggactacagacaagcccctttacctgtgtctcagttttcgtatctgtaaaataggcacagtggtttctgtcctgtctttctcacaggattactgtacagataaagtaagataaaggacacctgtcaaggagatatctgtaaacagttctacagacttcaggtaataatagcaagggaggatctcttagacctctgatctgtctgttagaatatactttttttttttttttttttcctgagatggagtttcgctcttgttgctcaggctggggtgcaatggtgctgtcttggctcactgcaacctctgcctcctgggttcgagtgattctcctgcctcagcctcccaagtagctgggactgcaggtgcgtgccatcatgcccagctaatttttgtacttttagtagagatggagtttcaccatgtagtccaggctggtttcaaacttctgacctcaggtgatccacctgccttggcctcccaaagtgctaggattacaggtgtgagccactgtgcccagccagaatatatcatttcactggactctgcaggtgctttggatgatcaaggaataggacatggctgtagaagtacttttcttcttcttttttgtttttttttgagacagagtcttacctgttgcccaggctggagtgcagtgacacaatcaaggctcactgtagcttcaacctccggggaacaagcaatcctcccacctcagccttctgagtagctgcgactacaggcataagccaccatacccagctttttttttttgccggggggagggtgggcgtagagatgggatcctcactatgttgctcaggccggtcttgaactcctgggctcaagccattctcccacattgtcttcccaaagtgctaggatttcaggcatgagccactgtgcccagcctgaagtacttttcttgaactcagcattgctgccctgaaccctcccccagctgccttccctactttgggagcctctatttctagaacaggaaaacgctaggctaaatatatgtcctaatggtctcttccatcggtgtgaaggaaagaaaatgggcccaatgttgttgcaaggattaggaaggtcctgccttgccacccagtgggtttagaaatccatctttacggcctccagagaagctggtgatcaggttcccagacatcagcaatcctgtttcctgaggagcttgtgggggctctctctggggatgatctgggtcctagacaaagagccacaactgatgggggtcactgggattgcagggggccatggctggctttttgtcctgggatgtcaggcaggtaccagatcctgagttcctgatgagctgatcctgggccaattcccattcctcgtccttggggacctggctattcttgccagtgaagtgacagctcccaaggcccagagcacccttgctgacatgtagacacagctgctttgcgatgttgtggcgaaggtccctctgagttgtgtactcaaagtactggttgccgccaaggccgtggcaggagtacatgatgaggggcttccccccgcggttgttctcacccacatccaggcattggttggtgccgaggttcttgatggcaccatagaaggtgggcgtcaggtcaggaacaaacatctctgggtagacattgtgcaggtaccaggaaaagttgtgacagtgcagttgttccctcagctgcagtcgttccgaaatgtcaccgaaggatttctcttgggccatctttgctgcctgcagatttctcctatagaaaatcttcttgtagctgtccatccagacctctgccaggcgcacttgattgcgagcaatgacactagtgcccttggggaaggtgtgggggctcttggtccggaacacatggcctacgacagagcaggggatgatctccagctggcccccacactgccacacccggaaggacatttccacgttctcccctccccagatctccatctgattatcataggtaccgatgtgctcaaagtaggacttggagatggagaagaggccaccagcaaacgtcggggatttgatggggtaggtttcatccttgcgcctctgcttctcatgtggaggaagtgtttcccagccgaaggtcaggctccagtcaaagttgcctcggctatggactctgcccctctggacgggcttggcgaactcaaaagtattaaggtcgatggtgacgatgtctgggctcaccaccactgtcttgtcctcagcgattcgagccaggaggggctccagccagccgtggaagcactcacagtgggcatccaggaacgtgagcacctccgcctgtgccacgctggcccccagcagccgggcggtgatcagccccttccgctcctcctgccgcaccaccctcaccacctgcagctgcttcacgtactgctccagcttctcctttaggtgctcctctgtgctggcatcatccaccagtatgatctccttgagcaagatggcaggggtggtgtgtaggacgctgtacactgttcgcagcagtgtggaccaggcttcgttgtggaacacaatgatcacgctggtggtggccagtggggggcagcgccggaacttctggtccacacactcaggtggtcgggtgtctggccccagggacctctgcagggagatccggtcgctggcaaaggcattgaaacagtgcttcttatagccttcttccttttcctgggtctccaggggggtccacttgctcttctgaaatgcttttccatctgccccaggggcattggggtcctgtggtggccgttcccagaagggcttcagttcagctggggtatagaacccagggaggcaggactggtttatggagaacagagtctgctgggcttctggagccctgatttggagcttgggcattgaatctctaaggttgttcatggcctccagcatgaggtccaggacgtgatccttccggctcaccagggacttcagccacggcttctctgtggcctcctctctgctgctcacatccctatgcaggaggaagaggaagagcacaaaggcgcagcccaccatggccaggcgcaggggcatgtggcgtctgcggaggagcctcatcctccagaaccaaggggcaccccagctgcgtcagctctgagtcctgagcccaaccctggagatagcttgatacgttgtggtggccacaagctggggcctcagcctgtcgcgccgaggcaaagccgcagccgcgccgcggggtggctcccgggttt

SEQ ID NO: 14633 - RNA, 3828 nt, Homo sapiens
  source 1..3828: mol_type = other RNA
gctgggattacaggcatgagccaccgtgcccggccctggctgttttcctatgctctgtggaggccagccagctagaaatgattagaatggaggaagagggaatgagaaggctggtggcgagtggtctagcgttcttgtggtgcagcggaaggagccctggctcagcattgaagaacgagcctcagtcttggctccagccatctgctagctatgggactacagacaagcccctttacctgtgtctcagttttcgtatctgtaaaataggcacagtggtttctgtcctgtctttctcacaggattactgtacagataaagtaagataaaggacacctgtcaaggagatatctgtaaacagttctacagacttcaggtaataatagcaagggaggatctcttagacctctgatctgtctgttagaatatactttttttttttttttttttcctgagatggagtttcgctcttgttgctcaggctggggtgcaatggtgctgtcttggctcactgcaacctctgcctcctgggttcgagtgattctcctgcctcagcctcccaagtagctgggactgcaggtgcgtgccatcatgcccagctaatttttgtacttttagtagagatggagtttcaccatgtagtccaggctggtttcaaacttctgacctcaggtgatccacctgccttggcctcccaaagtgctaggattacaggtgtgagccactgtgcccagccagaatatatcatttcactggactctgcaggtgctttggatgatcaaggaataggacatggctgtagaagtacttttcttcttcttttttgtttttttttgagacagagtcttacctgttgcccaggctggagtgcagtgacacaatcaaggctcactgtagcttcaacctccggggaacaagcaatcctcccacctcagccttctgagtagctgcgactacaggcataagccaccatacccagctttttttttttgccggggggagggtgggcgtagagatgggatcctcactatgttgctcaggccggtcttgaactcctgggctcaagccattctcccacattgtcttcccaaagtgctaggatttcaggcatgagccactgtgcccagcctgaagtacttttcttgaactcagcattgctgccctgaaccctcccccagctgccttccctactttgggagcctctatttctagaacaggaaaacgctaggctaaatatatgtcctaatggtctcttccatcggtgtgaaggaaagaaaatgggcccaatgttgttgcaaggattaggaaggtcctgccttgccacccagtgggtttagaaatccatctttacggcctccagagaagctggtgatcaggttcccagacatcagcaatcctgtttcctgaggagcttgtgggggctctctctggggatgatctgggtcctagacaaagagccacaactgatgggggtcactgggattgcagggggccatggctggctttttgtcctgggatgtcaggcaggtaccagatcctgagttcctgatgagctgatcctgggccaattcccattcctcgtccttggggacctggctattcttgccagtgaagtgacagctcccaaggcccagagcacccttgctgacatgtagacacagctgctttgcgatgttgtggcgaaggtccctctgagttgtgtactcaaagtactggttgccgccaaggccgtggcaggagtacatgatgaggggcttccccccgcggttgttctcacccacatccaggcattggttggtgccgaggttcttgatggcaccatagaaggtgggcgtcaggtcaggaacaaacatctctgggtagacattgtgcaggtaccaggaaaagttgtgacagtgcagttgttccctcagctgcagtcgttccgaaatgtcaccgaaggatttctcttgggccatctttgctgcctgcagatttctcctatagaaaatcttcttgtagctgtccatccagacctctgccaggcgcacttgattgcgagcaatgacactagtgcccttggggaaggtgtgggggctcttggtccggaacacatggcctacgacagagcaggggatgatctccagctggcccccacactgccacaccgatgtgctcaaagtaggacttggagatggagaagaggccaccagcaaacgtcggggatttgatggggtaggtttcatccttgcgcctctgcttctcatgtggaggaagtgtttcccagccgaaggtcaggctccagtcaaagttgcctcggctatggactctgcccctctggacgggcttggcgaactcaaaagtattaaggtcgatggtgacgatgtctgggctcaccaccactgtcttgtcctcagcgattcgagccaggaggggctccagccagccgtggaagcactcacagtgggcatccaggaacgtgagcacctccgcctgtgccacgctggcccccagcagccgggcggtgatcagccccttccgctcctcctgccgcaccaccctcaccacctgcagctgcttcacgtactgctccagcttctcctttaggtgctcctctgtgctggcatcatccaccagtatgatctccttgagcaagatggcaggggtggtgtgtaggacgctgtacactgttcgcagcagtgtggaccaggcttcgttgtggaacacaatgatcacgctggtggtggccagtggggggcagcgccggaacttctggtccacacactcaggtggtcgggtgtctggccccagggacctctgcagggagatccggtcgctggcaaaggcattgaaacagtgcttcttatagccttcttccttttcctgggtctccaggggggtccacttgctcttctgaaatgcttttccatctgccccaggggcattggggtcctgtggtggccgttcccagaagggcttcagttcagctggggtatagaacccagggaggcaggactggtttatggagaacagagtctgctgggcttctggagccctgatttggagcttgggcattgaatctctaaggttgttcatggcctccagcatgaggtccaggacgtgatccttccggctcaccagggacttcagccacggcttctctgtggcctcctctctgctgctcacatccctatgcaggaggaagaggaagagcacaaaggcgcagcccaccatggccaggcgcaggggcatgtggcgtctgcggaggagcctcatcctccagaaccaaggggcaccccagctgcgtcagctctgagtcctgagcccaaccctggagatagcttgatacgttgtggtggccacaagctggggcctcagccctgtgagaagcagaatcaaagaggtacccttgagtgctgaaggagccggcatgcaggaaactcagcaaatgggggagggcaacatctgtgaagaaatctcacgggggcagaaatgggccgaacactaactggcgagtaggagtcagcgaggcgaggtgagcacatttcaggcagaaggcacagtacctgcaatggtcccctccaggaaggcctcctgactgattcactcagaatcacctaggttactccaactctttcatcctggcactgcctcgtggtccctcacagcagggcctgtttttgcttcttttattttcccctctgcagacgtctgggtctgcgatgattggccctggatgcaagtaaaagctgtttctcctttttgtcagcctgggaatctgaacaactgtcgcgccgaggcaaagccgcagccgcgccgcggggtggctcccgggtttccccaccggacggc

SEQ ID NO: 14634 - RNA, 4409 nt, Homo sapiens
  source 1..4409: mol_type = other RNA
gctgggattacaggcatgagccaccgtgcccggccgcgagaataaactttcaaagtacccatttgtagagattttttaattgataaaattcactgagtagtgggcccttctgatgggcaggactttcagatcattcagatgacataattagtttcttaggagttctctatgctctacttgcaattctcataaattctgtttcacctctcaatttatactcatagatgtacactctaaaatgtggtcctgtggctggatggggtagcgcccaagtggaaaagcatatgggtgaaggtgctgccctgagtagccctttagcctttttagatgaaacttgaacttacagtagaacatttcccatacagagacccaaattaaattctataactctttacttcacaactagtggttggaggaggtggcatattggctcttctcacataaatatctataacagcggtgcctgtcctgggcttggtggatttgccatatttcaagttatcatcaattatatgcacaacaagatggtactgctgctgtacttcagctctacattcaaagttgaaaggattcttcacaattaattttggagtatttgaacctcgagttgggtcaaatccaaaatgatggttctcttttcctttaaaagtgataattgagaagttagaattattttaaggtatattgaaagattttctcaaactaccttaaattgctattaaaacacagtaggcgtaaatttttttaaaatttccattgcaccctgagtttttatatctatacatggcttataataaagctgagatcaaatgagcaacaatttcagttggttaggaaaaaaaaattttgaagattaagatcatgaatctgatcccatatatagccagcaagcctcaaattattatctaattgattctcctttccttctactcagatcaatttgattcccatcttcaacttagtctagatcaatatcaaatgggccggtcagatcataaatatctattgagccccttctaattttaagttatctccatagccctggagacattgttgatacacagggtccctaccttcatggagcttatcacccagcaagggaataagacatcaaactagtctttataatcaattggcaatgtccttactgatttccaagcttctactccttcagatacatgacagcaggtctgatctccataatttaaataggtctccacgttatgctgtctcatgatacccagtagttttcttttatagaacttatcacagtatgtaattttataattgctggtgttactactagtttagtaaacaatgagtgccgtgaatatctgtctcatatacttctgtgtacacatttccgagcacattgcctgatacatagttggtcccaatatatgcctttcgtaaaaaataagatggcttaagttgatatggatctgtgcaaatccaaaaataacacagtttgaaaccacgcatcctactgaatctgtactaatagcatcaaatggaaaggtggctgttgttatccagtaccatggacagcagacttcattccttgtaacttaaccttcaacatttcccatccaggttcaaagtccgttgtcaaagcatctgtaaaattactgatacttccattatgggaggaattagatttgatatgtgaaagtaaaaaagatgccttgaggaaacaatgctatagatattaaatagtttaactgttataaacataattatttctgaagttatacataatatctaacagggcaaaactaatgtcaatttgacatatgctcacgattaaaagaaataataaaattatgcaccagaaaccatctcaaaacgcatttcaaaatcttgtgactctccgtcgtggcagttcagggtgaagccattgacatttgtcccaagaacaacattgtcaaaaatgactgtcttatatagagagggtgtgcagacaggtgcttcatcattctcattttcaatgtcaacagtgatctgtcagccatgagggaagaagaaacatcaaatccacaccatgtgactacttatacacaatatcagaaataagcataagggtagagacggatcatttggaattattaaataaaaagtctagagatttggatttaaaaaaaatgttcctgcagattggaattctggccatcaatcaactagtcagtggtttattattcctgggttaactgtgacattcaatgtagccgttaggtaggattttggctcattagataagcttgtggaaagctcacaaattatgtaaatgatgagaaaaggaaagctgaagaatgatgcctctagaaattgtaatcccttgaactctttaaatatctatgcttaaaggcatagataaatttgcttcctctttctcaaaagaacttcctcagtactactctctcaaactcaatattttattggtaacaatatgattacttcaaagtatgctctgaccttaattagggactgttatcaaccttttcttaattaaaataccataaactaggaaactataatttacgtagaaaaagatcaaaatatcaagaatttttaaatgtcagtgattgaataccagtcagcctagaaaggttatctacccacttcttagatgactaataactgtctcaataatacttgcagaagaatccgtggtgcaccaatatttgcaagtattatctttttaaagtgttttatgtaatgttttaaaaacatagctaaattcttaaggaatggttcattctttaatgctacttctatagactgaatacagctatgtgtctcaccaagtatgtgagactttttacataataattaaacggattttaaggagatttctggaatagtccagtgctatttccattatatcacagaaagatatcaggaatctttattaaaatcctgggcctgacacttattgatgactttatttggcactagtgacttaccttttctttcttcaactgcaaaaagcagatctcaatctctaccttctcaggactgtcagaaggatcagttcattcattcagtgaatatttattgaatacttactatgtgccaagcactgatctagacaccacagaagctacagtggtaaaccaaaaacaaagaccctgatctaatataatttattctaatgacgaaagcaaagcaataactatactgacaaataaatatattaggcaaaatcataggataagctgatgctatttgggttaaggagatagagaatagctgatggaagtattttaagagggatttatttctttgacccactcacctattccctctctctcatgtttgttatatgtccttaagcatgtatgtatcctcatagaatatgtagcttttagttgtataattttgacttgcacaaatgatatggtgctatagaccttttgtgtttcttacttttctcacccagcgccatatatgtgctttccatgtttttgtttgcagaattcatttgctatttctggagtctgtattctgtagtatgcatctaccatatttgcttgttcatttcccatgatgaacacacatggattgcttcaaatgcccaccattacacacaatataaaaggcccttagaaacaaatttcatttgggcagagatatgattaaagtgagaatatgagccaatggaagataagcattacagtctttggcagaggttctgaggtaaaacattgttggtgtgttggaaaaacaacaaatgtttcatgtggctggattgaagtaagtaagagggagagagctaggagctaaagacaaattggtagccagggcccagatcatagagggcactgcagactttgaagatgacattggagcttaactaagcatgatgggaagccaatggagaatgttgaggaacaggatgatttatctttttaaaaggtcactctggctgtggtgtgaagagtaggctgtgaagggcacaagtaggaatgggggttctaatcaagaagctgctacactagaccaggtgaggtatggtaaaggcacagttggggtattagcagtagacaagttagaaaagtaagaagtggaaggacttaaggtacattctgaaattagagaagacagaaattgctgttggattggagaaataatttagggtacatgatagtgattaagtactcagacttaatccttctccttctttcagatgggtaatcttggataagctacctaactttgaagccttggaaataaaattcttccatctgttaaaaggagtatcagtaactattccataagatgagattaaattctaaatgagataatcaagggcatttcatagcacttgacttttattagattctcaataatgagtgggtgatgatgatagtgatgatgatgatgatgatagtgatgatgatgatgatgat

SEQ ID NO: 14635 - RNA, 2191 nt, Homo sapiens
  source 1..2191: mol_type = other RNA
gctgggattacaggcatgagccaccgtgcccggccgcttcgcatttttcttttgcaggttgcatgccagccaatattcctctgtgctgggaagggaaagtttgaggatgtatcaagaccatagcagtggatctcactgctcttgcctactcagggctttatctacacattgatagcccctcagaggaaaggcaccagccgaagagtcgacactggctctgggcttggatgctgcctctgataaacgctgggcactctgaccctgaagccagggagggagtgcttggcagctgcctgggcacactcccctcagtccagttgccaggcgaaattatacagtggatggcagctccacagagatgctaaagtttgaggtctaagtgtcagagagagctgacaatttttatgaggaaagtgaacaacaacaggtgtttatcagtacctgagaattatcatctagtttaattaagcaaaggtatcaggaggtctgtttcagctcattccctttagtatggccctaaaaaatcaacagaactgtcctacttcatgttgcccgactagcaggcaggtatgtgaacctaaagtagaagtcctagcttacatattattcataattaaacacagttcattttattattctggcaactagtgatatttcatgattataggccttaaaaatctaatacaagtacaattaaaaaaagacatagaatgcttacacaatacagaaggcactttgaggttacatgataaataaaaatacattaatagaggcaggattatttattggttccttcagtgtctgtgtccatggtgatcattgagagcccagttttgtacttcacctttggcgaatagtgtaaagaaaatggcaccaaaaacattaatagcagcagcaatatagaacacggtttgccattctccaacagtgttatcaggggtcagacttttagcaatgacgggcccaaccattcctggaatagtggcaaatgtatttgtgatgcccaggaggataccagcatacgaaggagcaatatccagatggttgatgctaaatccagaagagcaaaagcctcccagtgttgttgatatagttaggaaagcaacggccaaagaataatcacagccaatgaagccagcagctaccaggaatactgcaggtccaatcattcctataaggctaaaaattctgcgaacacataaagttgaaaaattccattttgcccttaaattgtcagcagcttgaccagacaggatcatacataaccaagagcctaaataaggcaatgaagataaaaacccattctcttgaacattgaaccttaggatctccttcatataagtaggcaataatgtcaataaagtataaaaagtccagttgtaagaaaagtgtgcaactacgatagcccaaagtggcagggattttaaaatgggtacccacggcactgacttctgtgaagaaagctgatttcttaatgatgaaagaatgtattccttttcataatgggaaattctcttgtgtttttgtggtgtgtcactaactaaccagatccacaaaagaaaccaaaatattccaatagtaccaaaaaagtagaagacataagtccaattcatatagtagcaaattattccagaaagaggaagagaaattactgtcccaagctgtgctcctgcatatgaaatgctaagaagtttgcttctttcaagagggggagcccaagaagaccacatggcatgcatggctggaaatgtaacaccctctcctagtccttctagtgctctgagtacaatgagtggtccaactcctaaatctgcagcaatgggagtgaacagggtgaggacagcagtgccaaggatcccaaatcctagcagcattttcccccctattttgctggcaacatatcctccaggaatctgtgtgatgatgtagccataaaaaaaggaaccgagaatccatccttgagtttctgcatcccattggtacttcttacccggcttcggcccgtggggcgcccggtagaagaggcgtgcggtccgtgctctcctcgccatcgttccgggccaggtctcgaaccggagacctcatgacgcctacgtgagcaggtgtactcgccacctggcagagaagggagcgccggcccgacagcccgaagcccccgggccgagctggctggaccgggcggggcgggggc

SEQ ID NO: 14636 - RNA, 2388 nt, Homo sapiens
  source 1..2388: mol_type = other RNA
gctgggattacaggcatgagccaccgtgcccggccgcttcgcatttttcttttgcaggttgcatgccagccaatattcctctgtgctgggaagggaaagtttgaggatgtatcaagaccatagcagtggatctcactgctcttgcctactcagggctttatctacacattgatagcccctcagaggaaaggcaccagccgaagagtcgacactggctctgggcttggatgctgcctctgataaacgctgggcactctgaccctgaagccagggagggagtgcttggcagctgcctgggcacactcccctcagtccagttgccaggcgaaattatacagtggatggcagctccacagagatgctaaagtttgaggtctaagtgtcagagagagctgacaatttttatgaggaaagtgaacaacaacaggtgtttatcagtacctgagaattatcatctagtttaattaagcaaaggtatcaggaggtctgtttcagctcattccctttagtatggccctaaaaaatcaacagaactgtcctacttcatgttgcccgactagcaggcaggtatgtgaacctaaagtagaagtcctagcttacatattattcataattaaacacagttcattttattattctggcaactagtgatatttcatgattataggccttaaaaatctaatacaagtacaattaaaaaaagacatagaatgcttacacaatacagaaggcactttgaggttacatgataaataaaaatacattaatagaggcaggattatttattggttccttcagtgtctgtgtccatggtgatcattgagagcccagttttgtacttcacctttggcgaatagtgtaaagaaaatggcaccaaaaacattaatagcagcagcaatatagaacacggtttgccattctccaacagtgttatcaggggtcagacttttagcaatgacgggcccaaccattcctggaatagtggcaaatgtatttgtgatgcccaggaggataccagcatacgaaggagcaatatccagatggttgatgctaaatccagaagagcaaaagcctcccagtgttgttgatatagttaggaaagcaacggccaaagaataatcacagccaatgaagccagcagctaccaggaatactgcaggtccaatcattcctataaggctaaaaattctgcgaacacataaagttgaaaaattccattttgcccttaaattgtcagcagcttgaccagacaggatcatacataaccaagagcctaaataaggcaatgaagataaaaacccattctcttgaacattgaaccttaggatctccttcatataagtaggcaataatgtcaataaagtataaaaagtccagttgtaagaaaagtgtgcaactacgatagcccaaagtggcagggattttaaaatgggtacccacggcactgacttctgtgaagaaagctgatttcttaatgatgaaagaatgtattccttttcataatgggaaattctcttgtgtttttgtggtgtgtcactaactaaccagatccacaaaagaaaccaaaatattccaatagtaccaaaaaagtagaagacataagtccaattcatatagtagcaaattattccagaaagaggaagagaaattactgtcccaagctgtgctcctgcatatgaaatgctaagaagtttgcttctttcaagagggggagcccaagaagaccacatggcatgcatggctggaaatgtaacaccctctcctagtccttctagtgctctgagtacaatgagtggtccaactcctaaatctgcagcaatgggagtgaacagggtgaggacagcagtgccaaggatcccaaatcctagcagcattttcccccctattttgctggcaacatatcctccaggaatctgtgtgatgatgtagccataaaaaaaggaaccgagaatccatccttgagtttctgcatcccattggtacttcttacccgtttgattatgatgaacttttatgggagcagaatgctctggacacgccttggaagttctattatcttctaaagttgtatttgaatctaccatatccactaacgcaacactcagattcacacgtaatgcatacacaatgaagaaaccaaaaaaggccaaaattgctaagttgtaacgagcagagcagcacactggagcggcttcggcccgtggggcgcccggtagaagaggcgtgcggtccgtgctctcctcgccatcgttccgggccaggtctcgaaccggagacctcatgacgcctacgtgagcaggtgtactcgccacctggcagagaagggagcgccggcccgacagcccgaagcccccgggccgagctggctggaccgggcggggcgggggc

SEQ ID NO: 14637 - RNA, 2409 nt, Homo sapiens
  source 1..2409: mol_type = other RNA
gctgggattacaggcatgagccaccgtgcccggccgcttcgcatttttcttttgcaggttgcatgccagccaatattcctctgtgctgggaagggaaagtttgaggatgtatcaagaccatagcagtggatctcactgctcttgcctactcagggctttatctacacattgatagcccctcagaggaaaggcaccagccgaagagtcgacactggctctgggcttggatgctgcctctgataaacgctgggcactctgaccctgaagccagggagggagtgcttggcagctgcctgggcacactcccctcagtccagttgccaggcgaaattatacagtggatggcagctccacagagatgctaaagtttgaggtctaagtgtcagagagagctgacaatttttatgaggaaagtgaacaacaacaggtgtttatcagtacctgagaattatcatctagtttaattaagcaaaggtatcaggaggtctgtttcagctcattccctttagtatggccctaaaaaatcaacagaactgtcctacttcatgttgcccgactagcaggcaggtatgtgaacctaaagtagaagtcctagcttacatattattcataattaaacacagttcattttattattctggcaactagtgatatttcatgattataggccttaaaaatctaatacaagtacaattaaaaaaagacatagaatgcttacacaatacagaaggcactttgaggttacatgataaataaaaatacattaatagaggcaggattatttattggttccttcagtgtctgtgtccatggtgatcattgagagcccagttttgtacttcacctttggcgaatagtgtaaagaaaatggcaccaaaaacattaatagcagcagcaatatagaacacggtttgccattctccaacagtgttatcaggggtcagacttttagcaatgacgggcccaaccattcctggaatagtggcaaatgtatttgtgatgcccaggaggataccagcatacgaaggagcaatatccagatggttgatgctaaatccagaagagcaaaagcctcccagtgttgttgatatagttaggaaagcaacggccaaagaataatcacagccaatgaagccagcagctaccaggaatactgcaggtccaatcattcctataaggctaaaaattctgcgaacacataaagttgaaaaattccattttgcccttaaattgtcagcagcttgaccagacaggatcatacataaccaagagcctaaataaggcaatgaagataaaaacccattctcttgaacattgaaccttaggatctccttcatataagtaggcaataatgtcaataaagtataaaaagtccagttgtaagaaaagtgtgcaactacgatagcccaaagtggcagggattttaaaatgggtacccacggcactgacttctgtgaagaaagctgatttcttaatgatgaaagaatgtattccttttcataatgggaaattctcttgtgtttttgtggtgtgtcactaactaaccagatccacaaaagaaaccaaaatattccaatagtaccaaaaaagtagaagacataagtccaattcatatagtagcaaattattccagaaagaggaagagaaattactgtcccaagctgtgctcctgcatatgaaatgctaagaagtttgcttctttcaagagggggagcccaagaagaccacatggcatgcatggctggaaatgtaacaccctctcctagtccttctagtgctctgagtacaatgagtggtccaactcctaaatctgcagcaatgggagtgaacagggtgaggacagcagtgccaaggatcccaaatcctagcagcattttcccccctattttgctggcaacatatcctccaggaatctgtgtgatgatgtagccataaaaaaaggaaccgagaatccatccttgagtttctgcatcccattggtacttcttacccgtttgattatgatgaacttttatgggagcagaatgctctggacacgccttggaagttctattatcttctaaagttgtatttgaatctaccatatccactaacgcaacactcagattcacacgtaatgcatacacaatgaagaaaccaaaaaaggccaaaattgctaagttgtaacgagcagagcagcacactggagctcgaagagtatcctcaaaggcggcttcggcccgtggggcgcccggtagaagaggcgtgcggtccgtgctctcctcgccatcgttccgggccaggtctcgaaccggagacctcatgacgcctacgtgagcaggtgtactcgccacctggcagagaagggagcgccggcccgacagcccgaagcccccgggccgagctggctggaccgggcggggcgggggc

SEQ ID NO: 14638 - RNA, 2385 nt, Homo sapiens
  source 1..2385: mol_type = other RNA
gctgggattacaggcatgagccaccgtgcccggccgcttcgcatttttcttttgcaggttgcatgccagccaatattcctctgtgctgggaagggaaagtttgaggatgtatcaagaccatagcagtggatctcactgctcttgcctactcagggctttatctacacattgatagcccctcagaggaaaggcaccagccgaagagtcgacactggctctgggcttggatgctgcctctgataaacgctgggcactctgaccctgaagccagggagggagtgcttggcagctgcctgggcacactcccctcagtccagttgccaggcgaaattatacagtggatggcagctccacagagatgctaaagtttgaggtctaagtgtcagagagagctgacaatttttatgaggaaagtgaacaacaacaggtgtttatcagtacctgagaattatcatctagtttaattaagcaaaggtatcaggaggtctgtttcagctcattccctttagtatggccctaaaaaatcaacagaactgtcctacttcatgttgcccgactagcaggcaggtatgtgaacctaaagtagaagtcctagcttacatattattcataattaaacacagttcattttattattctggcaactagtgatatttcatgattataggccttaaaaatctaatacaagtacaattaaaaaaagacatagaatgcttacacaatacagaaggcactttgaggttacatgataaataaaaatacattaatagaggcaggattatttattggttccttcagtgtctgtgtccatggtgatcattgagagcccagttttgtacttcacctttggcgaatagtgtaaagaaaatggcaccaaaaacattaatagcagcagcaatatagaacacggtttgccattctccaacagtgttatcaggggtcagacttttagcaatgacgggcccaaccattcctggaatagtggcaaatgtatttgtgatgcccaggaggataccagcatacgaaggagcaatatccagatggttgatgctaaatccagaagagcaaaagcctcccagtgttgttgatatagttaggaaagcaacggccaaagaataatcacagccaatgaagccagcagctaccaggaatactgcaggtccaatcattcctataaggctaaaaattctgcgaacacataaagttgaaaaattccattttgcccttaaattgtcagcagcttgaccagacaggatcatacataaccaagagcctaaataaggcaatgaagataaaaacccattctcttgaacattgaaccttaggatctccttcatataagtaggcaataatgtcaataaagtataaaaagtccagttgtaagaaaagtgtgcaactacgatagcccaaagtggcagggattttaaaatgggtacccacggcactgacttctgtgaagaaagctgatttcttaatgatgaaagaatgtattccttttcataatgggaaattctcttgtgtttttgtggtgtgtcactaactaaccagatccacaaaagaaaccaaaatattccaatagtaccaaaaaagtagaagacataagtccaattcatatagtagcaaattattccagaaagaggaagagaaattactgtcccaagctgtgctgcatatgaaatgctaagaagtttgcttctttcaagagggggagcccaagaagaccacatggcatgcatggctggaaatgtaacaccctctcctagtccttctagtgctctgagtacaatgagtggtccaactcctaaatctgcagcaatgggagtgaacagggtgaggacagcagtgccaaggatcccaaatcctagcagcattttcccccctattttgctggcaacatatcctccaggaatctgtgtgatgatgtagccataaaaaaaggaaccgagaatccatccttgagtttctgcatcccattggtacttcttacccgtttgattatgatgaacttttatgggagcagaatgctctggacacgccttggaagttctattatcttctaaagttgtatttgaatctaccatatccactaacgcaacactcagattcacacgtaatgcatacacaatgaagaaaccaaaaaaggccaaaattgctaagttgtaacgagcagagcagcacactggagcggcttcggcccgtggggcgcccggtagaagaggcgtgcggtccgtgctctcctcgccatcgttccgggccaggtctcgaaccggagacctcatgacgcctacgtgagcaggtgtactcgccacctggcagagaagggagcgccggcccgacagcccgaagcccccgggccgagctggctggaccgggcggggcgggggc

SEQ ID NO: 14639 - RNA, 2104 nt, Homo sapiens
  source 1..2104: mol_type = other RNA
gctgggattacaggcatgagccaccgtgcccggccgcttcgcatttttcttttgcaggttgcatgccagccaatattcctctgtgctgggaagggaaagtttgaggatgtatcaagaccatagcagtggatctcactgctcttgcctactcagggctttatctacacattgatagcccctcagaggaaaggcaccagccgaagagtcgacactggctctgggcttggatgctgcctctgataaacgctgggcactctgaccctgaagccagggagggagtgcttggcagctgcctgggcacactcccctcagtccagttgccaggcgaaattatacagtggatggcagctccacagagatgctaaagtttgaggtctaagtgtcagagagagctgacaatttttatgaggaaagtgaacaacaacaggtgtttatcagtacctgagaattatcatctagtttaattaagcaaaggtatcaggaggtctgtttcagctcattccctttagtatggccctaaaaaatcaacagaactgtcctacttcatgttgcccgactagcaggcaggtatgtgaacctaaagtagaagtcctagcttacatattattcataattaaacacagttcattttattattctggcaactagtgatatttcatgattataggccttaaaaatctaatacaagtacaattaaaaaaagacatagaatgcttacacaatacagaaggcactttgaggttacatgataaataaaaatacattaatagaggcaggattatttattggttccttcagtgtctgtgtccatggtgatcattgagagcccagttttgtacttcacctttggcgaatagtgtaaagaaaatggcaccaaaaacattaatagcagcagcaatatagaacacggtttgccattctccaacagtgttatcaggggtcagacttttagcaatgacgggcccaaccattcctggaatagtggcaaatgtatttgtgatgcccaggaggataccagcatacgaaggagcaatatccagatggttgatgctaaatccagaagagcaaaagcctcccagtgttgttgatatagttaggaaagcaacggccaaagaataatcacagccaatgaagccagcagctaccaggaatactgcaggtccaatcattcctataaggctaaaaattctgcgaacacataaagttgaaaaattccattttgcccttaaattgtcagcagcttgaccagacaggatcatacataaccaagagcctaaataaggcaatgaagataaaaacccattctcttgaacattgaaccttaggatctccttcatataagtaggcaataatgtcaataaagtataaaaagtccagttgtaagaaaagtgtgcaactacgatagcccaaagtggcagggattttaaaatgggtacccacggcactgacttctgtgaagaaagctgatttcttaatgatgaaagaatgtattccttttcataatgggaaattctcttgtgtttttgtggtgtgtcactaactaaccagatccacaaaagaaaccaaaatattccaatagtacctgcatatgaaatgctaagaagtttgcttctttcaagagggggagcccaagaagaccacatggcatgcatggctggaaatgtaacaccctctcctagtccttctagtgctctgagtacaatgagtggtccaactcctaaatctgcagcaatgggagtgaacagggtgaggacagcagtgccaaggatcccaaatcctagcagcattttcccccctattttgctggcaacatatcctccaggaatctgtgtgatgatgtagccataaaaaaaggaaccgagaatccatccttgagtttctgcatcccattggtacttcttacccggcttcggcccgtggggcgcccggtagaagaggcgtgcggtccgtgctctcctcgccatcgttccgggccaggtctcgaaccggagacctcatgacgcctacgtgagcaggtgtactcgccacctggcagagaagggagcgccggcccgacagcccgaagcccccgggccgagctggctggaccgggcggggcgggggc

SEQ ID NO: 14640 - RNA, 2301 nt, Homo sapiens
  source 1..2301: mol_type = other RNA
gctgggattacaggcatgagccaccgtgcccggccgcttcgcatttttcttttgcaggttgcatgccagccaatattcctctgtgctgggaagggaaagtttgaggatgtatcaagaccatagcagtggatctcactgctcttgcctactcagggctttatctacacattgatagcccctcagaggaaaggcaccagccgaagagtcgacactggctctgggcttggatgctgcctctgataaacgctgggcactctgaccctgaagccagggagggagtgcttggcagctgcctgggcacactcccctcagtccagttgccaggcgaaattatacagtggatggcagctccacagagatgctaaagtttgaggtctaagtgtcagagagagctgacaatttttatgaggaaagtgaacaacaacaggtgtttatcagtacctgagaattatcatctagtttaattaagcaaaggtatcaggaggtctgtttcagctcattccctttagtatggccctaaaaaatcaacagaactgtcctacttcatgttgcccgactagcaggcaggtatgtgaacctaaagtagaagtcctagcttacatattattcataattaaacacagttcattttattattctggcaactagtgatatttcatgattataggccttaaaaatctaatacaagtacaattaaaaaaagacatagaatgcttacacaatacagaaggcactttgaggttacatgataaataaaaatacattaatagaggcaggattatttattggttccttcagtgtctgtgtccatggtgatcattgagagcccagttttgtacttcacctttggcgaatagtgtaaagaaaatggcaccaaaaacattaatagcagcagcaatatagaacacggtttgccattctccaacagtgttatcaggggtcagacttttagcaatgacgggcccaaccattcctggaatagtggcaaatgtatttgtgatgcccaggaggataccagcatacgaaggagcaatatccagatggttgatgctaaatccagaagagcaaaagcctcccagtgttgttgatatagttaggaaagcaacggccaaagaataatcacagccaatgaagccagcagctaccaggaatactgcaggtccaatcattcctataaggctaaaaattctgcgaacacataaagttgaaaaattccattttgcccttaaattgtcagcagcttgaccagacaggatcatacataaccaagagcctaaataaggcaatgaagataaaaacccattctcttgaacattgaaccttaggatctccttcatataagtaggcaataatgtcaataaagtataaaaagtccagttgtaagaaaagtgtgcaactacgatagcccaaagtggcagggattttaaaatgggtacccacggcactgacttctgtgaagaaagctgatttcttaatgatgaaagaatgtattccttttcataatgggaaattctcttgtgtttttgtggtgtgtcactaactaaccagatccacaaaagaaaccaaaatattccaatagtacctgcatatgaaatgctaagaagtttgcttctttcaagagggggagcccaagaagaccacatggcatgcatggctggaaatgtaacaccctctcctagtccttctagtgctctgagtacaatgagtggtccaactcctaaatctgcagcaatgggagtgaacagggtgaggacagcagtgccaaggatcccaaatcctagcagcattttcccccctattttgctggcaacatatcctccaggaatctgtgtgatgatgtagccataaaaaaaggaaccgagaatccatccttgagtttctgcatcccattggtacttcttacccgtttgattatgatgaacttttatgggagcagaatgctctggacacgccttggaagttctattatcttctaaagttgtatttgaatctaccatatccactaacgcaacactcagattcacacgtaatgcatacacaatgaagaaaccaaaaaaggccaaaattgctaagttgtaacgagcagagcagcacactggagcggcttcggcccgtggggcgcccggtagaagaggcgtgcggtccgtgctctcctcgccatcgttccgggccaggtctcgaaccggagacctcatgacgcctacgtgagcaggtgtactcgccacctggcagagaagggagcgccggcccgacagcccgaagcccccgggccgagctggctggaccgggcggggcgggggc

SEQ ID NO: 14641 - RNA, 2229 nt, Homo sapiens
  source 1..2229: mol_type = other RNA
gctgggattacaggcatgagccaccgtgcccggccgcttcgcatttttcttttgcaggttgcatgccagccaatattcctctgtgctgggaagggaaagtttgaggatgtatcaagaccatagcagtggatctcactgctcttgcctactcagggctttatctacacattgatagcccctcagaggaaaggcaccagccgaagagtcgacactggctctgggcttggatgctgcctctgataaacgctgggcactctgaccctgaagccagggagggagtgcttggcagctgcctgggcacactcccctcagtccagttgccaggcgaaattatacagtggatggcagctccacagagatgctaaagtttgaggtctaagtgtcagagagagctgacaatttttatgaggaaagtgaacaacaacaggtgtttatcagtacctgagaattatcatctagtttaattaagcaaaggtatcaggaggtctgtttcagctcattccctttagtatggccctaaaaaatcaacagaactgtcctacttcatgttgcccgactagcaggcaggtatgtgaacctaaagtagaagtcctagcttacatattattcataattaaacacagttcattttattattctggcaactagtgatatttcatgattataggccttaaaaatctaatacaagtacaattaaaaaaagacatagaatgcttacacaatacagaaggcactttgaggttacatgataaataaaaatacattaatagaggcaggattatttattggttccttcagtgtctgtgtccatggtgatcattgagagcccagttttgtacttcacctttggcgaatagtgtaaagaaaatggcaccaaaaacattaatagcagcagcaatatagaacacggtttgccattctccaacagtgttatcaggggtcagacttttagcaatgacgggcccaaccattcctggaatagtggcaaatgtatttgtgatgcccaggaggataccagcatacgaaggagcaatatccagatggttgatgctaaatccagaagagcaaaagcctcccagtgttgttgatatagttaggaaagcaacggccaaagaataatcacagccaatgaagccagcagctaccaggaatactgcaggtccaatcattcctataaggctaaaaattctgcgaacacataaagttgaaaaattccattttgcccttaaattgtcagcagcttgaccagacaggatcatacataaccaagagcctaaataaggcaatgaagataaaaacccattctgatttcttaatgatgaaagaatgtattccttttcataatgggaaattctcttgtgtttttgtggtgtgtcactaactaaccagatccacaaaagaaaccaaaatattccaatagtaccaaaaaagtagaagacataagtccaattcatatagtagcaaattattccagaaagaggaagagaaattactgtcccaagctgtgctcctgcatatgaaatgctaagaagtttgcttctttcaagagggggagcccaagaagaccacatggcatgcatggctggaaatgtaacaccctctcctagtccttctagtgctctgagtacaatgagtggtccaactcctaaatctgcagcaatgggagtgaacagggtgaggacagcagtgccaaggatcccaaatcctagcagcattttcccccctattttgctggcaacatatcctccaggaatctgtgtgatgatgtagccataaaaaaaggaaccgagaatccatccttgagtttctgcatcccattggtacttcttacccgtttgattatgatgaacttttatgggagcagaatgctctggacacgccttggaagttctattatcttctaaagttgtatttgaatctaccatatccactaacgcaacactcagattcacacgtaatgcatacacaatgaagaaaccaaaaaaggccaaaattgctaagttgtaacgagcagagcagcacactggagcggcttcggcccgtggggcgcccggtagaagaggcgtgcggtccgtgctctcctcgccatcgttccgggccaggtctcgaaccggagacctcatgacgcctacgtgagcaggtgtactcgccacctggcagagaagggagcgccggcccgacagcccgaagcccccgggccgagctggctggaccgggcggggcgggggc

SEQ ID NO: 14642 - RNA, 2486 nt, Homo sapiens
  source 1..2486: mol_type = other RNA
gctgggattacaggcatgagccaccgtgcccggccgcttcgcatttttcttttgcaggttgcatgccagccaatattcctctgtgctgggaagggaaagtttgaggatgtatcaagaccatagcagtggatctcactgctcttgcctactcagggctttatctacacattgatagcccctcagaggaaaggcaccagccgaagagtcgacactggctctgggcttggatgctgcctctgataaacgctgggcactctgaccctgaagccagggagggagtgcttggcagctgcctgggcacactcccctcagtccagttgccaggcgaaattatacagtggatggcagctccacagagatgctaaagtttgaggtctaagtgtcagagagagctgacaatttttatgaggaaagtgaacaacaacaggtgtttatcagtacctgagaattatcatctagtttaattaagcaaaggtatcaggaggtctgtttcagctcattccctttagtatggccctaaaaaatcaacagaactgtcctacttcatgttgcccgactagcaggcaggtatgtgaacctaaagtagaagtcctagcttacatattattcataattaaacacagttcattttattattctggcaactagtgatatttcatgattataggccttaaaaatctaatacaagtacaattaaaaaaagacatagaatgcttacacaatacagaaggcactttgaggttacatgataaataaaaatacattaatagaggcaggattatttattggttccttcagtgtctgtgtccatggtgatcattgagagcccagttttgtacttcacctttggcgaatagtgtaaagaaaatggcaccaaaaacattaatagcagcagcaatatagaacacggtttgccattctccaacagtgttctgtaatcccagctattcgggaggctgaggcaggaaaatcgccggaacccgggaggcaaaggttgtggtgagctgagattgcgccattgtactccagcatcaggggtcagacttttagcaatgacgggcccaaccattcctggaatagtggcaaatgtatttgtgatgcccaggaggataccagcatacgaaggagcaatatccagatggttgatgctaaatccagaagagcaaaagcctcccagtgttgttgatatagttaggaaagcaacggccaaagaataatcacagccaatgaagccagcagctaccaggaatactgcaggtccaatcattcctataaggctaaaaattctgcgaacacataaagttgaaaaattccattttgcccttaaattgtcagcagcttgaccagacaggatcatacataaccaagagcctaaataaggcaatgaagataaaaacccattctcttgaacattgaaccttaggatctccttcatataagtaggcaataatgtcaataaagtataaaaagtccagttgtaagaaaagtgtgcaactacgatagcccaaagtggcagggattttaaaatgggtacccacggcactgacttctgtgaagaaagctgatttcttaatgatgaaagaatgtattccttttcataatgggaaattctcttgtgtttttgtggtgtgtcactaactaaccagatccacaaaagaaaccaaaatattccaatagtaccaaaaaagtagaagacataagtccaattcatatagtagcaaattattccagaaagaggaagagaaattactgtcccaagctgtgctcctgcatatgaaatgctaagaagtttgcttctttcaagagggggagcccaagaagaccacatggcatgcatggctggaaatgtaacaccctctcctagtccttctagtgctctgagtacaatgagtggtccaactcctaaatctgcagcaatgggagtgaacagggtgaggacagcagtgccaaggatcccaaatcctagcagcattttcccccctattttgctggcaacatatcctccaggaatctgtgtgatgatgtagccataaaaaaaggaaccgagaatccatccttgagtttctgcatcccattggtacttcttacccgtttgattatgatgaacttttatgggagcagaatgctctggacacgccttggaagttctattatcttctaaagttgtatttgaatctaccatatccactaacgcaacactcagattcacacgtaatgcatacacaatgaagaaaccaaaaaaggccaaaattgctaagttgtaacgagcagagcagcacactggagcggcttcggcccgtggggcgcccggtagaagaggcgtgcggtccgtgctctcctcgccatcgttccgggccaggtctcgaaccggagacctcatgacgcctacgtgagcaggtgtactcgccacctggcagagaagggagcgccggcccgacagcccgaagcccccgggccgagctggctggaccgggcggggcgggggc

SEQ ID NO: 14643 - RNA, 2297 nt, Homo sapiens
  source 1..2297: mol_type = other RNA
gctgggattacaggcatgagccaccgtgcccggccgcttcgcatttttcttttgcaggttgcatgccagccaatattcctctgtgctgggaagggaaagtttgaggatgtatcaagaccatagcagtggatctcactgctcttgcctactcagggctttatctacacattgatagcccctcagaggaaaggcaccagccgaagagtcgacactggctctgggcttggatgctgcctctgataaacgctgggcactctgaccctgaagccagggagggagtgcttggcagctgcctgggcacactcccctcagtccagttgccaggcgaaattatacagtggatggcagctccacagagatgctaaagtttgaggtctaagtgtcagagagagctgacaatttttatgaggaaagtgaacaacaacaggtgtttatcagtacctgagaattatcatctagtttaattaagcaaaggtatcaggaggtctgtttcagctcattccctttagtatggccctaaaaaatcaacagaactgtcctacttcatgttgcccgactagcaggcaggtatgtgaacctaaagtagaagtcctagcttacatattattcataattaaacacagttcattttattattctggcaactagtgatatttcatgattataggccttaaaaatctaatacaagtacaattaaaaaaagacatagaatgcttacacaatacagaaggcactttgaggttacatgataaataaaaatacattaatagaggcaggattatttattggttccttcagtgtctgtgtccatggtgatcattgagagcccagttttgtacttcacctttggcgaatagtgtaaagaaaatggcaccaaaaacattaatagcagcagcaatatagaacacggtttgccattctccaacagtgttgaaggagcaatatccagatggttgatgctaaatccagaagagcaaaagcctcccagtgttgttgatatagttaggaaagcaacggccaaagaataatcacagccaatgaagccagcagctaccaggaatactgcaggtccaatcattcctataaggctaaaaattctgcgaacacataaagttgaaaaattccattttgcccttaaattgtcagcagcttgaccagacaggatcatacataaccaagagcctaaataaggcaatgaagataaaaacccattctcttgaacattgaaccttaggatctccttcatataagtaggcaataatgtcaataaagtataaaaagtccagttgtaagaaaagtgtgcaactacgatagcccaaagtggcagggattttaaaatgggtacccacggcactgacttctgtgaagaaagctgatttcttaatgatgaaagaatgtattccttttcataatgggaaattctcttgtgtttttgtggtgtgtcactaactaaccagatccacaaaagaaaccaaaatattccaatagtaccaaaaaagtagaagacataagtccaattcatatagtagcaaattattccagaaagaggaagagaaattactgtcccaagctgtgctcctgcatatgaaatgctaagaagtttgcttctttcaagagggggagcccaagaagaccacatggcatgcatggctggaaatgtaacaccctctcctagtccttctagtgctctgagtacaatgagtggtccaactcctaaatctgcagcaatgggagtgaacagggtgaggacagcagtgccaaggatcccaaatcctagcagcattttcccccctattttgctggcaacatatcctccaggaatctgtgtgatgatgtagccataaaaaaaggaaccgagaatccatccttgagtttctgcatcccattggtacttcttacccgtttgattatgatgaacttttatgggagcagaatgctctggacacgccttggaagttctattatcttctaaagttgtatttgaatctaccatatccactaacgcaacactcagattcacacgtaatgcatacacaatgaagaaaccaaaaaaggccaaaattgctaagttgtaacgagcagagcagcacactggagcggcttcggcccgtggggcgcccggtagaagaggcgtgcggtccgtgctctcctcgccatcgttccgggccaggtctcgaaccggagacctcatgacgcctacgtgagcaggtgtactcgccacctggcagagaagggagcgccggcccgacagcccgaagcccccgggccgagctggctggaccgggcggggcgggggc

SEQ ID NO: 14644 - RNA, 3082 nt, Homo sapiens
  source 1..3082: mol_type = other RNA
gctgggattacaggcatgagccaccgtgcccggccggctacctcattctagtactgccccaacactgcctgccatttttgggtgctgagctaatcaattacctctggtctttagctcctttctggatgtcgtttcttagtgggtcaaatgagatatataaaaacttcctaaaaaatggatactttgctgtcttttctgtatctttcagttatcatcccaccacaattttcttttagtttacctcttccctctccacaaaagttgttctcaataaggtcaaggaaacatttgtattcattttctattgctgctgtaccaaattatcacaaacttggcttaaaacaacacaaatttattctctcatagttctataggccagaagtcagaaatcagtttcacagaactaaagtaaacgtgtcagcagggcttgctccttcgggaggctataggggataatctgttttctttttcttttcttagcttctggaggccattcacattccttggctcatggctgctttcttgtatcactccaaccttttgcttccattgtcgaatttcctactctctttaccctagtcaaatctccttctgactccctcttatagagacacctgtgattacattaggacctgcttagataatgcaatataattttcccatctcaagatccttaacttaaatctgcaaagtcctttatgcatataagtgacaggttccaggaattaggacctgggtatctttggggactattcttcctatagcagcactgattttctaattttcaaatctgatgtcttctgttcagtcctcatcctaactctcttgctatttgatactgtcagttactctgggaaaagctcctccctgactttcatgattattttcctctgatacgatatctttattgtctgtctctcccttaaaatgcaagactctgagagtaggaatcctggctatcttgtttgttgttttatccccagtgcttggaataatacctgccactatcaaatcacaaaaggcatcacgtaatgtaaattggatgagcttctcccattcctagttccaccaccactctctcattttccttcactagcaacttcctctattctcatgggtcaagattagtattctccatggtttgggaatagcttgcttttctccttatatgccaggtggccacatttccaaccatactcagtgggctctcaaatgtataccttaaccccagacctttgttttgcacttctaacttttatctttaccttgatatcccacaagcatggagaattcaccatgtcttacctttcccatccaccaagcacagcccaaaactaacttttccttcctcttacattctctgcctcagggaataaaaagtatcagaattcacccagtagtgtaagcaagaaaactgggagttatcccagaatccatgctttctctctactcccctctccacatcactaccgacccatccagtcagtcatgaagttttgtcaacctcactcctaaatatctcctgatatctctttctgtctgactcccattgctttggttcatgtccttattactcctatggagtaggatataagtgaacttaccaatgtgtccctcctgacttctcttgagtatggtagaatgtcacattcttaagctttttggaggcgtgccagagttgctggtcattgcctgtcctgcttctggcctctgccagtgggcagtgactgtgatttgcataccgcttccatagccagttggcccagggataggcttctgtcctaaaggtggctccttctatagatttggtcagccaacttaggtcatgggtgcctggttgtaaaatataagctgagtaaaattccttttaggatttcagaatagagaagcctgagaggctcagggtgctgtattgctgaacagaaaggttagcagtaatgatgggcataagcaggctgcagctatgaggaagcagatagtgtgtgtaagcaggggagctgtgagccaggagagaacaaggaagaaaataagccaaggcactgtgagaagggtgatgtttcagttttgggtggttctttaattgtacttctgaagcctggctgtattgtgattcctactgtcagatgtccatgagattgctgcattatttaaaaaaccccagtctgagtatacccttgtttcgtgcaataaactggccaaagagctatgtgttccagtaagctcataatgttatgaagagacatgtggaagaaagaggcactattctagagcagcaatatgaagtcccaaactattccactccttcataaggcattagcttgaagggggaaaaaaaggaagcttgtatcaccttttcctttggaggtgaatgatgagcttcttatatcaaagttaatctttatataaaaacaaattgatctttgcaaacataatttcagaaaggaaaagtaattgctgctacaaacatcacatgaaaatcacagtaataggtgacataacactgatacttgacagtgggataatcaaaccaccttttagatgccatgtttgtaggtatctacctttcattttgccagctgttgggacccatgggtttgctgaagatctgcaggattcctagtcacatgaccatattcctctcctgttttcataaggcttgagtacttccttggcttcatcacaaagggggcatgggtcagttccacatggctggggaggcctcataatgatggcggaaggcaaggaggagcaagtcacatcttacatggatggcagcaggcaaagagagaccttgtgctgagaaactcctttgtgaataaggtcaacacaggcagagttgtcttagaggcagagcaatttctcaagaagagtccaaaggaggatctggcaagttgcatgctatttccttgaaaccagagcatcttaattctgatccagatgatttctccccttcgaaataattgcaaacaagattaaaactgtattcaggaagtattccagctggcttttggcttcctctgatgtacagtcctgagcctcacgccgccaacgcctctgcttccgccctgcgccgggcacttcc

SEQ ID NO: 14645 - RNA, 3367 nt, Homo sapiens
  source 1..3367: mol_type = other RNA
gctgggattacaggcatgagccaccgtgcccggccggctacctcattctagtactgccccaacactgcctgccatttttgggtgctgagctaatcaattacctctggtctttagctcctttctggatgtcgtttcttagtgggtcaaatgagatatataaaaacttcctaaaaaatggatactttgctgtcttttctgtatctttcagttatcatcccaccacaattttcttttagtttacctcttccctctccacaaaagttgttctcaataaggtcaaggaaacatttgtattcattttctattgctgctgtaccaaattatcacaaacttggcttaaaacaacacaaatttattctctcatagttctataggccagaagtcagaaatcagtttcacagaactaaagtaaacgtgtcagcagggcttgctccttcgggaggctataggggataatctgttttctttttcttttcttagcttctggaggccattcacattccttggctcatggctgctttcttgtatcactccaaccttttgcttccattgtcgaatttcctactctctttaccctagtcaaatctccttctgactccctcttatagagacacctgtgattacattaggacctgcttagataatgcaatataattttcccatctcaagatccttaacttaaatctgcaaagtcctttatgcatataagtgacaggttccaggaattaggacctgggtatctttggggactattcttcctatagcagcactgattttctaattttcaaatctgatgtcttctgttcagtcctcatcctaactctcttgctatttgatactgtcagttactctgggaaaagctcctccctgactttcatgattattttcctctgatacgatatctttattgtctgtctctcccttaaaatgcaagactctgagagtaggaatcctggctatcttgtttgttgttttatccccagtgcttggaataatacctgccactatcaaatcacaaaaggcatcacgtaatgtaaattggatgagcttctcccattcctagttccaccaccactctctcattttccttcactagcaacttcctctattctcatgggtcaagattagtattctccatggtttgggaatagcttgcttttctccttatatgccaggtggccacatttccaaccatactcagtgggctctcaaatgtataccttaaccccagacctttgttttgcacttctaacttttatctttaccttgatatcccacaagcatggagaattcaccatgtcttacctttcccatccaccaagcacagcccaaaactaacttttccttcctcttacattctctgcctcagggaataaaaagtatcagaattcacccagtagtgtaagcaagaaaactgggagttatcccagaatccatgctttctctctactcccctctccacatcactaccgacccatccagtcagtcatgaagttttgtcaacctcactcctaaatatctcctgatatctctttctgtctgactcccattgctttggttcatgtccttattactcctatggagtaggatataagtgaacttaccaatgtgtccctcctgacttctcttgagtatggtagaatgtcacattcttaagctttttggaggcgtgccagagttgctggtcattgcctgtcctgcttctggcctctgccagtgggcagtgactgtgatttgcataccgcttccatagccagttggcccagggataggcttctgtcctaaaggtggctccttctatagatttggtcagccaacttaggtcatgggtgcctggttgtaaaatataagctgagtaaaattccttttaggatttcagaatagagaagcctgagaggctcagggtgctgtattgctgaacagaaaggttagcagtaatgatgggcataagcaggctgcagctatgaggaagcagatagtgtgtgtaagcaggggagctgtgagccaggagagaacaaggaagaaaataagccaaggcactgtgagaagggtgatgtttcagttttgggtggttctttaattgtacttctgaagcctggctgtattgtgattcctactgtcagatgtccatgagattgctgcattatttaaaaaaccccagtctgagtatacccttgtttcgtgcaataaactggccaaagagctatgtgttccagtaagctcataatgttatgaagagacatgtggaagaaagaggcactattctagagcagcaatatgaagtcccaaactattccactccttcataaggcattagcttgaagggggaaaaaaaggaagcttgtatcaccttttcctttggaggtgaatgatgagcttcttatatcaaagttaatctttatataaaaacaaattgatctttgcaaacataatttcagaaaggaaaagtaattgctgctacaaacatcacatgaaaatcacagtaataggtgacataacactgatacttgacagtgggataatcaaaccaccttttagatgccatgtttgtaggtatctacctttcattttgccagctgttgggacccatgggtttgctgaagatctgcaggattcctagtcacatgaccatattcctctctgaaataagaattgatgagtaagtttattgaagagctataggttaaaaccaacattaggtatatgtaaccaatactctaaatatgggataccttcagaaagcatctttctgtctccctctattcctatatatttggtggatgaatttttcactgtttaggataaaaacaacaggtcatatcaggactcttgaacattctcaggcaatagaatgccccacagtcacttgaaattgtttttggtgcatctaatcccatgtcataatcaaaacttaagacttggtttaaagttaagttgtatcttttccccgactgagaagccatgtgggggtgggaaggtgaggaaggggagcgtcttctccttgttcctggcagcttctgatccttgtagggttgcctgttttcataaggcttgagtacttccttggcttcatcacaaagggggcatgggtcctttgtgaataaggtcaacacaggcagagttgtcttagaggcagagcaatttctcaagaagagtccaaaggaggatctggcaagttgcatgctatttccttgaaaccagagcatcttaattctgatccagatgatttctccccttcgaaataattgcaaacaagattaaaactgtattcaggaagtattccagctggcttttggcttcctctgatgtacagtcctgagcctcacgccgccaacgcctctgcttccgccctgcgccgggcacttcc

SEQ ID NO: 14646 - RNA, 3275 nt, Homo sapiens
  source 1..3275: mol_type = other RNA
gctgggattacaggcatgagccaccgtgcccggccggctacctcattctagtactgccccaacactgcctgccatttttgggtgctgagctaatcaattacctctggtctttagctcctttctggatgtcgtttcttagtgggtcaaatgagatatataaaaacttcctaaaaaatggatactttgctgtcttttctgtatctttcagttatcatcccaccacaattttcttttagtttacctcttccctctccacaaaagttgttctcaataaggtcaaggaaacatttgtattcattttctattgctgctgtaccaaattatcacaaacttggcttaaaacaacacaaatttattctctcatagttctataggccagaagtcagaaatcagtttcacagaactaaagtaaacgtgtcagcagggcttgctccttcgggaggctataggggataatctgttttctttttcttttcttagcttctggaggccattcacattccttggctcatggctgctttcttgtatcactccaaccttttgcttccattgtcgaatttcctactctctttaccctagtcaaatctccttctgactccctcttatagagacacctgtgattacattaggacctgcttagataatgcaatataattttcccatctcaagatccttaacttaaatctgcaaagtcctttatgcatataagtgacaggttccaggaattaggacctgggtatctttggggactattcttcctatagcagcactgattttctaattttcaaatctgatgtcttctgttcagtcctcatcctaactctcttgctatttgatactgtcagttactctgggaaaagctcctccctgactttcatgattattttcctctgatacgatatctttattgtctgtctctcccttaaaatgcaagactctgagagtaggaatcctggctatcttgtttgttgttttatccccagtgcttggaataatacctgccactatcaaatcacaaaaggcatcacgtaatgtaaattggatgagcttctcccattcctagttccaccaccactctctcattttccttcactagcaacttcctctattctcatgggtcaagattagtattctccatggtttgggaatagcttgcttttctccttatatgccaggtggccacatttccaaccatactcagtgggctctcaaatgtataccttaaccccagacctttgttttgcacttctaacttttatctttaccttgatatcccacaagcatggagaattcaccatgtcttacctttcccatccaccaagcacagcccaaaactaacttttccttcctcttacattctctgcctcagggaataaaaagtatcagaattcacccagtagtgtaagcaagaaaactgggagttatcccagaatccatgctttctctctactcccctctccacatcactaccgacccatccagtcagtcatgaagttttgtcaacctcactcctaaatatctcctgatatctctttctgtctgactcccattgctttggttcatgtccttattactcctatggagtaggatataagtgaacttaccaatgtgtccctcctgacttctcttgagtatggtagaatgtcacattcttaagctttttggaggcgtgccagagttgctggtcattgcctgtcctgcttctggcctctgccagtgggcagtgactgtgatttgcataccgcttccatagccagttggcccagggataggcttctgtcctaaaggtggctccttctatagatttggtcagccaacttaggtcatgggtgcctggttgtaaaatataagctgagtaaaattccttttaggatttcagaatagagaagcctgagaggctcagggtgctgtattgctgaacagaaaggttagcagtaatgatgggcataagcaggctgcagctatgaggaagcagatagtgtgtgtaagcaggggagctgtgagccaggagagaacaaggaagaaaataagccaaggcactgtgagaagggtgatgtttcagttttgggtggttctttaattgtacttctgaagcctggctgtattgtgattcctactgtcagatgtccatgagattgctgcattatttaaaaaaccccagtctgagtatacccttgtttcgtgcaataaactggccaaagagctatgtgttccagtaagctcataatgttatgaagagacatgtggaagaaagaggcactattctagagcagcaatatgaagtcccaaactattccactccttcataaggcattagcttgaagggggaaaaaaaggaagcttgtatcaccttttcctttggaggtgaatgatgagcttcttatatcaaagttaatctttatataaaaacaaattgatctttgcaaacataatttcagaaaggaaaagtaattgctgctacaaacatcacatgaaaatcacagtaataggtgacataacactgatacttgacagtgggataatcaaaccaccttttagatgccatgtttgtaggtatctacctttcattttgccagctgttgggacccatgggtttgctgaagatctgcaggattcctagtcacatgaccatattcctctcttcagaaagcatctttctgtctccctctattcctatatatttggtggatgaatttttcactgtttaggataaaaacaacaggtcatatcaggactcttgaacattctcaggcaatagaatgccccacagtcacttgaaattgtttttggtgcatctaatcccatgtcataatcaaaacttaagacttggtttaaagttaagttgtatcttttccccgactgagaagccatgtgggggtgggaaggtgaggaaggggagcgtcttctccttgttcctggcagcttctgatccttgtagggttgcctgttttcataaggcttgagtacttccttggcttcatcacaaagggggcatgggtcctttgtgaataaggtcaacacaggcagagttgtcttagaggcagagcaatttctcaagaagagtccaaaggaggatctggcaagttgcatgctatttccttgaaaccagagcatcttaattctgatccagatgatttctccccttcgaaataattgcaaacaagattaaaactgtattcaggaagtattccagctggcttttggcttcctctgatgtacagtcctgagcctcacgccgccaacgcctctgcttccgccctgcgccgggcacttcc

SEQ ID NO: 14647 - RNA, 1474 nt, Homo sapiens
  source 1..1474: mol_type = other RNA
gctgggattacaggcatgagccaccgtgcccggcctacagttttcatgagtggctgtgaatccagagattggtctaattcttctgaatcagggcactctgcttaaggcaccaccaaatagatgtctcaccgtgatcctctggaataattgcattatttgttacattctttgcaactaaatgaattatgtgggtagaacaccacttgaatcacaaagtatcagcccgtgtgctagaagccaatttgatttgacaaaggtttgtccaacgacaattattatgcttatattcagatatgctgtttggctcattttattttgttctgttttgattaattgaattttgttatttttggttgattattttcaccacctttttccctgtgtgcataactcccacagacatgccttctacgccatcattatccttagtggaaatgaaatcccaaatatttgcagagggatttatgttgtagttattgttgctttcagttgctgctcttcgcttgtttgtaaaatagtctcactggctgttttctgggtttttgttttttttcttctactaataagtgcttccttggggcctgatgcaggtggcccatctgagtaaaagagtgcttgctgtgaacctgggaatggctctcccctgagatgacccagggttgcacagggcagtcgtcatcatcctccttgtgcaggggtgaccctcagacacagccaattaacccacgcagccctgctttcttgcagtcgtgaccatgatggtcagcgtgcccattccacgtccatgtgtggctccttcgctgctgccttcacagccccttctgactggtgtgggatgaatcaggtaagaagtcaccagggccattcattctggccccagatcacaccttccctgctcagaaatgacacctccctgcactcgcacccacagatggtcctgagtcagaagcctggcacctgggtcgggcagccgggtaagagtgtgcactttcatcgtctattcatacccgtcctgggaaaatctttccagcctgggaaatggcaacctgacacgtttcaccgggactcaacttcctgagcgtatgcacagaaaaccccacacccttcacctttattgaacaaggagggagcccgataagaatcgctgaagaaacgcggggagtgtcccgcacaaccggatgggtgtggcaggcagcgtgggcgagtagagtgacctggggcggaagaggtgtctgaatttgcgtggctccagcggctcaacccctccgagtcttcagtgcagtatagtgatccattatctccagtgtctaatttgggagcgggaccaggagtaaagttcatgaaatgttaggtgggttagagaccactgagccatcctctgcctgacatgggcatcttgaaactgccttgtggccatgtgctgcatccatggtcttgtccctggaaaagaaacaaaaagggacatgagaacagg

SEQ ID NO: 14648 - RNA, 1930 nt, Homo sapiens
  source 1..1930: mol_type = other RNA
gctgggattacaggcatgagccaccgtgcccggcctacagttttcatgagtggctgtgaatccagagattggtctaattcttctgaatcagggcactctgcttaaggcaccaccaaatagatgtctcaccgtgatcctctggaataattgcattatttgttacattctttgcaactaaatgaattatgtgggtagaacaccacttgaatcacaaagtatcagcccgtgtgctagaagccaatttgatttgacaaaggtttgtccaacgacaattattatgcttatattcagatatgctgtttggctcattttattttgttctgttttgattaattgaattttgttatttttggttgattattttcaccacctttttccctgtgtgcataactcccacagacatgccttctacgccatcattatccttagtggaaatgaaatcccaaatatttgcagagggatttatgttgtagttattgttgctttcagttgctgctcttcgcttgtttgtaaaatagtctcactggctgttttctgggtttttgttttttttcttctactaataagtgcttccttggggcctgatgcaggtggcccatctgagtaaaagagtgcttgctgtgaacctgggaatggctctcccctgagatgacccagggttgcacagggcagtcgtcatcatcctccttgtgcaggggtgaccctcagacacagccaattaacccacgcagccctgctttcttgcagtcgtgaccatgatggtcagcgtgcccattccacgtccatgtgtggctccttcgctgctgccttcacagccccttctgactggtgtgggatgaatcaggtaagaagtcaccagggccattcattctggccccagatcacaccttccctgctcagaaatgacacctccctgcactcgcacccacagatggtcctgagtcagaagcctggcacctgggtcgggcagccgggtaagagtgtgcactttcatcgtctattcatacccgtcctgggaaaatctttccagcctgggaaatggcaacctgacacgtttcaccgggactcaacttcctgagcgtatgcacagaaaaccccacacccttcacctttattgaacaaggagggagcccgataagaatcgctgaagaaacgcggggagtgtcccgcacaaccggatgggtgtggcaggcagcgtgggcgagtagagtgacctggggcggaagaggtgtctgaatttgcgtggctccagcggctcaacccctccgagtcttcagtgcagtatctgtgcaaaagagaaaagctttgtagatactctctgaaatcggcactgagcagatacccatttcttttcctttcgcatttgcagaatgtaatatttctaggggagcagaaagaattggttaggaaaaggctgttaaggaaggaggtaagtagacagagacggggtttgctggaaataatgaggaaaaagctcgaggccacttatgcacctgctgtcacgattcagctgggaccttctgaatcatacgaacccagaaaggacagctgtgctgtgtgcgttgtgcgaatgaccatttgctagaataacgtatctccagaataatttgtttaggggcaattttatgtgtgtacatggtattcacaaatgttttatccccacagttaattcaatgcagggacagttaaccctttttttcccagggaatttgggactgacctaaggactctctggcctccactcctattgccacacaagtttctgctgaggcaggaaccaccatgccttccagggacctccagtcaaaatcaatgaagtctgcaaacaatttcaactgtagtattgtagccccaataaataaagagcacttattaaaacatattgactcgaaaaatatttgacatggtgtgtttgtaacaggagaatggg

SEQ ID NO: 14649 - RNA, 5113 nt, Homo sapiens
  source 1..5113: mol_type = other RNA
gctgggattacaggcatgagccaccgtgcccggcctataacagtttcttatacatacgttactggccagcagtttcagctagcaacacaaatcaggtgagaggtgaagtgagtgataacctcatttcacctttctcacttgacacctttatctgttctttgttatggttcacagagtgttctactgatgtgtgagttcagtcatgctataaacctattttattttgtgggcctgtatttcgttattgaaccacagtcctggagccagccatcttctccacagattaagaggctgttgctagaactccaccatcaccacccatagaaaaagcactttaaattttcatgttgtggtaatggggtttgaaaggttggtagcatttttgcataagcagatcagcccattcccaagcggctttacacagcctctgacagtaacaaaccacgttctcattggtaccttaaagagtttaggagtcaaacccaaggatttgtccatgactgaaataagagcttaattataagtaattaagtcagcagatatttgagtacctgtaagcagcaggcgctgtgctaaaaagtggggacacagcagtgagcaagataggcatgtgcttatccttagataaacttcacttttaagactactactggagcctgaaagaggaaacagatgtagggtggtcaaaggtgtgacctagaggagcctgaagagcagaagtgccctgacttgaccaactcacagcagttcaagtaagatcctgttgagttaggtgtgctatgatatctgccccttcacagccatactgcacatgcaggctgtgtcacttcctaaagaggcgcccactctgcttgcttctctaccctgcagtcctcctttaaaccatctgcctaatcagctatgtatctgtactccctgtccctgtcctccgcccaattctgtatacgtttattctttgcataattcttaataagtagttgattggtgccctgtttcttaagaagtttcataatggaaagaggagaagctgatgaggagtctgcgtggagaagtgatggtaccacagaagtggaaggaggattagaaatgccagtcgatcaatctgtgagggctgtgggagataacagaaaaatggaggaaaaaaatcatagattatatagcatggtgttcgtggctgggatcaccaaatccctcttacccggggtaaaggactacatacaaggctgtgttaactttcattaaccttgaaagggaagaaatttaatttgaatttactgtgtggccggccctcttccaaaaagttcaagatgcacctaatgcaagaactaattcttgttctttttgtcacttccagataccaaggctcaaactgtttagcaggaatcactatccttcacctgtacaaagcattctgccacaccaggttataggacagattgccaccttctgtctcccccctcctcccacagactacctactaacagttcattcttcactcacttttctgtctctgaaacatccctttctttagttttctctaaccattattagcacctaatcccacccagattaaggcacctagagtgcccccaagacacaaaggtttcaagtcagtgaaagaaggtctgaccctccccacagatggctcacctttttcaggcaaatatgctcccaatggtggaagctaagatgatcgcaaggataatacagcagatcatgatcatgatcttcttctgctcatccagacaaggaaagaaagaatacatgagaaacatcatcgcaaaaagtattctgcagggagataagtgcatgtggacatggaagagggtgtgaaggaagagagcaacagaaggaaaaaggagatggatctggcttctaggacccagaatgccaacagaaatgttatttttggtgagacattcaagttagattaaaaggatgtttggtatggtcattccaccttctagataacatcgtgacagatctcccccatttcctcctaaagccagatactcccaaggactgaaccaaattcttttggggggaacacctcaaatctgaaacacaaacatagttacactgcattctgtgggagttaaaccatgttcaaaaattgcacttttgaaccatctgatccagcacatggcttaaaaaggtgtgaactgcattctaaaacctgaataaaaatcaccacatggtggcaccagatcattgtgtttctgcatcgagacagagccagaaccgtttcacaatcaatacaaagtcatttttatttttaaattagcaataaaataatcaagtttacatctaaaaaatacaaacaacaacaaaaaccttcacatgttgtattccaaactgtaagccccaggcctcaatgtcagaggagagcaaaggcctttagttattttgtctcttgttgctggagcccatccactgtctgacatcatagccatgggcaagaggatattgccttggctctgtctgagtgctggattgtgaccggccataagtagcctttgcaaaggaagctaatggacagtgcctgaattaagggtgcttaccctatcctagaaagcgttaaagtcaaagcggaaaatatacatggtacccaaaatcaaggagactgccagagaccagcaggggatctaagggatttaccactgggttagcacagacactacacttgaagatttcctagcggctgctgctgctgtttccatgataagaattcagtgagacaaagaacctgccaagctcattaaccgagtagcaggaagagctactgtgtagcctctggtgttccccaactgactcagccctgcagatgggacatcctgtaggtcatgtgaatatcaagttactgagggatgttctcaggacaagcctagcataggcaccaggtgggaaagggtgtcaaaaaattataccttctgtctgctaagcagaaaaacttaattgggatcaatttagctcactccagagttctcattttattctcccagtattcatccagaaaacaagtttcttgatgatatgggaagatcacatttccacagtgattcatttgcaggtaagcaaatgtcctttacccaatttttatcctagctcaaagttggctttttttttttgaggtcataatagcttccatttttatttcctacttcctgagacacacacacttatgtgtacatacatttcatacacaattagaatacatctggaacacatgagtgaatacaccagtgtcatgaaatatttccagagcttaggattctagcaccttgtcccttgcccaatttaaaatccctgattatttttggccccaagacaatagtctcacaaagcatcactttctaacaatgagcagccagtttctaagactcagacatggaaacatattccataccgtcagccttttgcaaagcataacctcagatgactgtatcatcctggtccctccttgagtaaatatgagagactacaacacagagaaaaatcaaagttgccccccaagctgaacaactaagagcttaatttaaggctgaatttcaaacaagtcagctctttagaccaaaatgacatctgccagtccctcatgttttcaggacatacggacaacaaacaggattggcatcctgccaggtagaagactcagatccaagccttcttgttgccaaacttagaagaatcattctgctttgttaaagatactcccctaaaaaaatacattgcagtttctgggagaatactccatgaggtagaaaaatacagcaccttgggagagtctcacaagagctttcccaagtgcaaggcataatctgacacacaacagggaggaagaaagctgggtgggtccacacagtccaggagaaaaggtacttgagagctggtggggcaggaggaggctctggggagaactcagggtcgcatcaggtagatcacattcccccagggctagattgttagctgagtcaggtccaagggtggttgcaaggaaacaaaggaacgggtcgcactcgctctcaggaaggccattcagactccattctcatctgaagacaagggtggccacaccagtctggagtgaaatcagtttatttcagtgcagcagcctcttaggccactcttaattcagcccaacggaaagtccaataatcaatgctaaaatgcccagcaacacaactactagcacaatgataattatcaatttctgattctccaccagcatggcgatgtccataaacatgtcgtgaagctccttgatgctgctctccagcctcacaatgtccttgtgtcgtccctcaatctcactgagggcttgcttggaaatctgtgagtcaatgatcccagaagtgaagatggccgggttgccactctccaacatctcctccagctcctcatcggttgtctttttgccagtaatttcgagctgccgctggattcgccctttgctgcgttctcggaagtccacttgagcttcattgtatttggtcatcacctccacaaacttccgagaaaggacagagtgctgggatttccgaatccgaaggtctgccgatgacctgacctcatcttcttcaatatgcttctccatgctcttcagtttgttccggacgttgttggcccttttcttaatctcagtcgtgagctgctctaggtcatccttggtttttggctctggaatcggtgcagagagaatgatactgtagagtttcttagcctcctctacatgttctgagatcttgtcaatgttaagccgagtttcctcaatctcagaaaagaactcgtccataaaagccgtgttgtcgatagcaatctcaaccgcatcagtatcatcatcctgtgtcagctgcttggccttcagctgctccagacggtccttcatcctgaagcccaggcgcccggaggcaggtagcgcgtcccaggtgagcgcgtcccaggtgagcgcttcccaggtgagctgccggaagcggcggccgggcccgccggggcgaaggagctggaggcgcaggcggcggcgggcggcggccgctagctaggaggagcgtccgaggccacgggagcctccgccgcgcagccccctccgcccccaccggcgcctcgcgctccaaat

SEQ ID NO: 14650 - RNA, 5226 nt, Homo sapiens
  source 1..5226: mol_type = other RNA
gctgggattacaggcatgagccaccgtgcccggcctataacagtttcttatacatacgttactggccagcagtttcagctagcaacacaaatcaggtgagaggtgaagtgagtgataacctcatttcacctttctcacttgacacctttatctgttctttgttatggttcacagagtgttctactgatgtgtgagttcagtcatgctataaacctattttattttgtgggcctgtatttcgttattgaaccacagtcctggagccagccatcttctccacagattaagaggctgttgctagaactccaccatcaccacccatagaaaaagcactttaaattttcatgttgtggtaatggggtttgaaaggttggtagcatttttgcataagcagatcagcccattcccaagcggctttacacagcctctgacagtaacaaaccacgttctcattggtaccttaaagagtttaggagtcaaacccaaggatttgtccatgactgaaataagagcttaattataagtaattaagtcagcagatatttgagtacctgtaagcagcaggcgctgtgctaaaaagtggggacacagcagtgagcaagataggcatgtgcttatccttagataaacttcacttttaagactactactggagcctgaaagaggaaacagatgtagggtggtcaaaggtgtgacctagaggagcctgaagagcagaagtgccctgacttgaccaactcacagcagttcaagtaagatcctgttgagttaggtgtgctatgatatctgccccttcacagccatactgcacatgcaggctgtgtcacttcctaaagaggcgcccactctgcttgcttctctaccctgcagtcctcctttaaaccatctgcctaatcagctatgtatctgtactccctgtccctgtcctccgcccaattctgtatacgtttattctttgcataattcttaataagtagttgattggtgccctgtttcttaagaagtttcataatggaaagaggagaagctgatgaggagtctgcgtggagaagtgatggtaccacagaagtggaaggaggattagaaatgccagtcgatcaatctgtgagggctgtgggagataacagaaaaatggaggaaaaaaatcatagattatatagcatggtgttcgtggctgggatcaccaaatccctcttacccggggtaaaggactacatacaaggctgtgttaactttcattaaccttgaaagggaagaaatttaatttgaatttactgtgtggccggccctcttccaaaaagttcaagatgcacctaatgcaagaactaattcttgttctttttgtcacttccagataccaaggctcaaactgtttagcaggaatcactatccttcacctgtacaaagcattctgccacaccaggttataggacagattgccaccttctgtctcccccctcctcccacagactacctactaacagttcattcttcactcacttttctgtctctgaaacatccctttctttagttttctctaaccattattagcacctaatcccacccagattaaggcacctagagtgcccccaagacacaaaggtttcaagtcagtgaaagaaggtctgaccctccccacagatggctcacctttttcaggcaaatatgctcccaatggtggaagctaagatgatcgcaaggataatacagcagatcatgatcatgatcttcttctgctcatccagacaaggaaagaaagaatacatgagaaacatcatcgcaaaaagtattctgcagggagataagtgcatgtggacatggaagagggtgtgaaggaagagagcaacagaaggaaaaaggagatggatctggcttctaggacccagaatgccaacagaaatgttatttttggtgagacattcaagttagattaaaaggatgtttggtatggtcattccaccttctagataacatcgtgacagatctcccccatttcctcctaaagccagatactcccaaggactgaaccaaattcttttggggggaacacctcaaatctgaaacacaaacatagttacactgcattctgtgggagttaaaccatgttcaaaaattgcacttttgaaccatctgatccagcacatggcttaaaaaggtgtgaactgcattctaaaacctgaataaaaatcaccacatggtggcaccagatcattgtgtttctgcatcgagacagagccagaaccgtttcacaatcaatacaaagtcatttttatttttaaattagcaataaaataatcaagtttacatctaaaaaatacaaacaacaacaaaaaccttcacatgttgtattccaaactgtaagccccaggcctcaatgtcagaggagagcaaaggcctttagttattttgtctcttgttgctggagcccatccactgtctgacatcatagccatgggcaagaggatattgccttggctctgtctgagtgctggattgtgaccggccataagtagcctttgcaaaggaagctaatggacagtgcctgaattaagggtgcttaccctatcctagaaagcgttaaagtcaaagcggaaaatatacatggtacccaaaatcaaggagactgccagagaccagcaggggatctaagggatttaccactgggttagcacagacactacacttgaagatttcctagcggctgctgctgctgtttccatgataagaattcagtgagacaaagaacctgccaagctcattaaccgagtagcaggaagagctactgtgtagcctctggtgttccccaactgactcagccctgcagatgggacatcctgtaggtcatgtgaatatcaagttactgagggatgttctcaggacaagcctagcataggcaccaggtgggaaagggtgtcaaaaaattataccttctgtctgctaagcagaaaaacttaattgggatcaatttagctcactccagagttctcattttattctcccagtattcatccagaaaacaagtttcttgatgatatgggaagatcacatttccacagtgattcatttgcaggtaagcaaatgtcctttacccaatttttatcctagctcaaagttggctttttttttttgaggtcataatagcttccatttttatttcctacttcctgagacacacacacttatgtgtacatacatttcatacacaattagaatacatctggaacacatgagtgaatacaccagtgtcatgaaatatttccagagcttaggattctagcaccttgtcccttgcccaatttaaaatccctgattatttttggccccaagacaatagtctcacaaagcatcactttctaacaatgagcagccagtttctaagactcagacatggaaacatattccataccgtcagccttttgcaaagcataacctcagatgactgtatcatcctggtccctccttgagtaaatatgagagactacaacacagagaaaaatcaaagttgccccccaagctgaacaactaagagcttaatttaaggctgaatttcaaacaagtcagctctttagaccaaaatgacatctgccagtccctcatgttttcaggacatacggacaacaaacaggattggcatcctgccaggtagaagactcagatccaagccttcttgttgccaaacttagaagaatcattctgctttgttaaagatactcccctaaaaaaatacattgcagtttctgggagaatactccatgaggtagaaaaatacagcaccttgggagagtctcacaagagctttcccaagtgcaaggcataatctgacacacaacagggaggaagaaagctgggtgggtccacacagtccaggagaaaaggtacttgagagctggtggggcaggaggaggctctggggagaactcagggtcgcatcaggtagatcacattcccccagggctagattgttagctgagtcaggtccaagggtggttgcaaggaaacaaaggaacgggtcgcactcgctctcaggaaggccattcagactccattctcatctgaagacaagggtggccacaccagtctggagtgaaatcagtttatttcagtgcagcagcctcttaggccactcttaattcagcccaacggaaagtccaataatcaatgctaaaatgcccagcaacacaactactagcacaatgataattatcaatttcttccgggcctgactctggtatttcacagcttttttcgtttcatctcgtgccttctccacgtggtccactgtgtgcatgacattcaactctatgttatctaacatctcaccctgattctccaccagcatggcgatgtccataaacatgtcgtgaagctccttgatgctgctctccagcctcacaatgtccttgtgtcgtccctcaatctcactgagggcttgcttggaaatctgtgagtcaatgatcccagaagtgaagatggccgggttgccactctccaacatctcctccagctcctcatcggttgtctttttgccagtaatttcgagctgccgctggattcgccctttgctgcgttctcggaagtccacttgagcttcattgtatttggtcatcacctccacaaacttccgagaaaggacagagtgctgggatttccgaatccgaaggtctgccgatgacctgacctcatcttcttcaatatgcttctccatgctcttcagtttgttccggacgttgttggcccttttcttaatctcagtcgtgagctgctctaggtcatccttggtttttggctctggaatcggtgcagagagaatgatactgtagagtttcttagcctcctctacatgttctgagatcttgtcaatgttaagccgagtttcctcaatctcagaaaagaactcgtccataaaagccgtgttgtcgatagcaatctcaaccgcatcagtatcatcatcctgtgtcagctgcttggccttcagctgctccagacggtccttcatcctgaagcccaggcgcccggaggcaggtagcgcgtcccaggtgagcgcgtcccaggtgagcgcttcccaggtgagctgccggaagcggcggccgggcccgccggggcgaaggagctggaggcgcaggcggcggcgggcggcggccgctagctaggaggagcgtccgaggccacgggagcctccgccgcgcagccccctccgcccccaccggcgcctcgcgctccaaatcc

SEQ ID NO: 14651 - RNA, 5112 nt, Homo sapiens
  source 1..5112: mol_type = other RNA
gctgggattacaggcatgagccaccgtgcccggcctataacagtttcttatacatacgttactggccagcagtttcagctagcaacacaaatcaggtgagaggtgaagtgagtgataacctcatttcacctttctcacttgacacctttatctgttctttgttatggttcacagagtgttctactgatgtgtgagttcagtcatgctataaacctattttattttgtgggcctgtatttcgttattgaaccacagtcctggagccagccatcttctccacagattaagaggctgttgctagaactccaccatcaccacccatagaaaaagcactttaaattttcatgttgtggtaatggggtttgaaaggttggtagcatttttgcataagcagatcagcccattcccaagcggctttacacagcctctgacagtaacaaaccacgttctcattggtaccttaaagagtttaggagtcaaacccaaggatttgtccatgactgaaataagagcttaattataagtaattaagtcagcagatatttgagtacctgtaagcagcaggcgctgtgctaaaaagtggggacacagcagtgagcaagataggcatgtgcttatccttagataaacttcacttttaagactactactggagcctgaaagaggaaacagatgtagggtggtcaaaggtgtgacctagaggagcctgaagagcagaagtgccctgacttgaccaactcacagcagttcaagtaagatcctgttgagttaggtgtgctatgatatctgccccttcacagccatactgcacatgcaggctgtgtcacttcctaaagaggcgcccactctgcttgcttctctaccctgcagtcctcctttaaaccatctgcctaatcagctatgtatctgtactccctgtccctgtcctccgcccaattctgtatacgtttattctttgcataattcttaataagtagttgattggtgccctgtttcttaagaagtttcataatggaaagaggagaagctgatgaggagtctgcgtggagaagtgatggtaccacagaagtggaaggaggattagaaatgccagtcgatcaatctgtgagggctgtgggagataacagaaaaatggaggaaaaaaatcatagattatatagcatggtgttcgtggctgggatcaccaaatccctcttacccggggtaaaggactacatacaaggctgtgttaactttcattaaccttgaaagggaagaaatttaatttgaatttactgtgtggccggccctcttccaaaaagttcaagatgcacctaatgcaagaactaattcttgttctttttgtcacttccagataccaaggctcaaactgtttagcaggaatcactatccttcacctgtacaaagcattctgccacaccaggttataggacagattgccaccttctgtctcccccctcctcccacagactacctactaacagttcattcttcactcacttttctgtctctgaaacatccctttctttagttttctctaaccattattagcacctaatcccacccagattaaggcacctagagtgcccccaagacacaaaggtttcaagtcagtgaaagaaggtctgaccctccccacagatggctcacctttttcaggcaaatatgctcccaatggtggaagctaagatgatcgcaaggataatacagcagatcatgatcatgatcttcttctgctcatccagacaaggaaagaaagaatacatgagaaacatcatcgcaaaaagtattctgcagggagataagtgcatgtggacatggaagagggtgtgaaggaagagagcaacagaaggaaaaaggagatggatctggcttctaggacccagaatgccaacagaaatgttatttttggtgagacattcaagttagattaaaaggatgtttggtatggtcattccaccttctagataacatcgtgacagatctcccccatttcctcctaaagccagatactcccaaggactgaaccaaattcttttggggggaacacctcaaatctgaaacacaaacatagttacactgcattctgtgggagttaaaccatgttcaaaaattgcacttttgaaccatctgatccagcacatggcttaaaaaggtgtgaactgcattctaaaacctgaataaaaatcaccacatggtggcaccagatcattgtgtttctgcatcgagacagagccagaaccgtttcacaatcaatacaaagtcatttttatttttaaattagcaataaaataatcaagtttacatctaaaaaatacaaacaacaacaaaaaccttcacatgttgtattccaaactgtaagccccaggcctcaatgtcagaggagagcaaaggcctttagttattttgtctcttgttgctggagcccatccactgtctgacatcatagccatgggcaagaggatattgccttggctctgtctgagtgctggattgtgaccggccataagtagcctttgcaaaggaagctaatggacagtgcctgaattaagggtgcttaccctatcctagaaagcgttaaagtcaaagcggaaaatatacatggtacccaaaatcaaggagactgccagagaccagcaggggatctaagggatttaccactgggttagcacagacactacacttgaagatttcctagcggctgctgctgctgtttccatgataagaattcagtgagacaaagaacctgccaagctcattaaccgagtagcaggaagagctactgtgtagcctctggtgttccccaactgactcagccctgcagatgggacatcctgtaggtcatgtgaatatcaagttactgagggatgttctcaggacaagcctagcataggcaccaggtgggaaagggtgtcaaaaaattataccttctgtctgctaagcagaaaaacttaattgggatcaatttagctcactccagagttctcattttattctcccagtattcatccagaaaacaagtttcttgatgatatgggaagatcacatttccacagtgattcatttgcaggtaagcaaatgtcctttacccaatttttatcctagctcaaagttggctttttttttttgaggtcataatagcttccatttttatttcctacttcctgagacacacacacttatgtgtacatacatttcatacacaattagaatacatctggaacacatgagtgaatacaccagtgtcatgaaatatttccagagcttaggattctagcaccttgtcccttgcccaatttaaaatccctgattatttttggccccaagacaatagtctcacaaagcatcactttctaacaatgagcagccagtttctaagactcagacatggaaacatattccataccgtcagccttttgcaaagcataacctcagatgactgtatcatcctggtccctccttgagtaaatatgagagactacaacacagagaaaaatcaaagttgccccccaagctgaacaactaagagcttaatttaaggctgaatttcaaacaagtcagctctttagaccaaaatgacatctgccagtccctcatgttttcaggacatacggacaacaaacaggattggcatcctgccaggtagaagactcagatccaagccttcttgttgccaaacttagaagaatcattctgctttgttaaagatactcccctaaaaaaatacattgcagtttctgggagaatactccatgaggtagaaaaatacagcaccttgggagagtctcacaagagctttcccaagtgcaaggcataatctgacacacaacagggaggaagaaagctgggtgggtccacacagtccaggagaaaaggtacttgagagctggtggggcaggaggaggctctggggagaactcagggtcgcatcaggtagatcacattcccccagggctagattgttagctgagtcaggtccaagggtggttgcaaggaaacaaaggaacgggtcgcactcgctctcaggaaggccattcagactccattctcatctgaagacaagggtggccacaccagtctggagtgaaatcagtttcttccgggcctgactctggtatttcacagcttttttcgtttcatctcgtgccttctccacgtggtccactgtgtgcatgacattcaactctatgttatctaacatctcaccctgattctccaccagcatggcgatgtccataaacatgtcgtgaagctccttgatgctgctctccagcctcacaatgtccttgtgtcgtccctcaatctcactgagggcttgcttggaaatctgtgagtcaatgatcccagaagtgaagatggccgggttgccactctccaacatctcctccagctcctcatcggttgtctttttgccagtaatttcgagctgccgctggattcgccctttgctgcgttctcggaagtccacttgagcttcattgtatttggtcatcacctccacaaacttccgagaaaggacagagtgctgggatttccgaatccgaaggtctgccgatgacctgacctcatcttcttcaatatgcttctccatgctcttcagtttgttccggacgttgttggcccttttcttaatctcagtcgtgagctgctctaggtcatccttggtttttggctctggaatcggtgcagagagaatgatactgtagagtttcttagcctcctctacatgttctgagatcttgtcaatgttaagccgagtttcctcaatctcagaaaagaactcgtccataaaagccgtgttgtcgatagcaatctcaaccgcatcagtatcatcatcctgtgtcagctgcttggccttcagctgctccagacggtccttcatcctgaagcccaggcgcccggaggcaggtagcgcgtcccaggtgagcgcgtcccaggtgagcgcttcccaggtgagctgccggaagcggcggccgggcccgccggggcgaaggagctggaggcgcaggcggcggcgggcggcggccgctagctaggaggagcgtccgaggccacgggagcctccgccgcgcagccccctccgcccccaccggcgcctcgcgctccaaatcc

SEQ ID NO: 14652 - RNA, 2510 nt, Homo sapiens
  source 1..2510: mol_type = other RNA
gctgggattacaggcatgagccaccgtgcccggcctataacagtttcttatacatacgttactggccagcagtttcagctagcaacacaaatcaggtgagaggtgaagtgagtgataacctcatttcacctttctcacttgacacctttatctgttctttgttatggttcacagagtgttctactgatgtgtgagttcagtcatgctataaacctattttattttgtgggcctgtatttcgttattgaaccacagtcctggagccagccatcttctccacagattaagaggctgttgctagaactccaccatcaccacccatagaaaaagcactttaaattttcatgttgtggtaatggggtttgaaaggttggtagcatttttgcataagcagatcagcccattcccaagcggctttacacagcctctgacagtaacaaaccacgttctcattggtaccttaaagagtttaggagtcaaacccaaggatttgtccatgactgaaataagagcttaattataagtaattaagtcagcagatatttgagtacctgtaagcagcaggcgctgtgctaaaaagtggggacacagcagtgagcaagataggcatgtgcttatccttagataaacttcacttttaagactactactggagcctgaaagaggaaacagatgtagggtggtcaaaggtgtgacctagaggagcctgaagagcagaagtgccctgacttgaccaactcacagcagttcaagtaagatcctgttgagttaggtgtgctatgatatctgccccttcacagccatactgcacatgcaggctgtgtcacttcctaaagaggcgcccactctgcttgcttctctaccctgcagtcctcctttaaaccatctgcctaatcagctatgtatctgtactccctgtccctgtcctccgcccaattctgtatacgtttattctttgcataattcttaataagtagttgattggtgccctgtttcttaagaagtttcataatggaaagaggagaagctgatgaggagtctgcgtggagaagtgatggtaccacagaagtggaaggaggattagaaatgccagtcgatcaatctgtgagggctgtgggagataacagaaaaatggaggaaaaaaatcatagattatatagcatggtgttcgtggctgggatcaccaaatccctcttacccggggtaaaggactacatacaaggctgtgttaactttcattaaccttgaaagggaagaaatttaatttgaatttactgtgtggccggccctcttccaaaaagttcaagatgcacctaatgcaagaactaattcttgttctttttgtcacttccagataccaaggctcaaactgtttagcaggaatcactatccttcacctgtacaaagcattctgccacaccaggttataggacagattgccaccttctgtctcccccctcctcccacagactacctactaacagttcattcttcactcacttttctgtctctgaaacatccctttctttagttttctctaaccattattagcacctaatcccacccagattaaggcacctagagtgcccccaagacacaaaggtttcaagtcagtgaaagaaggtctgaccctccccacagatggctcacctttttcaggcaaatatgctcccaatggtggaagctaagatgatcgcaaggataatacagcagatcatgatcatgatcttcttcttccgggcctgactctggtatttcacagcttttttcgtttcatctcgtgccttctccacgtggtccactgtgtgcatgacattcaactctatgttatctaacatctcaccctgattctccaccagcatggcgatgtccataaacatgtcgtgaagctccttgatgctgctctccagcctcacaatgtccttgtgtcgtccctcaatctcactgagggcttgcttggaaatctgtgagtcaatgatcccagaagtgaagatggccgggttgccactctccaacatctcctccagctcctcatcggttgtctttttgccagtaatttcgagctgccgctggattcgccctttgctgcgttctcggaagtccacttgagcttcattgtatttggtcatcacctccacaaacttccgagaaaggacagagtgctgggatttccgaatccgaaggtctgccgatgacctgacctcatcttcttcaatatgcttctccatgctcttcagtttgttccggacgttgttggcccttttcttaatctcagtcgtgagctgctctaggtcatccttggtttttggctctggaatcggtgcagagagaatgatactgtagagtttcttagcctcctctacatgttctgagatcttgtcaatgttaagccgagtttcctcaatctcagaaaagaactcgtccataaaagccgtgttgtcgatagcaatctcaaccgcatcagtatcatcatcctgtgtcagctgcttcatcatgggatggattaaagg

SEQ ID NO: 14653 - RNA, 2322 nt, Homo sapiens
  source 1..2322: mol_type = other RNA
gctgggattacaggcatgagccaccgtgcccggcctataacagtttcttatacatacgttactggccagcagtttcagctagcaacacaaatcaggtgagaggtgaagtgagtgataacctcatttcacctttctcacttgacacctttatctgttctttgttatggttcacagagtgttctactgatgtgtgagttcagtcatgctataaacctattttattttgtgggcctgtatttcgttattgaaccacagtcctggagccagccatcttctccacagattaagaggctgttgctagaactccaccatcaccacccatagaaaaagcactttaaattttcatgttgtggtaatggggtttgaaaggttggtagcatttttgcataagcagatcagcccattcccaagcggctttacacagcctctgacagtaacaaaccacgttctcattggtaccttaaagagtttaggagtcaaacccaaggatttgtccatgactgaaataagagcttaattataagtaattaagtcagcagatatttgagtacctgtaagcagcaggcgctgtgctaaaaagtggggacacagcagtgagcaagataggcatgtgcttatccttagataaacttcacttttaagactactactggagcctgaaagaggaaacagatgtagggtggtcaaaggtgtgacctagaggagcctgaagagcagaagtgccctgacttgaccaactcacagcagttcaagtaagatcctgttgagttaggtgtgctatgatatctgccccttcacagccatactgcacatgcaggctgtgtcacttcctaaagaggcgcccactctgcttgcttctctaccctgcagtcctcctttaaaccatctgcctaatcagctatgtatctgtactccctgtccctgtcctccgcccaattctgtatacgtttattctttgcataattcttaataagtagttgattggtgccctgtttcttaagaagtttcataatggaaagaggagaagctgatgaggagtctgcgtggagaagtgatggtaccacagaagtggaaggaggattagaaatgccagtcgatcaatctgtgagggctttttcaggcaaatatgctcccaatggtggaagctaagatgatcgcaaggataatacagcagatcatgatcatgatcttcttatttcagtgcagcagcctcttaggccactcttaattcagcccaacggaaagtccaataatcaatgctaaaatgcccagcaacacaactactagcacaatgataattatcaatttcttccgggcctgactctggtatttcacagcttttttcgtttcatctcgtgccttctccacgtggtccactgtgtgcatgacattcaactctatgttatctaacatctcaccctgattctccaccagcatggcgatgtccataaacatgtcgtgaagctccttgatgctgctctccagcctcacaatgtccttgtgtcgtccctcaatctcactgagggcttgcttggaaatctgtgagtcaatgatcccagaagtgaagatggccgggttgccactctccaacatctcctccagctcctcatcggttgtctttttgccagtaatttcgagctgccgctggattcgccctttgctgcgttctcggaagtccacttgagcttcattgtatttggtcatcacctccacaaacttccgagaaaggacagagtgctgggatttccgaatccgaaggtctgccgatgacctgacctcatcttcttcaatatgcttctccatgctcttcagtttgttccggacgttgttggcccttttcttaatctcagtcgtgagctgctctaggtcatccttggtttttggctctggaatcggtgcagagagaatgatactgtagagtttcttagcctcctctacatgttctgagatcttgtcaatgttaagccgagtttcctcaatctcagaaaagaactcgtccataaaagccgtgttgtcgatagcaatctcaaccgcatcagtatcatcatcctgtgtcagctgcttggccttcagctgctccagacggtccttcatcctgaagcccaggcgcccggaggcaggtagcgcgtcccaggtgagcgcgtcccaggtgagcgcttcccaggtgagctgccggaagcggcggccgggcccgccggggcgaaggagctggaggcgcaggcggcggcgggcggcggccgctagctaggaggagcgtccgaggccacgggagcctccgccgcgcagccccctccgcccccaccggcgcctcgcgctccaaat

SEQ ID NO: 14654 - RNA, 1971 nt, Homo sapiens
  source 1..1971: mol_type = other RNA
gctgggattacaggcatgagccaccgtgcccggcctataacagtttcttatacatacgttactggccagcagtttcagctagcaacacaaatcaggtgagaggtgaagtgagtgataacctcatttcacctttctcacttgacacctttatctgttctttgttatggttcacagagtgttctactgatgtgtgagttcagtcatgctataaacctattttattttgtgggcctgtatttcgttattgaaccacagtcctggagccagccatcttctccacagattaagaggctgttgctagaactccaccatcaccacccatagaaaaagcactttaaattttcatgttgtggtaatggggtttgaaaggttggtagcatttttgcataagcagatcagcccattcccaagcggctttacacagcctctgacagtaacaaaccacgttctcattggtaccttaaagagtttaggagtcaaacccaaggatttgtccatgactgaaataagagcttaattataagtaattaagtcagcagatatttgagtacctgtaagcagcaggcgctgtgctaaaaagtggggacacagcagtgagcaagataggcatgtgcttatccttagataaacttcacttttaagactactactggagcctgaaagaggaaacagatgtagggtggtcaaaggtgtgacctagaggagcctgaagagcagaagtgccctgacttgaccaactcacagcagttcaagtaagatcctgttgagttaggtgtgctatgatatctgccccttcacagccatactgcacatgcaggctgtgtcacttcctaaagaggcgcccactctgcttgcttctctaccctgcagtcctcctttaaaccatctgcctaatcagctatgtatctgtactccctgtccctgtcctccgcccaattctgtatacgtttattctttgcataattcttaataagtagttgattggtgccctgtttcttaagaagtttcataatggaaagaggagaagctgatgaggagtctgcgtggagaagtgatggtaccacagaagtggaaggaggattagaaatgccagtcgatcaatctgtgagggctttttcaggcaaatatgctcccaatggtggaagctaagatgatcgcaaggataatacagcagatcatgatcatgatcttcttcttccgggcctgactctggtatttcacagcttttttcgtttcatctcgtgccttctccacgtggtccactgtgtgcatgacattcaactctatgttatctaacatctcaccctgattctccaccagcatggcgatgtccataaacatgtcgtgaagctccttgatgctgctctccagcctcacaatgtccttgtgtcgtccctcaatctcactgagggcttgcttggaaatctgtgagtcaatgatcccagaagtgaagatggccgggttgccactctccaacatctcctccagctcctcatcggttgtctttttgccagtaatttcgagctgccgctggattcgccctttgctgcgttctcggaagtccacttgagcttcattgtatttggtcatcacctccacaaacttccgagaaaggacagagtgctgggatttccgaatccgaaggtctgccgatgacctgacctcatcttcttcaatatgcttctccatgctcttcagtttgttccggacgttgttggcccttttcttaatctcagtcgtgagctgctctaggtcatccttggtttttggctctggaatcggtgcagagagaatgatactgtagagtttcttagcctcctctacatgttctgagatcttgtcaatgttaagccgagtttcctcaatctcagaaaagaactcgtccataaaagccgtgttgtcgatagcaatctcaaccgcatcagtatcatcatcctgtgtcagctgcttcatcatgggatggattaaagg

SEQ ID NO: 14655 - RNA, 2208 nt, Homo sapiens
  source 1..2208: mol_type = other RNA
gctgggattacaggcatgagccaccgtgcccggcctataacagtttcttatacatacgttactggccagcagtttcagctagcaacacaaatcaggtgagaggtgaagtgagtgataacctcatttcacctttctcacttgacacctttatctgttctttgttatggttcacagagtgttctactgatgtgtgagttcagtcatgctataaacctattttattttgtgggcctgtatttcgttattgaaccacagtcctggagccagccatcttctccacagattaagaggctgttgctagaactccaccatcaccacccatagaaaaagcactttaaattttcatgttgtggtaatggggtttgaaaggttggtagcatttttgcataagcagatcagcccattcccaagcggctttacacagcctctgacagtaacaaaccacgttctcattggtaccttaaagagtttaggagtcaaacccaaggatttgtccatgactgaaataagagcttaattataagtaattaagtcagcagatatttgagtacctgtaagcagcaggcgctgtgctaaaaagtggggacacagcagtgagcaagataggcatgtgcttatccttagataaacttcacttttaagactactactggagcctgaaagaggaaacagatgtagggtggtcaaaggtgtgacctagaggagcctgaagagcagaagtgccctgacttgaccaactcacagcagttcaagtaagatcctgttgagttaggtgtgctatgatatctgccccttcacagccatactgcacatgcaggctgtgtcacttcctaaagaggcgcccactctgcttgcttctctaccctgcagtcctcctttaaaccatctgcctaatcagctatgtatctgtactccctgtccctgtcctccgcccaattctgtatacgtttattctttgcataattcttaataagtagttgattggtgccctgtttcttaagaagtttcataatggaaagaggagaagctgatgaggagtctgcgtggagaagtgatggtaccacagaagtggaaggaggattagaaatgccagtcgatcaatctgtgagggctttttcaggcaaatatgctcccaatggtggaagctaagatgatcgcaaggataatacagcagatcatgatcatgatcttcttcttccgggcctgactctggtatttcacagcttttttcgtttcatctcgtgccttctccacgtggtccactgtgtgcatgacattcaactctatgttatctaacatctcaccctgattctccaccagcatggcgatgtccataaacatgtcgtgaagctccttgatgctgctctccagcctcacaatgtccttgtgtcgtccctcaatctcactgagggcttgcttggaaatctgtgagtcaatgatcccagaagtgaagatggccgggttgccactctccaacatctcctccagctcctcatcggttgtctttttgccagtaatttcgagctgccgctggattcgccctttgctgcgttctcggaagtccacttgagcttcattgtatttggtcatcacctccacaaacttccgagaaaggacagagtgctgggatttccgaatccgaaggtctgccgatgacctgacctcatcttcttcaatatgcttctccatgctcttcagtttgttccggacgttgttggcccttttcttaatctcagtcgtgagctgctctaggtcatccttggtttttggctctggaatcggtgcagagagaatgatactgtagagtttcttagcctcctctacatgttctgagatcttgtcaatgttaagccgagtttcctcaatctcagaaaagaactcgtccataaaagccgtgttgtcgatagcaatctcaaccgcatcagtatcatcatcctgtgtcagctgcttggccttcagctgctccagacggtccttcatcctgaagcccaggcgcccggaggcaggtagcgcgtcccaggtgagcgcgtcccaggtgagcgcttcccaggtgagctgccggaagcggcggccgggcccgccggggcgaaggagctggaggcgcaggcggcggcgggcggcggccgctagctaggaggagcgtccgaggccacgggagcctccgccgcgcagccccctccgcccccaccggcgcctcgcgctccaaat

SEQ ID NO: 14656 - RNA, 4065 nt, Homo sapiens
  source 1..4065: mol_type = other RNA
gctgggattacaggcatgagccaccgtgcccggcctattttttaaattttttgcagagatgggatctccttatgttgcccaggctggtctcgaactcctgagctcaggtgatcccctcacttttgccttctaaagtgtgggattacaggcatgagccatggggcctggccagggagacttttctatccatgctgcacggcaatcttgtcctccttttgctagaagaaataagactcttggggctaggaagaaccttaaatgtcaaattccattttctcttgtcagatgacaaaagtaaatcagcatttcctttaaaaatcggagcactgactttggtcctattcaaaatagctaccttcaattagaattagggtaaaaaatgattcaccataatgttgtttaactttctctcttttttttttttttcaaattactagaattttattagccaagggatagcagctggaggagaaataacaaaaaaatacatcttaagaatccttaagtacagtgcatatttacaatttaagtgtcatattttagaaggccactgtccatcagctcagtaaatgtaccagcttctaaagccatgatgccataggtccatttgttgatgaaattcctacccactgtcctcgggcatctgactctggtctctgcactggcatcaagagaacgctgctcggtggtttaaggctaacaccttacagggtaacactgtaacactggccctggagccaggtgcttttctccatgaaaacttccaccttggtagctcagccgacatagacaacacacaaagcgcagctctgcacttctgtccttatcttcacacagtgacatccacaccaggtggccaaacagaagagaaggcagaggcccaccaagagctgatgctgcgcagtccttgggggatcatcctccggtctcactggggacgaacccaggttctggagcctctcccctgacagacagcttgtcaccggcacttatgggtcctctgggatttcagacaatacccaacttctgtaggttcagaaagtgctttcaagcaggcagtggcacccacacccggtgggacacacctcctgggtccgaaaccactccatcatgtggctggtgtggccaccgtgcccacaggtcaggcagaaattggacgatccccgcacagccacgtgacagatggcacactggaacgtgaagcctttgcagatggcacactgcgtgccacggacctcactccggcagtggctgcagtacacgccgaactcgatccctttgtgagggtcaggaggacaggagacaaacttcaacacttcagctcgcttctctctcagaccccaacggtagaggatttccccatagcatttcttaaagtcatcaaattgctgggtattggcggggtccaggagccttttatttttatcatgctggtcgcgttctcgctcacggggatcactgtaggtcagactcccaaagcggagctcttctggtgaggattctccccaaggggaggacaagtgctctgcctctcttcccgctatgttccagccgccagtgttgagccctgggtctgacatactggagcaggaaccagaagaggtaaagctaggatatcgactatgggacaccacaagattagaagaacggttaggaaaaggcccaaaggggtttggtagcccctgaggccgagactgggcttcaaacacgctacagagcatcgccagtgtctgaacatcccggagccggcaatagtgagccaacagggactccagcagctgccgcccaaatggatgtcgagcccagggtgtttccaaatctgggtcagatttcggaccaaggcaaagatctgtagctaccgtagccagcgaccaaacctggacaagatcctttcttccaacgagcaaggcagaggcggcattcttctgacatgtttcctgaatatcattcacattcaatatgtacagctctcccagcgatttgtgaacaggcaggaggcaagcaatatcctggatgatgactttcccagcagccttgatctgtcgattgccagagtctgatccctcacgcttacttttccatcgtcttgatttccgctccttgtagtagaaggagctgatggagacctgctctttctcgctgcgagtggggctcccactgtataaacgaaggttcccaggggcctctgtgcggatcttcatgggcgcgatcaagccagtgtgataagcagacaaggctgagagagatctcggagtaggctctgtgggagacaccgcccgatgcattgtcatgggccttgtgaaatataccaggtaacctgctccgcagaacctggccccagaagtcctaggaaagggaatgttggcgtcctggtacgacccgtaagccgtggtcacccgcgcaaacgtcggtaaggggggagtgacagagttggggagtgcaaacgggttgctggaagcgctgtcttcctggttcacaaaggactcaaggcaggagacgagctggcgcaggcagggctccaggcagctctggccacgcttcactttctgcagggctgtgtccttcaggatcttcagcagcttagctttcatggtggatgtgatggttgtggggttaataaactggaaggaaggggcggcgttgtttgggtactgtgcagggaacttcaccagcatcttgacacgatggttgctgcagtgcacagacactgtgcagctcctgtctgccgcatccatctccacattgacattccggatttgcacattgatcagggagaattcctgctgcaaggtctgaggcagccccagttgatctgatttcctctcttccaggagatttctagggggatcttcttttagggcttcttcctccccatggcttgcagtgtgctggtgatctgtatcttcagtgtgcagggtcttctcaggttccggcagaagggaaatactctcaatgaactcatcaacaccatctaatatgtcatttgcacaaagcctctgcatctgggaatccacccgccacattctcaaggtctgatcccgggaccacgtcaccagttgatagtccttggacccttccttctgcttcctccactggaactccaggaccacatcatcatgccccacgaaggtgtggactggggtgttcaagtcaaagacattccacaggagaaggctgttttccctccgcagctggggaaccatcacagtcaccaatccattgctgaaaggtgtgtatctggccttccagacaggcacctggcaaggaagaatattgaggtatttccgaggctggcggtaatcccagaacttcacagaattgtcttgactggaggtagcaagaatgtgctcgctgtctgggtgccagtccaggccatggattttggagaggtgggcggctagatattccactgctgtactgggtttcctcttatcccatatccgcacatcgccgtcatggctggtggcaaggcagttagcattttttttattccatttgacctgggaggcacccgcaacagcagacagtgcaacagtaggtttccttgtgtctttgatatcccaaatgtagatgtaggtgtccacagagctggtaaccaggaggtcaggctcaaacaccgcccagtccaagtcgctgatgacacgagtgtggccttgtaaggttgtgccaacttccccactgccgtctttccacttgtaaaggtctactcgttggttactcgaagccgcaaaatagtgtgcaaagctgtcatgaggattccactgcacagctccaatgtcccatttgctctggcgagagatctttcggtgaccttcgaaaggggcatctagattgacgatgtataagaatctgcggccagaaagcactgcatgctgcccaagacagtccacagacatcgcagttgcctgggagtcacggaactctacaaccacgttttcgctgctccatcgcgccgccatctcccccgcccggccgccgcggccccaggacggcgccctcccaccccgccgtccccagtatcccgggaccgtgcgccccacacagccagagaatcagccccgacac

SEQ ID NO: 14657 - RNA, 2285 nt, Homo sapiens
  source 1..2285: mol_type = other RNA
gctgggattacaggcatgagccaccgtgcccggcctgagtttctataatttaagcatctttaaggtaaagaaaaattgaaaatgagattacaggcaatttaacgcacaatttaatgaccagttcaatgagctggtttatttgcttgtaaaattattttatctaatgtaaaaatacttggtaaagaaaagttcttaatggggctggaagacaaaaagtctgcatttaaaaaaggttaacaaaatcaataatatatgggtaagcataggcacagaagaataaaaaatttaaaaatgttaaaatcaataataaagccactaataaccacaaaaggaaaactatggttctttttactttgtcaaagttctgcatctgttcccggttggtcagccaggattccatgtcctgggcagtctgaatgacaaatgcttcgtaatctgcaaacatctgtgtaaaacggttagcaaagacctctcggagctgtacattgagctggtagtcccttagttctgcctcttcacaatgcagttttaaatccttgtctttttcacccagagaagcagagaggtccattttttccacagccacaccagtacgcttggccagagcctgcaagcgggctatggtttcattgcccttcagtaactcatacatgctgatgttattagtacagacattgccgttctttttgtcattgaccaagtctttcagaaccatattcttcagtttgctggtactctcactgcaatgtaggctgccctcaggagggatcccaaattgaacaagaacctcagagagttcttggataaaatccactttattggggaactgtggaaattcttcaggcaactcaataaaatggttgtcaatgtccacaaaacacaaattagcctcttgaggaagttctagtttagaacggtcagttccttcttttgactgaaggcccatcagataagggacaggagcatcaagaaaatgtagcagagaagcaggtagaatgggcacataaacatgttgccattgaaatgggaacaaaagtgtggtgatgccttctgccacagtcatcaggcgttgataatcttgtgagtagagaaggatttgcatctctaaaagaacacaggtaaacacctgcaccaggttctctaatcccaggagctcaaatgcctcccgaagggggtaatcagagagggggagttcactgggcccaggcctctggcagatgacaggttcataaacaccataaaatttcagtgacctccctggaggtggaaggggtacttcataaagaatattgtggatatagctttcaagtggcaagggtggtggctgctgtgaggtaacagccttgtaaagctggataaggaatttcttgcaggcctgcatgaatggtaacggtgtgatcaagcatatactttttgaaacatacagggtgtctctgctaatatcataggagttgtatcgctggagtttcaaaagggaagttgtatctccttcatcaagactacttgccaatgagtccatactgcaggaagatgaagcatacacactgctgtaatgctcagcgttgtgcatctggtaaagtgtctgcattgctgtgcagatttgcttacttgtaacttcttcataaaaagtgagaacaaaaccataggtgcgagaaccatcttccctggtaattataaatgagtgaaactgggggtctttattgtccgtttgtgtcctgaaagatagccctttaggcatgcacaacatgttcaccgcatcttgatcaaaagggttccattctatattctgaggatagtgggcgagaactttggatttgaatgttcttctcaaaggactctggtcaaaattttcgcccgccagctcgtcaggctccagcccgctgtccgcgtcgatcccgcacagcacgaagtagtgcgcgaagcggcaggcggccggggaggagcccgagcccgggccgggcgccgcgcagctcccgctcatcccggccgcgctgctccaggggccgccgccgccgccgcccgggaaggctttctgcggaggctgccaccaccgctccggctgtggtctgtgcgcccgccctagggcgacactggcgcgcccatggccgcgcagccgcctctcgccgccgcagcctgcctcctcgctcggcgcgggggaagcggccgcgggctcgcgcgcggcgggtccggagcccggccgggtgggggaggggcgcggggggagtgtcggcctgagaggccctcgcagccgcagctgcgctcgcgagctgagagccgccgcgtct

SEQ ID NO: 14658 - RNA, 2351 nt, Homo sapiens
  source 1..2351: mol_type = other RNA
gctgggattacaggcatgagccaccgtgcccggcctgagtttctataatttaagcatctttaaggtaaagaaaaattgaaaatgagattacaggcaatttaacgcacaatttaatgaccagttcaatgagctggtttatttgcttgtaaaattattttatctaatgtaaaaatacttggtaaagaaaagttcttaatggggctggaagacaaaaagtctgcatttaaaaaaggttaacaaaatcaataatatatgggtaagcataggcacagaagaataaaaaatttaaaaatgttaaaatcaataataaagccactaataaccacaaaaggaaaactatggttctttttactttgtcaaagttctgcatctgttcccggttggtcagccaggattccatgtcctgggcagtctgaatgacaaatgcttcgtaatctgcaaacatctgtgtaaaacggttagcaaagacctctcggagctgtacattgagctggtagtcccttagttctgcctcttcacaatgcagttttaaatccttgtctttttcacccagagaagcagagaggtccattttttccacagccacaccagtacgcttggccagagcctgcaagcgggctatggtttcattgcccttcagtaactcatacatgctgatgttattagtacagacattgccgttctttttgtcattgaccaagtctttcagaaccatattcttcagtttgctggtactctcactgcaatgtaggctgccctcaggagggatcccaaattgaacaagaacctcagagagttcttggataaaatccactttattggggaactgtggaaattcttcaggcaactcaataaaatggttgtcaatgtccacaaaacacaaattagcctcttgaggaagttctagtttagaacggtcagttccttcttttgactgaaggcccatcagataagggacaggagcatcaagaaaatgtagcagagaagcaggtagaatgggcacataaacatgttgccattgaaatgggaacaaaagtgtggtgatgccttctgccacagtcatcaggcgttgataatcttgtgagtagagaaggatttgcatctctaaaagaacacaggtaaacacctgcaccaggttctctaatcccaggagctcaaatgcctcccgaagggggtaatcagagagggggagttcactgggcccaggcctctggcagatgacaggttcataaacaccataaaatttcagtgacctccctggaggtggaaggggtacttcataaagaatattgtggatatagctttcaagtggcaagggtggtggctgctgtgaggtaacagccttgtaaagctggataaggaatttcttgcaggcctgcatgaatggtaacggtgtgatcaagcatatactttttgaaacatacagggtgtctctgctaatatcataggagttgtatcgctggagtttcaaaagggaagttgtatctccttcatcaagactacttgccaatgagtccatactgcaggaagatgaagcatacacactgctgtaatgctcagcgttgtgcatctggtaaagtgtctgcattgctgtgcagatttgcttacttgtaacttcttcataaaaagtgagaacaaaaccataggtgcgagaaccatcttccctggtaattataaatgagtgaaactgggggtctttattgtccgtttgtgtcctgaaagatagccctttaggcatgcacaacatgttcaccgcatcttgatcaaaagggttccattctatattctgaggatagtgggcgagaactttggatttgaatgttcttctcaaaggactctggtcaaaattttcgcctgaagtcgtatttgcagcaccttggctcttgccatgacgatctgcttctagccattggtacaaaaccgccagctcgtcaggctccagcccgctgtccgcgtcgatcccgcacagcacgaagtagtgcgcgaagcggcaggcggccggggaggagcccgagcccgggccgggcgccgcgcagctcccgctcatcccggccgcgctgctccaggggccgccgccgccgccgcccgggaaggctttctgcggaggctgccaccaccgctccggctgtggtctgtgcgcccgccctagggcgacactggcgcgcccatggccgcgcagccgcctctcgccgccgcagcctgcctcctcgctcggcgcgggggaagcggccgcgggctcgcgcgcggcgggtccggagcccggccgggtgggggaggggcgcggggggagtgtcggcctgagaggccctcgcagccgcagctgcgctcgcgagctgagagccgccgcgtct

SEQ ID NO: 14659 - RNA, 1754 nt, Homo sapiens
  source 1..1754: mol_type = other RNA
gctgggattacaggcatgagccaccgtgcccggcctgagtttctataatttaagcatctttaaggtaaagaaaaattgaaaatgagattacaggcaatttaacgcacaatttaatgaccagttcaatgagctggtttatttgcttgtaaaattattttatctaatgtaaaaatacttggtaaagaaaagttcttaatggggctggaagacaaaaagtctgcatttaaaaaaggttaacaaaatcaataatatatgggtaagcataggcacagaagaataaaaaatttaaaaatgttaaaatcaataataaagccactaataaccacaaaaggaaaactatggttctttttactttgtcaaagttctgcatctgttcccggttggtcagccaggattccatgtcctgggcagtctgaatgacaaatgcttcgtaatctgcaaacatctgtgtaaaacggttagcaaagacctctcggagctgtacattgagctggtagtcccttagttctgcctcttcacaatgcagttttaaatccttgtctttttcacccagagaagcagagaggtccattttttccacagccacaccagtacgcttggccagagcctgcaagcgggctatggtttcattgcccttcagtaactcatacatgctgatgttattagtacagacattgccgttctttttgtcattgaccaagtctttcagaaccatattcttcagtttgctggtactctcactgcaatgtaggctgccctcaggagggatcccaaattgaacaagaacctcagagagttcttggataaaatccactttattggggaactgtggaaattcttcaggcaactcaataaaatggttgtcaatgtccacaaaacacaaattagcctcttgaggaagttctagtttagaacggtcagttccttcttttgactgaaggcccatcagataagggacaggagcatcaagaaaatgtagcagagaagcaggtagaatgggcacataaacatgttgccattgaaatgggaacaaaagtgtggtgatgccttctgccacagtcatcaggcgttgataatttgtaacttcttcataaaaagtgagaacaaaaccataggtgcgagaaccatcttccctggtaattataaatgagtgaaactgggggtctttattgtccgtttgtgtcctgaaagatagccctttaggcatgcacaacatgttcaccgcatcttgatcaaaagggttccattctatattctgaggatagtgggcgagaactttggatttgaatgttcttctcaaaggactctggtcaaaattttcgcccgccagctcgtcaggctccagcccgctgtccgcgtcgatcccgcacagcacgaagtagtgcgcgaagcggcaggcggccggggaggagcccgagcccgggccgggcgccgcgcagctcccgctcatcccggccgcgctgctccaggggccgccgccgccgccgcccgggaaggctttctgcggaggctgccaccaccgctccggctgtggtctgtgcgcccgccctagggcgacactggcgcgcccatggccgcgcagccgcctctcgccgccgcagcctgcctcctcgctcggcgcgggggaagcggccgcgggctcgcgcgcggcgggtccggagcccggccgggtgggggaggggcgcggggggagtgtcggcctgagaggccctcgcagccgcagctgcgctcgcgagctgagagccgccgcgtct

SEQ ID NO: 14660 - RNA, 2386 nt, Homo sapiens
  source 1..2386: mol_type = other RNA
gctgggattacaggcatgagccaccgtgcccggcctgatgttcacttattattgatacagttggattgatccctacgttggattttttgagtgttctgtttagtcctataaaagcagtagaaatctctaggccaacataagatgccacatggctcacaagggagttttgaagacatgaacatgcttctgagctcagcagtgtgtgtccctgcgggtcagggaagtcttgtgcacccactcagtgtgtgtccctgcgggtcggggagtcttgtgcacccactcagtgtgtgcagttggaagctggtcccttcagaaacctcagggaagagcccatctcgggcggctggaggcaggtggacaggacaccggggaggagtcttgaggtcgtctcctgttggtgggacgatcggtggcctccatggagagcggtgctggcaccttcactccctgcaccttcagtggtgctcaggcctcccctgaagctcctggcactcacagggttccagttcaatgctgtcgcttttcttgccttcacctgagaagccccttgaggaaagctggaggccccagggcaggccagtgttcagaggaaggagtcccggcctacacggcccgttgtccgcagagccagtgagtcagggtgctcagaagggtcctggtgtagctgctgactccatcgcagctgccctgagcactgctgaattcagaaaacagccttggaggaagcgtctctttatcccccgtacaaatgccgagacaggctccgggtggccagagcttcccgggtcagcccaggagatggcccagacccacagtgctctgggggcagcccaggccccgcccactgacagcactcatggcccctccggcggcagcttcagctcccctggggcagctctgatgcggggcaaaggcaggaagacgcccatgtgccatggcttctgcttcttcccaatgaactgcagttaattaaacaacacagacctgctgccaggagaaagtgtggcccctgggcacagggcccagtggggtggggagcaggggtgcggggagggcatggcccctctgcatgggtgtctgggcctcagctgtttcattatttgtaaatgaaagagcctggacctcaagttgtcttcagttttctgtctttaacactcttaagatttcattgttaatgtgattcaatcaatttggctaagttaggtgctgagctataattaattattttaacaaaagaagtaatacaatggatttttctcctgcttgttaaactaagtcatatgattataaaaatgaaactttatagatgcgactcccgccaaccctctccccagataccaagtgccgccctcggcagggatgcctgcatcaccccagtcatttagggtcatcaggggcccgagtaacgctggggcctgagcacgcggttggggtctccgtgtcccagccccccacccagccccgacctctgcgaacagcgccacacgtcccatggcttgtgtttcatgtgtatacttgaaggagcatgagtttcgtaaacatgctgctggctgttacattaaaaacatgagaaggtaacggcagcctccacacgccgccctctgctgtctgtgcctccgtgcccttggctgttcccaccccggggtctgcgggggtcagggcctgcctcctcttcctcagttggagtgaatttggggtctgactgagggcctcggccatcgtcaaatgtgacaaacacaggccctccccagagaccgcgtctccaggaagcacctgctcctctgggtttcgctgcagtcacctgagcaggtgctgggccaccgagcacttccatcacacagtggctggcggcggagccttgggtcgttttctgaaggtcaccaaccctttggcatcagagcaggcagagccttttgcatccccgccagtccccttgcccaggtggccccgggcaacctccaccctcaggcacccggtcccagttctgtttacagcttctcttttcctggcttctttccccatattgacaagatttcagtcttaggttggtcttgtctgctgtgctgctctgaggaagcctctcggctcctgggtgtgcaagaagccaagggcagccccttccctgtgagcgtgcgtgtccacacgcgtgtgcaggtggcacagagcatccagggctgtcatcagctgcttctggaccgcccaggtggctgcttgggagtttaccgtcacggcagtcctgtgctgccgtggaaacgcggggttgccgtgtggccgccgtggaaacgcggggttgccgtgtggccgccgtggaaacgcggggttgccgtgtggccgccgtggcgcggcagccatcgcctgcccggtgctgattgtgcctcctgtgtgc

SEQ ID NO: 14661 - RNA, 6926 nt, Homo sapiens
  source 1..6926: mol_type = other RNA
gctgggattacaggcatgagccaccgtgcccggcctggatatactttataatggtctcctggtcctaatgatatctttgggcaacttatttcttagtttttccctttcatcttgacaccttatatataaattcactttacaattcacaaagcacagttctacttacttattaattctcctaaccacctcatagatgggtattacaataccattttatgagtttcagaggggtttccttgtcccacacatattaggcttatgtcctggcagccccccattgaactctccaaacctgatcctttccactctgtgattttctctcttcatccctgctcaatctccctgcaccagcacccgattccattttattccagtcaacactaaacgcctgtgttcttaggtgctgattctagacagtgacagaggaaattttttaaggaccaaggacaagatatgtttttccttctggggacagatttgagctagttgctttttaaatattgttcctttgttattctgcctgataagacaaagtagtgggccttataaacaggatctcaccaggattgaatacctactatgctatgatattgtctagacactttattcattttatctcacttaccctgtaaaagcaggctctattatccccacaatacaaatgagttgatagaaatttagtgaagacaagacagttgtttaatgtcatatagctcctatgttcccatgttgaataaggattcaaaccccagtatctggctctacagcctgtggtacattacaccatgttgtccaacaagcatagctctcagggttacatggtttgttaaagtggttaaaaaccccaatcaaaggcccgtggaagttcttaagcaggggtaggttatgccagaaaaaaagtagtggctattcagctaattttctcacatttactcagtctttcccgtctgtaaaataaaaatgaatctaagttccagagaaaacaaatgggggcagtgtgagccaaggaagtgaataataataagcagaagagaaaggcagcctctgctcattggtagtcccaggaggtcggccttctgcagttgccaagcaacgagtgtaaacagcacaagatcatggccactaactacagtgccaaccaggtaagttcccattctccatttctttaacgtttacttttgtttttcagattctatctttggactgtcccctctcataggattctgatctttgaacagatagctgagagtggagtgagataatattttacctcctcagggatagagagagcccaggggcgatccaaaggtatctcttggttaaatttgtagggtgtaaaccagaagttggcaattttttttctgtaaaagggcggagtgtaaaaattttaggctttgcaggccaagtggcaaagtcaaaaatattctgtagctacttgcataattaaagaaaaacatttttccataacatttttgacaaattcaaaatataactgagtacaattttttgtactactaatgaaaataatggaattttgggggttgagaaaacatttcacttaactgggattcaaagttagtgttccatttgactgaatcaattgtaaatgttcatctataaaaatcacccttactctcaggccatccccaaacaggcagcaatatggatatggcccataggccatagtttaccaactcctgatctagaccagtgctgcccaacaaaaagagtgcgacccacaaatgtaattttaaattttctagtagctacatgaaaaaattaaaacataaaatttaaatatattgaatttaacccaataaatccaaatattatttcaacatttaatcagtatttaaaaaattataatcagacattttacgttctttttttgtactaaatctccaaaacctgctgggtgttgtagctcacgtctgtaatcccaacactttgggaggctgaggcacaaggatcgcttgaggccaggggtttgagaccaccctgggcaatatggtgagacctcgtctctacaagtaaatttaaaaattagctggacatggtggcatgcacctgtagtcccagctacctgtgagtctgagggaggaggatcgcttgaacccaggtgtccaaggctgcagtgagctaggatcatgccactgactccaacccaggtggcagaccaagatcctatctcaaaaaaaaaaagaaaagaaaaaaacttaaaaattcagcatatttcatatttacaaagcacctcaatttgaactagtcatatttcaggtgctcaacagctccatgtggctcccggctccatgctggacagcacacatctagaccaaacaaattacacccttgtcatagtgacttaaagcctacatggttggtcaggcctttggtcttcaaatctaaagaattgtgcctagtcttcatttcctgggtttggggccttgaagtctcatagggctacttatctttctctccacagtatgaaaaggctttctcatccaagtatctgcagaactggtctcccactaagccaacaaaagaggtattccatgttcagtgcacctacaagatagcctcatgctctccctgtcaattaactccttttagcattctctaaactcccatatccttctctgaccaagctccccaaatacttccctttttcccctcacaaacctttatctctcccacttgtaccccagagcatctcttctcatgaaggctacactcaaattattgccaacgatcgtggtcatctactgccttctgtgccccgttccaaggtgagatactatcttcactcctatcaagaaagtcaaataattaaggcacagaactgggagatgtgcagtctctcacagccattatcgggaaaattaaagtttaatctaattcatgttgtaatgtgagagcccctgaacttccggccagcttacccagcaggatagagttgtgtttagcacccttcagaagttcttaaattgatcaatgatctgtataaatgaaagccttcaggtgatgacatttgtgcagtgggtactcctttgccacactcggcctaaggatgtggaatttaagttggcagagtaaaggggatgaaaaaattaggcctgcaaagcctaaatgagggagggggataaggaagggtgggaagattatgctttcagtcttgtttcataaccatgcattcctaaaggtaaagaaaggaaataatacagaggtctaagtcagttactgggagtgagaagccctactgaggaatcccttttcatttttaggcaaatccttggggttccttcatgggcacctggcaaatgcctctgaagataccccctgctcgggtgaccctgacctcccgtacaactgctggtgctgcctccctcaccaaatggatacagaaaaatcctgatttactcaaggcctccaatgggctgtgtcctgaaatcttaggcaaggtatctattcttcccatctaacccaaaaccctgtagtctcaatttcttttcaacctcaaaaaatgtctattgttatgccaccactatcccagcatgggggacctctaaccaatttgtcttatcttgactagtccttaatcaccttctgaggcctgaagggatgggctaaggacatcatacccccaacagtagaaaatgatctaatctcaaggtgggggagggtggttagagaaatcaaatttaacttttcttatttgaaacttgatctactgcccatggtatggggagaaagggagttagaatcctgaggtgcattaggaatgatccgggcctgaccagagacatgactatctctcccactcttatcactgacagccccatgatccagacagtcagaagaaactcagaaagaagtctatcacaaagactgtacaacaagcacgaagtccaaccataattccaagctccccagctgccaacctcaattccccagatgaactccaaagctcacacccctctgcaggtcatactccaggtccccaaagaccagccaaatcctaagagcccacctggaagtccacgtatgctagaactctgggcagggcctaatctagctgaggtccagaaatacaaacctggaacttcatatggaccaagtggccacacactgaaaaacccgtatagcgactcagtgaaataaacaagagcccccagtcagaactgtgaaacagggaaattttggggtgggagtaaaagcaaatttggaaaataaacttttttttgttgaatcttttactgatctggattttccattcttgctatggctgcctcttgtaacacaattaggagaaggaaggtaggagaaaataaagtagggaaaagaacatacagtggtttgggtggaacacatttttacaagaattgagtcagttatactccagaaatgaccaagagaaagttggtctgaatcatggaaaaagggcagaacctcaaagaaccagtccctcaaccctacccactcattttttatcctgagcatggacaactaacaactacaaaatcagaaatagaattgagtagagtatgtatatgtgtgtttggagaaggtggggaagaaaaggtagggaaaaccaaagtagaagatactatgcttgtgtaagactttctatctaagcccaagtacaaatatagtttgaaaattgaagatattaaagtgattggaagacagagaagaaaaagacagtaagtagaaatttaaggcagaataacaaacatgatgctctgtcacaccccccacccacccactaccatgcttcaatcacccaaatggtacgaaaccaccaaaaaattcaactgccctacccattttccagcctctaacagctgtttatcattgaccccattttatattttcctggcactggctgttaaatttaatgcccttgccaaacctttcccagtcccaatgacaaagtgttctgtcatgatcacttgtccctcattccaaggacaaagtagagaacagctggtttaaaatggaggaaaggtacaaggacttcccagggcccctctagtaaaaagggaaaaccaatcattacttaaagccaaatactatttgggaccctgaatgaagactgttaaaacagcgggtccccaccttaactaaggtcttcctatccaattgacaccagccagttaacatttcccctcttcgacccacagctttaactggctggccaacaactcgaagtgacagatgagataagtctcttattccagagttcccaaaaactatcaaaacagcatgcctgctaaagcctggcctatatggattttaaaagcagcaagttttctcattaaattatacatttttgccaggttttcaacaatcccttcttttttaaaaaaaaactctatgcttcattcaccccaagcctataacctcaggtcatcatcccctagctgtcaccaacactggtcctctgtgcccctcaatgaatcataatttgctgaactgtaccatgaagcttataatcagtccttaatgggattttggtgcctataacccaaaagcactctacatgcgtcacttcttttctttttctccttccttctctgaggcttttctgtgatatttaaatctctggctaagttctatctgattccctgaaaacttttccaatgatgagatgtaggagaactgtttccctcctggtaaaggtcagattgcggggagagggaggatgtaaatgcctgagacccgagggaagaggaggaaattggttccttcccaacagccattttcttggtttctctagatttcaaggagagtcaaagataaaatgagtatttaattcagtttcagaaaaaaagggtacattacttcgatgagaaagcataaaattaagaggcttttctggaaatccaagaaaaagaaataaccattaatatgttcaatgataattttctagatcttcctcgtgtccaaagctatatattttctcctcaaaagcagctgctccaagaactaactagccctctttatctccctctagctgggacagactaattcccctccacccccacctctcttctttcaataacactgtgtaggtgttaatggcctgggctctcaccaatgaagagaattgtcctttaagccagcaacccacaggcagtggcacccaaagcctcaccaacccaccccccaacccggcccatccccagggcagaagccacagagctggcattgtttccactgtctcaggaagaaggagccaaaagctgaccctcagcacaaatcaaagcccaatatggagagagaataactgcttctaggccgagagtaggcaagctgtgggcaaaaaaggggagtttttgcagccacctcatctttagaaacaaggggaaaactagacccttttccactattatggtctaccaggtactctactgctccaaggagatctgaaaatacaaaaggatctaaacaaataaggagaacttttcccaggctggagataagaatgacaaacagaaagatgggtgaatgtaataatgtgtaggaagatgatgctgggagcctcctttcttcacatggctgccagccccatagaggacaacacagtaagaaccaggacaaccactccagactggtatagctggggaatcttcaggccttttcctaggtcccacatcaagtgtcggatcccattccaggtatgatacatgagagggaagacaagtgcaaacttagctgtgtggatcagtgctggccccagacacagggacttcacaagttccaaataagactcaaagttcccagggagtaacagggccgacatgccaaaaagagagacccctgcactcaaagcaataccagtgccacggtggcagatggacatcgccatgggaagagaccaactcagcaacagcgcagccatcttgggttccggtctggacggaagt

SEQ ID NO: 14662 - RNA, 7112 nt, Homo sapiens
  source 1..7112: mol_type = other RNA
gctgggattacaggcatgagccaccgtgcccggcctggatatactttataatggtctcctggtcctaatgatatctttgggcaacttatttcttagtttttccctttcatcttgacaccttatatataaattcactttacaattcacaaagcacagttctacttacttattaattctcctaaccacctcatagatgggtattacaataccattttatgagtttcagaggggtttccttgtcccacacatattaggcttatgtcctggcagccccccattgaactctccaaacctgatcctttccactctgtgattttctctcttcatccctgctcaatctccctgcaccagcacccgattccattttattccagtcaacactaaacgcctgtgttcttaggtgctgattctagacagtgacagaggaaattttttaaggaccaaggacaagatatgtttttccttctggggacagatttgagctagttgctttttaaatattgttcctttgttattctgcctgataagacaaagtagtgggccttataaacaggatctcaccaggattgaatacctactatgctatgatattgtctagacactttattcattttatctcacttaccctgtaaaagcaggctctattatccccacaatacaaatgagttgatagaaatttagtgaagacaagacagttgtttaatgtcatatagctcctatgttcccatgttgaataaggattcaaaccccagtatctggctctacagcctgtggtacattacaccatgttgtccaacaagcatagctctcagggttacatggtttgttaaagtggttaaaaaccccaatcaaaggcccgtggaagttcttaagcaggggtaggttatgccagaaaaaaagtagtggctattcagctaattttctcacatttactcagtctttcccgtctgtaaaataaaaatgaatctaagttccagagaaaacaaatgggggcagtgtgagccaaggaagtgaataataataagcagaagagaaaggcagcctctgctcattggtagtcccaggaggtcggccttctgcagttgccaagcaacgagtgtaaacagcacaagatcatggccactaactacagtgccaaccaggtaagttcccattctccatttctttaacgtttacttttgtttttcagattctatctttggactgtcccctctcataggattctgatctttgaacagatagctgagagtggagtgagataatattttacctcctcagggatagagagagcccaggggcgatccaaaggtatctcttggttaaatttgtagggtgtaaaccagaagttggcaattttttttctgtaaaagggcggagtgtaaaaattttaggctttgcaggccaagtggcaaagtcaaaaatattctgtagctacttgcataattaaagaaaaacatttttccataacatttttgacaaattcaaaatataactgagtacaattttttgtactactaatgaaaataatggaattttgggggttgagaaaacatttcacttaactgggattcaaagttagtgttccatttgactgaatcaattgtaaatgttcatctataaaaatcacccttactctcaggccatccccaaacaggcagcaatatggatatggcccataggccatagtttaccaactcctgatctagaccagtgctgcccaacaaaaagagtgcgacccacaaatgtaattttaaattttctagtagctacatgaaaaaattaaaacataaaatttaaatatattgaatttaacccaataaatccaaatattatttcaacatttaatcagtatttaaaaaattataatcagacattttacgttctttttttgtactaaatctccaaaacctgctgggtgttgtagctcacgtctgtaatcccaacactttgggaggctgaggcacaaggatcgcttgaggccaggggtttgagaccaccctgggcaatatggtgagacctcgtctctacaagtaaatttaaaaattagctggacatggtggcatgcacctgtagtcccagctacctgtgagtctgagggaggaggatcgcttgaacccaggtgtccaaggctgcagtgagctaggatcatgccactgactccaacccaggtggcagaccaagatcctatctcaaaaaaaaaaagaaaagaaaaaaacttaaaaattcagcatatttcatatttacaaagcacctcaatttgaactagtcatatttcaggtgctcaacagctccatgtggctcccggctccatgctggacagcacacatctagaccaaacaaattacacccttgtcatagtgacttaaagcctacatggttggtcaggcctttggtcttcaaatctaaagaattgtgcctagtcttcatttcctgggtttggggccttgaagtctcatagggctacttatctttctctccacagtatgaaaaggctttctcatccaagtatctgcagaactggtctcccactaagccaacaaaagaggtattccatgttcagtgcacctacaagatagcctcatgctctccctgtcaattaactccttttagcattctctaaactcccatatccttctctgaccaagctccccaaatacttccctttttcccctcacaaacctttatctctcccacttgtaccccagagcatctcttctcatgaaggctacactcaaattattgccaacgatcgtggtcatctactgccttctgtgccccgttccaaggtgagatactatcttcactcctatcaagaaagtcaaataattaaggcacagaactgggagatgtgcagtctctcacagccattatcgggaaaattaaagtttaatctaattcatgttgtaatgtgagagcccctgaacttccggccagcttacccagcaggatagagttgtgtttagcacccttcagaagttcttaaattgatcaatgatctgtataaatgaaagccttcaggtgatgacatttgtgcagtgggtactcctttgccacactcggcctaaggatgtggaatttaagttggcagagtaaaggggatgaaaaaattaggcctgcaaagcctaaatgagggagggggataaggaagggtgggaagattatgctttcagtcttgtttcataaccatgcattcctaaaggtaaagaaaggaaataatacagaggtctaagtcagttactgggagtgagaagccctactgaggaatcccttttcatttttaggcaaatccttggggttccttcatgggcacctggcaaatgcctctgaagataccccctgctcgggtgaccctgacctcccgtacaactgctggtgctgcctccctcaccaaatggatacagaaaaatcctgatttactcaaggcctccaatgggctgtgtcctgaaatcttaggcaaggtatctattcttcccatctaacccaaaaccctgtagtctcaatttcttttcaacctcaaaaaatgtctattgttatgccaccactatcccagcatgggggacctctaaccaatttgtcttatcttgactagtccttaatcaccttctgaggcctgaagggatgggctaaggacatcatacccccaacagtagaaaatgatctaatctcaaggtgggggagggtggttagagaaatcaaatttaacttttcttatttgaaacttgatctactgcccatggtatggggagaaagggagttagaatcctgaggtgcattaggaatgatccgggcctgaccagagacatgactatctctcccactcttatcactgacagccccatgatccagacagtcagaagaaactcagaaagaagtctatcacaaagactgtacaacaagcacgaagtccaaccataattccaagctccccagctgccaacctcaattccccagatgaactccaaagctcacacccctctgcaggtcatactccaggtccccaaagaccagccaaatcctaagagcccacctggaagtccacgtatgctagaactctgggcagggcctaatctagctgaggtccagaaatacaaacctggaacttcatatggaccaagtggccacacactgaaaaacccgtatagcgactcagtgaaataaacaagagcccccagtcagaactgtgaaacagggaaattttggggtgggagtaaaagcaaatttggaaaataaacttttttttgttgaatcttttactgatctggattttccattcttgctatggctgcctcttgtaacacaattaggagaaggaaggtaggagaaaataaagtagggaaaagaacatacagtggtttgggtggaacacatttttacaagaattgagtcagttatactccagaaatgaccaagagaaagttggtctgaatcatggaaaaagggcagaacctcaaagaaccagtccctcaaccctacccactcattttttatcctgagcatggacaactaacaactacaaaatcagaaatagaattgagtagagtatgtatatgtgtgtttggagaaggtggggaagaaaaggtagggaaaaccaaagtagaagatactatgcttgtgtaagactttctatctaagcccaagtacaaatatagtttgaaaattgaagatattaaagtgattggaagacagagaagaaaaagacagtaagtagaaatttaaggcagaataacaaacatgatgctctgtcacaccccccacccacccactaccatgcttcaatcacccaaatggtacgaaaccaccaaaaaattcaactgccctacccattttccagcctctaacagctgtttatcattgaccccattttatattttcctggcactggctgttaaatttaatgcccttgccaaacctttcccagtcccaatgacaaagtgttctgtcatgatcacttgtccctcattccaaggacaaagtagagaacagctggtttaaaatggaggaaaggtacaaggacttcccagggcccctctagtaaaaagggaaaaccaatcattacttaaagccaaatactatttgggaccctgaatgaagactgttaaaacagcgggtccccaccttaactaaggtcttcctatccaattgacaccagccagttaacatttcccctcttcgacccacagctttaactggctggccaacaactcgaagtgacagatgagataagtctcttattccagagttcccaaaaactatcaaaacagcatgcctgctaaagcctggcctatatggattttaaaagcagcaagttttctcattaaattatacatttttgccaggttttcaacaatcccttcttttttaaaaaaaaactctatgcttcattcaccccaagcctataacctcaggtcatcatcccctagctgtcaccaacactggtcctctgtgcccctcaatgaatcataatttgctgaactgtaccatgaagcttataatcagtccttaatgggattttggtgcctataacccaaaagcactctacatgcgtcacttcttttctttttctccttccttctctgaggcttttctgtgatatttaaatctctggctaagttctatctgattccctgaaaacttttccaatgatgagatgtaggagaactgtttccctcctggtaaaggtcagattgcggggagagggaggatgtaaatgcctgagacccgagggaagaggaggaaattggttccttcccaacagccattttcttggtttctctagatttcaaggagagtcaaagataaaatgagtatttaattcagtttcagaaaaaaagggtacattacttcgatgagaaagcataaaattaagaggcttttctggaaatccaagaaaaagaaataaccattaatatgttcaatgataattttctagatcttcctcgtgtccaaagctatatattttctcctcaaaagcagctgctccaagaactaactagccctctttatctccctctagctgggacagactaattcccctccacccccacctctcttctttcaataacactgtgtaggtgttaatggcctgggctctcaccaatgaagagaattgtcctttaagccagcaacccacaggcagtggcacccaaagcctcaccaacccaccccccaacccggcccatccccagggcagaagccacagagctggcattgtttccactgtctcaggaagaaggagccaaaagctgaccctcagcacaaatcaaagcccaatatggagagagaataactgcttctaggccgagagtaggcaagctgtgggcaaaaaaggggagtttttgcagccacctcatctttagaaacaaggggaaaactagacccttttccactattatggtctaccaggtactctactgctccaaggagatctgaaaatacaaaaggatctaaacaaataaggagaacttttcccaggctggagataagaatgacaaacagaaagatgggtgaatgtaataatgtgtaggaagatgatgctgggagcctcctttcttcacatggctgccagccccatagaggacaacacagtaagaaccaggacaaccactccagactggtatagctggggaatcttcaggccttttcctaggtcccacatcaagtgtcggatcccattccaggtatgatacatgagagggaagacaagtgcaaacttagctgtgtggatcagtgctggccccagacacagggacttcacaagttccaaataagactcaaagttcccagggagtaacagggccgacatgccaaaaagagagacccctgcactcaaagcaataccagtgccacggtggcagatggacatcgccatgggaagagaccaactttaccagactgcatcactgatagggctgtagatagtaatgtggggagacagaggacggtttgaacctatattcttattccagaaccgctccatctcttctttggccgtggttcccaaaggaacagcatttctgatacagagctgagggctaaagtgggctcggaggcaatgacgaccaacgtgtctcagcaacagcgcagccatcttgggttccggtctggacggaagt

SEQ ID NO: 14663 - RNA, 6983 nt, Homo sapiens
  source 1..6983: mol_type = other RNA
gctgggattacaggcatgagccaccgtgcccggcctggatatactttataatggtctcctggtcctaatgatatctttgggcaacttatttcttagtttttccctttcatcttgacaccttatatataaattcactttacaattcacaaagcacagttctacttacttattaattctcctaaccacctcatagatgggtattacaataccattttatgagtttcagaggggtttccttgtcccacacatattaggcttatgtcctggcagccccccattgaactctccaaacctgatcctttccactctgtgattttctctcttcatccctgctcaatctccctgcaccagcacccgattccattttattccagtcaacactaaacgcctgtgttcttaggtgctgattctagacagtgacagaggaaattttttaaggaccaaggacaagatatgtttttccttctggggacagatttgagctagttgctttttaaatattgttcctttgttattctgcctgataagacaaagtagtgggccttataaacaggatctcaccaggattgaatacctactatgctatgatattgtctagacactttattcattttatctcacttaccctgtaaaagcaggctctattatccccacaatacaaatgagttgatagaaatttagtgaagacaagacagttgtttaatgtcatatagctcctatgttcccatgttgaataaggattcaaaccccagtatctggctctacagcctgtggtacattacaccatgttgtccaacaagcatagctctcagggttacatggtttgttaaagtggttaaaaaccccaatcaaaggcccgtggaagttcttaagcaggggtaggttatgccagaaaaaaagtagtggctattcagctaattttctcacatttactcagtctttcccgtctgtaaaataaaaatgaatctaagttccagagaaaacaaatgggggcagtgtgagccaaggaagtgaataataataagcagaagagaaaggcagcctctgctcattggtagtcccaggaggtcggccttctgcagttgccaagcaacgagtgtaaacagcacaagatcatggccactaactacagtgccaaccaggtaagttcccattctccatttctttaacgtttacttttgtttttcagattctatctttggactgtcccctctcataggattctgatctttgaacagatagctgagagtggagtgagataatattttacctcctcagggatagagagagcccaggggcgatccaaaggtatctcttggttaaatttgtagggtgtaaaccagaagttggcaattttttttctgtaaaagggcggagtgtaaaaattttaggctttgcaggccaagtggcaaagtcaaaaatattctgtagctacttgcataattaaagaaaaacatttttccataacatttttgacaaattcaaaatataactgagtacaattttttgtactactaatgaaaataatggaattttgggggttgagaaaacatttcacttaactgggattcaaagttagtgttccatttgactgaatcaattgtaaatgttcatctataaaaatcacccttactctcaggccatccccaaacaggcagcaatatggatatggcccataggccatagtttaccaactcctgatctagaccagtgctgcccaacaaaaagagtgcgacccacaaatgtaattttaaattttctagtagctacatgaaaaaattaaaacataaaatttaaatatattgaatttaacccaataaatccaaatattatttcaacatttaatcagtatttaaaaaattataatcagacattttacgttctttttttgtactaaatctccaaaacctgctgggtgttgtagctcacgtctgtaatcccaacactttgggaggctgaggcacaaggatcgcttgaggccaggggtttgagaccaccctgggcaatatggtgagacctcgtctctacaagtaaatttaaaaattagctggacatggtggcatgcacctgtagtcccagctacctgtgagtctgagggaggaggatcgcttgaacccaggtgtccaaggctgcagtgagctaggatcatgccactgactccaacccaggtggcagaccaagatcctatctcaaaaaaaaaaagaaaagaaaaaaacttaaaaattcagcatatttcatatttacaaagcacctcaatttgaactagtcatatttcaggtgctcaacagctccatgtggctcccggctccatgctggacagcacacatctagaccaaacaaattacacccttgtcatagtgacttaaagcctacatggttggtcaggcctttggtcttcaaatctaaagaattgtgcctagtcttcatttcctgggtttggggccttgaagtctcatagggctacttatctttctctccacagtatgaaaaggctttctcatccaagtatctgcagaactggtctcccactaagccaacaaaagaggtattccatgttcagtgcacctacaagatagcctcatgctctccctgtcaattaactccttttagcattctctaaactcccatatccttctctgaccaagctccccaaatacttccctttttcccctcacaaacctttatctctcccacttgtaccccagagcatctcttctcatgaaggctacactcaaattattgccaacgatcgtggtcatctactgccttctgtgccccgttccaaggtgagatactatcttcactcctatcaagaaagtcaaataattaaggcacagaactgggagatgtgcagtctctcacagccattatcgggaaaattaaagtttaatctaattcatgttgtaatgtgagagcccctgaacttccggccagcttacccagcaggatagagttgtgtttagcacccttcagaagttcttaaattgatcaatgatctgtataaatgaaagccttcaggtgatgacatttgtgcagtgggtactcctttgccacactcggcctaaggatgtggaatttaagttggcagagtaaaggggatgaaaaaattaggcctgcaaagcctaaatgagggagggggataaggaagggtgggaagattatgctttcagtcttgtttcataaccatgcattcctaaaggtaaagaaaggaaataatacagaggtctaagtcagttactgggagtgagaagccctactgaggaatcccttttcatttttaggcaaatccttggggttccttcatgggcacctggcaaatgcctctgaagataccccctgctcgggtgaccctgacctcccgtacaactgctggtgctgcctccctcaccaaatggatacagaaaaatcctgatttactcaaggcctccaatgggctgtgtcctgaaatcttaggcaaggtatctattcttcccatctaacccaaaaccctgtagtctcaatttcttttcaacctcaaaaaatgtctattgttatgccaccactatcccagcatgggggacctctaaccaatttgtcttatcttgactagtccttaatcaccttctgaggcctgaagggatgggctaaggacatcatacccccaacagtagaaaatgatctaatctcaaggtgggggagggtggttagagaaatcaaatttaacttttcttatttgaaacttgatctactgcccatggtatggggagaaagggagttagaatcctgaggtgcattaggaatgatccgggcctgaccagagacatgactatctctcccactcttatcactgacagccccatgatccagacagtcagaagaaactcagaaagaagtctatcacaaagactgtacaacaagcacgaagtccaaccataattccaagctccccagctgccaacctcaattccccagatgaactccaaagctcacacccctctgcaggtcatactccaggtccccaaagaccagccaaatcctaagagcccacctggaagtccacgtatgctagaactctgggcagggcctaatctagctgaggtccagaaatacaaacctggaacttcatatggaccaagtggccacacactgaaaaacccgtatagcgactcagtgaaataaacaagagcccccagtcagaactgtgaaacagggaaattttggggtgggagtaaaagcaaatttggaaaataaacttttttttgttgaatcttttactgatctggattttccattcttgctatggctgcctcttgtaacacaattaggagaaggaaggtaggagaaaataaagtagggaaaagaacatacagtggtttgggtggaacacatttttacaagaattgagtcagttatactccagaaatgaccaagagaaagttggtctgaatcatggaaaaagggcagaacctcaaagaaccagtccctcaaccctacccactcattttttatcctgagcatggacaactaacaactacaaaatcagaaatagaattgagtagagtatgtatatgtgtgtttggagaaggtggggaagaaaaggtagggaaaaccaaagtagaagatactatgcttgtgtaagactttctatctaagcccaagtacaaatatagtttgaaaattgaagatattaaagtgattggaagacagagaagaaaaagacagtaagtagaaatttaaggcagaataacaaacatgatgctctgtcacaccccccacccacccactaccatgcttcaatcacccaaatggtacgaaaccaccaaaaaattcaactgccctacccattttccagcctctaacagctgtttatcattgaccccattttatattttcctggcactggctgttaaatttaatgcccttgccaaacctttcccagtcccaatgacaaagtgttctgtcatgatcacttgtccctcattccaaggacaaagtagagaacagctggtttaaaatggaggaaaggtacaaggacttcccagggcccctctagtaaaaagggaaaaccaatcattacttaaagccaaatactatttgggaccctgaatgaagactgttaaaacagcgggtccccaccttaactaaggtcttcctatccaattgacaccagccagttaacatttcccctcttcgacccacagctttaactggctggccaacaactcgaagtgacagatgagataagtctcttattccagagttcccaaaaactatcaaaacagcatgcctgctaaagcctggcctatatggattttaaaagcagcaagttttctcattaaattatacatttttgccaggttttcaacaatcccttcttttttaaaaaaaaactctatgcttcattcaccccaagcctataacctcaggtcatcatcccctagctgtcaccaacactggtcctctgtgcccctcaatgaatcataatttgctgaactgtaccatgaagcttataatcagtccttaatgggattttggtgcctataacccaaaagcactctacatgcgtcacttcttttctttttctccttccttctctgaggcttttctgtgatatttaaatctctggctaagttctatctgattccctgaaaacttttccaatgatgagatgtaggagaactgtttccctcctggtaaaggtcagattgcggggagagggaggatgtaaatgcctgagacccgagggaagaggaggaaattggttccttcccaacagccattttcttggtttctctagatttcaaggagagtcaaagataaaatgagtatttaattcagtttcagaaaaaaagggtacattacttcgatgagaaagcataaaattaagaggcttttctggaaatccaagaaaaagaaataaccattaatatgttcaatgataattttctagatcttcctcgtgtccaaagctatatattttctcctcaaaagcagctgctccaagaactaactagccctctttatctccctctagctgggacagactaattcccctccacccccacctctcttctttcaataacactgtgtaggtgttaatggcctgggctctcaccaatgaagagaattgtcctttaagccagcaacccacaggcagtggcacccaaagcctcaccaacccaccccccaacccggcccatccccagggcagaagccacagagctggcattgtttccactgtctcaggaagaaggagccaaaagctgaccctcagcacaaatcaaagcccaatatggagagagaataactgcttctaggccgagagtaggcaagctgtgggcaaaaaaggggagtttttgcagccacctcatctttagaaacaaggggaaaactagacccttttccactattatggtctaccaggtactctactgctccaaggagatctgaaaatacaaaaggatctaaacaaataaggagaacttttcccaggctggagataagaatgacaaacagaaagatgggtgaatgtaataatgtgtaggaagatgatgctgggagcctcctttcttcacatggctgccagccccatagaggacaacacagtaagaaccaggacaaccactccagactggtatagctggggaatcttcaggccttttcctaggtcccacatcaagtgtcggatcccattccaggtatgatacatgagagggaagacaagtgcaaacttagctgtgtggatcagtgctggccccagacacagggacttcacaagttccaaataagactcaaagttcccagggagtaacagggccgacatgccaaaaagagagacccctgcactcaaagcaataccagtgccacggtggcagatggacatcgccatgggaagagaccaatttctgatacagagctgagggctaaagtgggctcggaggcaatgacgaccaacgtgtctcagcaacagcgcagccatcttgggttccggtctggacggaagt

SEQ ID NO: 14664 - RNA, 6921 nt, Homo sapiens
  source 1..6921: mol_type = other RNA
gctgggattacaggcatgagccaccgtgcccggcctggatatactttataatggtctcctggtcctaatgatatctttgggcaacttatttcttagtttttccctttcatcttgacaccttatatataaattcactttacaattcacaaagcacagttctacttacttattaattctcctaaccacctcatagatgggtattacaataccattttatgagtttcagaggggtttccttgtcccacacatattaggcttatgtcctggcagccccccattgaactctccaaacctgatcctttccactctgtgattttctctcttcatccctgctcaatctccctgcaccagcacccgattccattttattccagtcaacactaaacgcctgtgttcttaggtgctgattctagacagtgacagaggaaattttttaaggaccaaggacaagatatgtttttccttctggggacagatttgagctagttgctttttaaatattgttcctttgttattctgcctgataagacaaagtagtgggccttataaacaggatctcaccaggattgaatacctactatgctatgatattgtctagacactttattcattttatctcacttaccctgtaaaagcaggctctattatccccacaatacaaatgagttgatagaaatttagtgaagacaagacagttgtttaatgtcatatagctcctatgttcccatgttgaataaggattcaaaccccagtatctggctctacagcctgtggtacattacaccatgttgtccaacaagcatagctctcagggttacatggtttgttaaagtggttaaaaaccccaatcaaaggcccgtggaagttcttaagcaggggtaggttatgccagaaaaaaagtagtggctattcagctaattttctcacatttactcagtctttcccgtctgtaaaataaaaatgaatctaagttccagagaaaacaaatgggggcagtgtgagccaaggaagtgaataataataagcagaagagaaaggcagcctctgctcattggtagtcccaggaggtcggccttctgcagttgccaagcaacgagtgtaaacagcacaagatcatggccactaactacagtgccaaccaggtaagttcccattctccatttctttaacgtttacttttgtttttcagattctatctttggactgtcccctctcataggattctgatctttgaacagatagctgagagtggagtgagataatattttacctcctcagggatagagagagcccaggggcgatccaaaggtatctcttggttaaatttgtagggtgtaaaccagaagttggcaattttttttctgtaaaagggcggagtgtaaaaattttaggctttgcaggccaagtggcaaagtcaaaaatattctgtagctacttgcataattaaagaaaaacatttttccataacatttttgacaaattcaaaatataactgagtacaattttttgtactactaatgaaaataatggaattttgggggttgagaaaacatttcacttaactgggattcaaagttagtgttccatttgactgaatcaattgtaaatgttcatctataaaaatcacccttactctcaggccatccccaaacaggcagcaatatggatatggcccataggccatagtttaccaactcctgatctagaccagtgctgcccaacaaaaagagtgcgacccacaaatgtaattttaaattttctagtagctacatgaaaaaattaaaacataaaatttaaatatattgaatttaacccaataaatccaaatattatttcaacatttaatcagtatttaaaaaattataatcagacattttacgttctttttttgtactaaatctccaaaacctgctgggtgttgtagctcacgtctgtaatcccaacactttgggaggctgaggcacaaggatcgcttgaggccaggggtttgagaccaccctgggcaatatggtgagacctcgtctctacaagtaaatttaaaaattagctggacatggtggcatgcacctgtagtcccagctacctgtgagtctgagggaggaggatcgcttgaacccaggtgtccaaggctgcagtgagctaggatcatgccactgactccaacccaggtggcagaccaagatcctatctcaaaaaaaaaaagaaaagaaaaaaacttaaaaattcagcatatttcatatttacaaagcacctcaatttgaactagtcatatttcaggtgctcaacagctccatgtggctcccggctccatgctggacagcacacatctagaccaaacaaattacacccttgtcatagtgacttaaagcctacatggttggtcaggcctttggtcttcaaatctaaagaattgtgcctagtcttcatttcctgggtttggggccttgaagtctcatagggctacttatctttctctccacagtatgaaaaggctttctcatccaagtatctgcagaactggtctcccactaagccaacaaaagaggtattccatgttcagtgcacctacaagatagcctcatgctctccctgtcaattaactccttttagcattctctaaactcccatatccttctctgaccaagctccccaaatacttccctttttcccctcacaaacctttatctctcccacttgtaccccagagcatctcttctcatgaaggctacactcaaattattgccaacgatcgtggtcatctactgccttctgtgccccgttccaaggtgagatactatcttcactcctatcaagaaagtcaaataattaaggcacagaactgggagatgtgcagtctctcacagccattatcgggaaaattaaagtttaatctaattcatgttgtaatgtgagagcccctgaacttccggccagcttacccagcaggatagagttgtgtttagcacccttcagaagttcttaaattgatcaatgatctgtataaatgaaagccttcaggtgatgacatttgtgcagtgggtactcctttgccacactcggcctaaggatgtggaatttaagttggcagagtaaaggggatgaaaaaattaggcctgcaaagcctaaatgagggagggggataaggaagggtgggaagattatgctttcagtcttgtttcataaccatgcattcctaaaggtaaagaaaggaaataatacagaggtctaagtcagttactgggagtgagaagccctactgaggaatcccttttcatttttaggcaaatccttggggttccttcatgggcacctggcaaatgcctctgaagataccccctgctcgggtgaccctgacctcccgtacaactgctggtgctgcctccctcaccaaatggatacagaaaaatcctgatttactcaaggcctccaatgggctgtgtcctgaaatcttaggcaaggtatctattcttcccatctaacccaaaaccctgtagtctcaatttcttttcaacctcaaaaaatgtctattgttatgccaccactatcccagcatgggggacctctaaccaatttgtcttatcttgactagtccttaatcaccttctgaggcctgaagggatgggctaaggacatcatacccccaacagtagaaaatgatctaatctcaaggtgggggagggtggttagagaaatcaaatttaacttttcttatttgaaacttgatctactgcccatggtatggggagaaagggagttagaatcctgaggtgcattaggaatgatccgggcctgaccagagacatgactatctctcccactcttatcactgacagccccatgatccagacagtcagaagaaactcagaaagaagtctatcacaaagactgtacaacaagcacgaagtccaaccataattccaagctccccagctgccaacctcaattccccagatgaactccaaagctcacacccctctgcaggtcatactccaggtccccaaagaccagccaaatcctaagagcccacctggaagtccacgtatgctagaactctgggcagggcctaatctagctgaggtccagaaatacaaacctggaacttcatatggaccaagtggccacacactgaaaaacccgtatagcgactcagtgaaataaacaagagcccccagtcagaactgtgaaacagggaaattttggggtgggagtaaaagcaaatttggaaaataaacttttttttgttgaatcttttactgatctggattttccattcttgctatggctgcctcttgtaacacaattaggagaaggaaggtaggagaaaataaagtagggaaaagaacatacagtggtttgggtggaacacatttttacaagaattgagtcagttatactccagaaatgaccaagagaaagttggtctgaatcatggaaaaagggcagaacctcaaagaaccagtccctcaaccctacccactcattttttatcctgagcatggacaactaacaactacaaaatcagaaatagaattgagtagagtatgtatatgtgtgtttggagaaggtggggaagaaaaggtagggaaaaccaaagtagaagatactatgcttgtgtaagactttctatctaagcccaagtacaaatatagtttgaaaattgaagatattaaagtgattggaagacagagaagaaaaagacagtaagtagaaatttaaggcagaataacaaacatgatgctctgtcacaccccccacccacccactaccatgcttcaatcacccaaatggtacgaaaccaccaaaaaattcaactgccctacccattttccagcctctaacagctgtttatcattgaccccattttatattttcctggcactggctgttaaatttaatgcccttgccaaacctttcccagtcccaatgacaaagtgttctgtcatgatcacttgtccctcattccaaggacaaagtagagaacagctggtttaaaatggaggaaaggtacaaggacttcccagggcccctctagtaaaaagggaaaaccaatcattacttaaagccaaatactatttgggaccctgaatgaagactgttaaaacagcgggtccccaccttaactaaggtcttcctatccaattgacaccagccagttaacatttcccctcttcgacccacagctttaactggctggccaacaactcgaagtgacagatgagataagtctcttattccagagttcccaaaaactatcaaaacagcatgcctgctaaagcctggcctatatggattttaaaagcagcaagttttctcattaaattatacatttttgccaggttttcaacaatcccttcttttttaaaaaaaaactctatgcttcattcaccccaagcctataacctcaggtcatcatcccctagctgtcaccaacactggtcctctgtgcccctcaatgaatcataatttgctgaactgtaccatgaagcttataatcagtccttaatgggattttggtgcctataacccaaaagcactctacatgcgtcacttcttttctttttctccttccttctctgaggcttttctgtgatatttaaatctctggctaagttctatctgattccctgaaaacttttccaatgatgagatgtaggagaactgtttccctcctggtaaaggtcagattgcggggagagggaggatgtaaatgcctgagacccgagggaagaggaggaaattggttccttcccaacagccattttcttggtttctctagatttcaaggagagtcaaagataaaatgagtatttaattcagtttcagaaaaaaagggtacattacttcgatgagaaagcataaaattaagaggcttttctggaaatccaagaaaaagaaataaccattaatatgttcaatgataattttctagatcttcctcgtgtccaaagctatatattttctcctcaaaagcagctgctccaagaactaactagccctctttatctccctctagctgggacagactaattcccctccacccccacctctcttctttcaataacactgtgtaggtgttaatggcctgggctctcaccaatgaagagaattgtcctttaagccagcaacccacaggcagtggcacccaaagcctcaccaacccaccccccaacccggcccatccccagggcagaagccacagagctggcattgtttccactgtctcaggaagaaggagccaaaagctgaccctcagcacaaatcaaagcccaatatggagagagaataactgcttctaggccgagagtaggcaagctgtgggcaaaaaaggggagtttttgcagccacctcatctttagaaacaaggggaaaactagacccttttccactattatggtctaccaggtactctactgctccaaggagatctgaaaatacaaaaggatctaaacaaataaggagaacttttcccaggctggagataagaatgacaaacagaaagatgggtgaatgtaataatgtgtaggaagatgatgctgggagcctcctttcttcacatggctgccagccccatagaggacaacacagtaagaaccaggacaaccactccagactggtatagctggggaatcttcaggccttttcctaggtcccacatctgcactcaaagcaataccagtgccacggtggcagatggacatcgccatgggaagagaccaactgtagatagtaatgtggggagacagaggacggtttgaacctatattcttattccagaaccgctccatctcttctttggccgtggttcccaaaggaacagcatttctgatacagagctgagggctaaagtgggctcggaggcaatgacgaccaacgtgtctcagcaacagcgcagccatcttgggttccggtctggacggaagt

SEQ ID NO: 14665 - RNA, 6819 nt, Homo sapiens
  source 1..6819: mol_type = other RNA
gctgggattacaggcatgagccaccgtgcccggcctggatatactttataatggtctcctggtcctaatgatatctttgggcaacttatttcttagtttttccctttcatcttgacaccttatatataaattcactttacaattcacaaagcacagttctacttacttattaattctcctaaccacctcatagatgggtattacaataccattttatgagtttcagaggggtttccttgtcccacacatattaggcttatgtcctggcagccccccattgaactctccaaacctgatcctttccactctgtgattttctctcttcatccctgctcaatctccctgcaccagcacccgattccattttattccagtcaacactaaacgcctgtgttcttaggtgctgattctagacagtgacagaggaaattttttaaggaccaaggacaagatatgtttttccttctggggacagatttgagctagttgctttttaaatattgttcctttgttattctgcctgataagacaaagtagtgggccttataaacaggatctcaccaggattgaatacctactatgctatgatattgtctagacactttattcattttatctcacttaccctgtaaaagcaggctctattatccccacaatacaaatgagttgatagaaatttagtgaagacaagacagttgtttaatgtcatatagctcctatgttcccatgttgaataaggattcaaaccccagtatctggctctacagcctgtggtacattacaccatgttgtccaacaagcatagctctcagggttacatggtttgttaaagtggttaaaaaccccaatcaaaggcccgtggaagttcttaagcaggggtaggttatgccagaaaaaaagtagtggctattcagctaattttctcacatttactcagtctttcccgtctgtaaaataaaaatgaatctaagttccagagaaaacaaatgggggcagtgtgagccaaggaagtgaataataataagcagaagagaaaggcagcctctgctcattggtagtcccaggaggtcggccttctgcagttgccaagcaacgagtgtaaacagcacaagatcatggccactaactacagtgccaaccaggtaagttcccattctccatttctttaacgtttacttttgtttttcagattctatctttggactgtcccctctcataggattctgatctttgaacagatagctgagagtggagtgagataatattttacctcctcagggatagagagagcccaggggcgatccaaaggtatctcttggttaaatttgtagggtgtaaaccagaagttggcaattttttttctgtaaaagggcggagtgtaaaaattttaggctttgcaggccaagtggcaaagtcaaaaatattctgtagctacttgcataattaaagaaaaacatttttccataacatttttgacaaattcaaaatataactgagtacaattttttgtactactaatgaaaataatggaattttgggggttgagaaaacatttcacttaactgggattcaaagttagtgttccatttgactgaatcaattgtaaatgttcatctataaaaatcacccttactctcaggccatccccaaacaggcagcaatatggatatggcccataggccatagtttaccaactcctgatctagaccagtgctgcccaacaaaaagagtgcgacccacaaatgtaattttaaattttctagtagctacatgaaaaaattaaaacataaaatttaaatatattgaatttaacccaataaatccaaatattatttcaacatttaatcagtatttaaaaaattataatcagacattttacgttctttttttgtactaaatctccaaaacctgctgggtgttgtagctcacgtctgtaatcccaacactttgggaggctgaggcacaaggatcgcttgaggccaggggtttgagaccaccctgggcaatatggtgagacctcgtctctacaagtaaatttaaaaattagctggacatggtggcatgcacctgtagtcccagctacctgtgagtctgagggaggaggatcgcttgaacccaggtgtccaaggctgcagtgagctaggatcatgccactgactccaacccaggtggcagaccaagatcctatctcaaaaaaaaaaagaaaagaaaaaaacttaaaaattcagcatatttcatatttacaaagcacctcaatttgaactagtcatatttcaggtgctcaacagctccatgtggctcccggctccatgctggacagcacacatctagaccaaacaaattacacccttgtcatagtgacttaaagcctacatggttggtcaggcctttggtcttcaaatctaaagaattgtgcctagtcttcatttcctgggtttggggccttgaagtctcatagggctacttatctttctctccacagtatgaaaaggctttctcatccaagtatctgcagaactggtctcccactaagccaacaaaagaggtattccatgttcagtgcacctacaagatagcctcatgctctccctgtcaattaactccttttagcattctctaaactcccatatccttctctgaccaagctccccaaatacttccctttttcccctcacaaacctttatctctcccacttgtaccccagagcatctcttctcatgaaggctacactcaaattattgccaacgatcgtggtcatctactgccttctgtgccccgttccaaggtgagatactatcttcactcctatcaagaaagtcaaataattaaggcacagaactgggagatgtgcagtctctcacagccattatcgggaaaattaaagtttaatctaattcatgttgtaatgtgagagcccctgaacttccggccagcttacccagcaggatagagttgtgtttagcacccttcagaagttcttaaattgatcaatgatctgtataaatgaaagccttcaggtgatgacatttgtgcagtgggtactcctttgccacactcggcctaaggatgtggaatttaagttggcagagtaaaggggatgaaaaaattaggcctgcaaagcctaaatgagggagggggataaggaagggtgggaagattatgctttcagtcttgtttcataaccatgcattcctaaaggtaaagaaaggaaataatacagaggtctaagtcagttactgggagtgagaagccctactgaggaatcccttttcatttttaggcaaatccttggggttccttcatgggcacctggcaaatgcctctgaagataccccctgctcgggtgaccctgacctcccgtacaactgctggtgctgcctccctcaccaaatggatacagaaaaatcctgatttactcaaggcctccaatgggctgtgtcctgaaatcttaggcaaggtatctattcttcccatctaacccaaaaccctgtagtctcaatttcttttcaacctcaaaaaatgtctattgttatgccaccactatcccagcatgggggacctctaaccaatttgtcttatcttgactagtccttaatcaccttctgaggcctgaagggatgggctaaggacatcatacccccaacagtagaaaatgatctaatctcaaggtgggggagggtggttagagaaatcaaatttaacttttcttatttgaaacttgatctactgcccatggtatggggagaaagggagttagaatcctgaggtgcattaggaatgatccgggcctgaccagagacatgactatctctcccactcttatcactgacagccccatgatccagacagtcagaagaaactcagaaagaagtctatcacaaagactgtacaacaagcacgaagtccaaccataattccaagctccccagctgccaacctcaattccccagatgaactccaaagctcacacccctctgcaggtcatactccaggtccccaaagaccagccaaatcctaagagcccacctggaagtccacgtatgctagaactctgggcagggcctaatctagctgaggtccagaaatacaaacctggaacttcatatggaccaagtggccacacactgaaaaacccgtatagcgactcagtgaaataaacaagagcccccagtcagaactgtgaaacagggaaattttggggtgggagtaaaagcaaatttggaaaataaacttttttttgttgaatcttttactgatctggattttccattcttgctatggctgcctcttgtaacacaattaggagaaggaaggtaggagaaaataaagtagggaaaagaacatacagtggtttgggtggaacacatttttacaagaattgagtcagttatactccagaaatgaccaagagaaagttggtctgaatcatggaaaaagggcagaacctcaaagaaccagtccctcaaccctacccactcattttttatcctgagcatggacaactaacaactacaaaatcagaaatagaattgagtagagtatgtatatgtgtgtttggagaaggtggggaagaaaaggtagggaaaaccaaagtagaagatactatgcttgtgtaagactttctatctaagcccaagtacaaatatagtttgaaaattgaagatattaaagtgattggaagacagagaagaaaaagacagtaagtagaaatttaaggcagaataacaaacatgatgctctgtcacaccccccacccacccactaccatgcttcaatcacccaaatggtacgaaaccaccaaaaaattcaactgccctacccattttccagcctctaacagctgtttatcattgaccccattttatattttcctggcactggctgttaaatttaatgcccttgccaaacctttcccagtcccaatgacaaagtgttctgtcatgatcacttgtccctcattccaaggacaaagtagagaacagctggtttaaaatggaggaaaggtacaaggacttcccagggcccctctagtaaaaagggaaaaccaatcattacttaaagccaaatactatttgggaccctgaatgaagactgttaaaacagcgggtccccaccttaactaaggtcttcctatccaattgacaccagccagttaacatttcccctcttcgacccacagctttaactggctggccaacaactcgaagtgacagatgagataagtctcttattccagagttcccaaaaactatcaaaacagcatgcctgctaaagcctggcctatatggattttaaaagcagcaagttttctcattaaattatacatttttgccaggttttcaacaatcccttcttttttaaaaaaaaactctatgcttcattcaccccaagcctataacctcaggtcatcatcccctagctgtcaccaacactggtcctctgtgcccctcaatgaatcataatttgctgaactgtaccatgaagcttataatcagtccttaatgggattttggtgcctataacccaaaagcactctacatgcgtcacttcttttctttttctccttccttctctgaggcttttctgtgatatttaaatctctggctaagttctatctgattccctgaaaacttttccaatgatgagatgtaggagaactgtttccctcctggtaaaggtcagattgcggggagagggaggatgtaaatgcctgagacccgagggaagaggaggaaattggttccttcccaacagccattttcttggtttctctagatttcaaggagagtcaaagataaaatgagtatttaattcagtttcagaaaaaaagggtacattacttcgatgagaaagcataaaattaagaggcttttctggaaatccaagaaaaagaaataaccattaatatgttcaatgataattttctagatcttcctcgtgtccaaagctatatattttctcctcaaaagcagctgctccaagaactaactagccctctttatctccctctagctgggacagactaattcccctccacccccacctctcttctttcaataacactgtgtaggtgttaatggcctgggctctcaccaatgaagagaattgtcctttaagccagcaacccacaggcagtggcacccaaagcctcaccaacccaccccccaacccggcccatccccagggcagaagccacagagctggcattgtttccactgtctcaggaagaaggagccaaaagctgaccctcagcacaaatcaaagcccaatatggagagagaataactgcttctaggccgagagtaggcaagctgtgggcaaaaaaggggagtttttgcagccacctcatctttagaaacaaggggaaaactagacccttttccactattatggtctaccaggtactctactgctccaaggagatctgaaaatacaaaaggatctaaacaaataaggagaacttttcccaggctggagataagaatgacaaacagaaagatgggtgaatgtaataatgtgtaggaagatgatgctgggagcctcctttcttcacatggctgccagccccatagaggacaacacagtaagaaccaggacaaccactccagactggtatagctggggaatcttcaggccttttcctaggtcccacatctgcactcaaagcaataccagtgccacggtggcagatggacatcgccatgggaagagaccaatttctgatacagagctgagggctaaagtgggctcggaggcaatgacgaccaacgtgtctcagcaacagcgcagccatcttgggttccggtctggacggaagt

SEQ ID NO: 14666 - RNA, 1247 nt, Homo sapiens
  source 1..1247: mol_type = other RNA
gctgggattacaggcatgagccaccgtgcccggccttctcttttctaaggtttaaaaaaaatgacactgaaatcctgaataacaattataattaagaaaggtacacaagaacatgccaagaattcatcctatcagcagatatgctgggtagtaatgaagtttgcttatcggtagcactcttttaatcaagttttccattctgaagactatttttggctttctcttgtctgatgtgagagatgactttgatgcaaccttttgaaattttgatcatccacatgacattcatcacatccaaaacaacacaactaatgacccaggataactggattaaaactccaagccttatgtagggttctgttccatacacggaatacatgaagccataatgaggaagcattgaggcaatccgcacgatgaagaatactactgtcatgagtattccattgataacgatagctttagaaaacttgggatacttcagagcttcaaagaaccaccgctgattcacaaacgggctggaaagctctgcaagcaggcgaaaattcccaatgtatgccagcactccatttttcagtacaaggtagtatgcatacagggacgcacaatgatgcattataaaaaatttgtcaccaatcactttccaatacaaaattataatggacaaatcagaaatgaggtagcctgaggcaatagcaatattcacgtttgcaagtgatggaccaccccaaagtggatcagctttagtagcctcatcgaataagaaaatgtacaggccaaaaataccaaccaccaaagaatggcatgtggatactacccttgagttccattcaatcttctttttgaagctgagactattgaaacctggagaaacttttgctgaaaaccagtaacttacaaagtagaaaagaagctgaaaggtgaaaaagctgatacaggtaacactgatgagcagttttgtgttgatctccatatttcttcaacctgtgccgggtcccggggcgagtcgcgcgcgggcggcggctgcgccgagccgggagagggcggcgggtgtctacaggagtctgctcatccgggccggcccgagggctggcgctggccagtgccgcccggtgagatgctcacgggagccagggaagccgcgggttccgggccgcttggaggtgcagtcgcggaggctccagctaccgcggcggccgtcgcgcccgcccggactgcgggctcgggttaccgcagagctgctcctt

SEQ ID NO: 14667 - RNA, 1349 nt, Homo sapiens
  source 1..1349: mol_type = other RNA
gctgggattacaggcatgagccaccgtgcccggccttctcttttctaaggtttaaaaaaaatgacactgaaatcctgaataacaattataattaagaaaggtacacaagaacatgccaagaattcatcctatcagcagatatgctgggtagtaatgaagtttgcttatcggtagcactcttttaatcaagttttccattctgaagactatttttggctttctcttgtctgatgtgagagatgactttgatgcaaccttttgaaattttgatcatccacatgacattcatcacatccaaaacaacacaactaatgacccaggataactggattaaaactccaagccttatgtagggttctgttccatacacggaatacatgaagccataatgaggaagcattgaggcaatccgcacgatgaagaatactactgtcatgagtattccattgataacgatagctttagaaaacttgggatacttcagagcttcaaagaaccaccgctgattcacaaacgggctggaaagctctgcaagcaggcgaaaattcccaatgtatgccagcactccatttttcagtacaaggtagtatgcatacagggacgcacaatgatgcattataaaaaatttgtcaccaatcactttccaatacaaaattataatggacaaatcagaaatgaggtagcctgaggcaatagcaatattcacgtttgcaagtgatggaccaccccaaagtggatcagctttagtagcctcatcgaataagaaaatgtacaggccaaaaataccaaccaccaaagaatggcatgtggatactacccttgagttccattcaatcttctttttgaagctgagactattgaaacctggagaaacttttgctgaaaaccagtaacttacaaagtagaaaagaagctgaaaggtgaaaaagctgatacaggtaacactgatgagcagttttgtgttgatctccatatttcttcaacttgtaatcccagctacttgggaggctgaggcacaagactcacttgaacccaggagacagaagttgccgtgagccaaggtagtgtgtctggaattggtgggttcttggtcttactgacttgaagaatgaagccgcggaccttcgcggtgagtgttacagctcttaaggtggcgcgtctggagtttgttccttctgatgttcggatgtgttcagagtttcttccttctggtaggttcgtggtcttgctggcttcaggagtgaagctgcagaccttcgcggtgagtgttacagctcataaaagcagtgtagacctaaagagtgagcagtagcaagatttattgcaaagaacgaaagaacaaagcttcc

SEQ ID NO: 14668 - RNA, 313 nt, Homo sapiens
  source 1..313: mol_type = other RNA
gctgggattacaggcatgagccaccgtgcccggcctttccagtggttttcgaagtgctcccgacagcctcccatgagggaaagtgtgggaatggggatagggggtgctggctggttgagataactctcattcttcctcatttcaactacgttaatctgttctacatactgaatttattggtaagctttgatctgaagggttccatacctttttcactgagagcctttccactcccctccccttctagtagtcgtgaacttcagaccctcgcttcgactcccactgccataactgtttttaaccaagcttccct

SEQ ID NO: 14669 - RNA, 471 nt, Homo sapiens
  source 1..471: mol_type = other RNA
gctgggattacaggcatgagccaccgtgcccggcctttccagtggttttcgaagtgctcccgacagcctcccatgagggaaagtgtgggaatggggatagggggtgctggctggttgagataactctcattcttcctcatttcaactacgttaatctgttctacatactgaatttattggtaagctttgatctgaagggttccatactcgatatgaaacaatgtgcagaaggacatcttctagtgttgtgtgccccaagcagactcctgacattaagcccttctttttcctagacattctagagccatcactgttgctctctggagagtcacaatgtccttagcaaagaaaggctatgagaagacctttttcactgagagcctttccactcccctccccttctagtagtcgtgaacttcagaccctcgcttcgactcccactgccataactgtttttaaccaagcttccct

SEQ ID NO: 14670 - RNA, 411 nt, Homo sapiens
  source 1..411: mol_type = other RNA
gctgggattacaggcatgagccaccgtgcccggctgctttcagagagttacccattaagtgctgcgtttggttcttgacaaaggacgccacaaggtccagttgatttgtctccactttccccacaaacacgttcagcgcgtagtcccggaagaaaggcccctccatgcccatcagcacggccccggcgcgcgcctgcagctgctccaactggaagcgactggggatgagggcggagcgcaggtgacccagggcctccagcaccaaggggtcgcactgcaggcagccccagcctccgggggcgcccaagcccgagagcagcagaagggtcaaagccagaggcatggcggggcctttgtgacgtcacagagagaacccggcccgccccgcctcccaggcgagggcgcggtcag

SEQ ID NO: 14671 - RNA, 9993 nt, Homo sapiens
  source 1..9993: mol_type = other RNA
gctgggattacaggcatgagccaccgtgcccggctttagttaactttttttaaagggacagatttattttgatagagccctaaaatgtgctgtgtatagtcaacaatacaataatcacagatttcttaactcaactgcttgtctgacaattaagcagaagggaacctttccctcctgctgatggccctgggggatgcagagatgataaagatgctgtcattgctctgggtcggggggaggtctcaacagagtgggatttgaggggcctgacactgctagggtccctggatgcctcatcgtataccttctttggaggatccactgtcctgtaggagtttgcagttttgctgaggagtcagcagtcgcacagggagagaaatggttatgaagaaaacaggaagcctgtaagtaactgaatgcaaagggaaaaggaactcccatttgctgtgtccctatgccatgctcttcatagatgttacctttttacctcatgtattggttccctgagattgctgtaatgacataccacaaacttgggggcttaacacaacagaaacatattctctcacagttctggaggccagaagtccaaagtcagtaccaccgggctgaatggaagcagtcagcaggcagtgctcccttgcaagcctccaggagagaacgtgtttctcatttcttccagcttctggggctgctggcattccttggcttggggcggccatcaccagtctctgcctctgtgctcacattgactctcctcctctttgtgccttctcaattctgtcggtgccaaatctccgtctgctttcctcttataaagatatgtgtgacggcatttagggcccaacctaatccaggataactctgctctctcaggaggcttaactgcacacctgcatagactcattttccaaataaggtagtatttacaggttccagggctatgaatctgatgccattgggcaccattattcagcctcctatgcctcagaaccatcctgtgatgaaggccttattatcttcctcatacagggagtcaggatcagagagggtaagtaccccaggccacacagataatatgtaatggcatcaggttttgaactcagggctgactccaaagcccatgcttgttttctgtgccctgccatatccctactaagtgccaagtgggtgggtgatgcctgctgtgaccacaagaggttcagacaagaaagcaatcaatgggaattagcattcattcatgagagctagcaggtggccaagcccagacaagggcagtctccattcctccttgactactgtcttcccaccctcaccatcaaggaagttcttcctgggtctaacctaagccccacgtggggtatggataggagctctgctgcctttcccttggacgcccctctccccagccccattttcctgatgagtgtttgtttctccacaggatatgggttgcttttcctgtcattagtcatcacacctgtcatccgggctaaactctccaagctggtgagagagacagagcagggtgagtgtcagaacccacctgtgtctggttcctcatgtccagtgctgcccgaaacgggctgatgggcagccatggctgggggaacagcttgccttcccccctctcaccctggagaagtaagtggccaaaacaaacacatttctgtgaaattgcccacaatgggcagaggatcatgccaccttggattttcaaaccgcagagttgggatttgcagtcagcagagcacaattatgttctttctagataaccagagcagaggatttactctctgcagacctcagcttttccgtctgtaagatgggtgtggtgatgccagagttccctgtttctctggggtcagcgtgtacaagcccagaagtgaacaaccttgtgacatgggtttcattttccacagttgacagataaagaaacagagacccagggggttacattggctcacccaaggttactcagtaaatggtggagctaggatgcaaacctacgtctgtgtttaaaagcagctggtctcaggatctgggttttagtccgagccctgccacaggcctgtttcttcatctgtgatgtgggtggtttgcttttgatgacatcacagacccctctagatgtgacagaatttaatctcaacttctgttgggttgttgcacattttgtaaactgtgggttctcctggtatatctataaagaacagcttctccagcctctgggtctttatgccccagtctggaaacattcatctttttccatctgtcctggaatgaggatctgatgatgacagagactctggtgccatacagagcccactgtgggttctggtgtccccagaatccatgtgtcttcattcattcacctaaactttttttcccagcactttctctgtgcccagagatgtcaagagaaacaggagaaaagaacagcccttactaactagctacttccaggggaccaggcccagtgatgggtgatttccatgtgaacttaatgttgctcacaatctaggaaataggtattatccttatttagcagaaggaggaacaggaacccaaaggataagaagctattcagtggtgacaccgctatgaatattggaactgatcagaccagcagttaatcccaaacaggagatgattccaaagaggataaaccagaaaaaagccatttccatcaagctttcatcagacaatatcacatgtactttttttttcttttatgtgctgggttctgtcagatcacatgtacttttaatgtggatttaatagcagccatttgtttagtagcccctctgtgccagctactgtccacatatgaccttactgaatccttgtcacagtacatgatgtagcaggatttactggtgaggaaggggagacataggttaagtgactactcccggtcacacagctgtgaggtggtggtgccagagttggaatatggccctttcggactccagagtatggtatttatttcttcacaggtgctctcttttctgctgtggcctgtgtgaatagcctggccatgctgacggcctccggcatcttcaactcactctacccagccactctgaactttatgaaggggttccccttcctcctgggagctggcctcctgctcatcccggctgttctgattgggtaatgcagggccctgaacccatgctcataatggagccctttctcttaaaagtttcctcttctcctcccaaccagaaatggcagcttcattcctggaatccttaccctctgggtgtcttgtcccaggttgcccctctccttgcagatggctgcctaatcctccaggagccattttccaagggcgagatggcgagctaggtggaggaaggatcaggctaacattgctgcttggcaaggctgtgttctctctcccagttcccctatttccctccattcccattttatagatggaactatggcagcagaactgtgttaaagggaaggccaggaagctttgtcagctagttgtggctgggccacaggctagcttgacccgctgactttttcctgtatgatattaagaattatatttcatggccgggcgtggaggctcttgcctgtaatcccgatcctgtgggaggctgaggcaggaggaccacttgagcccgggaattcaagatcagcctgggcaacatagcaagaccttgtctgtataaaaaatttaaaaaatcacccaggcatggtggtatgcactggtagtcccagctactaaggaggctgaggcaggaggatcacttgagcccaggagttcaagggtacagtgagctatgattatgtcactgccctccagcctggacaacagagcaagaccctgtctcttaaaaaaaaaaaagttattttccagagccatgtccctggatattgtcctccagctctcagcttctcagcttggggaaggaggaggttcaggagagctacctggaccagcccaccccagtaaatcctgtgtcacttctccagacaggccttgagggttccccacatgaaatccaaactctctctctggtctctcacaggatgctggaaaaggctgatcctcacctcgagttccagcagtttccccagagcccctgatctgcctggaccagaagacagagggcaagaggagcaaagtgaacaccaagcaactggaggtctgcagctggaagcccagcccacagcaggacaagcaactcttgtctaagggcagtgctctctttggacgaggtagtcaagagagaccaaggcaccaccccatccacagctgacccagcctctgtctaggatctagaatcataacccacacaggcccactgcaggacaggtggcagaggagctatttgggacaggagtcagttctccctttctgctatccatcacttataaccccacaggccagaggagaggtcctgagagaggtgacacttcagggaccagaggcagcacgagggctggcatctctccttccagcccaaactgcacagccccaaccaggttcccaacacgtgtagcagtcatcagccattccttaacaatgaatgtggtacctggttagtgccagccttgggaaggagggagggaggtaagaggggcttggtgatctctggaggaagagtgttgcctttgctgtggttggggaatcgatccttggctatggcctacccactcccctggctgaagagtgccaatcattacaaatcagcttcagcaaactgaaacaaaccttctggtgccttgggctttggggccctctgttttcctgctcccagtctgcctgccatacgttagacaacagaagctgctgggctgggcaggagccctgagctgcctggtggattggtaccaagtggggccagccagggcttctactgactcgctgtgcaaccttgagcaagccccactaggaacggctagatcagcaatgccccaaattgttgaatcgtggtgatcacatttggatggacaagttaggaaacttagctgattctctgagatacttcccacttcctcatacattctacaatgagatgcctctcttcatgggcctggggaaaggatgaatgagtgtggctggacttttgacctttaatgtccctgagcagttcttggcccttggggagaagtagggggaggatctggctgactcagccccaaccgaggggtagcagctgcagcccagccaagcagaacaccctggccctacagacctgtgtctgagcaggctttggaggaaaggccacttctgagtcctctgtctcaggagaagccaggcctaggtgcttgacctggtgatctgagctgtgtttgtcctagtatgggtggcagtcacctctgaacacactggccttggcttagaggaggcttgtgacttcagctgttccagctggggctggatgctggactctgattccctcagagagacagaagatcgggcagaggtcaaccagaaggccacacagggcagtggacaacagtggagggtataccaaatagaaataaaacgcaggaaacctctctgaatactgcccttggggacctcaggagggagtgggactgattggagacaaagagccagaaatcatcccctggagatactcagacactgtattgttattggcgctgtcctgtgagggcagtgtccaggctgccctgcttgtcatatccatgccctggctctggccccggtgagcacttgtgctgcatgaggaaaggaggatcaggtggggtcaaaaccaaagcatcgaggctggcactggccaagacagactctggcagggaggggagtggaaggaaggagccccaaacctggagtgagacctttgactttctgatgatgtggccaagaactaggagtcacctggccagcacagccaagagtggggctgggggcgcagccagctttaaggtgtcaacacctggcccttgcggggaaagagccttcagcagcccccacggcctggagcctgggtttattggagggtgctttcttaccctctgaacccagtggaggagggggcaatgggatattcctgctctgtatggcctctgggtcagctttttgttgcaaaatcctatcccccgctgctagattctttgaagcaagggagaagcaatagcccagcctcagaatgattctcaggaaagcaattccactgccagtggactgggtgccaggaggcctaggtctggatctggggctgccactaatgacaggaaagtgggcttatcctcaacctttctgagcctcagtgtcattatctgtaaaatggggatgataataccaggtagagttgctctgatgactggagaccatggagcggagtgtttgggaaatggcaaagatttgtgagggcttcgtgctttagagatttgctacccttaaccaccagcatcagctcacctgggaatctgtaagaaatgcagagtcctaggccccaccccagatctcctgattttaacaacattcccaggtgacttggatgcatgttaaagttggagaagctgccctaagtgacaaccctttgccttttcaggactttgcctctttccacagagctgcaggttctgtctaggctgcttttactgccatgggggctgcctggtccctgagtaagcagtgggtagccctggatggctgaggggctggggaagccagctgggccagaccaggaaggagcctgaggcacagcaccaaggcatggggtagggtgggctttgaggcacggcctccccatgcccagacccaggcccaaacaggaggctcctgtgcaccagcaagtgcagcaaagctggctgcagtgacaaggaagtcagagggagggctggtttgcctcaaccctcgccctggatgtggcaaaagataccacaccgaaggaagctgtaggggatctgggacttagtcaggctagctaagggcactgagtgattacagggcaaggccacagagcggcaggaagttgtaagtgcaggggccaggcacagtctgagtggagagccatgatggcactcatccctggctggctcctgggcccaggcccttgctcagaatacagtgcccaggcccgcctgggcattgccttaattcctgtctgaggctgccttccgtcatcctcctcaagctgactgctatcagcaggagaagggaatgcagaaccacccccaccccaactccagtgtctccagaactgagcagggaccctccccatgacggagacagacaacccaatggcagggcctgggggagttctaacctcccgtgcccaagcctgacttcccttccctctccagatactgaggaaagtgggttggaggtgggccatgagggtgggggacagggggagggagagccatttcctaagaagagcccaggttgtctcagcccagggagactggtttcaggagctgttccttcagaaaggacgatggaaatggaagtcacagcagggctggggaactggggactggttaggttggacccatgggtgcagcaccctccaaactggtgtcagagcctgcagatgagtcccgggaggagcggccctgcaggaagcggatgatcttctcaatggtggcctcctggtattcgtgggaccacttgataccgttgaaagtaagcacagcctgcatgtcctcaggcaggacctggggctcaggccactcgaagccatcaatgatgggcacaatgttcttgccgcagcttaaagcagtcacaatctccttatgcacccaatccttgcagtcatggtcttgcatgcacttgtccagtgctccaggtgatagcaccaacacaaagttgcgggcacccatgacactctggatgagtttgtcctcgaacttgcctgcttccagcttctccacatcaatgaagacactgaagccatgcagctgcaggtgcaccttcaggagactggccagctgggaacctgagttccggcggtagctgatgaagacatctggagtgtccccactgggtttgccaccagtacagggcagcggggagtgtagcatttctctggccgccgtgaggatgcgggcgcggtgcacgcccaggtggatgccgcagtcttccagcagctgctgctcagacacgcggtgcagcagggagcggtccaggccgcagctgaccaggccgtaggtgtactggcggaagcgcgggtccaggctgcccagccagtccgccaggttgctgcggtcgcacgtagaatagttggcgaaggtcttgagctccgtgagctccctaaagaacctcttgcgggtgatgcccgatttcatgcccaggtcggtctggagttcctcctccgtgagccgcagaagcaggtcgccatccacctgctgctcccggaagctctcgcagtacttggagaaaccgatctgctgcagccacgtctgaacctcggcctccttccagctgggcacggagggcaggatgggccgtggcacctcctcgcccagcaggcgcagcgcgcgcttggccagcgccgacttagtgccattggtagagtaggaaaccaggcgtttcaggctctggatggcgccgatgtcgctgaacaccttggtcttgccttgcaggctcttgatggcagcctcggcgcagaggtagaaagccccgatgcactgcgcctccaagcggttagagtcgagcaacggcacgaggcgctgcaggtcgtcgggcccgcggccctggcttgtgtcgctggcgtccaccagacagcgggcgaagcggccagggtccagcgaggccacaagcggctccacgagcgccagcgtgcccgagcgctccacctcgcgctccacctccttgttagtcgccaacaccgctactgcgaggcaggcgtgcagccgaagcagctcgtcctccttggagaaggcgagcgggaagagccactcggctgcgcgcttctctaccatgcgtcgctgcaccgcctggcccccgtgcagcgcgcagttgcccagcgccagcgcgcagtggcgcagcagcgcggggtccgtgcggcggcaccaatacagcaccgcgtccaggccgccggccgccaccagcctctggcatgtctcctccgaatgcttgaacatgtgctccaagatgcctgccacgctccgcgccagctctacgggttcgcgttccttcgccaggttcaggatcacgcccagcccaatgcgcgccacgcggtctcggttctcagccaccaggatctgctccagcaggcgcgcggcctgcacacgcgtctccaactccggcgcctgcagcagccgcaacagcaggtcgaggccgccatcgaggcggatggcgtcgcacagaccctgggctacctcgcggcccacggccggcagcagccaggcctcctccaccagttggaagacctcggccaggccggcgcccacggcccgcgcgccgcccgcctgcttcagcgcggacaaggcctgctgcagctccggcagcgcgcgctccagggcgtcctgcacctcggtgcctgcccccggcgacacttcgcggggcccgcggccacccgcagcccaccatgggcccgtgccaccgcccccatctggcccaggcaccgccagccgctcggcgcccggccgtgggcccgacatggcgaagaagcgacacagcttgtaggcggagagaagcagcgtcaggaccatgggcgcggggccgcgggggacatccccggcctggaggcggggccacgcggagagacccgggttttgggaaaagagggacccgagaggggtcggggaaagaagatggagggggaggaatggagagaagggtaccaggcaagggtgccggtcagaagtttgggggaggagtgtcggcaggatcgggggagcggttggcaaaggtgatgcaggcccagatgcagggagtgggcgaaaggagagagcgagcaggcgagggatggctccggacgccgtagggtagaggaggcggcggctggaacaaagcgtggcctgggcacgggctcggctgagctgggagat

SEQ ID NO: 14672 - RNA, 2228 nt, Homo sapiens
  source 1..2228: mol_type = other RNA
gctgggattacaggcatgagccaccgtgccctgcctgggcacttgttcttaaccagtggtgggaactttttcaaaatacagttatctgagaaatcacatgttaggatgcctgaaattacaggaaataatatttaaaatgcctattctttacaattagaaagtcatttgatgagtctggggcaaaatcctaacttaacatttttaacaaggaccccagaggattctgatgtgggtgatctatgtagatcaccctgtgaaaactactacccactaggtgattattttcttctttctcaagacctttccgtaactccaaccccataccatcaccaaactcacacacagctccctcactgtcaatttaagggaaagtacctaagaagcaaccatacggagggcaggactgacctctcagaagagtgagaccatcgtcaggagttggcctgtaagagaactagctcacctccacagctggcctgagatttcccccagaaaacagttcttgatctatttcaacacaaacgtaccatcatgtacccacaattctgtgtcacacagcataaccgtgataagctcagccaataatatttctttatgggccactgtagacattttcaaaaatcccaacacactgatagaacatctcattttcagtaatttaacacctagagaaagatctttcttgctgtgtctgtgcacacacttacctatcttctactgtcttattagaaggataaaaaactttgaatgaaaatccacttcttggaaaagagccagggtttatgcagaggcattcggtatttgtcgtagtgaaaggatcatatttgtctgcaatgacaagtagatcgggcacaggatacactctcaaagcatagtcatatgcccaatacactgggcagacataaagaggtaggggagtcagatgtccttgggataagatagtctttacaaagtgattaggaatagccaaattgctgctaggaaaacggacgcagtttctgcacattttatttactaagtcttcacggaagacagtaatttcctgtgtacagtactgaattctgcaaggattagtagtaaaaactgaaaatggtaccctttgtctgaattcattagtgatgctttcagcaagtggtggccttggtaagatggaaccaaatccaggatcctctggaccaggtacaaacacaaaacgactactttcaaagcttgaacttgattttttccatatggtgcagatgaaaaattaccacacagaataaagcaggttggaggtgctggtgaataaccagcaaacattatgcgaagtttttccaatacttccacctggtccaaccaaacatcagataaaaacacaaacatagcatctttattctcctcttctagctgttttagttttgcagaagtcttcacagatgtattagaaggacctccaaaaaaattaatatttccatagtatgccctagtagtactagagggctcagtgggtggaaatccaaaggcattgacatgaaacacttgatcttcaaaccaaccttctgctaagacaaagcatgcctctgtgtataaaccactatggaactgagctttactaaggtctagttggactgttccagtaggatcttccagaaaaaattttccctcttttaactgcgttatcattccaagaacaatcgcatctccgattttggttgtactacccaataaggtttctattgttttaagctggaatttgcttccgctttcatcagggtgagaacctatcaccggaggagtaaataattcatgcctgtgggtcctctggtgcaaaatggtatatcgctcacgaaacatctctgctttatctcttggtgttccaaataaatttggtgcagggtggttggtcattaacagaggaagaaatttttttctttctgaattgtacacaaagcgtggaatatcaaatgctcctatgatattgaaaacgtgctctatagtttcatcaacagactgactgcattcctggactgctgcttccaccacagatcgttcaatcatgtttgatgacaagggttgcttctcaactgcattaattatcttttccagtttatcttcaagctctaattcactgatagactgaagagcttctgtgaggtacttaatagcttcaccacggagcagcaagccccgcaacttgaaggcggagagcgcccggctccgcagccgctccggcgccatatttgcgattt

SEQ ID NO: 14673 - RNA, 2283 nt, Homo sapiens
  source 1..2283: mol_type = other RNA
gctgggattacaggcatgagccaccgtgccctgcctgggcacttgttcttaaccagtggtgggaactttttcaaaatacagttatctgagaaatcacatgttaggatgcctgaaattacaggaaataatatttaaaatgcctattctttacaattagaaagtcatttgatgagtctggggcaaaatcctaacttaacatttttaacaaggaccccagaggattctgatgtgggtgatctatgtagatcaccctgtgaaaactactacccactaggtgattattttcttctttctcaagacctttccgtaactccaaccccataccatcaccaaactcacacacagctccctcactgtcaatttaagggaaagtacctaagaagcaaccatacggagggcaggactgacctctcagaagagtgagaccatcgtcaggagttggcctgtaagagaactagctcacctccacagctggcctgagatttcccccagaaaacagttcttgatctatttcaacacaaacgtaccatcatgtacccacaattctgtgtcacacagcataaccgtgataagctcagccaataatatttctttatgggccactgtagacattttcaaaaatcccaacacactgatagaacatctcattttcagtaatttaacacctagagaaagatctttcttgctgtgtctgtgcacacacttacctatcttctactgtcttattagaaggataaaaaactttgaatgaaaatccacttcttggaaaagagccagggtttatgcagaggcattcggtatttgtcgtagtgaaaggatcatatttgtctgcaatgacaagtagatcgggcacaggatacactctcaaagcatagtcatatgcccaatacactgggcagacataaagaggtaggggagtcagatgtccttgggataagatagtctttacaaagtgattaggaatagccaaattgctgctaggaaaacggacgcagtttctgcacattttatttactaagtcttcacggaagacagtaatttcctgtgtacagtactgaattctgcaaggattagtagtaaaaactgaaaatggtaccctttgtctgaattcattagtgatgctttcagcaagtggtggccttggtaagatggaaccaaatccaggatcctctggaccaggtacaaacacaaaacgactactttggtgaatatctgggtattcacatattatatctgccaaagtttttagggaatctttcaaagcttgaacttgattttttccatatggtgcagatgaaaaattaccacacagaataaagcaggttggaggtgctggtgaataaccagcaaacattatgcgaagtttttccaatacttccacctggtccaaccaaacatcagataaaaacacaaacatagcatctttattctcctcttctagctgttttagttttgcagaagtcttcacagatgtattagaaggacctccaaaaaaattaatatttccatagtatgccctagtagtactagagggctcagtgggtggaaatccaaaggcattgacatgaaacacttgatcttcaaaccaaccttctgctaagacaaagcatgcctctgtgtataaaccactatggaactgagctttactaaggtctagttggactgttccagtaggatcttccagaaaaaattttccctcttttaactgcgttatcattccaagaacaatcgcatctccgattttggttgtactacccaataaggtttctattgttttaagctggaatttgcttccgctttcatcagggtgagaacctatcaccggaggagtaaataattcatgcctgtgggtcctctggtgcaaaatggtatatcgctcacgaaacatctctgctttatctcttggtgttccaaataaatttggtgcagggtggttggtcattaacagaggaagaaatttttttctttctgaattgtacacaaagcgtggaatatcaaatgctcctatgatattgaaaacgtgctctatagtttcatcaacagactgactgcattcctggactgctgcttccaccacagatcgttcaatcatgtttgatgacaagggttgcttctcaactgcattaattatcttttccagtttatcttcaagctctaattcactgatagactgaagagcttctgtgaggtacttaatagcttcaccacggagcagcaagccccgcaacttgaaggcggagagcgcccggctccgcagccgctccggcgccatatttgcgattt

SEQ ID NO: 14674 - RNA, 6381 nt, Homo sapiens
  source 1..6381: mol_type = other RNA
gctgggattacaggcatgagccaccgtgccggacctatttaaaaatctttttgaagtacagtactaataaactaaggactacctagagatcacacttttagatattatctattttaacatagattaaaaatactgtttatatgaaaattaagcttaaatacacgtataggtaataattattttgcccatatacaagtaatgtaaacagaggctatcaaggtgacccattatctactctaatttatatccactatgagcttcttcccagttgttatacaatgccatattttaattcctgactgaatggttaggaaagcaaaatgtaactctgtaaacttgatcagcactaatgtacaacatattatggagggtaaagtgaagcaagaatatattcaagtaaaataaaatgtctttcatgggcattcaaatcccacatctctctatatttctttcccaactaagagctataattaaaatcccatttattatttttctatagttcagaatcaacgtataaaatatgatgaaagtgaaactatctccctatatatcacatcatatatattgtgagaaagtcacttgttatatatggatatttcaattaactcataaatttttaaaaacatatcctccatacttatttctaacagaaaaaaataacaggaattattttactttactcacatggacaatgcagattttgtgggggtagaagtgtacacaactttgctggtcttcttcaacaaaattagtacagaattcctaatacaaagttaggttcaggacctcgaatggaacatgtctaagtgagaggcactgaagcttaggtttcattagcttcctgcgagatccacctatgcacagcaaacaactaatttttaatatttctctgactatattgcataacattaaaatattgttaccttcagtccatactatctttcatttcctgattctctggccttcggttttttatcttttcataccttatacctcaattacaaaagatcaactttaacaaaggtcagagttgctccctttcttagcagtatattcatctgcaaatcaagataaaataatgattttcctgtagactgattacagttcatgaggaattctgttatgtaattatactcttgttaaccctctattgatatgtcaaattgtaattggggaaacaattttaccagacacataagacgaacaggaaatctgtttcaacgtgaatatcttagtgttggagaaaccgtcatgcattgctaacgtaacctaataagctgtccaaattttgtgtccacagggctgaggagctacagtctaaatgcatacgcatgttgggaaccgaagtcagccatcttccctaggacaaatctttactcttctaaagaaggacaagaataaggtctactttcagctaaccatttataaggttcagttttcattggatcaaaggaatataatctaatactttttaaatggggtcaaaacagtattataaggaaaatatttactgcaaatatttataattgtgtaaggagaatcattctttttaaaatcaagttgtgttttagctttagaatcttttaaaatcacaagtatttgagaatccatccccacaaaaattaaaaaatactatattagttattttaaacagtattcattacttttactgtttatgttataataaacttatgtatataaacatttgaatatgcatggtacaaagtacaagtacagaacatgtagtaagtagtatgtgcatgtatgtgtgtgtgtgcatatcgtataaaaatatgagaaaaattttacttatataaaaacatatatataaataagtgttcaggagagtttttgagaatctgctttacatactgcaattttgagtgaaaattatggatattaatttcctgattaaaggaactgtgtcttctcatgatgagtcctaaaaataagccaaaatactacttaatctccatcactttttttcttaattactggctgactttttttctgcgtgaaatggcattacaatggcagggaaatttaataatgcaaaaatcacttttgaaaatgagaaagaataattctagttaccttttaaattgatacttttaaagagaaattcaaatcaaaaataaataaattaaagtctgagaccaatttgccactgtgaatataagcacattaaccccaggaagagccaagaactacacaaacctctctatgagaatttaccagtcttctttcatttggcaagaaaaagctcaggaaaatttgcttgtttaaattctatgagcctagtctatggggaaaaaaaaaataggaatatgaaagaaattcttacctccagcaacatatcatagggagagatgtggacaaatgaacaatatttactggaaataggaattataaatcaaattttgaaaaccctatgctaaggaaggaaggagttattataaattcactcagagacccaaacgttaggttcagctaaagaaatgtcagtcttggatatatattaaatgttttcaagagcaaaattgaaattactgaattggaaatgctccaaattataggtcatcatttctactttggacaattttttatgaattctatgtttgcctttaataattttaattggtataattctttcaaaaatccttattttcaaatggacaaaaattaaaggatgaaacatactctggccatgactaaccattttaccttagatgtttataaataacagttcaaaatttcatcattatattactctcatttgtaagttccactatatatatatatatatatatataaaaagtgtgtgtgtgtgtgtgtatatatatatatatatatatacacacacacacacacacacacatacacacacatatatatatatatataatcttttttttttggagatggagtctgactttgtcacccaggctggagtacagtggtgcaatcttggctcactgcaacctccgcctcccgggttcaagcaattctcctgcctcagcctcctcaatagctgagattaccagcatgtgccaccatgcccagctaattttgtatttttagtagagatggggtttctccatgttggtcaggctggtctagaactcccgacctcaggtgatccaccccctcagcctcccaaagtgctgggattacagatgtaagccaccatgcccggctcacagtattttctaatactggcaaaacaacatcttctgaacacaaacacttatccacagattctcatttcaattttcttcttatcagttgtctcttttgcaagttgaatgataattaaggtgtggaaattactgacaaagcctagatatagaagtggaaattttctagaaacatcagttgtaaatcttatttacagcgacatttcttttgcaatttttatgttaatatatgccttttcctaattaatctggacagtttcatctgaagagatattttaacagaagaatataaaatgtataaagaaaatgcacaaactgtcaaaattcatcatcgtgtaaaaatagccataaatttaaaaaacttcagaattactaacattgcatgtagatatgattacagatatgggactattattttgaacatcttctttgttggtgatttctctcatgttgataatgtaatttgaaggcttaaaatgcatatgtttagatagactcatcaggggtaagttattagtgaaacaggtggttgttctaatgaggatttaataccaaactaactcttgctctaagatgtgttatacactttcctgatcaaactgatgtgaaaaaaaaaaatgacagataactaaaacttcctgataatgaatgaaaaaacatctgacataataaattctcaaggatttttacttaaacataactcctggatgtgtctcataaacagtagcccctagaaactcttctttaatgtattcaacaatccccactgacctttgttcaaagtgctctgggtataatccattaaagcatgagtgtttgttatctaaattggtatctaaggggaagcaatgcaatgtcaatgtaaaataaatttctttctctcctctttgccataatcatgatgtatgctttttttcagaattgaaaacacttttcacagtatagacatctatagtgtgtaaaaccatctttacaaaacccatatatacagaaaaatctcagtcttcaatttgaaggttctttgccgtgctaacatatgttgtagagaatgaccacatagtaattgtctagtcttttctcctaaccccaataggtaggtatcagagactcaagaattgtgcgactcatagaataactgcatattcactttctataactacatagagttataactaaatttcttagaaattagttcgaatatgctaaaatatatgaataaaaataactgactccttttgtttatcaccaaagttgtaattctctagactttcagaaaatgaagtaaaaatccctattttgtgtctccccttgggcagattgccaagatctcaagtccattagttcataacttatcttcttctggtacaacttccagtattatttgtaatgttctggttattttctccgacattattctaaaccacctgggtttcttgtcccatataataaagagataatacgcagggactccagtcagagtgatgacgaagccaatccctgtactaaatgggtccgaatagagggaaagggcaaccatgaagaggcatgtgaaggaaaacaaagctgggatgaacagtggcaccttgaaaggacgatgcatatctgggcatttgtatcgaagataaatcagcccagcaactgccagcccaataaaaagccacctggcaaaactgaggaaattcaaaagactgtcgaggtctccagagaagagcattatcattgtcaaagggtgcaaaacaataacagctggtagaggagtgtgcttgcggacatgaatcatggagaggatttctggaaggtgaccctctcgagacgcaacatagaataacctggagacagcaaacacaccaccgttcatggagccaaagcaggagagggcaacaaagatcggaactgctaatgagaaatttcccagtagccgctcagaaaaggtcactgccactgcatttgaaagcagcagctcctcagcattaatggtcgtaaagtaggccacatttgtcagcacatagccaatggtgacaatggccatggatatacatattgcaaggggaatggttcattctccattgtccacagatgaagaactccataaaagaagagaagacagagagacttttcagggttttctacttcttcagtaacaaagttgaggtaaaaccagccagcatatgcatacattccataataaaaagccagtggcaaccgcgtaatacttgaatctcttcctgaaaaggcgtctttaaagttctgcgtttgacctttaattagctgcataactccagggactataattatcagaattgctgtgagcttgcaaaaggttaagaaaatctggatccgggcgctccagctgacactcatgctatttaggaccatcactacagttatgcccacagctgtaatgagcttgatcgcaagttcagggatttcacattgaataaaaaatggttccagaatgtagcgtccaaatgccagggatatcacagcagtagctgcagggcgtattatgaggagttccacccagactcgtacaaaagctggtaatggaccaaagacttccaaaatatatgtgtaatgacctccagatttctttatagttgttcccaattcagcataagacaaagctccaaatagtgacaggaccccacacaccgtccagatggtcagagacatgcccacgctgcccgtgttctggagcacgcccttaggagagatgaagattcctgctccaatgatggtgccaatgataatggagactcccctcagtaaagtgactttcctcttcagctgcactttctcctgcccaggtggctccttgttgcccagggaaggcagcctcccgttaacatttccctgcaggtaacctcctttggagatggtggacacaacaggctttctgaccatagtagggacacacgggggaaaaataaaacagagggaaagaaaacaaaactttcaactttggtgtctcttggtgttactgatcgatgtcttcctctgctttcagactgtctctctcagcgctatagtgttcacaggtgaaaactcaaaggtgtgctttttccttcacagcgatctaattactactcagaaacacctgtgtatgcatcgtgctctcaattctccacctcctcgttccaccactgctgctgctgctgctgctgccgccctatcattacaaacc

SEQ ID NO: 14675 - RNA, 6325 nt, Homo sapiens
  source 1..6325: mol_type = other RNA
gctgggattacaggcatgagccaccgtgccggacctatttaaaaatctttttgaagtacagtactaataaactaaggactacctagagatcacacttttagatattatctattttaacatagattaaaaatactgtttatatgaaaattaagcttaaatacacgtataggtaataattattttgcccatatacaagtaatgtaaacagaggctatcaaggtgacccattatctactctaatttatatccactatgagcttcttcccagttgttatacaatgccatattttaattcctgactgaatggttaggaaagcaaaatgtaactctgtaaacttgatcagcactaatgtacaacatattatggagggtaaagtgaagcaagaatatattcaagtaaaataaaatgtctttcatgggcattcaaatcccacatctctctatatttctttcccaactaagagctataattaaaatcccatttattatttttctatagttcagaatcaacgtataaaatatgatgaaagtgaaactatctccctatatatcacatcatatatattgtgagaaagtcacttgttatatatggatatttcaattaactcataaatttttaaaaacatatcctccatacttatttctaacagaaaaaaataacaggaattattttactttactcacatggacaatgcagattttgtgggggtagaagtgtacacaactttgctggtcttcttcaacaaaattagtacagaattcctaatacaaagttaggttcaggacctcgaatggaacatgtctaagtgagaggcactgaagcttaggtttcattagcttcctgcgagatccacctatgcacagcaaacaactaatttttaatatttctctgactatattgcataacattaaaatattgttaccttcagtccatactatctttcatttcctgattctctggccttcggttttttatcttttcataccttatacctcaattacaaaagatcaactttaacaaaggtcagagttgctccctttcttagcagtatattcatctgcaaatcaagataaaataatgattttcctgtagactgattacagttcatgaggaattctgttatgtaattatactcttgttaaccctctattgatatgtcaaattgtaattggggaaacaattttaccagacacataagacgaacaggaaatctgtttcaacgtgaatatcttagtgttggagaaaccgtcatgcattgctaacgtaacctaataagctgtccaaattttgtgtccacagggctgaggagctacagtctaaatgcatacgcatgttgggaaccgaagtcagccatcttccctaggacaaatctttactcttctaaagaaggacaagaataaggtctactttcagctaaccatttataaggttcagttttcattggatcaaaggaatataatctaatactttttaaatggggtcaaaacagtattataaggaaaatatttactgcaaatatttataattgtgtaaggagaatcattctttttaaaatcaagttgtgttttagctttagaatcttttaaaatcacaagtatttgagaatccatccccacaaaaattaaaaaatactatattagttattttaaacagtattcattacttttactgtttatgttataataaacttatgtatataaacatttgaatatgcatggtacaaagtacaagtacagaacatgtagtaagtagtatgtgcatgtatgtgtgtgtgtgcatatcgtataaaaatatgagaaaaattttacttatataaaaacatatatataaataagtgttcaggagagtttttgagaatctgctttacatactgcaattttgagtgaaaattatggatattaatttcctgattaaaggaactgtgtcttctcatgatgagtcctaaaaataagccaaaatactacttaatctccatcactttttttcttaattactggctgactttttttctgcgtgaaatggcattacaatggcagggaaatttaataatgcaaaaatcacttttgaaaatgagaaagaataattctagttaccttttaaattgatacttttaaagagaaattcaaatcaaaaataaataaattaaagtctgagaccaatttgccactgtgaatataagcacattaaccccaggaagagccaagaactacacaaacctctctatgagaatttaccagtcttctttcatttggcaagaaaaagctcaggaaaatttgcttgtttaaattctatgagcctagtctatggggaaaaaaaaaataggaatatgaaagaaattcttacctccagcaacatatcatagggagagatgtggacaaatgaacaatatttactggaaataggaattataaatcaaattttgaaaaccctatgctaaggaaggaaggagttattataaattcactcagagacccaaacgttaggttcagctaaagaaatgtcagtcttggatatatattaaatgttttcaagagcaaaattgaaattactgaattggaaatgctccaaattataggtcatcatttctactttggacaattttttatgaattctatgtttgcctttaataattttaattggtataattctttcaaaaatccttattttcaaatggacaaaaattaaaggatgaaacatactctggccatgactaaccattttaccttagatgtttataaataacagttcaaaatttcatcattatattactctcatttgtaagttccactatatatatatatatatatatataaaaagtgtgtgtgtgtgtgtgtatatatatatatatatatatacacacacacacacacacacacatacacacacatatatatatatatataatcttttttttttggagatggagtctgactttgtcacccaggctggagtacagtggtgcaatcttggctcactgcaacctccgcctcccgggttcaagcaattctcctgcctcagcctcctcaatagctgagattaccagcatgtgccaccatgcccagctaattttgtatttttagtagagatggggtttctccatgttggtcaggctggtctagaactcccgacctcaggtgatccaccccctcagcctcccaaagtgctgggattacagatgtaagccaccatgcccggctcacagtattttctaatactggcaaaacaacatcttctgaacacaaacacttatccacagattctcatttcaattttcttcttatcagttgtctcttttgcaagttgaatgataattaaggtgtggaaattactgacaaagcctagatatagaagtggaaattttctagaaacatcagttgtaaatcttatttacagcgacatttcttttgcaatttttatgttaatatatgccttttcctaattaatctggacagtttcatctgaagagatattttaacagaagaatataaaatgtataaagaaaatgcacaaactgtcaaaattcatcatcgtgtaaaaatagccataaatttaaaaaacttcagaattactaacattgcatgtagatatgattacagatatgggactattattttgaacatcttctttgttggtgatttctctcatgttgataatgtaatttgaaggcttaaaatgcatatgtttagatagactcatcaggggtaagttattagtgaaacaggtggttgttctaatgaggatttaataccaaactaactcttgctctaagatgtgttatacactttcctgatcaaactgatgtgaaaaaaaaaaatgacagataactaaaacttcctgataatgaatgaaaaaacatctgacataataaattctcaaggatttttacttaaacataactcctggatgtgtctcataaacagtagcccctagaaactcttctttaatgtattcaacaatccccactgacctttgttcaaagtgctctgggtataatccattaaagcatgagtgtttgttatctaaattggtatctaaggggaagcaatgcaatgtcaatgtaaaataaatttctttctctcctctttgccataatcatgatgtatgctttttttcagaattgaaaacacttttcacagtatagacatctatagtgtgtaaaaccatctttacaaaacccatatatacagaaaaatctcagtcttcaatttgaaggttctttgccgtgctaacatatgttgtagagaatgaccacatagtaattgtctagtcttttctcctaaccccaataggtaggtatcagagactcaagaattgtgcgactcatagaataactgcatattcactttctataactacatagagttataactaaatttcttagaaattagttcgaatatgctaaaatatatgaataaaaataactgactccttttgtttatcaccaaagttgtaattctctagactttcagaaaatgaagtaaaaatccctattttgtgtctccccttgggcagattgccaagatctcaagtccattagttcataacttatcttcttctggtacaacttccagtattatttgtaatgttctggttattttctccgacattattctaaaccacctgggtttcttgtcccatataataaagagataatacgcagggactccagtcagagtgatgacgaagccaatccctgtactaaatgggtccgaatagagggaaagggcaaccatgaagaggcatgtgaaggaaaacaaagctgggatgaacagtggcaccttgaaaggacgatgcatatctgggcatttgtatcgaagataaatcagcccagcaactgccagcccaataaaaagccacctggcaaaactgaggaaattcaaaagactgtcgaggtctccagagaagagcattatcattgtcaaagggtgcaaaacaataacagctggtagaggagtgtgcttgcggacatgaatcatggagaggatttctggaaggtgaccctctcgagacgcaacatagaataacctggagacagcaaacacaccaccgttcatggagccaaagcaggagagggcaacaaagatcggaactgctaatgagaaatttcccagtagccgctcagaaaaggtcactgccactgcatttgaaagcagcagctcctcagcattaatggtcgtaaagtaggccacatttgtcagcacatagccaatggtgacaatggccatggatatacatattgcaaggggaatggttttttcagggttttctacttcttcagtaacaaagttgaggtaaaaccagccagcatatgcatacattccataataaaaagccagtggcaaccgcgtaatacttgaatctcttcctgaaaaggcgtctttaaagttctgcgtttgacctttaattagctgcataactccagggactataattatcagaattgctgtgagcttgcaaaaggttaagaaaatctggatccgggcgctccagctgacactcatgctatttaggaccatcactacagttatgcccacagctgtaatgagcttgatcgcaagttcagggatttcacattgaataaaaaatggttccagaatgtagcgtccaaatgccagggatatcacagcagtagctgcagggcgtattatgaggagttccacccagactcgtacaaaagctggtaatggaccaaagacttccaaaatatatgtgtaatgacctccagatttctttatagttgttcccaattcagcataagacaaagctccaaatagtgacaggaccccacacaccgtccagatggtcagagacatgcccacgctgcccgtgttctggagcacgcccttaggagagatgaagattcctgctccaatgatggtgccaatgataatggagactcccctcagtaaagtgactttcctcttcagctgcactttctcctgcccaggtggctccttgttgcccagggaaggcagcctcccgttaacatttccctgcaggtaacctcctttggagatggtggacacaacaggctttctgaccatagtagggacacacgggggaaaaataaaacagagggaaagaaaacaaaactttcaactttggtgtctcttggtgttactgatcgatgtcttcctctgctttcagactgtctctctcagcgctatagtgttcacaggtgaaaactcaaaggtgtgctttttccttcacagcgatctaattactactcagaaacacctgtgtatgcatcgtgctctcaattctccacctcctcgttccaccactgctgctgctgctgctgctgccgccctatcattacaaacc

SEQ ID NO: 14676 - RNA, 6201 nt, Homo sapiens
  source 1..6201: mol_type = other RNA
gctgggattacaggcatgagccaccgtgccggacctatttaaaaatctttttgaagtacagtactaataaactaaggactacctagagatcacacttttagatattatctattttaacatagattaaaaatactgtttatatgaaaattaagcttaaatacacgtataggtaataattattttgcccatatacaagtaatgtaaacagaggctatcaaggtgacccattatctactctaatttatatccactatgagcttcttcccagttgttatacaatgccatattttaattcctgactgaatggttaggaaagcaaaatgtaactctgtaaacttgatcagcactaatgtacaacatattatggagggtaaagtgaagcaagaatatattcaagtaaaataaaatgtctttcatgggcattcaaatcccacatctctctatatttctttcccaactaagagctataattaaaatcccatttattatttttctatagttcagaatcaacgtataaaatatgatgaaagtgaaactatctccctatatatcacatcatatatattgtgagaaagtcacttgttatatatggatatttcaattaactcataaatttttaaaaacatatcctccatacttatttctaacagaaaaaaataacaggaattattttactttactcacatggacaatgcagattttgtgggggtagaagtgtacacaactttgctggtcttcttcaacaaaattagtacagaattcctaatacaaagttaggttcaggacctcgaatggaacatgtctaagtgagaggcactgaagcttaggtttcattagcttcctgcgagatccacctatgcacagcaaacaactaatttttaatatttctctgactatattgcataacattaaaatattgttaccttcagtccatactatctttcatttcctgattctctggccttcggttttttatcttttcataccttatacctcaattacaaaagatcaactttaacaaaggtcagagttgctccctttcttagcagtatattcatctgcaaatcaagataaaataatgattttcctgtagactgattacagttcatgaggaattctgttatgtaattatactcttgttaaccctctattgatatgtcaaattgtaattggggaaacaattttaccagacacataagacgaacaggaaatctgtttcaacgtgaatatcttagtgttggagaaaccgtcatgcattgctaacgtaacctaataagctgtccaaattttgtgtccacagggctgaggagctacagtctaaatgcatacgcatgttgggaaccgaagtcagccatcttccctaggacaaatctttactcttctaaagaaggacaagaataaggtctactttcagctaaccatttataaggttcagttttcattggatcaaaggaatataatctaatactttttaaatggggtcaaaacagtattataaggaaaatatttactgcaaatatttataattgtgtaaggagaatcattctttttaaaatcaagttgtgttttagctttagaatcttttaaaatcacaagtatttgagaatccatccccacaaaaattaaaaaatactatattagttattttaaacagtattcattacttttactgtttatgttataataaacttatgtatataaacatttgaatatgcatggtacaaagtacaagtacagaacatgtagtaagtagtatgtgcatgtatgtgtgtgtgtgcatatcgtataaaaatatgagaaaaattttacttatataaaaacatatatataaataagtgttcaggagagtttttgagaatctgctttacatactgcaattttgagtgaaaattatggatattaatttcctgattaaaggaactgtgtcttctcatgatgagtcctaaaaataagccaaaatactacttaatctccatcactttttttcttaattactggctgactttttttctgcgtgaaatggcattacaatggcagggaaatttaataatgcaaaaatcacttttgaaaatgagaaagaataattctagttaccttttaaattgatacttttaaagagaaattcaaatcaaaaataaataaattaaagtctgagaccaatttgccactgtgaatataagcacattaaccccaggaagagccaagaactacacaaacctctctatgagaatttaccagtcttctttcatttggcaagaaaaagctcaggaaaatttgcttgtttaaattctatgagcctagtctatggggaaaaaaaaaataggaatatgaaagaaattcttacctccagcaacatatcatagggagagatgtggacaaatgaacaatatttactggaaataggaattataaatcaaattttgaaaaccctatgctaaggaaggaaggagttattataaattcactcagagacccaaacgttaggttcagctaaagaaatgtcagtcttggatatatattaaatgttttcaagagcaaaattgaaattactgaattggaaatgctccaaattataggtcatcatttctactttggacaattttttatgaattctatgtttgcctttaataattttaattggtataattctttcaaaaatccttattttcaaatggacaaaaattaaaggatgaaacatactctggccatgactaaccattttaccttagatgtttataaataacagttcaaaatttcatcattatattactctcatttgtaagttccactatatatatatatatatatatataaaaagtgtgtgtgtgtgtgtgtatatatatatatatatatatacacacacacacacacacacacatacacacacatatatatatatatataatcttttttttttggagatggagtctgactttgtcacccaggctggagtacagtggtgcaatcttggctcactgcaacctccgcctcccgggttcaagcaattctcctgcctcagcctcctcaatagctgagattaccagcatgtgccaccatgcccagctaattttgtatttttagtagagatggggtttctccatgttggtcaggctggtctagaactcccgacctcaggtgatccaccccctcagcctcccaaagtgctgggattacagatgtaagccaccatgcccggctcacagtattttctaatactggcaaaacaacatcttctgaacacaaacacttatccacagattctcatttcaattttcttcttatcagttgtctcttttgcaagttgaatgataattaaggtgtggaaattactgacaaagcctagatatagaagtggaaattttctagaaacatcagttgtaaatcttatttacagcgacatttcttttgcaatttttatgttaatatatgccttttcctaattaatctggacagtttcatctgaagagatattttaacagaagaatataaaatgtataaagaaaatgcacaaactgtcaaaattcatcatcgtgtaaaaatagccataaatttaaaaaacttcagaattactaacattgcatgtagatatgattacagatatgggactattattttgaacatcttctttgttggtgatttctctcatgttgataatgtaatttgaaggcttaaaatgcatatgtttagatagactcatcaggggtaagttattagtgaaacaggtggttgttctaatgaggatttaataccaaactaactcttgctctaagatgtgttatacactttcctgatcaaactgatgtgaaaaaaaaaaatgacagataactaaaacttcctgataatgaatgaaaaaacatctgacataataaattctcaaggatttttacttaaacataactcctggatgtgtctcataaacagtagcccctagaaactcttctttaatgtattcaacaatccccactgacctttgttcaaagtgctctgggtataatccattaaagcatgagtgtttgttatctaaattggtatctaaggggaagcaatgcaatgtcaatgtaaaataaatttctttctctcctctttgccataatcatgatgtatgctttttttcagaattgaaaacacttttcacagtatagacatctatagtgtgtaaaaccatctttacaaaacccatatatacagaaaaatctcagtcttcaatttgaaggttctttgccgtgctaacatatgttgtagagaatgaccacatagtaattgtctagtcttttctcctaaccccaataggtaggtatcagagactcaagaattgtgcgactcatagaataactgcatattcactttctataactacatagagttataactaaatttcttagaaattagttcgaatatgctaaaatatatgaataaaaataactgactccttttgtttatcaccaaagttgtaattctctagactttcagaaaatgaagtaaaaatccctattttgtgtctccccttgggcagattgccaagatctcaagtccattagttcataacttatcttcttctggtacaacttccagtattatttgtaatgttctggttattttctccgacattattctaaaccacctgggtttcttgtcccatataataaagagataatacgcagggactccagtcagagtgatgacgaagccaatccctgtactaaatgggtccgaatagagggaaagggcaaccatgaagaggcatgtgaaggaaaacaaagctgggatgaacagtggcaccttgaaaggacgatgcatatctgggcatttgtatcgaagataaatcagcccagcaactgccagcccaataaaaagccacctggcaaaactgaggaaattcaaaagactgtcgaggtctccagagaagagcattatcattgtcaaagggtgcaaaacaataacagctggtagaggagtgtgcttgcggacatgaatcatggagaggatttctggaaggtgaccctctcgagacgcaacatagaataacctggagacagcaaacacaccaccgttcatggagccaaagcaggagagggcaacaaagatcggaactgctaatgagaaatttcccagtagccgctcagaaaaggtttttcagggttttctacttcttcagtaacaaagttgaggtaaaaccagccagcatatgcatacattccataataaaaagccagtggcaaccgcgtaatacttgaatctcttcctgaaaaggcgtctttaaagttctgcgtttgacctttaattagctgcataactccagggactataattatcagaattgctgtgagcttgcaaaaggttaagaaaatctggatccgggcgctccagctgacactcatgctatttaggaccatcactacagttatgcccacagctgtaatgagcttgatcgcaagttcagggatttcacattgaataaaaaatggttccagaatgtagcgtccaaatgccagggatatcacagcagtagctgcagggcgtattatgaggagttccacccagactcgtacaaaagctggtaatggaccaaagacttccaaaatatatgtgtaatgacctccagatttctttatagttgttcccaattcagcataagacaaagctccaaatagtgacaggaccccacacaccgtccagatggtcagagacatgcccacgctgcccgtgttctggagcacgcccttaggagagatgaagattcctgctccaatgatggtgccaatgataatggagactcccctcagtaaagtgactttcctcttcagctgcactttctcctgcccaggtggctccttgttgcccagggaaggcagcctcccgttaacatttccctgcaggtaacctcctttggagatggtggacacaacaggctttctgaccatagtagggacacacgggggaaaaataaaacagagggaaagaaaacaaaactttcaactttggtgtctcttggtgttactgatcgatgtcttcctctgctttcagactgtctctctcagcgctatagtgttcacaggtgaaaactcaaaggtgtgctttttccttcacagcgatctaattactactcagaaacacctgtgtatgcatcgtgctctcaattctccacctcctcgttccaccactgctgctgctgctgctgctgccgccctatcattacaaacc

SEQ ID NO: 14677 - RNA, 1049 nt, Homo sapiens
  source 1..1049: mol_type = other RNA
gctgggattacaggcatgagccaccgtgccgggctgaaaaataaccctttagatatctacagctttaaactgtgtgcagtcatgaaaagcagacattagaagtcattggcatttaataaattgcagtaaaattatacagtaaatacattacaatcattaataataggctttaatgagaagaatttaataaataatcattaaaaagacagcagaattttattctgttctcaatatgttgctgctcttcttatcaaatactataataaaactatatgactataatatagatttcaggagctaaaaaaagccttatattttcaaataaaagaacaatataaattttgcaaaatacaatgagcattactgaagtataaagtaaatatttggaattaaaatatatggtcatttagatacagactaaaaaagaatagaaatcttaatgattcctttctgcctacagtgagcttaaaattacaaccaaaaattttaataaatatgtagcacctacaagaaattttattaacagcttacataatgtgtaaatttgagcaatttattttagaacttttgaatctgaaaatcacctgcttgacattcatttgagaaagtgaaacataaaggagagtaacataagcaagacgacagaatgggaggttctgcatccacatcccccacgacataatgcagctgccacagcaaacataagtgcattcatgaaagccttggaatccagttcagagtttgtgacacccagctgagacttagatgacaggcctgcagaacttggttctctctatagtccctgaatcaggcaaaacacaccttctttccttctccagccatggtctggaagaaatcatttcccagcttccaggatgtcctggcaccttaactatgcgtccccaaggacctacagatcgcagggcaacaggggctgtgacagagtagcccagggctctcaaggtgcaggaggcgaaagaggagacagatcccaagctcctgtgccagcaccagcgagagacacagatcccgccaaatgcaggaagcca

SEQ ID NO: 14678 - RNA, 3118 nt, Homo sapiens
  source 1..3118: mol_type = other RNA
gctgggattacaggcatgagccaccgtgccgggctgaaaaataaccctttagatatctacagctttaaactgtgtgcagtcatgaaaagcagacattagaagtcattggcatttaataaattgcagtaaaattatacagtaaatacattacaatcattaataataggctttaatgagaagaatttaataaataatcattaaaaagacagcagaattttattctgttctcaatatgttgctgctcttcttatcaaatactataataaaactatatgactataatatagatttcaggagctaaaaaaagccttatattttcaaataaaagaacaatataaattttgcaaaatacaatgagcattactgaagtataaagtaaatatttggaattaaaatatatggtcatttagatacagactaaaaaagaatagaaatcttaatgattcctttctgcctacagtgagcttaaaattacaaccaaaaattttaataaatatgtagcacctacaagaaattttattaacagcttacataatgtgtaaatttgagcaatttattttagaacttttgaatctgaaaatcacctgcttgacattcatttgagaaagtgaaacataaaggagagtaacataagcaagacgacagaatgggaggttctgcatccacatcccccacgacataatgcagctgccacagcaaacataagtgcattcatgaaagccttggaatccagttcagagtttgtgacacccagctgagacttagatgacaggcctgcagaacttggttctctctatagtccctgaatcaggcaaaacacaccttctttccttctccagccatggtctggaagaaatcttcacattgatatgatgaaatgctaactaacaatatgaaaaatactaaagtataaatgtcactaaaatggtaaatacatactgaatttcagaatactataaattgttatcatcttaaactagactattaaaatacaagatgttttacataagtctcatgataaccagtaggaaaaaaaaatagtaaagaaaaagagaaagtaattaaagcatacacaaacaacaaaaattacacattggatatggtgtctcctgcttataattccaacactttgggaggccaaggtggaagaatcaaatctccttgggtgttgtggtacatgtctgcagtccaagctacttgggtggctaaggtgggacgattatttgagcccaggaggttaaggctacagtgagctgtgatatgccactgcacttcagtctgagcaagaaagcataactttgtctcaacaaaaatgaacaataccacaggaaagacagaaccagaaaaaaaagaagcaaacttaaaatggacagaaaactacaaatgtacaatagtaactgcttacctatcactaccttacaaataaaaagattaaagtatctactaaacagatactgctgtacactgaatgtcatctccaaaatttaggataaaatttaatagccaacatgttagaattaacaggtggaacctttaaaaattaattaagctataagcactctgccctcatgaatggattaacgttcttattatgggaatgggctaattataacaagaatggatctgttatatattaaaaaaaaaaagctctctctccctcacatctttgtgtatgttattatccagcaactagaccttcaacatataccagtataatgttgttttggcttcccagcctccagaatcatgagtcaaataaaattctattctttattaattaccagtgtgtgatattctgttatagcagccaaaagagactaaagcagacagagtggataaattaatcttttaaacctcataatatgctgcttacaagagactcaattatgaattaagagcataggctaaaagtgaaaggatagaaaatgatattccatgcaaataataaccaaaggagtgaaatggtaatgcttaaattagacaaaatagactttctagcaatgtctctcacaagaatgaaatgagtttaccatacaataatagaggttaatttctcaagagaatatagctttatatatttatgcacccaaaagggaggcttctaaatataaaaagcaaatattgccagaactgtagggagaagtagaaagaaacccaataatagaaaactttaacgaaatgtataataaaggacatatagttaacagcattgtaaattggcaagggaaagctggtctcatgtgttgcgtttgagaatgcagcaaagaaagtgggaactgataattttactgcaagcctgagttaggatgaaaaacagggtggtcgattagaggttccacttgccatacattaaaaaaacacaggagaaaaccagtcctcctctggagtgttaaaataattaaagatcagaaaattagtctaaagtggctctagtgccctgtgttcataggtaaaaaacaaaaaacaaacaaaaaaaaatctaaaacctaactcaaatatatttcctataaaacactatcttagcctgaagcaaaatgcaggtttaacccatgacaaacatgcaattaacctctgaatatgtaaccaggacatttccatctggatagttcaaataaggctaccatataactggaaccaattcttgaatttgggttgctttctcatgcatcttatgaaagcctttcctttatgcccctctggtggaccagaaatcatggctgggtgctttccatttcaccaatcactctttgttcagataaactgatgaaccttttaacatagactcccgttaatttttaacacgagagactgtggaccccacgggccgcagctcctcccacgcaaacacccactcgcggtttttccctgatgacccatctggcctccctgaacaatttgggaaatactcatggctgtgggcgcagagcagggcgctgcccagggacaggaccggatgggccggacgggacgtgggggtcctcgctgctggcccagcggccatcttgcagccacaggggactgagggccaagctgcgggagactcggagctaaccgtggggaggccggtcctgccggtttcacagtctgttctcccctctcgggatggcgaaccccgtat

SEQ ID NO: 14679 - RNA, 647 nt, Homo sapiens
  source 1..647: mol_type = other RNA
gctgggattacaggcatgagccaccgtgcctgaacttattttatagctctttggtctcctcccagatggcttggcaaacagcgattactgatgagtgttacccatcatgcaacaattctgctctcttttctgtcacacggtggtcagagactccagatagtcctccaatttaatgtaaaatgagacttgtttttgattgagggtctgaaggactctgcttcatgggtgacatccataaattttatgttccagcatatggtttatcttggtgaatgttccatgtgccctcagctattgcaccgacgcaccacgtgctctggtgcacatccaccgcctcttcctgcctcagtttctccttttgtaaaacaacagcttgtaaaggcctggggatcttctcatccacgggagttttctaaggatgcaggcgaaagaggtaggaaaagtactctgtctctgtcctgggtgttcgggatcaaggccttttgaaccaattccggaatccgccaccgggcggtggtaggagagagccagaggattcgtcagtaagtgtgcgtgcgtgacagagggcttttaaatagatcgctttgtatctagcacggtagcacctgcttctaagcttccaacggcagctcgagcaacgcgatcat

SEQ ID NO: 14680 - RNA, 4975 nt, Homo sapiens
  source 1..4975: mol_type = other RNA
gctgggattacaggcatgagccaccgtgcctgactgctgctttctaaataccatttcactcccacatttttctcccatcatgaaagtgtgtatcaggttggtttctctataaaaggaattatagctgaactagagctggaggagcataaccaccagcccaagagggaggggaaaagccggaaaggcgttgggcagggaggtggcttgggtacctggtttgaccacagttagaatatcatgattgtgttttgttagtctttaaatgattttgagtctgatagataactaaattctgattttaaaaactatttcagcaagagatttacattaaggctcatgaactaattcagatttttgttcgtgtctcttcaaaaattgctatcttagaaaagttagaattcaatgcccagttgaaaaattgcttggggcttgatagcaaatcaagtttcatcttatatacttttaatttgtaatataccaaagtcatttttgcaatactatattatgtactttcaagtatataattactgcttctttaaatacaaatgatcaagatattcagattattatgagttttttttggttatcatctattgctgctgcacaaattaccagatttcataattggtttaaataagcctccaatttgtttatatttattaacatgtatgattttgtgcatgtagaataagcttggcatagaaatggcctaaatgctcctgtagctcttcattcctttgtcgttctcactctccatgccagtatgtctcatttctagatcccatagaactttcaattgaaagtaataaccaaggcaactcactttccatgagtaatacaccacacttctagaaatcagcctatattactgtcacactggggattaagtaaaaaaaagagaaagaaggatgggaaggggagggaaggggaggggagcggaggaaagaagaaaaggaagggaaggggagggaaagggagagaaggggaggagagggaaaggagggaggaaggtaggaagaggagaaggaaggaagaaaggaaagaaatctgctcaccagagttgctattttttttttcttttctgtttagtgctttaccccttaattcttataggtaacggtctaatacagggtaactctcatagtggagaacttgagaagcattagtacttcaaattgagtcctaatggtaaaatttttttctgataaaaaaaggtactttgtagtgctgttaggaggtaacataatacctttactaccaatcttaggatcaattcaaggttcagtaaaaggaatgtatctggaattcttgattatagacatgaaaacactcttctgtcagcgttcatagtgagctgggaggttgcctacgcattaagacctagcttcataaaatgactcaaagccctaggcagtttctgggaaggactgggagtagcagtctcctggcaccccttgttcattcattcattcagtacctactatgtgctaggctttgaggatataacaatgaatttttcaaacaaattaaatagaccttggcctcaaagagctcacattctactagagaaggcacacatggagaagattataatacaatgttgtaaatccaatagtagagataaccagtttattttggggagcaaagagaaagggtccctaaccccagactgcctgcgaagaggtgaaatggaattgaatgggattatggtcagccaaggcttcctagtggagctgctacctgaactgagttttaagaggggtaggaaagaaaaaatgtagtgggtcataatggcattccagatacaggggacacaaacagctctgtgtttatgaactacaaccagttgttgacttttgtttcaagtggctccccttccccagtgctgtgtggacgatggactgaagaggagaaggctgggagcaagggaccagtaagctgttgcagcagtgcaggtgagatatgaggcctcaactctgcagtgttgacaaccatagagagcagagagcagaattcatcaatatttatcagcaccaatttttttttttaagacagagtctcacttcttcacccaggctggagtacaatggcgcaatcccggctcactgcaacctctgcctcccaggttcaagcgattctcctgcctcagcctccccagtagctgggattacaggcatgcaccaccacgcccgactaattttttttttttttttagtagagatggggtttcaccatgttggccaggctggtcttgagctcctgacctcaagtgatccgcccgccttggcctcccaaaatgctgggattacaggcatgagccaccatgcctggccaacaccaacctttagttacttgctgaatacacaggattaaggaggaagagaaagtatcaaggatgactcccaggttcctagcttggtggtcccagtaattgagagagagaatgcagcaggaagagcagctctagggggaacaggatgagtatctccacatgatgggttggaggtacctgtgagtcacatccaggtggatgtgtcctgtgggcagtgggacgcgagtctgaagctcaggcaagaggctagagttacatctttggagtcatcagcctaatggaggactgtggcatccaggtgccaaaagctagggaaacggctctggagagagaggggctttcttaattgacctgtatgctttgaagctctatagagacacaatcttatcccttcaggcctgtattttcttgggccactaagatgtggttacatattttctctcacatctcctagaacgtttgcaaaacaattcccagtcctatgatcatttctcccttcttctgagaactaattatatatggcacttaatatctattcacatgtagcactcatggtgaggtgttttttttgtttgtttgtttttgtttttttttttttgagacagagtcttactctgttgcccaagctggagtacaatggcactatctcggctcactgcaaactccgcctctagggttcaagcgattctcctgtctcagcctcctgaaaggctgcgattacaggtgcccgccaccacaccccgctaatatttagtagagacagggtttcaccatgttggtcaggctggttttgaactcctaacctcagggtgatccgcccaccttggcctcccaaagtgctgggattacaaggtgtgagccactgctcctggccttatggtgaagtcttgtatgtagaagatcaataaatgttcatcttcattgcttatattcatccggttctctgtatacaaaatgatcttctttttgcaggcatttttttgcttctcaagttttaacttcttacacattttaagactacttcaagattaatttgagtgtaaatgagcagtacttgttaggtaagtgtcttccattcaccgtcaagactgaatcattcttttcattatcaccacatattgcttattgtggaatttggaaacatccatttctcttcttcaggaagatcgtggagtttctccagtcaaggtcccactagagtgagttagggttgcagtaacctggagtgagcaatccctgattccaggtggtgatgtgggttgagtttcacattttactttatttgaagaatatgtgcaaaagactcactaaaaataagaacaaactaggctttgttgcagctgagtggtctggcaaatttctgtatagaggaatcattgggcatgaaggatttgatactgggatagaatccaattgcccttggaatggaagtagaatatcctttttaagagcactgaagttctgggatttctccggaataatcacctttgtgatgtgtggatcatgtccagggactgtaacatttattatataagacccaggcaagagaaggagataatactctccatatttgttggttctataggggcagatatgttttctgtcttggacttccacaattacattgggtaatggatttccattctgatcaaaaacttgaccctttacacctaggtgcacctgctttatatattcaattaatgaggctttgttattattccaaaaggatggaagcttctcctcacgaggatatttacagcatgacagctccaacgtaatttcaaaacactgggcccagatgtagttgtaatcttgcattccaccttggagtggataccaagagtatccatttgtaacaccattaggaaagttcattttgtttttacactcgtctcctttcttcatgttgggatttcttgaagcataggtatgtgcaagatattgaaaaacatcatcatcaggcgttaagcttcgggagtataatgccccagttgcttgaacaccattatcaaatgggtaactggccacgagggcaccaccatggaggtttgcagagaggacaaacgtctctgttttcagccacttcatgactgccacagtttcaggctgccttgagacattattatattcaaaagcatcggggaaatttcgattcaagtcatactggttataattttcccttccgatgctgtaataacagtcaggctttttgacggcttcaaatccatctgggttcatggaaggcatgatgtgtatccgggtactattgatcagatttgtgatttcagggtctttgccatcactggttacgagatagtcaatcagatggagcagcagctcccgcccaacagtctcatctccatgcatatttgccacgtatttgaactctggaatcccaattctgtgttcctttggaaaccgccccacaacaagaacccacaggtttctacctttcacagatttcccaatactgtgtaagtgagtgacagaactgtagttttgggcaacagtcttcaaaaacgcttccatcccttcctggcggtggtagttgaaatccagcgcagctaccaaaggcagcaacagccctagccagaggcacgggaagtccatgttcaggtcccaggcgcgcacctctacccaccc

SEQ ID NO: 14681 - RNA, 5246 nt, Homo sapiens
  source 1..5246: mol_type = other RNA
gctgggattacaggcatgagccaccgtgcctgactgctgctttctaaataccatttcactcccacatttttctcccatcatgaaagtgtgtatcaggttggtttctctataaaaggaattatagctgaactagagctggaggagcataaccaccagcccaagagggaggggaaaagccggaaaggcgttgggcagggaggtggcttgggtacctggtttgaccacagttagaatatcatgattgtgttttgttagtctttaaatgattttgagtctgatagataactaaattctgattttaaaaactatttcagcaagagatttacattaaggctcatgaactaattcagatttttgttcgtgtctcttcaaaaattgctatcttagaaaagttagaattcaatgcccagttgaaaaattgcttggggcttgatagcaaatcaagtttcatcttatatacttttaatttgtaatataccaaagtcatttttgcaatactatattatgtactttcaagtatataattactgcttctttaaatacaaatgatcaagatattcagattattatgagttttttttggttatcatctattgctgctgcacaaattaccagatttcataattggtttaaataagcctccaatttgtttatatttattaacatgtatgattttgtgcatgtagaataagcttggcatagaaatggcctaaatgctcctgtagctcttcattcctttgtcgttctcactctccatgccagtatgtctcatttctagatcccatagaactttcaattgaaagtaataaccaaggcaactcactttccatgagtaatacaccacacttctagaaatcagcctatattactgtcacactggggattaagtaaaaaaaagagaaagaaggatgggaaggggagggaaggggaggggagcggaggaaagaagaaaaggaagggaaggggagggaaagggagagaaggggaggagagggaaaggagggaggaaggtaggaagaggagaaggaaggaagaaaggaaagaaatctgctcaccagagttgctattttttttttcttttctgtttagtgctttaccccttaattcttataggtaacggtctaatacagggtaactctcatagtggagaacttgagaagcattagtacttcaaattgagtcctaatggtaaaatttttttctgataaaaaaaggtactttgtagtgctgttaggaggtaacataatacctttactaccaatcttaggatcaattcaaggttcagtaaaaggaatgtatctggaattcttgattatagacatgaaaacactcttctgtcagcgttcatagtgagctgggaggttgcctacgcattaagacctagcttcataaaatgactcaaagccctaggcagtttctgggaaggactgggagtagcagtctcctggcaccccttgttcattcattcattcagtacctactatgtgctaggctttgaggatataacaatgaatttttcaaacaaattaaatagaccttggcctcaaagagctcacattctactagagaaggcacacatggagaagattataatacaatgttgtaaatccaatagtagagataaccagtttattttggggagcaaagagaaagggtccctaaccccagactgcctgcgaagaggtgaaatggaattgaatgggattatggtcagccaaggcttcctagtggagctgctacctgaactgagttttaagaggggtaggaaagaaaaaatgtagtgggtcataatggcattccagatacaggggacacaaacagctctgtgtttatgaactacaaccagttgttgacttttgtttcaagtggctccccttccccagtgctgtgtggacgatggactgaagaggagaaggctgggagcaagggaccagtaagctgttgcagcagtgcaggtgagatatgaggcctcaactctgcagtgttgacaaccatagagagcagagagcagaattcatcaatatttatcagcaccaatttttttttttaagacagagtctcacttcttcacccaggctggagtacaatggcgcaatcccggctcactgcaacctctgcctcccaggttcaagcgattctcctgcctcagcctccccagtagctgggattacaggcatgcaccaccacgcccgactaattttttttttttttttagtagagatggggtttcaccatgttggccaggctggtcttgagctcctgacctcaagtgatccgcccgccttggcctcccaaaatgctgggattacaggcatgagccaccatgcctggccaacaccaacctttagttacttgctgaatacacaggattaaggaggaagagaaagtatcaaggatgactcccaggttcctagcttggtggtcccagtaattgagagagagaatgcagcaggaagagcagctctagggggaacaggatgagtatctccacatgatgggttggaggtacctgtgagtcacatccaggtggatgtgtcctgtgggcagtgggacgcgagtctgaagctcaggcaagaggctagagttacatctttggagtcatcagcctaatggaggactgtggcatccaggtgccaaaagctagggaaacggctctggagagagaggggctttcttaattgacctgtatgctttgaagctctatagagacacaatcttatcccttcaggcctgtattttcttgggccactaagatgtggttacatattttctctcacatctcctagaacgtttgcaaaacaattcccagtcctatgatcatttctcccttcttctgagaactaattatatatggcacttaatatctattcacatgtagcactcatggtgaggtgttttttttgtttgtttgtttttgtttttttttttttgagacagagtcttactctgttgcccaagctggagtacaatggcactatctcggctcactgcaaactccgcctctagggttcaagcgattctcctgtctcagcctcctgaaaggctgcgattacaggtgcccgccaccacaccccgctaatatttagtagagacagggtttcaccatgttggtcaggctggttttgaactcctaacctcagggtgatccgcccaccttggcctcccaaagtgctgggattacaaggtgtgagccactgctcctggccttatggtgaagtcttgtatgtagaagatcaataaatgttcatcttcattgcttatattcatccggttctctgtatacaaaatgatcttctttttgcaggcatttttttgcttctcaagttttaacttcttacacattttaagactacttcaagattaatttgagtgtaaatgagcagtacttgttaggtaagtgtcttccattcaccgtcaagactgaatcattcttttcattatcaccacatattgcttattgtggaatttggaaacatccatttctcttcttcaggaagatcgtggagtttctccagtcaaggtcccactagagtgagttagggttgcagtaacctggagtgagcaatccctgattccaggtggtgatgtgggttgagtttcacattttactttatttgaagaatatgtgcaaaagactcactaaaaataagaacaaactaggctttgttgcagctgagtggtctggcaaatttctgtatagaggaatcattgggcatgaaggatttgatactgggatagaatccaattgcccttggaatggaagtagaatatcctttttaagagcactgaagttctgggatttctccggaataatcacctttgtgatgtgtggatcatgtccagggactgtaacatttattatataagacccaggcaagagaaggagataatactctccatatttgttggttctataggggcagatatgttttctgtcttggacttccacaattacattgggtaatggatttccattctgatcaaaaacttgaccctttacacctaggtgcacctgctttatatattcaattaatgaggctttgttattattccaaaaggatggaagcttctcctcacgaggatatttacagcatgacagctccaacgtaatttcaaaacactgggcccagatgtagttgtaatcttgcattccaccttggagtggataccaagagtatccatttgtaacaccattaggaaagttcattttgtttttacactcgtctcctttcttcatgttgggatttcttgaagcataggtatgtgcaagatattgaaaaacatcatcatcaggcgttaagcttcgggagtataatgccccagttgcttgaacaccattatcaaatgggtaactggccacgagggcaccaccatggaggtttgcagagaggacaaacgtctctgttttcagccacttcatgactgccacagtttcaggctgccttgagacattattatattcaaaagcatcggggaaatttcgattcaagtcatactggttataattttcccttccgatgctgtaataacagtcaggctttttgacggcttcaaatccatctgggttcatggaaggcatgatgtgtatccgggtactattgatcagatttgtgatttcagggtctttgccatcactggttacgagatagtcaatcagatggagcagcagctcccgcccaacagtctcatctccatgcatatttgccacgtatttgaactctggaatcccaattctgtgttcctttggaaaccgccccacaacaagaacccacaggtttctacctttcacagatttcccaatactgtgtaagtgagtgacagaactgtagttttgggcaacagtcttcaaaaacgcttccatcccttcctggcggtggtagttgaaatccagcgcagctaccaaaggcagcaacagccctagccagaggcacgggaagtccatgttcttgtttgattgtaggtcataagacccccattccagaaagggtcctgtcccatacgcagaaggaagaaatgctgctcagagaggccaagaagaatctagacagacaggccttgctgggtttcctcactccatctgttaaagttacatcatacccttttgtccagtcatatttctaaacagctctacatactttttgaacctaagcataaaaatgtgcactttcctctgtcttcattctgaaggttcccatgtacacattaaatgcatttgtatgttatttctcctactagtctgccttttg

SEQ ID NO: 14682 - RNA, 4985 nt, Homo sapiens
  source 1..4985: mol_type = other RNA
gctgggattacaggcatgagccaccgtgcctgactgctgctttctaaataccatttcactcccacatttttctcccatcatgaaagtgtgtatcaggttggtttctctataaaaggaattatagctgaactagagctggaggagcataaccaccagcccaagagggaggggaaaagccggaaaggcgttgggcagggaggtggcttgggtacctggtttgaccacagttagaatatcatgattgtgttttgttagtctttaaatgattttgagtctgatagataactaaattctgattttaaaaactatttcagcaagagatttacattaaggctcatgaactaattcagatttttgttcgtgtctcttcaaaaattgctatcttagaaaagttagaattcaatgcccagttgaaaaattgcttggggcttgatagcaaatcaagtttcatcttatatacttttaatttgtaatataccaaagtcatttttgcaatactatattatgtactttcaagtatataattactgcttctttaaatacaaatgatcaagatattcagattattatgagttttttttggttatcatctattgctgctgcacaaattaccagatttcataattggtttaaataagcctccaatttgtttatatttattaacatgtatgattttgtgcatgtagaataagcttggcatagaaatggcctaaatgctcctgtagctcttcattcctttgtcgttctcactctccatgccagtatgtctcatttctagatcccatagaactttcaattgaaagtaataaccaaggcaactcactttccatgagtaatacaccacacttctagaaatcagcctatattactgtcacactggggattaagtaaaaaaaagagaaagaaggatgggaaggggagggaaggggaggggagcggaggaaagaagaaaaggaagggaaggggagggaaagggagagaaggggaggagagggaaaggagggaggaaggtaggaagaggagaaggaaggaagaaaggaaagaaatctgctcaccagagttgctattttttttttcttttctgtttagtgctttaccccttaattcttataggtaacggtctaatacagggtaactctcatagtggagaacttgagaagcattagtacttcaaattgagtcctaatggtaaaatttttttctgataaaaaaaggtactttgtagtgctgttaggaggtaacataatacctttactaccaatcttaggatcaattcaaggttcagtaaaaggaatgtatctggaattcttgattatagacatgaaaacactcttctgtcagcgttcatagtgagctgggaggttgcctacgcattaagacctagcttcataaaatgactcaaagccctaggcagtttctgggaaggactgggagtagcagtctcctggcaccccttgttcattcattcattcagtacctactatgtgctaggctttgaggatataacaatgaatttttcaaacaaattaaatagaccttggcctcaaagagctcacattctactagagaaggcacacatggagaagattataatacaatgttgtaaatccaatagtagagataaccagtttattttggggagcaaagagaaagggtccctaaccccagactgcctgcgaagaggtgaaatggaattgaatgggattatggtcagccaaggcttcctagtggagctgctacctgaactgagttttaagaggggtaggaaagaaaaaatgtagtgggtcataatggcattccagatacaggggacacaaacagctctgtgtttatgaactacaaccagttgttgacttttgtttcaagtggctccccttccccagtgctgtgtggacgatggactgaagaggagaaggctgggagcaagggaccagtaagctgttgcagcagtgcaggtgagatatgaggcctcaactctgcagtgttgacaaccatagagagcagagagcagaattcatcaatatttatcagcaccaatttttttttttaagacagagtctcacttcttcacccaggctggagtacaatggcgcaatcccggctcactgcaacctctgcctcccaggttcaagcgattctcctgcctcagcctccccagtagctgggattacaggcatgcaccaccacgcccgactaattttttttttttttttagtagagatggggtttcaccatgttggccaggctggtcttgagctcctgacctcaagtgatccgcccgccttggcctcccaaaatgctgggattacaggcatgagccaccatgcctggccaacaccaacctttagttacttgctgaatacacaggattaaggaggaagagaaagtatcaaggatgactcccaggttcctagcttggtggtcccagtaattgagagagagaatgcagcaggaagagcagctctagggggaacaggatgagtatctccacatgatgggttggaggtacctgtgagtcacatccaggtggatgtgtcctgtgggcagtgggacgcgagtctgaagctcaggcaagaggctagagttacatctttggagtcatcagcctaatggaggactgtggcatccaggtgccaaaagctagggaaacggctctggagagagaggggctttcttaattgacctgtatgctttgaagctctatagagacacaatcttatcccttcaggcctgtattttcttgggccactaagatgtggttacatattttctctcacatctcctagaacgtttgcaaaacaattcccagtcctatgatcatttctcccttcttctgagaactaattatatatggcacttaatatctattcacatgtagcactcatggtgaggtgttttttttgtttgtttgtttttgtttttttttttttgagacagagtcttactctgttgcccaagctggagtacaatggcactatctcggctcactgcaaactccgcctctagggttcaagcgattctcctgtctcagcctcctgaaaggctgcgattacaggtgcccgccaccacaccccgctaatatttagtagagacagggtttcaccatgttggtcaggctggttttgaactcctgacctcagggtgatccgcccaccttggcctcccaaagtgctgggattacaaggtgtgagccactgctcctggccttatggtgaagtcttgtatgtagaagatcaataaatgttcatcttcattgcttatattcatccggttctctgtatacaaaatgatcttctttttgcaggcatttttttgcttctcaagttttaacttcttacacattttaagactacttcaagattaatttgagtgtaaatgagcagtacttgttaggtaagtgtcttccattcaccgtcaagactgaatcattcttttcattatcaccacatattgcttattgtggaatttggaaacatccatttctcttcttcaggaagatcgtggagtttctccagtcaaggtcccactagagtgagttagggttgcagtaacctggagtgagcaatccctgattccaggtggtgatgtgggttgagtttcacattttactttatttgaagaatatgtgcaaaagactcactaaaaataagaacaaactaggctttgttgcagctgagtggtctggcaaatttctgtatagaggaatcattgggcatgaaggatttgatactgggatagaatccaattgcccttggaatggaagtagaatatcctttttaagagcactgaagttctgggatttctccggaataatcacctttgtgatgtgtggatcatgtccagggactgtaacatttattatataagacccaggcaagagaaggagataatactctccatatttgttggttctataggggcagatatgttttctgtcttggacttccacaattacattgggtaatggatttccattctgatcaaaaacttgaccctttacacctaggtgcacctgctttatatattcaattaatgaggctttgttattattccaaaaggatggaagcttctcctcacgaggatatttacagcatgacagctccaacgtaatttcaaaacactgggcccagatgtagttgtaatcttgcattccaccttggagtggataccaagagtatccatttgtaacaccattaggaaagttcattttgtttttacactcgtctcctttcttcatgttgggatttcttgaagcataggtatgtgcaagatattgaaaaacatcatcatcaggcgttaagcttcgggagtataatgccccagttgcttgaacaccattatcaaatgggtaactggccacgagggcaccaccatggaggtttgcagagaggacaaacgtctctgttttcagccacttcatgactgccacagtttcaggctgccttgagacattattatattcaaaagcatcggggaaatttcgattcaagtcatactggttataattttcccttccgatgctgtaataacagtcaggctttttgacggcttcaaatccatctgggttcatggaaggcatgatgtgtatccgggtactattgatcagatttgtgatttcagggtctttgccatcactggttacgagatagtcaatcagatggagcagcagctcccgcccaacagtctcatctccatgcatatttgccacgtatttgaactctggaatcccaattctgtgttcctttggaaaccgccccacaacaagaacccacaggtttctacctttcacagatttcccaatactgtgtaagtgagtgacagaactgtagttttgggcaacagtcttcaaaaacgcttccatcccttcctggcggtggtagttgaaatccagcgcagctaccaaaggcagcaacagccctagccagaggcacgggaagtccatgttctctacccacccgcggccgcccggcggggccgggtgttat

SEQ ID NO: 14683 - RNA, 1321 nt, Homo sapiens
  source 1..1321: mol_type = other RNA
gctgggattacaggcatgagccaccgtgcctggacagtgtcctttcaagcttctcatgcccttacttcctcctagacatggatgtggctcaagaatatcttttacccaagaggaaactttaactcggtcacagaacgccaggtttgggttgcagacgcttcttgtgggggagggaggtcttttcccctgtattcacagaagaggaggttgccaactggagatggttcatttccaagtttgtctggggtcccccagctatgcaggacccagaaagcagatgtctagacatccaggccaatggtctttcactactctgtgagtctcccgtgaacttcacctggaaccggtcctggcccagggctagctccttggtgagaaactcaaagaagtgggcgctgtggctgcggttgtcctcggcggtgcccactacgccgatggaggagatggacagctgcgcgcagggctcggtggacccgctcagcgccatggccaggcccggccgtaccgtcacgttcacgcggtccgcaggtttgcccaggatggaggcagcggcggcgcagagtcgtttctccagccccgcgggcactcggttggcgggcaaattcgtgtccagctccaggaacggcatggcgggcagaggaacggaaacagctctggcggaagaaaagctgggggtacccaaggctcgcggaccagggaggaggggcgaggcgccacagcaacctggcttctcattggctggacagagactcggcgctccccgattggctgcctagggtacctcccgcttctgcaaacaaaagtcacgtgtgccggctgatttccggaagtcccatcgtctccgccctacgtgtagccccacccactacaggtctttaacccggtagtggacccaccctgtctcccccgaccctcctgcctggcgccaggtgggtttccctctcaagcttccgcgctgtggtcgcccggttcctagccctattagaggtctgaacaccacacccccgacacacaaggacacacacacacctataggggtcttccccaggctcgaccctaataaccaatacaacgggagcttaaagtttttttgaatgatttgccaccatttcgaagtcaggcaatttcatgttcagtatggaaatctgcgcttgggcagtcaggagatgtggttactcgcgggggcgcgggtagggctaggctcacgacaatacctgtccctgcctggtccccattgacatctgcctgtgtagcctcttgtgccggtggtgagccactgtccaccagggggtggcaaaatatgttctttaaaacatggaaa

SEQ ID NO: 14684 - RNA, 956 nt, Homo sapiens
  source 1..956: mol_type = other RNA
gctgggattacaggcatgagccaccgtgcctggccaaaatcttctttttatatcaataaatgtccaaaggagagtaatttaaaattcttactgtttatttatatattgcatagctcaaaaagtttgaaaaaatgaagttttaacaggaagtcagtaaatgctcatagacccccttgtctctagcacttggagtccttagagatgggaatcttgacagcagaatttcagatgtttcaatcacttgccaaggaagtgccacacttgctcttcttcattactttctttatttggtgaagatgataccgattcaactaatgatcttgcttcctcttgagtgcaacggaaagggctatcagatatctgcacgtttgtgcaatttatagctcctccattacacttcttcataagcaatgctttccaacattgatgagtggatttaataacttcaagagcaaaagccttgtttttgaattctccattaaaagcaaactggttttctggttttccatctggtaccttatataatctaaaccaattaagagtagcttccaggtaacccggtttgaacttcttaacatcatcaatatcatgaaactttgaggcttcaggatcattcgcattgatagcaattaatttccaatctgtttcaccttcatcaataagagccaaaattccaaggatcttcacatgaataacttctccacaagaaagaatctctttagagttcaccttcagaggaatatcatgaaagggggaaatgtagtgaccagttacattcttaaagaagaggcggtaattctgcgagcagggctggccgcgctcctcagtgtggtacagggccatagcacggcgcgacccggtccctgcactggtccccaaccgcaggcacgcagcggctggggcacccgtgcgcagcagccgcagcagcgcgctcatggcgtcaatgacggtcctgc

SEQ ID NO: 14685 - RNA, 1175 nt, Homo sapiens
  source 1..1175: mol_type = other RNA
gctgggattacaggcatgagccaccgtgcctggccaaaatcttctttttatatcaataaatgtccaaaggagagtaatttaaaattcttactgtttatttatatattgcatagctcaaaaagtttgaaaaaatgaagttttaacaggaagtcagtaaatgctcatagacccccttgtctctagcacttggagtccttagagatgggaatcttgacagcagaatttcagatgtttcaatcacttgccaaggaagtgccacacttgctcttcttcattactttctttatttggtgaagatgataccgattcaactaatgatcttgcttcctcttgagtgcaacggaaagggctatcagatatctgcacgtttgtgcaatttatagctcctccattacacttcttcataagcaatgctttccaacattgatgagtggatttaataacttcaagagcaaaagccttgtttttgaattctccattaaaagcaaactggttttctggttttccatctggtaccttatataatctaaaccaattaagagtagcttccaggtaacccggtttgaacttcttaacatcatcaatatcatgaaactttgaggcttcaggatcattcgcattgatagcaattaatttccaatctgtttcaccttcatcaataagagccaaaattccaaggatcttcacatgaataacttctccacaagaaagaatctgagggagggtaccataattccatatataacccttgtaagggaagatattcgccacatagcgtagctttccatcctttacatattgtttaatgggattcattggctccttggtggcaatctccattttagcatttgtccaccgaggtatttctacaatcatattaaacagattctcatattcatcatttcgtgctttcttcataggaatgccattttcctctttagagttcaccttcagaggaatatcatgaaagggggaaatgtagtgaccagttacattcttaaagaagaggcggtaattctgcgagcagggctggccgcgctcctcagtgtggtacagggccatagcacggcgcgacccggtccctgcactggtccccaaccgcaggcacgcagcggctggggcacccgtgcgcagcagccgcagcagcgcgctcatggcgtcaatgacggtcctgc

SEQ ID NO: 14686 - RNA, 1254 nt, Homo sapiens
  source 1..1254: mol_type = other RNA
gctgggattacaggcatgagccaccgtgcctggccaaaatcttctttttatatcaataaatgtccaaaggagagtaatttaaaattcttactgtttatttatatattgcatagctcaaaaagtttgaaaaaatgaagttttaacaggaagtcagtaaatgctcatagacccccttgtctctagcacttggagtccttagagatgggaatcttgacagcagaatttcagatgtttcaatcacttgccaaggaagtgccacacttgctcttcttcattactttctttatttggtgaagatgataccgattcaactaatgatcttgcttcctcttgagtgcaacggaaagggctatcagatatctgcacgtttgtgcaatttatagctcctccattacacttcttcataagcaatgctttccaacattgatgagtggatttaataacttcaagagcaaaagccttgtttttgaattctccattaaaagcaaactggttttctggttttccatctggtaccttatataatctaaaccaattaagagtagcttccaggtaacccggtttgaacttcttaacatcatcaatatcatgaaactttgaggcttcaggatcattcgcattgatagcaattaatttccaatctgtttcaccttcatcaataagagccaaaattccaaggatcttcacatgaataacttctccacaagaaagaatctttgagcctatttcgcaaacatcaataggatcattatctccaaagcagttcgtgctcttatctttttcatggggatcttcccaagtctgagggagggtaccataattccatatataacccttgtaagggaagatattcgccacatagcgtagctttccatcctttacatattgtttaatgggattcattggctccttggtggcaatctccattttagcatttgtccaccgaggtatttctacaatcatattaaacagattctcatattcatcatttcgtgctttcttcataggaatgccattttcctctttagagttcaccttcagaggaatatcatgaaagggggaaatgtagtgaccagttacattcttaaagaagaggcggtaattctgcgagcagggctggccgcgctcctcagtgtggtacagggccatagcacggcgcgacccggtccctgcactggtccccaaccgcaggcacgcagcggctggggcacccgtgcgcagcagccgcagcagcgcgctcatggcgtcaatgac

SEQ ID NO: 14687 - RNA, 764 nt, Homo sapiens
  source 1..764: mol_type = other RNA
gctgggattacaggcatgagccaccgtgcctggccaaaatcttctttttatatcaataaatgtccaaaggagagtaatttaaaattcttactgtttatttatatattgcatagctcaaaaagtttgaaaaaatgaagttttaacaggaagtcagtaaatgctcatagacccccttgtctctagcacttggagtccttagagatgggaatcttgacagcagaatttcagatgtttcaatcacttgccaaggaagtgccacacttgctcttcttcattactttctttatttggtgaagatgataccgattcaactaatgatcttgcttcctcttgagtgcaacggaaagggctatcagatatctgcacgtttgtgcaatttatagctcctccattacacttcttcataagcaatgctttccaacattgatgagtggatttaataacttcaagagcaaaagccttgtttttgaattctccattaaaagcaaactggttttctggttttccatctggtaccttatataatctaaaccaattaagagtagcttccaggtaacccggtttgaacttcttaacatcatcaatattaaagaagaggcggtaattctgcgagcagggctggccgcgctcctcagtgtggtacagggccatagcacggcgcgacccggtccctgcactggtccccaaccgcaggcacgcagcggctggggcacccgtgcgcagcagccgcagcagcgcgctcatggcgtcaatgacggtcctgc

SEQ ID NO: 14688 - RNA, 560 nt, Homo sapiens
  source 1..560: mol_type = other RNA
gctgggattacaggcatgagccaccgtgcctggccaagattttatttttagtttacaattggaaggctagtgggccggtgcagaatctcgctgacttttgggtgagcatgttgagggccccctgcgtcagctgctcttctgttgaacggtgcagggtggggaggcctgggctgcactggccacacagtcccctcaagaagatcttctacgtgaaacaaaggagcactgagcgaggggagctctgctcagaaaggaccatcttgcatcactggtacggcccggcccgcgggtccctccgggtcaggacgcagacgcgcccgcggcggtaaccgggggcccgggggcctcgggcccaccccggccagaccccggggaggagcgcaggacactgcccgcgccgggactcggctgtttccgatcctcccgggcgtcctttaggagactcattcgcagccgacgttgcggaggcgcaggaaaagggcgagcaggtgcctcagggacaccacttccaaccgcacgccgatcgccggctccaccataaatagaaacgggtggtctct

SEQ ID NO: 14689 - RNA, 2658 nt, Homo sapiens
  source 1..2658: mol_type = other RNA
gctgggattacaggcatgagccaccgtgcctggccaccccaggaatatttgataacatcaacatcaaatcattcctgcctgccctcatgcagggacttctcacttagaaagttctatagacccaatgggcaggacaggaagatagagaagaaaacaccatctttaatcaacccgcctgcacagaaaccaggagagcactcccctccttgcaaggtcccagtgaaaagagaacctggtccccttgcaaaaaccatcttataaaaacaaaaggcttcaaagcaccagtggctacacccgttgagtagaaaggggcttgggggagagttggggtgagagaggtgagggctggaggcagggctggcccagtgaagggcagtagcttagcctgagggagctgcccccctctcaagctgtacccaccagctgggagctccatgcctgtgggggccagaggaactcctgggcctggctgcttgcatttgggatggtggggtggggttgccagccttgctcaggatattttggccttagagagtagggaatgatagattggagggtagtgggagaggagcggaatggtcaccacagacaggctcaggtgtgcaaaccatctgcaccatctgggtgccccccagttcctccatgtctcctgccctcctttctaacccagggccatgcctctttcacagatgaaatgctgagacctgatcctctctctatggacgcaccaggcagtgcgtgggatgcagcgtcctcaggagtgtctgtggagggaggtggggaaagtgttctcacctctacttgcccccaaggaagggtgagggtgctggcaatcccgactccccgactactcacacccccatctgccccttcagaactccttctgggcttgttagaggaggcttctggccattggattggttgtaaatgctggtgatctgtaaacactggagtctgggcagcgctgaccagcattgctcctctctgaaaccacaagccttccaactggtgaggtggatggagccgtcaggggtgagtggagttgtggaggtgatggggatacagtagaaccagcctcagggacctggaagggggtggagtgactgagttggggccccactttcctggaggagagagcttgaaagatttgccaagggtggacagaggctgagtgtaggaaggcttctctgtgggtggggctgaatttggggcttcatccatccagttcccaataagagaacgaatgggtatattgctttaagagaggcattggcaagtggtggtggtggtgtgtgaatatggtggagaccacataggtccaagatggaggggggcttggaaatggaactcagagagcagacactgggttttacagtcagaaactgcagaaagtacactgtgttcaaggcccacttccaccaaaaatctagctgtgtggcctcaagcaaatcacatctctgggcctcagttttaatgtactgcaaaatgagaattttaatcccagtctagctcagggaattgagttaaatgagaagtctaaaagagtccatttgctaagggattaattacttgaggtgcggaaaccgaggctcagagagggcaagggctttgctagacgtcacagtcagtgatggacctgcgattagaacccaggaatcctgctcctagttcacagtagctttccccagagctggtgagtgagtgtggtgggatgggatgggtctgatgtcctgctgtttttggacaggggggcaggatgctgggtgaagagtgaaagggagaggctggagaagagaggaaggccccagctcacgccaaggctgagattaaaaacaaacaaacaaaaaacaaaaaacccgtggtgcccctcccccgccccgccccactcctccgaagtccgggctgcgaagagccaagctcaaatccaagtccaagtccaagtccacgtccaagtccgcatctccagatgcagacgcggggttgggcacaggctgcagtgagcgcgcgggccaccagggggacacgcctgcgccttggcccgagctcgcggcagctgcggtcagcccagggcgaggcgccggggtgggcgcggggcagaggctaccccgacgtgtacagaggctgcagctgtaaatgcgacgtcttctggggcgcctggtatccgtaggagtcaaagccgccgatgaagtcaaagctgtcctcctcctccaggaacactttgctcacgtagcaggcgaacacgaagccgaacagtgccaggaagatctgcagggcgctgctgagggcttcaatgtaggggtagtcaagcaggcagccagtgacagagatgacatggtggtcctccagagccaggcgggagttcagaacaggtgtcaccaggcagcctggcccattctccatccaccaggagcggtgcagggatgtgttgaaggtcatgatgaagtcccggtccaggatgaggtaccgggagcggtactgcacggtgccaaagatgcccaggatgactgccatgatgtgcaggaagttggctaggatgggagcccactggtagcccaggaagtcaaagatctgccgctccagcgcagccaccagctgcaggcagcagaaggcgaccagcgtgcagcgcccgctgcacttgcccatggctccgggggctgc

SEQ ID NO: 14690 - RNA, 104 nt, Homo sapiens
  source 1..104: mol_type = other RNA
gctgggattacaggcatgagccaccgtgcctggccacgtccctattttagaaatgagaggagtgactgcacataggaaaaatgccacttttagcaattcaaagt

SEQ ID NO: 14691 - RNA, 1628 nt, Homo sapiens
  source 1..1628: mol_type = other RNA
gctgggattacaggcatgagccaccgtgcctggccacgtccctattttagaaatgagaggagtgactgcacataggaaaaatgccacttttagcaattcaaagtggaaaaacttcttttatataaaaattatcccaactcccaccccttggctctcagtgttgcatctcccacagaggtaaagttgtgccattttcccacggctttaaacaaagcaaaacaaaaccaccaatcctaataacccccctccttgccccgtctccacgctgtgcggagagggctctagcccctcagtcggacttctccttctccttcatgtgcaagaagacgatgctgaagatgaagagccccagcatcatggagaaggcgctggcgtagtaggggtaggccgaggggatgaagcgctcatactgcgtgtgctggagtggccgcacggatacctgagtggaagagtacaggtgtgtgtagcctagccggttgtaatccactttaaactggaatacaccatacacgtcgggcaacttgaactgaacactgtatttgccacctttcttcttcaggaaggtcctcacaaaaggatcaatgcggacaaactccagctgaatgtcatcgccatcaaaggggacccatttgccatttgagagctgctggatcacgatgctatactccactaggtcagtgacagtgtaggcattgggtggggctgtctcgcccacccgatgatgggacacaggccccacacggaggacaccctcctccttgaacacccagcgggagagggccacagctagttcatagttgcctgtctgggaatacctctgggagccgggcgccgccttctgcactgctgagttgaagaaggagtcgctgaagaagtcgagggagccgctgaagatgacgcgggcattgttcctggcctggagcccagcaatgaggagggtgttcttccccaccgcatgtggatactgggtgataggcttgtccgggaagaaggagtaagaggtggaagagcccgtcaggatgtccagcaccaaagggttatcaggatcggccaccatcccaacacctcgaaagaggatgggatttagagatgatttcccaacgatggttggggccttcagcaggttctcagtgtcagccacgatgagcgtatgctggccaaggtctgagatgtcatagttgtgatggtcaatgacagccgttttctcctcgtcaaactcaatcccgcactcactgcccagctctcgaagagggtcaccaatgtcggagctggcagctaccagcacactgcctccgccgtcaataaaggcactgatggtctccacgttgatgttgcctccaaaatcttctaccgaaggggagaaaatgatgagattgtcatagaggaattccccatactttatgagagacaggctggggtcatcagcggtcttgaatgtgagctcaaagccccggtccttcaggctccggaagaaaagcgaatgagtctcccgcacgttgaggttgtccagcagcactaaggtgcggggtccgctggcgcaaaccgcgccaagcaagggcagcagcaaccaaaagagggcccaagcccgggccgcggtgctgggctccatcttcctcctcctgccgaag

SEQ ID NO: 14692 - RNA, 3090 nt, Homo sapiens
  source 1..3090: mol_type = other RNA
gctgggattacaggcatgagccaccgtgcctggccatcctttatttgtgggggcaggagggaaggtctccctctgttgcccaagctggagtgcagtggtgagatctcagctcactgcaatgtccacctcccaggttcaatcgattcccgtgcctcagcctcccaagtagctgggataacaagcgtgggccaccatggctggctaatttttctatttttagtagagacggagtttcaccatgttgcacaggctggcctcgaactcctggtctcaagtgatccacccacctcagcctctcaaagtgctgagattacaggtgtgagtcaccgcgcccagcctattccatccttatctcagaagggcttactcttcaatgctaggcggtcacctgctctacagactagagggtccaagagcgactgtcattcaaacgctttagcagaagtagccaaggcgggtacctgagcttgtctgcaatgaagatgaccctcctctccagaagcagggaggcaaacacacagaccaggtggcggacgctgagggaggagaagagagactcaaagtccacgtgctcgagccgggagtccagcgggcggcacagttcgatcacctcagttcctgaacctggcaggaagttcttgacaaggatggttttgcccagggctgggaaaggggcttccatgacacttctcatgagtggctgaaccagggcaggagagatgcctcgtcttttttccacctcatccaagatccttgaaaagaggctgaagcatcccaggcggctcacaatgcagtaaacttcaggaaggcgcttccctttgcctccaggcagcagtcttcggcagtaaccgaaccttctgctcccatcttctccagttaagacaaatgagaatgtttcactggtgaactgctggacaggaacccaatccttggcatcgggaaaacagaactggggaatggccttcagttggtcctcagcttctctcatgaacttgaaagacctttccaacttcagagggaactgttgggtgagttctggcacgtaggcagccccggcctgcttcttgtgcaaagacacaaccacaaagtactcgaagagctgcctctcctggtactcgatgagttcccgggcaagtgatgggtaccgaggcgcctgcttcagccgggacttcacgttgaccaggcgctggctgtgagctttcagcttctcctctgtgtcactgtcagactcactgttctcatctgtcacttttcctgagttgctctccattgactgggacagcctcttcacccgtttctttcctctccggacctcataaatggcgttgattcgcaacaccagcttgggtatctttctcttcttcctgccgttctgtgggtctccaaggttaaagaaaatgtcatcagggctgctgggagtggagggagggctgattttggaaggggacccagttccatcccgactcagcttcctagtgtccagcagcttgaagttcctcctctctgaattttgtcggaaaaaagcaggtttggacaatgactgcttggtgagtgtgtcagggatggaagaggtgggagaagcaggaaaattcaagacacacttctttcccaggcagcgaccatgtaactcgatgtcctcataagggttctccttcattggcggatctagaatgtcttcatagacgttctcctccgataaagtgcgtgtcagccccagcttagtctgcgcgtaccagtccaccctgctgctctcagaggaagactgcagtaaatcttcaaactcataggactttctgtggtctgcactggatttctgtctcccggtccacagtcttctgttcacagaggaaggtgggggagaggagggcagaggcgggggaggtagagagggcagaggaggcagatttcttttctctttcctgaagccgatgccaggcttcccatctttgtccccttctccggcatgtttgaacgttctccggggttttggcagagggttgatgaagggctttgtgggggaaccctccgagcccctatacacgttctcaaggctccggtcccagggccttctgcatgaacctttcctgtcctccacaagctcaggggtgggctccctgccttccaggtccgaggggtggaccctctggctgacttctgagccactcccgcctcccaggttctcaggaagggtggaccctgcctctgccttgtcaggagggcagtgtggggagtaacaagtccctggtaactggggatccagccctgccgacccatccttcaaagcctgctcgagtttcttgacctgcttcagcacggagaggggatcgttctgaaagcgtagcttgccaagtcttggctctcggcctcggccccagctaggatccacttcccgttctggctggcttaggtcttgccccggctctgggtcctgtcccccgacgttcactgctcctttattcctctccttctctgtgctctctgttcctggcctcattccattcttagcctctgtgacctgagttctcaccccatcactactcctcctctccaccgtagaggacggcagataatcctcctgtccgtctgctctcctgctgggtgcaggagtgggcacctctttcttcccttcccattctgatatcttgtcctttatgttgagggacttgtgccggggtctggctctggcagatgggcaagggttctgaacacctctgagctgcttcttcccagccctgctggcttctgcagctgggtcactgatgatcatatccaagctgaacatatccattcttgactctagcgtgaggttgtggaggccttccaggggactccttctgaagcctgactcctgatcagtctctaggaatggaatggaggactaaagtggatgccttcgagggtctttctcagtccttggaccttccaccttgaccttgtcagccaatttgtagctcaggttttcagtctggctgtggctgcccttggccggcctgcacactgtcatcatgtcagtaccgaggggagttccaggtcacgcaggacaccgtcaaggaacacaggctgcacagcagaagtccgcagggaaatgcc

SEQ ID NO: 14693 - RNA, 11293 nt, Homo sapiens
  source 1..11293: mol_type = other RNA
gctgggattacaggcatgagccaccgtgcctggccatggcttctgtgtttcatttaacgctttgaaagccccatcttctcaaagattatatgaaaagcttattccagtttttaaaatatttgatacaagggtaatgtactttggtataaggagtgaggtatagatccagctttatatttttctttttttttttgagacggagtcttgccttgtcacccaggctggagtgcagtggcgcgatctcggctcactgcaatctccgcctcccgggttcatgccactctcctgcctcagtagctgggactacaggcgcccgccaccaagcccggctaattttttatatgtttagtagagacggggtttcaccacgttaaccaggatggtctcgatctcctgacctcaggatccgcccgcctcggcctcccaaagtgctgggatttcaggcgtgagccaccgcgcgcagcccagctttacatttttcagactggcctaccatgtctttgtcagacattgccatttacctacctagcatccattcttcctaacagatccctgacttcactcagggctgggatgtcccagcttaaaatactttccccaactctcttacagcaagggatggctatgtgattcagttctgtcccatgagacatggatggaagccactaagtggggcttccagagattttaaataaggacacctttgactgacatgctccatttggtctcttaagcttcatcttcttcctgcttgaaatgtagatgtaatacttagaggtgaaataacttttctgagacaatgaggatgaaagccactcaccaaagatggcagaatagagcaataaatggaccttgagttcttaataacactgttaaactgccatatcagttatggattatgtaaccttggatttattacgtgaaaaaataaactcacagtgaagctagtaatcacaggaatttttgtttcttgcaaccaaatatgttcctatctgatacagtatccccacttatttaatattccatctttttataccaatttgacatgctaccttcatcaccttcccatgtataattaattgggtataattctggaaaccctcctgtttcattgacctaaatgacttaaatttttaatagctaatataataacagccaatgtttgttgaatgccaaaactattctgtttattacattaattatctagttcatttaaccctcacaacagcgcttggagccttatttttttatttttttttgagacgaagttttgctcttcttgcccaggctggagtgcaatggtgacatctcagctcaccacactctccacctcccaggttcaagcgattctcctgtctcagcctccagagtagctgggattacaggcacgcgacaccacgcccagctaattttgtatttttagtagagatggggtttctccatgttggtcaggctggtctcaaactcccaacctcaggtgatctgccagcctctgcctcccaaagagctgggattacaggcgtaagccaccgcacctggccaaggaattctaaagctgttttaaaagactgcatttcagtatgcatccctaaacactatagcttaattttgcctgtgtttgaacttcatataaatgaagtaatacagtacaaattctttgtctttttcactcaacataatacttgtgaaattcttcatgtttttgtatgcggctttagttcatttattttcattgctgcataagattccattgtgtaattataccaacttgtctattctgtgttgatggacatgttcccgtttttggctatttgaataatgttaactgtgcacattcttgtacatatgtctcttatggtacatgtacatgcatttcggttgaatatatgtcaagagtataattgcatatcttggcctttagtattaaaagcacgtttctggctgggcgcagtggttcatgcctataatcccagcactttgggaggccaaggcgggcagatcacctgaggttagcagttcgagaccaacatggtgaaatcccgtctctactaaaaatacaaaaattagccgagtgtggcagtgggtgcctgtaatcccagctactcgggaggctgaggcaggagaatcgcttgaacccagaaggcagaggttgcagtgagccaagatcgcgccactgcactccagcctggcaacagagcaagactttgtctaataaaataaaataaagcacatttctgataccgtatttctactcaaaagctctgacaggctgggcacagtgtctcacgcctgtaatcccagcactttgggaggttgaggtgggcagatcaccggaggttgggagttcaagacccgcttggcctacatggagaaaccgtctttactaaaaacaaaaaaattagccgggtgtggtgatgggcacctgtaatcccagctacttgggaggctgaggcaggagaatcacttgaacctgggaggcagaggttgcagtgagccgagattgcaccactgcactccagcctcagcgagacagcgagactccatctcaacaaaaaagctctgacaaagaaagaatggcctagaatgtcaggtatggtgctgacatacctgttcaatttcattaaccactaaacttcaaactggttttctttttatatttttaaatttttttccccaagcaaactcacaaactgcgattctatctgaaagagtcttccctaccttctttgcctagttaacttttatttttccctaagatttcagcttaagcatcgttgcttcaaggaaggcttcttttatatacttgcttaccaccacaggcctctttttctcatttcttgaaatagttttacaatttgtgaaattaattggctgagtccccagcaaaataagctcattaaagtcagggtgtgtgtatattggggggggcggtctttttttttgagacagagtctcgctctgtcacccaggcgggagtgcagtggcgcgatctctgcttactgcaagctccgcctcccgggttcacaccattctcctgccgcagcctcccaagcagctgggactacaggcgcctgctaccacgcccggctaaattttgtatttttagtagagacggggtttcaccgtgttagccaggatggtctcgatcccctgacctcgtgatccacccgcctcggtctcccaaagtgctgggattgcaggcgtgagccaccgcgcccggcctattgggggtcttttttgcattatcactgtatccctacactcagcacagtactaggttcatacaggaaggggttaataaatatgtgattaatatctattgtcccttcacattcagggtgccaaattcaaaggctgtttcttctcaatgttttattattcaggccaccactagcacaatcctttgaaaataattttttttttttttttttttttttttttttttgagacggattctcgctctgtcgcccaggctggagtgcagtggcgcgatctcggctcactgcaacctccgcctcccgggtacacgccattctcctgcctcagcctcccgagtagctgagactacaggcgcccgctgccacgcccggctaatttttggtatttttagtagagtcagggtttcaccgtgttagccaggatggtctcgatctcctgacctcgtggtccgcccacctcggcctcccaaagtgctgggattacaggcgtgagccaccgcgcctggccgaaaatagatttttataaggtaaaagattttattaagtaccatttggtaaaaaaagattgaatgaggaatttagtacctaggcccatcatcataaacgtgagtatttttactgttttccatgaagagactataattatcacatgaagtaattctccataaggattacaaaacatatgagttgtttcattattaaatggtgcttactattaaaaagatactttacatggagaactaattccaccaaagtgagtaggtataaaatagagcaaaaatattgaacttaatcatttattcttcaacaagtgcttattatgcaaatagcagcaatctgcttttacattatctttttccctttatcaccagatgagaaatttctccccattatcattttgtgtaatttcacttgttcttgtgtaaatacttctgtttggtttttaataaaaattgctcagtggcaaatattacagaaaaaccaaggtttttattcttgataatttactgatagtctagtgttaacaaaattattacaggtgggaatgcttccttttttcgtaagtattaacaacttgtatatacactaattacaacttcaaaatattttacacaaatattctttttcatattagtatctaacttaattatctcagcaacagcattagtatagcatggactactataaaccaaacatcttcaaagtaaaaacttgcaaatatcttgctgaaaatagaaaagttgaaaccaagatactgccaatataaaaatgtaaagcagggaaatgttttaccactgccatcttccctatattctttctctaatgtaacctccaaactgtaacctcagcatatcaaaagaattttcaaagagaaaactaatcctaaatttcatgtttaataacatatgccttgtatagggaacattctcttaaccattttttaatcactacaacccagaaagacatggtttggtctaaaattttcaccagtttgttataaataaaatgtattcataagtagaactttcttcagaatgtattttttttaagagacaaggtcttacttactatgttgcccaggctggagtgcagtggttattcacaggcacgatcccacaaccgatcagcatgggagtttttatgtattgtagtgcaaaaatgtaggaatgtctagcttttttgatgtcaaagttgtaatttagggatttacttgaagagtgtcaagagattctcaaacacacaaaatgctgctaggaaattacagttgaaccttgaacaccacaaatttgaatagtgcgggtcaacttacatgcaatttttactttttttttcttttctgagacagggtctcactctgtcgcccaggctggcatgcagtggtgtgatcgcggctcactgcagcctcaacctcccaggctcaagcaattctcctgcctcacagcctcctgagtagctgggaccacaggcaggtgccacatgcccagctaatttttcttttgtagagatggggtctcactacgtcgaccaggctgattttgaactcctggccacaaaacagtcctcccgcctcagccttccaaagtgctgggattacaggtatgatactgtacccaggcatacaaacaatttttttttcccaaacaaactaggattgaaaatacagtactgtcaggatgcaaaacccatataaatgataggcctactttttgtatacttggattctgcagggaagactgtgagacttgagtatgggtggaatttggtatgcagtggttctggtaccaatccccttcgtatatagaggaacagctgtacacaaatgaggaatgaagcacttctaattcagggtattttctaaattaaagtattattatgattttttcagaggcaggatctcgctatcttgcccaggctggtctacaactcctgggttcaagcaatcctcctgccatggcctcccaaagttctgggattacaggcatgagccaccatgcctggctgtaattcaatttttaaagggaaatttaaaaatagtataaggctcaaaggttcaattaaagaaaccatttatgaaggagaataataaaatattactttgtgtacatatgtcagtgcagagaattgggtaagggtgatttttagctctgttaagacttgcttcagaatgccataccacagtctgaaagaatcatatgaaagtaagatattattttaaaaacaaaagtgccgggcacggtggcttaagcctgtaatcccagcactttgggaggccaaggtgggtggatcacctgaggtcaggagtttaagaccagcctggccaacatggtgaaaccctgtctccattaaaaatttaaaaaattagctgggcgtggtggcgggcaccggtaatcctagctattagggaggctgagacatgagaattgcttgaacccaggaatcagaggttgcagtgagctgagattgcgccacacactccagcctgggcgagagagcaagactccgtctccaaaaaaaaaaaaaaaaaaaaaaaaagggtcacaattccctaaagcctaaaactggataaaatgtgcactaacaaaaatgaatatttagaagtattcaactagttttgttcactatgaaaaataattttaagttgtagaagcattatttcattcaacattttgttacatcacaaaatttttaaatgactaaattttaaacaatatttaaacaaaaatatttacttcacattttaattcaatgcaaattttcactaatttagaagtctatgttaatacagattgagtataccctttccaaaatgcttgggaccagagtttctcaggtttcagactttttcagattttggaatatgtgcagaaatacagtggttgagttttcctaatccaaaaatctgaaatgcaaaatgctccaatgaacatttcctttaaagtgtcacatcggcactcaaaaatgttcttatctgaagcattctgaattttggattggggtgctcaatggctgtatgagtatttggggaattcctggaaatggacacattattacatataaaactgtcttacagaccttagaaataaggttttacaatggttcataagctttacaaatcttcctaaactactttttaaaaaacaatgcttaattatatagattttgattttttttttttttttttttgagacggagtctcactctgtcacctaggctggagtgcagtggcacgatcttggctcactgcaacctctgcctcccgggttcaagcgattctcctgcctcagcctcccaagtagctgggactacaggcgcccgccaccatgcccggctaatttattgtatttttagtagagacggggtttcaccatggtcttgatctcctgatctcgtgatccacccgcctcggcctcccaaagtgctgggattacaggcgtgagccaccgcgcccggcccagttctgtttttttgttttgttttgttttgtattttgtgtttttcttgagatggagtttcactcctgttgcccaggctggagtgcaatggcgcgatctcagctcaccgcaacctctgcctcctgggttcaagcaattctcctgtctcagcttccccagtagctgagattacaggtatgcaccaccatgcctggctaattttgtattcttagtagagatggggtttctccacattggtcaggctggtctcaaactcccaacctcaggtgatccacctgcctcggcctcccaaactgctgggattacaggcgtaagccaccatgcccagcctgttttaaaaattctaatgaactggcctggtgcggtggctgacacctgtaatcccggcactttgggaggctgaggcgggcggatcacgaggtcaggagatcgagaccatcctggttaacacggtgaaaccccatctctactaaaaatacaaaaaattagccaggcatggtggtgggcgcctgtagtcccagctactcgtgaggctgaggcagaagaatggtgcaaacccgggaggcagagcttgcagtgagccgagatcgtgccattgcactccagcttgggtgacagagtgactctgtctcaaacaacaacaacaaaattctaattaataattagattggaaatcattatttaaaaaattagttatgactcagaaaatattattatataaaaattcaaggagaggacattattagggtcatcttaccattattagccatagcagtactgtgtcttgcacacatctacaaatcatggttttttttttttttttttttttttttgagagagtcttgctctgttacccaggctggagtgcaatggcacaatcttggctcactgcaacctccacctccaagggttcaagcgattctccctgcctcagcctcctgagtagctgggattatacaggcgcctgccaccacgcccggctaatttttgtatttttagtagagacggggtttcgccatgttggccaggctggtctcaaactcctgactcaagctgctcatccactttggcctcccaaagtgctgggattacaggcgtgagccactgtgcctggcctacaaatcctgtttttaaactgacaatctgttctaactactttgctcattagcacacgaaaatgatactggttgagttcgaaacattgtaatttgtatttatagaaaccctaagtaagatagttcccaagattaaatgctattttaaaatactttttggaacaaaaatacctcattttatcttatatcattaggagtaaacatgatccatataagtgatttttaaaattcataccttaaagcaatgatagtttttaaaaattaaaccattttttaatagaggtgatcttaaaataccttcatttattgccttgtaaaattctacctcctggtcctgacccccaagctttctgtgaaagattccagggtcaacactatgaatgtcaaatattataatccattataacaaagtattaacctcagcaatttcttaagtgtaacaaatgtttatcttacggttgctgcttctgtaggcatagatatttcctgattacttcatattattctaacttctagaagtcctgtccctctggtgcttctcacctgtttttaaaaaaatcagtacatgtaattttctacattattctagctcaaaagtgctccacactttttctgcagcttaaaataagtttttctttctttccttttgggattaggggaaaggaagacggctgggcttgataacacactcatttgtaggtttgcttcagaggtgctggatatttcctgatgggtaagtttgctaaagaaatacataccaagaggtcgccatgttatcatactgaggacagcaggaaactcttccaggtgagaccagaaaggataatacaataatttgctaatagttaacagacatttgatattttatggacataaataaaatgatttacctactttacaaagtaatattaactacaggtgtatctaaaaacctatgaaattatttgcaacaaatatttcactgataaaaatttcttaatatttcccttagcaaaaactgtacatttgttagagagtacctgatacttgttaaaatatcaagtaatacaggacatggtgctgtaaaacaaaacacacaactgggaagtattttattttttctacttcatataacattgttcaacaccacaagattttaaaggtctctttccccaacttttatgatttagaagtaccacttaaaaatatttactgatgctgtaaatattactgtttttgtacatagtaaagattttaatgaatgccatatccattatacctcttgctcctttggtcagaaagataaacagaaactttaaatcagatgtttggacattcaaaaatggttttgaaaagtatacccaaacaaaccaaatatatatcagcaactattaaaaatcagttttagtagttattaagaattcttaacaaggaagtatcgaagcatgtgtgagattttaaaaactatatacaattttaaaaacaaatttaaatttttaaataaaaaagattaatggccaaattaaaaagtttgtgcatcagatttaatatcttaatgtttatcagaaatatattttgtgagtaagaattatttcataaatatatatgtataaatataaatatatatctgcaggatctgtgatgctggagaaaacattttgaagaaaaaaattgcacttttgattatcaagatattgtcaaatttaccctttaagtgaaatataattaccaatccaggtgcttttggcacaagtttttaggtgaatatcgacacaatcttaaaaacacaatgcttttgtattttattcactggaatatggagaatcaaacagaatttaaaattctgacccaaaaatcccagataactgcaattgcttaattaaatacaaaaaaaaattgttttaaaaagcgcttagacttccctttccatctggaacatgtaaaattttgcagcaacaggttttctccaattccttcagcaagaattcccagcctacacacaaatttaacaccatctttttctattcatgtataacttggatcacacaccagtatataacgacaaaaaataaatgtataataaaaagattggataaatcagaagaggctttttggtcttgaattcttcacccactaacaatgaagcagcactgtaggcagcccaaaacacaccaaacagttttataagtgtagacaccacttcaaatgatccaaccaccaaaagtacaggggctattacaatgagaggaagtaatgaatatcctataactccaaggacttggccatatgcaacttctccaccaagaactctggccagtaagaaaattgttagtgaaccaaatatccaaatggttataatccatgagaccaccctaaactgtccatataatgatatcatggaaaagaaaagaacaacagccagaggaccccaaaagtcaggattgtctctcaccacttgtctattaaaaccaagtgatggcattggcatcaaaacacatcggattttgtagtaaatatcctttagatcaatgtccaattcttccaagagtggcttgttatcttcaggatcatcatcttcaacttccagaagccagccataacctctttgtctcagaaatgtagtagctgtagattctttgataaaatctccaccaagatttaatttgacatctggggatgctattgaaccactgagatcttccgcgtctgctgaggagacaaaggtgaagtccccgttagtgggggcataggccgggggcgggcccggaggctgcatctcgcggcgactcccaaccggccgcggtagaagaggctgcggctgggcccagaccccgaggcggccgcggcggcgacccgcacgctcgccctacggtgcggcctacgagtctcgacgtgcaagctgcgagcgaggccagaaacgggcacagcgggccgctgagctgccccgagactaccccaccaaagtcttcttggtggcgaccacccaagcaccacgacgccggcaccctgacaggaccataacagtgac

SEQ ID NO: 14694 - RNA, 2188 nt, Homo sapiens
  source 1..2188: mol_type = other RNA
gctgggattacaggcatgagccaccgtgcctggcccaatcctcttaacataaacactttaacatcaattaatgcttgaactcaatgttaaatcaactcaaactcaagtcaatgctgaattgactctaatgacaattaatgcttgatggtttgctatactcattgcctgtgcatcaattatctcaaaaatgaattttctgatgttctgcaaggagtgacctcagactgaaaccttgtcacacttatgacatttgtaagatttctgtccagtagggattctctgatgcctaatgacttgtgaacgtgaagtaaagactttgccataattatcacacctgtgaggtttctctcctgtatgaattctcctatgttttgcctaggatgaagcttgactgaagaccttgcctcaatcatgacatttgtaaggtttctctccagtatgagttcgctgatgaactgcaagttatgaacgatgtctgaaaactttgccacatttattaacacttgtaagatctctcttcattacggattctccaatgatttgcaacagttctagcattaccaaaggcattgtgacaatcattgcattagtaaactttccctacaccatggattgcctgatggatggtgagtaagtggtgattgcccactaaaggctttgccacactcattacacttgtaaggtttctctccagggtgaattctagtatgtcctgcaaggtgtgaatcacacccaaaatccttatcacaaaccttacatttgtatggtttctctccagtatgaattcacctatgtctttcaagctgtgatttacgactgaaaactttgtcacaggtttttctccagtatgagttcactgatgaactgcaaggtatgaatgatgactgtaaaattggccacatttatcacacttgtaagatctctcttcattataggttctccaatgatttgcaagtgttgtagttttactggagactttgtggcagtcattacatctgtgagctttcactataccatggattgcttgatggtgaataggcgatgccctcaccctaaaggctttgccacactcattacacttgtaaggtttctctccagtgtgaatttcagtatgttctgcaaggagtgaattgagcccaaaaaccttttcacaaaccttacatttgtatggcttctccagtgtgaattctcctatgcattgcaaggtgtgatctgcaactgaaaacgttgtcacattctttacatttgtaaggtttctctccagtatgaattgcccacagactccaggttcctgtagttctcccacatcacagccctgtataaagcgttctgtgcagggtccaggcgtttccactccagcaaagagaactctatagccacatctctgaaagtcaagtatccctgaggaagagccatccctggctccttttctttgccttcttggtgtcttcctcaagtaacataagtctctggaaatcaatcccagggagaccaggttcctataattctccagcatcacgtctctgtatagagtcctctgagcagggtccaggcatttccactcctcctgagagaattctatggccacatccctgaatgtcagtagaccctgagaaagagccatccccgactcctttgctttcctcttcctcttctgggtttcttcctcaggtaccaagagtctttagaagtcaatcctgtatctcagctacttggtaggctgaggcacaagaatcacttgaacccaggagacagaggttgcagtgagccaagatcaggagactgcactcacagcctgaaggacagagtgagactcaggctgaggtgggagaattgcttgagcccggagagcagaggttgaagtgaatcaagatcgcacaactgccctccagcctgggggacacagcgaaactccatcacctccaccccccaaaaagttggaagctcactgaattaagatacaacttcaagaaatcataaaagcaatgcatgaagaacatgagaaggacaaccaacatacagaaattatgacgaactacacagaaactctcgggataaaaatacagtaactaaatggaaaaactcaatacatgggttcaaaatcagaattcattatgtaaattaaaaactagtgaagaggggtcaggcaaggtggctcacacctgtaatcccaggactctgggaggcc

SEQ ID NO: 14695 - RNA, 1895 nt, Homo sapiens
  source 1..1895: mol_type = other RNA
gctgggattacaggcatgagccaccgtgcctggcccaatcctcttaacataaacactttaacatcaattaatgcttgaactcaatgttaaatcaactcaaactcaagtcaatgctgaattgactctaatgacaattaatgcttgatggtttgctatactcattgcctgtgcatcaattatctcaaaaatgaattttctgatgttctgcaaggagtgacctcagactgaaaccttgtcacacttatgacatttgtaagatttctgtccagtagggattctctgatgcctaatgacttgtgaacgtgaagtaaagactttgccataattatcacacctgtgaggtttctctcctgtatgaattctcctatgttttgcctaggatgaagcttgactgaagaccttgcctcaatcatgacatttgtaaggtttctctccagtatgagttcgctgatgaactgcaagttatgaacgatgtctgaaaactttgccacatttattaacacttgtaagatctctcttcattacggattctccaatgatttgcaacagttctagcattaccaaaggcattgtgacaatcattgcattagtaaactttccctacaccatggattgcctgatggatggtgagtaagtggtgattgcccactaaaggctttgccacactcattacacttgtaaggtttctctccagggtgaattctagtatgtcctgcaaggtgtgaatcacacccaaaatccttatcacaaaccttacatttgtatggtttctctccagtatgaattcacctatgtctttcaagctgtgatttacgactgaaaactttgtcacaggtttttctccagtatgagttcactgatgaactgcaaggtatgaatgatgactgtaaaattggccacatttatcacacttgtaagatctctcttcattataggttctccaatgatttgcaagtgttgtagttttactggagactttgtggcagtcattacatctgtgagctttcactataccatggattgcttgatggtgaataggcgatgccctcaccctaaaggctttgccacactcattacacttgtaaggtttctctccagtgtgaatttcagtatgttctgcaaggagtgaattgagcccaaaaaccttttcacaaaccttacatttgtatggcttctccagtgtgaattctcctatgcattgcaaggtgtgatctgcaactgaaaacgttgtcacattctttacatttgtaaggtttctctccagtatgaattgcccacagactccaggttcctgtagttctcccacatcacagccctgtataaagcgttctgtgcagggtccaggcgtttccactccagcaaagagaactctatagccacatctctgaaagtcaagtatccctgaggaagagccatccctggctccttttctttgccttcttggtgtcttcctcaagtaacataagtctctggaaatcaatcccagggagaccaggttcctataattctccagcatcacgtctctgtatagagtcctctgagcagggtccaggcatttccactcctcctgagagaattctatggccacatccctgaatgtcagtagaccctgagaaagagccatccccgactcctttgctttcctcttcctcttctgggtttcttcctcaggtaccaagagtctttagaagtcaatcctgtatctcagctacttggtaggctgaggcacaagaatcacttgaacccaggagacagaggttgcagtgagccaagatcaggagactgcactcacagcctgaaggacagagtgagactgcgctgtggtgtgaccttcagtccctgccatccgcttccgggtctatgccaatcagcgcaggacagaggccaggcctggg

SEQ ID NO: 14696 - RNA, 3111 nt, Homo sapiens
  source 1..3111: mol_type = other RNA
gctgggattacaggcatgagccaccgtgcctggcccaatcctcttaacataaacactttaacatcaattaatgcttgaactcaatgttaaatcaactcaaactcaagtcaatgctgaattgactctaatgacaattaatgcttgatggtttgctatactcattgcctgtgcatcaattatctcaaaaatgaattttctgatgttctgcaaggagtgacctcagactgaaaccttgtcacacttatgacatttgtaagatttctgtccagtagggattctctgatgcctaatgacttgtgaacgtgaagtaaagactttgccataattatcacacctgtgaggtttctctcctgtatgaattctcctatgttttgcctaggatgaagcttgactgaagaccttgcctcaatcatgacatttgtaaggtttctctccagtatgagttcgctgatgaactgcaagttatgaacgatgtctgaaaactttgccacatttattaacacttgtaagatctctcttcattacggattctccaatgatttgcaacagttctagcattaccaaaggcattgtgacaatcattgcattagtaaactttccctacaccatggattgcctgatggatggtgagtaagtggtgattgcccactaaaggctttgccacactcattacacttgtaaggtttctctccagggtgaattctagtatgtcctgcaaggtgtgaatcacacccaaaatccttatcacaaaccttacatttgtatggtttctctccagtatgaattcacctatgtctttcaagctgtgatttacgactgaaaactttgtcacaggtttttctccagtatgagttcactgatgaactgcaaggtatgaatgatgactgtaaaattggccacatttatcacacttgtaagatctctcttcattataggttctccaatgatttgcaagtgttgtagttttactggagactttgtggcagtcattacatctgtgagctttcactataccatggattgcttgatggtgaataggcgatgccctcaccctaaaggctttgccacactcattacacttgtaaggtttctctccagtgtgaatttcagtatgttctgcaaggagtgaattgagcccaaaaaccttttcacaaaccttacatttgtatggcttctccagtgtgaattctcctatgcattgcaaggtgtgatctgcaactgaaaacgttgtcacattctttacatttgtaaggtttctctccagtatgaattgccttgtgaacaaaattacaacaaattagctgggtatggtggattccgcctgtagtctcagctgttctggaccctgaggcaggggaattgcttgaacccaaggcagagattgcagtgagctgagatcgcactgctgaaaagacacaaacaagttgaaagccactgtgactcggctcattgcaaactgcctcctgggctcaagcgattctcctgcctcaacctttcgagtagctgggactgcaggtgcacaccaccatgcctggctaagttttgtatttttagtagagacagggttttgtgatgctggccagactggtctcgaactccttactgcaaaaaaatgaatatataatacatagaagtatatgtatttctatgaaatatataacacatagaaatgaataagttgaaagcctctgtgtcttaaacaaatgacagtagaactaaaatatgggaaggtcgggcatggtggttcacacctgtaatcccagcactttggaagtccaaggcaggtggatcacgaggtcaggagttcaagaccattgtggccaacatggtgaaaacctgtctctactaaaaatacaaaaattagctgggcatggtggcatgtgcctgcaatcccagctactcaggagactgaggcaggagaattgcttgaactgggacctgggaggcagaggttgcagtgagccgagatggtgccactgcactccagcctgggctacagagcaagactccatctcaaaaaaggaaaaaaaaaaaaaaagaactaaaatatgggaatctcattcaacctcacaagctccctcaataagaatgatgaaaagtgtaactgttacagggttgatcccacaacaaactgaacaaagcttttcttgttaaaaatgaacaatgccaggtgcggtggctcaagcctgtaatcccagcactttagaggccgaggcgggtgggtatggaggtcaggagttcgagacgagcctggccaacatggcaaaaccctatctccactaaagatacaaaataacatgctgggcatggtggcacgtgcctggaatcccagctgtgtacatcaaaagcacgtatggggcaaaatcacaaaagagaatacaaaaccaggaaaagccaagatacacaaggacagattcttcatgtctggaggaacattttcctcacccacagactccaggttcctgtagttctcccacatcacagccctgtataaagcgttctgtgcagggtccaggcgtttccactccagcaaagagaactctatagccacatctctgaaagtcaagtatccctgaggaagagccatccctggctccttttctttgccttcttggtgtcttcctcaagtaacataagtctctggaaatcaatcccagggagaccaggttcctataattctccagcatcacgtctctgtatagagtcctctgagcagggtccaggcatttccactcctcctgagagaattctatggccacatccctgaatgtcagtagaccctgagaaagagccatccccgactcctttgctttcctcttcctcttctgggtttcttcctcaggtaccaagagtctttagaagtcaatcctgtatctcagctacttggtaggctgaggcacaagaatcacttgaacccaggagacagaggttgcagtgagccaagatcaggagactgcactcacagcctgaaggacagagtgagactcaggctgaggtgggagaattgcttgagcccggagagcagaggttgaagtgaatcaagatcgcacaactgccctccagcgcgctgtggtgtgaccttcagtccctgccatccgcttccgggtctat

SEQ ID NO: 14697 - RNA, 3102 nt, Homo sapiens
  source 1..3102: mol_type = other RNA
gctgggattacaggcatgagccaccgtgcctggcccaatcctcttaacataaacactttaacatcaattaatgcttgaactcaatgttaaatcaactcaaactcaagtcaatgctgaattgactctaatgacaattaatgcttgatggtttgctatactcattgcctgtgcatcaattatctcaaaaatgaattttctgatgttctgcaaggagtgacctcagactgaaaccttgtcacacttatgacatttgtaagatttctgtccagtagggattctctgatgcctaatgacttgtgaacgtgaagtaaagactttgccataattatcacacctgtgaggtttctctcctgtatgaattctcctatgttttgcctaggatgaagcttgactgaagaccttgcctcaatcatgacatttgtaaggtttctctccagtatgagttcgctgatgaactgcaagttatgaacgatgtctgaaaactttgccacatttattaacacttgtaagatctctcttcattacggattctccaatgatttgcaacagttctagcattaccaaaggcattgtgacaatcattgcattagtaaactttccctacaccatggattgcctgatggatggtgagtaagtggtgattgcccactaaaggctttgccacactcattacacttgtaaggtttctctccagggtgaattctagtatgtcctgcaaggtgtgaatcacacccaaaatccttatcacaaaccttacatttgtatggtttctctccagtatgaattcacctatgtctttcaagctgtgatttacgactgaaaactttgtcacaggtttttctccagtatgagttcactgatgaactgcaaggtatgaatgatgactgtaaaattggccacatttatcacacttgtaagatctctcttcattataggttctccaatgatttgcaagtgttgtagttttactggagactttgtggcagtcattacatctgtgagctttcactataccatggattgcttgatggtgaataggcgatgccctcaccctaaaggctttgccacactcattacacttgtaaggtttctctccagtgtgaatttcagtatgttctgcaaggagtgaattgagcccaaaaaccttttcacaaaccttacatttgtatggcttctccagtgtgaattctcctatgcattgcaaggtgtgatctgcaactgaaaacgttgtcacattctttacatttgtaaggtttctctccagtatgaattgccttgtgaacaaaattacaacaaattagctgggtatggtggattccgcctgtagtctcagctgttctggaccctgaggcaggggaattgcttgaacccaaggcagagattgcagtgagctgagatcgcactgctgaaaagacacaaacaagttgaaagccactgtgactcggctcattgcaaactgcctcctgggctcaagcgattctcctgcctcaacctttcgagtagctgggactgcaggtgcacaccaccatgcctggctaagttttgtatttttagtagagacagggttttgtgatgctggccagactggtctcgaactccttactgcaaaaaaatgaatatataatacatagaagtatatgtatttctatgaaatatataacacatagaaatgaataagttgaaagcctctgtgtcttaaacaaatgacagtagaactaaaatatgggaaggtcgggcatggtggttcacacctgtaatcccagcactttggaagtccaaggcaggtggatcacgaggtcaggagttcaagaccattgtggccaacatggtgaaaacctgtctctactaaaaatacaaaaattagctgggcatggtggcatgtgcctgcaatcccagctactcaggagactgaggcaggagaattgcttgaactgggacctgggaggcagaggttgcagtgagccgagatggtgccactgcactccagcctgggctacagagcaagactccatctcaaaaaaggaaaaaaaaaaaaaaagaactaaaatatgggaatctcattcaacctcacaagctccctcaataagaatgatgaaaagtgtaactgttacagggttgatcccacaacaaactgaacaaagcttttcttgttaaaaatgaacaatgccaggtgcggtggctcaagcctgtaatcccagcactttagaggccgaggcgggtgggtatggaggtcaggagttcgagacgagcctggccaacatggcaaaaccctatctccactaaagatacaaaataacatgctgggcatggtggcacgtgcctggaatcccagctgtgtacatcaaaagcacgtatggggcaaaatcacaaaagagaatacaaaaccaggaaaagccaagatacacaaggacagattcttcatgtctggaggaacattttcctcacccacagactccaggttcctgtagttctcccacatcacagccctgtataaagcgttctgtgcagggtccaggcgtttccactccagcaaagagaactctatagccacatctctgaaagtcaagtatccctgaggaagagccatccctggctccttttctttgccttcttggtgtcttcctcaagtaacataagtctctggaaatcaatcccagggagaccaggttcctataattctccagcatcacgtctctgtatagagtcctctgagcagggtccaggcatttccactcctcctgagagaattctatggccacatccctgaatgtcagtagaccctgagaaagagccatccccgactcctttgctttcctcttcctcttctgggtttcttcctcaggtaccaagagtctttagaagtcaatcctgtatctcagctacttggtaggctgaggcacaagaatcacttgaacccaggagacagaggttgcagtgagccaagatcaggagactgcactcacagcctgaaggacagagtgagactccggacgtctcaatttgctctgggttgagaaagaggggccgcaatttccaggtctgtggggactcaacgtccccggtatagcagcaccacaggactgggaagcacacataaaacag

SEQ ID NO: 14698 - RNA, 3033 nt, Homo sapiens
  source 1..3033: mol_type = other RNA
gctgggattacaggcatgagccaccgtgcctggcccaatcctcttaacataaacactttaacatcaattaatgcttgaactcaatgttaaatcaactcaaactcaagtcaatgctgaattgactctaatgacaattaatgcttgatggtttgctatactcattgcctgtgcatcaattatctcaaaaatgaattttctgatgttctgcaaggagtgacctcagactgaaaccttgtcacacttatgacatttgtaagatttctgtccagtagggattctctgatgcctaatgacttgtgaacgtgaagtaaagactttgccataattatcacacctgtgaggtttctctcctgtatgaattctcctatgttttgcctaggatgaagcttgactgaagaccttgcctcaatcatgacatttgtaaggtttctctccagtatgagttcgctgatgaactgcaagttatgaacgatgtctgaaaactttgccacatttattaacacttgtaagatctctcttcattacggattctccaatgatttgcaacagttctagcattaccaaaggcattgtgacaatcattgcattagtaaactttccctacaccatggattgcctgatggatggtgagtaagtggtgattgcccactaaaggctttgccacactcattacacttgtaaggtttctctccagggtgaattctagtatgtcctgcaaggtgtgaatcacacccaaaatccttatcacaaaccttacatttgtatggtttctctccagtatgaattcacctatgtctttcaagctgtgatttacgactgaaaactttgtcacaggtttttctccagtatgagttcactgatgaactgcaaggtatgaatgatgactgtaaaattggccacatttatcacacttgtaagatctctcttcattataggttctccaatgatttgcaagtgttgtagttttactggagactttgtggcagtcattacatctgtgagctttcactataccatggattgcttgatggtgaataggcgatgccctcaccctaaaggctttgccacactcattacacttgtaaggtttctctccagtgtgaatttcagtatgttctgcaaggagtgaattgagcccaaaaaccttttcacaaaccttacatttgtatggcttctccagtgtgaattctcctatgcattgcaaggtgtgatctgcaactgaaaacgttgtcacattctttacatttgtaaggtttctctccagtatgaattgccttgtgaacaaaattacaacaaattagctgggtatggtggattccgcctgtagtctcagctgttctggaccctgaggcaggggaattgcttgaacccaaggcagagattgcagtgagctgagatcgcactgctgaaaagacacaaacaagttgaaagccactgtgactcggctcattgcaaactgcctcctgggctcaagcgattctcctgcctcaacctttcgagtagctgggactgcaggtgcacaccaccatgcctggctaagttttgtatttttagtagagacagggttttgtgatgctggccagactggtctcgaactccttactgcaaaaaaatgaatatataatacatagaagtatatgtatttctatgaaatatataacacatagaaatgaataagttgaaagcctctgtgtcttaaacaaatgacagtagaactaaaatatgggaaggtcgggcatggtggttcacacctgtaatcccagcactttggaagtccaaggcaggtggatcacgaggtcaggagttcaagaccattgtggccaacatggtgaaaacctgtctctactaaaaatacaaaaattagctgggcatggtggcatgtgcctgcaatcccagctactcaggagactgaggcaggagaattgcttgaactgggacctgggaggcagaggttgcagtgagccgagatggtgccactgcactccagcctgggctacagagcaagactccatctcaaaaaaggaaaaaaaaaaaaaaagaactaaaatatgggaatctcattcaacctcacaagctccctcaataagaatgatgaaaagtgtaactgttacagggttgatcccacaacaaactgaacaaagcttttcttgttaaaaatgaacaatgccaggtgcggtggctcaagcctgtaatcccagcactttagaggccgaggcgggtgggtatggaggtcaggagttcgagacgagcctggccaacatggcaaaaccctatctccactaaagatacaaaataacatgctgggcatggtggcacgtgcctggaatcccagctgtgtacatcaaaagcacgtatggggcaaaatcacaaaagagaatacaaaaccaggaaaagccaagatacacaaggacagattcttcatgtctggaggaacattttcctcacccacagactccaggttcctgtagttctcccacatcacagccctgtataaagcgttctgtgcagggtccaggcgtttccactccagcaaagagaactctatagccacatctctgaaagtcaagtatccctgaggaagagccatccctggctccttttctttgccttcttggtgtcttcctcaagtaacataagtctctggaaatcaatcccagggagaccaggttcctataattctccagcatcacgtctctgtatagagtcctctgagcagggtccaggcatttccactcctcctgagagaattctatggccacatccctgaatgtcagtagaccctgagaaagagccatccccgactcctttgctttcctcttcctcttctgggtttcttcctcaggtaccaagagtctttagaagtcaatcctgtatctcagctacttggtaggctgaggcacaagaatcacttgaacccaggagacagaggttgcagtgagccaagatcaggagactgcactcacagcctgaaggacagagtgagactgcgctgtggtgtgaccttcagtccctgccatccgcttccgggtctat

SEQ ID NO: 14699 - RNA, 1965 nt, Homo sapiens
  source 1..1965: mol_type = other RNA
gctgggattacaggcatgagccaccgtgcctggcccagtctgcattcttaatctctgcaaatccttggcatccaagctttctgaattactttataaaagcaatattaattatatcaacaatttcatcagagccttggtagagagacagaattgtgctctgcagtaaaattttcaggtggtctcctatagttaacttttcatccatggcacaattaatgtttacatttgaaataaatgaataaaatgcatttttgtcttaaatagactgttgaggtcccaacatgatacagggatctcccctagaagatttgggattttctagtccaaatgtgatgaaaggaagctcactgtatttggatgccgcacaattcttttctggatcgctctgatttagggaaaattctatcattttatactgatgtgatatcttccttaccaatccctctttctgcatgtccctaaaactcttctcccctgttaaatattagtctttactttggcacataagtgattcttagaacactttgaacaccattctatagatatccttaaatttaaaaccacccctttgaagttaaaagtttaaaatggatataagaccagagatttatttgacaagagtcatagactgaggtacggtccagatataaaaggagggatttagcaggatttttaatgagtaagcccagctcagcaagaatctgacagaagtagaaattatgtgagatcttttcatagttaccccaaatcatgaaagtgtctaaaagttcttgtgatttctctttagtggaactagagaacattcaggtaattgaccgtccctaagtgagtaatatgtgtgctggtctgtaaatcagatgagccctgtgagtttgtcatggagatggtgtcagaagacattgtcataaaattattactaaattatacaattgtcctgttttacctgctttacctcctactgtctttattttctcttctacattgatttctcccagtcttgttgccacgcctcataatgcaataatgatctctatggcttcagctgagttcttgctttggactataacacattgtccatcatacagtttagttatgttaagcccttcaaatagaattttggagcacagatggcagtcactactgtaggtaacctggtcactgccacaaataggttcactgggcttgatgtaggataaaaaccagcacttatttacattcttgaggcattcaactattgttttgtctagctgacctctttcagaggccataggaagggggaagtcaattgcaaaggccatccacatggaggtagctagaacaaggatggcgtctgagcagatccccttcatggtgacagaagaactgctgtgactcccatggttgctctgagaaactggctgaacaggatggtttttgttgatagtttgttcataatgaactaggaaggaaggcaaagcttatttgtcttttcaaggttccaatgccctttaagattagttggccttcaatagatccagatgacagagaggtatgcttcctcaatgcctcccttagtctctccagaaaggcagtaggattttcttcctttcccgatgtagcagtcctgcacctgttttcctgcccttcttgaccacaaagaaaggggtctgggctgctggattctagtggtcctttaccagcgtgcctgacattgcctttgcactcaggagtgagttctagagctgggctgggtttctgagtatttcataacaacccagttgccccatcaagatgcattttcataaacaacagttcttatgcaaattcgtttcagagagggtgtaggtaaccttttgagtcaggattgagatagagtttttgcccactagggcctttgtccttttcctttgtaggaatatgccttaattatcgaacttaagattttgttgccctggattaagtccttttgggtacgaaatatgagag

SEQ ID NO: 14700 - RNA, 1939 nt, Homo sapiens
  source 1..1939: mol_type = other RNA
gctgggattacaggcatgagccaccgtgcctggcccagtctgcattcttaatctctgcaaatccttggcatccaagctttctgaattactttataaaagcaatattaattatatcaacaatttcatcagagccttggtagagagacagaattgtgctctgcagtaaaattttcaggtggtctcctatagttaacttttcatccatggcacaattaatgtttacatttgaaataaatgaataaaatgcatttttgtcttaaatagactgttgaggtcccaacatgatacagggatctcccctagaagatttgggattttctagtccaaatgtgatgaaaggaagctcactgtatttggatgccgcacaattcttttctggatcgctctgatttagggaaaattctatcattttatactgatgtgatatcttccttaccaatccctctttctgcatgtccctaaaactcttctcccctgttaaatattagtctttactttggcacataagtgattcttagaacactttgaacaccattctatagatatccttaaatttaaaaccacccctttgaagttaaaagtttaaaatggatataagaccagagatttatttgacaagagtcatagactgaggtacggtccagatataaaaggagggatttagcaggatttttaatgagtaagcccagctcagcaagaatctgacagaagtagaaattatgtgagatcttttcatagttaccccaaatcatgaaagtgtctaaaagttcttgtgatttctctttagtggaactagagaacattcaggtaattgaccgtccctaagtgagtaatatgtgtgctggtctgtaaatcagatgagccctgtgagtttgtcatggagatggtgtcagaagacattgtcataaaattattactaaattatacaattgtcctgttttacctgctttacctcctactgtctttattttctcttctacattgatttctcccagtcttgttgccacgcctcataatgcaataatgatctctatggcttcagctgagttcttgctttggactataacacattgtccatcatacagtttagttatgttaagcccttcaaatagaattttggagcacagatggcagtcactactgtaggtaacctggtcactgccacaaataggttcactgggcttgatgtaggataaaaaccagcacttatttacattcttgaggcattcaactattgttttgtctagctgacctctttcagaggccataggaagggggaagtcaattgcaaaggccatccacatggaggtagctagaacaaggatggcgtctgagcagatccccttcatggtgacagaagaactgctgtgactcccatggttgctctgagaaactggctgaacaggatggtttttgttgatagtttgttcataatgaactaggaaggaaggcaaagcttatttgtcttttcaaggttccaatgccttatatggaatcctccaagttcagtcttatttagcagagctgagaaatctggagatagagtgctcatttcccttaaatgatagcttgttctaccatttgaacaaaaatttctcaaaacgctaacattttttaaagcagaagttcagaagttattggttatcataaattcctcaggtctaagtcctaaatgaatggccttaactggggacatgccacatagttctgggaggtcaagtgtattttctcagcactgctctgatcaaccacagtgtctaccatggtggtcttcagaatttttgcttttaatccctctaaatttggtgcctgcttatatatatttttaagttacatgtaaaattttccatcagaaattttaataggctgggtactgtggctcaagcctgtaatctcagcactttgggaagctgaggcaggcggatcgcttgaggctagg

SEQ ID NO: 14701 - RNA, 2338 nt, Homo sapiens
  source 1..2338: mol_type = other RNA
gctgggattacaggcatgagccaccgtgcctggccctcagggtacttttaataaagtgctagctaggcaagcctattcttcctctcaagagtaggtgttccacttttgaacacctatgccaggcaccggctatagtgcctacaagaggatgatatgtggacatgaccactttccctgactacatcagtggttctcaactggggatgattttgcaatgtctgcttatgggacatttggtaatgtctagagacatttgtggttgtcacaactagtggaggggtactacctgcatgtagtgggtagagtccagagatgctactaagtatcctataatgcataggacagctgcccacaacaaagaattatctcactcaaaatgtcaatagggtcgaggttgagaaatcctggtctaggctgggtgtggtggctcatgactgtaatcccagcattttgggaggccaaggcaggaggatcacttgagcccaccaggagttcaagaccagcctgggcaatgtagggagatctccacaaaaaataaaaataaattagctgcactatagtccttgttacacagaaggctgacgtgggagcatcacttgaacgtaggaagtgagtgagctgtgattgcactactgcactccagtctgggcaacagagtgagaccctggctcaaacaaaacaaaaacaaaagcattgaaagaaagaaagaggccgggcgcggtggctcacgcctgtaatcccagcactttgggaggccgaggcgggcagatcacggggtcaggagatcgagaccatcctgactaacacggtgaaaccctgtctctactaaaaatacaaaaaattagccaggcttggtggcgggcgcctgtagtcccagctactcggcaggctgaggcaggagaatggcatgaatccaggaggcggagctggcagtgagccgagatcgtgccaccacactccagcctgggcaacagagcgagactctggtactcctgcaccacctcctccaaaggcagcacgctgtgctgtttgtggctcctggattctcggcacaccacacagatggcctctttgtccacctcacagaagagtttcagggcttcctggtgtttaaagcacatgccctgatcattactccggtttccccgataaggagtggggcacatctggcgaattatctggaccatgttggccagctgcaagttgggacgaaagctgcgacgtgtaaagctctttcggcactgggggcaggtgaactgccctggaaggggcaaggaaggaggcgggtggatgtcaggatacagctcttcatcttcgtcctcatcgtatgcttccagtatttcttcttctcggtagacatcaattctcaggtcaggtctcaagcctcctaggtaatagtcctgatcttcctcttcttcttcttcctcctcgtcccacatatagtctacgttgtcccaattagttataccactgtcaccgagccagagttcatcgtcatcttggtcttggaacaactcttcgtcagcattcccccgatacaacacctctcgaatggagccgtcccatccatccatggcccccaccgcttcctcgtcctcctcctcctcccattcatcttcctcctcgttctggtcctcctcgtcctccttactccacagctgggtcacacaccctcggcagaagttgtgcccacagctgatggacacggggtccttgaagtaatccaagcagatggcacacaccgcttcctcctgaagggtctgcatggggctgggagtagtggcataaccagccatcttaatgcccgccggcaggtgtagatacgtcagcttggagctgaggagcggggacgcgcctgcaggcctgcctccaaactactctggtgacccgaggctgtcctcaaccttgctcttcttcctcggggccgcaggggagctttgaccccctctctcagggtgcgaacgcccagatccagactcacagcctctctctgggatcggtggggacagagcaggctgcagcccccagctgctcggtcctgtcacgtctctcgctaccctcagggtgtgccctacactgcggcgtccgcctcagatgcagccgctggctaccctgcccgaggcgacgcaaaatgacgtctcgctcctgcacacgctctggagagacgctctaggccggcggaggaccacgtctctatggtgtgccgggggccgcgcgggccgggagttgggtgggctgggggacaggcgcgcccgcgccgcccgctccagctgggctagtgctgcacattccggccagcccctcctcaagaccccattcccaagccccttctcagctc

SEQ ID NO: 14702 - RNA, 1446 nt, Homo sapiens
  source 1..1446: mol_type = other RNA
gctgggattacaggcatgagccaccgtgcctggccgagaccccatctctttaaaaaaaccaaaaatgtttattagatgaatgagagaatcctgacatgagcagacacctcgtgctgtgttgtggaggcggacaggccctgtggggagtggggacacactcgtgtggcagcttcccccagccccaacgccccacccctgcttccctaggctgcaggccaacttcaccatccgggaagatgccaaccccagctcccgacagcgaggactcaagcgcttccaggctaacccggaggccaactggggtccccggcctcgtgcccggccagggtgagtggtggtaaggtgggggtggggctcagccagggaaagaaggggtaaagggcagatggggtcccacctactcctcccctcgcacaggggcaaggcggccgacgaagctatggaggagagacgcaggctgcttcagaacaagcggaaggagccgccggaagatgtggcccagcgggctgcccggctcaagacatttccttgcaagaggtttaaggaggtgaggtccctcctccctttcctccactgcaggacacatgagtctcccctttgggcaacagggagagaattgggggagctggggccaggcaagtgtttgggagtgggcttcccatcccaggaaaggatcccatcaggggctgctgagctccgggcaggggttcacacccaccatcttcccaccagggcacctgtcaacgcggggaccagtgctgctactcccacagccccccgacacccagggtttctgctgatgctgcccctgactgtccagagacctccaaccagaccccccctggacctggggctgccgctgggccaggcatagactgaaccaataaagagatgtcacgtcaccttctcccgattgcctgtggtttgtgtattggtccatacagctgcatgactgggatctgttcctctggggatcgttcgcccctgcctggctggagtgttgagtcttcagcgctctccaggccacgggcttgcgcatagtggggcgctcctgcccggtagcccccacgtgtcttcgcgccgctgcctcctcgccgcctggtttctttggcccagctctccaggggccacagtggcggaagctggaccggaaccaggcgccctgtgcatccgctccagaccaggtgcttcctgccctgaggcccggggcgaggggggcgtgcacacaaagagggacctcgcaggctgctgcccagacacccagtgagggggagctgtacccctccctgccctccagagtggggtttagtaacgttaacgaagagtcctggggcaggatcccctctctggctcctgctcccttcatccccatctgtaatgaggctaatcttaggaccctccttgtagcgatatcagagttagcgcttaattttttttttttttttt

SEQ ID NO: 14703 - RNA, 5859 nt, Homo sapiens
  source 1..5859: mol_type = other RNA
gctgggattacaggcatgagccaccgtgcctggccggtttctatttttataatgcaaaaataataatcatggcaatgggaattcagggattgtatgtagtcagaagggctaagaagtagggagaaatgatgccattttagagcctgggcagctgaggcagagaagaaacgaatccatctgtggagctgacccaggtgcaagctcccaggatctgccagtctcagtcgcatggtttcatcctgaaagcagctgcccttacttaagggacaaagtcttttaggagctgcccacaaatacttggaaaacaaggcttcaaaatccagaagcaacaatgcaaatttcagaatggtgctgtgagaaaggaaaaatgttagagtcacaggagtttgccctttaattgtaagcaagacttcttgattctaaaaaatttctgtagtttattcagtttgctaattcagaagaaagtgtgcattgcatgagatcaaagaattgaaaattttaaaatgatttgggttgtagctggctcccaactgcaggtgagtcactaatctccaatgtttggatactgtatttgtgtttgttttgagacagagtcttgctctgtcgcccaggctggagtgcagtggtacaatcgaggctcactgcaacctctgcttcctgggctcaagggattcgtgtgtctcagcctccctagtagctgggattacaggcgccggccaccatgcccagctaattgtttttgtttttagtggagacggggtttcaccatgttggccaggctggtcttgaattcctgacctcaggtgatccacctgcctcagctttccaaagtggtgggattacaggcgtgagccactgtgtcccgcctgtttcctgtatgtggataaatctcaggacaagatgaagctgggacaggctcctcctactaccagtgacgcatgcatgcctttggctacaacaaaggccttttaagaacttcaatctccaagtctggtgggaggctttgtcttgcctcgtcagcctggaggttctgttttgaaagagcaaagcagcagactgaaattgaatgggttgcaaaggagaaacctttagagctatagaaaactttctatctatcgaaataggccatttccaacagaggcctgaatttagaaactcctagagctggctggaactttagaggataaccacagtggtccgtaaccctcttaggaagcactgggttggatacacaccctaaggggagtaggttgggttaggaacccttccagtcacctttctttgctctataggtcatcttatgaaggctaatcaccctccttttcattctagattattgctgtgttgcatacacgtgactgcaattaagtgttaaatctcacatctgtggaagttttggtagctcacttctgataagattggccagccgggtgcggtggctcacacctgtaatcccagcactttgggaggctgaggtgggtggatcatgaggtcaggagttcgagaccagcctgaccaacatggtgaaacaccgtctctactaaaaataaaaaaattagctgggcatagtggtgggtgcctgtaatcccagctactcaggagactgacacaggagaatcgcttgaacctgggaggtgggggttgcagcgagctgagatcatgccactgcactccagcctggctggcagagagctactctgtctcaaaaaaaaaaaaaaaaaaaaaatcggccagagggctcatggggaaaaaagtcacttgtgtgtagttcccgctctgtgacccactaaaagctctgcgtttaagggcagggaagcatggtccagccctgttatcccccaaaaggacacatacaaagctcagttcttgagctgtgcttatgcaatactatagtgatcagtaagctgaatgtatttgcttcacttctaaccttttttaaaagtgatcttgaggaatgctttgttgatcttgaattaataattcaaaaagggggtgggggaagatggggtatttctaagaaatgcagaatatttcagttttgaatattaaatctcttacaactacaaaccccttcatagtctccatccattcagaaaaacaaagccaaaggagaatttcttgtggaaaaaaactaaggaagttccccacataaccagccgaagaggaaaggctttccctgtcctctctcaagaggaagccacagcagccgtttgtcatgttactgctaccctggcttttaaaaagtgacagggagcaggactttagattaggactttggtggatactctgtatagttgagtataaaatccctacaatgagttagacttagtttcctagataaataaacgtgtctacataaaattttatatatatattttttcttccagttaacagtcttttctcttgggtgggtagaccaaacccaagatccaaccttccccttacttcccaccaagtagtaccaaaaacaactttccccctccactaagtccttagggaagcaggaaggctagtgcagcagctgtcagggataaaggcacaggcagagctggggtgacggagttgtctgggacaggctaccactggcccactggagtcacggaaccctgacaccaccctcagcaggggaggttcccgatcaccctcaagttctcccatcccatagttagatcttttaaaggcacatctagaagtggtgcaactggaggcaggggtaagctgtacacagttgccacgcaggggttaaggggctgcaggactccatggtacagaggaatggaagtgtccttgccctcttccagactcggggcagggggagacagcggggagatgggctcctggaacccagcctgtttctgtagagccccagaggggccaacaacaggaaagaccagagtcgtggtcagtagtgcacatgcttaacaggtctttggtgcttgggtagcagcatctcttatgtacaaaggcttctgaagccagcaaagctgggaaagtcatctcctgcacagtcgcggcctgactcctctcctggtgctggccatcggctcacaagcccctgggctccagaaccagccagttctcagtgaccatctgcacatcctggccactcagaggctcccgcagcctcaccttcacctccagcttccccccggtgggcttccttccatccaggacctccacaatttctctgatctcacactcattctccagccgctccagtttcaggtgtgctgtgccaaccagcttgtcgcttctgaagaaggaccctttgtggaagatctcaaacttgatgcctttgctctggatcaccctcttgaagccccggtggtttcggttgatgtttagtttgaagagttgatcaaattctggagagtttgtgttcttcaccacagctgttttgcttttttgagcctggtccgagttagggtagtgaaactcaaaccgcacaaaagcatccaggtcatcgggagtcacccctggaggggctgggaggttcattccccggacaatgatcagatgcatttctgtgctgttgagttctgagaagatcctcacagtctggaatgtcttcaactcaaagtggtgggtgggagggtcgaggccctgagcctgggccagctgcaggatctccagctgtttcttgcggtcctgagcaagcttctcaaatcgggtggtctcagccacgttgccctggtgcatgaactgcttggagaacagcaggcacttctcttgttgctccagaagcattttttgcagctgggcatacacctcctccgccttctgggagagtcgcaggtcctcatggtggatgaggatgaagtcaccctcctcatccgtcaagggcgaaggcaccttggacagatcaacaggtctgccagatcgggcctggatgatctgagcctcaagccatttggctacccgcagataggctttggcctgctccaggtcctggctgcgcttggcctgcagggctgcccgctgatactgcagtttccgtgcctccagcagtgccagctgctcccgcacagatggactcggtgactccttagaacttgaggccctgggctcaggcaggcgctgggatgaagggactgtgggccgtgcaggtttcttggccactggggcctgtgctgggggctcaccctgcaggtgcccaggaggctcgtcctcgtctttatcagccggggctgaatcctctgcagaggccagtttctctgcagctgccaatgtcgctgccactgcgtcctcctcaacacccatagtggactccaggccagggatggggggaaatcctggaggaacaggcaattcagcaaagttgactttccgtcctgctcggtgtgctcgaatagcatcttgatattgcttggcaatgcgctcatgcatccgagccttgcgctcgtccccaccactccgggcctggatgcccgcctcgcggtacttgttcagcctctgctgcagggcatccagcactgtctgtgactctgtaggggccactggggttgctgggacgtcaggggccatcactggctgcactcgctccacggctgggggaatgactgagggtgctgtgggagcctgagaagcctgctggggcttcagatcctcaggtgccgggggcatggcactcagatccacgggctgccccttctccagggcctccaggacagcaccgaatctcttcccaatcctcatgagctctcgggcacggtctagctctccagcccgcttggcactgagggcagccactttgtactctctctgtcgggatgacagcagggcccgcgggtctgggtctaagtctgaaacgggctgggcagaaatgccagggaggctggtctcaggttgggaggggttgtctgactccaaggcagggggagctggagggtctgtctcagggctcctgttggctggttcctggggggccaggggccgctttcctaaggccactggaggtgggatctcatcctcattgatctttctgcctctcctcacagaggctagctgcgactccaaggtcttcaggccgcgctcgcagcgcctggctttggctgcttcgcctgcctccttggcactggccgcagcctctcggtagttgtgaatccgttcctccagcaaagcgtgtagcccctgagatgctccggcctgagctgctggggctgaagctgtcaggacggctgtctgcactggaggttcagtgtcttctaggccgttctcctcctcagagccgcctgggtcagctacctcatcaccatccaggggctcagtctcctcgtccacacctaagacctcctgcagctccgtcagcagctctgcatcttcctccagcccttcctcctcctcctcctcctccacatcccgcatacagtctgccgccaacttctcgatgtgggccatgggcaggggggcctgccccttgggtgctggcttcttgcctgtggtttgtgcttcccctgtgagagccagcagctcagcctccaggtcctcatcatcttcagcctcatccatgcccagcagcatgtcctcagggccaaactccataaagagccccatctgcttggcagcggccaccccttggcctctggcctgagggcccttccgaggtcttggccctggcatcatggcagcctagatacctcgcggtgaatccgagccaaaccccggccttgtctcacccggcaccgccctgggctcccgcgggccctgggccgcagcggtagcgacaggaagcgccagcaggggaggtggctcgcgcgcaacacgtgaccccactggccggcggccggcagtgcgcatgtgcacggctacgcgggcggggggctccaacaggtgacaccggggcggggttcgcagcgcgca

SEQ ID NO: 14704 - RNA, 6648 nt, Homo sapiens
  source 1..6648: mol_type = other RNA
gctgggattacaggcatgagccaccgtgcctggccggtttctatttttataatgcaaaaataataatcatggcaatgggaattcagggattgtatgtagtcagaagggctaagaagtagggagaaatgatgccattttagagcctgggcagctgaggcagagaagaaacgaatccatctgtggagctgacccaggtgcaagctcccaggatctgccagtctcagtcgcatggtttcatcctgaaagcagctgcccttacttaagggacaaagtcttttaggagctgcccacaaatacttggaaaacaaggcttcaaaatccagaagcaacaatgcaaatttcagaatggtgctgtgagaaaggaaaaatgttagagtcacaggagtttgccctttaattgtaagcaagacttcttgattctaaaaaatttctgtagtttattcagtttgctaattcagaagaaagtgtgcattgcatgagatcaaagaattgaaaattttaaaatgatttgggttgtagctggctcccaactgcaggtgagtcactaatctccaatgtttggatactgtatttgtgtttgttttgagacagagtcttgctctgtcgcccaggctggagtgcagtggtacaatcgaggctcactgcaacctctgcttcctgggctcaagggattcgtgtgtctcagcctccctagtagctgggattacaggcgccggccaccatgcccagctaattgtttttgtttttagtggagacggggtttcaccatgttggccaggctggtcttgaattcctgacctcaggtgatccacctgcctcagctttccaaagtggtgggattacaggcgtgagccactgtgtcccgcctgtttcctgtatgtggataaatctcaggacaagatgaagctgggacaggctcctcctactaccagtgacgcatgcatgcctttggctacaacaaaggccttttaagaacttcaatctccaagtctggtgggaggctttgtcttgcctcgtcagcctggaggttctgttttgaaagagcaaagcagcagactgaaattgaatgggttgcaaaggagaaacctttagagctatagaaaactttctatctatcgaaataggccatttccaacagaggcctgaatttagaaactcctagagctggctggaactttagaggataaccacagtggtccgtaaccctcttaggaagcactgggttggatacacaccctaaggggagtaggttgggttaggaacccttccagtcacctttctttgctctataggtcatcttatgaaggctaatcaccctccttttcattctagattattgctgtgttgcatacacgtgactgcaattaagtgttaaatctcacatctgtggaagttttggtagctcacttctgataagattggccagccgggtgcggtggctcacacctgtaatcccagcactttgggaggctgaggtgggtggatcatgaggtcaggagttcgagaccagcctgaccaacatggtgaaacaccgtctctactaaaaataaaaaaattagctgggcatagtggtgggtgcctgtaatcccagctactcaggagactgacacaggagaatcgcttgaacctgggaggtgggggttgcagcgagctgagatcatgccactgcactccagcctggctggcagagagctactctgtctcaaaaaaaaaaaaaaaaaaaaaatcggccagagggctcatggggaaaaaagtcacttgtgtgtagttcccgctctgtgacccactaaaagctctgcgtttaagggcagggaagcatggtccagccctgttatcccccaaaaggacacatacaaagctcagttcttgagctgtgcttatgcaatactatagtgatcagtaagctgaatgtatttgcttcacttctaaccttttttaaaagtgatcttgaggaatgctttgttgatcttgaattaataattcaaaaagggggtgggggaagatggggtatttctaagaaatgcagaatatttcagttttgaatattaaatctcttacaactacaaaccccttcatagtctccatccattcagaaaaacaaagccaaaggagaatttcttgtggaaaaaaactaaggaagttccccacataaccagccgaagaggaaaggctttccctgtcctctctcaagaggaagccacagcagccgtttgtcatgttactgctaccctggcttttaaaaagtgacagggagcaggactttagattaggactttggtggatactctgtatagttgagtataaaatccctacaatgagttagacttagtttcctagataaataaacgtgtctacataaaattttatatatatattttttcttccagttaacagtcttttctcttgggtgggtagaccaaacccaagatccaaccttccccttacttcccaccaagtagtaccaaaaacaactttccccctccactaagtccttagggaagcaggaaggctagtgcagcagctgtcagggataaaggcacaggcagagctggggtgacggagttgtctgggacaggctaccactggcccactggagtcacggaaccctgacaccaccctcagcaggggaggttcccgatcaccctcaagttctcccatcccatagttagatcttttaaaggcacatctagaagtggtgcaactggaggcaggggtaagctgtacacagttgccacgcaggggttaaggggctgcaggactccatggtacagaggaatggaagtgtccttgccctcttccagactcggggcagggggagacagcggggagatgggctcctggaacccagcctgtttctgtagagccccagaggggccaacaacaggaaagaccagagtcgtggtcagtagtgcacatgcttaacaggtctttggtgcttgggtagcagcatctcttatgtacaaaggcttctgaagccagcaaagctgggaaagtcatctcctgcacagtcgcggcctgactcctctcctggtgctggccatcggctcacaagcccctgggctccagaaccagccagttctcagtgaccatctgcacatcctggccactcagaggctcccgcagcctcaccttcacctccagcttccccccggtgggcttccttccatccaggacctgtgaggaccacagagagggaaatggtaactaaggggacagagatggggagcaggcaggtccctacattcccaggaaagaagtgagaggagctaagatgtcctgtggcatgaacacaggaatctccattcatgaaaaccctaccctcccagtatttggaggaggaggtggtggtggttttaggtgagtcttattaaaaaagtaataaataaatccagacaagcatcctagagctctgttcattttctcctcaatccccacggcaacttctggaagaaacattggcttgaagaagcagccttccactgacccaaaccctcacttcacagatggccaagagagagaagcagatgactctatgtggcagagtcagcactggaaccccaaacccagggttccttcccattcaccacgctactccctcttttgggcagaagatgaggcagtcaattagggcacaaagcagtacaataggcccaagaagtccaaccaccctcagtggctccaatagagaccagggcccgcataagaacaacttccccaggcaggcagtagggccaggtgtgctacagtgggaagagccccagcctacataggttatcagtaaggagctggtcgtagctctgccaaggacacaccatatgagcttacagaaccccctttcctctcggacctgagtttcctcatttgtcagaggcaaggtcgtatagtccttgcctgtggaatccattgagttcatggaaacaaggaggctgccttctcctgggtccctctgtgagatttctcagaccttctgaacctctccatctccacaatttctctgatctcacactcattctccagccgctccagtttcaggtgtgctgtgccaaccagcttgtcgcttctgaagaaggaccctttgtggaagatctcaaacttgatgcctttgctctggatcaccctcttgaagccccggtggtttcggttgatgtttagtttgaagagttgatcaaattctggagagtttgtgttcttcaccacagctgttttgcttttttgagcctggtccgagttagggtagtgaaactcaaaccgcacaaaagcatccaggtcatcgggagtcacccctggaggggctgggaggttcattccccggacaatgatcagatgcatttctgtgctgttgagttctgagaagatcctcacagtctggaatgtcttcaactcaaagtggtgggtgggagggtcgaggccctgagcctgggccagctgcaggatctccagctgtttcttgcggtcctgagcaagcttctcaaatcgggtggtctcagccacgttgccctggtgcatgaactgcttggagaacagcaggcacttctcttgttgctccagaagcattttttgcagctgggcatacacctcctccgccttctgggagagtcgcaggtcctcatggtggatgaggatgaagtcaccctcctcatccgtcaagggcgaaggcaccttggacagatcaacaggtctgccagatcgggcctggatgatctgagcctcaagccatttggctacccgcagataggctttggcctgctccaggtcctggctgcgcttggcctgcagggctgcccgctgatactgcagtttccgtgcctccagcagtgccagctgctcccgcacagatggactcggtgactccttagaacttgaggccctgggctcaggcaggcgctgggatgaagggactgtgggccgtgcaggtttcttggccactggggcctgtgctgggggctcaccctcgtcctcgtctttatcagccggggctgaatcctctgcagaggccagtttctctgcagctgccaatgtcgctgccactgcgtcctcctcaacacccatagtggactccaggccagggatggggggaaatcctggaggaacaggcaattcagcaaagttgactttccgtcctgctcggtgtgctcgaatagcatcttgatattgcttggcaatgcgctcatgcatccgagccttgcgctcgtccccaccactccgggcctggatgcccgcctcgcggtacttgttcagcctctgctgcagggcatccagcactgtctgtgactctgtaggggccactggggttgctgggacgtcaggggccatcactggctgcactcgctccacggctgggggaatgactgagggtgctgtgggagcctgagaagcctgctggggcttcagatcctcaggtgccgggggcatggcactcagatccacgggctgccccttctccagggcctccaggacagcaccgaatctcttcccaatcctcatgagctctcgggcacggtctagctctccagcccgcttggcactgagggcagccactttgtactctctctgtcgggatgacagcagggcccgcgggtctgggtctaagtctgaaacgggctgggcagaaatgccagggaggctggtctcaggttgggaggggttgtctgactccaaggcagggggagctggagggtctgtctcagggctcctgttggctggttcctggggggccaggggccgctttcctaaggccactggaggtgggatctcatcctcattgatctttctgcctctcctcacagaggctagctgcgactccaaggtcttcaggccgcgctcgcagcgcctggctttggctgcttcgcctgcctccttggcactggccgcagcctctcggtagttgtgaatccgttcctccagcaaagcgtgtagcccctgagatgctccggcctgagctgctggggctgaagctgtcaggacggctgtctgcactggaggttcagtgtcttctaggccgttctcctcctcagagccgcctgggtcagctacctcatcaccatccaggggctcagtctcctcgtccacacctaagacctcctgcagctccgtcagcagctctgcatcttcctccagcccttcctcctcctcctcctcctccacatcccgcatacagtctgccgccaacttctcgatgtgggccatgggcaggggggcctgccccttgggtgctggcttcttgcctgtggtttgtgcttcccctgtgagagccagcagctcagcctccaggtcctcatcatcttcagcctcatccatgcccagcagcatgtcctcagggccaaactccataaagagccccatctgcttggcagcggccaccccttggcctctggcctgagggcccttccgaggtcttggccctggcatcatggcagcctagatacctcgcggtgaatccgagccaaaccccggccttgtctcacccggcaccgccctgggctcccgcgggccctgggccgcagcggtagcgacaggaagcgccagcaggggaggtggctcgcgcgcaacacgtgaccccactggccggcggccggcagtgcgcatgtgcacggctacgcgggcggggggctccaacaggtgacaccggggcggggttcgcagcgcgca

SEQ ID NO: 14705 - RNA, 5949 nt, Homo sapiens
  source 1..5949: mol_type = other RNA
gctgggattacaggcatgagccaccgtgcctggccggtttctatttttataatgcaaaaataataatcatggcaatgggaattcagggattgtatgtagtcagaagggctaagaagtagggagaaatgatgccattttagagcctgggcagctgaggcagagaagaaacgaatccatctgtggagctgacccaggtgcaagctcccaggatctgccagtctcagtcgcatggtttcatcctgaaagcagctgcccttacttaagggacaaagtcttttaggagctgcccacaaatacttggaaaacaaggcttcaaaatccagaagcaacaatgcaaatttcagaatggtgctgtgagaaaggaaaaatgttagagtcacaggagtttgccctttaattgtaagcaagacttcttgattctaaaaaatttctgtagtttattcagtttgctaattcagaagaaagtgtgcattgcatgagatcaaagaattgaaaattttaaaatgatttgggttgtagctggctcccaactgcaggtgagtcactaatctccaatgtttggatactgtatttgtgtttgttttgagacagagtcttgctctgtcgcccaggctggagtgcagtggtacaatcgaggctcactgcaacctctgcttcctgggctcaagggattcgtgtgtctcagcctccctagtagctgggattacaggcgccggccaccatgcccagctaattgtttttgtttttagtggagacggggtttcaccatgttggccaggctggtcttgaattcctgacctcaggtgatccacctgcctcagctttccaaagtggtgggattacaggcgtgagccactgtgtcccgcctgtttcctgtatgtggataaatctcaggacaagatgaagctgggacaggctcctcctactaccagtgacgcatgcatgcctttggctacaacaaaggccttttaagaacttcaatctccaagtctggtgggaggctttgtcttgcctcgtcagcctggaggttctgttttgaaagagcaaagcagcagactgaaattgaatgggttgcaaaggagaaacctttagagctatagaaaactttctatctatcgaaataggccatttccaacagaggcctgaatttagaaactcctagagctggctggaactttagaggataaccacagtggtccgtaaccctcttaggaagcactgggttggatacacaccctaaggggagtaggttgggttaggaacccttccagtcacctttctttgctctataggtcatcttatgaaggctaatcaccctccttttcattctagattattgctgtgttgcatacacgtgactgcaattaagtgttaaatctcacatctgtggaagttttggtagctcacttctgataagattggccagccgggtgcggtggctcacacctgtaatcccagcactttgggaggctgaggtgggtggatcatgaggtcaggagttcgagaccagcctgaccaacatggtgaaacaccgtctctactaaaaataaaaaaattagctgggcatagtggtgggtgcctgtaatcccagctactcaggagactgacacaggagaatcgcttgaacctgggaggtgggggttgcagcgagctgagatcatgccactgcactccagcctggctggcagagagctactctgtctcaaaaaaaaaaaaaaaaaaaaaatcggccagagggctcatggggaaaaaagtcacttgtgtgtagttcccgctctgtgacccactaaaagctctgcgtttaagggcagggaagcatggtccagccctgttatcccccaaaaggacacatacaaagctcagttcttgagctgtgcttatgcaatactatagtgatcagtaagctgaatgtatttgcttcacttctaaccttttttaaaagtgatcttgaggaatgctttgttgatcttgaattaataattcaaaaagggggtgggggaagatggggtatttctaagaaatgcagaatatttcagttttgaatattaaatctcttacaactacaaaccccttcatagtctccatccattcagaaaaacaaagccaaaggagaatttcttgtggaaaaaaactaaggaagttccccacataaccagccgaagaggaaaggctttccctgtcctctctcaagaggaagccacagcagccgtttgtcatgttactgctaccctggcttttaaaaagtgacagggagcaggactttagattaggactttggtggatactctgtatagttgagtataaaatccctacaatgagttagacttagtttcctagataaataaacgtgtctacataaaattttatatatatattttttcttccagttaacagtcttttctcttgggtgggtagaccaaacccaagatccaaccttccccttacttcccaccaagtagtaccaaaaacaactttccccctccactaagtccttagggaagcaggaaggctagtgcagcagctgtcagggataaaggcacaggcagagctggggtgacggagttgtctgggacaggctaccactggcccactggagtcacggaaccctgacaccaccctcagcaggggaggttcccgatcaccctcaagttctcccatcccatagttagatcttttaaaggcacatctagaagtggtgcaactggaggcaggggtaagctgtacacagttgccacgcaggggttaaggggctgcaggactccatggtacagaggaatggaagtgtccttgccctcttccagactcggggcagggggagacagcggggagatgggctcctggaacccagcctgtttctgtagagccccagaggggccaacaacaggaaagaccagagtcgtggtcagtagtgcacatgcttaacaggtctttggtgcttgggtagcagcatctcttatgtacaaaggcttctgaagccagcaaagctgggaaagtcatctcctgcacagtcgcggcctgactcctctcctggtgctggccatcggctcacaagcccctgggctccagaaccagccagttctcagtgaccatctgcacatcctggccactcagaggctcccgcagcctcaccttcacctccagcttccccccggtgggcttccttccatccaggacctgtggaatccattgagttcatggaaacaaggaggctgccttctcctgggtccctctgtgagatttctcagaccttctgaacctctccatctccacaatttctctgatctcacactcattctccagccgctccagtttcaggtgtgctgtgccaaccagcttgtcgcttctgaagaaggaccctttgtggaagatctcaaacttgatgcctttgctctggatcaccctcttgaagccccggtggtttcggttgatgtttagtttgaagagttgatcaaattctggagagtttgtgttcttcaccacagctgttttgcttttttgagcctggtccgagttagggtagtgaaactcaaaccgcacaaaagcatccaggtcatcgggagtcacccctggaggggctgggaggttcattccccggacaatgatcagatgcatttctgtgctgttgagttctgagaagatcctcacagtctggaatgtcttcaactcaaagtggtgggtgggagggtcgaggccctgagcctgggccagctgcaggatctccagctgtttcttgcggtcctgagcaagcttctcaaatcgggtggtctcagccacgttgccctggtgcatgaactgcttggagaacagcaggcacttctcttgttgctccagaagcattttttgcagctgggcatacacctcctccgccttctgggagagtcgcaggtcctcatggtggatgaggatgaagtcaccctcctcatccgtcaagggcgaaggcaccttggacagatcaacaggtctgccagatcgggcctggatgatctgagcctcaagccatttggctacccgcagataggctttggcctgctccaggtcctggctgcgcttggcctgcagggctgcccgctgatactgcagtttccgtgcctccagcagtgccagctgctcccgcacagatggactcggtgactccttagaacttgaggccctgggctcaggcaggcgctgggatgaagggactgtgggccgtgcaggtttcttggccactggggcctgtgctgggggctcaccctgcaggtgcccaggaggctcgtcctcgtctttatcagccggggctgaatcctctgcagaggccagtttctctgcagctgccaatgtcgctgccactgcgtcctcctcaacacccatagtggactccaggccagggatggggggaaatcctggaggaacaggcaattcagcaaagttgactttccgtcctgctcggtgtgctcgaatagcatcttgatattgcttggcaatgcgctcatgcatccgagccttgcgctcgtccccaccactccgggcctggatgcccgcctcgcggtacttgttcagcctctgctgcagggcatccagcactgtctgtgactctgtaggggccactggggttgctgggacgtcaggggccatcactggctgcactcgctccacggctgggggaatgactgagggtgctgtgggagcctgagaagcctgctggggcttcagatcctcaggtgccgggggcatggcactcagatccacgggctgccccttctccagggcctccaggacagcaccgaatctcttcccaatcctcatgagctctcgggcacggtctagctctccagcccgcttggcactgagggcagccactttgtactctctctgtcgggatgacagcagggcccgcgggtctgggtctaagtctgaaacgggctgggcagaaatgccagggaggctggtctcaggttgggaggggttgtctgactccaaggcagggggagctggagggtctgtctcagggctcctgttggctggttcctggggggccaggggccgctttcctaaggccactggaggtgggatctcatcctcattgatctttctgcctctcctcacagaggctagctgcgactccaaggtcttcaggccgcgctcgcagcgcctggctttggctgcttcgcctgcctccttggcactggccgcagcctctcggtagttgtgaatccgttcctccagcaaagcgtgtagcccctgagatgctccggcctgagctgctggggctgaagctgtcaggacggctgtctgcactggaggttcagtgtcttctaggccgttctcctcctcagagccgcctgggtcagctacctcatcaccatccaggggctcagtctcctcgtccacacctaagacctcctgcagctccgtcagcagctctgcatcttcctccagcccttcctcctcctcctcctcctccacatcccgcatacagtctgccgccaacttctcgatgtgggccatgggcaggggggcctgccccttgggtgctggcttcttgcctgtggtttgtgcttcccctgtgagagccagcagctcagcctccaggtcctcatcatcttcagcctcatccatgcccagcagcatgtcctcagggccaaactccataaagagccccatctgcttggcagcggccaccccttggcctctggcctgagggcccttccgaggtcttggccctggcatcatggcagcctagatacctcgcggtgaatccgagccaaaccccggccttgtctcacccggcaccgccctgggctcccgcgggccctgggccgcagcggtagcgacaggaagcgccagcaggggaggtggctcgcgcgcaacacgtgaccccactggccggcggccggcagtgcgcatgtgcacggctacgcgggcggggggctccaacaggtgacaccggggcggggttcgcagcgcgca

SEQ ID NO: 14706 - RNA, 5823 nt, Homo sapiens
  source 1..5823: mol_type = other RNA
gctgggattacaggcatgagccaccgtgcctggccggtttctatttttataatgcaaaaataataatcatggcaatgggaattcagggattgtatgtagtcagaagggctaagaagtagggagaaatgatgccattttagagcctgggcagctgaggcagagaagaaacgaatccatctgtggagctgacccaggtgcaagctcccaggatctgccagtctcagtcgcatggtttcatcctgaaagcagctgcccttacttaagggacaaagtcttttaggagctgcccacaaatacttggaaaacaaggcttcaaaatccagaagcaacaatgcaaatttcagaatggtgctgtgagaaaggaaaaatgttagagtcacaggagtttgccctttaattgtaagcaagacttcttgattctaaaaaatttctgtagtttattcagtttgctaattcagaagaaagtgtgcattgcatgagatcaaagaattgaaaattttaaaatgatttgggttgtagctggctcccaactgcaggtgagtcactaatctccaatgtttggatactgtatttgtgtttgttttgagacagagtcttgctctgtcgcccaggctggagtgcagtggtacaatcgaggctcactgcaacctctgcttcctgggctcaagggattcgtgtgtctcagcctccctagtagctgggattacaggcgccggccaccatgcccagctaattgtttttgtttttagtggagacggggtttcaccatgttggccaggctggtcttgaattcctgacctcaggtgatccacctgcctcagctttccaaagtggtgggattacaggcgtgagccactgtgtcccgcctgtttcctgtatgtggataaatctcaggacaagatgaagctgggacaggctcctcctactaccagtgacgcatgcatgcctttggctacaacaaaggccttttaagaacttcaatctccaagtctggtgggaggctttgtcttgcctcgtcagcctggaggttctgttttgaaagagcaaagcagcagactgaaattgaatgggttgcaaaggagaaacctttagagctatagaaaactttctatctatcgaaataggccatttccaacagaggcctgaatttagaaactcctagagctggctggaactttagaggataaccacagtggtccgtaaccctcttaggaagcactgggttggatacacaccctaaggggagtaggttgggttaggaacccttccagtcacctttctttgctctataggtcatcttatgaaggctaatcaccctccttttcattctagattattgctgtgttgcatacacgtgactgcaattaagtgttaaatctcacatctgtggaagttttggtagctcacttctgataagattggccagccgggtgcggtggctcacacctgtaatcccagcactttgggaggctgaggtgggtggatcatgaggtcaggagttcgagaccagcctgaccaacatggtgaaacaccgtctctactaaaaataaaaaaattagctgggcatagtggtgggtgcctgtaatcccagctactcaggagactgacacaggagaatcgcttgaacctgggaggtgggggttgcagcgagctgagatcatgccactgcactccagcctggctggcagagagctactctgtctcaaaaaaaaaaaaaaaaaaaaaatcggccagagggctcatggggaaaaaagtcacttgtgtgtagttcccgctctgtgacccactaaaagctctgcgtttaagggcagggaagcatggtccagccctgttatcccccaaaaggacacatacaaagctcagttcttgagctgtgcttatgcaatactatagtgatcagtaagctgaatgtatttgcttcacttctaaccttttttaaaagtgatcttgaggaatgctttgttgatcttgaattaataattcaaaaagggggtgggggaagatggggtatttctaagaaatgcagaatatttcagttttgaatattaaatctcttacaactacaaaccccttcatagtctccatccattcagaaaaacaaagccaaaggagaatttcttgtggaaaaaaactaaggaagttccccacataaccagccgaagaggaaaggctttccctgtcctctctcaagaggaagccacagcagccgtttgtcatgttactgctaccctggcttttaaaaagtgacagggagcaggactttagattaggactttggtggatactctgtatagttgagtataaaatccctacaatgagttagacttagtttcctagataaataaacgtgtctacataaaattttatatatatattttttcttccagttaacagtcttttctcttgggtgggtagaccaaacccaagatccaaccttccccttacttcccaccaagtagtaccaaaaacaactttccccctccactaagtccttagggaagcaggaaggctagtgcagcagctgtcagggataaaggcacaggcagagctggggtgacggagttgtctgggacaggctaccactggcccactggagtcacggaaccctgacaccaccctcagcaggggaggttcccgatcaccctcaagttctcccatcccatagttagatcttttaaaggcacatctagaagtggtgcaactggaggcaggggtaagctgtacacagttgccacgcaggggttaaggggctgcaggactccatggtacagaggaatggaagtgtccttgccctcttccagactcggggcagggggagacagcggggagatgggctcctggaacccagcctgtttctgtagagccccagaggggccaacaacaggaaagaccagagtcgtggtcagtagtgcacatgcttaacaggtctttggtgcttgggtagcagcatctcttatgtacaaaggcttctgaagccagcaaagctgggaaagtcatctcctgcacagtcgcggcctgactcctctcctggtgctggccatcggctcacaagcccctgggctccagaaccagccagttctcagtgaccatctgcacatcctggccactcagaggctcccgcagcctcaccttcacctccagcttccccccggtgggcttccttccatccaggacctgtggaatccattgagttcatggaaacaaggaggctgccttctcctgggtccctctgtgagatttctcagaccttctgaacctctccatctccacaatttctctgatctcacactcattctccagccgctccagtttcaggtgtgctgtgccaaccagcttgtcgcttctgaagaaggaccctttgtggaagatctcaaacttgatgcctttgctctggatcaccctcttgaagccccggtggtttcggttgatgtttagtttgaagagttgatcaaattctggagagtttgtgttcttcaccacagctgttttgcttttttgagcctggtccgagttagggtagtgaaactcaaaccgcacaaaagcatccaggtcatcgggagtcacccctggaggggctgggaggttcattccccggacaatgatcagatgcatttctgtgctgttgagttctgagaagatcctcacagtctggaatgtcttcaactcaaagtggtgggtgggagggtcgaggccctgagcctgggccagctgcaggatctccagctgtttcttgcggtcctgagcaagcttctcaaatcgggtggtctcagccacgttgccctggtgcatgaactgcttggagaacagcaggcacttcttggacagatcaacaggtctgccagatcgggcctggatgatctgagcctcaagccatttggctacccgcagataggctttggcctgctccaggtcctggctgcgcttggcctgcagggctgcccgctgatactgcagtttccgtgcctccagcagtgccagctgctcccgcacagatggactcggtgactccttagaacttgaggccctgggctcaggcaggcgctgggatgaagggactgtgggccgtgcaggtttcttggccactggggcctgtgctgggggctcaccctgcaggtgcccaggaggctcgtcctcgtctttatcagccggggctgaatcctctgcagaggccagtttctctgcagctgccaatgtcgctgccactgcgtcctcctcaacacccatagtggactccaggccagggatggggggaaatcctggaggaacaggcaattcagcaaagttgactttccgtcctgctcggtgtgctcgaatagcatcttgatattgcttggcaatgcgctcatgcatccgagccttgcgctcgtccccaccactccgggcctggatgcccgcctcgcggtacttgttcagcctctgctgcagggcatccagcactgtctgtgactctgtaggggccactggggttgctgggacgtcaggggccatcactggctgcactcgctccacggctgggggaatgactgagggtgctgtgggagcctgagaagcctgctggggcttcagatcctcaggtgccgggggcatggcactcagatccacgggctgccccttctccagggcctccaggacagcaccgaatctcttcccaatcctcatgagctctcgggcacggtctagctctccagcccgcttggcactgagggcagccactttgtactctctctgtcgggatgacagcagggcccgcgggtctgggtctaagtctgaaacgggctgggcagaaatgccagggaggctggtctcaggttgggaggggttgtctgactccaaggcagggggagctggagggtctgtctcagggctcctgttggctggttcctggggggccaggggccgctttcctaaggccactggaggtgggatctcatcctcattgatctttctgcctctcctcacagaggctagctgcgactccaaggtcttcaggccgcgctcgcagcgcctggctttggctgcttcgcctgcctccttggcactggccgcagcctctcggtagttgtgaatccgttcctccagcaaagcgtgtagcccctgagatgctccggcctgagctgctggggctgaagctgtcaggacggctgtctgcactggaggttcagtgtcttctaggccgttctcctcctcagagccgcctgggtcagctacctcatcaccatccaggggctcagtctcctcgtccacacctaagacctcctgcagctccgtcagcagctctgcatcttcctccagcccttcctcctcctcctcctcctccacatcccgcatacagtctgccgccaacttctcgatgtgggccatgggcaggggggcctgccccttgggtgctggcttcttgcctgtggtttgtgcttcccctgtgagagccagcagctcagcctccaggtcctcatcatcttcagcctcatccatgcccagcagcatgtcctcagggccaaactccataaagagccccatctgcttggcagcggccaccccttggcctctggcctgagggcccttccgaggtcttggccctggcatcatggcagcctagatacctcgcggtgaatccgagccaaaccccggccttgtctcacccggcaccgccctgggctcccgcgggccctgggccgcagcggtagcgacaggaagcgccagcaggggaggtggctcgcgcgcaacacgtgaccccactggccggcggccggcagtgcgcatgtgcacggctacgcgggcggggggctccaacaggtgacaccggggcggggttcgcagcgcgca

SEQ ID NO: 14707 - RNA, 752 nt, Homo sapiens
  source 1..752: mol_type = other RNA
gctgggattacaggcatgagccaccgtgcctggcctaaaataattctttttaaggcccttctacaacaccccaaatgtagaactgagttgctgtattaaatttgacatttaaatcttggttaaaacaacaacaaaaaaagggataaagaatatttactgtgttttttgctttatttattcagagagtgaaactgtgttacagtgagctaaatttttagctgtacttagaatgtgctccctcctacatttcactctggaaaagtgaagtatcttatcatttcttagaaacctggatgtgaaactagtcaatattaagatcttatacacatcctgagtgatgcccaatttaaggctttgaatagctattcatgtaagttgacttttctgtgcatttgtatcggggaggatccagttcaggttgatgtcctgggaaccagtgaggctctcgcttaaatcctgggaaggcaagggtttgggctgcacgatattcctcaggtcatatctttcctggttccagttgcccatcagggtacggtttgaataggtattctcattagtggtgcatcgccatccatactggaaaaacttggacatattattccaatctgtccacacttcaccatggccatctgcattaacaaggctgccacagtgtgggtttgtgaggaaacaggcgaggttctgtctctggaagagaaattttgagcagcagagacactgggaggcagccatttcagacgaggtgaaaaaag

SEQ ID NO: 14708 - RNA, 819 nt, Homo sapiens
  source 1..819: mol_type = other RNA
gctgggattacaggcatgagccaccgtgcctggcctaaaataattctttttaaggcccttctacaacaccccaaatgtagaactgagttgctgtattaaatttgacatttaaatcttggttaaaacaacaacaaaaaaagggataaagaatatttactgtgttttttgctttatttattcagagagtgaaactgtgttacagtgagctaaatttttagctgtacttagaatgtgctccctcctacatttcactctggaaaagtgaagtatcttatcatttcttagaaacctggatgtgaaactagtcaatattaagatcttatacacatcctgagtgatgcccaatttaaggctttgaatagctattcatgtaagttgacttttctgtgcatttgtatcggggaggatccagttcaggttgatgtcctgggaaccagtgaggctctcgcttaaatctatgtgttgaaagtggcattttgttgttgtagcttgtatcatatgttgtttcaaagtagtgtccaaactgggaaggcaagggtttgggctgcacgatattcctcaggtcatatctttcctggttccagttgcccatcagggtacggtttgaataggtattctcattagtggtgcatcgccatccatactggaaaaacttggacatattattccaatctgtccacacttcaccatggccatctgcattaacaaggctgccacagtgtgggtttgtgaggaaacaggcgaggttctgtctctggaagagaaattttgagcagcagagacactgggaggcagccatttcagacgaggtgaaaaaag

SEQ ID NO: 14709 - RNA, 11949 nt, Homo sapiens
  source 1..11949: mol_type = other RNA
gctgggattacaggcatgagccaccgtgcctggcctaaactaactcttttacatttgttgagacagtgcacttctatttcaggagtcagatactcatctaagtatatattgtaaaagctgtatctatactaatatttttgtctgcttgatcaatagttgaaatcttccattatgatggtagacttgtcaaaacttccctatagttctgtcatttgtttttaacaagtctgttttgttaggtaggtagcagtttcaaattatacaatttgggtgatttaaaccttttttcattataaagtgactcatttacaatgcattctatcttagggaccattttagctgatgtatagctacttcagctttctcttggtcatatctacctacgacaagttgagcatccctaatctgaaaatccaaaatgctccaaaatctgaaacattttaagcaccaacatgatgctcaagggaaatacaccttttctgagttctaaatgttatatagtgcatagaactggatttgttgttgttgttgttttgttttagagacagagtctcactctgtgccccaggctggagtgcagtggcatgatcttggctcactgcaacctccacctcccaggttcaagcaactctcctgcctcagcttcccaagtagttgggattactggcatgtgccaccagacccagctaatttttgtatttttagtagagaccgggttttgccatgttggccagggtggtctggaactcctgatctcaggtgatccgcctgccttggcctcccaaagtgttgggattacaggcatgagccaccacacttggcctaaaactggatttttttttttttttttttttttttttttttttgagatgaagtctcgctctgtcgcccaggctggaatgcagtggcacgatctcggctcactgcaagcttcacctcctgggttcatgccattctcctgcctcagcctccggagtagctgggactataggcgcctgccaccatgcccggctaattttttgtatttttgtagagatgaggtttcaccgtgttggccaggatagtcttgatctcctgacctcgtgatccgcccccctcggcctccccaagtgctgagattatagacgtgagccatcgcgcctggctagaactggatatttaaaatccagtaaatatttggtaaatttactacatcccatatatttcaactagtaataaattcggatttacttgtcgtcatcttcttttgtgtttatgttagccttatttttctaattcggcagtccccaaccttgttggcaccagggactgatttttgtggaagacaatttttccactgatgcggtttttttcccatggatgggggccggggcgggcatggttttgggattaaactgttccacctcagaaaatcaggcagtagattctcataaggagcacgcaacctagatccctcacatgcgcagttcacaatagagtttgtgctgctgtgagaatctaatgcagcagctgatctgacaggaggcggtgctcagggtaggtttgccgctcgcttcctgctgtgcagccaggtcctgaacaggtcagggacaggcagcctgggggggttggggacctctgctgtgttgttttcccctgttgttcttgctgctactaaactgataaagctttctttattttccctctacaactttggaagttacacattttgattctttagtaattatgctaaaaaacgacagctttcatacttaaagcctaaagttaatcaagatctttatactctgctcccaaagaaatggaaagctcttagaacactgtaattctgatcactgaactactgttttcagcatcttttgtttttgagacagggtctcactctgttgcccagactggagtgcactagtgcaatgaatcatagctcactacagttttgaactctgggcttaagggatcctcctgcctctgcctgccaagtagctgggactacaggcatgctactgtgcatggccaacttttttattttttttagagaccaggtctcactatgttgcccaggctggtctcaaactcctgggctcaaacgatcctcctgccttggccttccaaagtgctgggattacaggtgtgaaccaccatgcccagccggtttttaattttttaatatgcctccaaaggagacattatcatggttttctactgttcatattgggttatatttgcccggatcttcatcagtcttttttgttaatcactgtctattatgtatcacttcttccttcattgagtttttaaaattcatgtggcatatatttcagtaggcttttcagtgagggtctgttatcctgaagtctctcagtctttgagaagtctttaattcactttcattcttggatgataactagaaatcaaattccagattgacagttatttttctctattattttgaagctactgtattgtctctgatttctatggctgctatggagaacttctaccagcaggttagattcttgtgggtaaactctctttttctttctggttgcttttaagctttttctctttgtctctgttgttctgcagtattatttttatttatccctggctcgctgcatttcctaaatgtgaagattcatgtctcattaatcattttcagccattatcacttttaatattgccttgctcccctactcgattctctcctcctagaacttctacaggacatacgctgaatattctcattcaatttttcatgcctcttaacacgtattctccatcactactccattcttgctaatttccccaacttcattttatagtttattcttttttttttttttttgagatggagtctcactctgtcacccacactggagtgcaatggcacgatcttggctcactgcaacctccacctcccgggttcaagcgattctcctgcttcagcctctcaagtagctgggattacaggtgcacgccaccaggcccagctaattttttttgttttttttaatagagacagggtttcaccatgtgtaccaggttggtcttgaactcctgacctcatggtccacccgcctcagcctcccaaagtgctaggattacaggcatgagccaccgcgcccagtccggtttattcattttctgtgtcctaatatcttcattaagttaatttccagtacagttgtacctcagtatctgcagggagttggttccaggatccctttgactatcaaaatccacagatgctcaagggccctatataaaatggtgtcttttctggtgttttttgtttttgttttttgagacaaggtctcattctgttgccaggctggagagcagtggctcagtcacagctcactgtagcctcgacctcctgggctcaggtgattctcccacctcaacctaccaagtagctgggactataggcacgtgccactatgcctggtcaatttttgtattttgtgtagacagggttttgccatgttgcccaggctggtctacaactcctgggctcaagcagtctgcccacctccatcccccaaaaacgttgggattacacgtgtgagccaccatgccaggcctggagtagtatttgcatgtaacctatgcacatcctcccatatactttaagtcatctctggattacttataatatctaatacaatataaatactatgtaaatagttgttacactgtattttaaaatatgtatatttttattgttgtattattttttcaaatctttcccatcacattagttgattctgaagatgcagagcccgtaaatatggacggccaactatgttgtatttctcatttctgaaaattctatttagtttctaaagtttgtttccttcttctaaatatatttaaatatactttatttgtagcctctgcttaataattctattatctaaagtccttgggggtttaaatcttattgccttctgactcttatgataaattgtttccttgcatgttctattattttgaattgtgatctcaacttcattggggtttcatatgtggatatcctgttaggtctgagttaacatgcaacaatctagaaattctgtttccttctggcaactgccctagaaatacttttcatattaagttcacaggattcgcagaccacacaggtagtataaatttgaatcccaaactggtgaaaaggtaggtctatggtgacaaattcccaggaatgacttttattctctgtaccatgagtccaagctaacacaagcactagagggtggattttgttttttaatccttccattgagggtgaatgtctttaaaggtcctggctttgtatgtggatctcaatccaacttctcaccttgtaggggggcctaagactttacctcgagtgtccttgcgtgacctttaaaacccgagcatactggttacagaaactagggactgtctttacgcccaggcagtcacaaagcataaaccacacaccatactgttgttaaatttcctgtttagggctccgcccaggctggaatgcaatggcatgatctcagctcactgcaacctccatctcccaggttcaaatgattctgcctcagcctcccaagtagctgggattaccggcatgcgccaccatgcccagctaatttttatatttttagaagagatggattttcaccatgttggccaggctagtctcaaactcctgacctcaagtgatccgcctgcctcagcctcccaaagtgctgggattacaggcgtgagccaccaggcctggcggaaccttgatcttttaaatgtgaatttcagatatttctattacctgtaaggagagaggtggggaagacgaaggttgaagggaatattgaataaataactcctgtgtactagccctcaatacatgagatatttgataacagctatacaaaacaagccatgttaatagatgagaaattaaagctcagaaaggtcaaataatttcgctaaggtcacaatgtactattacacccgaattcacgttggaattaactagtcagatccattttcattctggacatggtggtgtatgcctgtagtcccagctatttgggggcctgaagtgagaggactgcttgtgcctaggaattcatgtacagcctgggcaacatagcaagaaactgcttctaaaaataaataggctgggtgcagtggctcacgcctgtaatcccagcactttgggaggtggaggcaggtggatcacttgaggtcaggagttcaagaccagcctggccaacacggcgaaaccccatctctactaaaaatacaaaaaattagctgggtgtggtggtgcgtgcctgtaatcccagttacttgggaggctgaggcaggagaagagctttaacccaggaagcagaggttgtggtgagctgagatcacgtcactgcactccagcctgggcaacagagcaagactctgtctcaaataaaaataaataactttgggaggccgaagtgggaggatcccgaggtcgagatcgagaccatcctggctaacacagtgaaaccccatctctactaaaaatacaaaaaattagctgggcatggtggcaggcacctgtagtctcccagctacttggaaggctgaggcagaagaattgcttgaacctgggaggcggaggttgcagtgagccgagatcgtgccactgcattccagcctgggcaacagagagagactccatctcaaaaaattaaaaataagttaacaaataatcaattttcttcctctacagcagaggtcagcaaacttattctgttaaaggccaaacagtaaatattttaggcctcataagccatatggtattggctgcaactattcagttttactgttgtatcattaaagcagccactgaaaagtgtaaacaaatgagcatgactgtgttcccataaaactttaaggacattgacatttgaatttcataaaattttcacatataacaatactattattacttggatcttttccccaaccatataaaaatttaaaacccgttgctaatgcatgggtcttacaaaaacagcctggagttgacccacgggccgtggtttgctgacccttatcatacaccataacacctccttggaagtacacctctctaatgcctttgttccaaacaatactgggttaggaaagacatggaaaaaggaaaatgagatacattattttttgtaccctatgggggattgaggggttgttgctacatagccccctcaatttgtgctgtagcaatatgcagttaagatccttattctaatgttaaatgtctcttctgtggcttatcctaactttaaaaaaaaaaaaaagaagccatcttacgtaaatgaacttacaattttaagacagggtctcactctgtcacccaggctggagtgcagtggtacaatcacggctcattgcagcctcgacctctcaggctcgagagatcctcccaccccaacttcccaagtagctgggactacaggtgtgcaccactatgcctagctcatcttttttttttttttttttttcctttaaaagatatggagtctcgctattttgcccaggctggtcttgaactcctggactcaagcaatccacctgcctcagcctcccagagtgttgggattacaggtgtgagccactgtgcccggcctgaattatcttcttattgtaaaatttcctttaatgcttaatagttgatgtatattaagtgctaactaaatgttcactgataaacattaatcagatgctgctaaatattgtctttctttattcacagatgatagtcaatgggcacaacatataagtagttacaatgaaatgagaagcaatatagcagtcaggctatatgcatgatttaacaacaaaattatcacttccttttaatttagaataagggacaatttaaaaagcatctcttggccctatcatttctgttccagtagttagtgttcatatgtgaatactaagtttgacattcctttctcccatagaaccattttggtgatttggatggtggccactacactgctttctgcaagaattcagtcacccaggcctgatatagctttgataacacacgagtcagtgagattccagatacttctgttcaaaatgctatggatctcctgttctatagctgccagcccttttccataccaatacaaaagcgttaagagccaggaaaatggtgtttcctgaacactgcaaaacaagcagtcagcatctggtggtagagttttgcttggtcattaaactcttagaacttacttgcatcattaacatttttatgccttgtgggcatgttatacaacctttcatcttaagataaatctgtcgtccagaagatgggtcttggttcactaaaaaaggcagtgtgaatataatgcaatgctaatggatgcaggccttcaaaacactgcaattatatagtgagttcaggtttcaaaattcagtgtttatcagaaaatatctcataatcatatatattcaacaaattattttccaaagatactcatgaagctaaacaaaaataatttttgttcaaatggctcgatgagtttaagaatatgatttgaatatatttgatataataatttagccaagaagtggtctcttagactaattgtaaaacatgaaaagttgtcagcttcacaatttgaaccccatcctttcatcttctccctgagagcctgctaatggtggtctctttctgaagcacttttagaatcttatttttatatggagtgttttactgactatatatatagcaactgagtccctcggttaaataaattataagctcctttaaccctcttaatacatcactctgtaaagatgtagtttataatgcagttcactttgcaatcatgcctgactcccggcatttttactttaatatttagaatgaatattctcaatatgtgagaatactagtcttgaaagaatgactctgggtgttattatatagcacgtgtgtatataaaatctatggttttactgtcctatatttgataatacaatattaaagacagaacacccacagggttataaattatttttctcattaagattttaatgtagctgtaaatgaaattctcgttttaaaaaaattaaagtttccatttttttttttagaataaagatttagtgcacaaatacagcccaaagccaacagaaaaattgctttgccctgtcatttccctaagaaagcactgaagttaactcaaaataggctgaaagaaaaaaagcaatcctctgagttctaggtttcacaaaaggaccacgtgttaaactatgtacatcgatttgatgtgcaagtatgcaataaatatgtacacatacattcctatctgctttacatcattctagagtattcatagtatatcaagatgggatttagaaatgtgaaaaggccataacagtgaaaaggaaaaaaaaaagataacaatagtttttagaccagtcgaataataatgcttagctagttaattattttaactttggagcagactaaaaaagttgttttgaaataaatggtacctgtaagtgatgattactgcaatacttgttaaatgttatttgtcagcactgaccggaattatatagtgctagtaacacagctcccactgtcctagaattcctctaaatggccagctatagctaccattatcctgataagcatttcaagagttgtgttgctgagccttttaaaagataactagtttataacctatgtctccttatgtggctacatcagttactcgtggtcccaatgaagtataaaagaggatataagctgctgaagatttcacagaagaaacggagatatcagaaacttcatgatcatcaaacttaaaccaccgttgtcttgctgcatttttacaataggctgtgtagtggcctccatccagcccaccgtagtgatttgaaacagaaaacaaattatatttcttcaaattgttctttggaccaataacatactgtgacaagtcaagattttctaacgggaagtccacagatgtctgtaatttttgtttccacctgccatcgtaggaaaaacgtttcagatgcactaaaagcacaggtggtaacttccagatttctatcttttttagagaatcccgtcgagctctgcaatgactgcagtaaaatctgttgttatctgtgagtttttcttctttggaaaataatctaaggcaatcctgtaatgtacatttacttgtggatgctagtggtagagacaaatacatgaaggcctcaaatgtcctagactttttgtgacatgtgaggcactgtactgtagatttgaattgaccctgaaaaagtgcaacaataatagactcattgagctgcttgtgtttctgccaggcatgttctgcagctttaaagtcatcgagatgatcattattttcttctttatatctcttccgattatcagctttatttagatcttcatggagaccatccattaggaacagaagcaattcttgtgaatcttgctgactgtatcctgcaaactggtcattgatcttcccaatggtgattttaaagtcctttggactgatatatctatactgtcctgtccacagggctttcatgattataccaaattcttctgccacttcacctttatgccccaacaaatttgacctgttaatatcatcctgataacagtttcggttgaaataatcagccaaatgtggagcgttacataggcactgcaatattgagttcatataacaagtatttcctaagttacgaagtccagtaagagctggtccagaacctccaaaaacaggattgaggttccgaatctgagaagcagaaagccttgagatctcagctttaggataacatgttggcttgttttcccgattaactgttggagttactgttggcttcctcttctcttcctcttgaatagcctgggttatatctggggaggagtaggagcgcttcagtttggaaggttccctatcccgctcagcaggaatctgtggcttggctttatgagttggaggggtggaaggaggtgcagatgaaggagccatttccggtgggtacatatgaacagtgttggtgggtgaatgataataacgaaaggttccagtgattgggtcaagaaacttggcccagcctgaaggcagtcctggtacgatcctccccatttcttcacttcgtgctcttgtcaaaggttctcgttgagccttgcctgaacctgaatcccctgtcacagatgtatggggcacatctcctgttgactttttctgtatttctggggttggacaccttttccccctatcttctacagatttcttggcatcagaagtttcatgttcacttttactttgtctttttactcctgttatttctttgcccctctttgctgaggtttctttatcttctttcttggcctgttcactttctttcttctccatttcttcttttgctttttgttgcttctctgtaatttcattttcttcagcttcttgtttctttttggctttttgttcttgttcttccttcctcagtttctctttctgttcctcttgctgcctttcccgaagttctttttcttgtttgtttttttccattagaagagcagtttctgcatgaatacgagccttttcttcatctgttaacatgagagttggagaaaaaactactggcttggtggaacgatcaggaataacttttccactctgaggagattgttgctcatggtttgtactttcagattttattctatgctcttcaggcaatttgactgctggttttttagtacgatcaatctgtggaacattctttatactaggcactggctgaattatgggtgaaacatcagatttagaagcagcaactggttcaactggagttgatatattcagtggtcccattctctcattttgaccacttatcaattctatattttcatctacttctatagatgcaggtggcgtctgggcagcaggtttagaaggaattgattcttccaatgagggataagtaaaatccaatgagatagacacctcttcattctggcgtcgtgggggtggagtgaccttagcatttgttgtatactggggataacaaaggagccagttttcatagcctccctctaaaaccaaaggctcattgcgcaggacagttttactttcccacttgaaaagtgcatctttcagactccggagagttgttccaatctgtaaatctttggcagaactaaaccagtcaagaagtaccacatactccacattccccctcttcttccatgtgtctttagaatcatctggcaggtgtgcttcaatccaactagcagtgactcctggactgatggcttcttcaggaacactgagagaatgtaaaatacaggaatcctgataatcctgcattcttcgagcatccattataatcaagctgatgtttttatccgtcatcattgtgtatagttcctttgctgtgattgctcctttctctttggtctcacatttttcattcttttcaccattgctcttttgggttttgtctttggaatccaaaacattctccaaagagcctttagccaatgtgccaccatcctctcttcctgtttcctgccttttttgttgtagccgctgtgcttcctcctgcctgtctttttcctcaagttttttccggacttcagcttcttcatatctcttagtgcttattttctctggtttaacttctgtcttcttattaaggtcttttagtgaagaactgaggtagagttctttaggaactgaagccacagcaggcatgatgaattatctttacttttccactttcacaatggatgctatatttccttacaagtgcttctttccgtgacgccgggcgcgcttcactaacgccagccttctcgccaaatgcccatctcccaagaactcgagggagaattagccttggctaccaggacggaagccagcccagctc

SEQ ID NO: 14710 - RNA, 12267 nt, Homo sapiens
  source 1..12267: mol_type = other RNA
gctgggattacaggcatgagccaccgtgcctggcctaaactaactcttttacatttgttgagacagtgcacttctatttcaggagtcagatactcatctaagtatatattgtaaaagctgtatctatactaatatttttgtctgcttgatcaatagttgaaatcttccattatgatggtagacttgtcaaaacttccctatagttctgtcatttgtttttaacaagtctgttttgttaggtaggtagcagtttcaaattatacaatttgggtgatttaaaccttttttcattataaagtgactcatttacaatgcattctatcttagggaccattttagctgatgtatagctacttcagctttctcttggtcatatctacctacgacaagttgagcatccctaatctgaaaatccaaaatgctccaaaatctgaaacattttaagcaccaacatgatgctcaagggaaatacaccttttctgagttctaaatgttatatagtgcatagaactggatttgttgttgttgttgttttgttttagagacagagtctcactctgtgccccaggctggagtgcagtggcatgatcttggctcactgcaacctccacctcccaggttcaagcaactctcctgcctcagcttcccaagtagttgggattactggcatgtgccaccagacccagctaatttttgtatttttagtagagaccgggttttgccatgttggccagggtggtctggaactcctgatctcaggtgatccgcctgccttggcctcccaaagtgttgggattacaggcatgagccaccacacttggcctaaaactggatttttttttttttttttttttttttttttttttgagatgaagtctcgctctgtcgcccaggctggaatgcagtggcacgatctcggctcactgcaagcttcacctcctgggttcatgccattctcctgcctcagcctccggagtagctgggactataggcgcctgccaccatgcccggctaattttttgtatttttgtagagatgaggtttcaccgtgttggccaggatagtcttgatctcctgacctcgtgatccgcccccctcggcctccccaagtgctgagattatagacgtgagccatcgcgcctggctagaactggatatttaaaatccagtaaatatttggtaaatttactacatcccatatatttcaactagtaataaattcggatttacttgtcgtcatcttcttttgtgtttatgttagccttatttttctaattcggcagtccccaaccttgttggcaccagggactgatttttgtggaagacaatttttccactgatgcggtttttttcccatggatgggggccggggcgggcatggttttgggattaaactgttccacctcagaaaatcaggcagtagattctcataaggagcacgcaacctagatccctcacatgcgcagttcacaatagagtttgtgctgctgtgagaatctaatgcagcagctgatctgacaggaggcggtgctcagggtaggtttgccgctcgcttcctgctgtgcagccaggtcctgaacaggtcagggacaggcagcctgggggggttggggacctctgctgtgttgttttcccctgttgttcttgctgctactaaactgataaagctttctttattttccctctacaactttggaagttacacattttgattctttagtaattatgctaaaaaacgacagctttcatacttaaagcctaaagttaatcaagatctttatactctgctcccaaagaaatggaaagctcttagaacactgtaattctgatcactgaactactgttttcagcatcttttgtttttgagacagggtctcactctgttgcccagactggagtgcactagtgcaatgaatcatagctcactacagttttgaactctgggcttaagggatcctcctgcctctgcctgccaagtagctgggactacaggcatgctactgtgcatggccaacttttttattttttttagagaccaggtctcactatgttgcccaggctggtctcaaactcctgggctcaaacgatcctcctgccttggccttccaaagtgctgggattacaggtgtgaaccaccatgcccagccggtttttaattttttaatatgcctccaaaggagacattatcatggttttctactgttcatattgggttatatttgcccggatcttcatcagtcttttttgttaatcactgtctattatgtatcacttcttccttcattgagtttttaaaattcatgtggcatatatttcagtaggcttttcagtgagggtctgttatcctgaagtctctcagtctttgagaagtctttaattcactttcattcttggatgataactagaaatcaaattccagattgacagttatttttctctattattttgaagctactgtattgtctctgatttctatggctgctatggagaacttctaccagcaggttagattcttgtgggtaaactctctttttctttctggttgcttttaagctttttctctttgtctctgttgttctgcagtattatttttatttatccctggctcgctgcatttcctaaatgtgaagattcatgtctcattaatcattttcagccattatcacttttaatattgccttgctcccctactcgattctctcctcctagaacttctacaggacatacgctgaatattctcattcaatttttcatgcctcttaacacgtattctccatcactactccattcttgctaatttccccaacttcattttatagtttattcttttttttttttttttgagatggagtctcactctgtcacccacactggagtgcaatggcacgatcttggctcactgcaacctccacctcccgggttcaagcgattctcctgcttcagcctctcaagtagctgggattacaggtgcacgccaccaggcccagctaattttttttgttttttttaatagagacagggtttcaccatgtgtaccaggttggtcttgaactcctgacctcatggtccacccgcctcagcctcccaaagtgctaggattacaggcatgagccaccgcgcccagtccggtttattcattttctgtgtcctaatatcttcattaagttaatttccagtacagttgtacctcagtatctgcagggagttggttccaggatccctttgactatcaaaatccacagatgctcaagggccctatataaaatggtgtcttttctggtgttttttgtttttgttttttgagacaaggtctcattctgttgccaggctggagagcagtggctcagtcacagctcactgtagcctcgacctcctgggctcaggtgattctcccacctcaacctaccaagtagctgggactataggcacgtgccactatgcctggtcaatttttgtattttgtgtagacagggttttgccatgttgcccaggctggtctacaactcctgggctcaagcagtctgcccacctccatcccccaaaaacgttgggattacacgtgtgagccaccatgccaggcctggagtagtatttgcatgtaacctatgcacatcctcccatatactttaagtcatctctggattacttataatatctaatacaatataaatactatgtaaatagttgttacactgtattttaaaatatgtatatttttattgttgtattattttttcaaatctttcccatcacattagttgattctgaagatgcagagcccgtaaatatggacggccaactatgttgtatttctcatttctgaaaattctatttagtttctaaagtttgtttccttcttctaaatatatttaaatatactttatttgtagcctctgcttaataattctattatctaaagtccttgggggtttaaatcttattgccttctgactcttatgataaattgtttccttgcatgttctattattttgaattgtgatctcaacttcattggggtttcatatgtggatatcctgttaggtctgagttaacatgcaacaatctagaaattctgtttccttctggcaactgccctagaaatacttttcatattaagttcacaggattcgcagaccacacaggtagtataaatttgaatcccaaactggtgaaaaggtaggtctatggtgacaaattcccaggaatgacttttattctctgtaccatgagtccaagctaacacaagcactagagggtggattttgttttttaatccttccattgagggtgaatgtctttaaaggtcctggctttgtatgtggatctcaatccaacttctcaccttgtaggggggcctaagactttacctcgagtgtccttgcgtgacctttaaaacccgagcatactggttacagaaactagggactgtctttacgcccaggcagtcacaaagcataaaccacacaccatactgttgttaaatttcctgtttagggctccgcccaggctggaatgcaatggcatgatctcagctcactgcaacctccatctcccaggttcaaatgattctgcctcagcctcccaagtagctgggattaccggcatgcgccaccatgcccagctaatttttatatttttagaagagatggattttcaccatgttggccaggctagtctcaaactcctgacctcaagtgatccgcctgcctcagcctcccaaagtgctgggattacaggcgtgagccaccaggcctggcggaaccttgatcttttaaatgtgaatttcagatatttctattacctgtaaggagagaggtggggaagacgaaggttgaagggaatattgaataaataactcctgtgtactagccctcaatacatgagatatttgataacagctatacaaaacaagccatgttaatagatgagaaattaaagctcagaaaggtcaaataatttcgctaaggtcacaatgtactattacacccgaattcacgttggaattaactagtcagatccattttcattctggacatggtggtgtatgcctgtagtcccagctatttgggggcctgaagtgagaggactgcttgtgcctaggaattcatgtacagcctgggcaacatagcaagaaactgcttctaaaaataaataggctgggtgcagtggctcacgcctgtaatcccagcactttgggaggtggaggcaggtggatcacttgaggtcaggagttcaagaccagcctggccaacacggcgaaaccccatctctactaaaaatacaaaaaattagctgggtgtggtggtgcgtgcctgtaatcccagttacttgggaggctgaggcaggagaagagctttaacccaggaagcagaggttgtggtgagctgagatcacgtcactgcactccagcctgggcaacagagcaagactctgtctcaaataaaaataaataactttgggaggccgaagtgggaggatcccgaggtcgagatcgagaccatcctggctaacacagtgaaaccccatctctactaaaaatacaaaaaattagctgggcatggtggcaggcacctgtagtctcccagctacttggaaggctgaggcagaagaattgcttgaacctgggaggcggaggttgcagtgagccgagatcgtgccactgcattccagcctgggcaacagagagagactccatctcaaaaaattaaaaataagttaacaaataatcaattttcttcctctacagcagaggtcagcaaacttattctgttaaaggccaaacagtaaatattttaggcctcataagccatatggtattggctgcaactattcagttttactgttgtatcattaaagcagccactgaaaagtgtaaacaaatgagcatgactgtgttcccataaaactttaaggacattgacatttgaatttcataaaattttcacatataacaatactattattacttggatcttttccccaaccatataaaaatttaaaacccgttgctaatgcatgggtcttacaaaaacagcctggagttgacccacgggccgtggtttgctgacccttatcatacaccataacacctccttggaagtacacctctctaatgcctttgttccaaacaatactgggttaggaaagacatggaaaaaggaaaatgagatacattattttttgtaccctatgggggattgaggggttgttgctacatagccccctcaatttgtgctgtagcaatatgcagttaagatccttattctaatgttaaatgtctcttctgtggcttatcctaactttaaaaaaaaaaaaaagaagccatcttacgtaaatgaacttacaattttaagacagggtctcactctgtcacccaggctggagtgcagtggtacaatcacggctcattgcagcctcgacctctcaggctcgagagatcctcccaccccaacttcccaagtagctgggactacaggtgtgcaccactatgcctagctcatcttttttttttttttttttttcctttaaaagatatggagtctcgctattttgcccaggctggtcttgaactcctggactcaagcaatccacctgcctcagcctcccagagtgttgggattacaggtgtgagccactgtgcccggcctgaattatcttcttattgtaaaatttcctttaatgcttaatagttgatgtatattaagtgctaactaaatgttcactgataaacattaatcagatgctgctaaatattgtctttctttattcacagatgatagtcaatgggcacaacatataagtagttacaatgaaatgagaagcaatatagcagtcaggctatatgcatgatttaacaacaaaattatcacttccttttaatttagaataagggacaatttaaaaagcatctcttggccctatcatttctgttccagtagttagtgttcatatgtgaatactaagtttgacattcctttctcccatagaaccattttggtgatttggatggtggccactacactgctttctgcaagaattcagtcacccaggcctgatatagctttgataacacacgagtcagtgagattccagatacttctgttcaaaatgctatggatctcctgttctatagctgccagcccttttccataccaatacaaaagcgttaagagccaggaaaatggtgtttcctgaacactgcaaaacaagcagtcagcatctggtggtagagttttgcttggtcattaaactcttagaacttacttgcatcattaacatttttatgccttgtgggcatgttatacaacctttcatcttaagataaatctgtcgtccagaagatgggtcttggttcactaaaaaaggcagtgtgaatataatgcaatgctaatggatgcaggccttcaaaacactgcaattatatagtgagttcaggtttcaaaattcagtgtttatcagaaaatatctcataatcatatatattcaacaaattattttccaaagatactcatgaagctaaacaaaaataatttttgttcaaatggctcgatgagtttaagaatatgatttgaatatatttgatataataatttagccaagaagtggtctcttagactaattgtaaaacatgaaaagttgtcagcttcacaatttgaaccccatcctttcatcttctccctgagagcctgctaatggtggtctctttctgaagcacttttagaatcttatttttatatggagtgttttactgactatatatatagcaactgagtccctcggttaaataaattataagctcctttaaccctcttaatacatcactctgtaaagatgtagtttataatgcagttcactttgcaatcatgcctgactcccggcatttttactttaatatttagaatgaatattctcaatatgtgagaatactagtcttgaaagaatgactctgggtgttattatatagcacgtgtgtatataaaatctatggttttactgtcctatatttgataatacaatattaaagacagaacacccacagggttataaattatttttctcattaagattttaatgtagctgtaaatgaaattctcgttttaaaaaaattaaagtttccatttttttttttagaataaagatttagtgcacaaatacagcccaaagccaacagaaaaattgctttgccctgtcatttccctaagaaagcactgaagttaactcaaaataggctgaaagaaaaaaagcaatcctctgagttctaggtttcacaaaaggaccacgtgttaaactatgtacatcgatttgatgtgcaagtatgcaataaatatgtacacatacattcctatctgctttacatcattctagagtattcatagtatatcaagatgggatttagaaatgtgaaaaggccataacagtgaaaaggaaaaaaaaaagataacaatagtttttagaccagtcgaataataatgcttagctagttaattattttaactttggagcagactaaaaaagttgttttgaaataaatggtacctgtaagtgatgattactgcaatacttgttaaatgttatttgtcagcactgaccggaattatatagtgctagtaacacagctcccactgtcctagaattcctctaaatggccagctatagctaccattatcctgataagcatttcaagagttgtgttgctgagccttttaaaagataactagtttataacctatgtctccttatgtggctacatcagttactcgtggtcccaatgaagtataaaagaggatataagctgctgaagatttcacagaagaaacggagatatcagaaacttcatgatcatcaaacttaaaccaccgttgtcttgctgcatttttacaataggctgtgtagtggcctccatccagcccaccgtagtgatttgaaacagaaaacaaattatatttcttcaaattgttctttggaccaataacatactgtgacaagtcaagattttctaacgggaagtccacagatgtctgtaatttttgtttccacctgccatcgtaggaaaaacgtttcagatgcactaaaagcacaggtggtaacttccagatttctatcttttttagagaatcccgtcgagctctgcaatgactgcagtaaaatctgttgttatctgtgagtttttcttctttggaaaataatctaaggcaatcctgtaatgtacatttacttgtggatgctagtggtagagacaaatacatgaaggcctcaaatgtcctagactttttgtgacatgtgaggcactgtactgtagatttgaattgaccctgaaaaagtgcaacaataatagactcattgagctgcttgtgtttctgccaggcatgttctgcagctttaaagtcatcgagatgatcattattttcttctttatatctcttccgattatcagctttatttagatcttcatggagaccatccattaggaacagaagcaattcttgtgaatcttgctgactgtatcctgcaaactggtcattgatcttcccaatggtgattttaaagtcctttggactgatatatctatactgtcctgtccacagggctttcatgattataccaaattcttctgccacttcacctttatgccccaacaaatttgacctgttaatatcatcctgataacagtttcggttgaaataatcagccaaatgtggagcgttacataggcactgcaatattgagttcatataacaagtatttcctaagttacgaagtccagtaagagctggtccagaacctccaaaaacaggattgaggttccgaatctgagaagcagaaagccttgagatctcagctttaggataacatgttggcttgttttcccgattaactgttggagttactgttggcttcctcttctcttcctcttgaatagcctgggttatatctggggaggagtaggagcgcttcagtttggaaggttccctatcccgctcagcaggaatctgtggcttggctttatgagttggaggggtggaaggaggtgcagatgaaggagccatttccggtgggtacatatgaacagtgttggtgggtgaatgataataacgaaaggttccagtgattgggtcaagaaacttggcccagcctgaaggcagtcctggtacgatcctccccatttcttcacttcgtgctcttgtcaaaggttctcgttgagctttatttctttcggtatcgtctgtatcctctctaaaagttcctgtccttagaattccactttctggttgtcctttaatcttaaatggcttgcctgaacctgaatcccctgtcacagatgtatggggcacatctcctgttgactttttctgtatttctggggttggacaccttttccccctatcttctacagatttcttggcatcagaagtttcatgttcacttttactttgtctttttactcctgttatttctttgcccctctttgctgaggtttctttatcttctttcttggcctgttcactttctttcttctccatttcttcttttgctttttgttgcttctctgtaatttcattttcttcagcttcttgtttctttttggctttttgttcttgttcttccttcctcagtttctctttctgttcctcttgctgcctttcccgaagttctttttcttgtttgtttttttccattagaagagcagtttctgcatgaatacgagccttttcttcatctgttaacatgagagttggagaaaaaactactggcttggtggaacgatcaggaataacttttccactctgaggagattgttgctcatggtttgtactttcagattttattctatgctcttcaggcaatttgactgctggttttttagtacgatcaatctgtggaacattctttatactaggcactggctgaattatgggtgaaacatcagatttagaagcagcaactggttcaactggagttgatatattcagtggtcccattctctcattttgaccacttatcaattctatattttcatctacttctatagatgcaggtggcgtctgggcagcaggtttagaaggaattgattcttccaatgagggataagtaaaatccaatgagatagacacctcttcattctggcgtcgtgggggtggagtgaccttagcatttgttgtatactggggataacaaaggagccagttttcatagcctccctctaaaaccaaaggctcattgcgcaggacagttttactttcccacttgaaaagtgcatctttcagactccggagagttgttccaatctgtaaatctttggcagaactaaaccagtcaagaagtaccacatactccacattccccctcttcttccatgtgtctttagaatcatctggcaggtgtgcttcaatccaactagcagtgactcctggactgatggcttcttcaggaacactgagagaatgtaaaatacaggaatcctgataatcctgcattcttcgagcatccattataatcaagctgatgtttttatccgtcatcattgtgtatagttcctttgctgtgattgctcctttctctttggtctcacatttttcattcttttcaccattgctcttttgggttttgtctttggaatccaaaacattctccaaagagcctttagccaatgtgccaccatcctctcttcctgtttcctgccttttttgttgtagccgctgtgcttcctcctgcctgtctttttcctcaagttttttccggacttcagcttcttcatatcttaatttaaggctttcagagagtctttcagcttcttcgacagcttttttgatgtttccaggtccaagtattgaatggaaataatcctgctgttgcttgaaatcaggtctttttttgataagattataaacagtcacgtatttcatatatagtacataggccctttcctcatcacgatctaatctgcattcttctgctgtcttaaagatcttcagggcactgtgcacataactcttagtgcttattttctctggtttaacttctgtcttcttattaaggtcttttagtgaagaactgaggtagagttctttaggaactgaagccacagcaggcatgatgaattatctttacttttccactttcacaatggatgctatatttccttacaagtgcttctttccgtgacgccgggcgcgcttcactaacgccagccttctcgccaaatgcccatctcccaagaactcgagggagaattagccttggctaccaggacggaagccagcccagctc

SEQ ID NO: 14711 - RNA, 12407 nt, Homo sapiens
  source 1..12407: mol_type = other RNA
gctgggattacaggcatgagccaccgtgcctggcctaaactaactcttttacatttgttgagacagtgcacttctatttcaggagtcagatactcatctaagtatatattgtaaaagctgtatctatactaatatttttgtctgcttgatcaatagttgaaatcttccattatgatggtagacttgtcaaaacttccctatagttctgtcatttgtttttaacaagtctgttttgttaggtaggtagcagtttcaaattatacaatttgggtgatttaaaccttttttcattataaagtgactcatttacaatgcattctatcttagggaccattttagctgatgtatagctacttcagctttctcttggtcatatctacctacgacaagttgagcatccctaatctgaaaatccaaaatgctccaaaatctgaaacattttaagcaccaacatgatgctcaagggaaatacaccttttctgagttctaaatgttatatagtgcatagaactggatttgttgttgttgttgttttgttttagagacagagtctcactctgtgccccaggctggagtgcagtggcatgatcttggctcactgcaacctccacctcccaggttcaagcaactctcctgcctcagcttcccaagtagttgggattactggcatgtgccaccagacccagctaatttttgtatttttagtagagaccgggttttgccatgttggccagggtggtctggaactcctgatctcaggtgatccgcctgccttggcctcccaaagtgttgggattacaggcatgagccaccacacttggcctaaaactggatttttttttttttttttttttttttttttttttgagatgaagtctcgctctgtcgcccaggctggaatgcagtggcacgatctcggctcactgcaagcttcacctcctgggttcatgccattctcctgcctcagcctccggagtagctgggactataggcgcctgccaccatgcccggctaattttttgtatttttgtagagatgaggtttcaccgtgttggccaggatagtcttgatctcctgacctcgtgatccgcccccctcggcctccccaagtgctgagattatagacgtgagccatcgcgcctggctagaactggatatttaaaatccagtaaatatttggtaaatttactacatcccatatatttcaactagtaataaattcggatttacttgtcgtcatcttcttttgtgtttatgttagccttatttttctaattcggcagtccccaaccttgttggcaccagggactgatttttgtggaagacaatttttccactgatgcggtttttttcccatggatgggggccggggcgggcatggttttgggattaaactgttccacctcagaaaatcaggcagtagattctcataaggagcacgcaacctagatccctcacatgcgcagttcacaatagagtttgtgctgctgtgagaatctaatgcagcagctgatctgacaggaggcggtgctcagggtaggtttgccgctcgcttcctgctgtgcagccaggtcctgaacaggtcagggacaggcagcctgggggggttggggacctctgctgtgttgttttcccctgttgttcttgctgctactaaactgataaagctttctttattttccctctacaactttggaagttacacattttgattctttagtaattatgctaaaaaacgacagctttcatacttaaagcctaaagttaatcaagatctttatactctgctcccaaagaaatggaaagctcttagaacactgtaattctgatcactgaactactgttttcagcatcttttgtttttgagacagggtctcactctgttgcccagactggagtgcactagtgcaatgaatcatagctcactacagttttgaactctgggcttaagggatcctcctgcctctgcctgccaagtagctgggactacaggcatgctactgtgcatggccaacttttttattttttttagagaccaggtctcactatgttgcccaggctggtctcaaactcctgggctcaaacgatcctcctgccttggccttccaaagtgctgggattacaggtgtgaaccaccatgcccagccggtttttaattttttaatatgcctccaaaggagacattatcatggttttctactgttcatattgggttatatttgcccggatcttcatcagtcttttttgttaatcactgtctattatgtatcacttcttccttcattgagtttttaaaattcatgtggcatatatttcagtaggcttttcagtgagggtctgttatcctgaagtctctcagtctttgagaagtctttaattcactttcattcttggatgataactagaaatcaaattccagattgacagttatttttctctattattttgaagctactgtattgtctctgatttctatggctgctatggagaacttctaccagcaggttagattcttgtgggtaaactctctttttctttctggttgcttttaagctttttctctttgtctctgttgttctgcagtattatttttatttatccctggctcgctgcatttcctaaatgtgaagattcatgtctcattaatcattttcagccattatcacttttaatattgccttgctcccctactcgattctctcctcctagaacttctacaggacatacgctgaatattctcattcaatttttcatgcctcttaacacgtattctccatcactactccattcttgctaatttccccaacttcattttatagtttattcttttttttttttttttgagatggagtctcactctgtcacccacactggagtgcaatggcacgatcttggctcactgcaacctccacctcccgggttcaagcgattctcctgcttcagcctctcaagtagctgggattacaggtgcacgccaccaggcccagctaattttttttgttttttttaatagagacagggtttcaccatgtgtaccaggttggtcttgaactcctgacctcatggtccacccgcctcagcctcccaaagtgctaggattacaggcatgagccaccgcgcccagtccggtttattcattttctgtgtcctaatatcttcattaagttaatttccagtacagttgtacctcagtatctgcagggagttggttccaggatccctttgactatcaaaatccacagatgctcaagggccctatataaaatggtgtcttttctggtgttttttgtttttgttttttgagacaaggtctcattctgttgccaggctggagagcagtggctcagtcacagctcactgtagcctcgacctcctgggctcaggtgattctcccacctcaacctaccaagtagctgggactataggcacgtgccactatgcctggtcaatttttgtattttgtgtagacagggttttgccatgttgcccaggctggtctacaactcctgggctcaagcagtctgcccacctccatcccccaaaaacgttgggattacacgtgtgagccaccatgccaggcctggagtagtatttgcatgtaacctatgcacatcctcccatatactttaagtcatctctggattacttataatatctaatacaatataaatactatgtaaatagttgttacactgtattttaaaatatgtatatttttattgttgtattattttttcaaatctttcccatcacattagttgattctgaagatgcagagcccgtaaatatggacggccaactatgttgtatttctcatttctgaaaattctatttagtttctaaagtttgtttccttcttctaaatatatttaaatatactttatttgtagcctctgcttaataattctattatctaaagtccttgggggtttaaatcttattgccttctgactcttatgataaattgtttccttgcatgttctattattttgaattgtgatctcaacttcattggggtttcatatgtggatatcctgttaggtctgagttaacatgcaacaatctagaaattctgtttccttctggcaactgccctagaaatacttttcatattaagttcacaggattcgcagaccacacaggtagtataaatttgaatcccaaactggtgaaaaggtaggtctatggtgacaaattcccaggaatgacttttattctctgtaccatgagtccaagctaacacaagcactagagggtggattttgttttttaatccttccattgagggtgaatgtctttaaaggtcctggctttgtatgtggatctcaatccaacttctcaccttgtaggggggcctaagactttacctcgagtgtccttgcgtgacctttaaaacccgagcatactggttacagaaactagggactgtctttacgcccaggcagtcacaaagcataaaccacacaccatactgttgttaaatttcctgtttagggctccgcccaggctggaatgcaatggcatgatctcagctcactgcaacctccatctcccaggttcaaatgattctgcctcagcctcccaagtagctgggattaccggcatgcgccaccatgcccagctaatttttatatttttagaagagatggattttcaccatgttggccaggctagtctcaaactcctgacctcaagtgatccgcctgcctcagcctcccaaagtgctgggattacaggcgtgagccaccaggcctggcggaaccttgatcttttaaatgtgaatttcagatatttctattacctgtaaggagagaggtggggaagacgaaggttgaagggaatattgaataaataactcctgtgtactagccctcaatacatgagatatttgataacagctatacaaaacaagccatgttaatagatgagaaattaaagctcagaaaggtcaaataatttcgctaaggtcacaatgtactattacacccgaattcacgttggaattaactagtcagatccattttcattctggacatggtggtgtatgcctgtagtcccagctatttgggggcctgaagtgagaggactgcttgtgcctaggaattcatgtacagcctgggcaacatagcaagaaactgcttctaaaaataaataggctgggtgcagtggctcacgcctgtaatcccagcactttgggaggtggaggcaggtggatcacttgaggtcaggagttcaagaccagcctggccaacacggcgaaaccccatctctactaaaaatacaaaaaattagctgggtgtggtggtgcgtgcctgtaatcccagttacttgggaggctgaggcaggagaagagctttaacccaggaagcagaggttgtggtgagctgagatcacgtcactgcactccagcctgggcaacagagcaagactctgtctcaaataaaaataaataactttgggaggccgaagtgggaggatcccgaggtcgagatcgagaccatcctggctaacacagtgaaaccccatctctactaaaaatacaaaaaattagctgggcatggtggcaggcacctgtagtctcccagctacttggaaggctgaggcagaagaattgcttgaacctgggaggcggaggttgcagtgagccgagatcgtgccactgcattccagcctgggcaacagagagagactccatctcaaaaaattaaaaataagttaacaaataatcaattttcttcctctacagcagaggtcagcaaacttattctgttaaaggccaaacagtaaatattttaggcctcataagccatatggtattggctgcaactattcagttttactgttgtatcattaaagcagccactgaaaagtgtaaacaaatgagcatgactgtgttcccataaaactttaaggacattgacatttgaatttcataaaattttcacatataacaatactattattacttggatcttttccccaaccatataaaaatttaaaacccgttgctaatgcatgggtcttacaaaaacagcctggagttgacccacgggccgtggtttgctgacccttatcatacaccataacacctccttggaagtacacctctctaatgcctttgttccaaacaatactgggttaggaaagacatggaaaaaggaaaatgagatacattattttttgtaccctatgggggattgaggggttgttgctacatagccccctcaatttgtgctgtagcaatatgcagttaagatccttattctaatgttaaatgtctcttctgtggcttatcctaactttaaaaaaaaaaaaaagaagccatcttacgtaaatgaacttacaattttaagacagggtctcactctgtcacccaggctggagtgcagtggtacaatcacggctcattgcagcctcgacctctcaggctcgagagatcctcccaccccaacttcccaagtagctgggactacaggtgtgcaccactatgcctagctcatcttttttttttttttttttttcctttaaaagatatggagtctcgctattttgcccaggctggtcttgaactcctggactcaagcaatccacctgcctcagcctcccagagtgttgggattacaggtgtgagccactgtgcccggcctgaattatcttcttattgtaaaatttcctttaatgcttaatagttgatgtatattaagtgctaactaaatgttcactgataaacattaatcagatgctgctaaatattgtctttctttattcacagatgatagtcaatgggcacaacatataagtagttacaatgaaatgagaagcaatatagcagtcaggctatatgcatgatttaacaacaaaattatcacttccttttaatttagaataagggacaatttaaaaagcatctcttggccctatcatttctgttccagtagttagtgttcatatgtgaatactaagtttgacattcctttctcccatagaaccattttggtgatttggatggtggccactacactgctttctgcaagaattcagtcacccaggcctgatatagctttgataacacacgagtcagtgagattccagatacttctgttcaaaatgctatggatctcctgttctatagctgccagcccttttccataccaatacaaaagcgttaagagccaggaaaatggtgtttcctgaacactgcaaaacaagcagtcagcatctggtggtagagttttgcttggtcattaaactcttagaacttacttgcatcattaacatttttatgccttgtgggcatgttatacaacctttcatcttaagataaatctgtcgtccagaagatgggtcttggttcactaaaaaaggcagtgtgaatataatgcaatgctaatggatgcaggccttcaaaacactgcaattatatagtgagttcaggtttcaaaattcagtgtttatcagaaaatatctcataatcatatatattcaacaaattattttccaaagatactcatgaagctaaacaaaaataatttttgttcaaatggctcgatgagtttaagaatatgatttgaatatatttgatataataatttagccaagaagtggtctcttagactaattgtaaaacatgaaaagttgtcagcttcacaatttgaaccccatcctttcatcttctccctgagagcctgctaatggtggtctctttctgaagcacttttagaatcttatttttatatggagtgttttactgactatatatatagcaactgagtccctcggttaaataaattataagctcctttaaccctcttaatacatcactctgtaaagatgtagtttataatgcagttcactttgcaatcatgcctgactcccggcatttttactttaatatttagaatgaatattctcaatatgtgagaatactagtcttgaaagaatgactctgggtgttattatatagcacgtgtgtatataaaatctatggttttactgtcctatatttgataatacaatattaaagacagaacacccacagggttataaattatttttctcattaagattttaatgtagctgtaaatgaaattctcgttttaaaaaaattaaagtttccatttttttttttagaataaagatttagtgcacaaatacagcccaaagccaacagaaaaattgctttgccctgtcatttccctaagaaagcactgaagttaactcaaaataggctgaaagaaaaaaagcaatcctctgagttctaggtttcacaaaaggaccacgtgttaaactatgtacatcgatttgatgtgcaagtatgcaataaatatgtacacatacattcctatctgctttacatcattctagagtattcatagtatatcaagatgggatttagaaatgtgaaaaggccataacagtgaaaaggaaaaaaaaaagataacaatagtttttagaccagtcgaataataatgcttagctagttaattattttaactttggagcagactaaaaaagttgttttgaaataaatggtacctgtaagtgatgattactgcaatacttgttaaatgttatttgtcagcactgaccggaattatatagtgctagtaacacagctcccactgtcctagaattcctctaaatggccagctatagctaccattatcctgataagcatttcaagagttgtgttgctgagccttttaaaagataactagtttataacctatgtctccttatgtggctacatcagttactcgtggtcccaatgaagtataaaagaggatataagctgctgaagatttcacagaagaaacggagatatcagaaacttcatgatcatcaaacttaaaccaccgttgtcttgctgcatttttacaataggctgtgtagtggcctccatccagcccaccgtagtgatttgaaacagaaaacaaattatatttcttcaaattgttctttggaccaataacatactgtgacaagtcaagattttctaacgggaagtccacagatgtctgtaatttttgtttccacctgccatcgtaggaaaaacgtttcagatgcactaaaagcacaggtggtaacttccagatttctatcttttttagagaatcccgtcgagctctgcaatgactgcagtaaaatctgttgttatctgtgagtttttcttctttggaaaataatctaaggcaatcctgtaatgtacatttacttgtggatgctagtggtagagacaaatacatgaaggcctcaaatgtcctagactttttgtgacatgtgaggcactgtactgtagatttgaattgaccctgaaaaagtgcaacaataatagactcattgagctgcttgtgtttctgccaggcatgttctgcagctttaaagtcatcgagatgatcattattttcttctttatatctcttccgattatcagctttatttagatcttcatggagaccatccattaggaacagaagcaattcttgtgaatcttgctgactgtatcctgcaaactggtcattgatcttcccaatggtgattttaaagtcctttggactgatatatctatactgtcctgtccacagggctttcatgattataccaaattcttctgccacttcacctttatgccccaacaaatttgacctgttaatatcatcctgataacagtttcggttgaaataatcagccaaatgtggagcgttacataggcactgcaatattgagttcatataacaagtatttcctaagttacgaagtccagtaagagctggtccagaacctccaaaaacaggattgaggttccgaatctgagaagcagaaagccttgagatctcagctttaggataacatgttggcttgttttcccgattaactgttggagttactgttggcttcctcttctcttcctcttgaatagcctgggttatatctggggaggagtaggagcgcttcagtttggaaggttccctatcccgctcagcaggaatctgtggcttggctttatgagttggaggggtggaaggaggtgcagatgaaggagccatttccggtgggtacatatgaacagtgttggtgggtgaatgataataacgaaaggttccagtgattgggtcaagaaacttggcccagcctgaaggcagtcctggtacgatcctccccatttcttcacttcgtgctcttgtcaaaggttctcgttgagctttatttctttcggtatcgtctgtatcctctctaaaagttcctgtccttagaattccactttctggttgtcctttaatcttaaatggcttgcctgaacctgaatcccctgtcacagatgtatggggcacatctcctgttgactttttctgtatttctggggttggacaccttttccccctatcttctacagatttcttggcatcagaagtttcatgttcacttttactttgtctttttactcctgttatttctttgcccctctttgctgaggtttctttatcttctttcttggcctgttcactttctttcttctccatttcttcttttgctttttgttgcttctctgtaatttcattttcttcagcttcttgtttctttttggctttttgttcttgttcttccttcctcagtttctctttctgttcctcttgctgcctttcccgaagttctttttcttgtttgtttttttccattagaagagcagtttctgcatgaatacgagccttttcttcatctgttaacatgagagttggagaaaaaactactggcttggtggaacgatcaggaataacttttccactctgaggagattgttgctcatggtttgtactttcagattttattctatgctcttcaggcaatttgactgctggttttttagtacgatcaatctgtggaacattctttatactaggcactggctgaattatgggtgaaacatcagatttagaagcagcaactggttcaactggagttgatatattcagtggtcccattctctcattttgaccacttatcaattctatattttcatctacttctatagatgcaggtggcgtctgggcagcaggtttagaaggaattgattcttccaatgagggataagtaaaatccaatgagatagacacctcttcattctggcgtcgtgggggtggagtgaccttagcatttgttgtatactggggataacaaaggagccagttttcatagcctccctctaaaaccaaaggctcattgcgcaggacagttttactttcccacttgaaaagtgcatctttcagactccggagagttgttccaatctgtaaatctttggcagaactaaaccagtcaagaagtaccacatactccacattccccctcttcttccatgtgtctttagaatcatctggcaggtgtgcttcaatccaactagcagtgactcctggactgatggcttcttcaggaacactgagagaatgtaaaatacaggaatcctgataatcctgcattcttcgagcatccattataatcaagctgatgtttttatccgtcatcattgtgtatagttcctttgctgtgattgctcctttctctttggtctcacatttttcattcttttcaccattgctcttttgggttttgtctttggaatccaaaacattctccaaagagcctttagccaatgtgccaccatcctctcttcctgtttcctgccttttttgttgtagccgctgtgcttcctcctgcctgtctttttcctcaagttttttccggacttcagcttcttcatatcttaatttaaggctttcagagagtctttcagcttcttcgacagcttttttgatgtttccaggtccaagtattgaatggaaataatcctgctgttgcttgaaatcaggtctttttttgataagattataaacagtcacgtatttcatatatagtacataggccctttcctcatcacgatctaatctgcattcttctgctgtcttaaagatcttcagggcactgtgcacataactcttagtgcttattttctctggtttaacttctgtcttcttattaaggtcttttagtgaagaactgaggtagagttctttaggaactgaagccacagcaggcatgatgaattatctttacttttccactttcacaatggatgctatatttccttacaagtgcttctttcctttaggagttgtcccactcctctccgcggacagagcttgtctccggggtaaccagcagctggtggaaggaaaggcgttcatcgttcacagcggacgacttcccagagaacaggtgctagggcccaagacccgcactcaccgtgacgccgggcgcgcttcactaacgccagccttctcgccaaatgcccatctcccaagaactcgagggagaattagccttggctaccaggacggaagccagcccagctc

SEQ ID NO: 14712 - RNA, 2471 nt, Homo sapiens
  source 1..2471: mol_type = other RNA
gctgggattacaggcatgagccaccgtgcctggcctataacatgtattcttgtgtcttcccattttactggcctctgagttagttctttgaaagtcactgtagttctgcacttggattctgatttcagatcctagccccatcaccaactgtgcgtgactttggatgaattagtctgagcctcagtttcctcatcagatttgtaattaggtcaaataactcaatatccctgagccccagttttcttgcatgtataatagggatattaatccccattcacaaggttgtcatgagagatatgtgaaacaccaggtcgtatgcctagtcagtgcctgacatattagtaactgcttcttaggggactgatcagtcctccttcctcttttcattgtccacagctgcatctggccactgctccacaccggcctcctggatataggatgaattccaggagttggcaaagtggaagttgtatatggtttatagagaggtgcctggtattgagtgttgctgtcactgaccaatgccataacttgggacaaaccacttcacttctctgagtctctcttctcatctgtcatttaacatgataacatagtacctacctgtgtaggttagtacaagatccaaagagattaactaaaacaaacacacaaaagcaaaagcaaacaaacaaaaaacatgattcttgtagtaaatagttatttaataataactgaattatgctacttggggtcttgctttgcccatgtgtaaatttagaattttgtcccataacattctggaaaaaaaatccattattcatatcttttgtgaaatgctgagtacagtctcctcctttcttagaaattcataagacattatcatattaaaggctctgagatatcccatgagaaaaaaaatctgtttaactttatttaatcctgtatttttcaaatttatttggccacaccttcaaataactattaatgtctcatgggaggtaatgttctgaagaacacactttcgaccaattgggccaagtggtcttttggttcacctggagctgtcatcctgagttaaagaatagccattgcttatcagagcctcttctttaatcaccagcacaaggaatgcaatgaaaactcatgtttttgcataaaatggtgcctttggttgtgtttcttctataacgcaggaaatagtaaatgtgtatattctcaaaccccacgatattagccatgcaggctgttggatgttctgcctcctgatgtgtgtgtgtgtatatatgtgtgtgtgtgtgtgtgtgtgcatgtacccacatgtgtgcacgcatgtacccacatgtgtgcacacagcacctttctcttcctcttgaggctgtcagagtcacgcacctggggcattacaagtcctgggtacctctataactattccctttcttctcacaagagtgcctttgacctctttctgttaaatcccctagaaacatttcagtcctccctctttctggaactggaacccttgggtctccaccttgggtccctgctgcaaaggggaaattggggtcttgggaaattattcccaagggaaagcgtgaagtcattgggtaagcatagatttgagattctgacttcctcaaacataaattgggaatagctgaccctttcaccagtgagggctagcacacattttgttggcttatgcccatggggctgagacccaagtaggcggtcagggaagccttcctcaccatctgcttaagacgcatctgccgaatactcagtatctcagtgcacttattcacaccctctttcattctccaaaacatctcgctttcaacggcaaattataggcgaccctacccattcctctcctaaagtcccttattaagaaggctggaagtctcaggggtgagcagcaagggaaagaggaagtctgtttccagtggtgttcatggcccatacagccaacagagggcgctcccacaccacgcaacactggggtccaaggatccaggcaggccctggggaaggcggccagctgacctttctccaggctgttcttgggttgccagagcagcggaggtgtcagctgagagtggtcacagcctggggaggagaaggcagggagagaggctggggcacccgaaggggaggaggagctggcagggaaaacacacagacacatttcacagaggcagagacacaggggaacacacagaatatgcagttgtacctacaaacaacaaatgcaacataccccacacagacacagcatgcagccaggggatttagagaaatcatatagggtgcagactcacaaatgaatgcaatccatcccatacaggtatacacaatgcagtcacctcagccagctaaacaaaaacaaaggcaacacacagataccaacacatataaacatgcatgtgagcacatcacccaacagggacattcaagctatgtgcagccaacgaaaggcagataacaaagag

SEQ ID NO: 14713 - RNA, 2955 nt, Homo sapiens
  source 1..2955: mol_type = other RNA
gctgggattacaggcatgagccaccgtgcctggcctgaagatggcacttttaaaaagatttttttctaagtaaaatggcccccaaagagcccaatgatttttttaagggtttatttttcattttaaaaaaactggataaaaatgaaagctgtaaaatatgggaagaggagcaagagagctgctgagtttgcatttgaaattgtgaggggctggggaggacacgaccaggtagagaggacccctacccactagtccctgctctcacagcttgcgctccccacactcaggctgcaccaccagggaacacaggacagaagtctagaggacaagagaccaaactcaagtcttctttcttgtggttggttgggtgtttacatgtgcaagtgtagtaagccacaccccacagacataaggtgcctgtctgtggatgccataggcatgctcctaagctcagtctctggtgaccccgagtctctgggcaggccacgggccttcacttctccactttcttggctttcttgaggatgttgcattttttcctgttagggcagtggcactgctcgtcgttgctggggatacattcgcagtgccacacctcctccaccttctccacggggtagacggcttccacctagtggcagatgagccgcagctgcgtagggtccagctgcttcttgttgcaagcccgaaaattgttgtactgcagctggaggttctcggcggtggaggagccccgcggcaaagttgcccacggagaggctctgctgcacgatcttgcacacctccttgtcggacagcaggtagggagagcgcaccgggaagctcagtgagggaccaccacctcatccaaggggatcttgcagaagtccttgctgctcctctcgggggcagcgggggaccctcagactcctctctgaacctctcaggattgattgcatagctcctcatgtctttacactcggggccagcacgtggaccttgcactgctgctggtaggagcgcctctgttcctgttccagtgcaggttgcccatgaactcaagggtccagacgcgattgtttttggtgcagaggtagagcaggtgcacttagtggcgaatgagcttgatgcaggacgggtccagctgcttcttgcccagggagtcgctgcagctgtgctgcttgtgcaggttgtcatgggtgaagagcttggggaataggggcaccagcaggcgcgaggtgaagttgccgatggacaggctgctctcgtagatactgtgaagatgctcgttgctgagcaggccgtcggcgccgggcacctccaagttgggctggggatctccaatttgaccaagtcgataggtaccagtcagatcttcttggagcggcaccgctcgcccttgaagctatcctccaccctgattactgagatgtcatcgggcaggctggaggagttgtagcagttgtcgcgtggggggctcgccttcgctgcctgcgtccagccccaggccctgaagcttgtcgttgatgcactgggcgcaccgctgcagccaggcctcctcctcctgcatgtgggggaagtagacctccgtgaagttgcagatgatctgcagcctctgcgggtccaggtcctgcttgccgccaggcctcctcctcctgcatgtgggggaagtagacctccgtgaagttgcagatgatctgcagcctctgcgggtccagctcctgcttgccgccgtccccgtagcagctgtcctgctcgcccagcttgcggtagtggaagagctcagggaagagccagtggaggaggaagacggcaaactcgcctgtgaagaggcttcatgcaggaactaagtgagggcctacatgtccaccacgtggtctgaggcgatggtgctgctccagtccagagacaggccctcctcctcgtctttgtggtccaggaagtggccggggtccactgctcagcctcaagctggcagcctggccaccgggctggctgttctccatctcccgctgggcccagaagtggctgaagaacttattcagctggggcaagcactcggcctgtcacacagccctctccttcaccgaggggtagtagacctccatgtagttgtggatgagctgcaggtgcagtgactccagcttaagcttggcctcaaagctgcaggcactgcagcctcgggagaagttgactgtggctgaagagcttggggaagagctgcaccagcgggcagcaggccaggaccccgcctgacaggctctggtccaagatctgcttaagctccatgcccgtgagctgctacggggtggtgggggtcggctggaatttggccaccatctcagtggggttcaccttcagggagagcaggtccactttgctgtgtagctgggacctgttggacgtgagggtgttgagcatgtagaacatctcctggatcaggaagtagatgttagggtcactgttggtggctgccccagtgctgccacagtcccacttctatggctcattcaggagcctaagcagcgaggggctgttgctggaatttgccttctggaagagctcatacgtgtttagcaggtcccccgagggagggttcttcttctccatgaccttgtgggagatgccatacagaggcttcttgtagtaaggggtggtggcatggttgcggggctcctccttgcctggccacacagagcccgagctcctgccttgccggcctgctctccattgccttggcagggcgagctgttctcgggttccacatgcctgctaggagcgcctctgggatcagctacctcctctccacgctggggatggagtctggctggccattgctgaccagctgagtcctggagggcagtaaagacgctgtccagaaggtgcttctcagaagtcctggaattcacggagcagcctagagcagcatctttggcctctgtctccactctcacttcttagaagttcttctacatc

SEQ ID NO: 14714 - RNA, 3196 nt, Homo sapiens
  source 1..3196: mol_type = other RNA
gctgggattacaggcatgagccaccgtgcctggcctgcgagtttaattattttttcgggggtgggtgaacttctcgcagcggcccccttgtgggggtaacccggtggcgggtttcacttcggggtttggaggggaagttggagtctgtggggcgggtcccgcccggccccgaatgtcacggccgaggttctcggaagcagcagagtgaagttccttcctgccctgaccccaggtctatggcttaaaaatcagggtgcccaggctggggccgcgcagcccaggggccctctgtaaacatggcaggtgcagccagaaggggcttccgggaccccgggggacctgcggtgggcagggcagagggtcagggtgaccagagccatggagagggcaatgcccggaggacacgtagatatggggtgggggagttaggacccccaacatggagagagacaggggccaagaaagacagagaaaaggagacagagggagatctggagaatgggggagggaaggaaagagaaagagggtgagagaaccccaaacaagagccagagccggagaaatgaggacccctggatgtggctggtctggtccgtggctcccgccgccgcagcctccggcgcagacgggcccaggggcggctctgcttggggcgggtcctcggtgctcagcgggcggcaggcggcgggccggggcccggggcgcgcactgggtgcgccagggtgacggtgagcgcgtcgttgtgctgcaccagcgaggcgtgctggtagtgcagcaccagctccttcagcgacccgtacaggttgtagggctccgcgaagccgaagccggtggccgtgcggtagatgacgcagtgcttggtgtcgccgtccactaccacggagcaggcgtagcagccccgctggctgctctcgcggatgaggaaggtgccatcccgcttgccactcagcatctcctctgcctgcgtgcggttgatcttgcccacgtaccaagtgcgttcctcgtggtgcgggagatcgtcctcgtcctccatgagtgcgtactggtcactcctcagtctcatttttaatccccagccactcgttgattttcttctgccgggcgcctttctgggtgagccacacgaggtactggtctcggatcttgcgcagctgcatgaggtccggcttgaggctgttcatgcgcttgtcgatctctctgttgtccgaggcctgggcccgcagctgctgctccagcttcgtgcggctctcatggatctcggcaatgcgggacttgagccgctcggagttcagcaggatcctttgcatctctttctcgttgccctcacgccggaagcgctccaggtattccttgctgcatttctcttgagtctggccctgctcttcaaagatcttgatagtctcattgaaggcctcaattgcagtacgcttcatctgcagctcctgggaggtccgtgtgtactcttcataaagctggtcatactcgcggctcttgtcctggtactgctggtgatagaccttaagctgggcgcccactgcctccacgctgtcctccttgacaatctggtcctgctggtatttggacacagggtagaggagccgtgtgtccagcttggcattgtactgggccagagactcgtggcggtagtgattgatgaggtccacaacggagcagaaggtgagtggctctgagaagccatagtgcccatctcggtggaagaccttgatcagcttattgttcccgcctttcctgagggtcagcgtgtactcgccctggatcttgctagaagcatctcggactaggaaggtgccatcgggagtgtcccggagtttctcgttcacctcctcccttgaaatgtccccccagtaccactcagcatcctgcagggagggtgggctccctccattggccaggactgtggaggccggctttgccttggggggtttaggcggcagcgctgggggcgcaacctcctgctcttccaagtgttcctgaagcagcttctccaccagcagcgccgggaagtcagggctgggctcactccccgcagggcccggcgcgcctcggccgaggcctcgggggtcacgagcggcgcgggcagtgccagcaggaagctcttaatgccgtcagccagggctgccgtgtcccactgatccacgtcgctcagggaccagtctgtacgcggtgcgggcagctccgggcggtagtgagattcgctgtccagccctgtcctttcaatggcctccacaagcttcaccagaagagggggagccacatcaggtggggagaactgctcgggcaagtcggggagtgtgaggcctggctcaggggccccatcacggggcctggcgggcagtgggcgggggccccgtgggcgagggccgggccgggccagggccacgggccccaggaactccacataggtgccagggaagtcacctcgctgccgtgtgcgctcgttgaggccgggcatccagcccacgctctgtgggcagcgctcgccaccctcggccacgcccagcgcctgcaaggccgcccggctcactaccagcacgtcgccgggcagcagctccaggtcctccggccgctcccggcggaacgggtacagagcgcggtactggaagccctcagggcccgccatggccgcgtgagtggggtggggtctggatggttaggtggctgcttggagccccactggccccattggttgaagcagggctgggagggtccgctgggttggcttggggtgctgggacctctatctccagcagtcacaggcgaccacaggggccgctcatgcctcgcttcaaattattccatgacccttacaagggccactcgtcactgggtccaccattcgtcagctggtgggagggagttggtggtgtggtgtcaggtcactgggccattgagtcctccatcagcaggtgaggctggggcaggccgctcacgccctcacacggagggccatgggcgcccaaggctggcggctctgctggctgcaccagacaagggagccaagggtgcaggctgccaccatgctcggccagctgaggacgccgacctggtcgcggccgccaccgccgccgcagccgccgtcacaccaagccaagcccgccccgtggctccaccgcggccaccgtcgccgcagccgcgggatccccgcctccgccgccgccacggttccgagcggcct

SEQ ID NO: 14715 - RNA, 3458 nt, Homo sapiens
  source 1..3458: mol_type = other RNA
gctgggattacaggcatgagccaccgtgcctggcctgcgagtttaattattttttcgggggtgggtgaacttctcgcagcggcccccttgtgggggtaacccggtggcgggtttcacttcggggtttggaggggaagttggagtctgtggggcgggtcccgcccggccccgaatgtcacggccgaggttctcggaagcagcagagtgaagttccttcctgccctgaccccaggtctatggcttaaaaatcagggtgcccaggctggggccgcgcagcccaggggccctctgtaaacatggcaggtgcagccagaaggggcttccgggaccccgggggacctgcggtgggcagggcagagggtcagggtgaccagagccatggagagggcaatgcccggaggacacgtagatatggggtgggggagttaggacccccaacatggagagagacaggggccaagaaagacagagaaaaggagacagagggagatctggagaatgggggagggaaggaaagagaaagagggtgagagaaccccaaacaagagccagagccggagaaatgaggacccctggatgtggctggtctggtccgtggctcccgccgccgcagcctccggcgcagacgggcccaggggcggctctgcttggggcgggtcctcggtgctcagcgggcggcaggcggcgggccggggcccggggcgcgcactgggtgcgccagggtgacggtgagcgcgtcgttgtgctgcaccagcgaggcgtgctggtagtgcagcaccagctccttcagcgacccgtacaggttgtagggctccgcgaagccgaagccggtggccgtgcggtagatgacgcagtgcttggtgtcgccgtccactaccacggagcaggcgtagcagccccgctggctgctctcgcggatgaggaaggtgccatcccgcttgccactcagcatctcctctgcctgcgtgcggttgatcttgcccacgtaccaagtgcgttcctcgtggtgcgggagatcgtcctcgtcctccatgagtgcgtactggtcctcagtctcatttttaatccccagccactcgttgattttcttctgccgggcgcctttctgggtgagccacacgaggtactggtctcggatcttgcgcagctgcatgaggtccggcttgaggctgttcatgcgcttgtcgatctctctgttgtccgaggcctgggcccgcagctgctgctccagcttcgtgcggctctcatggatctcggcaatgcgggacttgagccgctcggagttcagcaggatcctttgcatctctttctcgttgccctcacgccggaagcgctccaggtattccttgctgcatttctcttgagtctggccctgctcttcaaagatcttgatagtctcattgaaggcctcaattgcagtacgcttcatctgcagctcctggaggagggggcgcagctcagcacctcctgggactccccaaaaggccctgggaggtccgtgtgtactcttcataaagctggtcatactcgcggctcttgtcctggtactgctggtgatagaccttaagctgggcgcccactgcctccacgctgtcctccttgacaatctggtcctgctggtatttggacacagggtagaggagccgtgtgtccagcttggcattgtactgggccagagactcgtggcggtagtgattgatgaggtccacaacggagcagaaggtgagtggctctgagaagccatagtgcccatctcggtggaagaccttgatcagcttattgttcccgcctttcctgagggtcagcgtgtactcgccctggatcttgctagaagcatctcggactaggaaggtgccatcgggagtgtcccggagtttctcgttcacctcctcccttgaaatgtccccccagtaccactcagcatcctgcagggagggtgggctccctccattggccaggactgtggaggccggctttgccttggggggtttaggcggcagcgctgggggcgcaacctcctgctcttccaagtgttcctgaagcagcttctccaccagcagcgccgggaagtcagggctgggctcactcccgtcgggagcgccccctggcggcggcgaggacggcggcggcggcgcgcgcagcagcagcggcccaaaggtggcgcccagggcccggaccgcgggacccagggccggggcgcggctggccacgcggcccaggtgctggagcaggaagcgcagcgtgagcgcgcggtgcagcggcagcgtcggtggctccagcgccggccccacgggccccgcggcctcccgcagggcccggcgcgcctcggccgaggcctcgggggtcacgagcggcgcgggcagtgccagcaggaagctcttaatgccgtcagccagggctgccgtgtcccactgatccacgtcgctcagggaccagtctgtacgcggtgcgggcagctccgggcggtagtgagattcgctgtccagccctgtcctttcaatggcctccacaagcttcaccagaagagggggagccacatcaggtggggagaactgctcgggcaagtcggggagtgtgaggcctggctcaggggccccatcacggggcctggcgggcagtgggcgggggccccgtgggcgagggccgggccgggccagggccacgggccccaggaactccacataggtgccagggaagtcacctcgctgccgtgtgcgctcgttgaggccgggcatccagcccacgctctgtgggcagcgctcgccaccctcggccacgcccagcgcctgcaaggccgcccggctcactaccagcacgtcgccgggcagcagctccaggtcctccggccgctcccggcggaacgggtacagagcgcggtactggaagccctcagggcccgccatggccgcgtgagtggggtggggtctggatggttaggtggctgcttggagccccactggccccattggttgaagcagggctgggagggtccgctgggttggcttggggtgctgggacctctatctccagcagtcacaggcgaccacaggggccgctcatgcctcgcttcaaattattccatgacccttacaagggccactcgtcactgggtccaccattcgtcagctggtgggagggagttggtggtgtggtgtcaggtcactgggccattgagtcctccatcagcaggtgaggctggggcaggccgctcacgccctcacacggagggccatgggcgcccaaggctggcggctctgctggctgcaccagacaagggagccaagggtgcaggctgccaccatgctcggccagctgaggacgccgacctggtcgcggccgccaccgccgccgcagccgccgtcacaccaagccaagcccgccccgtggctccaccgcggccaccgtcgccgcagccgcgggatccccgcctccgccgccgccacggttccgagcggcct

SEQ ID NO: 14716 - RNA, 3409 nt, Homo sapiens
  source 1..3409: mol_type = other RNA
gctgggattacaggcatgagccaccgtgcctggcctgcgagtttaattattttttcgggggtgggtgaacttctcgcagcggcccccttgtgggggtaacccggtggcgggtttcacttcggggtttggaggggaagttggagtctgtggggcgggtcccgcccggccccgaatgtcacggccgaggttctcggaagcagcagagtgaagttccttcctgccctgaccccaggtctatggcttaaaaatcagggtgcccaggctggggccgcgcagcccaggggccctctgtaaacatggcaggtgcagccagaaggggcttccgggaccccgggggacctgcggtgggcagggcagagggtcagggtgaccagagccatggagagggcaatgcccggaggacacgtagatatggggtgggggagttaggacccccaacatggagagagacaggggccaagaaagacagagaaaaggagacagagggagatctggagaatgggggagggaaggaaagagaaagagggtgagagaaccccaaacaagagccagagccggagaaatgaggacccctggatgtggctggtctggtccgtggctcccgccgccgcagcctccggcgcagacgggcccaggggcggctctgcttggggcgggtcctcggtgctcagcgggcggcaggcggcgggccggggcccggggcgcgcactgggtgcgccagggtgacggtgagcgcgtcgttgtgctgcaccagcgaggcgtgctggtagtgcagcaccagctccttcagcgacccgtacaggttgtagggctccgcgaagccgaagccggtggccgtgcggtagatgacgcagtgcttggtgtcgccgtccactaccacggagcaggcgtagcagccccgctggctgctctcgcggatgaggaaggtgccatcccgcttgccactcagcatctcctctgcctgcgtgcggttgatcttgcccacgtaccaagtgcgttcctcgtggtgcgggagatcgtcctcgtcctccatgagtgcgtactggtcctcagtctcatttttaatccccagccactcgttgattttcttctgccgggcgcctttctgggtgagccacacgaggtactggtctcggatcttgcgcagctgcatgaggtccggcttgaggctgttcatgcgcttgtcgatctctctgttgtccgaggcctgggcccgcagctgctgctccagcttcgtgcggctctcatggatctcggcaatgcgggacttgagccgctcggagttcagcaggatcctttgcatctctttctcgttgccctcacgccggaagcgctccaggtattccttgctgcatttctcttgagtctggccctgctcttcaaagatcttgatagtctcattgaaggcctcaattgcagtacgcttcatctgcagctcctgggaggtccgtgtgtactcttcataaagctggtcatactcgcggctcttgtcctggtactgctggtgatagaccttaagctgggcgcccactgcctccacgctgtcctccttgacaatctggtcctgctggtatttggacacagggtagaggagccgtgtgtccagcttggcattgtactgggccagagactcgtggcggtagtgattgatgaggtccacaacggagcagaaggtgagtggctctgagaagccatagtgcccatctcggtggaagaccttgatcagcttattgttcccgcctttcctgagggtcagcgtgtactcgccctggatcttgctagaagcatctcggactaggaaggtgccatcgggagtgtcccggagtttctcgttcacctcctcccttgaaatgtccccccagtaccactcagcatcctgcagggagggtgggctccctccattggccaggactgtggaggccggctttgccttggggggtttaggcggcagcgctgggggcgcaacctcctgctcttccaagtgttcctgaagcagcttctccaccagcagcgccgggaagtcagggctgggctcactcccgtcgggagcgccccctggcggcggcgaggacggcggcggcggcgcgcgcagcagcagcggcccaaaggtggcgcccagggcccggaccgcgggacccagggccggggcgcggctggccacgcggcccaggtgctggagcaggaagcgcagcgtgagcgcgcggtgcagcggcagcgtcggtggctccagcgccggccccacgggccccgcggcctcccgcagggcccggcgcgcctcggccgaggcctcgggggtcacgagcggcgcgggcagtgccagcaggaagctcttaatgccgtcagccagggctgccgtgtcccactgatccacgtcgctcagggaccagtctgtacgcggtgcgggcagctccgggcggtagtgagattcgctgtccagccctgtcctttcaatggcctccacaagcttcaccagaagagggggagccacatcaggtggggagaactgctcgggcaagtcggggagtgtgaggcctggctcaggggccccatcacggggcctggcgggcagtgggcgggggccccgtgggcgagggccgggccgggccagggccacgggccccaggaactccacataggtgccagggaagtcacctcgctgccgtgtgcgctcgttgaggccgggcatccagcccacgctctgtgggcagcgctcgccaccctcggccacgcccagcgcctgcaaggccgcccggctcactaccagcacgtcgccgggcagcagctccaggtcctccggccgctcccggcggaacgggtacagagcgcggtactggaagccctcagggcccgccatggccgcgtgagtggggtggggtctggatggttaggtggctgcttggagccccactggccccattggttgaagcagggctgggagggtccgctgggttggcttggggtgctgggacctctatctccagcagtcacaggcgaccacaggggccgctcatgcctcgcttcaaattattccatgacccttacaagggccactcgtcactgggtccaccattcgtcagctggtgggagggagttggtggtgtggtgtcaggtcactgggccattgagtcctccatcagcaggtgaggctggggcaggccgctcacgccctcacacggagggccatgggcgcccaaggctggcggctctgctggctgcaccagacaagggagccaagggtgcaggctgccaccatgctcggccagctgaggacgccgacctggtcgcggccgccaccgccgccgcagccgccgtcacaccaagccaagcccgccccgtggctccaccgcggccaccgtcgccgcagccgcgggatccccgcctccgccgccgccacggttccgagcggcct

SEQ ID NO: 14717 - RNA, 351 nt, Homo sapiens
  source 1..351: mol_type = other RNA
gctgggattacaggcatgagccaccgtgcctggcctgcttgttgttttcatctcatcctgatttctgaatacaggagaggagctgagttggtgttcactaacaagcacagaagctttgttacatttacagtgtcattcttggcaaaacctgaatggtatgtttgtggggtgatgaggttcagtcccctgtgacctgtgcatctggccaacactgtggtgacatccttaggaatccccgtggattccagagaagaaagtagatgggagcaagtgtccagtacagcaacagcgtattaggaggagacagcaaaatgcctaggcagatacggaagggtccctggagaatctcca

SEQ ID NO: 14718 - RNA, 1646 nt, Homo sapiens
  source 1..1646: mol_type = other RNA
gctgggattacaggcatgagccaccgtgcctggcctgtggccatgttttaacaccaccacaattgccatgggttgccaggcagcctggcagaggaacactgcaaggacccgtcccttcatggcagattcagaaaggctgaaaggcgttatggtcagtcagggaagacccaggagccactcaggcccacacagacctctctgtgtgccactggcctcttgcacccctcctttgactgtgacgttctcccctggagggatcaagaggtcaaaccaggcactcagaaaggcaagggccatagtagggtgaccttgagtgagccacatgatgtctgggagctttgcattccttgcctgcatcatggcagatgtttcctctctcccacggttctggggaagaacagaggagagaatgtatatgaaacccattcacccagtaggttcctggccaaagcaggtttccttccaaggggaatggggtggggcgggggtgccacaggcagggagaagatctgagggcctgactcactgggttctctcccagggacttaaccagggtggcgtgtctgcacttgaagctgcagcaggcacctctcaggcctgtggctcccagctctaattacagatttctggacatgtttcctgtttgggagctggcagtgtccccgcagaggatccacagataatgagcagctggcttcagaggctccatccatggggcactgacctgggagcaggcccaagcaggcccgcctcagacagcagaaggccctcaaaggtcatctggtctcaattcttccccacatcacactcacacaggaccaacaccgtgatcaccatgaccagtctctgcttgcacggttccagtgatgggcagctcaccacttcacagccagtctgctaatctctagacatcactcaagacagcactggaagcacttcccaaatcagtttgtcctttaacttctagctattgatccccaggtccaccaagaacaatgaaacatggaacagaagaagggcgcagaccctgggatcaagaagaactggctttggttccaatcttagtttttacgcttgcagtcttggtctctttgatcctcaatattcttctctccagagatgttaatgttctagggtggggcctgagatgttgcacttctaaccagctcccagctgtggctgaagctgttgctccacaggccacactttgagtgttgtggaagaaagcagacagtcaacttacaacaccttcaatattcaggtcaggcactaacttgctgcatggccttaaacatgtcctttctgttttctgggtcttatcttcccatctgtaaaacaaggtagatggattaggtcttgcctagagaaggaactgacattacctgagccactgatatgtttatttattaacttttctctccaaaatatttgattgagcaattcctatgaaccaggacctgatctatagcactgcacaggagagatgaaacaaagctcatgcctcgtggagctggccccatgctttgcacgaaatgcctgattcctatgatctcatttagcctttactacagtcacccacaggagttgggtgccatcatccttgctttacagataagaaaactgaggcatcggcagggtgcggtggc

SEQ ID NO: 14719 - RNA, 1962 nt, Homo sapiens
  source 1..1962: mol_type = other RNA
gctgggattacaggcatgagccaccgtgcctggccttccatgttgcttttttaaggctagtcaagtgaagcagtgggaatgagaaggaacacagaaatctgttaaatgattgtgatcaattggttgtaaacatcactgcacttggactagcctcgtgtcattttttaatggaaacatgatttgttttcttcttgtcatcatcttaagaataaaaagagtatttgacctttgctcaaaataattttctctttgggttacaatctgaagggcattaattatgaagatattgttataattaatgcccactgtctaaaggagaattctcagccagttcagacctaaagagagcaagatgtcgtttgagctttttcttctcctctgtctgttcacacaatttgacttcaatgttgccatcactgaatgcttctcctttggtttcctccactggattctctctgagggaaaactttgctttcttccgcatcattgtaattcctgaatttccatgcctttgtgctggagagaaggttttatttactatgcaataacaaactgcagacaaaacattttttttgaagttttcattcataaatgcatagacaatgggattacagatggagttggaaaatccaataatttgcacgatagcaaaaatcatcttgattgtgacatcatcatattccttttcaaaattactgtattcaatcatcatatggacaacatggaatggtgcccagcacacagcaaagagagccaccactgtcaccatcataatgacagctcgtttcttcttcctggctattttggacatttcttttccatgaatagttcgaagcactgaaccatccccaactcttttctttatccaaagttcataaccaattttactgtacagaataagcatcaccataagaggcaggaggaagaggatgacaaggatgaaggtggtgtagatcttctggtgcacagggctggtccactcttctaagcagcagatgtgttccttttcatataggaagtcatatttgatctcaagttgttgcacgtgccacatgggtgatcctacgatgactgccaccagccagaccacacctagcattgtgaaagcccttcggttggtgtattgccacttcattttaaaaggatgcacaagtccctggtgcctttccacagcaatgcaggtcatagtgaggatttctgtcacaacagcggtagactggacaaatggcaccatcttgcaaatgaaagcaccccccagccagttgtcggaaatgttctggagcatggtgacgggaatgcagaagaaggtgatgagcaggtcactgagcgccaaggagcagataaagatgttggtgacggtgcgcatggccttgctgcgggtcaccacgtagaacaccagagcattgccaaagagcgccagggcgaagatgagcacgccggtgagcacgagggccagcttggcgcgtcccggcagctctggggtgtagacgagcggtcgcagccggtacagagcgatgaactgctcccgcgtcaggttgtggtcccgcagcagccgagagaactgctccggggtaatgttaagcgcctgcattgctgtgcgctcccgggacgcggggccaccgcccgctactggctggccatccgcatctgcggggcagcgagggcttcgggggaccagccggaggccgcctcccttcctctactctggagtcagccgcgcgggagggctctaggctgcaccccgggaggttcgggaaaggagagcagctcagggatcaaacccacgataaagaggcgggaagccaaagcactgggagactcgatctcagtgaccaaaaaatgttcgcggttcaaataaagttcttcccttgctcttccctaaggcgaggcgccgccacggtctggggtgctggagcgccacgcgagggtcctggcgcctctggctccccgccttctggccat

SEQ ID NO: 14720 - RNA, 842 nt, Homo sapiens
  source 1..842: mol_type = other RNA
gctgggattacaggcatgagccaccgtgcctggccttgtacacttactgtacagtcaatttacctgccactgatgtcatccacactgtggctgtgggtgctgaggtttggtgctgcctgcttggagctgtggcaccagcctctgggctcctgactcaagcacagggggcttcaggacctccgtgttctcttggcctctcccagtctgagctgttttatctgcaaggagtgcttgcagatttgggaaaggaaataggaacacgttgtgtaagcaaacaccaagaatgcagcattccctgcagtgagggtcccaccacaggcacacagcagcaggtggctgacacacggtctgtaagatggaagagatgcggacgcccagggacaggttcacggggcccagtggccaatggcctgttttgccttgcagaggtggtttcataagtcagttcacagtataccaccggctccgccagcaggtccgcggggtgggtgcggcgggagctgtggagatgcgtgggaataacgccgacaccccaggctgcagcatcctgagctccagggccgcggtccgactcctcccccggtcccaggcttcatcctggcctgggcttctccgaggcagggctggggccgcactgtgtgaggggctcaggctcagggcggtcccaggcctgggtggggcccagaggtgcctctgcttcacaggaaatcgtgagcgtgttcatagacgtgcagtcgcctgctttgtgttccttcatgcactttcatcagggatcttttctgattgtaagtgatgcttatgtcccactgtgccagtcgtccacagccctggggggatctgag

SEQ ID NO: 14721 - RNA, 2934 nt, Homo sapiens
  source 1..2934: mol_type = other RNA
gctgggattacaggcatgagccaccgtgcctggcctttttcttttttaaacagggtcttgctctgtcacccagactagaggtgcagtggcacagtcatggctcactgcagcctcaatctcctgggctcaagtgatcctcaagggcctccagagtagcccaccaccatgcctggcttttttttttttttttttttttgtaagtagagacacatttcactgtgttggccaggctggtgtcgaactcctgggctcaagccattgcccacctcaaagtgctgggattacaagtgtgagccaccacacccaaccaggttatttgaacatttttaagtactgtattttctctattgtaatattgactgtcatctctgtgcaggttttttagtggttgctctaggttgaaacgctttgaattcttaggtatctaagagtgagcattttctttttttgactgctatactctcaccagttgccagcttctcatataaatattgtaaatgctctcgtttaggtaactcagcttctggagttgagggaacttcaaaatcagaagagctctgggaatctgcatttgtgctaagatttagcaaacttttttcctcgggtatatgtgtctcactgcttagagtagttggttctccagtactaggaactattgtcacatctttatctctgcttttcaaatcagagtaagtatcctttgggcaaattacattttgttccatgagagaggcaggaatattctctttgattgttggtctgtagtcagctttgtccaaggaagtaatatccccactgtttctctcttgggaagataacaaaacagtatcagattggctgtcccagccttgacttccttgttctgttatgtgtgttgactgggaagaattctgggaggagatgtgagttgattctccatcagagtcactgaaaagctttggtgactgagatccccctgccactgtggaggaagggaagttttccaaactctcatctgtgatttcatcatttcttttaaagaatacttcccactggggtacatccccatcagccttttgcaggtgaagtacagagcccagatctccttgcagtgaagctgggattcctacttcttcttcactttcactgttggattcttcacaatctacaaagtttgtgaaacgagagctctgcatacactctgctctgcagcatcctggggtttgtctcagtttttcaggctgcttttctgatactgcagtcattgaaaatacctcagggtgaaaagtttccgggtatggaactttgtgccttaaaggtattggcagaggatcatcaaagagatagtcatcttcctcctcgtgccaggaacagtgtcttgtcctggtcccaacagccagagtggaaaacctcatgatccatgggcatttgtaaaagaaccaagaagagccttgcctcagtagtggggaaaattaaccatatactaaatgctactctgttcctgagtctcggtgaactgttctagctctcttcagttttcccagtggtttatactttggctccgtactttgggaagaccggcataaaggctttaagatttcgacaactttatccatagttgtgccaactggaatgacatttggatatgcgttcacaggacagaggtagctcaagaaatctttaatctcactgtaggaggagtgaaaagaaaaacaagctctgtatgaactctctccagtcctcacaattacatttgtttttctgctcctttctccaaaccacatggtggatggcttaatgctgattatgtggagtggaattctatttctggaagtaattccacagggtaatttgctccactgaaaatattcctctgccttgggatgccggcatgcatggatctgagtgttgcggtctgttgtgagatgatgaaggatctcaggcatgttcctaaacatgtctagcttattcacatgaacctggactcctaattcttcactaaggttggtgaacagatattcatagccataagccgctttgcagttcagccacacaacatggtacgggctccgagtgatccagcttcggaccagctctaagactccacttaaacactcctcccgacttggaatttggtaaaatcttggatcacagaacgtagtatccaaatatacactttggatgtctttgactctgcccccggagtgcagaagctccattctagcagcttctccttgcgccaatctgaagtctcctgtgtacaggacagttccattattgccctgaaataaaaacataactgatcccggacagtgaccagctggtaagagagtcacaacaatctcttccttctctcctgatgcttcatccactaaagatatctgggtaggagtctcgatttcaatagatatcttctggcttaactcagagtctggggcagggccgcagcaacatcagcttctgctgggtgcccgtgtgcagctcctccgagtcctggggcaggtgcatgtgcttcagagccaaagcgggagaccagcaaattcgtttcttccaaaatctgtatttcgggctcgttaacaacaactccttagtcacaggtgaacagtatagataaaccttcaagctggctggaatcctggtcctgccacttactggctgtgtgacactgggcaactaatttaacctctctggttcctcagtttcctcatctgcactccaaccttcttttcaaggtaggggctcttaatcctttcatgtgatctttgtggcagtgggacaggaagtaggcgcgggccctcaggttctccctatcgaagcggtctatggagatagttggatactcggccatctgcccctcgaaagaactcatagcgccgccgatcccagagtccgggaccccaaaaccgcagctgaagccaaggccagccctgaccgcgccgccacttccgggaagcc

SEQ ID NO: 14722 - RNA, 2712 nt, Homo sapiens
  source 1..2712: mol_type = other RNA
gctgggattacaggcatgagccaccgtgcctggcctttttcttttttaaacagggtcttgctctgtcacccagactagaggtgcagtggcacagtcatggctcactgcagcctcaatctcctgggctcaagtgatcctcaagggcctccagagtagcccaccaccatgcctggcttttttttttttttttttttttgtaagtagagacacatttcactgtgttggccaggctggtgtcgaactcctgggctcaagccattgcccacctcaaagtgctgggattacaagtgtgagccaccacacccaaccaggttatttgaacatttttaagtactgtattttctctattgtaatattgactgtcatctctgtgcaggttttttagtggttgctctaggttgaaacgctttgaattcttaggtatctaagagtgagcattttctttttttgactgctatactctcaccagttgccagcttctcatataaatattgtaaatgctctcgtttaggtaactcagcttctggagttgagggaacttcaaaatcagaagagctctgggaatctgcatttgtgctaagatttagcaaacttttttcctcgggtatatgtgtctcactgcttagagtagttggttctccagtactaggaactattgtcacatctttatctctgcttttcaaatcagagtaagtatcctttgggcaaattacattttgttccatgagagaggcaggaatattctctttgattgttggtctgtagtcagctttgtccaaggaagtaatatccccactgtttctctcttgggaagataacaaaacagtatcagattggctgtcccagccttgacttccttgttctgttatgtgtgttgactgggaagaattctgggaggagatgtgagttgattctccatcagagtcactgaaaagctttggtgactgagatccccctgccactgtggaggaagggaagttttccaaactctcatctgtgatttcatcatttcttttaaagaatacttcccactggggtacatccccatcagccttttgcaggtgaagtacagagcccagatctccttgcagtgaagctgggattcctacttcttcttcactttcactgttggattcttcacaatctacaaagtttgtgaaacgagagctctgcatacactctgctctgcagcatcctggggtttgtctcagtttttcaggctgcttttctgatactgcagtcattgaaaatacctcagggtgaaaagtttccgggtatggaactttgtgccttaaaggtattggcagaggatcatcaaagagatagtcatcttcctcctctgagtctcggtgaactgttctagctctcttcagttttcccagtggtttatactttggctccgtactttgggaagaccggcataaaggctttaagatttcgacaactttatccatagttgtgccaactggaatgacatttggatatgcgttcacaggacagaggtagctcaagaaatctttaatctcactgtaggaggagtgaaaagaaaaacaagctctgtatgaactctctccagtcctcacaattacatttgtttttctgctcctttctccaaaccacatggtggatggcttaatgctgattatgtggagtggaattctatttctggaagtaattccacagggtaatttgctccactgaaaatattcctctgccttgggatgccggcatgcatggatctgagtgttgcggtctgttgtgagatgatgaaggatctcaggcatgttcctaaacatgtctagcttattcacatgaacctggactcctaattcttcactaaggttggtgaacagatattcatagccataagccgctttgcagttcagccacacaacatggtacgggctccgagtgatccagcttcggaccagctctaagactccacttaaacactcctcccgacttggaatttggtaaaatcttggatcacagaacgtagtatccaaatatacactttggatgtctttgactctgcccccggagtgcagaagctccattctagcagcttctccttgcgccaatctgaagtctcctgtgtacaggacagttccattattgccctgaaataaaaacataactgatcccggacagtgaccagctggtaagagagtcacaacaatctcttccttctctcctgatgcttcatccactaaagatatctgggtaggagtctcgatttcaatagatataattcgtttcttccaaaatctgtatttcgggctcgttaacaacaactccttagtcacaggtgaacagtatagataaaccttcaagctatgcacaccatttcagtgccaccaagagcacaaggtgggggtggaaacacggtgtccctggacctcctccaacagtggtccctcaccattgttacttggaaatacgcgcttgtatgtgatcaggtgtgtctgcactccaaccttcttttcaaggtaggggctcttaatcctttcatgtgatctttgtggcagtgggacaggaagtaggcgcgggccctcaggttctccctatcgaagcggtctatggagatagttggatactcggccatctgcccctcgaaagaactcatagcgccgccgatcccagagtccgggaccccaaaaccgcagctgaagccaaggccagccctgaccgcgccgccacttccgggaagcc

SEQ ID NO: 14723 - RNA, 2581 nt, Homo sapiens
  source 1..2581: mol_type = other RNA
gctgggattacaggcatgagccaccgtgcctggcctttttcttttttaaacagggtcttgctctgtcacccagactagaggtgcagtggcacagtcatggctcactgcagcctcaatctcctgggctcaagtgatcctcaagggcctccagagtagcccaccaccatgcctggcttttttttttttttttttttttgtaagtagagacacatttcactgtgttggccaggctggtgtcgaactcctgggctcaagccattgcccacctcaaagtgctgggattacaagtgtgagccaccacacccaaccaggttatttgaacatttttaagtactgtattttctctattgtaatattgactgtcatctctgtgcaggttttttagtggttgctctaggttgaaacgctttgaattcttaggtatctaagagtgagcattttctttttttgactgctatactctcaccagttgccagcttctcatataaatattgtaaatgctctcgtttaggtaactcagcttctggagttgagggaacttcaaaatcagaagagctctgggaatctgcatttgtgctaagatttagcaaacttttttcctcgggtatatgtgtctcactgcttagagtagttggttctccagtactaggaactattgtcacatctttatctctgcttttcaaatcagagtaagtatcctttgggcaaattacattttgttccatgagagaggcaggaatattctctttgattgttggtctgtagtcagctttgtccaaggaagtaatatccccactgtttctctcttgggaagataacaaaacagtatcagattggctgtcccagccttgacttccttgttctgttatgtgtgttgactgggaagaattctgggaggagatgtgagttgattctccatcagagtcactgaaaagctttggtgactgagatccccctgccactgtggaggaagggaagttttccaaactctcatctgtgatttcatcatttcttttaaagaatacttcccactggggtacatccccatcagccttttgcaggtgaagtacagagcccagatctccttgcagtgaagctgggattcctacttcttcttcactttcactgttggattcttcacaatctacaaagtttgtgaaacgagagctctgcatacactctgctctgcagcatcctggggtttgtctcagtttttcaggctgcttttctgatactgcagtcattgaaaatacctcagggtgaaaagtttccgggtatggaactttgtgccttaaaggtattggcagaggatcatcaaagagatagtcatcttcctcctctgagtctcggtgaactgttctagctctcttcagttttcccagtggtttatactttggctccgtactttgggaagaccggcataaaggctttaagatttcgacaactttatccatagttgtgccaactggaatgacatttggatatgcgttcacaggacagaggtagctcaagaaatctttaatctcactgtaggaggagtgaaaagaaaaacaagctctgtatgaactctctccagtcctcacaattacatttgtttttctgctcctttctccaaaccacatggtggatggcttaatgctgattatgtggagtggaattctatttctggaagtaattccacagggtaatttgctccactgaaaatattcctctgccttgggatgccggcatgcatggatctgagtgttgcggtctgttgtgagatgatgaaggatctcaggcatgttcctaaacatgtctagcttattcacatgaacctggactcctaattcttcactaaggttggtgaacagatattcatagccataagccgctttgcagttcagccacacaacatggtacgggctccgagtgatccagcttcggaccagctctaagactccacttaaacactcctcccgacttggaatttggtaaaatcttggatcacagaacgtagtatccaaatatacactttggatgtctttgactctgcccccggagtgcagaagctccattctagcagcttctccttgcgccaatctgaagtctcctgtgtacaggacagttccattattgccctgaaataaaaacataactgatcccggacagtgaccagctggtaagagagtcacaacaatctcttccttctctcctgatgcttcatccactaaagatatctgggtaggagtctcgatttcaatagatataattcgtttcttccaaaatctgtatttcgggctcgttaacaacaactccttagtcacaggtgaacagtatagataaaccttcaagctgcactccaaccttcttttcaaggtaggggctcttaatcctttcatgtgatctttgtggcagtgggacaggaagtaggcgcgggccctcaggttctccctatcgaagcggtctatggagatagttggatactcggccatctgcccctcgaaagaactcatagcgccgccgatcccagagtccgggaccccaaaaccgcagctgaagccaaggccagccctgaccgcgccgccacttccgggaagcc

SEQ ID NO: 14724 - RNA, 2666 nt, Homo sapiens
  source 1..2666: mol_type = other RNA
gctgggattacaggcatgagccaccgtgcctggcctttttcttttttaaacagggtcttgctctgtcacccagactagaggtgcagtggcacagtcatggctcactgcagcctcaatctcctgggctcaagtgatcctcaagggcctccagagtagcccaccaccatgcctggcttttttttttttttttttttttgtaagtagagacacatttcactgtgttggccaggctggtgtcgaactcctgggctcaagccattgcccacctcaaagtgctgggattacaagtgtgagccaccacacccaaccaggttatttgaacatttttaagtactgtattttctctattgtaatattgactgtcatctctgtgcaggttttttagtggttgctctaggttgaaacgctttgaattcttaggtatctaagagtgagcattttctttttttgactgctatactctcaccagttgccagcttctcatataaatattgtaaatgctctcgtttaggtaactcagcttctggagttgagggaacttcaaaatcagaagagctctgggaatctgcatttgtgctaagatttagcaaacttttttcctcgggtatatgtgtctcactgcttagagtagttggttctccagtactaggaactattgtcacatctttatctctgcttttcaaatcagagtaagtatcctttgggcaaattacattttgttccatgagagaggcaggaatattctctttgattgttggtctgtagtcagctttgtccaaggaagtaatatccccactgtttctctcttgggaagataacaaaacagtatcagattggctgtcccagccttgacttccttgttctgttatgtgtgttgactgggaagaattctgggaggagatgtgagttgattctccatcagagtcactgaaaagctttggtgactgagatccccctgccactgtggaggaagggaagttttccaaactctcatctgtgatttcatcatttcttttaaagaatacttcccactggggtacatccccatcagccttttgcaggtgaagtacagagcccagatctccttgcagtgaagctgggattcctacttcttcttcactttcactgttggattcttcacaatctacaaagtttgtgaaacgagagctctgcatacactctgctctgcagcatcctggggtttgtctcagtttttcaggctgcttttctgatactgcagtcattgaaaatacctcagggtgaaaagtttccgggtatggaactttgtgccttaaaggtattggcagaggatcatcaaagagatagtcatcttcctcctctgagtctcggtgaactgttctagctctcttcagttttcccagtggtttatactttggctccgtactttgggaagaccggcataaaggctttaagatttcgacaactttatccatagttgtgccaactggaatgacatttggatatgcgttcacaggacagaggtagctcaagaaatctttaatctcactgtaggaggagtgaaaagaaaaacaagctctgtatgaactctctccagtcctcacaattacatttgtttttctgctcctttctccaaaccacatggtggatggcttaatgctgattatgtggagtggaattctatttctggaagtaattccacagggtaatttgctccactgaaaatattcctctgccttgggatgccggcatgcatggatctgagtgttgcggtctgttgtgagatgatgaaggatctcaggcatgttcctaaacatgtctagcttattcacatgaacctggactcctaattcttcactaaggttggtgaacagatattcatagccataagccgctttgcagttcagccacacaacatggtacgggctccgagtgatccagcttcggaccagctctaagactccacttaaacactcctcccgacttggaatttggtaaaatcttggatcacagaacgtagtatccaaatatacactttggatgtctttgactctgcccccggagtgcagaagctccattctagcagcttctccttgcgccaatctgaagtctcctgtgtacaggacagttccattattgccctgaaataaaaacataactgatcccggacagtgaccagctggtaagagagtcacaacaatctcttccttctctcctgatgcttcatccactaaagatatctgggtaggagtctcgatttcaatagatataattcgtttcttccaaaatctgtatttcgggctcgttaacaacaactccttagtcacaggtgaacagtatagataaaccttcaagctggctggaatcctggtcctgccacttactggctgtgtgacactgggcaactaatttaacctctctggttcctcagtttcctcatctgcactccaaccttcttttcaaggtaggggctcttaatcctttcatgtgatctttgtggcagtgggacaggaagtaggcgcgggccctcaggttctccctatcgaagcggtctatggagatagttggatactcggccatctgcccctcgaaagaactcatagcgccgccgatcccagagtccgggaccccaaaaccgcagctgaagccaaggccagccctgaccgcgccgccacttccgggaagcc

SEQ ID NO: 14725 - RNA, 2496 nt, Homo sapiens
  source 1..2496: mol_type = other RNA
gctgggattacaggcatgagccaccgtgcctggcctttttcttttttaaacagggtcttgctctgtcacccagactagaggtgcagtggcacagtcatggctcactgcagcctcaatctcctgggctcaagtgatcctcaagggcctccagagtagcccaccaccatgcctggcttttttttttttttttttttttgtaagtagagacacatttcactgtgttggccaggctggtgtcgaactcctgggctcaagccattgcccacctcaaagtgctgggattacaagtgtgagccaccacacccaaccaggttatttgaacatttttaagtactgtattttctctattgtaatattgactgtcatctctgtgcaggttttttagtggttgctctaggttgaaacgctttgaattcttaggtatctaagagtgagcattttctttttttgactgctatactctcaccagttgccagcttctcatataaatattgtaaatgctctcgtttaggtaactcagcttctggagttgagggaacttcaaaatcagaagagctctgggaatctgcatttgtgctaagatttagcaaacttttttcctcgggtatatgtgtctcactgcttagagtagttggttctccagtactaggaactattgtcacatctttatctctgcttttcaaatcagagtaagtatcctttgggcaaattacattttgttccatgagagaggcaggaatattctctttgattgttggtctgtagtcagctttgtccaaggaagtaatatccccactgtttctctcttgggaagataacaaaacagtatcagattggctgtcccagccttgacttccttgttctgttatgtgtgttgactgggaagaattctgggaggagatgtgagttgattctccatcagagtcactgaaaagctttggtgactgagatccccctgccactgtggaggaagggaagttttccaaactctcatctgtgatttcatcatttcttttaaagaatacttcccactggggtacatccccatcagccttttgcaggtgaagtacagagcccagatctccttgcagtgaagctgggattcctacttcttcttcactttcactgttggattcttcacaatctacaaagtttgtgaaacgagagctctgcatacactctgctctgcagcatcctggggtttgtctcagtttttcaggctgcttttctgatactgcagtcattgaaaatacctcagggtgaaaagtttccgggtatggaactttgtgccttaaaggtattggcagaggatcatcaaagagatagtcatcttcctcctctgagtctcggtgaactgttctagctctcttcagttttcccagtggtttatactttggctccgtactttgggaagaccggcataaaggctttaagatttcgacaactttatccatagttgtgccaactggaatgacatttggatatgcgttcacaggacagaggtagctcaagaaatctttaatctcactgtaggaggagtgaaaagaaaaacaagctctgtatgaactctctccagtcctcacaattacatttgtttttctgctcctttctccaaaccacatggtggatggcttaatgctgattatgtggagtggaattctatttctggaagtaattccacagggtaatttgctccactgaaaatattcctctgccttgggatgccggcatgcatggatctgagtgttgcggtctgttgtgagatgatgaaggatctcaggcatgttcctaaacatgtctagcttattcacatgaacctggactcctaattcttcactaaggttggtgaacagatattcatagccataagccgctttgcagttcagccacacaacatggtacgggctccgagtgatccagcttcggaccagctctaagactccacttaaacactcctcccgacttggaatttggtaaaatcttggatcacagaacgtagtatccaaatatacactttggatgtctttgactctgcccccggagtgcagaagctccattctagcagcttctccttgcgccaatctgaagtctcctgtgtacaggacagttccattattgccctgaaataaaaacataactgatcccggacagtgaccagctggtaagagagtcacaacaatctcttccttctctcctgatgcttcatccactaaagatatctgggtaggagtctcgatttcaatagatataattcgtttcttccaaaatctgtatttcgggctcgttaacaacaactccttagtcacaggtgaacagtatagataaaccttcaagctttgtggcagtgggacaggaagtaggcgcgggccctcaggttctccctatcgaagcggtctatggagatagttggatactcggccatctgcccctcgaaagaactcatagcgccgccgatcccagagtccgggaccccaaaaccgcagctgaagccaaggc

SEQ ID NO: 14726 - RNA, 3034 nt, Homo sapiens
  source 1..3034: mol_type = other RNA
gctgggattacaggcatgagccaccgtgcctggcctttttcttttttaaacagggtcttgctctgtcacccagactagaggtgcagtggcacagtcatggctcactgcagcctcaatctcctgggctcaagtgatcctcaagggcctccagagtagcccaccaccatgcctggcttttttttttttttttttttttgtaagtagagacacatttcactgtgttggccaggctggtgtcgaactcctgggctcaagccattgcccacctcaaagtgctgggattacaagtgtgagccaccacacccaaccaggttatttgaacatttttaagtactgtattttctctattgtaatattgactgtcatctctgtgcaggttttttagtggttgctctaggttgaaacgctttgaattcttaggtatctaagagtgagcattttctttttttgactgctatactctcaccagttgccagcttctcatataaatattgtaaatgctctcgtttaggtaactcagcttctggagttgagggaacttcaaaatcagaagagctctgggaatctgcatttgtgctaagatttagcaaacttttttcctcgggtatatgtgtctcactgcttagagtagttggttctccagtactaggaactattgtcacatctttatctctgcttttcaaatcagagtaagtatcctttgggcaaattacattttgttccatgagagaggcaggaatattctctttgattgttggtctgtagtcagctttgtccaaggaagtaatatccccactgtttctctcttgggaagataacaaaacagtatcagattggctgtcccagccttgacttccttgttctgttatgtgtgttgactgggaagaattctgggaggagatgtgagttgattctccatcagagtcactgaaaagctttggtgactgagatccccctgccactgtggaggaagggaagttttccaaactctcatctgtgatttcatcatttcttttaaagaatacttcccactggggtacatccccatcagccttttgcaggtgaagtacagagcccagatctccttgcagtgaagctgggattcctacttcttcttcactttcactgttggattcttcacaatctacaaagtttgtgaaacgagagctctgcatacactctgctctgcagcatcctggggtttgtctcagtttttcaggctgcttttctgatactgcagtcattgaaaatacctcagggtgaaaagtttccgggtatggaactttgtgccttaaaggtattggcagaggatcatcaaagagatagtcatcttcctcctctgagtctcggtgaactgttctagctctcttcagttttcccagtggtttatactttggctccgtactttgggaagaccggcataaaggctttaagatttcgacaactttatccatagttgtgccaactggaatgacatttggatatgcgttcacaggacagaggtagctcaagaaatctttaatctcactgtaggaggagtgaaaagaaaaacaagctctgtatgaactctctccagtcctcacaattacatttgtttttctgctcctttctccaaaccacatggtggatggcttaatgctgattatgtggagtggaattctatttctggaagtaattccacagggtaatttgctccactgaaaatattcctctgccttgggatgccggcatgcatggatctgagtgttgcggtctgttgtgagatgatgaaggatctcaggcatgttcctaaacatgtctagcttattcacatgaacctggactcctaattcttcactaaggttggtgaacagatattcatagccataagccgctttgcagttcagccacacaacatggtacgggctccgagtgatccagcttcggaccagctctaagactccacttaaacactcctcccgacttggaatttggtaaaatcttggatcacagaacgtagtatccaaatatacactttggatgtctttgactctgcccccggagtgcagaagctccattctagcagcttctccttgcgccaatctgaagtctcctgtgtacaggacagttccattattgccctgaaataaaaacataactgatcccggacagtgaccagctggtaagagagtcacaacaatctcttccttctctcctgatgcttcatccactaaagatatctgggtaggagtctcgatttcaatagatatcttctggcttaactcagagtctggggcagggccgcagcaacatcagcttctgctgggtgcccgtgtgcagctcctccgagtcctggggcaggtgcatgtgcttcagagccaaagcgggagaccagcactattgaggccagaggaagtgagagacagaagtgggtttcggtctgtcctagtgggccattctgccttccagtttgtctctgttcccctccacttctcttccagctttccttcctgactgctggccgggctgacctgtagtaacttcaagctgaatgccagagacaacaggaacaaccctgctgttgtgactgctaattcgtttcttccaaaatctgtatttcgggctcgttaacaacaactccttagtcacaggtgaacagtatagataaaccttcaagctatgcacaccatttcagtgccaccaagagcacaaggtgggggtggaaacacggtgtccctggacctcctccaacagtggtccctcaccattgttacttggaaatacgcgcttgtatgtgatcaggtgtgtctgcactccaaccttcttttcaaggtaggggctcttaatcctttcatgtgatctttgtggcagtgggacaggaagtaggcgcgggccctcaggttctccctatcgaagcggtctatggagatagttggatactcggccatctgcccctcgaaagaactcatagcgccgccgatcccagagtccgggaccccaaaaccgcagctgaagccaaggccagccctgaccgcgccgccacttccgggaagcc

SEQ ID NO: 14727 - RNA, 2988 nt, Homo sapiens
  source 1..2988: mol_type = other RNA
gctgggattacaggcatgagccaccgtgcctggcctttttcttttttaaacagggtcttgctctgtcacccagactagaggtgcagtggcacagtcatggctcactgcagcctcaatctcctgggctcaagtgatcctcaagggcctccagagtagcccaccaccatgcctggcttttttttttttttttttttttgtaagtagagacacatttcactgtgttggccaggctggtgtcgaactcctgggctcaagccattgcccacctcaaagtgctgggattacaagtgtgagccaccacacccaaccaggttatttgaacatttttaagtactgtattttctctattgtaatattgactgtcatctctgtgcaggttttttagtggttgctctaggttgaaacgctttgaattcttaggtatctaagagtgagcattttctttttttgactgctatactctcaccagttgccagcttctcatataaatattgtaaatgctctcgtttaggtaactcagcttctggagttgagggaacttcaaaatcagaagagctctgggaatctgcatttgtgctaagatttagcaaacttttttcctcgggtatatgtgtctcactgcttagagtagttggttctccagtactaggaactattgtcacatctttatctctgcttttcaaatcagagtaagtatcctttgggcaaattacattttgttccatgagagaggcaggaatattctctttgattgttggtctgtagtcagctttgtccaaggaagtaatatccccactgtttctctcttgggaagataacaaaacagtatcagattggctgtcccagccttgacttccttgttctgttatgtgtgttgactgggaagaattctgggaggagatgtgagttgattctccatcagagtcactgaaaagctttggtgactgagatccccctgccactgtggaggaagggaagttttccaaactctcatctgtgatttcatcatttcttttaaagaatacttcccactggggtacatccccatcagccttttgcaggtgaagtacagagcccagatctccttgcagtgaagctgggattcctacttcttcttcactttcactgttggattcttcacaatctacaaagtttgtgaaacgagagctctgcatacactctgctctgcagcatcctggggtttgtctcagtttttcaggctgcttttctgatactgcagtcattgaaaatacctcagggtgaaaagtttccgggtatggaactttgtgccttaaaggtattggcagaggatcatcaaagagatagtcatcttcctcctctgagtctcggtgaactgttctagctctcttcagttttcccagtggtttatactttggctccgtactttgggaagaccggcataaaggctttaagatttcgacaactttatccatagttgtgccaactggaatgacatttggatatgcgttcacaggacagaggtagctcaagaaatctttaatctcactgtaggaggagtgaaaagaaaaacaagctctgtatgaactctctccagtcctcacaattacatttgtttttctgctcctttctccaaaccacatggtggatggcttaatgctgattatgtggagtggaattctatttctggaagtaattccacagggtaatttgctccactgaaaatattcctctgccttgggatgccggcatgcatggatctgagtgttgcggtctgttgtgagatgatgaaggatctcaggcatgttcctaaacatgtctagcttattcacatgaacctggactcctaattcttcactaaggttggtgaacagatattcatagccataagccgctttgcagttcagccacacaacatggtacgggctccgagtgatccagcttcggaccagctctaagactccacttaaacactcctcccgacttggaatttggtaaaatcttggatcacagaacgtagtatccaaatatacactttggatgtctttgactctgcccccggagtgcagaagctccattctagcagcttctccttgcgccaatctgaagtctcctgtgtacaggacagttccattattgccctgaaataaaaacataactgatcccggacagtgaccagctggtaagagagtcacaacaatctcttccttctctcctgatgcttcatccactaaagatatctgggtaggagtctcgatttcaatagatatcttctggcttaactcagagtctggggcagggccgcagcaacatcagcttctgctgggtgcccgtgtgcagctcctccgagtcctggggcaggtgcatgtgcttcagagccaaagcgggagaccagcactattgaggccagaggaagtgagagacagaagtgggtttcggtctgtcctagtgggccattctgccttccagtttgtctctgttcccctccacttctcttccagctttccttcctgactgctggccgggctgacctgtagtaacttcaagctgaatgccagagacaacaggaacaaccctgctgttgtgactgctaattcgtttcttccaaaatctgtatttcgggctcgttaacaacaactccttagtcacaggtgaacagtatagataaaccttcaagctggctggaatcctggtcctgccacttactggctgtgtgacactgggcaactaatttaacctctctggttcctcagtttcctcatctgcactccaaccttcttttcaaggtaggggctcttaatcctttcatgtgatctttgtggcagtgggacaggaagtaggcgcgggccctcaggttctccctatcgaagcggtctatggagatagttggatactcggccatctgcccctcgaaagaactcatagcgccgccgatcccagagtccgggaccccaaaaccgcagctgaagccaaggccagccctgaccgcgccgccacttccgggaagcc

SEQ ID NO: 14728 - RNA, 2525 nt, Homo sapiens
  source 1..2525: mol_type = other RNA
gctgggattacaggcatgagccaccgtgcctggcctttttcttttttaaacagggtcttgctctgtcacccagactagaggtgcagtggcacagtcatggctcactgcagcctcaatctcctgggctcaagtgatcctcaagggcctccagagtagcccaccaccatgcctggcttttttttttttttttttttttgtaagtagagacacatttcactgtgttggccaggctggtgtcgaactcctgggctcaagccattgcccacctcaaagtgctgggattacaagtgtgagccaccacacccaaccaggttatttgaacatttttaagtactgtattttctctattgtaatattgactgtcatctctgtgcaggttttttagtggttgctctaggttgaaacgctttgaattcttaggtatctaagagtgagcattttctttttttgactgctatactctcaccagttgccagcttctcatataaatattgtaaatgctctcgtttaggtaactcagcttctggagttgagggaacttcaaaatcagaagagctctgggaatctgcatttgtgctaagatttagcaaacttttttcctcgggtatatgtgtctcactgcttagagtagttggttctccagtactaggaactattgtcacatctttatctctgcttttcaaatcagagtaagtatcctttgggcaaattacattttgttccatgagagaggcaggaatattctctttgattgttggtctgtagtcagctttgtccaaggaagtaatatccccactgtttctctcttgggaagataacaaaacagtatcagattggctgtcccagccttgacttccttgttctgttatgtgtgttgactgggaagaattctgggaggagatgtgagttgattctccatcagagtcactgaaaagctttggtgactgagatccccctgccactgtggaggaagggaagttttccaaactctcatctgtgatttcatcatttcttttaaagaatacttcccactggggtacatccccatcagccttttgcaggtgaagtacagagcccagatctccttgcagtgaagctgggattcctacttcttcttcactttcactgttggattcttcacaatctacaaagtttgtgaaacgagagctctgcatacactctgctctgcagcatcctggggtttgtctcagtttttcaggctgcttttctgatactgcagtcattgaaaatacctcagggtgaaaagtttccgggtatggaactttgtgccttaaaggtattggcagaggatcatcaaagagatagtcatcttcctcctctgagtctcggtgaactgttctagctctcttcagttttcccagtggtttatactttggctccgtactttgggaagaccggcataaaggctttaagatttcgacaactttatccatagttgtgccaactggaatgacatttggatatgcgttcacaggacagaggtagctcaagaaatctttaatctcactgtaggaggagtgaaaagaaaaacaagctctgtatgaactctctccagtcctcacaattacatttgtttttctgctcctttctccaaaccacatggtggatggcttaatgctgattatgtggagtggaattctatttctggaagtaattccacagggtaatttgctccactgaaaatattcctctgccttgggatgccggcatgcatggatctgagtgttgcggtctgttgtgagatgatgaaggatctcaggcatgttcctaaacatgtctagcttattcacatgaacctggactcctaattcttcactaaggttggtgaacagatattcatagccataagccgctttgcagttcagccacacaacatggtacgggctccgagtgatccagcttcggaccagctctaagactccacttaaacactcctcccgacttggaatttggtaaaatcttggatcacagaacgtagtatccaaatatacactttggatgtctttgactctgcccccggagtgcagaagctccattctagcagcttctccttgcgccaatctgaagtctcctgtgtacaggacagttccattattgccctgaaataaaaacctctcctgatgcttcatccactaaagatatctgggtaggagtctcgatttcaatagatataattcgtttcttccaaaatctgtatttcgggctcgttaacaacaactccttagtcacaggtgaacagtatagataaaccttcaagctgcactccaaccttcttttcaaggtaggggctcttaatcctttcatgtgatctttgtggcagtgggacaggaagtaggcgcgggccctcaggttctccctatcgaagcggtctatggagatagttggatactcggccatctgcccctcgaaagaactcatagcgccgccgatcccagagtccgggaccccaaaaccgcagctgaagccaaggccagccctgaccgcgccgccacttccgggaagcc

SEQ ID NO: 14729 - RNA, 2473 nt, Homo sapiens
  source 1..2473: mol_type = other RNA
gctgggattacaggcatgagccaccgtgcctggcctttttcttttttaaacagggtcttgctctgtcacccagactagaggtgcagtggcacagtcatggctcactgcagcctcaatctcctgggctcaagtgatcctcaagggcctccagagtagcccaccaccatgcctggcttttttttttttttttttttttgtaagtagagacacatttcactgtgttggccaggctggtgtcgaactcctgggctcaagccattgcccacctcaaagtgctgggattacaagtgtgagccaccacacccaaccaggttatttgaacatttttaagtactgtattttctctattgtaatattgactgtcatctctgtgcaggttttttagtggttgctctaggttgaaacgctttgaattcttaggtatctaagagtgagcattttctttttttgactgctatactctcaccagttgccagcttctcatataaatattgtaaatgctctcgtttaggtaactcagcttctggagttgagggaacttcaaaatcagaagagctctgggaatctgcatttgtgctaagatttagcaaacttttttcctcgggtatatgtgtctcactgcttagagtagttggttctccagtactaggaactattgtcacatctttatctctgcttttcaaatcagagtaagtatcctttgggcaaattacattttgttccatgagagaggcaggaatattctctttgattgttggtctgtagtcagctttgtccaaggaagtaatatccccactgtttctctcttgggaagataacaaaacagtatcagattggctgtcccagccttgacttccttgttctgttatgtgtgttgactgggaagaattctgggaggagatgtgagttgattctccatcagagtcactgaaaagctttggtgactgagatccccctgccactgtggaggaagggaagttttccaaactctcatctgtgatttcatcatttcttttaaagaatacttcccactggggtacatccccatcagccttttgcaggtgaagtacagagcccagatctccttgcagtgaagctgggattcctacttcttcttcactttcactgttggattcttcacaatctacaaagtttgtgaaacgagagctctgcatacactctgctctgcagcatcctggggtttgtctcagtttttcaggctgcttttctgatactgcagtcattgaaaatacctcagggtgaaaagtttccgggtatggaactttgtgccttaaaggtattggcagaggatcatcaaagagatagtcatcttcctcctctgagtctcggtgaactgttctagctctcttcagttttcccagtggtttatactttggctccgtactttgggaagaccggcataaaggctttaagatttcgacaactttatccatagttgtgccaactggaatgacatttggatatgcgttcacaggacagaggtagctcaagaaatctttaatctcactgtaggaggagtgaaaagaaaaacaagctctgtatgaactctctccagtcctcacaattacatttgtttttctgctcctttctccaaaccacatggtggatggcttaatgctgattatgtggagtggaattctatttctggaagtaattccacagggtaatttgctccactgaaaatattcctctgccttgggatgccggcatgcatggatctgagtgttgcggtctgttgtgagatgatgaaggatctcaggcatgttcctaaacatgtctagcttattcacatgaacctggactcctaattcttcactaaggttggtgaacagatattcatagccataagccgctttgcagttcagccacacaacatggtacgggctccgagtgatccagcttcggaccagctctaagactccacttaaacactcctcccgacttggaatttggtaaaatcttggatcacagaacgtagtatccaaatatacactttggatgtctttgactctgcccccggagtgcagaagctccattctagcagcttctccttgcgccaatctgaagtctcctgtgtacaggacagttccattattgccctgaaataaaaacctctcctgatgcttcatccactaaagatatctgggtaggagtctcgatttcaatagatataattcgtttcttccaaaatctgtatttcgggctcgttaacaacaactccttagtcacaggtgaacagtatagataaaccttcaagctttgtggcagtgggacaggaagtaggcgcgggccctcaggttctccctatcgaagcggtctatggagatagttggatactcggccatctgcccctcgaaagaactcatagcgccgccgatcccagagtccgggaccccaaaaccgcagctgaagccaaggccagccctgaccgcgccgccacttccgggaagcc

SEQ ID NO: 14730 - RNA, 2440 nt, Homo sapiens
  source 1..2440: mol_type = other RNA
gctgggattacaggcatgagccaccgtgcctggcctttttcttttttaaacagggtcttgctctgtcacccagactagaggtgcagtggcacagtcatggctcactgcagcctcaatctcctgggctcaagtgatcctcaagggcctccagagtagcccaccaccatgcctggcttttttttttttttttttttttgtaagtagagacacatttcactgtgttggccaggctggtgtcgaactcctgggctcaagccattgcccacctcaaagtgctgggattacaagtgtgagccaccacacccaaccaggttatttgaacatttttaagtactgtattttctctattgtaatattgactgtcatctctgtgcaggttttttagtggttgctctaggttgaaacgctttgaattcttaggtatctaagagtgagcattttctttttttgactgctatactctcaccagttgccagcttctcatataaatattgtaaatgctctcgtttaggtaactcagcttctggagttgagggaacttcaaaatcagaagagctctgggaatctgcatttgtgctaagatttagcaaacttttttcctcgggtatatgtgtctcactgcttagagtagttggttctccagtactaggaactattgtcacatctttatctctgcttttcaaatcagagtaagtatcctttgggcaaattacattttgttccatgagagaggcaggaatattctctttgattgttggtctgtagtcagctttgtccaaggaagtaatatccccactgtttctctcttgggaagataacaaaacagtatcagattggctgtcccagccttgacttccttgttctgttatgtgtgttgactgggaagaattctgggaggagatgtgagttgattctccatcagagtcactgaaaagctttggtgactgagatccccctgccactgtggaggaagggaagttttccaaactctcatctgtgatttcatcatttcttttaaagaatacttcccactggggtacatccccatcagccttttgcaggtgaagtacagagcccagatctccttgcagtgaagctgggattcctacttcttcttcactttcactgttggattcttcacaatctacaaagtttgtgaaacgagagctctgcatacactctgctctgcagcatcctggggtttgtctcagtttttcaggctgcttttctgatactgcagtcattgaaaatacctcagggtgaaaagtttccgggtatggaactttgtgccttaaaggtattggcagaggatcatcaaagagatagtcatcttcctcctctgagtctcggtgaactgttctagctctcttcagttttcccagtggtttatactttggctccgtactttgggaagaccggcataaaggctttaagatttcgacaactttatccatagttgtgccaactggaatgacatttggatatgcgttcacaggacagaggtagctcaagaaatctttaatctcactgtaggaggagtgaaaagaaaaacaagctctgtatgaactctctccagtcctcacaattacatttgtttttctgctcctttctccaaaccacatggtggatggcttaatgctgattatgtggagtggaattctatttctggaagtaattccacagggtaatttgctccactgaaaatattcctctgccttgggatgccggcatgcatggatctgagtgttgcggtctgttgtgagatgatgaaggatctcaggcatgttcctaaacatgtctagcttattcacatgaacctggactcctaattcttcactaaggttggtgaacagatattcatagccataagccgctttgcagttcagccacacaacatggtacgggctccgagtgatccagcttcggaccagctctaagactccacttaaacactcctcccgacttggaatttggtaaaatcttggatcacagaacgtagtatccaaatatacactttggatgtctttgactctgcccccggagtgcagaagctccattctagcagcttctccttgcgccaatctgaagtctcctgtgtacaggacagttccattattgccctgaaataaaaacctctcctgatgcttcatccactaaagatatctgggtaggagtctcgatttcaatagatatctgcactccaaccttcttttcaaggtaggggctcttaatcctttcatgtgatctttgtggcagtgggacaggaagtaggcgcgggccctcaggttctccctatcgaagcggtctatggagatagttggatactcggccatctgcccctcgaaagaactcatagcgccgccgatcccagagtccgggaccccaaaaccgcagctgaagccaaggccagccctgaccgcgccgccacttccgggaagcc

SEQ ID NO: 14731 - RNA, 2982 nt, Homo sapiens
  source 1..2982: mol_type = other RNA
gctgggattacaggcatgagccaccgtgcctggcctttttcttttttaaacagggtcttgctctgtcacccagactagaggtgcagtggcacagtcatggctcactgcagcctcaatctcctgggctcaagtgatcctcaagggcctccagagtagcccaccaccatgcctggcttttttttttttttttttttttgtaagtagagacacatttcactgtgttggccaggctggtgtcgaactcctgggctcaagccattgcccacctcaaagtgctgggattacaagtgtgagccaccacacccaaccaggttatttgaacatttttaagtactgtattttctctattgtaatattgactgtcatctctgtgcaggttttttagtggttgctctaggttgaaacgctttgaattcttaggtatctaagagtgagcattttctttttttgactgctatactctcaccagttgccagcttctcatataaatattgtaaatgctctcgtttaggtaactcagcttctggagttgagggaacttcaaaatcagaagagctctgggaatctgcatttgtgctaagatttagcaaacttttttcctcgggtatatgtgtctcactgcttagagtagttggttctccagtactaggaactattgtcacatctttatctctgcttttcaaatcagagtaagtatcctttgggcaaattacattttgttccatgagagaggcaggaatattctctttgattgttggtctgtagtcagctttgtccaaggaagtaatatccccactgtttctctcttgggaagataacaaaacagtatcagattggctgtcccagccttgacttccttgttctgttatgtgtgttgactgggaagaattctgggaggagatgtgagttgattctccatcagagtcactgaaaagctttggtgactgagatccccctgccactgtggaggaagggaagttttccaaactctcatctgtgatttcatcatttcttttaaagaatacttcccactggggtacatccccatcagccttttgcaggtgaagtacagagcccagatctccttgcagtgaagctgggattcctacttcttcttcactttcactgttggattcttcacaatctacaaagtttgtgaaacgagagctctgcatacactctgctctgcagcatcctggggtttgtctcagtttttcaggctgcttttctgatactgcagtcattgaaaatacctcagggtgaaaagtttccgggtatggaactttgtgccttaaaggtattggcagaggatcatcaaagagatagtcatcttcctcctctgagtctcggtgaactgttctagctctcttcagttttcccagtggtttatactttggctccgtactttgggaagaccggcataaaggctttaagccctttcgaaggcctcactgccaactgcctcctcctggcagattccgggaagcctttaggatgatatttcgacaactttatccatagttgtgccaactggaatgacatttggatatgcgttcacaggacagaggtagctcaagaaatctttaatctcactgtaggaggagtgaaaagaaaaacaagctctgtatgaactctctccagtcctcacaattacatttgtttttctgctcctttctccaaaccacatggtggatggcttaatgctgattatgtggagtggaattctatttctggaagtaattccacagggtaatttgctccactgaaaatattcctctgccttgggatgccggcatgcatggatctgagtgttgcggtctgttgtgagatgatgaaggatctcaggcatgttcctaaacatgtctagcttattcacatgaacctggactcctaattcttcactaaggttggtgaacagatattcatagccataagccgctttgcagttcagccacacaacatggtacgggctccgagtgatccagcttcggaccagctctaagactccacttaaacactcctcccgacttggaatttggtaaaatcttggatcacagaacgtagtatccaaatatacactttggatgtctttgactctgcccccggagtgcagaagctccattctagcagcttctccttgcgccaatctgaagtctcctgtgtacaggacagttccattattgccctgaaataaaaacataactgatcccggacagtgaccagctggtaagagagtcacaacaatctcttccttctctcctgatgcttcatccactaaagatatctgggtaggagtctcgatttcaatagatataattcgtttcttccaaaatctgtatttcgggctcgttaacaacaactccttagtcacaggtgaacagtatagataaaccttcaagctgcactccaaccttcttttcaaggtaggggctcttaatcctttcatgtgatctttgtggcagtgggacaggaagtaggcgcgggccctcaggttctccctatcgaagcggtctatggagatagttggatactcggccatctgcccctcgaaagaactcatagcgccgccgatcccagagtccgggaccccaaaaccgcagctgaagccaaggccagccctgaccgcgccgccacttccgggaagccgcgcgctgcctcgccattgggcggccgaacgcagccacgtccaatcagaggagtccggagaccgggggcaaagtcaaggagcatccggtcgggttctaggcgcccgctgcttgggtttaaatcacccgcgcttcgctgcacgcgatgggccctgagccctgcccagtgcaaggctcattcccgcccaacaaacacaggtgttgctctggtaaggcgttgcccatgtctgtggaggtgcagtcgcgggaagggaaatcgaaactcccagagcaggtggccccagccgacgaggtgagtgggctgcggaactgcgcttagaaatcattcttcgttccg

SEQ ID NO: 14732 - RNA, 2675 nt, Homo sapiens
  source 1..2675: mol_type = other RNA
gctgggattacaggcatgagccaccgtgcctggcctttttcttttttaaacagggtcttgctctgtcacccagactagaggtgcagtggcacagtcatggctcactgcagcctcaatctcctgggctcaagtgatcctcaagggcctccagagtagcccaccaccatgcctggcttttttttttttttttttttttgtaagtagagacacatttcactgtgttggccaggctggtgtcgaactcctgggctcaagccattgcccacctcaaagtgctgggattacaagtgtgagccaccacacccaaccaggttatttgaacatttttaagtactgtattttctctattgtaatattgactgtcatctctgtgcaggttttttagtggttgctctaggttgaaacgctttgaattcttaggtatctaagagtgagcattttctttttttgactgctatactctcaccagttgccagcttctcatataaatattgtaaatgctctcgtttaggtaactcagcttctggagttgagggaacttcaaaatcagaagagctctgggaatctgcatttgtgctaagatttagcaaacttttttcctcgggtatatgtgtctcactgcttagagtagttggttctccagtactaggaactattgtcacatctttatctctgcttttcaaatcagagtaagtatcctttgggcaaattacattttgttccatgagagaggcaggaatattctctttgattgttggtctgtagtcagctttgtccaaggaagtaatatccccactgtttctctcttgggaagataacaaaacagtatcagattggctgtcccagccttgacttccttgttctgttatgtgtgttgactgggaagaattctgggaggagatgtgagttgattctccatcagagtcactgaaaagctttggtgactgagatccccctgccactgtggaggaagggaagttttccaaactctcatctgtgatttcatcatttcttttaaagaatacttcccactggggtacatccccatcagccttttgcaggtgaagtacagagcccagatctccttgcagtgaagctgggattcctacttcttcttcactttcactgttggattcttcacaatctacaaagtttgtgaaacgagagctctgcatacactctgctctgcagcatcctggggtttgtctcagtttttcaggctgcttttctgatactgcagtcattgaaaatacctcagggtgaaaagtttccgggtatggaactttgtgccttaaaggtattggcagaggatcatcaaagagatagtcatcttcctcctctgagtctcggtgaactgttctagctctcttcagttttcccagtggtttatactttggctccgtactttgggaagaccggcataaaggctttaagccctttcgaaggcctcactgccaactgcctcctcctggcagattccgggaagcctttaggatgatatttcgacaactttatccatagttgtgccaactggaatgacatttggatatgcgttcacaggacagaggtagctcaagaaatctttaatctcactgtaggaggagtgaaaagaaaaacaagctctgtatgaactctctccagtcctcacaattacatttgtttttctgctcctttctccaaaccacatggtggatggcttaatgctgattatgtggagtggaattctatttctggaagtaattccacagggtaatttgctccactgaaaatattcctctgccttgggatgccggcatgcatggatctgagtgttgcggtctgttgtgagatgatgaaggatctcaggcatgttcctaaacatgtctagcttattcacatgaacctggactcctaattcttcactaaggttggtgaacagatattcatagccataagccgctttgcagttcagccacacaacatggtacgggctccgagtgatccagcttcggaccagctctaagactccacttaaacactcctcccgacttggaatttggtaaaatcttggatcacagaacgtagtatccaaatatacactttggatgtctttgactctgcccccggagtgcagaagctccattctagcagcttctccttgcgccaatctgaagtctcctgtgtacaggacagttccattattgccctgaaataaaaacctctcctgatgcttcatccactaaagatatctgggtaggagtctcgatttcaatagatataattcgtttcttccaaaatctgtatttcgggctcgttaacaacaactccttagtcacaggtgaacagtatagataaaccttcaagctggctggaatcctggtcctgccacttactggctgtgtgacactgggcaactaatttaacctctctggttcctcagtttcctcatctgcactccaaccttcttttcaaggtaggggctcttaatcctttcatgtgatctttgtggcagtgggacaggaagtaggcgcgggccctcaggttctccctatcgaagcggtctatggagatagttggatactcggccatctgcccctcgaaagaactcatagcgccgccgatcccagagtccgggaccccaaaaccgcagctgaagccaaggccagccctgaccgcgccgccacttccgggaagcc

SEQ ID NO: 14733 - RNA, 2696 nt, Homo sapiens
  source 1..2696: mol_type = other RNA
gctgggattacaggcatgagccaccgtgcctggcgtttgtttcccttctgtacagggagtttggggttgggtgaaaagacatctaagggtctttctatcccaggggtgtgtggtcccaggcagggagtcaggaggggcgccgtacgggaggttggcttgtcagcagcatagatggggtcactaaggccggcggttgggtgaccctcagcgctgggcccgaggtcgcgctagagacggaggccggggccgaggcagacaggccaaactgggcctggccagccgggagagggggaggcggcccaggaagagagggaggctgagacagaaagatgggcggggcacagggatgtctgcaaagaaggcacggtcccgagggggtgacagggctccctcctcagagagttccaggtcccgggccacggccaggatctcctggcgggcggctgtgttgcgcaggccacggatgtcgaggagggctgccacgtgcttctgcctgatgtctgggtagtcgcgcaccaacactcccacctccacctggatgctgggcgtgtcttccagctgcatgacttcagccaaatggggcaccacggcatccagccacgaggcctgggactccagccgccggaacagcctctgcagttgcgccgcgtcctcccggagcctgccggccacgcggctgcgggtccgcgccgagctgcagcgcaggcgcccacggagcaggggccgcacgtactcgaccagcgcccgccggtgtagctcggctaccagcgcctggtaaggctcgtcctgcattctgcgcagggccagggcctgggcacccagcgtgcccacgatgccatccagggcctccgggctgctcagccacttccggcgcatcagcttgttgaagtgtggctgcagctcctggaacagcaggttggccacgacacggtggcagagccgggtcacatggtccagagcactagcagatgcttcccgggccggctcgctttctgggggccccacccgggccaggcgctcggccagagctctcagtggggggccgcagttgaccagggcgatggtcttgctgatataggtgtcaggtagcatctcccggactgctgggttctcatggaatcgctccacacgctgctggaagctctgcaggaactctgccagcccgcctaggcagcagtgggccatccgctccccaaactcctggctgatgcggggtgctcgctctgtgtgctcttccagcagctcacacacatcctgggccaggctgctgggctggtcctccaggctcccccagtgctcttcgtcctcctgcagcacacggagaagggcagcccgggtctgagccttaacatctgtgacgcattcatcctccaaaccccgcagggtgccaggggagagaaggggccccagctccccattctccagggcggccatgtccaccagccctaggacctctctggggtagacctgattgtgccagtgcagcagcgcgtagcggtcggccagcggcagcctgcgacgggcggaggcccccagccactcggccagggccccgtggtagccgcgcaggtagacgccgaaggcgcccaggccggcggggtaggcgggcgccaggcggccccgcaccacggccatatcctccagcagccgcgcccgcagcgcctccagctgcccggccaggcccccgggcgccccgggagccgctgcctctaggcgctcccgggccgcgcgcgccacggcttcggcccagcgtgcgcgtagtttgcgggccgccccgggaccccgacgcccgtcggccgcctcctcctgtaccagcacctggcccagctgcgccaccgcgccagccccggcgcacgctcccggcccggggcccgccagcgtctcgcgcaccagcgcccacagctcgcgctgcagggcctcgtacagcagcgccacgtcccgcgcccggcggcccccgccagcgccctcggccttgggaggcccaggcgcgccgcccctcgacggcgccagctcctcggcctctagctccaggatgtgctcgtccgcacgcgctagttcgcgctgctggatcaggctcaggatctccagcactgacaatggctccttcatctttgggggctctgggaccttgggtgggggctctggagctgcctcgcctgcaggcaccactctctcagccagggacgcacgctggggcttggatccacgccccagtctcaggaaggccagtctccgggcggcctcccccgctgcctcctcgtcgccgtgggctcgggtcccatgcagccgggccaggaggccaaaatctgctgagctcctgcgtatccctggtaccagcacacggcccaagaaagagcggggctgcccatccccagggctgcctgcccgccggcccggggcccagcccagccggaagggggccaggcccgcaagcttctccagggtggcgcggcggcgacaagatgttccattggggagggaccccagctccccggcctcttcttcctccagccctgaaacttcttcaaaggggttccgagaggacctcaggggcagggtccccgcccggggcaccttagggtctgacactcccagattcttcaggataggcattttgacaggtggggacctctgtcctcctgcccgtccttctgttcccgctgctgtcctgtccccaggctacttcagccaggact

SEQ ID NO: 14734 - RNA, 2545 nt, Homo sapiens
  source 1..2545: mol_type = other RNA
gctgggattacaggcatgagccaccgtgcctggctaagctttccattctcagtgaagaaagtgatctgttctcttccccattggttgcaataagcagactggacatcatactatgactagaaaaggcaatcctcagctttctctaatcctctgaatggaattgggttaggtttggagaggagaggtgggttcatggaaaggaattaccatcatggtgccaagactactgagtgtcaaaccacttcagaatatggatacggagggagaatattattctcctttaagaagtagtgcctgtgtctgtcttttttgcgggcttatgtggattacatctgcattccacacatcacagctacctctgtcctgatggctattcctctaggaaaagctaaggagcaatctacgaagacaatgaatacataagggagattgtttacaaaagaaaagtgttccagtgggtatagaggaaaaaatggtcagaggtgaggtagaaattttttactttccccaattaatgaacaccttttcccttcaaccttctacaggctgtttattcttgctcctgtaggaaggcgtggcaaggtatcagctttctctttgctacccactgctacttttagaccactgtgcttccatcctcttgcaaaaattcttctccctttgaagcttatgccatctggctttactgccctttaacaccttttttttttctttttctttttgtagtgcagtggcaataatcatagctcactgcagcctcaaactcctgggctcaagtgatcctccaaacccagccttcagcacctattaacctctttttgtgccaactcttactatcatcctgggaggttttacaaaaacccatgaaaaatacagttagttcctgacctccaactccaacgaatactcccactttcaattccttaatttcaccatttctagaaaaacaggtttttgttgatggcagcttcagggccatagtaaggactgggagagggtagcattcttcttctttttttttgaaacagggtctcgctatgtcactcaggttggagtgcaatggtgccatcaggactcactgcaacctcaaactcctcagtctcaggtgatcctcccacctcagcctcccaaatagctgggactacaggcaagtgcacacccacctaattaaaaaaaaattttgtagaaatggggtctctcactatgttgcccaggctgatcttgaactcctggccaaagtattgggattacaggtgtgagccaccacacccagccagggtatcattattaagtgtagtaagattgatggtgccagcactggctggtgttgacttgaagactcactgaaagactgggactggcagccatgatgcataagggcagaatagcctgggggttgtactgcccagtgatacttggggaaaggttcaagatctggatttgactcttgtgccaagcttccaagaaacctaggttcagaggtaagagcacctttcctatcagctgcctctgtggggacatctgacactttcaacatccacccccttgaaatactcttccctttgattctgtgacaattatctcccaggttttcttcttcttcactcgctgttccttttcaaagattctccaagagctctttttctacttgtgccttaaatgttggaatttccgagagcactcttcttagccctctgctcttttctggggagcttatccaaatctatggcttcaactaccaccgaaatgttgatgtttcagaatttctggcctatatatcacagggctttctaaaaagtagttttctggccaggtaccatggctcacgcctgtaatcccagcactttaggaggccgaggagagtggatcacgaggtcaagagtttgagaccagcctggccaacataacgaaaccccgtctctactaaaaatacaaaaaattagccaggcatggtggcgtgcacctgtagtcccagctactcaagaggctgaggcaggagaattgcttgaacctgggaatcagaggttgcaatgagctgagatgtgccactgcactccagcctgggtgacagagcgagactgtctcaaaaaagaaaaaaaaaaagtagctttctgtaaaataatatgtgcataataaaataatttcaagcaataaagatagatgtaaaatgaaaagtataagtcttatccctcctaggcccactcttcataattttttaatgcatgtgtaaatgtgtcatatttattctgtgcttgctttttttctccacttatatttttctcttaagttttagatctgtgtattaaacatgccactaggacatatctatctagctatctcacaggtacctaaaacttcttcaccttctttggaattctccctcctgcaacaccctaccactagtctcctttttacatcaacaccatgaaaaaactgtctttatacgttgtgccttctcaattcaatctggtttctatccaccataactacaaaacagctttctccaaatttcctaaatgacctccttgttgcagtatcttttttg

SEQ ID NO: 14735 - RNA, 2253 nt, Homo sapiens
  source 1..2253: mol_type = other RNA
gctgggattacaggcatgagccaccgtgcctggtgaattatgtctgtaagtatgaaaaaaagcagctaagatcatgaagaggatacagacacttttgtgactagaaaagccaagtatcataactttggcttccatgacattgaaatgcaactccaagtaggttgctgggatgaccctcccttaaaacataaccctgaatatctgctttggactgcctggccttggtctcttccattctacccagcaaaggccttaactttcatagccagacagtgaataagcagtggagagggaagtggagagtgaggtggggaggacttcctgatgacatcatggttttagtcagtgcatgagagcatgctgagaatgtctgatggacttaaccacacactcagctgcagagcaggcgcccaccttcacttcagtgggatggatcccagagtgagccatgtcaaacaaggtctgagttcactgaggagatagactctgatggtagaggcatgaaccaaatagccctcccaaggggagctggatggcctactgacagaattgcaggctcaagaatgagaaagacctgggcttaaaccccctggctgtgtcactctgggtaagtgactaaattctctgtgcctcagtttttccctttaagaacatgaaggcagaggacaagcctgtccaataaggctgagaaataagcaggctgatgtgtgtcaaggactggggagttcacttcaggtcctgccgtgcaccagtccctgccctagtccacagcttccgctctcaagaagctcgtggagaggagccagctgcactgacaatgttggcatgacatggggtgctaacgacattttgtccagcatgaataagggctcagggaagacttcctggaggcgaggttgatgctggaactgggaaggaccttgtttctccttcgtctccaataaacacaagtttttaaagcagaaaggataagagaaggccatcatgccacagtgctgaatcaaggcatgcctcctctggagaaacaactgtctccgtaagcattcggcattaatcccacgacatcttggtgagcgagttcagtgtggcaatacccgatcttcagctgccgcatcatcgctgtgcaggagtcagcccttcaggcctcgcaggagcggctgggtccccacctccaggcactacccgggcagagcatttcgtaggcctttttcttccgcttttgcctggactcaatcatgcgaacaatggcgtcctcttcataggtgtggccacacactttatttttcactggcttcttcatttcctcctttgtaatggggcaggtgaagttggtctgactttgggtcacaattatatcttcatccactccttctgttccgtcagcttctctgtcagcttgaagaccacattgcttctttagttctttcagctgttgtttaaactgtacaaatttttcattattttgaaagtctgcatcagaattcttgctctgtaaagccaaaaatttcttctctaccaataattttaaatctggtattttttctggacgttcttctttcacatgatttattgtagattgaacagcctttacataatggtttagttgccgatccaatgtagcaaattcaaccattgccttgtccatactatattcactactcacttcagctttccagtaaagaaacttgacaaacactactagggccaggtgatcaaggttgacattactggtcatgttgatgacttgcactagctttgatatgacgtgatgagaagggcccttgacctctgtgctcttcttcccaaaaacctgtaacgcaaatctaatcataataagacatcagacaaactccagctgagagacattctacaaaacacctaagcaggattcctcaaaactgtcaggattacaagaaaaaaaaaagcgaaaccaactaagaagcgtctacgaagatgatgattaaatgcaatgtgatatcctggattggatcccagacaacgttctttaaaaggatatcagtgaaatccaaataaagtctggagcttactatttagtttagtcaacaggaatgtaccagagttgttccttagttttgacaaatgtaccatggtagtataagatcttcttaacaactgagggaactgtgtgagggtatgggtatatgggaactccactatctacaactttggtaaatctaacatcattccaaaataaaaaacttattgaaaaaataaaaaggatagagagagatt

SEQ ID NO: 14736 - RNA, 223 nt, Homo sapiens
  source 1..223: mol_type = other RNA
gctgggattacaggcatgagccaccgtgcttggcaggtcctggggggtagacaacacacctggaggccacacgcatgctggtcagggagctcaggcagggagagagaggcactcgtgggccaacaccttttttaggtccagcactgttatccaaccatgtttcttggaaatttgctgtaagaggattgctggtgtggatttgctgaacggaaaccatttctgc

SEQ ID NO: 14737 - RNA, 557 nt, Homo sapiens
  source 1..557: mol_type = other RNA
gctgggattacaggcatgagccaccgtgcttggcccagagcattaattttcttacaaacagcagcccccagtttagctgggctggaccagctgcttggagaggggttcttgatgaaaacctgtctgcacagactcccatgaggatgtccttggatctcaatcggtattctcactttctgccagtcttggattatcctggagtctcccagaaggattttcaggtcatgtgctatattagctcatccttagggaagaacgttccaattgaagaagccatctgactctcccccaggtgtgtggtcatcttctttgctcatgcagcctgtattccacccgaatgtaagcttctgtgggcaggaggctcatctgtcttgttcgctgccgtgttgctactgccaagcagtccccagtaggctggtcatggctggtgtccattacatatttgtgcagcgtatgggtgaacatacacacatccttttgctcacagttctggaggctgggaattccaagatcaaggcattggcaaactcgtatctggcaagggcctgcttcttttt

SEQ ID NO: 14738 - RNA, 1496 nt, Homo sapiens
  source 1..1496: mol_type = other RNA
gctgggattacaggcatgagccaccgtgcttggcccagagcattaattttcttacaaacagcagcccccagtttagctgggctggaccagctgcttggagaggggttcttgatgaaaacctgtctgcacagactcccatgaggatgtccttggatctcaatcggtattctcactttctgccagtcttggattatcctggagtctcccagaaggattttcaggtcatgtgctatattagctcatccttagggaagaacgttccaattgaagaagccatctgactctcccccaggtgtgtggtcatcttctttgctcatgcagcctgtattccacccgaatgtaagcttctgtgggcaggaggctcatctgtcttgttcgctgccgtgttgctactgccaagcagtccccagtaggctggtcatggctggtgtccattacatatttgtgcagcgtatgggtgaacatacacacatccttttgctcacagttctggaggctgggaattccaagatcaaggcattggcaaactcgtatctggcaagggcctgcttcttttttcactgtatcttcacatggcagaagcagcaaatgagctctctgggttctcttttataaggttactaatcccattcatgagggctccaccctcatgacctgatcacctaccaaagatttaccttctaataccattaccttggagattaggattttgacatgaattttgggacacagactataacacagaggaattagaatagtaaatgagaagagaaagaaattgtgtggctggagagagaggcagcatagtttttctatagacttgtaggcctatatgtatcagagagctattgttgcatatcaaattcccccaaaaggtagtgacttaaaacaatagtcccttattacttcatgatttggcaggctggcagtctaggctagactcagctgggaggcgttctggatctaggctgagctcccttatgcatctggagtcagctgtgggtcagcagatgcctctgcttctggggtaggctggttgttggctggggcacctcagctctcttccacatggtctctcatcctccattaggctagcccaggcaggattgttcacatggtggcagggttctaagagaaagttgctgcatgcaaagcctcttgagactcatgcttagaactgtcacgccataatttctgccacatctattggccaaagcaagtcccatggccagcctagattcaaggggtgaggaaatagattttaactcttgatgggaggagctgccaagccacattgtaaagggggcaagatagagggaggggtgaattatcaagggcatttttgcaaccaggtaggaaatttgtgtggttggaagtcacaggagatttttaagcagggaccagcaataacagggcacatagccaaggtcatttgtgctgcactgtgatggaaactttcaagagcttgtgtcttaccttgccgttgtggttatgag

SEQ ID NO: 14739 - RNA, 2169 nt, Homo sapiens
  source 1..2169: mol_type = other RNA
gctgggattacaggcatgagccaccgtgtccagccttaggttttctagtttagaagacattttgtgtacccttctaggcctctgagcaagaagtttcttcattaggctctccgtgttactttatactttttacttacgttcacagtggtcctaaaaccaagatgcagccctaagcacctcataggagaagctgtattttttttttttttttttgagatggagtcttgctctggcacccaggctggagtgcagtggtgcgatctcagctcactgcagcgtccgaggaggagctgtagtttaaaggaagatactcaatactctaggaagcagatcatcaaaattttaaaaagcggctgggtgcggtggctcatgcctgtaatcccagcactttaaggaggctgaggcgggcggatcaccttaggtcaggagttcaagaccagcctggccaatgtggtgaaaccctgtctctactaaaaatacaaaaattagccaggcgtggtggcaggcacctgtaatcccaggtactcaggaggctgaggcaggagaatcgattgaactcgggaggcggaggttgcaatgaaccgagatcatgccattgcactccagcctgggtgacaagcaaaactctatctcaaaaaaaaaaatgtttaaaaggaagatatagaaatatggaatgcttatacagtattatttcatagtttttttaaatgtcatgtttctaatgtttagataatcttgaaagaaattctcctcacttcccctttatcctccatctttcatcaaaggaaaaaaaatcaaagcagtacaagtactcctttttttttcccccaattaatccaagttccttagaaatgttgctgtttgggtgagaattctactgattatcccgacttcacagccagcaatgacactttcagcagaaagttttcttggcataaactctttagttctcagactgcttactcataagttcttcttgagaacttgtcagcgacgcaatctgttttgtcttgaagagcacaagactcagacggttgtcactttggggagagcacatagcatctcaaacagcaggttagccgccagcagggctgtgttcccagaaagatcatacggtggtgaaacttcgacaagatcacagcccatcacgttcaggccttgacaacccctgatgatctccagagcctgactaggagtgagaccagcaatttcaggtgtccctgtccctggcgcataggcaggatccagagcgtcaatatcaaagctgatataaatgggtttgcctcccatctgctgcctgacttcccccatcagaggaaccagcgacttcatccagcagtcttcagccaggactacccggaagccctggctccggttgtatctgtagggatccaaggtcgtggaagagccccggatgccaatctgcaccacacgcttacagtccaggagaccctcatccacacaccggcggaagggcgccccgtggtagagcttctctcctagggccttgtcggtcgtgtccgtgtgcgcatccacgtgcagcagccccactgggccatgcttttttgccatcgcttgcaatatgggatatgtgattgtgtgatctccacccaaggtcagaggaatacagccagctgctacaattttctcataggcctcttgaattcgccggcagctgtcctgaaggttgtaaagattgacattcacatcgcctaggtctgcaaccatgagggactggaaggggagggcccccgtgctaggattgactgtcccaagcatcactgattcttcccggatgcggcgaggtccgaatctcgccccaggccggttggaggtcccagtatccaggggcaccccgatgaaggcagcgtccagcccctcgggggaggtctgcaccggcaggcgcatcatggagcagacgcccaccggccgggccacgaactcggggctggggggctggttccggggcgcgtcggaagcctggcggctctggcggcgccccggatgaaagagccctgcggcaggacgcgcgcccacgccgggccccgggccccgggcgcacccggacgccagcagcctcagcattgccgcgcgcggccaagacctcaccgaccaaaccgcccgcgaggccgccgcgatctggctggtcccgaacggcgaggcgagtgt

SEQ ID NO: 14740 - RNA, 7718 nt, Homo sapiens
  source 1..7718: mol_type = other RNA
gctgggattacaggcatgagccaccgtgtccagtcacagcccagcaatagtaacagccttgatcttgatagtctcttaatagcatgtctcataaatagtttattccggaagttggaaattgtaaaatttaatataaaataaaaattttaaagcttataaaatcaaaagttccatttagtttgtttttacgtacatcgtcttattccaaaagaatctgaagtggttggcagaggaatgtgtacaggagtaaccatgaacagaaataatcctataaaacaaaatactagatgaatgccgggcgcggtggctcacgcctgtaatcccagcactttgggaggctgaggcaggcagatcacctgaggtcgggagttcaggactagcctgaccaacacggagaaaccccatctctactaaaaatacaaaatttgccgggcatggtggcgcacgcctgtaatcccagctactaaggaggctaaggcaggagaatcgcttgaaaccaggaggcagaggttgcggtgagccaagattgtgccattgcactccagcctgggcaacgagcaaaattccatctcaaaaaaaaaaaaaagaaaccgtcgaatggacactaattttttttaaaagaaaagctcacgtgcacagggagtagaataaatcaaagattacacttctaccctaaagttagaaaaggcaggctttctatggttaggaggaaaaatctaccaacacctttaaataaaaaatgctttaactaaaacaagattttgctgaaatccttccaaggcagaaaaaactatgaaaaccagaaaccaaggttggggggtggggtgtcatgtttaaaatgaagcagcactaagcaacatttctccagctttcaccttgcccagagtcttgtagatgaatatcaaaaacaaattaaaatccacagagcagaatttttcttccacttgtttaaaggaaactgttataagcagaactgtccaaagggccatatcaaagaaaacgggttctaaagtgaaacctaaaacattccagtaaccaaatacctgagagaagctgtgaggaagtgcatgtggaaggctgacacatttctgagtttccatagactcttgcagcttctatgttcagtgagaaaaaaaatccccaggcaatggctcctactagaagtttaaggaattctaaattgctcttcagtaattctcagccttgagtgcccattaaaattacctgaaaaggtctttttttttttttaataccaatgctggaccccatccaagatcaattaaattgaaatcccttggtacaaggcccaggcattagtattttttaaagctcccagaggttctaatgtgctgccagtgctgagatccacttagcaacctacaaaaatgctgaaaaagtcaaggatgactgtaattactgtgtgtttgaaattcagttgtgacagaaaatgatttttctgggaggtaaatttttttcactagtgctaggctgcctttcttttcatgtgcttatgccctctactatacagtactgaaatccctcaagataataagaacaacaccatttattgagcacttacatggtatcaagcactgtgctgggcactacccacccccatctccacacacaatcactgatgtccattattctgcaaaaataagtattaaacccattaatctgaaacagctgataagaaggcgtttcgttggcccctatcacaaagcaagaagttacagaattgggattagaacctacatgtatctgattacgaagcaatgctttttattttcctttaattttatgtatttatgttgcaaaaggtaatagagttacatgtttcacaggtttataaaggtttatatggtatacataaggcatataaaaattaatctcactgatgatttttttctatcacaactgaagttcaaatacatagtaaccacgattatccttgattcctatcacttagcctctcctatcacccagccaacaattctactccctggagacaaacttagcagtttcttgtttatataatatatttacaagcaaatacatgtaagaatatgtgacataccatacatttgaattcctccccaccccattttaaataatttcaacaactgcatagttcacacactattttgcacatggcttttttcactttaacagtgcatctcaaagattattccatatcaataaactttttaaatttttttttgtaatacatagtattccattgtactgatgtaccatcactttaaaaccagtctattattgatagacatttgattttttctatttgctgttataaaaatgttagaatgaataaccttgagctacataattttataaatacatacagataattacacctatagattaaatgcctagatgtcaaaagccatgccctttcactactctatgctatctcaggattctaagaaacaactcacaatcagacttataatgacttatacttattttatttaaaaactttaaatacccaaattatgctttttgttttattttaaaatattggaatttttttttcagaatatgctcaaaaaccaaacagtctgagagagggttttaagccaaggtaaaatgactttaaaaccagtggcataaacactgtgctggctgtctcttcccgttcagaaggtatctgcccccgaagactccatgtcctcctgcattgtgctgagactcagagactgagagcagtcctcgaggttcactgacggcagcatcactgacatcttggcagggggcatctgtgaagcggagagtggcactgctttcccacctgaaaatacacatgtgaggtacggattaagctcaatttgtgtccgatccatatcacctggtgaaacttgttgctgtgaaggtgcaatatcagatttatttctaacacgtaggtaactttgtgatggtttgtgttcaacttgcttaacatcctgattttgctttagttggtactgggaaaaatcttcagcggctactggtaaattaacatcattttcttgtgctgtcagaagtgttgtgggaagaaccagcttagaatttggctccaactccaattctcccaaactcattggaccatgactagcacatgaatcttcataaatactacctgaaactgtgtcaaattgccgagataatggtttaggatcacattgttgatccaaagactgtgtattagtgacaggtggctgcatatagagagaatgtcccattaagatgttctctgctgccgctgttagctggggtctttgtccttcactaagttcacccacactgttttccaagtccatttcaacggcatcatgcagagtgctggataagctatcattaaggtttgtcaggtacagtcctatatcttctaaaatcttgggggccaatttttgaccacagctaaataaaatctctccttcagagatgggtttatctaaagtttcagtttcagtgacagtaacactcaatgtgctctccagtgttgatgaatcagaacctggcatctgtgagggggaaggggccttggtgccggcaggaaatggcataaagggaactggctctggaggtggaggctgagcagggaaatccatactctctggttcttcatccttagccacagacattacaatagctcttggatgaagttcttcttgaggtgagttagggttctcttcttccagtggcaggtctccatcaccccatggcttgggaagctctgggcttgataccttcaatttatcaatggaaatatctgacaaagttggggtaaaaactgccgccgctggaggaggtgtagtagtaggggtaactgttggagtattaacaagcatgatggcaggcatatcatctcctttttcagcacatatttctttcacaggaaaagccatatcatgatccgaatcacagggagaagaatctggagtctttaccaaaacacactccttagcaggtgatgaaggtgagcaaggaggcgtaggctgtggggtaggcagtggggtgcacactcttgccggcaaatatgtttcatttgttgaagcatccccagaaacacctgtagcaacaggaccttgcttctttgcttctctgtcacccagcatgacagcaatggtctcagcaagagcttcgttaacaaaatgtttaatcacatttgagttcacaggaacaccagcatcaacaaaaagctggagggcgccactgcttgttccttccacaatgtcagaagtcagtggttcacttgtctcactgactgaaacactgatactaggtgcaatctgttgctggactggaaagagcccagagataattcttgacattatttcttgctctacccattgaattaagctattttccagtgtttcttttctctcaattactttatccagaatatcagcagtgggctgaaaagtagaagcaactggcggaaatggaggaccattatattttgtagaatcagctttaacacttctgttaaactccagaattggttcagagtctggaatttcatcacatttttcttcttcctgtatgacatcgattatttcatcaaagttagttcctggaaacttcacctcttcttcatctaccttcataatttctggagtctttatccaagtttgcacaggaggaagagatgcttctttggggctagacagaggtgaaaggacatcagcactactatttgaaatgctgtcaatatctacactgggtaatacctgcacagtaagctgaggaggatcctttttttctgacttcatttctacaatggctatgttaggtttctttactccagtttctacttttcgagatgatggaggaatagaagtagtcacagttacagggtgtggcttgctgacaatcactccagcaggtggcatggtatcactattactttgggtttgtcctaaaagaattgccataggaatcagatgaccttccaatgtacctgaaaaagtaggcatttctctacttgggctgaacaaatattgctgatcgccatgaggtaacacaggaacagaatgtttcattttagaatccatcttcttaggttttgttgcatagaagtcagtctgtgttcttattgactttaccttagtgcctttaactcgttctattacttttggtctctgtggtctggacttaggagatggagaattaaatctgagatatggtccttttttaagagtgcttcgatggccctgataaactggctttccatagacttgtaacatataatcttcatcttgtattactgtggttgctttcaaaagcccttcctttctctctttctgtaaacttgaagcaggcatgcccctcataggtagatttctaaaatgctcttctatttgcttttgagaatgttttcttggaattacagatttgttgacagttttatcttgtgtgttggttctaatatctttagtcatattctgacctttcttggttctctgattcttctgatcaaatcttttttgttcataatctgttcttgacagttcatcctgaatttctgcagaaatagttttaatccattcatccactgtctttctgatcctaattttctctgacatctctctgttggtagataaagcattgataagcgaatacatggcagctccatcttttgcacgaataatagcttccaggttttcttcaagtacttttttattgttttgtactcctctcaaaatcttctcagcatctttcaatacagatcttgttgtattggttgtttgaagcttaacagaattctgtggaagatctggaagcttcaacatactcagagattcttttggctggaccatgctatttgtttctttctctttttggccaaggtcatgaagaacatcatcagacttctgcatagtcactttagttgtttctagctcttcacaggaaggaaatctgtttgttttctcaggagtccatcctatttttgacctagttagtgaggtggtgtttgatgattcactttttcttgtcaaagaatcattattattcaaaatttgttccaatagtcttacatttcctctgtgacacgacacttccatattttctttttcttccaaaagattttccctctttgatagttcatcatcccttgaaacaggtacaggagcaaatctgcgaggtgctggtgtctccaaaggagatttctgtttatcaaaactcgtatcttcaacttcttttaaaggtgcttgtttggaagcaaatgtgttatataaagatggattacagctaccaagattagggtgttctggttttacggaatacttttccactgctctggaggagggcatactaacaggctgaaaactactagtcttgagtgcagcactaataaaatgagtctgaatatctatttgttgttgttgtaacttttcaagatgccttatgtgctgctccataaacacattcatttgcttttcgtgatcatgacaatgtaatttctcttgtttcctctgaatgcttgtttgctgctctgtaacacgttgcaggtgtttatcagtctcctgtaatttactaagtaattctgtaacagaattgacttttgcttccaaatcactctgcacctttatcaacggagctgcggttgcaatggcagcagcagttgctgcagccacggttgtagctgaatcaattccactgggtgaaattctagtctcctgagtaacagcatccttctctatgcctgcatcttctaacagatgtacctttacttccttaaaaacaggcatgctttgagctttttgctttaaaactgttcttagagcatctttctgtcccattgtatactgagaaatgaagatgtcatttgctttttgcttgttgttctcttctattttatccaaaggcaacacttgcactgcaacgtctttagaaaaatcactttctgacaccatgggattttctaatagaggctggtaacaatttctagcagaagttaagtctgatgaaccacgtgatgttccattcaaactagtccccgttccaacaggaagacgtttatttgcagacaatgccggaggaacacagggcaactcatctttcagcaaaaccaaatgatctccatgattttgagaaactacctcacgaagtctcttcactggcatcttaatcttttttttcttctccaagctgacctcagagcctttcatattgttggtcacaaaacaagtcccacacttaaggacggaaaaactttctctgtttccttaagacttcagaacaaaattttcacctctttgcaataactgtttttaaaatgtcgaacatccacaaagctgaaaatctaaattctgatattgaatccaggattagagctgactataaagtcatatttacccattaatcccactcagtctattaatacaccacgccaaaatgtgaaagtggggatgacaagagaatggccacaggagcaacaataaccataacagtgcactccccaaccccagagctggtagggcaaaaccaaacacatgtagtggcgggcttaaaatttgttgagaagaggcagtcaagcaaataaaagcgaaatgctatttttaaaataatgacccacataagaagcgtaatagctttcttcagccacagagtcttacacacccctccagatgcaatcgtcggaaacataaattcacccctacgtatctccagaacgcccgagacccgcaccgtcgtgggtgtaatctgacaacagc

SEQ ID NO: 14741 - RNA, 7622 nt, Homo sapiens
  source 1..7622: mol_type = other RNA
gctgggattacaggcatgagccaccgtgtccagtcacagcccagcaatagtaacagccttgatcttgatagtctcttaatagcatgtctcataaatagtttattccggaagttggaaattgtaaaatttaatataaaataaaaattttaaagcttataaaatcaaaagttccatttagtttgtttttacgtacatcgtcttattccaaaagaatctgaagtggttggcagaggaatgtgtacaggagtaaccatgaacagaaataatcctataaaacaaaatactagatgaatgccgggcgcggtggctcacgcctgtaatcccagcactttgggaggctgaggcaggcagatcacctgaggtcgggagttcaggactagcctgaccaacacggagaaaccccatctctactaaaaatacaaaatttgccgggcatggtggcgcacgcctgtaatcccagctactaaggaggctaaggcaggagaatcgcttgaaaccaggaggcagaggttgcggtgagccaagattgtgccattgcactccagcctgggcaacgagcaaaattccatctcaaaaaaaaaaaaaagaaaccgtcgaatggacactaattttttttaaaagaaaagctcacgtgcacagggagtagaataaatcaaagattacacttctaccctaaagttagaaaaggcaggctttctatggttaggaggaaaaatctaccaacacctttaaataaaaaatgctttaactaaaacaagattttgctgaaatccttccaaggcagaaaaaactatgaaaaccagaaaccaaggttggggggtggggtgtcatgtttaaaatgaagcagcactaagcaacatttctccagctttcaccttgcccagagtcttgtagatgaatatcaaaaacaaattaaaatccacagagcagaatttttcttccacttgtttaaaggaaactgttataagcagaactgtccaaagggccatatcaaagaaaacgggttctaaagtgaaacctaaaacattccagtaaccaaatacctgagagaagctgtgaggaagtgcatgtggaaggctgacacatttctgagtttccatagactcttgcagcttctatgttcagtgagaaaaaaaatccccaggcaatggctcctactagaagtttaaggaattctaaattgctcttcagtaattctcagccttgagtgcccattaaaattacctgaaaaggtctttttttttttttaataccaatgctggaccccatccaagatcaattaaattgaaatcccttggtacaaggcccaggcattagtattttttaaagctcccagaggttctaatgtgctgccagtgctgagatccacttagcaacctacaaaaatgctgaaaaagtcaaggatgactgtaattactgtgtgtttgaaattcagttgtgacagaaaatgatttttctgggaggtaaatttttttcactagtgctaggctgcctttcttttcatgtgcttatgccctctactatacagtactgaaatccctcaagataataagaacaacaccatttattgagcacttacatggtatcaagcactgtgctgggcactacccacccccatctccacacacaatcactgatgtccattattctgcaaaaataagtattaaacccattaatctgaaacagctgataagaaggcgtttcgttggcccctatcacaaagcaagaagttacagaattgggattagaacctacatgtatctgattacgaagcaatgctttttattttcctttaattttatgtatttatgttgcaaaaggtaatagagttacatgtttcacaggtttataaaggtttatatggtatacataaggcatataaaaattaatctcactgatgatttttttctatcacaactgaagttcaaatacatagtaaccacgattatccttgattcctatcacttagcctctcctatcacccagccaacaattctactccctggagacaaacttagcagtttcttgtttatataatatatttacaagcaaatacatgtaagaatatgtgacataccatacatttgaattcctccccaccccattttaaataatttcaacaactgcatagttcacacactattttgcacatggcttttttcactttaacagtgcatctcaaagattattccatatcaataaactttttaaatttttttttgtaatacatagtattccattgtactgatgtaccatcactttaaaaccagtctattattgatagacatttgattttttctatttgctgttataaaaatgttagaatgaataaccttgagctacataattttataaatacatacagataattacacctatagattaaatgcctagatgtcaaaagccatgccctttcactactctatgctatctcaggattctaagaaacaactcacaatcagacttataatgacttatacttattttatttaaaaactttaaatacccaaattatgctttttgttttattttaaaatattggaatttttttttcagaatatgctcaaaaaccaaacagtctgagagagggttttaagccaaggtaaaatgactttaaaaccagtggcataaacactgtgctggctgtctcttcccgttcagaaggtatctgcccccgaagactccatgtcctcctgcattgtgctgagactcagagactgagagcagtcctcgaggttcactgacggcagcatcactgacatcttggcagggggcatctgtgaagcggagagtggcactgctttcccacctgaaaatacacatgtgaggtacggattaagctcaatttgtgtccgatccatatcacctggtgaaacttgttgctgtgaaggtgcaatatcagatttatttctaacacgtaggtaactttgtgatggtttgtgttcaacttgcttaacatcctgattttgctttagttggtactgggaaaaatcttcagcggctactggtaaattaacatcattttcttgtgctgtcagaagtgttgtgggaagaaccagcttagaatttggctccaactccaattctcccaaactcattggaccatgactagcacatgaatcttcataaatactacctgaaactgtgtcaaattgccgagataatggtttaggatcacattgttgatccaaagactgtgtattagtgacaggtggctgcatatagagagaatgtcccattaagatgttctctgctgccgctgttagctggggtctttgtccttcactaagttcacccacactgttttccaagtcctctgaatgatagactgcttgctgggaaactgctgactcctggttttgtttagcaaaagaaagaattgcatctgcatgaaattttttatgggacatcctaatcacttgcccttcactaggaggatcatcctccatttcaacggcatcatgcagagtgctggataagctatcattaaggtttgtcaggtacagtcctatatcttctaaaatcttgggggccaatttttgaccacagctaaataaaatctctccttcagagatgggtttatctaaagtttcagtttcagtgacagtaacactcaatgtgctctccagtgttgatgaatcagaacctggcatctgtgagggggaaggggccttggtgccggcaggaaatggcataaagggaactggctctggaggtggaggctgagcagggaaatccatactctctggttcttcatccttagccacagacattacaatagctcttggatgaagttcttcttgaggtgagttagggttctcttcttccagtggcaggtctccatcaccccatggcttgggaagctctgggcttgataccttcaatttatcaatggaaatatctgacaaagttggggtaaaaactgccgccgctggaggaggtgtagtagtaggggtaactgttggagtattaacaagcatgatggcaggcatatcatctcctttttcagcacatatttctttcacaggaaaagccatatcatgatccgaatcacagggagaagaatctggagtctttaccaaaacacactccttagcaggtgatgaaggtgagcaaggaggcgtaggctgtggggtaggcagtggggtgcacactcttgccggcaaatatgtttcatttgttgaagcatccccagaaacacctgtagcaacaggaccttgcttctttgcttctctgtcacccagcatgacagcaatggtctcagcaagagcttcgttaacaaaatgtttaatcacatttgagttcacaggaacaccagcatcaacaaaaagctggagggcgccactgcttgttccttccacaatgtcagaagtcagtggttcacttgtctcactgactgaaacactgatactaggtgcaatctgttgctggactggaaagagcccagagataattcttgacattatttcttgctctacccattgaattaagctattttccagtgtttcttttctctcaattactttatccagaatatcagcagtgggctgaaaagtagaagcaactggcggaaatggaggaccattatattttgtagaatcagctttaacacttctgttaaactccagaattggttcagagtctggaatttcatcacatttttcttcttcctgtatgacatcgattatttcatcaaagttagttcctggaaacttcacctcttcttcatctaccttcataatttctggagtctttatccaagtttgcacaggaggaagagatgcttctttggggctagacagaggtgaaaggacatcagcactactatttgaaatgctgtcaatatctacactgggtaatacctgcacagtaagctgaggaggatcctttttttctgacttcatttctacaatggctatgttaggtttctttactccagtttctacttttcgagatgatggaggaatagaagtagtcacagttacagggtgtggcttgctgacaatcactccagcaggtggcatggtatcactattactttgggtttgtcctaaaagaattgccataggaatcagatgaccttccaatgtacctgaaaaagtaggcatttctctacttgggctgaacaaatattgctgatcgccatgaggtaacacaggaacagaatgtttcattttagaatccatcttcttaggttttgttgcatagaagtcagtctgtgttcttattgactttaccttagtgcctttaactcgttctattacttttggtctctgtggtctggacttaggagatggagaattaaatctgagatatggtccttttttaagagtgcttcgatggccctgataaactggctttccatagacttgtaacatataatcttcatcttgtattactgtggttgctttcaaaagcccctgaatttctgcagaaatagttttaatccattcatccactgtctttctgatcctaattttctctgacatctctctgttggtagataaagcattgataagcgaatacatggcagctccatcttttgcacgaataatagcttccaggttttcttcaagtacttttttattgttttgtactcctctcaaaatcttctcagcatctttcaatacagatcttgttgtattggttgtttgaagcttaacagaattctgtggaagatctggaagcttcaacatactcagagattcttttggctggaccatgctatttgtttctttctctttttggccaaggtcatgaagaacatcatcagacttctgcatagtcactttagttgtttctagctcttcacaggaaggaaatctgtttgttttctcaggagtccatcctatttttgacctagttagtgaggtggtgtttgatgattcactttttcttgtcaaagaatcattattattcaaaatttgttccaatagtcttacatttcctctgtgacacgacacttccatattttctttttcttccaaaagattttccctctttgatagttcatcatcccttgaaacaggtacaggagcaaatctgcgaggtgctggtgtctccaaaggagatttctgtttatcaaaactcgtatcttcaacttcttttaaaggtgcttgtttggaagcaaatgtgttatataaagatggattacagctaccaagattagggtgttctggttttacggaatacttttccactgctctggaggagggcatactaacaggctgaaaactactagtcttgagtgcagcactaataaaatgagtctgaatatctatttgttgttgttgtaacttttcaagatgccttatgtgctgctccataaacacattcatttgcttttcgtgatcatgacaatgtaatttctcttgtttcctctgaatgcttgtttgctgctctgtaacacgttgcaggtgtttatcagtctcctgtaatttactaagtaattctgtaacagaattgacttttgcttccaaatcactctgcacctttatcaacggagctgcggttgcaatggcagcagcagttgctgcagccacggttgtagctgaatcaattccactgggtgaaattctagtctcctgagtaacagcatccttctctatgcctgcatcttctaacagatgtacctttacttccttaaaaacaggcatgctttgagctttttgctttaaaactgttcttagagcatctttctgtcccattgtatactgagaaatgaagatgtcatttgctttttgcttgttgttctcttctattttatccaaaggcaacacttgcactgcaacgtctttagaaaaatcactttctgacaccatgggattttctaatagaggctggtaacaatttctagcagaagttaagtctgatgaaccacgtgatgttccattcaaactagtccccgttccaacaggaagacgtttatttgcagacaatgccggaggaacacagggcaactcatctttcagcaaaaccaaatgatctccatgattttgagaaactacctcacgaagtctcttcactggcatcttaatcttttttttcttctccaagctgacctcagagcctttcatattgttggtcacaaaacaagtcccacacttaaggacggaaaaactttctctgtttccttaagacttcagaacaaaattttcacctctttgcaataactgtttttaaaatgtcgaacatccacaaagctgaaaatctaaattctgatattgaatccaggattagagctgactataaagtcatatttacccattaatcccactcagtctattaatacaccacgccaaaatgtgaaagtggggatgacaagagaatggccacaggagcaacaataaccataacagtgcactccccaaccccagagctggtagggcaaaaccaaacacatgtagtggcgggcttaaaatttgttgagaagaggcagtcaagcaaataaaagcgaaatgctatttttaaaataatgacccacataagaagcgtaatagctttcttcagccacagagtcttacacacccctccagatgcaatcgtcggaaacataaattcacccctacgtatctccagaacgcccgagacccgcaccgtcgtgggtgtaatctgacaacagc

SEQ ID NO: 14742 - RNA, 7466 nt, Homo sapiens
  source 1..7466: mol_type = other RNA
gctgggattacaggcatgagccaccgtgtccagtcacagcccagcaatagtaacagccttgatcttgatagtctcttaatagcatgtctcataaatagtttattccggaagttggaaattgtaaaatttaatataaaataaaaattttaaagcttataaaatcaaaagttccatttagtttgtttttacgtacatcgtcttattccaaaagaatctgaagtggttggcagaggaatgtgtacaggagtaaccatgaacagaaataatcctataaaacaaaatactagatgaatgccgggcgcggtggctcacgcctgtaatcccagcactttgggaggctgaggcaggcagatcacctgaggtcgggagttcaggactagcctgaccaacacggagaaaccccatctctactaaaaatacaaaatttgccgggcatggtggcgcacgcctgtaatcccagctactaaggaggctaaggcaggagaatcgcttgaaaccaggaggcagaggttgcggtgagccaagattgtgccattgcactccagcctgggcaacgagcaaaattccatctcaaaaaaaaaaaaaagaaaccgtcgaatggacactaattttttttaaaagaaaagctcacgtgcacagggagtagaataaatcaaagattacacttctaccctaaagttagaaaaggcaggctttctatggttaggaggaaaaatctaccaacacctttaaataaaaaatgctttaactaaaacaagattttgctgaaatccttccaaggcagaaaaaactatgaaaaccagaaaccaaggttggggggtggggtgtcatgtttaaaatgaagcagcactaagcaacatttctccagctttcaccttgcccagagtcttgtagatgaatatcaaaaacaaattaaaatccacagagcagaatttttcttccacttgtttaaaggaaactgttataagcagaactgtccaaagggccatatcaaagaaaacgggttctaaagtgaaacctaaaacattccagtaaccaaatacctgagagaagctgtgaggaagtgcatgtggaaggctgacacatttctgagtttccatagactcttgcagcttctatgttcagtgagaaaaaaaatccccaggcaatggctcctactagaagtttaaggaattctaaattgctcttcagtaattctcagccttgagtgcccattaaaattacctgaaaaggtctttttttttttttaataccaatgctggaccccatccaagatcaattaaattgaaatcccttggtacaaggcccaggcattagtattttttaaagctcccagaggttctaatgtgctgccagtgctgagatccacttagcaacctacaaaaatgctgaaaaagtcaaggatgactgtaattactgtgtgtttgaaattcagttgtgacagaaaatgatttttctgggaggtaaatttttttcactagtgctaggctgcctttcttttcatgtgcttatgccctctactatacagtactgaaatccctcaagataataagaacaacaccatttattgagcacttacatggtatcaagcactgtgctgggcactacccacccccatctccacacacaatcactgatgtccattattctgcaaaaataagtattaaacccattaatctgaaacagctgataagaaggcgtttcgttggcccctatcacaaagcaagaagttacagaattgggattagaacctacatgtatctgattacgaagcaatgctttttattttcctttaattttatgtatttatgttgcaaaaggtaatagagttacatgtttcacaggtttataaaggtttatatggtatacataaggcatataaaaattaatctcactgatgatttttttctatcacaactgaagttcaaatacatagtaaccacgattatccttgattcctatcacttagcctctcctatcacccagccaacaattctactccctggagacaaacttagcagtttcttgtttatataatatatttacaagcaaatacatgtaagaatatgtgacataccatacatttgaattcctccccaccccattttaaataatttcaacaactgcatagttcacacactattttgcacatggcttttttcactttaacagtgcatctcaaagattattccatatcaataaactttttaaatttttttttgtaatacatagtattccattgtactgatgtaccatcactttaaaaccagtctattattgatagacatttgattttttctatttgctgttataaaaatgttagaatgaataaccttgagctacataattttataaatacatacagataattacacctatagattaaatgcctagatgtcaaaagccatgccctttcactactctatgctatctcaggattctaagaaacaactcacaatcagacttataatgacttatacttattttatttaaaaactttaaatacccaaattatgctttttgttttattttaaaatattggaatttttttttcagaatatgctcaaaaaccaaacagtctgagagagggttttaagccaaggtaaaatgactttaaaaccagtggcataaacactgtgctggctgtctcttcccgttcagaaggtatctgcccccgaagactccatgtcctcctgcattgtgctgagactcagagactgagagcagtcctcgaggttcactgacggcagcatcactgacatcttggcagggggcatctgtgaagcggagagtggcactgctttcccacctgaaaatacacatgtgaggtacggattaagctcaatttgtgtccgatccatatcacctggtgaaacttgttgctgtgaaggtgcaatatcagatttatttctaacacgtaggtaactttgtgatggtttgtgttcaacttgcttaacatcctgattttgctttagttggtactgggaaaaatcttcagcggctactggtaaattaacatcattttcttgtgctgtcagaagtgttgtgggaagaaccagcttagaatttggctccaactccaattctcccaaactcattggaccatgactagcacatgaatcttcataaatactacctgaaactgtgtcaaattgccgagataatggtttaggatcacattgttgatccaaagactgtgtattagtgacaggtggctgcatatagagagaatgtcccattaagatgttctctgctgccgctgttagctggggtctttgtccttcactaagttcacccacactgttttccaagtcctctgaatgatagactgcttgctgggaaactgctgactcctggttttgtttagcaaaagaaagaattgcatctgcatgaaattttttatgggacatcctaatcacttgcccttcactaggaggatcatcctccatttcaacggcatcatgcagagtgctggataagctatcattaaggtttgtcaggtacagtcctatatcttctaaaatcttgggggccaatttttgaccacagctaaataaaatctctccttcagagatgggtttatctaaagtttcagtttcagtgacagtaacactcaatgtgctctccagtgttgatgaatcagaacctggcatctgtgagggggaaggggccttggtgccggcaggaaatggcataaagggaactggctctggaggtggaggctgagcagggaaatccatactctctggttcttcatccttagccacagacattacaatagctcttggatgaagttcttcttgaggtgagttagggttctcttcttccagtggcaggtctccatcaccccatggcttgggaagctctgggcttgataccttcaatttatcaatggaaatatctgacaaagttggggtaaaaactgccgccgctggaggaggtgtagtagtaggggtaactgttggagtattaacaagcatgatggcaggcatatcatctcctttttcagcacatatttctttcacaggaaaagccatatcatgatccgaatcacagggagaagaatctggagtctttaccaaaacacactccttagcaggtgatgaaggtgagcaaggaggcgtaggctgtggggtaggcagtggggtgcacactcttgccggcaaatatgtttcatttgttgaagcatccccagaaacacctgtagcaacaggaccttgcttctttgcttctctgtcacccagcatgacagcaatggtctcagcaagagcttcgttaacaaaatgtttaatcacatttgagttcacaggaacaccagcatcaacaaaaagctggagggcgccactgcttgttccttccacaatgtcagaagtcagtggttcacttgtctcactgactgaaacactgatactaggtgcaatctgttgctggactggaaagagcccagagataattcttgacattatttcttgctctacccattgaattaagctattttccagtgtttcttttctctcaattactttatccagaatatcagcagtgggctgaaaagtagaagcaactggcggaaatggaggaccattatattttgtagaatcagctttaacacttctgttaaactccagaattggttcagagtctggaatttcatcacatttttcttcttcctgtatgacatcgattatttcatcaaagttagttcctggaaacttcacctcttcttcatctaccttcataatttctggagtctttatccaagtttgcacaggaggaagagatgcttctttggggctagacagaggtgaaaggacatcagcactactatttgaaatgctgtcaatatctacactgggtaatacctgcacagtaagctgaggaggatcctttttttctgacttcatttctacaatggctatgttaggtttctttactccagtttctacttttcgagatgatggaggaatagaagtagtcacagttacagggtgtggcttgctgacaatcactccagcaggtggcatggtatcactattactttgggtttgtcctaaaagaattgccataggaatcagatgaccttccaatgtacctgaaaaagtaggcatttctctacttgggctgaacaaatattgctgatcgccatgaggtaacacaggaacagaatgtttcattttagaatccatcttcttaggttttgttgcatagaagtcagtctgtgttcttattgactttaccttagtgcctttaactcgttctattacttttggtctctgtggtctggacttaggagatggagaattaaatctgagatatggtccttttttaagagtgcttcgatggccctgataaactggctttccatagacttgtaacatataatcttcatcttgtattactgtggttgctttcaaaagcccttcctttctctctttctgtaaacttgaagcaggcatgcccctcataggtagatttctaaaatgctcttctatttgcttttgagaatgttttcttggaattacagatttgttgacagttttatcttgtgtgttggttctaatatctttagtcatattctgacctttcttggttctctgattcttctgatcaaatcttttttgttcataatctgttcttgacagttcatcctgaatttctgcagaaatagttttaatccattcatccactgtctttctgatcctaattttctctgacatctctctgttggtagataaagcattgataagcgaatacatggcagctccatcttttgcacgaataatagcttccaggttttcttcaagtacttttttattgttttgtactcctctcaaaatcttctcagcatctttcaatacagatcttgttgtattggttgtttgaagcttaacagaattctgtggaagatctggaagcttcaacatactcagagattcttttggctggaccatgctatttgtttctttctctttttggccaaggtcatgaagaacatcatcagacttctgcatagtcactttagttgtttctagctcttcacaggaaggaaatctgtttgttttctcaggagtccatcctatttttgacctagttagtgaggtggtgtttgatgattcactttttcttgtcaaagaatcattattattcaaaatttgttccaatagtcttacatttcctctgtgacacgacacttccatattttctttttcttccaaaagattttccctctttgatagttcatcatcccttgaaacaggtacaggagcaaatctgcgaggtgctggtgtctccaaaggagatttctgtttatcaaaactcgtatcttcaacttcttttaaaggtgcttgtttggaagcaaatgtgttatataaagatggattacagctaccaagattagggtgttctggttttacggaatacttttccactgctctggaggagggcatactaacaggctgaaaactactagtcttgagtgcagcactaataaaatgagtctgaatatctatttgttgttgttgtaacttttcaagatgccttatgtgctgctccataaacacattcatttgcttttcgtgatcatgacaatgtaatttctcttgtttcctctgaatgcttgtttgctgctctgtaacacgttgcaggtgtttatcagtctcctgtaatttactaagtaattctgtaacagaattgacttttgcttccaaatcactctgcacctttatcaacggagctgcggttgcaatggcagcagcagttgctgcagccacggttgtagctgaatcaattccactgggtgaaattctagtctcctgagtaacagcatccttctctatgcctgcatcttctaacagatgtacctttacttccttaaaaacaggcatgctttgagctctgtagtcccagctactcgggaggctgaggtgggaggatctcatgagcctgaggaggtagagactgcagtgagttgtgatcaccccactgtgatcactccagcctgtgagacaaagtgagacattttgctttaaaactgttcttagagcatctttctgtcccattgtatactgagaaatgaagatgtcatttgctttttgcttgttgttctcttctattttatccaaaggcaacacttgcactgcaacgtctttagaaaaatcactttctgacaccatgggattttctaatagaggctggtaacaatttctagcagaagttaagtctgatgaacccaaaacatccaaccagaaagctaagcgctctctggtgctcttccattcctctccgggtggaaacaaactccggacataacaggggtttatttatttatttattttaaggtagcacattgccgcacaagaccgctctacagtctcatccaagacttgaagagctcccgacttgtaatactacttgtgtttaccagggactgttgacactgcttcgcttccgaagaccgttagggacgt

SEQ ID NO: 14743 - RNA, 7535 nt, Homo sapiens
  source 1..7535: mol_type = other RNA
gctgggattacaggcatgagccaccgtgtccagtcacagcccagcaatagtaacagccttgatcttgatagtctcttaatagcatgtctcataaatagtttattccggaagttggaaattgtaaaatttaatataaaataaaaattttaaagcttataaaatcaaaagttccatttagtttgtttttacgtacatcgtcttattccaaaagaatctgaagtggttggcagaggaatgtgtacaggagtaaccatgaacagaaataatcctataaaacaaaatactagatgaatgccgggcgcggtggctcacgcctgtaatcccagcactttgggaggctgaggcaggcagatcacctgaggtcgggagttcaggactagcctgaccaacacggagaaaccccatctctactaaaaatacaaaatttgccgggcatggtggcgcacgcctgtaatcccagctactaaggaggctaaggcaggagaatcgcttgaaaccaggaggcagaggttgcggtgagccaagattgtgccattgcactccagcctgggcaacgagcaaaattccatctcaaaaaaaaaaaaaagaaaccgtcgaatggacactaattttttttaaaagaaaagctcacgtgcacagggagtagaataaatcaaagattacacttctaccctaaagttagaaaaggcaggctttctatggttaggaggaaaaatctaccaacacctttaaataaaaaatgctttaactaaaacaagattttgctgaaatccttccaaggcagaaaaaactatgaaaaccagaaaccaaggttggggggtggggtgtcatgtttaaaatgaagcagcactaagcaacatttctccagctttcaccttgcccagagtcttgtagatgaatatcaaaaacaaattaaaatccacagagcagaatttttcttccacttgtttaaaggaaactgttataagcagaactgtccaaagggccatatcaaagaaaacgggttctaaagtgaaacctaaaacattccagtaaccaaatacctgagagaagctgtgaggaagtgcatgtggaaggctgacacatttctgagtttccatagactcttgcagcttctatgttcagtgagaaaaaaaatccccaggcaatggctcctactagaagtttaaggaattctaaattgctcttcagtaattctcagccttgagtgcccattaaaattacctgaaaaggtctttttttttttttaataccaatgctggaccccatccaagatcaattaaattgaaatcccttggtacaaggcccaggcattagtattttttaaagctcccagaggttctaatgtgctgccagtgctgagatccacttagcaacctacaaaaatgctgaaaaagtcaaggatgactgtaattactgtgtgtttgaaattcagttgtgacagaaaatgatttttctgggaggtaaatttttttcactagtgctaggctgcctttcttttcatgtgcttatgccctctactatacagtactgaaatccctcaagataataagaacaacaccatttattgagcacttacatggtatcaagcactgtgctgggcactacccacccccatctccacacacaatcactgatgtccattattctgcaaaaataagtattaaacccattaatctgaaacagctgataagaaggcgtttcgttggcccctatcacaaagcaagaagttacagaattgggattagaacctacatgtatctgattacgaagcaatgctttttattttcctttaattttatgtatttatgttgcaaaaggtaatagagttacatgtttcacaggtttataaaggtttatatggtatacataaggcatataaaaattaatctcactgatgatttttttctatcacaactgaagttcaaatacatagtaaccacgattatccttgattcctatcacttagcctctcctatcacccagccaacaattctactccctggagacaaacttagcagtttcttgtttatataatatatttacaagcaaatacatgtaagaatatgtgacataccatacatttgaattcctccccaccccattttaaataatttcaacaactgcatagttcacacactattttgcacatggcttttttcactttaacagtgcatctcaaagattattccatatcaataaactttttaaatttttttttgtaatacatagtattccattgtactgatgtaccatcactttaaaaccagtctattattgatagacatttgattttttctatttgctgttataaaaatgttagaatgaataaccttgagctacataattttataaatacatacagataattacacctatagattaaatgcctagatgtcaaaagccatgccctttcactactctatgctatctcaggattctaagaaacaactcacaatcagacttataatgacttatacttattttatttaaaaactttaaatacccaaattatgctttttgttttattttaaaatattggaatttttttttcagaatatgctcaaaaaccaaacagtctgagagagggttttaagccaaggtaaaatgactttaaaaccagtggcataaacactgtgctggctgtctcttcccgttcagaaggtatctgcccccgaagactccatgtcctcctgcattgtgctgagactcagagactgagagcagtcctcgaggttcactgacggcagcatcactgacatcttggcagggggcatctgtgaagcggagagtggcactgctttcccacctgaaaatacacatgtgaggtacggattaagctcaatttgtgtccgatccatatcacctggtgaaacttgttgctgtgaaggtgcaatatcagatttatttctaacacgtaggtaactttgtgatggtttgtgttcaacttgcttaacatcctgattttgctttagttggtactgggaaaaatcttcagcggctactggtaaattaacatcattttcttgtgctgtcagaagtgttgtgggaagaaccagcttagaatttggctccaactccaattctcccaaactcattggaccatgactagcacatgaatcttcataaatactacctgaaactgtgtcaaattgccgagataatggtttaggatcacattgttgatccaaagactgtgtattagtgacaggtggctgcatatagagagaatgtcccattaagatgttctctgctgccgctgttagctggggtctttgtccttcactaagttcacccacactgttttccaagtcctctgaatgatagactgcttgctgggaaactgctgactcctggttttgtttagcaaaagaaagaattgcatctgcatgaaattttttatgggacatcctaatcacttgcccttcactaggaggatcatcctccatttcaacggcatcatgcagagtgctggataagctatcattaaggtttgtcaggtacagtcctatatcttctaaaatcttgggggccaatttttgaccacagctaaataaaatctctccttcagagatgggtttatctaaagtttcagtttcagtgacagtaacactcaatgtgctctccagtgttgatgaatcagaacctggcatctgtgagggggaaggggccttggtgccggcaggaaatggcataaagggaactggctctggaggtggaggctgagcagggaaatccatactctctggttcttcatccttagccacagacattacaatagctcttggatgaagttcttcttgaggtgagttagggttctcttcttccagtggcaggtctccatcaccccatggcttgggaagctctgggcttgataccttcaatttatcaatggaaatatctgacaaagttggggtaaaaactgccgccgctggaggaggtgtagtagtaggggtaactgttggagtattaacaagcatgatggcaggcatatcatctcctttttcagcacatatttctttcacaggaaaagccatatcatgatccgaatcacagggagaagaatctggagtctttaccaaaacacactccttagcaggtgatgaaggtgagcaaggaggcgtaggctgtggggtaggcagtggggtgcacactcttgccggcaaatatgtttcatttgttgaagcatccccagaaacacctgtagcaacaggaccttgcttctttgcttctctgtcacccagcatgacagcaatggtctcagcaagagcttcgttaacaaaatgtttaatcacatttgagttcacaggaacaccagcatcaacaaaaagctggagggcgccactgcttgttccttccacaatgtcagaagtcagtggttcacttgtctcactgactgaaacactgatactaggtgcaatctgttgctggactggaaagagcccagagataattcttgacattatttcttgctctacccattgaattaagctattttccagtgtttcttttctctcaattactttatccagaatatcagcagtgggctgaaaagtagaagcaactggcggaaatggaggaccattatattttgtagaatcagctttaacacttctgttaaactccagaattggttcagagtctggaatttcatcacatttttcttcttcctgtatgacatcgattatttcatcaaagttagttcctggaaacttcacctcttcttcatctaccttcataatttctggagtctttatccaagtttgcacaggaggaagagatgcttctttggggctagacagaggtgaaaggacatcagcactactatttgaaatgctgtcaatatctacactgggtaatacctgcacagtaagctgaggaggatcctttttttctgacttcatttctacaatggctatgttaggtttctttactccagtttctacttttcgagatgatggaggaatagaagtagtcacagttacagggtgtggcttgctgacaatcactccagcaggtggcatggtatcactattactttgggtttgtcctaaaagaattgccataggaatcagatgaccttccaatgtacctgaaaaagtaggcatttctctacttgggctgaacaaatattgctgatcgccatgaggtaacacaggaacagaatgtttcattttagaatccatcttcttaggttttgttgcatagaagtcagtctgtgttcttattgactttaccttagtgcctttaactcgttctattacttttggtctctgtggtctggacttaggagatggagaattaaatctgagatatggtccttttttaagagtgcttcgatggccctgataaactggctttccatagacttgtaacatataatcttcatcttgtattactgtggttgctttcaaaagcccttcctttctctctttctgtaaacttgaagcaggcatgcccctcataggtagatttctaaaatgctcttctatttgcttttgagaatgttttcttggaattacagatttgttgacagttttatcttgtgtgttggttctaatatctttagtcatattctgacctttcttggttctctgattcttctgatcaaatcttttttgttcataatctgttcttgacagttcatcctgaatttctgcagaaatagttttaatccattcatccactgtctttctgatcctaattttctctgacatctctctgttggtagataaagcattgataagcgaatacatggcagctccatcttttgcacgaataatagcttccaggttttcttcaagtacttttttattgttttgtactcctctcaaaatcttctcagcatctttcaatacagatcttgttgtattggttgtttgaagcttaacagaattctgtggaagatctggaagcttcaacatactcagagattcttttggctggaccatgctatttgtttctttctctttttggccaaggtcatgaagaacatcatcagacttctgcatagtcactttagttgtttctagctcttcacaggaaggaaatctgtttgttttctcaggagtccatcctatttttgacctagttagtgaggtggtgtttgatgattcactttttcttgtcaaagaatcattattattcaaaatttgttccaatagtcttacatttcctctgtgacacgacacttccatattttctttttcttccaaaagattttccctctttgatagttcatcatcccttgaaacaggtacaggagcaaatctgcgaggtgctggtgtctccaaaggagatttctgtttatcaaaactcgtatcttcaacttcttttaaaggtgcttgtttggaagcaaatgtgttatataaagatggattacagctaccaagattagggtgttctggttttacggaatacttttccactgctctggaggagggcatactaacaggctgaaaactactagtcttgagtgcagcactaataaaatgagtctgaatatctatttgttgttgttgtaacttttcaagatgccttatgtgctgctccataaacacattcatttgcttttcgtgatcatgacaatgtaatttctcttgtttcctctgaatgcttgtttgctgctctgtaacacgttgcaggtgtttatcagtctcctgtaatttactaagtaattctgtaacagaattgacttttgcttccaaatcactctgcacctttatcaacggagctgcggttgcaatggcagcagcagttgctgcagccacggttgtagctgaatcaattccactgggtgaaattctagtctcctgagtaacagcatccttctctatgcctgcatcttctaacagatgtacctttacttccttaaaaacaggcatgctttgagctttttgctttaaaactgttcttagagcatctttctgtcccattgtatactgagaaatgaagatgtcatttgctttttgcttgttgttctcttctattttatccaaaggcaacacttgcactgcaacgtctttagaaaaatcactttctgacaccatgggattttctaatagaggctggtaacaatttctagcagaagttaagtctgatgaaccacgtgatgttccattcaaactagtccccgttccaacaggaagacgtttatttgcagacaatgccggaggaacacagggcaactcatctttcagcaaaaccaaatgatctccatgattttgagaaactacctcacgaagtctcttcactggcatcttaatcttttttttcttctccaagctgacctcagagcccaaaacatccaaccagaaagctaagcgctctctggtgctcttccattcctctccgggtggaaacaaactccggacataacaggggtttatttatttatttattttaaggtagcacattgccgcacaagaccgctctacagtctcatccaagacttgaagagctcccgacttgtaatactacttgtgtttaccagggactgttgacactgcttcgcttccgaagaccgttagggacgt

SEQ ID NO: 14744 - RNA, 7850 nt, Homo sapiens
  source 1..7850: mol_type = other RNA
gctgggattacaggcatgagccaccgtgtccagtcacagcccagcaatagtaacagccttgatcttgatagtctcttaatagcatgtctcataaatagtttattccggaagttggaaattgtaaaatttaatataaaataaaaattttaaagcttataaaatcaaaagttccatttagtttgtttttacgtacatcgtcttattccaaaagaatctgaagtggttggcagaggaatgtgtacaggagtaaccatgaacagaaataatcctataaaacaaaatactagatgaatgccgggcgcggtggctcacgcctgtaatcccagcactttgggaggctgaggcaggcagatcacctgaggtcgggagttcaggactagcctgaccaacacggagaaaccccatctctactaaaaatacaaaatttgccgggcatggtggcgcacgcctgtaatcccagctactaaggaggctaaggcaggagaatcgcttgaaaccaggaggcagaggttgcggtgagccaagattgtgccattgcactccagcctgggcaacgagcaaaattccatctcaaaaaaaaaaaaaagaaaccgtcgaatggacactaattttttttaaaagaaaagctcacgtgcacagggagtagaataaatcaaagattacacttctaccctaaagttagaaaaggcaggctttctatggttaggaggaaaaatctaccaacacctttaaataaaaaatgctttaactaaaacaagattttgctgaaatccttccaaggcagaaaaaactatgaaaaccagaaaccaaggttggggggtggggtgtcatgtttaaaatgaagcagcactaagcaacatttctccagctttcaccttgcccagagtcttgtagatgaatatcaaaaacaaattaaaatccacagagcagaatttttcttccacttgtttaaaggaaactgttataagcagaactgtccaaagggccatatcaaagaaaacgggttctaaagtgaaacctaaaacattccagtaaccaaatacctgagagaagctgtgaggaagtgcatgtggaaggctgacacatttctgagtttccatagactcttgcagcttctatgttcagtgagaaaaaaaatccccaggcaatggctcctactagaagtttaaggaattctaaattgctcttcagtaattctcagccttgagtgcccattaaaattacctgaaaaggtctttttttttttttaataccaatgctggaccccatccaagatcaattaaattgaaatcccttggtacaaggcccaggcattagtattttttaaagctcccagaggttctaatgtgctgccagtgctgagatccacttagcaacctacaaaaatgctgaaaaagtcaaggatgactgtaattactgtgtgtttgaaattcagttgtgacagaaaatgatttttctgggaggtaaatttttttcactagtgctaggctgcctttcttttcatgtgcttatgccctctactatacagtactgaaatccctcaagataataagaacaacaccatttattgagcacttacatggtatcaagcactgtgctgggcactacccacccccatctccacacacaatcactgatgtccattattctgcaaaaataagtattaaacccattaatctgaaacagctgataagaaggcgtttcgttggcccctatcacaaagcaagaagttacagaattgggattagaacctacatgtatctgattacgaagcaatgctttttattttcctttaattttatgtatttatgttgcaaaaggtaatagagttacatgtttcacaggtttataaaggtttatatggtatacataaggcatataaaaattaatctcactgatgatttttttctatcacaactgaagttcaaatacatagtaaccacgattatccttgattcctatcacttagcctctcctatcacccagccaacaattctactccctggagacaaacttagcagtttcttgtttatataatatatttacaagcaaatacatgtaagaatatgtgacataccatacatttgaattcctccccaccccattttaaataatttcaacaactgcatagttcacacactattttgcacatggcttttttcactttaacagtgcatctcaaagattattccatatcaataaactttttaaatttttttttgtaatacatagtattccattgtactgatgtaccatcactttaaaaccagtctattattgatagacatttgattttttctatttgctgttataaaaatgttagaatgaataaccttgagctacataattttataaatacatacagataattacacctatagattaaatgcctagatgtcaaaagccatgccctttcactactctatgctatctcaggattctaagaaacaactcacaatcagacttataatgacttatacttattttatttaaaaactttaaatacccaaattatgctttttgttttattttaaaatattggaatttttttttcagaatatgctcaaaaaccaaacagtctgagagagggttttaagccaaggtaaaatgactttaaaaccagtggcataaacactgtgctggctgtctcttcccgttcagaaggtatctgcccccgaagactccatgtcctcctgcattgtgctgagactcagagactgagagcagtcctcgaggttcactgacggcagcatcactgacatcttggcagggggcatctgtgaagcggagagtggcactgctttcccacctgaaaatacacatgtgaggtacggattaagctcaatttgtgtccgatccatatcacctggtgaaacttgttgctgtgaaggtgcaatatcagatttatttctaacacgtaggtaactttgtgatggtttgtgttcaacttgcttaacatcctgattttgctttagttggtactgggaaaaatcttcagcggctactggtaaattaacatcattttcttgtgctgtcagaagtgttgtgggaagaaccagcttagaatttggctccaactccaattctcccaaactcattggaccatgactagcacatgaatcttcataaatactacctgaaactgtgtcaaattgccgagataatggtttaggatcacattgttgatccaaagactgtgtattagtgacaggtggctgcatatagagagaatgtcccattaagatgttctctgctgccgctgttagctggggtctttgtccttcactaagttcacccacactgttttccaagtcctctgaatgatagactgcttgctgggaaactgctgactcctggttttgtttagcaaaagaaagaattgcatctgcatgaaattttttatgggacatcctaatcacttgcccttcactaggaggatcatcctccatttcaacggcatcatgcagagtgctggataagctatcattaaggtttgtcaggtacagtcctatatcttctaaaatcttgggggccaatttttgaccacagctaaataaaatctctccttcagagatgggtttatctaaagtttcagtttcagtgacagtaacactcaatgtgctctccagtgttgatgaatcagaacctggcatctgtgagggggaaggggccttggtgccggcaggaaatggcataaagggaactggctctggaggtggaggctgagcagggaaatccatactctctggttcttcatccttagccacagacattacaatagctcttggatgaagttcttcttgaggtgagttagggttctcttcttccagtggcaggtctccatcaccccatggcttgggaagctctgggcttgataccttcaatttatcaatggaaatatctgacaaagttggggtaaaaactgccgccgctggaggaggtgtagtagtaggggtaactgttggagtattaacaagcatgatggcaggcatatcatctcctttttcagcacatatttctttcacaggaaaagccatatcatgatccgaatcacagggagaagaatctggagtctttaccaaaacacactccttagcaggtgatgaaggtgagcaaggaggcgtaggctgtggggtaggcagtggggtgcacactcttgccggcaaatatgtttcatttgttgaagcatccccagaaacacctgtagcaacaggaccttgcttctttgcttctctgtcacccagcatgacagcaatggtctcagcaagagcttcgttaacaaaatgtttaatcacatttgagttcacaggaacaccagcatcaacaaaaagctggagggcgccactgcttgttccttccacaatgtcagaagtcagtggttcacttgtctcactgactgaaacactgatactaggtgcaatctgttgctggactggaaagagcccagagataattcttgacattatttcttgctctacccattgaattaagctattttccagtgtttcttttctctcaattactttatccagaatatcagcagtgggctgaaaagtagaagcaactggcggaaatggaggaccattatattttgtagaatcagctttaacacttctgttaaactccagaattggttcagagtctggaatttcatcacatttttcttcttcctgtatgacatcgattatttcatcaaagttagttcctggaaacttcacctcttcttcatctaccttcataatttctggagtctttatccaagtttgcacaggaggaagagatgcttctttggggctagacagaggtgaaaggacatcagcactactatttgaaatgctgtcaatatctacactgggtaatacctgcacagtaagctgaggaggatcctttttttctgacttcatttctacaatggctatgttaggtttctttactccagtttctacttttcgagatgatggaggaatagaagtagtcacagttacagggtgtggcttgctgacaatcactccagcaggtggcatggtatcactattactttgggtttgtcctaaaagaattgccataggaatcagatgaccttccaatgtacctgaaaaagtaggcatttctctacttgggctgaacaaatattgctgatcgccatgaggtaacacaggaacagaatgtttcattttagaatccatcttcttaggttttgttgcatagaagtcagtctgtgttcttattgactttaccttagtgcctttaactcgttctattacttttggtctctgtggtctggacttaggagatggagaattaaatctgagatatggtccttttttaagagtgcttcgatggccctgataaactggctttccatagacttgtaacatataatcttcatcttgtattactgtggttgctttcaaaagcccttcctttctctctttctgtaaacttgaagcaggcatgcccctcataggtagatttctaaaatgctcttctatttgcttttgagaatgttttcttggaattacagatttgttgacagttttatcttgtgtgttggttctaatatctttagtcatattctgacctttcttggttctctgattcttctgatcaaatcttttttgttcataatctgttcttgacagttcatcctgaatttctgcagaaatagttttaatccattcatccactgtctttctgatcctaattttctctgacatctctctgttggtagataaagcattgataagcgaatacatggcagctccatcttttgcacgaataatagcttccaggttttcttcaagtacttttttattgttttgtactcctctcaaaatcttctcagcatctttcaatacagatcttgttgtattggttgtttgaagcttaacagaattctgtggaagatctggaagcttcaacatactcagagattcttttggctggaccatgctatttgtttctttctctttttggccaaggtcatgaagaacatcatcagacttctgcatagtcactttagttgtttctagctcttcacaggaaggaaatctgtttgttttctcaggagtccatcctatttttgacctagttagtgaggtggtgtttgatgattcactttttcttgtcaaagaatcattattattcaaaatttgttccaatagtcttacatttcctctgtgacacgacacttccatattttctttttcttccaaaagattttccctctttgatagttcatcatcccttgaaacaggtacaggagcaaatctgcgaggtgctggtgtctccaaaggagatttctgtttatcaaaactcgtatcttcaacttcttttaaaggtgcttgtttggaagcaaatgtgttatataaagatggattacagctaccaagattagggtgttctggttttacggaatacttttccactgctctggaggagggcatactaacaggctgaaaactactagtcttgagtgcagcactaataaaatgagtctgaatatctatttgttgttgttgtaacttttcaagatgccttatgtgctgctccataaacacattcatttgcttttcgtgatcatgacaatgtaatttctcttgtttcctctgaatgcttgtttgctgctctgtaacacgttgcaggtgtttatcagtctcctgtaatttactaagtaattctgtaacagaattgacttttgcttccaaatcactctgcacctttatcaacggagctgcggttgcaatggcagcagcagttgctgcagccacggttgtagctgaatcaattccactgggtgaaattctagtctcctgagtaacagcatccttctctatgcctgcatcttctaacagatgtacctttacttccttaaaaacaggcatgctttgagctttttgctttaaaactgttcttagagcatctttctgtcccattgtatactgagaaatgaagatgtcatttgctttttgcttgttgttctcttctattttatccaaaggcaacacttgcactgcaacgtctttagaaaaatcactttctgacaccatgggattttctaatagaggctggtaacaatttctagcagaagttaagtctgatgaaccacgtgatgttccattcaaactagtccccgttccaacaggaagacgtttatttgcagacaatgccggaggaacacagggcaactcatctttcagcaaaaccaaatgatctccatgattttgagaaactacctcacgaagtctcttcactggcatcttaatcttttttttcttctccaagctgacctcagagcctttcatattgttggtcacaaaacaagtcccacacttaaggacggaaaaactttctctgtttccttaagacttcagaacaaaattttcacctctttgcaataactgtttttaaaatgtcgaacatccacaaagctgaaaatctaaattctgatattgaatccaggattagagctgactataaagtcatatttacccattaatcccactcagtctattaatacaccacgccaaaatgtgaaagtggggatgacaagagaatggccacaggagcaacaataaccataacagtgcactccccaaccccagagctggtagggcaaaaccaaacacatgtagtggcgggcttaaaatttgttgagaagaggcagtcaagcaaataaaagcgaaatgctatttttaaaataatgacccacataagaagcgtaatagctttcttcagccacagagtcttacacacccctccagatgcaatcgtcggaaacataaattcacccctacgtatctccagaacgcccgagacccgcaccgtcgtgggtgtaatctgacaacagc

SEQ ID NO: 14745 - RNA, 7343 nt, Homo sapiens
  source 1..7343: mol_type = other RNA
gctgggattacaggcatgagccaccgtgtccagtcacagcccagcaatagtaacagccttgatcttgatagtctcttaatagcatgtctcataaatagtttattccggaagttggaaattgtaaaatttaatataaaataaaaattttaaagcttataaaatcaaaagttccatttagtttgtttttacgtacatcgtcttattccaaaagaatctgaagtggttggcagaggaatgtgtacaggagtaaccatgaacagaaataatcctataaaacaaaatactagatgaatgccgggcgcggtggctcacgcctgtaatcccagcactttgggaggctgaggcaggcagatcacctgaggtcgggagttcaggactagcctgaccaacacggagaaaccccatctctactaaaaatacaaaatttgccgggcatggtggcgcacgcctgtaatcccagctactaaggaggctaaggcaggagaatcgcttgaaaccaggaggcagaggttgcggtgagccaagattgtgccattgcactccagcctgggcaacgagcaaaattccatctcaaaaaaaaaaaaaagaaaccgtcgaatggacactaattttttttaaaagaaaagctcacgtgcacagggagtagaataaatcaaagattacacttctaccctaaagttagaaaaggcaggctttctatggttaggaggaaaaatctaccaacacctttaaataaaaaatgctttaactaaaacaagattttgctgaaatccttccaaggcagaaaaaactatgaaaaccagaaaccaaggttggggggtggggtgtcatgtttaaaatgaagcagcactaagcaacatttctccagctttcaccttgcccagagtcttgtagatgaatatcaaaaacaaattaaaatccacagagcagaatttttcttccacttgtttaaaggaaactgttataagcagaactgtccaaagggccatatcaaagaaaacgggttctaaagtgaaacctaaaacattccagtaaccaaatacctgagagaagctgtgaggaagtgcatgtggaaggctgacacatttctgagtttccatagactcttgcagcttctatgttcagtgagaaaaaaaatccccaggcaatggctcctactagaagtttaaggaattctaaattgctcttcagtaattctcagccttgagtgcccattaaaattacctgaaaaggtctttttttttttttaataccaatgctggaccccatccaagatcaattaaattgaaatcccttggtacaaggcccaggcattagtattttttaaagctcccagaggttctaatgtgctgccagtgctgagatccacttagcaacctacaaaaatgctgaaaaagtcaaggatgactgtaattactgtgtgtttgaaattcagttgtgacagaaaatgatttttctgggaggtaaatttttttcactagtgctaggctgcctttcttttcatgtgcttatgccctctactatacagtactgaaatccctcaagataataagaacaacaccatttattgagcacttacatggtatcaagcactgtgctgggcactacccacccccatctccacacacaatcactgatgtccattattctgcaaaaataagtattaaacccattaatctgaaacagctgataagaaggcgtttcgttggcccctatcacaaagcaagaagttacagaattgggattagaacctacatgtatctgattacgaagcaatgctttttattttcctttaattttatgtatttatgttgcaaaaggtaatagagttacatgtttcacaggtttataaaggtttatatggtatacataaggcatataaaaattaatctcactgatgatttttttctatcacaactgaagttcaaatacatagtaaccacgattatccttgattcctatcacttagcctctcctatcacccagccaacaattctactccctggagacaaacttagcagtttcttgtttatataatatatttacaagcaaatacatgtaagaatatgtgacataccatacatttgaattcctccccaccccattttaaataatttcaacaactgcatagttcacacactattttgcacatggcttttttcactttaacagtgcatctcaaagattattccatatcaataaactttttaaatttttttttgtaatacatagtattccattgtactgatgtaccatcactttaaaaccagtctattattgatagacatttgattttttctatttgctgttataaaaatgttagaatgaataaccttgagctacataattttataaatacatacagataattacacctatagattaaatgcctagatgtcaaaagccatgccctttcactactctatgctatctcaggattctaagaaacaactcacaatcagacttataatgacttatacttattttatttaaaaactttaaatacccaaattatgctttttgttttattttaaaatattggaatttttttttcagaatatgctcaaaaaccaaacagtctgagagagggttttaagccaaggtaaaatgactttaaaaccagtggcataaacactgtgctggctgtctcttcccgttcagaaggtatctgcccccgaagactccatgtcctcctgcattgtgctgagactcagagactgagagcagtcctcgaggttcactgacggcagcatcactgacatcttggcagggggcatctgtgaagcggagagtggcactgctttcccacctgaaaatacacatgtgaggtacggattaagctcaatttgtgtccgatccatatcacctggtgaaacttgttgctgtgaaggtgcaatatcagatttatttctaacacgtaggtaactttgtgatggtttgtgttcaacttgcttaacatcctgattttgctttagttggtactgggaaaaatcttcagcggctactggtaaattaacatcattttcttgtgctgtcagaagtgttgtgggaagaaccagcttagaatttggctccaactccaattctcccaaactcattggaccatgactagcacatgaatcttcataaatactacctgaaactgtgtcaaattgccgagataatggtttaggatcacattgttgatccaaagactgtgtattagtgacaggtggctgcatatagagagaatgtcccattaagatgttctctgctgccgctgttagctggggtctttgtccttcactaagttcacccacactgttttccaagtcctctgaatgatagactgcttgctgggaaactgctgactcctggttttgtttagcaaaagaaagaattgcatctgcatgaaattttttatgggacatcctaatcacttgcccttcactaggaggatcatcctccatttcaacggcatcatgcagagtgctggataagctatcattaaggtttgtcaggtacagtcctatatcttctaaaatcttgggggccaatttttgaccacagctaaataaaatctctccttcagagatgggtttatctaaagtttcagtttcagtgacagtaacactcaatgtgctctccagtgttgatgaatcagaacctggcatctgtgagggggaaggggccttggtgccggcaggaaatggcataaagggaactggctctggaggtggaggctgagcagggaaatccatactctctggttcttcatccttagccacagacattacaatagctcttggatgaagttcttcttgaggtgagttagggttctcttcttccagtggcaggtctccatcaccccatggcttgggaagctctgggcttgataccttcaatttatcaatggaaatatctgacaaagttggggtaaaaactgccgccgctggaggaggtgtagtagtaggggtaactgttggagtattaacaagcatgatggcaggcatatcatctcctttttcagcacatatttctttcacaggaaaagccatatcatgatccgaatcacagggagaagaatctggagtctttaccaaaacacactccttagcaggtgatgaaggtgagcaaggaggcgtaggctgtggggtaggcagtggggtgcacactcttgccggcaaatatgtttcatttgttgaagcatccccagaaacacctgtagcaacaggaccttgcttctttgcttctctgtcacccagcatgacagcaatggtctcagcaagagcttcgttaacaaaatgtttaatcacatttgagttcacaggaacaccagcatcaacaaaaagctggagggcgccactgcttgttccttccacaatgtcagaagtcagtggttcacttgtctcactgactgaaacactgatactaggtgcaatctgttgctggactggaaagagcccagagataattcttgacattatttcttgctctacccattgaattaagctattttccagtgtttcttttctctcaattactttatccagaatatcagcagtgggctgaaaagtagaagcaactggcggaaatggaggaccattatattttgtagaatcagctttaacacttctgttaaactccagaattggttcagagtctggaatttcatcacatttttcttcttcctgtatgacatcgattatttcatcaaagttagttcctggaaacttcacctcttcttcatctaccttcataatttctggagtctttatccaagtttgcacaggaggaagagatgcttctttggggctagacagaggtgaaaggacatcagcactactatttgaaatgctgtcaatatctacactgggtaatacctgcacagtaagctgaggaggatcctttttttctgacttcatttctacaatggctatgttaggtttctttactccagtttctacttttcgagatgatggaggaatagaagtagtcacagttacagggtgtggcttgctgacaatcactccagcaggtggcatggtatcactattactttgggtttgtcctaaaagaattgccataggaatcagatgaccttccaatgtacctgaaaaagtaggcatttctctacttgggctgaacaaatattgctgatcgccatgaggtaacacaggaacagaatgtttcattttagaatccatcttcttaggttttgttgcatagaagtcagtctgtgttcttattgactttaccttagtgcctttaactcgttctattacttttggtctctgtggtctggacttaggagatggagaattaaatctgagatatggtccttttttaagagtgcttcgatggccctgataaactggctttccatagacttgtaacatataatcttcatcttgtattactgtggttgctttcaaaagcccttcctttctctctttctgtaaacttgaagcaggcatgcccctcataggtagatttctaaaatgctcttctatttgcttttgagaatgttttcttggaattacagatttgttgacagttttatcttgtgtgttggttctaatatctttagtcatattctgacctttcttggttctctgattcttctgatcaaatcttttttgttcataatctgttcttgacagttcatcctgaatttctgcagaaatagttttaatccattcatccactgtctttctgatcctaattttctctgacatctctctgttggtagataaagcattgataagcgaatacatggcagctccatcttttgcacgaataatagcttccaggttttcttcaagtacttttttattgttttgtactcctctcaaaatcttctcagcatctttcaatacagatcttgttgtattggttgtttgaagcttaacagaattctgtggaagatctggaagcttcaacatactcagagattcttttggctggaccatgctatttgtttctttctctttttggccaaggtcatgaagaacatcatcagacttctgcatagtcactttagttgtttctagctcttcacaggaaggaaatctgtttgttttctcaggagtccatcctatttttgacctagttagtgaggtggtgtttgatgattcactttttcttgtcaaagaatcattattattcaaaatttgttccaatagtcttacatttcctctgtgacacgacacttccatattttctttttcttccaaaagattttccctctttgatagttcatcatcccttgaaacaggtacaggagcaaatctgcgaggtgctggtgtctccaaaggagatttctgtttatcaaaactcgtatcttcaacttcttttaaaggtgcttgtttggaagcaaatgtgttatataaagatggattacagctaccaagattagggtgttctggttttacggaatacttttccactgctctggaggagggcatactaacaggctgaaaactactagtcttgagtgcagcactaataaaatgagtctgaatatctatttgttgttgttgtaacttttcaagatgccttatgtgctgctccataaacacattcatttgcttttcgtgatcatgacaatgtaatttctcttgtttcctctgaatgcttgtttgctgctctgtaacacgttgcaggtgtttatcagtctcctgtaatttactaagtaattctgtaacagaattgacttttgcttccaaatcactctgcacctttatcaacggagctgcggttgcaatggcagcagcagttgctgcagccacggttgtagctgaatcaattccactgggtgaaattctagtctcctgagtaacagcatccttctctatgcctgcatcttctaacagatgtacctttacttccttaaaaacaggcatgctttgagctttttgctttaaaactgttcttagagcatctttctgtcccattgtatactgagaaatgaagatgtcatttgctttttgcttgttgttctcttctattttatccaaaggcaacacttgcactgcaacgtctttagaaaaatcactttctgacaccatgggattttctaatagaggctggtaacaatttctagcagaagttaagtctgatgaacccaaaacatccaaccagaaagctaagcgctctctggtgctcttccattcctctccgggtggaaacaaactccggacataacaggggtttatttatttatttattttaaggtagcacattgccgcacaagaccgctctacagtctcatccaagacttgaagagctcccgacttgtaatactacttgtgtttaccagggactgttgacactgcttcgcttccgaagaccgttagggacgt

SEQ ID NO: 14746 - RNA, 7200 nt, Homo sapiens
  source 1..7200: mol_type = other RNA
gctgggattacaggcatgagccaccgtgtccagtcacagcccagcaatagtaacagccttgatcttgatagtctcttaatagcatgtctcataaatagtttattccggaagttggaaattgtaaaatttaatataaaataaaaattttaaagcttataaaatcaaaagttccatttagtttgtttttacgtacatcgtcttattccaaaagaatctgaagtggttggcagaggaatgtgtacaggagtaaccatgaacagaaataatcctataaaacaaaatactagatgaatgccgggcgcggtggctcacgcctgtaatcccagcactttgggaggctgaggcaggcagatcacctgaggtcgggagttcaggactagcctgaccaacacggagaaaccccatctctactaaaaatacaaaatttgccgggcatggtggcgcacgcctgtaatcccagctactaaggaggctaaggcaggagaatcgcttgaaaccaggaggcagaggttgcggtgagccaagattgtgccattgcactccagcctgggcaacgagcaaaattccatctcaaaaaaaaaaaaaagaaaccgtcgaatggacactaattttttttaaaagaaaagctcacgtgcacagggagtagaataaatcaaagattacacttctaccctaaagttagaaaaggcaggctttctatggttaggaggaaaaatctaccaacacctttaaataaaaaatgctttaactaaaacaagattttgctgaaatccttccaaggcagaaaaaactatgaaaaccagaaaccaaggttggggggtggggtgtcatgtttaaaatgaagcagcactaagcaacatttctccagctttcaccttgcccagagtcttgtagatgaatatcaaaaacaaattaaaatccacagagcagaatttttcttccacttgtttaaaggaaactgttataagcagaactgtccaaagggccatatcaaagaaaacgggttctaaagtgaaacctaaaacattccagtaaccaaatacctgagagaagctgtgaggaagtgcatgtggaaggctgacacatttctgagtttccatagactcttgcagcttctatgttcagtgagaaaaaaaatccccaggcaatggctcctactagaagtttaaggaattctaaattgctcttcagtaattctcagccttgagtgcccattaaaattacctgaaaaggtctttttttttttttaataccaatgctggaccccatccaagatcaattaaattgaaatcccttggtacaaggcccaggcattagtattttttaaagctcccagaggttctaatgtgctgccagtgctgagatccacttagcaacctacaaaaatgctgaaaaagtcaaggatgactgtaattactgtgtgtttgaaattcagttgtgacagaaaatgatttttctgggaggtaaatttttttcactagtgctaggctgcctttcttttcatgtgcttatgccctctactatacagtactgaaatccctcaagataataagaacaacaccatttattgagcacttacatggtatcaagcactgtgctgggcactacccacccccatctccacacacaatcactgatgtccattattctgcaaaaataagtattaaacccattaatctgaaacagctgataagaaggcgtttcgttggcccctatcacaaagcaagaagttacagaattgggattagaacctacatgtatctgattacgaagcaatgctttttattttcctttaattttatgtatttatgttgcaaaaggtaatagagttacatgtttcacaggtttataaaggtttatatggtatacataaggcatataaaaattaatctcactgatgatttttttctatcacaactgaagttcaaatacatagtaaccacgattatccttgattcctatcacttagcctctcctatcacccagccaacaattctactccctggagacaaacttagcagtttcttgtttatataatatatttacaagcaaatacatgtaagaatatgtgacataccatacatttgaattcctccccaccccattttaaataatttcaacaactgcatagttcacacactattttgcacatggcttttttcactttaacagtgcatctcaaagattattccatatcaataaactttttaaatttttttttgtaatacatagtattccattgtactgatgtaccatcactttaaaaccagtctattattgatagacatttgattttttctatttgctgttataaaaatgttagaatgaataaccttgagctacataattttataaatacatacagataattacacctatagattaaatgcctagatgtcaaaagccatgccctttcactactctatgctatctcaggattctaagaaacaactcacaatcagacttataatgacttatacttattttatttaaaaactttaaatacccaaattatgctttttgttttattttaaaatattggaatttttttttcagaatatgctcaaaaaccaaacagtctgagagagggttttaagccaaggtaaaatgactttaaaaccagtggcataaacactgtgctggctgtctcttcccgttcagaaggtatctgcccccgaagactccatgtcctcctgcattgtgctgagactcagagactgagagcagtcctcgaggttcactgacggcagcatcactgacatcttggcagggggcatctgtgaagcggagagtggcactgctttcccacctgaaaatacacatgtgaggtacggattaagctcaatttgtgtccgatccatatcacctggtgaaacttgttgctgtgaaggtgcaatatcagatttatttctaacacgtaggtaactttgtgatggtttgtgttcaacttgcttaacatcctgattttgctttagttggtactgggaaaaatcttcagcggctactggtaaattaacatcattttcttgtgctgtcagaagtgttgtgggaagaaccagcttagaatttggctccaactccaattctcccaaactcattggaccatgactagcacatgaatcttcataaatactacctgaaactgtgtcaaattgccgagataatggtttaggatcacattgttgatccaaagactgtgtattagtgacaggtggctgcatatagagagaatgtcccattaagatgttctctgctgccgctgttagctggggtctttgtccttcactaagttcacccacactgttttccaagtcctctgaatgatagactgcttgctgggaaactgctgactcctggttttgtttagcaaaagaaagaattgcatctgcatgaaattttttatgggacatcctaatcacttgcccttcactaggaggatcatcctccatttcaacggcatcatgcagagtgctggataagctatcattaaggtttgtcaggtacagtcctatatcttctaaaatcttgggggccaatttttgaccacagctaaataaaatctctccttcagagatgggtttatctaaagtttcagtttcagtgacagtaacactcaatgtgctctccagtgttgatgaatcagaacctggcatctgtgagggggaaggggccttggtgccggcaggaaatggcataaagggaactggctctggaggtggaggctgagcagggaaatccatactctctggttcttcatccttagccacagacattacaatagctcttggatgaagttcttcttgaggtgagttagggttctcttcttccagtggcaggtctccatcaccccatggcttgggaagctctgggcttgataccttcaatttatcaatggaaatatctgacaaagttggggtaaaaactgccgccgctggaggaggtgtagtagtaggggtaactgttggagtattaacaagcatgatggcaggcatatcatctcctttttcagcacatatttctttcacaggaaaagccatatcatgatccgaatcacagggagaagaatctggagtctttaccaaaacacactccttagcaggtgatgaaggtgagcaaggaggcgtaggctgtggggtaggcagtggggtgcacactcttgccggcaaatatgtttcatttgttgaagcatccccagaaacacctgtagcaacaggaccttgcttctttgcttctctgtcacccagcatgacagcaatggtctcagcaagagcttcgttaacaaaatgtttaatcacatttgagttcacaggaacaccagcatcaacaaaaagctggagggcgccactgcttgttccttccacaatgtcagaagtcagtggttcacttgtctcactgactgaaacactgatactaggtgcaatctgttgctggactggaaagagcccagagataattcttgacattatttcttgctctacccattgaattaagctattttccagtgtttcttttctctcaattactttatccagaatatcagcagtgggctgaaaagtagaagcaactggcggaaatggaggaccattatattttgtagaatcagctttaacacttctgttaaactccagaattggttcagagtctggaatttcatcacatttttcttcttcctgtatgacatcgattatttcatcaaagttagttcctggaaacttcacctcttcttcatctaccttcataatttctggagtctttatccaagtttgcacaggaggaagagatgcttctttggggctagacagaggtgaaaggacatcagcactactatttgaaatgctgtcaatatctacactgggtaatacctgcacagtaagctgaggaggatcctttttttctgacttcatttctacaatggctatgttaggtttctttactccagtttctacttttcgagatgatggaggaatagaagtagtcacagttacagggtgtggcttgctgacaatcactccagcaggtggcatggtatcactattactttgggtttgtcctaaaagaattgccataggaatcagatgaccttccaatgtacctgaaaaagtaggcatttctctacttgggctgaacaaatattgctgatcgccatgaggtaacacaggaacagaatgtttcattttagaatccatcttcttaggttttgttgcatagaagtcagtctgtgttcttattgactttaccttagtgcctttaactcgttctattacttttggtctctgtggtctggacttaggagatggagaattaaatctgagatatggtccttttttaagagtgcttcgatggccctgataaactggctttccatagacttgtaacatataatcttcatcttgtattactgtggttgctttcaaaagcccttcctttctctctttctgtaaacttgaagcaggcatgcccctcataggtagatttctaaaatgctcttctatttgcttttgagaatgttttcttggaattacagatttgttgacagttttatcttgtgtgttggttctaatatctttagtcatattctgacctttcttggttctctgattcttctgatcaaatcttttttgttcataatctgttcttgacagttcatcctgaatttctgcagaaatagttttaatccattcatccactgtctttctgatcctaattttctctgacatctctctgttggtagataaagcattgataagcgaatacatggcagctccatcttttgcacgaataatagcttccaggttttcttcaagtacttttttattgttttgtactcctctcaaaatcttctcagcatctttcaatacagatcttgttgtattggttgtttgaagcttaacagaattctgtggaagatctggaagcttcaacatactcagagattcttttggctggaccatgctatttgtttctttctctttttggccaaggtcatgaagaacatcatcagacttctgcatagtcactttagttgtttctagctcttcacaggaaggaaatctgtttgttttctcaggagtccatcctatttttgacctagttagtgaggtggtgtttgatgattcactttttcttgtcaaagaatcattattattcaaaatttgttccaatagtcttacatttcctctgtgacacgacacttccatattttctttttcttccaaaagattttccctctttgatagttcatcatcccttgaaacaggtacaggagcaaatctgcgaggtgctggtgtctccaaaggagatttctgtttatcaaaactcgtatcttcaacttcttttaaaggtgcttgtttggaagcaaatgtgttatataaagatggattacagctaccaagattagggtgttctggttttacggaatacttttccactgctctggaggagggcatactaacaggctgaaaactactagtcttgagtgcagcactaataaaatgagtctgaatatctatttgttgttgttgtaacttttcaagatgccttatgtgctgctccataaacacattcatttgcttttcgtgatcatgacaatgtaatttctcttgtttcctctgaatgcttgtttgctgctctgtaacacgttgcaggtgtttatcagtctcctgtaatttactaagtaattctgtaacagaattgacttttgcttccaaatcactctgcacctttatcaacggagctgcggttgcaatggcagcagcagttgctgcagccacggttgtagctgaatcaattccactgggtgaaattctagtctcctgagtaacagcatccttctctatgcctgcatcttctaacagatgtacctttacttccttaaaaacaggcatgctttgagctttttgctttaaaactgttcttagagcatctttctgtcccattgtatactgagaaatgaagatgtcatttgctttttgcttgttgttctcttctattttatccaaaggcaacacttgcactgcaacgtctttagaaaaatcactttctgacaccatgggattttctaatagaggctggtaacaatttctagcagaagttaagtctgatgaacccctccagatgcaatcgtcggaaacataaattcacccctacgtatctccagaacgcccgagacccgcaccgtcgtgggtgtaatctgacaacagc

SEQ ID NO: 14747 - RNA, 7777 nt, Homo sapiens
  source 1..7777: mol_type = other RNA
gctgggattacaggcatgagccaccgtgtccagtcacagcccagcaatagtaacagccttgatcttgatagtctcttaatagcatgtctcataaatagtttattccggaagttggaaattgtaaaatttaatataaaataaaaattttaaagcttataaaatcaaaagttccatttagtttgtttttacgtacatcgtcttattccaaaagaatctgaagtggttggcagaggaatgtgtacaggagtaaccatgaacagaaataatcctataaaacaaaatactagatgaatgccgggcgcggtggctcacgcctgtaatcccagcactttgggaggctgaggcaggcagatcacctgaggtcgggagttcaggactagcctgaccaacacggagaaaccccatctctactaaaaatacaaaatttgccgggcatggtggcgcacgcctgtaatcccagctactaaggaggctaaggcaggagaatcgcttgaaaccaggaggcagaggttgcggtgagccaagattgtgccattgcactccagcctgggcaacgagcaaaattccatctcaaaaaaaaaaaaaagaaaccgtcgaatggacactaattttttttaaaagaaaagctcacgtgcacagggagtagaataaatcaaagattacacttctaccctaaagttagaaaaggcaggctttctatggttaggaggaaaaatctaccaacacctttaaataaaaaatgctttaactaaaacaagattttgctgaaatccttccaaggcagaaaaaactatgaaaaccagaaaccaaggttggggggtggggtgtcatgtttaaaatgaagcagcactaagcaacatttctccagctttcaccttgcccagagtcttgtagatgaatatcaaaaacaaattaaaatccacagagcagaatttttcttccacttgtttaaaggaaactgttataagcagaactgtccaaagggccatatcaaagaaaacgggttctaaagtgaaacctaaaacattccagtaaccaaatacctgagagaagctgtgaggaagtgcatgtggaaggctgacacatttctgagtttccatagactcttgcagcttctatgttcagtgagaaaaaaaatccccaggcaatggctcctactagaagtttaaggaattctaaattgctcttcagtaattctcagccttgagtgcccattaaaattacctgaaaaggtctttttttttttttaataccaatgctggaccccatccaagatcaattaaattgaaatcccttggtacaaggcccaggcattagtattttttaaagctcccagaggttctaatgtgctgccagtgctgagatccacttagcaacctacaaaaatgctgaaaaagtcaaggatgactgtaattactgtgtgtttgaaattcagttgtgacagaaaatgatttttctgggaggtaaatttttttcactagtgctaggctgcctttcttttcatgtgcttatgccctctactatacagtactgaaatccctcaagataataagaacaacaccatttattgagcacttacatggtatcaagcactgtgctgggcactacccacccccatctccacacacaatcactgatgtccattattctgcaaaaataagtattaaacccattaatctgaaacagctgataagaaggcgtttcgttggcccctatcacaaagcaagaagttacagaattgggattagaacctacatgtatctgattacgaagcaatgctttttattttcctttaattttatgtatttatgttgcaaaaggtaatagagttacatgtttcacaggtttataaaggtttatatggtatacataaggcatataaaaattaatctcactgatgatttttttctatcacaactgaagttcaaatacatagtaaccacgattatccttgattcctatcacttagcctctcctatcacccagccaacaattctactccctggagacaaacttagcagtttcttgtttatataatatatttacaagcaaatacatgtaagaatatgtgacataccatacatttgaattcctccccaccccattttaaataatttcaacaactgcatagttcacacactattttgcacatggcttttttcactttaacagtgcatctcaaagattattccatatcaataaactttttaaatttttttttgtaatacatagtattccattgtactgatgtaccatcactttaaaaccagtctattattgatagacatttgattttttctatttgctgttataaaaatgttagaatgaataaccttgagctacataattttataaatacatacagataattacacctatagattaaatgcctagatgtcaaaagccatgccctttcactactctatgctatctcaggattctaagaaacaactcacaatcagacttataatgacttatacttattttatttaaaaactttaaatacccaaattatgctttttgttttattttaaaatattggaatttttttttcagaatatgctcaaaaaccaaacagtctgagagagggttttaagccaaggtaaaatgactttaaaaccagtggcataaacactgtgctggctgtctcttcccgttcagaaggtatctgcccccgaagactccatgtcctcctgcattgtgctgagactcagagactgagagcagtcctcgaggttcactgacggcagcatcactgacatcttggcagggggcatctgtgaagcggagagtggcactgctttcccacctgggtgatgaaataatctgtatgacaaacctccacagcccgagtttacctatacaggaaaccttcttcacatgtacccccaaacctgaaaatacacatgtgaggtacggattaagctcaatttgtgtccgatccatatcacctggtgaaacttgttgctgtgaaggtgcaatatcagatttatttctaacacgtaggtaactttgtgatggtttgtgttcaacttgcttaacatcctgattttgctttagttggtactgggaaaaatcttcagcggctactggtaaattaacatcattttcttgtgctgtcagaagtgttgtgggaagaaccagcttagaatttggctccaactccaattctcccaaactcattggaccatgactagcacatgaatcttcataaatactacctgaaactgtgtcaaattgccgagataatggtttaggatcacattgttgatccaaagactgtgtattagtgacaggtggctgcatatagagagaatgtcccattaagatgttctctgctgccgctgttagctggggtctttgtccttcactaagttcacccacactgttttccaagtcctctgaatgatagactgcttgctgggaaactgctgactcctggttttgtttagcaaaagaaagaattgcatctgcatgaaattttttatgggacatcctaatcacttgcccttcactaggaggatcatcctccatttcaacggcatcatgcagagtgctggataagctatcattaaggtttgtcaggtacagtcctatatcttctaaaatcttgggggccaatttttgaccacagctaaataaaatctctccttcagagatgggtttatctaaagtttcagtttcagtgacagtaacactcaatgtgctctccagtgttgatgaatcagaacctggcatctgtgagggggaaggggccttggtgccggcaggaaatggcataaagggaactggctctggaggtggaggctgagcagggaaatccatactctctggttcttcatccttagccacagacattacaatagctcttggatgaagttcttcttgaggtgagttagggttctcttcttccagtggcaggtctccatcaccccatggcttgggaagctctgggcttgataccttcaatttatcaatggaaatatctgacaaagttggggtaaaaactgccgccgctggaggaggtgtagtagtaggggtaactgttggagtattaacaagcatgatggcaggcatatcatctcctttttcagcacatatttctttcacaggaaaagccatatcatgatccgaatcacagggagaagaatctggagtctttaccaaaacacactccttagcaggtgatgaaggtgagcaaggaggcgtaggctgtggggtaggcagtggggtgcacactcttgccggcaaatatgtttcatttgttgaagcatccccagaaacacctgtagcaacaggaccttgcttctttgcttctctgtcacccagcatgacagcaatggtctcagcaagagcttcgttaacaaaatgtttaatcacatttgagttcacaggaacaccagcatcaacaaaaagctggagggcgccactgcttgttccttccacaatgtcagaagtcagtggttcacttgtctcactgactgaaacactgatactaggtgcaatctgttgctggactggaaagagcccagagataattcttgacattatttcttgctctacccattgaattaagctattttccagtgtttcttttctctcaattactttatccagaatatcagcagtgggctgaaaagtagaagcaactggcggaaatggaggaccattatattttgtagaatcagctttaacacttctgttaaactccagaattggttcagagtctggaatttcatcacatttttcttcttcctgtatgacatcgattatttcatcaaagttagttcctggaaacttcacctcttcttcatctaccttcataatttctggagtctttatccaagtttgcacaggaggaagagatgcttctttggggctagacagaggtgaaaggacatcagcactactatttgaaatgctgtcaatatctacactgggtaatacctgcacagtaagctgaggaggatcctttttttctgacttcatttctacaatggctatgttaggtttctttactccagtttctacttttcgagatgatggaggaatagaagtagtcacagttacagggtgtggcttgctgacaatcactccagcaggtggcatggtatcactattactttgggtttgtcctaaaagaattgccataggaatcagatgaccttccaatgtacctgaaaaagtaggcatttctctacttgggctgaacaaatattgctgatcgccatgaggtaacacaggaacagaatgtttcattttagaatccatcttcttaggttttgttgcatagaagtcagtctgtgttcttattgactttaccttagtgcctttaactcgttctattacttttggtctctgtggtctggacttaggagatggagaattaaatctgagatatggtccttttttaagagtgcttcgatggccctgataaactggctttccatagacttgtaacatataatcttcatcttgtattactgtggttgctttcaaaagcccttcctttctctctttctgtaaacttgaagcaggcatgcccctcataggtagatttctaaaatgctcttctatttgcttttgagaatgttttcttggaattacagatttgttgacagttttatcttgtgtgttggttctaatatctttagtcatattctgacctttcttggttctctgattcttctgatcaaatcttttttgttcataatctgttcttgacagttcatcctgaatttctgcagaaatagttttaatccattcatccactgtctttctgatcctaattttctctgacatctctctgttggtagataaagcattgataagcgaatacatggcagctccatcttttgcacgaataatagcttccaggttttcttcaagtacttttttattgttttgtactcctctcaaaatcttctcagcatctttcaatacagatcttgttgtattggttgtttgaagcttaacagaattctgtggaagatctggaagcttcaacatactcagagattcttttggctggaccatgctatttgtttctttctctttttggccaaggtcatgaagaacatcatcagacttctgcatagtcactttagttgtttctagctcttcacaggaaggaaatctgtttgttttctcaggagtccatcctatttttgacctagttagtgaggtggtgtttgatgattcactttttcttgtcaaagaatcattattattcaaaatttgttccaatagtcttacatttcctctgtgacacgacacttccatattttctttttcttccaaaagattttccctctttgatagttcatcatcccttgaaacaggtacaggagcaaatctgcgaggtgctggtgtctccaaaggagatttctgtttatcaaaactcgtatcttcaacttcttttaaaggtgcttgtttggaagcaaatgtgttatataaagatggattacagctaccaagattagggtgttctggttttacggaatacttttccactgctctggaggagggcatactaacaggctgaaaactactagtcttgagtgcagcactaataaaatgagtctgaatatctatttgttgttgttgtaacttttcaagatgccttatgtgctgctccataaacacattcatttgcttttcgtgatcatgacaatgtaatttctcttgtttcctctgaatgcttgtttgctgctctgtaacacgttgcaggtgtttatcagtctcctgtaatttactaagtaattctgtaacagaattgacttttgcttccaaatcactctgcacctttatcaacggagctgcggttgcaatggcagcagcagttgctgcagccacggttgtagctgaatcaattccactgggtgaaattctagtctcctgagtaacagcatccttctctatgcctgcatcttctaacagatgtacctttacttccttaaaaacaggcatgctttgagctctgtagtcccagctactcgggaggctgaggtgggaggatctcatgagcctgaggaggtagagactgcagtgagttgtgatcaccccactgtgatcactccagcctgtgagacaaagtgagacattttgctttaaaactgttcttagagcatctttctgtcccattgtatactgagaaatgaagatgtcatttgctttttgcttgttgttctcttctattttatccaaaggcaacacttgcactgcaacgtctttagaaaaatcactttctgacaccatgggattttctaatagaggctggtaacaatttctagcagaagttaagtctgatgaaccacgtgatgttccattcaaactagtccccgttccaacaggaagacgtttatttgcagacaatgccggaggaacacagggcaactcatctttcagcaaaaccaaatgatctccatgattttgagaaactacctcacgaagtctcttcactggcatcttaatcttttttttcttctccaagctgacctcagagcctttcatattgttggtcacaaaacaagtcccacaccaaaacatccaaccagaaagctaagcgctctctggtgctcttccattcctctccgggtggaaacaaactccggacataacaggggtttatttatttatttattttaaggtagcacattgccgcacaagaccgctctacagtctcatccaagacttgaagagctcccgacttgtaatactacttgtgtttaccagggactgttgacactgcttcgcttccgaagaccgttagggacgt

SEQ ID NO: 14748 - RNA, 7935 nt, Homo sapiens
  source 1..7935: mol_type = other RNA
gctgggattacaggcatgagccaccgtgtccagtcacagcccagcaatagtaacagccttgatcttgatagtctcttaatagcatgtctcataaatagtttattccggaagttggaaattgtaaaatttaatataaaataaaaattttaaagcttataaaatcaaaagttccatttagtttgtttttacgtacatcgtcttattccaaaagaatctgaagtggttggcagaggaatgtgtacaggagtaaccatgaacagaaataatcctataaaacaaaatactagatgaatgccgggcgcggtggctcacgcctgtaatcccagcactttgggaggctgaggcaggcagatcacctgaggtcgggagttcaggactagcctgaccaacacggagaaaccccatctctactaaaaatacaaaatttgccgggcatggtggcgcacgcctgtaatcccagctactaaggaggctaaggcaggagaatcgcttgaaaccaggaggcagaggttgcggtgagccaagattgtgccattgcactccagcctgggcaacgagcaaaattccatctcaaaaaaaaaaaaaagaaaccgtcgaatggacactaattttttttaaaagaaaagctcacgtgcacagggagtagaataaatcaaagattacacttctaccctaaagttagaaaaggcaggctttctatggttaggaggaaaaatctaccaacacctttaaataaaaaatgctttaactaaaacaagattttgctgaaatccttccaaggcagaaaaaactatgaaaaccagaaaccaaggttggggggtggggtgtcatgtttaaaatgaagcagcactaagcaacatttctccagctttcaccttgcccagagtcttgtagatgaatatcaaaaacaaattaaaatccacagagcagaatttttcttccacttgtttaaaggaaactgttataagcagaactgtccaaagggccatatcaaagaaaacgggttctaaagtgaaacctaaaacattccagtaaccaaatacctgagagaagctgtgaggaagtgcatgtggaaggctgacacatttctgagtttccatagactcttgcagcttctatgttcagtgagaaaaaaaatccccaggcaatggctcctactagaagtttaaggaattctaaattgctcttcagtaattctcagccttgagtgcccattaaaattacctgaaaaggtctttttttttttttaataccaatgctggaccccatccaagatcaattaaattgaaatcccttggtacaaggcccaggcattagtattttttaaagctcccagaggttctaatgtgctgccagtgctgagatccacttagcaacctacaaaaatgctgaaaaagtcaaggatgactgtaattactgtgtgtttgaaattcagttgtgacagaaaatgatttttctgggaggtaaatttttttcactagtgctaggctgcctttcttttcatgtgcttatgccctctactatacagtactgaaatccctcaagataataagaacaacaccatttattgagcacttacatggtatcaagcactgtgctgggcactacccacccccatctccacacacaatcactgatgtccattattctgcaaaaataagtattaaacccattaatctgaaacagctgataagaaggcgtttcgttggcccctatcacaaagcaagaagttacagaattgggattagaacctacatgtatctgattacgaagcaatgctttttattttcctttaattttatgtatttatgttgcaaaaggtaatagagttacatgtttcacaggtttataaaggtttatatggtatacataaggcatataaaaattaatctcactgatgatttttttctatcacaactgaagttcaaatacatagtaaccacgattatccttgattcctatcacttagcctctcctatcacccagccaacaattctactccctggagacaaacttagcagtttcttgtttatataatatatttacaagcaaatacatgtaagaatatgtgacataccatacatttgaattcctccccaccccattttaaataatttcaacaactgcatagttcacacactattttgcacatggcttttttcactttaacagtgcatctcaaagattattccatatcaataaactttttaaatttttttttgtaatacatagtattccattgtactgatgtaccatcactttaaaaccagtctattattgatagacatttgattttttctatttgctgttataaaaatgttagaatgaataaccttgagctacataattttataaatacatacagataattacacctatagattaaatgcctagatgtcaaaagccatgccctttcactactctatgctatctcaggattctaagaaacaactcacaatcagacttataatgacttatacttattttatttaaaaactttaaatacccaaattatgctttttgttttattttaaaatattggaatttttttttcagaatatgctcaaaaaccaaacagtctgagagagggttttaagccaaggtaaaatgactttaaaaccagtggcataaacactgtgctggctgtctcttcccgttcagaaggtatctgcccccgaagactccatgtcctcctgcattgtgctgagactcagagactgagagcagtcctcgaggttcactgacggcagcatcactgacatcttggcagggggcatctgtgaagcggagagtggcactgctttcccacctgggtgatgaaataatctgtatgacaaacctccacagcccgagtttacctatacaggaaaccttcttcacatgtacccccaaacctgaaaatacacatgtgaggtacggattaagctcaatttgtgtccgatccatatcacctggtgaaacttgttgctgtgaaggtgcaatatcagatttatttctaacacgtaggtaactttgtgatggtttgtgttcaacttgcttaacatcctgattttgctttagttggtactgggaaaaatcttcagcggctactggtaaattaacatcattttcttgtgctgtcagaagtgttgtgggaagaaccagcttagaatttggctccaactccaattctcccaaactcattggaccatgactagcacatgaatcttcataaatactacctgaaactgtgtcaaattgccgagataatggtttaggatcacattgttgatccaaagactgtgtattagtgacaggtggctgcatatagagagaatgtcccattaagatgttctctgctgccgctgttagctggggtctttgtccttcactaagttcacccacactgttttccaagtcctctgaatgatagactgcttgctgggaaactgctgactcctggttttgtttagcaaaagaaagaattgcatctgcatgaaattttttatgggacatcctaatcacttgcccttcactaggaggatcatcctccatttcaacggcatcatgcagagtgctggataagctatcattaaggtttgtcaggtacagtcctatatcttctaaaatcttgggggccaatttttgaccacagctaaataaaatctctccttcagagatgggtttatctaaagtttcagtttcagtgacagtaacactcaatgtgctctccagtgttgatgaatcagaacctggcatctgtgagggggaaggggccttggtgccggcaggaaatggcataaagggaactggctctggaggtggaggctgagcagggaaatccatactctctggttcttcatccttagccacagacattacaatagctcttggatgaagttcttcttgaggtgagttagggttctcttcttccagtggcaggtctccatcaccccatggcttgggaagctctgggcttgataccttcaatttatcaatggaaatatctgacaaagttggggtaaaaactgccgccgctggaggaggtgtagtagtaggggtaactgttggagtattaacaagcatgatggcaggcatatcatctcctttttcagcacatatttctttcacaggaaaagccatatcatgatccgaatcacagggagaagaatctggagtctttaccaaaacacactccttagcaggtgatgaaggtgagcaaggaggcgtaggctgtggggtaggcagtggggtgcacactcttgccggcaaatatgtttcatttgttgaagcatccccagaaacacctgtagcaacaggaccttgcttctttgcttctctgtcacccagcatgacagcaatggtctcagcaagagcttcgttaacaaaatgtttaatcacatttgagttcacaggaacaccagcatcaacaaaaagctggagggcgccactgcttgttccttccacaatgtcagaagtcagtggttcacttgtctcactgactgaaacactgatactaggtgcaatctgttgctggactggaaagagcccagagataattcttgacattatttcttgctctacccattgaattaagctattttccagtgtttcttttctctcaattactttatccagaatatcagcagtgggctgaaaagtagaagcaactggcggaaatggaggaccattatattttgtagaatcagctttaacacttctgttaaactccagaattggttcagagtctggaatttcatcacatttttcttcttcctgtatgacatcgattatttcatcaaagttagttcctggaaacttcacctcttcttcatctaccttcataatttctggagtctttatccaagtttgcacaggaggaagagatgcttctttggggctagacagaggtgaaaggacatcagcactactatttgaaatgctgtcaatatctacactgggtaatacctgcacagtaagctgaggaggatcctttttttctgacttcatttctacaatggctatgttaggtttctttactccagtttctacttttcgagatgatggaggaatagaagtagtcacagttacagggtgtggcttgctgacaatcactccagcaggtggcatggtatcactattactttgggtttgtcctaaaagaattgccataggaatcagatgaccttccaatgtacctgaaaaagtaggcatttctctacttgggctgaacaaatattgctgatcgccatgaggtaacacaggaacagaatgtttcattttagaatccatcttcttaggttttgttgcatagaagtcagtctgtgttcttattgactttaccttagtgcctttaactcgttctattacttttggtctctgtggtctggacttaggagatggagaattaaatctgagatatggtccttttttaagagtgcttcgatggccctgataaactggctttccatagacttgtaacatataatcttcatcttgtattactgtggttgctttcaaaagcccttcctttctctctttctgtaaacttgaagcaggcatgcccctcataggtagatttctaaaatgctcttctatttgcttttgagaatgttttcttggaattacagatttgttgacagttttatcttgtgtgttggttctaatatctttagtcatattctgacctttcttggttctctgattcttctgatcaaatcttttttgttcataatctgttcttgacagttcatcctgaatttctgcagaaatagttttaatccattcatccactgtctttctgatcctaattttctctgacatctctctgttggtagataaagcattgataagcgaatacatggcagctccatcttttgcacgaataatagcttccaggttttcttcaagtacttttttattgttttgtactcctctcaaaatcttctcagcatctttcaatacagatcttgttgtattggttgtttgaagcttaacagaattctgtggaagatctggaagcttcaacatactcagagattcttttggctggaccatgctatttgtttctttctctttttggccaaggtcatgaagaacatcatcagacttctgcatagtcactttagttgtttctagctcttcacaggaaggaaatctgtttgttttctcaggagtccatcctatttttgacctagttagtgaggtggtgtttgatgattcactttttcttgtcaaagaatcattattattcaaaatttgttccaatagtcttacatttcctctgtgacacgacacttccatattttctttttcttccaaaagattttccctctttgatagttcatcatcccttgaaacaggtacaggagcaaatctgcgaggtgctggtgtctccaaaggagatttctgtttatcaaaactcgtatcttcaacttcttttaaaggtgcttgtttggaagcaaatgtgttatataaagatggattacagctaccaagattagggtgttctggttttacggaatacttttccactgctctggaggagggcatactaacaggctgaaaactactagtcttgagtgcagcactaataaaatgagtctgaatatctatttgttgttgttgtaacttttcaagatgccttatgtgctgctccataaacacattcatttgcttttcgtgatcatgacaatgtaatttctcttgtttcctctgaatgcttgtttgctgctctgtaacacgttgcaggtgtttatcagtctcctgtaatttactaagtaattctgtaacagaattgacttttgcttccaaatcactctgcacctttatcaacggagctgcggttgcaatggcagcagcagttgctgcagccacggttgtagctgaatcaattccactgggtgaaattctagtctcctgagtaacagcatccttctctatgcctgcatcttctaacagatgtacctttacttccttaaaaacaggcatgctttgagctttttgctttaaaactgttcttagagcatctttctgtcccattgtatactgagaaatgaagatgtcatttgctttttgcttgttgttctcttctattttatccaaaggcaacacttgcactgcaacgtctttagaaaaatcactttctgacaccatgggattttctaatagaggctggtaacaatttctagcagaagttaagtctgatgaaccacgtgatgttccattcaaactagtccccgttccaacaggaagacgtttatttgcagacaatgccggaggaacacagggcaactcatctttcagcaaaaccaaatgatctccatgattttgagaaactacctcacgaagtctcttcactggcatcttaatcttttttttcttctccaagctgacctcagagcctttcatattgttggtcacaaaacaagtcccacacttaaggacggaaaaactttctctgtttccttaagacttcagaacaaaattttcacctctttgcaataactgtttttaaaatgtcgaacatccacaaagctgaaaatctaaattctgatattgaatccaggattagagctgactataaagtcatatttacccattaatcccactcagtctattaatacaccacgccaaaatgtgaaagtggggatgacaagagaatggccacaggagcaacaataaccataacagtgcactccccaaccccagagctggtagggcaaaaccaaacacatgtagtggcgggcttaaaatttgttgagaagaggcagtcaagcaaataaaagcgaaatgctatttttaaaataatgacccacataagaagcgtaatagctttcttcagccacagagtcttacacacccctccagatgcaatcgtcggaaacataaattcacccctacgtatctccagaacgcccgagacccgcaccgtcgtgggtgtaatctgacaacagc

SEQ ID NO: 14749 - RNA, 7784 nt, Homo sapiens
  source 1..7784: mol_type = other RNA
gctgggattacaggcatgagccaccgtgtccagtcacagcccagcaatagtaacagccttgatcttgatagtctcttaatagcatgtctcataaatagtttattccggaagttggaaattgtaaaatttaatataaaataaaaattttaaagcttataaaatcaaaagttccatttagtttgtttttacgtacatcgtcttattccaaaagaatctgaagtggttggcagaggaatgtgtacaggagtaaccatgaacagaaataatcctataaaacaaaatactagatgaatgccgggcgcggtggctcacgcctgtaatcccagcactttgggaggctgaggcaggcagatcacctgaggtcgggagttcaggactagcctgaccaacacggagaaaccccatctctactaaaaatacaaaatttgccgggcatggtggcgcacgcctgtaatcccagctactaaggaggctaaggcaggagaatcgcttgaaaccaggaggcagaggttgcggtgagccaagattgtgccattgcactccagcctgggcaacgagcaaaattccatctcaaaaaaaaaaaaaagaaaccgtcgaatggacactaattttttttaaaagaaaagctcacgtgcacagggagtagaataaatcaaagattacacttctaccctaaagttagaaaaggcaggctttctatggttaggaggaaaaatctaccaacacctttaaataaaaaatgctttaactaaaacaagattttgctgaaatccttccaaggcagaaaaaactatgaaaaccagaaaccaaggttggggggtggggtgtcatgtttaaaatgaagcagcactaagcaacatttctccagctttcaccttgcccagagtcttgtagatgaatatcaaaaacaaattaaaatccacagagcagaatttttcttccacttgtttaaaggaaactgttataagcagaactgtccaaagggccatatcaaagaaaacgggttctaaagtgaaacctaaaacattccagtaaccaaatacctgagagaagctgtgaggaagtgcatgtggaaggctgacacatttctgagtttccatagactcttgcagcttctatgttcagtgagaaaaaaaatccccaggcaatggctcctactagaagtttaaggaattctaaattgctcttcagtaattctcagccttgagtgcccattaaaattacctgaaaaggtctttttttttttttaataccaatgctggaccccatccaagatcaattaaattgaaatcccttggtacaaggcccaggcattagtattttttaaagctcccagaggttctaatgtgctgccagtgctgagatccacttagcaacctacaaaaatgctgaaaaagtcaaggatgactgtaattactgtgtgtttgaaattcagttgtgacagaaaatgatttttctgggaggtaaatttttttcactagtgctaggctgcctttcttttcatgtgcttatgccctctactatacagtactgaaatccctcaagataataagaacaacaccatttattgagcacttacatggtatcaagcactgtgctgggcactacccacccccatctccacacacaatcactgatgtccattattctgcaaaaataagtattaaacccattaatctgaaacagctgataagaaggcgtttcgttggcccctatcacaaagcaagaagttacagaattgggattagaacctacatgtatctgattacgaagcaatgctttttattttcctttaattttatgtatttatgttgcaaaaggtaatagagttacatgtttcacaggtttataaaggtttatatggtatacataaggcatataaaaattaatctcactgatgatttttttctatcacaactgaagttcaaatacatagtaaccacgattatccttgattcctatcacttagcctctcctatcacccagccaacaattctactccctggagacaaacttagcagtttcttgtttatataatatatttacaagcaaatacatgtaagaatatgtgacataccatacatttgaattcctccccaccccattttaaataatttcaacaactgcatagttcacacactattttgcacatggcttttttcactttaacagtgcatctcaaagattattccatatcaataaactttttaaatttttttttgtaatacatagtattccattgtactgatgtaccatcactttaaaaccagtctattattgatagacatttgattttttctatttgctgttataaaaatgttagaatgaataaccttgagctacataattttataaatacatacagataattacacctatagattaaatgcctagatgtcaaaagccatgccctttcactactctatgctatctcaggattctaagaaacaactcacaatcagacttataatgacttatacttattttatttaaaaactttaaatacccaaattatgctttttgttttattttaaaatattggaatttttttttcagaatatgctcaaaaaccaaacagtctgagagagggttttaagccaaggtaaaatgactttaaaaccagtggcataaacactgtgctggctgtctcttcccgttcagaaggtatctgcccccgaagactccatgtcctcctgcattgtgctgagactcagagactgagagcagtcctcgaggttcactgacggcagcatcactgacatcttggcagggggcatctgtgaagcggagagtggcactgctttcccaccttgttgctgtgaaggtgcaatatcagatttatttctaacacgtaggtaactttgtgatggtttgtgttcaacttgcttaacatcctgattttgctttagttggtactgggaaaaatcttcagcggctactggtaaattaacatcattttcttgtgctgtcagaagtgttgtgggaagaaccagcttagaatttggctccaactccaattctcccaaactcattggaccatgactagcacatgaatcttcataaatactacctgaaactgtgtcaaattgccgagataatggtttaggatcacattgttgatccaaagactgtgtattagtgacaggtggctgcatatagagagaatgtcccattaagatgttctctgctgccgctgttagctggggtctttgtccttcactaagttcacccacactgttttccaagtcctctgaatgatagactgcttgctgggaaactgctgactcctggttttgtttagcaaaagaaagaattgcatctgcatgaaattttttatgggacatcctaatcacttgcccttcactaggaggatcatcctccatttcaacggcatcatgcagagtgctggataagctatcattaaggtttgtcaggtacagtcctatatcttctaaaatcttgggggccaatttttgaccacagctaaataaaatctctccttcagagatgggtttatctaaagtttcagtttcagtgacagtaacactcaatgtgctctccagtgttgatgaatcagaacctggcatctgtgagggggaaggggccttggtgccggcaggaaatggcataaagggaactggctctggaggtggaggctgagcagggaaatccatactctctggttcttcatccttagccacagacattacaatagctcttggatgaagttcttcttgaggtgagttagggttctcttcttccagtggcaggtctccatcaccccatggcttgggaagctctgggcttgataccttcaatttatcaatggaaatatctgacaaagttggggtaaaaactgccgccgctggaggaggtgtagtagtaggggtaactgttggagtattaacaagcatgatggcaggcatatcatctcctttttcagcacatatttctttcacaggaaaagccatatcatgatccgaatcacagggagaagaatctggagtctttaccaaaacacactccttagcaggtgatgaaggtgagcaaggaggcgtaggctgtggggtaggcagtggggtgcacactcttgccggcaaatatgtttcatttgttgaagcatccccagaaacacctgtagcaacaggaccttgcttctttgcttctctgtcacccagcatgacagcaatggtctcagcaagagcttcgttaacaaaatgtttaatcacatttgagttcacaggaacaccagcatcaacaaaaagctggagggcgccactgcttgttccttccacaatgtcagaagtcagtggttcacttgtctcactgactgaaacactgatactaggtgcaatctgttgctggactggaaagagcccagagataattcttgacattatttcttgctctacccattgaattaagctattttccagtgtttcttttctctcaattactttatccagaatatcagcagtgggctgaaaagtagaagcaactggcggaaatggaggaccattatattttgtagaatcagctttaacacttctgttaaactccagaattggttcagagtctggaatttcatcacatttttcttcttcctgtatgacatcgattatttcatcaaagttagttcctggaaacttcacctcttcttcatctaccttcataatttctggagtctttatccaagtttgcacaggaggaagagatgcttctttggggctagacagaggtgaaaggacatcagcactactatttgaaatgctgtcaatatctacactgggtaatacctgcacagtaagctgaggaggatcctttttttctgacttcatttctacaatggctatgttaggtttctttactccagtttctacttttcgagatgatggaggaatagaagtagtcacagttacagggtgtggcttgctgacaatcactccagcaggtggcatggtatcactattactttgggtttgtcctaaaagaattgccataggaatcagatgaccttccaatgtacctgaaaaagtaggcatttctctacttgggctgaacaaatattgctgatcgccatgaggtaacacaggaacagaatgtttcattttagaatccatcttcttaggttttgttgcatagaagtcagtctgtgttcttattgactttaccttagtgcctttaactcgttctattacttttggtctctgtggtctggacttaggagatggagaattaaatctgagatatggtccttttttaagagtgcttcgatggccctgataaactggctttccatagacttgtaacatataatcttcatcttgtattactgtggttgctttcaaaagcccttcctttctctctttctgtaaacttgaagcaggcatgcccctcataggtagatttctaaaatgctcttctatttgcttttgagaatgttttcttggaattacagatttgttgacagttttatcttgtgtgttggttctaatatctttagtcatattctgacctttcttggttctctgattcttctgatcaaatcttttttgttcataatctgttcttgacagttcatcctgaatttctgcagaaatagttttaatccattcatccactgtctttctgatcctaattttctctgacatctctctgttggtagataaagcattgataagcgaatacatggcagctccatcttttgcacgaataatagcttccaggttttcttcaagtacttttttattgttttgtactcctctcaaaatcttctcagcatctttcaatacagatcttgttgtattggttgtttgaagcttaacagaattctgtggaagatctggaagcttcaacatactcagagattcttttggctggaccatgctatttgtttctttctctttttggccaaggtcatgaagaacatcatcagacttctgcatagtcactttagttgtttctagctcttcacaggaaggaaatctgtttgttttctcaggagtccatcctatttttgacctagttagtgaggtggtgtttgatgattcactttttcttgtcaaagaatcattattattcaaaatttgttccaatagtcttacatttcctctgtgacacgacacttccatattttctttttcttccaaaagattttccctctttgatagttcatcatcccttgaaacaggtacaggagcaaatctgcgaggtgctggtgtctccaaaggagatttctgtttatcaaaactcgtatcttcaacttcttttaaaggtgcttgtttggaagcaaatgtgttatataaagatggattacagctaccaagattagggtgttctggttttacggaatacttttccactgctctggaggagggcatactaacaggctgaaaactactagtcttgagtgcagcactaataaaatgagtctgaatatctatttgttgttgttgtaacttttcaagatgccttatgtgctgctccataaacacattcatttgcttttcgtgatcatgacaatgtaatttctcttgtttcctctgaatgcttgtttgctgctctgtaacacgttgcaggtgtttatcagtctcctgtaatttactaagtaattctgtaacagaattgacttttgcttccaaatcactctgcacctttatcaacggagctgcggttgcaatggcagcagcagttgctgcagccacggttgtagctgaatcaattccactgggtgaaattctagtctcctgagtaacagcatccttctctatgcctgcatcttctaacagatgtacctttacttccttaaaaacaggcatgctttgagctttttgctttaaaactgttcttagagcatctttctgtcccattgtatactgagaaatgaagatgtcatttgctttttgcttgttgttctcttctattttatccaaaggcaacacttgcactgcaacgtctttagaaaaatcactttctgacaccatgggattttctaatagaggctggtaacaatttctagcagaagttaagtctgatgaaccacgtgatgttccattcaaactagtccccgttccaacaggaagacgtttatttgcagacaatgccggaggaacacagggcaactcatctttcagcaaaaccaaatgatctccatgattttgagaaactacctcacgaagtctcttcactggcatcttaatcttttttttcttctccaagctgacctcagagcctttcatattgttggtcacaaaacaagtcccacacttaaggacggaaaaactttctctgtttccttaagacttcagaacaaaattttcacctctttgcaataactgtttttaaaatgtcgaacatccacaaagctgaaaatctaaattctgatattgaatccaggattagagctgactataaagtcatatttacccattaatcccactcagtctattaatacaccacgccaaaatgtgaaagtggggatgacaagagaatggccacaggagcaacaataaccataacagtgcactccccaaccccagagctggtagggcaaaaccaaacacatgtagtggcgggcttaaaatttgttgagaagaggcagtcaagcaaataaaagcgaaatgctatttttaaaataatgacccacataagaagcgtaatagctttcttcagccacagagtcttacacacccctccagatgcaatcgtcggaaacataaattcacccctacgtatctccagaacgcccgagacccgcaccgtcgtgggtgtaatctgacaacagc

SEQ ID NO: 14750 - RNA, 7134 nt, Homo sapiens
  source 1..7134: mol_type = other RNA
gctgggattacaggcatgagccaccgtgtccagtcacagcccagcaatagtaacagccttgatcttgatagtctcttaatagcatgtctcataaatagtttattccggaagttggaaattgtaaaatttaatataaaataaaaattttaaagcttataaaatcaaaagttccatttagtttgtttttacgtacatcgtcttattccaaaagaatctgaagtggttggcagaggaatgtgtacaggagtaaccatgaacagaaataatcctataaaacaaaatactagatgaatgccgggcgcggtggctcacgcctgtaatcccagcactttgggaggctgaggcaggcagatcacctgaggtcgggagttcaggactagcctgaccaacacggagaaaccccatctctactaaaaatacaaaatttgccgggcatggtggcgcacgcctgtaatcccagctactaaggaggctaaggcaggagaatcgcttgaaaccaggaggcagaggttgcggtgagccaagattgtgccattgcactccagcctgggcaacgagcaaaattccatctcaaaaaaaaaaaaaagaaaccgtcgaatggacactaattttttttaaaagaaaagctcacgtgcacagggagtagaataaatcaaagattacacttctaccctaaagttagaaaaggcaggctttctatggttaggaggaaaaatctaccaacacctttaaataaaaaatgctttaactaaaacaagattttgctgaaatccttccaaggcagaaaaaactatgaaaaccagaaaccaaggttggggggtggggtgtcatgtttaaaatgaagcagcactaagcaacatttctccagctttcaccttgcccagagtcttgtagatgaatatcaaaaacaaattaaaatccacagagcagaatttttcttccacttgtttaaaggaaactgttataagcagaactgtccaaagggccatatcaaagaaaacgggttctaaagtgaaacctaaaacattccagtaaccaaatacctgagagaagctgtgaggaagtgcatgtggaaggctgacacatttctgagtttccatagactcttgcagcttctatgttcagtgagaaaaaaaatccccaggcaatggctcctactagaagtttaaggaattctaaattgctcttcagtaattctcagccttgagtgcccattaaaattacctgaaaaggtctttttttttttttaataccaatgctggaccccatccaagatcaattaaattgaaatcccttggtacaaggcccaggcattagtattttttaaagctcccagaggttctaatgtgctgccagtgctgagatccacttagcaacctacaaaaatgctgaaaaagtcaaggatgactgtaattactgtgtgtttgaaattcagttgtgacagaaaatgatttttctgggaggtaaatttttttcactagtgctaggctgcctttcttttcatgtgcttatgccctctactatacagtactgaaatccctcaagataataagaacaacaccatttattgagcacttacatggtatcaagcactgtgctgggcactacccacccccatctccacacacaatcactgatgtccattattctgcaaaaataagtattaaacccattaatctgaaacagctgataagaaggcgtttcgttggcccctatcacaaagcaagaagttacagaattgggattagaacctacatgtatctgattacgaagcaatgctttttattttcctttaattttatgtatttatgttgcaaaaggtaatagagttacatgtttcacaggtttataaaggtttatatggtatacataaggcatataaaaattaatctcactgatgatttttttctatcacaactgaagttcaaatacatagtaaccacgattatccttgattcctatcacttagcctctcctatcacccagccaacaattctactccctggagacaaacttagcagtttcttgtttatataatatatttacaagcaaatacatgtaagaatatgtgacataccatacatttgaattcctccccaccccattttaaataatttcaacaactgcatagttcacacactattttgcacatggcttttttcactttaacagtgcatctcaaagattattccatatcaataaactttttaaatttttttttgtaatacatagtattccattgtactgatgtaccatcactttaaaaccagtctattattgatagacatttgattttttctatttgctgttataaaaatgttagaatgaataaccttgagctacataattttataaatacatacagataattacacctatagattaaatgcctagatgtcaaaagccatgccctttcactactctatgctatctcaggattctaagaaacaactcacaatcagacttataatgacttatacttattttatttaaaaactttaaatacccaaattatgctttttgttttattttaaaatattggaatttttttttcagaatatgctcaaaaaccaaacagtctgagagagggttttaagccaaggtaaaatgactttaaaaccagtggcataaacactgtgctggctgtctcttcccgttcagaaggtatctgcccccgaagactccatgtcctcctgcattgtgctgagactcagagactgagagcagtcctcgaggttcactgacggcagcatcactgacatcttggcagggggcatctgtgaagcggagagtggcactgctttcccaccttgttgctgtgaaggtgcaatatcagatttatttctaacacgtaggtaactttgtgatggtttgtgttcaacttgcttaacatcctgattttgctttagttggtactgggaaaaatcttcagcggctactggtaaattaacatcattttcttgtgctgtcagaagtgttgtgggaagaaccagcttagaatttggctccaactccaattctcccaaactcattggaccatgactagcacatgaatcttcataaatactacctgaaactgtgtcaaattgccgagataatggtttaggatcacattgttgatccaaagactgtgtattagtgacaggtggctgcatatagagagaatgtcccattaagatgttctctgctgccgctgttagctggggtctttgtccttcactaagttcacccacactgttttccaagtcctctgaatgatagactgcttgctgggaaactgctgactcctggttttgtttagcaaaagaaagaattgcatctgcatgaaattttttatgggacatcctaatcacttgcccttcactaggaggatcatcctccatttcaacggcatcatgcagagtgctggataagctatcattaaggtttgtcaggtacagtcctatatcttctaaaatcttgggggccaatttttgaccacagctaaataaaatctctccttcagagatgggtttatctaaagtttcagtttcagtgacagtaacactcaatgtgctctccagtgttgatgaatcagaacctggcatctgtgagggggaaggggccttggtgccggcaggaaatggcataaagggaactggctctggaggtggaggctgagcagggaaatccatactctctggttcttcatccttagccacagacattacaatagctcttggatgaagttcttcttgaggtgagttagggttctcttcttccagtggcaggtctccatcaccccatggcttgggaagctctgggcttgataccttcaatttatcaatggaaatatctgacaaagttggggtaaaaactgccgccgctggaggaggtgtagtagtaggggtaactgttggagtattaacaagcatgatggcaggcatatcatctcctttttcagcacatatttctttcacaggaaaagccatatcatgatccgaatcacagggagaagaatctggagtctttaccaaaacacactccttagcaggtgatgaaggtgagcaaggaggcgtaggctgtggggtaggcagtggggtgcacactcttgccggcaaatatgtttcatttgttgaagcatccccagaaacacctgtagcaacaggaccttgcttctttgcttctctgtcacccagcatgacagcaatggtctcagcaagagcttcgttaacaaaatgtttaatcacatttgagttcacaggaacaccagcatcaacaaaaagctggagggcgccactgcttgttccttccacaatgtcagaagtcagtggttcacttgtctcactgactgaaacactgatactaggtgcaatctgttgctggactggaaagagcccagagataattcttgacattatttcttgctctacccattgaattaagctattttccagtgtttcttttctctcaattactttatccagaatatcagcagtgggctgaaaagtagaagcaactggcggaaatggaggaccattatattttgtagaatcagctttaacacttctgttaaactccagaattggttcagagtctggaatttcatcacatttttcttcttcctgtatgacatcgattatttcatcaaagttagttcctggaaacttcacctcttcttcatctaccttcataatttctggagtctttatccaagtttgcacaggaggaagagatgcttctttggggctagacagaggtgaaaggacatcagcactactatttgaaatgctgtcaatatctacactgggtaatacctgcacagtaagctgaggaggatcctttttttctgacttcatttctacaatggctatgttaggtttctttactccagtttctacttttcgagatgatggaggaatagaagtagtcacagttacagggtgtggcttgctgacaatcactccagcaggtggcatggtatcactattactttgggtttgtcctaaaagaattgccataggaatcagatgaccttccaatgtacctgaaaaagtaggcatttctctacttgggctgaacaaatattgctgatcgccatgaggtaacacaggaacagaatgtttcattttagaatccatcttcttaggttttgttgcatagaagtcagtctgtgttcttattgactttaccttagtgcctttaactcgttctattacttttggtctctgtggtctggacttaggagatggagaattaaatctgagatatggtccttttttaagagtgcttcgatggccctgataaactggctttccatagacttgtaacatataatcttcatcttgtattactgtggttgctttcaaaagcccttcctttctctctttctgtaaacttgaagcaggcatgcccctcataggtagatttctaaaatgctcttctatttgcttttgagaatgttttcttggaattacagatttgttgacagttttatcttgtgtgttggttctaatatctttagtcatattctgacctttcttggttctctgattcttctgatcaaatcttttttgttcataatctgttcttgacagttcatcctgaatttctgcagaaatagttttaatccattcatccactgtctttctgatcctaattttctctgacatctctctgttggtagataaagcattgataagcgaatacatggcagctccatcttttgcacgaataatagcttccaggttttcttcaagtacttttttattgttttgtactcctctcaaaatcttctcagcatctttcaatacagatcttgttgtattggttgtttgaagcttaacagaattctgtggaagatctggaagcttcaacatactcagagattcttttggctggaccatgctatttgtttctttctctttttggccaaggtcatgaagaacatcatcagacttctgcatagtcactttagttgtttctagctcttcacaggaaggaaatctgtttgttttctcaggagtccatcctatttttgacctagttagtgaggtggtgtttgatgattcactttttcttgtcaaagaatcattattattcaaaatttgttccaatagtcttacatttcctctgtgacacgacacttccatattttctttttcttccaaaagattttccctctttgatagttcatcatcccttgaaacaggtacaggagcaaatctgcgaggtgctggtgtctccaaaggagatttctgtttatcaaaactcgtatcttcaacttcttttaaaggtgcttgtttggaagcaaatgtgttatataaagatggattacagctaccaagattagggtgttctggttttacggaatacttttccactgctctggaggagggcatactaacaggctgaaaactactagtcttgagtgcagcactaataaaatgagtctgaatatctatttgttgttgttgtaacttttcaagatgccttatgtgctgctccataaacacattcatttgcttttcgtgatcatgacaatgtaatttctcttgtttcctctgaatgcttgtttgctgctctgtaacacgttgcaggtgtttatcagtctcctgtaatttactaagtaattctgtaacagaattgacttttgcttccaaatcactctgcacctttatcaacggagctgcggttgcaatggcagcagcagttgctgcagccacggttgtagctgaatcaattccactgggtgaaattctagtctcctgagtaacagcatccttctctatgcctgcatcttctaacagatgtacctttacttccttaaaaacaggcatgctttgagctttttgctttaaaactgttcttagagcatctttctgtcccattgtatactgagaaatgaagatgtcatttgctttttgcttgttgttctcttctattttatccaaaggcaacacttgcactgcaacgtctttagaaaaatcactttctgacaccatgggattttctaatagaggctggtaacaatttctagcagaagttaagtctgatgaacccctccagatgcaatcgtcggaaacataaattcacccctacgtatctccagaacgcccgagacccgcaccgtcgtgggtgtaatctgacaacagc

SEQ ID NO: 14751 - RNA, 3167 nt, Homo sapiens
  source 1..3167: mol_type = other RNA
gctgggattacaggcatgagccaccgtgtccggcaacactcttaatatgagtgacttcaaagcttttgaagcctctatccccgctggcagtggtgtgcccctgggctctccctagactaggctaaagcccctgccaaccactctcccagcaccctgcacttaccttttcatgacacccatcacttttagacttacaggttgaattgctgccttccttgctaggctgtaagttccccgatggacataactgcatctgcctggtgtgctgttgtttccctggtgtctgaacagagtcaggctcctgacaggcccccgctatttggagctgagtcaataggatgtgcaaactgagggagaggaaagggtggaggaaaactcgcagacctcagaggcctggggagaggaaaagtgtcttgctcaagtcacatactaggcaggaagagatcatggttcctgctcagaatctttgactctcagtcagggcctttcccactcactatactgtgctagaaagaggctacgaaacccacagaaaagtgttctatagttaaataagcttgaaaaactctggattaaacaaaatgaaaggagtttctttgccactggtcttttcagggcctttaacatgctcctgtgcccgtgcttctggaagaaggtcacacacagtactccatgctctctgaccctggaactctgcctgtgaggcggtctgaaacctccagcaccaccccccagctatgtgtcacaattatttattaaatgtgacacagcagagagatttgttgccattttttttagtggctaggaaaatccttttgtacaaataaaaataattcaaaaccccaatatatgaatgggataaaaatgcagctgctctggttgaagggggtactggggatccatctggagctgtcctttcactgctgctatgcaaagaacccttgcttcctgtagagcgcagttcgaaaatcactgatgcagaattggcacatgaggttgaagctaggaggcttctagtgctggctctgccatggactgttttaccctgggcaagtcatttagtctcactgggcttcagtttcccgtgtatacgataagtctgtcacactgtatgtttcttagagtcctgaactttcagctttgatatggtgaagagtacatttctatgactataaaagtctaactctaagattccatggcttaatattccaattctgggactgcctgtagctagcccaagctggtgcagcacgctagagcccaggctgttgaaggcagaattcattaactgcagtgcgctgcccaggggcactgggttcctgggataggggtgccaggttcctggggtgggtggaccgtgatcggcagccgctcagtgggacaagctgggagagggacccaggtctcctgactcctgctctatctttagatctccatagcaaccatcaccagggcaccaagctgaaggcacaggctgagtggctgcctgcaggaggagggaggggcgtttccttcccgtgcctcttcttttgctaggctcgatttttgagccaggaaaggggactgagaatgaagctgttcacagcaagaaaggcttggggccaatacaagacagtcgagggccccaccttgctctcaggatgtggtcaagtcatagaacccaagaccttcatgtgtcaggctcatggcactggaggaaaggcagaatcctcctccaaagagctctaagcctctcccgtgtccttccctacacactcaggagcccctaatccgagatggtgctgaggccacagttggagcccccattagatcctctaatcggaggggccagggaagctcctcccgactcttcccctgcccaactcctactcctcctggggctcagcctggacttggcttcctctgaagagtcctccctgactcccaggctggttgctcacctcctcagggcccctacagcccatcctccttctacatagtaggaggccaggaggagtgattaacctcatggggcagatgagaagtagaggttctgagcagtaaagacacttgcccaaggtcacctggcaaatgagcagcaggaccaggcctggactccgtgtcttctgattccagtctgtgctccttcctgggtcccagtagcaggctcatggcctaggctttggaagagaggccagggctagaagaggaaataggagtcctcagtgaggcctgcgcacagtaagcacctggctatgtctttggtgaactcagccgagccacagaccagtgcgaatggctttctccgacagcagctgaccagctctttaattaggtcctggcccaggtggccaaagtgggttttctcttggtaactccagggaagctgctctgaggagctctcctggctgagtacaaagaaggtacggacattccagaaacgggcctgctcttggaggaaggttttcaggtagatgctctcaaaggtcttgaagcaaccgaccagagtgacaaaagtctcgtcattctcattgtctgtgatgctctgcaggataggcaccatgggggccaggcccgtgcccgcagccagcaagaggagctcaccatactggtttggtttatagaagaaatctccgaaaggtcctcgccagaaagctgtgtctcctactctccaggactcaacataccgggacatcagccccatctggtagcactgtgactctggcccacgcagcaggctcctgtccttgctggcttgggctgcctcccaccttgccagatctcggtgatagaggtcaaacacacagggtgagcagccactgccgcagcactgggaaggcaagggttctgtgggccgtagctgcatccaggcttcctcagtgtcgtcgtcctcttccctctcagccatcatcagtggggcttgggcagcctagaaggaacaactgggtgctcttccagaacaggccaggctctatgagaccacgggcgcaggccctgctccttggccagcattttgtagagacagggtctcactatgttgccagtctggtctcgaactcctggcctcaagtgatcttctcatctcagtctcccaaagtgctgagattacaggcatgagccaccatgtctggccctactcgcctgcgcttcacctcacgtgaggattttccaggttcctcccagtctct

SEQ ID NO: 14752 - RNA, 3404 nt, Homo sapiens
  source 1..3404: mol_type = other RNA
gctgggattacaggcatgagccaccgtgtccggcaacactcttaatatgagtgacttcaaagcttttgaagcctctatccccgctggcagtggtgtgcccctgggctctccctagactaggctaaagcccctgccaaccactctcccagcaccctgcacttaccttttcatgacacccatcacttttagacttacaggttgaattgctgccttccttgctaggctgtaagttccccgatggacataactgcatctgcctggtgtgctgttgtttccctggtgtctgaacagagtcaggctcctgacaggcccccgctatttggagctgagtcaataggatgtgcaaactgagggagaggaaagggtggaggaaaactcgcagacctcagaggcctggggagaggaaaagtgtcttgctcaagtcacatactaggcaggaagagatcatggttcctgctcagaatctttgactctcagtcagggcctttcccactcactatactgtgctagaaagaggctacgaaacccacagaaaagtgttctatagttaaataagcttgaaaaactctggattaaacaaaatgaaaggagtttctttgccactggtcttttcagggcctttaacatgctcctgtgcccgtgcttctggaagaaggtcacacacagtactccatgctctctgaccctggaactctgcctgtgaggcggtctgaaacctccagcaccaccccccagctatgtgtcacaattatttattaaatgtgacacagcagagagatttgttgccattttttttagtggctaggaaaatccttttgtacaaataaaaataattcaaaaccccaatatatgaatgggataaaaatgcagctgctctggttgaagggggtactggggatccatctggagctgtcctttcactgctgctatgcaaagaacccttgcttcctgtagagcgcagttcgaaaatcactgatgcagaattggcacatgaggttgaagctaggaggcttctagtgctggctctgccatggactgttttaccctgggcaagtcatttagtctcactgggcttcagtttcccgtgtatacgataagtctgtcacactgtatgtttcttagagtcctgaactttcagctttgatatggtgaagagtacatttctatgactataaaagtctaactctaagattccatggcttaatattccaattctgggactgcctgtagctagcccaagctggtgcagcacgctagagcccaggctgttgaaggcagaattcattaactgcagtgcgctgcccaggggcactgggttcctgggataggggtgccaggttcctggggtgggtggaccgtgatcggcagccgctcagtgggacaagctgggagagggacccaggtctcctgactcctgctctatctttagatctccatagcaaccatcaccagggcaccaagctgaaggcacaggctgagtggctgcctgcaggaggagggaggggcgtttccttcccgtgcctcttcttttgctaggctcgatttttgagccaggaaaggggactgagaatgaagctgttcacagcaagaaaggcttggggccaatacaagacagtcgagggccccaccttgctctcaggatgtggtcaagtcatagaacccaagaccttcatgtgtcaggctcatggcactggaggaaaggcagaatcctcctccaaagagctctaagcctctcccgtgtccttccctacacactcaggagcccctaatccgagatggtgctgaggccacagttggagcccccattagatcctctaatcggaggggccagggaagctcctcccgactcttcccctgcccaactcctactcctcctggggctcagcctggacttggcttcctctgaagagtcctccctgactcccaggctggttgctcacctcctcagggcccctacagcccatcctccttctacatagtaggaggccaggaggagtgattaacctcatggggcagatgagaagtagaggttctgagcagtaaagacacttgcccaaggtcacctggcaaatgagcagcaggaccaggcctggactccgtgtcttctgattccagtctgtgctccttcctgggtcccagtagcaggctcatggcctaggctttggaagagaggccagggctagaagaggaaataggagtcctcagtgaggcctgcgcacagtaagcacctggctatgtctttggtgaactcagccgagccacagaccagtgcgaatggctttctccgacagcagctgaccagctctttaattaggtcctggcccaggtggccaaagtgggttttctcttggtaactccagggaagctgctctgaggagctctcctggctgagtacaaagaaggtacggacattccagaaacgggcctgctcttggaggaaggttttcaggtagatgctctcaaaggtcttgaagcaaccgaccagagtgacaaaagtctcgtcattctcattgtctgtgatgctctgcaggataggcaccatgggggccaggcccgtgcccgcagccagcaagaggagctcaccatactggtttggtttatagaagaaatctccgaaaggtcctcgccagaaagctgtgtctcctactctccaggactcaacataccgggacatcagccccatctggtagcacttaattaacacttcaaagtatccttctgcgttggcagggctgatgggcgtataggctctctgaatttctaagtcatctactatccctcgtaggatgaggtgctggccgggccgcaggccaagctggctgttcccgggtagagcaaaccggacacggtaggtgtccttagtgagcctgtccatggcaatgatgcagaaggccacgaaggtctctgggttcagcttggaggggcagctctgtgactctggcccacgcagcaggctcctgtccttgctggcttgggctgcctcccaccttgccagatctcggtgatagaggtcaaacacacagggtgagcagccactgccgcagcactgggaaggcaagggttctgtgggccgtagctgcatccaggcttcctcagtgtcgtcgtcctcttccctctcagccatcatcagtggggcttgggcagcctagaaggaacaactgggtgctcttccagaacaggccaggctctatgagaccacgggcgcaggccctgctccttggccagcattttgtagagacagggtctcactatgttgccagtctggtctcgaactcctggcctcaagtgatcttctcatctcagtctcccaaagtgctgagattacaggcatgagccaccatgtctggccctactcgcctgcgcttcacctcacgtgaggattttccaggttcctcccagtctct

SEQ ID NO: 14753 - RNA, 3255 nt, Homo sapiens
  source 1..3255: mol_type = other RNA
gctgggattacaggcatgagccaccgtgtccggcaacactcttaatatgagtgacttcaaagcttttgaagcctctatccccgctggcagtggtgtgcccctgggctctccctagactaggctaaagcccctgccaaccactctcccagcaccctgcacttaccttttcatgacacccatcacttttagacttacaggttgaattgctgccttccttgctaggctgtaagttccccgatggacataactgcatctgcctggtgtgctgttgtttccctggtgtctgaacagagtcaggctcctgacaggcccccgctatttggagctgagtcaataggatgtgcaaactgagggagaggaaagggtggaggaaaactcgcagacctcagaggcctggggagaggaaaagtgtcttgctcaagtcacatactaggcaggaagagatcatggttcctgctcagaatctttgactctcagtcagggcctttcccactcactatactgtgctagaaagaggctacgaaacccacagaaaagtgttctatagttaaataagcttgaaaaactctggattaaacaaaatgaaaggagtttctttgccactggtcttttcagggcctttaacatgctcctgtgcccgtgcttctggaagaaggtcacacacagtactccatgctctctgaccctggaactctgcctgtgaggcggtctgaaacctccagcaccaccccccagctatgtgtcacaattatttattaaatgtgacacagcagagagatttgttgccattttttttagtggctaggaaaatccttttgtacaaataaaaataattcaaaaccccaatatatgaatgggataaaaatgcagctgctctggttgaagggggtactggggatccatctggagctgtcctttcactgctgctatgcaaagaacccttgcttcctgtagagcgcagttcgaaaatcactgatgcagaattggcacatgaggttgaagctaggaggcttctagtgctggctctgccatggactgttttaccctgggcaagtcatttagtctcactgggcttcagtttcccgtgtatacgataagtctgtcacactgtatgtttcttagagtcctgaactttcagctttgatatggtgaagagtacatttctatgactataaaagtctaactctaagattccatggcttaatattccaattctgggactgcctgtagctagcccaagctggtgcagcacgctagagcccaggctgttgaaggcagaattcattaactgcagtgcgctgcccaggggcactgggttcctgggataggggtgccaggttcctggggtgggtggaccgtgatcggcagccgctcagtgggacaagctgggagagggacccaggtctcctgactcctgctctatctttagatctccatagcaaccatcaccagggcaccaagctgaaggcacaggctgagtggctgcctgcaggaggagggaggggcgtttccttcccgtgcctcttcttttgctaggctcgatttttgagccaggaaaggggactgagaatgaagctgttcacagcaagaaaggcttggggccaatacaagacagtcgagggccccaccttgctctcaggatgtggtcaagtcatagaacccaagaccttcatgtgtcaggctcatggcactggaggaaaggcagaatcctcctccaaagagctctaagcctctcccgtgtccttccctacacactcaggagcccctaatccgagatggtgctgaggccacagttggagcccccattagatcctctaatcggaggggccagggaagctcctcccgactcttcccctgcccaactcctactcctcctggggctcagcctggacttggcttcctctgaagagtcctccctgactcccaggctggttgctcacctcctcagggcccctacagcccatcctccttctacatagtaggaggccaggaggagtgattaacctcatggggcagatgagaagtagaggttctgagcagtaaagacacttgcccaaggtcacctggcaaatgagcagcaggaccaggcctggactccgtgtcttctgattccagtctgtgctccttcctgggtcccagtagcaggctcatggcctaggctttggaagagaggccagggctagaagaggaaataggagtcctcagtgaggcctgcgcacagtaagcacctggctatgtctttggtgaactcagccgagccacagaccagtgcgaatggctttctccgacagcagctgaccagctctttaattaggtcctggcccaggtggccaaagtgggttttctcttggtaactccagggaagctgctctgaggagctctcctggctgagtacaaagaaggtacggacattccagaaacgggcctgctcttggaggaaggttttcaggtagatgctctcaaaggtcttgaagcaaccgaccagagtgacaaaagtctcgtcattctcattgtctgtgatgctctgcaggataggcaccatgggggccaggcccgtgcccgcagccagcaagaggagctcaccatactggtttggtttatagaagaaatctccgaaaggtcctcgccagaaagctgtgtctcctactctccaggactcaacataccgggacatcagccccatctggtagcacttaattaacacttcaaagtatccttctgcgttggcagggctgatgggcgtataggctctctgaatttctaagtcatctactatccctctgtgactctggcccacgcagcaggctcctgtccttgctggcttgggctgcctcccaccttgccagatctcggtgatagaggtcaaacacacagggtgagcagccactgccgcagcactgggaaggcaagggttctgtgggccgtagctgcatccaggcttcctcagtgtcgtcgtcctcttccctctcagccatcatcagtggggcttgggcagcctagaaggaacaactgggtgctcttccagaacaggccaggctctatgagaccacgggcgcaggccctgctccttggccagcattttgtagagacagggtctcactatgttgccagtctggtctcgaactcctggcctcaagtgatcttctcatctcagtctcccaaagtgctgagattacaggcatgagccaccatgtctggccctactcgcctgcgcttcacctcacgtgaggattttccaggttcctcccagtctct

SEQ ID NO: 14754 - RNA, 1838 nt, Homo sapiens
  source 1..1838: mol_type = other RNA
gctgggattacaggcatgagccacctcacccagcctcctcatcaccttctaacccactcttatcattttcttgttctgattgctttaccagctaactagaatgtttgggacgtggcagggcaggcagggggatggaggggccctggggacagtgtggctaaccagcctgtgcctgacctggagggcttggagctcatgccaggtgcctggcccgatgtcgccgacccggagccggttgtgcgccaggctgagctcccgcagttggtccaggccggccagaggctcgggctcgagcatccgcagctggttgcgttgcagctgcagggtgcgcaggccagtgggcaggcccatgggcagccgggttagctgattccctgccaggtcgaggctgcgcagggcacgcaaccggcggaaggcccggtggtgcacacgggcgctggccaggcggttataggccaggttaagctccgtcaggcccggtgtggcgaccaggtcacgggcacccagcgcggccacgtggttgtggggcagcaccagggcacgcaggcggcggggcagggctggaggcacgcggtccagcccattgccatagaggtgcagcgtgtgcaggccccgcagcggccgcagagccccggcgggcagccctgagctccccagctggttgtgctgcagcaacaaatagcgcagaccacgcgccccgtgcagccgagccgcctccacctgccggatgcggttgcggcccaggtgcaggatagccagggtccggggcaggccggcgggcactgtggtcagctggttgtgggagagatccaggtattcaaggctatgcagcttgctgaaggtggtggcatccaggccactgtctgtcagctggttgtgctggaggtagagctcacggagttgagtctggcggctcagggctcctcggggcaccttggagatgagattgttctgcaggtggagccgctcgagtgagggcggcaggctgggcggcaggtagctgagctggttgttggagaggctgagggtggcgatggcctcggagccgcggaaggcgtcggggggcaggccagcgttgctcagctggttgttgtggaggtacacggacctgagtgccggcttctccccaaaggtgagggggaagatctccatcacttggttggcagccagatccgcgacacggagggaccggggcagaaactgaggggccactgagagcttgttgtgagccacgcagaggtgctgcagctgggtgagggactcgaaggcctcgtcaggcaggccttcggaggagatgaggttgttgtggaggttgagggttcgcaggccactgaggcgggacagctcattgtaggggagttcctggagctggttgttctgcagggagaggtgctgagcggctctggtgatgttgtccgggaacactcgaaggtccaagccatcacagtccacagtgtcgactcgggggcaggagcagcgcaggggacaggcccggggcaggggctgcaagctctcccccaggtgggggaaggcagcgtcttccaagccggcgacgggcgggggccccggcaacagcaggagcagcagcaggctcggccacatggccagccctgactctgccatctcgcccaagctgctgaccaggacttcctaatggaaaccaggcggtcacctcctggagcctctgctgtggccaccaccgccccccatctccagacccatgccaccccccacaacagcctgttctcccggggctttgggggagctggcccacccccttccccgccctggggaggacgggcaggcggccggatggggtggtgaggacaggccagccc

SEQ ID NO: 14755 - RNA, 1864 nt, Homo sapiens
  source 1..1864: mol_type = other RNA
gctgggattacaggcatgagccacctcacccagcctcctcatcaccttctaacccactcttatcattttcttgttctgattgctttaccagctaactagaatgtttgggacgtggcagggcaggcagggggatggaggggccctggggacagtgtggctaaccagcctgtgcctgacctggagggcttggagctcatgccaggtgcctggcccgatgtcgccgacccggagccggttgtgcgccaggctgagctcccgcagttggtccaggccggccagaggctcgggctcgagcatccgcagctggttgcgttgcagctgcagggtgcgcaggccagtgggcaggcccatgggcagccgggttagctgattccctgccaggtcgaggctgcgcagggcacgcaaccggcggaaggcccggtggtgcacacgggcgctggccaggcggttataggccaggttaagctccgtcaggcccggtgtggcgaccaggtcacgggcacccagcgcggccacgtggttgtggggcagcaccagggcacgcaggcggcggggcagggctggaggcacgcggtccagcccattgccatagaggtgcagcgtgtgcaggccccgcagcggccgcagagccccggcgggcagccctgagctccccagctggttgtgctgcagcaacaaatagcgcagaccacgcgccccgtgcagccgagccgcctccacctgccggatgcggttgcggcccaggtgcaggatagccagggtccggggcaggccggcgggcactgtggtcagctggttgtgggagagatccaggtattcaaggctatgcagcttgctgaaggtggtggcatccaggccactgtctgtcagctggttgtgctggaggtagagctcacggagttgagtctggcggctcagggctcctcggggcaccttggagatgagattgttctgcaggtggagccgctcgagtgagggcggcaggctgggcggcaggtagctgagctggttgttggagaggctgagggtggcgatggcctcggagccgcggaaggcgtcggggggcaggccagcgttgctcagctggttgttgtggaggtacacggacctgagtgccggcttctccccaaaggtgagggggaagatctccatcacttggttggcagccagatccgcgacacggagggaccggggcagaaactgaggggccactgagagcttgttgtgagccacgcagaggtgctgcagctgggtgagggactcgaaggcctcgtcaggcaggccttcggaggagatgaggttgttgtggaggttgagggttcgcaggccactgaggcgggacagctcattgtaggggagttcctggagctggttgttctgcagggagaggtgctgagcggctctggtgatgttgtccgggaacactcgaaggtccaagccatcacagtccacagtgtcgactcgggggcaggagcagcgcaggggacaggcccggggcaggggctgcaagctctcccccaggtgggggaaggcagcgtcttccaagccggcgacgggcgggggccccggcaacagcaggagcagcagcaggctcggccactgggtgggcctccccattgaaagtgtgggagctccctggatagggctgagtcttcccccgcagagtgagagttaccgaagcaggctctgtctcctccatcagactggaaactcccagagctgggggatgatgtctctctcccccatcagtttgggagctctggagggcagaaatgtggatctcttgcaggtgggcagtaactggggcaaggctgtgtctctgtggacagggactgcgccttctccgtgaggctggtagctttgt

SEQ ID NO: 14756 - RNA, 1754 nt, Homo sapiens
  source 1..1754: mol_type = other RNA
gctgggattacaggcatgagccacctcacccagcctcctcatcaccttctaacccactcttatcattttcttgttctgattgctttaccagctaactagaatgtttgggacgtggcagggcaggcagggggatggaggggccctggggacagtgtggctaaccagcctgtgcctgacctggagggcttggagctcatgccaggtgcctggcccgatgtcgccgacccggagccggttgtgcgccaggctgagctcccgcagttggtccaggccggccagaggctcgggctcgagcatccgcagctggttgcgttgcagctgcagggtgcgcaggccagtgggcaggcccatgggcagccgggttagctgattccctgccaggtcgaggctgcgcagggcacgcaaccggcggaaggcccggtggtgcacacgggcgctggccaggcggttataggccaggttaagctccgtcaggcccggtgtggcgaccaggtcacgggcacccagcgcggccacgtggttgtggggcagcaccagggcacgcaggcggcggggcagggctggaggcacgcggtccagcccattgccatagaggtgcagcgtgtgcaggccccgcagcggccgcagagccccggcgggcagccctgagctccccagctggttgtgctgcagcaacaaatagcgcagaccacgcgccccgtgcagccgagccgcctccacctgccggatgcggttgcggcccaggtgcaggatagccagggtccggggcaggccggcgggcactgtggtcagctggttgtgggagagatccaggtattcaaggctatgcagcttgctgaaggtggtggcatccaggccactgtctgtcagctggttgtgctggaggtagagctcacggagttgagtctggcggctcagggctcctcggggcaccttggagatgagattgttctgcaggtggagccgctcgagtgagggcggcaggctgggcggcaggtagctgagctggttgttggagaggctgagggtggcgatggcctcggagccgcggaaggcgtcggggggcaggccagcgttgctcagctggttgttgtggaggtacacggaccttgttgtgagccacgcagaggtgctgcagctgggtgagggactcgaaggcctcgtcaggcaggccttcggaggagatgaggttgttgtggaggttgagggttcgcaggccactgaggcgggacagctcattgtaggggagttcctggagctggttgttctgcagggagaggtgctgagcggctctggtgatgttgtccgggaacactcgaaggtccaagccatcacagtccacagtgtcgactcgggggcaggagcagcgcaggggacaggcccggggcaggggctgcaagctctcccccaggtgggggaaggcagcgtcttccaagccggcgacgggcgggggccccggcaacagcaggagcagcagcaggctcggccactgggtgggcctccccattgaaagtgtgggagctccctggatagggctgagtcttcccccgcagagtgagagttaccgaagcaggctctgtctcctccatcagactggaaactcccagagctgggggatgatgtctctctcccccatcagtttgggagctctggagggcagaaatgtggatctcttgcaggtgggcagtaactggggcaaggctgtgtctctgtggacagggactgcgccttctccgtgaggctggtagctttgt

SEQ ID NO: 14757 - RNA, 1563 nt, Homo sapiens
  source 1..1563: mol_type = other RNA
gctgggattacaggcatgagccacctcacccagcctcctcatcaccttctaacccactcttatcattttcttgttctgattgctttaccagctaactagaatgtttgggacgtggcagggcaggcagggggatggaggggccctggggacagtgtggctaaccagcctgtgcctgacctggagggcttggagctcatgccaggtgcctggcccgatgtcgccgacccggagccggttgtgcgccaggctgagctcccgcagttggtccaggccggccagaggctcgggctcgagcatccgcagctggttgcgttgcagctgcagggtgcgcaggccagtgggcaggcccatgggcagccgggttagctgattccctgccaggtcgaggctgcgcagggcacgcaaccggcggaaggcccggtggtgcacacgggcgctggccaggcggttataggccaggttaagctccgtcaggcccggtgtggcgaccaggtcacgggcacccagcgcggccacgtggttgtggggcagcaccagggcacgcaggcggcggggcagggctggaggcacgcggtccagcccattgccatagaggtgcagcgtgtgcaggccccgcagcggccgcagagccccggcgggcagccctgagctccccagctggttgtgctgcagcaacaaatagcgcagaccacgcgccccgtgcagccgagccgcctccacctgccggatgcggttgcggcccaggtgcaggatagccagggtccggggcaggccggcgggcactgtggtcagctggttgtgggagagatccaggtattcaaggctatgcagcttgctgaaggtggtggcatccaggccactgtctgtcagctggttgtgctggaggtagagctcacggagttgagtctggcggctcagggctcctcggggcaccttggagatgagattgttcttgttgtgagccacgcagaggtgctgcagctgggtgagggactcgaaggcctcgtcaggcaggccttcggaggagatgaggttgttgtggaggttgagggttcgcaggccactgaggcgggacagctcattgtaggggagttcctggagctggttgttctgcagggagaggtgctgagcggctctggtgatgttgtccgggaacactcgaaggtccaagccatcacagtccacagtgtcgactcgggggcaggagcagcgcaggggacaggcccggggcaggggctgcaagctctcccccaggtgggggaaggcagcgtcttccaagccggcgacgggcgggggccccggcaacagcaggagcagcagcaggctcggccacatggccagccctgactctgccatctcgcccaagctgctgaccaggacttcctaatggaaaccaggcggtcacctcctggagcctctgctgtggccaccaccgccccccatctccagacccatgccaccccccacaacagcctgttctcccggggctttgggggagctggcccacccccttccccgccctggggaggacgggcaggcggccggatggggtggtgaggacag

SEQ ID NO: 14758 - RNA, 1597 nt, Homo sapiens
  source 1..1597: mol_type = other RNA
gctgggattacaggcatgagccacctcacccagcctcctcatcaccttctaacccactcttatcattttcttgttctgattgctttaccagctaactagaatgtttgggacgtggcagggcaggcagggggatggaggggccctggggacagtgtggctaaccagcctgtgcctgacctggagggcttggagctcatgccaggtgcctggcccgatgtcgccgacccggagccggttgtgcgccaggctgagctcccgcagttggtccaggccggccagaggctcgggctcgagcatccgcagctggttgcgttgcagctgcagggtgcgcaggccagtgggcaggcccatgggcagccgggttagctgattccctgccaggtcgaggctgcgcagggcacgcaaccggcggaaggcccggtggtgcacacgggcgctggccaggcggttataggccaggttaagctccgtcaggcccggtgtggcgaccaggtcacgggcacccagcgcggccacgtggttgtggggcagcaccagggcacgcaggcggcggggcagggctggaggcacgcggtccagcccattgccatagaggtgcagcgtgtgcaggccccgcagcggccgcagagccccggcgggcagccctgagctccccagctggttgtgctgcagcaacaaatagcgcagaccacgcgccccgtgcagccgagccgcctccacctgccggatgcggttgcggcccaggtgcaggatagccagggtccggggcaggccggcgggcactgtggtcagctggttgtgggagagatccaggtattcaaggctatgcagcttgctgaaggtggtggcatccaggccactgtctgtcagctggttgtgctggaggtagagctcacggagttgagtctggcggctcagggctcctcggggcaccttggagatgagattgttcttgttgtgagccacgcagaggtgctgcagctgggtgagggactcgaaggcctcgtcaggcaggccttcggaggagatgaggttgttgtggaggttgagggttcgcaggccactgaggcgggacagctcattgtaggggagttcctggagctggttgttctgcagggagaggtgctgagcggctctggtgatgttgtccgggaacactcgaaggtccaagccatcacagtccacagtgtcgactcgggggcaggagcagcgcaggggacaggcccggggcaggggctgcaagctctcccccaggtgggggaaggcagcgtcttccaagccggcgacgggcgggggccccggcaacagcaggagcagcagcaggctcggccactgggtgggcctccccattgaaagtgtgggagctccctggatagggctgagtcttcccccgcagagtgagagttaccgaagcaggctctgtctcctccatcagactggaaactcccagagctgggggatgatgtctctctcccccatcagtttgggagctctggagggcagaaatgtggatctcttgcaggtgggcagtaactggggcaaggctgtgtctctgtggacagggactgcgccttctccgtgaggctggtagctttgt

SEQ ID NO: 14759 - RNA, 10264 nt, Homo sapiens
  source 1..10264: mol_type = other RNA
gctgggattacaggcatgagccacctcacccggccaataaagcttttagaagaatataagaatatcttcataaccttggtgtgaacatttattaaatacgacgcaaaagtattagcaattaaataaaagactggtatattggacttcataaaatttttggtcatcaaaggaaagcacttagaaagtagaaaagcaaactaaagagaagacatttatggtaaaatatcagacaaaaaccctcatatccataaaatataaaagactcctgcaagtcagtaagaaaaaaagacaacccaataaatatgaacaaatgacttgaacaggcacttaattgaggatagccaaatgactaataaaaatataaaaaggtgttccacacatcactacttatcaggaaaatacaccttaaaatctcagtgaaatacaaaatcaccagaatggttaaaaccacaatcaaatatacacatttgtcagagtggctaaactactagggctgatggtaccaagcactgatgaggatgtggaagaactagaacacttacacattattggtgggtatgtaaattggtacaaccattgttgaaaaccatttggtaatatcttctacagctaaatatatattcatcttatgactcagtagtttcactccttttttttgtctgtttttttgagacagggtctcactctatcgcccaggatggaatgtagtggtgcgatcaaggctcactgcagccagctgtttcacttttaagtggacacacaagagaaatgagtgtacgtgtccattaaaatatatgcacaagaatgcttatggctgctttaaacacaaaagctaaaaattacaaacaaccaaaatgtctatcagtgggagaatggataaattgtgatgtatttatctgatggaatactacagagcaacgaaaaagaacaaactactgttattgctacatgcaacaacatagatgcatttcacagacataatgctgatcaaattaaaccagacacaaaaacctatagactggataattccatgtataggaatgtcaacaacagtgacagaggtcagagtggtggttatgtatgaggactgactgggagcctcatcttgatctgaatgatggttatatgggcgcatatatatgtaaacatttattgagctgtatatttcagacctgtgcactttacacaccatgttgcaataacattttaaacaatatgatcactatctatatgtagttttagtgctccatttggactggtctctggccactggatgtcagtgtttggagcagtgggcagcaggaaaagctggggaaggagtgggaaaacagaggagagagctatcacatgggcttcctagagaaaaataagcactttatgaagcttataagttcctttatgtacacagtagacaaagccttttaaagagatttgtccatacgggcactgaaataacatttttgtaaagtagccttctctatgttgattgcagatgtttctatctcagaatttaagtctacttgctttctcacacagcatcattatttccttattcctaataattttcatcacaaacatttcccagctctgtcccaatcaagttcttatttctctgaacggaattacaatttataaatgtaggtccacatgcagatatcttaataagtagtgaaataccagtgtagaaatacacaaatgagtgtggacacaccatagaaaagcagaaaaatacgagaaaaagtgcatgtacggagtatgggatgaactgatgcagttaaggaagacaactcacaaagcaactcacggctgggcaaagctgggaggctgaggcgggaggattgcttgaagccaggagtttgagactagcctgggcaccatactgataccttgtagctattaaaaaaaaattagctgggcatggtggctcatgcctgtagtctacttagtcagctgcttaggaggctgaggtacaaggattgcttgagcccaggaggtggaggttgcagtgagctgtgatcacgccactgcactccggccagggtgacagagtgagaccctgtctcacacaaaggcaactcatttgagctgaggcttggctatacttttaattgtccacatagaatagaggaaaaacaatgtttttcatcttttttaatcttccatttaccttttagtaagacaaattcttatctttatgtaaaactgtggaagagcagttacatagattgttgcagcttagattattttcaagaagtttaaattctacacataaggatacataccatttttaccagctatactttaaaatgccagtctttaaaaattcctctatgtgtatatgtggtttcttcttcttttcaaaaattcatgcctgtgaagtttttaggaatatttttcaaaactttagtactgaggcattaactgtttatgtgacacagcacctttaaatttctgtttttattcagccaaagaatgagaattattgtacattgctagtatttataatttcagcaaataggatagcagtatagtacctaaaataaactattaggaataactgaatgcctaccacagcaacagagctttaatgaggttaattgtcacatacatatccattccaacatagcagtgcacatttcacatgaccagcctcttatgtagttaaaaataaaactgcagttttaaaatgtcaagttcctcaaccttactggattttaaaacaaagcaaacaaaagaaacaaggattttctaatctatctataagcagaaatgtcagaaaataaagctacagtattccataaaacttaaaatttccttttctaagtcatgacatttctcttttgttctgttttctttttcttctaatattaagaaaatttaaaacgtaaatgaaaaaactgcttaatgtggcaaggaacaagaatgaaactagatttttttttttagtaaaggggcaaattgtataccaacatataaattaaaagtgttatgcaatgagaaacaataatggaaacagcataatactacatactatcccagtttcctgtgctctgaagaacagctgctatactaaatactaacttgacttatctgaagtattcaatactttctgataacccaagcagcattatattaatagttagaatactactacaaaatgtccttctacctctcccacaagaaatacaccaggaaacttaagcctgatgaataactactaagaatcttgtcttttaatacaagtctccttctagacacaaaatcctagctttttgtaatgtggttaaaaggagtaatggaaaagaaatgactgccaataaacatttcctattttgcactagggtgaagaaaccaagacacaaacatttggaagccactttagtttcttattccttttcaccctaatagtaggaaaatattaggcacctacttaattcacaaattcatgaaacagggtggacaacagccttgtgtaggggaagcatttggaatggtaatcaactacttaattacataacagggagctgggcatacaaagaaaagggctcagaagaaatatcttgaaaagtaagcaatatagaaggtgaggacagaagtgaggctaatcaaatgttcttagcaagatgttgcccccctgaaaatatgctcccccaataaaacacgtaaataactactcttaaggaaaatattttctctaaagaatgtcacaatttggagtgaagttacttaacaaaacagggaataaaacctttaatgttggctgtagcagttattttctttgggtagattatacttaaaatatttccttcatacatacttctgttaaaatttttttttcccattcttgagttttacaatgtctcctatccaaacttcaaatttcattagagccggctacatttgttttagtgccagatacaggtatcaagtgatgacagacacttacgtgaggtatacaatcaattaaagactggaaattggggtattatcatgtaagacatttgagaggccaaaagtcatataattttaagatacttcatgatgttacagtaataattcatctatataacaattattttgacataagtggcatatcagaatttaacttatttacttagatcttaaggaatattagatgtattctcacatgaacactcaaatcatgctattattatcagtcactgggagaacagccaaagtaatcaggcagtctaaggcacatatagacccaataatttagaaattttcaccattatgaggtaccctgtttttaataaatatgacaataacaggcgcttgaaatgggggcaaggtgaataagtatccagtcaattgtatacttttataaagtagtgtatttgagaacataaactgagatacaaaaggaatttccttactttaaaaaaagtgacttctatcttagtagatttctttaaaataacttaccttatatttaaaagttagtcatttacatacttaagaaatcaacagtaatctaaaaaaattaaaaggcagttttcttgggtaatgaacctgtgactccaagacagacaacaatgtggaaattaactcaggagactgactttctattctagtaattcagtggtttcttactttataaaggtttggaagaattaatgaatttctttttttcttaagacagggtctcgctctgttgcccaggctggagtgcagtggtgtgatcacagctcactgcagcctcgaactcctgggctcaagcgatcctccacatgttggcctcccatgagccaccatgctcagctaatttttatttttatttttggagagacagtgtctcactatgttgcccaggttggtctctaactcctggtttcaagtgattctccagtcttatactcccaaagcacaaggattacaggcctgagccaccacactcagccaatcaatttcaaaatgctaattaacctctttcagacacacgatctggcagagtaattagaagaaactggtctttcttaacatctttcctctattatcttccttttcttattcttgcctctcaatttgtcatatacagttacaaaatatatgaatcaggatttatgttggcatgaaaattatatgcaatacaatcagtaagtgaagaagggagggggtggtgtggctctagtcccaaagttaatgtcataaggagaaataatgtaagtatttgtatttcttagatcttcttctattttactcttaataccaaaaaaagagtcctatcatttaactttttatatattttgtagtgtttatttttgatgtgaccaaatgaaagctttctgaattttaaagtgcaattcactgtatgttaatacacagcctgcataggacctaactgcttcaaacttggcatcaaatgctgtctttttggtacttataagtagggtgtagataaagatatttgacaagagtgcaacagtgtttgttaaggtcttttcaaaagcccatttgagattattcaggcaggctcatcagttgacagctagcctatctttccttcttcctgttagtctgactgcctttttacccatttcatcgcctgtcgaatcctcctcaagaagaggcaagggaaataaatgaaaatgaaacccattaatttccaatattcacaatgaaatcaatcacatcatcaatctgtatactgtctgaccatttttctggatcattttctattagcaacatagtccctttagtttgtactttataactagtattttctaccaggatgcacagtttaaaaaatggcttgaagagccaaatatgttcccaatatgtccaatataattataaatatggtcattttcttgattactagagatctgtgcctgatggaatcacattttgtgaattagcaatagtttggtaataattcacacaaaatttcccataattactaggaataactgaaagctgggagtagaaaactttcattaactcaatattatgtagccatttgggccagcaaaaagtgtaaaatattattcccaataaccactgtggacaaaatgtgaacaggataatataatattttgaaaatattttaatatttgccattttttgcctgtgctattaatatatacattgatttagtaataaatatactactattacatagagtgcaatatttttagtattcataactggttgaaattaatgctgctataacctcaagaaaggaataaataaatatcatgtccaaattccaaactaatgctcaaaaggttatcattaacaaaaactataaaataaacatgttgggcattatctctttaagcatgattcctgtaaacaaagcaaaaaaatcacttttctcagtcctgacatttcacatgatggctttaaaagaaaatataacacacaaaccctatcacttcttttttttttttttttttttttgcatagggaacgaattaattgtatttttaaatgcagcaatcttttaatgaaatgttttcatcacatagtacttgttttctgtatgaattcagaacttttgagcaataaaagtgctctgcataagtttataaaatatgctttctggatttaaaatttaacagaaaaatttccaaacaagtcataggtatgattctaaaatattatgtacataatatatgactacaggaggaaattcctcactgtagtacaacacagtgtacaaatatgaagcacagtgtttagtttaatttccctttaggttttcctcacattggtgcataagtggctgactacatgacacaacatgccccattctacttgttgcatacaaagtagaagaggaatgtgaggacaaatttaaagtagaaaatgaaaataaatggcaaaaatacagtgcaaatgctttaaacagtgcactttataaaatagtttgctttattcatacttttttataaagtgcaatattacttaaaacagagagacatgtaccttaatattctgcaataaccattaaaacaaattgccaggaaagagcagtgcaaaattaaaaacatacacatagcttagcatgcatctcagatggatcccgaatacagagtatgggaccttgagttcttatatctttttttttttttttcactttttagaaaaagtttaataatagcaggttatcatcatatgtaaccataaaataaaaacaataagttaaaatcttctctcaagaaataagtatatgccacacataaaattcattacagaatcttttttgaaaacagacccctttctctgataaatcattgtttgaagggtgcaaatttcaaaaacccacattgtccacaaggcaaagcaaaaggtatcatcacagtatgagtcatttcttgttggcagacatctggaaaacctgtgacttacaagcagctcaaatctagccctaattaaatttacaggaacctttgctctttcaagaatagtcttgttggcatcatgctaggttgctaaaaagagtaatatgtgctctattcacagtaacattctctgtccagtgcttttgaatgaggataaccaaacaggttttcctgaaaaaaatcattaggaggcagattccaatgagaccaacgggaaacatttttaaaagcataaaagatcgcctcaggcatatgctgagggaataaaggtgcaatggatcactgatacactcctaccatgcctaagctactgagtccgagaactggaagagggtctccgggttattgctgtcggcaggattgctgggctgcagtgtcttggtgggtgtagttttaccgtgagaatgagaggaagaagaatgggaactctcactggaactgctgcgcgtctcggtactggtgctagtctttttcatttttcttctcttagccaaaggggccttatcaacattctgaaggcaaaacccctctctcttgtatttgttaaaggcgtggaaggttgctttcacacaggtatgcacggcagctccggaagatcctagaatatccggagtcatcagaggattggaggacagctgacttccatcttgtagccattcattgtacctcaagccagacattttaagccttttgtttggatctactgtgagaagtccttggatcaaatctttagcctcttgggatacattcttccaggcttctccttcaaaggagaaatctccctttttaattttcttcatgatttccaccgcgctggtacacgtcaaacttcggtcatgagattggaagggaaccaaaatgacgcccaagctccacaggtcacaggactcatcgtagccgttctgattcaagagctctggggcggcataatgaagggtgaagcatggagtcttcaggggctgattatccggtggctttagccgtgcaaatccaaaatcaattattttaatttccaaattgtcattttcatcggtgaacaataaattctcaggtttcagatccctgtgcaccactccaacatcatgcatgtggcttacagctgaaacaagcttcctcatgatgtagctggcttccgtctcactgaagtgcttctttttcttaatgcgctcaaacagttctcctccattcagaagttccatcactagaaacgtgtgaagctgatcatgaaaaacttcatgcaacttcacaatattggggtgtccttcacagagtttcagagctgttatttccttttgagtattggcttccatccttttgctgattattttgactgcaaaagcttggttactttttttatgcacacactttcgacaaattgaaaaactaccttctcccaggggtttgtccttcaaatctaggtcatagtgttgatagaatggagagtccttcatcattgcactcctggcaacatttgtcactccaggacgttcaactcccatgtgaaactgaagagggtctatgacagctgcattacgcttgaataggatggaaggagcaacaaaggaatagccctgaaacagcttctcagaactctggggcagggctgcgggagaataagtgggatccatttctgtgaactcttctgcaaagttactcacatctaattcatctcgaatgactggcttaaatggtgcaggcacttttttggcggctaaatcatcccaatttattttctgaaagaagagatgttctttgatttcatctgcatcacgtggaccacatcccaatctcttcttgggatctttcatcaaaagacgctgaattaggtctttcgctaaagcactcatttcttggggatatggaggctcactttttaatattctcctagatatctcagcttgggaatttttttctccatcaacagtgaaaggagatgctccagttagtaattcatacattagaacacccaaactccaccagtcaactgccttgtcatgtcctgaatctccccctctgacaatatctggtgccatgtattcaatagttccacaaaaggaatatgctctttcagtttcatcagccacaaactccttactcagaccaaaatctgtcagcaccacatggccattagaatcaagtagaatattctcaagcttaatatcacgatatataatccccaacttgtggagatgttcgagggcaagcacaatctctccaacataaatctgcacctcatgctctgtgaaacgctctctttgagaaagatgagtaaaaagttcaccaccatttatataatctaaaatgagatgaagtttggtttctgtctggaaagcataatgtaatgttaccaaaaatggcgactgcctaatgtgttccaggacttgtcgttctgtccttgtatgctctgtggttttggccttttgaacgattgttgcctttttcaaaactttcatggcatacagctttccagtatcatggccacttattttacgaactagaaatacttttccataagctccagttcctaggaccttcaggagctcaaaattttctattcccaccttctcagcatgtcctgtcaaattagcagtccgcagctcgtgcttgacagtgaggagctgctctcctccgtcgccgccgtccgcgctggtccccgcggcgccgccgctgctgccaccctcctcctccatcttctcctttttttccgatcccgcgggtcgctacgaggggaacccaggagacagcggacgcccgtcccctcgcagccgctgccgcggccccaggagtcggggtgcggcggctccagaactcggacgcaaagacgagtctctttcccgctctggccgcacggctcgctcctcgcctcctcccccttcggcgggcaccgctagtaccgc

SEQ ID NO: 14760 - RNA, 10322 nt, Homo sapiens
  source 1..10322: mol_type = other RNA
gctgggattacaggcatgagccacctcacccggccaataaagcttttagaagaatataagaatatcttcataaccttggtgtgaacatttattaaatacgacgcaaaagtattagcaattaaataaaagactggtatattggacttcataaaatttttggtcatcaaaggaaagcacttagaaagtagaaaagcaaactaaagagaagacatttatggtaaaatatcagacaaaaaccctcatatccataaaatataaaagactcctgcaagtcagtaagaaaaaaagacaacccaataaatatgaacaaatgacttgaacaggcacttaattgaggatagccaaatgactaataaaaatataaaaaggtgttccacacatcactacttatcaggaaaatacaccttaaaatctcagtgaaatacaaaatcaccagaatggttaaaaccacaatcaaatatacacatttgtcagagtggctaaactactagggctgatggtaccaagcactgatgaggatgtggaagaactagaacacttacacattattggtgggtatgtaaattggtacaaccattgttgaaaaccatttggtaatatcttctacagctaaatatatattcatcttatgactcagtagtttcactccttttttttgtctgtttttttgagacagggtctcactctatcgcccaggatggaatgtagtggtgcgatcaaggctcactgcagccagctgtttcacttttaagtggacacacaagagaaatgagtgtacgtgtccattaaaatatatgcacaagaatgcttatggctgctttaaacacaaaagctaaaaattacaaacaaccaaaatgtctatcagtgggagaatggataaattgtgatgtatttatctgatggaatactacagagcaacgaaaaagaacaaactactgttattgctacatgcaacaacatagatgcatttcacagacataatgctgatcaaattaaaccagacacaaaaacctatagactggataattccatgtataggaatgtcaacaacagtgacagaggtcagagtggtggttatgtatgaggactgactgggagcctcatcttgatctgaatgatggttatatgggcgcatatatatgtaaacatttattgagctgtatatttcagacctgtgcactttacacaccatgttgcaataacattttaaacaatatgatcactatctatatgtagttttagtgctccatttggactggtctctggccactggatgtcagtgtttggagcagtgggcagcaggaaaagctggggaaggagtgggaaaacagaggagagagctatcacatgggcttcctagagaaaaataagcactttatgaagcttataagttcctttatgtacacagtagacaaagccttttaaagagatttgtccatacgggcactgaaataacatttttgtaaagtagccttctctatgttgattgcagatgtttctatctcagaatttaagtctacttgctttctcacacagcatcattatttccttattcctaataattttcatcacaaacatttcccagctctgtcccaatcaagttcttatttctctgaacggaattacaatttataaatgtaggtccacatgcagatatcttaataagtagtgaaataccagtgtagaaatacacaaatgagtgtggacacaccatagaaaagcagaaaaatacgagaaaaagtgcatgtacggagtatgggatgaactgatgcagttaaggaagacaactcacaaagcaactcacggctgggcaaagctgggaggctgaggcgggaggattgcttgaagccaggagtttgagactagcctgggcaccatactgataccttgtagctattaaaaaaaaattagctgggcatggtggctcatgcctgtagtctacttagtcagctgcttaggaggctgaggtacaaggattgcttgagcccaggaggtggaggttgcagtgagctgtgatcacgccactgcactccggccagggtgacagagtgagaccctgtctcacacaaaggcaactcatttgagctgaggcttggctatacttttaattgtccacatagaatagaggaaaaacaatgtttttcatcttttttaatcttccatttaccttttagtaagacaaattcttatctttatgtaaaactgtggaagagcagttacatagattgttgcagcttagattattttcaagaagtttaaattctacacataaggatacataccatttttaccagctatactttaaaatgccagtctttaaaaattcctctatgtgtatatgtggtttcttcttcttttcaaaaattcatgcctgtgaagtttttaggaatatttttcaaaactttagtactgaggcattaactgtttatgtgacacagcacctttaaatttctgtttttattcagccaaagaatgagaattattgtacattgctagtatttataatttcagcaaataggatagcagtatagtacctaaaataaactattaggaataactgaatgcctaccacagcaacagagctttaatgaggttaattgtcacatacatatccattccaacatagcagtgcacatttcacatgaccagcctcttatgtagttaaaaataaaactgcagttttaaaatgtcaagttcctcaaccttactggattttaaaacaaagcaaacaaaagaaacaaggattttctaatctatctataagcagaaatgtcagaaaataaagctacagtattccataaaacttaaaatttccttttctaagtcatgacatttctcttttgttctgttttctttttcttctaatattaagaaaatttaaaacgtaaatgaaaaaactgcttaatgtggcaaggaacaagaatgaaactagatttttttttttagtaaaggggcaaattgtataccaacatataaattaaaagtgttatgcaatgagaaacaataatggaaacagcataatactacatactatcccagtttcctgtgctctgaagaacagctgctatactaaatactaacttgacttatctgaagtattcaatactttctgataacccaagcagcattatattaatagttagaatactactacaaaatgtccttctacctctcccacaagaaatacaccaggaaacttaagcctgatgaataactactaagaatcttgtcttttaatacaagtctccttctagacacaaaatcctagctttttgtaatgtggttaaaaggagtaatggaaaagaaatgactgccaataaacatttcctattttgcactagggtgaagaaaccaagacacaaacatttggaagccactttagtttcttattccttttcaccctaatagtaggaaaatattaggcacctacttaattcacaaattcatgaaacagggtggacaacagccttgtgtaggggaagcatttggaatggtaatcaactacttaattacataacagggagctgggcatacaaagaaaagggctcagaagaaatatcttgaaaagtaagcaatatagaaggtgaggacagaagtgaggctaatcaaatgttcttagcaagatgttgcccccctgaaaatatgctcccccaataaaacacgtaaataactactcttaaggaaaatattttctctaaagaatgtcacaatttggagtgaagttacttaacaaaacagggaataaaacctttaatgttggctgtagcagttattttctttgggtagattatacttaaaatatttccttcatacatacttctgttaaaatttttttttcccattcttgagttttacaatgtctcctatccaaacttcaaatttcattagagccggctacatttgttttagtgccagatacaggtatcaagtgatgacagacacttacgtgaggtatacaatcaattaaagactggaaattggggtattatcatgtaagacatttgagaggccaaaagtcatataattttaagatacttcatgatgttacagtaataattcatctatataacaattattttgacataagtggcatatcagaatttaacttatttacttagatcttaaggaatattagatgtattctcacatgaacactcaaatcatgctattattatcagtcactgggagaacagccaaagtaatcaggcagtctaaggcacatatagacccaataatttagaaattttcaccattatgaggtaccctgtttttaataaatatgacaataacaggcgcttgaaatgggggcaaggtgaataagtatccagtcaattgtatacttttataaagtagtgtatttgagaacataaactgagatacaaaaggaatttccttactttaaaaaaagtgacttctatcttagtagatttctttaaaataacttaccttatatttaaaagttagtcatttacatacttaagaaatcaacagtaatctaaaaaaattaaaaggcagttttcttgggtaatgaacctgtgactccaagacagacaacaatgtggaaattaactcaggagactgactttctattctagtaattcagtggtttcttactttataaaggtttggaagaattaatgaatttctttttttcttaagacagggtctcgctctgttgcccaggctggagtgcagtggtgtgatcacagctcactgcagcctcgaactcctgggctcaagcgatcctccacatgttggcctcccatgagccaccatgctcagctaatttttatttttatttttggagagacagtgtctcactatgttgcccaggttggtctctaactcctggtttcaagtgattctccagtcttatactcccaaagcacaaggattacaggcctgagccaccacactcagccaatcaatttcaaaatgctaattaacctctttcagacacacgatctggcagagtaattagaagaaactggtctttcttaacatctttcctctattatcttccttttcttattcttgcctctcaatttgtcatatacagttacaaaatatatgaatcaggatttatgttggcatgaaaattatatgcaatacaatcagtaagtgaagaagggagggggtggtgtggctctagtcccaaagttaatgtcataaggagaaataatgtaagtatttgtatttcttagatcttcttctattttactcttaataccaaaaaaagagtcctatcatttaactttttatatattttgtagtgtttatttttgatgtgaccaaatgaaagctttctgaattttaaagtgcaattcactgtatgttaatacacagcctgcataggacctaactgcttcaaacttggcatcaaatgctgtctttttggtacttataagtagggtgtagataaagatatttgacaagagtgcaacagtgtttgttaaggtcttttcaaaagcccatttgagattattcaggcaggctcatcagttgacagctagcctatctttccttcttcctgttagtctgactgcctttttacccatttcatcgcctgtcgaatcctcctcaagaagaggcaagggaaataaatgaaaatgaaacccattaatttccaatattcacaatgaaatcaatcacatcatcaatctgtatactgtctgaccatttttctggatcattttctattagcaacatagtccctttagtttgtactttataactagtattttctaccaggatgcacagtttaaaaaatggcttgaagagccaaatatgttcccaatatgtccaatataattataaatatggtcattttcttgattactagagatctgtgcctgatggaatcacattttgtgaattagcaatagtttggtaataattcacacaaaatttcccataattactaggaataactgaaagctgggagtagaaaactttcattaactcaatattatgtagccatttgggccagcaaaaagtgtaaaatattattcccaataaccactgtggacaaaatgtgaacaggataatataatattttgaaaatattttaatatttgccattttttgcctgtgctattaatatatacattgatttagtaataaatatactactattacatagagtgcaatatttttagtattcataactggttgaaattaatgctgctataacctcaagaaaggaataaataaatatcatgtccaaattccaaactaatgctcaaaaggttatcattaacaaaaactataaaataaacatgttgggcattatctctttaagcatgattcctgtaaacaaagcaaaaaaatcacttttctcagtcctgacatttcacatgatggctttaaaagaaaatataacacacaaaccctatcacttcttttttttttttttttttttttgcatagggaacgaattaattgtatttttaaatgcagcaatcttttaatgaaatgttttcatcacatagtacttgttttctgtatgaattcagaacttttgagcaataaaagtgctctgcataagtttataaaatatgctttctggatttaaaatttaacagaaaaatttccaaacaagtcataggtatgattctaaaatattatgtacataatatatgactacaggaggaaattcctcactgtagtacaacacagtgtacaaatatgaagcacagtgtttagtttaatttccctttaggttttcctcacattggtgcataagtggctgactacatgacacaacatgccccattctacttgttgcatacaaagtagaagaggaatgtgaggacaaatttaaagtagaaaatgaaaataaatggcaaaaatacagtgcaaatgctttaaacagtgcactttataaaatagtttgctttattcatacttttttataaagtgcaatattacttaaaacagagagacatgtaccttaatattctgcaataaccattaaaacaaattgccaggaaagagcagtgcaaaattaaaaacatacacatagcttagcatgcatctcagatggatcccgaatacagagtatgggaccttgagttcttatatctttttttttttttttcactttttagaaaaagtttaataatagcaggttatcatcatatgtaaccataaaataaaaacaataagttaaaatcttctctcaagaaataagtatatgccacacataaaattcattacagaatcttttttgaaaacagacccctttctctgataaatcattgtttgaagggtgcaaatttcaaaaacccacattgtccacaaggcaaagcaaaaggtatcatcacagtatgagtcatttcttgttggcagacatctggaaaacctgtgacttacaagcagctcaaatctagccctaattaaatttacaggaacctttgctctttcaagaatagtcttgttggcatcatgctaggttgctaaaaagagtaatatgtgctctattcacagtaacattctctgtccagtgcttttgaatgaggataaccaaacaggttttcctgaaaaaaatcattaggaggcagattccaatgagaccaacgggaaacatttttaaaagcataaaagatcgcctcaggcatatgctgagggaataaaggtgcaatggatcactgatacactcctaccatgcctaagctactgagtccgagaactggaagagggtctccgggttattgctgtcggcaggattgctgggctgcagtgtcttggtgggtgtagttttaccgtgagaatgagaggaagaagaatgggaactctcactggaactgctgcgcgtctcggtactggtgctagtctttttcatttttcttctcttagccaaaggggccttatcaacattctgaaggcaaaacccctctctcttgtatttgttaaaggcgtggaaggttgctttcacacaggtatgcacggcagctccggaagatcctagaatatccggagtcatcagaggattggaggacagctgacttccatcttgtagccattcattgtacctcaagccagacattttaagccttttgtttggatctactgtgagaagtccttggatcaaatctttagcctcttgggatacattcttccaggcttctccttcaaaggagaaatctccctttttaattttcttcatgatttccaccgcgctggtacacgtcaaacttcggtcatgagattggaagggaacctgtcctgacaacattgtgtacaaaatgacgcccaagctccacaggtcacaggactcatcgtagccgttctgattcaagagctctggggcggcataatgaagggtgaagcatggagtcttcaggggctgattatccggtggctttagccgtgcaaatccaaaatcaattattttaatttccaaattgtcattttcatcggtgaacaataaattctcaggtttcagatccctgtgcaccactccaacatcatgcatgtggcttacagctgaaacaagcttcctcatgatgtagctggcttccgtctcactgaagtgcttctttttcttaatgcgctcaaacagttctcctccattcagaagttccatcactagaaacgtgtgaagctgatcatgaaaaacttcatgcaacttcacaatattggggtgtccttcacagagtttcagagctgttatttccttttgagtattggcttccatccttttgctgattattttgactgcaaaagcttggttactttttttatgcacacactttcgacaaattgaaaaactaccttctcccaggggtttgtccttcaaatctaggtcatagtgttgatagaatggagagtccttcatcattgcactcctggcaacatttgtcactccaggacgttcaactcccatgtgaaactgaagagggtctatgacagctgcattacgcttgaataggatggaaggagcaacaaaggaatagccctgaaacagcttctcagaactctggggcagggctgcgggagaataagtgggatccatttctgtgaactcttctgcaaagttactcacatctaattcatctcgaatgactggcttaaatggtgcaggcacttttttggcggctaaatcatcccaatttattttctgaaagaagagatgttctttgatttcatctgcatcacgtggaccacatcccaatctcttcttgggatctttcatcaaaagacgctgaattaggtctttcgctaaagcactcatttcttggggatatggaggctcactttttaatattctcctagatatctcagcttgggaatttttttctccatcaacagtgaaaggagatgctccagttagtaattcatacattagaacacccaaactccaccagtcaactgccttgtcatgtcctgaatctccccctctgacaatatctggtgccatgtattcaatagttccacaaaaggaatatgctctttcagtcttgaacaaacaaacaaaaaagggatttgatttcaagttcatcagccacaaactccttactcagaccaaaatctgtcagcaccacatggccattagaatcaagtagaatattctcaagcttaatatcacgatatataatccccaacttgtggagatgttcgagggcaagcacaatctctccaacataaatctgcacctcatgctctgtgaaacgctctctttgagaaagatgagtaaaaagttcaccaccatttatataatctaaaatgagatgaagtttggtttctgtctggaaagcataatgtaatgttaccaaaaatggcgactgcctaatgtgttccaggacttgtcgttctgtccttgtatgctctgtggttttggccttttgaacgattgttgcctttttcaaaactttcatggcatacagctttccagtatcatggccacttattttacgaactagaaatacttttccataagctccagttcctaggaccttcaggagctcaaaattttctattcccaccttctcagcatgtcctgtcaaattagcagtccgcagctcgtgcttgacagtgaggagctgctctcctccgtcgccgccgtccgcgctggtccccgcggcgccgccgctgctgccaccctcctcctccatcttctcctttttttccgatcccgcgggtcgctacgaggggaacccaggagacagcggacgcccgtcccctcgcagccgctgccgcggccccaggagtcggggtgcggcggctccagaactcggacgcaaagacgagtctctttcccgctctggccgcacggctcgctcctcgcctcctcccccttcggcgggcaccgctagtaccgc

SEQ ID NO: 14761 - RNA, 10177 nt, Homo sapiens
  source 1..10177: mol_type = other RNA
gctgggattacaggcatgagccacctcacccggccaataaagcttttagaagaatataagaatatcttcataaccttggtgtgaacatttattaaatacgacgcaaaagtattagcaattaaataaaagactggtatattggacttcataaaatttttggtcatcaaaggaaagcacttagaaagtagaaaagcaaactaaagagaagacatttatggtaaaatatcagacaaaaaccctcatatccataaaatataaaagactcctgcaagtcagtaagaaaaaaagacaacccaataaatatgaacaaatgacttgaacaggcacttaattgaggatagccaaatgactaataaaaatataaaaaggtgttccacacatcactacttatcaggaaaatacaccttaaaatctcagtgaaatacaaaatcaccagaatggttaaaaccacaatcaaatatacacatttgtcagagtggctaaactactagggctgatggtaccaagcactgatgaggatgtggaagaactagaacacttacacattattggtgggtatgtaaattggtacaaccattgttgaaaaccatttggtaatatcttctacagctaaatatatattcatcttatgactcagtagtttcactccttttttttgtctgtttttttgagacagggtctcactctatcgcccaggatggaatgtagtggtgcgatcaaggctcactgcagccagctgtttcacttttaagtggacacacaagagaaatgagtgtacgtgtccattaaaatatatgcacaagaatgcttatggctgctttaaacacaaaagctaaaaattacaaacaaccaaaatgtctatcagtgggagaatggataaattgtgatgtatttatctgatggaatactacagagcaacgaaaaagaacaaactactgttattgctacatgcaacaacatagatgcatttcacagacataatgctgatcaaattaaaccagacacaaaaacctatagactggataattccatgtataggaatgtcaacaacagtgacagaggtcagagtggtggttatgtatgaggactgactgggagcctcatcttgatctgaatgatggttatatgggcgcatatatatgtaaacatttattgagctgtatatttcagacctgtgcactttacacaccatgttgcaataacattttaaacaatatgatcactatctatatgtagttttagtgctccatttggactggtctctggccactggatgtcagtgtttggagcagtgggcagcaggaaaagctggggaaggagtgggaaaacagaggagagagctatcacatgggcttcctagagaaaaataagcactttatgaagcttataagttcctttatgtacacagtagacaaagccttttaaagagatttgtccatacgggcactgaaataacatttttgtaaagtagccttctctatgttgattgcagatgtttctatctcagaatttaagtctacttgctttctcacacagcatcattatttccttattcctaataattttcatcacaaacatttcccagctctgtcccaatcaagttcttatttctctgaacggaattacaatttataaatgtaggtccacatgcagatatcttaataagtagtgaaataccagtgtagaaatacacaaatgagtgtggacacaccatagaaaagcagaaaaatacgagaaaaagtgcatgtacggagtatgggatgaactgatgcagttaaggaagacaactcacaaagcaactcacggctgggcaaagctgggaggctgaggcgggaggattgcttgaagccaggagtttgagactagcctgggcaccatactgataccttgtagctattaaaaaaaaattagctgggcatggtggctcatgcctgtagtctacttagtcagctgcttaggaggctgaggtacaaggattgcttgagcccaggaggtggaggttgcagtgagctgtgatcacgccactgcactccggccagggtgacagagtgagaccctgtctcacacaaaggcaactcatttgagctgaggcttggctatacttttaattgtccacatagaatagaggaaaaacaatgtttttcatcttttttaatcttccatttaccttttagtaagacaaattcttatctttatgtaaaactgtggaagagcagttacatagattgttgcagcttagattattttcaagaagtttaaattctacacataaggatacataccatttttaccagctatactttaaaatgccagtctttaaaaattcctctatgtgtatatgtggtttcttcttcttttcaaaaattcatgcctgtgaagtttttaggaatatttttcaaaactttagtactgaggcattaactgtttatgtgacacagcacctttaaatttctgtttttattcagccaaagaatgagaattattgtacattgctagtatttataatttcagcaaataggatagcagtatagtacctaaaataaactattaggaataactgaatgcctaccacagcaacagagctttaatgaggttaattgtcacatacatatccattccaacatagcagtgcacatttcacatgaccagcctcttatgtagttaaaaataaaactgcagttttaaaatgtcaagttcctcaaccttactggattttaaaacaaagcaaacaaaagaaacaaggattttctaatctatctataagcagaaatgtcagaaaataaagctacagtattccataaaacttaaaatttccttttctaagtcatgacatttctcttttgttctgttttctttttcttctaatattaagaaaatttaaaacgtaaatgaaaaaactgcttaatgtggcaaggaacaagaatgaaactagatttttttttttagtaaaggggcaaattgtataccaacatataaattaaaagtgttatgcaatgagaaacaataatggaaacagcataatactacatactatcccagtttcctgtgctctgaagaacagctgctatactaaatactaacttgacttatctgaagtattcaatactttctgataacccaagcagcattatattaatagttagaatactactacaaaatgtccttctacctctcccacaagaaatacaccaggaaacttaagcctgatgaataactactaagaatcttgtcttttaatacaagtctccttctagacacaaaatcctagctttttgtaatgtggttaaaaggagtaatggaaaagaaatgactgccaataaacatttcctattttgcactagggtgaagaaaccaagacacaaacatttggaagccactttagtttcttattccttttcaccctaatagtaggaaaatattaggcacctacttaattcacaaattcatgaaacagggtggacaacagccttgtgtaggggaagcatttggaatggtaatcaactacttaattacataacagggagctgggcatacaaagaaaagggctcagaagaaatatcttgaaaagtaagcaatatagaaggtgaggacagaagtgaggctaatcaaatgttcttagcaagatgttgcccccctgaaaatatgctcccccaataaaacacgtaaataactactcttaaggaaaatattttctctaaagaatgtcacaatttggagtgaagttacttaacaaaacagggaataaaacctttaatgttggctgtagcagttattttctttgggtagattatacttaaaatatttccttcatacatacttctgttaaaatttttttttcccattcttgagttttacaatgtctcctatccaaacttcaaatttcattagagccggctacatttgttttagtgccagatacaggtatcaagtgatgacagacacttacgtgaggtatacaatcaattaaagactggaaattggggtattatcatgtaagacatttgagaggccaaaagtcatataattttaagatacttcatgatgttacagtaataattcatctatataacaattattttgacataagtggcatatcagaatttaacttatttacttagatcttaaggaatattagatgtattctcacatgaacactcaaatcatgctattattatcagtcactgggagaacagccaaagtaatcaggcagtctaaggcacatatagacccaataatttagaaattttcaccattatgaggtaccctgtttttaataaatatgacaataacaggcgcttgaaatgggggcaaggtgaataagtatccagtcaattgtatacttttataaagtagtgtatttgagaacataaactgagatacaaaaggaatttccttactttaaaaaaagtgacttctatcttagtagatttctttaaaataacttaccttatatttaaaagttagtcatttacatacttaagaaatcaacagtaatctaaaaaaattaaaaggcagttttcttgggtaatgaacctgtgactccaagacagacaacaatgtggaaattaactcaggagactgactttctattctagtaattcagtggtttcttactttataaaggtttggaagaattaatgaatttctttttttcttaagacagggtctcgctctgttgcccaggctggagtgcagtggtgtgatcacagctcactgcagcctcgaactcctgggctcaagcgatcctccacatgttggcctcccatgagccaccatgctcagctaatttttatttttatttttggagagacagtgtctcactatgttgcccaggttggtctctaactcctggtttcaagtgattctccagtcttatactcccaaagcacaaggattacaggcctgagccaccacactcagccaatcaatttcaaaatgctaattaacctctttcagacacacgatctggcagagtaattagaagaaactggtctttcttaacatctttcctctattatcttccttttcttattcttgcctctcaatttgtcatatacagttacaaaatatatgaatcaggatttatgttggcatgaaaattatatgcaatacaatcagtaagtgaagaagggagggggtggtgtggctctagtcccaaagttaatgtcataaggagaaataatgtaagtatttgtatttcttagatcttcttctattttactcttaataccaaaaaaagagtcctatcatttaactttttatatattttgtagtgtttatttttgatgtgaccaaatgaaagctttctgaattttaaagtgcaattcactgtatgttaatacacagcctgcataggacctaactgcttcaaacttggcatcaaatgctgtctttttggtacttataagtagggtgtagataaagatatttgacaagagtgcaacagtgtttgttaaggtcttttcaaaagcccatttgagattattcaggcaggctcatcagttgacagctagcctatctttccttcttcctgttagtctgactgcctttttacccatttcatcgcctgtcgaatcctcctcaagaagaggcaagggaaataaatgaaaatgaaacccattaatttccaatattcacaatgaaatcaatcacatcatcaatctgtatactgtctgaccatttttctggatcattttctattagcaacatagtccctttagtttgtactttataactagtattttctaccaggatgcacagtttaaaaaatggcttgaagagccaaatatgttcccaatatgtccaatataattataaatatggtcattttcttgattactagagatctgtgcctgatggaatcacattttgtgaattagcaatagtttggtaataattcacacaaaatttcccataattactaggaataactgaaagctgggagtagaaaactttcattaactcaatattatgtagccatttgggccagcaaaaagtgtaaaatattattcccaataaccactgtggacaaaatgtgaacaggataatataatattttgaaaatattttaatatttgccattttttgcctgtgctattaatatatacattgatttagtaataaatatactactattacatagagtgcaatatttttagtattcataactggttgaaattaatgctgctataacctcaagaaaggaataaataaatatcatgtccaaattccaaactaatgctcaaaaggttatcattaacaaaaactataaaataaacatgttgggcattatctctttaagcatgattcctgtaaacaaagcaaaaaaatcacttttctcagtcctgacatttcacatgatggctttaaaagaaaatataacacacaaaccctatcacttcttttttttttttttttttttttgcatagggaacgaattaattgtatttttaaatgcagcaatcttttaatgaaatgttttcatcacatagtacttgttttctgtatgaattcagaacttttgagcaataaaagtgctctgcataagtttataaaatatgctttctggatttaaaatttaacagaaaaatttccaaacaagtcataggtatgattctaaaatattatgtacataatatatgactacaggaggaaattcctcactgtagtacaacacagtgtacaaatatgaagcacagtgtttagtttaatttccctttaggttttcctcacattggtgcataagtggctgactacatgacacaacatgccccattctacttgttgcatacaaagtagaagaggaatgtgaggacaaatttaaagtagaaaatgaaaataaatggcaaaaatacagtgcaaatgctttaaacagtgcactttataaaatagtttgctttattcatacttttttataaagtgcaatattacttaaaacagagagacatgtaccttaatattctgcaataaccattaaaacaaattgccaggaaagagcagtgcaaaattaaaaacatacacatagcttagcatgcatctcagatggatcccgaatacagagtatgggaccttgagttcttatatctttttttttttttttcactttttagaaaaagtttaataatagcaggttatcatcatatgtaaccataaaataaaaacaataagttaaaatcttctctcaagaaataagtatatgccacacataaaattcattacagaatcttttttgaaaacagacccctttctctgataaatcattgtttgaagggtgcaaatttcaaaaacccacattgtccacaaggcaaagcaaaaggtatcatcacagtatgagtcatttcttgttggcagacatctggaaaacctgtgacttacaagcagctcaaatctagccctaattaaatttacaggaacctttgctctttcaagaatagtcttgttggcatcatgctaggttgctaaaaagagtaatatgtgctctattcacagtaacattctctgtccagtgcttttgaatgaggataaccaaacaggttttcctgaaaaaaatcattaggaggcagattccaatgagaccaacgggaaacatttttaaaagcataaaagatcgcctcaggcatatgctgagggaataaaggtgcaatggatcactgatacactcctaccatgcctaagctactgagtccgagaactggaagagggtctccgggttattgctgtcggcaggattgctgggctgcagtgtcttggtgggtgtagttttaccgtgagaatgagaggaagaagaatgggaactctcactggaactgctgcgcgtctcggtactggtgctagtctttttcatttttcttctcttagccaaaggggccttatcaacattctgaaggcaaaacccctctctcttgtatttgttaaaggcgtggaaggttgctttcacacaggtatgcacggcagctccggaagatcctagaatatccggagtcatcagaggattggaggacagctgacttccatcttgtagccattcattgtacctcaagccagacattttaagccttttgtttggatctactgtgagaagtccttggatcaaatctttagcctcttgggatacattcttccaggcttctccttcaaaggagaaatctccctttttaattttcttcatgatttccaccgcgctggtacacgtcaaacttcggtcatgagattggaagggaacctgtcctgacaacattgtgtacaaaatgacgcccaagctccacaggtcacaggactcatcgtagccgttctgattcaagagctctggggcggcataatgaagggtgaagcatggagtcttcaggggctgattatccggtggctttagccgtgcaaatccaaaatcaattattttaatttccaaattgtcattttcatcggtgaacaataaattctcaggtttcagatccctgtgcaccactccaacatcatgcatgtggcttacagctgaaacaagcttcctcatgatgtagctggcttccgtctcactgaagtgcttctttttcttaatgcgctcaaacagttctcctccattcagaagttccatcactagaaacgtgtgaagctgatcatgaaaaacttcatgcaacttcacaatattggggtgtccttcacagagtttcagagctgttatttccttttgagtattggcttccatccttttgctgattattttgactgcaaaagcttggttactttttttatgcacacactttcgacaaattgaaaaactaccttctcccaggggtttgtccttcaaatctaggtcatagtgttgatagaatggagagtccttcatcattgcactcctggcaacatttgtcactccaggacgttcaactcccatgtgaaactgaagagggtctatgacagctgcattacgcttgaataggatggaaggagcaacaaaggaatagccctgaaacagcttctcagaactctggggcagggctgcgggagaataagtgggatccatttctgtgaactcttctgcaaagttactcacatctaattcatctcgaatgactggcttaaatggtgcaggcacttttttggcggctaaatcatcccaatttattttctgaaagaagagatgttctttgatttcatctgcatcacgtggaccacatcccaatctcttcttgggatctttcatcaaaagacgctgaattaggtctttcgctaaagcactcatttcttggggatatggaggctcactttttaatattctcctagatatctcagcttgggaatttttttctccatcaacagtgaaaggagatgctccagttagtaattcatacattagaacacccaaactccaccagtcaactgccttgtcatgtcctgaatctccccctctgacaatatctggtgccatgtattcaatagttccacaaaaggaatatgctctttcagtcttgtggagatgttcgagggcaagcacaatctctccaacataaatctgcacctcatgctctgtgaaacgctctctttgagaaagatgagtaaaaagttcaccaccatttatataatctaaaatgagatgaagtttggtttctgtctggaaagcataatgtaatgttaccaaaaatggcgactgcctaatgtgttccaggacttgtcgttctgtccttgtatgctctgtggttttggccttttgaacgattgttgcctttttcaaaactttcatggcatacagctttccagtatcatggccacttattttacgaactagaaatacttttccataagctccagttcctaggaccttcaggagctcaaaattttctattcccaccttctcagcatgtcctgtcaaattagcagtccgcagctcgtgcttgacagtgaggagctgctctcctccgtcgccgccgtccgcgctggtccccgcggcgccgccgctgctgccaccctcctcctccatcttctcctttttttccgatcccgcgggtcgctacgaggggaacccaggagacagcggacgcccgtcccctcgcagccgctgccgcggccccaggagtcggggtgcggcggctccagaactcggacgcaaagacgagtctctttcccgctctggccgcacggctcgctcctcgcctcctcccccttcggcgggcaccgctagtaccgc

SEQ ID NO: 14762 - RNA, 10285 nt, Homo sapiens
  source 1..10285: mol_type = other RNA
gctgggattacaggcatgagccacctcacccggccaataaagcttttagaagaatataagaatatcttcataaccttggtgtgaacatttattaaatacgacgcaaaagtattagcaattaaataaaagactggtatattggacttcataaaatttttggtcatcaaaggaaagcacttagaaagtagaaaagcaaactaaagagaagacatttatggtaaaatatcagacaaaaaccctcatatccataaaatataaaagactcctgcaagtcagtaagaaaaaaagacaacccaataaatatgaacaaatgacttgaacaggcacttaattgaggatagccaaatgactaataaaaatataaaaaggtgttccacacatcactacttatcaggaaaatacaccttaaaatctcagtgaaatacaaaatcaccagaatggttaaaaccacaatcaaatatacacatttgtcagagtggctaaactactagggctgatggtaccaagcactgatgaggatgtggaagaactagaacacttacacattattggtgggtatgtaaattggtacaaccattgttgaaaaccatttggtaatatcttctacagctaaatatatattcatcttatgactcagtagtttcactccttttttttgtctgtttttttgagacagggtctcactctatcgcccaggatggaatgtagtggtgcgatcaaggctcactgcagccagctgtttcacttttaagtggacacacaagagaaatgagtgtacgtgtccattaaaatatatgcacaagaatgcttatggctgctttaaacacaaaagctaaaaattacaaacaaccaaaatgtctatcagtgggagaatggataaattgtgatgtatttatctgatggaatactacagagcaacgaaaaagaacaaactactgttattgctacatgcaacaacatagatgcatttcacagacataatgctgatcaaattaaaccagacacaaaaacctatagactggataattccatgtataggaatgtcaacaacagtgacagaggtcagagtggtggttatgtatgaggactgactgggagcctcatcttgatctgaatgatggttatatgggcgcatatatatgtaaacatttattgagctgtatatttcagacctgtgcactttacacaccatgttgcaataacattttaaacaatatgatcactatctatatgtagttttagtgctccatttggactggtctctggccactggatgtcagtgtttggagcagtgggcagcaggaaaagctggggaaggagtgggaaaacagaggagagagctatcacatgggcttcctagagaaaaataagcactttatgaagcttataagttcctttatgtacacagtagacaaagccttttaaagagatttgtccatacgggcactgaaataacatttttgtaaagtagccttctctatgttgattgcagatgtttctatctcagaatttaagtctacttgctttctcacacagcatcattatttccttattcctaataattttcatcacaaacatttcccagctctgtcccaatcaagttcttatttctctgaacggaattacaatttataaatgtaggtccacatgcagatatcttaataagtagtgaaataccagtgtagaaatacacaaatgagtgtggacacaccatagaaaagcagaaaaatacgagaaaaagtgcatgtacggagtatgggatgaactgatgcagttaaggaagacaactcacaaagcaactcacggctgggcaaagctgggaggctgaggcgggaggattgcttgaagccaggagtttgagactagcctgggcaccatactgataccttgtagctattaaaaaaaaattagctgggcatggtggctcatgcctgtagtctacttagtcagctgcttaggaggctgaggtacaaggattgcttgagcccaggaggtggaggttgcagtgagctgtgatcacgccactgcactccggccagggtgacagagtgagaccctgtctcacacaaaggcaactcatttgagctgaggcttggctatacttttaattgtccacatagaatagaggaaaaacaatgtttttcatcttttttaatcttccatttaccttttagtaagacaaattcttatctttatgtaaaactgtggaagagcagttacatagattgttgcagcttagattattttcaagaagtttaaattctacacataaggatacataccatttttaccagctatactttaaaatgccagtctttaaaaattcctctatgtgtatatgtggtttcttcttcttttcaaaaattcatgcctgtgaagtttttaggaatatttttcaaaactttagtactgaggcattaactgtttatgtgacacagcacctttaaatttctgtttttattcagccaaagaatgagaattattgtacattgctagtatttataatttcagcaaataggatagcagtatagtacctaaaataaactattaggaataactgaatgcctaccacagcaacagagctttaatgaggttaattgtcacatacatatccattccaacatagcagtgcacatttcacatgaccagcctcttatgtagttaaaaataaaactgcagttttaaaatgtcaagttcctcaaccttactggattttaaaacaaagcaaacaaaagaaacaaggattttctaatctatctataagcagaaatgtcagaaaataaagctacagtattccataaaacttaaaatttccttttctaagtcatgacatttctcttttgttctgttttctttttcttctaatattaagaaaatttaaaacgtaaatgaaaaaactgcttaatgtggcaaggaacaagaatgaaactagatttttttttttagtaaaggggcaaattgtataccaacatataaattaaaagtgttatgcaatgagaaacaataatggaaacagcataatactacatactatcccagtttcctgtgctctgaagaacagctgctatactaaatactaacttgacttatctgaagtattcaatactttctgataacccaagcagcattatattaatagttagaatactactacaaaatgtccttctacctctcccacaagaaatacaccaggaaacttaagcctgatgaataactactaagaatcttgtcttttaatacaagtctccttctagacacaaaatcctagctttttgtaatgtggttaaaaggagtaatggaaaagaaatgactgccaataaacatttcctattttgcactagggtgaagaaaccaagacacaaacatttggaagccactttagtttcttattccttttcaccctaatagtaggaaaatattaggcacctacttaattcacaaattcatgaaacagggtggacaacagccttgtgtaggggaagcatttggaatggtaatcaactacttaattacataacagggagctgggcatacaaagaaaagggctcagaagaaatatcttgaaaagtaagcaatatagaaggtgaggacagaagtgaggctaatcaaatgttcttagcaagatgttgcccccctgaaaatatgctcccccaataaaacacgtaaataactactcttaaggaaaatattttctctaaagaatgtcacaatttggagtgaagttacttaacaaaacagggaataaaacctttaatgttggctgtagcagttattttctttgggtagattatacttaaaatatttccttcatacatacttctgttaaaatttttttttcccattcttgagttttacaatgtctcctatccaaacttcaaatttcattagagccggctacatttgttttagtgccagatacaggtatcaagtgatgacagacacttacgtgaggtatacaatcaattaaagactggaaattggggtattatcatgtaagacatttgagaggccaaaagtcatataattttaagatacttcatgatgttacagtaataattcatctatataacaattattttgacataagtggcatatcagaatttaacttatttacttagatcttaaggaatattagatgtattctcacatgaacactcaaatcatgctattattatcagtcactgggagaacagccaaagtaatcaggcagtctaaggcacatatagacccaataatttagaaattttcaccattatgaggtaccctgtttttaataaatatgacaataacaggcgcttgaaatgggggcaaggtgaataagtatccagtcaattgtatacttttataaagtagtgtatttgagaacataaactgagatacaaaaggaatttccttactttaaaaaaagtgacttctatcttagtagatttctttaaaataacttaccttatatttaaaagttagtcatttacatacttaagaaatcaacagtaatctaaaaaaattaaaaggcagttttcttgggtaatgaacctgtgactccaagacagacaacaatgtggaaattaactcaggagactgactttctattctagtaattcagtggtttcttactttataaaggtttggaagaattaatgaatttctttttttcttaagacagggtctcgctctgttgcccaggctggagtgcagtggtgtgatcacagctcactgcagcctcgaactcctgggctcaagcgatcctccacatgttggcctcccatgagccaccatgctcagctaatttttatttttatttttggagagacagtgtctcactatgttgcccaggttggtctctaactcctggtttcaagtgattctccagtcttatactcccaaagcacaaggattacaggcctgagccaccacactcagccaatcaatttcaaaatgctaattaacctctttcagacacacgatctggcagagtaattagaagaaactggtctttcttaacatctttcctctattatcttccttttcttattcttgcctctcaatttgtcatatacagttacaaaatatatgaatcaggatttatgttggcatgaaaattatatgcaatacaatcagtaagtgaagaagggagggggtggtgtggctctagtcccaaagttaatgtcataaggagaaataatgtaagtatttgtatttcttagatcttcttctattttactcttaataccaaaaaaagagtcctatcatttaactttttatatattttgtagtgtttatttttgatgtgaccaaatgaaagctttctgaattttaaagtgcaattcactgtatgttaatacacagcctgcataggacctaactgcttcaaacttggcatcaaatgctgtctttttggtacttataagtagggtgtagataaagatatttgacaagagtgcaacagtgtttgttaaggtcttttcaaaagcccatttgagattattcaggcaggctcatcagttgacagctagcctatctttccttcttcctgttagtctgactgcctttttacccatttcatcgcctgtcgaatcctcctcaagaagaggcaagggaaataaatgaaaatgaaacccattaatttccaatattcacaatgaaatcaatcacatcatcaatctgtatactgtctgaccatttttctggatcattttctattagcaacatagtccctttagtttgtactttataactagtattttctaccaggatgcacagtttaaaaaatggcttgaagagccaaatatgttcccaatatgtccaatataattataaatatggtcattttcttgattactagagatctgtgcctgatggaatcacattttgtgaattagcaatagtttggtaataattcacacaaaatttcccataattactaggaataactgaaagctgggagtagaaaactttcattaactcaatattatgtagccatttgggccagcaaaaagtgtaaaatattattcccaataaccactgtggacaaaatgtgaacaggataatataatattttgaaaatattttaatatttgccattttttgcctgtgctattaatatatacattgatttagtaataaatatactactattacatagagtgcaatatttttagtattcataactggttgaaattaatgctgctataacctcaagaaaggaataaataaatatcatgtccaaattccaaactaatgctcaaaaggttatcattaacaaaaactataaaataaacatgttgggcattatctctttaagcatgattcctgtaaacaaagcaaaaaaatcacttttctcagtcctgacatttcacatgatggctttaaaagaaaatataacacacaaaccctatcacttcttttttttttttttttttttttgcatagggaacgaattaattgtatttttaaatgcagcaatcttttaatgaaatgttttcatcacatagtacttgttttctgtatgaattcagaacttttgagcaataaaagtgctctgcataagtttataaaatatgctttctggatttaaaatttaacagaaaaatttccaaacaagtcataggtatgattctaaaatattatgtacataatatatgactacaggaggaaattcctcactgtagtacaacacagtgtacaaatatgaagcacagtgtttagtttaatttccctttaggttttcctcacattggtgcataagtggctgactacatgacacaacatgccccattctacttgttgcatacaaagtagaagaggaatgtgaggacaaatttaaagtagaaaatgaaaataaatggcaaaaatacagtgcaaatgctttaaacagtgcactttataaaatagtttgctttattcatacttttttataaagtgcaatattacttaaaacagagagacatgtaccttaatattctgcaataaccattaaaacaaattgccaggaaagagcagtgcaaaattaaaaacatacacatagcttagcatgcatctcagatggatcccgaatacagagtatgggaccttgagttcttatatctttttttttttttttcactttttagaaaaagtttaataatagcaggttatcatcatatgtaaccataaaataaaaacaataagttaaaatcttctctcaagaaataagtatatgccacacataaaattcattacagaatcttttttgaaaacagacccctttctctgataaatcattgtttgaagggtgcaaatttcaaaaacccacattgtccacaaggcaaagcaaaaggtatcatcacagtatgagtcatttcttgttggcagacatctggaaaacctgtgacttacaagcagctcaaatctagccctaattaaatttacaggaacctttgctctttcaagaatagtcttgttggcatcatgctaggttgctaaaaagagtaatatgtgctctattcacagtaacattctctgtccagtgcttttgaatgaggataaccaaacaggttttcctgaaaaaaatcattaggaggcagattccaatgagaccaacgggaaacatttttaaaagcataaaagatcgcctcaggcatatgctgagggaataaaggtgcaatggatcactgatacactcctaccatgcctaagctactgagtccgagaactggaagagggtctccgggttattgctgtcggcaggattgctgggctgcagtgtcttggtgggtgtagttttaccgtgagaatgagaggaagaagaatgggaactctcactggaactgctgcgcgtctcggtactggtgctagtctttttcatttttcttctcttagccaaaggggccttatcaacattctgaaggcaaaacccctctctcttgtatttgttaaaggcgtggaaggttgctttcacacaggtatgcacggcagctccggaagatcctagaatatccggagtcatcagaggattggaggacagctgacttccatcttgtagccattcattgtacctcaagccagacattttaagccttttgtttggatctactgtgagaagtccttggatcaaatctttagcctcttgggatacattcttccaggcttctccttcaaaggagaaatctccctttttaattttcttcatgatttccaccgcgctggtacacgtcaaacttcggtcatgagattggaagggaacctgtcctgacaacattgtgtacaaaatgacgcccaagctccacaggtcacaggactcatcgtagccgttctgattcaagagctctggggcggcataatgaagggtgaagcatggagtcttcaggggctgattatccggtggctttagccgtgcaaatccaaaatcaattattttaatttccaaattgtcattttcatcggtgaacaataaattctcaggtttcagatccctgtgcaccactccaacatcatgcatgtggcttacagctgaaacaagcttcctcatgatgtagctggcttccgtctcactgaagtgcttctttttcttaatgcgctcaaacagttctcctccattcagaagttccatcactagaaacgtgtgaagctgatcatgaaaaacttcatgcaacttcacaatattggggtgtccttcacagagtttcagagctgttatttccttttgagtattggcttccatccttttgctgattattttgactgcaaaagcttggttactttttttatgcacacactttcgacaaattgaaaaactaccttctcccaggggtttgtccttcaaatctaggtcatagtgttgatagaatggagagtccttcatcattgcactcctggcaacatttgtcactccaggacgttcaactcccatgtgaaactgaagagggtctatgacagctgcattacgcttgaataggatggaaggagcaacaaaggaatagccctgaaacagcttctcagaactctggggcagggctgcgggagaataagtgggatccatttctgtgaactcttctgcaaagttactcacatctaattcatctcgaatgactggcttaaatggtgcaggcacttttttggcggctaaatcatcccaatttattttctgaaagaagagatgttctttgatttcatctgcatcacgtggaccacatcccaatctcttcttgggatctttcatcaaaagacgctgaattaggtctttcgctaaagcactcatttcttggggatatggaggctcactttttaatattctcctagatatctcagcttgggaatttttttctccatcaacagtgaaaggagatgctccagttagtaattcatacattagaacacccaaactccaccagtcaactgccttgtcatgtcctgaatctccccctctgacaatatctggtgccatgtattcaatagttccacaaaaggaatatgctctttcagtttcatcagccacaaactccttactcagaccaaaatctgtcagcaccacatggccattagaatcaagtagaatattctcaagcttaatatcacgatatataatccccaacttgtggagatgttcgagggcaagcacaatctctccaacataaatctgcacctcatgctctgtgaaacgctctctttgagaaagatgagtaaaaagttcaccaccatttatataatctaaaatgagatgaagtttggtttctgtctggaaagcataatgtaatgttaccaaaaatggcgactgcctaatgtgttccaggacttgtcgttctgtccttgtatgctctgtggttttggccttttgaacgattgttgcctttttcaaaactttcatggcatacagctttccagtatcatggccacttattttacgaactagaaatacttttccataagctccagttcctaggaccttcaggagctcaaaattttctattcccaccttctcagcatgtcctgtcaaattagcagtccgcagctcgtgcttgacagtgaggagctgctctcctccgtcgccgccgtccgcgctggtccccgcggcgccgccgctgctgccaccctcctcctccatcttctcctttttttccgatcccgcgggtcgctacgaggggaacccaggagacagcggacgcccgtcccctcgcagccgctgccgcggccccaggagtcggggtgcggcggctccagaactcggacgcaaagacgagtctctttcccgctctggccgcacggctcgctcctcgcctcctcccccttcggcgggcaccgctagtaccgc

SEQ ID NO: 14763 - RNA, 10425 nt, Homo sapiens
  source 1..10425: mol_type = other RNA
gctgggattacaggcatgagccacctcacccggccaataaagcttttagaagaatataagaatatcttcataaccttggtgtgaacatttattaaatacgacgcaaaagtattagcaattaaataaaagactggtatattggacttcataaaatttttggtcatcaaaggaaagcacttagaaagtagaaaagcaaactaaagagaagacatttatggtaaaatatcagacaaaaaccctcatatccataaaatataaaagactcctgcaagtcagtaagaaaaaaagacaacccaataaatatgaacaaatgacttgaacaggcacttaattgaggatagccaaatgactaataaaaatataaaaaggtgttccacacatcactacttatcaggaaaatacaccttaaaatctcagtgaaatacaaaatcaccagaatggttaaaaccacaatcaaatatacacatttgtcagagtggctaaactactagggctgatggtaccaagcactgatgaggatgtggaagaactagaacacttacacattattggtgggtatgtaaattggtacaaccattgttgaaaaccatttggtaatatcttctacagctaaatatatattcatcttatgactcagtagtttcactccttttttttgtctgtttttttgagacagggtctcactctatcgcccaggatggaatgtagtggtgcgatcaaggctcactgcagccagctgtttcacttttaagtggacacacaagagaaatgagtgtacgtgtccattaaaatatatgcacaagaatgcttatggctgctttaaacacaaaagctaaaaattacaaacaaccaaaatgtctatcagtgggagaatggataaattgtgatgtatttatctgatggaatactacagagcaacgaaaaagaacaaactactgttattgctacatgcaacaacatagatgcatttcacagacataatgctgatcaaattaaaccagacacaaaaacctatagactggataattccatgtataggaatgtcaacaacagtgacagaggtcagagtggtggttatgtatgaggactgactgggagcctcatcttgatctgaatgatggttatatgggcgcatatatatgtaaacatttattgagctgtatatttcagacctgtgcactttacacaccatgttgcaataacattttaaacaatatgatcactatctatatgtagttttagtgctccatttggactggtctctggccactggatgtcagtgtttggagcagtgggcagcaggaaaagctggggaaggagtgggaaaacagaggagagagctatcacatgggcttcctagagaaaaataagcactttatgaagcttataagttcctttatgtacacagtagacaaagccttttaaagagatttgtccatacgggcactgaaataacatttttgtaaagtagccttctctatgttgattgcagatgtttctatctcagaatttaagtctacttgctttctcacacagcatcattatttccttattcctaataattttcatcacaaacatttcccagctctgtcccaatcaagttcttatttctctgaacggaattacaatttataaatgtaggtccacatgcagatatcttaataagtagtgaaataccagtgtagaaatacacaaatgagtgtggacacaccatagaaaagcagaaaaatacgagaaaaagtgcatgtacggagtatgggatgaactgatgcagttaaggaagacaactcacaaagcaactcacggctgggcaaagctgggaggctgaggcgggaggattgcttgaagccaggagtttgagactagcctgggcaccatactgataccttgtagctattaaaaaaaaattagctgggcatggtggctcatgcctgtagtctacttagtcagctgcttaggaggctgaggtacaaggattgcttgagcccaggaggtggaggttgcagtgagctgtgatcacgccactgcactccggccagggtgacagagtgagaccctgtctcacacaaaggcaactcatttgagctgaggcttggctatacttttaattgtccacatagaatagaggaaaaacaatgtttttcatcttttttaatcttccatttaccttttagtaagacaaattcttatctttatgtaaaactgtggaagagcagttacatagattgttgcagcttagattattttcaagaagtttaaattctacacataaggatacataccatttttaccagctatactttaaaatgccagtctttaaaaattcctctatgtgtatatgtggtttcttcttcttttcaaaaattcatgcctgtgaagtttttaggaatatttttcaaaactttagtactgaggcattaactgtttatgtgacacagcacctttaaatttctgtttttattcagccaaagaatgagaattattgtacattgctagtatttataatttcagcaaataggatagcagtatagtacctaaaataaactattaggaataactgaatgcctaccacagcaacagagctttaatgaggttaattgtcacatacatatccattccaacatagcagtgcacatttcacatgaccagcctcttatgtagttaaaaataaaactgcagttttaaaatgtcaagttcctcaaccttactggattttaaaacaaagcaaacaaaagaaacaaggattttctaatctatctataagcagaaatgtcagaaaataaagctacagtattccataaaacttaaaatttccttttctaagtcatgacatttctcttttgttctgttttctttttcttctaatattaagaaaatttaaaacgtaaatgaaaaaactgcttaatgtggcaaggaacaagaatgaaactagatttttttttttagtaaaggggcaaattgtataccaacatataaattaaaagtgttatgcaatgagaaacaataatggaaacagcataatactacatactatcccagtttcctgtgctctgaagaacagctgctatactaaatactaacttgacttatctgaagtattcaatactttctgataacccaagcagcattatattaatagttagaatactactacaaaatgtccttctacctctcccacaagaaatacaccaggaaacttaagcctgatgaataactactaagaatcttgtcttttaatacaagtctccttctagacacaaaatcctagctttttgtaatgtggttaaaaggagtaatggaaaagaaatgactgccaataaacatttcctattttgcactagggtgaagaaaccaagacacaaacatttggaagccactttagtttcttattccttttcaccctaatagtaggaaaatattaggcacctacttaattcacaaattcatgaaacagggtggacaacagccttgtgtaggggaagcatttggaatggtaatcaactacttaattacataacagggagctgggcatacaaagaaaagggctcagaagaaatatcttgaaaagtaagcaatatagaaggtgaggacagaagtgaggctaatcaaatgttcttagcaagatgttgcccccctgaaaatatgctcccccaataaaacacgtaaataactactcttaaggaaaatattttctctaaagaatgtcacaatttggagtgaagttacttaacaaaacagggaataaaacctttaatgttggctgtagcagttattttctttgggtagattatacttaaaatatttccttcatacatacttctgttaaaatttttttttcccattcttgagttttacaatgtctcctatccaaacttcaaatttcattagagccggctacatttgttttagtgccagatacaggtatcaagtgatgacagacacttacgtgaggtatacaatcaattaaagactggaaattggggtattatcatgtaagacatttgagaggccaaaagtcatataattttaagatacttcatgatgttacagtaataattcatctatataacaattattttgacataagtggcatatcagaatttaacttatttacttagatcttaaggaatattagatgtattctcacatgaacactcaaatcatgctattattatcagtcactgggagaacagccaaagtaatcaggcagtctaaggcacatatagacccaataatttagaaattttcaccattatgaggtaccctgtttttaataaatatgacaataacaggcgcttgaaatgggggcaaggtgaataagtatccagtcaattgtatacttttataaagtagtgtatttgagaacataaactgagatacaaaaggaatttccttactttaaaaaaagtgacttctatcttagtagatttctttaaaataacttaccttatatttaaaagttagtcatttacatacttaagaaatcaacagtaatctaaaaaaattaaaaggcagttttcttgggtaatgaacctgtgactccaagacagacaacaatgtggaaattaactcaggagactgactttctattctagtaattcagtggtttcttactttataaaggtttggaagaattaatgaatttctttttttcttaagacagggtctcgctctgttgcccaggctggagtgcagtggtgtgatcacagctcactgcagcctcgaactcctgggctcaagcgatcctccacatgttggcctcccatgagccaccatgctcagctaatttttatttttatttttggagagacagtgtctcactatgttgcccaggttggtctctaactcctggtttcaagtgattctccagtcttatactcccaaagcacaaggattacaggcctgagccaccacactcagccaatcaatttcaaaatgctaattaacctctttcagacacacgatctggcagagtaattagaagaaactggtctttcttaacatctttcctctattatcttccttttcttattcttgcctctcaatttgtcatatacagttacaaaatatatgaatcaggatttatgttggcatgaaaattatatgcaatacaatcagtaagtgaagaagggagggggtggtgtggctctagtcccaaagttaatgtcataaggagaaataatgtaagtatttgtatttcttagatcttcttctattttactcttaataccaaaaaaagagtcctatcatttaactttttatatattttgtagtgtttatttttgatgtgaccaaatgaaagctttctgaattttaaagtgcaattcactgtatgttaatacacagcctgcataggacctaactgcttcaaacttggcatcaaatgctgtctttttggtacttataagtagggtgtagataaagatatttgacaagagtgcaacagtgtttgttaaggtcttttcaaaagcccatttgagattattcaggcaggctcatcagttgacagctagcctatctttccttcttcctgttagtctgactgcctttttacccatttcatcgcctgtcgaatcctcctcaagaagaggcaagggaaataaatgaaaatgaaacccattaatttccaatattcacaatgaaatcaatcacatcatcaatctgtatactgtctgaccatttttctggatcattttctattagcaacatagtccctttagtttgtactttataactagtattttctaccaggatgcacagtttaaaaaatggcttgaagagccaaatatgttcccaatatgtccaatataattataaatatggtcattttcttgattactagagatctgtgcctgatggaatcacattttgtgaattagcaatagtttggtaataattcacacaaaatttcccataattactaggaataactgaaagctgggagtagaaaactttcattaactcaatattatgtagccatttgggccagcaaaaagtgtaaaatattattcccaataaccactgtggacaaaatgtgaacaggataatataatattttgaaaatattttaatatttgccattttttgcctgtgctattaatatatacattgatttagtaataaatatactactattacatagagtgcaatatttttagtattcataactggttgaaattaatgctgctataacctcaagaaaggaataaataaatatcatgtccaaattccaaactaatgctcaaaaggttatcattaacaaaaactataaaataaacatgttgggcattatctctttaagcatgattcctgtaaacaaagcaaaaaaatcacttttctcagtcctgacatttcacatgatggctttaaaagaaaatataacacacaaaccctatcacttcttttttttttttttttttttttgcatagggaacgaattaattgtatttttaaatgcagcaatcttttaatgaaatgttttcatcacatagtacttgttttctgtatgaattcagaacttttgagcaataaaagtgctctgcataagtttataaaatatgctttctggatttaaaatttaacagaaaaatttccaaacaagtcataggtatgattctaaaatattatgtacataatatatgactacaggaggaaattcctcactgtagtacaacacagtgtacaaatatgaagcacagtgtttagtttaatttccctttaggttttcctcacattggtgcataagtggctgactacatgacacaacatgccccattctacttgttgcatacaaagtagaagaggaatgtgaggacaaatttaaagtagaaaatgaaaataaatggcaaaaatacagtgcaaatgctttaaacagtgcactttataaaatagtttgctttattcatacttttttataaagtgcaatattacttaaaacagagagacatgtaccttaatattctgcaataaccattaaaacaaattgccaggaaagagcagtgcaaaattaaaaacatacacatagcttagcatgcatctcagatggatcccgaatacagagtatgggaccttgagttcttatatctttttttttttttttcactttttagaaaaagtttaataatagcaggttatcatcatatgtaaccataaaataaaaacaataagttaaaatcttctctcaagaaataagtatatgccacacataaaattcattacagaatcttttttgaaaacagacccctttctctgataaatcattgtttgaagggtgcaaatttcaaaaacccacattgtccacaaggcaaagcaaaaggtatcatcacagtatgagtcatttcttgttggcagacatctggaaaacctgtgacttacaagcagctcaaatctagccctaattaaatttacaggaacctttgctctttcaagaatagtcttgttggcatcatgctaggttgctaaaaagagtaatatgtgctctattcacagtaacattctctgtccagtgcttttgaatgaggataaccaaacaggttttcctgaaaaaaatcattaggaggcagattccaatgagaccaacgggaaacatttttaaaagcataaaagatcgcctcaggcatatgctgagggaataaaggtgcaatggatcactgatacactcctaccatgcctaagctactgagtccgagaactggaagagggtctccgggttattgctgtcggcaggattgctgggctgcagtgtcttggtgggtgtagttttaccgtgagaatgagaggaagaagaatgggaactctcactggaactgctgcgcgtctcggtactggtgctagtctttttcatttttcttctcttagccaaaggggccttatcaacattctgaaggcaaaacccctctctcttgtatttgttaaaggcgtggaaggttgctttcacacaggtatgcacggcagctccggaagatcctagaatatccggagtcatcagaggattggaggacagctgacttccatcttgtagccattcattgtacctcaagccagacattttaagccttttgtttggatctactgtgagaagtccttggatcaaatctttagcctcttgggatacattcttccaggcttctccttcaaaggagaaatctccctttttaattttcttcatgatttccaccgcgctggtacacgtcaaacttcggtcatgagattggaagggaacctgtcctgacaacattgtgtacaaaatgacgcccaagctccacaggtcacaggactcatcgtagccgttctgattcaagagctctggggcggcataatgaagggtgaagcatggagtcttcaggggctgattatccggtggctttagccgtgcaaatccaaaatcaattattttaatttccaaattgtcattttcatcggtgaacaataaattctcaggtttcagatccctgtgcaccactccaacatcatgcatgtggcttacagctgaaacaagcttcctcatgatgtagctggcttccgtctcactgaagtgcttctttttcttaatgcgctcaaacagttctcctccattcagaagttccatcactagaaacgtgtgaagctgatcatgaaaaacttcatgcaacttcacaatattggggtgtccttcacagagtttcagagctgttatttccttttgagtattggcttccatccttttgctgattattttgactgcaaaagcttggttactttttttatgcacacactttcgacaaattgaaaaactaccttctcccaggggtttgtccttcaaatctaggtcatagtgttgatagaatggagagtccttcatcattgcactcctggcaacatttgtcactccaggacgttcaactcccatgtgaaactgaagagggtctatgacagctgcattacgcttgaataggatggaaggagcaacaaaggaatagccctgaaacagcttctcagaactctggggcagggctgcgggagaataagtgggatccatttctgtgaactcttctgcaaagttactcacatctaattcatctcgaatgactggcttaaatggtgcaggcacttttttggcggctaaatcatcccaatttattttctgaaagaagagatgttctttgatttcatctgcatcacgtggaccacatcccaatctcttcttgggatctttcatcaaaagacgctgaattaggtctttcgctaaagcactcatttcttggggatatggaggctcactttttaatattctcctagatatctcagcttgggaatttttttctccatcaacagtgaaaggagatgctccagttagtaattcatacattagaacacccaaactccaccagtcaactgccttgtcatgtcctgaatctccccctctgacaatatctggtgccatgtattcaatagttccacaaaaggaatatgctctttcagtttcatcagccacaaactccttactcagaccaaaatctgtcagcaccacatggccattagaatcaagtagaatattctcaagcttaatatcacgatatataatccccaacttgtggagatgttcgagggcaagcacaatctctccaacataaatctgcacctcatgctctgtgaaacgctctctttgagaaagatgagtaaaaagttcaccaccatttatataatctaaaatgagatgaagtttggtttctgtctggaaagcataatgtaatgttaccaaaaatggcgactgcctaatgtgttccaggacttgtcgttctgtccttgtatgctctgtggttttggccttttgaacgattgttgcctttttcaaaactttcatggcatacagctttccagtatcatggccacttattttacgaactagaaatacttttccataagctccagttcctaggaccttcaggagctcaaaattttctattcccaccttctcagcatgtcctgtcaaattagctgggtatggtagtgggtgcctgtaatcccagccacttgggaggctgaggcaggagaatcacttgaacccaggaggcggaggttatagtgagccgagatcagcaccacactccagcctgggcaacagagtagactcgtctcagtccgcagctcgtgcttgacagtgaggagctgctctcctccgtcgccgccgtccgcgctggtccccgcggcgccgccgctgctgccaccctcctcctccatcttctcctttttttccgatcccgcgggtcgctacgaggggaacccaggagacagcggacgcccgtcccctcgcagccgctgccgcggccccaggagtcggggtgcggcggctccagaactcggacgcaaagacgagtctctttcccgctctggccgcacggctcgctcctcgcctcctcccccttcggcgggcaccgctagtaccgc

SEQ ID NO: 14764 - RNA, 10082 nt, Homo sapiens
  source 1..10082: mol_type = other RNA
gctgggattacaggcatgagccacctcacccggccaataaagcttttagaagaatataagaatatcttcataaccttggtgtgaacatttattaaatacgacgcaaaagtattagcaattaaataaaagactggtatattggacttcataaaatttttggtcatcaaaggaaagcacttagaaagtagaaaagcaaactaaagagaagacatttatggtaaaatatcagacaaaaaccctcatatccataaaatataaaagactcctgcaagtcagtaagaaaaaaagacaacccaataaatatgaacaaatgacttgaacaggcacttaattgaggatagccaaatgactaataaaaatataaaaaggtgttccacacatcactacttatcaggaaaatacaccttaaaatctcagtgaaatacaaaatcaccagaatggttaaaaccacaatcaaatatacacatttgtcagagtggctaaactactagggctgatggtaccaagcactgatgaggatgtggaagaactagaacacttacacattattggtgggtatgtaaattggtacaaccattgttgaaaaccatttggtaatatcttctacagctaaatatatattcatcttatgactcagtagtttcactccttttttttgtctgtttttttgagacagggtctcactctatcgcccaggatggaatgtagtggtgcgatcaaggctcactgcagccagctgtttcacttttaagtggacacacaagagaaatgagtgtacgtgtccattaaaatatatgcacaagaatgcttatggctgctttaaacacaaaagctaaaaattacaaacaaccaaaatgtctatcagtgggagaatggataaattgtgatgtatttatctgatggaatactacagagcaacgaaaaagaacaaactactgttattgctacatgcaacaacatagatgcatttcacagacataatgctgatcaaattaaaccagacacaaaaacctatagactggataattccatgtataggaatgtcaacaacagtgacagaggtcagagtggtggttatgtatgaggactgactgggagcctcatcttgatctgaatgatggttatatgggcgcatatatatgtaaacatttattgagctgtatatttcagacctgtgcactttacacaccatgttgcaataacattttaaacaatatgatcactatctatatgtagttttagtgctccatttggactggtctctggccactggatgtcagtgtttggagcagtgggcagcaggaaaagctggggaaggagtgggaaaacagaggagagagctatcacatgggcttcctagagaaaaataagcactttatgaagcttataagttcctttatgtacacagtagacaaagccttttaaagagatttgtccatacgggcactgaaataacatttttgtaaagtagccttctctatgttgattgcagatgtttctatctcagaatttaagtctacttgctttctcacacagcatcattatttccttattcctaataattttcatcacaaacatttcccagctctgtcccaatcaagttcttatttctctgaacggaattacaatttataaatgtaggtccacatgcagatatcttaataagtagtgaaataccagtgtagaaatacacaaatgagtgtggacacaccatagaaaagcagaaaaatacgagaaaaagtgcatgtacggagtatgggatgaactgatgcagttaaggaagacaactcacaaagcaactcacggctgggcaaagctgggaggctgaggcgggaggattgcttgaagccaggagtttgagactagcctgggcaccatactgataccttgtagctattaaaaaaaaattagctgggcatggtggctcatgcctgtagtctacttagtcagctgcttaggaggctgaggtacaaggattgcttgagcccaggaggtggaggttgcagtgagctgtgatcacgccactgcactccggccagggtgacagagtgagaccctgtctcacacaaaggcaactcatttgagctgaggcttggctatacttttaattgtccacatagaatagaggaaaaacaatgtttttcatcttttttaatcttccatttaccttttagtaagacaaattcttatctttatgtaaaactgtggaagagcagttacatagattgttgcagcttagattattttcaagaagtttaaattctacacataaggatacataccatttttaccagctatactttaaaatgccagtctttaaaaattcctctatgtgtatatgtggtttcttcttcttttcaaaaattcatgcctgtgaagtttttaggaatatttttcaaaactttagtactgaggcattaactgtttatgtgacacagcacctttaaatttctgtttttattcagccaaagaatgagaattattgtacattgctagtatttataatttcagcaaataggatagcagtatagtacctaaaataaactattaggaataactgaatgcctaccacagcaacagagctttaatgaggttaattgtcacatacatatccattccaacatagcagtgcacatttcacatgaccagcctcttatgtagttaaaaataaaactgcagttttaaaatgtcaagttcctcaaccttactggattttaaaacaaagcaaacaaaagaaacaaggattttctaatctatctataagcagaaatgtcagaaaataaagctacagtattccataaaacttaaaatttccttttctaagtcatgacatttctcttttgttctgttttctttttcttctaatattaagaaaatttaaaacgtaaatgaaaaaactgcttaatgtggcaaggaacaagaatgaaactagatttttttttttagtaaaggggcaaattgtataccaacatataaattaaaagtgttatgcaatgagaaacaataatggaaacagcataatactacatactatcccagtttcctgtgctctgaagaacagctgctatactaaatactaacttgacttatctgaagtattcaatactttctgataacccaagcagcattatattaatagttagaatactactacaaaatgtccttctacctctcccacaagaaatacaccaggaaacttaagcctgatgaataactactaagaatcttgtcttttaatacaagtctccttctagacacaaaatcctagctttttgtaatgtggttaaaaggagtaatggaaaagaaatgactgccaataaacatttcctattttgcactagggtgaagaaaccaagacacaaacatttggaagccactttagtttcttattccttttcaccctaatagtaggaaaatattaggcacctacttaattcacaaattcatgaaacagggtggacaacagccttgtgtaggggaagcatttggaatggtaatcaactacttaattacataacagggagctgggcatacaaagaaaagggctcagaagaaatatcttgaaaagtaagcaatatagaaggtgaggacagaagtgaggctaatcaaatgttcttagcaagatgttgcccccctgaaaatatgctcccccaataaaacacgtaaataactactcttaaggaaaatattttctctaaagaatgtcacaatttggagtgaagttacttaacaaaacagggaataaaacctttaatgttggctgtagcagttattttctttgggtagattatacttaaaatatttccttcatacatacttctgttaaaatttttttttcccattcttgagttttacaatgtctcctatccaaacttcaaatttcattagagccggctacatttgttttagtgccagatacaggtatcaagtgatgacagacacttacgtgaggtatacaatcaattaaagactggaaattggggtattatcatgtaagacatttgagaggccaaaagtcatataattttaagatacttcatgatgttacagtaataattcatctatataacaattattttgacataagtggcatatcagaatttaacttatttacttagatcttaaggaatattagatgtattctcacatgaacactcaaatcatgctattattatcagtcactgggagaacagccaaagtaatcaggcagtctaaggcacatatagacccaataatttagaaattttcaccattatgaggtaccctgtttttaataaatatgacaataacaggcgcttgaaatgggggcaaggtgaataagtatccagtcaattgtatacttttataaagtagtgtatttgagaacataaactgagatacaaaaggaatttccttactttaaaaaaagtgacttctatcttagtagatttctttaaaataacttaccttatatttaaaagttagtcatttacatacttaagaaatcaacagtaatctaaaaaaattaaaaggcagttttcttgggtaatgaacctgtgactccaagacagacaacaatgtggaaattaactcaggagactgactttctattctagtaattcagtggtttcttactttataaaggtttggaagaattaatgaatttctttttttcttaagacagggtctcgctctgttgcccaggctggagtgcagtggtgtgatcacagctcactgcagcctcgaactcctgggctcaagcgatcctccacatgttggcctcccatgagccaccatgctcagctaatttttatttttatttttggagagacagtgtctcactatgttgcccaggttggtctctaactcctggtttcaagtgattctccagtcttatactcccaaagcacaaggattacaggcctgagccaccacactcagccaatcaatttcaaaatgctaattaacctctttcagacacacgatctggcagagtaattagaagaaactggtctttcttaacatctttcctctattatcttccttttcttattcttgcctctcaatttgtcatatacagttacaaaatatatgaatcaggatttatgttggcatgaaaattatatgcaatacaatcagtaagtgaagaagggagggggtggtgtggctctagtcccaaagttaatgtcataaggagaaataatgtaagtatttgtatttcttagatcttcttctattttactcttaataccaaaaaaagagtcctatcatttaactttttatatattttgtagtgtttatttttgatgtgaccaaatgaaagctttctgaattttaaagtgcaattcactgtatgttaatacacagcctgcataggacctaactgcttcaaacttggcatcaaatgctgtctttttggtacttataagtagggtgtagataaagatatttgacaagagtgcaacagtgtttgttaaggtcttttcaaaagcccatttgagattattcaggcaggctcatcagttgacagctagcctatctttccttcttcctgttagtctgactgcctttttacccatttcatcgcctgtcgaatcctcctcaagaagaggcaagggaaataaatgaaaatgaaacccattaatttccaatattcacaatgaaatcaatcacatcatcaatctgtatactgtctgaccatttttctggatcattttctattagcaacatagtccctttagtttgtactttataactagtattttctaccaggatgcacagtttaaaaaatggcttgaagagccaaatatgttcccaatatgtccaatataattataaatatggtcattttcttgattactagagatctgtgcctgatggaatcacattttgtgaattagcaatagtttggtaataattcacacaaaatttcccataattactaggaataactgaaagctgggagtagaaaactttcattaactcaatattatgtagccatttgggccagcaaaaagtgtaaaatattattcccaataaccactgtggacaaaatgtgaacaggataatataatattttgaaaatattttaatatttgccattttttgcctgtgctattaatatatacattgatttagtaataaatatactactattacatagagtgcaatatttttagtattcataactggttgaaattaatgctgctataacctcaagaaaggaataaataaatatcatgtccaaattccaaactaatgctcaaaaggttatcattaacaaaaactataaaataaacatgttgggcattatctctttaagcatgattcctgtaaacaaagcaaaaaaatcacttttctcagtcctgacatttcacatgatggctttaaaagaaaatataacacacaaaccctatcacttcttttttttttttttttttttttgcatagggaacgaattaattgtatttttaaatgcagcaatcttttaatgaaatgttttcatcacatagtacttgttttctgtatgaattcagaacttttgagcaataaaagtgctctgcataagtttataaaatatgctttctggatttaaaatttaacagaaaaatttccaaacaagtcataggtatgattctaaaatattatgtacataatatatgactacaggaggaaattcctcactgtagtacaacacagtgtacaaatatgaagcacagtgtttagtttaatttccctttaggttttcctcacattggtgcataagtggctgactacatgacacaacatgccccattctacttgttgcatacaaagtagaagaggaatgtgaggacaaatttaaagtagaaaatgaaaataaatggcaaaaatacagtgcaaatgctttaaacagtgcactttataaaatagtttgctttattcatacttttttataaagtgcaatattacttaaaacagagagacatgtaccttaatattctgcaataaccattaaaacaaattgccaggaaagagcagtgcaaaattaaaaacatacacatagcttagcatgcatctcagatggatcccgaatacagagtatgggaccttgagttcttatatctttttttttttttttcactttttagaaaaagtttaataatagcaggttatcatcatatgtaaccataaaataaaaacaataagttaaaatcttctctcaagaaataagtatatgccacacataaaattcattacagaatcttttttgaaaacagacccctttctctgataaatcattgtttgaagggtgcaaatttcaaaaacccacattgtccacaaggcaaagcaaaaggtatcatcacagtatgagtcatttcttgttggcagacatctggaaaacctgtgacttacaagcagctcaaatctagccctaattaaatttacaggaacctttgctctttcaagaatagtcttgttggcatcatgctaggttgctaaaaagagtaatatgtgctctattcacagtaacattctctgtccagtgcttttgaatgaggataaccaaacaggttttcctgaaaaaaatcattaggaggcagattccaatgagaccaacgggaaacatttttaaaagcataaaagatcgcctcaggcatatgctgagggaataaaggtgcaatggatcactgatacactcctaccatgcctaagctactgagtccgagaactggaagagggtctccgggttattgctgtcggcaggattgctgggctgcagtgtcttggtgggtgtagttttaccgtgagaatgagaggaagaagaatgggaactctcactggaactgctgcgcgtctcggtactggtgctagtctttttcatttttcttctcttagccaaaggggccttatcaacattctgaaggcaaaacccctctctcttgtatttgttaaaggcgtggaaggttgctttcacacaggtatgcacggcagctccggaagatcctagaatatccggagtcatcagaggattggaggacagctgacttccatcttgtagccattcattgtacctcaagccagacattttaagccttttgtttggatctactgtgagaagtccttggatcaaatctttagcctcttgggatacattcttccaggcttctccttcaaaggagaaatctccctttttaattttcttcatgatttccaccgcgctggtacacgtcaaacttcggtcatgagattggaagggaacctgtcctgacaacattgtgtacaaaatgacgcccaagctccacaggtcacaggactcatcgtagccgttctgattcaagagctctggggcggcataatgaagggtgaagcatggagtcttcaggggctgattatccggtggctttagccgtgcaaatccaaaatcaattattttaatttccaaattgtcattttcatcggtgaacaataaattctcaggtttcagatccctgtgcaccactccaacatcatgcatgtggcttacagctgaaacaagcttcctcatgatgtagctggcttccgtctcactgaagtgcttctttttcttaatgcgctcaaacagttctcctccattcagaagttccatcactagaaacgtgtgaagctgatcatgaaaaacttcatgcaacttcacaatattggggtgtccttcacagagtttcagagctgttatttccttttgagtattggcttccatccttttgctgattattttgactgcaaaagcttggttactttttttatgcacacactttcgacaaattgaaaaactaccttctcccaggggtttgtccttcaaatctaggtcatagtgttgatagaatggagagtccttcatcattgcactcctggcaacatttgtcactccaggacgttcaactcccatgtgaaactgaagagggtctatgacagctgcattacgcttgaataggatggaaggagcaacaaaggaatagccctgaaacagcttctcagaactctggggcagggctgcgggagaataagtgggatccatttctgtgaactcttctgcaaagttactcacatctaattcatctcgaatgactggcttaaatggtgcaggcacttttttggcggctaaatcatcccaatttattttctgaaagaagagatgttctttgatttcatctgcatcacgtggaccacatcccaatctcttcttgggatctttcatcaaaagacgctgaattaggtctttcgctaaagcactcatttcttggggatatggaggctcactttttaatattctcctagatatctcagcttgggaatttttttctccatcaacagtgaaaggagatgctccagttagtaattcatacattagaacacccaaactccaccagtcaactgccttgtcatgtcctgaatctccccctctgacaatatctggtgccatgtattcaatagttccacaaaaggaatatgctctttcagtttcatcagccacaaactccttactcagaccaaaatctgtcagcaccacatggccattagaatcaagtagaatattctcaagcttaatatcacgatatataatccccaacttgtggagatgttcgagggcaagcacaatctctccaacataaatctgcacctcatgctctgtgaaacgctctctttgagaaagatgagtaaaaagttcaccaccatttatataatctaaaatgagatgaagtttggtttctgtctggaaagcataatgtaatgttaccaaaaatggcgactgcctaatgtgttccaggacttgtcgttctgtccttgtatgctctgtggttttggccttttgaacgattgttgcctttttcaaaactttcatggcatacagctttccagtatcatggccacttattttacgaactagaaatacttttccataagctccagttcctaggaccttcaggagctcaaaattttctattcccaccttctcagcatgtcctgtcaaattagctgtgcgggaagggggagcagcgacatcctcggaggtgcgtgccacgggcagcggtcggcggctgcgctggccccgatgcctggtgcccgccgctcattcccgggct

SEQ ID NO: 14765 - RNA, 10066 nt, Homo sapiens
  source 1..10066: mol_type = other RNA
gctgggattacaggcatgagccacctcacccggccaataaagcttttagaagaatataagaatatcttcataaccttggtgtgaacatttattaaatacgacgcaaaagtattagcaattaaataaaagactggtatattggacttcataaaatttttggtcatcaaaggaaagcacttagaaagtagaaaagcaaactaaagagaagacatttatggtaaaatatcagacaaaaaccctcatatccataaaatataaaagactcctgcaagtcagtaagaaaaaaagacaacccaataaatatgaacaaatgacttgaacaggcacttaattgaggatagccaaatgactaataaaaatataaaaaggtgttccacacatcactacttatcaggaaaatacaccttaaaatctcagtgaaatacaaaatcaccagaatggttaaaaccacaatcaaatatacacatttgtcagagtggctaaactactagggctgatggtaccaagcactgatgaggatgtggaagaactagaacacttacacattattggtgggtatgtaaattggtacaaccattgttgaaaaccatttggtaatatcttctacagctaaatatatattcatcttatgactcagtagtttcactccttttttttgtctgtttttttgagacagggtctcactctatcgcccaggatggaatgtagtggtgcgatcaaggctcactgcagccagctgtttcacttttaagtggacacacaagagaaatgagtgtacgtgtccattaaaatatatgcacaagaatgcttatggctgctttaaacacaaaagctaaaaattacaaacaaccaaaatgtctatcagtgggagaatggataaattgtgatgtatttatctgatggaatactacagagcaacgaaaaagaacaaactactgttattgctacatgcaacaacatagatgcatttcacagacataatgctgatcaaattaaaccagacacaaaaacctatagactggataattccatgtataggaatgtcaacaacagtgacagaggtcagagtggtggttatgtatgaggactgactgggagcctcatcttgatctgaatgatggttatatgggcgcatatatatgtaaacatttattgagctgtatatttcagacctgtgcactttacacaccatgttgcaataacattttaaacaatatgatcactatctatatgtagttttagtgctccatttggactggtctctggccactggatgtcagtgtttggagcagtgggcagcaggaaaagctggggaaggagtgggaaaacagaggagagagctatcacatgggcttcctagagaaaaataagcactttatgaagcttataagttcctttatgtacacagtagacaaagccttttaaagagatttgtccatacgggcactgaaataacatttttgtaaagtagccttctctatgttgattgcagatgtttctatctcagaatttaagtctacttgctttctcacacagcatcattatttccttattcctaataattttcatcacaaacatttcccagctctgtcccaatcaagttcttatttctctgaacggaattacaatttataaatgtaggtccacatgcagatatcttaataagtagtgaaataccagtgtagaaatacacaaatgagtgtggacacaccatagaaaagcagaaaaatacgagaaaaagtgcatgtacggagtatgggatgaactgatgcagttaaggaagacaactcacaaagcaactcacggctgggcaaagctgggaggctgaggcgggaggattgcttgaagccaggagtttgagactagcctgggcaccatactgataccttgtagctattaaaaaaaaattagctgggcatggtggctcatgcctgtagtctacttagtcagctgcttaggaggctgaggtacaaggattgcttgagcccaggaggtggaggttgcagtgagctgtgatcacgccactgcactccggccagggtgacagagtgagaccctgtctcacacaaaggcaactcatttgagctgaggcttggctatacttttaattgtccacatagaatagaggaaaaacaatgtttttcatcttttttaatcttccatttaccttttagtaagacaaattcttatctttatgtaaaactgtggaagagcagttacatagattgttgcagcttagattattttcaagaagtttaaattctacacataaggatacataccatttttaccagctatactttaaaatgccagtctttaaaaattcctctatgtgtatatgtggtttcttcttcttttcaaaaattcatgcctgtgaagtttttaggaatatttttcaaaactttagtactgaggcattaactgtttatgtgacacagcacctttaaatttctgtttttattcagccaaagaatgagaattattgtacattgctagtatttataatttcagcaaataggatagcagtatagtacctaaaataaactattaggaataactgaatgcctaccacagcaacagagctttaatgaggttaattgtcacatacatatccattccaacatagcagtgcacatttcacatgaccagcctcttatgtagttaaaaataaaactgcagttttaaaatgtcaagttcctcaaccttactggattttaaaacaaagcaaacaaaagaaacaaggattttctaatctatctataagcagaaatgtcagaaaataaagctacagtattccataaaacttaaaatttccttttctaagtcatgacatttctcttttgttctgttttctttttcttctaatattaagaaaatttaaaacgtaaatgaaaaaactgcttaatgtggcaaggaacaagaatgaaactagatttttttttttagtaaaggggcaaattgtataccaacatataaattaaaagtgttatgcaatgagaaacaataatggaaacagcataatactacatactatcccagtttcctgtgctctgaagaacagctgctatactaaatactaacttgacttatctgaagtattcaatactttctgataacccaagcagcattatattaatagttagaatactactacaaaatgtccttctacctctcccacaagaaatacaccaggaaacttaagcctgatgaataactactaagaatcttgtcttttaatacaagtctccttctagacacaaaatcctagctttttgtaatgtggttaaaaggagtaatggaaaagaaatgactgccaataaacatttcctattttgcactagggtgaagaaaccaagacacaaacatttggaagccactttagtttcttattccttttcaccctaatagtaggaaaatattaggcacctacttaattcacaaattcatgaaacagggtggacaacagccttgtgtaggggaagcatttggaatggtaatcaactacttaattacataacagggagctgggcatacaaagaaaagggctcagaagaaatatcttgaaaagtaagcaatatagaaggtgaggacagaagtgaggctaatcaaatgttcttagcaagatgttgcccccctgaaaatatgctcccccaataaaacacgtaaataactactcttaaggaaaatattttctctaaagaatgtcacaatttggagtgaagttacttaacaaaacagggaataaaacctttaatgttggctgtagcagttattttctttgggtagattatacttaaaatatttccttcatacatacttctgttaaaatttttttttcccattcttgagttttacaatgtctcctatccaaacttcaaatttcattagagccggctacatttgttttagtgccagatacaggtatcaagtgatgacagacacttacgtgaggtatacaatcaattaaagactggaaattggggtattatcatgtaagacatttgagaggccaaaagtcatataattttaagatacttcatgatgttacagtaataattcatctatataacaattattttgacataagtggcatatcagaatttaacttatttacttagatcttaaggaatattagatgtattctcacatgaacactcaaatcatgctattattatcagtcactgggagaacagccaaagtaatcaggcagtctaaggcacatatagacccaataatttagaaattttcaccattatgaggtaccctgtttttaataaatatgacaataacaggcgcttgaaatgggggcaaggtgaataagtatccagtcaattgtatacttttataaagtagtgtatttgagaacataaactgagatacaaaaggaatttccttactttaaaaaaagtgacttctatcttagtagatttctttaaaataacttaccttatatttaaaagttagtcatttacatacttaagaaatcaacagtaatctaaaaaaattaaaaggcagttttcttgggtaatgaacctgtgactccaagacagacaacaatgtggaaattaactcaggagactgactttctattctagtaattcagtggtttcttactttataaaggtttggaagaattaatgaatttctttttttcttaagacagggtctcgctctgttgcccaggctggagtgcagtggtgtgatcacagctcactgcagcctcgaactcctgggctcaagcgatcctccacatgttggcctcccatgagccaccatgctcagctaatttttatttttatttttggagagacagtgtctcactatgttgcccaggttggtctctaactcctggtttcaagtgattctccagtcttatactcccaaagcacaaggattacaggcctgagccaccacactcagccaatcaatttcaaaatgctaattaacctctttcagacacacgatctggcagagtaattagaagaaactggtctttcttaacatctttcctctattatcttccttttcttattcttgcctctcaatttgtcatatacagttacaaaatatatgaatcaggatttatgttggcatgaaaattatatgcaatacaatcagtaagtgaagaagggagggggtggtgtggctctagtcccaaagttaatgtcataaggagaaataatgtaagtatttgtatttcttagatcttcttctattttactcttaataccaaaaaaagagtcctatcatttaactttttatatattttgtagtgtttatttttgatgtgaccaaatgaaagctttctgaattttaaagtgcaattcactgtatgttaatacacagcctgcataggacctaactgcttcaaacttggcatcaaatgctgtctttttggtacttataagtagggtgtagataaagatatttgacaagagtgcaacagtgtttgttaaggtcttttcaaaagcccatttgagattattcaggcaggctcatcagttgacagctagcctatctttccttcttcctgttagtctgactgcctttttacccatttcatcgcctgtcgaatcctcctcaagaagaggcaagggaaataaatgaaaatgaaacccattaatttccaatattcacaatgaaatcaatcacatcatcaatctgtatactgtctgaccatttttctggatcattttctattagcaacatagtccctttagtttgtactttataactagtattttctaccaggatgcacagtttaaaaaatggcttgaagagccaaatatgttcccaatatgtccaatataattataaatatggtcattttcttgattactagagatctgtgcctgatggaatcacattttgtgaattagcaatagtttggtaataattcacacaaaatttcccataattactaggaataactgaaagctgggagtagaaaactttcattaactcaatattatgtagccatttgggccagcaaaaagtgtaaaatattattcccaataaccactgtggacaaaatgtgaacaggataatataatattttgaaaatattttaatatttgccattttttgcctgtgctattaatatatacattgatttagtaataaatatactactattacatagagtgcaatatttttagtattcataactggttgaaattaatgctgctataacctcaagaaaggaataaataaatatcatgtccaaattccaaactaatgctcaaaaggttatcattaacaaaaactataaaataaacatgttgggcattatctctttaagcatgattcctgtaaacaaagcaaaaaaatcacttttctcagtcctgacatttcacatgatggctttaaaagaaaatataacacacaaaccctatcacttcttttttttttttttttttttttgcatagggaacgaattaattgtatttttaaatgcagcaatcttttaatgaaatgttttcatcacatagtacttgttttctgtatgaattcagaacttttgagcaataaaagtgctctgcataagtttataaaatatgctttctggatttaaaatttaacagaaaaatttccaaacaagtcataggtatgattctaaaatattatgtacataatatatgactacaggaggaaattcctcactgtagtacaacacagtgtacaaatatgaagcacagtgtttagtttaatttccctttaggttttcctcacattggtgcataagtggctgactacatgacacaacatgccccattctacttgttgcatacaaagtagaagaggaatgtgaggacaaatttaaagtagaaaatgaaaataaatggcaaaaatacagtgcaaatgctttaaacagtgcactttataaaatagtttgctttattcatacttttttataaagtgcaatattacttaaaacagagagacatgtaccttaatattctgcaataaccattaaaacaaattgccaggaaagagcagtgcaaaattaaaaacatacacatagcttagcatgcatctcagatggatcccgaatacagagtatgggaccttgagttcttatatctttttttttttttttcactttttagaaaaagtttaataatagcaggttatcatcatatgtaaccataaaataaaaacaataagttaaaatcttctctcaagaaataagtatatgccacacataaaattcattacagaatcttttttgaaaacagacccctttctctgataaatcattgtttgaagggtgcaaatttcaaaaacccacattgtccacaaggcaaagcaaaaggtatcatcacagtatgagtcatttcttgttggcagacatctggaaaacctgtgacttacaagcagctcaaatctagccctaattaaatttacaggaacctttgctctttcaagaatagtcttgttggcatcatgctaggttgctaaaaagagtaatatgtgctctattcacagtaacattctctgtccagtgcttttgaatgaggataaccaaacaggttttcctgaaaaaaatcattaggaggcagattccaatgagaccaacgggaaacatttttaaaagcataaaagatcgcctcaggcatatgctgagggaataaaggtgcaatggatcactgatacactcctaccatgcctaagctactgagtccgagaactggaagagggtctccgggttattgctgtcggcaggattgctgggctgcagtgtcttggtgggtgtagttttaccgtgagaatgagaggaagaagaatgggaactctcactggaactgctgcgcgtctcggtactggtgctagtctttttcatttttcttctcttagccaaaggggccttatcaacattctgaaggcaaaacccctctctcttgtatttgttaaaggcgtggaaggttgctttcacacaggtatgcacggcagctccggaagatcctagaatatccggagtcatcagaggattggaggacagctgacttccatcttgtagccattcattgtacctcaagccagacattttaagccttttgtttggatctactgtgagaagtccttggatcaaatctttagcctcttgggatacattcttccaggcttctccttcaaaggagaaatctccctttttaattttcttcatgatttccaccgcgctggtacacgtcaaacttcggtcatgagattggaagggaacctgtcctgacaacattgtgtacaaaatgacgcccaagctccacaggtcacaggactcatcgtagccgttctgattcaagagctctggggcggcataatgaagggtgaagcatggagtcttcaggggctgattatccggtggctttagccgtgcaaatccaaaatcaattattttaatttccaaattgtcattttcatcggtgaacaataaattctcaggtttcagatccctgtgcaccactccaacatcatgcatgtggcttacagctgaaacaagcttcctcatgatgtagctggcttccgtctcactgaagtgcttctttttcttaatgcgctcaaacagttctcctccattcagaagttccatcactagaaacgtgtgaagctgatcatgaaaaacttcatgcaacttcacaatattggggtgtccttcacagagtttcagagctgttatttccttttgagtattggcttccatccttttgctgattattttgactgcaaaagcttggttactttttttatgcacacactttcgacaaattgaaaaactaccttctcccaggggtttgtccttcaaatctaggtcatagtgttgatagaatggagagtccttcatcattgcactcctggcaacatttgtcactccaggacgttcaactcccatgtgaaactgaagagggtctatgacagctgcattacgcttgaataggatggaaggagcaacaaaggaatagccctgaaacagcttctcagaactctggggcagggctgcgggagaataagtgggatccatttctgtgaactcttctgcaaagttactcacatctaattcatctcgaatgactggcttaaatggtgcaggcacttttttggcggctaaatcatcccaatttattttctgaaagaagagatgttctttgatttcatctgcatcacgtggaccacatcccaatctcttcttgggatctttcatcaaaagacgctgaattaggtctttcgctaaagcactcatttcttggggatatggaggctcactttttaatattctcctagatatctcagcttgggaatttttttctccatcaacagtgaaaggagatgctccagttagtaattcatacattagaacacccaaactccaccagtcaactgccttgtcatgtcctgaatctccccctctgacaatatctggtgccatgtattcaatagttccacaaaaggaatatgctctttcagtttcatcagccacaaactccttactcagaccaaaatctgtcagcaccacatggccattagaatcaagtagaatattctcaagcttaatatcacgatatataatccccaacttgtggagatgttcgagggcaagcacaatctctccaacataaatctgcacctcatgctctgtgaaacgctctctttgagaaagatgagtaaaaagttcaccaccatttatataatctccagttcctaggaccttcaggagctcaaaattttctattcccaccttctcagcatgtcctgtcaaattagcagtccgcagctcgtgcttgacagtgaggagctgctctcctccgtcgccgccgtccgcgctggtccccgcggcgccgccgctgctgccaccctcctcctccatcttctcctttttttccgatcccgcgggtcgctacgaggggaacccaggagacagcggacgcccgtcccctcgcagccgctgccgcggccccaggagtcggggtgcggcggctccagaactcggacgcaaagacgagtctctttcccgctctggccgcacggctcgctcctcgcctcctcccccttcggcgggcaccgctagtaccgc

SEQ ID NO: 14766 - RNA, 9791 nt, Homo sapiens
  source 1..9791: mol_type = other RNA
gctgggattacaggcatgagccacctcacccggccaataaagcttttagaagaatataagaatatcttcataaccttggtgtgaacatttattaaatacgacgcaaaagtattagcaattaaataaaagactggtatattggacttcataaaatttttggtcatcaaaggaaagcacttagaaagtagaaaagcaaactaaagagaagacatttatggtaaaatatcagacaaaaaccctcatatccataaaatataaaagactcctgcaagtcagtaagaaaaaaagacaacccaataaatatgaacaaatgacttgaacaggcacttaattgaggatagccaaatgactaataaaaatataaaaaggtgttccacacatcactacttatcaggaaaatacaccttaaaatctcagtgaaatacaaaatcaccagaatggttaaaaccacaatcaaatatacacatttgtcagagtggctaaactactagggctgatggtaccaagcactgatgaggatgtggaagaactagaacacttacacattattggtgggtatgtaaattggtacaaccattgttgaaaaccatttggtaatatcttctacagctaaatatatattcatcttatgactcagtagtttcactccttttttttgtctgtttttttgagacagggtctcactctatcgcccaggatggaatgtagtggtgcgatcaaggctcactgcagccagctgtttcacttttaagtggacacacaagagaaatgagtgtacgtgtccattaaaatatatgcacaagaatgcttatggctgctttaaacacaaaagctaaaaattacaaacaaccaaaatgtctatcagtgggagaatggataaattgtgatgtatttatctgatggaatactacagagcaacgaaaaagaacaaactactgttattgctacatgcaacaacatagatgcatttcacagacataatgctgatcaaattaaaccagacacaaaaacctatagactggataattccatgtataggaatgtcaacaacagtgacagaggtcagagtggtggttatgtatgaggactgactgggagcctcatcttgatctgaatgatggttatatgggcgcatatatatgtaaacatttattgagctgtatatttcagacctgtgcactttacacaccatgttgcaataacattttaaacaatatgatcactatctatatgtagttttagtgctccatttggactggtctctggccactggatgtcagtgtttggagcagtgggcagcaggaaaagctggggaaggagtgggaaaacagaggagagagctatcacatgggcttcctagagaaaaataagcactttatgaagcttataagttcctttatgtacacagtagacaaagccttttaaagagatttgtccatacgggcactgaaataacatttttgtaaagtagccttctctatgttgattgcagatgtttctatctcagaatttaagtctacttgctttctcacacagcatcattatttccttattcctaataattttcatcacaaacatttcccagctctgtcccaatcaagttcttatttctctgaacggaattacaatttataaatgtaggtccacatgcagatatcttaataagtagtgaaataccagtgtagaaatacacaaatgagtgtggacacaccatagaaaagcagaaaaatacgagaaaaagtgcatgtacggagtatgggatgaactgatgcagttaaggaagacaactcacaaagcaactcacggctgggcaaagctgggaggctgaggcgggaggattgcttgaagccaggagtttgagactagcctgggcaccatactgataccttgtagctattaaaaaaaaattagctgggcatggtggctcatgcctgtagtctacttagtcagctgcttaggaggctgaggtacaaggattgcttgagcccaggaggtggaggttgcagtgagctgtgatcacgccactgcactccggccagggtgacagagtgagaccctgtctcacacaaaggcaactcatttgagctgaggcttggctatacttttaattgtccacatagaatagaggaaaaacaatgtttttcatcttttttaatcttccatttaccttttagtaagacaaattcttatctttatgtaaaactgtggaagagcagttacatagattgttgcagcttagattattttcaagaagtttaaattctacacataaggatacataccatttttaccagctatactttaaaatgccagtctttaaaaattcctctatgtgtatatgtggtttcttcttcttttcaaaaattcatgcctgtgaagtttttaggaatatttttcaaaactttagtactgaggcattaactgtttatgtgacacagcacctttaaatttctgtttttattcagccaaagaatgagaattattgtacattgctagtatttataatttcagcaaataggatagcagtatagtacctaaaataaactattaggaataactgaatgcctaccacagcaacagagctttaatgaggttaattgtcacatacatatccattccaacatagcagtgcacatttcacatgaccagcctcttatgtagttaaaaataaaactgcagttttaaaatgtcaagttcctcaaccttactggattttaaaacaaagcaaacaaaagaaacaaggattttctaatctatctataagcagaaatgtcagaaaataaagctacagtattccataaaacttaaaatttccttttctaagtcatgacatttctcttttgttctgttttctttttcttctaatattaagaaaatttaaaacgtaaatgaaaaaactgcttaatgtggcaaggaacaagaatgaaactagatttttttttttagtaaaggggcaaattgtataccaacatataaattaaaagtgttatgcaatgagaaacaataatggaaacagcataatactacatactatcccagtttcctgtgctctgaagaacagctgctatactaaatactaacttgacttatctgaagtattcaatactttctgataacccaagcagcattatattaatagttagaatactactacaaaatgtccttctacctctcccacaagaaatacaccaggaaacttaagcctgatgaataactactaagaatcttgtcttttaatacaagtctccttctagacacaaaatcctagctttttgtaatgtggttaaaaggagtaatggaaaagaaatgactgccaataaacatttcctattttgcactagggtgaagaaaccaagacacaaacatttggaagccactttagtttcttattccttttcaccctaatagtaggaaaatattaggcacctacttaattcacaaattcatgaaacagggtggacaacagccttgtgtaggggaagcatttggaatggtaatcaactacttaattacataacagggagctgggcatacaaagaaaagggctcagaagaaatatcttgaaaagtaagcaatatagaaggtgaggacagaagtgaggctaatcaaatgttcttagcaagatgttgcccccctgaaaatatgctcccccaataaaacacgtaaataactactcttaaggaaaatattttctctaaagaatgtcacaatttggagtgaagttacttaacaaaacagggaataaaacctttaatgttggctgtagcagttattttctttgggtagattatacttaaaatatttccttcatacatacttctgttaaaatttttttttcccattcttgagttttacaatgtctcctatccaaacttcaaatttcattagagccggctacatttgttttagtgccagatacaggtatcaagtgatgacagacacttacgtgaggtatacaatcaattaaagactggaaattggggtattatcatgtaagacatttgagaggccaaaagtcatataattttaagatacttcatgatgttacagtaataattcatctatataacaattattttgacataagtggcatatcagaatttaacttatttacttagatcttaaggaatattagatgtattctcacatgaacactcaaatcatgctattattatcagtcactgggagaacagccaaagtaatcaggcagtctaaggcacatatagacccaataatttagaaattttcaccattatgaggtaccctgtttttaataaatatgacaataacaggcgcttgaaatgggggcaaggtgaataagtatccagtcaattgtatacttttataaagtagtgtatttgagaacataaactgagatacaaaaggaatttccttactttaaaaaaagtgacttctatcttagtagatttctttaaaataacttaccttatatttaaaagttagtcatttacatacttaagaaatcaacagtaatctaaaaaaattaaaaggcagttttcttgggtaatgaacctgtgactccaagacagacaacaatgtggaaattaactcaggagactgactttctattctagtaattcagtggtttcttactttataaaggtttggaagaattaatgaatttctttttttcttaagacagggtctcgctctgttgcccaggctggagtgcagtggtgtgatcacagctcactgcagcctcgaactcctgggctcaagcgatcctccacatgttggcctcccatgagccaccatgctcagctaatttttatttttatttttggagagacagtgtctcactatgttgcccaggttggtctctaactcctggtttcaagtgattctccagtcttatactcccaaagcacaaggattacaggcctgagccaccacactcagccaatcaatttcaaaatgctaattaacctctttcagacacacgatctggcagagtaattagaagaaactggtctttcttaacatctttcctctattatcttccttttcttattcttgcctctcaatttgtcatatacagttacaaaatatatgaatcaggatttatgttggcatgaaaattatatgcaatacaatcagtaagtgaagaagggagggggtggtgtggctctagtcccaaagttaatgtcataaggagaaataatgtaagtatttgtatttcttagatcttcttctattttactcttaataccaaaaaaagagtcctatcatttaactttttatatattttgtagtgtttatttttgatgtgaccaaatgaaagctttctgaattttaaagtgcaattcactgtatgttaatacacagcctgcataggacctaactgcttcaaacttggcatcaaatgctgtctttttggtacttataagtagggtgtagataaagatatttgacaagagtgcaacagtgtttgttaaggtcttttcaaaagcccatttgagattattcaggcaggctcatcagttgacagctagcctatctttccttcttcctgttagtctgactgcctttttacccatttcatcgcctgtcgaatcctcctcaagaagaggcaagggaaataaatgaaaatgaaacccattaatttccaatattcacaatgaaatcaatcacatcatcaatctgtatactgtctgaccatttttctggatcattttctattagcaacatagtccctttagtttgtactttataactagtattttctaccaggatgcacagtttaaaaaatggcttgaagagccaaatatgttcccaatatgtccaatataattataaatatggtcattttcttgattactagagatctgtgcctgatggaatcacattttgtgaattagcaatagtttggtaataattcacacaaaatttcccataattactaggaataactgaaagctgggagtagaaaactttcattaactcaatattatgtagccatttgggccagcaaaaagtgtaaaatattattcccaataaccactgtggacaaaatgtgaacaggataatataatattttgaaaatattttaatatttgccattttttgcctgtgctattaatatatacattgatttagtaataaatatactactattacatagagtgcaatatttttagtattcataactggttgaaattaatgctgctataacctcaagaaaggaataaataaatatcatgtccaaattccaaactaatgctcaaaaggttatcattaacaaaaactataaaataaacatgttgggcattatctctttaagcatgattcctgtaaacaaagcaaaaaaatcacttttctcagtcctgacatttcacatgatggctttaaaagaaaatataacacacaaaccctatcacttcttttttttttttttttttttttgcatagggaacgaattaattgtatttttaaatgcagcaatcttttaatgaaatgttttcatcacatagtacttgttttctgtatgaattcagaacttttgagcaataaaagtgctctgcataagtttataaaatatgctttctggatttaaaatttaacagaaaaatttccaaacaagtcataggtatgattctaaaatattatgtacataatatatgactacaggaggaaattcctcactgtagtacaacacagtgtacaaatatgaagcacagtgtttagtttaatttccctttaggttttcctcacattggtgcataagtggctgactacatgacacaacatgccccattctacttgttgcatacaaagtagaagaggaatgtgaggacaaatttaaagtagaaaatgaaaataaatggcaaaaatacagtgcaaatgctttaaacagtgcactttataaaatagtttgctttattcatacttttttataaagtgcaatattacttaaaacagagagacatgtaccttaatattctgcaataaccattaaaacaaattgccaggaaagagcagtgcaaaattaaaaacatacacatagcttagcatgcatctcagatggatcccgaatacagagtatgggaccttgagttcttatatctttttttttttttttcactttttagaaaaagtttaataatagcaggttatcatcatatgtaaccataaaataaaaacaataagttaaaatcttctctcaagaaataagtatatgccacacataaaattcattacagaatcttttttgaaaacagacccctttctctgataaatcattgtttgaagggtgcaaatttcaaaaacccacattgtccacaaggcaaagcaaaaggtatcatcacagtatgagtcatttcttgttggcagacatctggaaaacctgtgacttacaagcagctcaaatctagccctaattaaatttacaggaacctttgctctttcaagaatagtcttgttggcatcatgctaggttgctaaaaagagtaatatgtgctctattcacagtaacattctctgtccagtgcttttgaatgaggataaccaaacaggttttcctgaaaaaaatcattaggaggcagattccaatgagaccaacgggaaacatttttaaaagcataaaagatcgcctcaggcatatgctgagggaataaaggtgcaatggatcactgatacactcctaccatgcctaagctactgagtccgagaactggaagagggtctccgggttattgctgtcggcaggattgctgggctgcagtgtcttggtgggtgtagttttaccgtgagaatgagaggaagaagaatgggaactctcactggaactgctgcgcgtctcggtactggtgctagtctttttcatttttcttctcttagccaaaggggccttatcaacattctgaaggcaaaacccctctctcttgtatttgttaaaggcgtggaaggttgctttcacacaggtatgcacggcagctccggaagatcctagaatatccggagtcatcagaggattggaggacagctgacttccatcttgtagccattcattgtacctcaagccagacattttaagccttttgtttggatctactgtgagaagtccttggatcaaatctttagcctcttgggatacattcttccaggcttctccttcaaaggagaaatctccctttttaattttcttcatgatttccaccgcgctggtacacgtcaaacttcggtcatgagattggaagggaacctgtcctgacaacattgtgtacaaaatgacgcccaagctccacaggtcacaggactcatcgtagccgttctgattcaagagctctggggcggcataatgaagggtgaagcatggagtcttcaggggctgattatccggtggctttagccgtgcaaatccaaaatcaattattttaatttccaaattgtcattttcatcggtgaacaataaattctcaggtttcagatccctgtgcaccactccaacatcatgcatgtggcttacagctgaaacaagcttcctcatgatgtagctggcttccgtctcactgaagtgcttctttttcttaatgcgctcaaacagttctcctccattcagaagttccatcactagaaacgtgtgaagctgatcatgaaaaacttcatgcaacttcacaatattggggtgtccttcacagagtttcagagctgttatttccttttgagtattggcttccatccttttgctgattattttgactgcaaaagcttggttactttttttatgcacacactttcgacaaattgaaaaactaccttctcccaggggtttgtccttcaaatctaggtcatagtgttgatagaatggagagtccttcatcattgcactcctggcaacatttgtcactccaggacgttcaactcccatgtgaaactgaagagggtctatgacagctgcattacgcttgaataggatggaaggagcaacaaaggaatagccctgaaacagcttctcagaactctggggcagggctgcgggagaataagtgggatccatttctgtgaactcttctgcaaagttactcacatctaattcatctcgaatgactggcttaaatggtgcaggcacttttttggcggctaaatcatcccaatttattttctgaaagaagagatgttctttgatttcatctgcatcacgtggaccacatcccaatctcttcttgggatctttcatcaaaagacgctgaattaggtctttcgctaaagcactcatttcttggggatatggaggctcactttttaatattctcctagatatctcagcttgggaatttttttctccatcaacagtgaaaggagatgctccagttagtaattcatacattagaacacccaaactccaccagtcaactgccttgtcatgtcctgaatctccccctctgacaatatctggtgccatgtattcaatagttccacaaaaggaatatgctctttcagtttcatcagccacaaactccttactcagaccaaaatctgtcagcaccacatggccattagaatcaagtagaatattctcaagcttaatatcacgatatataatccccaacttgtggagatgttcgagggcaagcacaatctctccaacataaatctgcacctcatgctctgtgaaacgctctctttgagaaagatgagtaaaaagttcaccaccatttatataatctgtgcgggaagggggagcagcgacatcctcggaggtgcgtgccacgggcagcggtcggcggctgcgctggccccgatgcctggtgcccgccgctcattcccgggct

SEQ ID NO: 14767 - RNA, 10201 nt, Homo sapiens
  source 1..10201: mol_type = other RNA
gctgggattacaggcatgagccacctcacccggccaataaagcttttagaagaatataagaatatcttcataaccttggtgtgaacatttattaaatacgacgcaaaagtattagcaattaaataaaagactggtatattggacttcataaaatttttggtcatcaaaggaaagcacttagaaagtagaaaagcaaactaaagagaagacatttatggtaaaatatcagacaaaaaccctcatatccataaaatataaaagactcctgcaagtcagtaagaaaaaaagacaacccaataaatatgaacaaatgacttgaacaggcacttaattgaggatagccaaatgactaataaaaatataaaaaggtgttccacacatcactacttatcaggaaaatacaccttaaaatctcagtgaaatacaaaatcaccagaatggttaaaaccacaatcaaatatacacatttgtcagagtggctaaactactagggctgatggtaccaagcactgatgaggatgtggaagaactagaacacttacacattattggtgggtatgtaaattggtacaaccattgttgaaaaccatttggtaatatcttctacagctaaatatatattcatcttatgactcagtagtttcactccttttttttgtctgtttttttgagacagggtctcactctatcgcccaggatggaatgtagtggtgcgatcaaggctcactgcagccagctgtttcacttttaagtggacacacaagagaaatgagtgtacgtgtccattaaaatatatgcacaagaatgcttatggctgctttaaacacaaaagctaaaaattacaaacaaccaaaatgtctatcagtgggagaatggataaattgtgatgtatttatctgatggaatactacagagcaacgaaaaagaacaaactactgttattgctacatgcaacaacatagatgcatttcacagacataatgctgatcaaattaaaccagacacaaaaacctatagactggataattccatgtataggaatgtcaacaacagtgacagaggtcagagtggtggttatgtatgaggactgactgggagcctcatcttgatctgaatgatggttatatgggcgcatatatatgtaaacatttattgagctgtatatttcagacctgtgcactttacacaccatgttgcaataacattttaaacaatatgatcactatctatatgtagttttagtgctccatttggactggtctctggccactggatgtcagtgtttggagcagtgggcagcaggaaaagctggggaaggagtgggaaaacagaggagagagctatcacatgggcttcctagagaaaaataagcactttatgaagcttataagttcctttatgtacacagtagacaaagccttttaaagagatttgtccatacgggcactgaaataacatttttgtaaagtagccttctctatgttgattgcagatgtttctatctcagaatttaagtctacttgctttctcacacagcatcattatttccttattcctaataattttcatcacaaacatttcccagctctgtcccaatcaagttcttatttctctgaacggaattacaatttataaatgtaggtccacatgcagatatcttaataagtagtgaaataccagtgtagaaatacacaaatgagtgtggacacaccatagaaaagcagaaaaatacgagaaaaagtgcatgtacggagtatgggatgaactgatgcagttaaggaagacaactcacaaagcaactcacggctgggcaaagctgggaggctgaggcgggaggattgcttgaagccaggagtttgagactagcctgggcaccatactgataccttgtagctattaaaaaaaaattagctgggcatggtggctcatgcctgtagtctacttagtcagctgcttaggaggctgaggtacaaggattgcttgagcccaggaggtggaggttgcagtgagctgtgatcacgccactgcactccggccagggtgacagagtgagaccctgtctcacacaaaggcaactcatttgagctgaggcttggctatacttttaattgtccacatagaatagaggaaaaacaatgtttttcatcttttttaatcttccatttaccttttagtaagacaaattcttatctttatgtaaaactgtggaagagcagttacatagattgttgcagcttagattattttcaagaagtttaaattctacacataaggatacataccatttttaccagctatactttaaaatgccagtctttaaaaattcctctatgtgtatatgtggtttcttcttcttttcaaaaattcatgcctgtgaagtttttaggaatatttttcaaaactttagtactgaggcattaactgtttatgtgacacagcacctttaaatttctgtttttattcagccaaagaatgagaattattgtacattgctagtatttataatttcagcaaataggatagcagtatagtacctaaaataaactattaggaataactgaatgcctaccacagcaacagagctttaatgaggttaattgtcacatacatatccattccaacatagcagtgcacatttcacatgaccagcctcttatgtagttaaaaataaaactgcagttttaaaatgtcaagttcctcaaccttactggattttaaaacaaagcaaacaaaagaaacaaggattttctaatctatctataagcagaaatgtcagaaaataaagctacagtattccataaaacttaaaatttccttttctaagtcatgacatttctcttttgttctgttttctttttcttctaatattaagaaaatttaaaacgtaaatgaaaaaactgcttaatgtggcaaggaacaagaatgaaactagatttttttttttagtaaaggggcaaattgtataccaacatataaattaaaagtgttatgcaatgagaaacaataatggaaacagcataatactacatactatcccagtttcctgtgctctgaagaacagctgctatactaaatactaacttgacttatctgaagtattcaatactttctgataacccaagcagcattatattaatagttagaatactactacaaaatgtccttctacctctcccacaagaaatacaccaggaaacttaagcctgatgaataactactaagaatcttgtcttttaatacaagtctccttctagacacaaaatcctagctttttgtaatgtggttaaaaggagtaatggaaaagaaatgactgccaataaacatttcctattttgcactagggtgaagaaaccaagacacaaacatttggaagccactttagtttcttattccttttcaccctaatagtaggaaaatattaggcacctacttaattcacaaattcatgaaacagggtggacaacagccttgtgtaggggaagcatttggaatggtaatcaactacttaattacataacagggagctgggcatacaaagaaaagggctcagaagaaatatcttgaaaagtaagcaatatagaaggtgaggacagaagtgaggctaatcaaatgttcttagcaagatgttgcccccctgaaaatatgctcccccaataaaacacgtaaataactactcttaaggaaaatattttctctaaagaatgtcacaatttggagtgaagttacttaacaaaacagggaataaaacctttaatgttggctgtagcagttattttctttgggtagattatacttaaaatatttccttcatacatacttctgttaaaatttttttttcccattcttgagttttacaatgtctcctatccaaacttcaaatttcattagagccggctacatttgttttagtgccagatacaggtatcaagtgatgacagacacttacgtgaggtatacaatcaattaaagactggaaattggggtattatcatgtaagacatttgagaggccaaaagtcatataattttaagatacttcatgatgttacagtaataattcatctatataacaattattttgacataagtggcatatcagaatttaacttatttacttagatcttaaggaatattagatgtattctcacatgaacactcaaatcatgctattattatcagtcactgggagaacagccaaagtaatcaggcagtctaaggcacatatagacccaataatttagaaattttcaccattatgaggtaccctgtttttaataaatatgacaataacaggcgcttgaaatgggggcaaggtgaataagtatccagtcaattgtatacttttataaagtagtgtatttgagaacataaactgagatacaaaaggaatttccttactttaaaaaaagtgacttctatcttagtagatttctttaaaataacttaccttatatttaaaagttagtcatttacatacttaagaaatcaacagtaatctaaaaaaattaaaaggcagttttcttgggtaatgaacctgtgactccaagacagacaacaatgtggaaattaactcaggagactgactttctattctagtaattcagtggtttcttactttataaaggtttggaagaattaatgaatttctttttttcttaagacagggtctcgctctgttgcccaggctggagtgcagtggtgtgatcacagctcactgcagcctcgaactcctgggctcaagcgatcctccacatgttggcctcccatgagccaccatgctcagctaatttttatttttatttttggagagacagtgtctcactatgttgcccaggttggtctctaactcctggtttcaagtgattctccagtcttatactcccaaagcacaaggattacaggcctgagccaccacactcagccaatcaatttcaaaatgctaattaacctctttcagacacacgatctggcagagtaattagaagaaactggtctttcttaacatctttcctctattatcttccttttcttattcttgcctctcaatttgtcatatacagttacaaaatatatgaatcaggatttatgttggcatgaaaattatatgcaatacaatcagtaagtgaagaagggagggggtggtgtggctctagtcccaaagttaatgtcataaggagaaataatgtaagtatttgtatttcttagatcttcttctattttactcttaataccaaaaaaagagtcctatcatttaactttttatatattttgtagtgtttatttttgatgtgaccaaatgaaagctttctgaattttaaagtgcaattcactgtatgttaatacacagcctgcataggacctaactgcttcaaacttggcatcaaatgctgtctttttggtacttataagtagggtgtagataaagatatttgacaagagtgcaacagtgtttgttaaggtcttttcaaaagcccatttgagattattcaggcaggctcatcagttgacagctagcctatctttccttcttcctgttagtctgactgcctttttacccatttcatcgcctgtcgaatcctcctcaagaagaggcaagggaaataaatgaaaatgaaacccattaatttccaatattcacaatgaaatcaatcacatcatcaatctgtatactgtctgaccatttttctggatcattttctattagcaacatagtccctttagtttgtactttataactagtattttctaccaggatgcacagtttaaaaaatggcttgaagagccaaatatgttcccaatatgtccaatataattataaatatggtcattttcttgattactagagatctgtgcctgatggaatcacattttgtgaattagcaatagtttggtaataattcacacaaaatttcccataattactaggaataactgaaagctgggagtagaaaactttcattaactcaatattatgtagccatttgggccagcaaaaagtgtaaaatattattcccaataaccactgtggacaaaatgtgaacaggataatataatattttgaaaatattttaatatttgccattttttgcctgtgctattaatatatacattgatttagtaataaatatactactattacatagagtgcaatatttttagtattcataactggttgaaattaatgctgctataacctcaagaaaggaataaataaatatcatgtccaaattccaaactaatgctcaaaaggttatcattaacaaaaactataaaataaacatgttgggcattatctctttaagcatgattcctgtaaacaaagcaaaaaaatcacttttctcagtcctgacatttcacatgatggctttaaaagaaaatataacacacaaaccctatcacttcttttttttttttttttttttttgcatagggaacgaattaattgtatttttaaatgcagcaatcttttaatgaaatgttttcatcacatagtacttgttttctgtatgaattcagaacttttgagcaataaaagtgctctgcataagtttataaaatatgctttctggatttaaaatttaacagaaaaatttccaaacaagtcataggtatgattctaaaatattatgtacataatatatgactacaggaggaaattcctcactgtagtacaacacagtgtacaaatatgaagcacagtgtttagtttaatttccctttaggttttcctcacattggtgcataagtggctgactacatgacacaacatgccccattctacttgttgcatacaaagtagaagaggaatgtgaggacaaatttaaagtagaaaatgaaaataaatggcaaaaatacagtgcaaatgctttaaacagtgcactttataaaatagtttgctttattcatacttttttataaagtgcaatattacttaaaacagagagacatgtaccttaatattctgcaataaccattaaaacaaattgccaggaaagagcagtgcaaaattaaaaacatacacatagcttagcatgcatctcagatggatcccgaatacagagtatgggaccttgagttcttatatctttttttttttttttcactttttagaaaaagtttaataatagcaggttatcatcatatgtaaccataaaataaaaacaataagttaaaatcttctctcaagaaataagtatatgccacacataaaattcattacagaatcttttttgaaaacagacccctttctctgataaatcattgtttgaagggtgcaaatttcaaaaacccacattgtccacaaggcaaagcaaaaggtatcatcacagtatgagtcatttcttgttggcagacatctggaaaacctgtgacttacaagcagctcaaatctagccctaattaaatttacaggaacctttgctctttcaagaatagtcttgttggcatcatgctaggttgctaaaaagagtaatatgtgctctattcacagtaacattctctgtccagtgcttttgaatgaggataaccaaacaggttttcctgaaaaaaatcattaggaggcagattccaatgagaccaacgggaaacatttttaaaagcataaaagatcgcctcaggcatatgctgagggaataaaggtgcaatggatcactgatacactcctaccatgcctaagctactgagtccgagaactggaagagggtctccgggttattgctgtcggcaggattgctgggctgcagtgtcttggtgggtgtagttttaccgtgagaatgagaggaagaagaatgggaactctcactggaactgctgcgcgtctcggtactggtgctagtctttttcatttttcttctcttagccaaaggggccttatcaacattctgaaggcaaaacccctctctcttgtatttgttaaaggcgtggaaggttgctttcacacaggtatgcacggcagctccggaagatcctagaatatccggagtcatcagaggattggaggacagctgacttccatcttgtagccattcattgtacctcaagccagacattttaagccttttgtttggatctactgtgagaagtccttggatcaaatctttagcctcttgggatacattcttccaggcttctccttcaaaggagaaatctccctttttaattttcttcatgatttccaccgcgctggtacacgtcaaacttcggtcatgagattggaagggaacctgtcctgacaacattgtgtacaaaatgacgcccaagctccacaggtcacaggactcatcgtagccgttctgattcaagagctctggggcggcataatgaagggtgaagcatggagtcttcaggggctgattatccggtggctttagccgtgcaaatccaaaatcaattattttaatttccaaattgtcattttcatcggtgaacaataaattctcaggtttcagatccctgtgcaccactccaacatcatgcatgtggcttacagctgaaacaagcttcctcatgatgtagctggcttccgtctcactgaagtgcttctttttcttaatgcgctcaaacagttctcctccattcagaagttccatcactagaaacgtgtgaagctgatcatgaaaaacttcatgcaacttcacaatattggggtgtccttcacagagtttcagagctgttatttccttttgagtattggcttccatccttttgctgattattttgactgcaaaagcttggttactttttttatgcacacactttcgacaaattgaaaaactaccttctcccaggggtttgtccttcaaatctaggtcatagtgttgatagaatggagagtccttcatcattgcactcctggcaacatttgtcactccaggacgttcaactcccatgtgaaactgaagagggtctatgacagctgcattacgcttgaataggatggaaggagcaacaaaggaatagccctgaaacagcttctcagaactctggggcagggctgcgggagaataagtgggatccatttctgtgaactcttctgcaaagttactcacatctaattcatctcgaatgactggcttaaatggtgcaggcacttttttggcggctaaatcatcccaatttattttctgaaagaagagatgttctttgatttcatctgcatcacgtggaccacatcccaatctcttcttgggatctttcatcaaaagacgctgaattaggtctttcgctaaagcactcatttcttggggatatggaggctcactttttaatattctcctagatatctcagcttgggaatttttttctccatcaacagtgaaaggagatgctccagttagtaattcatacattagaacacccaaactccaccagtcaactgcttcatcagccacaaactccttactcagaccaaaatctgtcagcaccacatggccattagaatcaagtagaatattctcaagcttaatatcacgatatataatccccaacttgtggagatgttcgagggcaagcacaatctctccaacataaatctgcacctcatgctctgtgaaacgctctctttgagaaagatgagtaaaaagttcaccaccatttatataatctaaaatgagatgaagtttggtttctgtctggaaagcataatgtaatgttaccaaaaatggcgactgcctaatgtgttccaggacttgtcgttctgtccttgtatgctctgtggttttggccttttgaacgattgttgcctttttcaaaactttcatggcatacagctttccagtatcatggccacttattttacgaactagaaatacttttccataagctccagttcctaggaccttcaggagctcaaaattttctattcccaccttctcagcatgtcctgtcaaattagcagtccgcagctcgtgcttgacagtgaggagctgctctcctccgtcgccgccgtccgcgctggtccccgcggcgccgccgctgctgccaccctcctcctccatcttctcctttttttccgatcccgcgggtcgctacgaggggaacccaggagacagcggacgcccgtcccctcgcagccgctgccgcggccccaggagtcggggtgcggcggctccagaactcggacgcaaagacgagtctctttcccgctctggccgcacggctcgctcctcgcctcctcccccttcggcgggcaccgctagtaccgc

SEQ ID NO: 14768 - RNA, 10472 nt, Homo sapiens
  source 1..10472: mol_type = other RNA
gctgggattacaggcatgagccacctcacccggccaataaagcttttagaagaatataagaatatcttcataaccttggtgtgaacatttattaaatacgacgcaaaagtattagcaattaaataaaagactggtatattggacttcataaaatttttggtcatcaaaggaaagcacttagaaagtagaaaagcaaactaaagagaagacatttatggtaaaatatcagacaaaaaccctcatatccataaaatataaaagactcctgcaagtcagtaagaaaaaaagacaacccaataaatatgaacaaatgacttgaacaggcacttaattgaggatagccaaatgactaataaaaatataaaaaggtgttccacacatcactacttatcaggaaaatacaccttaaaatctcagtgaaatacaaaatcaccagaatggttaaaaccacaatcaaatatacacatttgtcagagtggctaaactactagggctgatggtaccaagcactgatgaggatgtggaagaactagaacacttacacattattggtgggtatgtaaattggtacaaccattgttgaaaaccatttggtaatatcttctacagctaaatatatattcatcttatgactcagtagtttcactccttttttttgtctgtttttttgagacagggtctcactctatcgcccaggatggaatgtagtggtgcgatcaaggctcactgcagccagctgtttcacttttaagtggacacacaagagaaatgagtgtacgtgtccattaaaatatatgcacaagaatgcttatggctgctttaaacacaaaagctaaaaattacaaacaaccaaaatgtctatcagtgggagaatggataaattgtgatgtatttatctgatggaatactacagagcaacgaaaaagaacaaactactgttattgctacatgcaacaacatagatgcatttcacagacataatgctgatcaaattaaaccagacacaaaaacctatagactggataattccatgtataggaatgtcaacaacagtgacagaggtcagagtggtggttatgtatgaggactgactgggagcctcatcttgatctgaatgatggttatatgggcgcatatatatgtaaacatttattgagctgtatatttcagacctgtgcactttacacaccatgttgcaataacattttaaacaatatgatcactatctatatgtagttttagtgctccatttggactggtctctggccactggatgtcagtgtttggagcagtgggcagcaggaaaagctggggaaggagtgggaaaacagaggagagagctatcacatgggcttcctagagaaaaataagcactttatgaagcttataagttcctttatgtacacagtagacaaagccttttaaagagatttgtccatacgggcactgaaataacatttttgtaaagtagccttctctatgttgattgcagatgtttctatctcagaatttaagtctacttgctttctcacacagcatcattatttccttattcctaataattttcatcacaaacatttcccagctctgtcccaatcaagttcttatttctctgaacggaattacaatttataaatgtaggtccacatgcagatatcttaataagtagtgaaataccagtgtagaaatacacaaatgagtgtggacacaccatagaaaagcagaaaaatacgagaaaaagtgcatgtacggagtatgggatgaactgatgcagttaaggaagacaactcacaaagcaactcacggctgggcaaagctgggaggctgaggcgggaggattgcttgaagccaggagtttgagactagcctgggcaccatactgataccttgtagctattaaaaaaaaattagctgggcatggtggctcatgcctgtagtctacttagtcagctgcttaggaggctgaggtacaaggattgcttgagcccaggaggtggaggttgcagtgagctgtgatcacgccactgcactccggccagggtgacagagtgagaccctgtctcacacaaaggcaactcatttgagctgaggcttggctatacttttaattgtccacatagaatagaggaaaaacaatgtttttcatcttttttaatcttccatttaccttttagtaagacaaattcttatctttatgtaaaactgtggaagagcagttacatagattgttgcagcttagattattttcaagaagtttaaattctacacataaggatacataccatttttaccagctatactttaaaatgccagtctttaaaaattcctctatgtgtatatgtggtttcttcttcttttcaaaaattcatgcctgtgaagtttttaggaatatttttcaaaactttagtactgaggcattaactgtttatgtgacacagcacctttaaatttctgtttttattcagccaaagaatgagaattattgtacattgctagtatttataatttcagcaaataggatagcagtatagtacctaaaataaactattaggaataactgaatgcctaccacagcaacagagctttaatgaggttaattgtcacatacatatccattccaacatagcagtgcacatttcacatgaccagcctcttatgtagttaaaaataaaactgcagttttaaaatgtcaagttcctcaaccttactggattttaaaacaaagcaaacaaaagaaacaaggattttctaatctatctataagcagaaatgtcagaaaataaagctacagtattccataaaacttaaaatttccttttctaagtcatgacatttctcttttgttctgttttctttttcttctaatattaagaaaatttaaaacgtaaatgaaaaaactgcttaatgtggcaaggaacaagaatgaaactagatttttttttttagtaaaggggcaaattgtataccaacatataaattaaaagtgttatgcaatgagaaacaataatggaaacagcataatactacatactatcccagtttcctgtgctctgaagaacagctgctatactaaatactaacttgacttatctgaagtattcaatactttctgataacccaagcagcattatattaatagttagaatactactacaaaatgtccttctacctctcccacaagaaatacaccaggaaacttaagcctgatgaataactactaagaatcttgtcttttaatacaagtctccttctagacacaaaatcctagctttttgtaatgtggttaaaaggagtaatggaaaagaaatgactgccaataaacatttcctattttgcactagggtgaagaaaccaagacacaaacatttggaagccactttagtttcttattccttttcaccctaatagtaggaaaatattaggcacctacttaattcacaaattcatgaaacagggtggacaacagccttgtgtaggggaagcatttggaatggtaatcaactacttaattacataacagggagctgggcatacaaagaaaagggctcagaagaaatatcttgaaaagtaagcaatatagaaggtgaggacagaagtgaggctaatcaaatgttcttagcaagatgttgcccccctgaaaatatgctcccccaataaaacacgtaaataactactcttaaggaaaatattttctctaaagaatgtcacaatttggagtgaagttacttaacaaaacagggaataaaacctttaatgttggctgtagcagttattttctttgggtagattatacttaaaatatttccttcatacatacttctgttaaaatttttttttcccattcttgagttttacaatgtctcctatccaaacttcaaatttcattagagccggctacatttgttttagtgccagatacaggtatcaagtgatgacagacacttacgtgaggtatacaatcaattaaagactggaaattggggtattatcatgtaagacatttgagaggccaaaagtcatataattttaagatacttcatgatgttacagtaataattcatctatataacaattattttgacataagtggcatatcagaatttaacttatttacttagatcttaaggaatattagatgtattctcacatgaacactcaaatcatgctattattatcagtcactgggagaacagccaaagtaatcaggcagtctaaggcacatatagacccaataatttagaaattttcaccattatgaggtaccctgtttttaataaatatgacaataacaggcgcttgaaatgggggcaaggtgaataagtatccagtcaattgtatacttttataaagtagtgtatttgagaacataaactgagatacaaaaggaatttccttactttaaaaaaagtgacttctatcttagtagatttctttaaaataacttaccttatatttaaaagttagtcatttacatacttaagaaatcaacagtaatctaaaaaaattaaaaggcagttttcttgggtaatgaacctgtgactccaagacagacaacaatgtggaaattaactcaggagactgactttctattctagtaattcagtggtttcttactttataaaggtttggaagaattaatgaatttctttttttcttaagacagggtctcgctctgttgcccaggctggagtgcagtggtgtgatcacagctcactgcagcctcgaactcctgggctcaagcgatcctccacatgttggcctcccatgagccaccatgctcagctaatttttatttttatttttggagagacagtgtctcactatgttgcccaggttggtctctaactcctggtttcaagtgattctccagtcttatactcccaaagcacaaggattacaggcctgagccaccacactcagccaatcaatttcaaaatgctaattaacctctttcagacacacgatctggcagagtaattagaagaaactggtctttcttaacatctttcctctattatcttccttttcttattcttgcctctcaatttgtcatatacagttacaaaatatatgaatcaggatttatgttggcatgaaaattatatgcaatacaatcagtaagtgaagaagggagggggtggtgtggctctagtcccaaagttaatgtcataaggagaaataatgtaagtatttgtatttcttagatcttcttctattttactcttaataccaaaaaaagagtcctatcatttaactttttatatattttgtagtgtttatttttgatgtgaccaaatgaaagctttctgaattttaaagtgcaattcactgtatgttaatacacagcctgcataggacctaactgcttcaaacttggcatcaaatgctgtctttttggtacttataagtagggtgtagataaagatatttgacaagagtgcaacagtgtttgttaaggtcttttcaaaagcccatttgagattattcaggcaggctcatcagttgacagctagcctatctttccttcttcctgttagtctgactgcctttttacccatttcatcgcctgtcgaatcctcctcaagaagaggcaagggaaataaatgaaaatgaaacccattaatttccaatattcacaatgaaatcaatcacatcatcaatctgtatactgtctgaccatttttctggatcattttctattagcaacatagtccctttagtttgtactttataactagtattttctaccaggatgcacagtttaaaaaatggcttgaagagccaaatatgttcccaatatgtccaatataattataaatatggtcattttcttgattactagagatctgtgcctgatggaatcacattttgtgaattagcaatagtttggtaataattcacacaaaatttcccataattactaggaataactgaaagctgggagtagaaaactttcattaactcaatattatgtagccatttgggccagcaaaaagtgtaaaatattattcccaataaccactgtggacaaaatgtgaacaggataatataatattttgaaaatattttaatatttgccattttttgcctgtgctattaatatatacattgatttagtaataaatatactactattacatagagtgcaatatttttagtattcataactggttgaaattaatgctgctataacctcaagaaaggaataaataaatatcatgtccaaattccaaactaatgctcaaaaggttatcattaacaaaaactataaaataaacatgttgggcattatctctttaagcatgattcctgtaaacaaagcaaaaaaatcacttttctcagtcctgacatttcacatgatggctttaaaagaaaatataacacacaaaccctatcacttcttttttttttttttttttttttgcatagggaacgaattaattgtatttttaaatgcagcaatcttttaatgaaatgttttcatcacatagtacttgttttctgtatgaattcagaacttttgagcaataaaagtgctctgcataagtttataaaatatgctttctggatttaaaatttaacagaaaaatttccaaacaagtcataggtatgattctaaaatattatgtacataatatatgactacaggaggaaattcctcactgtagtacaacacagtgtacaaatatgaagcacagtgtttagtttaatttccctttaggttttcctcacattggtgcataagtggctgactacatgacacaacatgccccattctacttgttgcatacaaagtagaagaggaatgtgaggacaaatttaaagtagaaaatgaaaataaatggcaaaaatacagtgcaaatgctttaaacagtgcactttataaaatagtttgctttattcatacttttttataaagtgcaatattacttaaaacagagagacatgtaccttaatattctgcaataaccattaaaacaaattgccaggaaagagcagtgcaaaattaaaaacatacacatagcttagcatgcatctcagatggatcccgaatacagagtatgggaccttgagttcttatatctttttttttttttttcactttttagaaaaagtttaataatagcaggttatcatcatatgtaaccataaaataaaaacaataagttaaaatcttctctcaagaaataagtatatgccacacataaaattcattacagaatcttttttgaaaacagacccctttctctgataaatcattgtttgaagggtgcaaatttcaaaaacccacattgtccacaaggcaaagcaaaaggtatcatcacagtatgagtcatttcttgttggcagacatctggaaaacctgtgacttacaagcagctcaaatctagccctaattaaatttacaggaacctttgctctttcaagaatagtcttgttggcatcatgctaggttgctaaaaagagtaatatgtgctctattcacagtaacattctctgtccagtgcttttgaatgaggataaccaaacaggttttcctgaaaaaaatcattaggaggcagattccaatgagaccaacgggaaacatttttaaaagcataaaagatcgcctcaggcatatgctgagggaataaaggtgcaatggatcactgatacactcctaccatgcctaagctactgagtccgagaactggaagagggtctccgggttattgctgtcggcaggattgctgggctgcagtgtcttggtgggtgtagttttaccgtgagaatgagaggaagaagaatgggaactctcactggaactgctgcgcgtctcggtactggtgctagtctttttcatttttcttctcttagccaaaggggccttatcaacattctgaaggcaaaacccctctctcttgtatttgttaaaggcgtggaaggttgctttcacacaggtatgcacggcagctccggaagatcctagaatatccggagtcatcagaggattggaggacagctgacttccatcttgtagccattcattgtacctcaagccagacattttaagccttttgtttggatctactgtgagaagtccttggatcaaatctttagcctcttgggatacattcttccaggcttctccttcaaaggagaaatctccctttttaattttcttcatgatttccaccgcgctggtacacgtcaaacttcggtcatgagattggaagggaacctgtcctgacaacattgtgtacaaaatgacgcccaagctccacaggtcacaggactcatcgtagccgttctgattcaagagctctggggcggcataatgaagggtgaagcatggagtcttcaggggctgattatccggtggctttagccgtgcaaatccaaaatcaattattttaatttccaaattgtcattttcatcggtgaacaataaattctcaggtttcagatccctgtgcaccactccaacatcatgcatgtggcttacagctgaaacaagcttcctcatgatgtagctggcttccgtctcactgaagtgcttctttttcttaatgcgctcaaacagttctcctccattcagaagttccatcactagaaacgtgtgaagctgatcatgaaaaacttcatgcaacttcacaatattggggtgtccttcacagagtttcagagctgttatttccttttgagtattggcttccatccttttgctgattattttgactgcaaaagcttggttactttttttatgcacacactttcgacaaattgaaaaactaccttctcccaggggtttgtccttcaaatctaggtcatagtgttgatagaatggagagtccttcatcattgcactcctggcaacatttgtcactccaggacgttcaactcccatgtgaaactgaagagggtctatgacagctgcattacgcttgaataggatggaaggagcaacaaaggaatagccctgaaacagcttctcagaactctggggcagggctgcgggagaataagtgggatccatttctgtgaactcttctgcaaagttactcacatctaattcatctcgaatgactggcttaaatggtgcaggcacttttttggcggctaaatcatcccaatttattttctgaaagaagagatgttctttgatttcatctgcatcacgtggaccacatcccaatctcttcttgggatctttcatcaaaagacgctgaattaggtctttcgctaaagcactcatttcttggggatatggaggctcactttttaatattctcctcatttatttttccgcctctcaaagaacactgtccttcacttccagatgtccaatgtcttcaaatctgttgtttcatatattttgcccattgttaaaattgtttcaggcaggaaagtaaatctggtccctgtttattccatcttctttggaagtggaatctctatttttaatttttaatgtcaaatctagatatctcagcttgggaatttttttctccatcaacagtgaaaggagatgctccagttagtaattcatacattagaacacccaaactccaccagtcaactgccttgtcatgtcctgaatctccccctctgacaatatctggtgccatgtattcaatagttccacaaaaggaatatgctctttcagtttcatcagccacaaactccttactcagaccaaaatctgtcagcaccacatggccattagaatcaagtagaatattctcaagcttaatatcacgatatataatccccaacttgtggagatgttcgagggcaagcacaatctctccaacataaatctgcacctcatgctctgtgaaacgctctctttgagaaagatgagtaaaaagttcaccaccatttatataatctaaaatgagatgaagtttggtttctgtctggaaagcataatgtaatgttaccaaaaatggcgactgcctaatgtgttccaggacttgtcgttctgtccttgtatgctctgtggttttggccttttgaacgattgttgcctttttcaaaactttcatggcatacagctttccagtatcatggccacttattttacgaactagaaatacttttccataagctccagttcctaggaccttcaggagctcaaaattttctattcccaccttctcagcatgtcctgtcaaattagcagtccgcagctcgtgcttgacagtgaggagctgctctcctccgtcgccgccgtccgcgctggtccccgcggcgccgccgctgctgccaccctcctcctccatcttctcctttttttccgatcccgcgggtcgctacgaggggaacccaggagacagcggacgcccgtcccctcgcagccgctgccgcggccccaggagtcggggtgcggcggctccagaactcggacgcaaagacgagtctctttcccgctctggccgcacggctcgctcctcgcctcctcccccttcggcgggcaccgctagtaccgc

SEQ ID NO: 14769 - RNA, 10445 nt, Homo sapiens
  source 1..10445: mol_type = other RNA
gctgggattacaggcatgagccacctcacccggccaataaagcttttagaagaatataagaatatcttcataaccttggtgtgaacatttattaaatacgacgcaaaagtattagcaattaaataaaagactggtatattggacttcataaaatttttggtcatcaaaggaaagcacttagaaagtagaaaagcaaactaaagagaagacatttatggtaaaatatcagacaaaaaccctcatatccataaaatataaaagactcctgcaagtcagtaagaaaaaaagacaacccaataaatatgaacaaatgacttgaacaggcacttaattgaggatagccaaatgactaataaaaatataaaaaggtgttccacacatcactacttatcaggaaaatacaccttaaaatctcagtgaaatacaaaatcaccagaatggttaaaaccacaatcaaatatacacatttgtcagagtggctaaactactagggctgatggtaccaagcactgatgaggatgtggaagaactagaacacttacacattattggtgggtatgtaaattggtacaaccattgttgaaaaccatttggtaatatcttctacagctaaatatatattcatcttatgactcagtagtttcactccttttttttgtctgtttttttgagacagggtctcactctatcgcccaggatggaatgtagtggtgcgatcaaggctcactgcagccagctgtttcacttttaagtggacacacaagagaaatgagtgtacgtgtccattaaaatatatgcacaagaatgcttatggctgctttaaacacaaaagctaaaaattacaaacaaccaaaatgtctatcagtgggagaatggataaattgtgatgtatttatctgatggaatactacagagcaacgaaaaagaacaaactactgttattgctacatgcaacaacatagatgcatttcacagacataatgctgatcaaattaaaccagacacaaaaacctatagactggataattccatgtataggaatgtcaacaacagtgacagaggtcagagtggtggttatgtatgaggactgactgggagcctcatcttgatctgaatgatggttatatgggcgcatatatatgtaaacatttattgagctgtatatttcagacctgtgcactttacacaccatgttgcaataacattttaaacaatatgatcactatctatatgtagttttagtgctccatttggactggtctctggccactggatgtcagtgtttggagcagtgggcagcaggaaaagctggggaaggagtgggaaaacagaggagagagctatcacatgggcttcctagagaaaaataagcactttatgaagcttataagttcctttatgtacacagtagacaaagccttttaaagagatttgtccatacgggcactgaaataacatttttgtaaagtagccttctctatgttgattgcagatgtttctatctcagaatttaagtctacttgctttctcacacagcatcattatttccttattcctaataattttcatcacaaacatttcccagctctgtcccaatcaagttcttatttctctgaacggaattacaatttataaatgtaggtccacatgcagatatcttaataagtagtgaaataccagtgtagaaatacacaaatgagtgtggacacaccatagaaaagcagaaaaatacgagaaaaagtgcatgtacggagtatgggatgaactgatgcagttaaggaagacaactcacaaagcaactcacggctgggcaaagctgggaggctgaggcgggaggattgcttgaagccaggagtttgagactagcctgggcaccatactgataccttgtagctattaaaaaaaaattagctgggcatggtggctcatgcctgtagtctacttagtcagctgcttaggaggctgaggtacaaggattgcttgagcccaggaggtggaggttgcagtgagctgtgatcacgccactgcactccggccagggtgacagagtgagaccctgtctcacacaaaggcaactcatttgagctgaggcttggctatacttttaattgtccacatagaatagaggaaaaacaatgtttttcatcttttttaatcttccatttaccttttagtaagacaaattcttatctttatgtaaaactgtggaagagcagttacatagattgttgcagcttagattattttcaagaagtttaaattctacacataaggatacataccatttttaccagctatactttaaaatgccagtctttaaaaattcctctatgtgtatatgtggtttcttcttcttttcaaaaattcatgcctgtgaagtttttaggaatatttttcaaaactttagtactgaggcattaactgtttatgtgacacagcacctttaaatttctgtttttattcagccaaagaatgagaattattgtacattgctagtatttataatttcagcaaataggatagcagtatagtacctaaaataaactattaggaataactgaatgcctaccacagcaacagagctttaatgaggttaattgtcacatacatatccattccaacatagcagtgcacatttcacatgaccagcctcttatgtagttaaaaataaaactgcagttttaaaatgtcaagttcctcaaccttactggattttaaaacaaagcaaacaaaagaaacaaggattttctaatctatctataagcagaaatgtcagaaaataaagctacagtattccataaaacttaaaatttccttttctaagtcatgacatttctcttttgttctgttttctttttcttctaatattaagaaaatttaaaacgtaaatgaaaaaactgcttaatgtggcaaggaacaagaatgaaactagatttttttttttagtaaaggggcaaattgtataccaacatataaattaaaagtgttatgcaatgagaaacaataatggaaacagcataatactacatactatcccagtttcctgtgctctgaagaacagctgctatactaaatactaacttgacttatctgaagtattcaatactttctgataacccaagcagcattatattaatagttagaatactactacaaaatgtccttctacctctcccacaagaaatacaccaggaaacttaagcctgatgaataactactaagaatcttgtcttttaatacaagtctccttctagacacaaaatcctagctttttgtaatgtggttaaaaggagtaatggaaaagaaatgactgccaataaacatttcctattttgcactagggtgaagaaaccaagacacaaacatttggaagccactttagtttcttattccttttcaccctaatagtaggaaaatattaggcacctacttaattcacaaattcatgaaacagggtggacaacagccttgtgtaggggaagcatttggaatggtaatcaactacttaattacataacagggagctgggcatacaaagaaaagggctcagaagaaatatcttgaaaagtaagcaatatagaaggtgaggacagaagtgaggctaatcaaatgttcttagcaagatgttgcccccctgaaaatatgctcccccaataaaacacgtaaataactactcttaaggaaaatattttctctaaagaatgtcacaatttggagtgaagttacttaacaaaacagggaataaaacctttaatgttggctgtagcagttattttctttgggtagattatacttaaaatatttccttcatacatacttctgttaaaatttttttttcccattcttgagttttacaatgtctcctatccaaacttcaaatttcattagagccggctacatttgttttagtgccagatacaggtatcaagtgatgacagacacttacgtgaggtatacaatcaattaaagactggaaattggggtattatcatgtaagacatttgagaggccaaaagtcatataattttaagatacttcatgatgttacagtaataattcatctatataacaattattttgacataagtggcatatcagaatttaacttatttacttagatcttaaggaatattagatgtattctcacatgaacactcaaatcatgctattattatcagtcactgggagaacagccaaagtaatcaggcagtctaaggcacatatagacccaataatttagaaattttcaccattatgaggtaccctgtttttaataaatatgacaataacaggcgcttgaaatgggggcaaggtgaataagtatccagtcaattgtatacttttataaagtagtgtatttgagaacataaactgagatacaaaaggaatttccttactttaaaaaaagtgacttctatcttagtagatttctttaaaataacttaccttatatttaaaagttagtcatttacatacttaagaaatcaacagtaatctaaaaaaattaaaaggcagttttcttgggtaatgaacctgtgactccaagacagacaacaatgtggaaattaactcaggagactgactttctattctagtaattcagtggtttcttactttataaaggtttggaagaattaatgaatttctttttttcttaagacagggtctcgctctgttgcccaggctggagtgcagtggtgtgatcacagctcactgcagcctcgaactcctgggctcaagcgatcctccacatgttggcctcccatgagccaccatgctcagctaatttttatttttatttttggagagacagtgtctcactatgttgcccaggttggtctctaactcctggtttcaagtgattctccagtcttatactcccaaagcacaaggattacaggcctgagccaccacactcagccaatcaatttcaaaatgctaattaacctctttcagacacacgatctggcagagtaattagaagaaactggtctttcttaacatctttcctctattatcttccttttcttattcttgcctctcaatttgtcatatacagttacaaaatatatgaatcaggatttatgttggcatgaaaattatatgcaatacaatcagtaagtgaagaagggagggggtggtgtggctctagtcccaaagttaatgtcataaggagaaataatgtaagtatttgtatttcttagatcttcttctattttactcttaataccaaaaaaagagtcctatcatttaactttttatatattttgtagtgtttatttttgatgtgaccaaatgaaagctttctgaattttaaagtgcaattcactgtatgttaatacacagcctgcataggacctaactgcttcaaacttggcatcaaatgctgtctttttggtacttataagtagggtgtagataaagatatttgacaagagtgcaacagtgtttgttaaggtcttttcaaaagcccatttgagattattcaggcaggctcatcagttgacagctagcctatctttccttcttcctgttagtctgactgcctttttacccatttcatcgcctgtcgaatcctcctcaagaagaggcaagggaaataaatgaaaatgaaacccattaatttccaatattcacaatgaaatcaatcacatcatcaatctgtatactgtctgaccatttttctggatcattttctattagcaacatagtccctttagtttgtactttataactagtattttctaccaggatgcacagtttaaaaaatggcttgaagagccaaatatgttcccaatatgtccaatataattataaatatggtcattttcttgattactagagatctgtgcctgatggaatcacattttgtgaattagcaatagtttggtaataattcacacaaaatttcccataattactaggaataactgaaagctgggagtagaaaactttcattaactcaatattatgtagccatttgggccagcaaaaagtgtaaaatattattcccaataaccactgtggacaaaatgtgaacaggataatataatattttgaaaatattttaatatttgccattttttgcctgtgctattaatatatacattgatttagtaataaatatactactattacatagagtgcaatatttttagtattcataactggttgaaattaatgctgctataacctcaagaaaggaataaataaatatcatgtccaaattccaaactaatgctcaaaaggttatcattaacaaaaactataaaataaacatgttgggcattatctctttaagcatgattcctgtaaacaaagcaaaaaaatcacttttctcagtcctgacatttcacatgatggctttaaaagaaaatataacacacaaaccctatcacttcttttttttttttttttttttttgcatagggaacgaattaattgtatttttaaatgcagcaatcttttaatgaaatgttttcatcacatagtacttgttttctgtatgaattcagaacttttgagcaataaaagtgctctgcataagtttataaaatatgctttctggatttaaaatttaacagaaaaatttccaaacaagtcataggtatgattctaaaatattatgtacataatatatgactacaggaggaaattcctcactgtagtacaacacagtgtacaaatatgaagcacagtgtttagtttaatttccctttaggttttcctcacattggtgcataagtggctgactacatgacacaacatgccccattctacttgttgcatacaaagtagaagaggaatgtgaggacaaatttaaagtagaaaatgaaaataaatggcaaaaatacagtgcaaatgctttaaacagtgcactttataaaatagtttgctttattcatacttttttataaagtgcaatattacttaaaacagagagacatgtaccttaatattctgcaataaccattaaaacaaattgccaggaaagagcagtgcaaaattaaaaacatacacatagcttagcatgcatctcagatggatcccgaatacagagtatgggaccttgagttcttatatctttttttttttttttcactttttagaaaaagtttaataatagcaggttatcatcatatgtaaccataaaataaaaacaataagttaaaatcttctctcaagaaataagtatatgccacacataaaattcattacagaatcttttttgaaaacagacccctttctctgataaatcattgtttgaagggtgcaaatttcaaaaacccacattgtccacaaggcaaagcaaaaggtatcatcacagtatgagtcatttcttgttggcagacatctggaaaacctgtgacttacaagcagctcaaatctagccctaattaaatttacaggaacctttgctctttcaagaatagtcttgttggcatcatgctaggttgctaaaaagagtaatatgtgctctattcacagtaacattctctgtccagtgcttttgaatgaggataaccaaacaggttttcctgaaaaaaatcattaggaggcagattccaatgagaccaacgggaaacatttttaaaagcataaaagatcgcctcaggcatatgctgagggaataaaggtgcaatggatcactgatacactcctaccatgcctaagctactgagtccgagaactggaagagggtctccgggttattgctgtcggcaggattgctgggctgcagtgtcttggtgggtgtagttttaccgtgagaatgagaggaagaagaatgggaactctcactggaactgctgcgcgtctcggtactggtgctagtctttttcatttttcttctcttagccaaaggggccttatcaacattctgaaggcaaaacccctctctcttgtatttgttaaaggcgtggaaggttgctttcacacaggtatgcacggcagctccggaagatcctagaatatccggagtcatcagaggattggaggacagctgacttccatcttgtagccattcattgtacctcaagccagacattttaagccttttgtttggatctactgtgagaagtccttggatcaaatctttagcctcttgggatacattcttccaggcttctccttcaaaggagaaatctccctttttaattttcttcatgatttccaccgcgctggtacacgtcaaacttcggtcatgagattggaagggaacctgtcctgacaacattgtgtacaaaatgacgcccaagctccacaggtcacaggactcatcgtagccgttctgattcaagagctctggggcggcataatgaagggtgaagcatggagtcttcaggggctgattatccggtggctttagccgtgcaaatccaaaatcaattattttaatttccaaattgtcattttcatcggtgaacaataaattctcaggtttcagatccctgtgcaccactccaacatcatgcatgtggcttacagctgaaacaagcttcctcatgatgtagctggcttccgtctcactgaagtgcttctttttcttaatgcgctcaaacagttctcctccattcagaagttccatcactagaaacgtgtgaagctgatcatgaaaaacttcatgcaacttcacaatattggggtgtccttcacagagtttcagagctgttatttccttttgagtattggcttccatccttttgctgattattttgactgcaaaagcttggttactttttttatgcacacactttcgacaaattgaaaaactaccttctcccaggggtttgtccttcaaatctaggtcatagtgttgatagaatggagagtccttcatcattgcactcctggcaacatttgtcactccaggacgttcaactcccatgtgaaactgaagagggtctatgacagctgcattacgcttgaataggatggaaggagcaacaaaggaatagccctgaaacagcttctcagaactctggggcagggctgcgggagaataagtgggatccatttctgtgaactcttctgcaaagttactcacatctaattcatctcgaatgactggcttaaatggtgcaggcacttttttggcggctaaatcatcccaatttattttctgaaagaagagatgttctttgatttcatctgcatcacgtggaccacatcccaatctcttcttgggatctttcatcaaaagacgctgaattaggtctttcgctaaagcactcatttcttggggatatggaggctcactttttaatattctcctgtaggcagacaaaacttgctagatatctcagcttgggaatttttttctccatcaacagtgaaaggagatgctccagttagtaattcatacattagaacacccaaactccaccagtcaactgccttgtcatgtcctgaatctccccctctgacaatatctggtgccatgtattcaatagttccacaaaaggaatatgctctttcagtttcatcagccacaaactccttactcagaccaaaatctgtcagcaccacatggccattagaatcaagtagaatattctcaagcttaatatcacgatatataatccccaacttgtggagatgttcgagggcaagcacaatctctccaacataaatctgcacctcatgctctgtgaaacgctctctttgagaaagatgagtaaaaagttcaccaccatttatataatctaaaatgagatgaagtttggtttctgtctggaaagcataatgtaatgttaccaaaaatggcgactgcctaatgtgttccaggacttgtcgttctgtccttgtatgctctgtggttttggccttttgaacgattgttgcctttttcaaaactttcatggcatacagctttccagtatcatggccacttattttacgaactagaaatacttttccataagctccagttcctaggaccttcaggagctcaaaattttctattcccaccttctcagcatgtcctgtcaaattagctgggtatggtagtgggtgcctgtaatcccagccacttgggaggctgaggcaggagaatcacttgaacccaggaggcggaggttatagtgagccgagatcagcaccacactccagcctgggcaacagagtagactcgtctcagtccgcagctcgtgcttgacagtgaggagctgctctcctccgtcgccgccgtccgcgctggtccccgcggcgccgccgctgctgccaccctcctcctccatcttctcctttttttccgatcccgcgggtcgctacgaggggaacccaggagacagcggacgcccgtcccctcgcagccgctgccgcggccccaggagtcggggtgcggcggctccagaactcggacgcaaagacgagtctctttcccgctctggccgcacggctcgctcctcgcctcctcccccttcggcgggcaccgctagtaccgc

SEQ ID NO: 14770 - RNA, 10181 nt, Homo sapiens
  source 1..10181: mol_type = other RNA
gctgggattacaggcatgagccacctcacccggccaataaagcttttagaagaatataagaatatcttcataaccttggtgtgaacatttattaaatacgacgcaaaagtattagcaattaaataaaagactggtatattggacttcataaaatttttggtcatcaaaggaaagcacttagaaagtagaaaagcaaactaaagagaagacatttatggtaaaatatcagacaaaaaccctcatatccataaaatataaaagactcctgcaagtcagtaagaaaaaaagacaacccaataaatatgaacaaatgacttgaacaggcacttaattgaggatagccaaatgactaataaaaatataaaaaggtgttccacacatcactacttatcaggaaaatacaccttaaaatctcagtgaaatacaaaatcaccagaatggttaaaaccacaatcaaatatacacatttgtcagagtggctaaactactagggctgatggtaccaagcactgatgaggatgtggaagaactagaacacttacacattattggtgggtatgtaaattggtacaaccattgttgaaaaccatttggtaatatcttctacagctaaatatatattcatcttatgactcagtagtttcactccttttttttgtctgtttttttgagacagggtctcactctatcgcccaggatggaatgtagtggtgcgatcaaggctcactgcagccagctgtttcacttttaagtggacacacaagagaaatgagtgtacgtgtccattaaaatatatgcacaagaatgcttatggctgctttaaacacaaaagctaaaaattacaaacaaccaaaatgtctatcagtgggagaatggataaattgtgatgtatttatctgatggaatactacagagcaacgaaaaagaacaaactactgttattgctacatgcaacaacatagatgcatttcacagacataatgctgatcaaattaaaccagacacaaaaacctatagactggataattccatgtataggaatgtcaacaacagtgacagaggtcagagtggtggttatgtatgaggactgactgggagcctcatcttgatctgaatgatggttatatgggcgcatatatatgtaaacatttattgagctgtatatttcagacctgtgcactttacacaccatgttgcaataacattttaaacaatatgatcactatctatatgtagttttagtgctccatttggactggtctctggccactggatgtcagtgtttggagcagtgggcagcaggaaaagctggggaaggagtgggaaaacagaggagagagctatcacatgggcttcctagagaaaaataagcactttatgaagcttataagttcctttatgtacacagtagacaaagccttttaaagagatttgtccatacgggcactgaaataacatttttgtaaagtagccttctctatgttgattgcagatgtttctatctcagaatttaagtctacttgctttctcacacagcatcattatttccttattcctaataattttcatcacaaacatttcccagctctgtcccaatcaagttcttatttctctgaacggaattacaatttataaatgtaggtccacatgcagatatcttaataagtagtgaaataccagtgtagaaatacacaaatgagtgtggacacaccatagaaaagcagaaaaatacgagaaaaagtgcatgtacggagtatgggatgaactgatgcagttaaggaagacaactcacaaagcaactcacggctgggcaaagctgggaggctgaggcgggaggattgcttgaagccaggagtttgagactagcctgggcaccatactgataccttgtagctattaaaaaaaaattagctgggcatggtggctcatgcctgtagtctacttagtcagctgcttaggaggctgaggtacaaggattgcttgagcccaggaggtggaggttgcagtgagctgtgatcacgccactgcactccggccagggtgacagagtgagaccctgtctcacacaaaggcaactcatttgagctgaggcttggctatacttttaattgtccacatagaatagaggaaaaacaatgtttttcatcttttttaatcttccatttaccttttagtaagacaaattcttatctttatgtaaaactgtggaagagcagttacatagattgttgcagcttagattattttcaagaagtttaaattctacacataaggatacataccatttttaccagctatactttaaaatgccagtctttaaaaattcctctatgtgtatatgtggtttcttcttcttttcaaaaattcatgcctgtgaagtttttaggaatatttttcaaaactttagtactgaggcattaactgtttatgtgacacagcacctttaaatttctgtttttattcagccaaagaatgagaattattgtacattgctagtatttataatttcagcaaataggatagcagtatagtacctaaaataaactattaggaataactgaatgcctaccacagcaacagagctttaatgaggttaattgtcacatacatatccattccaacatagcagtgcacatttcacatgaccagcctcttatgtagttaaaaataaaactgcagttttaaaatgtcaagttcctcaaccttactggattttaaaacaaagcaaacaaaagaaacaaggattttctaatctatctataagcagaaatgtcagaaaataaagctacagtattccataaaacttaaaatttccttttctaagtcatgacatttctcttttgttctgttttctttttcttctaatattaagaaaatttaaaacgtaaatgaaaaaactgcttaatgtggcaaggaacaagaatgaaactagatttttttttttagtaaaggggcaaattgtataccaacatataaattaaaagtgttatgcaatgagaaacaataatggaaacagcataatactacatactatcccagtttcctgtgctctgaagaacagctgctatactaaatactaacttgacttatctgaagtattcaatactttctgataacccaagcagcattatattaatagttagaatactactacaaaatgtccttctacctctcccacaagaaatacaccaggaaacttaagcctgatgaataactactaagaatcttgtcttttaatacaagtctccttctagacacaaaatcctagctttttgtaatgtggttaaaaggagtaatggaaaagaaatgactgccaataaacatttcctattttgcactagggtgaagaaaccaagacacaaacatttggaagccactttagtttcttattccttttcaccctaatagtaggaaaatattaggcacctacttaattcacaaattcatgaaacagggtggacaacagccttgtgtaggggaagcatttggaatggtaatcaactacttaattacataacagggagctgggcatacaaagaaaagggctcagaagaaatatcttgaaaagtaagcaatatagaaggtgaggacagaagtgaggctaatcaaatgttcttagcaagatgttgcccccctgaaaatatgctcccccaataaaacacgtaaataactactcttaaggaaaatattttctctaaagaatgtcacaatttggagtgaagttacttaacaaaacagggaataaaacctttaatgttggctgtagcagttattttctttgggtagattatacttaaaatatttccttcatacatacttctgttaaaatttttttttcccattcttgagttttacaatgtctcctatccaaacttcaaatttcattagagccggctacatttgttttagtgccagatacaggtatcaagtgatgacagacacttacgtgaggtatacaatcaattaaagactggaaattggggtattatcatgtaagacatttgagaggccaaaagtcatataattttaagatacttcatgatgttacagtaataattcatctatataacaattattttgacataagtggcatatcagaatttaacttatttacttagatcttaaggaatattagatgtattctcacatgaacactcaaatcatgctattattatcagtcactgggagaacagccaaagtaatcaggcagtctaaggcacatatagacccaataatttagaaattttcaccattatgaggtaccctgtttttaataaatatgacaataacaggcgcttgaaatgggggcaaggtgaataagtatccagtcaattgtatacttttataaagtagtgtatttgagaacataaactgagatacaaaaggaatttccttactttaaaaaaagtgacttctatcttagtagatttctttaaaataacttaccttatatttaaaagttagtcatttacatacttaagaaatcaacagtaatctaaaaaaattaaaaggcagttttcttgggtaatgaacctgtgactccaagacagacaacaatgtggaaattaactcaggagactgactttctattctagtaattcagtggtttcttactttataaaggtttggaagaattaatgaatttctttttttcttaagacagggtctcgctctgttgcccaggctggagtgcagtggtgtgatcacagctcactgcagcctcgaactcctgggctcaagcgatcctccacatgttggcctcccatgagccaccatgctcagctaatttttatttttatttttggagagacagtgtctcactatgttgcccaggttggtctctaactcctggtttcaagtgattctccagtcttatactcccaaagcacaaggattacaggcctgagccaccacactcagccaatcaatttcaaaatgctaattaacctctttcagacacacgatctggcagagtaattagaagaaactggtctttcttaacatctttcctctattatcttccttttcttattcttgcctctcaatttgtcatatacagttacaaaatatatgaatcaggatttatgttggcatgaaaattatatgcaatacaatcagtaagtgaagaagggagggggtggtgtggctctagtcccaaagttaatgtcataaggagaaataatgtaagtatttgtatttcttagatcttcttctattttactcttaataccaaaaaaagagtcctatcatttaactttttatatattttgtagtgtttatttttgatgtgaccaaatgaaagctttctgaattttaaagtgcaattcactgtatgttaatacacagcctgcataggacctaactgcttcaaacttggcatcaaatgctgtctttttggtacttataagtagggtgtagataaagatatttgacaagagtgcaacagtgtttgttaaggtcttttcaaaagcccatttgagattattcaggcaggctcatcagttgacagctagcctatctttccttcttcctgttagtctgactgcctttttacccatttcatcgcctgtcgaatcctcctcaagaagaggcaagggaaataaatgaaaatgaaacccattaatttccaatattcacaatgaaatcaatcacatcatcaatctgtatactgtctgaccatttttctggatcattttctattagcaacatagtccctttagtttgtactttataactagtattttctaccaggatgcacagtttaaaaaatggcttgaagagccaaatatgttcccaatatgtccaatataattataaatatggtcattttcttgattactagagatctgtgcctgatggaatcacattttgtgaattagcaatagtttggtaataattcacacaaaatttcccataattactaggaataactgaaagctgggagtagaaaactttcattaactcaatattatgtagccatttgggccagcaaaaagtgtaaaatattattcccaataaccactgtggacaaaatgtgaacaggataatataatattttgaaaatattttaatatttgccattttttgcctgtgctattaatatatacattgatttagtaataaatatactactattacatagagtgcaatatttttagtattcataactggttgaaattaatgctgctataacctcaagaaaggaataaataaatatcatgtccaaattccaaactaatgctcaaaaggttatcattaacaaaaactataaaataaacatgttgggcattatctctttaagcatgattcctgtaaacaaagcaaaaaaatcacttttctcagtcctgacatttcacatgatggctttaaaagaaaatataacacacaaaccctatcacttcttttttttttttttttttttttgcatagggaacgaattaattgtatttttaaatgcagcaatcttttaatgaaatgttttcatcacatagtacttgttttctgtatgaattcagaacttttgagcaataaaagtgctctgcataagtttataaaatatgctttctggatttaaaatttaacagaaaaatttccaaacaagtcataggtatgattctaaaatattatgtacataatatatgactacaggaggaaattcctcactgtagtacaacacagtgtacaaatatgaagcacagtgtttagtttaatttccctttaggttttcctcacattggtgcataagtggctgactacatgacacaacatgccccattctacttgttgcatacaaagtagaagaggaatgtgaggacaaatttaaagtagaaaatgaaaataaatggcaaaaatacagtgcaaatgctttaaacagtgcactttataaaatagtttgctttattcatacttttttataaagtgcaatattacttaaaacagagagacatgtaccttaatattctgcaataaccattaaaacaaattgccaggaaagagcagtgcaaaattaaaaacatacacatagcttagcatgcatctcagatggatcccgaatacagagtatgggaccttgagttcttatatctttttttttttttttcactttttagaaaaagtttaataatagcaggttatcatcatatgtaaccataaaataaaaacaataagttaaaatcttctctcaagaaataagtatatgccacacataaaattcattacagaatcttttttgaaaacagacccctttctctgataaatcattgtttgaagggtgcaaatttcaaaaacccacattgtccacaaggcaaagcaaaaggtatcatcacagtatgagtcatttcttgttggcagacatctggaaaacctgtgacttacaagcagctcaaatctagccctaattaaatttacaggaacctttgctctttcaagaatagtcttgttggcatcatgctaggttgctaaaaagagtaatatgtgctctattcacagtaacattctctgtccagtgcttttgaatgaggataaccaaacaggttttcctgaaaaaaatcattaggaggcagattccaatgagaccaacgggaaacatttttaaaagcataaaagatcgcctcaggcatatgctgagggaataaaggtgcaatggatcactgatacactcctaccatgcctaagctactgagtccgagaactggaagagggtctccgggttattgctgtcggcaggattgctgggctgcagtgtcttggtgggtgtagttttaccgtgagaatgagaggaagaagaatgggaactctcactggaactgctgcgcgtctcggtactggtgctagtctttttcatttttcttctcttagccaaaggggccttatcaacattctgaaggcaaaacccctctctcttgtatttgttaaaggcgtggaaggttgctttcacacaggtatgcacggcagctccggaagatcctagaatatccggagtcatcagaggattggaggacagctgacttccatcttgtagccattcattgtacctcaagccagacattttaagccttttgtttggatctactgtgagaagtccttggatcaaatctttagcctcttgggatacattcttccaggcttctccttcaaaggagaaatctccctttttaattttcttcatgatttccaccgcgctggtacacgtcaaacttcggtcatgagattggaagggaacctgtcctgacaacattgtgtacaaaatgacgcccaagctccacaggtcacaggactcatcgtagccgttctgattcaagagctctggggcggcataatgaagggtgaagcatggagtcttcaggggctgattatccggtggctttagccgtgcaaatccaaaatcaattattttaatttccaaattgtcattttcatcggtgaacaataaattctcaggtttcagatccctgtgcaccactccaacatcatgcatgtggcttacagctgaaacaagcttcctcatgatgtagctggcttccgtctcactgaagtgcttctttttcttaatgcgctcaaacagttctcctccattcagaagttccatcactagaaacgtgtgaagctgatcatgaaaaacttcatgcaacttcacaatattggggtgtccttcacagagtttcagagctgttatttccttttgagtattggcttccatccttttgctgattattttgactgcaaaagcttggttactttttttatgcacacactttcgacaaattgaaaaactaccttctcccaggggtttgtccttcaaatctaggtcatagtgttgatagaatggagagtccttcatcattgcactcctggcaacatttgtcactccaggacgttcaactcccatgtgaaactgaagagggtctatgacagctgcattacgcttgaataggatggaaggagcaacaaaggaatagccctgaaacagcttctcagaactctggggcagggctgcgggagaataagtgggatccatttctgtgaactcttctgcaaagttactcacatctaattcatctcgaatgactggcttaaatggtgcaggcacttttttggcggctaaatcatcccaatttattttctgaaagaagagatgttctttgatttcatctgcatcacgtggaccacatcccaatctcttcttgggatctttcatcaaaagacgctgaattaggtctttcgctaaagcactcatttcttggggatatggaggctcactttttaatattctccttgtcatgtcctgaatctccccctctgacaatatctggtgccatgtattcaatagttccacaaaaggaatatgctctttcagtttcatcagccacaaactccttactcagaccaaaatctgtcagcaccacatggccattagaatcaagtagaatattctcaagcttaatatcacgatatataatccccaacttgtggagatgttcgagggcaagcacaatctctccaacataaatctgcacctcatgctctgtgaaacgctctctttgagaaagatgagtaaaaagttcaccaccatttatataatctaaaatgagatgaagtttggtttctgtctggaaagcataatgtaatgttaccaaaaatggcgactgcctaatgtgttccaggacttgtcgttctgtccttgtatgctctgtggttttggccttttgaacgattgttgcctttttcaaaactttcatggcatacagctttccagtatcatggccacttattttacgaactagaaatacttttccataagctccagttcctaggaccttcaggagctcaaaattttctattcccaccttctcagcatgtcctgtcaaattagcagtccgcagctcgtgcttgacagtgaggagctgctctcctccgtcgccgccgtccgcgctggtccccgcggcgccgccgctgctgccaccctcctcctccatcttctcctttttttccgatcccgcgggtcgctacgaggggaacccaggagacagcggacgcccgtcccctcgcagccgctgccgcggccccaggagtcggggtgcggcggctccagaactcggacgcaaagacgagtctctttcccgctctggccgcacggctcgctcctcgcctcctcccccttcggcgggcaccgctagtaccgc

SEQ ID NO: 14771 - RNA, 10123 nt, Homo sapiens
  source 1..10123: mol_type = other RNA
gctgggattacaggcatgagccacctcacccggccaataaagcttttagaagaatataagaatatcttcataaccttggtgtgaacatttattaaatacgacgcaaaagtattagcaattaaataaaagactggtatattggacttcataaaatttttggtcatcaaaggaaagcacttagaaagtagaaaagcaaactaaagagaagacatttatggtaaaatatcagacaaaaaccctcatatccataaaatataaaagactcctgcaagtcagtaagaaaaaaagacaacccaataaatatgaacaaatgacttgaacaggcacttaattgaggatagccaaatgactaataaaaatataaaaaggtgttccacacatcactacttatcaggaaaatacaccttaaaatctcagtgaaatacaaaatcaccagaatggttaaaaccacaatcaaatatacacatttgtcagagtggctaaactactagggctgatggtaccaagcactgatgaggatgtggaagaactagaacacttacacattattggtgggtatgtaaattggtacaaccattgttgaaaaccatttggtaatatcttctacagctaaatatatattcatcttatgactcagtagtttcactccttttttttgtctgtttttttgagacagggtctcactctatcgcccaggatggaatgtagtggtgcgatcaaggctcactgcagccagctgtttcacttttaagtggacacacaagagaaatgagtgtacgtgtccattaaaatatatgcacaagaatgcttatggctgctttaaacacaaaagctaaaaattacaaacaaccaaaatgtctatcagtgggagaatggataaattgtgatgtatttatctgatggaatactacagagcaacgaaaaagaacaaactactgttattgctacatgcaacaacatagatgcatttcacagacataatgctgatcaaattaaaccagacacaaaaacctatagactggataattccatgtataggaatgtcaacaacagtgacagaggtcagagtggtggttatgtatgaggactgactgggagcctcatcttgatctgaatgatggttatatgggcgcatatatatgtaaacatttattgagctgtatatttcagacctgtgcactttacacaccatgttgcaataacattttaaacaatatgatcactatctatatgtagttttagtgctccatttggactggtctctggccactggatgtcagtgtttggagcagtgggcagcaggaaaagctggggaaggagtgggaaaacagaggagagagctatcacatgggcttcctagagaaaaataagcactttatgaagcttataagttcctttatgtacacagtagacaaagccttttaaagagatttgtccatacgggcactgaaataacatttttgtaaagtagccttctctatgttgattgcagatgtttctatctcagaatttaagtctacttgctttctcacacagcatcattatttccttattcctaataattttcatcacaaacatttcccagctctgtcccaatcaagttcttatttctctgaacggaattacaatttataaatgtaggtccacatgcagatatcttaataagtagtgaaataccagtgtagaaatacacaaatgagtgtggacacaccatagaaaagcagaaaaatacgagaaaaagtgcatgtacggagtatgggatgaactgatgcagttaaggaagacaactcacaaagcaactcacggctgggcaaagctgggaggctgaggcgggaggattgcttgaagccaggagtttgagactagcctgggcaccatactgataccttgtagctattaaaaaaaaattagctgggcatggtggctcatgcctgtagtctacttagtcagctgcttaggaggctgaggtacaaggattgcttgagcccaggaggtggaggttgcagtgagctgtgatcacgccactgcactccggccagggtgacagagtgagaccctgtctcacacaaaggcaactcatttgagctgaggcttggctatacttttaattgtccacatagaatagaggaaaaacaatgtttttcatcttttttaatcttccatttaccttttagtaagacaaattcttatctttatgtaaaactgtggaagagcagttacatagattgttgcagcttagattattttcaagaagtttaaattctacacataaggatacataccatttttaccagctatactttaaaatgccagtctttaaaaattcctctatgtgtatatgtggtttcttcttcttttcaaaaattcatgcctgtgaagtttttaggaatatttttcaaaactttagtactgaggcattaactgtttatgtgacacagcacctttaaatttctgtttttattcagccaaagaatgagaattattgtacattgctagtatttataatttcagcaaataggatagcagtatagtacctaaaataaactattaggaataactgaatgcctaccacagcaacagagctttaatgaggttaattgtcacatacatatccattccaacatagcagtgcacatttcacatgaccagcctcttatgtagttaaaaataaaactgcagttttaaaatgtcaagttcctcaaccttactggattttaaaacaaagcaaacaaaagaaacaaggattttctaatctatctataagcagaaatgtcagaaaataaagctacagtattccataaaacttaaaatttccttttctaagtcatgacatttctcttttgttctgttttctttttcttctaatattaagaaaatttaaaacgtaaatgaaaaaactgcttaatgtggcaaggaacaagaatgaaactagatttttttttttagtaaaggggcaaattgtataccaacatataaattaaaagtgttatgcaatgagaaacaataatggaaacagcataatactacatactatcccagtttcctgtgctctgaagaacagctgctatactaaatactaacttgacttatctgaagtattcaatactttctgataacccaagcagcattatattaatagttagaatactactacaaaatgtccttctacctctcccacaagaaatacaccaggaaacttaagcctgatgaataactactaagaatcttgtcttttaatacaagtctccttctagacacaaaatcctagctttttgtaatgtggttaaaaggagtaatggaaaagaaatgactgccaataaacatttcctattttgcactagggtgaagaaaccaagacacaaacatttggaagccactttagtttcttattccttttcaccctaatagtaggaaaatattaggcacctacttaattcacaaattcatgaaacagggtggacaacagccttgtgtaggggaagcatttggaatggtaatcaactacttaattacataacagggagctgggcatacaaagaaaagggctcagaagaaatatcttgaaaagtaagcaatatagaaggtgaggacagaagtgaggctaatcaaatgttcttagcaagatgttgcccccctgaaaatatgctcccccaataaaacacgtaaataactactcttaaggaaaatattttctctaaagaatgtcacaatttggagtgaagttacttaacaaaacagggaataaaacctttaatgttggctgtagcagttattttctttgggtagattatacttaaaatatttccttcatacatacttctgttaaaatttttttttcccattcttgagttttacaatgtctcctatccaaacttcaaatttcattagagccggctacatttgttttagtgccagatacaggtatcaagtgatgacagacacttacgtgaggtatacaatcaattaaagactggaaattggggtattatcatgtaagacatttgagaggccaaaagtcatataattttaagatacttcatgatgttacagtaataattcatctatataacaattattttgacataagtggcatatcagaatttaacttatttacttagatcttaaggaatattagatgtattctcacatgaacactcaaatcatgctattattatcagtcactgggagaacagccaaagtaatcaggcagtctaaggcacatatagacccaataatttagaaattttcaccattatgaggtaccctgtttttaataaatatgacaataacaggcgcttgaaatgggggcaaggtgaataagtatccagtcaattgtatacttttataaagtagtgtatttgagaacataaactgagatacaaaaggaatttccttactttaaaaaaagtgacttctatcttagtagatttctttaaaataacttaccttatatttaaaagttagtcatttacatacttaagaaatcaacagtaatctaaaaaaattaaaaggcagttttcttgggtaatgaacctgtgactccaagacagacaacaatgtggaaattaactcaggagactgactttctattctagtaattcagtggtttcttactttataaaggtttggaagaattaatgaatttctttttttcttaagacagggtctcgctctgttgcccaggctggagtgcagtggtgtgatcacagctcactgcagcctcgaactcctgggctcaagcgatcctccacatgttggcctcccatgagccaccatgctcagctaatttttatttttatttttggagagacagtgtctcactatgttgcccaggttggtctctaactcctggtttcaagtgattctccagtcttatactcccaaagcacaaggattacaggcctgagccaccacactcagccaatcaatttcaaaatgctaattaacctctttcagacacacgatctggcagagtaattagaagaaactggtctttcttaacatctttcctctattatcttccttttcttattcttgcctctcaatttgtcatatacagttacaaaatatatgaatcaggatttatgttggcatgaaaattatatgcaatacaatcagtaagtgaagaagggagggggtggtgtggctctagtcccaaagttaatgtcataaggagaaataatgtaagtatttgtatttcttagatcttcttctattttactcttaataccaaaaaaagagtcctatcatttaactttttatatattttgtagtgtttatttttgatgtgaccaaatgaaagctttctgaattttaaagtgcaattcactgtatgttaatacacagcctgcataggacctaactgcttcaaacttggcatcaaatgctgtctttttggtacttataagtagggtgtagataaagatatttgacaagagtgcaacagtgtttgttaaggtcttttcaaaagcccatttgagattattcaggcaggctcatcagttgacagctagcctatctttccttcttcctgttagtctgactgcctttttacccatttcatcgcctgtcgaatcctcctcaagaagaggcaagggaaataaatgaaaatgaaacccattaatttccaatattcacaatgaaatcaatcacatcatcaatctgtatactgtctgaccatttttctggatcattttctattagcaacatagtccctttagtttgtactttataactagtattttctaccaggatgcacagtttaaaaaatggcttgaagagccaaatatgttcccaatatgtccaatataattataaatatggtcattttcttgattactagagatctgtgcctgatggaatcacattttgtgaattagcaatagtttggtaataattcacacaaaatttcccataattactaggaataactgaaagctgggagtagaaaactttcattaactcaatattatgtagccatttgggccagcaaaaagtgtaaaatattattcccaataaccactgtggacaaaatgtgaacaggataatataatattttgaaaatattttaatatttgccattttttgcctgtgctattaatatatacattgatttagtaataaatatactactattacatagagtgcaatatttttagtattcataactggttgaaattaatgctgctataacctcaagaaaggaataaataaatatcatgtccaaattccaaactaatgctcaaaaggttatcattaacaaaaactataaaataaacatgttgggcattatctctttaagcatgattcctgtaaacaaagcaaaaaaatcacttttctcagtcctgacatttcacatgatggctttaaaagaaaatataacacacaaaccctatcacttcttttttttttttttttttttttgcatagggaacgaattaattgtatttttaaatgcagcaatcttttaatgaaatgttttcatcacatagtacttgttttctgtatgaattcagaacttttgagcaataaaagtgctctgcataagtttataaaatatgctttctggatttaaaatttaacagaaaaatttccaaacaagtcataggtatgattctaaaatattatgtacataatatatgactacaggaggaaattcctcactgtagtacaacacagtgtacaaatatgaagcacagtgtttagtttaatttccctttaggttttcctcacattggtgcataagtggctgactacatgacacaacatgccccattctacttgttgcatacaaagtagaagaggaatgtgaggacaaatttaaagtagaaaatgaaaataaatggcaaaaatacagtgcaaatgctttaaacagtgcactttataaaatagtttgctttattcatacttttttataaagtgcaatattacttaaaacagagagacatgtaccttaatattctgcaataaccattaaaacaaattgccaggaaagagcagtgcaaaattaaaaacatacacatagcttagcatgcatctcagatggatcccgaatacagagtatgggaccttgagttcttatatctttttttttttttttcactttttagaaaaagtttaataatagcaggttatcatcatatgtaaccataaaataaaaacaataagttaaaatcttctctcaagaaataagtatatgccacacataaaattcattacagaatcttttttgaaaacagacccctttctctgataaatcattgtttgaagggtgcaaatttcaaaaacccacattgtccacaaggcaaagcaaaaggtatcatcacagtatgagtcatttcttgttggcagacatctggaaaacctgtgacttacaagcagctcaaatctagccctaattaaatttacaggaacctttgctctttcaagaatagtcttgttggcatcatgctaggttgctaaaaagagtaatatgtgctctattcacagtaacattctctgtccagtgcttttgaatgaggataaccaaacaggttttcctgaaaaaaatcattaggaggcagattccaatgagaccaacgggaaacatttttaaaagcataaaagatcgcctcaggcatatgctgagggaataaaggtgcaatggatcactgatacactcctaccatgcctaagctactgagtccgagaactggaagagggtctccgggttattgctgtcggcaggattgctgggctgcagtgtcttggtgggtgtagttttaccgtgagaatgagaggaagaagaatgggaactctcactggaactgctgcgcgtctcggtactggtgctagtctttttcatttttcttctcttagccaaaggggccttatcaacattctgaaggcaaaacccctctctcttgtatttgttaaaggcgtggaaggttgctttcacacaggtatgcacggcagctccggaagatcctagaatatccggagtcatcagaggattggaggacagctgacttccatcttgtagccattcattgtacctcaagccagacattttaagccttttgtttggatctactgtgagaagtccttggatcaaatctttagcctcttgggatacattcttccaggcttctccttcaaaggagaaatctccctttttaattttcttcatgatttccaccgcgctggtacacgtcaaacttcggtcatgagattggaagggaacctgtcctgacaacattgtgtacaaaatgacgcccaagctccacaggtcacaggactcatcgtagccgttctgattcaagagctctggggcggcataatgaagggtgaagcatggagtcttcaggggctgattatccggtggctttagccgtgcaaatccaaaatcaattattttaatttccaaattgtcattttcatcggtgaacaataaattctcaggtttcagatccctgtgcaccactccaacatcatgcatgtggcttacagctgaaacaagcttcctcatgatgtagctggcttccgtctcactgaagtgcttctttttcttaatgcgctcaaacagttctcctccattcagaagttccatcactagaaacgtgtgaagctgatcatgaaaaacttcatgcaacttcacaatattggggtgtccttcacagagtttcagagctgttatttccttttgagtattggcttccatccttttgctgattattttgactgcaaaagcttggttactttttttatgcacacactttcgacaaattgaaaaactaccttctcccaggggtttgtccttcaaatctaggtcatagtgttgatagaatggagagtccttcatcattgcactcctggcaacatttgtcactccaggacgttcaactcccatgtgaaactgaagagggtctatgacagctgcattacgcttgaataggatggaaggagcaacaaaggaatagccctgaaagaagagatgttctttgatttcatctgcatcacgtggaccacatcccaatctcttcttgggatctttcatcaaaagacgctgaattaggtctttcgctaaagcactcatttcttggggatatggaggctcactttttaatattctcctagatatctcagcttgggaatttttttctccatcaacagtgaaaggagatgctccagttagtaattcatacattagaacacccaaactccaccagtcaactgccttgtcatgtcctgaatctccccctctgacaatatctggtgccatgtattcaatagttccacaaaaggaatatgctctttcagtttcatcagccacaaactccttactcagaccaaaatctgtcagcaccacatggccattagaatcaagtagaatattctcaagcttaatatcacgatatataatccccaacttgtggagatgttcgagggcaagcacaatctctccaacataaatctgcacctcatgctctgtgaaacgctctctttgagaaagatgagtaaaaagttcaccaccatttatataatctaaaatgagatgaagtttggtttctgtctggaaagcataatgtaatgttaccaaaaatggcgactgcctaatgtgttccaggacttgtcgttctgtccttgtatgctctgtggttttggccttttgaacgattgttgcctttttcaaaactttcatggcatacagctttccagtatcatggccacttattttacgaactagaaatacttttccataagctccagttcctaggaccttcaggagctcaaaattttctattcccaccttctcagcatgtcctgtcaaattagcagtccgcagctcgtgcttgacagtgaggagctgctctcctccgtcgccgccgtccgcgctggtccccgcggcgccgccgctgctgccaccctcctcctccatcttctcctttttttccgatcccgcgggtcgctacgaggggaacccaggagacagcggacgcccgtcccctcgcagccgctgccgcggccccaggagtcggggtgcggcggctccagaactcggacgcaaagacgagtctctttcccgctctggccgcacggctcgctcctcgcctcctcccccttcggcgggcaccgctagtaccgc

SEQ ID NO: 14772 - RNA, 4853 nt, Homo sapiens
  source 1..4853: mol_type = other RNA
gctgggattacaggcatgagccacctcacccggcccttttaatcattcttaatgggcttataagcagttattaagtcccccttcagccttctcagaacctcattttacttgcattgaagctgagagcttccaaggaaagcatttgactccgggccccacagatttgcaatgccttaaatgggcaatcagccacttcactcactttaacctgcataaatgaacagttctgccttcttttgcaaagtttaaatccattcaagggagttccctggcaaccaacccttattaataaatcacgctcaatctaggccaggacaggcattttgcaaatgcttcttttgcttgagaagtgacactggcactaggcacacagtaaacaagctgctgctctctctgaagctctacatttgctggatccagtctgtctcccacaggaccttgtggacctggtaggctctcacctgactccccagttgggaagggagtgcttccctaatgaacactcacctggacctttcttagggttactggactagggtcgcagcagctgggcagcagggcatagagctcgagtgaagcttgctcaggctctgctaggcacacattggaaagttacatttcctattccatcataataccatttattcccagttcattgctcatgcctacaggtggaagtctgagttttatgtctagatggggcttccagtatgtccccactcagagtcctgcagttccttccaatcataggaagtgggaaggagcaaggcaggtaggttgtaaggctgatggtgtttcagctttgaggaaaaagtgatttcacttcaatagtaattttaaccagaatggctaaagttaaaaggattgacaatcccaagtgttggcaaggatagagagcaattgcaactctcagtgtttgctgctggaatgtgaatcagagccaccactttggaactctttggcagatccagcaattgctccagcaatcccactcttagatatatgagcaaaaaagtgagtgtttatgttcaccaaaagacatgtacaagaaagttcatagtgttgtaattcacttttattttttttttctgagatggagtcttgctttgtcacccaggctagagtgcagtggcacaatctcaactcactgtaacctccacctctcaggtttaagcagttctccctacctcagcctcccaagtagctgggattacatgtgcccaccaccacaccaagctaatttttgtattttttagtagagacagggttttgccatctaggccaggctgatcttgaactcctgaccttaggtgatctgcccaccttggcaaagtgctggcattacaggcatgagccatcatgccctgcctgtagttcacttttaagtatattttttaaaagtaaaaaatctgaagcagctgccacccaagtgtagaatagataaattgtgatataatcatagaatgaaaccagacataaccatgaagagaactgaactactgctagacaggacaacgtggatgaatctcacatgcaggatgctgatccggacaccacaagaaaaaacaaaagaaggtgcctactgagttttcttctttccagatgaccaactcttaacttactcatctgtttttttcactgttctgcttcttttgaagaagatttgaggtgacttacaaaggtgtatggcatatttataactgaagaaatctgggtgatgttaaaacgagggcaggaaaataaggtggaaaccagatgtaaggatagtcttcactatttatgtcaggaattcctacaaactttctatggtgaacagaatagagcttcctagcagtcaatgcaaagaagaaacacaacaattccacaccccaaagttaacagtcttgcttatcagaagcacaggtagttctgaaatctgatagaaaatgttcctgtatcatttcagaacacgcaactatgtgatcaaacccctttctatttgtttaaaaatttgtcaaacatcccatgtttgaccctggatgtctgaatcccctcagcccacattttcccccctacaccatgcccacaccatccccatagaatttagggtgaggcagcatctcagtgattgacaggcccctccttagaccccgtttactttcctgggtgtggtttggggtaagccctgttcatgaaggctggatttctgttctttgggttgcccagcttgccaccctcatttctggaacccagaccagcatcctcagcccacgctttgccactcagctcatcttcttcccagttggcacttctcagtgaccccatcccttccccagcagtgactctgcgtggggcagctccctggtggctggactctttccattttggcatttgggttagtggatctttccactttctggctccagtttttgagttgaattcatatgtttccccggtcactggatctatggcttctccatcaaagatagtgttcatctggatagtttccaccacgacgtctctctctgcagtcttcgtttagaggttccttgttcttcccagtcttgcaggggcagtgtctgtggatggctttggccaataggacgaccaggtacacgaggagacccagaagcaatatggagcccaaagtgatgacaaacggcacgtaccatgcagatggagagtaaacgtttttcctcaggacctgataggtgaccctgggcctgggggtcgtggtgatgatagtggttgggtggggaatgactttaatactcagtgtcactgttcctgtctcaacaagagcctccgctttcttcctgtcagacatcaagttgtcatcagttacgtagacaagtagcttgtagtcccagatcttatcaaacccaccagcatagtcaaagcgagatgtaagcagcaggcgtgtgacattggaaccagcattgggagagaaggtgaaatgattgttgacgttacctgggccaatggaataacggaaagatctggggctggaatcaaggtcggtacatgtcagcttgaaattctgaatatttgtgccaactttcagatccactgggagggccaggaaataagagtttggagtacaaattggcttttcatcattttcttcaaggatgttcacagtaacagtgacagagcttgtgtcttcgttgttggtggcctggattctgagaatatagatgggggttgtttcacagtccactttagttaccagctggagttctcctgtcttgggattaatccaaaatacatttggatactggaggctggcccctccagtggagatggagtacaggaggctgctctgggggaggtctttatcagtggctcgcacctgtcccactcgggttctggcgggccttctttctgacacatcaaatacataggatggcctatcaaaaatgagaggaaactcattttctgggcttgttaggatataaacgtagacgttatttttatagtaagggggggccacatcctgcacctggattatcaccgtatatttattgccggctgctaggttacttggattttcgtagtctagatcaccaatcagcacaatcttcccagagccagctggatcctgtaaaaatctgctgccgctccccactccagatggcatggtgaagttgaatctgttgtttggtgcctcactgtcatcatcaaagcagaacttgtttaggtcaagaagcaacgtccccttggctgttctttccggcaccataatgctgaaggtgaacttttggcatgtggcaggattgtcgttgacgtcttccacaatgaaggttatctggatgcgattctcctgacccccatatggtctgtccttcactagaacttccagggaaatggtgggattttgtctcaattcacctgcatctcggtctatcctttgggccacttggattgtaccagtcaactgatttatcatgaaatatttgctaacagtggtaatgctgtagaggaggtggctgggaaaaccttcatcatcaggatcctccgctgtgatattggccacgatggttcctggactcagttcctccaggactgtgtacactcgtgtcgggctggtaaagcgagggacttcgtcgttgaggttcacgatgttcacctggagctctgtggaggctttgaggcctccactgtccctcacctccacgatgagatggaaacttctgtgtcctgcttcaaagtccaattctgttgtggagaagagggtgccattagcagacattctgaagctctttgggggagaaatcaggaaataactgaggggaatgtttcggcttgtgtcttctggatcgaaggcctcaacctggtaaatgaatccagggtttgctctttctactatgtagaggtgtagaccttctgccaagttgccttgaaactgaggtggctcgttcacatctgttacctggacagtcaggacttgcaggtctgtgacaccaacctcatccttcacataaatctgcaaatcaaatatgtttggtcctgtttcaaaatctagttgttccatcccagtggtgacaacctcaaagtaggtgcctgacagccaattcaccctaaaagcttcagtgaggggatttgagttgactatctggggaaatcctgggatcacaggtgacaatgatgctgataacttcacagaaaacttgtgcactgaagtcccaggtggagaattctctgccacattgcctgtagcaggtaagaggattaggtgtagtgcttctccccctgacatggcacccaggagagccaggagaatgattgcttcctgcatacttgatggtcacaactgtgcgtgcttccagcacattagccacagcctgaatcccgtctcacacccaaagtttatt

SEQ ID NO: 14773 - RNA, 4602 nt, Homo sapiens
  source 1..4602: mol_type = other RNA
gctgggattacaggcatgagccacctcacccggcccttttaatcattcttaatgggcttataagcagttattaagtcccccttcagccttctcagaacctcattttacttgcattgaagctgagagcttccaaggaaagcatttgactccgggccccacagatttgcaatgccttaaatgggcaatcagccacttcactcactttaacctgcataaatgaacagttctgccttcttttgcaaagtttaaatccattcaagggagttccctggcaaccaacccttattaataaatcacgctcaatctaggccaggacaggcattttgcaaatgcttcttttgcttgagaagtgacactggcactaggcacacagtaaacaagctgctgctctctctgaagctctacatttgctggatccagtctgtctcccacaggaccttgtggacctggtaggctctcacctgactccccagttgggaagggagtgcttccctaatgaacactcacctggacctttcttagggttactggactagggtcgcagcagctgggcagcagggcatagagctcgagtgaagcttgctcaggctctgctaggcacacattggaaagttacatttcctattccatcataataccatttattcccagttcattgctcatgcctacaggtggaagtctgagttttatgtctagatggggcttccagtatgtccccactcagagtcctgcagttccttccaatcataggaagtgggaaggagcaaggcaggtaggttgtaaggctgatggtgtttcagctttgaggaaaaagtgatttcacttcaatagtaattttaaccagaatggctaaagttaaaaggattgacaatcccaagtgttggcaaggatagagagcaattgcaactctcagtgtttgctgctggaatgtgaatcagagccaccactttggaactctttggcagatccagcaattgctccagcaatcccactcttagatatatgagcaaaaaagtgagtgtttatgttcaccaaaagacatgtacaagaaagttcatagtgttgtaattcacttttattttttttttctgagatggagtcttgctttgtcacccaggctagagtgcagtggcacaatctcaactcactgtaacctccacctctcaggtttaagcagttctccctacctcagcctcccaagtagctgggattacatgtgcccaccaccacaccaagctaatttttgtattttttagtagagacagggttttgccatctaggccaggctgatcttgaactcctgaccttaggtgatctgcccaccttggcaaagtgctggcattacaggcatgagccatcatgccctgcctgtagttcacttttaagtatattttttaaaagtaaaaaatctgaagcagctgccacccaagtgtagaatagataaattgtgatataatcatagaatgaaaccagacataaccatgaagagaactgaactactgctagacaggacaacgtggatgaatctcacatgcaggatgctgatccggacaccacaagaaaaaacaaaagaaggtgcctactgagttttcttctttccagatgaccaactcttaacttactcatctgtttttttcactgttctgcttcttttgaagaagatttgaggtgacttacaaaggtgtatggcatatttataactgaagaaatctgggtgatgttaaaacgagggcaggaaaataaggtggaaaccagatgtaaggatagtcttcactatttatgtcaggaattcctacaaactttctatggtgaacagaatagagcttcctagcagtcaatgcaaagaagaaacacaacaattccacaccccaaagttaacagtcttgcttatcagaagcacaggtagttctgaaatctgatagaaaatgttcctgtatcatttcagaacacgcaactatgtgatcaaacccctttctatttgtttaaaaatttgtcaaacatcccatgtttgaccctggatgtctgaatcccctcagcccacattttcccccctacaccatgcccacaccatccccatagaatttagggtgaggcagcatctcagtgattgacaggcccctccttagaccccgtttactttcctgggtgtggtttggggtaagccctgttcatgaaggctggatttctgttctttgggttgcccagcttgccaccctcatttctggaacccagaccagcatcctcagcccacgctttgccactcagctcatcttcttcccagttggcacttctcagtgaccccatcccttccccagcagtgactctgcgtggggcagctccctggtggctggactctttccattttggcatttgggttagtggatctttccactttctggctccagtttttgagttgaattcatatgtttccccggtcactggatctatggcttctccatcaaagatagtgttcatctggatagtttccaccacgacgtctctctctgcagtcttcgtttagaggttccttgttcttcccagtcttgcaggggcagtgtctgtggatggctttggccaataggacgaccaggtacacgaggagacccagaagcaatatggagcccaaagtgatgacaaacggcacgtaccatgcagatggagagtaaacgtttttcctcaggacctgataggtgaccctgggctgggccaatggaataacggaaagatctggggctggaatcaaggtcggtacatgtcagcttgaaattctgaatatttgtgccaactttcagatccactgggagggccaggaaataagagtttggagtacaaattggcttttcatcattttcttcaaggatgttcacagtaacagtgacagagcttgtgtcttcgttgttggtggcctggattctgagaatatagatgggggttgtttcacagtccactttagttaccagctggagttctcctgtcttgggattaatccaaaatacatttggatactggaggctggcccctccagtggagatggagtacaggaggctgctctgggggaggtctttatcagtggctcgcacctgtcccactcgggttctggcgggccttctttctgacacatcaaatacataggatggcctatcaaaaatgagaggaaactcattttctgggcttgttaggatataaacgtagacgttatttttatagtaagggggggccacatcctgcacctggattatcaccgtatatttattgccggctgctaggttacttggattttcgtagtctagatcaccaatcagcacaatcttcccagagccagctggatcctgtaaaaatctgctgccgctccccactccagatggcatggtgaagttgaatctgttgtttggtgcctcactgtcatcatcaaagcagaacttgtttaggtcaagaagcaacgtccccttggctgttctttccggcaccataatgctgaaggtgaacttttggcatgtggcaggattgtcgttgacgtcttccacaatgaaggttatctggatgcgattctcctgacccccatatggtctgtccttcactagaacttccagggaaatggtgggattttgtctcaattcacctgcatctcggtctatcctttgggccacttggattgtaccagtcaactgatttatcatgaaatatttgctaacagtggtaatgctgtagaggaggtggctgggaaaaccttcatcatcaggatcctccgctgtgatattggccacgatggttcctggactcagttcctccaggactgtgtacactcgtgtcgggctggtaaagcgagggacttcgtcgttgaggttcacgatgttcacctggagctctgtggaggctttgaggcctccactgtccctcacctccacgatgagatggaaacttctgtgtcctgcttcaaagtccaattctgttgtggagaagagggtgccattagcagacattctgaagctctttgggggagaaatcaggaaataactgaggggaatgtttcggcttgtgtcttctggatcgaaggcctcaacctggtaaatgaatccagggtttgctctttctactatgtagaggtgtagaccttctgccaagttgccttgaaactgaggtggctcgttcacatctgttacctggacagtcaggacttgcaggtctgtgacaccaacctcatccttcacataaatctgcaaatcaaatatgtttggtcctgtttcaaaatctagttgttccatcccagtggtgacaacctcaaagtaggtgcctgacagccaattcaccctaaaagcttcagtgaggggatttgagttgactatctggggaaatcctgggatcacaggtgacaatgatgctgataacttcacagaaaacttgtgcactgaagtcccaggtggagaattctctgccacattgcctgtagcaggtaagaggattaggtgtagtgcttctccccctgacatggcacccaggagagccaggagaatgattgcttcctgcatacttgatggtcacaactgtgcgtgcttccagcacattagccacagcctgaatcccgtctcacacccaaagtttatt

SEQ ID NO: 14774 - RNA, 5015 nt, Homo sapiens
  source 1..5015: mol_type = other RNA
gctgggattacaggcatgagccacctcacccggcccttttaatcattcttaatgggcttataagcagttattaagtcccccttcagccttctcagaacctcattttacttgcattgaagctgagagcttccaaggaaagcatttgactccgggccccacagatttgcaatgccttaaatgggcaatcagccacttcactcactttaacctgcataaatgaacagttctgccttcttttgcaaagtttaaatccattcaagggagttccctggcaaccaacccttattaataaatcacgctcaatctaggccaggacaggcattttgcaaatgcttcttttgcttgagaagtgacactggcactaggcacacagtaaacaagctgctgctctctctgaagctctacatttgctggatccagtctgtctcccacaggaccttgtggacctggtaggctctcacctgactccccagttgggaagggagtgcttccctaatgaacactcacctggacctttcttagggttactggactagggtcgcagcagctgggcagcagggcatagagctcgagtgaagcttgctcaggctctgctaggcacacattggaaagttacatttcctattccatcataataccatttattcccagttcattgctcatgcctacaggtggaagtctgagttttatgtctagatggggcttccagtatgtccccactcagagtcctgcagttccttccaatcataggaagtgggaaggagcaaggcaggtaggttgtaaggctgatggtgtttcagctttgaggaaaaagtgatttcacttcaatagtaattttaaccagaatggctaaagttaaaaggattgacaatcccaagtgttggcaaggatagagagcaattgcaactctcagtgtttgctgctggaatgtgaatcagagccaccactttggaactctttggcagatccagcaattgctccagcaatcccactcttagatatatgagcaaaaaagtgagtgtttatgttcaccaaaagacatgtacaagaaagttcatagtgttgtaattcacttttattttttttttctgagatggagtcttgctttgtcacccaggctagagtgcagtggcacaatctcaactcactgtaacctccacctctcaggtttaagcagttctccctacctcagcctcccaagtagctgggattacatgtgcccaccaccacaccaagctaatttttgtattttttagtagagacagggttttgccatctaggccaggctgatcttgaactcctgaccttaggtgatctgcccaccttggcaaagtgctggcattacaggcatgagccatcatgccctgcctgtagttcacttttaagtatattttttaaaagtaaaaaatctgaagcagctgccacccaagtgtagaatagataaattgtgatataatcatagaatgaaaccagacataaccatgaagagaactgaactactgctagacaggacaacgtggatgaatctcacatgcaggatgctgatccggacaccacaagaaaaaacaaaagaaggtgcctactgagttttcttctttccagatgaccaactcttaacttactcatctgtttttttcactgttctgcttcttttgaagaagatttgaggtgacttacaaaggtgtatggcatatttataactgaagaaatctgggtgatgttaaaacgagggcaggaaaataaggtggaaaccagatgtaaggatagtcttcactatttatgtcaggaattcctacaaactttctatggtgaacagaatagagcttcctagcagtcaatgcaaagaagaaacacaacaattccacaccccaaagttaacagtcttgcttatcagaagcacaggtagttctgaaatctgatagaaaatgttcctgtatcatttcagaacacgcaactatgtgatcaaacccctttctatttgtttaaaaatttgtcaaacatcccatgtttgaccctggatgtctgaatcccctcagcccacattttcccccctacaccatgcccacaccatccccatagaatttagggtgaggcagcatctcagtgattgacaggcccctccttagaccccgtttactttcctgggtgtggtttggggtaagccctgttcatgaaggctggatttctgttctttgggttgcccagcttgccaccctcatttctggaacccagaccagcatcctcagcccacgctttgccactcagctcatcttcttcccagttggcacttctcagtgaccccatcccttccccagcagtgactctgcgtggggcagctccctggtggctggactctttccattttggcatttgggttagtggatctttccactttctggctccagtttttgagttgaattcatatgtttccccggtcactggatctatggcttctccatcaaagatagtgttcatctggatagtttccaccacgacgtctctctctgcagtcttcgtttctccgcttccttccagccacagaagatgcagctgaaaatgctccaagatgtgatcgcggcctgattctttgccgagtaggaacctttttacgtagcacaacagagcaagcaaaaaacaacagacaagggaaacaggtactgtacatacctcctttctttgtcagaggttccttgttcttcccagtcttgcaggggcagtgtctgtggatggctttggccaataggacgaccaggtacacgaggagacccagaagcaatatggagcccaaagtgatgacaaacggcacgtaccatgcagatggagagtaaacgtttttcctcaggacctgataggtgaccctgggcctgggggtcgtggtgatgatagtggttgggtggggaatgactttaatactcagtgtcactgttcctgtctcaacaagagcctccgctttcttcctgtcagacatcaagttgtcatcagttacgtagacaagtagcttgtagtcccagatcttatcaaacccaccagcatagtcaaagcgagatgtaagcagcaggcgtgtgacattggaaccagcattgggagagaaggtgaaatgattgttgacgttacctgggccaatggaataacggaaagatctggggctggaatcaaggtcggtacatgtcagcttgaaattctgaatatttgtgccaactttcagatccactgggagggccaggaaataagagtttggagtacaaattggcttttcatcattttcttcaaggatgttcacagtaacagtgacagagcttgtgtcttcgttgttggtggcctggattctgagaatatagatgggggttgtttcacagtccactttagttaccagctggagttctcctgtcttgggattaatccaaaatacatttggatactggaggctggcccctccagtggagatggagtacaggaggctgctctgggggaggtctttatcagtggctcgcacctgtcccactcgggttctggcgggccttctttctgacacatcaaatacataggatggcctatcaaaaatgagaggaaactcattttctgggcttgttaggatataaacgtagacgttatttttatagtaagggggggccacatcctgcacctggattatcaccgtatatttattgccggctgctaggttacttggattttcgtagtctagatcaccaatcagcacaatcttcccagagccagctggatcctgtaaaaatctgctgccgctccccactccagatggcatggtgaagttgaatctgttgtttggtgcctcactgtcatcatcaaagcagaacttgtttaggtcaagaagcaacgtccccttggctgttctttccggcaccataatgctgaaggtgaacttttggcatgtggcaggattgtcgttgacgtcttccacaatgaaggttatctggatgcgattctcctgacccccatatggtctgtccttcactagaacttccagggaaatggtgggattttgtctcaattcacctgcatctcggtctatcctttgggccacttggattgtaccagtcaactgatttatcatgaaatatttgctaacagtggtaatgctgtagaggaggtggctgggaaaaccttcatcatcaggatcctccgctgtgatattggccacgatggttcctggactcagttcctccaggactgtgtacactcgtgtcgggctggtaaagcgagggacttcgtcgttgaggttcacgatgttcacctggagctctgtggaggctttgaggcctccactgtccctcacctccacgatgagatggaaacttctgtgtcctgcttcaaagtccaattctgttgtggagaagagggtgccattagcagacattctgaagctctttgggggagaaatcaggaaataactgaggggaatgtttcggcttgtgtcttctggatcgaaggcctcaacctggtaaatgaatccagggtttgctctttctactatgtagaggtgtagaccttctgccaagttgccttgaaactgaggtggctcgttcacatctgttacctggacagtcaggacttgcaggtctgtgacaccaacctcatccttcacataaatctgcaaatcaaatatgtttggtcctgtttcaaaatctagttgttccatcccagtggtgacaacctcaaagtaggtgcctgacagccaattcaccctaaaagcttcagtgaggggatttgagttgactatctggggaaatcctgggatcacaggtgacaatgatgctgataacttcacagaaaacttgtgcactgaagtcccaggtggagaattctctgccacattgcctgtagcaggtaagaggattaggtgtagtgcttctccccctgacatggcacccaggagagccaggagaatgattgcttcctgcatacttgatggtcacaactgtgcgtgcttccagcacattagccacagcctgaatcccgtctcacacccaaagtttatt

SEQ ID NO: 14775 - RNA, 4483 nt, Homo sapiens
  source 1..4483: mol_type = other RNA
gctgggattacaggcatgagccacctcacccggcccttttaatcattcttaatgggcttataagcagttattaagtcccccttcagccttctcagaacctcattttacttgcattgaagctgagagcttccaaggaaagcatttgactccgggccccacagatttgcaatgccttaaatgggcaatcagccacttcactcactttaacctgcataaatgaacagttctgccttcttttgcaaagtttaaatccattcaagggagttccctggcaaccaacccttattaataaatcacgctcaatctaggccaggacaggcattttgcaaatgcttcttttgcttgagaagtgacactggcactaggcacacagtaaacaagctgctgctctctctgaagctctacatttgctggatccagtctgtctcccacaggaccttgtggacctggtaggctctcacctgactccccagttgggaagggagtgcttccctaatgaacactcacctggacctttcttagggttactggactagggtcgcagcagctgggcagcagggcatagagctcgagtgaagcttgctcaggctctgctaggcacacattggaaagttacatttcctattccatcataataccatttattcccagttcattgctcatgcctacaggtggaagtctgagttttatgtctagatggggcttccagtatgtccccactcagagtcctgcagttccttccaatcataggaagtgggaaggagcaaggcaggtaggttgtaaggctgatggtgtttcagctttgaggaaaaagtgatttcacttcaatagtaattttaaccagaatggctaaagttaaaaggattgacaatcccaagtgttggcaaggatagagagcaattgcaactctcagtgtttgctgctggaatgtgaatcagagccaccactttggaactctttggcagatccagcaattgctccagcaatcccactcttagatatatgagcaaaaaagtgagtgtttatgttcaccaaaagacatgtacaagaaagttcatagtgttgtaattcacttttattttttttttctgagatggagtcttgctttgtcacccaggctagagtgcagtggcacaatctcaactcactgtaacctccacctctcaggtttaagcagttctccctacctcagcctcccaagtagctgggattacatgtgcccaccaccacaccaagctaatttttgtattttttagtagagacagggttttgccatctaggccaggctgatcttgaactcctgaccttaggtgatctgcccaccttggcaaagtgctggcattacaggcatgagccatcatgccctgcctgtagttcacttttaagtatattttttaaaagtaaaaaatctgaagcagctgccacccaagtgtagaatagataaattgtgatataatcatagaatgaaaccagacataaccatgaagagaactgaactactgctagacaggacaacgtggatgaatctcacatgcaggatgctgatccggacaccacaagaaaaaacaaaagaaggtgcctactgagttttcttctttccagatgaccaactcttaacttactcatctgtttttttcactgttctgcttcttttgaagaagatttgaggtgacttacaaaggtgtatggcatatttataactgaagaaatctgggtgatgttaaaacgagggcaggaaaataaggtggaaaccagatgtaaggatagtcttcactatttatgtcaggaattcctacaaactttctatggtgaacagaatagagcttcctagcagtcaatgcaaagaagaaacacaacaattccacaccccaaagttaacagtcttgcttatcagaagcacaggtagttctgaaatctgatagaaaatgttcctgtatcatttcagaacacgcaactatgtgatcaaacccctttctatttgtttaaaaatttgtcaaacatcccatgtttgaccctggatgtctgaatcccctcagcccacattttcccccctacaccatgcccacaccatccccatagaatttagggtgaggcagcatctcagtgattgacaggcccctccttagaccccgtttactttcctgggtgtggtttggggtaagccctgttcatgaaggctggatttctgttctttgggttgcccagcttgccaccctcatttctggaacccagaccagcatcctcagcccacgctttgccactcagctcatcttcttcccagttggcacttctcagtgaccccatcccttccccagcagtgactctgcgtggggcagctccctggtggctggactctttccattttggcatttgggttagtggatctttccactttctggctccagtttttgagttgaattcatatgtttccccggtcactggatctatggcttctccatcaaagatagtgttcatctggatagtttccaccacgacgtctctctctgcagtcttcgtttctcctttctttgtcagaggttccttgttcttcccagtcttgcaggggcagtgtctgtggatggctttggccaataggacgaccaggtacacgaggagacccagaagcaatatggagcccaaagtgatgacaaacggcacgtaccatgcagatggagagtaaacgtttttcctcaggacctgataggtgaccctgggcctgggggtcgtggtgatgatagtggttgggtggggaatgactttaatactcagtgtcactgttcctgtctcaacaagagcctccgctttcttcctgggccaatggaataacggaaagatctggggctggaatcaaggtcggtacatgtcagcttgaaattctgaatatttgtgccaactttcagatccactgggagggccaggaaataagagtttggagtacaaattggcttttcatcattttcttcaaggatgttcacagtaaccgggccttctttctgacacatcaaatacataggatggcctatcaaaaatgagaggaaactcattttctgggcttgttaggatataaacgtagacgttatttttatagtaagggggggccacatcctgcacctggattatcaccgtatatttattgccggctgctaggttacttggattttcgtagtctagatcaccaatcagcacaatcttcccagagccagctggatcctgtaaaaatctgctgccgctccccactccagatggcatggtgaagttgaatctgttgtttggtgcctcactgtcatcatcaaagcagaacttgtttaggtcaagaagcaacgtccccttggctgttctttccggcaccataatgctgaaggtgaacttttggcatgtggcaggattgtcgttgacgtcttccacaatgaaggttatctggatgcgattctcctgacccccatatggtctgtccttcactagaacttccagggaaatggtgggattttgtctcaattcacctgcatctcggtctatcctttgggccacttggattgtaccagtcaactgatttatcatgaaatatttgctaacagtggtaatgctgtagaggaggtggctgggaaaaccttcatcatcaggatcctccgctgtgatattggccacgatggttcctggactcagttcctccaggactgtgtacactcgtgtcgggctggtaaagcgagggacttcgtcgttgaggttcacgatgttcacctggagctctgtggaggctttgaggcctccactgtccctcacctccacgatgagatggaaacttctgtgtcctgcttcaaagtccaattctgttgtggagaagagggtgccattagcagacattctgaagctctttgggggagaaatcaggaaataactgaggggaatgtttcggcttgtgtcttctggatcgaaggcctcaacctggtaaatgaatccagggtttgctctttctactatgtagaggtgtagaccttctgccaagttgccttgaaactgaggtggctcgttcacatctgttacctggacagtcaggacttgcaggtctgtgacaccaacctcatccttcacataaatctgcaaatcaaatatgtttggtcctgtttcaaaatctagttgttccatcccagtggtgacaacctcaaagtaggtgcctgacagccaattcaccctaaaagcttcagtgaggggatttgagttgactatctggggaaatcctgggatcacaggtgacaatgatgctgataacttcacagaaaacttgtgcactgaagtcccaggtggagaattctctgccacattgcctgtagcaggtaagaggattaggtgtagtgcttctccccctgacatggcacccaggagagccaggagaatgattgcttcctgcatacttgatggtcacaactgtgcgtgcttccagcacattagccacagcctgaatcccgtctcacacccaaagtttatt

SEQ ID NO: 14776 - RNA, 4468 nt, Homo sapiens
  source 1..4468: mol_type = other RNA
gctgggattacaggcatgagccacctcacccggcccttttaatcattcttaatgggcttataagcagttattaagtcccccttcagccttctcagaacctcattttacttgcattgaagctgagagcttccaaggaaagcatttgactccgggccccacagatttgcaatgccttaaatgggcaatcagccacttcactcactttaacctgcataaatgaacagttctgccttcttttgcaaagtttaaatccattcaagggagttccctggcaaccaacccttattaataaatcacgctcaatctaggccaggacaggcattttgcaaatgcttcttttgcttgagaagtgacactggcactaggcacacagtaaacaagctgctgctctctctgaagctctacatttgctggatccagtctgtctcccacaggaccttgtggacctggtaggctctcacctgactccccagttgggaagggagtgcttccctaatgaacactcacctggacctttcttagggttactggactagggtcgcagcagctgggcagcagggcatagagctcgagtgaagcttgctcaggctctgctaggcacacattggaaagttacatttcctattccatcataataccatttattcccagttcattgctcatgcctacaggtggaagtctgagttttatgtctagatggggcttccagtatgtccccactcagagtcctgcagttccttccaatcataggaagtgggaaggagcaaggcaggtaggttgtaaggctgatggtgtttcagctttgaggaaaaagtgatttcacttcaatagtaattttaaccagaatggctaaagttaaaaggattgacaatcccaagtgttggcaaggatagagagcaattgcaactctcagtgtttgctgctggaatgtgaatcagagccaccactttggaactctttggcagatccagcaattgctccagcaatcccactcttagatatatgagcaaaaaagtgagtgtttatgttcaccaaaagacatgtacaagaaagttcatagtgttgtaattcacttttattttttttttctgagatggagtcttgctttgtcacccaggctagagtgcagtggcacaatctcaactcactgtaacctccacctctcaggtttaagcagttctccctacctcagcctcccaagtagctgggattacatgtgcccaccaccacaccaagctaatttttgtattttttagtagagacagggttttgccatctaggccaggctgatcttgaactcctgaccttaggtgatctgcccaccttggcaaagtgctggcattacaggcatgagccatcatgccctgcctgtagttcacttttaagtatattttttaaaagtaaaaaatctgaagcagctgccacccaagtgtagaatagataaattgtgatataatcatagaatgaaaccagacataaccatgaagagaactgaactactgctagacaggacaacgtggatgaatctcacatgcaggatgctgatccggacaccacaagaaaaaacaaaagaaggtgcctactgagttttcttctttccagatgaccaactcttaacttactcatctgtttttttcactgttctgcttcttttgaagaagatttgaggtgacttacaaaggtgtatggcatatttataactgaagaaatctgggtgatgttaaaacgagggcaggaaaataaggtggaaaccagatgtaaggatagtcttcactatttatgtcaggaattcctacaaactttctatggtgaacagaatagagcttcctagcagtcaatgcaaagaagaaacacaacaattccacaccccaaagttaacagtcttgcttatcagaagcacaggtagttctgaaatctgatagaaaatgttcctgtatcatttcagaacacgcaactatgtgatcaaacccctttctatttgtttaaaaatttgtcaaacatcccatgtttgaccctggatgtctgaatcccctcagcccacattttcccccctacaccatgcccacaccatccccatagaatttagggtgaggcagcatctcagtgattgacaggcccctccttagaccccgtttactttcctgggtgtggtttggggtaagccctgttcatgaaggctggatttctgttctttgggttgcccagcttgccaccctcatttctggaacccagaccagcatcctcagcccacgctttgccactcagctcatcttcttcccagttggcacttctcagtgaccccatcccttccccagcagtgactctgcgtggggcagctccctggtggctggactctttccattttggcatttgggttagtggatctttccactttctggctccagtttttgagttgaattcatatgtttccccggtcactggatctatggcttctccatcaaagatagtgttcatctggatagtttccaccacgacgtctctctctgcagtcttcgtttctcctttctttgtcagaggttccttgttcttcccagtcttgcaggggcagtgtctgtggatggctttggccaataggacgaccaggtacacgaggagacccagaagcaatatggagcccaaagtgatgacaaacggcacgtaccatgcagatggagagtaaacgtttttcctcaggacctgataggtgaccctgggcctgggggtcgtggtgatgatagtggttgggtggggaatgactttaatactcagtgtcactgttcctgtctcaacaagagcctccgctttcttcctgtcagacatcaagttgtcatcagttacgtagacaagtagcttgtagtcccagatcttatcaaacccaccagcatagtcaaagcgagatgtaagcagcaggcgtgtgacattggaaccagcattgggagagaaggtgaaatgattgttgacgttaccgggccttctttctgacacatcaaatacataggatggcctatcaaaaatgagaggaaactcattttctgggcttgttaggatataaacgtagacgttatttttatagtaagggggggccacatcctgcacctggattatcaccgtatatttattgccggctgctaggttacttggattttcgtagtctagatcaccaatcagcacaatcttcccagagccagctggatcctgtaaaaatctgctgccgctccccactccagatggcatggtgaagttgaatctgttgtttggtgcctcactgtcatcatcaaagcagaacttgtttaggtcaagaagcaacgtccccttggctgttctttccggcaccataatgctgaaggtgaacttttggcatgtggcaggattgtcgttgacgtcttccacaatgaaggttatctggatgcgattctcctgacccccatatggtctgtccttcactagaacttccagggaaatggtgggattttgtctcaattcacctgcatctcggtctatcctttgggccacttggattgtaccagtcaactgatttatcatgaaatatttgctaacagtggtaatgctgtagaggaggtggctgggaaaaccttcatcatcaggatcctccgctgtgatattggccacgatggttcctggactcagttcctccaggactgtgtacactcgtgtcgggctggtaaagcgagggacttcgtcgttgaggttcacgatgttcacctggagctctgtggaggctttgaggcctccactgtccctcacctccacgatgagatggaaacttctgtgtcctgcttcaaagtccaattctgttgtggagaagagggtgccattagcagacattctgaagctctttgggggagaaatcaggaaataactgaggggaatgtttcggcttgtgtcttctggatcgaaggcctcaacctggtaaatgaatccagggtttgctctttctactatgtagaggtgtagaccttctgccaagttgccttgaaactgaggtggctcgttcacatctgttacctggacagtcaggacttgcaggtctgtgacaccaacctcatccttcacataaatctgcaaatcaaatatgtttggtcctgtttcaaaatctagttgttccatcccagtggtgacaacctcaaagtaggtgcctgacagccaattcaccctaaaagcttcagtgaggggatttgagttgactatctggggaaatcctgggatcacaggtgacaatgatgctgataacttcacagaaaacttgtgcactgaagtcccaggtggagaattctctgccacattgcctgtagcaggtaagaggattaggtgtagtgcttctccccctgacatggcacccaggagagccaggagaatgattgcttcctgcatacttgatggtcacaactgtgcgtgcttccagcacattagccacagcctgaatcccgtctcacacccaaagtttatt

SEQ ID NO: 14777 - RNA, 4651 nt, Homo sapiens
  source 1..4651: mol_type = other RNA
gctgggattacaggcatgagccacctcacccggcccttttaatcattcttaatgggcttataagcagttattaagtcccccttcagccttctcagaacctcattttacttgcattgaagctgagagcttccaaggaaagcatttgactccgggccccacagatttgcaatgccttaaatgggcaatcagccacttcactcactttaacctgcataaatgaacagttctgccttcttttgcaaagtttaaatccattcaagggagttccctggcaaccaacccttattaataaatcacgctcaatctaggccaggacaggcattttgcaaatgcttcttttgcttgagaagtgacactggcactaggcacacagtaaacaagctgctgctctctctgaagctctacatttgctggatccagtctgtctcccacaggaccttgtggacctggtaggctctcacctgactccccagttgggaagggagtgcttccctaatgaacactcacctggacctttcttagggttactggactagggtcgcagcagctgggcagcagggcatagagctcgagtgaagcttgctcaggctctgctaggcacacattggaaagttacatttcctattccatcataataccatttattcccagttcattgctcatgcctacaggtggaagtctgagttttatgtctagatggggcttccagtatgtccccactcagagtcctgcagttccttccaatcataggaagtgggaaggagcaaggcaggtaggttgtaaggctgatggtgtttcagctttgaggaaaaagtgatttcacttcaatagtaattttaaccagaatggctaaagttaaaaggattgacaatcccaagtgttggcaaggatagagagcaattgcaactctcagtgtttgctgctggaatgtgaatcagagccaccactttggaactctttggcagatccagcaattgctccagcaatcccactcttagatatatgagcaaaaaagtgagtgtttatgttcaccaaaagacatgtacaagaaagttcatagtgttgtaattcacttttattttttttttctgagatggagtcttgctttgtcacccaggctagagtgcagtggcacaatctcaactcactgtaacctccacctctcaggtttaagcagttctccctacctcagcctcccaagtagctgggattacatgtgcccaccaccacaccaagctaatttttgtattttttagtagagacagggttttgccatctaggccaggctgatcttgaactcctgaccttaggtgatctgcccaccttggcaaagtgctggcattacaggcatgagccatcatgccctgcctgtagttcacttttaagtatattttttaaaagtaaaaaatctgaagcagctgccacccaagtgtagaatagataaattgtgatataatcatagaatgaaaccagacataaccatgaagagaactgaactactgctagacaggacaacgtggatgaatctcacatgcaggatgctgatccggacaccacaagaaaaaacaaaagaaggtgcctactgagttttcttctttccagatgaccaactcttaacttactcatctgtttttttcactgttctgcttcttttgaagaagatttgaggtgacttacaaaggtgtatggcatatttataactgaagaaatctgggtgatgttaaaacgagggcaggaaaataaggtggaaaccagatgtaaggatagtcttcactatttatgtcaggaattcctacaaactttctatggtgaacagaatagagcttcctagcagtcaatgcaaagaagaaacacaacaattccacaccccaaagttaacagtcttgcttatcagaagcacaggtagttctgaaatctgatagaaaatgttcctgtatcatttcagaacacgcaactatgtgatcaaacccctttctatttgtttaaaaatttgtcaaacatcccatgtttgaccctggatgtctgaatcccctcagcccacattttcccccctacaccatgcccacaccatccccatagaatttagggtgaggcagcatctcagtgattgacaggcccctccttagaccccgtttactttcctgggtgtggtttggggtaagccctgttcatgaaggctggatttctgttctttgggttgcccagcttgccaccctcatttctggaacccagaccagcatcctcagcccacgctttgccactcagctcatcttcttcccagttggcacttctcagtgaccccatcccttccccagcagtgactctgcgtggggcagctccctggtggctggactctttccattttggcatttgggttagtggatctttccactttctggctccagtttttgagttgaattcatatgtttccccggtcactggatctatggcttctccatcaaagatagtgttcatctggatagtttccaccacgacgtctctctctgcagtcttcgtttctcctttctttgtcagaggttccttgttcttcccagtcttgcaggggcagtgtctgtggatggctttggccaataggacgaccaggtacacgaggagacccagaagcaatatggagcccaaagtgatgacaaacggcacgtaccatgcagatggagagtaaacgtttttcctcaggacctgataggtgaccctgggcctgggggtcgtggtgatgatagtggttgggtggggaatgactttaatactcagtgtcactgttcctgtctcaacaagagcctccgctttcttcctgtcagacatcaagttgtcatcagttacgtagacaagtagcttgtagtcccagatcttatcaaacccaccagcatagtcaaagcgagatgtaagcagcaggcgtgtgacattggaaccagcattgggagagaaggtgaaatgattgttgacgttaccgggccttctttctgacacatcaaatacataggatggcctatcaaaaatgagaggaaactcattttctgggcttgttaggatataaacgtagacgttatttttatagtaagggggggccacatcctgcacctggattatcaccgtatatttattgccggctgctaggttacttggattttcgtagtctagatcaccaatcagcacaatcttcccagagccagctggatcctgtaaaaatctgctgccgctccccactccagatggcatggtgaagttgaatctgttgtttggtgcctcactgtcatcatcaaagcagaacttgtttaggtcaagaagcaacgtccccttggctgttctttccggcaccataatgctgaaggtgaacttttggcatgtggcaggattgtcgttgacgtcttccacaatgaaggttatctggatgcgattctcctgacccccatatggtctgtccttcactagaacttccagggaaatggtgggattttgtctcaattcacctgcatctcggtctatcctttgggccacttggattgtaccagtcaactgatttatcatgaaatatttgctaacagtggtaatgctgtagaggaggtggctgggaaaaccttcatcatcaggatcctccgctgtgatattggccacgatggttcctggactcagttcctccaggactgtgtacactcgtgtcgggctggtaaagcgagggacttcgtcgttgaggttcacgatgttcacctggagctctgtggaggctttgaggcctccactgtccctcacctccacgatgagatggaaacttctgtgtcctgcttcaaagtccaattctgttgtggagaagagggtgccattagcagacattctgaagctctttgggggagaaatcaggaaataactgaggggaatgtttcggcttgtgtcttctggatcgaaggcctcaacctggtaaatgaatccagggtttgctctttctactatgtagaggtgtagaccttctgccaagttgccttgaaactgaggtggctcgttcacatctgttacctggacagtcaggacttgcaggtctgtgacaccaacctcatccttcacataaatctgcaaatcaaatatgtttggtcctgtttcaaaatctagttgttccatcccagtggtgacaacctgcgtttcagaacgacatctacccactggtttcagctcctagagcaacaactgcagaatctccatggtccaaagtcctccaggaaagagaagaaaggggtgacgggggtgagggctgggaggcgaggtcaccagggtcccttccctggctcgggtgggggtggggggcgcaacccctcacggctcctccccaccaagccgtcgggaccccagcgggggcgcctcgcgttgggcgacagggacgcggggagagagcgacaagctggaagcaagggctgcctgcaaaactttcggtcctccagcggcaactctgcgggaaagaccacccttccttcggccccgcgtcgggcctatccccgtgtgccccgacccctgcgccccaggcttgggcggcgccgctgcatcccggctgccgggcgcgctgcagccttcgctctcccgcacgcggcgctcgcccgtccgcgctgcccctccccggcaggcgggcggccccggcgggcgggcgggc

SEQ ID NO: 14778 - RNA, 4553 nt, Homo sapiens
  source 1..4553: mol_type = other RNA
gctgggattacaggcatgagccacctcacccggcccttttaatcattcttaatgggcttataagcagttattaagtcccccttcagccttctcagaacctcattttacttgcattgaagctgagagcttccaaggaaagcatttgactccgggccccacagatttgcaatgccttaaatgggcaatcagccacttcactcactttaacctgcataaatgaacagttctgccttcttttgcaaagtttaaatccattcaagggagttccctggcaaccaacccttattaataaatcacgctcaatctaggccaggacaggcattttgcaaatgcttcttttgcttgagaagtgacactggcactaggcacacagtaaacaagctgctgctctctctgaagctctacatttgctggatccagtctgtctcccacaggaccttgtggacctggtaggctctcacctgactccccagttgggaagggagtgcttccctaatgaacactcacctggacctttcttagggttactggactagggtcgcagcagctgggcagcagggcatagagctcgagtgaagcttgctcaggctctgctaggcacacattggaaagttacatttcctattccatcataataccatttattcccagttcattgctcatgcctacaggtggaagtctgagttttatgtctagatggggcttccagtatgtccccactcagagtcctgcagttccttccaatcataggaagtgggaaggagcaaggcaggtaggttgtaaggctgatggtgtttcagctttgaggaaaaagtgatttcacttcaatagtaattttaaccagaatggctaaagttaaaaggattgacaatcccaagtgttggcaaggatagagagcaattgcaactctcagtgtttgctgctggaatgtgaatcagagccaccactttggaactctttggcagatccagcaattgctccagcaatcccactcttagatatatgagcaaaaaagtgagtgtttatgttcaccaaaagacatgtacaagaaagttcatagtgttgtaattcacttttattttttttttctgagatggagtcttgctttgtcacccaggctagagtgcagtggcacaatctcaactcactgtaacctccacctctcaggtttaagcagttctccctacctcagcctcccaagtagctgggattacatgtgcccaccaccacaccaagctaatttttgtattttttagtagagacagggttttgccatctaggccaggctgatcttgaactcctgaccttaggtgatctgcccaccttggcaaagtgctggcattacaggcatgagccatcatgccctgcctgtagttcacttttaagtatattttttaaaagtaaaaaatctgaagcagctgccacccaagtgtagaatagataaattgtgatataatcatagaatgaaaccagacataaccatgaagagaactgaactactgctagacaggacaacgtggatgaatctcacatgcaggatgctgatccggacaccacaagaaaaaacaaaagaaggtgcctactgagttttcttctttccagatgaccaactcttaacttactcatctgtttttttcactgttctgcttcttttgaagaagatttgaggtgacttacaaaggtgtatggcatatttataactgaagaaatctgggtgatgttaaaacgagggcaggaaaataaggtggaaaccagatgtaaggatagtcttcactatttatgtcaggaattcctacaaactttctatggtgaacagaatagagcttcctagcagtcaatgcaaagaagaaacacaacaattccacaccccaaagttaacagtcttgcttatcagaagcacaggtagttctgaaatctgatagaaaatgttcctgtatcatttcagaacacgcaactatgtgatcaaacccctttctatttgtttaaaaatttgtcaaacatcccatgtttgaccctggatgtctgaatcccctcagcccacattttcccccctacaccatgcccacaccatccccatagaatttagggtgaggcagcatctcagtgattgacaggcccctccttagaccccgtttactttcctgggtgtggtttggggtaagccctgttcatgaaggctggatttctgttctttgggttgcccagcttgccaccctcatttctggaacccagaccagcatcctcagcccacgctttgccactcagctcatcttcttcccagttggcacttctcagtgaccccatcccttccccagcagtgactctgcgtggggcagctccctggtggctggactctttccattttggcatttgggttagtggatctttccactttctggctccagtttttgagttgaattcatatgtttccccggtcactggatctatggcttctccatcaaagatagtgttcatctggatagtttccaccacgacgtctctctctgcagtcttcgtttctcctttctttgtcagaggttccttgttcttcccagtcttgcaggggcagtgtctgtggatggctttggccaataggacgaccaggtacacgaggagacccagaagcaatatggagcccaaagtgatgacaaacggcacgtaccatgcagatggagagtaaacgtttttcctcaggacctgataggtgaccctgggcctgggggtcgtggtgatgatagtggttgggtggggaatgactttaatactcagtgtcactgttcctgtctcaacaagagcctccgctttcttcctgtcagacatcaagttgtcatcagttacgtagacaagtagcttgtagtcccagatcttatcaaacccaccagcatagtcaaagcgagatgtaagcagcaggcgtgtgacattggaaccagcattgggagagaaggtgaaatgattgttgacgttaccgggccttctttctgacacatcaaatacataggatggcctatcaaaaatgagaggaaactcattttctgggcttgttaggatataaacgtagacgttatttttatagtaagggggggccacatcctgcacctggattatcaccgtatatttattgccggctgctaggttacttggattttcgtagtctagatcaccaatcagcacaatcttcccagagccagctggatcctgtaaaaatctgctgccgctccccactccagatggcatggtgaagttgaatctgttgtttggtgcctcactgtcatcatcaaagcagaacttgtttaggtcaagaagcaacgtccccttggctgttctttccggcaccataatgctgaaggtgaacttttggcatgtggcaggattgtcgttgacgtcttccacaatgaaggttatctggatgcgattctcctgacccccatatggtctgtccttcactagaacttccagggaaatggtgggattttgtctcaattcacctgcatctcggtctatcctttgggccacttggattgtaccagtcaactgatttatcatgaaatatttgctaacagtggtaatgctgtagaggaggtggctgggaaaaccttcatcatcaggatcctccgctgtgatattggccacgatggttcctggactcagttcctccaggactgtgtacactcgtgtcgggctggtaaagcgagggacttcgtcgttgaggttcacgatgttcacctggagctctgtggaggctttgaggcctccactgtccctcacctccacgatgagatggaaacttctgtgtcctgcttcaaagtccaattctgttgtggagaagagggtgccattagcagacattctgaagctctttgggggagaaatcaggaaatacttctgccaagttgccttgaaactgaggtggctcgttcacatctgttacctggacagtcaggacttgcaggtctgtgacaccaacctcatccttcacataaatctgcaaatcaaatatgtttggtcctgtttcaaaatctagttgttccatcccagtggtgacaacctgcgtttcagaacgacatctacccactggtttcagctcctagagcaacaactgcagaatctccatggtccaaagtcctccaggaaagagaagaaaggggtgacgggggtgagggctgggaggcgaggtcaccagggtcccttccctggctcgggtgggggtggggggcgcaacccctcacggctcctccccaccaagccgtcgggaccccagcgggggcgcctcgcgttgggcgacagggacgcggggagagagcgacaagctggaagcaagggctgcctgcaaaactttcggtcctccagcggcaactctgcgggaaagaccacccttccttcggccccgcgtcgggcctatccccgtgtgccccgacccctgcgccccaggcttgggcggcgccgctgcatcccggctgccgggcgcgctgcagccttcgctctcccgcacgcggcgctcgcccgtccgcgctgcccctccccggcaggcgggcggccccggcgggcgggcgggc

SEQ ID NO: 14779 - RNA, 4353 nt, Homo sapiens
  source 1..4353: mol_type = other RNA
gctgggattacaggcatgagccacctcacccggcccttttaatcattcttaatgggcttataagcagttattaagtcccccttcagccttctcagaacctcattttacttgcattgaagctgagagcttccaaggaaagcatttgactccgggccccacagatttgcaatgccttaaatgggcaatcagccacttcactcactttaacctgcataaatgaacagttctgccttcttttgcaaagtttaaatccattcaagggagttccctggcaaccaacccttattaataaatcacgctcaatctaggccaggacaggcattttgcaaatgcttcttttgcttgagaagtgacactggcactaggcacacagtaaacaagctgctgctctctctgaagctctacatttgctggatccagtctgtctcccacaggaccttgtggacctggtaggctctcacctgactccccagttgggaagggagtgcttccctaatgaacactcacctggacctttcttagggttactggactagggtcgcagcagctgggcagcagggcatagagctcgagtgaagcttgctcaggctctgctaggcacacattggaaagttacatttcctattccatcataataccatttattcccagttcattgctcatgcctacaggtggaagtctgagttttatgtctagatggggcttccagtatgtccccactcagagtcctgcagttccttccaatcataggaagtgggaaggagcaaggcaggtaggttgtaaggctgatggtgtttcagctttgaggaaaaagtgatttcacttcaatagtaattttaaccagaatggctaaagttaaaaggattgacaatcccaagtgttggcaaggatagagagcaattgcaactctcagtgtttgctgctggaatgtgaatcagagccaccactttggaactctttggcagatccagcaattgctccagcaatcccactcttagatatatgagcaaaaaagtgagtgtttatgttcaccaaaagacatgtacaagaaagttcatagtgttgtaattcacttttattttttttttctgagatggagtcttgctttgtcacccaggctagagtgcagtggcacaatctcaactcactgtaacctccacctctcaggtttaagcagttctccctacctcagcctcccaagtagctgggattacatgtgcccaccaccacaccaagctaatttttgtattttttagtagagacagggttttgccatctaggccaggctgatcttgaactcctgaccttaggtgatctgcccaccttggcaaagtgctggcattacaggcatgagccatcatgccctgcctgtagttcacttttaagtatattttttaaaagtaaaaaatctgaagcagctgccacccaagtgtagaatagataaattgtgatataatcatagaatgaaaccagacataaccatgaagagaactgaactactgctagacaggacaacgtggatgaatctcacatgcaggatgctgatccggacaccacaagaaaaaacaaaagaaggtgcctactgagttttcttctttccagatgaccaactcttaacttactcatctgtttttttcactgttctgcttcttttgaagaagatttgaggtgacttacaaaggtgtatggcatatttataactgaagaaatctgggtgatgttaaaacgagggcaggaaaataaggtggaaaccagatgtaaggatagtcttcactatttatgtcaggaattcctacaaactttctatggtgaacagaatagagcttcctagcagtcaatgcaaagaagaaacacaacaattccacaccccaaagttaacagtcttgcttatcagaagcacaggtagttctgaaatctgatagaaaatgttcctgtatcatttcagaacacgcaactatgtgatcaaacccctttctatttgtttaaaaatttgtcaaacatcccatgtttgaccctggatgtctgaatcccctcagcccacattttcccccctacaccatgcccacaccatccccatagaatttagggtgaggcagcatctcagtgattgacaggcccctccttagaccccgtttactttcctgggtgtggtttggggtaagccctgttcatgaaggctggatttctgttctttgggttgcccagcttgccaccctcatttctggaacccagaccagcatcctcagcccacgctttgccactcagctcatcttcttcccagttggcacttctcagtgaccccatcccttccccagcagtgactctgcgtggggcagctccctggtggctggactctttccattttggcatttgggttagtggatctttccactttctggctccagtttttgagttgaattcatatgtttccccggtcactggatctatggcttctccatcaaagatagtgttcatctggatagtttccaccacgacgtctctctctgcagtcttcgtttctcctttctttgtcagaggttccttgttcttcccagtcttgcaggggcagtgtctgtggatggctttggccaataggacgaccaggtacacgaggagacccagaagcaatatggagcccaaagtgatgacaaacggcacgtaccatgcagatggagagtaaacgtttttcctcaggacctgataggtgaccctgggcctgggggtcgtggtgatgatagtggttgggtggggaatgactttaatactcagtgtcactgttcctgtctcaacaagagcctccgctttcttcctgtcagacatcaagttgtcatcagttacgtagacaagtagcttgtagtcccagatcttatcaaacccaccagcatagtcaaagcgagatgtaagcagcaggcgtgtgacattggaaccagcattgggagagaaggtgaaatgattgttgacgttaccgggccttctttctgacacatcaaatacataggatggcctatcaaaaatgagaggaaactcattttctgggcttgttaggatataaacgtagacgttatttttatagtaagggggggccacatcctgcacctggattatcaccgtatatttattgccggctgctaggttacttggattttcgtagtctagatcaccaatcagcacaatcttcccagagccagctggatcctgtaaaaatctgctgccgctccccactccagatggcatggtgaagttgaatctgttgtttggtgcctcactgtcatcatcaaagcagaacttgtttaggtcaagaagcaacgtccccttggctgttctttccggcaccataatgctgaaggtgaacttttggcatgtggcaggattgtcgttgacgtcttccacaatgaaggttatctggatgcgattctcctgacccccatatggtctgtccttcactagaacttccagggaaatggtgggattttgtctcaattcacctgcatctcggtctatcctttgggccacttggattgtaccagtcaactgatttatcatgaaatatttgctaacagtggtaatgctgtagaggaggtggctgggaaaaccttcatcatcaggatcctccgctgtgatattggccacgatggttcctggactcagttcctccaggactgtgtacactcgtgtcgggcttctgccaagttgccttgaaactgaggtggctcgttcacatctgttacctggacagtcaggacttgcaggtctgtgacaccaacctcatccttcacataaatctgcaaatcaaatatgtttggtcctgtttcaaaatctagttgttccatcccagtggtgacaacctgcgtttcagaacgacatctacccactggtttcagctcctagagcaacaactgcagaatctccatggtccaaagtcctccaggaaagagaagaaaggggtgacgggggtgagggctgggaggcgaggtcaccagggtcccttccctggctcgggtgggggtggggggcgcaacccctcacggctcctccccaccaagccgtcgggaccccagcgggggcgcctcgcgttgggcgacagggacgcggggagagagcgacaagctggaagcaagggctgcctgcaaaactttcggtcctccagcggcaactctgcgggaaagaccacccttccttcggccccgcgtcgggcctatccccgtgtgccccgacccctgcgccccaggcttgggcggcgccgctgcatcccggctgccgggcgcgctgcagccttcgctctcccgcacgcggcgctcgcccgtccgcgctgcccctccccggcaggcgggcggccccggcgggcgggcgggc

SEQ ID NO: 14780 - RNA, 7418 nt, Homo sapiens
  source 1..7418: mol_type = other RNA
gctgggattacaggcatgagccacctcacccggcccttttaatcattcttaatgggcttataagcagttattaagtcccccttcagccttctcagaacctcattttacttgcattgaagctgagagcttccaaggaaagcatttgactccgggccccacagatttgcaatgccttaaatgggcaatcagccacttcactcactttaacctgcataaatgaacagttctgccttcttttgcaaagtttaaatccattcaagggagttccctggcaaccaacccttattaataaatcacgctcaatctaggccaggacaggcattttgcaaatgcttcttttgcttgagaagtgacactggcactaggcacacagtaaacaagctgctgctctctctgaagctctacatttgctggatccagtctgtctcccacaggaccttgtggacctggtaggctctcacctgactccccagttgggaagggagtgcttccctaatgaacactcacctggacctttcttagggttactggactagggtcgcagcagctgggcagcagggcatagagctcgagtgaagcttgctcaggctctgctaggcacacattggaaagttacatttcctattccatcataataccatttattcccagttcattgctcatgcctacaggtggaagtctgagttttatgtctagatggggcttccagtatgtccccactcagagtcctgcagttccttccaatcataggaagtgggaaggagcaaggcaggtaggttgtaaggctgatggtgtttcagctttgaggaaaaagtgatttcacttcaatagtaattttaaccagaatggctaaagttaaaaggattgacaatcccaagtgttggcaaggatagagagcaattgcaactctcagtgtttgctgctggaatgtgaatcagagccaccactttggaactctttggcagatccagcaattgctccagcaatcccactcttagatatatgagcaaaaaagtgagtgtttatgttcaccaaaagacatgtacaagaaagttcatagtgttgtaattcacttttattttttttttctgagatggagtcttgctttgtcacccaggctagagtgcagtggcacaatctcaactcactgtaacctccacctctcaggtttaagcagttctccctacctcagcctcccaagtagctgggattacatgtgcccaccaccacaccaagctaatttttgtattttttagtagagacagggttttgccatctaggccaggctgatcttgaactcctgaccttaggtgatctgcccaccttggcaaagtgctggcattacaggcatgagccatcatgccctgcctgtagttcacttttaagtatattttttaaaagtaaaaaatctgaagcagctgccacccaagtgtagaatagataaattgtgatataatcatagaatgaaaccagacataaccatgaagagaactgaactactgctagacaggacaacgtggatgaatctcacatgcaggatgctgatccggacaccacaagaaaaaacaaaagaaggtgcctactgagttttcttctttccagatgaccaactcttaacttactcatctgtttttttcactgttctgcttcttttgaagaagatttgaggtgacttacaaaggtgtatggcatatttataactgaagaaatctgggtgatgttaaaacgagggcaggaaaataaggtggaaaccagatgtaaggatagtcttcactatttatgtcaggaattcctacaaactttctatggtgaacagaatagagcttcctagcagtcaatgcaaagaagaaacacaacaattccacaccccaaagttaacagtcttgcttatcagaagcacaggtagttctgaaatctgatagaaaatgttcctgtatcatttcagaacacgcaactatgtgatcaaacccctttctatttgtttaaaaatttgtcaaacatcccatgtttgaccctggatgtctgaatcccctcagcccacattttcccccctacaccatgcccacaccatccccatagaatttagggtgaggcagcatctcagtgattgacaggcccctccttagaccccgtttactttcctgggtgtggtttggggtaagccctgttcatgaaggctggatttctgttctttgggttgcccagcttgccaccctcatttctggaacccagaccagcatcctcagcccacgctttgccactcagctcatcttcttcccagttggcacttctcagtgaccccatcccttccccagcagtgactctgcgtggggcagctccctggtggctggactctttccattttggcatttgggttagtggatctttccactttctggctccagtttttgagttgaattcatatgtttccccggtcactggatctatggcttctccatcaaagatagtgttcatctggatagtttccaccacgacgtctctctctgcagtcttcgtttctcctttctttgtcagaggttccttgttcttcccagtcttgcaggggcagtgtctgtggatggctttggccaataggacgaccaggtacacgaggagacccagaagcaatatggagcccaaagtgatgacaaacggcacgtaccatgcagatggagagtaaacgtttttcctcaggacctgataggtgaccctgggcctgggggtcgtggtgatgatagtggttgggtggggaatgactttaatactcagtgtcactgttcctgtctcaacaagagcctccgctttcttcctgtcagacatcaagttgtcatcagttacgtagacaagtagcttgtagtcccagatcttatcaaacccaccagcatagtcaaagcgagatgtaagcagcaggcgtgtgacattggaaccagcattgggagagaaggtgaaatgattgttgacgttacctgggccaatggaataacggaaagatctggggctggaatcaaggtcggtacatgtcagcttgaaattctgaatatttgtgccaactttcagatccactgggagggccaggaaataagagtttggagtacaaattggcttttcatcattttcttcaaggatgttcacagtaacagtgacagagcttgtgtcttcgttgttggtggcctggattctgagaatatagatgggggttgtttcacagtccactttagttaccagctggagttctcctgtcttgggattaatccaaaatacatttggatactggaggctggcccctccagtggagatggagtacaggaggctgctctgggggaggtctttatcagtggctcgcacctgtcccactcgggttctggcgggccttctttctgacacatcaaatacataggatggcctatcaaaaatgagaggaaactcattttctgggcttgttaggatataaacgtagacgttatttttatagtaagggggggccacatcctgcacctggattatcaccgtatatttattgccggctgctaggttacttggattttcgtagtctagatcaccaatcagcacaatcttcccagagccagctggatcctgtaaaaatctgctgccgctccccactccagatggcatggtgaagttgaatctgttgtttggtgcctcactgtcatcatcaaagcagaacttgtttaggtcaagaagcaacgtccccttggctgttctttccggcaccataatgccccaaactcagagccttccgatcaagcccagcttgctgtaggaggctctgaggaagaccaatgaacaccttgagacttccattcattgaggggctttctcatgtctccaggtttcagttcctccatctataaaatggacataaatgatatcaattagtttttactacataacacactgtcccaaaactgagtgaattaaaacaacaagcatttatggtttctcacagtactataggttttcccacagtcctttcggttttagtttggcttagctggtctctgtggtcactgacagcttggctggggctggacagtctaggatggcctcactcacatgcctggtggtgggaaggtgcttgatttctgcttcttcttgtcctcatcttctaggaggctagtctaggctcattgcatggaggtctctggttccaaaagtaacaagagagggcaagtcccaaggcacatgcatttttcaagcctccgttgtgccatgtttgtgaatgctccagtggtcaaagcaattcacgtggtcaagctcagattcaaggagacccatctcttgatggagctaatagcaaaatcacattgcaaaggagcatgcataaagagcaagcagggaggaatttgcggcttttctttcttttttgtttgttttggctacctatcttaatcatattttgccttggtagaatttcttacaaaaatatatcgtggctgtcatgagaatgtgcctggaagacctttaaccatgagagcataactgaccatcggcctcagctgctgggctctgaaatccatcactgtgtttgtggtgaggccacgtaccaacaactggtcatggcaaagatactaaggctcattcctgtcctatgtcagttgacactggctccaggacccccaatgccctagctgaacactccttaactgcatggcagcctagaatatgtccaactaccttttctccctctttccttcactcagatcagccttgcatcatgatctgatgacttgcccagccttgtccatctctctccccattttctgccacaggcatctcccctaataatagccttgcacatttaatcccatcttagcatctggttcttggagcatacacttctctctgcaaccaaactctgttcccttctttgttccacatcctcttttcatggcagataaaatcagctctgggctcagtgcatacggagcaaagtctgacagcaagaatggtcatgggccactgaggataacaggtttgcttgctggagcgtgtaatggagtctccacgatgcctcattggcaaagatcacctctgtatttcagcaggattggagtctgaacattcctgccttgattgcacaatgtcatggtttcattcatagggacttagaagagacaccacttattaaacaccaactgcatgctgtatcataccaagcactttaaaaacactatctctaatttcctcatctcagagaggtttgtattcttgtccccactgcacaggggaagaaagagtggttccgagcattttcaaggcctgtccaggaaagtggatgtatccagacttgatcctctgcagtgttagagtcactgtaaactttaacttccatgcataagtatccaggctcacagatggtttggggatctaagccttgatttcaactctgcagaagccaggagattgcatcatttaaagaatccaaggtcccgaagccagacatttcaggcactccaacagaggcctcctcacttggccctccagggctgcttggcctgttctctcattcgtccctgacagttggtattcttcccctaaacgcctaacttggaaagccactcccctcattcagcaatccctgcctcaaaagcgagctgccctcgctcccagccatcagaccatgtttctctccccatgcaaagttgactgtgtccagcccattctgaatcagccaaactgctccgcctcttgctcacaaacagcttgcaaagcgctttcactgaatcgcctgacaatttacaaccagagcgggggttgtcacgtgcctcggatgcctccgtcgggccctgggctcattcatcatcagcctgggaaagcctcaggggccacggtacgaaaggctgggagcctgcaggagcccgcgcgggcagcagggggcgcccgcctcctccacgccgccctcctccctgcgggagcacagcacaccgcctccagcagccgcgctgacctcacccgctctgccacctgctctcaagaactccacagcagagaccgcgcccacagcctccaaggaaggaacaaacattcaagagcaagtgtcagagactgtggcagaaccatgccattgtcactttgttctgttttgacctgcttgcgtgcttggctttgacatagttggactggagaaggtataaggctgggaggatggcgggtgctgcaggtcagggcttctcagccctctccgcacccgcccttatgcagccttgggacgcgaggctgggctttaggctgaagacctccgcccctggaactgcagaggaggggtccctttcgttgcccttcctcacatcttggcgttcatagggtggctgagagttcctcccgctagaagagcccaaagagggaacttgagccttggttagattatcttcagtaataaatgcagttagtccagctacggatttcacattggccttcagggctaatctggagggaagattatcaagtgcaggactctgtttggtcttgcctggacagtctaggatattcgaattgcagtttcaccagctaatatggaacacagtctgcaaactgtcctcccatactccaggggactctggactgcaggaagccaaatatacaattaacagatatgcactgaagagagaaaatggacaaggaagatttgagacagcacagccctctccaggcattctcacttcttaaccttcaccccctacctcttagggcagaggaacaaggaagagcaggagggcagaagagggcaggagcttcccaggatgtactggaaccacccaagagttctagcacagatttaaaatgtcaaagaaagtgtaagtgtgatgctgcaaattgtctccactccatcccctgggcccagacatctctcaatttatgcacgtaaaggtgtggaagtcacaatcctaactacccatgcagctgtccccacccatctaatggacttgtagggcttaggttgggataggaacctactacatgcttaagattgtgactgacgttattggggtgtcagcaggaagcagctggtgaattaggatcattctaggaggggtcagtaaagggactatgaagaaggtgctcacagagtatatggaaatctcatcagatggtgcaatatctcagggctcgtgagagtgaagcacccttaccaccactaggcccagggaagccagtggaggaagcaggtcctgcgacagagagctgcttttgggaatggagatcttcaggcagggaagggatgcacccagctcacaaagagagagcctgaccctcctctccttctctttccaggactccccattggccaactagaagctggaaggcaagggagttggttggtatctgatatggtttggctgtgtccccacccaaatctcatcttgaactcccacatgttgtgagagggacccagtagg

SEQ ID NO: 14781 - RNA, 4276 nt, Homo sapiens
  source 1..4276: mol_type = other RNA
gctgggattacaggcatgagccacctcacccggcccttttaatcattcttaatgggcttataagcagttattaagtcccccttcagccttctcagaacctcattttacttgcattgaagctgagagcttccaaggaaagcatttgactccgggccccacagatttgcaatgccttaaatgggcaatcagccacttcactcactttaacctgcataaatgaacagttctgccttcttttgcaaagtttaaatccattcaagggagttccctggcaaccaacccttattaataaatcacgctcaatctaggccaggacaggcattttgcaaatgcttcttttgcttgagaagtgacactggcactaggcacacagtaaacaagctgctgctctctctgaagctctacatttgctggatccagtctgtctcccacaggaccttgtggacctggtaggctctcacctgactccccagttgggaagggagtgcttccctaatgaacactcacctggacctttcttagggttactggactagggtcgcagcagctgggcagcagggcatagagctcgagtgaagcttgctcaggctctgctaggcacacattggaaagttacatttcctattccatcataataccatttattcccagttcattgctcatgcctacaggtggaagtctgagttttatgtctagatggggcttccagtatgtccccactcagagtcctgcagttccttccaatcataggaagtgggaaggagcaaggcaggtaggttgtaaggctgatggtgtttcagctttgaggaaaaagtgatttcacttcaatagtaattttaaccagaatggctaaagttaaaaggattgacaatcccaagtgttggcaaggatagagagcaattgcaactctcagtgtttgctgctggaatgtgaatcagagccaccactttggaactctttggcagatccagcaattgctccagcaatcccactcttagatatatgagcaaaaaagtgagtgtttatgttcaccaaaagacatgtacaagaaagttcatagtgttgtaattcacttttattttttttttctgagatggagtcttgctttgtcacccaggctagagtgcagtggcacaatctcaactcactgtaacctccacctctcaggtttaagcagttctccctacctcagcctcccaagtagctgggattacatgtgcccaccaccacaccaagctaatttttgtattttttagtagagacagggttttgccatctaggccaggctgatcttgaactcctgaccttaggtgatctgcccaccttggcaaagtgctggcattacaggcatgagccatcatgccctgcctgtagttcacttttaagtatattttttaaaagtaaaaaatctgaagcagctgccacccaagtgtagaatagataaattgtgatataatcatagaatgaaaccagacataaccatgaagagaactgaactactgctagacaggacaacgtggatgaatctcacatgcaggatgctgatccggacaccacaagaaaaaacaaaagaaggtgcctactgagttttcttctttccagatgaccaactcttaacttactcatctgtttttttcactgttctgcttcttttgaagaagatttgaggtgacttacaaaggtgtatggcatatttataactgaagaaatctgggtgatgttaaaacgagggcaggaaaataaggtggaaaccagatgtaaggatagtcttcactatttatgtcaggaattcctacaaactttctatggtgaacagaatagagcttcctagcagtcaatgcaaagaagaaacacaacaattccacaccccaaagttaacagtcttgcttatcagaagcacaggtagttctgaaatctgatagaaaatgttcctgtatcatttcagaacacgcaactatgtgatcaaacccctttctatttgtttaaaaatttgtcaaacatcccatgtttgaccctggatgtctgaatcccctcagcccacattttcccccctacaccatgcccacaccatccccatagaatttagggtgaggcagcatctcagtgattgacaggcccctccttagaccccgtttactttcctgggtgtggtttggggtaagccctgttcatgaaggctggatttctgttctttgggttgcccagcttgccaccctcatttctggaacccagaccagcatcctcagcccacgctttgccactcagctcatcttcttcccagttggcacttctcagtgaccccatcccttccccagcagtgactctgcgtggggcagctccctggtggctggactctttccattttggcatttgggttagtggatctttccactttctggctccagtttttgagttgaattcatatgtttccccggtcactggatctatggcttctccatcaaagatagtgttcatctggatagtttccaccacgacgtctctctctgcagtcttcgtttctcctttctttgtcagaggttccttgttcttcccagtcttgcaggggcagtgtctgtggatggctttggccaataggacgaccaggtacacgaggagacccagaagcaatatggagcccaaagtgatgacaaacggcacgtaccatgcagatggagagtaaacgtttttcctcaggacctgataggtgaccctgggcctgggggtcgtggtgatgatagtggttgggtggggaatgactttaatactcagtgtcactgttcctgtctcaacaagagcctccgctttcttcctgtcagacatcaagttgtcatcagttacgtagacaagtagcttgtagtcccagatcttatcaaacccaccagcatagtcaaagcgagatgtaagcagcaggcgtgtgacattggaaccagcattgggagagaaggtgaaatgattgttgacgttacctgggccaatggaataacggaaagatctggggctggaatcaaggtcggtacatgtcagcttgaaattctgaatatttgtgccaactttcagatccactgggagggccaggaaataagagtttggagtacaaattggcttttcatcattttcttcaaggatgttcacagtaacagtgacagagcttgtgtcttcgttgttggtggcctggattctgagaatatagatgggggttgtttcacagtccactttagttaccagctggagttctcctgtcttgggattaatccaaaatacatttggatactggaggctggcccctccagtggagatggagtacaggaggctgctctgggggaggtctttatcagtggctcgcacctgtcccactcgggttctggcgggccttctttctgacacatcaaatacataggatggcctatcaaaaatgagaggaaactcattttctgggcttgttaggatataaacgtagacgttatttttatagtaagggggggccacatcctgcacctggattatcaccgtatatttattgccggctgctaggttacttggattttcgtagtctagatcaccaatcagcacaatcttcccagagccagctggatcctgtaaaaatctgctgccgctccccactccagatggcatggtgaagttgaatctgttgtttggtgcctcactgtcatcatcaaagcagaacttgtttaggtcaagaagcaacgtccccttggctgttctttccggcaccataatgctgaaggtgaacttttggcatgtggcaggattgtcgttgacgtcttccacaatgaaggttatctggatgcgattctcctgacccccatatggtctgtccttcactagaacttccagggaaatggtgggattttgtctcaattcacctgcatctcggtctatcctttgggccacttggattgtaccagtcaactgaggggaatgtttcggcttgtgtcttctggatcgaaggcctcaacctggtaaatgaatccagggtttgctctttctactatgtagaggtgtagaccttctgccaagttgccttgaaactgaggtggctcgttcacatctgttacctggacagtcaggacttgcaggtctgtgacaccaacctcatccttcacataaatctgcaaatcaaatatgtttggtcctgtttcaaaatctagttgttccatcccagtggtgacaacctgacatggcacccaggagagccaggagaatgattgcttcctgcatacttgatggtcacaactgtgcgtgcttccagcacatt

SEQ ID NO: 14782 - RNA, 4846 nt, Homo sapiens
  source 1..4846: mol_type = other RNA
gctgggattacaggcatgagccacctcacccggcccttttaatcattcttaatgggcttataagcagttattaagtcccccttcagccttctcagaacctcattttacttgcattgaagctgagagcttccaaggaaagcatttgactccgggccccacagatttgcaatgccttaaatgggcaatcagccacttcactcactttaacctgcataaatgaacagttctgccttcttttgcaaagtttaaatccattcaagggagttccctggcaaccaacccttattaataaatcacgctcaatctaggccaggacaggcattttgcaaatgcttcttttgcttgagaagtgacactggcactaggcacacagtaaacaagctgctgctctctctgaagctctacatttgctggatccagtctgtctcccacaggaccttgtggacctggtaggctctcacctgactccccagttgggaagggagtgcttccctaatgaacactcacctggacctttcttagggttactggactagggtcgcagcagctgggcagcagggcatagagctcgagtgaagcttgctcaggctctgctaggcacacattggaaagttacatttcctattccatcataataccatttattcccagttcattgctcatgcctacaggtggaagtctgagttttatgtctagatggggcttccagtatgtccccactcagagtcctgcagttccttccaatcataggaagtgggaaggagcaaggcaggtaggttgtaaggctgatggtgtttcagctttgaggaaaaagtgatttcacttcaatagtaattttaaccagaatggctaaagttaaaaggattgacaatcccaagtgttggcaaggatagagagcaattgcaactctcagtgtttgctgctggaatgtgaatcagagccaccactttggaactctttggcagatccagcaattgctccagcaatcccactcttagatatatgagcaaaaaagtgagtgtttatgttcaccaaaagacatgtacaagaaagttcatagtgttgtaattcacttttattttttttttctgagatggagtcttgctttgtcacccaggctagagtgcagtggcacaatctcaactcactgtaacctccacctctcaggtttaagcagttctccctacctcagcctcccaagtagctgggattacatgtgcccaccaccacaccaagctaatttttgtattttttagtagagacagggttttgccatctaggccaggctgatcttgaactcctgaccttaggtgatctgcccaccttggcaaagtgctggcattacaggcatgagccatcatgccctgcctgtagttcacttttaagtatattttttaaaagtaaaaaatctgaagcagctgccacccaagtgtagaatagataaattgtgatataatcatagaatgaaaccagacataaccatgaagagaactgaactactgctagacaggacaacgtggatgaatctcacatgcaggatgctgatccggacaccacaagaaaaaacaaaagaaggtgcctactgagttttcttctttccagatgaccaactcttaacttactcatctgtttttttcactgttctgcttcttttgaagaagatttgaggtgacttacaaaggtgtatggcatatttataactgaagaaatctgggtgatgttaaaacgagggcaggaaaataaggtggaaaccagatgtaaggatagtcttcactatttatgtcaggaattcctacaaactttctatggtgaacagaatagagcttcctagcagtcaatgcaaagaagaaacacaacaattccacaccccaaagttaacagtcttgcttatcagaagcacaggtagttctgaaatctgatagaaaatgttcctgtatcatttcagaacacgcaactatgtgatcaaacccctttctatttgtttaaaaatttgtcaaacatcccatgtttgaccctggatgtctgaatcccctcagcccacattttcccccctacaccatgcccacaccatccccatagaatttagggtgaggcagcatctcagtgattgacaggcccctccttagaccccgtttactttcctgggtgtggtttggggtaagccctgttcatgaaggctggatttctgttctttgggttgcccagcttgccaccctcatttctggaacccagaccagcatcctcagcccacgctttgccactcagctcatcttcttcccagttggcacttctcagtgaccccatcccttccccagcagtgactctgcgtggggcagctccctggtggctggactctttccattttggcatttgggttagtggatctttccactttctggctccagtttttgagttgaattcatatgtttccccggtcactggatctatggcttctccatcaaagatagtgttcatctggatagtttccaccacgacgtctctctctgcagtcttcgtttctcctttctttgtcagaggttccttgttcttcccagtcttgcaggggcagtgtctgtggatggctttggccaataggacgaccaggtacacgaggagacccagaagcaatatggagcccaaagtgatgacaaacggcacgtaccatgcagatggagagtaaacgtttttcctcaggacctgataggtgaccctgggcctgggggtcgtggtgatgatagtggttgggtggggaatgactttaatactcagtgtcactgttcctgtctcaacaagagcctccgctttcttcctgtcagacatcaagttgtcatcagttacgtagacaagtagcttgtagtcccagatcttatcaaacccaccagcatagtcaaagcgagatgtaagcagcaggcgtgtgacattggaaccagcattgggagagaaggtgaaatgattgttgacgttacctgggccaatggaataacggaaagatctggggctggaatcaaggtcggtacatgtcagcttgaaattctgaatatttgtgccaactttcagatccactgggagggccaggaaataagagtttggagtacaaattggcttttcatcattttcttcaaggatgttcacagtaacagtgacagagcttgtgtcttcgttgttggtggcctggattctgagaatatagatgggggttgtttcacagtccactttagttaccagctggagttctcctgtcttgggattaatccaaaatacatttggatactggaggctggcccctccagtggagatggagtacaggaggctgctctgggggaggtctttatcagtggctcgcacctgtcccactcgggttctggcgggccttctttctgacacatcaaatacataggatggcctatcaaaaatgagaggaaactcattttctgggcttgttaggatataaacgtagacgttatttttatagtaagggggggccacatcctgcacctggattatcaccgtatatttattgccggctgctaggttacttggattttcgtagtctagatcaccaatcagcacaatcttcccagagccagctggatcctgtaaaaatctgctgccgctccccactccagatggcatggtgaagttgaatctgttgtttggtgcctcactgtcatcatcaaagcagaacttgtttaggtcaagaagcaacgtccccttggctgttctttccggcaccataatgctgaaggtgaacttttggcatgtggcaggattgtcgttgacgtcttccacaatgaaggttatctggatgcgattctcctgacccccatatggtctgtccttcactagaacttccagggaaatggtgggattttgtctcaattcacctgcatctcggtctatcctttgggccacttggattgtaccagtcaactgatttatcatgaaatatttgctaacagtggtaatgctgtagaggaggtggctgggaaaaccttcatcatcaggatcctccgctgtgatattggccacgatggttcctggactcagttcctccaggactgtgtacactcgtgtcgggctggtaaagcgagggacttcgtcgttgaggttcacgatgttcacctggagctctgtggaggctttgaggcctccactgtccctcacctccacgatgagatggaaacttctgtgtcctgcttcaaagtccaattctgttgtggagaagagggtgccattagcagacattctgaagctctttgggggagaaatcaggaaataactgaggggaatgtttcggcttgtgtcttctggatcgaaggcctcaacctggtaaatgaatccagggtttgctctttctactatgtagaggtgtagaccttctgccaagttgccttgaaactgaggtggctcgttcacatctgttacctggacagtcaggacttgcaggtctgtgacaccaacctcatccttcacataaatctgcaaatcaaatatgtttggtcctgtttcaaaatctagttgttccatcccagtggtgacaacctcaaagtaggtgcctgacagccaattcaccctaaaagcttcagtgaggggatttgagttgactatctggggaaatcctgggatcacaggtgacaatgatgctgataacttcacagaaaacttgtgcactgaagtcccaggtggagaattctctgccacattgcctgtagcaggtaagaggattaggtgtagtgcttctccccctgacatggcacccaggagagccaggagaatgattgcttcctgcatacttgatggtcacaactgtgcgtgcttccagcacattagccacagcctgaatccc

SEQ ID NO: 14783 - RNA, 4643 nt, Homo sapiens
  source 1..4643: mol_type = other RNA
gctgggattacaggcatgagccacctcacccggcccttttaatcattcttaatgggcttataagcagttattaagtcccccttcagccttctcagaacctcattttacttgcattgaagctgagagcttccaaggaaagcatttgactccgggccccacagatttgcaatgccttaaatgggcaatcagccacttcactcactttaacctgcataaatgaacagttctgccttcttttgcaaagtttaaatccattcaagggagttccctggcaaccaacccttattaataaatcacgctcaatctaggccaggacaggcattttgcaaatgcttcttttgcttgagaagtgacactggcactaggcacacagtaaacaagctgctgctctctctgaagctctacatttgctggatccagtctgtctcccacaggaccttgtggacctggtaggctctcacctgactccccagttgggaagggagtgcttccctaatgaacactcacctggacctttcttagggttactggactagggtcgcagcagctgggcagcagggcatagagctcgagtgaagcttgctcaggctctgctaggcacacattggaaagttacatttcctattccatcataataccatttattcccagttcattgctcatgcctacaggtggaagtctgagttttatgtctagatggggcttccagtatgtccccactcagagtcctgcagttccttccaatcataggaagtgggaaggagcaaggcaggtaggttgtaaggctgatggtgtttcagctttgaggaaaaagtgatttcacttcaatagtaattttaaccagaatggctaaagttaaaaggattgacaatcccaagtgttggcaaggatagagagcaattgcaactctcagtgtttgctgctggaatgtgaatcagagccaccactttggaactctttggcagatccagcaattgctccagcaatcccactcttagatatatgagcaaaaaagtgagtgtttatgttcaccaaaagacatgtacaagaaagttcatagtgttgtaattcacttttattttttttttctgagatggagtcttgctttgtcacccaggctagagtgcagtggcacaatctcaactcactgtaacctccacctctcaggtttaagcagttctccctacctcagcctcccaagtagctgggattacatgtgcccaccaccacaccaagctaatttttgtattttttagtagagacagggttttgccatctaggccaggctgatcttgaactcctgaccttaggtgatctgcccaccttggcaaagtgctggcattacaggcatgagccatcatgccctgcctgtagttcacttttaagtatattttttaaaagtaaaaaatctgaagcagctgccacccaagtgtagaatagataaattgtgatataatcatagaatgaaaccagacataaccatgaagagaactgaactactgctagacaggacaacgtggatgaatctcacatgcaggatgctgatccggacaccacaagaaaaaacaaaagaaggtgcctactgagttttcttctttccagatgaccaactcttaacttactcatctgtttttttcactgttctgcttcttttgaagaagatttgaggtgacttacaaaggtgtatggcatatttataactgaagaaatctgggtgatgttaaaacgagggcaggaaaataaggtggaaaccagatgtaaggatagtcttcactatttatgtcaggaattcctacaaactttctatggtgaacagaatagagcttcctagcagtcaatgcaaagaagaaacacaacaattccacaccccaaagttaacagtcttgcttatcagaagcacaggtagttctgaaatctgatagaaaatgttcctgtatcatttcagaacacgcaactatgtgatcaaacccctttctatttgtttaaaaatttgtcaaacatcccatgtttgaccctggatgtctgaatcccctcagcccacattttcccccctacaccatgcccacaccatccccatagaatttagggtgaggcagcatctcagtgattgacaggcccctccttagaccccgtttactttcctgggtgtggtttggggtaagccctgttcatgaaggctggatttctgttctttgggttgcccagcttgccaccctcatttctggaacccagaccagcatcctcagcccacgctttgccactcagctcatcttcttcccagttggcacttctcagtgaccccatcccttccccagcagtgactctgcgtggggcagctccctggtggctggactctttccattttggcatttgggttagtggatctttccactttctggctccagtttttgagttgaattcatatgtttccccggtcactggatctatggcttctccatcaaagatagtgttcatctggatagtttccaccacgacgtctctctctgcagtcttcgtttctcctttctttgtcagaggttccttgttcttcccagtcttgcaggggcagtgtctgtggatggctttggccaataggacgaccaggtacacgaggagacccagaagcaatatggagcccaaagtgatgacaaacggcacgtaccatgcagatggagagtaaacgtttttcctcaggacctgataggtgaccctgggcctgggggtcgtggtgatgatagtggttgggtggggaatgactttaatactcagtgtcactgttcctgtctcaacaagagcctccgctttcttcctgtcagacatcaagttgtcatcagttacgtagacaagtagcttgtagtcccagatcttatcaaacccaccagcatagtcaaagcgagatgtaagcagcaggcgtgtgacattggaaccagcattgggagagaaggtgaaatgattgttgacgttacctgggccaatggaataacggaaagatctggggctggaatcaaggtcggtacatgtcagcttgaaattctgaatatttgtgccaactttcagatccactgggagggccaggaaataagagtttggagtacaaattggcttttcatcattttcttcaaggatgttcacagtaacagtgacagagcttgtgtcttcgttgttggtggcctggattctgagaatatagatgggggttgtttcacagtccactttagttaccagctggagttctcctgtcttgggattaatccaaaatacatttggatactggaggctggcccctccagtggagatggagtacaggaggctgctctgggggaggtctttatcagtggctcgcacctgtcccactcgggttctggcgggccttctttctgacacatcaaatacataggatggcctatcaaaaatgagaggaaactcattttctgggcttgttaggatataaacgtagacgttatttttatagtaagggggggccacatcctgcacctggattatcaccgtatatttattgccggctgctaggttacttggattttcgtagtctagatcaccaatcagcacaatcttcccagagccagctggatcctgtaaaaatctgctgccgctccccactccagatggcatggtgaagttgaatctgttgtttggtgcctcactgtcatcatcaaagcagaacttgtttaggtcaagaagcaacgtccccttggctgttctttccggcaccataatgctgaaggtgaacttttggcatgtggcaggattgtcgttgacgtcttccacaatgaaggttatctggatgcgattctcctgacccccatatggtctgtccttcactagaacttccagggaaatggtgggattttgtctcaattcacctgcatctcggtctatcctttgggccacttggattgtaccagtcaactgatttatcatgaaatatttgctaacagtggtaatgctgtagaggaggtggctgggaaaaccttcatcatcaggatcctccgctgtgatattggccacgatggttcctggactcagttcctccaggactgtgtacactcgtgtcgggctggtaaagcgagggacttcgtcgttgaggttcacgatgttcacctggagctctgtggaggctttgaggcctccactgtccctcacctccacgatgagatggaaacttctgtgtcctgcttcaaagtccaattctgttgtggagaagagggtgccattagcagacattctgaagctctttgggggagaaatcaggaaataactgaggggaatgtttcggcttgtgtcttctggatcgaaggcctcaacctggtaaatgaatccagggtttgctctttctactatgtagaggtgtagaccttctgccaagttgccttgaaactgaggtggctcgttcacatctgttacctggacagtcaggacttgcaggtctgtgacaccaacctcatccttcacataaatctgcaaatcaaatatgtttggtcctgtttcaaaatctagttgttccatcccagtggtgacaacctgacatggcacccaggagagccaggagaatgattgcttcctgcatacttgatggtcacaactgtgcgtgcttccagcacattagccacagcctgaatccc

SEQ ID NO: 14784 - RNA, 5050 nt, Homo sapiens
  source 1..5050: mol_type = other RNA
gctgggattacaggcatgagccacctcacccggcccttttaatcattcttaatgggcttataagcagttattaagtcccccttcagccttctcagaacctcattttacttgcattgaagctgagagcttccaaggaaagcatttgactccgggccccacagatttgcaatgccttaaatgggcaatcagccacttcactcactttaacctgcataaatgaacagttctgccttcttttgcaaagtttaaatccattcaagggagttccctggcaaccaacccttattaataaatcacgctcaatctaggccaggacaggcattttgcaaatgcttcttttgcttgagaagtgacactggcactaggcacacagtaaacaagctgctgctctctctgaagctctacatttgctggatccagtctgtctcccacaggaccttgtggacctggtaggctctcacctgactccccagttgggaagggagtgcttccctaatgaacactcacctggacctttcttagggttactggactagggtcgcagcagctgggcagcagggcatagagctcgagtgaagcttgctcaggctctgctaggcacacattggaaagttacatttcctattccatcataataccatttattcccagttcattgctcatgcctacaggtggaagtctgagttttatgtctagatggggcttccagtatgtccccactcagagtcctgcagttccttccaatcataggaagtgggaaggagcaaggcaggtaggttgtaaggctgatggtgtttcagctttgaggaaaaagtgatttcacttcaatagtaattttaaccagaatggctaaagttaaaaggattgacaatcccaagtgttggcaaggatagagagcaattgcaactctcagtgtttgctgctggaatgtgaatcagagccaccactttggaactctttggcagatccagcaattgctccagcaatcccactcttagatatatgagcaaaaaagtgagtgtttatgttcaccaaaagacatgtacaagaaagttcatagtgttgtaattcacttttattttttttttctgagatggagtcttgctttgtcacccaggctagagtgcagtggcacaatctcaactcactgtaacctccacctctcaggtttaagcagttctccctacctcagcctcccaagtagctgggattacatgtgcccaccaccacaccaagctaatttttgtattttttagtagagacagggttttgccatctaggccaggctgatcttgaactcctgaccttaggtgatctgcccaccttggcaaagtgctggcattacaggcatgagccatcatgccctgcctgtagttcacttttaagtatattttttaaaagtaaaaaatctgaagcagctgccacccaagtgtagaatagataaattgtgatataatcatagaatgaaaccagacataaccatgaagagaactgaactactgctagacaggacaacgtggatgaatctcacatgcaggatgctgatccggacaccacaagaaaaaacaaaagaaggtgcctactgagttttcttctttccagatgaccaactcttaacttactcatctgtttttttcactgttctgcttcttttgaagaagatttgaggtgacttacaaaggtgtatggcatatttataactgaagaaatctgggtgatgttaaaacgagggcaggaaaataaggtggaaaccagatgtaaggatagtcttcactatttatgtcaggaattcctacaaactttctatggtgaacagaatagagcttcctagcagtcaatgcaaagaagaaacacaacaattccacaccccaaagttaacagtcttgcttatcagaagcacaggtagttctgaaatctgatagaaaatgttcctgtatcatttcagaacacgcaactatgtgatcaaacccctttctatttgtttaaaaatttgtcaaacatcccatgtttgaccctggatgtctgaatcccctcagcccacattttcccccctacaccatgcccacaccatccccatagaatttagggtgaggcagcatctcagtgattgacaggcccctccttagaccccgtttactttcctgggtgtggtttggggtaagccctgttcatgaaggctggatttctgttctttgggttgcccagcttgccaccctcatttctggaacccagaccagcatcctcagcccacgctttgccactcagctcatcttcttcccagttggcacttctcagtgaccccatcccttccccagcagtgactctgcgtggggcagctccctggtggctggactctttccattttggcatttgggttagtggatctttccactttctggctccagtttttgagttgaattcatatgtttccccggtcactggatctatggcttctccatcaaagatagtgttcatctggatagtttccaccacgacgtctctctctgcagtcttcgtttctcctttctttgtcagaggttccttgttcttcccagtcttgcaggggcagtgtctgtggatggctttggccaataggacgaccaggtacacgaggagacccagaagcaatatggagcccaaagtgatgacaaacggcacgtaccatgcagatggagagtaaacgtttttcctcaggacctgataggtgaccctgggcctgggggtcgtggtgatgatagtggttgggtggggaatgactttaatactcagtgtcactgttcctgtctcaacaagagcctccgctttcttcctgtcagacatcaagttgtcatcagttacgtagacaagtagcttgtagtcccagatcttatcaaacccaccagcatagtcaaagcgagatgtaagcagcaggcgtgtgacattggaaccagcattgggagagaaggtgaaatgattgttgacgttacctgggccaatggaataacggaaagatctggggctggaatcaaggtcggtacatgtcagcttgaaattctgaatatttgtgccaactttcagatccactgggagggccaggaaataagagtttggagtacaaattggcttttcatcattttcttcaaggatgttcacagtaacagtgacagagcttgtgtcttcgttgttggtggcctggattctgagaatatagatgggggttgtttcacagtccactttagttaccagctggagttctcctgtcttgggattaatccaaaatacatttggatactggaggctggcccctccagtggagatggagtacaggaggctgctctgggggaggtctttatcagtggctcgcacctgtcccactcgggttctggcgggccttctttctgacacatcaaatacataggatggcctatcaaaaatgagaggaaactcattttctgggcttgttaggatataaacgtagacgttatttttatagtaagggggggccacatcctgcacctggattatcaccgtatatttattgccggctgctaggttacttggattttcgtagtctagatcaccaatcagcacaatcttcccagagccagctggatcctgtaaaaatctgctgccgctccccactccagatggcatggtgaagttgaatctgttgtttggtgcctcactgtcatcatcaaagcagaacttgtttaggtcaagaagcaacgtccccttggctgttctttccggcaccataatgctgaaggtgaacttttggcatgtggcaggattgtcgttgacgtcttccacaatgaaggttatctggatgcgattctcctgacccccatatggtctgtccttcactagaacttccagggaaatggtgggattttgtctcaattcacctgcatctcggtctatcctttgggccacttggattgtaccagtcaactgatttatcatgaaatatttgctaacagtggtaatgctgtagaggaggtggctgggaaaaccttcatcatcaggatcctccgctgtgatattggccacgatggttcctggactcagttcctccaggactgtgtacactcgtgtcgggctggtaaagcgagggacttcgtcgttgaggttcacgatgttcacctggagctctgtggaggctttgaggcctccactgtccctcacctccacgatgagatggaaacttctgtgtcctgcttcaaagtccaattctgttgtggagaagagggtgccattagcagacattctgaagctctttgggggagaaatcaggaaataactgaggggaatgtttcggcttgtgtcttctggatcgaaggcctcaacctggtaaatgaatccagggtttgctctttctactatgtagaggtgtagaccttctgccaagttgccttgaaactgaggtggctcgttcacatctgttacctggacagtcaggacttgcaggtctgtgacaccaacctcatccttcacataaatctgcaaatcaaatatgtttggtcctgtttcaaaatctagttgttccatcccagtggtgacaacctgcgtttcagaacgacatctacccactggtttcagctcctagagcaacaactgcagaatctccatggtccaaagtcctccaggaaagagaagaaaggggtgacgggggtgagggctgggaggcgaggtcaccagggtcccttccctggctcgggtgggggtggggggcgcaacccctcacggctcctccccaccaagccgtcgggaccccagcgggggcgcctcgcgttgggcgacagggacgcggggagagagcgacaagctggaagcaagggctgcctgcaaaactttcggtcctccagcggcaactctgcgggaaagaccacccttccttcggccccgcgtcgggcctatccccgtgtgccccgacccctgcgccccaggcttgggcggcgccgctgcatcccggctgccgggcgcgctgcagccttcgctctcccgcacgcggcgctcgcccgtccgcgctgcccctccccggcaggcgggcggccccggcgggcgggcgggc

SEQ ID NO: 14785 - RNA, 4358 nt, Homo sapiens
  source 1..4358: mol_type = other RNA
gctgggattacaggcatgagccacctcacccggcccttttaatcattcttaatgggcttataagcagttattaagtcccccttcagccttctcagaacctcattttacttgcattgaagctgagagcttccaaggaaagcatttgactccgggccccacagatttgcaatgccttaaatgggcaatcagccacttcactcactttaacctgcataaatgaacagttctgccttcttttgcaaagtttaaatccattcaagggagttccctggcaaccaacccttattaataaatcacgctcaatctaggccaggacaggcattttgcaaatgcttcttttgcttgagaagtgacactggcactaggcacacagtaaacaagctgctgctctctctgaagctctacatttgctggatccagtctgtctcccacaggaccttgtggacctggtaggctctcacctgactccccagttgggaagggagtgcttccctaatgaacactcacctggacctttcttagggttactggactagggtcgcagcagctgggcagcagggcatagagctcgagtgaagcttgctcaggctctgctaggcacacattggaaagttacatttcctattccatcataataccatttattcccagttcattgctcatgcctacaggtggaagtctgagttttatgtctagatggggcttccagtatgtccccactcagagtcctgcagttccttccaatcataggaagtgggaaggagcaaggcaggtaggttgtaaggctgatggtgtttcagctttgaggaaaaagtgatttcacttcaatagtaattttaaccagaatggctaaagttaaaaggattgacaatcccaagtgttggcaaggatagagagcaattgcaactctcagtgtttgctgctggaatgtgaatcagagccaccactttggaactctttggcagatccagcaattgctccagcaatcccactcttagatatatgagcaaaaaagtgagtgtttatgttcaccaaaagacatgtacaagaaagttcatagtgttgtaattcacttttattttttttttctgagatggagtcttgctttgtcacccaggctagagtgcagtggcacaatctcaactcactgtaacctccacctctcaggtttaagcagttctccctacctcagcctcccaagtagctgggattacatgtgcccaccaccacaccaagctaatttttgtattttttagtagagacagggttttgccatctaggccaggctgatcttgaactcctgaccttaggtgatctgcccaccttggcaaagtgctggcattacaggcatgagccatcatgccctgcctgtagttcacttttaagtatattttttaaaagtaaaaaatctgaagcagctgccacccaagtgtagaatagataaattgtgatataatcatagaatgaaaccagacataaccatgaagagaactgaactactgctagacaggacaacgtggatgaatctcacatgcaggatgctgatccggacaccacaagaaaaaacaaaagaaggtgcctactgagttttcttctttccagatgaccaactcttaacttactcatctgtttttttcactgttctgcttcttttgaagaagatttgaggtgacttacaaaggtgtatggcatatttataactgaagaaatctgggtgatgttaaaacgagggcaggaaaataaggtggaaaccagatgtaaggatagtcttcactatttatgtcaggaattcctacaaactttctatggtgaacagaatagagcttcctagcagtcaatgcaaagaagaaacacaacaattccacaccccaaagttaacagtcttgcttatcagaagcacaggtagttctgaaatctgatagaaaatgttcctgtatcatttcagaacacgcaactatgtgatcaaacccctttctatttgtttaaaaatttgtcaaacatcccatgtttgaccctggatgtctgaatcccctcagcccacattttcccccctacaccatgcccacaccatccccatagaatttagggtgaggcagcatctcagtgattgacaggcccctccttagaccccgtttactttcctgggtgtggtttggggtaagccctgttcatgaaggctggatttctgttctttgggttgcccagcttgccaccctcatttctggaacccagaccagcatcctcagcccacgctttgccactcagctcatcttcttcccagttggcacttctcagtgaccccatcccttccccagcagtgactctgcgtggggcagctccctggtggctggactctttccattttggcatttgggttagtggatctttccactttctggctccagtttttgagttgaattcatatgtttccccggtcactggatctatggcttctccatcaaagatagtgttcatctggatagtttccaccacgacgtctctctctgcagtcttcgtttctcctttctttgtcagaggttccttgttcttcccagtcttgcaggggcagtgtctgtggatggctttggccaataggacgaccaggtacacgaggagacccagaagcaatatggagcccaaagtgatgacaaacggcacgtaccatgcagatggagagtaaacgtttttcctcaggacctgataggtgaccctgggcctgggggtcgtggtgatgatagtggttgggtggggaatgactttaatactcagtgtcactgttcctgtctcaacaagagcctccgctttcttcctgtcagacatcaagttgtcatcagttacgtagacaagtagcttgtagtcccagatcttatcaaacccaccagcatagtcaaagcgagatgtaagcagcaggcgtgtgacattggaaccagcattgggagagaaggtgaaatgattgttgacgttacctgggccaatggaataacggaaagatctggggctggaatcaaggtcggtacatgtcagcttgaaattctgaatatttgtgccaactttcagatccactgggagggccaggaaataagagtttggagtacaaattggcttttcatcattttcttcaaggatgttcacagtaacagtgacagagcttgtgtcttcgttgttggtggcctggattctgagaatatagatgggggttgtttcacagtccactttagttaccagctggagttctcctgtcttgggattaatccaaaatacatttggatactggaggctggcccctccagtggagatggagtacaggaggctgctctgggggaggtctttatcagtggctcgcacctgtcccactcgggttctggcgggccttctttctgacacatcaaatacataggatggcctatcaaaaatgagaggaaactcattttctgggcttgttaggatataaacgtagacgttatttttatagtaagggggggccacatcctgcacctggattatcaccgtatatttattgccggctgctaggttacttggattttcgtagtctagatcaccaatcagcacaatcttcccagagccagctggatcctgtaaaaatctgctgccgctccccactccagatggcatggtgaagttgaatctgttgtttggtgcctcactgtcatcatcaaagcagaacttgtttaggtcaagaagcaacgtccccttggctgttctttccggcaccataatgctgaaggtgaacttttggcatgtggcaggattgtcgttgacgtcttccacaatgaaggttatctggatgcgattctcctgacccccatatggtctgtccttcactagaacttccagggaaatggtgggattttgtctcaattcacctgcatctcggtctatcctttgggccacttggattgtaccagtcaactgatttatcatgaaatatttgctaacagtggtaatgctgtagaggaggtggctgggaaaaccttcatcatcaggatcctccgctgtgatattggccacgatggttcctggactcagttcctccaggactgtgtacactcgtgtcgggctggtaaagcgagggacttcgtcgttgaggttcacgatgttcacctggagctctgtggaggctttgaggcctccactgtccctcacctccacgatgagatggaaacttctgtgtcctgcttcaaagtccaattctgttgtggagaagagggtgccattagcagacattctgaagctctttgggggagaaatcaggaaataatgtttatattcatttcttccaaagggctttaaggttagaaggtttcattatttcctgctaggatgagggatgttctatc

SEQ ID NO: 14786 - RNA, 7066 nt, Homo sapiens
  source 1..7066: mol_type = other RNA
gctgggattacaggcatgagccacctcacccggcccttttaatcattcttaatgggcttataagcagttattaagtcccccttcagccttctcagaacctcattttacttgcattgaagctgagagcttccaaggaaagcatttgactccgggccccacagatttgcaatgccttaaatgggcaatcagccacttcactcactttaacctgcataaatgaacagttctgccttcttttgcaaagtttaaatccattcaagggagttccctggcaaccaacccttattaataaatcacgctcaatctaggccaggacaggcattttgcaaatgcttcttttgcttgagaagtgacactggcactaggcacacagtaaacaagctgctgctctctctgaagctctacatttgctggatccagtctgtctcccacaggaccttgtggacctggtaggctctcacctgactccccagttgggaagggagtgcttccctaatgaacactcacctggacctttcttagggttactggactagggtcgcagcagctgggcagcagggcatagagctcgagtgaagcttgctcaggctctgctaggcacacattggaaagttacatttcctattccatcataataccatttattcccagttcattgctcatgcctacaggtggaagtctgagttttatgtctagatggggcttccagtatgtccccactcagagtcctgcagttccttccaatcataggaagtgggaaggagcaaggcaggtaggttgtaaggctgatggtgtttcagctttgaggaaaaagtgatttcacttcaatagtaattttaaccagaatggctaaagttaaaaggattgacaatcccaagtgttggcaaggatagagagcaattgcaactctcagtgtttgctgctggaatgtgaatcagagccaccactttggaactctttggcagatccagcaattgctccagcaatcccactcttagatatatgagcaaaaaagtgagtgtttatgttcaccaaaagacatgtacaagaaagttcatagtgttgtaattcacttttattttttttttctgagatggagtcttgctttgtcacccaggctagagtgcagtggcacaatctcaactcactgtaacctccacctctcaggtttaagcagttctccctacctcagcctcccaagtagctgggattacatgtgcccaccaccacaccaagctaatttttgtattttttagtagagacagggttttgccatctaggccaggctgatcttgaactcctgaccttaggtgatctgcccaccttggcaaagtgctggcattacaggcatgagccatcatgccctgcctgtagttcacttttaagtatattttttaaaagtaaaaaatctgaagcagctgccacccaagtgtagaatagataaattgtgatataatcatagaatgaaaccagacataaccatgaagagaactgaactactgctagacaggacaacgtggatgaatctcacatgcaggatgctgatccggacaccacaagaaaaaacaaaagaaggtgcctactgagttttcttctttccagatgaccaactcttaacttactcatctgtttttttcactgttctgcttcttttgaagaagatttgaggtgacttacaaaggtgtatggcatatttataactgaagaaatctgggtgatgttaaaacgagggcaggaaaataaggtggaaaccagatgtaaggatagtcttcactatttatgtcaggaattcctacaaactttctatggtgaacagaatagagcttcctagcagtcaatgcaaagaagaaacacaacaattccacaccccaaagttaacagtcttgcttatcagaagcacaggtagttctgaaatctgatagaaaatgttcctgtatcatttcagaacacgcaactatgtgatcaaacccctttctatttgtttaaaaatttgtcaaacatcccatgtttgaccctggatgtctgaatcccctcagcccacattttcccccctacaccatgcccacaccatccccatagaatttagggtgaggcagcatctcagtgattgacaggcccctccttagaccccgtttactttcctgggtgtggtttggggtaagccctgttcatgaaggctggatttctgttctttgggttgcccagcttgccaccctcatttctggaacccagaccagcatcctcagcccacgctttgccactcagctcatcttcttcccagttggcacttctcagtgaccccatcccttccccagcagtgactctgcgtggggcagctccctggtggctggactctttccattttggcatttgggttagtggatctttccactttctggctccagtttttgagttgaattcatatgtttccccggtcactggatctatggcttctccatcaaagatagtgttcatctggatagtttccaccacgacgtctctctctgcagtcttcgtttctcctttctttgtcagaggttccttgttcttcccagtcttgcaggggcagtgtctgtggatggctttggccaataggacgaccaggtacacgaggagacccagaagcaatatggagcccaaagtgatgacaaacggcacgtaccatgcagatggagagtaaacgtttttcctcaggacctgataggtgaccctgggcctgggggtcgtggtgatgatagtggttgggtggggaatgactttaatactcagtgtcactgttcctgtctcaacaagagcctccgctttcttcctgtcagacatcaagttgtcatcagttacgtagacaagtagcttgtagtcccagatcttatcaaacccaccagcatagtcaaagcgagatgtaagcagcaggcgtgtgacattggaaccagcattgggagagaaggtgaaatgattgttgacgttacctgggccaatggaataacggaaagatctggggctggaatcaaggtcggtacatgtcagcttgaaattctgaatatttgtgccaactttcagatccactgggagggccaggaaataagagtttggagtacaaattggcttttcatcattttcttcaaggatgttcacagtaacagtgacagagcttgtgtcttcgttgttggtggcctggattctgagaatatagatgggggttgtttcacagtccactttagttaccagctggagttctcctgtcttgggattaatccaaaatacatttggatactggaggctggcccctccagtggagatggagtacaggaggctgctctgggggaggtctttatcagtggctcgcacctgtcccactcgggttctggcgggccttctttctgacacatcaaatacataggatggcctatcaaaaatgagaggaaactcattttctgggcttgttaggatataaacgtagacgttatttttatagtaagggggggccacatcctgcacctggattatcaccgtatatttattgccggctgctaggttacttggattttcgtagtctagatcaccaatcagcacaatcttcccagagccagctggatcctgtaaaaatctgctgccgctccccactccagatggcatggtgaagttgaatctgttgtttggtgcctcactgtcatcatcaaagcagaacttgtttaggtcaagaagcaacgtccccttggctgttctttccggcaccataatgctgaaggtgaacttttggcatgtggcaggattgtcgttgacgtcttccacaatgaaggttatctggatgcgattctcctgacccccatatggtctgtccttcactagaacttccagggaaatggtgggattttgtctcaattcacctgcatctcggtctatcctttgggccacttggattgtaccagtcaactgatttatcatgaaatatttgctaacagtggtaatgctgtagaggaggtggctgggaaaaccttcatcatcaggatcctccgctgtgatattggccacgatggttcctggactcagttcctccaggactgtgtacactcgtgtcgggctggtaaagcgagggacttcgtcgttgaggttcacgatgttcacctggagctctgtggaggctttgaggcctccactgtccctcacctccacgatgagatggaaacttctgtgtcctgcttcaaagtccaattctgttgtggagaagagggtgccattagcagacattctgaagctctttgggggagaaatcaggaaataccttgattgtgccttggtgtagggagaaaggaaggtgagagggagctggcccagtttccagaaatgtcagctccctggggtacgaggggaacgccacctccaggcttgcttccccactgcagtaggagtcaccgaccaatgattcaacctgtgccactttgcagctatcagttgctttcagtagaaacaaacaacaagaattcagcttcttgtcttttatagaatagagcagtcaactaccaggccaccgcaggctgagtttccagaaggaaagacccttattcggcccacatccagggagtgtcaatggctccacaagccactgagtacatggccccaaacccaccccagagggccagagcactcaggactgtggcaagttacaaatatgttgccacattcctatatttttcaatggaagctgaatattttgtaaaagcctcaattcctctctttgttttcccctattccaccctcgtctcagctcagaggtgggacgtggaggaggaaggaggaagagtgcctagaagaaaaaaaactatcgttaaaaaactacccactgcaagtccttaacgtggctcctgctcgtggttcattgttctgaggatgagctaagtgggttacaggcaagtacttgaatgtttttaagaagagacacgatgacaaatgcaaaatgctattattaatgtaatccttcaccgataaagctgcagatcctatgccctcacattctgtcattctttttccataattggcctgggttctgtgctgcaagattcaggctttgctaatcttaataacaatgatccccatctatttgagagtgtcccaccccacatgcaaacagccagcagtgaccacatatttggagtgggaattgtccagtacctttgctttttccttttatgagcctttgaacaagaacctggagtagaatgaagaatgccttttgctaagacttcaggtggtgactcctgactcctgagttggcaggcagacaccaggggagctgaatgactggggcaggtgggggtgtatggtggggacagggatgctgtcactcagaaaagcaaggggtaggaagccagtggcagaacttgccagaacagagtagaagggaggtgggtcaggagacctgggttctcactggagttacctgacccctcagttccctccctcatccagaaatcaaggactgcccaatggacctgaaagatcccatccagctgggacccttgatagggccaggtctggcatatgatgaccactttatacacaggaaaaccaaaactcacaactggctgccacttcctagagctatgagcaagataaagacagaaagagaaggatggcccctgctgcgctcccaaaagtccaggtagtagctaggttattgctctcttaatttaatcctttgtctgccttggtgaagacaaagcacatttcattttatgcaaaagcccttcctcaatggaaaggccaaaagaaagccccttaatggagaaattgctgtactagatcattttgcctccagctgagagattgattaacatcctgggagtctccaaggaggctcttctgcagtcacggtggccatttccaagcagagggggaagcagagagtgtgggagttgaatgggaggagggtggtctcaaagagcctccttcagaaagtggagaagaggtgggggggtgggtacccaaagaagaaatgccagtaaaaataattattcacatgcagatcatccttctctatgttctgagcccattattaatgcatacctccaagccaagccccggctctacctgcatgcccaccacaacacagaaggtgcccaggaagggggaaccaatgctagatctaagcctgtgcctggccaatgcagtagccactaccctcacgtacgtgtgactatgagcattgaaatgtggctggtctgcacggagatgatctgtaagtgtaaaatgcacactgagtttggacaccgagtatggaaaaagaaggcaaaatatctcattaatcattttatgttgactatgctgaaatattttgagtatactgagttaaataagctattaaaattaatttcatttattttgttttactttcaatgtggctactagaacatttaaaattacatgtgcaggactcatttctggctcacagtatagctttattggacagagccggtccaatattgatcagtgttggtccaaacaatgtaccagcacatgctttttaagtttcactaaaaagaagggagcaaatacaagtggcttccagattagtacctgtttttcattaactgtgatacagtttcactttattaagctggagaagagttgtaagatttgtcattttaaaggggttgaggtttcaaaatgcatcctatagctatttttaaaaatccattattcattctctagttgctgccaccagcagggtgactcgtggaccccaccaggttaagatgacagacacaaaccaagcctaggtcgcttcaggcatgtgctttagtgttttgttaaactctgtccttgtttgttcagtccagtggttcttgaagtacatggtacatcagaatcaccggggaggtttgtattcaaactcagcattctcaggcaatgtccaggaatctgcatttttaaaatcagcctaagtatgttctaatgcctgaacacacttctaaagcctgcaaaacacttataaaccggtgtttccactgggtgtggtggctcatgtctgtaatcctagcactttgggaggccaaggcaggtggatggcttg

SEQ ID NO: 14787 - RNA, 5155 nt, Homo sapiens
  source 1..5155: mol_type = other RNA
gctgggattacaggcatgagccacctcacccggcccttttaatcattcttaatgggcttataagcagttattaagtcccccttcagccttctcagaacctcattttacttgcattgaagctgagagcttccaaggaaagcatttgactccgggccccacagatttgcaatgccttaaatgggcaatcagccacttcactcactttaacctgcataaatgaacagttctgccttcttttgcaaagtttaaatccattcaagggagttccctggcaaccaacccttattaataaatcacgctcaatctaggccaggacaggcattttgcaaatgcttcttttgcttgagaagtgacactggcactaggcacacagtaaacaagctgctgctctctctgaagctctacatttgctggatccagtctgtctcccacaggaccttgtggacctggtaggctctcacctgactccccagttgggaagggagtgcttccctaatgaacactcacctggacctttcttagggttactggactagggtcgcagcagctgggcagcagggcatagagctcgagtgaagcttgctcaggctctgctaggcacacattggaaagttacatttcctattccatcataataccatttattcccagttcattgctcatgcctacaggtggaagtctgagttttatgtctagatggggcttccagtatgtccccactcagagtcctgcagttccttccaatcataggaagtgggaaggagcaaggcaggtaggttgtaaggctgatggtgtttcagctttgaggaaaaagtgatttcacttcaatagtaattttaaccagaatggctaaagttaaaaggattgacaatcccaagtgttggcaaggatagagagcaattgcaactctcagtgtttgctgctggaatgtgaatcagagccaccactttggaactctttggcagatccagcaattgctccagcaatcccactcttagatatatgagcaaaaaagtgagtgtttatgttcaccaaaagacatgtacaagaaagttcatagtgttgtaattcacttttattttttttttctgagatggagtcttgctttgtcacccaggctagagtgcagtggcacaatctcaactcactgtaacctccacctctcaggtttaagcagttctccctacctcagcctcccaagtagctgggattacatgtgcccaccaccacaccaagctaatttttgtattttttagtagagacagggttttgccatctaggccaggctgatcttgaactcctgaccttaggtgatctgcccaccttggcaaagtgctggcattacaggcatgagccatcatgccctgcctgtagttcacttttaagtatattttttaaaagtaaaaaatctgaagcagctgccacccaagtgtagaatagataaattgtgatataatcatagaatgaaaccagacataaccatgaagagaactgaactactgctagacaggacaacgtggatgaatctcacatgcaggatgctgatccggacaccacaagaaaaaacaaaagaaggtgcctactgagttttcttctttccagatgaccaactcttaacttactcatctgtttttttcactgttctgcttcttttgaagaagatttgaggtgacttacaaaggtgtatggcatatttataactgaagaaatctgggtgatgttaaaacgagggcaggaaaataaggtggaaaccagatgtaaggatagtcttcactatttatgtcaggaattcctacaaactttctatggtgaacagaatagagcttcctagcagtcaatgcaaagaagaaacacaacaattccacaccccaaagttaacagtcttgcttatcagaagcacaggtagttctgaaatctgatagaaaatgttcctgtatcatttcagaacacgcaactatgtgatcaaacccctttctatttgtttaaaaatttgtcaaacatcccatgtttgaccctggatgtctgaatcccctcagcccacattttcccccctacaccatgcccacaccatccccatagaatttagggtgaggcagcatctcagtgattgacaggcccctccttagaccccgtttactttcctgggtgtggtttggggtaagccctgttcatgaaggctggatttctgttctttgggttgcccagcttgccaccctcatttctggaacccagaccagcatcctcagcccacgctttgccactcagctcatcttcttcccagttggcacttctcagtgaccccatcccttccccagcagtgactctgcgtggggcagctccctggtggctggactctttccattttggcatttgggttagtggatctttccactttctggctccagtttttgagttgaattcatatgtttccccggtcactggatctatggcttctccatcaaagatagtgttcatctggatagtttccaccacgacgtctctctctgcagtcttcgtttctcctttctttgtcagaggttccttgttcttcccagtcttgcaggggcagtgtctgtggatggctttggccaataggacgaccaggtacacgaggagacccagaagcaatatggagcccaaagtgatgacaaacggcacgtaccatgcagatggagagtaaacgtttttcctcaggacctgataggtgaccctgggcctgggggtcgtggtgatgatagtggttgggtggggaatgactttaatactcagtgtcactgttcctgtctcaacaagagcctccgctttcttcctgtcagacatcaagttgtcatcagttacgtagacaagtagcttgtagtcccagatcttatcaaacccaccagcatagtcaaagcgagatgtaagcagcaggcgtgtgacattggaaccagcattgggagagaaggtgaaatgattgttgacgttacctgggccaatggaataacggaaagatctggggctggaatcaaggtcggtacatgtcagcttgaaattctgaatatttgtgccaactttcagatccactgggagggccaggaaataagagtttggagtacaaattggcttttcatcattttcttcaaggatgttcacagtaacagtgacagagcttgtgtcttcgttgttggtggcctggattctgagaatatagatgggggttgtttcacagtccactttagttaccagctggagttctcctgtcttgggattaatccaaaatacatttggatactggaggctggcccctccagtggagatggagtacaggaggctgctctgggggaggtctttatcagtggctcgcacctgtcccactcgggttctggcgggccttctttctgacacatcaaatacataggatggcctatcaaaaatgagaggaaactcattttctgggcttgttaggatataaacgtagacgttatttttatagtaagggggggccacatcctgcacctggattatcaccgtatatttattgccggctgctaggttacttggattttcgtagtctagatcaccaatcagcacaatcttcccagagccagctggatcctgtaaaaatctgctgccgctccccactccagatggcatggtgaagttgaatctgttgtttggtgcctcactgtcatcatcaaagcagaacttgtttaggtcaagaagcaacgtccccttggctgttctttccggcaccataatgctgaaggtgaacttttggcatgtggcaggattgtcgttgacgtcttccacaatgaaggttatctggatgcgattctcctgacccccatatggtctgtccttcactagaacttccagggaaatggtgggattttgtctcaattcacctgcatctcggtctatcctttgggccacttggattgtaccagtcaactgatttatcatgaaatatttgctaacagtggtaatgctgtagaggaggtggctgggaaaaccttcatcatcaggatcctccgctgtgatattggccacgatggttcctggactcagttcctccaggactgtgtacactcgtgtcgggctggtaaagcgagggacttcgtcgttgaggttcacgatgttcacctggagctctgtggaggctttgaggcctccactgtccctcacctccacgatgagatggaaacttctgtgtcctgcttcaaagtccaattctgttgtggagaagagggtgccattagcagacattctgaagctctttgggggagaaatcaggaaatacttctgccaagttgccttgaaactgaggtggctcgttcacatctgttacctggacagtcaggacttgcaggtctgtgacaccaacctcatccttcacataaatctgcaaatcaaatatgtttggtcctgtttcaaaatctagttgttccatcccagtggtgacaacctcaaagtaggtgcctgacagccaattcaccctaaaagcttcagtgaggggatttgagttgactatctggggaaatcctgggatcacaggtgacaatgatgctgataacttcacagaaaacttgtgcactgaagtcccaggtggagaattctctgccacattgcctgtagcaggtaagaggattaggtgtagtgcttctccccctgcgtttcagaacgacatctacccactggtttcagctcctagagcaacaactgcagaatctccatggtccaaagtcctccaggaaagagaagaaaggggtgacgggggtgagggctgggaggcgaggtcaccagggtcccttccctggctcgggtgggggtggggggcgcaacccctcacggctcctccccaccaagccgtcgggaccccagcgggggcgcctcgcgttgggcgacagggacgcggggagagagcgacaagctggaagcaagggctgcctgcaaaactttcggtcctccagcggcaactctgcgggaaagaccacccttccttcggccccgcgtcgggcctatccccgtgtgccccgacccctgcgccccaggcttgggcggcgccgctgcatcccggctgccgggcgcgctgcagccttcgctctcccgcacgcggcgctcgcccgtccgcgctgcccctccccggcaggcgggcggccccggcgggcgggcgggc

SEQ ID NO: 14788 - RNA, 4955 nt, Homo sapiens
  source 1..4955: mol_type = other RNA
gctgggattacaggcatgagccacctcacccggcccttttaatcattcttaatgggcttataagcagttattaagtcccccttcagccttctcagaacctcattttacttgcattgaagctgagagcttccaaggaaagcatttgactccgggccccacagatttgcaatgccttaaatgggcaatcagccacttcactcactttaacctgcataaatgaacagttctgccttcttttgcaaagtttaaatccattcaagggagttccctggcaaccaacccttattaataaatcacgctcaatctaggccaggacaggcattttgcaaatgcttcttttgcttgagaagtgacactggcactaggcacacagtaaacaagctgctgctctctctgaagctctacatttgctggatccagtctgtctcccacaggaccttgtggacctggtaggctctcacctgactccccagttgggaagggagtgcttccctaatgaacactcacctggacctttcttagggttactggactagggtcgcagcagctgggcagcagggcatagagctcgagtgaagcttgctcaggctctgctaggcacacattggaaagttacatttcctattccatcataataccatttattcccagttcattgctcatgcctacaggtggaagtctgagttttatgtctagatggggcttccagtatgtccccactcagagtcctgcagttccttccaatcataggaagtgggaaggagcaaggcaggtaggttgtaaggctgatggtgtttcagctttgaggaaaaagtgatttcacttcaatagtaattttaaccagaatggctaaagttaaaaggattgacaatcccaagtgttggcaaggatagagagcaattgcaactctcagtgtttgctgctggaatgtgaatcagagccaccactttggaactctttggcagatccagcaattgctccagcaatcccactcttagatatatgagcaaaaaagtgagtgtttatgttcaccaaaagacatgtacaagaaagttcatagtgttgtaattcacttttattttttttttctgagatggagtcttgctttgtcacccaggctagagtgcagtggcacaatctcaactcactgtaacctccacctctcaggtttaagcagttctccctacctcagcctcccaagtagctgggattacatgtgcccaccaccacaccaagctaatttttgtattttttagtagagacagggttttgccatctaggccaggctgatcttgaactcctgaccttaggtgatctgcccaccttggcaaagtgctggcattacaggcatgagccatcatgccctgcctgtagttcacttttaagtatattttttaaaagtaaaaaatctgaagcagctgccacccaagtgtagaatagataaattgtgatataatcatagaatgaaaccagacataaccatgaagagaactgaactactgctagacaggacaacgtggatgaatctcacatgcaggatgctgatccggacaccacaagaaaaaacaaaagaaggtgcctactgagttttcttctttccagatgaccaactcttaacttactcatctgtttttttcactgttctgcttcttttgaagaagatttgaggtgacttacaaaggtgtatggcatatttataactgaagaaatctgggtgatgttaaaacgagggcaggaaaataaggtggaaaccagatgtaaggatagtcttcactatttatgtcaggaattcctacaaactttctatggtgaacagaatagagcttcctagcagtcaatgcaaagaagaaacacaacaattccacaccccaaagttaacagtcttgcttatcagaagcacaggtagttctgaaatctgatagaaaatgttcctgtatcatttcagaacacgcaactatgtgatcaaacccctttctatttgtttaaaaatttgtcaaacatcccatgtttgaccctggatgtctgaatcccctcagcccacattttcccccctacaccatgcccacaccatccccatagaatttagggtgaggcagcatctcagtgattgacaggcccctccttagaccccgtttactttcctgggtgtggtttggggtaagccctgttcatgaaggctggatttctgttctttgggttgcccagcttgccaccctcatttctggaacccagaccagcatcctcagcccacgctttgccactcagctcatcttcttcccagttggcacttctcagtgaccccatcccttccccagcagtgactctgcgtggggcagctccctggtggctggactctttccattttggcatttgggttagtggatctttccactttctggctccagtttttgagttgaattcatatgtttccccggtcactggatctatggcttctccatcaaagatagtgttcatctggatagtttccaccacgacgtctctctctgcagtcttcgtttctcctttctttgtcagaggttccttgttcttcccagtcttgcaggggcagtgtctgtggatggctttggccaataggacgaccaggtacacgaggagacccagaagcaatatggagcccaaagtgatgacaaacggcacgtaccatgcagatggagagtaaacgtttttcctcaggacctgataggtgaccctgggcctgggggtcgtggtgatgatagtggttgggtggggaatgactttaatactcagtgtcactgttcctgtctcaacaagagcctccgctttcttcctgtcagacatcaagttgtcatcagttacgtagacaagtagcttgtagtcccagatcttatcaaacccaccagcatagtcaaagcgagatgtaagcagcaggcgtgtgacattggaaccagcattgggagagaaggtgaaatgattgttgacgttacctgggccaatggaataacggaaagatctggggctggaatcaaggtcggtacatgtcagcttgaaattctgaatatttgtgccaactttcagatccactgggagggccaggaaataagagtttggagtacaaattggcttttcatcattttcttcaaggatgttcacagtaacagtgacagagcttgtgtcttcgttgttggtggcctggattctgagaatatagatgggggttgtttcacagtccactttagttaccagctggagttctcctgtcttgggattaatccaaaatacatttggatactggaggctggcccctccagtggagatggagtacaggaggctgctctgggggaggtctttatcagtggctcgcacctgtcccactcgggttctggcgggccttctttctgacacatcaaatacataggatggcctatcaaaaatgagaggaaactcattttctgggcttgttaggatataaacgtagacgttatttttatagtaagggggggccacatcctgcacctggattatcaccgtatatttattgccggctgctaggttacttggattttcgtagtctagatcaccaatcagcacaatcttcccagagccagctggatcctgtaaaaatctgctgccgctccccactccagatggcatggtgaagttgaatctgttgtttggtgcctcactgtcatcatcaaagcagaacttgtttaggtcaagaagcaacgtccccttggctgttctttccggcaccataatgctgaaggtgaacttttggcatgtggcaggattgtcgttgacgtcttccacaatgaaggttatctggatgcgattctcctgacccccatatggtctgtccttcactagaacttccagggaaatggtgggattttgtctcaattcacctgcatctcggtctatcctttgggccacttggattgtaccagtcaactgatttatcatgaaatatttgctaacagtggtaatgctgtagaggaggtggctgggaaaaccttcatcatcaggatcctccgctgtgatattggccacgatggttcctggactcagttcctccaggactgtgtacactcgtgtcgggcttctgccaagttgccttgaaactgaggtggctcgttcacatctgttacctggacagtcaggacttgcaggtctgtgacaccaacctcatccttcacataaatctgcaaatcaaatatgtttggtcctgtttcaaaatctagttgttccatcccagtggtgacaacctcaaagtaggtgcctgacagccaattcaccctaaaagcttcagtgaggggatttgagttgactatctggggaaatcctgggatcacaggtgacaatgatgctgataacttcacagaaaacttgtgcactgaagtcccaggtggagaattctctgccacattgcctgtagcaggtaagaggattaggtgtagtgcttctccccctgcgtttcagaacgacatctacccactggtttcagctcctagagcaacaactgcagaatctccatggtccaaagtcctccaggaaagagaagaaaggggtgacgggggtgagggctgggaggcgaggtcaccagggtcccttccctggctcgggtgggggtggggggcgcaacccctcacggctcctccccaccaagccgtcgggaccccagcgggggcgcctcgcgttgggcgacagggacgcggggagagagcgacaagctggaagcaagggctgcctgcaaaactttcggtcctccagcggcaactctgcgggaaagaccacccttccttcggccccgcgtcgggcctatccccgtgtgccccgacccctgcgccccaggcttgggcggcgccgctgcatcccggctgccgggcgcgctgcagccttcgctctcccgcacgcggcgctcgcccgtccgcgctgcccctccccggcaggcgggcggccccggcgggcgggcgggc

SEQ ID NO: 14789 - RNA, 4884 nt, Homo sapiens
  source 1..4884: mol_type = other RNA
gctgggattacaggcatgagccacctcacccggcccttttaatcattcttaatgggcttataagcagttattaagtcccccttcagccttctcagaacctcattttacttgcattgaagctgagagcttccaaggaaagcatttgactccgggccccacagatttgcaatgccttaaatgggcaatcagccacttcactcactttaacctgcataaatgaacagttctgccttcttttgcaaagtttaaatccattcaagggagttccctggcaaccaacccttattaataaatcacgctcaatctaggccaggacaggcattttgcaaatgcttcttttgcttgagaagtgacactggcactaggcacacagtaaacaagctgctgctctctctgaagctctacatttgctggatccagtctgtctcccacaggaccttgtggacctggtaggctctcacctgactccccagttgggaagggagtgcttccctaatgaacactcacctggacctttcttagggttactggactagggtcgcagcagctgggcagcagggcatagagctcgagtgaagcttgctcaggctctgctaggcacacattggaaagttacatttcctattccatcataataccatttattcccagttcattgctcatgcctacaggtggaagtctgagttttatgtctagatggggcttccagtatgtccccactcagagtcctgcagttccttccaatcataggaagtgggaaggagcaaggcaggtaggttgtaaggctgatggtgtttcagctttgaggaaaaagtgatttcacttcaatagtaattttaaccagaatggctaaagttaaaaggattgacaatcccaagtgttggcaaggatagagagcaattgcaactctcagtgtttgctgctggaatgtgaatcagagccaccactttggaactctttggcagatccagcaattgctccagcaatcccactcttagatatatgagcaaaaaagtgagtgtttatgttcaccaaaagacatgtacaagaaagttcatagtgttgtaattcacttttattttttttttctgagatggagtcttgctttgtcacccaggctagagtgcagtggcacaatctcaactcactgtaacctccacctctcaggtttaagcagttctccctacctcagcctcccaagtagctgggattacatgtgcccaccaccacaccaagctaatttttgtattttttagtagagacagggttttgccatctaggccaggctgatcttgaactcctgaccttaggtgatctgcccaccttggcaaagtgctggcattacaggcatgagccatcatgccctgcctgtagttcacttttaagtatattttttaaaagtaaaaaatctgaagcagctgccacccaagtgtagaatagataaattgtgatataatcatagaatgaaaccagacataaccatgaagagaactgaactactgctagacaggacaacgtggatgaatctcacatgcaggatgctgatccggacaccacaagaaaaaacaaaagaaggtgcctactgagttttcttctttccagatgaccaactcttaacttactcatctgtttttttcactgttctgcttcttttgaagaagatttgaggtgacttacaaaggtgtatggcatatttataactgaagaaatctgggtgatgttaaaacgagggcaggaaaataaggtggaaaccagatgtaaggatagtcttcactatttatgtcaggaattcctacaaactttctatggtgaacagaatagagcttcctagcagtcaatgcaaagaagaaacacaacaattccacaccccaaagttaacagtcttgcttatcagaagcacaggtagttctgaaatctgatagaaaatgttcctgtatcatttcagaacacgcaactatgtgatcaaacccctttctatttgtttaaaaatttgtcaaacatcccatgtttgaccctggatgtctgaatcccctcagcccacattttcccccctacaccatgcccacaccatccccatagaatttagggtgaggcagcatctcagtgattgacaggcccctccttagaccccgtttactttcctgggtgtggtttggggtaagccctgttcatgaaggctggatttctgttctttgggttgcccagcttgccaccctcatttctggaacccagaccagcatcctcagcccacgctttgccactcagctcatcttcttcccagttggcacttctcagtgaccccatcccttccccagcagtgactctgcgtggggcagctccctggtggctggactctttccattttggcatttgggttagtggatctttccactttctggctccagtttttgagttgaattcatatgtttccccggtcactggatctatggcttctccatcaaagatagtgttcatctggatagtttccaccacgacgtctctctctgcagtcttcgtttctcctttctttgtcagaggttccttgttcttcccagtcttgcaggggcagtgtctgtggatggctttggccaataggacgaccaggtacacgaggagacccagaagcaatatggagcccaaagtgatgacaaacggcacgtaccatgcagatggagagtaaacgtttttcctcaggacctgataggtgaccctgggcctgggggtcgtggtgatgatagtggttgggtggggaatgactttaatactcagtgtcactgttcctgtctcaacaagagcctccgctttcttcctgtcagacatcaagttgtcatcagttacgtagacaagtagcttgtagtcccagatcttatcaaacccaccagcatagtcaaagcgagatgtaagcagcaggcgtgtgacattggaaccagcattgggagagaaggtgaaatgattgttgacgttacctgggccaatggaataacggaaagatctggggctggaatcaaggtcggtacatgtcagcttgaaattctgaatatttgtgccaactttcagatccactgggagggccaggaaataagagtttggagtacaaattggcttttcatcattttcttcaaggatgttcacagtaacagtgacagagcttgtgtcttcgttgttggtggcctggattctgagaatatagatgggggttgtttcacagtccactttagttaccagctggagttctcctgtcttgggattaatccaaaatacatttggatactggaggctggcccctccagtggagatggagtacaggaggctgctctgggggaggtctttatcagtggctcgcacctgtcccactcgggttctggctggaggaataaagtaccgggccttctttctgacacatcaaatacataggatggcctatcaaaaatgagaggaaactcattttctgggcttgttaggatataaacgtagacgttatttttatagtaagggggggccacatcctgcacctggattatcaccgtatatttattgccggctgctaggttacttggattttcgtagtctagatcaccaatcagcacaatcttcccagagccagctggatcctgtaaaaatctgctgccgctccccactccagatggcatggtgaagttgaatctgttgtttggtgcctcactgtcatcatcaaagcagaacttgtttaggtcaagaagcaacgtccccttggctgttctttccggcaccataatgctgaaggtgaacttttggcatgtggcaggattgtcgttgacgtcttccacaatgaaggttatctggatgcgattctcctgacccccatatggtctgtccttcactagaacttccagggaaatggtgggattttgtctcaattcacctgcatctcggtctatcctttgggccacttggattgtaccagtcaactgatttatcatgaaatatttgctaacagtggtaatgctgtagaggaggtggctgggaaaaccttcatcatcaggatcctccgctgtgatattggccacgatggttcctggactcagttcctccaggactgtgtacactcgtgtcgggctggtaaagcgagggacttcgtcgttgaggttcacgatgttcacctggagctctgtggaggctttgaggcctccactgtccctcacctccacgatgagatggaaacttctgtgtcctgcttcaaagtccaattctgttgtggagaagagggtgccattagcagacattctgaagctctttgggggagaaatcaggaaataactgaggggaatgtttcggcttgtgtcttctggatcgaaggcctcaacctggtaaatgaatccagggtttgctctttctactatgtagaggtgtagaccttctgccaagttgccttgaaactgaggtggctcgttcacatctgttacctggacagtcaggacttgcaggtctgtgacaccaacctcatccttcacataaatctgcaaatcaaatatgtttggtcctgtttcaaaatctagttgttccatcccagtggtgacaacctcaaagtaggtgcctgacagccaattcaccctaaaagcttcagtgaggggatttgagttgactatctggggaaatcctgggatcacaggtgacaatgatgctgataacttcacagaaaacttgtgcactgaagtcccaggtggagaattctctgccacattgcctgtagcaggtaagaggattaggtgtagtgcttctccccctgacatggcacccaggagagccaggagaatgattgcttcctgcatacttgatggtcacaactgtgcgtgcttccagcacattagccacagcctgaatcccgtctcacacccaaagtttatt

SEQ ID NO: 14790 - RNA, 4640 nt, Homo sapiens
  source 1..4640: mol_type = other RNA
gctgggattacaggcatgagccacctcacccggcccttttaatcattcttaatgggcttataagcagttattaagtcccccttcagccttctcagaacctcattttacttgcattgaagctgagagcttccaaggaaagcatttgactccgggccccacagatttgcaatgccttaaatgggcaatcagccacttcactcactttaacctgcataaatgaacagttctgccttcttttgcaaagtttaaatccattcaagggagttccctggcaaccaacccttattaataaatcacgctcaatctaggccaggacaggcattttgcaaatgcttcttttgcttgagaagtgacactggcactaggcacacagtaaacaagctgctgctctctctgaagctctacatttgctggatccagtctgtctcccacaggaccttgtggacctggtaggctctcacctgactccccagttgggaagggagtgcttccctaatgaacactcacctggacctttcttagggttactggactagggtcgcagcagctgggcagcagggcatagagctcgagtgaagcttgctcaggctctgctaggcacacattggaaagttacatttcctattccatcataataccatttattcccagttcattgctcatgcctacaggtggaagtctgagttttatgtctagatggggcttccagtatgtccccactcagagtcctgcagttccttccaatcataggaagtgggaaggagcaaggcaggtaggttgtaaggctgatggtgtttcagctttgaggaaaaagtgatttcacttcaatagtaattttaaccagaatggctaaagttaaaaggattgacaatcccaagtgttggcaaggatagagagcaattgcaactctcagtgtttgctgctggaatgtgaatcagagccaccactttggaactctttggcagatccagcaattgctccagcaatcccactcttagatatatgagcaaaaaagtgagtgtttatgttcaccaaaagacatgtacaagaaagttcatagtgttgtaattcacttttattttttttttctgagatggagtcttgctttgtcacccaggctagagtgcagtggcacaatctcaactcactgtaacctccacctctcaggtttaagcagttctccctacctcagcctcccaagtagctgggattacatgtgcccaccaccacaccaagctaatttttgtattttttagtagagacagggttttgccatctaggccaggctgatcttgaactcctgaccttaggtgatctgcccaccttggcaaagtgctggcattacaggcatgagccatcatgccctgcctgtagttcacttttaagtatattttttaaaagtaaaaaatctgaagcagctgccacccaagtgtagaatagataaattgtgatataatcatagaatgaaaccagacataaccatgaagagaactgaactactgctagacaggacaacgtggatgaatctcacatgcaggatgctgatccggacaccacaagaaaaaacaaaagaaggtgcctactgagttttcttctttccagatgaccaactcttaacttactcatctgtttttttcactgttctgcttcttttgaagaagatttgaggtgacttacaaaggtgtatggcatatttataactgaagaaatctgggtgatgttaaaacgagggcaggaaaataaggtggaaaccagatgtaaggatagtcttcactatttatgtcaggaattcctacaaactttctatggtgaacagaatagagcttcctagcagtcaatgcaaagaagaaacacaacaattccacaccccaaagttaacagtcttgcttatcagaagcacaggtagttctgaaatctgatagaaaatgttcctgtatcatttcagaacacgcaactatgtgatcaaacccctttctatttgtttaaaaatttgtcaaacatcccatgtttgaccctggatgtctgaatcccctcagcccacattttcccccctacaccatgcccacaccatccccatagaatttagggtgaggcagcatctcagtgattgacaggcccctccttagaccccgtttactttcctgggtgtggtttggggtaagccctgttcatgaaggctggatttctgttctttgggttgcccagcttgccaccctcatttctggaacccagaccagcatcctcagcccacgctttgccactcagctcatcttcttcccagttggcacttctcagtgaccccatcccttccccagcagtgactctgcgtggggcagctccctggtggctggactctttccattttggcatttgggttagtggatctttccactttctggctccagtttttgagttgaattcatatgtttccccggtcactggatctatggcttctccatcaaagatagtgttcatctggatagtttccaccacgacgtctctctctgcagtcttcgtttctcctttctttgtcagaggttccttgttcttcccagtcttgcaggggcagtgtctgtggatggctttggccaataggacgaccaggtacacgaggagacccagaagcaatatggagcccaaagtgatgacaaacggcacgtaccatgcagatggagagtaaacgtttttcctcaggacctgataggtgaccctgggcctgggggtcgtggtgatgatagtggttgggtggggaatgactttaatactcagtgtcactgttcctgtctcaacaagagcctccgctttcttcctgtcagacatcaagttgtcatcagttacgtagacaagtagcttgtagtcccagatcttatcaaacccaccagcatagtcaaagcgagatgtaagcagcaggcgtgtgacattggaaccagcattgggagagaaggtgaaatgattgttgacgttacctgggccaatggaataacggaaagatctggggctggaatcaaggtcggtacatgtcagcttgaaattctgaatatttgtgccaactttcagatccactgggagggccaggaaataagagtttggagtacaaattggcttttcatcattttcttcaaggatgttcacagtaaccgggccttctttctgacacatcaaatacataggatggcctatcaaaaatgagaggaaactcattttctgggcttgttaggatataaacgtagacgttatttttatagtaagggggggccacatcctgcacctggattatcaccgtatatttattgccggctgctaggttacttggattttcgtagtctagatcaccaatcagcacaatcttcccagagccagctggatcctgtaaaaatctgctgccgctccccactccagatggcatggtgaagttgaatctgttgtttggtgcctcactgtcatcatcaaagcagaacttgtttaggtcaagaagcaacgtccccttggctgttctttccggcaccataatgctgaaggtgaacttttggcatgtggcaggattgtcgttgacgtcttccacaatgaaggttatctggatgcgattctcctgacccccatatggtctgtccttcactagaacttccagggaaatggtgggattttgtctcaattcacctgcatctcggtctatcctttgggccacttggattgtaccagtcaactgatttatcatgaaatatttgctaacagtggtaatgctgtagaggaggtggctgggaaaaccttcatcatcaggatcctccgctgtgatattggccacgatggttcctggactcagttcctccaggactgtgtacactcgtgtcgggctggtaaagcgagggacttcgtcgttgaggttcacgatgttcacctggagctctgtggaggctttgaggcctccactgtccctcacctccacgatgagatggaaacttctgtgtcctgcttcaaagtccaattctgttgtggagaagagggtgccattagcagacattctgaagctctttgggggagaaatcaggaaataactgaggggaatgtttcggcttgtgtcttctggatcgaaggcctcaacctggtaaatgaatccagggtttgctctttctactatgtagaggtgtagaccttctgccaagttgccttgaaactgaggtggctcgttcacatctgttacctggacagtcaggacttgcaggtctgtgacaccaacctcatccttcacataaatctgcaaatcaaatatgtttggtcctgtttcaaaatctagttgttccatcccagtggtgacaacctcaaagtaggtgcctgacagccaattcaccctaaaagcttcagtgaggggatttgagttgactatctggggaaatcctgggatcacaggtgacaatgatgctgataacttcacagaaaacttgtgcactgaagtcccaggtggagaattctctgccacattgcctgtagcaggtaagaggattaggtgtagtgcttctccccctgacatggcacccaggagagccaggagaatgattgcttcctgcatacttgatggtcacaactgtgcgtgcttccagcacattagccacagcctgaatcccgtctcacacccaaagtttatt

SEQ ID NO: 14791 - RNA, 4968 nt, Homo sapiens
  source 1..4968: mol_type = other RNA
gctgggattacaggcatgagccacctcacccggcccttttaatcattcttaatgggcttataagcagttattaagtcccccttcagccttctcagaacctcattttacttgcattgaagctgagagcttccaaggaaagcatttgactccgggccccacagatttgcaatgccttaaatgggcaatcagccacttcactcactttaacctgcataaatgaacagttctgccttcttttgcaaagtttaaatccattcaagggagttccctggcaaccaacccttattaataaatcacgctcaatctaggccaggacaggcattttgcaaatgcttcttttgcttgagaagtgacactggcactaggcacacagtaaacaagctgctgctctctctgaagctctacatttgctggatccagtctgtctcccacaggaccttgtggacctggtaggctctcacctgactccccagttgggaagggagtgcttccctaatgaacactcacctggacctttcttagggttactggactagggtcgcagcagctgggcagcagggcatagagctcgagtgaagcttgctcaggctctgctaggcacacattggaaagttacatttcctattccatcataataccatttattcccagttcattgctcatgcctacaggtggaagtctgagttttatgtctagatggggcttccagtatgtccccactcagagtcctgcagttccttccaatcataggaagtgggaaggagcaaggcaggtaggttgtaaggctgatggtgtttcagctttgaggaaaaagtgatttcacttcaatagtaattttaaccagaatggctaaagttaaaaggattgacaatcccaagtgttggcaaggatagagagcaattgcaactctcagtgtttgctgctggaatgtgaatcagagccaccactttggaactctttggcagatccagcaattgctccagcaatcccactcttagatatatgagcaaaaaagtgagtgtttatgttcaccaaaagacatgtacaagaaagttcatagtgttgtaattcacttttattttttttttctgagatggagtcttgctttgtcacccaggctagagtgcagtggcacaatctcaactcactgtaacctccacctctcaggtttaagcagttctccctacctcagcctcccaagtagctgggattacatgtgcccaccaccacaccaagctaatttttgtattttttagtagagacagggttttgccatctaggccaggctgatcttgaactcctgaccttaggtgatctgcccaccttggcaaagtgctggcattacaggcatgagccatcatgccctgcctgtagttcacttttaagtatattttttaaaagtaaaaaatctgaagcagctgccacccaagtgtagaatagataaattgtgatataatcatagaatgaaaccagacataaccatgaagagaactgaactactgctagacaggacaacgtggatgaatctcacatgcaggatgctgatccggacaccacaagaaaaaacaaaagaaggtgcctactgagttttcttctttccagatgaccaactcttaacttactcatctgtttttttcactgttctgcttcttttgaagaagatttgaggtgacttacaaaggtgtatggcatatttataactgaagaaatctgggtgatgttaaaacgagggcaggaaaataaggtggaaaccagatgtaaggatagtcttcactatttatgtcaggaattcctacaaactttctatggtgaacagaatagagcttcctagcagtcaatgcaaagaagaaacacaacaattccacaccccaaagttaacagtcttgcttatcagaagcacaggtagttctgaaatctgatagaaaatgttcctgtatcatttcagaacacgcaactatgtgatcaaacccctttctatttgtttaaaaatttgtcaaacatcccatgtttgaccctggatgtctgaatcccctcagcccacattttcccccctacaccatgcccacaccatccccatagaatttagggtgaggcagcatctcagtgattgacaggcccctccttagaccccgtttactttcctgggtgtggtttggggtaagccctgttcatgaaggctggatttctgttctttgggttgcccagcttgccaccctcatttctggaacccagaccagcatcctcagcccacgctttgccactcagctcatcttcttcccagttggcacttctcagtgaccccatcccttccccagcagtgactctgcgtggggcagctccctggtggctggactctttccattttggcatttgggttagtggatctttccactttctggctccagtttttgagttgaattcatatgtttccccggtcactggatctatggcttctccatcaaagatagtgttcatctggatagtttccaccacgacgtctctctctgcagtcttcgtttctcctttctttgtcagaggttccttgttcttcccagtcttgcaggggcagtgtctgtggatggctttggccaataggacgaccaggtacacgaggagacccagaagcaatatggagcccaaagtgatgacaaacggcacgtaccatgcagatggagagtaaacgtttttcctcaggacctgataggtgaccctgggcctgggggtcgtggtgatgatagtggttgggtggggaatgactttaatactcagtgtcactgttcctgtctcaacaagagcctccgctttcttcctgtcagacatcaagttgtcatcagttacgtagacaagtagcttgtagtcccagatcttatcaaacccaccagcatagtcaaagcgagatgtaagcagcaggcgtgtgacattggaaccagcattgggagagaaggtgaaatgattgttgacgttacctgggccaatggaataacggaaagatctggggctggaatcaaggtcggtacatgtcagcttgaaattctgaatatttgtgccaactttcagatccactgggagggccaggaaataagagtttggagtacaaattggcttttcatcattttcttcaaggatgttcacagtaacctgcagatgacaccgagttgtttttccaggaaggtgtggatttacggtgtctccatgtgccaccttgcctgctgccccttgtaaatggaacttctttaactagtgacagagcttgtgtcttcgttgttggtggcctggattctgagaatatagatgggggttgtttcacagtccactttagttaccagctggagttctcctgtcttgggattaatccaaaatacatttggatactggaggctggcccctccagtggagatggagtacaggaggctgctctgggggaggtctttatcagtggctcgcacctgtcccactcgggttctggcgggccttctttctgacacatcaaatacataggatggcctatcaaaaatgagaggaaactcattttctgggcttgttaggatataaacgtagacgttatttttatagtaagggggggccacatcctgcacctggattatcaccgtatatttattgccggctgctaggttacttggattttcgtagtctagatcaccaatcagcacaatcttcccagagccagctggatcctgtaaaaatctgctgccgctccccactccagatggcatggtgaagttgaatctgttgtttggtgcctcactgtcatcatcaaagcagaacttgtttaggtcaagaagcaacgtccccttggctgttctttccggcaccataatgctgaaggtgaacttttggcatgtggcaggattgtcgttgacgtcttccacaatgaaggttatctggatgcgattctcctgacccccatatggtctgtccttcactagaacttccagggaaatggtgggattttgtctcaattcacctgcatctcggtctatcctttgggccacttggattgtaccagtcaactgatttatcatgaaatatttgctaacagtggtaatgctgtagaggaggtggctgggaaaaccttcatcatcaggatcctccgctgtgatattggccacgatggttcctggactcagttcctccaggactgtgtacactcgtgtcgggctggtaaagcgagggacttcgtcgttgaggttcacgatgttcacctggagctctgtggaggctttgaggcctccactgtccctcacctccacgatgagatggaaacttctgtgtcctgcttcaaagtccaattctgttgtggagaagagggtgccattagcagacattctgaagctctttgggggagaaatcaggaaataactgaggggaatgtttcggcttgtgtcttctggatcgaaggcctcaacctggtaaatgaatccagggtttgctctttctactatgtagaggtgtagaccttctgccaagttgccttgaaactgaggtggctcgttcacatctgttacctggacagtcaggacttgcaggtctgtgacaccaacctcatccttcacataaatctgcaaatcaaatatgtttggtcctgtttcaaaatctagttgttccatcccagtggtgacaacctcaaagtaggtgcctgacagccaattcaccctaaaagcttcagtgaggggatttgagttgactatctggggaaatcctgggatcacaggtgacaatgatgctgataacttcacagaaaacttgtgcactgaagtcccaggtggagaattctctgccacattgcctgtagcaggtaagaggattaggtgtagtgcttctccccctgacatggcacccaggagagccaggagaatgattgcttcctgcatacttgatggtcacaactgtgcgtgcttccagcacattagccacagcctgaatcccgtctcacacccaaagtttatt

SEQ ID NO: 14792 - RNA, 4217 nt, Homo sapiens
  source 1..4217: mol_type = other RNA
gctgggattacaggcatgagccacctcacccggcccttttaatcattcttaatgggcttataagcagttattaagtcccccttcagccttctcagaacctcattttacttgcattgaagctgagagcttccaaggaaagcatttgactccgggccccacagatttgcaatgccttaaatgggcaatcagccacttcactcactttaacctgcataaatgaacagttctgccttcttttgcaaagtttaaatccattcaagggagttccctggcaaccaacccttattaataaatcacgctcaatctaggccaggacaggcattttgcaaatgcttcttttgcttgagaagtgacactggcactaggcacacagtaaacaagctgctgctctctctgaagctctacatttgctggatccagtctgtctcccacaggaccttgtggacctggtaggctctcacctgactccccagttgggaagggagtgcttccctaatgaacactcacctggacctttcttagggttactggactagggtcgcagcagctgggcagcagggcatagagctcgagtgaagcttgctcaggctctgctaggcacacattggaaagttacatttcctattccatcataataccatttattcccagttcattgctcatgcctacaggtggaagtctgagttttatgtctagatggggcttccagtatgtccccactcagagtcctgcagttccttccaatcataggaagtgggaaggagcaaggcaggtaggttgtaaggctgatggtgtttcagctttgaggaaaaagtgatttcacttcaatagtaattttaaccagaatggctaaagttaaaaggattgacaatcccaagtgttggcaaggatagagagcaattgcaactctcagtgtttgctgctggaatgtgaatcagagccaccactttggaactctttggcagatccagcaattgctccagcaatcccactcttagatatatgagcaaaaaagtgagtgtttatgttcaccaaaagacatgtacaagaaagttcatagtgttgtaattcacttttattttttttttctgagatggagtcttgctttgtcacccaggctagagtgcagtggcacaatctcaactcactgtaacctccacctctcaggtttaagcagttctccctacctcagcctcccaagtagctgggattacatgtgcccaccaccacaccaagctaatttttgtattttttagtagagacagggttttgccatctaggccaggctgatcttgaactcctgaccttaggtgatctgcccaccttggcaaagtgctggcattacaggcatgagccatcatgccctgcctgtagttcacttttaagtatattttttaaaagtaaaaaatctgaagcagctgccacccaagtgtagaatagataaattgtgatataatcatagaatgaaaccagacataaccatgaagagaactgaactactgctagacaggacaacgtggatgaatctcacatgcaggatgctgatccggacaccacaagaaaaaacaaaagaaggtgcctactgagttttcttctttccagatgaccaactcttaacttactcatctgtttttttcactgttctgcttcttttgaagaagatttgaggtgacttacaaaggtgtatggcatatttataactgaagaaatctgggtgatgttaaaacgagggcaggaaaataaggtggaaaccagatgtaaggatagtcttcactatttatgtcaggaattcctacaaactttctatggtgaacagaatagagcttcctagcagtcaatgcaaagaagaaacacaacaattccacaccccaaagttaacagtcttgcttatcagaagcacaggtagttctgaaatctgatagaaaatgttcctgtatcatttcagaacacgcaactatgtgatcaaacccctttctatttgtttaaaaatttgtcaaacatcccatgtttgaccctggatgtctgaatcccctcagcccacattttcccccctacaccatgcccacaccatccccatagaatttagggtgaggcagcatctcagtgattgacaggcccctccttagaccccgtttactttcctgggtgtggtttggggtaagccctgttcatgaaggctggatttctgttctttgggttgcccagcttgccaccctcatttctggaacccagaccagcatcctcagcccacgctttgccactcagctcatcttcttcccagttggcacttctcagtgaccccatcccttccccagcagtgactctgcgtggggcagctccctggtggctggactctttccattttggcatttgggttagtggatctttccactttctggctccagtttttgagttgaattcatatgtttccccggtcactggatctatggcttctccatcaaagatagtgttcatctggatagtttccaccacgacgtctctctctgcagtcttcgtttctcctttctttgtcagaggttccttgttcttcccagtcttgcaggggcagtgtctgtggatggctttggccaataggacgaccaggtacacgaggagacccagaagcaatatggagcccaaagtgatgacaaacggcacgtaccatgcagatggagagtaaacgtttttcctcaggacctgataggtgaccctgggcgggccttctttctgacacatcaaatacataggatggcctatcaaaaatgagaggaaactcattttctgggcttgttaggatataaacgtagacgttatttttatagtaagggggggccacatcctgcacctggattatcaccgtatatttattgccggctgctaggttacttggattttcgtagtctagatcaccaatcagcacaatcttcccagagccagctggatcctgtaaaaatctgctgccgctccccactccagatggcatggtgaagttgaatctgttgtttggtgcctcactgtcatcatcaaagcagaacttgtttaggtcaagaagcaacgtccccttggctgttctttccggcaccataatgctgaaggtgaacttttggcatgtggcaggattgtcgttgacgtcttccacaatgaaggttatctggatgcgattctcctgacccccatatggtctgtccttcactagaacttccagggaaatggtgggattttgtctcaattcacctgcatctcggtctatcctttgggccacttggattgtaccagtcaactgatttatcatgaaatatttgctaacagtggtaatgctgtagaggaggtggctgggaaaaccttcatcatcaggatcctccgctgtgatattggccacgatggttcctggactcagttcctccaggactgtgtacactcgtgtcgggctggtaaagcgagggacttcgtcgttgaggttcacgatgttcacctggagctctgtggaggctttgaggcctccactgtccctcacctccacgatgagatggaaacttctgtgtcctgcttcaaagtccaattctgttgtggagaagagggtgccattagcagacattctgaagctctttgggggagaaatcaggaaataactgaggggaatgtttcggcttgtgtcttctggatcgaaggcctcaacctggtaaatgaatccagggtttgctctttctactatgtagaggtgtagaccttctgccaagttgccttgaaactgaggtggctcgttcacatctgttacctggacagtcaggacttgcaggtctgtgacaccaacctcatccttcacataaatctgcaaatcaaatatgtttggtcctgtttcaaaatctagttgttccatcccagtggtgacaacctcaaagtaggtgcctgacagccaattcaccctaaaagcttcagtgaggggatttgagttgactatctggggaaatcctgggatcacaggtgacaatgatgctgataacttcacagaaaacttgtgcactgaagtcccaggtggagaattctctgccacattgcctgtagcaggtaagaggattaggtgtagtgcttctccccctgacatggcacccaggagagccaggagaatgattgcttcctgcatacttgatggtcacaactgtgcgtgcttccagcacattagccacagcctgaatcccgtctcacacccaaagtttatt

SEQ ID NO: 14793 - RNA, 4616 nt, Homo sapiens
  source 1..4616: mol_type = other RNA
gctgggattacaggcatgagccacctcacccggcccttttaatcattcttaatgggcttataagcagttattaagtcccccttcagccttctcagaacctcattttacttgcattgaagctgagagcttccaaggaaagcatttgactccgggccccacagatttgcaatgccttaaatgggcaatcagccacttcactcactttaacctgcataaatgaacagttctgccttcttttgcaaagtttaaatccattcaagggagttccctggcaaccaacccttattaataaatcacgctcaatctaggccaggacaggcattttgcaaatgcttcttttgcttgagaagtgacactggcactaggcacacagtaaacaagctgctgctctctctgaagctctacatttgctggatccagtctgtctcccacaggaccttgtggacctggtaggctctcacctgactccccagttgggaagggagtgcttccctaatgaacactcacctggacctttcttagggttactggactagggtcgcagcagctgggcagcagggcatagagctcgagtgaagcttgctcaggctctgctaggcacacattggaaagttacatttcctattccatcataataccatttattcccagttcattgctcatgcctacaggtggaagtctgagttttatgtctagatggggcttccagtatgtccccactcagagtcctgcagttccttccaatcataggaagtgggaaggagcaaggcaggtaggttgtaaggctgatggtgtttcagctttgaggaaaaagtgatttcacttcaatagtaattttaaccagaatggctaaagttaaaaggattgacaatcccaagtgttggcaaggatagagagcaattgcaactctcagtgtttgctgctggaatgtgaatcagagccaccactttggaactctttggcagatccagcaattgctccagcaatcccactcttagatatatgagcaaaaaagtgagtgtttatgttcaccaaaagacatgtacaagaaagttcatagtgttgtaattcacttttattttttttttctgagatggagtcttgctttgtcacccaggctagagtgcagtggcacaatctcaactcactgtaacctccacctctcaggtttaagcagttctccctacctcagcctcccaagtagctgggattacatgtgcccaccaccacaccaagctaatttttgtattttttagtagagacagggttttgccatctaggccaggctgatcttgaactcctgaccttaggtgatctgcccaccttggcaaagtgctggcattacaggcatgagccatcatgccctgcctgtagttcacttttaagtatattttttaaaagtaaaaaatctgaagcagctgccacccaagtgtagaatagataaattgtgatataatcatagaatgaaaccagacataaccatgaagagaactgaactactgctagacaggacaacgtggatgaatctcacatgcaggatgctgatccggacaccacaagaaaaaacaaaagaaggtgcctactgagttttcttctttccagatgaccaactcttaacttactcatctgtttttttcactgttctgcttcttttgaagaagatttgaggtgacttacaaaggtgtatggcatatttataactgaagaaatctgggtgatgttaaaacgagggcaggaaaataaggtggaaaccagatgtaaggatagtcttcactatttatgtcaggaattcctacaaactttctatggtgaacagaatagagcttcctagcagtcaatgcaaagaagaaacacaacaattccacaccccaaagttaacagtcttgcttatcagaagcacaggtagttctgaaatctgatagaaaatgttcctgtatcatttcagaacacgcaactatgtgatcaaacccctttctatttgtttaaaaatttgtcaaacatcccatgtttgaccctggatgtctgaatcccctcagcccacattttcccccctacaccatgcccacaccatccccatagaatttagggtgaggcagcatctcagtgattgacaggcccctccttagaccccgtttactttcctgggtgtggtttggggtaagccctgttcatgaaggctggatttctgttctttgggttgcccagcttgccaccctcatttctggaacccagaccagcatcctcagcccacgctttgccactcagctcatcttcttcccagttggcacttctcagtgaccccatcccttccccagcagtgactctgcgtggggcagctccctggtggctggactctttccattttggcatttgggttagtggatctttccactttctggctccagtttttgagttgaattcatatgtttccccggtcactggatctatggcttctccatcaaagatagtgttcatctggatagtttccaccacgacgtctctctctgcagtcttcgtttctcctttctttgtcagaggttccttgttcttcccagtcttgcaggggcagtgtctgtggatggctttggccaataggacgaccaggtacacgaggagacccagaagcaatatggagcccaaagtgatgacaaacggcacgtaccatgcagatggagagtaaacgtttttcctcaggacctgataggtgaccctgggctgggccaatggaataacggaaagatctggggctggaatcaaggtcggtacatgtcagcttgaaattctgaatatttgtgccaactttcagatccactgggagggccaggaaataagagtttggagtacaaattggcttttcatcattttcttcaaggatgttcacagtaacagtgacagagcttgtgtcttcgttgttggtggcctggattctgagaatatagatgggggttgtttcacagtccactttagttaccagctggagttctcctgtcttgggattaatccaaaatacatttggatactggaggctggcccctccagtggagatggagtacaggaggctgctctgggggaggtctttatcagtggctcgcacctgtcccactcgggttctggcgggccttctttctgacacatcaaatacataggatggcctatcaaaaatgagaggaaactcattttctgggcttgttaggatataaacgtagacgttatttttatagtaagggggggccacatcctgcacctggattatcaccgtatatttattgccggctgctaggttacttggattttcgtagtctagatcaccaatcagcacaatcttcccagagccagctggatcctgtaaaaatctgctgccgctccccactccagatggcatggtgaagttgaatctgttgtttggtgcctcactgtcatcatcaaagcagaacttgtttaggtcaagaagcaacgtccccttggctgttctttccggcaccataatgctgaaggtgaacttttggcatgtggcaggattgtcgttgacgtcttccacaatgaaggttatctggatgcgattctcctgacccccatatggtctgtccttcactagaacttccagggaaatggtgggattttgtctcaattcacctgcatctcggtctatcctttgggccacttggattgtaccagtcaactgatttatcatgaaatatttgctaacagtggtaatgctgtagaggaggtggctgggaaaaccttcatcatcaggatcctccgctgtgatattggccacgatggttcctggactcagttcctccaggactgtgtacactcgtgtcgggctggtaaagcgagggacttcgtcgttgaggttcacgatgttcacctggagctctgtggaggctttgaggcctccactgtccctcacctccacgatgagatggaaacttctgtgtcctgcttcaaagtccaattctgttgtggagaagagggtgccattagcagacattctgaagctctttgggggagaaatcaggaaataactgaggggaatgtttcggcttgtgtcttctggatcgaaggcctcaacctggtaaatgaatccagggtttgctctttctactatgtagaggtgtagaccttctgccaagttgccttgaaactgaggtggctcgttcacatctgttacctggacagtcaggacttgcaggtctgtgacaccaacctcatccttcacataaatctgcaaatcaaatatgtttggtcctgtttcaaaatctagttgttccatcccagtggtgacaacctcaaagtaggtgcctgacagccaattcaccctaaaagcttcagtgaggggatttgagttgactatctggggaaatcctgggatcacaggtgacaatgatgctgataacttcacagaaaacttgtgcactgaagtcccaggtggagaattctctgccacattgcctgtagcaggtaagaggattaggtgtagtgcttctccccctgacatggcacccaggagagccaggagaatgattgcttcctgcatacttgatggtcacaactgtgcgtgcttccagcacattagccacagcctgaatcccgtctcacacccaaagtttatt

SEQ ID NO: 14794 - RNA, 4633 nt, Homo sapiens
  source 1..4633: mol_type = other RNA
gctgggattacaggcatgagccacctcacccggcccttttaatcattcttaatgggcttataagcagttattaagtcccccttcagccttctcagaacctcattttacttgcattgaagctgagagcttccaaggaaagcatttgactccgggccccacagatttgcaatgccttaaatgggcaatcagccacttcactcactttaacctgcataaatgaacagttctgccttcttttgcaaagtttaaatccattcaagggagttccctggcaaccaacccttattaataaatcacgctcaatctaggccaggacaggcattttgcaaatgcttcttttgcttgagaagtgacactggcactaggcacacagtaaacaagctgctgctctctctgaagctctacatttgctggatccagtctgtctcccacaggaccttgtggacctggtaggctctcacctgactccccagttgggaagggagtgcttccctaatgaacactcacctggacctttcttagggttactggactagggtcgcagcagctgggcagcagggcatagagctcgagtgaagcttgctcaggctctgctaggcacacattggaaagttacatttcctattccatcataataccatttattcccagttcattgctcatgcctacaggtggaagtctgagttttatgtctagatggggcttccagtatgtccccactcagagtcctgcagttccttccaatcataggaagtgggaaggagcaaggcaggtaggttgtaaggctgatggtgtttcagctttgaggaaaaagtgatttcacttcaatagtaattttaaccagaatggctaaagttaaaaggattgacaatcccaagtgttggcaaggatagagagcaattgcaactctcagtgtttgctgctggaatgtgaatcagagccaccactttggaactctttggcagatccagcaattgctccagcaatcccactcttagatatatgagcaaaaaagtgagtgtttatgttcaccaaaagacatgtacaagaaagttcatagtgttgtaattcacttttattttttttttctgagatggagtcttgctttgtcacccaggctagagtgcagtggcacaatctcaactcactgtaacctccacctctcaggtttaagcagttctccctacctcagcctcccaagtagctgggattacatgtgcccaccaccacaccaagctaatttttgtattttttagtagagacagggttttgccatctaggccaggctgatcttgaactcctgaccttaggtgatctgcccaccttggcaaagtgctggcattacaggcatgagccatcatgccctgcctgtagttcacttttaagtatattttttaaaagtaaaaaatctgaagcagctgccacccaagtgtagaatagataaattgtgatataatcatagaatgaaaccagacataaccatgaagagaactgaactactgctagacaggacaacgtggatgaatctcacatgcaggatgctgatccggacaccacaagaaaaaacaaaagaaggtgcctactgagttttcttctttccagatgaccaactcttaacttactcatctgtttttttcactgttctgcttcttttgaagaagatttgaggtgacttacaaaggtgtatggcatatttataactgaagaaatctgggtgatgttaaaacgagggcaggaaaataaggtggaaaccagatgtaaggatagtcttcactatttatgtcaggaattcctacaaactttctatggtgaacagaatagagcttcctagcagtcaatgcaaagaagaaacacaacaattccacaccccaaagttaacagtcttgcttatcagaagcacaggtagttctgaaatctgatagaaaatgttcctgtatcatttcagaacacgcaactatgtgatcaaacccctttctatttgtttaaaaatttgtcaaacatcccatgtttgaccctggatgtctgaatcccctcagcccacattttcccccctacaccatgcccacaccatccccatagaatttagggtgaggcagcatctcagtgattgacaggcccctccttagaccccgtttactttcctgggtgtggtttggggtaagccctgttcatgaaggctggatttctgttctttgggttgcccagcttgccaccctcatttctggaacccagaccagcatcctcagcccacgctttgccactcagctcatcttcttcccagttggcacttctcagtgaccccatcccttccccagcagtgactctgcgtggggcagctccctggtggctggactctttccattttggcatttgggttagtggatctttccactttctggctccagtttttgagttgaattcatatgtttccccggtcactggatctatggcttctccatcaaagatagtgttcatctggatagtttccaccacgacgtctctctctgcagtcttcgtttctcctttctttgtcagaggttccttgttcttcccagtcttgcaggggcagtgtctgtggatggctttggccaataggacgaccaggtacacgaggagacccagaagcaatatggagcccaaagtgatgacaaacggcacgtaccatgcagatggagagtaaacgtttttcctcaggacctgataggtgaccctgggctgggccaatggaataacggaaagatctggggctggaatcaaggtcggtacatgtcagcttgaaattctgaatatttgtgccaactttcagatccactgggagggccaggaaataagagtttggagtacaaattggcttttcatcattttcttcaaggatgttcacagtaacagtgacagagcttgtgtcttcgttgttggtggcctggattctgagaatatagatgggggttgtttcacagtccactttagttaccagctggagttctcctgtcttgggattaatccaaaatacatttggatactggaggctggcccctccagtggagatggagtacaggaggctgctctgggggaggtctttatcagtggctcgcacctgtcccactcgggttctggctggaggaataaagtaccgggccttctttctgacacatcaaatacataggatggcctatcaaaaatgagaggaaactcattttctgggcttgttaggatataaacgtagacgttatttttatagtaagggggggccacatcctgcacctggattatcaccgtatatttattgccggctgctaggttacttggattttcgtagtctagatcaccaatcagcacaatcttcccagagccagctggatcctgtaaaaatctgctgccgctccccactccagatggcatggtgaagttgaatctgttgtttggtgcctcactgtcatcatcaaagcagaacttgtttaggtcaagaagcaacgtccccttggctgttctttccggcaccataatgctgaaggtgaacttttggcatgtggcaggattgtcgttgacgtcttccacaatgaaggttatctggatgcgattctcctgacccccatatggtctgtccttcactagaacttccagggaaatggtgggattttgtctcaattcacctgcatctcggtctatcctttgggccacttggattgtaccagtcaactgatttatcatgaaatatttgctaacagtggtaatgctgtagaggaggtggctgggaaaaccttcatcatcaggatcctccgctgtgatattggccacgatggttcctggactcagttcctccaggactgtgtacactcgtgtcgggctggtaaagcgagggacttcgtcgttgaggttcacgatgttcacctggagctctgtggaggctttgaggcctccactgtccctcacctccacgatgagatggaaacttctgtgtcctgcttcaaagtccaattctgttgtggagaagagggtgccattagcagacattctgaagctctttgggggagaaatcaggaaataactgaggggaatgtttcggcttgtgtcttctggatcgaaggcctcaacctggtaaatgaatccagggtttgctctttctactatgtagaggtgtagaccttctgccaagttgccttgaaactgaggtggctcgttcacatctgttacctggacagtcaggacttgcaggtctgtgacaccaacctcatccttcacataaatctgcaaatcaaatatgtttggtcctgtttcaaaatctagttgttccatcccagtggtgacaacctcaaagtaggtgcctgacagccaattcaccctaaaagcttcagtgaggggatttgagttgactatctggggaaatcctgggatcacaggtgacaatgatgctgataacttcacagaaaacttgtgcactgaagtcccaggtggagaattctctgccacattgcctgtagcaggtaagaggattaggtgtagtgcttctccccctgacatggcacccaggagagccaggagaatgattgcttcctgcatacttgatggtcacaactgtgcgtgcttccagcacattagccacagcctgaatcccgtctcacacccaaagtttatt

SEQ ID NO: 14795 - RNA, 4389 nt, Homo sapiens
  source 1..4389: mol_type = other RNA
gctgggattacaggcatgagccacctcacccggcccttttaatcattcttaatgggcttataagcagttattaagtcccccttcagccttctcagaacctcattttacttgcattgaagctgagagcttccaaggaaagcatttgactccgggccccacagatttgcaatgccttaaatgggcaatcagccacttcactcactttaacctgcataaatgaacagttctgccttcttttgcaaagtttaaatccattcaagggagttccctggcaaccaacccttattaataaatcacgctcaatctaggccaggacaggcattttgcaaatgcttcttttgcttgagaagtgacactggcactaggcacacagtaaacaagctgctgctctctctgaagctctacatttgctggatccagtctgtctcccacaggaccttgtggacctggtaggctctcacctgactccccagttgggaagggagtgcttccctaatgaacactcacctggacctttcttagggttactggactagggtcgcagcagctgggcagcagggcatagagctcgagtgaagcttgctcaggctctgctaggcacacattggaaagttacatttcctattccatcataataccatttattcccagttcattgctcatgcctacaggtggaagtctgagttttatgtctagatggggcttccagtatgtccccactcagagtcctgcagttccttccaatcataggaagtgggaaggagcaaggcaggtaggttgtaaggctgatggtgtttcagctttgaggaaaaagtgatttcacttcaatagtaattttaaccagaatggctaaagttaaaaggattgacaatcccaagtgttggcaaggatagagagcaattgcaactctcagtgtttgctgctggaatgtgaatcagagccaccactttggaactctttggcagatccagcaattgctccagcaatcccactcttagatatatgagcaaaaaagtgagtgtttatgttcaccaaaagacatgtacaagaaagttcatagtgttgtaattcacttttattttttttttctgagatggagtcttgctttgtcacccaggctagagtgcagtggcacaatctcaactcactgtaacctccacctctcaggtttaagcagttctccctacctcagcctcccaagtagctgggattacatgtgcccaccaccacaccaagctaatttttgtattttttagtagagacagggttttgccatctaggccaggctgatcttgaactcctgaccttaggtgatctgcccaccttggcaaagtgctggcattacaggcatgagccatcatgccctgcctgtagttcacttttaagtatattttttaaaagtaaaaaatctgaagcagctgccacccaagtgtagaatagataaattgtgatataatcatagaatgaaaccagacataaccatgaagagaactgaactactgctagacaggacaacgtggatgaatctcacatgcaggatgctgatccggacaccacaagaaaaaacaaaagaaggtgcctactgagttttcttctttccagatgaccaactcttaacttactcatctgtttttttcactgttctgcttcttttgaagaagatttgaggtgacttacaaaggtgtatggcatatttataactgaagaaatctgggtgatgttaaaacgagggcaggaaaataaggtggaaaccagatgtaaggatagtcttcactatttatgtcaggaattcctacaaactttctatggtgaacagaatagagcttcctagcagtcaatgcaaagaagaaacacaacaattccacaccccaaagttaacagtcttgcttatcagaagcacaggtagttctgaaatctgatagaaaatgttcctgtatcatttcagaacacgcaactatgtgatcaaacccctttctatttgtttaaaaatttgtcaaacatcccatgtttgaccctggatgtctgaatcccctcagcccacattttcccccctacaccatgcccacaccatccccatagaatttagggtgaggcagcatctcagtgattgacaggcccctccttagaccccgtttactttcctgggtgtggtttggggtaagccctgttcatgaaggctggatttctgttctttgggttgcccagcttgccaccctcatttctggaacccagaccagcatcctcagcccacgctttgccactcagctcatcttcttcccagttggcacttctcagtgaccccatcccttccccagcagtgactctgcgtggggcagctccctggtggctggactctttccattttggcatttgggttagtggatctttccactttctggctccagtttttgagttgaattcatatgtttccccggtcactggatctatggcttctccatcaaagatagtgttcatctggatagtttccaccacgacgtctctctctgcagtcttcgtttctcctttctttgtcagaggttccttgttcttcccagtcttgcaggggcagtgtctgtggatggctttggccaataggacgaccaggtacacgaggagacccagaagcaatatggagcccaaagtgatgacaaacggcacgtaccatgcagatggagagtaaacgtttttcctcaggacctgataggtgaccctgggctgggccaatggaataacggaaagatctggggctggaatcaaggtcggtacatgtcagcttgaaattctgaatatttgtgccaactttcagatccactgggagggccaggaaataagagtttggagtacaaattggcttttcatcattttcttcaaggatgttcacagtaaccgggccttctttctgacacatcaaatacataggatggcctatcaaaaatgagaggaaactcattttctgggcttgttaggatataaacgtagacgttatttttatagtaagggggggccacatcctgcacctggattatcaccgtatatttattgccggctgctaggttacttggattttcgtagtctagatcaccaatcagcacaatcttcccagagccagctggatcctgtaaaaatctgctgccgctccccactccagatggcatggtgaagttgaatctgttgtttggtgcctcactgtcatcatcaaagcagaacttgtttaggtcaagaagcaacgtccccttggctgttctttccggcaccataatgctgaaggtgaacttttggcatgtggcaggattgtcgttgacgtcttccacaatgaaggttatctggatgcgattctcctgacccccatatggtctgtccttcactagaacttccagggaaatggtgggattttgtctcaattcacctgcatctcggtctatcctttgggccacttggattgtaccagtcaactgatttatcatgaaatatttgctaacagtggtaatgctgtagaggaggtggctgggaaaaccttcatcatcaggatcctccgctgtgatattggccacgatggttcctggactcagttcctccaggactgtgtacactcgtgtcgggctggtaaagcgagggacttcgtcgttgaggttcacgatgttcacctggagctctgtggaggctttgaggcctccactgtccctcacctccacgatgagatggaaacttctgtgtcctgcttcaaagtccaattctgttgtggagaagagggtgccattagcagacattctgaagctctttgggggagaaatcaggaaataactgaggggaatgtttcggcttgtgtcttctggatcgaaggcctcaacctggtaaatgaatccagggtttgctctttctactatgtagaggtgtagaccttctgccaagttgccttgaaactgaggtggctcgttcacatctgttacctggacagtcaggacttgcaggtctgtgacaccaacctcatccttcacataaatctgcaaatcaaatatgtttggtcctgtttcaaaatctagttgttccatcccagtggtgacaacctcaaagtaggtgcctgacagccaattcaccctaaaagcttcagtgaggggatttgagttgactatctggggaaatcctgggatcacaggtgacaatgatgctgataacttcacagaaaacttgtgcactgaagtcccaggtggagaattctctgccacattgcctgtagcaggtaagaggattaggtgtagtgcttctccccctgacatggcacccaggagagccaggagaatgattgcttcctgcatacttgatggtcacaactgtgcgtgcttccagcacattagccacagcctgaatcccgtctcacacccaaagtttatt

SEQ ID NO: 14796 - RNA, 5077 nt, Homo sapiens
  source 1..5077: mol_type = other RNA
gctgggattacaggcatgagccacctcacccggcccttttaatcattcttaatgggcttataagcagttattaagtcccccttcagccttctcagaacctcattttacttgcattgaagctgagagcttccaaggaaagcatttgactccgggccccacagatttgcaatgccttaaatgggcaatcagccacttcactcactttaacctgcataaatgaacagttctgccttcttttgcaaagtttaaatccattcaagggagttccctggcaaccaacccttattaataaatcacgctcaatctaggccaggacaggcattttgcaaatgcttcttttgcttgagaagtgacactggcactaggcacacagtaaacaagctgctgctctctctgaagctctacatttgctggatccagtctgtctcccacaggaccttgtggacctggtaggctctcacctgactccccagttgggaagggagtgcttccctaatgaacactcacctggacctttcttagggttactggactagggtcgcagcagctgggcagcagggcatagagctcgagtgaagcttgctcaggctctgctaggcacacattggaaagttacatttcctattccatcataataccatttattcccagttcattgctcatgcctacaggtggaagtctgagttttatgtctagatggggcttccagtatgtccccactcagagtcctgcagttccttccaatcataggaagtgggaaggagcaaggcaggtaggttgtaaggctgatggtgtttcagctttgaggaaaaagtgatttcacttcaatagtaattttaaccagaatggctaaagttaaaaggattgacaatcccaagtgttggcaaggatagagagcaattgcaactctcagtgtttgctgctggaatgtgaatcagagccaccactttggaactctttggcagatccagcaattgctccagcaatcccactcttagatatatgagcaaaaaagtgagtgtttatgttcaccaaaagacatgtacaagaaagttcatagtgttgtaattcacttttattttttttttctgagatggagtcttgctttgtcacccaggctagagtgcagtggcacaatctcaactcactgtaacctccacctctcaggtttaagcagttctccctacctcagcctcccaagtagctgggattacatgtgcccaccaccacaccaagctaatttttgtattttttagtagagacagggttttgccatctaggccaggctgatcttgaactcctgaccttaggtgatctgcccaccttggcaaagtgctggcattacaggcatgagccatcatgccctgcctgtagttcacttttaagtatattttttaaaagtaaaaaatctgaagcagctgccacccaagtgtagaatagataaattgtgatataatcatagaatgaaaccagacataaccatgaagagaactgaactactgctagacaggacaacgtggatgaatctcacatgcaggatgctgatccggacaccacaagaaaaaacaaaagaaggtgcctactgagttttcttctttccagatgaccaactcttaacttactcatctgtttttttcactgttctgcttcttttgaagaagatttgaggtgacttacaaaggtgtatggcatatttataactgaagaaatctgggtgatgttaaaacgagggcaggaaaataaggtggaaaccagatgtaaggatagtcttcactatttatgtcaggaattcctacaaactttctatggtgaacagaatagagcttcctagcagtcaatgcaaagaagaaacacaacaattccacaccccaaagttaacagtcttgcttatcagaagcacaggtagttctgaaatctgatagaaaatgttcctgtatcatttcagaacacgcaactatgtgatcaaacccctttctatttgtttaaaaatttgtcaaacatcccatgtttgaccctggatgtctgaatcccctcagcccacattttcccccctacaccatgcccacaccatccccatagaatttagggtgaggcagcatctcagtgattgacaggcccctccttagaccccgtttactttcctgggtgtggtttggggtaagccctgttcatgaaggctggatttctgttctttgggttgcccagcttgccaccctcatttctggaacccagaccagcatcctcagcccacgctttgccactcagctcatcttcttcccagttggcacttctcagtgaccccatcccttccccagcagtgactctgcgtggggcagctccctggtggctggactctttccattttggcatttgggttagtggatctttccactttctggctccagtttttgagttgaattcatatgtttccccggtcactggatctatggcttctccatcaaagatagtgttcatctggatagtttccaccacgacgtctctctctgcagtcttcgtttctcctttctttgtcagaggttccttgttcttcccagtcttgcaggggcagtgtctgtggatggctttggccaataggacgaccaggtacacgaggagacccagaagcaatatggagcccaaagtgatgacaaacggcacgtaccatgcagatggagagtaaacgtttttcctcaggacctgataggtgaccctgggctgggccaatggaataacggaaagatctggggctggaatcaaggtcggtacatgtcagcttgaaattctgaatatttgtgccaactttcagatccactgggagggccaggaaataagagtttggagtacaaattggcttttcatcattttcttcaaggatgttcacagtaacctagagtagcaagaaggtggtcattctcaatagctaaaactcattgagtgcttactgtgtgtaggcagttttcaggctaagcacttttcataaattagctcatttaaactcacatgagatagctaacatgattattcccattttatggtgagaaaatggaagtttagagagactaggtaattgatctaagatcattcagctagtgaatggcagagttgggatttgaattcaggtctgtcctactccaaatcctatgctattaacttctacaccatatgcatgtgtgtgtgcacatttagtgtatgtataccttgccccccccccacacacacacacatgcacctggacacataggctcacctgcagatgacaccgagttgtttttccaggaaggtgtggatttacggtgtctccatgtgccaccttgcctgctgccccttgtaaatggaacttctttaactagtgacagagcttgtgtcttcgttgttggtggcctggattctgagaatatagatgggggttgtttcacagtccactttagttaccagctggagttctcctgtcttgggattaatccaaaatacatttggatactggaggctggcccctccagtggagatggagtacaggaggctgctctgggggaggtctttatcagtggctcgcacctgtcccactcgggttctggcgggccttctttctgacacatcaaatacataggatggcctatcaaaaatgagaggaaactcattttctgggcttgttaggatataaacgtagacgttatttttatagtaagggggggccacatcctgcacctggattatcaccgtatatttattgccggctgctaggttacttggattttcgtagtctagatcaccaatcagcacaatcttcccagagccagctggatcctgtaaaaatctgctgccgctccccactccagatggcatggtgaagttgaatctgttgtttggtgcctcactgtcatcatcaaagcagaacttgtttaggtcaagaagcaacgtccccttggctgttctttccggcaccataatgctgaaggtgaacttttggcatgtggcaggattgtcgttgacgtcttccacaatgaaggttatctggatgcgattctcctgacccccatatggtctgtccttcactagaacttccagggaaatggtgggattttgtctcaattcacctgcatctcggtctatcctttgggccacttggattgtaccagtcaactgatttatcatgaaatatttgctaacagtggtaatgctgtagaggaggtggctgggaaaaccttcatcatcaggatcctccgctgtgatattggccacgatggttcctggactcagttcctccaggactgtgtacactcgtgtcgggctggtaaagcgagggacttcgtcgttgaggttcacgatgttcacctggagctctgtggaggctttgaggcctccactgtccctcacctccacgatgagatggaaacttctgtgtcctgcttcaaagtccaattctgttgtggagaagagggtgccattagcagacattctgaagctctttgggggagaaatcaggaaataactgaggggaatgtttcggcttgtgtcttctggatcgaaggcctcaacctggtaaatgaatccagggtttgctctttctactatgtagaggtgtagaccttctgccaagttgccttgaaactgaggtggctcgttcacatctgttacctggacagtcaggacttgcaggtctgtgacaccaacctcatccttcacataaatctgcaaatcaaatatgtttggtcctgtttcaaaatctagttgttccatcccagtggtgacaacctcaaagtaggtgcctgacagccaattcaccctaaaagcttcagtgaggggatttgagttgactatctggggaaatcctgggatcacaggtgacaatgatgctgataacttcacagaaaacttgtgcactgaagtcccaggtggagaattctctgccacattgcctgtagcaggtaagaggattaggtgtagtgcttctccccctgacatggcacccaggagagccaggagaatgattgcttcctgcatacttgatggtcacaactgtgcgtgcttccagcacattagccacagcctgaatcccgtctcacacccaaagtttatt

SEQ ID NO: 14797 - RNA, 4717 nt, Homo sapiens
  source 1..4717: mol_type = other RNA
gctgggattacaggcatgagccacctcacccggcccttttaatcattcttaatgggcttataagcagttattaagtcccccttcagccttctcagaacctcattttacttgcattgaagctgagagcttccaaggaaagcatttgactccgggccccacagatttgcaatgccttaaatgggcaatcagccacttcactcactttaacctgcataaatgaacagttctgccttcttttgcaaagtttaaatccattcaagggagttccctggcaaccaacccttattaataaatcacgctcaatctaggccaggacaggcattttgcaaatgcttcttttgcttgagaagtgacactggcactaggcacacagtaaacaagctgctgctctctctgaagctctacatttgctggatccagtctgtctcccacaggaccttgtggacctggtaggctctcacctgactccccagttgggaagggagtgcttccctaatgaacactcacctggacctttcttagggttactggactagggtcgcagcagctgggcagcagggcatagagctcgagtgaagcttgctcaggctctgctaggcacacattggaaagttacatttcctattccatcataataccatttattcccagttcattgctcatgcctacaggtggaagtctgagttttatgtctagatggggcttccagtatgtccccactcagagtcctgcagttccttccaatcataggaagtgggaaggagcaaggcaggtaggttgtaaggctgatggtgtttcagctttgaggaaaaagtgatttcacttcaatagtaattttaaccagaatggctaaagttaaaaggattgacaatcccaagtgttggcaaggatagagagcaattgcaactctcagtgtttgctgctggaatgtgaatcagagccaccactttggaactctttggcagatccagcaattgctccagcaatcccactcttagatatatgagcaaaaaagtgagtgtttatgttcaccaaaagacatgtacaagaaagttcatagtgttgtaattcacttttattttttttttctgagatggagtcttgctttgtcacccaggctagagtgcagtggcacaatctcaactcactgtaacctccacctctcaggtttaagcagttctccctacctcagcctcccaagtagctgggattacatgtgcccaccaccacaccaagctaatttttgtattttttagtagagacagggttttgccatctaggccaggctgatcttgaactcctgaccttaggtgatctgcccaccttggcaaagtgctggcattacaggcatgagccatcatgccctgcctgtagttcacttttaagtatattttttaaaagtaaaaaatctgaagcagctgccacccaagtgtagaatagataaattgtgatataatcatagaatgaaaccagacataaccatgaagagaactgaactactgctagacaggacaacgtggatgaatctcacatgcaggatgctgatccggacaccacaagaaaaaacaaaagaaggtgcctactgagttttcttctttccagatgaccaactcttaacttactcatctgtttttttcactgttctgcttcttttgaagaagatttgaggtgacttacaaaggtgtatggcatatttataactgaagaaatctgggtgatgttaaaacgagggcaggaaaataaggtggaaaccagatgtaaggatagtcttcactatttatgtcaggaattcctacaaactttctatggtgaacagaatagagcttcctagcagtcaatgcaaagaagaaacacaacaattccacaccccaaagttaacagtcttgcttatcagaagcacaggtagttctgaaatctgatagaaaatgttcctgtatcatttcagaacacgcaactatgtgatcaaacccctttctatttgtttaaaaatttgtcaaacatcccatgtttgaccctggatgtctgaatcccctcagcccacattttcccccctacaccatgcccacaccatccccatagaatttagggtgaggcagcatctcagtgattgacaggcccctccttagaccccgtttactttcctgggtgtggtttggggtaagccctgttcatgaaggctggatttctgttctttgggttgcccagcttgccaccctcatttctggaacccagaccagcatcctcagcccacgctttgccactcagctcatcttcttcccagttggcacttctcagtgaccccatcccttccccagcagtgactctgcgtggggcagctccctggtggctggactctttccattttggcatttgggttagtggatctttccactttctggctccagtttttgagttgaattcatatgtttccccggtcactggatctatggcttctccatcaaagatagtgttcatctggatagtttccaccacgacgtctctctctgcagtcttcgtttctcctttctttgtcagaggttccttgttcttcccagtcttgcaggggcagtgtctgtggatggctttggccaataggacgaccaggtacacgaggagacccagaagcaatatggagcccaaagtgatgacaaacggcacgtaccatgcagatggagagtaaacgtttttcctcaggacctgataggtgaccctgggctgggccaatggaataacggaaagatctggggctggaatcaaggtcggtacatgtcagcttgaaattctgaatatttgtgccaactttcagatccactgggagggccaggaaataagagtttggagtacaaattggcttttcatcattttcttcaaggatgttcacagtaacctgcagatgacaccgagttgtttttccaggaaggtgtggatttacggtgtctccatgtgccaccttgcctgctgccccttgtaaatggaacttctttaactagtgacagagcttgtgtcttcgttgttggtggcctggattctgagaatatagatgggggttgtttcacagtccactttagttaccagctggagttctcctgtcttgggattaatccaaaatacatttggatactggaggctggcccctccagtggagatggagtacaggaggctgctctgggggaggtctttatcagtggctcgcacctgtcccactcgggttctggcgggccttctttctgacacatcaaatacataggatggcctatcaaaaatgagaggaaactcattttctgggcttgttaggatataaacgtagacgttatttttatagtaagggggggccacatcctgcacctggattatcaccgtatatttattgccggctgctaggttacttggattttcgtagtctagatcaccaatcagcacaatcttcccagagccagctggatcctgtaaaaatctgctgccgctccccactccagatggcatggtgaagttgaatctgttgtttggtgcctcactgtcatcatcaaagcagaacttgtttaggtcaagaagcaacgtccccttggctgttctttccggcaccataatgctgaaggtgaacttttggcatgtggcaggattgtcgttgacgtcttccacaatgaaggttatctggatgcgattctcctgacccccatatggtctgtccttcactagaacttccagggaaatggtgggattttgtctcaattcacctgcatctcggtctatcctttgggccacttggattgtaccagtcaactgatttatcatgaaatatttgctaacagtggtaatgctgtagaggaggtggctgggaaaaccttcatcatcaggatcctccgctgtgatattggccacgatggttcctggactcagttcctccaggactgtgtacactcgtgtcgggctggtaaagcgagggacttcgtcgttgaggttcacgatgttcacctggagctctgtggaggctttgaggcctccactgtccctcacctccacgatgagatggaaacttctgtgtcctgcttcaaagtccaattctgttgtggagaagagggtgccattagcagacattctgaagctctttgggggagaaatcaggaaataactgaggggaatgtttcggcttgtgtcttctggatcgaaggcctcaacctggtaaatgaatccagggtttgctctttctactatgtagaggtgtagaccttctgccaagttgccttgaaactgaggtggctcgttcacatctgttacctggacagtcaggacttgcaggtctgtgacaccaacctcatccttcacataaatctgcaaatcaaatatgtttggtcctgtttcaaaatctagttgttccatcccagtggtgacaacctcaaagtaggtgcctgacagccaattcaccctaaaagcttcagtgaggggatttgagttgactatctggggaaatcctgggatcacaggtgacaatgatgctgataacttcacagaaaacttgtgcactgaagtcccaggtggagaattctctgccacattgcctgtagcaggtaagaggattaggtgtagtgcttctccccctgacatggcacccaggagagccaggagaatgattgcttcctgcatacttgatggtcacaactgtgcgtgcttccagcacattagccacagcctgaatcccgtctcacacccaaagtttatt

SEQ ID NO: 14798 - RNA, 1375 nt, Homo sapiens
  source 1..1375: mol_type = other RNA
gctgggattacaggcatgagccacctcacctggccagtttgcccatttttaaattagatttttgtttctgttgttgagttgtaagagttttctgcacattctggatactaaccccttaccagatacatgatttgcaaatatttcctcccattctttagctgcctttttgctctgttgatggtgccctttgatgcacaaaagttttaaattttcatcgaccttagtatttattttttcttttattggctgtgcttttgttaccaagaaattcttgccatccatatacagacggacctttttattcttttttttttcttcagcaaatcccaggcatcgcgtcactccctcttccccttcagtctgtctctcacagcatgggatctttcttgcgggccccagtgtcactgtcccatccacgcacccagcagtggtctctgggtggaatctgaaacccctccattagcacatgtcccaaattatctcagaaatgtcttttcacggtggtgactttgacccaggacccacgtggcacttggtagatatgtccccaggtctccagtctgagccatctcccgtgtttcctgccagcaacgtgttatagggacagggtaggttgttagagggacagggtaggttggccataggctacccccaacccccgatgtgccttctgcctcctgtggtgtcatcggccagtccttgggtccttcccacttcctataaatggaggtgagctcttgcagcgctgttaatgttgggcccagccacacgcaggtgctgtgagcttcacaccccatctccccaggaggcagaaactgtgctcgccaccgctgtgacaaaagctgcacacaggatccaggtggtgatggtgaatccttcctcttgaagctcctcaccggctggtcacccaggggcctctctctggggtgggccctgcagacattgaggagtacactgaggcttgcaggcttgcatctgatgacttcctaatcctggcatgccttcgcagtgatgagctgagattcttccatctcgaagaactttcacatatcaaataagatgacttggttaagctgaacactgtggcaactgctttccttctctgagacttgtgttttccaagacgggcgcagatgggcgctcagcacgggccgggcgtgatccaattacacagcagatttcagacgcccagacttggagctggggaagcctggcgccctggggagaacactgccttatttgctttagaaaagtcagctctcctgttcctaaggcctcctggatgggggcccgcctcttccccttggtggtttgctggggtgggagttcgcgtttcgcggtcctctgaagggctctcgctgctgcttctgtcatt

SEQ ID NO: 14799 - RNA, 2652 nt, Homo sapiens
  source 1..2652: mol_type = other RNA
gctgggattacaggcatgagccacctcacctggcctacatccttattctttacagcataatattctgtagtgtaaatgtgtcacactttaccatactcttattgagggtgcaattaactcattaatggatcaagtaattaatgcccagtgtggcaaggaaacagagacacgatcatgtttctacagtactggtagagtttttaactgatacagtccccaaaaggtataagatatcaaagatcttaaaaacatatgtactctgtagtcctagttgcttaggaggctgaggaaggaggactcctagagcccaggaattcagtggtgcggtgagctatgattgcaccactgcactccaacctgggcaatggagtgagatactgcctctaaaaaccaagcaaccaacatacaaaaatctgtgctctttaattcatgtatagaaattccacgtataaaaattccatgtatagaaatttatcttaagataattatatggctgggcacggtggctcatgcctatagtctcagcaccttgggaggctgaggcaggaggattactggagtccagaagttccagaacagcctaagcaacatggtgagacatcgtctctatttaaaaaaatacaaaaaaactccccgtctctataaaaagtacaaaaagttagccaggcgtggtggcgcacacctgtgatcccagctacacaggaggctgagactgtggaatcacttgagcgtgggaggctgaggctgcagtgagccatgatcgtgccgctgtactccagcctgggtgtcagagcaagaccctgcctcagaaaaaaacaaaaaaaaaaggataattagataattatagaagagcctaatgattactctgcaagaatcattatgggtgccttatttggaagcgtaaaaatgttggaaataacccaaatatccagcattaggggaaatggttgagaaaattacaaatccatccagtggaatctacagggccattagcagtgcaagcaggtggtgaagggaccttcatcttatttgcagagaggccatgcataggcatgctagcaggtgtatttttcattgtactttcactgaccttacaatatgtggaaatggttcttcaattctggcaatagaataactcctcgtcctggttctggtgaaggcatgacagctgtgggcatgcatgtgtgtgctggtgtatatgcacacacacatacatgctcaaactcttaaacaggagcttctgcaaacgtgtaataagctggagaaagtcattttcatcagcatcacctccatgaagagcactgggtttatttgaaagaaatttcttgatgaattgcttagaagaggatatgagatcacaaatgatctcagtgtgttcagaactgccttgcaagaggcaagcaggggcctctttcagtttactccagaggaagtgagaaaacagaagagggagtgggaagatgtgtcggggagtccccaagacacgctcaggtatgacgatttgctgcaaagaatcgcagaactcaaaaaagctgttgtattcacagttacagcttaacacagtggaaggatgcggattaaaaatcagcaaaggggccaggcgcggtggctcatgcctgtaatcccagcactttgggaggtcgaggccggcggccttgtcacttgagctcaggagttcgagaccagcctggccaacatggcaaaaccccgtctctactaacatataagaattagccaggcatggtggttggcacctgtaatcccagctccttgggaggctgaagcagaagaatcacgtgaacctgggaggtggaggttgcaatgagccgagatccagccaccgcactccaaccttggtgacagagtgagactccatctcaaaaataaataaatagataaacaaaatcagcaaaggaaaaaggtgctcagggcagaatccaggcaggagcttgcagctgtaccctcctagatagtcatatgtgcagtgcttaagtctcccagcaatgatgtgtgacaacacacgcaaaacactgccaaccaggggaactcacctgagccttagtgtccatggcttttcttggggatcagttacccagtgtccagcccctccagaggtcaggctgatacagcatgaccgcaggcacccaccataaatcatgttgttagcatcaactacccggcatggcccaaggccccagatatacagaagccctcttatcaggcagaatattttaagccgttagcagttatcctgcaggaacaggtgaagagccagtccttcctctgagatgtgcagggtttaaccatcccaagcctcttgagataaccctttctgtaaatgaaggtcgagttttgcatcagagaaaacgtgtttgattgaggccagggtggtggagaacggaagtgacgacagacagaagccagcagaagtaaggcacgaggctccacagaatcacgggatggttgcagccagattctaacatcagaggggcaggatttgaagtggagaggctgatatgatgctgacagggggtaccagcacccccaggccatcgtaattagcatctggccgtgatcccagtctcctggcagcacattcctcatcttcctcgccagccaatctcctttccccagcaaccctccgacagcact

SEQ ID NO: 14800 - RNA, 1397 nt, Homo sapiens
  source 1..1397: mol_type = other RNA
gctgggattacaggcatgagccacctcattgggcctcccccattcaatttcagtgacatgactgactccccacccacccatgccattgagatgcccttttcagaccctcagagcctctcgcgtcaaggaagccaattcactacccactgggccagctggcgtgggccgccccaactgcccaggaagccccactcagaccatgaccttgctgcctgtgcagtccaggccccggcaagggccaggcatggaacatatgctcagagcgatgggggtcagggccaaggccacagagcaagatgcagaggagcccaggctgggaccggttctgcctgaacatgagcccctcggagcaggggccccgccactcagcgccgggtcctcaggccaggcatgccctgtgcgaggaagggccccgggcctcccaccagagctagaggaggggtggctggcaaagggaggctgaggaggaacggagggttgaggggctggggacttgcggccaggtaggcacaagcacatgaatcaactccaactggaagcagagaaaaagcagtaaaaccaaatgtccttagaaattcctttagtgctcagctgtccatgaaaacaggataagcggcttcctccgtctgtgctcagcagggcagggtggaggcgctgcgctcaggccaggaggacctcgaatcaggacggggtggggcggggctctgagctggggaagcggctccagcgttgctactttagggcgtccaggtgggtgcagacctgggagaagacactgtccacggagccctcagcgttgaccttgcgcacaatgccacgtttctcatagaaggcgatgacaggttctgtggccttgtaataggtctccagccgctttttgatggtctcctcattgtcgtccacacgcccgctggtctctccacgtttcaagagccgctgggtcatggtctcagggcctgcgtccacatacagcagcagtgtgggctgtccaatccgtcgctcaaactcttctccttgctgcacctcccgcgggtagccatcaatcaggaagcctttggaagtattgactttggccaccatggcatcccggagcatgtccaacactgtctccagtggaaccagctgccccttctccatgatttccgacagcttcttgcccctggccgagcctgagctgacctcggaccgcaggaggtccccggtggagaggtgggtgtagccatacttctgcacgatcttctcacactgggtgcccttccctgagccaggcccacccaccacaaagatgatcttggttttcttcagcttctctctggctctcagatcgtcttctctgcgggggtcactcgaggagcagcagcccatggtcccgtcctgccgtgtctcctgtgcaccct

SEQ ID NO: 14801 - RNA, 1402 nt, Homo sapiens
  source 1..1402: mol_type = other RNA
gctgggattacaggcatgagccacctcattgggcctcccccattcaatttcagtgacatgactgactccccacccacccatgccattgagatgcccttttcagaccctcagagcctctcgcgtcaaggaagccaattcactacccactgggccagctggcgtgggccgccccaactgcccaggaagccccactcagaccatgaccttgctgcctgtgcagtccaggccccggcaagggccaggcatggaacatatgctcagagcgatgggggtcagggccaaggccacagagcaagatgcagaggagcccaggctgggaccggttctgcctgaacatgagcccctcggagcaggggccccgccactcagcgccgggtcctcaggccaggcatgccctgtgcgaggaagggccccgggcctcccaccagagctagaggaggggtggctggcaaagggaggctgaggaggaacggagggttgaggggctggggacttgcggccaggtaggcacaagcacatgaatcaactccaactggaagcagagaaaaagcagtaaaaccaaatgtccttagaaattcctttagtgctcagctgtccatgaaaacaggataagcggcttcctccgtctgtgctcagcagggcagggtggaggcgctgcgctcaggccaggaggacctcgaatcaggacggggtggggcggggctctgagctggggaagcggctccagcgttgctactttagggcgtccaggtgggtgcagacctgggagaagacactgtccacggagccctcagcgttgaccttgcgcacaatgccacgtttctcatagaaggcgatgacaggttctgtggccttgtaataggtctccagccgctttttgatggtctcctcattgtcgtccacacgcccgctggtctctccacgtttcaagagccgctgggtcatggtctcagggcctgcgtccacatacagcagcagtgtgggctgtccaatccgtcgctcaaactcttctccttgctgcacctcccgcgggtagccatcaatcaggaagcctttggaagtattgactttggccaccatggcatcccggagcatgtccaacactgtctccagtggaaccagctgccccttctccatgatttccgacagcttcttgcccctggccgagcctgagctgacctcggaccgcaggaggtccccggtggagaggtgggtgtagccatacttctgcacgatcttctcacactgggtgcccttccctgagccaggcccacccaccacaaagatgatcttggttttcttcagcttctcttccatcctgccgaggtcccgggagccgtgtcagtgctctggggaggggtgcgggtgggcgccggggccagtgcgtgccctgcccgtcctc

SEQ ID NO: 14802 - RNA, 1457 nt, Homo sapiens
  source 1..1457: mol_type = other RNA
gctgggattacaggcatgagccacctcattgggcctcccccattcaatttcagtgacatgactgactccccacccacccatgccattgagatgcccttttcagaccctcagagcctctcgcgtcaaggaagccaattcactacccactgggccagctggcgtgggccgccccaactgcccaggaagccccactcagaccatgaccttgctgcctgtgcagtccaggccccggcaagggccaggcatggaacatatgctcagagcgatgggggtcagggccaaggccacagagcaagatgcagaggagcccaggctgggaccggttctgcctgaacatgagcccctcggagcaggggccccgccactcagcgccgggtcctcaggccaggcatgccctgtgcgaggaagggccccgggcctcccaccagagctagaggaggggtggctggcaaagggaggctgaggaggaacggagggttgaggggctggggacttgcggccaggtaggcacaagcacatgaatcaactccaactggaagcagagaaaaagcagtaaaaccaaatgtccttagaaattcctttagtgctcagctgtccatgaaaacaggataagcggcttcctccgtctgtgctcagcagggcagggtggaggcgctgcgctcaggccaggaggacctcgaatcaggacggggtggggcggggctctgagctggggaagcggctccagcgttgctactttagggcgtccaggtgggtgcagacctgggagaagacactgtccacggagccctcagcgttgaccttgcgcacaatgccacgtttctcatagaaggcgatgacgggttctgtggccttgtaataggtctccagccgctttttgatggtctcctcattgtcgtccacacgcccgctggtctctccacgtttcaagagccgctgggtcatggtctcagggcctgcgtccacatacagcagcagtgtgggctgtccaatccgtcgctcaaactcttctccttgctgcacctcccgcgggtagccatcaatcaggaagcctttggaagtattgactttggccaccatggcatcccggagcatgtccaacactgtctccagtggaaccagctgccccttctccatgatttccgacagcttcttgcccctggccgagcctgagctgacctcggaccgcaggaggtccccggtggagaggtgggtgtagccatacttctgcacgatcttctcacactgggtgcccttccctgagccaggcccacccaccacaaagatgatcttggttttcttcagcttctcttccatcctgccgaggtcccgggagccgtgtcagtgctttgggaggctgaggcagaagaatagcttgaacccaggaggcagaggttgcggtgagccgagatcacgccattgcactccagactgggcaacaaggcaagaagagcgaa

SEQ ID NO: 14803 - RNA, 1050 nt, Homo sapiens
  source 1..1050: mol_type = other RNA
gctgggattacaggcatgagccacctcgcccaaccaggaagcttttcttcagtctctttctggagaacactcagccaggctgtaggtccccaggaaaagcccaagcttccatttaaggatttgcatttcctgaatttgcctttgcatcttcggtggtggcccaggaaattcgaatccagaggaaagaagcacgcggcagcgctgggtcttgcaggcatcatagctctcattcttgtatccggcacacagcatatttttggtaagttttggaaacatctttgaacactcctcccagtccatgatgaccattggcgctttcatcagatccgttttcacagagtttttgtcagcagcattggtctggccccaacctgccacccagcattcgcgccatgtggcagggccgggctgcgtggggaggcagatgggcaccttcaggtcatcgagcttgatgggcgaagccagcagcagcaaggcaatgtcattgtccatgttggctctcttaaagtctttgtgaagaatgatgctggcgacctcctttatttccatggatgggctagttaagtcgttggtccccagcacgacactcagttcttctggaaacagctcctcggaatataagcagtgagccgcagtgagaatccaccacttgttgaggatggagccgccacagaaaggttcacttcttgcctgaatactcacctgccacggaaactcacccacctccgcctccatcccccctgtgattctggaataccgagttcttccctcgaaaatagatctgtcaccacattcactgactgggctggggggatgagggggctgagggcggtgggctcccctagccctgcctaggatagccactccagcctctgggagaggagtccgtggaccgagctgagttcccgtgaccagggacaggagcagcaacactgagaacaggagcatggccctgggctgtgctgtgggcccgggggtgacagaggccagggctgaggcagtgaggctgagagcctccagctcagatccagagcccccaagtgatgtcac

SEQ ID NO: 14804 - RNA, 959 nt, Homo sapiens
  source 1..959: mol_type = other RNA
gctgggattacaggcatgagccacctcgcccatcctcaatatatatttttcactgagatctaaatcacataccatagaattttaatgtgtacagttcagtggtttttagtcttttcacaataaattgagtttttgagtagacaatgcattcatatggcttaaaattcaacgattaccaaggaatatacacggaaacatcttccttccccgcatcccgcatacatagatcatattatctatttcttgactatactcatagatattttatgcaaatacaagcaaatgtattccgtccctttttaatctacatggtggagaactatatgtactgttcagcatcttgcttttttacttaacttggaggtcctgctggtaccgagctttctcattccttctggtggctgcctggtattctagtctatggatggataaatatttattgatggatatttaggttgttgctacacctcagcttttgcaaacaaatgctgcaaagaagaacctggtgcatgagacattttgcatgttcgggcagatctgtagaagtaattcccagaagggcgcatgttttttacattttgacagttcttgctaaatggccctttatagaggttacaccagttttaattcccatcagaatttatttccaaacctatcatgagatacgccagcactgacaagaatcctcactgcggcattgttcatcgcgccccaaactggaaacagctcaatcgatcctcagcggaacggagaaatcatggcctcttcacgcgatgaaatattatgctttcttccttcctttctcggtgaagtgaagggtcacctctcattgtggaagaaggactagtaaagccagctttaaatgaacattactgggttggcctatgccaggcaggcgcgaggtctctattccccatgtgacaatcaagctgggtgcgttcacgcccaggatgctgggg

SEQ ID NO: 14805 - RNA, 3844 nt, Homo sapiens
  source 1..3844: mol_type = other RNA
gctgggattacaggcatgagccacctcgcctggcccctcctcttgttttttgcctgtcacgtatttgttttgttggaaacccgagacattggtcctatagacctcactctattctggattttgctgactgcatccccatggagtttgtttgtgtgtttgtttgttatgaagtcttgctctgtcacccaggctggagtgtaatggcggatcacagctcactgcagcctcaacctcccagacttaagcaatcctccagcctcagcctcccaaatagctaggactacaggcatgcaccaccacactcagctaagttttttgatttttagtagacaggatctcactgtgttgcccaagcttgtctcaaactcctggcctcaagcaatcctcctgcctcaacctccccagagtgctgaaattacaggtgtgagccaccacgcccagcccccatggagttttgacatctccctgtataccacatatttcctataaaccagtagcgaacctagaaacttgtccagctgaatctccatttctttggcgtggatgcttcctgggtggcgccctgcacttcctgctacatcacaccaggaggcccccgtgtctggctgcttcccttcctgttcagtgagactcagcagcgggcacaggtgctacccccagcccgcactttgctattcaccctgtgctgatccccaggcagagccacacttcacgagagggtcacactgtatgtatacccagggaataagaggtcacttcaagtcgcttagttattctcaatatttttaaatttcagtctcaaacagaatgcaatttcatctagtttataaaacttaatatacgtatactgctacctcaaagtaatcaatccaacacttggccagttaatatgacctaatttcacatttacctgtacatttacagcattcatactagagttattctgctaccacacagagatttcaactttattatatactttaacaaaaatggtatgtgaaatggatattatgtctatttacttaagggttattttgcagagtgacttactaaatggaaaaaaaactgtatggtctatattagtaagaaagtaatttttggagaaggattatgtaaaaggaattacagaattgggaataagctgtttcaggcatgatgacaaggcaagagcatcaggaaatcacggtgtttcctcttagcaaccggtgagcagcaggaaaggcaacagaactcctcaggacccagcactcccggagccacggcttcccagagagcctggcacaggcacacaactgggtgagggttcttgtgtggatatttaaaacaacaccatcaagataaaaatattgttgtatctgtagcatctctatttatgtatttattttcccttgaaataaaaatgttctaaagttacattgttttccatgctgcctgttttattacttctcacaacttaggcaacaaaattttacgtcatcatatttccagttcttatacgtctgctctactctgtatttagatttggttagaaaatctgattattcttgatttcaccaggagctttcttttttatttatttattatttatttattatttatttcttccaaataaaaactaatagtcaacttcattaggcattatgactagaaaattaagcactcgttgtggagagaaaagtattcttatacagccattttattttattttattttattttattttattttattttatttttgagaaagggtctcactctgtcacccaggctgaagtgcagtggtgccatcatagatagctcactgcagacccaacctcctgagctcaaacgatcctcctgcctcagtcttccgagtaactaggaccataggtgtgcaccaccacgcccggctaatttttgtatttttggtagagacagggtttcaccatgttgctcaggctggtctcgaacttctggctcaagcaatcctcccaccttgacctcccaaagtgctgggattacaggcgtgagccaccgcacccggccagcccttttaagtttgagccctttaacaggatctaaatctggtgctcaggataaaatgttgcctctggtgctttcttcccataattacagtattacagaggcattcttaatgttccctcttcaaattagaaacagtaagttgaaattgccttcaacttactgttgatggcaatttgagcccagatgccagtattagagaacatatattgaagaactgaatttgtaagtaaaccaccatttccctgtacaagtaaatgcacaggatactgccagtcattaaatattgagtctagcacaatgtatgaagcataaaaattcactgccactggtttttaaacagctgtttcccccaaagaaagggcaacttctggtatgcaccagtaaaatagcaacctttttacattactttgcataaagatttacaagtgtcccaggacctgggaggccagtctataacaagacagcctttagcgacatcgctttccttctccacggtgatcagcgaacacaaatacccactgtgtgtcggcgagctggtctgctacatcagcccaggtttaaaatctaggcttactttctgttaacaaatcgcacgtggatgggcccccctggcgtcaggagcccgtgggtttttgcatgaacagcattggtctgagaagatgttttgatctcaaaatgttgaagcaactggatcacgacgaggtgaatctccagttctgcaattctccgccctatgcagctgcgaaccccatgaccaaaggggatggatccaaaattgtcaactctatctaagtctcctttccgcagccagcgctcaggccggaactccttggcccgagggaagttctcatcctggtacgatgtggcatagtggcaaagggccagctgggtgcctttcggaatcagatacccgccaataaccaggtcttcctgggtgacccggccgttccctggcagcactggaaacagcctcagggtttccttaaggagagctctgaccagcgggaccttggggacatcagctgcagttggaacatgcctttcccctaaattcttcacaatctcccggtacaccgtctgctgcacttctgggtgccttgccaggaggtacacagtccaagacaaggtgaaggacgtcgtgtcgacgccggccagcagcatctcagtcacgttggcgtagatctcctgcagcgtcagagcctggctaaggaagaggtatgtgagaagtcccccgctcaccctccggcctcggtccatttggtactgtatgtccctcaacttgttgtcaacatgaatttggctgaatttgaagagtccatcccaggacctgcagaattcccgccagggctttgggatgaaggggcgaagccatctggggatggcgcctgcatacatggaggtcttgaacatgctaaacatgagctccagggcctcgatgtattccacagtcagctgtgggatgctgttttccaggcagcccaaacgactctcataaaggatggtggccactccttccattgaatatttgaagaaaagatcattgacattggtcacggtttctccatcttctgcctggctcctgaggaggtagattcttttaattaagtcagcaataacttggttgacttctccagaataaatggccacatctttcggtttcagaattctttgtctcaatacgcttctcatcttgagccactgttcaccctcccacggagccagcgtcgcccctcctggctcctgacgggacaactctgcacggaggaggagccagaaagcccagcagggctctcatgtctgggagatcgcacaaggagact

SEQ ID NO: 14806 - RNA, 4046 nt, Homo sapiens
  source 1..4046: mol_type = other RNA
gctgggattacaggcatgagccacctcgcctggcccctcctcttgttttttgcctgtcacgtatttgttttgttggaaacccgagacattggtcctatagacctcactctattctggattttgctgactgcatccccatggagtttgtttgtgtgtttgtttgttatgaagtcttgctctgtcacccaggctggagtgtaatggcggatcacagctcactgcagcctcaacctcccagacttaagcaatcctccagcctcagcctcccaaatagctaggactacaggcatgcaccaccacactcagctaagttttttgatttttagtagacaggatctcactgtgttgcccaagcttgtctcaaactcctggcctcaagcaatcctcctgcctcaacctccccagagtgctgaaattacaggtgtgagccaccacgcccagcccccatggagttttgacatctccctgtataccacatatttcctataaaccagtagcgaacctagaaacttgtccagctgaatctccatttctttggcgtggatgcttcctgggtggcgccctgcacttcctgctacatcacaccaggaggcccccgtgtctggctgcttcccttcctgttcagtgagactcagcagcgggcacaggtgctacccccagcccgcactttgctattcaccctgtgctgatccccaggcagagccacacttcacgagagggtcacactgtatgtatacccagggaataagaggtcacttcaagtcgcttagttattctcaatatttttaaatttcagtctcaaacagaatgcaatttcatctagtttataaaacttaatatacgtatactgctacctcaaagtaatcaatccaacacttggccagttaatatgacctaatttcacatttacctgtacatttacagcattcatactagagttattctgctaccacacagagatttcaactttattatatactttaacaaaaatggtatgtgaaatggatattatgtctatttacttaagggttattttgcagagtgacttactaaatggaaaaaaaactgtatggtctatattagtaagaaagtaatttttggagaaggattatgtaaaaggaattacagaattgggaataagctgtttcaggcatgatgacaaggcaagagcatcaggaaatcacggtgtttcctcttagcaaccggtgagcagcaggaaaggcaacagaactcctcaggacccagcactcccggagccacggcttcccagagagcctggcacaggcacacaactgggtgagggttcttgtgtggatatttaaaacaacaccatcaagataaaaatattgttgtatctgtagcatctctatttatgtatttattttcccttgaaataaaaatgttctaaagttacattgttttccatgctgcctgttttattacttctcacaacttaggcaacaaaattttacgtcatcatatttccagttcttatacgtctgctctactctgtatttagatttggttagaaaatctgattattcttgatttcaccaggagctttcttttttatttatttattatttatttattatttatttcttccaaataaaaactaatagtcaacttcattaggcattatgactagaaaattaagcactcgttgtggagagaaaagtattcttatacagccattttattttattttattttattttattttattttattttatttttgagaaagggtctcactctgtcacccaggctgaagtgcagtggtgccatcatagatagctcactgcagacccaacctcctgagctcaaacgatcctcctgcctcagtcttccgagtaactaggaccataggtgtgcaccaccacgcccggctaatttttgtatttttggtagagacagggtttcaccatgttgctcaggctggtctcgaacttctggctcaagcaatcctcccaccttgacctcccaaagtgctgggattacaggcgtgagccaccgcacccggccagcccttttaagtttgagccctttaacaggatctaaatctggtgctcaggataaaatgttgcctctggtgctttcttcccataattacagtattacagaggcattcttaatgttccctcttcaaattagaaacagtaagttgaaattgccttcaacttactgttgatggcaatttgagcccagatgccagtattagagaacatatattgaagaactgaatttgtaagtaaaccaccatttccctgtacaagtaaatgcacaggatactgccagtcattaaatattgagtctagcacaatgtatgaagcataaaaattcactgccactggtttttaaacagctgtttcccccaaagaaagggcaacttctggtatgcaccagtaaaatagcaacctttttacattactttgcataaagatttacaagtgtcccaggacctgggaggccagtctataacaagacagcctttagcgacatcgctttccttctccacggtgatcagcgaacacaaatacccactgtgtgtcggcgagctggtctgctacatcagcccaggtttaaaatctaggcttactttctgttaacaaatcgcacgtggatgggcccccctggcgtcaggagcccgtgggtttttgcatgaacagcattggtctgagaagatgttttgatctcaaaatgttgaagcaactggatcacgacgaggtgaatctccagttctgcaattctccgccctatgcagctgcgaaccccatgaccaaaggggatggatccaaaattgtcaactctatctaagtctcctttccgcagccagcgctcaggccggaactccttggcccgagggaagttctcatcctggtacgatgtggcatagtggcaaagggccagctgggtgcctttcggaatcagatacccgccaataaccaggtcttcctgggtgacccggccgttccctggcagcactggaaacagcctcagggtttccttaaggagagctctgaccagcgggaccttggggacatcagctgcagttggaacatgcctttcccctaaattcttcacaatctcccggtacaccgtctgctgcacttctgggtgccttgccaggaggtacacagtccaagacaaggtgaaggacgtcgtgtcgacgccggccagcagcatctcagtcacgttggcgtagatctcctgcagcgtcagagcctggctaaggaagaggtatgtgagaagtcccccgctcaccctccggcctcggtccatttggtactgtatgtccctcaacttgttgtcaacatgaatttggctgaatttgaagagtccatcccaggacctgcagaattcccgccagggctttgggatgaaggggcgaagccatctggggatggcgcctgcatacatggaggtcttgaacatgctaaacatgagctccagggcctcgatgtattccacagtcagctgtgggatgctgttttccaggcagcccaaacgactctcataaaggatggtggccactccttccattgaatatttgaagaaaagatcattgacattggtcacggtttctccatcttctgcctggctcctgaggaggtagattcttttaattaagtcagcaataacttggttgacttctccagaataaatggccacatctttcggtttcagaattctttgtctcaatacgcttctcatcttgagccactgttcaccctccctggatctcgtggatgcggctgaagccgtccctgcagaagaactccgccaggttggcgagggtcctcggccccggcatggcggcgaggctccggggaccctcggctcggccccctcccggcggcgaccccggccgcccggcgcctttgtcctcggcccgcgcccccgccgggagccgtgcgcccgcgggttgaggccgccgcggggccccgccgcccaggagcccaccccgctcgggcgccggccgcagcccggctctcaggatccgcgccagcagggccatggcgctcgtctgcatcggcttgtttgtct

SEQ ID NO: 14807 - RNA, 4237 nt, Homo sapiens
  source 1..4237: mol_type = other RNA
gctgggattacaggcatgagccacctcgcctggcccctcctcttgttttttgcctgtcacgtatttgttttgttggaaacccgagacattggtcctatagacctcactctattctggattttgctgactgcatccccatggagtttgtttgtgtgtttgtttgttatgaagtcttgctctgtcacccaggctggagtgtaatggcggatcacagctcactgcagcctcaacctcccagacttaagcaatcctccagcctcagcctcccaaatagctaggactacaggcatgcaccaccacactcagctaagttttttgatttttagtagacaggatctcactgtgttgcccaagcttgtctcaaactcctggcctcaagcaatcctcctgcctcaacctccccagagtgctgaaattacaggtgtgagccaccacgcccagcccccatggagttttgacatctccctgtataccacatatttcctataaaccagtagcgaacctagaaacttgtccagctgaatctccatttctttggcgtggatgcttcctgggtggcgccctgcacttcctgctacatcacaccaggaggcccccgtgtctggctgcttcccttcctgttcagtgagactcagcagcgggcacaggtgctacccccagcccgcactttgctattcaccctgtgctgatccccaggcagagccacacttcacgagagggtcacactgtatgtatacccagggaataagaggtcacttcaagtcgcttagttattctcaatatttttaaatttcagtctcaaacagaatgcaatttcatctagtttataaaacttaatatacgtatactgctacctcaaagtaatcaatccaacacttggccagttaatatgacctaatttcacatttacctgtacatttacagcattcatactagagttattctgctaccacacagagatttcaactttattatatactttaacaaaaatggtatgtgaaatggatattatgtctatttacttaagggttattttgcagagtgacttactaaatggaaaaaaaactgtatggtctatattagtaagaaagtaatttttggagaaggattatgtaaaaggaattacagaattgggaataagctgtttcaggcatgatgacaaggcaagagcatcaggaaatcacggtgtttcctcttagcaaccggtgagcagcaggaaaggcaacagaactcctcaggacccagcactcccggagccacggcttcccagagagcctggcacaggcacacaactgggtgagggttcttgtgtggatatttaaaacaacaccatcaagataaaaatattgttgtatctgtagcatctctatttatgtatttattttcccttgaaataaaaatgttctaaagttacattgttttccatgctgcctgttttattacttctcacaacttaggcaacaaaattttacgtcatcatatttccagttcttatacgtctgctctactctgtatttagatttggttagaaaatctgattattcttgatttcaccaggagctttcttttttatttatttattatttatttattatttatttcttccaaataaaaactaatagtcaacttcattaggcattatgactagaaaattaagcactcgttgtggagagaaaagtattcttatacagccattttattttattttattttattttattttattttattttatttttgagaaagggtctcactctgtcacccaggctgaagtgcagtggtgccatcatagatagctcactgcagacccaacctcctgagctcaaacgatcctcctgcctcagtcttccgagtaactaggaccataggtgtgcaccaccacgcccggctaatttttgtatttttggtagagacagggtttcaccatgttgctcaggctggtctcgaacttctggctcaagcaatcctcccaccttgacctcccaaagtgctgggattacaggcgtgagccaccgcacccggccagcccttttaagtttgagccctttaacaggatctaaatctggtgctcaggataaaatgttgcctctggtgctttcttcccataattacagtattacagaggcattcttaatgttccctcttcaaattagaaacagtaagttgaaattgccttcaacttactgttgatggcaatttgagcccagatgccagtattagagaacatatattgaagaactgaatttgtaagtaaaccaccatttccctgtacaagtaaatgcacaggatactgccagtcattaaatattgagtctagcacaatgtatgaagcataaaaattcactgccactggtttttaaacagctgtttcccccaaagaaagggcaacttctggtatgcaccagtaaaatagcaacctttttacattactttgcataaagatttacaagtgtcccaggacctgggaggccagtctataacaagacagcctttagcgacatcgctttccttctccacggtgatcagcgaacacaaatacccactgtgtgtcggcgagctggtctgctacatcagcccaggtttaaaatctaggcttactttctgttaacaaatcgcacgtggatgggcccccctggcgtcaggagcccgtgggtttttgcatgaacagcattggtctgagaagatgttttgatctcaaaatgttgaagcaactggatcacgacgaggtgaatctccagttctgcaattctccgccctatgcagctgcgaaccccatgaccaaaggggatggatccaaaattgtcaactctatctaagtctcctttccgcagccagcgctcaggccggaactccttggcccgagggaagttctcatcctggtacgatgtggcatagtggcaaagggccagctgggtgcctttcggaatcagatacccgccaataaccaggtcttcctgggtgacccggccgttccctggcagcactggaaacagcctcagggtttccttaaggagagctctgaccagcgggaccttggggacatcagctgcagttggaacatgcctttcccctaaattcttcacaatctcccggtacaccgtctgctgcacttctgggtgccttgccaggaggtacacagtccaagacaaggtgaaggacgtcgtgtcgacgccggccagcagcatctcagtcacgttggcgtagatctcctgcagcgtcagagcctggctaaggaagaggtatgtgagaagtcccccgctcaccctccggcctcggtccatttggtactgtatgtccctcaacttgttgtcaacatgaatttggctgaatttgaagagtccatcccaggacctgcagaattcccgccagggctttgggatgaaggggcgaagccatctggggatggcgcctgcatacatggaggtcttgaacatgctaaacatgagctccagggcctcgatgtattccacagtcagctgtgggatgctgttttccaggcagcccaaacgactctcataaaggatggtggccactccttccattgaatatttgaagaaaagatcattgacattggtcacggtttctccatcttctgcctggctcctgaggaggtagattcttttaattaagtcagcaataacttggttgacttctccagaataaatggccacatctttcggtttcagaattctttgtctcaatacgcttctcatcttgagccactgttcaccctccgccgagatgagcccggtggctctcccccgcaagtctcggtactcccgccaggactccatgttggctctctggggcgcagcgccctccgcccggagcacctgagccaccatatcgcggtctgcaatagatactacaaactgaggaccaaagtgagacttgaagatttttccatattcccgtgtgtgcttctgctggatctcgtggatgcggctgaagccgtccctgcagaagaactccgccaggttggcgagggtcctcggccccggcatggcggcgaggctccggggaccctcggctcggccccctcccggcggcgaccccggccgcccggcgcctttgtcctcggcccgcgcccccgccgggagccgtgcgcccgcgggttgaggccgccgcggggccccgccgcccaggagcccaccccgctcgggcgccggccgcagcccggctctcaggatccgcgccagcagggccatggcgctcgtctgcatcggcttgtttgtct

SEQ ID NO: 14808 - RNA, 3934 nt, Homo sapiens
  source 1..3934: mol_type = other RNA
gctgggattacaggcatgagccacctcgcctggcccctcctcttgttttttgcctgtcacgtatttgttttgttggaaacccgagacattggtcctatagacctcactctattctggattttgctgactgcatccccatggagtttgtttgtgtgtttgtttgttatgaagtcttgctctgtcacccaggctggagtgtaatggcggatcacagctcactgcagcctcaacctcccagacttaagcaatcctccagcctcagcctcccaaatagctaggactacaggcatgcaccaccacactcagctaagttttttgatttttagtagacaggatctcactgtgttgcccaagcttgtctcaaactcctggcctcaagcaatcctcctgcctcaacctccccagagtgctgaaattacaggtgtgagccaccacgcccagcccccatggagttttgacatctccctgtataccacatatttcctataaaccagtagcgaacctagaaacttgtccagctgaatctccatttctttggcgtggatgcttcctgggtggcgccctgcacttcctgctacatcacaccaggaggcccccgtgtctggctgcttcccttcctgttcagtgagactcagcagcgggcacaggtgctacccccagcccgcactttgctattcaccctgtgctgatccccaggcagagccacacttcacgagagggtcacactgtatgtatacccagggaataagaggtcacttcaagtcgcttagttattctcaatatttttaaatttcagtctcaaacagaatgcaatttcatctagtttataaaacttaatatacgtatactgctacctcaaagtaatcaatccaacacttggccagttaatatgacctaatttcacatttacctgtacatttacagcattcatactagagttattctgctaccacacagagatttcaactttattatatactttaacaaaaatggtatgtgaaatggatattatgtctatttacttaagggttattttgcagagtgacttactaaatggaaaaaaaactgtatggtctatattagtaagaaagtaatttttggagaaggattatgtaaaaggaattacagaattgggaataagctgtttcaggcatgatgacaaggcaagagcatcaggaaatcacggtgtttcctcttagcaaccggtgagcagcaggaaaggcaacagaactcctcaggacccagcactcccggagccacggcttcccagagagcctggcacaggcacacaactgggtgagggttcttgtgtggatatttaaaacaacaccatcaagataaaaatattgttgtatctgtagcatctctatttatgtatttattttcccttgaaataaaaatgttctaaagttacattgttttccatgctgcctgttttattacttctcacaacttaggcaacaaaattttacgtcatcatatttccagttcttatacgtctgctctactctgtatttagatttggttagaaaatctgattattcttgatttcaccaggagctttcttttttatttatttattatttatttattatttatttcttccaaataaaaactaatagtcaacttcattaggcattatgactagaaaattaagcactcgttgtggagagaaaagtattcttatacagccattttattttattttattttattttattttattttattttatttttgagaaagggtctcactctgtcacccaggctgaagtgcagtggtgccatcatagatagctcactgcagacccaacctcctgagctcaaacgatcctcctgcctcagtcttccgagtaactaggaccataggtgtgcaccaccacgcccggctaatttttgtatttttggtagagacagggtttcaccatgttgctcaggctggtctcgaacttctggctcaagcaatcctcccaccttgacctcccaaagtgctgggattacaggcgtgagccaccgcacccggccagcccttttaagtttgagccctttaacaggatctaaatctggtgctcaggataaaatgttgcctctggtgctttcttcccataattacagtattacagaggcattcttaatgttccctcttcaaattagaaacagtaagttgaaattgccttcaacttactgttgatggcaatttgagcccagatgccagtattagagaacatatattgaagaactgaatttgtaagtaaaccaccatttccctgtacaagtaaatgcacaggatactgccagtcattaaatattgagtctagcacaatgtatgaagcataaaaattcactgccactggtttttaaacagctgtttcccccaaagaaagggcaacttctggtatgcaccagtaaaatagcaacctttttacattactttgcataaagatttacaagtgtcccaggacctgggaggccagtctataacaagacagcctttagcgacatcgctttccttctccacggtgatcagcgaacacaaatacccactgtgtgtcggcgagctggtctgctacatcagcccaggtttaaaatctaggcttactttctgttaacaaatcgcacgtggatgggcccccctggcgtcaggagcccgtgggtttttgcatgaacagcattggtctgagaagatgttttgatctcaaaatgttgaagcaactggatcacgacgaggtgaatctccagttctgcaattctccgccctatgcagctgcgaaccccatgaccaaaggggatggatccaaaattgtcaactctatctaagtctcctttccgcagccagcgctcaggccggaactccttggcccgagggaagttctcatcctggtacgatgtggcatagtggcaaagggccagctgggtgcctttcggaatcagatacccgccaataaccaggtcttcctgggtgacccggccgttccctggcagcactggaaacagcctcagggtttccttaaggagagctctgaccagcgggaccttggggacatcagctgcagttggaacatgcctttcccctaaattcttcacaatctcccggtacaccgtctgctgcacttctgggtgccttgccaggaggtacacagtccaagacaaggtgaaggacgtcgtgtcgacgccggccagcagcatctcagtcacgttggcgtagatctcctgcagcgtcagagcctggctaaggaagaggtatgtgagaagtcccccgctcaccctccggcctcggtccatttggtactgtatgtccctcaacttgttgtcaacatgaatttggctgaatttgaagagtccatcccaggacctgcagaattcccgccagggctttgggatgaaggggcgaagccatctggggatggcgcctgcatacatggaggtcttgaacatgctaaacatgagctccagggcctcgatgtattccacagtcagctgtgggatgctgttttccaggcagcccaaacgactctcataaaggatggtggccactccttccattgaatatttgaagaaaagatcattgacattggtcacggtttctccatcttctgcctggctcctgaggaggtagattcttttaattaagtcagcaataacttggttgacttctccagaataaatggccacatctttcggtttcagaattctttgtctcaatacgcttctcatcttgagccactgttcaccctccgccgagatgagcccggtggctctcccccgcaagtctcggtactcccgccaggactccatgttggctctctggggcgcagcgccctccgcccggagcacctgagccaccatatcgcggtctggatctcgtggatgcggctgaagccgtccctgcagaagaactccgccaggttggcgagggtcctcggccccggcatggc

SEQ ID NO: 14809 - RNA, 1476 nt, Homo sapiens
  source 1..1476: mol_type = other RNA
gctgggattacaggcatgagccacctcgcctggcctcttatctttcttaagtagtgttcttagttgttttcctttaagctgttaaaccccctcattcaatgatacctggaggattgagctgggctggatgttcaacaagatttgtgattccaaaataatcttctctcttgggattttcctagatcaaagccattggggattatgtaagagtcccaccactcaatttcaggaatatctccttcctttagctccttcttaggagcaatgagggcaagcctagtcgaagtatggatgcctgtttttcgagctgcttgtgaaatctctgcctgtagcttctccagttgagcctttgtccgtaatcgctgagcaatcttctcaaatttgcccttgtcatggaatttaaaagtgcgtctctggcgctgggaaggggcaatggagactcgggggtcaaaaaaggtattggattccatgtcttctgatggcttttcctttagttgttgcttgaattgttccctcttcacagcacgaatattggctttcagagtaggcatgcggtgtgtcagctcaatctccttgcctgttgcatctacagtgcgcccttgctcatccaggatcagtggtgtaggtttcgtttggtcttttaactccaccttcgggggagcaatgcccatggcatggagattagccaggcccaccatgttggcattgccgatgagtcctggcttcagtgccagctgggcttggattcgagcttgcagttcagctgctttccttgccttctcaatggcatcattcatgaaagtggcagcctgggagggctgaatagtgttgccaataggaagtcgttctggttgggaggaagaaggagtctttggctgaggtgtaggggggctaatgaagctcagctgttttttcctctcctcgatttgtcgtgttgctgcctccatcatctgtttgatctggagcttagtcagcatgccagggctctctgatggaggcccagggatcacctctggctcttcttccacctcctcaaaacggggtattcgtcgcttctttactcctgatgattctttagagatctcagagtcatcaccaaacacctcctttagctctcgttttctgctcctgtcactgctagacttggaatgcctagagcttcggccttcctccacagcctcaaacagtttgtccacaaatcggagagtagaatcatcaagaaaaggtttcagatgatcggctgccttcttcttgtccatgcccttccccacacagttcaatgctgctgtgaccaccgtaggctctgagaaacccaggaccctcttcactgtcttctctatccatggtttcagctcatccagctccctctttgacagtgccatttttcaggaaaaagagaacaatagctcaaacaggactcaatactacacctcacaaacttcagcccctgagacggagcccgaacgttacaccgga

SEQ ID NO: 14810 - RNA, 1481 nt, Homo sapiens
  source 1..1481: mol_type = other RNA
gctgggattacaggcatgagccacctcgcctggcctcttatctttcttaagtagtgttcttagttgttttcctttaagctgttaaaccccctcattcaatgatacctggaggattgagctgggctggatgttcaacaagatttgtgattccaaaataatcttctctcttgggattttcctctgtaagatcaaagccattggggattatgtaagagtcccaccactcaatttcaggaatatctccttcctttagctccttcttaggagcaatgagggcaagcctagtcgaagtatggatgcctgtttttcgagctgcttgtgaaatctctgcctgtagcttctccagttgagcctttgtccgtaatcgctgagcaatcttctcaaatttgcccttgtcatggaatttaaaagtgcgtctctggcgctgggaaggggcaatggagactcgggggtcaaaaaaggtattggattccatgtcttctgatggcttttcctttagttgttgcttgaattgttccctcttcacagcacgaatattggctttcagagtaggcatgcggtgtgtcagctcaatctccttgcctgttgcatctacagtgcgcccttgctcatccaggatcagtggtgtaggtttcgtttggtcttttaactccaccttcgggggagcaatgcccatggcatggagattagccaggcccaccatgttggcattgccgatgagtcctggcttcagtgccagctgggcttggattcgagcttgcagttcagctgctttccttgccttctcaatggcatcattcatgaaagtggcagcctgggagggctgaatagtgttgccaataggaagtcgttctggttgggaggaagaaggagtctttggctgaggtgtaggggggctaatgaagctcagctgttttttcctctcctcgatttgtcgtgttgctgcctccatcatctgtttgatctggagcttagtcagcatgccagggctctctgatggaggcccagggatcacctctggctcttcttccacctcctcaaaacggggtattcgtcgcttctttactcctgatgattctttagagatctcagagtcatcaccaaacacctcctttagctctcgttttctgctcctgtcactgctagacttggaatgcctagagcttcggccttcctccacagcctcaaacagtttgtccacaaatcggagagtagaatcatcaagaaaaggtttcagatgatcggctgccttcttcttgtccatgcccttccccacacagttcaatgctgctgtgaccaccgtaggctctgagaaacccaggaccctcttcactgtcttctctatccatggtttcagctcatccagctccctctttgacagtgccatttttcaggaaaaagagaacaatagctcaaacaggactcaatactacacctcacaaacttcagcccctgagacggagcccgaacgttacaccgga

SEQ ID NO: 14811 - RNA, 1314 nt, Homo sapiens
  source 1..1314: mol_type = other RNA
gctgggattacaggcatgagccacctcgcctggcctcttatctttcttaagtagtgttcttagttgttttcctttaagctgttaaaccccctcattcaatgatacctggaggattgagctgggctggatgttcaacaagatttgtgattccaaaataatcttctctcttgggattttcctctgtactttgtccgtaatcgctgagcaatcttctcaaatttgcccttgtcatggaatttaaaagtgcgtctctggcgctgggaaggggcaatggagactcgggggtcaaaaaaggtattggattccatgtcttctgatggcttttcctttagttgttgcttgaattgttccctcttcacagcacgaatattggctttcagagtaggcatgcggtgtgtcagctcaatctccttgcctgttgcatctacagtgcgcccttgctcatccaggatcagtggtgtaggtttcgtttggtcttttaactccaccttcgggggagcaatgcccatggcatggagattagccaggcccaccatgttggcattgccgatgagtcctggcttcagtgccagctgggcttggattcgagcttgcagttcagctgctttccttgccttctcaatggcatcattcatgaaagtggcagcctgggagggctgaatagtgttgccaataggaagtcgttctggttgggaggaagaaggagtctttggctgaggtgtaggggggctaatgaagctcagctgttttttcctctcctcgatttgtcgtgttgctgcctccatcatctgtttgatctggagcttagtcagcatgccagggctctctgatggaggcccagggatcacctctggctcttcttccacctcctcaaaacggggtattcgtcgcttctttactcctgatgattctttagagatctcagagtcatcaccaaacacctcctttagctctcgttttctgctcctgtcactgctagacttggaatgcctagagcttcggccttcctccacagcctcaaacagtttgtccacaaatcggagagtagaatcatcaagaaaaggtttcagatgatcggctgccttcttcttgtccatgcccttccccacacagttcaatgctgctgtgaccaccgtaggctctgagaaacccaggaccctcttcactgtcttctctatccatggtttcagctcatccagctccctctttgacagtgccatttttcaggaaaaagagaacaatagctcaaacaggactcaatactacacctcacaaacttcagcccctgagacggagcccgaacgttacaccgga

SEQ ID NO: 14812 - RNA, 1319 nt, Homo sapiens
  source 1..1319: mol_type = other RNA
gctgggattacaggcatgagccacctctcccagtctcagttattattttaataaatgagactgaacgtcctcttataaggctcactcccttgttcctactacatttgctctgtttaagtatctctttaaattcttcagttaagatcatcccttttatcagaaacctagacaccacaaagtagctttctcacctttaattctccatagggatcactattatactataatatttgcatacgtatgtgtatatatgtatttgcttttttaaaaaagtaaaaatgctcttctcactctttgtcgatataggcacccaggtacgtagttagaaattaaataaaggccacaataatttcccaaggaagatcattaaaaagaaaaatcctttcttcctctaatatcacatagctggcctttatggcatgccagctaagaaaaaaggtattgcctatggtgacaggaagactcaatctttctctctttgggttgtagctgaatttctatcaaaagtcctagtaaaatatataactcctcatttgttctaagccaagtcttttcttcagttttccttcaaacaatacctttactttcccattagaatatgaagaattggagactgtgaacagcaaggtttggggtgggtatcagtcacttcaaatctggctatgcagagagagggaaagacatggcagaatagcaggggtggagggtgagtgaaatgtatcttcattgggagtattgaaagagagcaagtttttcaaagttgttgccggtatctcatgaaagcccaggctgctaccatggtgagggcaaacactggcaccagcaccataaatatgggaataccacttgggtccccttcacctcgatgtcctataggtccattctgcacctgtaacctgtgctgcactctcagagacacagcatagcctgcattacgaaagaggtctacagcatcctggtgcagcaggttctttaggtcttggccatttaccgaaaggatcttatcaccctcctggagccgcccatccagggccgcagccccattttctttgatgcggctgacgtagatgccactgtcgttggagacatactgctgatctgtcccaccgacgatgttgaagcccagccctgagggccctctggtaagattgatctcttcctcagtgaccaaataatccactcttccgttcatgttttacagctcgtctggcttcctacttgggtcagctggagtgcagcacaggtgaaggtgaatcaatctcggcgctgcgcccacagcacagcggtttcggtttcagcagcctcgagacccggaaaag

SEQ ID NO: 14813 - RNA, 526 nt, Homo sapiens
  source 1..526: mol_type = other RNA
gctgggattacaggcatgagccacctggaggaattcttggccccggcctctgtgtccccgcagcactgggtctcgtttgtctctgtgactctgcactcatctttgaatcctgaatgtccagctgaaagcccaggagagtcgatgcttcatagaggaagccctgagccaccgtggatgtaacagcccatctcaaggcacccaagcagtttccaggctcacagcggctgccctgctagtcttggacctcttcctaatggcatcctgggtgtcagtgctggtgatggctggtactgctgacggtttcccactttctgcactcctgagaatctcggcaggcgtacctagaccggagcttctccaacttctccgagcctatgaatcacctgcagatccttcattcatgcaacttgggctttttcagattctgatacaggacacagcttctgttctgattctggcatgatcctgtagtcttggccatctcctccctcatgcaattcttgtgtcaattctaatgacctctctt

SEQ ID NO: 14814 - RNA, 730 nt, Homo sapiens
  source 1..730: mol_type = other RNA
gctgggattacaggcatgagccacctggaggaattcttggccccggcctctgtgtccccgcagcactgggtctcgtttgtctctgtgactctgcactcatctttgaatcctgaatgtccagctgaaagcccaggagagtcgatgcttcatagaggaagccctgagccaccgtggatgtaacagcccatctcaaggcacccaagcagtttccaggctcacagcggctgccctgctagtcttggacctcttcctaatggcatcctgggtgtcagtgctggtgatggctggtactgctgacggtttcccactttctgcactcctgagaatctcggcaggcgtacctagaccggagcttctccaacttctccgagcctatgaatcacctgcagatctggagtgctgttccgtccacagcctgccagacaggttctagacctgcaccagatacacatgctgtctgctactagcttctttgaggctaagagagcaaagtcatgattcaggttcccttataggcttatgaatgtcacatagaagaaacccatctttccagttgtctggatgacaaaatacaagctcttggccacagcagggtccttcattcatgcaacttgggctttttcagattctgatacaggacacagcttctgttctgattctggcatgatcctgtagtcttggccatctcctccctcatgcaattcttgtgtcaattctaatgacctctctt

SEQ ID NO: 14815 - RNA, 779 nt, Homo sapiens
  source 1..779: mol_type = other RNA
gctgggattacaggcatgagccacctggaggaattcttggccccggcctctgtgtccccgcagcactgggtctcgtttgtctctgtgactctgcactcatctttgaatcctgaatgtccagctgaaagcccaggagagtcgatgcttcatagaggaagccctgagccaccgtggatgtaacagcccatctcaaggcacccaagcagtttccaggctcacagcggctgccctgctagtcttggacctcttcctaatggcatcctgggtgtcagtgctggtgatggctggtactgctgacggtttcccactttctgcactcctgagaatctcggcaggcgtacctagaccggagcttctccaacttctccgagcctatgaatcacctgcagatctggagtgctgttccgtccacagcctgccagacaggttctagacctgcaccagatacacatgctgtctgctactagcttctttgaggctaagagagcaaagtcatgattcaggttcccttataggcttatgaatgtcacatagaagaaacccatctttccagttgtctggatgacaaaatacaagctcttggccacagcagggtctgagagaaagaatgtggatgtatcaggccaaccttcattcatgcaacttgggctttttcagattctgatacaggacacagcttctgttctgattctggcacacagagctgacgtgaacaggagtgtgcttgagggtggcgcttgacacaagtatcaatgtgcttttgtcttccagaaaaaaac

SEQ ID NO: 14816 - RNA, 762 nt, Homo sapiens
  source 1..762: mol_type = other RNA
gctgggattacaggcatgagccacctggaggaattcttggccccggcctctgtgtccccgcagcactgggtctcgtttgtctctgtgactctgcactcatctttgaatcctgaatgtccagctgaaagcccaggagagtcgatgcttcatagaggaagccctgagccaccgtggatgtaacagcccatctcaaggcacccaagcagtttccaggctcacagcggctgccctgctagtcttggacctcttcctaatggcatcctgggtgtcagtgctggtgatggctggtactgctgacggtttcccactttctgcactcctgagaatctcggcaggcgtacctagaccggagcttctccaacttctccgagcctatgaatcacctgcagatctggagtgctgttccgtccacagcctgccagacaggttctagacctgcaccagatacacatgctgtctgctactagcttctttgaggctaagagagcaaagtcatgattcaggttcccttataggcttatgaatgtcacatagaagaaacccatctttccagttgtctggatgacaaaatacaagctcttggccacagcagggtctgagagaaagaatgtggatgtatcaggccaaccttcattcatgcaacttgggctttttcagattctgatacaggacacagcttctgttctgattctggcatgatcctgtagtcttggccatctcctccctcatgcaattcttgtgtcaattctaatgacctctctt

SEQ ID NO: 14817 - RNA, 518 nt, Homo sapiens
  source 1..518: mol_type = other RNA
gctgggattacaggcatgagccaccttgcacagcctcagcccactttctctatagttttttccagagggaaggggggataattttttgtaatgtgattaaatttatcaaactttttttaatgacatgcatttttcatcacagctaaacatttttctcactcagaatatagagaaattcactcataatttcttattgtcctgaagaaattcttatgcataccaaagtgccagtttatgatccaagtttgtaaagtgatgtcaaacattgcattgtttaacatgagacatttaataatcagtcatgttcatagttttcttaattcttctaaatgatgtcaatctgatatcttcttgcctttctaagagaagacaacataaatcattatgatgcagcccacaatccagccaatcaggagaagaataggaaccagaaggtgtgaaaatgtagaccccgctttttcagccattattcctgttggtgggtggctaggtcaggccacgcttacctctttcttttg

SEQ ID NO: 14818 - RNA, 596 nt, Homo sapiens
  source 1..596: mol_type = other RNA
gctgggattacaggcatgagccaccttgcccggccccaattcggaattcttaacacagtcttctgagtagtgtcaccagttgatcatatcagaatttttgaaagccgttggctgtcctgtagactgtcccctccgacattgtccacagcaccaaatctggcctgcagatggtgtggggccatctcatcagcaggcaggtctgtcccaggtcctgattctgcccagggaactggcagttcctgagaagtgagaggtatgcagttacctctcaacacctcttcagtccgtatcccccagagcatttaaggtctttctctgtgtttctgaggtgcacatccttgttcctgtgactttgacacctctgttaatgggtctgtaataaaaattcctctggttcgggtgagtcccattcccatctctctcatttcaactgctccagtggaaatgtggtctggaatatgcatgaaaggggtggatccagaatgtacgaagaaaccaagaagaagcttttcacgggatctactcggatgtctgggatctggccactaccgcaggctcgagacaacccaggtgcgtatgcgccgcgcacacggaac

SEQ ID NO: 14819 - RNA, 3405 nt, Homo sapiens
  source 1..3405: mol_type = other RNA
gctgggattacaggcatgagccaccttgcccggccccaattcggaattcttaacacagtcttctgagtagtgtcaccagttgatcatatcagaatttttgaaagccgttggctgtcctgtagactgtcccctccgacattgtccacagcaccaaatctggcctgcagatggtgtggggccatctcatcagcaggcaggtctgtcccaggtcctgattctgcccagggaactggcagttcctgagaagtgagaggtatgcagttacctctcaacacctcttcagtccgtatcccccagagcatttaaggtctttcttcgctgcagaacgccttgccagcttgcttcctggctgggcctgctgtctgcacagttgccctgcccaggtctaagaccgtggggcgtggtcacaggtactattttaggactcctctcaccacaggcactgaacttggggctgcatatatatcaccccattactcctcagaagatactgtaacgtaggtatcttttattggctgtattgaggcttaatgcatccattttaggtgtacaatttgatgagttttgacaaaagtatagtcttgtaaccacaatcacgatgttcatgacacagaatattcccatcaccccaggaagaagttcctgcctctttgcagaccatcctcccctcttggcccctggctatatgttttgccttcactagaatttcatataaatgaaatttatgtaagatgtaatttttgtctggcttctttcactgagcacagtgcttctgaaattcgttcatgtcatcagtggtttgctcttttctctgctaaccagttgatgaatatttaggttgtttatgactattatgaataaagcgtgtagaaacatacatgtacaattatttgtgtgaacgtgttttcatttctcctgaggaaatacctaacactggaattgctgtttcattaagttattgttattcccattttatagataaaagattgaagctcaaagaggtgaagcagcttgcctgagctcacacagcatggcaaaaattcaaagccatgtctgagctctacaccaggtagtcacttgtacaaaaaaggtaatttttggagtcaaaggtccttgattggtagataaattaccacatatgggctgaattccactgtattctggtttgtagcttgtggaaatagacactgagcccaagttgctgagcactacacgcagagaggtcactctttgaaggcatttcagcaggtgacttctgggagcttaggctgcaggtctgcaaggtttttgttagtgttgtgaaggtagtgttggccaggtttctccactgtaaagtcatgattactccactataattactaaattgagaggagagacattgagactaagaatccgattcattgagctttcacccactagtttcaatacccagcgtgaattcctaactcctttcctttcccatttactagttgtattattctgttagggagagcttttccttcttcctcagttatgtttatataactatgtcctcaaggattttattctatggaatctaatccattaccatcattgttttaatgtttgatgtgttccaactttggccagaagcagtctcattaaactgacttctatgtccttttaacgtgctcctgtgattctctgagcacttccttactctcaggtataagatattccaagctcttgctcttctcctgtaccagccctggtcccttttagtagagaatgacatttagaaaccaagatctgggtgtgagatgaacttctgggtactgggatgtcacagcttctacgccacctcagtctgcaggtttttaaggcagcaagtgaggtgaaaggcagggccatgagattggagttgtaagctacggactcagcaaaatcaggctgctggtggtaggatgtctataacaagtgcagtgagctcactcatgggctcacagggtggtggaactgggcagtcagtccaaccaggcagtggtttctccactcagaaacacctctgtaggccgggcacggtgactcacgcctgtaatcccagcactttgggaggctgaggcaggcagatcacctgaggtcaggagttcaagaccagcctggccaacatggcaaaaaactctgtctctactaaaaatacaaaaattagctaggcgtggtggcatgcacctgtaatcccagctacttgggaggctgaggcaggagaatcacttgaacccgggaggcggaggttgcagtgagccaaaattgtgccactgcactccagcctgggcaacagagtgagactctgcctcaaaaaaaaaaaaaaaaaaaaagaaagaaagaaagaaagaaacacctttgtaaattttacacatttataaatctttcagctctttctgccttgctgtaaattacttccatgacagaggacctgggaggctggttttctaggatggtgggagggtcagggacagtgtgggggacacatggagaagggtggcctcaggggcttcacattgtggactgccacggtgatgggaaacttcacagatctctcttggcagacactctgctgtcctcaaggctgatcagctggctggcttgggagagagccaatgactggaggggacctcaggaatcagaggtggtgactcatagtgggaggccacagtctcagagtctggttctctgaaaagaaccacgccttccgatggtgtttggcaccttccattctgaagggcctgctggctctggggtccaccggggctgaggcagtcctgggcctgttgtgggcagtgggtgggaacaagtgccatctatctccagtggctttcatgtgcgtcaccctgctggcctccaccacaatcttgggagcaggatgcctttttttgtcttccagacattgaggctgagaagagcaggcacaggtctccgccgactctcgtgttcttcacagtgcagcctggccagagttacctggcccagctggcagccggcgtgtgaggccacagggagcctgctctctgaaactgagcagccttggcagtctggagggcccaggggacagtggcattctgcttctcaggacagactctgtgcagctgagcttcagccaggctagcctctgtgtttctgaggtgcacatccttgttcctgtgactttgacacctctgttaatgggtctgtaataaaaattcctctggttcgggtgagtcccattcccatctctctcatttcaactgctccagtggaaatgtggtctggaatatgcatgaaaggggtggatccagaatgtacgaagaaaccaagaagaagcttttcacgggatctactcggatgtctgggatctggccactaccgcaggctcgagacaacccaggtgcgtatgcgccgcgcacacggaac

SEQ ID NO: 14820 - RNA, 3298 nt, Homo sapiens
  source 1..3298: mol_type = other RNA
gctgggattacaggcatgagccaccttgccctccaggattcacattatttatgaagataaaacagtccagagaagcccctataccgggcaatttatttactgcctcttatttaatattcacaatatatttctagggaatgggctcatttataggtaaacatttatagatgtataagggaggctcagtgacatgagaaaagccacctgctggaaggtcaggcatggagggaaggagaagggctgatcttgcccaatccctgccctggaccagaaccaaaggctgagcaagtagaggaggtcctacctgtgatgtgcaggattctagggatgcccagtcacaggggagctcttggcctgtttggtgatactgcccacctgttgtactagtgagagagaggcactttgtacgtcctcaccctgcacacatttgtggctctgataaacttggagtagccaagaactagcccagcccccagatctggtgggggtgggcgatgctcctgagtccaagtgatccagttggccaggggcatctggttctcagtgtcagtaccagtccagatgagccccccatcccatgagctctccccatgattggagtttgagtatttttatctagaatctaacaagatccctgatgtaataataataataataataataataataataataatgggagaggggctgagtgagaaactgaggaggagggagccttgataagtccttgggctccaggcccctggaagaccttccctgcagaatggacccttccacctgggtgggtgtatacctggttctcaggggcagggggcagccagggagagagaggacactgatgccctcacacagctgctcctgttccagcagctcaaggcctgatccaagacacagaagaagccaatatgtctgcccctcaaactgggtggtaagcaagccccccaggggacaccaagaagggggattcagacaccctagacgttacctcctccttcagtctggtcttcagtatgtttcttcccaaacacccattcctaccccaggacaggaaacccaagaccagaaaagtgtcttctcacttgtcactaactgggcacaaaaggaaggtctaaagatcgtgagtgggtgggtgaggggacaagtgaattataagtaaattaatgagtaagagaatgaatgaataaacaagttagcacataaatgagtggctaaatgaataaatgaatgaaaggatggatgggtggatgagtagatgaatgggtggatgaaaggaaggatgtgtagatggatgggtgaggatggatggatggatgggtaaatggatgaggatgagtggatgcaaggaaggaagacaggatggatggatgaatgggaatggatgaggatggatggatggatggagaataaattgatgtatgaatggatgaatggataggtgtgtggatgggaaaatggatagaagcaagaaagaatgggtggatggatggataggtgaggatgggtggatgagtggatgaggatggatggatgcatgcatagataggtggatgggtggatgaatgaatggatggatggatagatagaaggaaaaacaaatgcatggatgaatgagaatggatggctagatagaaagaaggaagaacaaatgcatggatgaatgagaatagatgcatggataaatggaggatggataaatggacagatggatggctgaatggatggacggatggatgaatggatggatggatagatggacggatggatggatggatggatggatggatggatggatggacggacaagtggatgaatggatggagggatggatggatggatggatggatggatggatggaatggatggatggattgatggatggatgaatagatgggtggatggatggatggatggatggatagatggataaggatggagggactaatggatggatggataaggattgatgaatgaatgaatggatgaataaatgaggatgaatggatgaatggatggctatagggaagaatagataaatggaaaggaggaaggaagagggaaaagtgacaacccaaagcatagattttaaggcaaggcaagagccatggtagaatccaagatgggctcccatccactccacccctaggaggtctggtatggaagctgtgaagtggaccttccaagccagggcacccctacttcctacaggccttcccagattgctgatcaagaccaagctactcatccctcagacaaacctatattccgcccccaaacacccccttgcaagcctagcccttcccagaggaagccctcagaggggcgcctgaccaccctcccagccacgaggtaccctgcctgaggctcgggacttgatgcgcagtttgtggggcagagagggctgacccagaccctcaggactgttccctggggcagggcaggtcaccccaggagacagacccatgggatcagcagtgggtgtcagcaacacatctgatggccctgaagcccggcatccagagggcactggtgaccacagcccccagcagggtctgagctctggtctggaccctacatgcccctccaagaggtgacagctgaagagggcaggtgggagggcagtctgcaaggccatgtcaattctgttgagggtaggagatgcagactcttggggggacctaggagaagtggccaagccagtccatctgggagccagcaggcagccccgacatcctggaatcccagcatccagggaacgtggccttaagaggcagctgtgagagccagacaaggatgagagtgcttcagccccaggccgggggtccccagtccagggggcttccaatagcagagcctgcaggggcaaggcccggggcccaccagtcaggggcaggaggccaaagcgaagcttgagcgccttcagctcacccttgagcagggcattctcctccatcagtgcagccagcctgccctcaatggctgcatcattgagacgtcgcttttccctggatctcttggctgcttcattgttcttcctccgcttctcccagtaaactgtgtccttcttttcttctggcatgaactcccgctggcgacgtatggaggggcccctgccccgagccccccacaaggtcttgctatgactctgagacacatctggcaggcccgagaaacccacatccatagctgcttggagaaccttattccttataggagaatcacaaagtacattgaaggctctgagaaatcctgctctggacgctgtctccccggtgagtcccacgtgagcctcatcagcctt

SEQ ID NO: 14821 - RNA, 3703 nt, Homo sapiens
  source 1..3703: mol_type = other RNA
gctgggattacaggcatgagccaccttgccctccaggattcacattatttatgaagataaaacagtccagagaagcccctataccgggcaatttatttactgcctcttatttaatattcacaatatatttctagggaatgggctcatttataggtaaacatttatagatgtataagggaggctcagtgacatgagaaaagccacctgctggaaggtcaggcatggagggaaggagaagggctgatcttgcccaatccctgccctggaccagaaccaaaggctgagcaagtagaggaggtcctacctgtgatgtgcaggattctagggatgcccagtcacaggggagctcttggcctgtttggtgatactgcccacctgttgtactagtgagagagaggcactttgtacgtcctcaccctgcacacatttgtggctctgataaacttggagtagccaagaactagcccagcccccagatctggtgggggtgggcgatgctcctgagtccaagtgatccagttggccaggggcatctggttctcagtgtcagtaccagtccagatgagccccccatcccatgagctctccccatgattggagtttgagtatttttatctagaatctaacaagatccctgatgtaataataataataataataataataataataataatgggagaggggctgagtgagaaactgaggaggagggagccttgataagtccttgggctccaggcccctggaagaccttccctgcagaatggacccttccacctgggtgggtgtatacctggttctcaggggcagggggcagccagggagagagaggacactgatgccctcacacagctgctcctgttccagcagctcaaggcctgatccaagacacagaagaagccaatatgtctgcccctcaaactgggtggtaagcaagccccccaggggacaccaagaagggggattcagacaccctagacgttacctcctccttcagtctggtcttcagtatgtttcttcccaaacacccattcctaccccaggacaggaaacccaagaccagaaaagtgtcttctcacttgtcactaactgggcacaaaaggaaggtctaaagatcgtgagtgggtgggtgaggggacaagtgaattataagtaaattaatgagtaagagaatgaatgaataaacaagttagcacataaatgagtggctaaatgaataaatgaatgaaaggatggatgggtggatgagtagatgaatgggtggatgaaaggaaggatgtgtagatggatgggtgaggatggatggatggatgggtaaatggatgaggatgagtggatgcaaggaaggaagacaggatggatggatgaatgggaatggatgaggatggatggatggatggagaataaattgatgtatgaatggatgaatggataggtgtgtggatgggaaaatggatagaagcaagaaagaatgggtggatggatggataggtgaggatgggtggatgagtggatgaggatggatggatgcatgcatagataggtggatgggtggatgaatgaatggatggatggatagatagaaggaaaaacaaatgcatggatgaatgagaatggatggctagatagaaagaaggaagaacaaatgcatggatgaatgagaatagatgcatggataaatggaggatggataaatggacagatggatggctgaatggatggacggatggatgaatggatggatggatagatggacggatggatggatggatggatggatggatggatggatggacggacaagtggatgaatggatggagggatggatggatggatggatggatggatggatggaatggatggatggattgatggatggatgaatagatgggtggatggatggatggatggatggatagatggataaggatggagggactaatggatggatggataaggattgatgaatgaatgaatggatgaataaatgaggatgaatggatgaatggatggctatagggaagaatagataaatggaaaggaggaaggaagagggaaaagtgacaacccaaagcatagattttaaggcaaggcaagagccatggtagaatccaagatgggctcccatccactccacccctaggaggtctggtatggaagctgtgaagtggaccttccaagccagggcacccctacttcctacaggccttcccagattgctgatcaagaccaagctactcatccctcagacaaacctatattccgcccccaaacacccccttgcaagcctagcccttcccagaggaagccctcagaggggcgcctgaccaccctcccagccacgaggtaccctgcctgaggctcgggacttgatgcgcagtttgtggggcagagagggctgacccagaccctcaggactgttccctggggcagggcaggtcaccccaggagacagacccatgggatcagcagtgggtgtcagcaacacatctgatggccctgaagcccggcatccagagggcactggtgaccacagcccccagcagggtctgagctctggtctggaccctacatgcccctccaagaggtgacagctgaagagggcaggtgggagggcagtctgcaaggccatgtcaattctgttgagggtaggagatgcagactcttggggggacctaggagaagtggccaagccagtccatctgggagccagcaggcagccccgacatcctggaatcccagcatccagggaacgtggccttaagaggcagctgtgagagccagacaaggatgagagtgcttcagccccaggccgggggtccccagtccagggggcttccaatagcagagcctgcaggggcaaggcccggggcccaccagtcaggggcaggaggccaaagcgaagcttgagcgccttcagctcacccttgagcagggcattctcctccatcagtgcagccagcctgccctcaatggctgcatcattgagacgtcgcttttccctggatctcttggctgcttcattgttcttcctccgcttctcccagtaaactgtgtccttcttttcttctggcatgaactcccgctggcgacgtatggaggggcccctgccccgagccccccacaaggtcttgctatgactctgagacacatctggcaggcccgagaaacccacatccatagctgcttggagaactgttgagaaggtcagcagacaagcccagggctcagttcaattggagttccaaggtaagattcttggaaacccagagggagacagaaggatgactgaaccttattccttataggagaatcacaaagtacattgaaggctctgagaaatccctcacaccaaaacttgcacatcaacgtctggcacattatttatcatcgcctatgaatttgggcattcgtcaccaaaactggaaacaactcacgtgtctcccgtttttagagcatagagggtaacttcctgatgttgccatggcatctgtaaaccgtcagggggctggtgggagtgtagcagtgaggacaatcagaggtcactcatgtcatcatcttggtcttgatgggtttgggccggcttctttacttgcttcctgctccttgctcctcctggctctccagtcttccacccaagccctcaggttcccctagagctctttcccacttcctagtccccagccatggcagagaactctgt

SEQ ID NO: 14822 - RNA, 3867 nt, Homo sapiens
  source 1..3867: mol_type = other RNA
gctgggattacaggcatgagccaccttgccctccaggattcacattatttatgaagataaaacagtccagagaagcccctataccgggcaatttatttactgcctcttatttaatattcacaatatatttctagggaatgggctcatttataggtaaacatttatagatgtataagggaggctcagtgacatgagaaaagccacctgctggaaggtcaggcatggagggaaggagaagggctgatcttgcccaatccctgccctggaccagaaccaaaggctgagcaagtagaggaggtcctacctgtgatgtgcaggattctagggatgcccagtcacaggggagctcttggcctgtttggtgatactgcccacctgttgtactagtgagagagaggcactttgtacgtcctcaccctgcacacatttgtggctctgataaacttggagtagccaagaactagcccagcccccagatctggtgggggtgggcgatgctcctgagtccaagtgatccagttggccaggggcatctggttctcagtgtcagtaccagtccagatgagccccccatcccatgagctctccccatgattggagtttgagtatttttatctagaatctaacaagatccctgatgtaataataataataataataataataataataataatgggagaggggctgagtgagaaactgaggaggagggagccttgataagtccttgggctccaggcccctggaagaccttccctgcagaatggacccttccacctgggtgggtgtatacctggttctcaggggcagggggcagccagggagagagaggacactgatgccctcacacagctgctcctgttccagcagctcaaggcctgatccaagacacagaagaagccaatatgtctgcccctcaaactgggtggtaagcaagccccccaggggacaccaagaagggggattcagacaccctagacgttacctcctccttcagtctggtcttcagtatgtttcttcccaaacacccattcctaccccaggacaggaaacccaagaccagaaaagtgtcttctcacttgtcactaactgggcacaaaaggaaggtctaaagatcgtgagtgggtgggtgaggggacaagtgaattataagtaaattaatgagtaagagaatgaatgaataaacaagttagcacataaatgagtggctaaatgaataaatgaatgaaaggatggatgggtggatgagtagatgaatgggtggatgaaaggaaggatgtgtagatggatgggtgaggatggatggatggatgggtaaatggatgaggatgagtggatgcaaggaaggaagacaggatggatggatgaatgggaatggatgaggatggatggatggatggagaataaattgatgtatgaatggatgaatggataggtgtgtggatgggaaaatggatagaagcaagaaagaatgggtggatggatggataggtgaggatgggtggatgagtggatgaggatggatggatgcatgcatagataggtggatgggtggatgaatgaatggatggatggatagatagaaggaaaaacaaatgcatggatgaatgagaatggatggctagatagaaagaaggaagaacaaatgcatggatgaatgagaatagatgcatggataaatggaggatggataaatggacagatggatggctgaatggatggacggatggatgaatggatggatggatagatggacggatggatggatggatggatggatggatggatggatggacggacaagtggatgaatggatggagggatggatggatggatggatggatggatggatggaatggatggatggattgatggatggatgaatagatgggtggatggatggatggatggatggatagatggataaggatggagggactaatggatggatggataaggattgatgaatgaatgaatggatgaataaatgaggatgaatggatgaatggatggctatagggaagaatagataaatggaaaggaggaaggaagagggaaaagtgacaacccaaagcatagattttaaggcaaggcaagagccatggtagaatccaagatgggctcccatccactccacccctaggaggtctggtatggaagctgtgaagtggaccttccaagccagggcacccctacttcctacaggccttcccagattgctgatcaagaccaagctactcatccctcagacaaacctatattccgcccccaaacacccccttgcaagcctagcccttcccagaggaagccctcagaggggcgcctgaccaccctcccagccacgaggtaccctgcctgaggctcgggacttgatgcgcagtttgtggggcagagagggctgacccagaccctcaggactgttccctggggcagggcaggtcaccccaggagacagacccatgggatcagcagtgggtgtcagcaacacatctgatggccctgaagcccggcatccagagggcactggtgaccacagcccccagcagggtctgagctctggtctggaccctacatgcccctccaagaggtgacagctgaagagggcaggtgggagggcagtctgcaaggccatgtcaattctgttgagggtaggagatgcagactcttggggggacctaggagaagtggccaagccagtccatctgggagccagcaggcagccccgacatcctggaatcccagcatccagggaacgtggccttaagaggcagctgtgagagccagacaaggatgagagtgcttcagccccaggccgggggtccccagtccagggggcttccaatagcagagcctgcaggggcaaggcccggggcccaccagtcaggggcaggaggccaaagcgaagcttgagcgccttcagctcacccttgagcagggcattctcctccatcagtgcagccagcctgccctcaatggctgcatcattgagacgtcgcttttccctggatctcttggctgcttcattgttcttcctccgcttctcccagtaaactgtgtccttcttttcttctggcatgaactcccgctggcgacgtatggaggggcccctgccccgagccccccacaaggtcttgctatgactctgagacacatctggcaggcccgagaaacccacatccatagctgcttggagaactgttgagaaggtcagcagacaagcccagggctcagttcaattggagttccaaggtaagattcttggaaacccagagggagacagaaggatgactgaaccttattccttataggagaatcacaaagtacattgaaggctctgagaaatctgcagacttgaccaactcttcatctttatttctgccttcctggcccaccagggcaggcatttgggtctgttttgttcgccgctgcaacccccagtgcttggaatggagcctggcacgcaggaggtgttcgttccgtaaatatttgttgaatgaatgaatccacacctcacaccaaaacttgcacatcaacgtctggcacattatttatcatcgcctatgaatttgggcattcgtcaccaaaactggaaacaactcacgtgtctcccgtttttagagcatagagggtaacttcctgatgttgccatggcatctgtaaaccgtcagggggctggtgggagtgtagcagtgaggacaatcagaggtcactcatgtcatcatcttggtcttgatgggtttgggccggcttctttacttgcttcctgctccttgctcctcctggctctccagtcttccacccaagccctcaggttcccctagagctctttcccacttcctagtccccagccatggcagagaactctgt

SEQ ID NO: 14823 - RNA, 2269 nt, Homo sapiens
  source 1..2269: mol_type = other RNA
gctgggattacaggcatgagccacgacacctggcctcagaagggatttctgaccccaagagggagagactcctaaaatttgaggttaaatgtcaaagtgtgtcactttctttaacagaatagagatttattaccttgtttccaagatgccatcaattataagatcacaagtttttgagaggaagtaaagaactacaattatattaatgaacccatcaattgcaagatatgttctgatttcagaatcattaaaatgtgaagaaatgtctatcttgcaattgaaaaaaaagcctataataataataatgttggctcctaggctgggcaccatagtccatgcctgtaatcccagcactttgggaggccaaagcagaaggatcacttgaggccaggggttcaagaccagcctgggcaacacagcgagaccccatctctacaaaaataaaaaataaaaaaattagcctggtgaggtgacacatacctgtagtcccagctactctggaggctgaggagggagcatcccttgagcccaggagttcaaggctgcagcgagctgtgagcgtgccactgcactccagcccaggtgacagattgaggctctgtctcaaaaaaaaaaaaaaaagaaaagaaaaaagaaaagaaaaagaatcctggttcccatttattaagcatctcctgggtgccaggcgctatactccagatgttttcctaagtccttcacttgttatagtgccccaatgaggcaggtgttatcatttccacttcatggttaggaaactgaatataaagaggttgagtcacttttccaaggccacacaaccaggaagtagggcttggatggtaggacttcttaattccagatactttctcttcttggtagattgttctccaggctaaggagtcacagacgaggttgctatagaatagaaatgggttgtgaatgtgttgctttgaacatgtcttgaatctgcaaggtgaccaggaaggacaaaggtaacatagatagagttgtaatctaattaatctccaaatactggtccttggagggaaggcattaacaggacagtcagcgtgctcagaatccagataaaggggagccaaagaccaagaccgtcagggttgatacagcccagagtgggagaaggaccctgatcagccaccaggatcattccaggcccacggacaacacaacaagctcctaccctagaggccactattctgcagagtcaccctattccatcactgactctttactaatgaagcagaaatcttttgaggataatttagttcttcttgcaacctttcttcaagaggggaaaatgtgctgagcaattgtcatgagccagcaggcagagatgtagtactggaacaagttatacgttaacaaggttttctggttagttagtccaagttagttcccctgtgcctggttatgggattgaatgttttgctctgtgaagcagtggatacggcgcttcatctgatatgaaccccgtgacagatcctattgtgatactctcagcagtgctccctgacacctggctcctgggctatctgtctatctgtctaactacagtgtgggggaaagccaagcccacattggtggattcccaacatagctctacctcatcagatgacaaaagaatgttctgcagctttttggtggggtggcggcagggatgtggacacagttggggtagggcagggcagacaaggttgaggattgctggaagcatcagagattgcgtcaaagatgtctctgtcgacctgaccagaagaagctcattgtgaagctgccagagagtgtgcctctgggtcttgactctggagaggctctttggacagtggtggagatagcgccagggtagaggtcatcgcgtctccacctggacgtcaacaggactgaaggtcacagttgctgggtgttggctgccgttgctgtttgggcccacggcagaaggggcggttggcttggggcccttgggctctagttcccgcctcgtcctcattttcctgttgtacatcttcagcaggatcagaaccacggtgaagatgatgatgacaaccaccacaacggcagcaacaatggctccagaactcttatacaggaagtcttctcccctggtggtcatgttcagtgagaagaaggtggtatcccccagaggggtggctgtggtcatctcgatcctgctctgtcgagccccgctcggcctcccgccggcaccgccgcgctcccagccagggtccccgccgccgcccggcgctgccac

SEQ ID NO: 14824 - RNA, 2795 nt, Homo sapiens
  source 1..2795: mol_type = other RNA
gctgggattacaggcatgagccacgatccttagtatctatgtaacagagtcatacaaatacgttgaactggtttgtcagtaaggttggcaatatggagaaagatggaaatttagacattaaaagatttaaaagtcaagttggtttttgctttagcttgtcattcatcattagttccagttccagactcaacttattcagctactgatgtgtagaacctaaagaattatggatgtttttctaaaagtaagggttggtttttttgggagggtggtttagacaacactctatgttttattactctttttagtggtggaatttttgttagtccttttgcaaattttgagaattttaacatctactttttccccctcgttctttccaaatgaaaactgttaccattatttctgttttgaaagtagtatcaaaggctgtctgtatttatgtgagcaacatgccaaatattttgatagcttgtactctatctctcccattccatattttggtataattattagggagcagatcagaaattttgctacatctgatcaataattatgatttttcttaaccttagaggaattagaactgtgtcattcagtgatgtgtaatactaatacatagttttaatatctttggttatttgaaccaccaaactctctagtagttaattttaagacttatgttaattatcaaaactgcagtgtctcactgtgtaaccatttctgaggcacctgtaaataatatctgatgttacagagatgatcccagaaaaagccttcagtgaaggaaaaaacttaaaacttactatacacgtagcctcatcaaatttgtttccccaaatgtagatatgagagaaagtgagatttgttttcattgattgtgaaagtgcaacaagtccttctccctctatgttgttgctgactactgacaacctgaaaccaataattccacaaggaaagaatacaaaaattagcaacatttattacaaacactttcttgtgtagtcttagcattattcttcagtatgttgtaatgtagtggtaaaaatactgaccatttaattcctaaaatccaagaaacttagttttctaattagatccttaaggtacttagtagagctaactacattttgaaagtcttctgttttatattattcagtaaatgtttgggtggatagcagatatatttttctggataaatgcatccaagtattttattctttagttcattcttacttttaaaagtcttgatcatattgaatgcttctgagttttctattagaattcaggataagtaatataagcaatgcaaattttctcattaatttgaaggaatcgttaatagaatcagtctaattgtaaaagacattacatttgaaaaatagaaatgtaaatgtttactgtaacttaatactatgtcagtttagaagctgagttttcatatttcattataatcttaagagttaaggggattgaggttagtatttaaaaatttgcttttctgttattttgattaaatataaaaccatactaacgctttaagactcctgttgtgtgaagtaagagtttcactgagatagtttgcgcctgcattttctattctgttaaaggaaagatctattacttccagggtagtgttgcttttcagtacatcagccaaatacaccattccatcatgagttattttgttgcagctgacatcaaggtagcgcaggctactgttcagatacagtgcatcacataactgttgtataccactgttttttatatcatgcttacacatgtgtagtgcaacaagacagtgattttctttcaacatgcggcctacatggactgtagactcttcctgttcactgtacagtataggtcggtttaggtttattgccttaattgcttggttttgagttagtactgtagcaaatgctatcacactttgcattcccagatcacagtcacccagatctaatttctctaatgatgaattaatttgcagcattgcagcaaaaaacattccacctttattttcaattttgtttccagtcattcttaggtatttcagagtccgattcttatgtagcactttagcaatcaattctccaccttcgggcccaatatcattaaacatgaggtttaagtaaatgagattaagttgtttctgaagcagtttcgcagcatagtatgcaccaacatcacatagaaggttatatccaacatccaaaccattaatatacagacaattctttaaaattttggaaagaatccaaaaatcttcacctgtaactctttctactggcactaagcgattgttaccagcaatgtttaatgtgattcctgctgctagcccctttttaatttcttcatccacttcttggagtatatgcaatataaaaggattaattttctgggatttttccatacacagattagaataatgtttctggagaccagattctggagattagtccgcctgcagctgtgaggcggctacacgagcctcggcgccagcctgcttcgagtcccgctggctgtgcctgcccgggccctgaggcctcactgctaaggcagtgaccgcctactctgtggaggtcctttgtcaccctgccctggttaaaggcagcctgagggagggcgtcctggctcctttgcagggaggagttcccgaggtttgaggggctccgctgctgagctagggctggggctacaaagaagattatgacaaagcccgctcctacaaagtgtgcaccggcctgccgggccagcgaagaagcagagtagcatcagcacatgataaaggc

SEQ ID NO: 14825 - RNA, 2955 nt, Homo sapiens
  source 1..2955: mol_type = other RNA
gctgggattacaggcatgagccacgatccttagtatctatgtaacagagtcatacaaatacgttgaactggtttgtcagtaaggttggcaatatggagaaagatggaaatttagacattaaaagatttaaaagtcaagttggtttttgctttagcttgtcattcatcattagttccagttccagactcaacttattcagctactgatgtgtagaacctaaagaattatggatgtttttctaaaagtaagggttggtttttttgggagggtggtttagacaacactctatgttttattactctttttagtggtggaatttttgttagtccttttgcaaattttgagaattttaacatctactttttccccctcgttctttccaaatgaaaactgttaccattatttctgttttgaaagtagtatcaaaggctgtctgtatttatgtgagcaacatgccaaatattttgatagcttgtactctatctctcccattccatattttggtataattattagggagcagatcagaaattttgctacatctgatcaataattatgatttttcttaaccttagaggaattagaactgtgtcattcagtgatgtgtaatactaatacatagttttaatatctttggttatttgaaccaccaaactctctagtagttaattttaagacttatgttaattatcaaaactgcagtgtctcactgtgtaaccatttctgaggcacctgtaaataatatctgatgttacagagatgatcccagaaaaagccttcagtgaaggaaaaaacttaaaacttactatacacgtagcctcatcaaatttgtttccccaaatgtagatatgagagaaagtgagatttgttttcattgattgtgaaagtgcaacaagtccttctccctctatgttgttgctgactactgacaacctgaaaccaataattccacaaggaaagaatacaaaaattagcaacatttattacaaacactttcttgtgtagtcttagcattattcttcagtatgttgtaatgtagtggtaaaaatactgaccatttaattcctaaaatccaagaaacttagttttctaattagatccttaaggtacttagtagagctaactacattttgaaagtcttctgttttatattattcagtaaatgtttgggtggatagcagatatatttttctggataaatgcatccaagtattttattctttagttcattcttacttttaaaagtcttgatcatattgaatgcttctgagttttctattagaattcaggataagtaatataagcaatgcaaattttctcattaatttgaaggaatcgttaatagaatcagtctaattgtaaaagacattacatttgaaaaatagaaatgtaaatgtttactgtaacttaatactatgtcagtttagaagctgagttttcatatttcattataatcttaagagttaaggggattgaggttagtatttaaaaatttgcttttctgttattttgattaaatataaaaccatactaacgctttaagactcctgttgtgtgaagtaagagtttcactgagatagtttgcgcctgcattttctattctgttaaaggaaagatctattacttccagggtagtgttgcttttcagtacatcagccaaatacaccattccatcatgagttattttgttgcagctgacatcaaggtagcgcaggctactgttcagatacagtgcatcacataactgttgtataccactgttttttatatcatgcttacacatgtgtagtgcaacaagacagtgattttctttcaacatgcggcctacatggactgtagactcttcctgttcactgtacagtataggtcggtttaggtttattgccttaattgcttggttttgagttagtactgtagcaaatgctatcacactttgcattcccagatcacagtcacccagatctaatttctctaatgatgaattaatttgcagcattgcagcaaaaaacattccacctttattttcaattttgtttccagtcattcttaggtatttcagagtccgattcttatgtagcactttagcaatcaattctccaccttcgggcccaatatcattaaacatgaggtttaagtaaatgagattaagttgtttctgaagcagtttcgcagcatagtatgcaccaacatcacatagaaggttatatccaacatccaaaccattaatatacagacaattctttaaaattttggaaagaatccaaaaatcttcacctgtaactctttctactggcactaagcgattgttaccagcaatgtttaatgtgattcctgctgctagcccctttttaatttcttcatccacttcttggagtatatgcaatataaaaggattaattttctgggatttttccatacacagattagaataatgtttctggagaccagattctggagattcgcgctggaccgccagggccgcgcccggagtactggcctgagtggaggcccaagccggggacctggccggcgcacgggcggcctcccgggagctccccatgctcctctcacccactggccgcggcggctgcgctgccatggcgaccgcgcgcgcacttacagtccgcctgcagctgtgaggcggctacacgagcctcggcgccagcctgcttcgagtcccgctggctgtgcctgcccgggccctgaggcctcactgctaaggcagtgaccgcctactctgtggaggtcctttgtcaccctgccctggttaaaggcagcctgagggagggcgtcctggctcctttgcagggaggagttcccgaggtttgaggggctccgctgctgagctagggctggggctacaaagaagattatgacaaagcccgctcctacaaagtgtgcaccggcctgccgggccagcgaagaagcagagtagcatcagcacatgataaaggc

SEQ ID NO: 14826 - RNA, 1234 nt, Homo sapiens
  source 1..1234: mol_type = other RNA
gctgggattacaggcatgagccacgctcccagcctctactgactttcttatccctccgaccttggcctgagcgttacccaaggaataaggaatgaccaaagattttgaagtggaaagagcgctggacgtggaagttggagagtatggttcggagcttagacatcttagctacttcccagagcctgagtttcttcatcctatggcacatgtaggatccacctttcttcactcggtctttcccagaagggggaccttttgggttaagcgtttcttcaacagaatgatgaacagtccaccagtctgaagtccattcccatgcgttccccactatgttgtataagccataaccattgggagggaaggcatcaacaggcgcagttccttggaagccatcctcaccagtgttggtcaccggaaactcgccctgccaaatgttggcataatgctggcctttgggctgcagtttgttgccccaggggaaaagtctattatgcaggcctcctcgacagctgtattcccactcagcttccgtgggcagccgcttccctgcccaagtgcagtaggcaaccgcatcattccaggacacatggagaactggatgatccggcctgtgcagaatagtagagtcaggcccttctgggtgtctccagttagcgcctttcacaggtaaccaccagggagcagctgcaactgcctgttgaatattggtcttcacttgctcactcaacatgccttcaaagacaaaggagtcgccaaacttctcagcctctgtcaaatagccagttgagttcacaaacttctcaaattcagtattactgacttcataggcatccatgtaaaaggcatcaatagtaactctcctcgcaggtgcttccccatcctgctttatctgaggatcatctgtgcccattgtaaatactccagcagggatggggaccatctttgagtgcgcgagttgccgctctccgggtacggggcccggagcgttagcctcccgcgagtatcggtgagcggctgccgaactgccatgggcgccaggccgctggggcgtgccgcagccgcaagaacccgcaagggaccccgcgcccgcaccggtcccggcctcctggctccctgccgctccacacagcagcgagagcagcagcagcaagaggacgagacccagctcagggcaacgtccacacaccagccctagtgcgggcgcagccatgttgtcccgcgggccatgtgaccc

SEQ ID NO: 14827 - RNA, 4853 nt, Homo sapiens
  source 1..4853: mol_type = other RNA
gctgggattacaggcatgagccacggcacccagccctgagtagactttctaatgagcgtaatatgggagaaagggcaggggtggttgtggaactctctctccagcgtttgagactcacatgaggtaaaagccacttcatcttatctggaggtcttgaggcaaagttggctataggctaaactatgaagctatctctccattacagcacctcactgaagcttaaagtgctaaatagtagggcaatatttcagaatttcaggtgtttgggagatagggaaggaatttttctggaattctgtcagcatggaggtgagtggggcctctatgggtaaacaagtctgtgggtttttgccttgccctccattgtcttctccactccacagtttatcccagaaatgtttccccaacactagcttcccagtctcactttgttctttgttcagggggaggataacaggagactatgaagatgactctaccccactggtgatcctggcctcaggatttatttcccatgtgacgcagagtgaggaggcacattcccatttttgagacctcatttcttgcaacatcaatttttctgattagcaccataaaaagttttaacaccatgaccgtttaggttagattactttgaggaaaaaggtagacacaatccaatcactttttttttcatttatagaagagcctacaattattttagtttttcattcatatgtgcatccttcacatgtcactatactttcagattaagctcagtggcacagagcttatttaaacaattctgaactgcaccatgaattaataggcttcccaagctttttcttccacgcccaagaaacttcaggcctttacctgagtaaaaactaaacttgactttaaaataagccaaaaccaaaataaaacccaaacaaccaaaccccattaaaataaaaagcaataaacctaagaacaagcatatatattgtggtggttctgtggtagacaaacgtaccagaagcctttgaagcttaacattattgaaggtttctgtacattactgggtaactaaaatcaactttcacttgatggaaagctgaaagttctgaaaaatgatttatactgactgtgggaaggttaaacctggggtctgatttaaagagggtggaggataggattgatagagagaaaacagagcccagatgtaaaagaggtatctctggtgcacagtgatatgcaaggcctatagacttggtaggtcaggatgctacaggggctaacaaggggaaactgatatttacaggatgtgtttactatgtgccaagcctttccctgaaaggcacctgaaatacaagataacatttgctaatcctcacaaccaccctatggtgtcataattattgtcctcattttactggtaaggaaaaggcagttatacatctcatttgaagcttaaagagcacaatatgtgaggaagactggatttgaacccaggaccatttcactccattaccgatattctttcccctgtattactacatttcccataaacctaattcatagttgctgtttaagtcgatctgaagttttggtatgatctttcaaagcctaaatctggacttataaaacacaatagatggtactctaggctgtagaacttcctttctgaggggagagaaaatttcatttacttggttttacagaaaactgaccagcttgagcagcttttcagggtttctttaagaatatggcaattgagagtgagtcaaaacatcttgtacaactataaaactgcagaagaatttgtctcatggcacagaaataaaagggtaactactacttttaaagtttagactgtgagttaaattgtcaacatgtttaccaagttcttattaggagctcttaacacaaaattttaaaacggtgtttaagtattcatttttttaaaagtaccaaaaagtatcattttaatagcttaacattccctcaataaatgaactatacttttgtacttcatgcttaagttagagtaaattgctttagttgtcagaatgtgctatgctatcttggttacacatctttttatctggaacagttcttccccagaccctctctcactcccaaaactggagttacatgactcccaaatacagtaccttgtattttccccatcacaccacgaatcctactataggataattgcttaattttctgtatcctttaatggtctttaagctctgcaggggcaagaactgtgtgcatattgttcaggacagtatccccagttgaccagcacagtatctggccctcaacaaatgtttgttgaatgaatgaattagaacagaagtcttaacatggaaacaatgatttatagcaatggccccaacagcaattttctagcttccaatgtgtcactaataatttcattagtatgtgtttcataagcagagatcctcatcaagatagcctgtgttcattaataaattttcaatgttttaatagtaagctcagagtgacccaatttattttgttcgtatacaatttataatgtagttgcattattccgtatttgtatacaaatctgctgttcaataagaacacattctctttactgtaccacagtacagtaaatggatccaatcccaattatgcattaaattgtgccaactgaataatcttaaaaactttatgtttaatgaagtaaatttgtcctagattttctagaaccttaactacaaatttatcagagaaatacggtattgcttttcaagaactagttgttcttaaatttaaaagaaaccattcagtagtgtttaaaaaaccaaacaactctgaaaataacccatcaaaacataatattaaaatcatttgatttctgttggaaaaccaggtaaacatagtttaaatgcgtttttgtctatgaaagcattcagaaaattctacttttcacaaaagaggtttatatcctacagctctttttaagaccgaaagtttaaaataaattttaattttattctttggctattatttatacctaataaatgagtcgctgatatcaattcacaatagatttattttacataaaagaaaaagcttgctgttaatgaaaaatccagtagaaaacagttctgctttaagttgaggctcaaaagtagaagctgcttattagtgaaacctcaataaaaagagaattttgtaagaaaacattcttggcatgaaagctctaacataaattctgtaatgaaatatttaccatgcaactttattggcagaaaggccagtttctgatggctggtattttcagtctcttaacacattaacatggaagatacttaacctgctttatttagagttaattgtatataaatacaaagtcatgatgggcaacctttccatagtccacctacttaattgagcagttctaagtaggtaattggcaccttgcccttctggtttcccctttcccccattagccagtctgaatccattccaacaacactgaacacagtgatcacctcatctgccagaagtgataattcagtactgtttgctgcatcataatcatagagaaccctggcctttctgctgccactacactccttaaggtcactgaggttggaaggagaggtgattactaggccacttgttgaagccatggcagaagaaccaatcgcatttggtaaaactgatggtacaggtgtcacagaagtctgattgttgttactaagataattggatggaaaacttcccagttgtttctggaggtccaacatatactggtaacactgtgcatagtaagtcatctgggcttctacaaagtcattcagacagcgaaggtgatgggcatgtgtactgctgattccctctagcagaagtctggtaatctctgcttgacgatcaaattcactttgagttattcttaattcctgttcagacataatgttatctccttcaaggcgagctgagtttagttgtgaatttctagtttctgcagcttttgccttttttagtctcgtttttgcagcatccaaatccagtctcttattttgcaatagtttcctttctttagcaattgttttgtaatctccttctataaagtttcttaaaggagtaagaaaatttaaggctgacgtttgaatcagttctctgtctgctgttccaattcttttttgggtttctccacatttaataagggcattaccataagctgttcctgggccaaactcagtccctgcatcaatcatatattgtcccaaaagttctgggttgtttatacgacttggagcttttctatccagtttctcataaacaaattcttctatcctggcatttggatttggctgcaataacacttcagtttgtttcattattttttctgtccatattttggtacattcagctttgctaaggaggttctctaagtgagcatccaattctgtcttctcagcctggccaagcttttcttctgtgaactgcacggcgcgactgaggaaggtgcctgcgtcggccgccagcttcttcacgttgaagtccatgatattcatcctaggcggcagccgggcggagccggccgacctagcggcggcgaggcggaggtgccgcggccgggctggggcgcagggctagagcggcgagggcagacgtggtaggtggagggaggcggcgccagccccgcagccgcagctgtcgtttccgtgaacggggaggatgaaggcggggcgagggaggagaacaagcgcgcggcggcagcgccaaggatgggtcagtcggctcggagaacggccgctaacgtcgacgatgggccccgcgggcgagccggagatggacgggcgaccccgccgtgtggacccgggtcccaagggaaaaacaagcgc

SEQ ID NO: 14828 - RNA, 4895 nt, Homo sapiens
  source 1..4895: mol_type = other RNA
gctgggattacaggcatgagccacggcacccagccctgagtagactttctaatgagcgtaatatgggagaaagggcaggggtggttgtggaactctctctccagcgtttgagactcacatgaggtaaaagccacttcatcttatctggaggtcttgaggcaaagttggctataggctaaactatgaagctatctctccattacagcacctcactgaagcttaaagtgctaaatagtagggcaatatttcagaatttcaggtgtttgggagatagggaaggaatttttctggaattctgtcagcatggaggtgagtggggcctctatgggtaaacaagtctgtgggtttttgccttgccctccattgtcttctccactccacagtttatcccagaaatgtttccccaacactagcttcccagtctcactttgttctttgttcagggggaggataacaggagactatgaagatgactctaccccactggtgatcctggcctcaggatttatttcccatgtgacgcagagtgaggaggcacattcccatttttgagacctcatttcttgcaacatcaatttttctgattagcaccataaaaagttttaacaccatgaccgtttaggttagattactttgaggaaaaaggtagacacaatccaatcactttttttttcatttatagaagagcctacaattattttagtttttcattcatatgtgcatccttcacatgtcactatactttcagattaagctcagtggcacagagcttatttaaacaattctgaactgcaccatgaattaataggcttcccaagctttttcttccacgcccaagaaacttcaggcctttacctgagtaaaaactaaacttgactttaaaataagccaaaaccaaaataaaacccaaacaaccaaaccccattaaaataaaaagcaataaacctaagaacaagcatatatattgtggtggttctgtggtagacaaacgtaccagaagcctttgaagcttaacattattgaaggtttctgtacattactgggtaactaaaatcaactttcacttgatggaaagctgaaagttctgaaaaatgatttatactgactgtgggaaggttaaacctggggtctgatttaaagagggtggaggataggattgatagagagaaaacagagcccagatgtaaaagaggtatctctggtgcacagtgatatgcaaggcctatagacttggtaggtcaggatgctacaggggctaacaaggggaaactgatatttacaggatgtgtttactatgtgccaagcctttccctgaaaggcacctgaaatacaagataacatttgctaatcctcacaaccaccctatggtgtcataattattgtcctcattttactggtaaggaaaaggcagttatacatctcatttgaagcttaaagagcacaatatgtgaggaagactggatttgaacccaggaccatttcactccattaccgatattctttcccctgtattactacatttcccataaacctaattcatagttgctgtttaagtcgatctgaagttttggtatgatctttcaaagcctaaatctggacttataaaacacaatagatggtactctaggctgtagaacttcctttctgaggggagagaaaatttcatttacttggttttacagaaaactgaccagcttgagcagcttttcagggtttctttaagaatatggcaattgagagtgagtcaaaacatcttgtacaactataaaactgcagaagaatttgtctcatggcacagaaataaaagggtaactactacttttaaagtttagactgtgagttaaattgtcaacatgtttaccaagttcttattaggagctcttaacacaaaattttaaaacggtgtttaagtattcatttttttaaaagtaccaaaaagtatcattttaatagcttaacattccctcaataaatgaactatacttttgtacttcatgcttaagttagagtaaattgctttagttgtcagaatgtgctatgctatcttggttacacatctttttatctggaacagttcttccccagaccctctctcactcccaaaactggagttacatgactcccaaatacagtaccttgtattttccccatcacaccacgaatcctactataggataattgcttaattttctgtatcctttaatggtctttaagctctgcaggggcaagaactgtgtgcatattgttcaggacagtatccccagttgaccagcacagtatctggccctcaacaaatgtttgttgaatgaatgaattagaacagaagtcttaacatggaaacaatgatttatagcaatggccccaacagcaattttctagcttccaatgtgtcactaataatttcattagtatgtgtttcataagcagagatcctcatcaagatagcctgtgttcattaataaattttcaatgttttaatagtaagctcagagtgacccaatttattttgttcgtatacaatttataatgtagttgcattattccgtatttgtatacaaatctgctgttcaataagaacacattctctttactgtaccacagtacagtaaatggatccaatcccaattatgcattaaattgtgccaactgaataatcttaaaaactttatgtttaatgaagtaaatttgtcctagattttctagaaccttaactacaaatttatcagagaaatacggtattgcttttcaagaactagttgttcttaaatttaaaagaaaccattcagtagtgtttaaaaaaccaaacaactctgaaaataacccatcaaaacataatattaaaatcatttgatttctgttggaaaaccaggtaaacatagtttaaatgcgtttttgtctatgaaagcattcagaaaattctacttttcacaaaagaggtttatatcctacagctctttttaagaccgaaagtttaaaataaattttaattttattctttggctattatttatacctaataaatgagtcgctgatatcaattcacaatagatttattttacataaaagaaaaagcttgctgttaatgaaaaatccagtagaaaacagttctgctttaagttgaggctcaaaagtagaagctgcttattagtgaaacctcaataaaaagagaattttgtaagaaaacattcttggcatgaaagctctaacataaattctgtaatgaaatatttaccatgcaactttattggcagaaaggccagtttctgatggctggtattttcagtctcttaacacattaacatggaagatacttaacctgctttatttagagttaattgtatataaatacaaagtcatgatgggcaacctttccatagtccacctacttaattgagcagttctaagtaggtaattggcaccttgcccttctggtttcccctttcccccattagccagtctgaatccattccaacaacactgaacacagtgatcacctcatctgccagaagtgataattcagtactgtttgctgcatcataatcatagagaaccctggcctttctgctgccactacactccttaaggtcactgaggttggaaggagaggtgattactaggccacttgttgaagccatggcagaagaaccaatcgcatttggtaaaactgatggtacaggtgtcacagaagtctgattgttgttactaagataattggatggaaaacttcccagttgtttctggaggtccaacatatactggtaacactgtgcatagtaagtcatctgggcttctacaaagtcattcagacagcgaaggtgatgggcatgtgtactgctgattccctctagcagaagtctggtaatctctgcttgacgatcaaattcactttgagttattcttaattcctgttcagacttcagccattttacatgcaggaagttgagcatgtaagagaaatttaccataatgttatctccttcaaggcgagctgagtttagttgtgaatttctagtttctgcagcttttgccttttttagtctcgtttttgcagcatccaaatccagtctcttattttgcaatagtttcctttctttagcaattgttttgtaatctccttctataaagtttcttaaaggagtaagaaaatttaaggctgacgtttgaatcagttctctgtctgctgttccaattcttttttgggtttctccacatttaataagggcattaccataagctgttcctgggccaaactcagtccctgcatcaatcatatattgtcccaaaagttctgggttgtttatacgacttggagcttttctatccagtttctcataaacaaattcttctatcctggcatttggatttggctgcaataacacttcagtttgtttcattattttttctgtccatattttggtacattcagctttgctaaggaggttctctaagtgagcatccaattctgtcttctcagcctggccaagcttttcttctgtgaactgcacggcgcgactgaggaaggtgcctgcgtcggccgccagcttcttcacgttgaagtccatgatattcatcctaggcggcagccgggcggagccggccgacctagcggcggcgaggcggaggtgccgcggccgggctggggcgcagggctagagcggcgagggcagacgtggtaggtggagggaggcggcgccagccccgcagccgcagctgtcgtttccgtgaacggggaggatgaaggcggggcgagggaggagaacaagcgcgcggcggcagcgccaaggatgggtcagtcggctcggagaacggccgctaacgtcgacgatgggccccgcgggcgagccggagatggacgggcgaccccgccgtgtggacccgggtcccaagggaaaaac

SEQ ID NO: 14829 - RNA, 4666 nt, Homo sapiens
  source 1..4666: mol_type = other RNA
gctgggattacaggcatgagccacggcacccagccctgagtagactttctaatgagcgtaatatgggagaaagggcaggggtggttgtggaactctctctccagcgtttgagactcacatgaggtaaaagccacttcatcttatctggaggtcttgaggcaaagttggctataggctaaactatgaagctatctctccattacagcacctcactgaagcttaaagtgctaaatagtagggcaatatttcagaatttcaggtgtttgggagatagggaaggaatttttctggaattctgtcagcatggaggtgagtggggcctctatgggtaaacaagtctgtgggtttttgccttgccctccattgtcttctccactccacagtttatcccagaaatgtttccccaacactagcttcccagtctcactttgttctttgttcagggggaggataacaggagactatgaagatgactctaccccactggtgatcctggcctcaggatttatttcccatgtgacgcagagtgaggaggcacattcccatttttgagacctcatttcttgcaacatcaatttttctgattagcaccataaaaagttttaacaccatgaccgtttaggttagattactttgaggaaaaaggtagacacaatccaatcactttttttttcatttatagaagagcctacaattattttagtttttcattcatatgtgcatccttcacatgtcactatactttcagattaagctcagtggcacagagcttatttaaacaattctgaactgcaccatgaattaataggcttcccaagctttttcttccacgcccaagaaacttcaggcctttacctgagtaaaaactaaacttgactttaaaataagccaaaaccaaaataaaacccaaacaaccaaaccccattaaaataaaaagcaataaacctaagaacaagcatatatattgtggtggttctgtggtagacaaacgtaccagaagcctttgaagcttaacattattgaaggtttctgtacattactgggtaactaaaatcaactttcacttgatggaaagctgaaagttctgaaaaatgatttatactgactgtgggaaggttaaacctggggtctgatttaaagagggtggaggataggattgatagagagaaaacagagcccagatgtaaaagaggtatctctggtgcacagtgatatgcaaggcctatagacttggtaggtcaggatgctacaggggctaacaaggggaaactgatatttacaggatgtgtttactatgtgccaagcctttccctgaaaggcacctgaaatacaagataacatttgctaatcctcacaaccaccctatggtgtcataattattgtcctcattttactggtaaggaaaaggcagttatacatctcatttgaagcttaaagagcacaatatgtgaggaagactggatttgaacccaggaccatttcactccattaccgatattctttcccctgtattactacatttcccataaacctaattcatagttgctgtttaagtcgatctgaagttttggtatgatctttcaaagcctaaatctggacttataaaacacaatagatggtactctaggctgtagaacttcctttctgaggggagagaaaatttcatttacttggttttacagaaaactgaccagcttgagcagcttttcagggtttctttaagaatatggcaattgagagtgagtcaaaacatcttgtacaactataaaactgcagaagaatttgtctcatggcacagaaataaaagggtaactactacttttaaagtttagactgtgagttaaattgtcaacatgtttaccaagttcttattaggagctcttaacacaaaattttaaaacggtgtttaagtattcatttttttaaaagtaccaaaaagtatcattttaatagcttaacattccctcaataaatgaactatacttttgtacttcatgcttaagttagagtaaattgctttagttgtcagaatgtgctatgctatcttggttacacatctttttatctggaacagttcttccccagaccctctctcactcccaaaactggagttacatgactcccaaatacagtaccttgtattttccccatcacaccacgaatcctactataggataattgcttaattttctgtatcctttaatggtctttaagctctgcaggggcaagaactgtgtgcatattgttcaggacagtatccccagttgaccagcacagtatctggccctcaacaaatgtttgttgaatgaatgaattagaacagaagtcttaacatggaaacaatgatttatagcaatggccccaacagcaattttctagcttccaatgtgtcactaataatttcattagtatgtgtttcataagcagagatcctcatcaagatagcctgtgttcattaataaattttcaatgttttaatagtaagctcagagtgacccaatttattttgttcgtatacaatttataatgtagttgcattattccgtatttgtatacaaatctgctgttcaataagaacacattctctttactgtaccacagtacagtaaatggatccaatcccaattatgcattaaattgtgccaactgaataatcttaaaaactttatgtttaatgaagtaaatttgtcctagattttctagaaccttaactacaaatttatcagagaaatacggtattgcttttcaagaactagttgttcttaaatttaaaagaaaccattcagtagtgtttaaaaaaccaaacaactctgaaaataacccatcaaaacataatattaaaatcatttgatttctgttggaaaaccaggtaaacatagtttaaatgcgtttttgtctatgaaagcattcagaaaattctacttttcacaaaagaggtttatatcctacagctctttttaagaccgaaagtttaaaataaattttaattttattctttggctattatttatacctaataaatgagtcgctgatatcaattcacaatagatttattttacataaaagaaaaagcttgctgttaatgaaaaatccagtagaaaacagttctgctttaagttgaggctcaaaagtagaagctgcttattagtgaaacctcaataaaaagagaattttgtaagaaaacattcttggcatgaaagctctaacataaattctgtaatgaaatatttaccatgcaactttattggcagaaaggccagtttctgatggctggtattttcagtctcttaacacattaacatggaagatacttaacctgctttatttagagttaattgtatataaatacaaagtcatgatgggcaacctttccatagtccacctacttaattgagcagttctaagtaggtaattggcaccttgcccttctggtttcccctttcccccattagccagtctgaatccattccaacaacactgaacacagtgatcacctcatctgccagaagtgataattcagtactgtttgctgcatcataatcatagagaaccctggcctttctgctgccactacactccttaaggtcactgaggttggaaggagaggtgattactaggccacttgttgaagccatggcagaagaaccaatcgcatttggtaaaactgatggtacaggtgtcacagaagtctgattgttgttactaagataattggatggaaaacttcccagttgtttctggaggtccaacatatactggtaacactgtgcatagtaagtcatctgggcttctacaaagtcattcagacagcgaaggtgatgggcatgtgtactgctgattccctctagcagaagtctggtaatctctgcttgacgatcaaattcactttgagttattcttaattcctgttcagatgaatttctagtttctgcagcttttgccttttttagtctcgtttttgcagcatccaaatccagtctcttattttgcaatagtttcctttctttagcaattgttttgtaatctccttctataaagtttcttaaaggagtaagaaaatttaaggctgacgtttgaatcagttctctgtctgctgttccaattcttttttgggtttctccacatttaataagggcattaccataagctgttcctgggccaaactcagtccctgcatcaatcatatattgtcccaaaagttctgggttgtttatacgacttggagcttttctatccagtttctcataaacaaattcttctatcctggcatctgcacggcgcgactgaggaaggtgcctgcgtcggccgccagcttcttcacgttgaagtccatgatattcatcctaggcggcagccgggcggagccggccgacctagcggcggcgaggcggaggtgccgcggccgggctggggcgcagggctagagcggcgagggcagacgtggtaggtggagggaggcggcgccagccccgcagccgcagctgtcgtttccgtgaacggggaggatgaaggcggggcgagggaggagaacaagcgcgcggcggcagcgccaaggatgggtcagtcggctcggagaacggccgctaacgtcgacgatgggccccgcgggcgagccggagatggacgggcgaccccgccgtgtggacccgggtcccaagggaaaaac

SEQ ID NO: 14830 - RNA, 4808 nt, Homo sapiens
  source 1..4808: mol_type = other RNA
gctgggattacaggcatgagccacggcacccagccctgagtagactttctaatgagcgtaatatgggagaaagggcaggggtggttgtggaactctctctccagcgtttgagactcacatgaggtaaaagccacttcatcttatctggaggtcttgaggcaaagttggctataggctaaactatgaagctatctctccattacagcacctcactgaagcttaaagtgctaaatagtagggcaatatttcagaatttcaggtgtttgggagatagggaaggaatttttctggaattctgtcagcatggaggtgagtggggcctctatgggtaaacaagtctgtgggtttttgccttgccctccattgtcttctccactccacagtttatcccagaaatgtttccccaacactagcttcccagtctcactttgttctttgttcagggggaggataacaggagactatgaagatgactctaccccactggtgatcctggcctcaggatttatttcccatgtgacgcagagtgaggaggcacattcccatttttgagacctcatttcttgcaacatcaatttttctgattagcaccataaaaagttttaacaccatgaccgtttaggttagattactttgaggaaaaaggtagacacaatccaatcactttttttttcatttatagaagagcctacaattattttagtttttcattcatatgtgcatccttcacatgtcactatactttcagattaagctcagtggcacagagcttatttaaacaattctgaactgcaccatgaattaataggcttcccaagctttttcttccacgcccaagaaacttcaggcctttacctgagtaaaaactaaacttgactttaaaataagccaaaaccaaaataaaacccaaacaaccaaaccccattaaaataaaaagcaataaacctaagaacaagcatatatattgtggtggttctgtggtagacaaacgtaccagaagcctttgaagcttaacattattgaaggtttctgtacattactgggtaactaaaatcaactttcacttgatggaaagctgaaagttctgaaaaatgatttatactgactgtgggaaggttaaacctggggtctgatttaaagagggtggaggataggattgatagagagaaaacagagcccagatgtaaaagaggtatctctggtgcacagtgatatgcaaggcctatagacttggtaggtcaggatgctacaggggctaacaaggggaaactgatatttacaggatgtgtttactatgtgccaagcctttccctgaaaggcacctgaaatacaagataacatttgctaatcctcacaaccaccctatggtgtcataattattgtcctcattttactggtaaggaaaaggcagttatacatctcatttgaagcttaaagagcacaatatgtgaggaagactggatttgaacccaggaccatttcactccattaccgatattctttcccctgtattactacatttcccataaacctaattcatagttgctgtttaagtcgatctgaagttttggtatgatctttcaaagcctaaatctggacttataaaacacaatagatggtactctaggctgtagaacttcctttctgaggggagagaaaatttcatttacttggttttacagaaaactgaccagcttgagcagcttttcagggtttctttaagaatatggcaattgagagtgagtcaaaacatcttgtacaactataaaactgcagaagaatttgtctcatggcacagaaataaaagggtaactactacttttaaagtttagactgtgagttaaattgtcaacatgtttaccaagttcttattaggagctcttaacacaaaattttaaaacggtgtttaagtattcatttttttaaaagtaccaaaaagtatcattttaatagcttaacattccctcaataaatgaactatacttttgtacttcatgcttaagttagagtaaattgctttagttgtcagaatgtgctatgctatcttggttacacatctttttatctggaacagttcttccccagaccctctctcactcccaaaactggagttacatgactcccaaatacagtaccttgtattttccccatcacaccacgaatcctactataggataattgcttaattttctgtatcctttaatggtctttaagctctgcaggggcaagaactgtgtgcatattgttcaggacagtatccccagttgaccagcacagtatctggccctcaacaaatgtttgttgaatgaatgaattagaacagaagtcttaacatggaaacaatgatttatagcaatggccccaacagcaattttctagcttccaatgtgtcactaataatttcattagtatgtgtttcataagcagagatcctcatcaagatagcctgtgttcattaataaattttcaatgttttaatagtaagctcagagtgacccaatttattttgttcgtatacaatttataatgtagttgcattattccgtatttgtatacaaatctgctgttcaataagaacacattctctttactgtaccacagtacagtaaatggatccaatcccaattatgcattaaattgtgccaactgaataatcttaaaaactttatgtttaatgaagtaaatttgtcctagattttctagaaccttaactacaaatttatcagagaaatacggtattgcttttcaagaactagttgttcttaaatttaaaagaaaccattcagtagtgtttaaaaaaccaaacaactctgaaaataacccatcaaaacataatattaaaatcatttgatttctgttggaaaaccaggtaaacatagtttaaatgcgtttttgtctatgaaagcattcagaaaattctacttttcacaaaagaggtttatatcctacagctctttttaagaccgaaagtttaaaataaattttaattttattctttggctattatttatacctaataaatgagtcgctgatatcaattcacaatagatttattttacataaaagaaaaagcttgctgttaatgaaaaatccagtagaaaacagttctgctttaagttgaggctcaaaagtagaagctgcttattagtgaaacctcaataaaaagagaattttgtaagaaaacattcttggcatgaaagctctaacataaattctgtaatgaaatatttaccatgcaactttattggcagaaaggccagtttctgatggctggtattttcagtctcttaacacattaacatggaagatacttaacctgctttatttagagttaattgtatataaatacaaagtcatgatgggcaacctttccatagtccacctacttaattgagcagttctaagtaggtaattggcaccttgcccttctggtttcccctttcccccattagccagtctgaatccattccaacaacactgaacacagtgatcacctcatctgccagaagtgataattcagtactgtttgctgcatcataatcatagagaaccctggcctttctgctgccactacactccttaaggtcactgaggttggaaggagaggtgattactaggccacttgttgaagccatggcagaagaaccaatcgcatttggtaaaactgatggtacaggtgtcacagaagtctgattgttgttactaagataattggatggaaaacttcccagttgtttctggaggtccaacatatactggtaacactgtgcatagtaagtcatctgggcttctacaaagtcattcagacagcgaaggtgatgggcatgtgtactgctgattccctctagcagaagtctggtaatctctgcttgacgatcaaattcactttgagttattcttaattcctgttcagatgaatttctagtttctgcagcttttgccttttttagtctcgtttttgcagcatccaaatccagtctcttattttgcaatagtttcctttctttagcaattgttttgtaatctccttctataaagtttcttaaaggagtaagaaaatttaaggctgacgtttgaatcagttctctgtctgctgttccaattcttttttgggtttctccacatttaataagggcattaccataagctgttcctgggccaaactcagtccctgcatcaatcatatattgtcccaaaagttctgggttgtttatacgacttggagcttttctatccagtttctcataaacaaattcttctatcctggcatttggatttggctgcaataacacttcagtttgtttcattattttttctgtccatattttggtacattcagctttgctaaggaggttctctaagtgagcatccaattctgtcttctcagcctggccaagcttttcttctgtgaactgcacggcgcgactgaggaaggtgcctgcgtcggccgccagcttcttcacgttgaagtccatgatattcatcctaggcggcagccgggcggagccggccgacctagcggcggcgaggcggaggtgccgcggccgggctggggcgcagggctagagcggcgagggcagacgtggtaggtggagggaggcggcgccagccccgcagccgcagctgtcgtttccgtgaacggggaggatgaaggcggggcgagggaggagaacaagcgcgcggcggcagcgccaaggatgggtcagtcggctcggagaacggccgctaacgtcgacgatgggccccgcgggcgagccggagatggacgggcgaccccgccgtgtggacccgggtcccaagggaaaaac

SEQ ID NO: 14831 - RNA, 4705 nt, Homo sapiens
  source 1..4705: mol_type = other RNA
gctgggattacaggcatgagccacggcacccagccctgagtagactttctaatgagcgtaatatgggagaaagggcaggggtggttgtggaactctctctccagcgtttgagactcacatgaggtaaaagccacttcatcttatctggaggtcttgaggcaaagttggctataggctaaactatgaagctatctctccattacagcacctcactgaagcttaaagtgctaaatagtagggcaatatttcagaatttcaggtgtttgggagatagggaaggaatttttctggaattctgtcagcatggaggtgagtggggcctctatgggtaaacaagtctgtgggtttttgccttgccctccattgtcttctccactccacagtttatcccagaaatgtttccccaacactagcttcccagtctcactttgttctttgttcagggggaggataacaggagactatgaagatgactctaccccactggtgatcctggcctcaggatttatttcccatgtgacgcagagtgaggaggcacattcccatttttgagacctcatttcttgcaacatcaatttttctgattagcaccataaaaagttttaacaccatgaccgtttaggttagattactttgaggaaaaaggtagacacaatccaatcactttttttttcatttatagaagagcctacaattattttagtttttcattcatatgtgcatccttcacatgtcactatactttcagattaagctcagtggcacagagcttatttaaacaattctgaactgcaccatgaattaataggcttcccaagctttttcttccacgcccaagaaacttcaggcctttacctgagtaaaaactaaacttgactttaaaataagccaaaaccaaaataaaacccaaacaaccaaaccccattaaaataaaaagcaataaacctaagaacaagcatatatattgtggtggttctgtggtagacaaacgtaccagaagcctttgaagcttaacattattgaaggtttctgtacattactgggtaactaaaatcaactttcacttgatggaaagctgaaagttctgaaaaatgatttatactgactgtgggaaggttaaacctggggtctgatttaaagagggtggaggataggattgatagagagaaaacagagcccagatgtaaaagaggtatctctggtgcacagtgatatgcaaggcctatagacttggtaggtcaggatgctacaggggctaacaaggggaaactgatatttacaggatgtgtttactatgtgccaagcctttccctgaaaggcacctgaaatacaagataacatttgctaatcctcacaaccaccctatggtgtcataattattgtcctcattttactggtaaggaaaaggcagttatacatctcatttgaagcttaaagagcacaatatgtgaggaagactggatttgaacccaggaccatttcactccattaccgatattctttcccctgtattactacatttcccataaacctaattcatagttgctgtttaagtcgatctgaagttttggtatgatctttcaaagcctaaatctggacttataaaacacaatagatggtactctaggctgtagaacttcctttctgaggggagagaaaatttcatttacttggttttacagaaaactgaccagcttgagcagcttttcagggtttctttaagaatatggcaattgagagtgagtcaaaacatcttgtacaactataaaactgcagaagaatttgtctcatggcacagaaataaaagggtaactactacttttaaagtttagactgtgagttaaattgtcaacatgtttaccaagttcttattaggagctcttaacacaaaattttaaaacggtgtttaagtattcatttttttaaaagtaccaaaaagtatcattttaatagcttaacattccctcaataaatgaactatacttttgtacttcatgcttaagttagagtaaattgctttagttgtcagaatgtgctatgctatcttggttacacatctttttatctggaacagttcttccccagaccctctctcactcccaaaactggagttacatgactcccaaatacagtaccttgtattttccccatcacaccacgaatcctactataggataattgcttaattttctgtatcctttaatggtctttaagctctgcaggggcaagaactgtgtgcatattgttcaggacagtatccccagttgaccagcacagtatctggccctcaacaaatgtttgttgaatgaatgaattagaacagaagtcttaacatggaaacaatgatttatagcaatggccccaacagcaattttctagcttccaatgtgtcactaataatttcattagtatgtgtttcataagcagagatcctcatcaagatagcctgtgttcattaataaattttcaatgttttaatagtaagctcagagtgacccaatttattttgttcgtatacaatttataatgtagttgcattattccgtatttgtatacaaatctgctgttcaataagaacacattctctttactgtaccacagtacagtaaatggatccaatcccaattatgcattaaattgtgccaactgaataatcttaaaaactttatgtttaatgaagtaaatttgtcctagattttctagaaccttaactacaaatttatcagagaaatacggtattgcttttcaagaactagttgttcttaaatttaaaagaaaccattcagtagtgtttaaaaaaccaaacaactctgaaaataacccatcaaaacataatattaaaatcatttgatttctgttggaaaaccaggtaaacatagtttaaatgcgtttttgtctatgaaagcattcagaaaattctacttttcacaaaagaggtttatatcctacagctctttttaagaccgaaagtttaaaataaattttaattttattctttggctattatttatacctaataaatgagtcgctgatatcaattcacaatagatttattttacataaaagaaaaagcttgctgttaatgaaaaatccagtagaaaacagttctgctttaagttgaggctcaaaagtagaagctgcttattagtgaaacctcaataaaaagagaattttgtaagaaaacattcttggcatgaaagctctaacataaattctgtaatgaaatatttaccatgcaactttattggcagaaaggccagtttctgatggctggtattttcagtctcttaacacattaacatggaagatacttaacctgctttatttagagttaattgtatataaatacaaagtcatgatgggcaacctttccatagtccacctacttaattgagcagttctaagtaggtaattggcaccttgcccttctggtttcccctttcccccattagccagtctgaatccattccaacaacactgaacacagtgatcacctcatctgccagaagtgataattcagtactgtttgctgcatcataatcatagagaaccctggcctttctgctgccactacactccttaaggtcactgaggttggaaggagaggtgattactaggccacttgttgaagccatggcagaagaaccaatcgcatttggtaaaactgatggtacaggtgtcacagaagtctgattgttgttactaagataattggatggaaaacttcccagttgtttctggaggtccaacatatactggtaacactgtgcatagtaagtcatctgggcttctacaaagtcattcagacagcgaaggtgatgggcatgtgtactgctgattccctctagcagaagtctggtaatctctgcttgacgatcaaattcactttgagttattcttaattcctgttcagattttgtcacctcctctgcccaaatcataatgttatctccttcaaggcgagctgagtttagttgtgaatttctagtttctgcagcttttgccttttttagtctcgtttttgcagcatccaaatccagtctcttattttgcaatagtttcctttctttagcaattgttttgtaatctccttctataaagtttcttaaaggagtaagaaaatttaaggctgacgtttgaatcagttctctgtctgctgttccaattcttttttgggtttctccacatttaataagggcattaccataagctgttcctgggccaaactcagtccctgcatcaatcatatattgtcccaaaagttctgggttgtttatacgacttggagcttttctatccagtttctcataaacaaattcttctatcctggcatctgcacggcgcgactgaggaaggtgcctgcgtcggccgccagcttcttcacgttgaagtccatgatattcatcctaggcggcagccgggcggagccggccgacctagcggcggcgaggcggaggtgccgcggccgggctggggcgcagggctagagcggcgagggcagacgtggtaggtggagggaggcggcgccagccccgcagccgcagctgtcgtttccgtgaacggggaggatgaaggcggggcgagggaggagaacaagcgcgcggcggcagcgccaaggatgggtcagtcggctcggagaacggccgctaacgtcgacgatgggccccgcgggcgagccggagatggacgggcgaccccgccgtgt

SEQ ID NO: 14832 - RNA, 4871 nt, Homo sapiens
  source 1..4871: mol_type = other RNA
gctgggattacaggcatgagccacggcacccagccctgagtagactttctaatgagcgtaatatgggagaaagggcaggggtggttgtggaactctctctccagcgtttgagactcacatgaggtaaaagccacttcatcttatctggaggtcttgaggcaaagttggctataggctaaactatgaagctatctctccattacagcacctcactgaagcttaaagtgctaaatagtagggcaatatttcagaatttcaggtgtttgggagatagggaaggaatttttctggaattctgtcagcatggaggtgagtggggcctctatgggtaaacaagtctgtgggtttttgccttgccctccattgtcttctccactccacagtttatcccagaaatgtttccccaacactagcttcccagtctcactttgttctttgttcagggggaggataacaggagactatgaagatgactctaccccactggtgatcctggcctcaggatttatttcccatgtgacgcagagtgaggaggcacattcccatttttgagacctcatttcttgcaacatcaatttttctgattagcaccataaaaagttttaacaccatgaccgtttaggttagattactttgaggaaaaaggtagacacaatccaatcactttttttttcatttatagaagagcctacaattattttagtttttcattcatatgtgcatccttcacatgtcactatactttcagattaagctcagtggcacagagcttatttaaacaattctgaactgcaccatgaattaataggcttcccaagctttttcttccacgcccaagaaacttcaggcctttacctgagtaaaaactaaacttgactttaaaataagccaaaaccaaaataaaacccaaacaaccaaaccccattaaaataaaaagcaataaacctaagaacaagcatatatattgtggtggttctgtggtagacaaacgtaccagaagcctttgaagcttaacattattgaaggtttctgtacattactgggtaactaaaatcaactttcacttgatggaaagctgaaagttctgaaaaatgatttatactgactgtgggaaggttaaacctggggtctgatttaaagagggtggaggataggattgatagagagaaaacagagcccagatgtaaaagaggtatctctggtgcacagtgatatgcaaggcctatagacttggtaggtcaggatgctacaggggctaacaaggggaaactgatatttacaggatgtgtttactatgtgccaagcctttccctgaaaggcacctgaaatacaagataacatttgctaatcctcacaaccaccctatggtgtcataattattgtcctcattttactggtaaggaaaaggcagttatacatctcatttgaagcttaaagagcacaatatgtgaggaagactggatttgaacccaggaccatttcactccattaccgatattctttcccctgtattactacatttcccataaacctaattcatagttgctgtttaagtcgatctgaagttttggtatgatctttcaaagcctaaatctggacttataaaacacaatagatggtactctaggctgtagaacttcctttctgaggggagagaaaatttcatttacttggttttacagaaaactgaccagcttgagcagcttttcagggtttctttaagaatatggcaattgagagtgagtcaaaacatcttgtacaactataaaactgcagaagaatttgtctcatggcacagaaataaaagggtaactactacttttaaagtttagactgtgagttaaattgtcaacatgtttaccaagttcttattaggagctcttaacacaaaattttaaaacggtgtttaagtattcatttttttaaaagtaccaaaaagtatcattttaatagcttaacattccctcaataaatgaactatacttttgtacttcatgcttaagttagagtaaattgctttagttgtcagaatgtgctatgctatcttggttacacatctttttatctggaacagttcttccccagaccctctctcactcccaaaactggagttacatgactcccaaatacagtaccttgtattttccccatcacaccacgaatcctactataggataattgcttaattttctgtatcctttaatggtctttaagctctgcaggggcaagaactgtgtgcatattgttcaggacagtatccccagttgaccagcacagtatctggccctcaacaaatgtttgttgaatgaatgaattagaacagaagtcttaacatggaaacaatgatttatagcaatggccccaacagcaattttctagcttccaatgtgtcactaataatttcattagtatgtgtttcataagcagagatcctcatcaagatagcctgtgttcattaataaattttcaatgttttaatagtaagctcagagtgacccaatttattttgttcgtatacaatttataatgtagttgcattattccgtatttgtatacaaatctgctgttcaataagaacacattctctttactgtaccacagtacagtaaatggatccaatcccaattatgcattaaattgtgccaactgaataatcttaaaaactttatgtttaatgaagtaaatttgtcctagattttctagaaccttaactacaaatttatcagagaaatacggtattgcttttcaagaactagttgttcttaaatttaaaagaaaccattcagtagtgtttaaaaaaccaaacaactctgaaaataacccatcaaaacataatattaaaatcatttgatttctgttggaaaaccaggtaaacatagtttaaatgcgtttttgtctatgaaagcattcagaaaattctacttttcacaaaagaggtttatatcctacagctctttttaagaccgaaagtttaaaataaattttaattttattctttggctattatttatacctaataaatgagtcgctgatatcaattcacaatagatttattttacataaaagaaaaagcttgctgttaatgaaaaatccagtagaaaacagttctgctttaagttgaggctcaaaagtagaagctgcttattagtgaaacctcaataaaaagagaattttgtaagaaaacattcttggcatgaaagctctaacataaattctgtaatgaaatatttaccatgcaactttattggcagaaaggccagtttctgatggctggtattttcagtctcttaacacattaacatggaagatacttaacctgctttatttagagttaattgtatataaatacaaagtcatgatgggcaacctttccatagtccacctacttaattgagcagttctaagtaggtaattggcaccttgcccttctggtttcccctttcccccattagccagtctgaatccattccaacaacactgaacacagtgatcacctcatctgccagaagtgataattcagtactgtttgctgcatcataatcatagagaaccctggcctttctgctgccactacactccttaaggtcactgaggttggaaggagaggtgattactaggccacttgttgaagccatggcagaagaaccaatcgcatttggtaaaactgatggtacaggtgtcacagaagtctgattgttgttactaagataattggatggaaaacttcccagttgtttctggaggtccaacatatactggtaacactgtgcatagtaagtcatctgggcttctacaaagtcattcagacagcgaaggtgatgggcatgtgtactgctgattccctctagcagaagtctggtaatctctgcttgacgatcaaattcactttgagttattcttaattcctgttcagattttgtcacctcctctgcccaaatcataatgttatctccttcaaggcgagctgagtttagttgtgaatttctagtttctgcagcttttgccttttttagtctcgtttttgcagcatccaaatccagtctcttattttgcaatagtttcctttctttagcaattgttttgtaatctccttctataaagtttcttaaaggagtaagaaaatttaaggctgacgtttgaatcagttctctgtctgctgttccaattcttttttgggtttctccacatttaataagggcattaccataagctgttcctgggccaaactcagtccctgcatcaatcatatattgtcccaaaagttctgggttgtttatacgacttggagcttttctatccagtttctcataaacaaattcttctatcctggcatttggatttggctgcaataacacttcagtttgtttcattattttttctgtccatattttggtacattcagctttgctaaggaggttctctaagtgagcatccaattctgtcttctcagcctggccaagcttttcttctgtgaactgcacggcgcgactgaggaaggtgcctgcgtcggccgccagcttcttcacgttgaagtccatgatattcatcctaggcggcagccgggcggagccggccgacctagcggcggcgaggcggaggtgccgcggccgggctggggcgcagggctagagcggcgagggcagacgtggtaggtggagggaggcggcgccagccccgcagccgcagctgtcgtttccgtgaacggggaggatgaaggcggggcgagggaggagaacaagcgcgcggcggcagcgccaaggatgggtcagtcggctcggagaacggccgctaacgtcgacgatgggccccgcgggcgagccggagatggacgggcgaccccgccgtgtggacccgggtcccaagggaaaaac

SEQ ID NO: 14833 - RNA, 4753 nt, Homo sapiens
  source 1..4753: mol_type = other RNA
gctgggattacaggcatgagccacggcacccagccctgagtagactttctaatgagcgtaatatgggagaaagggcaggggtggttgtggaactctctctccagcgtttgagactcacatgaggtaaaagccacttcatcttatctggaggtcttgaggcaaagttggctataggctaaactatgaagctatctctccattacagcacctcactgaagcttaaagtgctaaatagtagggcaatatttcagaatttcaggtgtttgggagatagggaaggaatttttctggaattctgtcagcatggaggtgagtggggcctctatgggtaaacaagtctgtgggtttttgccttgccctccattgtcttctccactccacagtttatcccagaaatgtttccccaacactagcttcccagtctcactttgttctttgttcagggggaggataacaggagactatgaagatgactctaccccactggtgatcctggcctcaggatttatttcccatgtgacgcagagtgaggaggcacattcccatttttgagacctcatttcttgcaacatcaatttttctgattagcaccataaaaagttttaacaccatgaccgtttaggttagattactttgaggaaaaaggtagacacaatccaatcactttttttttcatttatagaagagcctacaattattttagtttttcattcatatgtgcatccttcacatgtcactatactttcagattaagctcagtggcacagagcttatttaaacaattctgaactgcaccatgaattaataggcttcccaagctttttcttccacgcccaagaaacttcaggcctttacctgagtaaaaactaaacttgactttaaaataagccaaaaccaaaataaaacccaaacaaccaaaccccattaaaataaaaagcaataaacctaagaacaagcatatatattgtggtggttctgtggtagacaaacgtaccagaagcctttgaagcttaacattattgaaggtttctgtacattactgggtaactaaaatcaactttcacttgatggaaagctgaaagttctgaaaaatgatttatactgactgtgggaaggttaaacctggggtctgatttaaagagggtggaggataggattgatagagagaaaacagagcccagatgtaaaagaggtatctctggtgcacagtgatatgcaaggcctatagacttggtaggtcaggatgctacaggggctaacaaggggaaactgatatttacaggatgtgtttactatgtgccaagcctttccctgaaaggcacctgaaatacaagataacatttgctaatcctcacaaccaccctatggtgtcataattattgtcctcattttactggtaaggaaaaggcagttatacatctcatttgaagcttaaagagcacaatatgtgaggaagactggatttgaacccaggaccatttcactccattaccgatattctttcccctgtattactacatttcccataaacctaattcatagttgctgtttaagtcgatctgaagttttggtatgatctttcaaagcctaaatctggacttataaaacacaatagatggtactctaggctgtagaacttcctttctgaggggagagaaaatttcatttacttggttttacagaaaactgaccagcttgagcagcttttcagggtttctttaagaatatggcaattgagagtgagtcaaaacatcttgtacaactataaaactgcagaagaatttgtctcatggcacagaaataaaagggtaactactacttttaaagtttagactgtgagttaaattgtcaacatgtttaccaagttcttattaggagctcttaacacaaaattttaaaacggtgtttaagtattcatttttttaaaagtaccaaaaagtatcattttaatagcttaacattccctcaataaatgaactatacttttgtacttcatgcttaagttagagtaaattgctttagttgtcagaatgtgctatgctatcttggttacacatctttttatctggaacagttcttccccagaccctctctcactcccaaaactggagttacatgactcccaaatacagtaccttgtattttccccatcacaccacgaatcctactataggataattgcttaattttctgtatcctttaatggtctttaagctctgcaggggcaagaactgtgtgcatattgttcaggacagtatccccagttgaccagcacagtatctggccctcaacaaatgtttgttgaatgaatgaattagaacagaagtcttaacatggaaacaatgatttatagcaatggccccaacagcaattttctagcttccaatgtgtcactaataatttcattagtatgtgtttcataagcagagatcctcatcaagatagcctgtgttcattaataaattttcaatgttttaatagtaagctcagagtgacccaatttattttgttcgtatacaatttataatgtagttgcattattccgtatttgtatacaaatctgctgttcaataagaacacattctctttactgtaccacagtacagtaaatggatccaatcccaattatgcattaaattgtgccaactgaataatcttaaaaactttatgtttaatgaagtaaatttgtcctagattttctagaaccttaactacaaatttatcagagaaatacggtattgcttttcaagaactagttgttcttaaatttaaaagaaaccattcagtagtgtttaaaaaaccaaacaactctgaaaataacccatcaaaacataatattaaaatcatttgatttctgttggaaaaccaggtaaacatagtttaaatgcgtttttgtctatgaaagcattcagaaaattctacttttcacaaaagaggtttatatcctacagctctttttaagaccgaaagtttaaaataaattttaattttattctttggctattatttatacctaataaatgagtcgctgatatcaattcacaatagatttattttacataaaagaaaaagcttgctgttaatgaaaaatccagtagaaaacagttctgctttaagttgaggctcaaaagtagaagctgcttattagtgaaacctcaataaaaagagaattttgtaagaaaacattcttggcatgaaagctctaacataaattctgtaatgaaatatttaccatgcaactttattggcagaaaggccagtttctgatggctggtattttcagtctcttaacacattaacatggaagatacttaacctgctttatttagagttaattgtatataaatacaaagtcatgatgggcaacctttccatagtccacctacttaattgagcagttctaagtaggtaattggcaccttgcccttctggtttcccctttcccccattagccagtctgaatccattccaacaacactgaacacagtgatcacctcatctgccagaagtgataattcagtactgtttgctgcatcataatcatagagaaccctggcctttctgctgccactacactccttaaggtcactgaggttggaaggagaggtgattactaggccacttgttgaagccatggcagaagaaccaatcgcatttggtaaaactgatggtacaggtgtcacagaagtctgattgttgttactaagataattggatggaaaacttcccagttgtttctggaggtccaacatatactggtaacactgtgcatagtaagtcatctgggcttctacaaagtcattcagacagcgaaggtgatgggcatgtgtactgctgattccctctagcagaagtctggtaatctctgcttgacgatcaaattcactttgagttattcttaattcctgttcagattttgtcacctcctctgcccaaatcttcagccattttacatgcaggaagttgagcatgtaagagaaatttaccataatgttatctccttcaaggcgagctgagtttagttgtgaatttctagtttctgcagcttttgccttttttagtctcgtttttgcagcatccaaatccagtctcttattttgcaatagtttcctttctttagcaattgttttgtaatctccttctataaagtttcttaaaggagtaagaaaatttaaggctgacgtttgaatcagttctctgtctgctgttccaattcttttttgggtttctccacatttaataagggcattaccataagctgttcctgggccaaactcagtccctgcatcaatcatatattgtcccaaaagttctgggttgtttatacgacttggagcttttctatccagtttctcataaacaaattcttctatcctggcatctgcacggcgcgactgaggaaggtgcctgcgtcggccgccagcttcttcacgttgaagtccatgatattcatcctaggcggcagccgggcggagccggccgacctagcggcggcgaggcggaggtgccgcggccgggctggggcgcagggctagagcggcgagggcagacgtggtaggtggagggaggcggcgccagccccgcagccgcagctgtcgtttccgtgaacggggaggatgaaggcggggcgagggaggagaacaagcgcgcggcggcagcgccaaggatgggtcagtcggctcggagaacggccgctaacgtcgacgatgggccccgcgggcgagccggagatggacgggcgaccccgccgtgt

SEQ ID NO: 14834 - RNA, 4925 nt, Homo sapiens
  source 1..4925: mol_type = other RNA
gctgggattacaggcatgagccacggcacccagccctgagtagactttctaatgagcgtaatatgggagaaagggcaggggtggttgtggaactctctctccagcgtttgagactcacatgaggtaaaagccacttcatcttatctggaggtcttgaggcaaagttggctataggctaaactatgaagctatctctccattacagcacctcactgaagcttaaagtgctaaatagtagggcaatatttcagaatttcaggtgtttgggagatagggaaggaatttttctggaattctgtcagcatggaggtgagtggggcctctatgggtaaacaagtctgtgggtttttgccttgccctccattgtcttctccactccacagtttatcccagaaatgtttccccaacactagcttcccagtctcactttgttctttgttcagggggaggataacaggagactatgaagatgactctaccccactggtgatcctggcctcaggatttatttcccatgtgacgcagagtgaggaggcacattcccatttttgagacctcatttcttgcaacatcaatttttctgattagcaccataaaaagttttaacaccatgaccgtttaggttagattactttgaggaaaaaggtagacacaatccaatcactttttttttcatttatagaagagcctacaattattttagtttttcattcatatgtgcatccttcacatgtcactatactttcagattaagctcagtggcacagagcttatttaaacaattctgaactgcaccatgaattaataggcttcccaagctttttcttccacgcccaagaaacttcaggcctttacctgagtaaaaactaaacttgactttaaaataagccaaaaccaaaataaaacccaaacaaccaaaccccattaaaataaaaagcaataaacctaagaacaagcatatatattgtggtggttctgtggtagacaaacgtaccagaagcctttgaagcttaacattattgaaggtttctgtacattactgggtaactaaaatcaactttcacttgatggaaagctgaaagttctgaaaaatgatttatactgactgtgggaaggttaaacctggggtctgatttaaagagggtggaggataggattgatagagagaaaacagagcccagatgtaaaagaggtatctctggtgcacagtgatatgcaaggcctatagacttggtaggtcaggatgctacaggggctaacaaggggaaactgatatttacaggatgtgtttactatgtgccaagcctttccctgaaaggcacctgaaatacaagataacatttgctaatcctcacaaccaccctatggtgtcataattattgtcctcattttactggtaaggaaaaggcagttatacatctcatttgaagcttaaagagcacaatatgtgaggaagactggatttgaacccaggaccatttcactccattaccgatattctttcccctgtattactacatttcccataaacctaattcatagttgctgtttaagtcgatctgaagttttggtatgatctttcaaagcctaaatctggacttataaaacacaatagatggtactctaggctgtagaacttcctttctgaggggagagaaaatttcatttacttggttttacagaaaactgaccagcttgagcagcttttcagggtttctttaagaatatggcaattgagagtgagtcaaaacatcttgtacaactataaaactgcagaagaatttgtctcatggcacagaaataaaagggtaactactacttttaaagtttagactgtgagttaaattgtcaacatgtttaccaagttcttattaggagctcttaacacaaaattttaaaacggtgtttaagtattcatttttttaaaagtaccaaaaagtatcattttaatagcttaacattccctcaataaatgaactatacttttgtacttcatgcttaagttagagtaaattgctttagttgtcagaatgtgctatgctatcttggttacacatctttttatctggaacagttcttccccagaccctctctcactcccaaaactggagttacatgactcccaaatacagtaccttgtattttccccatcacaccacgaatcctactataggataattgcttaattttctgtatcctttaatggtctttaagctctgcaggggcaagaactgtgtgcatattgttcaggacagtatccccagttgaccagcacagtatctggccctcaacaaatgtttgttgaatgaatgaattagaacagaagtcttaacatggaaacaatgatttatagcaatggccccaacagcaattttctagcttccaatgtgtcactaataatttcattagtatgtgtttcataagcagagatcctcatcaagatagcctgtgttcattaataaattttcaatgttttaatagtaagctcagagtgacccaatttattttgttcgtatacaatttataatgtagttgcattattccgtatttgtatacaaatctgctgttcaataagaacacattctctttactgtaccacagtacagtaaatggatccaatcccaattatgcattaaattgtgccaactgaataatcttaaaaactttatgtttaatgaagtaaatttgtcctagattttctagaaccttaactacaaatttatcagagaaatacggtattgcttttcaagaactagttgttcttaaatttaaaagaaaccattcagtagtgtttaaaaaaccaaacaactctgaaaataacccatcaaaacataatattaaaatcatttgatttctgttggaaaaccaggtaaacatagtttaaatgcgtttttgtctatgaaagcattcagaaaattctacttttcacaaaagaggtttatatcctacagctctttttaagaccgaaagtttaaaataaattttaattttattctttggctattatttatacctaataaatgagtcgctgatatcaattcacaatagatttattttacataaaagaaaaagcttgctgttaatgaaaaatccagtagaaaacagttctgctttaagttgaggctcaaaagtagaagctgcttattagtgaaacctcaataaaaagagaattttgtaagaaaacattcttggcatgaaagctctaacataaattctgtaatgaaatatttaccatgcaactttattggcagaaaggccagtttctgatggctggtattttcagtctcttaacacattaacatggaagatacttaacctgctttatttagagttaattgtatataaatacaaagtcatgatgggcaacctttccatagtccacctacttaattgagcagttctaagtaggtaattggcaccttgcccttctggtttcccctttcccccattagccagtctgaatccattccaacaacactgaacacagtgatcacctcatctgccagaagtgataattcagtactgtttgctgcatcataatcatagagaaccctggcctttctgctgccactacactccttaaggtcactgaggttggaaggagaggtgattactaggccacttgttgaagccatggcagaagaaccaatcgcatttggtaaaactgatggtacaggtgtcacagaagtctgattgttgttactaagataattggatggaaaacttcccagttgtttctggaggtccaacatatactggtaacactgtgcatagtaagtcatctgggcttctacaaagtcattcagacagcgaaggtgatgggcatgtgtactgctgattccctctagcagaagtctggtaatctctgcttgacgatcaaattcactttgagttattcttaattcctgttcagattttgtcacctcctctgcccaaatcttcagccattttacatgcaggaagttgagcatgtaagagaaatttaccataatgttatctccttcaaggcgagctgagtttagttgtgaatttctagtttctgcagcttttgccttttttagtctcgtttttgcagcatccaaatccagtctcttattttgcaatagtttcctttctttagcaattgttttgtaatctccttctataaagtttcttaaaggagtaagaaaatttaaggctgacgtttgaatcagttctctgtctgctgttccaattcttttttgggtttctccacatttaataagggcattaccataagctgttcctgggccaaactcagtccctgcatcaatcatatattgtcccaaaagttctgggttgtttatacgacttggagcttttctatccagtttctcataaacaaattcttctatcctggcatttggatttggctgcaataacacttcagtttgtttcattattttttctgtccatattttggtacattcagctttgctaaggaggttctctaagtgagcatccaattctgtcttctcagcctggccaagcttttcttctgtgaactgcacggcgcgactgaggaaggtgcctgcgtcggccgccagcttcttcacgttgaagtccatgatattcatcctaggcggcagccgggcggagccggccgacctagcggcggcgaggcggaggtgccgcggccgggctggggcgcagggctagagcggcgagggcagacgtggtaggtggagggaggcggcgccagccccgcagccgcagctgtcgtttccgtgaacggggaggatgaaggcggggcgagggaggagaacaagcgcgcggcggcagcgccaaggatgggtcagtcggctcggagaacggccgctaacgtcgacgatgggccccgcgggcgagccggagatggacgggcgaccccgccgtgtggacccgggtcccaagggaaaaacaagcgc

SEQ ID NO: 14835 - RNA, 2333 nt, Homo sapiens
  source 1..2333: mol_type = other RNA
gctgggattacaggcatgagccacggcgccaggctgcatggtcattttttagggagctgggaaaactggacatgcccccaagccccagggtcttccaaatccgattgcagcccccacatggccaatgctgtatcagcaggtgggcccgggaccctgctcatcccttcagccccatcctgcccctgcaaccttgcccgggggcaggtgcccccttcgatgatctcaggtcagcatgacaaatcgtttggagacctgggcaatctggtttaacttaaaccttctcctaggacacaagccctggcagaaatccactggtaaaatgacacccgggcaacagtcaaggttttatttccagttaggtcccaggatgggggaagggagaggagaagtcacaggccattgatcccaactgtcatcccctagggagaccatatcccacaccccagggcctgggccatgcctcttttcctccttcaccctggagtcctgggaagttgatttgagaagatgctaggaacacaatgaaagccaattcatccgatccagttttcaagggttatttattaaaccccttggttctgaccccaagctaagtgggactcagcatcagaccctgcactcagagagccccctgacttggggaagacagagtcagagaaaggcagccccagtgtggccagggctcagctggaaggaaggacaaggggctgggagaacccagagttcaagagatctgggaaacagggaacggcattccagacggagggcacaccttgggcatgggtaaggaaagcccatcgtgtgttctaggaagcatggatggatgaaacggggtcccagccgctatggacagccccgagtttcacctgtaaaaggcaggattatttgtttttaattttaattttaatttttttgagacagtcttgctctgtcgcccaggctagagtgcagtggcacgatcttggctcaccgcaagctccgcctcccaagttcacgccattctcctgcctcagcctcccgagttgctgggactacaggtgcccaccaccacgcctggctaattttttatatttttagtagagacagggtttcaccatgttagccaagatggtctcgatctcctgacctcgtgatccgcccacctgggcctcccaaagtgctgggattacaggcgtgagcccccgcacccggccaaaggcaggattatttgttaagcgggttgcagtgttctaccagaccccccaccctcaacccaagcccctggtctcactgggacttggccactgccaggagcgtctggcccttcacggcttcaggcccagcacagcgcgtgtcattctgggaaaacatcttgtctttttgggcctgaagccaacgatagaggtcgctcaggttctggtcacagatccaggggttgccggagatgtcgaagccatcccgcatgtcccagtttggctgccctagggatgcccagagcccctcgggcacgctggccagtgagttattggagaggtccagcatgtccagctgccgcaggccctggaaggcaccggctgccaccctggccagcttgttgccgttcaggaagaggtagcgcaggtccggctgcggcaagaggagatcttttcccagtacttgcaatttgttgccttctagatgtagccgttctaattgcagcggacccctcaggaggtcaggtggcaaggtctccaactggttctccccaaggtcaagggtgcgcaggagggtgaagttggccagcagcccggggggcagtttccggaggcggttcccagacaggtccagatgccccagagctttcaggccgtgtagccacgagacctccaggacctccagctggttttctttcaataccagggtgtccagggtggctgaggcctggaagaggcccgggggcagcccggtcagggcgtttcgggttagatccagcaccctcagctgcggcactggccgcaggaattcgggcgagaggctttccagcccattgctggagaggtgcaattcttggagcttagaggcgccctggaggaggttggctggcaggtgggtcaggttgaagaattccacggccaggtgcacggtgtcggctggcaggtagccggggatttcggcaggtggttgacaggagatggagctgccatggtctgagcggaacacctggcagtctttggggctcagggtgaccccccaggctgaggctgccaacagcagcagcaggaacagagttctagaaacatggggttgaatgccccctgggctttttggtcgctgtctgctccaagaggacatggtagctctgctcttttgcttct

SEQ ID NO: 14836 - RNA, 2953 nt, Homo sapiens
  source 1..2953: mol_type = other RNA
gctgggattacaggcatgagccacggcgccctgcccaagctactgttattaactattttgttcaaagagggatagctgacttctgaatgtggtgcaggggaaacctgcattcaggtacagcatctgcactagggaaggtgagagaaaatctgtagctgctccatgtacatgagacatcagagcactagccggtttggtggtctgtcttccagctcgaagcatgcaaatggcacagcccagcctcttagatccaccaaatgctaccactggaagggaccttccagaccagcatttctcaacacccacagggattcacagctgttccataatccagagatcctgcagtcagataaacttgggcagcacaggtctagatcaagtcaaacaggtttctttattttggaacttcttggagccattactgtgcccacacatatcaagaaactgctgaagggaccaaattgtgcatttctctctaatgtccttgacattagagcatttctagaccagtgttcttccagccatacttttcgaaaccttaattaaaagcagcatctctcagacttgaccatgtgcctggtgatcacctggggggctggttacagtgtcgtttattggatgcctctcccagagttttggcatttctgacaagttcccaggtgatgccgttggtccaggaacctgagaaccactggtctaggcttaccccttcattccccagagaagaaaacagtccaaccagagagtatttgctttcagtagtgactattaattgagccagtcacctgctaagcacttttcgtgactctttctaagggcaagtatgatagtgggattcagcccctagaaaggggatagcgcaatgcaaatcattactgtagagttttaccctgtgccagtcactcaccactgcagaagggttggtacttcaggcagggcgtcctcccgagactagtcaaggtcttcctgtccttggcatcagtattaggaacataaattctgtctgtatttaatcctctgggccttcatttttcatctatggacgatctgaggggaagagaaaattcgggtccttgtgttccacttgtccagttgagaaattcacgtggaactctgcccatggtcgttaattccaagttaggaacttgggccaaatgcttaaagtcaacccaaacttctcttctgagcaaaaaggaaggccgagccgtgccattcccacgtgcttctaaatggccagcagagccaccagaaacgggcagaggcgagaacatgacttcaacttggtgtttctggtggatatgttttcagacacccagaagaactgcgaagagacagcttctctgtatagcatccctcggagatgctgcagacttggttccaggccatcgcaataaagcaaatatcacagtaaagtgggtcacacaaatgttttggtttcccagtgcatattaaaatgtttatgctacatgatagtagaaagtgagcaatagcattatgtcttaaagaatccaattatatactttaatttaaaatatattattgccaaaaagtgagcacatgctgttggaaaaacggcaccaacagatctgcttgaagcagggttcccacaaaccttcaatatggaaaagaaactccactgtatctgtgaaaacacataaagcaagtacaataaaatgaggtgtgcctgtaatatgaccgtccaacacaagtaaccttccatcagtgttcccacaaacactgtatcctcaacatgtcacccgatgatgcaaccccagtaccttgagatggggtatatggaggatttgctcttacatgtagtagactgagtgggtcgaggcttaacaaaagaaactgcaagtgaatgagataaagctacggaattttgttgagtacagcaatttagtgagtcacttcattttgctagatcttcatttctgaaatgaattttagacaaaataactgaaatcaattatcaggccagcccacgaagtactgctgagcacaggcattgctagaagtcacaaccaataacacaactggcagtaagcgccttatcacagagatggagaacctgatcacagagcccacgacggaggccctgatgcccatctccctgcaaagcagatgagatgtccaaactgtacttccagacctggcccataaaataagatggagtgtggagatcacaaaagtaggtacctacctggagataagctaactctagattttttacaggaaagctagtttcatgccataagatattaaagctcttccttaccagaaaaaaaccttatacaaagcaagacaggctgtatttcctgtgttctaaattatcgtgggaacctcagttacatcctctcctgccatgttttggggcttggaggtaagaaagaggtaaagcaaacagataacactgtaaagggatgagaggtaagtagaaaagagaaaacaactgaaaaagcaaaaaaaggttctttgtcgtctgcacaaagcacttcctgctctgggtttccatcatgccttttctgagaaccaacacctcgtttcctaatccactactatcccatgctgtgacgggaggaccatgaccaccagcacaaaggaccacagcagaacataaacagtgcaggtgaggaaaatgcaaactttgccgtagaaagcagaaccatgtgaatttcccgtgagtcaccctcactctaaagaacactcacatatttggtaatggctctcatgagctgggccggtgacagagggcatctccaccagaaccatctccggtcaggccacatgagggtggaggcatggtatagctgacgttcaggttgacgaggagacactacaaaggcttgccatcctggaatttaccaaacccaagaagctggacactgatactttttttttttttttaagacggagtctcgttctgtcaccaggctggagtgcagtggcacga

SEQ ID NO: 14837 - RNA, 6382 nt, Homo sapiens
  source 1..6382: mol_type = other RNA
gctgggattacaggcatgagccacggcgcctgaccacacctggctaatctttttaaaaagtttttgtacagacagggtctccctatattggtcaggcttgtctcgaactcctgggttccagcaatcctccagcctcagccttcccaagtgctggtattacatggatgagccactgcacctggctaattttactttaaaggaatctttctactattttatcattaagtatgacatttgtgttttcagaacatatattccctaccaagttacaggagttaattttaattcccaacttaatagtattttagtgtcatctatgggtgttaaattccatcaagtgatttatcagcatatactgagataatccttatgagttttatctggtagttaattaaaatattttctaatattaaatcttccaaacatactcttctgttttttgagacagggtctagttctgtcacccagggtggagtacagtggtacgatctcagctcactgcaacttccgcctcctagattcaagtgattctcccgtcccagcctcccaagtagctgggattataggtgtcagttaccatgccctgctatttttttgtatttttagtagagaggggtttcaccatgttggccaggctggtctcaaactcctgacctcaggtgatccaccatctcagcctcctgaagtgctgggattataggtgtgagccaccgtgcctggccccatatatctctttttaagtgggcatactgccattataaataatagtgattctgctggtaatgaacaaaggatgctggatccactaatagtctgttaaacctaatatcatgactttcttgttagctatacattggtttgctataattccatttagaatttttaaacctatgttcacaaatatggatttttaaacctatgttcacaaatatggatttttaaacctatgttcacaaatatggtttgcaagtcattttttctcctaaatttctatttgatggggaagttgtaaaatattggggttatttttccttggattttccttataataactattcctgaaaagtctctggaatgtctttcttttctggggctggggtagaaggactagatagatttacaaaccagtaactcaatttctgttttgtaaaattttcatttcattaaataataagtcctaatcaagtattattctttcccacagtatgtgagtgctgtcctcaatactgtcaacacttctggcttctaccaggcaaggctgcatgtagatttgcatctgaaaaaacaacaaactaaaatctaaccctaggtagtagtaaactgaatataaactttctcttatgaatttattctgtcttctttggtacatcaataataatatacacctttacagtatttcccagattgggggatacactttagcaagtatctgcgattatttgtttatgtaagatgtcccttcccttctgtgaatcatcattcttcaccccaagtatcttgagattggattctgtataagcagaatacaacagttaggcattcaggtatcattaaattcctccgcttcaaggatgaaaatttctttgggtatctaatagagtacaaagcagaaggtgtttcagaaatatttgcagtattgaatccgcatattcctccaagatagccctaatctaactggcagggtcccactcttcccagattaatgcccactcacataacaaacctgatgaggtagtgaagaaaactaactttgtgagtaagcaactggcagagtttttcaccactgtgactctatagctacatgtaactaagtagtatcactgacacataatcttaaattgaagttttaagatcattattctccatgttatacatgggtatcaaaagcattcccctcttgaccactccagaattctgtttaaaatttttcaatgacaacttatccatttccccaaagcctcagtgagcacatgatgccaacaattcatttcatgacttcatagcatgggccaagtttcttgcttaaaagacttccatcctgtcttgggaaacaaccatttccaaatatccacatatccttgcaagtttctgcctactcctctaccacccatttctgaagccatctgatttagtaagctgtatgcaaaagatacacaatggctaatgcaatcaaacaaggaatgtattaaaagcacacccaatagctcaaaataaaagacaagtgaacaaagttaagaaaatgacagtaacaaaagctgttctgggaacctctattgaaatagctacttattacatcaacatgctaccacagaacaaaagctcatgttgcttttctgaacttgaaaaacccattaacaatgtacagttctgagcctcagctgaccatagtgctcatgccaagtcctgagcagggcatcttgaatggtggttccctcatgactacatacaccgttagggaatgtttcgttaagaggaaatcaagatgttctaacctgtgaaggtagaatagattccaggctacacaaacacatgaagtgtgccttatattgattactaaagaggttgctgccaagactgcttccaaagggcagaagatagccctaaaaaatgtttgcagtgtggaaatgcatttttagtaagtcatattctagtaacaagttgcatttggtaagacacaaagaaacaatgttggtatgcagagtagaaatctctggaagatgatattgtcatatcagagatattgtcagtatcagagatactgaaatctctggaagatgatttttgtctcacatatggcattcgcaagtaaaatgccaaactgcaaaattcatattatgtagtacacataggaagatatctaaatatccctgtaggctctgggatgttatttcttattcttaacctccttactagattcacttgtacaatgaaataatctgtatcttattatttataattgagaattttctcaaaccttttcctgaaattttggaacacctggaataaaatttcttaaaatgattcctaaaagaaataattcttcaaaattaatattaagatataataacaggttggtttttttttttttttttttttttttttttagaatgaagcttctaaggtgaggttaacagtccagctgtggtttatttggtacattcataagatgttcactcctatatatattttttccctaggggtttctcatttctagatttacactttcccttatagcatggtccctccaaggtatatgcttccgatacataaaatgtttgtaattttgttaattctgccattcattagctcaataatttctctcattaaaattctgtaaactatgaatttcaaagaagtctattctatattcatctggttcatgaagtttcctctttgtgaatcttattttagtaaaatgactttacaacgtttaacatggttcctcacctgtatgaactttttaaaaaaaggtatgacttgctgctaaaaattttcagagtggttactaaattcagttttcctgtgtattgtctactatctttttgcatgtaaagaacagctttctgtggatgcctttccatatgctgtgcattcataaagtttctattcagtatgagttttctggaagatgacaagatgattccacttacagagtttctctttatatatgattgtttctatctcttgtgaatccacttttcagagtttcgtaaaattatcaatgtttgtcatctacatgagttctctgatgcataatgagctgtgacttccaacaaaaggctttcccacattcagtgcacttacaaggcttctctcctgtatgtgttctctgatgtgcactgagaattgatttttgagagaaggttttcccacattcattgcacccatagggtttctctcctgaatgagttctttgatgtacaatgagttgagaattcctaatgaaggcttttccacactcactgcattcatatggtttctctcttgtgtgcattctctggtgtacaagaaggcgtaatttcccactgaaggatttctcacattgactgcatttataagggttgacccctgcatgagttcgctcatgtacaatgagtagtgatttccaaatgaaggctttcccacattcattacattcatatggtttttcacctgaatgagttctcatgtgtataattaggtatgacttgctgctaaaagctttcccacattcactgcacccataaggcttttcccctgcatgagttcgctgatgtgaaatgagctggtctttcctattaaaggctttcccacattcactgcattcatagggattttctcctgtgtgaattctctgatgcacaatgagttgtgaattgaaactaaaggatttcccgcattccctgcactcatgtggtttctctcctgtatgagttctcatatgtataataaggtatgacttgctcctgaaggctttcccacactcactgcatccatatggttttactcctgtgtgacttctctgatgtacaatgagctgggacttcaaactaaaggtttttgcacattgactgcatccatagggttttactccagtgtgcactcctttatgtacaatgagctgtgatttgaacgtaaaggcttttccacattcattacaactatagggtttctctcctgtatgagttctctgatgtacaatcaggtttgactttgtattaaaggctttctgacactcactacattcaaatggtttctcccctgtatgagttctctggtgtataataagctgtgactttaaaccaaaagcctttccacagtcggtgcattcataaggcttctctcctgcatgagttctctggtgtgaaataagctggtatttccgactgaaggctttcccacattcatggcattcataggggttctctcctgtatgaatcctctgatgtataatgagctgtgatttaaaactgaaggctttcccacaattgttgcattcatggagtttttctcctgtatgagtccttgtatgtataataaggtatgacttgctcctgaaggctttgccacattcattgcatacataaggtttcattcctgtgtgacttctctgatgtacaatgagctgtgatttcaaactgaatcctttaccacactgaatacacccatagggctttactcctgtgtgaatcccctgatgtacaatgagctgtgacttgaatgtaaaggcttttccacaatcactacaaacataaggtttctcccctgtatgggttctctgatgtaccataaggtttgactttgtattaaaggctttctgacattcattgcattcatatggtttctctcctgtatgaattctttcatgtataatgagctgtgattttaaaccaaaagctttcccacattcattacacacatatggtttctgtcctgaatgagttttctggtgtgaaacaagctggtctttcctactgaagactttcccacattcacagcactcatagggattctcacctgtgtgaattctctgatgtataacaagctgtgaatggaaactgaatgttttcctgcattcactgcattcatgtagtttctctcctgtatgaattctctgatgtacaatgaggtatgatttactactgaagtctttcccacattcattacaaccatagggtttctcttcggcatgagtttgctgatgcactagaaggtatgacttgctgctgaaggctttctcacaacagctgcatccaaagggtttttcgcccatatacatttgttggcacataagttgcgatttcttattgacggtttttccagattcaatactttcacagtattttattccaataacagtttgctcatgtttagaatggaagaatgattttccatgtacctgaaacccattaggattatttctagcataatcactagtgaaatctatatatttcaaactctttccatgcgtgccacatttatgaggtttttgtcttgaaagatactttgtactaagaagacatagttttccaaatgtagtgcattcaaagctttttgccgtacttcccagcttgtctttattttcctgatgccaatccataagatcatcaattttccagactgtgtccaaatagaagctgtccggaccctggtggccatccctacggtcagttttgtgtgcctcgctggaagtgacaggacgcgagggatgctccggctcctccaaaccctgaaggggcagcagaatagagtccagggtactgcctccacctccagatctgcagccagaagggttcgcaaccactccagactcggctggcccgttgaccacgacgggcgatgaacgctatctgaggaacaaggatctcgccatcggcgcggaacaatggcggccgctacgtat

SEQ ID NO: 14838 - RNA, 6583 nt, Homo sapiens
  source 1..6583: mol_type = other RNA
gctgggattacaggcatgagccacggcgcctgaccacacctggctaatctttttaaaaagtttttgtacagacagggtctccctatattggtcaggcttgtctcgaactcctgggttccagcaatcctccagcctcagccttcccaagtgctggtattacatggatgagccactgcacctggctaattttactttaaaggaatctttctactattttatcattaagtatgacatttgtgttttcagaacatatattccctaccaagttacaggagttaattttaattcccaacttaatagtattttagtgtcatctatgggtgttaaattccatcaagtgatttatcagcatatactgagataatccttatgagttttatctggtagttaattaaaatattttctaatattaaatcttccaaacatactcttctgttttttgagacagggtctagttctgtcacccagggtggagtacagtggtacgatctcagctcactgcaacttccgcctcctagattcaagtgattctcccgtcccagcctcccaagtagctgggattataggtgtcagttaccatgccctgctatttttttgtatttttagtagagaggggtttcaccatgttggccaggctggtctcaaactcctgacctcaggtgatccaccatctcagcctcctgaagtgctgggattataggtgtgagccaccgtgcctggccccatatatctctttttaagtgggcatactgccattataaataatagtgattctgctggtaatgaacaaaggatgctggatccactaatagtctgttaaacctaatatcatgactttcttgttagctatacattggtttgctataattccatttagaatttttaaacctatgttcacaaatatggatttttaaacctatgttcacaaatatggatttttaaacctatgttcacaaatatggtttgcaagtcattttttctcctaaatttctatttgatggggaagttgtaaaatattggggttatttttccttggattttccttataataactattcctgaaaagtctctggaatgtctttcttttctggggctggggtagaaggactagatagatttacaaaccagtaactcaatttctgttttgtaaaattttcatttcattaaataataagtcctaatcaagtattattctttcccacagtatgtgagtgctgtcctcaatactgtcaacacttctggcttctaccaggcaaggctgcatgtagatttgcatctgaaaaaacaacaaactaaaatctaaccctaggtagtagtaaactgaatataaactttctcttatgaatttattctgtcttctttggtacatcaataataatatacacctttacagtatttcccagattgggggatacactttagcaagtatctgcgattatttgtttatgtaagatgtcccttcccttctgtgaatcatcattcttcaccccaagtatcttgagattggattctgtataagcagaatacaacagttaggcattcaggtatcattaaattcctccgcttcaaggatgaaaatttctttgggtatctaatagagtacaaagcagaaggtgtttcagaaatatttgcagtattgaatccgcatattcctccaagatagccctaatctaactggcagggtcccactcttcccagattaatgcccactcacataacaaacctgatgaggtagtgaagaaaactaactttgtgagtaagcaactggcagagtttttcaccactgtgactctatagctacatgtaactaagtagtatcactgacacataatcttaaattgaagttttaagatcattattctccatgttatacatgggtatcaaaagcattcccctcttgaccactccagaattctgtttaaaatttttcaatgacaacttatccatttccccaaagcctcagtgagcacatgatgccaacaattcatttcatgacttcatagcatgggccaagtttcttgcttaaaagacttccatcctgtcttgggaaacaaccatttccaaatatccacatatccttgcaagtttctgcctactcctctaccacccatttctgaagccatctgatttagtaagctgtatgcaaaagatacacaatggctaatgcaatcaaacaaggaatgtattaaaagcacacccaatagctcaaaataaaagacaagtgaacaaagttaagaaaatgacagtaacaaaagctgttctgggaacctctattgaaatagctacttattacatcaacatgctaccacagaacaaaagctcatgttgcttttctgaacttgaaaaacccattaacaatgtacagttctgagcctcagctgaccatagtgctcatgccaagtcctgagcagggcatcttgaatggtggttccctcatgactacatacaccgttagggaatgtttcgttaagaggaaatcaagatgttctaacctgtgaaggtagaatagattccaggctacacaaacacatgaagtgtgccttatattgattactaaagaggttgctgccaagactgcttccaaagggcagaagatagccctaaaaaatgtttgcagtgtggaaatgcatttttagtaagtcatattctagtaacaagttgcatttggtaagacacaaagaaacaatgttggtatgcagagtagaaatctctggaagatgatattgtcatatcagagatattgtcagtatcagagatactgaaatctctggaagatgatttttgtctcacatatggcattcgcaagtaaaatgccaaactgcaaaattcatattatgtagtacacataggaagatatctaaatatccctgtaggctctgggatgttatttcttattcttaacctccttactagattcacttgtacaatgaaataatctgtatcttattatttataattgagaattttctcaaaccttttcctgaaattttggaacacctggaataaaatttcttaaaatgattcctaaaagaaataattcttcaaaattaatattaagatataataacaggttggtttttttttttttttttttttttttttttagaatgaagcttctaaggtgaggttaacagtccagctgtggtttatttggtacattcataagatgttcactcctatatatattttttccctaggggtttctcatttctagatttacactttcccttatagcatggtccctccaaggtatatgcttccgatacataaaatgtttgtaattttgttaattctgccattcattagctcaataatttctctcattaaaattctgtaaactatgaatttcaaagaagtctattctatattcatctggttcatgaagtttcctctttgtgaatcttattttagtaaaatgactttacaacgtttaacatggttcctcacctgtatgaactttttaaaaaaaggtatgacttgctgctaaaaattttcagagtggttactaaattcagttttcctgtgtattgtctactatctttttgcatgtaaagaacagctttctgtggatgcctttccatatgctgtgcattcataaagtttctattcagtatgagttttctggaagatgacaagatgattccacttacagagtttctctttatatatgattgtttctatctcttgtgaatccacttttcagagtttcgtaaaattatcaatgtttgtcatctacatgagttctctgatgcataatgagctgtgacttccaacaaaaggctttcccacattcagtgcacttacaaggcttctctcctgtatgtgttctctgatgtgcactgagaattgatttttgagagaaggttttcccacattcattgcacccatagggtttctctcctgaatgagttctttgatgtacaatgagttgagaattcctaatgaaggcttttccacactcactgcattcatatggtttctctcttgtgtgcattctctggtgtacaagaaggcgtaatttcccactgaaggatttctcacattgactgcatttataagggttgacccctgcatgagttcgctcatgtacaatgagtagtgatttccaaatgaaggctttcccacattcattacattcatatggtttttcacctgaatgagttctcatgtgtataattaggtatgacttgctgctaaaagctttcccacattcactgcacccataaggcttttcccctgcatgagttcgctgatgtgaaatgagctggtctttcctattaaaggctttcccacattcactgcattcatagggattttctcctgtgtgaattctctgatgcacaatgagttgtgaattgaaactaaaggatttcccgcattccctgcactcatgtggtttctctcctgtatgagttctcatatgtataataaggtatgacttgctcctgaaggctttcccacactcactgcatccatatggttttactcctgtgtgacttctctgatgtacaatgagctgggacttcaaactaaaggtttttgcacattgactgcatccatagggttttactccagtgtgcactcctttatgtacaatgagctgtgatttgaacgtaaaggcttttccacattcattacaactatagggtttctctcctgtatgagttctctgatgtacaatcaggtttgactttgtattaaaggctttctgacactcactacattcaaatggtttctcccctgtatgagttctctggtgtataataagctgtgactttaaaccaaaagcctttccacagtcggtgcattcataaggcttctctcctgcatgagttctctggtgtgaaataagctggtatttccgactgaaggctttcccacattcatggcattcataggggttctctcctgtatgaatcctctgatgtataatgagctgtgatttaaaactgaaggctttcccacaattgttgcattcatggagtttttctcctgtatgagtccttgtatgtataataaggtatgacttgctcctgaaggctttgccacattcattgcatacataaggtttcattcctgtgtgacttctctgatgtacaatgagctgtgatttcaaactgaatcctttaccacactgaatacacccatagggctttactcctgtgtgaatcccctgatgtacaatgagctgtgacttgaatgtaaaggcttttccacaatcactacaaacataaggtttctcccctgtatgggttctctgatgtaccataaggtttgactttgtattaaaggctttctgacattcattgcattcatatggtttctctcctgtatgaattctttcatgtataatgagctgtgattttaaaccaaaagctttcccacattcattacacacatatggtttctgtcctgaatgagttttctggtgtgaaacaagctggtctttcctactgaagactttcccacattcacagcactcatagggattctcacctgtgtgaattctctgatgtataacaagctgtgaatggaaactgaatgttttcctgcattcactgcattcatgtagtttctctcctgtatgaattctctgatgtacaatgaggtatgatttactactgaagtctttcccacattcattacaaccatagggtttctcttcggcatgagtttgctgatgcactagaaggtatgacttgctgctgaaggctttctcacaacagctgcatccaaagggtttttcgcccatatacatttgttggcacataagttgcgatttcttattgacggtttttccagattcaatactttcacagtattttattccaataacagtttgctcatgtttagaatggaagaatgattttccatgtacctgaaacccattaggattatttctagcataatcactagtgaaatctatatatttcaaactctttccatgcgtgccacatttatgaggtttttgtcttgaaagatactttgtactaagaagacatagttttccaaatgtagtgcattcaaagctttttgccgtacttcccagcttgtctttattttcctgatgccaatccataagatcatcaattttccagactgtgtccaggacttggtgatttttggctgctcttgggaaataaacagccactctaggactttctctattctgcgactcttctgcttctgcctgggtgttccagggagaggttgcagaccaggagtcccttggcccaagatggattcctgaccttggagctttctgatcctatcccatgaactgtttcgttcttggagaggtgggacccaaatagaagctgtccggaccctggtggccatccctacggtcagttttgtgtgcctcgctggaagtgacaggacgcgagggatgctccggctcctccaaaccctgaaggggcagcagaatagagtccagggtactgcctccacctccagatctgcagccagaagggttcgcaaccactccagactcggctggcccgttgaccacgacgggcgatgaacgctatctgaggaacaaggatctcgccatcggcgcggaacaatggcggccgctacgtat

SEQ ID NO: 14839 - RNA, 6711 nt, Homo sapiens
  source 1..6711: mol_type = other RNA
gctgggattacaggcatgagccacggcgcctgaccacacctggctaatctttttaaaaagtttttgtacagacagggtctccctatattggtcaggcttgtctcgaactcctgggttccagcaatcctccagcctcagccttcccaagtgctggtattacatggatgagccactgcacctggctaattttactttaaaggaatctttctactattttatcattaagtatgacatttgtgttttcagaacatatattccctaccaagttacaggagttaattttaattcccaacttaatagtattttagtgtcatctatgggtgttaaattccatcaagtgatttatcagcatatactgagataatccttatgagttttatctggtagttaattaaaatattttctaatattaaatcttccaaacatactcttctgttttttgagacagggtctagttctgtcacccagggtggagtacagtggtacgatctcagctcactgcaacttccgcctcctagattcaagtgattctcccgtcccagcctcccaagtagctgggattataggtgtcagttaccatgccctgctatttttttgtatttttagtagagaggggtttcaccatgttggccaggctggtctcaaactcctgacctcaggtgatccaccatctcagcctcctgaagtgctgggattataggtgtgagccaccgtgcctggccccatatatctctttttaagtgggcatactgccattataaataatagtgattctgctggtaatgaacaaaggatgctggatccactaatagtctgttaaacctaatatcatgactttcttgttagctatacattggtttgctataattccatttagaatttttaaacctatgttcacaaatatggatttttaaacctatgttcacaaatatggatttttaaacctatgttcacaaatatggtttgcaagtcattttttctcctaaatttctatttgatggggaagttgtaaaatattggggttatttttccttggattttccttataataactattcctgaaaagtctctggaatgtctttcttttctggggctggggtagaaggactagatagatttacaaaccagtaactcaatttctgttttgtaaaattttcatttcattaaataataagtcctaatcaagtattattctttcccacagtatgtgagtgctgtcctcaatactgtcaacacttctggcttctaccaggcaaggctgcatgtagatttgcatctgaaaaaacaacaaactaaaatctaaccctaggtagtagtaaactgaatataaactttctcttatgaatttattctgtcttctttggtacatcaataataatatacacctttacagtatttcccagattgggggatacactttagcaagtatctgcgattatttgtttatgtaagatgtcccttcccttctgtgaatcatcattcttcaccccaagtatcttgagattggattctgtataagcagaatacaacagttaggcattcaggtatcattaaattcctccgcttcaaggatgaaaatttctttgggtatctaatagagtacaaagcagaaggtgtttcagaaatatttgcagtattgaatccgcatattcctccaagatagccctaatctaactggcagggtcccactcttcccagattaatgcccactcacataacaaacctgatgaggtagtgaagaaaactaactttgtgagtaagcaactggcagagtttttcaccactgtgactctatagctacatgtaactaagtagtatcactgacacataatcttaaattgaagttttaagatcattattctccatgttatacatgggtatcaaaagcattcccctcttgaccactccagaattctgtttaaaatttttcaatgacaacttatccatttccccaaagcctcagtgagcacatgatgccaacaattcatttcatgacttcatagcatgggccaagtttcttgcttaaaagacttccatcctgtcttgggaaacaaccatttccaaatatccacatatccttgcaagtttctgcctactcctctaccacccatttctgaagccatctgatttagtaagctgtatgcaaaagatacacaatggctaatgcaatcaaacaaggaatgtattaaaagcacacccaatagctcaaaataaaagacaagtgaacaaagttaagaaaatgacagtaacaaaagctgttctgggaacctctattgaaatagctacttattacatcaacatgctaccacagaacaaaagctcatgttgcttttctgaacttgaaaaacccattaacaatgtacagttctgagcctcagctgaccatagtgctcatgccaagtcctgagcagggcatcttgaatggtggttccctcatgactacatacaccgttagggaatgtttcgttaagaggaaatcaagatgttctaacctgtgaaggtagaatagattccaggctacacaaacacatgaagtgtgccttatattgattactaaagaggttgctgccaagactgcttccaaagggcagaagatagccctaaaaaatgtttgcagtgtggaaatgcatttttagtaagtcatattctagtaacaagttgcatttggtaagacacaaagaaacaatgttggtatgcagagtagaaatctctggaagatgatattgtcatatcagagatattgtcagtatcagagatactgaaatctctggaagatgatttttgtctcacatatggcattcgcaagtaaaatgccaaactgcaaaattcatattatgtagtacacataggaagatatctaaatatccctgtaggctctgggatgttatttcttattcttaacctccttactagattcacttgtacaatgaaataatctgtatcttattatttataattgagaattttctcaaaccttttcctgaaattttggaacacctggaataaaatttcttaaaatgattcctaaaagaaataattcttcaaaattaatattaagatataataacaggttggtttttttttttttttttttttttttttttagaatgaagcttctaaggtgaggttaacagtccagctgtggtttatttggtacattcataagatgttcactcctatatatattttttccctaggggtttctcatttctagatttacactttcccttatagcatggtccctccaaggtatatgcttccgatacataaaatgtttgtaattttgttaattctgccattcattagctcaataatttctctcattaaaattctgtaaactatgaatttcaaagaagtctattctatattcatctggttcatgaagtttcctctttgtgaatcttattttagtaaaatgactttacaacgtttaacatggttcctcacctgtatgaactttttaaaaaaaggtatgacttgctgctaaaaattttcagagtggttactaaattcagttttcctgtgtattgtctactatctttttgcatgtaaagaacagctttctgtggatgcctttccatatgctgtgcattcataaagtttctattcagtatgagttttctggaagatgacaagatgattccacttacagagtttctctttatatatgattgtttctatctcttgtgaatccacttttcagagtttcgtaaaattatcaatgtttgtcatctacatgagttctctgatgcataatgagctgtgacttccaacaaaaggctttcccacattcagtgcacttacaaggcttctctcctgtatgtgttctctgatgtgcactgagaattgatttttgagagaaggttttcccacattcattgcacccatagggtttctctcctgaatgagttctttgatgtacaatgagttgagaattcctaatgaaggcttttccacactcactgcattcatatggtttctctcttgtgtgcattctctggtgtacaagaaggcgtaatttcccactgaaggatttctcacattgactgcatttataagggttgacccctgcatgagttcgctcatgtacaatgagtagtgatttccaaatgaaggctttcccacattcattacattcatatggtttttcacctgaatgagttctcatgtgtataattaggtatgacttgctgctaaaagctttcccacattcactgcacccataaggcttttcccctgcatgagttcgctgatgtgaaatgagctggtctttcctattaaaggctttcccacattcactgcattcatagggattttctcctgtgtgaattctctgatgcacaatgagttgtgaattgaaactaaaggatttcccgcattccctgcactcatgtggtttctctcctgtatgagttctcatatgtataataaggtatgacttgctcctgaaggctttcccacactcactgcatccatatggttttactcctgtgtgacttctctgatgtacaatgagctgggacttcaaactaaaggtttttgcacattgactgcatccatagggttttactccagtgtgcactcctttatgtacaatgagctgtgatttgaacgtaaaggcttttccacattcattacaactatagggtttctctcctgtatgagttctctgatgtacaatcaggtttgactttgtattaaaggctttctgacactcactacattcaaatggtttctcccctgtatgagttctctggtgtataataagctgtgactttaaaccaaaagcctttccacagtcggtgcattcataaggcttctctcctgcatgagttctctggtgtgaaataagctggtatttccgactgaaggctttcccacattcatggcattcataggggttctctcctgtatgaatcctctgatgtataatgagctgtgatttaaaactgaaggctttcccacaattgttgcattcatggagtttttctcctgtatgagtccttgtatgtataataaggtatgacttgctcctgaaggctttgccacattcattgcatacataaggtttcattcctgtgtgacttctctgatgtacaatgagctgtgatttcaaactgaatcctttaccacactgaatacacccatagggctttactcctgtgtgaatcccctgatgtacaatgagctgtgacttgaatgtaaaggcttttccacaatcactacaaacataaggtttctcccctgtatgggttctctgatgtaccataaggtttgactttgtattaaaggctttctgacattcattgcattcatatggtttctctcctgtatgaattctttcatgtataatgagctgtgattttaaaccaaaagctttcccacattcattacacacatatggtttctgtcctgaatgagttttctggtgtgaaacaagctggtctttcctactgaagactttcccacattcacagcactcatagggattctcacctgtgtgaattctctgatgtataacaagctgtgaatggaaactgaatgttttcctgcattcactgcattcatgtagtttctctcctgtatgaattctctgatgtacaatgaggtatgatttactactgaagtctttcccacattcattacaaccatagggtttctcttcggcatgagtttgctgatgcactagaaggtatgacttgctgctgaaggctttctcacaacagctgcatccaaagggtttttcgcccatatacatttgttggcacataagttgcgatttcttattgacggtttttccagattcaatactttcacagtattttattccaataacagtttgctcatgtttagaatggaagaatgattttccatgtacctgaaacccattaggattatttctagcataatcactagtgaaatctatatatttcaaactctttccatgcgtgccacatttatgaggtttttgtcttgaaagatactttgtactaagaagacatagttttccaaatgtagtgcattcaaagctttttgccgtacttcccagcttgtctttattttcctgatgccaatccataagatcatcaattttccagactgtgtctccagaggatgcagcaacaaggcgtcatcttggaagcacagagcaggccctcaccagacaccaaacctgccagcaccttggctttggactttccagccttcaaaattggacaggtctgatttggaacttgggcctgcaccatacacagctcttctccttgttccaacttgaagatgatatcaggtttggtgtgttggtaccctagggacaccaggttgctatagttctccaacatcacactcctgtacaggcacttctgtgctgggtctagcagctgccactcctcccaggtaaaatccacaaacacatccatgaatgacaaaggtccccaaatagaagctgtccggaccctggtggccatccctacggtcagttttgtgtgcctcgctggaagtgacaggacgcgagggatgctccggctcctccaaaccctgaaggggcagcagaatagagtccagggtactgcctccacctccagatctgcagccagaagggttcgcaaccactccagactcggctggcccgttgaccacgacgggcgatgaacgctatctgaggaacaaggatctcgccatcggcgcggaacaatggcggccgctacgtat

SEQ ID NO: 14840 - RNA, 6912 nt, Homo sapiens
  source 1..6912: mol_type = other RNA
gctgggattacaggcatgagccacggcgcctgaccacacctggctaatctttttaaaaagtttttgtacagacagggtctccctatattggtcaggcttgtctcgaactcctgggttccagcaatcctccagcctcagccttcccaagtgctggtattacatggatgagccactgcacctggctaattttactttaaaggaatctttctactattttatcattaagtatgacatttgtgttttcagaacatatattccctaccaagttacaggagttaattttaattcccaacttaatagtattttagtgtcatctatgggtgttaaattccatcaagtgatttatcagcatatactgagataatccttatgagttttatctggtagttaattaaaatattttctaatattaaatcttccaaacatactcttctgttttttgagacagggtctagttctgtcacccagggtggagtacagtggtacgatctcagctcactgcaacttccgcctcctagattcaagtgattctcccgtcccagcctcccaagtagctgggattataggtgtcagttaccatgccctgctatttttttgtatttttagtagagaggggtttcaccatgttggccaggctggtctcaaactcctgacctcaggtgatccaccatctcagcctcctgaagtgctgggattataggtgtgagccaccgtgcctggccccatatatctctttttaagtgggcatactgccattataaataatagtgattctgctggtaatgaacaaaggatgctggatccactaatagtctgttaaacctaatatcatgactttcttgttagctatacattggtttgctataattccatttagaatttttaaacctatgttcacaaatatggatttttaaacctatgttcacaaatatggatttttaaacctatgttcacaaatatggtttgcaagtcattttttctcctaaatttctatttgatggggaagttgtaaaatattggggttatttttccttggattttccttataataactattcctgaaaagtctctggaatgtctttcttttctggggctggggtagaaggactagatagatttacaaaccagtaactcaatttctgttttgtaaaattttcatttcattaaataataagtcctaatcaagtattattctttcccacagtatgtgagtgctgtcctcaatactgtcaacacttctggcttctaccaggcaaggctgcatgtagatttgcatctgaaaaaacaacaaactaaaatctaaccctaggtagtagtaaactgaatataaactttctcttatgaatttattctgtcttctttggtacatcaataataatatacacctttacagtatttcccagattgggggatacactttagcaagtatctgcgattatttgtttatgtaagatgtcccttcccttctgtgaatcatcattcttcaccccaagtatcttgagattggattctgtataagcagaatacaacagttaggcattcaggtatcattaaattcctccgcttcaaggatgaaaatttctttgggtatctaatagagtacaaagcagaaggtgtttcagaaatatttgcagtattgaatccgcatattcctccaagatagccctaatctaactggcagggtcccactcttcccagattaatgcccactcacataacaaacctgatgaggtagtgaagaaaactaactttgtgagtaagcaactggcagagtttttcaccactgtgactctatagctacatgtaactaagtagtatcactgacacataatcttaaattgaagttttaagatcattattctccatgttatacatgggtatcaaaagcattcccctcttgaccactccagaattctgtttaaaatttttcaatgacaacttatccatttccccaaagcctcagtgagcacatgatgccaacaattcatttcatgacttcatagcatgggccaagtttcttgcttaaaagacttccatcctgtcttgggaaacaaccatttccaaatatccacatatccttgcaagtttctgcctactcctctaccacccatttctgaagccatctgatttagtaagctgtatgcaaaagatacacaatggctaatgcaatcaaacaaggaatgtattaaaagcacacccaatagctcaaaataaaagacaagtgaacaaagttaagaaaatgacagtaacaaaagctgttctgggaacctctattgaaatagctacttattacatcaacatgctaccacagaacaaaagctcatgttgcttttctgaacttgaaaaacccattaacaatgtacagttctgagcctcagctgaccatagtgctcatgccaagtcctgagcagggcatcttgaatggtggttccctcatgactacatacaccgttagggaatgtttcgttaagaggaaatcaagatgttctaacctgtgaaggtagaatagattccaggctacacaaacacatgaagtgtgccttatattgattactaaagaggttgctgccaagactgcttccaaagggcagaagatagccctaaaaaatgtttgcagtgtggaaatgcatttttagtaagtcatattctagtaacaagttgcatttggtaagacacaaagaaacaatgttggtatgcagagtagaaatctctggaagatgatattgtcatatcagagatattgtcagtatcagagatactgaaatctctggaagatgatttttgtctcacatatggcattcgcaagtaaaatgccaaactgcaaaattcatattatgtagtacacataggaagatatctaaatatccctgtaggctctgggatgttatttcttattcttaacctccttactagattcacttgtacaatgaaataatctgtatcttattatttataattgagaattttctcaaaccttttcctgaaattttggaacacctggaataaaatttcttaaaatgattcctaaaagaaataattcttcaaaattaatattaagatataataacaggttggtttttttttttttttttttttttttttttagaatgaagcttctaaggtgaggttaacagtccagctgtggtttatttggtacattcataagatgttcactcctatatatattttttccctaggggtttctcatttctagatttacactttcccttatagcatggtccctccaaggtatatgcttccgatacataaaatgtttgtaattttgttaattctgccattcattagctcaataatttctctcattaaaattctgtaaactatgaatttcaaagaagtctattctatattcatctggttcatgaagtttcctctttgtgaatcttattttagtaaaatgactttacaacgtttaacatggttcctcacctgtatgaactttttaaaaaaaggtatgacttgctgctaaaaattttcagagtggttactaaattcagttttcctgtgtattgtctactatctttttgcatgtaaagaacagctttctgtggatgcctttccatatgctgtgcattcataaagtttctattcagtatgagttttctggaagatgacaagatgattccacttacagagtttctctttatatatgattgtttctatctcttgtgaatccacttttcagagtttcgtaaaattatcaatgtttgtcatctacatgagttctctgatgcataatgagctgtgacttccaacaaaaggctttcccacattcagtgcacttacaaggcttctctcctgtatgtgttctctgatgtgcactgagaattgatttttgagagaaggttttcccacattcattgcacccatagggtttctctcctgaatgagttctttgatgtacaatgagttgagaattcctaatgaaggcttttccacactcactgcattcatatggtttctctcttgtgtgcattctctggtgtacaagaaggcgtaatttcccactgaaggatttctcacattgactgcatttataagggttgacccctgcatgagttcgctcatgtacaatgagtagtgatttccaaatgaaggctttcccacattcattacattcatatggtttttcacctgaatgagttctcatgtgtataattaggtatgacttgctgctaaaagctttcccacattcactgcacccataaggcttttcccctgcatgagttcgctgatgtgaaatgagctggtctttcctattaaaggctttcccacattcactgcattcatagggattttctcctgtgtgaattctctgatgcacaatgagttgtgaattgaaactaaaggatttcccgcattccctgcactcatgtggtttctctcctgtatgagttctcatatgtataataaggtatgacttgctcctgaaggctttcccacactcactgcatccatatggttttactcctgtgtgacttctctgatgtacaatgagctgggacttcaaactaaaggtttttgcacattgactgcatccatagggttttactccagtgtgcactcctttatgtacaatgagctgtgatttgaacgtaaaggcttttccacattcattacaactatagggtttctctcctgtatgagttctctgatgtacaatcaggtttgactttgtattaaaggctttctgacactcactacattcaaatggtttctcccctgtatgagttctctggtgtataataagctgtgactttaaaccaaaagcctttccacagtcggtgcattcataaggcttctctcctgcatgagttctctggtgtgaaataagctggtatttccgactgaaggctttcccacattcatggcattcataggggttctctcctgtatgaatcctctgatgtataatgagctgtgatttaaaactgaaggctttcccacaattgttgcattcatggagtttttctcctgtatgagtccttgtatgtataataaggtatgacttgctcctgaaggctttgccacattcattgcatacataaggtttcattcctgtgtgacttctctgatgtacaatgagctgtgatttcaaactgaatcctttaccacactgaatacacccatagggctttactcctgtgtgaatcccctgatgtacaatgagctgtgacttgaatgtaaaggcttttccacaatcactacaaacataaggtttctcccctgtatgggttctctgatgtaccataaggtttgactttgtattaaaggctttctgacattcattgcattcatatggtttctctcctgtatgaattctttcatgtataatgagctgtgattttaaaccaaaagctttcccacattcattacacacatatggtttctgtcctgaatgagttttctggtgtgaaacaagctggtctttcctactgaagactttcccacattcacagcactcatagggattctcacctgtgtgaattctctgatgtataacaagctgtgaatggaaactgaatgttttcctgcattcactgcattcatgtagtttctctcctgtatgaattctctgatgtacaatgaggtatgatttactactgaagtctttcccacattcattacaaccatagggtttctcttcggcatgagtttgctgatgcactagaaggtatgacttgctgctgaaggctttctcacaacagctgcatccaaagggtttttcgcccatatacatttgttggcacataagttgcgatttcttattgacggtttttccagattcaatactttcacagtattttattccaataacagtttgctcatgtttagaatggaagaatgattttccatgtacctgaaacccattaggattatttctagcataatcactagtgaaatctatatatttcaaactctttccatgcgtgccacatttatgaggtttttgtcttgaaagatactttgtactaagaagacatagttttccaaatgtagtgcattcaaagctttttgccgtacttcccagcttgtctttattttcctgatgccaatccataagatcatcaattttccagactgtgtctccagaggatgcagcaacaaggcgtcatcttggaagcacagagcaggccctcaccagacaccaaacctgccagcaccttggctttggactttccagccttcaaaattggacaggtctgatttggaacttgggcctgcaccatacacagctcttctccttgttccaacttgaagatgatatcaggtttggtgtgttggtaccctagggacaccaggttgctatagttctccaacatcacactcctgtacaggcacttctgtgctgggtctagcagctgccactcctcccaggtaaaatccacaaacacatccatgaatgacaaaggtccccaggacttggtgatttttggctgctcttgggaaataaacagccactctaggactttctctattctgcgactcttctgcttctgcctgggtgttccagggagaggttgcagaccaggagtcccttggcccaagatggattcctgaccttggagctttctgatcctatcccatgaactgtttcgttcttggagaggtgggacccaaatagaagctgtccggaccctggtggccatccctacggtcagttttgtgtgcctcgctggaagtgacaggacgcgagggatgctccggctcctccaaaccctgaaggggcagcagaatagagtccagggtactgcctccacctccagatctgcagccagaagggttcgcaaccactccagactcggctggcccgttgaccacgacgggcgatgaacgctatctgaggaacaaggatctcgccatcggcgcggaacaatggcggccgctacgtat

SEQ ID NO: 14841 - RNA, 6478 nt, Homo sapiens
  source 1..6478: mol_type = other RNA
gctgggattacaggcatgagccacggcgcctgaccacacctggctaatctttttaaaaagtttttgtacagacagggtctccctatattggtcaggcttgtctcgaactcctgggttccagcaatcctccagcctcagccttcccaagtgctggtattacatggatgagccactgcacctggctaattttactttaaaggaatctttctactattttatcattaagtatgacatttgtgttttcagaacatatattccctaccaagttacaggagttaattttaattcccaacttaatagtattttagtgtcatctatgggtgttaaattccatcaagtgatttatcagcatatactgagataatccttatgagttttatctggtagttaattaaaatattttctaatattaaatcttccaaacatactcttctgttttttgagacagggtctagttctgtcacccagggtggagtacagtggtacgatctcagctcactgcaacttccgcctcctagattcaagtgattctcccgtcccagcctcccaagtagctgggattataggtgtcagttaccatgccctgctatttttttgtatttttagtagagaggggtttcaccatgttggccaggctggtctcaaactcctgacctcaggtgatccaccatctcagcctcctgaagtgctgggattataggtgtgagccaccgtgcctggccccatatatctctttttaagtgggcatactgccattataaataatagtgattctgctggtaatgaacaaaggatgctggatccactaatagtctgttaaacctaatatcatgactttcttgttagctatacattggtttgctataattccatttagaatttttaaacctatgttcacaaatatggatttttaaacctatgttcacaaatatggatttttaaacctatgttcacaaatatggtttgcaagtcattttttctcctaaatttctatttgatggggaagttgtaaaatattggggttatttttccttggattttccttataataactattcctgaaaagtctctggaatgtctttcttttctggggctggggtagaaggactagatagatttacaaaccagtaactcaatttctgttttgtaaaattttcatttcattaaataataagtcctaatcaagtattattctttcccacagtatgtgagtgctgtcctcaatactgtcaacacttctggcttctaccaggcaaggctgcatgtagatttgcatctgaaaaaacaacaaactaaaatctaaccctaggtagtagtaaactgaatataaactttctcttatgaatttattctgtcttctttggtacatcaataataatatacacctttacagtatttcccagattgggggatacactttagcaagtatctgcgattatttgtttatgtaagatgtcccttcccttctgtgaatcatcattcttcaccccaagtatcttgagattggattctgtataagcagaatacaacagttaggcattcaggtatcattaaattcctccgcttcaaggatgaaaatttctttgggtatctaatagagtacaaagcagaaggtgtttcagaaatatttgcagtattgaatccgcatattcctccaagatagccctaatctaactggcagggtcccactcttcccagattaatgcccactcacataacaaacctgatgaggtagtgaagaaaactaactttgtgagtaagcaactggcagagtttttcaccactgtgactctatagctacatgtaactaagtagtatcactgacacataatcttaaattgaagttttaagatcattattctccatgttatacatgggtatcaaaagcattcccctcttgaccactccagaattctgtttaaaatttttcaatgacaacttatccatttccccaaagcctcagtgagcacatgatgccaacaattcatttcatgacttcatagcatgggccaagtttcttgcttaaaagacttccatcctgtcttgggaaacaaccatttccaaatatccacatatccttgcaagtttctgcctactcctctaccacccatttctgaagccatctgatttagtaagctgtatgcaaaagatacacaatggctaatgcaatcaaacaaggaatgtattaaaagcacacccaatagctcaaaataaaagacaagtgaacaaagttaagaaaatgacagtaacaaaagctgttctgggaacctctattgaaatagctacttattacatcaacatgctaccacagaacaaaagctcatgttgcttttctgaacttgaaaaacccattaacaatgtacagttctgagcctcagctgaccatagtgctcatgccaagtcctgagcagggcatcttgaatggtggttccctcatgactacatacaccgttagggaatgtttcgttaagaggaaatcaagatgttctaacctgtgaaggtagaatagattccaggctacacaaacacatgaagtgtgccttatattgattactaaagaggttgctgccaagactgcttccaaagggcagaagatagccctaaaaaatgtttgcagtgtggaaatgcatttttagtaagtcatattctagtaacaagttgcatttggtaagacacaaagaaacaatgttggtatgcagagtagaaatctctggaagatgatattgtcatatcagagatattgtcagtatcagagatactgaaatctctggaagatgatttttgtctcacatatggcattcgcaagtaaaatgccaaactgcaaaattcatattatgtagtacacataggaagatatctaaatatccctgtaggctctgggatgttatttcttattcttaacctccttactagattcacttgtacaatgaaataatctgtatcttattatttataattgagaattttctcaaaccttttcctgaaattttggaacacctggaataaaatttcttaaaatgattcctaaaagaaataattcttcaaaattaatattaagatataataacaggttggtttttttttttttttttttttttttttttagaatgaagcttctaaggtgaggttaacagtccagctgtggtttatttggtacattcataagatgttcactcctatatatattttttccctaggggtttctcatttctagatttacactttcccttatagcatggtccctccaaggtatatgcttccgatacataaaatgtttgtaattttgttaattctgccattcattagctcaataatttctctcattaaaattctgtaaactatgaatttcaaagaagtctattctatattcatctggttcatgaagtttcctctttgtgaatcttattttagtaaaatgactttacaacgtttaacatggttcctcacctgtatgaactttttaaaaaaaggtatgacttgctgctaaaaattttcagagtggttactaaattcagttttcctgtgtattgtctactatctttttgcatgtaaagaacagctttctgtggatgcctttccatatgctgtgcattcataaagtttctattcagtatgagttttctggaagatgacaagatgattccacttacagagtttctctttatatatgattgtttctatctcttgtgaatccacttttcagagtttcgtaaaattatcaatgtttgtcatctacatgagttctctgatgcataatgagctgtgacttccaacaaaaggctttcccacattcagtgcacttacaaggcttctctcctgtatgtgttctctgatgtgcactgagaattgatttttgagagaaggttttcccacattcattgcacccatagggtttctctcctgaatgagttctttgatgtacaatgagttgagaattcctaatgaaggcttttccacactcactgcattcatatggtttctctcttgtgtgcattctctggtgtacaagaaggcgtaatttcccactgaaggatttctcacattgactgcatttataagggttgacccctgcatgagttcgctcatgtacaatgagtagtgatttccaaatgaaggctttcccacattcattacattcatatggtttttcacctgaatgagttctcatgtgtataattaggtatgacttgctgctaaaagctttcccacattcactgcacccataaggcttttcccctgcatgagttcgctgatgtgaaatgagctggtctttcctattaaaggctttcccacattcactgcattcatagggattttctcctgtgtgaattctctgatgcacaatgagttgtgaattgaaactaaaggatttcccgcattccctgcactcatgtggtttctctcctgtatgagttctcatatgtataataaggtatgacttgctcctgaaggctttcccacactcactgcatccatatggttttactcctgtgtgacttctctgatgtacaatgagctgggacttcaaactaaaggtttttgcacattgactgcatccatagggttttactccagtgtgcactcctttatgtacaatgagctgtgatttgaacgtaaaggcttttccacattcattacaactatagggtttctctcctgtatgagttctctgatgtacaatcaggtttgactttgtattaaaggctttctgacactcactacattcaaatggtttctcccctgtatgagttctctggtgtataataagctgtgactttaaaccaaaagcctttccacagtcggtgcattcataaggcttctctcctgcatgagttctctggtgtgaaataagctggtatttccgactgaaggctttcccacattcatggcattcataggggttctctcctgtatgaatcctctgatgtataatgagctgtgatttaaaactgaaggctttcccacaattgttgcattcatggagtttttctcctgtatgagtccttgtatgtataataaggtatgacttgctcctgaaggctttgccacattcattgcatacataaggtttcattcctgtgtgacttctctgatgtacaatgagctgtgatttcaaactgaatcctttaccacactgaatacacccatagggctttactcctgtgtgaatcccctgatgtacaatgagctgtgacttgaatgtaaaggcttttccacaatcactacaaacataaggtttctcccctgtatgggttctctgatgtaccataaggtttgactttgtattaaaggctttctgacattcattgcattcatatggtttctctcctgtatgaattctttcatgtataatgagctgtgattttaaaccaaaagctttcccacattcattacacacatatggtttctgtcctgaatgagttttctggtgtgaaacaagctggtctttcctactgaagactttcccacattcacagcactcatagggattctcacctgtgtgaattctctgatgtataacaagctgtgaatggaaactgaatgttttcctgcattcactgcattcatgtagtttctctcctgtatgaattctctgatgtacaatgaggtatgatttactactgaagtctttcccacattcattacaaccatagggtttctcttcggcatgagtttgctgatgcactagaaggtatgacttgctgctgaaggctttctcacaacagctgcatccaaagggtttttcgcccatatacatttgttggcacataagttgcgatttcttattgacggtttttccagattcaatactttcacagtattttattccaataacagtttgctcatgtttagaatggaagaatgattttccatgtacctgaaacccattaggattatttctagcataatcactagtgaaatctatatatttcaaactctttccatgcgtgccacatttatgaggtttttgtcttgaaagatactttgtactaagaagacatagttttccaaatgtagtgcattcaaagctttttgccgtacttcccagcttgtctttattttcctgatgccaatccataagatcatcaattttccagactgtgtttggacaggtctgatttggaacttgggcctgcaccatacacagctcttctccttgttccaacttgaagatgatatcaggtttggtgtgttggtaccccaaatagaagctgtccggaccctggtggccatccctacggtcagttttgtgtgcctcgctggaagtgacaggacgcgagggatgctccggctcctccaaaccctgaaggggcagcagaatagagtccagggtactgcctccacctccagatctgcagccagaagggttcgcaaccactccagactcggctggcccgttgaccacgacgggcgatgaacgctatctgaggaacaaggatctcgccatcggcgcggaacaatggcggccgctacgtat

SEQ ID NO: 14842 - RNA, 6679 nt, Homo sapiens
  source 1..6679: mol_type = other RNA
gctgggattacaggcatgagccacggcgcctgaccacacctggctaatctttttaaaaagtttttgtacagacagggtctccctatattggtcaggcttgtctcgaactcctgggttccagcaatcctccagcctcagccttcccaagtgctggtattacatggatgagccactgcacctggctaattttactttaaaggaatctttctactattttatcattaagtatgacatttgtgttttcagaacatatattccctaccaagttacaggagttaattttaattcccaacttaatagtattttagtgtcatctatgggtgttaaattccatcaagtgatttatcagcatatactgagataatccttatgagttttatctggtagttaattaaaatattttctaatattaaatcttccaaacatactcttctgttttttgagacagggtctagttctgtcacccagggtggagtacagtggtacgatctcagctcactgcaacttccgcctcctagattcaagtgattctcccgtcccagcctcccaagtagctgggattataggtgtcagttaccatgccctgctatttttttgtatttttagtagagaggggtttcaccatgttggccaggctggtctcaaactcctgacctcaggtgatccaccatctcagcctcctgaagtgctgggattataggtgtgagccaccgtgcctggccccatatatctctttttaagtgggcatactgccattataaataatagtgattctgctggtaatgaacaaaggatgctggatccactaatagtctgttaaacctaatatcatgactttcttgttagctatacattggtttgctataattccatttagaatttttaaacctatgttcacaaatatggatttttaaacctatgttcacaaatatggatttttaaacctatgttcacaaatatggtttgcaagtcattttttctcctaaatttctatttgatggggaagttgtaaaatattggggttatttttccttggattttccttataataactattcctgaaaagtctctggaatgtctttcttttctggggctggggtagaaggactagatagatttacaaaccagtaactcaatttctgttttgtaaaattttcatttcattaaataataagtcctaatcaagtattattctttcccacagtatgtgagtgctgtcctcaatactgtcaacacttctggcttctaccaggcaaggctgcatgtagatttgcatctgaaaaaacaacaaactaaaatctaaccctaggtagtagtaaactgaatataaactttctcttatgaatttattctgtcttctttggtacatcaataataatatacacctttacagtatttcccagattgggggatacactttagcaagtatctgcgattatttgtttatgtaagatgtcccttcccttctgtgaatcatcattcttcaccccaagtatcttgagattggattctgtataagcagaatacaacagttaggcattcaggtatcattaaattcctccgcttcaaggatgaaaatttctttgggtatctaatagagtacaaagcagaaggtgtttcagaaatatttgcagtattgaatccgcatattcctccaagatagccctaatctaactggcagggtcccactcttcccagattaatgcccactcacataacaaacctgatgaggtagtgaagaaaactaactttgtgagtaagcaactggcagagtttttcaccactgtgactctatagctacatgtaactaagtagtatcactgacacataatcttaaattgaagttttaagatcattattctccatgttatacatgggtatcaaaagcattcccctcttgaccactccagaattctgtttaaaatttttcaatgacaacttatccatttccccaaagcctcagtgagcacatgatgccaacaattcatttcatgacttcatagcatgggccaagtttcttgcttaaaagacttccatcctgtcttgggaaacaaccatttccaaatatccacatatccttgcaagtttctgcctactcctctaccacccatttctgaagccatctgatttagtaagctgtatgcaaaagatacacaatggctaatgcaatcaaacaaggaatgtattaaaagcacacccaatagctcaaaataaaagacaagtgaacaaagttaagaaaatgacagtaacaaaagctgttctgggaacctctattgaaatagctacttattacatcaacatgctaccacagaacaaaagctcatgttgcttttctgaacttgaaaaacccattaacaatgtacagttctgagcctcagctgaccatagtgctcatgccaagtcctgagcagggcatcttgaatggtggttccctcatgactacatacaccgttagggaatgtttcgttaagaggaaatcaagatgttctaacctgtgaaggtagaatagattccaggctacacaaacacatgaagtgtgccttatattgattactaaagaggttgctgccaagactgcttccaaagggcagaagatagccctaaaaaatgtttgcagtgtggaaatgcatttttagtaagtcatattctagtaacaagttgcatttggtaagacacaaagaaacaatgttggtatgcagagtagaaatctctggaagatgatattgtcatatcagagatattgtcagtatcagagatactgaaatctctggaagatgatttttgtctcacatatggcattcgcaagtaaaatgccaaactgcaaaattcatattatgtagtacacataggaagatatctaaatatccctgtaggctctgggatgttatttcttattcttaacctccttactagattcacttgtacaatgaaataatctgtatcttattatttataattgagaattttctcaaaccttttcctgaaattttggaacacctggaataaaatttcttaaaatgattcctaaaagaaataattcttcaaaattaatattaagatataataacaggttggtttttttttttttttttttttttttttttagaatgaagcttctaaggtgaggttaacagtccagctgtggtttatttggtacattcataagatgttcactcctatatatattttttccctaggggtttctcatttctagatttacactttcccttatagcatggtccctccaaggtatatgcttccgatacataaaatgtttgtaattttgttaattctgccattcattagctcaataatttctctcattaaaattctgtaaactatgaatttcaaagaagtctattctatattcatctggttcatgaagtttcctctttgtgaatcttattttagtaaaatgactttacaacgtttaacatggttcctcacctgtatgaactttttaaaaaaaggtatgacttgctgctaaaaattttcagagtggttactaaattcagttttcctgtgtattgtctactatctttttgcatgtaaagaacagctttctgtggatgcctttccatatgctgtgcattcataaagtttctattcagtatgagttttctggaagatgacaagatgattccacttacagagtttctctttatatatgattgtttctatctcttgtgaatccacttttcagagtttcgtaaaattatcaatgtttgtcatctacatgagttctctgatgcataatgagctgtgacttccaacaaaaggctttcccacattcagtgcacttacaaggcttctctcctgtatgtgttctctgatgtgcactgagaattgatttttgagagaaggttttcccacattcattgcacccatagggtttctctcctgaatgagttctttgatgtacaatgagttgagaattcctaatgaaggcttttccacactcactgcattcatatggtttctctcttgtgtgcattctctggtgtacaagaaggcgtaatttcccactgaaggatttctcacattgactgcatttataagggttgacccctgcatgagttcgctcatgtacaatgagtagtgatttccaaatgaaggctttcccacattcattacattcatatggtttttcacctgaatgagttctcatgtgtataattaggtatgacttgctgctaaaagctttcccacattcactgcacccataaggcttttcccctgcatgagttcgctgatgtgaaatgagctggtctttcctattaaaggctttcccacattcactgcattcatagggattttctcctgtgtgaattctctgatgcacaatgagttgtgaattgaaactaaaggatttcccgcattccctgcactcatgtggtttctctcctgtatgagttctcatatgtataataaggtatgacttgctcctgaaggctttcccacactcactgcatccatatggttttactcctgtgtgacttctctgatgtacaatgagctgggacttcaaactaaaggtttttgcacattgactgcatccatagggttttactccagtgtgcactcctttatgtacaatgagctgtgatttgaacgtaaaggcttttccacattcattacaactatagggtttctctcctgtatgagttctctgatgtacaatcaggtttgactttgtattaaaggctttctgacactcactacattcaaatggtttctcccctgtatgagttctctggtgtataataagctgtgactttaaaccaaaagcctttccacagtcggtgcattcataaggcttctctcctgcatgagttctctggtgtgaaataagctggtatttccgactgaaggctttcccacattcatggcattcataggggttctctcctgtatgaatcctctgatgtataatgagctgtgatttaaaactgaaggctttcccacaattgttgcattcatggagtttttctcctgtatgagtccttgtatgtataataaggtatgacttgctcctgaaggctttgccacattcattgcatacataaggtttcattcctgtgtgacttctctgatgtacaatgagctgtgatttcaaactgaatcctttaccacactgaatacacccatagggctttactcctgtgtgaatcccctgatgtacaatgagctgtgacttgaatgtaaaggcttttccacaatcactacaaacataaggtttctcccctgtatgggttctctgatgtaccataaggtttgactttgtattaaaggctttctgacattcattgcattcatatggtttctctcctgtatgaattctttcatgtataatgagctgtgattttaaaccaaaagctttcccacattcattacacacatatggtttctgtcctgaatgagttttctggtgtgaaacaagctggtctttcctactgaagactttcccacattcacagcactcatagggattctcacctgtgtgaattctctgatgtataacaagctgtgaatggaaactgaatgttttcctgcattcactgcattcatgtagtttctctcctgtatgaattctctgatgtacaatgaggtatgatttactactgaagtctttcccacattcattacaaccatagggtttctcttcggcatgagtttgctgatgcactagaaggtatgacttgctgctgaaggctttctcacaacagctgcatccaaagggtttttcgcccatatacatttgttggcacataagttgcgatttcttattgacggtttttccagattcaatactttcacagtattttattccaataacagtttgctcatgtttagaatggaagaatgattttccatgtacctgaaacccattaggattatttctagcataatcactagtgaaatctatatatttcaaactctttccatgcgtgccacatttatgaggtttttgtcttgaaagatactttgtactaagaagacatagttttccaaatgtagtgcattcaaagctttttgccgtacttcccagcttgtctttattttcctgatgccaatccataagatcatcaattttccagactgtgtttggacaggtctgatttggaacttgggcctgcaccatacacagctcttctccttgttccaacttgaagatgatatcaggtttggtgtgttggtaccccaggacttggtgatttttggctgctcttgggaaataaacagccactctaggactttctctattctgcgactcttctgcttctgcctgggtgttccagggagaggttgcagaccaggagtcccttggcccaagatggattcctgaccttggagctttctgatcctatcccatgaactgtttcgttcttggagaggtgggacccaaatagaagctgtccggaccctggtggccatccctacggtcagttttgtgtgcctcgctggaagtgacaggacgcgagggatgctccggctcctccaaaccctgaaggggcagcagaatagagtccagggtactgcctccacctccagatctgcagccagaagggttcgcaaccactccagactcggctggcccgttgaccacgacgggcgatgaacgctatctgaggaacaaggatctcgccatcggcgcggaacaatggcggccgctacgtat

SEQ ID NO: 14843 - RNA, 6747 nt, Homo sapiens
  source 1..6747: mol_type = other RNA
gctgggattacaggcatgagccacggcgcctgaccacacctggctaatctttttaaaaagtttttgtacagacagggtctccctatattggtcaggcttgtctcgaactcctgggttccagcaatcctccagcctcagccttcccaagtgctggtattacatggatgagccactgcacctggctaattttactttaaaggaatctttctactattttatcattaagtatgacatttgtgttttcagaacatatattccctaccaagttacaggagttaattttaattcccaacttaatagtattttagtgtcatctatgggtgttaaattccatcaagtgatttatcagcatatactgagataatccttatgagttttatctggtagttaattaaaatattttctaatattaaatcttccaaacatactcttctgttttttgagacagggtctagttctgtcacccagggtggagtacagtggtacgatctcagctcactgcaacttccgcctcctagattcaagtgattctcccgtcccagcctcccaagtagctgggattataggtgtcagttaccatgccctgctatttttttgtatttttagtagagaggggtttcaccatgttggccaggctggtctcaaactcctgacctcaggtgatccaccatctcagcctcctgaagtgctgggattataggtgtgagccaccgtgcctggccccatatatctctttttaagtgggcatactgccattataaataatagtgattctgctggtaatgaacaaaggatgctggatccactaatagtctgttaaacctaatatcatgactttcttgttagctatacattggtttgctataattccatttagaatttttaaacctatgttcacaaatatggatttttaaacctatgttcacaaatatggatttttaaacctatgttcacaaatatggtttgcaagtcattttttctcctaaatttctatttgatggggaagttgtaaaatattggggttatttttccttggattttccttataataactattcctgaaaagtctctggaatgtctttcttttctggggctggggtagaaggactagatagatttacaaaccagtaactcaatttctgttttgtaaaattttcatttcattaaataataagtcctaatcaagtattattctttcccacagtatgtgagtgctgtcctcaatactgtcaacacttctggcttctaccaggcaaggctgcatgtagatttgcatctgaaaaaacaacaaactaaaatctaaccctaggtagtagtaaactgaatataaactttctcttatgaatttattctgtcttctttggtacatcaataataatatacacctttacagtatttcccagattgggggatacactttagcaagtatctgcgattatttgtttatgtaagatgtcccttcccttctgtgaatcatcattcttcaccccaagtatcttgagattggattctgtataagcagaatacaacagttaggcattcaggtatcattaaattcctccgcttcaaggatgaaaatttctttgggtatctaatagagtacaaagcagaaggtgtttcagaaatatttgcagtattgaatccgcatattcctccaagatagccctaatctaactggcagggtcccactcttcccagattaatgcccactcacataacaaacctgatgaggtagtgaagaaaactaactttgtgagtaagcaactggcagagtttttcaccactgtgactctatagctacatgtaactaagtagtatcactgacacataatcttaaattgaagttttaagatcattattctccatgttatacatgggtatcaaaagcattcccctcttgaccactccagaattctgtttaaaatttttcaatgacaacttatccatttccccaaagcctcagtgagcacatgatgccaacaattcatttcatgacttcatagcatgggccaagtttcttgcttaaaagacttccatcctgtcttgggaaacaaccatttccaaatatccacatatccttgcaagtttctgcctactcctctaccacccatttctgaagccatctgatttagtaagctgtatgcaaaagatacacaatggctaatgcaatcaaacaaggaatgtattaaaagcacacccaatagctcaaaataaaagacaagtgaacaaagttaagaaaatgacagtaacaaaagctgttctgggaacctctattgaaatagctacttattacatcaacatgctaccacagaacaaaagctcatgttgcttttctgaacttgaaaaacccattaacaatgtacagttctgagcctcagctgaccatagtgctcatgccaagtcctgagcagggcatcttgaatggtggttccctcatgactacatacaccgttagggaatgtttcgttaagaggaaatcaagatgttctaacctgtgaaggtagaatagattccaggctacacaaacacatgaagtgtgccttatattgattactaaagaggttgctgccaagactgcttccaaagggcagaagatagccctaaaaaatgtttgcagtgtggaaatgcatttttagtaagtcatattctagtaacaagttgcatttggtaagacacaaagaaacaatgttggtatgcagagtagaaatctctggaagatgatattgtcatatcagagatattgtcagtatcagagatactgaaatctctggaagatgatttttgtctcacatatggcattcgcaagtaaaatgccaaactgcaaaattcatattatgtagtacacataggaagatatctaaatatccctgtaggctctgggatgttatttcttattcttaacctccttactagattcacttgtacaatgaaataatctgtatcttattatttataattgagaattttctcaaaccttttcctgaaattttggaacacctggaataaaatttcttaaaatgattcctaaaagaaataattcttcaaaattaatattaagatataataacaggttggtttttttttttttttttttttttttttttagaatgaagcttctaaggtgaggttaacagtccagctgtggtttatttggtacattcataagatgttcactcctatatatattttttccctaggggtttctcatttctagatttacactttcccttatagcatggtccctccaaggtatatgcttccgatacataaaatgtttgtaattttgttaattctgccattcattagctcaataatttctctcattaaaattctgtaaactatgaatttcaaagaagtctattctatattcatctggttcatgaagtttcctctttgtgaatcttattttagtaaaatgactttacaacgtttaacatggttcctcacctgtatgaactttttaaaaaaaggtatgacttgctgctaaaaattttcagagtggttactaaattcagttttcctgtgtattgtctactatctttttgcatgtaaagaacagctttctgtggatgcctttccatatgctgtgcattcataaagtttctattcagtatgagttttctggaagatgacaagatgattccacttacagagtttctctttatatatgattgtttctatctcttgtgaatccacttttcagagtttcgtaaaattatcaatgtttgtcatctacatgagttctctgatgcataatgagctgtgacttccaacaaaaggctttcccacattcagtgcacttacaaggcttctctcctgtatgtgttctctgatgtgcactgagaattgatttttgagagaaggttttcccacattcattgcacccatagggtttctctcctgaatgagttctttgatgtacaatgagttgagaattcctaatgaaggcttttccacactcactgcattcatatggtttctctcttgtgtgcattctctggtgtacaagaaggcgtaatttcccactgaaggatttctcacattgactgcatttataagggttgacccctgcatgagttcgctcatgtacaatgagtagtgatttccaaatgaaggctttcccacattcattacattcatatggtttttcacctgaatgagttctcatgtgtataattaggtatgacttgctgctaaaagctttcccacattcactgcacccataaggcttttcccctgcatgagttcgctgatgtgaaatgagctggtctttcctattaaaggctttcccacattcactgcattcatagggattttctcctgtgtgaattctctgatgcacaatgagttgtgaattgaaactaaaggatttcccgcattccctgcactcatgtggtttctctcctgtatgagttctcatatgtataataaggtatgacttgctcctgaaggctttcccacactcactgcatccatatggttttactcctgtgtgacttctctgatgtacaatgagctgggacttcaaactaaaggtttttgcacattgactgcatccatagggttttactccagtgtgcactcctttatgtacaatgagctgtgatttgaacgtaaaggcttttccacattcattacaactatagggtttctctcctgtatgagttctctgatgtacaatcaggtttgactttgtattaaaggctttctgacactcactacattcaaatggtttctcccctgtatgagttctctggtgtataataagctgtgactttaaaccaaaagcctttccacagtcggtgcattcataaggcttctctcctgcatgagttctctggtgtgaaataagctggtatttccgactgaaggctttcccacattcatggcattcataggggttctctcctgtatgaatcctctgatgtataatgagctgtgatttaaaactgaaggctttcccacaattgttgcattcatggagtttttctcctgtatgagtccttgtatgtataataaggtatgacttgctcctgaaggctttgccacattcattgcatacataaggtttcattcctgtgtgacttctctgatgtacaatgagctgtgatttcaaactgaatcctttaccacactgaatacacccatagggctttactcctgtgtgaatcccctgatgtacaatgagctgtgacttgaatgtaaaggcttttccacaatcactacaaacataaggtttctcccctgtatgggttctctgatgtaccataaggtttgactttgtattaaaggctttctgacattcattgcattcatatggtttctctcctgtatgaattctttcatgtataatgagctgtgattttaaaccaaaagctttcccacattcattacacacatatggtttctgtcctgaatgagttttctggtgtgaaacaagctggtctttcctactgaagactttcccacattcacagcactcatagggattctcacctgtgtgaattctctgatgtataacaagctgtgaatggaaactgaatgttttcctgcattcactgcattcatgtagtttctctcctgtatgaattctctgatgtacaatgaggtatgatttactactgaagtctttcccacattcattacaaccatagggtttctcttcggcatgagtttgctgatgcactagaaggtatgacttgctgctgaaggctttctcacaacagctgcatccaaagggtttttcgcccatatacatttgttggcacataagttgcgatttcttattgacggtttttccagattcaatactttcacagtattttattccaataacagtttgctcatgtttagaatggaagaatgattttccatgtacctgaaacccattaggattatttctagcataatcactagtgaaatctatatatttcaaactctttccatgcgtgccacatttatgaggtttttgtcttgaaagatactttgtactaagaagacatagttttccaaatgtagtgcattcaaagctttttgccgtacttcccagcttgtctttattttcctgatgccaatccataagatcatcaattttccagactgtgtttggacaggtctgatttggaacttgggcctgcaccatacacagctcttctccttgttccaacttgaagatgatatcaggtttggtgtgttggtaccctagggacaccaggttgctatagttctccaacatcacactcctgtacaggcacttctgtgctgggtctagcagctgccactcctcccaggtaaaatccacaaacacatccatgaatgacaaaggtccccaggacttggtgatttttggctgctcttgggaaataaacagccactctaggactttctctattctgcgactcttctgcttctgcctgggtgttccagggagaggttgcagaccaggagtcccttggcccaagatggattcctgaccttggagctttctgatcctatcccatgaactgtttcgttcttggagaggtgggacccaaatagaagctgtccggaccctggtggccatccctacggtcagttttgtgtgcctcgctggaagtgacaggacgcgagggatgctccagatctgcagccagaagggttcgcaaccactccagactcggctggcccgttgaccacgacgggcgatgaacgctatctgaggaacaaggatctcgccatcggcgcggaacaatggcggccgctacgtat

SEQ ID NO: 14844 - RNA, 6806 nt, Homo sapiens
  source 1..6806: mol_type = other RNA
gctgggattacaggcatgagccacggcgcctgaccacacctggctaatctttttaaaaagtttttgtacagacagggtctccctatattggtcaggcttgtctcgaactcctgggttccagcaatcctccagcctcagccttcccaagtgctggtattacatggatgagccactgcacctggctaattttactttaaaggaatctttctactattttatcattaagtatgacatttgtgttttcagaacatatattccctaccaagttacaggagttaattttaattcccaacttaatagtattttagtgtcatctatgggtgttaaattccatcaagtgatttatcagcatatactgagataatccttatgagttttatctggtagttaattaaaatattttctaatattaaatcttccaaacatactcttctgttttttgagacagggtctagttctgtcacccagggtggagtacagtggtacgatctcagctcactgcaacttccgcctcctagattcaagtgattctcccgtcccagcctcccaagtagctgggattataggtgtcagttaccatgccctgctatttttttgtatttttagtagagaggggtttcaccatgttggccaggctggtctcaaactcctgacctcaggtgatccaccatctcagcctcctgaagtgctgggattataggtgtgagccaccgtgcctggccccatatatctctttttaagtgggcatactgccattataaataatagtgattctgctggtaatgaacaaaggatgctggatccactaatagtctgttaaacctaatatcatgactttcttgttagctatacattggtttgctataattccatttagaatttttaaacctatgttcacaaatatggatttttaaacctatgttcacaaatatggatttttaaacctatgttcacaaatatggtttgcaagtcattttttctcctaaatttctatttgatggggaagttgtaaaatattggggttatttttccttggattttccttataataactattcctgaaaagtctctggaatgtctttcttttctggggctggggtagaaggactagatagatttacaaaccagtaactcaatttctgttttgtaaaattttcatttcattaaataataagtcctaatcaagtattattctttcccacagtatgtgagtgctgtcctcaatactgtcaacacttctggcttctaccaggcaaggctgcatgtagatttgcatctgaaaaaacaacaaactaaaatctaaccctaggtagtagtaaactgaatataaactttctcttatgaatttattctgtcttctttggtacatcaataataatatacacctttacagtatttcccagattgggggatacactttagcaagtatctgcgattatttgtttatgtaagatgtcccttcccttctgtgaatcatcattcttcaccccaagtatcttgagattggattctgtataagcagaatacaacagttaggcattcaggtatcattaaattcctccgcttcaaggatgaaaatttctttgggtatctaatagagtacaaagcagaaggtgtttcagaaatatttgcagtattgaatccgcatattcctccaagatagccctaatctaactggcagggtcccactcttcccagattaatgcccactcacataacaaacctgatgaggtagtgaagaaaactaactttgtgagtaagcaactggcagagtttttcaccactgtgactctatagctacatgtaactaagtagtatcactgacacataatcttaaattgaagttttaagatcattattctccatgttatacatgggtatcaaaagcattcccctcttgaccactccagaattctgtttaaaatttttcaatgacaacttatccatttccccaaagcctcagtgagcacatgatgccaacaattcatttcatgacttcatagcatgggccaagtttcttgcttaaaagacttccatcctgtcttgggaaacaaccatttccaaatatccacatatccttgcaagtttctgcctactcctctaccacccatttctgaagccatctgatttagtaagctgtatgcaaaagatacacaatggctaatgcaatcaaacaaggaatgtattaaaagcacacccaatagctcaaaataaaagacaagtgaacaaagttaagaaaatgacagtaacaaaagctgttctgggaacctctattgaaatagctacttattacatcaacatgctaccacagaacaaaagctcatgttgcttttctgaacttgaaaaacccattaacaatgtacagttctgagcctcagctgaccatagtgctcatgccaagtcctgagcagggcatcttgaatggtggttccctcatgactacatacaccgttagggaatgtttcgttaagaggaaatcaagatgttctaacctgtgaaggtagaatagattccaggctacacaaacacatgaagtgtgccttatattgattactaaagaggttgctgccaagactgcttccaaagggcagaagatagccctaaaaaatgtttgcagtgtggaaatgcatttttagtaagtcatattctagtaacaagttgcatttggtaagacacaaagaaacaatgttggtatgcagagtagaaatctctggaagatgatattgtcatatcagagatattgtcagtatcagagatactgaaatctctggaagatgatttttgtctcacatatggcattcgcaagtaaaatgccaaactgcaaaattcatattatgtagtacacataggaagatatctaaatatccctgtaggctctgggatgttatttcttattcttaacctccttactagattcacttgtacaatgaaataatctgtatcttattatttataattgagaattttctcaaaccttttcctgaaattttggaacacctggaataaaatttcttaaaatgattcctaaaagaaataattcttcaaaattaatattaagatataataacaggttggtttttttttttttttttttttttttttttagaatgaagcttctaaggtgaggttaacagtccagctgtggtttatttggtacattcataagatgttcactcctatatatattttttccctaggggtttctcatttctagatttacactttcccttatagcatggtccctccaaggtatatgcttccgatacataaaatgtttgtaattttgttaattctgccattcattagctcaataatttctctcattaaaattctgtaaactatgaatttcaaagaagtctattctatattcatctggttcatgaagtttcctctttgtgaatcttattttagtaaaatgactttacaacgtttaacatggttcctcacctgtatgaactttttaaaaaaaggtatgacttgctgctaaaaattttcagagtggttactaaattcagttttcctgtgtattgtctactatctttttgcatgtaaagaacagctttctgtggatgcctttccatatgctgtgcattcataaagtttctattcagtatgagttttctggaagatgacaagatgattccacttacagagtttctctttatatatgattgtttctatctcttgtgaatccacttttcagagtttcgtaaaattatcaatgtttgtcatctacatgagttctctgatgcataatgagctgtgacttccaacaaaaggctttcccacattcagtgcacttacaaggcttctctcctgtatgtgttctctgatgtgcactgagaattgatttttgagagaaggttttcccacattcattgcacccatagggtttctctcctgaatgagttctttgatgtacaatgagttgagaattcctaatgaaggcttttccacactcactgcattcatatggtttctctcttgtgtgcattctctggtgtacaagaaggcgtaatttcccactgaaggatttctcacattgactgcatttataagggttgacccctgcatgagttcgctcatgtacaatgagtagtgatttccaaatgaaggctttcccacattcattacattcatatggtttttcacctgaatgagttctcatgtgtataattaggtatgacttgctgctaaaagctttcccacattcactgcacccataaggcttttcccctgcatgagttcgctgatgtgaaatgagctggtctttcctattaaaggctttcccacattcactgcattcatagggattttctcctgtgtgaattctctgatgcacaatgagttgtgaattgaaactaaaggatttcccgcattccctgcactcatgtggtttctctcctgtatgagttctcatatgtataataaggtatgacttgctcctgaaggctttcccacactcactgcatccatatggttttactcctgtgtgacttctctgatgtacaatgagctgggacttcaaactaaaggtttttgcacattgactgcatccatagggttttactccagtgtgcactcctttatgtacaatgagctgtgatttgaacgtaaaggcttttccacattcattacaactatagggtttctctcctgtatgagttctctgatgtacaatcaggtttgactttgtattaaaggctttctgacactcactacattcaaatggtttctcccctgtatgagttctctggtgtataataagctgtgactttaaaccaaaagcctttccacagtcggtgcattcataaggcttctctcctgcatgagttctctggtgtgaaataagctggtatttccgactgaaggctttcccacattcatggcattcataggggttctctcctgtatgaatcctctgatgtataatgagctgtgatttaaaactgaaggctttcccacaattgttgcattcatggagtttttctcctgtatgagtccttgtatgtataataaggtatgacttgctcctgaaggctttgccacattcattgcatacataaggtttcattcctgtgtgacttctctgatgtacaatgagctgtgatttcaaactgaatcctttaccacactgaatacacccatagggctttactcctgtgtgaatcccctgatgtacaatgagctgtgacttgaatgtaaaggcttttccacaatcactacaaacataaggtttctcccctgtatgggttctctgatgtaccataaggtttgactttgtattaaaggctttctgacattcattgcattcatatggtttctctcctgtatgaattctttcatgtataatgagctgtgattttaaaccaaaagctttcccacattcattacacacatatggtttctgtcctgaatgagttttctggtgtgaaacaagctggtctttcctactgaagactttcccacattcacagcactcatagggattctcacctgtgtgaattctctgatgtataacaagctgtgaatggaaactgaatgttttcctgcattcactgcattcatgtagtttctctcctgtatgaattctctgatgtacaatgaggtatgatttactactgaagtctttcccacattcattacaaccatagggtttctcttcggcatgagtttgctgatgcactagaaggtatgacttgctgctgaaggctttctcacaacagctgcatccaaagggtttttcgcccatatacatttgttggcacataagttgcgatttcttattgacggtttttccagattcaatactttcacagtattttattccaataacagtttgctcatgtttagaatggaagaatgattttccatgtacctgaaacccattaggattatttctagcataatcactagtgaaatctatatatttcaaactctttccatgcgtgccacatttatgaggtttttgtcttgaaagatactttgtactaagaagacatagttttccaaatgtagtgcattcaaagctttttgccgtacttcccagcttgtctttattttcctgatgccaatccataagatcatcaattttccagactgtgtttggacaggtctgatttggaacttgggcctgcaccatacacagctcttctccttgttccaacttgaagatgatatcaggtttggtgtgttggtaccctagggacaccaggttgctatagttctccaacatcacactcctgtacaggcacttctgtgctgggtctagcagctgccactcctcccaggtaaaatccacaaacacatccatgaatgacaaaggtccccaggacttggtgatttttggctgctcttgggaaataaacagccactctaggactttctctattctgcgactcttctgcttctgcctgggtgttccagggagaggttgcagaccaggagtcccttggcccaagatggattcctgaccttggagctttctgatcctatcccatgaactgtttcgttcttggagaggtgggacccaaatagaagctgtccggaccctggtggccatccctacggtcagttttgtgtgcctcgctggaagtgacaggacgcgagggatgctccggctcctccaaaccctgaaggggcagcagaatagagtccagggtactgcctccacctccagatctgcagccagaagggttcgcaaccactccagactcggctggcccgttgaccacgacgggcgatgaacgctatctgaggaacaaggatctcgccatcggcgcggaacaatggcggccgctacgtat

SEQ ID NO: 14845 - RNA, 6754 nt, Homo sapiens
  source 1..6754: mol_type = other RNA
gctgggattacaggcatgagccacggcgcctgaccacacctggctaatctttttaaaaagtttttgtacagacagggtctccctatattggtcaggcttgtctcgaactcctgggttccagcaatcctccagcctcagccttcccaagtgctggtattacatggatgagccactgcacctggctaattttactttaaaggaatctttctactattttatcattaagtatgacatttgtgttttcagaacatatattccctaccaagttacaggagttaattttaattcccaacttaatagtattttagtgtcatctatgggtgttaaattccatcaagtgatttatcagcatatactgagataatccttatgagttttatctggtagttaattaaaatattttctaatattaaatcttccaaacatactcttctgttttttgagacagggtctagttctgtcacccagggtggagtacagtggtacgatctcagctcactgcaacttccgcctcctagattcaagtgattctcccgtcccagcctcccaagtagctgggattataggtgtcagttaccatgccctgctatttttttgtatttttagtagagaggggtttcaccatgttggccaggctggtctcaaactcctgacctcaggtgatccaccatctcagcctcctgaagtgctgggattataggtgtgagccaccgtgcctggccccatatatctctttttaagtgggcatactgccattataaataatagtgattctgctggtaatgaacaaaggatgctggatccactaatagtctgttaaacctaatatcatgactttcttgttagctatacattggtttgctataattccatttagaatttttaaacctatgttcacaaatatggatttttaaacctatgttcacaaatatggatttttaaacctatgttcacaaatatggtttgcaagtcattttttctcctaaatttctatttgatggggaagttgtaaaatattggggttatttttccttggattttccttataataactattcctgaaaagtctctggaatgtctttcttttctggggctggggtagaaggactagatagatttacaaaccagtaactcaatttctgttttgtaaaattttcatttcattaaataataagtcctaatcaagtattattctttcccacagtatgtgagtgctgtcctcaatactgtcaacacttctggcttctaccaggcaaggctgcatgtagatttgcatctgaaaaaacaacaaactaaaatctaaccctaggtagtagtaaactgaatataaactttctcttatgaatttattctgtcttctttggtacatcaataataatatacacctttacagtatttcccagattgggggatacactttagcaagtatctgcgattatttgtttatgtaagatgtcccttcccttctgtgaatcatcattcttcaccccaagtatcttgagattggattctgtataagcagaatacaacagttaggcattcaggtatcattaaattcctccgcttcaaggatgaaaatttctttgggtatctaatagagtacaaagcagaaggtgtttcagaaatatttgcagtattgaatccgcatattcctccaagatagccctaatctaactggcagggtcccactcttcccagattaatgcccactcacataacaaacctgatgaggtagtgaagaaaactaactttgtgagtaagcaactggcagagtttttcaccactgtgactctatagctacatgtaactaagtagtatcactgacacataatcttaaattgaagttttaagatcattattctccatgttatacatgggtatcaaaagcattcccctcttgaccactccagaattctgtttaaaatttttcaatgacaacttatccatttccccaaagcctcagtgagcacatgatgccaacaattcatttcatgacttcatagcatgggccaagtttcttgcttaaaagacttccatcctgtcttgggaaacaaccatttccaaatatccacatatccttgcaagtttctgcctactcctctaccacccatttctgaagccatctgatttagtaagctgtatgcaaaagatacacaatggctaatgcaatcaaacaaggaatgtattaaaagcacacccaatagctcaaaataaaagacaagtgaacaaagttaagaaaatgacagtaacaaaagctgttctgggaacctctattgaaatagctacttattacatcaacatgctaccacagaacaaaagctcatgttgcttttctgaacttgaaaaacccattaacaatgtacagttctgagcctcagctgaccatagtgctcatgccaagtcctgagcagggcatcttgaatggtggttccctcatgactacatacaccgttagggaatgtttcgttaagaggaaatcaagatgttctaacctgtgaaggtagaatagattccaggctacacaaacacatgaagtgtgccttatattgattactaaagaggttgctgccaagactgcttccaaagggcagaagatagccctaaaaaatgtttgcagtgtggaaatgcatttttagtaagtcatattctagtaacaagttgcatttggtaagacacaaagaaacaatgttggtatgcagagtagaaatctctggaagatgatattgtcatatcagagatattgtcagtatcagagatactgaaatctctggaagatgatttttgtctcacatatggcattcgcaagtaaaatgccaaactgcaaaattcatattatgtagtacacataggaagatatctaaatatccctgtaggctctgggatgttatttcttattcttaacctccttactagattcacttgtacaatgaaataatctgtatcttattatttataattgagaattttctcaaaccttttcctgaaattttggaacacctggaataaaatttcttaaaatgattcctaaaagaaataattcttcaaaattaatattaagatataataacaggttggtttttttttttttttttttttttttttttagaatgaagcttctaaggtgaggttaacagtccagctgtggtttatttggtacattcataagatgttcactcctatatatattttttccctaggggtttctcatttctagatttacactttcccttatagcatggtccctccaaggtatatgcttccgatacataaaatgtttgtaattttgttaattctgccattcattagctcaataatttctctcattaaaattctgtaaactatgaatttcaaagaagtctattctatattcatctggttcatgaagtttcctctttgtgaatcttattttagtaaaatgactttacaacgtttaacatggttcctcacctgtatgaactttttaaaaaaaggtatgacttgctgctaaaaattttcagagtggttactaaattcagttttcctgtgtattgtctactatctttttgcatgtaaagaacagctttctgtggatgcctttccatatgctgtgcattcataaagtttctattcagtatgagttttctggaagatgacaagatgattccacttacagagtttctctttatatatgattgtttctatctcttgtgaatccacttttcagagtttcgtaaaattatcaatgtttgtcatctacatgagttctctgatgcataatgagctgtgacttccaacaaaaggctttcccacattcagtgcacttacaaggcttctctcctgtatgtgttctctgatgtgcactgagaattgatttttgagagaaggttttcccacattcattgcacccatagggtttctctcctgaatgagttctttgatgtacaatgagttgagaattcctaatgaaggcttttccacactcactgcattcatatggtttctctcttgtgtgcattctctggtgtacaagaaggcgtaatttcccactgaaggatttctcacattgactgcatttataagggttgacccctgcatgagttcgctcatgtacaatgagtagtgatttccaaatgaaggctttcccacattcattacattcatatggtttttcacctgaatgagttctcatgtgtataattaggtatgacttgctgctaaaagctttcccacattcactgcacccataaggcttttcccctgcatgagttcgctgatgtgaaatgagctggtctttcctattaaaggctttcccacattcactgcattcatagggattttctcctgtgtgaattctctgatgcacaatgagttgtgaattgaaactaaaggatttcccgcattccctgcactcatgtggtttctctcctgtatgagttctcatatgtataataaggtatgacttgctcctgaaggctttcccacactcactgcatccatatggttttactcctgtgtgacttctctgatgtacaatgagctgggacttcaaactaaaggtttttgcacattgactgcatccatagggttttactccagtgtgcactcctttatgtacaatgagctgtgatttgaacgtaaaggcttttccacattcattacaactatagggtttctctcctgtatgagttctctgatgtacaatcaggtttgactttgtattaaaggctttctgacactcactacattcaaatggtttctcccctgtatgagttctctggtgtataataagctgtgactttaaaccaaaagcctttccacagtcggtgcattcataaggcttctctcctgcatgagttctctggtgtgaaataagctggtatttccgactgaaggctttcccacattcatggcattcataggggttctctcctgtatgaatcctctgatgtataatgagctgtgatttaaaactgaaggctttcccacaattgttgcattcatggagtttttctcctgtatgagtccttgtatgtataataaggtatgacttgctcctgaaggctttgccacattcattgcatacataaggtttcattcctgtgtgacttctctgatgtacaatgagctgtgatttcaaactgaatcctttaccacactgaatacacccatagggctttactcctgtgtgaatcccctgatgtacaatgagctgtgacttgaatgtaaaggcttttccacaatcactacaaacataaggtttctcccctgtatgggttctctgatgtaccataaggtttgactttgtattaaaggctttctgacattcattgcattcatatggtttctctcctgtatgaattctttcatgtataatgagctgtgattttaaaccaaaagctttcccacattcattacacacatatggtttctgtcctgaatgagttttctggtgtgaaacaagctggtctttcctactgaagactttcccacattcacagcactcatagggattctcacctgtgtgaattctctgatgtataacaagctgtgaatggaaactgaatgttttcctgcattcactgcattcatgtagtttctctcctgtatgaattctctgatgtacaatgaggtatgatttactactgaagtctttcccacattcattacaaccatagggtttctcttcggcatgagtttgctgatgcactagaaggtatgacttgctgctgaaggctttctcacaacagctgcatccaaagggtttttcgcccatatacatttgttggcacataagttgcgatttcttattgacggtttttccagattcaatactttcacagtattttattccaataacagtttgctcatgtttagaatggaagaatgattttccatgtacctgaaacccattaggattatttctagcataatcactagtgaaatctatatatttcaaactctttccatgcgtgccacatttatgaggtttttgtcttgaaagatactttgtactaagaagacatagttttccaaatgtagtgcattcaaagctttttgccgtacttcccagcttgtctttattttcctgatgccaatccataagatcatcaattttccagactgtgtttggacaggtctgatttggaacttgggcctgcaccatacacagctcttctccttgttccaacttgaagatgatatcaggtttggtgtgttggtaccctagggacaccaggttgctatagttctccaacatcacactcctgtacaggcacttctgtgctgggtctagcagctgccactcctcccaggtaaaatccacaaacacatccatgaatgacaaaggtccccaggacttggtgatttttggctgctcttgggaaataaacagccactctaggactttctctattctgcgactcttctgcttctgcctgggtgttccagggagaggttgcagaccaggagtcccttggcccaagatggattcctgaccttggagctttctgatcctatcccatgaactgtttcgttcttggagaggtgggacctgtggaccaaatagaagctgtccggaccctggtggccatccctacggtcagttttgtgtgcctcgctggaagtgacaggacgcgagggatgctccagatctgcagccagaagggttcgcaaccactccagactcggctggcccgttgaccacgacgggcgatgaacgctatctgaggaacaaggatctcgccatcggcgcggaacaatggcggccgctacgtat

SEQ ID NO: 14846 - RNA, 2650 nt, Homo sapiens
  source 1..2650: mol_type = other RNA
gctgggattacaggcatgagccacggcgctagcctcctaaacaattttaaacatgaaagtggtttggaggcgatttagaatttgggtcaaaactagtgagtttcaaacacttatatctgcaatgtaacttataaggcagaaaaggcagacttttccctactcccgccttttttttttcttttattgctgatcttcttggttctaaaaatttgttcagaaagcctgatggttgtttaaatgcttagcaccatgacacacgtgtaataaaaattgcataaatggaccaggcacggtggctcatgcctgtaatcccagcactttggaaggccaaggaggctggatcctctgaggtcaggagttcgagatcattctggccaacatgatgaaaccctgtctctactaaaaaaatacaaaaaattagctgagcatagtggcggacacctgtaatcccagctactcgtgaggctgaggcgggagaattgcttgaacccggaaggtggaggttacagtgagccgagatttcaccatcgcactccagcctgggcaacaagagcaaagctccatctcaaaaaaaaaaaaaaaaattgcataaatatgttaaatcacctggcaaatgattttcttcccctggtgtctatgtgttccatactattgtaggctctttaactggtaaaacagctaccccaattcagagatccagtacttaatgcatcacatttccagagttatgagaaaacagctaaacctgtgagttagactcactttgtttccccacggaggaaataaaaacccacgatttgaaacctttggaaaacataggaaatgcaacatttggaagtataacatagaaacaagagataatcatacaatgcttccaaatgaagtctcacgttggatttgctggtttttaagacagattcccctcttctggacagctgtgatggccaagatagaagttcatttgctatgtttccagggactattctctttgatgtatacaggatttatggggtctaaaaagaacatacaattataaagtgttcatatttgagagaaaactgcaatgatcagaaggattgagccagttttagcataaaaaattaggactacattaatgatgaggttgactatacacagtttggagtgagagagttactctacccagtatcactgacatgttggaatgccagatgaaactgaaacagaaaaattgtcttggggtctaaaagacgtctgatgtgctgatgtctgttcagtcttctgcactcatgggcgtaaactctcaaagagcaccactgggtcttagtccgtggcataaagactattctcaatgtagatattgtcttctgcttggacttccttttcaactgcattttgcaaagctttaatttgaaggctgctaaatgaaacattttggcaatgatgacacccaaaagagcaagaagcaccaagacagaaatacagactccagcatagattcctttagtggtattggccgtcagtagactatgttctaggaacagttgagtttgattgttattccaaaggccatctgaagactctgtcacggtgtcattcccatctgttgtgtaagagtacaatggtgagctggtgggttctctccttattgctccctgcagtgtcgtagggtgggtttctgctggctgaggtgaagatggtgaagtggctactggttcatggttctgcctgggcaaaggcattggaggaacaaaggtagagacagttgttgtcactggaacacttgttgttgttggaatgctcgttgtcgttggaacgctcgttgtcgttgaaacagtcattgtcgtcagaacagtcgttgtcgttggaatgctcattgttgttggaacagttgtcgttggaacagtcgtcattggaacagtcgttgtcgttggaacagtggtgctcgttcgaacagtcgtgacggttggaacagttgtgacaattggagtagtcgtgaccttgggtggcacaatctccaatgatacggtgattttcatgtcattgaaccacccacggtgctcaacacggcaacaatatacgccactgtcagacacagctgtattttctatggtcaaagagacatcccttcttgaaaggtcccccaatagcttatagcgtgtgtccttccgataggtgacgtgggttccattggtccagacaatgccattttggcatgtgaatagagaacatgagcctctattccagcacatggatgtgacagctccactgtagtggcagggtagtgtgacagatggacctgcctctccaccaacctttacagaaccagctacagaatctgccagatgtaggatgaggcttaagatgaccacttgaggatgcattatgggatcagccggttagttagaaggcggttttccagcttctcctccctcctcctggtctgtttgtagccctcctccaaagatctttatagattaagactactttctcccagaattccattctttatctctttgccacacctttacataagaatacggggaagcacgtttgaacattacatttctccagttggctgatctttttactggatttgatccacttacaaatttaaacagattacagggagattgttacagtacttgttctctactgggcatttgttttg

SEQ ID NO: 14847 - RNA, 2771 nt, Homo sapiens
  source 1..2771: mol_type = other RNA
gctgggattacaggcatgagccacggcgctagcctcctaaacaattttaaacatgaaagtggtttggaggcgatttagaatttgggtcaaaactagtgagtttcaaacacttatatctgcaatgtaacttataaggcagaaaaggcagacttttccctactcccgccttttttttttcttttattgctgatcttcttggttctaaaaatttgttcagaaagcctgatggttgtttaaatgcttagcaccatgacacacgtgtaataaaaattgcataaatggaccaggcacggtggctcatgcctgtaatcccagcactttggaaggccaaggaggctggatcctctgaggtcaggagttcgagatcattctggccaacatgatgaaaccctgtctctactaaaaaaatacaaaaaattagctgagcatagtggcggacacctgtaatcccagctactcgtgaggctgaggcgggagaattgcttgaacccggaaggtggaggttacagtgagccgagatttcaccatcgcactccagcctgggcaacaagagcaaagctccatctcaaaaaaaaaaaaaaaaattgcataaatatgttaaatcacctggcaaatgattttcttcccctggtgtctatgtgttccatactattgtaggctctttaactggtaaaacagctaccccaattcagagatccagtacttaatgcatcacatttccagagttatgagaaaacagctaaacctgtgagttagactcactttgtttccccacggaggaaataaaaacccacgatttgaaacctttggaaaacataggaaatgcaacatttggaagtataacatagaaacaagagataatcatacaatgcttccaaatgaagtctcacgttggatttgctggtttttaagacagattcccctcttctggacagctgtgatggccaagatagaagttcatttgctatgtttccagggactattctctttgatgtatacaggatttatggggtctaaaaagaacatacaattataaagtgttcatatttgagagaaaactgcaatgatcagaaggattgagccagttttagcataaaaaattaggactacattaatgatgaggttgactatacacagtttggagtgagagagttactctacccagtatcactgacatgttggaatgccagatgaaactgaaacagaaaaattgtcttggggtctaaaagacgtctgatgtgctgatgtctgttcagtcttctgcactcatgggcgtaaactctcaaagagcaccactgggtcttagtccgtggcataaagactattctcaatgtagatattgtcttctgcttggacttccttttcaactgcattttgcaaagctttaatttgaaggctgctaaatgaaacattttggcaatgatgacacccaaaagagcaagaagcaccaagacagaaatacagactccagcatagattcctttagtggtattggccgtcagtagactatgttctaggaacagttgagtttgattgttattccaaaggccatctgaagactctgtcacggtgtcattcccatctgttgtgtaagagtacaatggtgagctggtgggttctctccttattgctccctgcagtgtcgtagggtgggtttctgctggctgaggtgaagatggtgaagtggctactggttcatggttctgcctgggcaaaggcattggaggaacaaaggtagagacagttgttgtcactggaacacttgttgttgttggaatgctcgttgtcgttggaacgctcgttgtcgttgaaacagtcattgtcgtcagaacagtcgttgtcgttggaatgctcattgttgttggaacagttgtcgttggaacagtcgtcattggaacagtcgttgtcgttggaacagtggtgctcgttcgaacagtcgtgacggttggaacagttgtgacaattggagtagtcgtgaccttgggtggcacaatctccaatgatacggtgattttcatgtcattgaaccacccacggtgctcaacacggcaacaatatacgccactgtcagacacagctgtattttctatggtcaaagagacatcccttcttgaaaggtcccccaatagcttatagcgtgtgtccttccgataggtgacgtgggttccattggtccagacaatgccattttggcatgtgaatagagaacatgagcctctattccagcacatggatgtgacagctccactgtagtggcagggtagtgtgacagatggacctgcctctccaccaacctttacagaaccagctacagaatctgccagatgtaggatgaggcttaagatgaccacttgaggatgcattatgggatcagcctgaaggaaaatgagcagacaggctggttggtaccctccaccagatggtatctgatcaagtcttaaatctcagattgcaacttatcttttcacccagttggttgattcatatgagcctgctcggttagttagaaggcggttttccagcttctcctccctcctcctggtctgtttgtagccctcctccaaagatctttatagattaagactactttctcccagaattccattctttatctctttgccacacctttacataagaatacggggaagcacgtttgaacattacatttctccagttggctgatctttttactggatttgatccacttacaaatttaaacagattacagggagattgttacagtacttgttctctactgggcatttgttttg

SEQ ID NO: 14848 - RNA, 2774 nt, Homo sapiens
  source 1..2774: mol_type = other RNA
gctgggattacaggcatgagccacggcgctagcctcctaaacaattttaaacatgaaagtggtttggaggcgatttagaatttgggtcaaaactagtgagtttcaaacacttatatctgcaatgtaacttataaggcagaaaaggcagacttttccctactcccgccttttttttttcttttattgctgatcttcttggttctaaaaatttgttcagaaagcctgatggttgtttaaatgcttagcaccatgacacacgtgtaataaaaattgcataaatggaccaggcacggtggctcatgcctgtaatcccagcactttggaaggccaaggaggctggatcctctgaggtcaggagttcgagatcattctggccaacatgatgaaaccctgtctctactaaaaaaatacaaaaaattagctgagcatagtggcggacacctgtaatcccagctactcgtgaggctgaggcgggagaattgcttgaacccggaaggtggaggttacagtgagccgagatttcaccatcgcactccagcctgggcaacaagagcaaagctccatctcaaaaaaaaaaaaaaaaattgcataaatatgttaaatcacctggcaaatgattttcttcccctggtgtctatgtgttccatactattgtaggctctttaactggtaaaacagctaccccaattcagagatccagtacttaatgcatcacatttccagagttatgagaaaacagctaaacctgtgagttagactcactttgtttccccacggaggaaataaaaacccacgatttgaaacctttggaaaacataggaaatgcaacatttggaagtataacatagaaacaagagataatcatacaatgcttccaaatgaagtctcacgttggatttgctggtttttaagacagattcccctcttctggacagctgtgatggccaagatagaagttcatttgctatgtttccagggactattctctttgatgtatacaggatttatggggtctaaaaagaacatacaattataaagtgttcatatttgagagaaaactgcaatgatcagaaggattgagccagttttagcataaaaaattaggactacattaatgatgaggttgactatacacagtttggagtgagagagttactctacccagtatcactgacatgttggaatgccagatgaaactgaaacagaaaaattgtcttggggtctaaaagacgtctgatgtgctgatgtctgttcagtcttctgcactcatgggcgtaaactctcaaagagcaccactgggtcttagtccgtggcataaagactattctcaatgtagatattgtcttctgcttggacttccttttcaactgcattttgcaaagctttaatttgaaggctgctaaatgaaacattttggcaatgatgacacccaaaagagcaagaagcaccaagacagaaatacagactccagcatagattcctttagtggtattggccgtcagtagactatgttctaggaacagttgagtttgattgttattccaaaggccatctgaagactctgtcacggtgtcattcccatctgttgtgtaagagtacaatggtgagctggtgggttctctccttattgctccctgcagtgtcgtagggtgggtttctgctggctgaggtgaagatggtgaagtggctactggttcatggttctgcctgggcaaaggcattggaggaacaaaggtagagacagttgttgtcactggaacacttgttgttgttggaatgctcgttgtcgttggaacgctcgttgtcgttgaaacagtcattgtcgtcagaacagtcgttgtcgttggaatgctcattgttgttggaacagttgtcgttggaacagtcgtcattggaacagtcgttgtcgttggaacagtggtgctcgttcgaacagtcgtgacggttggaacagttgtgacaattggagtagtcgtgaccttgggtggcacaatctccaatgatacggtgattttcatgtcattgaaccacccacggtgctcaacacggcaacaatatacgccactgtcagacacagctgtattttctatggtcaaagagacatcccttcttgaaaggtcccccaatagcttatagcgtgtgtccttccgataggtgacgtgggttccattggtccagacaatgccattttggcatgtgaatagagaacatgagcctctattccagcacatggatgtgacagctccactgtagtggcagggtagtgtgacagatggacctgcctctccaccaacctttacagaaccagctacagaatctgccagatgtaggatgaggcttaagatgaccacttgaggatgcattatgggatcagcctgaaggaaaatgagcagacaggctggttggtaccctccaccagatggtatctgatcaagtcttaaatctcagattgcaacttatcttttcacccagttggttgattcatatgagcctgctctgcggttagttagaaggcggttttccagcttctcctccctcctcctggtctgtttgtagccctcctccaaagatctttatagattaagactactttctcccagaattccattctttatctctttgccacacctttacataagaatacggggaagcacgtttgaacattacatttctccagttggctgatctttttactggatttgatccacttacaaatttaaacagattacagggagattgttacagtacttgttctctactgggcatttgttttg

SEQ ID NO: 14849 - RNA, 2702 nt, Homo sapiens
  source 1..2702: mol_type = other RNA
gctgggattacaggcatgagccacggcgctagcctcctaaacaattttaaacatgaaagtggtttggaggcgatttagaatttgggtcaaaactagtgagtttcaaacacttatatctgcaatgtaacttataaggcagaaaaggcagacttttccctactcccgccttttttttttcttttattgctgatcttcttggttctaaaaatttgttcagaaagcctgatggttgtttaaatgcttagcaccatgacacacgtgtaataaaaattgcataaatggaccaggcacggtggctcatgcctgtaatcccagcactttggaaggccaaggaggctggatcctctgaggtcaggagttcgagatcattctggccaacatgatgaaaccctgtctctactaaaaaaatacaaaaaattagctgagcatagtggcggacacctgtaatcccagctactcgtgaggctgaggcgggagaattgcttgaacccggaaggtggaggttacagtgagccgagatttcaccatcgcactccagcctgggcaacaagagcaaagctccatctcaaaaaaaaaaaaaaaaattgcataaatatgttaaatcacctggcaaatgattttcttcccctggtgtctatgtgttccatactattgtaggctctttaactggtaaaacagctaccccaattcagagatccagtacttaatgcatcacatttccagagttatgagaaaacagctaaacctgtgagttagactcactttgtttccccacggaggaaataaaaacccacgatttgaaacctttggaaaacataggaaatgcaacatttggaagtataacatagaaacaagagataatcatacaatgcttccaaatgaagtctcacgttggatttgctggtttttaagacagattcccctcttctggacagctgtgatggccaagatagaagttcatttgctatgtttccagggactattctctttgatgtatacaggatttatggggtctaaaaagaacatacaattataaagtgttcatatttgagagaaaactgcaatgatcagaaggattgagccagttttagcataaaaaattaggactacattaatgatgaggttgactatacacagtttggagtgagagagttactctacccagtatcactgacatgttggaatgccagatgaaactgaaacagaaaaattgtcttggggtctaaaagacgtctgatgtgctgatgtctgttcagtcttctgcactcatgggcgtaaactctcaaagagcaccactgggtcttagtccgtggcataaagactattctcaatgtagatattgtcttctgcttggacttccttttcaactgcattttgcaaagctttaatttgaaggctgctaaatgaaacattttggcaatgatgacacccaaaagagcaagaagcaccaagacagaaatacagactccagcatagattcctttagtggtattggccgtcagtagactatgttctaggaacagttgagtttgattgttattccaaaggccatctgaagactctgtcacggtgtcattcccatctgttgtgtaagagtacaatggtgagctggtgggttctctccttattgctccctgcagtgtcgtagggtgggtttctgctggctgaggtgaagatggtgaagtggctactggttcatggttctgcctgggcaaaggcattggaggaacaaaggtagagacagttgttgtcactggaacacttgttgttgttggaatgctcgttgtcgttggaacgctcgttgtcgttgaaacagtcattgtcgtcagaacagtcgttgtcgttggaatgctcattgttgttggaacagttgtcgttggaacagtcgtcattggaacagtcgttgtcgttggaacagtggtgctcgttcgaacagtcgtgacggttggaacagttgtgacaattggagtagtcgtgaccttgggtggcacaatctccaatgatacggtgattttcatgtcattgaaccacccacggtgctcaacacggcaacaatatacgccactgtcagacacagctgtattttctatggtcaaagagacatcccttcttgaaaggtcccccaatagcttatagcgtgtgtccttccgataggtgacgtgggttccattggtccagacaatgccattttggcatgtgaatagagaacatgagcctctattccagcacatggatgtgacagctccactgtagtggcagggtagtgtgacagatggacctgcctctccaccaacctttacagaaccagctacagaatctgccagatgtaggatgaggcttaagatgaccacttgaggatgcattatgggatcagcctgaaggaaaatgagcagacaggctggttggtaccctccaccagatggtatctgatcaagtcttaaatctcagattgcaacttatcttttcacccagttggttgattcatatgagcctgctctggttcagatccaggctctgtcactcacaatgctgggtaaccctgagagttcctgagttctcttcaaacctctatttcctcagttgtaaaatagcactaaaaatgcttcctctatctcccaccaaggattgatataataagcaaaaagggccacggaagaacttggaaaactaaacctacatcatatgcagtaatagcactagct

SEQ ID NO: 14850 - RNA, 2578 nt, Homo sapiens
  source 1..2578: mol_type = other RNA
gctgggattacaggcatgagccacggcgctagcctcctaaacaattttaaacatgaaagtggtttggaggcgatttagaatttgggtcaaaactagtgagtttcaaacacttatatctgcaatgtaacttataaggcagaaaaggcagacttttccctactcccgccttttttttttcttttattgctgatcttcttggttctaaaaatttgttcagaaagcctgatggttgtttaaatgcttagcaccatgacacacgtgtaataaaaattgcataaatggaccaggcacggtggctcatgcctgtaatcccagcactttggaaggccaaggaggctggatcctctgaggtcaggagttcgagatcattctggccaacatgatgaaaccctgtctctactaaaaaaatacaaaaaattagctgagcatagtggcggacacctgtaatcccagctactcgtgaggctgaggcgggagaattgcttgaacccggaaggtggaggttacagtgagccgagatttcaccatcgcactccagcctgggcaacaagagcaaagctccatctcaaaaaaaaaaaaaaaaattgcataaatatgttaaatcacctggcaaatgattttcttcccctggtgtctatgtgttccatactattgtaggctctttaactggtaaaacagctaccccaattcagagatccagtacttaatgcatcacatttccagagttatgagaaaacagctaaacctgtgagttagactcactttgtttccccacggaggaaataaaaacccacgatttgaaacctttggaaaacataggaaatgcaacatttggaagtataacatagaaacaagagataatcatacaatgcttccaaatgaagtctcacgttggatttgctggtttttaagacagattcccctcttctggacagctgtgatggccaagatagaagttcatttgctatgtttccagggactattctctttgatgtatacaggatttatggggtctaaaaagaacatacaattataaagtgttcatatttgagagaaaactgcaatgatcagaaggattgagccagttttagcataaaaaattaggactacattaatgatgaggttgactatacacagtttggagtgagagagttactctacccagtatcactgacatgttggaatgccagatgaaactgaaacagaaaaattgtcttggggtctaaaagacgtctgatgtgctgatgtctgttcagtcttctgcactcatgggcgtaaactctcaaagagcaccactgggtcttagtccgtggcataaagactattctcaatgtagatattgtcttctgcttggacttccttttcaactgcattttgcaaagctttaatttgaaggctgctaaatgaaacattttggcaatgatgacacccaaaagagcaagaagcaccaagacagaaatacagactccagcatagattcctttagtggtattggccgtcagtagactatgttctaggaacagttgagtttgattgttattccaaaggccatctgaagactctgtcacggtgtcattcccatctgttgtgtaagagtacaatggtgagctggtgggttctctccttattgctccctgcagtgtcgtagggtgggtttctgctggctgaggtgaagatggtgaagtggctactggttcatggttctgcctgggcaaaggcattggaggaacaaaggtagagacagttgttgtcactggaacacttgttgttgttggaatgctcgttgtcgttggaacgctcgttgtcgttgaaacagtcattgtcgtcagaacagtcgttgtcgttggaatgctcattgttgttggaacagttgtcgttggaacagtcgtcattggaacagtcgttgtcgttggaacagtggtgctcgttcgaacagtcgtgacggttggaacagttgtgacaattggagtagtcgtgaccttgggtggcacaatctccaatgatacggtgattttcatgtcattgaaccacccacggtgctcaacacggcaacaatatacgccactgtcagacacagctgtattttctatggtcaaagagacatcccttcttgaaaggtcccccaatagcttatagcgtgtgtccttccgataggtgacgtgggttccattggtccagacaatgccattttggcatgtgaatagagaacatgagcctctattccagcacatggatgtgacagctccactgtagtggcagggtagtgtgacagatggacctgcctctccaccaacctttacagaaccagctacagaatctgccagatgtaggatgaggcttaagatgaccacttgaggatgcattatgggatcagcgttcagatccaggctctgtcactcacaatgctgggtaaccctgagagttcctgagttctcttcaaacctctatttcctcagttgtaaaatagcactaaaaatgcttcctctatctcccaccaaggattgatataataagcaaaaagggccacggaagaacttggaaaactaaacctacatcatatgcagtaatagcactagct

SEQ ID NO: 14851 - RNA, 2025 nt, Homo sapiens
  source 1..2025: mol_type = other RNA
gctgggattacaggcatgagccacggcgctagcctcctaaacaattttaaacatgaaagtggtttggaggcgatttagaatttgggtcaaaactagtgagtttcaaacacttatatctgcaatgtaacttataaggcagaaaaggcagacttttccctactcccgccttttttttttcttttattgctgatcttcttggttctaaaaatttgttcagaaagcctgatggttgtttaaatgcttagcaccatgacacacgtgtaataaaaattgcataaatggaccaggcacggtggctcatgcctgtaatcccagcactttggaaggccaaggaggctggatcctctgaggtcaggagttcgagatcattctggccaacatgatgaaaccctgtctctactaaaaaaatacaaaaaattagctgagcatagtggcggacacctgtaatcccagctactcgtgaggctgaggcgggagaattgcttgaacccggaaggtggaggttacagtgagccgagatttcaccatcgcactccagcctgggcaacaagagcaaagctccatctcaaaaaaaaaaaaaaaaattgcataaatatgttaaatcacctggcaaatgattttcttcccctggtgtctatgtgttccatactattgtaggctctttaactggtaaaacagctaccccaattcagagatccagtacttaatgcatcacatttccagagttatgagaaaacagctaaacctgtgagttagactcactttgtttccccacggaggaaataaaaacccacgatttgaaacctttggaaaacataggaaatgcaacatttggaagtataacatagaaacaagagataatcatacaatgcttccaaatgaagtctcacgttggatttgctggtttttaagacagattcccctcttctggacagctgtgatggccaagatagaagttcatttgctatgtttccagggactattctctttgatgtatacaggatttatggggtctaaaaagaacatacaattataaagtgttcatatttgagagaaaactgcaatgatcagaaggattgagccagttttagcataaaaaattaggactacattaatgatgaggttgactatacacagtttggagtgagagagttactctacccagtatcactgacatgttggaatgccagatgaaactgaaacagaaaaattgtcttggggtctaaaagacgtctgatgtgctgatgtctgttcagtcttctgcactcatgggcgtaaactctcaaagagcaccactgggtcttagtccgtggcataaagactattctcaatgtagatattgtcttctgcttggacttccttttcaactgcattttgcaaagctttaatttgaaggctgctaaatgaaacattttggcaatgatgacacccaaaagagcaagaagcaccaagacagaaatacagactccagcatagattcctttagtggtattggccgtcagtagactatgttctaggaacagttgagtttgattgttattccaaaggccatctgaagactctgtcacggtgtcattcccatctgttgtgtaagagtacaatggtgagctggtgggttctctccttattgctccctgcagtgtcgtagggtgggtttctgctggctgaggtgaagatggtgaagtggctactggttcatggttctgcctgggcaaaggcattggaggaacaaaggtagagacagttgttgtcactggaacacttgttgttgttggaatgctcgttgtcgttggaacgctcgttgtcgttgaaacagtcattgtcgtcagaacagtcgttgtcgttggaatgctcattgttgttggaacagttgtcgttggaacagtcgtcattggaacagtcgttgtcgttggaacagtggtgctcgttcgaacagtcgtgacggttggaacagttgtgacaattggagtagtcgtgaccttggtctgtcatccaggccggactgcagtggcatgatcaactcac

SEQ ID NO: 14852 - RNA, 2702 nt, Homo sapiens
  source 1..2702: mol_type = other RNA
gctgggattacaggcatgagccacggcgctagcctcctaaacaattttaaacatgaaagtggtttggaggcgatttagaatttgggtcaaaactagtgagtttcaaacacttatatctgcaatgtaacttataaggcagaaaaggcagacttttccctactcccgccttttttttttcttttattgctgatcttcttggttctaaaaatttgttcagaaagcctgatggttgtttaaatgcttagcaccatgacacacgtgtaataaaaattgcataaatggaccaggcacggtggctcatgcctgtaatcccagcactttggaaggccaaggaggctggatcctctgaggtcaggagttcgagatcattctggccaacatgatgaaaccctgtctctactaaaaaaatacaaaaaattagctgagcatagtggcggacacctgtaatcccagctactcgtgaggctgaggcgggagaattgcttgaacccggaaggtggaggttacagtgagccgagatttcaccatcgcactccagcctgggcaacaagagcaaagctccatctcaaaaaaaaaaaaaaaaattgcataaatatgttaaatcacctggcaaatgattttcttcccctggtgtctatgtgttccatactattgtaggctctttaactggtaaaacagctaccccaattcagagatccagtacttaatgcatcacatttccagagttatgagaaaacagctaaacctgtgagttagactcactttgtttccccacggaggaaataaaaacccacgatttgaaacctttggaaaacataggaaatgcaacatttggaagtataacatagaaacaagagataatcatacaatgcttccaaatgaagtctcacgttggatttgctggtttttaagacagattcccctcttctggacagctgtgatggccaagatagaagttcatttgctatgtttccagggactattctctttgatgtatacaggatttatggggtctaaaaagaacatacaattataaagtgttcatatttgagagaaaactgcaatgatcagaaggattgagccagttttagcataaaaaattaggactacattaatgatgaggttgactatacacagtttggagtgagagagttactctacccagtatcactgacatgttggaatgccagatgaaactgaaacagaaaaattgtcttggggtctaaaagacgtctgatgtgctgatgtctgttcagtcttctgcactcatgggcgtaaactctcaaagagcaccactgggtcttagtccgtggcataaagactattctcaatgtagatattgtcttctgcttggacttccttttcaactgcattttgcaaagctttaatttgaaggctgctaaatgaaacattttggcaatgatgacacccaaaagagcaagaagcaccaagacagaaatacagactccagcatagattcctttagtggtattggccgtcagtagactatgttctaggaacagttgagtttgattgttattccaaaggccatctgaagactctgtcacggtgtcattcccatctgttgtgtaagagtacaatggtgagctggtgggttctctccttattgctccctgcagtgtcgtagggtgggtttctgctggctgaggtgaagatggtgaagtggctggttcatggttctgcctgggcaaaggcattggaggaacaaaggtagagacagttgttgtcactggaacacttgttgttgttggaatgctcgttgtcgttggaacgctcgttgtcgttgaaacagtcattgtcgtcagaacagtcgttgtcgttggaatgctcattgttgttggaacagttgtcgttggaacagtcgtcattggaacagtcgttgtcgttggaacagtggtgctcgttcgaacagtcgtgacggttggaacagttgtgacaattggagtagtcgtgaccttgggtggcacaatctccaatgatacggtgattttcatgtcattgaaccacccacggtgctcaacacggcaacaatatacgccactgtcagacacagctgtattttctatggtcaaagagacatcccttcttgaaaggtcccccaatagcttatagcgtgtgtccttccgataggtgacgtgggttccattggtccagacaatgccattttggcatgtgaatagagaacatgagcctctattccagcacatggatgtgacagctccactgtagtggcagggtagtgtgacagatggacctgcctctccaccaacctttacagaaccagctacagaatctgccagatgtaggatgaggcttaagatgaccacttgaggatgcattatgggatcagcctgaaggaaaatgagcagacaggctggttggtaccctccaccagatggtatctgatcaagtcttaaatctcagattgcaacttatcttttcacccagttggttgattcatatgagcctgctctggttcagatccaggctctgtcactcacaatgctgggtaaccctgagagttcctgagttctcttcaaacctctatttcctcagttgtaaaatagcactaaaaatgcttcctctatctcccaccaaggattgatataataagcaaaaagggccacggaagaacttggaaaactaaacctacatcatatgcagtaatagcactagctgag

SEQ ID NO: 14853 - RNA, 437 nt, Homo sapiens
  source 1..437: mol_type = other RNA
gctgggattacaggcatgagccacggggcctggcctaaaattgttgtttttaaaaaaattccaaatggttagaatgttttgcttcatttgtggctattcacttctagttttattactttgtgctaagtaaatatgacctgtacaatttttttttttgacggagtctcactctgtcgcccaggctggagtgcagtggagcaatctcggctcgctgcaacctctgcctcccaggttcaagcagttctcctgcctgagcgtcccaagtagctgggactacaggtgcccgccaccacacccagctaatttttttgtattttagtagagatggggtttcatcttgcccaagctggttgggaactcctgagctcaggcaatctgcccacctcggcctcccaaagtgctgggattacaggcgtgagccaccgcgcccggccaac

SEQ ID NO: 14854 - RNA, 2236 nt, Homo sapiens
  source 1..2236: mol_type = other RNA
gctgggattacaggcatgagccacggtgcccagcctgttccagcctttttgttaaaactacagagtgaatggccccagaggggaagtttcatttctgggtctcttttcagcccctttctgccttccccccacaaactcagacaaatggacatggcctggaaaacccagtgtggctgctgagctccccgcgggtgggaagaggatcaaaaacaaagtctgatcatcccatagccttgctggccaagaccaagaaccgagctgggcaacagtgagctgcaggcttcgctttccctgcgggctccatgccccggctgcacggggaggtgttctaggcggccgccggccagagcctttgagagtggaaccttcctcgtgttcaattagaggacccagacttgggaacagagccgtaaccacacttccagccttggacacaggaacaaacgaaaaataatttttctgtgtcagacacctgaatcctgagggcatgtcaggatctattttcagatatctacattctgtcttcatccaacacctttgctgtgaggtcaacttgaatattccactgtgactcttccccaacccagtctcctccctcccagaggcagagccaaatggcccgagagtgtgacaagttgagacctgtaggacagacagcaggttgcctgcccaacaagcgattctgcccttctttctttccaaaataaccctgattccatctgggcagcaaattcctcagataaaagactttatgattctctatctcttgcagacagaatggtcacagagaggtatgtagaagcccttggatgaagcttccaggaaagatcttaaaggaccaactcagctagaagacgcgtcctttcgcccttcatcctctctctctgcctgcctaaaacatgacacgatggctggcactgtagcagctatcttgaatcatgaggcttctttaaagatagaaggtctgtgctaaggatgacgaagaagagtgacagaagaaagctgggtgcctgatgactttgtggagccacccattccagccgagaccaccagcctctgaaattcttctacaggtgcccgcgtggtacttgagggcgctcacgttgcgtctgtgggccgtgaacgtgcgcacacactcccctgtgtctgccagccagcacttgacggtcctgtccgcgctgccagagtacacgagtcggttcaccagctccagacagatgacggagccccggtgctcccggaacacccgcagctgctccccactcaggatgtcccaggcacggatggtggcgtcggtgctgcctgtgaaggccgtgtggccgggcgtgtctagcactaggcacagcactgcacccgtgtggccccgcagcgtctggtggcagcagccgctggccacctgccacaccttggctgtgccatctgtgctgccggtcaccagaagccccccggccgcggcctcctccgcgcagggagtgctggggaggtcccacggggcagagtaggctagggtcagcacgcagttgcggtggccccggaactcccgggacatctgccccttgtccacactccagacccgagctgtccggtcataggagctgctgaagagctggttgttggcaaccaggatcctgttcacgatggacgtgtgtcctcggtacacctgcagacactgcccggtcagcacgtcccacctcctgatggtgcagtcggcgctgcatgtgaaggcagcctcatcctccagctggcagaaggtcacatagctttcatgtccttgcaggagcgcgcagcactggccgtccgcggtgctccagagccgggccgtgccgtcctcgctgcccgtcagcaggcgctgcccgtcggggctcaggctcagccagttgatgcccccgcggtggtcggcgcagaccctcagggccgacccgccgccccccatcccgctggcagggcggggaacaagaaggagctgcgccccgctagggaggggcgccccggggtccgcgcggcggctccgtacgactgcggcccgcggccatcgcggggaacggggagcccgactcctgcggaggcacgcggcgaggggagggtgaaggaccctagctccccgctgcctccagcctctgggcccgcgaacccagggcgctgcggggggcggcccactcgggacctccgccctgggtagagtcctgggcgcgcgggcagagagaacccccttcccagcaccgctcggaggatccac

SEQ ID NO: 14855 - RNA, 1302 nt, Homo sapiens
  source 1..1302: mol_type = other RNA
gctgggattacaggcatgagccacggtgcccggccacatttgcattactaagggcctttaaatattgacgttattaaaatgacaaacccacacaaaaatgcaggaaagttggccgggcgcagtggctcacacctgtaatcccagcactttgggaggctgaggcgggtggatcatgaggtcaagggatcaagaccatcctggccaacatggtgaaaccctgtctctactaaagatacaaaatcagccaggcttggtggtgtgcgcctgtagtcccagctactccggaggctgaggcaggaattgcttgaacccgggaggcagaggttacagtgaactgagattgtgccactgcactccagtctggcaacagagcaagactctatctcccaaaaaaaaaaaaaaaaaaaaaaaaagggcagggaggtgaaatgacctctgtttacatccaacttgctcggctgctgtcctcccacagccgacagagatggaaatcttagagtaaaatatgcaaatcatattaaataaaaacccaaatgaacgaactctgcgctatcttgctcaacgtactaggacaaacttccatattccccctaaacgcccctgagaccatggctgacagaaccacctgctactttcaacacagaaaattcaattttcctttaccttcaaaccgaaaacctttattgagaggcagcatttggcaaagcaggggctaaaagcccagggtaattcaaggctcaaaactcatgtcctcagctctgcacatgtcggaatgggacataactcaccacggtgagacccactggctggtccactgtggcgcacgtcatccacgccaccacctacttacctccagcggagccctatctcgccgcagcttgactgccttgacttctgtagaaaattctatttcaataacagtcttcttcttcaggtcatcccagatcattactttgttgggagggtatttcggcttttttccaccaccaactaaagctaaatagttgcagcgaaataacatttcaacatggccaactcctccttctagaaattcttgtttctctttttcttttagtggatcagtgttatagactcggaatccattttccatcccacacgcaaagcatccgtggtcctggttgaagccggcgtagagcagcccgttgccgtgagggttacacggcaggaggttcatggcgccgccgtgctgggtcgccgctcctcagcgctgcatgcctctcgctggggacggcggcctggtcccttcgggccggcgctgaggccgccgcggccggaagtgcc

SEQ ID NO: 14856 - RNA, 916 nt, Homo sapiens
  source 1..916: mol_type = other RNA
gctgggattacaggcatgagccacggtgcctggcccctcaaagttagccattttcttattggctatttttcaaattaggttgatcccaactttacactattgaaaacaccattgcctgaatattatcatacacctatctttatctaaatctgattatttccttagaatctattactagaagtggaattatggaaccaaaaccctccctgttctaaatttagctgaaaaatgtttttccccgggtgatacagcttatgataggcacaggaagataggtaggaggaaatagcagtgtggtggttttggattaatttattaatttacaacaaagactttttaagcacctactaggttggacctcaggggaaatcactggagagttgtatcacagggactttctggacttgagcctggggtgtaaagcaggcaatatgtaaagcgtttgggcttcctttctgtccttgttgaatccagtttgtgcagggactctccactcttggcgtcttaatccattttttgttgcgtgactgcagacacttgttcctcattttatcccactgcttggtgcacaggagacatttattaaatgtttgttgaatgaatgaatgacaagcacttgtcacaacggtaactctgtgaagactaggatcctatccattttgttcattacaaaattccgcctaagccttgaacaaggctatgagttataagtgcaaagcgatttagaggaaggaggggtaactaaactgactgaagaagctaagggaagcctcacagataaaattacatctaaactgaaactgaaaggaaggtggaaaactaaaaagatcaacaagggaaggactgcagacagaatatcgcgaggtattggtcagccaagatggcttctaacactggccgccacacttaatatggc

SEQ ID NO: 14857 - RNA, 553 nt, Homo sapiens
  source 1..553: mol_type = other RNA
gctgggattacaggcatgagccacggtgcctggcccctcaaagttagccattttcttattggctatttttcaaattaggttgatcccaactttacactattgaaaacaccattgcctgaatattatcatacacctatctttatctaaatctgattatttccttagaatctattactagaagtggaattatggaaccaaaaccctccctgttctaaatttagctgaaaaatgtttttccccgggtgatacagcttatgataggcacaggaagataggtaggaggaaatagcagtgtggtggttttggattaatttattaatttacaacaaagactttttaagcacctactaggttggacctcaggggaaatcactggagagttgtatcacagggactttctggacttgagcctggggtgtaaagcaggcaatatgtaaagcgtttgggcttcctttctgtccttgttgaatccagtttgtgcagggactctccactcttggcgtcttaatccattttttgttgctgtggtgggctattgtgcccagtgcgcctg

SEQ ID NO: 14858 - RNA, 2749 nt, Homo sapiens
  source 1..2749: mol_type = other RNA
gctgggattacaggcatgagccacggtgcctggctatcacgcaattcttaagtgcttattccagtagcagaagagattagaaaggctggctttttccaacagtgggagcttgaatctggaaagtcttaaagttgttgtaatttcacactactaagaagcactttgctcatgcaactgaaaaaaaaattaagtgcctacctgggtgattccagggcacttataagcaactaagactaattagaagtcctcatagcctctaatgaaaagataggaagtaattcgctctatgatacaaaaattcctggatgtttggaattgttttacatcattgggcacaggattccttactgggagcttttgctttcccagggccaaagtccctgttctatgtcacacattgtggagggcaggggacaaatggatacagagcttggtatccactgatatggctcccacaaagacatttgggaggatgagtaaggaaagagagaggcaaaatctcagtaccagttgtaactggaaaatgtcatttacatggaatgagaacttacatggggcgagctgagaagcactttcagttgaagcaaatagaaaaattaaggcactttcctttacttttagttatttttaaacacgtatctttatgctcagatctttcttttataactgggttataactggggagaataaaaggatccgggcatgagagaaagtgaaatcaagggaggaagagggcatgcaatgggggaagggaggagcaggaatgtccactttactgaatacaaaatactgtaaaagatggatcctgccatattcttcccccaatcaacttggatgaaaaacagaaatactacattcttaaacacagttcatttttagtttgtcgtggcaatacatggaaaaaaatcaggccactactaagcatctatagagtgtatctttggcaaaaatgtggacctgcaacaattcagatggttttctttcaattaggttcaaaaatcatggctctgtaaatttccaaaacttttaaagtcttctcatgtcttcttataatcgggcattcagaggtacgtgttggttctaatagctttggtagaaacatgctgaaaatagaaatgaatataaaatgccttgtctttaggctaatttggtatggattagtaaggcctgagtgaactggaaattagtacatttcttgaaataatacaaatgaatgtgagacacatgggtagaacagcagattcagaaaaaaaggttagtattgtagtcccaagttttataaaagacatcaagtaaggccagcaatagaggaatcaagtttctttttcgggttccctggggtgatttcctatcagcttcacgttcatgagctggggatttgtaaaatgtgagatggcctttgactttgtttttgatgcgatcagcagcggcactgtctgcaatccaggcccagcattctcagacagcgtgcagtacggatgcttctggctggcagggaggtcgtggcagtgggctgactagtgtgctgtgttgggagggctcagagggtgatggggcaagcctccgtgcaaagggagttcctttctggtcgtgccctcctttttggctggagcttggccacagagattggctgccattctcatccctggatggggtggaggcaggtcccagacaacctcagataattgaacagcagctgtgaccctcagaacagcgtttcttctttttcttggggtggaaaatggtgaggattgcttcatcaaaaaccgctttgagacctttctgagtcagagctgaacattccaagtagcactgtgctccgatcgcttttgcgagcttcacaccatgctcgtaagtgagaggtttctctttcatatacagcaaacgggccaaggtttttgggtcatcacggagatcaatctgggtccctatgaggacataaggcacgtgaggcatgcagtccttgagctcggggacccattcctcctggacattgtggtaagaggcagggtttacgacagagaagcagatcaaaaacacatccgtgttggggtaggagagtggcctcagctggttgtagtcctcctgtcccgcggtgtcatacagtccgagcaagtgttgcttgcctcccacagtcacagtaactgcatagtggtcaaacacagtgggcacgtattcctctgggaaggcgtcgttggcgtagctcatcagcaggcaggttttccccacggcaccgtcccccaccaccacacacttcaacatcttcttctcgtcgttgcccctgcagccgcagctgctgtcagttccctctttgcagttcattcttgcggctccagctgctggggactcctgctgctattgcttctcctgctttttccaaagcacatgaagcggcagaaagccagtgccaggcttgagtttactctgtctgactttgggtaccttggatcatacagacatgtccgaggctgggatatgtcctgttgcttaccatgctggtaaagaaaggtaacacacacttgagggagttatgaaaagggtctgcccctttccgctctcagtgtgagttaagaaaccctcattttcacagaattcgaggggcttcctaacagcctagaaatttcagcagcctgagggttttactctgctctccctgtctctagcctggcaaaagatacggtggaattttgctaaatctttctcattttccaagtcacatctaacatggaggaaagctgggctttttaat

SEQ ID NO: 14859 - RNA, 2615 nt, Homo sapiens
  source 1..2615: mol_type = other RNA
gctgggattacaggcatgagccacggtgcctggctatcacgcaattcttaagtgcttattccagtagcagaagagattagaaaggctggctttttccaacagtgggagcttgaatctggaaagtcttaaagttgttgtaatttcacactactaagaagcactttgctcatgcaactgaaaaaaaaattaagtgcctacctgggtgattccagggcacttataagcaactaagactaattagaagtcctcatagcctctaatgaaaagataggaagtaattcgctctatgatacaaaaattcctggatgtttggaattgttttacatcattgggcacaggattccttactgggagcttttgctttcccagggccaaagtccctgttctatgtcacacattgtggagggcaggggacaaatggatacagagcttggtatccactgatatggctcccacaaagacatttgggaggatgagtaaggaaagagagaggcaaaatctcagtaccagttgtaactggaaaatgtcatttacatggaatgagaacttacatggggcgagctgagaagcactttcagttgaagcaaatagaaaaattaaggcactttcctttacttttagttatttttaaacacgtatctttatgctcagatctttcttttataactgggttataactggggagaataaaaggatccgggcatgagagaaagtgaaatcaagggaggaagagggcatgcaatgggggaagggaggagcaggaatgtccactttactgaatacaaaatactgtaaaagatggatcctgccatattcttcccccaatcaacttggatgaaaaacagaaatactacattcttaaacacagttcatttttagtttgtcgtggcaatacatggaaaaaaatcaggccactactaagcatctatagagtgtatctttggcaaaaatgtggacctgcaacaattcagatggttttctttcaattaggttcaaaaatcatggctctgtaaatttccaaaacttttaaagtcttctcatgtcttcttataatcgggcattcagaggtacgtgttggttctaatagctttggtagaaacatgctgaaaatagaaatgaatataaaatgccttgtctttaggctaatttggtatggattagtaaggcctgagtgaactggaaattagtacatttcttgaaataatacaaatgaatgtgagacacatgggtagaacagcagattcagaaaaaaaggttagtattgtagtcccaagttttataaaagacatcaagtaaggccagcaatagaggaatcaagtttctttttcgggttccctggggtgatttcctatcagcttcacgttcatgagctggggatttgtaaaatgtgagatggcctttgactttgtttttgatgcgatcagcagcggcactgtctgcaatccaggcccagcattctcagacagcgtgcagtacggatgcttctggctggcagggaggtcgtggcagtgggctgactagtgtgctgtgttgggagggctcagagggtgatggggcaagcctccgtgcaaagggagttcctttctggtcgtgccctcctttttggctggagcttggccacagagattggctgccattctcatccctggatggggtggaggcaggtcccagacaacctcagataattgaacagcagctgtgaccctcagaacagcgtttcttctttttcttggggtggaaaatggtgaggattgcttcatcaaaaaccgctttgagacctttctgagtcagagctgaacattccaagtagcactgtgctccgatcgcttttgcgagcttcacaccatgctcgtaagtgagaggtttctctttcatatacagcaaacgggccaaggtttttgggtcatcacggagatcaatctgtcccgcggtgtcatacagtccgagcaagtgttgcttgcctcccacagtcacagtaactgcatagtggtcaaacacagtgggcacgtattcctctgggaaggcgtcgttggcgtagctcatcagcaggcaggttttccccacggcaccgtcccccaccaccacacacttcaacatcttcttctcgtcgttgcccctgcagccgcagctgctgtcagttccctctttgcagttcattcttgcggctccagctgctggggactcctgctgctattgcttctcctgctttttccaaagcacatgaagcggcagaaagccagtgccaggcttgagtttactctgtctgactttgggtaccttggatcatacagacatgtccgaggctgggatatgtcctgttgcttaccatgctggtaaagaaaggtaacacacacttgagggagttatgaaaagggtctgcccctttccgctctcagtgtgagttaagaaaccctcattttcacagaattcgaggggcttcctaacagcctagaaatttcagcagcctgagggttttactctgctctccctgtctctagcctggcaaaagatacggtggaattttgctaaatctttctcattttccaagtcacatctaacatggaggaaagctgggctttttaatggagtttttttccctttgcttcctccagctt

SEQ ID NO: 14860 - RNA, 2910 nt, Homo sapiens
  source 1..2910: mol_type = other RNA
gctgggattacaggcatgagccacggtgcctggctatcacgcaattcttaagtgcttattccagtagcagaagagattagaaaggctggctttttccaacagtgggagcttgaatctggaaagtcttaaagttgttgtaatttcacactactaagaagcactttgctcatgcaactgaaaaaaaaattaagtgcctacctgggtgattccagggcacttataagcaactaagactaattagaagtcctcatagcctctaatgaaaagataggaagtaattcgctctatgatacaaaaattcctggatgtttggaattgttttacatcattgggcacaggattccttactgggagcttttgctttcccagggccaaagtccctgttctatgtcacacattgtggagggcaggggacaaatggatacagagcttggtatccactgatatggctcccacaaagacatttgggaggatgagtaaggaaagagagaggcaaaatctcagtaccagttgtaactggaaaatgtcatttacatggaatgagaacttacatggggcgagctgagaagcactttcagttgaagcaaatagaaaaattaaggcactttcctttacttttagttatttttaaacacgtatctttatgctcagatctttcttttataactgggttataactggggagaataaaaggatccgggcatgagagaaagtgaaatcaagggaggaagagggcatgcaatgggggaagggaggagcaggaatgtccactttactgaatacaaaatactgtaaaagatggatcctgccatattcttcccccaatcaacttggatgaaaaacagaaatactacattcttaaacacagttcatttttagtttgtcgtggcaatacatggaaaaaaatcaggccactactaagcatctatagagtgtatctttggcaaaaatgtggacctgcaacaattcagatggttttctttcaattaggttcaaaaatcatggctctgtaaatttccaaaacttttaaagtcttctcatgtcttcttataatcgggcattcagaggtacgtgttggttctaatagctttggtagaaacatgctgaaaatagaaatgaatataaaatgccttgtctttaggctaatttggtatggattagtaaggcctgagtgaactggaaattagtacatttcttgaaataatacaaatgaatgtgagacacatgggtagaacagcagattcagaaaaaaaggttagtattgtagtcccaagttttataaaagacatcaagtaaggccagcaatagaggaatcaagtttctttttcgggttccctggggtgatttcctatcagcttcacgttcatgagctggggatttgtaaaatgtgagatggcctttgactttgtttttgatgcgatcagcagcggcactgtctgcaatccaggcccagcattctcagacagcgtgcagtacggatgcttctggctggcagggaggtcgtggcagtgggctgactagtgtgctgtgttgggagggctcagagggtgatggggcaagcctccgtgcaaagggagttcctttctggtcgtgccctcctttttggctggagcttggccacagagattggctgccattctcatccctggatggggtggaggcaggtcccagacaacctcagataattgaacagcagctgtgaccctcagaacagcgtttcttctttttcttggggtggaaaatggtgaggattgcttcatcaaaaaccgctttgagacctttctgagtcagagctgaacattccaagtagcactgtgctccgatctggagtcctgcaggaggggcagggcactccccatcctcctgcccccagtgtgcagctgacagcatgtcaggctttgcctttcgatggagcgggaggagcccaagcttgtctcttccaattcagacatttcgcttttgcgagcttcacaccatgctcgtaagtgagaggtttctctttcatatacagcaaacgggccaaggtttttgggtcatcacggagatcaatctgggtccctatgaggacataaggcacgtgaggcatgcagtccttgagctcggggacccattcctcctggacattgtggtaagaggcagggtttacgacagagaagcagatcaaaaacacatccgtgttggggtaggagagtggcctcagctggttgtagtcctcctgtcccgcggtgtcatacagtccgagcaagtgttgcttgcctcccacagtcacagtaactgcatagtggtcaaacacagtgggcacgtattcctctgggaaggcgtcgttggcgtagctcatcagcaggcaggttttccccacggcaccgtcccccaccaccacacacttcaacatcttcttctcgtcgttgcccctgcagccgcagctgctgtcagttccctctttgcagttcattcttgcggctccagctgctggggactcctgctgctattgcttctcctgctttttccaaagcacatgaagcggcagaaagccagtgccaggcttgagtttactctgtctgactttgggtaccttggatcatacagacatgtccgaggctgggatatgtcctgttgcttaccatgctggtaaagaaaggtaacacacacttgagggagttatgaaaagggtctgcccctttccgctctcagtgtgagttaagaaaccctcattttcacagaattcgaggggcttcctaacagcctagaaatttcagcagcctgagggttttactctgctctccctgtctctagcctggcaaaagatacggtggaattttgctaaatctttctcattttccaagtcacatctaacatggaggaaagctgggctttttaatggagtttttttccctttgcttcctccagctt

SEQ ID NO: 14861 - RNA, 2900 nt, Homo sapiens
  source 1..2900: mol_type = other RNA
gctgggattacaggcatgagccacggtgcctggctatcacgcaattcttaagtgcttattccagtagcagaagagattagaaaggctggctttttccaacagtgggagcttgaatctggaaagtcttaaagttgttgtaatttcacactactaagaagcactttgctcatgcaactgaaaaaaaaattaagtgcctacctgggtgattccagggcacttataagcaactaagactaattagaagtcctcatagcctctaatgaaaagataggaagtaattcgctctatgatacaaaaattcctggatgtttggaattgttttacatcattgggcacaggattccttactgggagcttttgctttcccagggccaaagtccctgttctatgtcacacattgtggagggcaggggacaaatggatacagagcttggtatccactgatatggctcccacaaagacatttgggaggatgagtaaggaaagagagaggcaaaatctcagtaccagttgtaactggaaaatgtcatttacatggaatgagaacttacatggggcgagctgagaagcactttcagttgaagcaaatagaaaaattaaggcactttcctttacttttagttatttttaaacacgtatctttatgctcagatctttcttttataactgggttataactggggagaataaaaggatccgggcatgagagaaagtgaaatcaagggaggaagagggcatgcaatgggggaagggaggagcaggaatgtccactttactgaatacaaaatactgtaaaagatggatcctgccatattcttcccccaatcaacttggatgaaaaacagaaatactacattcttaaacacagttcatttttagtttgtcgtggcaatacatggaaaaaaatcaggccactactaagcatctatagagtgtatctttggcaaaaatgtggacctgcaacaattcagatggttttctttcaattaggttcaaaaatcatggctctgtaaatttccaaaacttttaaagtcttctcatgtcttcttataatcgggcattcagaggtacgtgttggttctaatagctttggtagaaacatgctgaaaatagaaatgaatataaaatgccttgtctttaggctaatttggtatggattagtaaggcctgagtgaactggaaattagtacatttcttgaaataatacaaatgaatgtgagacacatgggtagaacagcagattcagaaaaaaaggttagtattgtagtcccaagttttataaaagacatcaagtaaggccagcaatagaggaatcaagtttctttttcgggttccctggggtgatttcctatcagcttcacgttcatgagctggggatttgtaaaatgtgagatggcctttgactttgtttttgatgcgatcagcagcggcactgtctgcaatccaggcccagcattctcagacagcgtgcagtacggatgcttctggctggcagggaggtcgtggcagtgggctgactagtgtgctgtgttgggagggctcagagggtgatggggcaagcctccgtgcaaagggagttcctttctggtcgtgccctcctttttggctggagcttggccacagagattggctgccattctcatccctggatggggtggaggcaggtcccagacaacctcagataattgaacagcagctgtgaccctcagaacagcgtttcttctttttcttggggtggaaaatggtgaggattgcttcatcaaaaaccgctttgagacctttctgagtcagagctgaacattccaagtagcactgtgctccgatttaggatcctaaggactccatggacgtctggcgctagttagtattgacattactgtgcatagaagtaggaagagttcagtatctcgatcaggtgttgtgagaggttctcatgcaggataccgcttttgcgagcttcacaccatgctcgtaagtgagaggtttctctttcatatacagcaaacgggccaaggtttttgggtcatcacggagatcaatctgggtccctatgaggacataaggcacgtgaggcatgcagtccttgagctcggggacccattcctcctggacattgtggtaagaggcagggtttacgacagagaagcagatcaaaaacacatccgtgttggggtaggagagtggcctcagctggttgtagtcctcctgtcccgcggtgtcatacagtccgagcaagtgttgcttgcctcccacagtcacagtaactgcatagtggtcaaacacagtgggcacgtattcctctgggaaggcgtcgttggcgtagctcatcagcaggcaggttttccccacggcaccgtcccccaccaccacacacttcaacatcttcttctcgtcgttgcccctgcagccgcagctgctgtcagttccctctttgcagttcattcttgcggctccagctgctggggactcctgctgctattgcttctcctgctttttccaaagcacatgaagcggcagaaagccagtgccaggcttgagtttactctgtctgactttgggtaccttggatcatacagacatgtccgaggctgggatatgtcctgttgcttaccatgctggtaaagaaaggtaacacacacttgagggagttatgaaaagggtctgcccctttccgctctcagtgtgagttaagaaaccctcattttcacagaattcgaggggcttcctaacagcctagaaatttcagcagcctgagggttttactctgctctccctgtctctagcctggcaaaagatacggtggaattttgctaaatctttctcattttccaagtcacatctaacatggaggaaagctgggctttttaatggagtttttttccctttgcttcctccagctt

SEQ ID NO: 14862 - RNA, 983 nt, Homo sapiens
  source 1..983: mol_type = other RNA
gctgggattacaggcatgagccacgtgcccagcctttatttttaagtagtgaagagccttcttggtcatgctaaggaatttttattaaactgatgaccagagcagccactagaaattttaaacagggtgacatcctatctgcatttaagcttttttatttttttaagaatcaagtgaatacaattttagagattgctaaatccagagaggtccagtgggaaaactggtagccattggatttgagttgtaaacacgtaacagctgaacttacgtatatgaacactgccataggaactgaggtctgtgaatccaaaaatgtaggcaaaacttcctgttgaacatttttctggggaaaccaccatagcttttatcaaatgcttaaaggtatggaacattctaaaaggaaggtgatattcaaacctaaaagtgtatcaacggtatccacatggagaagagggtcaaggatgggggaacaaagactggtaggtgggaaggtcaaaaagaaaatgggaaaaccagcaatgggaaaatttttttttttctttttttgagacagtcttgctatgttgctcaggctggatcagtgcagtagcacaatctcggctcagtgcagtggcacaatctcggctcactgcaacctctgcctcctgggttcaagtgattctcctgtctcagcctcccaagtagctgggattacaggtgcccgccaccacgcctggctaatttttatattttgagtagaggcggggtttcaccacgttggccaggctggtctcgaactcctgaccttaagtgatctgcccgtcttggcctcccagagtgctgggattacaggtgtgcgcaggaagaaaatttcaatggacgaggtagtcaacaaaatgaagtcaagaaaatatgtaagactcagaaatactctaactgttgacctaagaacagctgagtatgggtgccaacacctggtgcaatgggtagtgtggatgaga

SEQ ID NO: 14863 - RNA, 3123 nt, Homo sapiens
  source 1..3123: mol_type = other RNA
gctgggattacaggcatgagccactaatacccagccaagagcacacatttaggatagaacttgagcatacttttgttctggaagaggacagaaatagagcaagggacaggaaacaacaaacaaaacccagtagcagtgagttagcttctgtcccgtctccacccttgtaagtaggacactggcttaacaattagttttattatcagccctcactgtttaaatcttagcagagaaaaagaaaagctgttgaagagaataaaattaagaaacataaaaagggaaaacttgattatcaccagtttctggatttttagttttcttcttctaactgaagttcactcagatctagggaatagcattaagcttaacgtgaaagtggggggaaaaatgtggcacattgaagtggcaggtagctgtaaagagaagagggaagcatttttaaactgtagtaaggtttatccgagagtgattacttttataaggaagagattctatgaaaatgcagcaaggaggctggtccgtggagtaccacaaagctggggaactgcagttttcatgctgattctctatctttaccactctgggtcaattgtggcagagaagctgttttatcttccttgggcatgggagaggaaaggaggagggatgcatatgactcagtttttaaatcagtaccttacagggttatttagtaaagtggtaaggcttctgtaaaatgctttgagtgactaggaaacaaatcagaggcaaaataacaacataaaataataacaccaaacatcagagaactgaagggaagaggagcgagtcactgaaaaccagggacaccagttgtccaggtcaccaacagcttcctggtgctcccccaccccacagtctgctgtgagctctttcacctagaatgagcctagagaatggcctagtggggcaagggacctagcactggctctcagccacaactaacaccacatcccaaattacccctccagaacagatgccgagggacactagaagcgaggagtagttgggatacttttgctacaccttctatcttgagagaaagagatttaaaccaatagtataatacatcagttgaaatacatctgacgataataacaaagatgcattgacctataaaaagtcatttaatgcatattccagatggccaatacaagctggttaggtaattagcccttgaagaattcttttataatcatataaaaatgttttgtcttgtttaaaaaaagtctactctaacaaaaacatccaccaatgggcttgcattttttccatttgcaggtttgtaagatcataaaaatatacacatatgcatctctgggcatatctctgtccactagctaatcagttttggcaatacactgcataggggtatactaccattggtttctgacattaagttagctttaagcttattggctattccaacaactggaggcagcttagaacccaatccctggaaagcacttgcaggattaactacccgtttccctgacaccttgtctatggtggtgagaggtctggggacagacttgctaatccaagggtgtcttaatgcttgagctggggtcaagcgggcagaggggtcccagtgaagacaccttttcaagaactctataaacaagtagtcatcacaccctttcagtgctgtcccccagtctttgctgcctgggggaccccgctttttacccctacgtgagcgaccccccacaagcacaaccctcccatctgcctgggtagtcacagagcagtagcggggtatgcccttggaattaataaagtacttggcacgtttggattgctccagaagttttggtggtggcatccctagaagctccatcatgcaggccaactggtctccttcatcctctccagggaagagaggctgtcctgttaaaagttctgcaaggatgcagccaaaactccatatgtcaattggtgtgctgtagcggcttcctaagatgatttctggagctctgtagaaccgagactggatatatgtgtagagcttctggtactcgaaacagctggacccaaagtcaatgaccttggttgaactgcgcccgtggtgtttcaggagaatgttttctggcttcagatcgcagtgaataatcttatttttgtggagggcatccaaagattgcaagatggactgggcaaacttgcgtaccaactggacgctaaaaccctgaaacttattttttttaatcagctcataaaggtctatgctcagcaattcaaaggccatgcaaacatggttccggaatgtgaaactttccagcatgtggataacgttcatactaccagttttatcctgtttcttaagatgctccaaaatccggatctcctcagctgcttgacgatgaaagcgcttctcattgcgcaccatttttagggccacgtactgtcgaagtttgtgatcatagaccctggccacctgcccaaaactccccttgccaataattttcagcacctcatatcgataagctagatggtctcgaggtacatgaatataggccccatctgcatcatcataccctccattattgggaccaccaataactccatgtcttttcttggcatttggacctacaaagtaaatttctggataattaattatttccagtttctcataggcagtgaggtggtgtttatattgcttcagggcttgttctggagtcagaggcaccactttgggtgccttggatgaactgttggattttactgtattcaagcaatctgaacttttaccctgagaaacagtaggagagcatttttcagagtcactgatgccatctgactgaatagtattggattttctgttgccaaattcttgaaacagctgttctaccttcatctcacctccatccaaaaagtgctgagtatgatctcctgtaaactgctcagtggtcatatttagtcttctgggtggaggtggttcagaaggattgcagagtacatttgaacaggggggacatttggtttcatctatcatcatgaaggtgtcatagacaccatcccccaaccccgatctagggtttcagagggaatccaggggtggaaattcttcttgctctaactccgctctagccccgtcccccgcgc

SEQ ID NO: 14864 - RNA, 3289 nt, Homo sapiens
  source 1..3289: mol_type = other RNA
gctgggattacaggcatgagccactaatacccagccaagagcacacatttaggatagaacttgagcatacttttgttctggaagaggacagaaatagagcaagggacaggaaacaacaaacaaaacccagtagcagtgagttagcttctgtcccgtctccacccttgtaagtaggacactggcttaacaattagttttattatcagccctcactgtttaaatcttagcagagaaaaagaaaagctgttgaagagaataaaattaagaaacataaaaagggaaaacttgattatcaccagtttctggatttttagttttcttcttctaactgaagttcactcagatctagggaatagcattaagcttaacgtgaaagtggggggaaaaatgtggcacattgaagtggcaggtagctgtaaagagaagagggaagcatttttaaactgtagtaaggtttatccgagagtgattacttttataaggaagagattctatgaaaatgcagcaaggaggctggtccgtggagtaccacaaagctggggaactgcagttttcatgctgattctctatctttaccactctgggtcaattgtggcagagaagctgttttatcttccttgggcatgggagaggaaaggaggagggatgcatatgactcagtttttaaatcagtaccttacagggttatttagtaaagtggtaaggcttctgtaaaatgctttgagtgactaggaaacaaatcagaggcaaaataacaacataaaataataacaccaaacatcagagaactgaagggaagaggagcgagtcactgaaaaccagggacaccagttgtccaggtcaccaacagcttcctggtgctcccccaccccacagtctgctgtgagctctttcacctagaatgagcctagagaatggcctagtggggcaagggacctagcactggctctcagccacaactaacaccacatcccaaattacccctccagaacagatgccgagggacactagaagcgaggagtagttgggatacttttgctacaccttctatcttgagagaaagagatttaaaccaatagtataatacatcagttgaaatacatctgacgataataacaaagatgcattgacctataaaaagtcatttaatgcatattccagatggccaatacaagctggttaggtaattagcccttgaagaattcttttataatcatataaaaatgttttgtcttgtttaaaaaaagtctactctaacaaaaacatccaccaatgggcttgcattttttccatttgcaggtttgtaagatcataaaaatatacacatatgcatctctgggcatatctctgtccactagctaatcagttttggcaatacactgcataggggtatactaccattggtttctgacattaagttagctttaagcttattggctattccaacaactggaggcagcttagaacccaatccctggaaagcacttgcaggattaactacccgtttccctgacaccttgtctatggtggtgagaggtctggggacagacttgctaatccaagggtgtcttaatgcttgagctggggtcaagcgggcagaggggtcccagtgaagacaccttttcaagaactctataaacaagtagtcatcacaccctttcagtgctgtcccccagtctttgctgcctgggggaccccgctttttacccctacgtgagcgaccccccacaagcacaaccctcccatctgcctgggtagtcacagagcagtagcggggtatgcccttggaattaataaagtacttggcacgtttggattgctccagaagttttggtggtggcatccctagaagctccatcatgcaggccaactggtctccttcatcctctccagggaagagaggctgtcctgttaaaagttctgcaaggatgcagccaaaactccatatgtcaattggtgtgctgtagcggcttcctaagatgatttctggagctctgtagaaccgagactggatatatgtgtagagcttctggtactcgaaacagctggacccaaagtcaatgaccttggttgaactgcgcccgtggtgtttcaggagaatgttttctggcttcagatcgcagtgaataatcttatttttgtggagggcatccaaagattgcaagatggactgggcaaacttgcgtaccaactggacgctaaaaccctgaaacttattttttttaatcagctcataaaggtctatgctcagcaattcaaaggccatgcaaacatggttccggaatgtgaaactttccagcatgtggataacgttcatactaccagttttatcctgtttcttaagatgctccaaaatccggatctcctcagctgcttgacgatgaaagcgcttctcattgcgcaccatttttagggccacgtactgtcgaagtttgtgatcatagaccctggccacctgcccaaaactccccttgccaataattttcagcacctcatatcgataagctagatggtctcgaggtacatgaatataggccccatctgcatcatcataccctccattattgggaccaccaataactccatgtcttttcttggcatttggacctacaaagtaaatttctggataattaattatttccagtttctcataggcagtgaggtggtgtttatattgcttcagggcttgttctggagtcagaggcaccactttgggtgccttggatgaactgttggattttactgtattcaagcaatctgaacttttaccctgagaaacagtaggagagcatttttcagagtcactgatgccatctgactgaatagtattggattttctgttgccaaattcttgaaacagctgttctaccttcatctcacctccatccaaaaagtgctgagtatgatctcctgtaaactgctcagtggtcatatttagtcttctgggtggaggtggttcagaaggattgcagagtacatttgaacaggggggacatttggtttcatctatcatcatgaaggtgtcatagacaccatcccccaacctccgctgctggggcgggagcccggccccaggcggccccgcatccttccgcccaggcccacgagctgtgcctcccatctcctagctcgggaccccgcgcggggagaggcgccagttgggggtccggtcggccacgccacctacgccgggacggctgcctccgcggcgcgacgctcccacgggtactctcgaccagacactgcagctcagcgcactttcgctcccgactggccccggctgggaagt

SEQ ID NO: 14865 - RNA, 3383 nt, Homo sapiens
  source 1..3383: mol_type = other RNA
gctgggattacaggcatgagccactaatacccagccaagagcacacatttaggatagaacttgagcatacttttgttctggaagaggacagaaatagagcaagggacaggaaacaacaaacaaaacccagtagcagtgagttagcttctgtcccgtctccacccttgtaagtaggacactggcttaacaattagttttattatcagccctcactgtttaaatcttagcagagaaaaagaaaagctgttgaagagaataaaattaagaaacataaaaagggaaaacttgattatcaccagtttctggatttttagttttcttcttctaactgaagttcactcagatctagggaatagcattaagcttaacgtgaaagtggggggaaaaatgtggcacattgaagtggcaggtagctgtaaagagaagagggaagcatttttaaactgtagtaaggtttatccgagagtgattacttttataaggaagagattctatgaaaatgcagcaaggaggctggtccgtggagtaccacaaagctggggaactgcagttttcatgctgattctctatctttaccactctgggtcaattgtggcagagaagctgttttatcttccttgggcatgggagaggaaaggaggagggatgcatatgactcagtttttaaatcagtaccttacagggttatttagtaaagtggtaaggcttctgtaaaatgctttgagtgactaggaaacaaatcagaggcaaaataacaacataaaataataacaccaaacatcagagaactgaagggaagaggagcgagtcactgaaaaccagggacaccagttgtccaggtcaccaacagcttcctggtgctcccccaccccacagtctgctgtgagctctttcacctagaatgagcctagagaatggcctagtggggcaagggacctagcactggctctcagccacaactaacaccacatcccaaattacccctccagaacagatgccgagggacactagaagcgaggagtagttgggatacttttgctacaccttctatcttgagagaaagagatttaaaccaatagtataatacatcagttgaaatacatctgacgataataacaaagatgcattgacctataaaaagtcatttaatgcatattccagatggccaatacaagctggttaggtaattagcccttgaagaattcttttataatcatataaaaatgttttgtcttgtttaaaaaaagtctactctaacaaaaacatccaccaatgggcttgcattttttccatttgcaggtttgtaagatcataaaaatatacacatatgcatctctgggcatatctctgtccactagctaatcagttttggcaatacactgcataggggtatactaccattggtttctgacattaagttagctttaagcttattggctattccaacaactggaggcagcttagaacccaatccctggaaagcacttgcaggattaactacccgtttccctgacaccttgtctatggtggtgagaggtctggggacagacttgctaatccaagggtgtcttaatgcttgagctggggtcaagcgggcagaggggtcccagtgaagacaccttttcaagaactctataaacaagtagtcatcacaccctttcagtgctgtcccccagtctttgctgcctgggggaccccgctttttacccctacgtgagcgaccccccacaagcacaaccctcccatctgcctgggtagtcacagagcagtagcggggtatgcccttggaattaataaagtacttggcacgtttggattgctccagaagttttggtggtggcatccctagaagctccatcatgcaggccaactggtctccttcatcctctccagggaagagaggctgtcctgttaaaagttctgcaaggatgcagccaaaactccatatgtcaattggtgtgctgtagcggcttcctaagatgatttctggagctctgtagaaccgagactggatatatgtgtagagcttctggtactcgaaacagctggacccaaagtcaatgaccttggttgaactgcgcccgtggtgtttcaggagaatgttttctggcttcagatcgcagtgaataatcttatttttgtggagggcatccaaagattgcaagatggactgggcaaacttgcgtaccaactggacgctaaaaccctgaaacttattttttttaatcagctcataaaggtctatgctcagcaattcaaaggccatgcaaacatggttccggaatgtgaaactttccagcatgtggataacgttcatactaccagttttatcctgtttcttaagatgctccaaaatccggatctcctcagctgcttgacgatgaaagcgcttctcattgcgcaccatttttagggccacgtactgtcgaagtttgtgatcatagaccctggccacctgcccaaaactccccttgccaataattttcagcacctcatatcgataagctagatggtctcgaggtacatgaatataggccccatctgcatcatcataccctccattattgggaccaccaataactccatgtcttttcttggcatttggacctacaaagtaaatttctggataattaattatttccagtttctcataggcagtgaggtggtgtttatattgcttcagggcttgttctggagtcagaggcaccactttgggtgccttggatgaactgttggattttactgtattcaagcaatctgaacttttaccctgagaaacagtaggagagcatttttcagagtcactgatgccatctgactgaatagtattggattttctgttgccaaattcttgaaacagctgttctaccttcatctcacctccatccaaaaagtgctgagtatgatctcctgtaaactgctcagtggtcatatttagtcttctgggtggaggtggttcagaaggattgcagagtacatttgaacaggggggacatttggtttcatctatcatcatgaaggtgtcatagacaccatcccccaacttctctttccacttcattttctggtggatggtggaggcaaaattctaaatgattaaggatcacttctctgttctttaacactgtggctccaccactccgctgctggggcgggagcccggccccaggcggccccgcatccttccgcccaggcccacgagctgtgcctcccatctcctagctcgggaccccgcgcggggagaggcgccagttgggggtccggtcggccacgccacctacgccgggacggctgcctccgcggcgcgacgctcccacgggtactctcgaccagacactgcagctcagcgcactttcgctcccgactggccccggctgggaagt

SEQ ID NO: 14866 - RNA, 1557 nt, Homo sapiens
  source 1..1557: mol_type = other RNA
gctgggattacaggcatgagccactacacccagaagtgtggctatttttaaaaaacacagtgctgtgttctttccggaaagagaagtcttcaatggtctggcttgagacccacagggctctgcagacagcctgtgctgtggggtcctaagccggatccccatctggtggcacatgccctcccaagggtccccagtggccttggaggtctcagagactccctttgctgctggaaggaagtccatgctcccagatgctcatggcctgagtcctgaggaatgcgctcctggtccccgttctgcaggtgtcacatgtgcatggggctcccaggggtcctgcgtcctcccctggctccccctctccagaccctgcgactcctcctgggccagccacccctgggctgatagacattttgttgctgttgccgatggtggcgtcctcgagaaagcacgatttcatgtggattctctgggcggcttccccctcagggtgagttcctggactgggaattcttgcttcaaacgaagcttctgggccggcagcagtggcagagactggggggctgccaggggggatgtgggcagggccctcggacgggacgccgtggagcctcatctcattgctgtgtcccagctgcacccgtctcagtatggactgctccatgtggatgtcctggggcccccagggatcaactagggtcccccaagttgaggaatcacctggtgccattgaagggaggtggcgtggaccggcggaaccgtcctccctggagactgtctgtcttgtaatgatgttcccgtgtccaatctggatggcttcggagtttgcaatggaaatccagctgttgggtccattctggcagatcatgttgattggattgtgctggtaaataattgaggctgactttgctcttcttccagaatcttctgggcggtaaatcgtccatgctttggactgctcatccatgtccagaaggtgcctgctcttcatcctgtacaagtctcggttcacatcttttgctgtcctcattcccagtgcttgggcgatgaccagggccctctggggaccattgtctttgagaaacctgtagatgtcttcctcccgttgttggctgaactgagggccaggggtctctggaattgtagctgcatgttgctggggcctctcggcagggctggacaaggccagctctgcaggaccctcgccttcaggatcagtcccgcccaagcaccaggtggcaggggatgtgagggagactttcaactcctttttcattcggtagaggacttggttgagctccctcttgggtgcttggcattccttcaccagctgggcaagtttcaccggggagccagcctctgtcagcacctgcaggattctttgttcaaggtggccttctctgcccgggtcagcaggagcctgggccatgctgacagcagctgcaaggagtcggagagacttggcaggtgtgcaggcttctgcactgtggccctgagagggtgggctaggtcgaggctggggcttctgaagtggccgagcctggtgcttcttgcagctct

SEQ ID NO: 14867 - RNA, 3879 nt, Homo sapiens
  source 1..3879: mol_type = other RNA
gctgggattacaggcatgagccactacacccagcaactgtcaacttgtaatacaaaaataccttcaagctgataatcaagaacatttagtgactttaaaaagctgacagaatatttccatgctacacaaaacagttctatacacagctttacagttttaaagttctttgctggcacttgactttatagttaacacaatgactactgatatcaacgaaatactgtttttagcttatatatattttcaaaatcagtattacctcacaaaacagtaaagaaatatcacttctgctgaagaatcctctaagatgaacaccaaaactgtacagctaaaacatattgagaatcatgtaaatgtttaaggcaatagataaaaatttatacaatccagtgaaatttatacatgtccagcagaaaaaaaaggattattcctgattaaatgaagcatgtatcaggtttagatcaacaatacaaacctacaaagcaagttacttcttttttaaggttttttgatgatttggtgacacaactagaatataaccttttagatgaaaattggtgactttgcaaatacacattctaaattccaaaattaaaacgaaacttcttttcaaacagtagaatcctggtttgttgtttttactgtcaatgagcttatagctattctctgtattattataaatgaagtcaccactcagtcaccctaatacacatatggttttttttcttttttttttttccttttttttttttttttttttttgagacggagtctcactctgtcatccaggctggagtgcagtggcccagtctcggctctctgcagcctctgactcccgggtttcagcaattctcctgcctcagcctcctgggtagctgggattacaggcgcatgccaccacgcccagctaatttttgtatttttagtagagacggggtttcaccatgttggccaggctggtcttgaactgacctcaggtgatccacctgcctcggcctcccaaagtgctaggattacaggcgtgagccaccgcgcccagcctgcatttttttcttcatagaagaaaacaaaagtaaaacttcccaaattatgtttaacttataacacattttgtaaagaccccttaggttaaccattttggaagtctacattgttctgaagaaaaagatatgctttcaaaacactatctagcaattcctaatcatttttctattataaaaattaaaattcaaaagttattgccacagtgcttgtggcagtaaacagaatgtaaaatgtatcaaaagactaaattagtgtcatgaaacataaacatactaaataatcaaataaatactggacccttagcacagaaaattattaaaaggttgatttgagtgttaaaatttgtaacattaaattaccttcgtatttcaaacattactttttctaaaccaaaccagaagttaatcaacttttcctctcctttaggaacaaaaaggatatttaagatattttccaaaacagtaaaaacaacttagtgtttcaatctagttacaacaaaccctgttgatcctgtgcatttcactgaggcgctacacgcacccaaaaatcatcatcagaaagagaacttgaacttcctgactcagagtctggctcactgaatccacctaagtcccattcagtgctagactcacttggtatttcttcttcttcagtgaggaaactctgaccaggttcaaggcaggaaggataaacacgagcagagaggcaaaaaaagttagaatcaaactgcaagaggcctaatgtggtacctatattaatccattggtctcccctaatatcatattcatacacagtcacccggttctttttccactgtggggtgcgagaggtgatgagcaacaatttttggccatgcttgataattctgtagttgttggtctctgagaccaagggaatattattcatttgcctccattctgccctaactgggttgtagaccttcatgactgggatatcacagatacaatagatctcctcattgaagacgcaggcttcctgaaagtcattgcgcttcagagaaacgcacttcagccacatattgtggctaggatcataacagaacatgcgcttactgttgagagcatagagatagtctcgaattaccattaggtcaaaggataaaaaagaatggggcagtggagccaccaatgcccactggtttctcttaacattgtagcattccacttccttcaacttaactccagtaatagggtctcgcccccccaaaatgtagatatagccattgagatatgccacatccatgccctcacgacacagcaagcgatctgcaagttgctgccaactattctgagctggtttatacacccagaggtctgtcctgggctgagcagctagatagatgtcatggtcaggagagatacagacagctaaagtggtgacagtcctagtgtgagccagacaggtcaaaggtgacggcactttgtaaaggtcccccgagtatggatcacagcagagaaagggatctctggggtgtccaaagaagatcaccatctccttggcacacatacccagtctctggggtggattttctgctgcagatacaagagagttgctgctgctactgctgctgctgctgtttggcactggcaccagagacttgtacaacaggtcaccatagcgcatctgcagggccccttcaataacgtccaggcagtacttcttcacgatgggcttggtcagcagcccttctaagtagtcctgatcttcttcagtgaagtgcatccagcgcacgcacttgaagacttctgcagcactgggaccccgctctttgggagcagcctccagccactgcactgccacatggcacactgtctgctcactctccacgtccagactatccaagcgcaggacagccagcagctgggccagggtcagatctgctagagtctcctcccgaattgaacccatgtggctgagttgcttgaagttctgagctatataggactgggcctgggatcgcagcttgcgatggccaaaggcatctgcaaacttgaggatggcggtgcagttggtcaggtcaagacgtcgggctaagaaggaggcacaggcttcccgcacatattccagctgtagcatgtcggaggccgcgtacaggcgctccacgttggcctcactgagagacacacgacccgtgtagcagtagtcgaccaacacctcgaaggactcggcgtccacatcgtgcatggtcacgctggcctgctggctctcgtacatgccacctgtgaacatgctcttgaagtagggacatgccgcggccagcacattgcggttgcaggggaacaggcgacccgtgccaggcccgctgccaggcgtcaccacctcgatggtcacatcacacagcagccgcgcatcgtagaaggacttgagctgtgccagcagggctgcagaatgggccgtgtcctttaattcctctggacccgtgaaaaaggccgaaactgtgggtttgtgaatcttcttgggccgcttcccaccacggggactggctaggcggcgagagcgcggggcgtcttcccgggactgcatggtggagatggcgacgggcgctgatggcgagaaacgctgcaggacccggctctggctcctcctcaaccttccctcgctgacgctaagatagcagcgtctccgaagagacagcagcacgagcccatttactgaattcaaccctaccccgcagaaccgcctcccgttatcgtttagacagtggctgactcaccctctctcactcccgcgtcctttctccgcgtctgctcgccttcacaggacccgctggcttggagccgcagaagccgctactgcagcgtgggcgacaatgct

SEQ ID NO: 14868 - RNA, 2126 nt, Homo sapiens
  source 1..2126: mol_type = other RNA
gctgggattacaggcatgagccactacaccccgccagtattaactataataatagtccaatgctgcatccaggctattactgatgatgatgcctttaagacctaaacccctctgcctacttcaatgaatgaaccagaaatgttatcctcagcaaagagacctacagagttacttttgtgtataaaagctccctgtgtaggcatctgcatttgttagaaataccagaaattcagtgttaatcatcagtgtaagcataagatacatatatcttcccctaccatgtgatgaaaggacttagttgaaattatgtgggcattgccagttaccacaaaaagcttggttaaggcccattttcattcactaaggaacatcttgggatgaacttgagtttttattaggttattgtgggtagctatgactcattactaagctacaagagccaaattaattctggtttcagttagaactctattcacagttctaaagcatgcaaatccactcagccacctttatgaatttctcacaaagtctaaagtacaactgcttgccagttaacacttccttacggtttgaaggtttcagaaagatgtaacaataatatgttacaaaagtctcgtttgtcaggttataattgactgtaaacaggtttgggggagggagaggcacacatcataagacattacataacaatgttttgtgccagattttttagtccatttgtgcaggtaaaaagctaactcttaaagggccaaagaacagagacatttgtcttccaccttattccactccaaactcaggctgtcttggcagtggaggatactgttctatgtcagataatacagaaatatttggcatcacttccattaaattctttcctgcagcacacattattcatgtcctcttcactgtcacttgctcttgccagactgtcgaaagggtggttgaagtgttcttgctggtcagaagaaactgctccaaagaacatgcaagaaaactttctgagacacagagaccctggcacttcctctgtgttgctgacactgctttctgatacttcactgacatctccatccactcttttcattgcagggctgccacagttttccaatgcagatatgtttgtgagagtctccttaggataaagccttcttggtgctgctttttttgaaatacattccagggcctggccagttacatttttgccagcctttttttcaatcagatctgacctttttcgtttctgtgaaagacacagtgactgtggtgaagatgctctactttgttcatcagctaatgtggccaaaataaagttagcttccactaacatatcatcaatactcaaagccagaggtttcccagggaaatcaaaataaatggatataggagcatgtgtagcttctgaaaatgtcagtattcccttcaattctttgaaacaaaatgttatctcagtgtccattccaatttgaaagaagtcaaactcatctgagccaacaaacatctcactgtgtacagcattgctcaaatccattgattcctcattagaactcttgaggcaaaaattcagtggagtaacagcaagagtaacttcctcttgacttgatgtaaaaagaacaatggcatcagcaagcaatcttggttgaatcattagcgtattagtacaaacattcttgtcaaaaataacttgcaaaggctgactttcttgaaaacatatattatgagttcttttaataccatgtctgtagaagaattgaataactactttgcatttatcagatctggtgaatattctgcacttctctatatttctttcaagggaattcagacatctaaagatgggcaaaattgacttcattcccaatttgcattttaaatgcagtgttgtgtcaagttcattttcactcattttcactaaagctgaccattgataatgctgaaaaaacacaggagagaacaggacacatccatatgctgaccgagaagaattcacacatcttagagcaagaccttttttagatgggtctagccagaactcgtcactaattcgtgatagagcttgaactgctttcccaaatactttcacctgactgccgctcatcacgcacttcagcatggctgccatccgccct

SEQ ID NO: 14869 - RNA, 2876 nt, Homo sapiens
  source 1..2876: mol_type = other RNA
gctgggattacaggcatgagccactacaccccgccagtattaactataataatagtccaatgctgcatccaggctattactgatgatgatgcctttaagacctaaacccctctgcctacttcaatgaatgaaccagaaatgttatcctcagcaaagagacctacagagttacttttgtgtataaaagctccctgtgtaggcatctgcatttgttagaaataccagaaattcagtgttaatcatcagtgtaagcataagatacatatatcttcccctaccatgtgatgaaaggacttagttgaaattatgtgggcattgccagttaccacaaaaagcttggttaaggcccattttcattcactaaggaacatcttgggatgaacttgagtttttattaggttattgtgggtagctatgactcattactaagctacaagagccaaattaattctggtttcagttagaactctattcacagttctaaagcatgcaaatccactcagccacctttatgaatttctcacaaagtctaaagtacaactgcttgccagttaacacttccttacggtttgaaggtttcagaaagatgtaacaataatatgttacaaaagtctcgtttgtcaggttataattgactgtaaacaggtttgggggagggagaggcacacatcataagacattacataacaatgttttgtgccagattttttagtccatttgtgcaggtaaaaagctaactcttaaagggccaaagaacagagacatttgtcttccaccttattccactccaaactcaggctgtcttggcagtggaggatactgttctatgtcagataatacagaaatatttggcatcacttccattaaattctttcctgcagcacactgcaaaataaaaaatcacatctgaaaatcagaacaatttgaggttaggaaataaaattttacaatatgtaaaaacactccaggttgggcgcagtggctcaagtctgtaatcccagcactttgggaggccgaggtgggcagatcacttgaggccaggagttcaagaccaccctggccaacatggcgaaaccctgtctctacaaaataccagaaattagccaggcatggtggcacgcacctgcaatcccagctgcacgggaggctgaggcaggagaatcgcttggacctgggaggcagatgttgcagtgagcagagattgcaccactgcacttgagcctgagtgacaaagtgagactccgtctaaaaaagccaagtgaaagtgactatatatttttactcttgatcttttttccagggtttattctacttaaagtcttaaaatataaaaaacaatgcacaaaaaaggccatggtattacatgagaaaactaaaatccaaatgtttgcaatcaaatacaaaagatacctgactacaaatcacaaaattccatttcaagccatcttgatggcactctaaatggctgttgaataaagtttaaatacctttataaaactagcaaagatgttaaaagctctagggtgaacgtgcattgaattgaagaactctaatgggcttttttccttcacagaaaactcttctgcctcacaagtagcataatggatttaaagcaagttacatacacttgacaaacagctatttctagatatggttgttgtacaagatgatgtggtttaaaagcccatcctccattaaaaggaagtcctggacaacctcttttagacactaaacatgcaaactcgtgcttgaggggcaaatgagccagtcactgggctggggcccagctcagccatcattaagcattagaatatagagaaactgccattattcatgtcctcttcactgtcacttgctcttgccagactgtcgaaagggtggttgaagtgttcttgctggtcagaagaaactgctccaaagaacatgcaagaaaactttctgagacacagagaccctggcacttcctctgtgttgctgacactgctttctgatacttcactgacatctccatccactcttttcattgcagggctgccacagttttccaatgcagatatgtttgtgagagtctccttaggataaagccttcttggtgctgctttttttgaaatacattccagggcctggccagttacatttttgccagcctttttttcaatcagatctgacctttttcgtttctgtgaaagacacagtgactgtggtgaagatgctctactttgttcatcagctaatgtggccaaaataaagttagcttccactaacatatcatcaatactcaaagccagaggtttcccagggaaatcaaaataaatggatataggagcatgtgtagcttctgaaaatgtcagtattcccttcaattctttgaaacaaaatgttatctcagtgtccattccaatttgaaagaagtcaaactcatctgagccaacaaacatctcactgtgtacagcattgctcaaatcatgtctgtagaagaattgaataactactttgcatttatcagatctggtgaatattctgcacttctctatatttctttcaagggaattcagacatctaaagatgggcaaaattgacttcattcccaatttgcattttaaatgcagtgttgtgtcaagttcattttcactcattttcactaaagctgaccattgataatgctgaaaaaacacaggagagaacaggacacatccatatgctgaccgagaagaattcacacatcttagagcaagaccttttttagatgggtctagccagaactcgtcactaattcgtgatagagcttgaactgctttcccaaatactttcacctgactgccgctcatcacgcacttcagcatggctgccatccgccctaaaaagcaggctcggaa

SEQ ID NO: 14870 - RNA, 2989 nt, Homo sapiens
  source 1..2989: mol_type = other RNA
gctgggattacaggcatgagccactacaccccgccagtattaactataataatagtccaatgctgcatccaggctattactgatgatgatgcctttaagacctaaacccctctgcctacttcaatgaatgaaccagaaatgttatcctcagcaaagagacctacagagttacttttgtgtataaaagctccctgtgtaggcatctgcatttgttagaaataccagaaattcagtgttaatcatcagtgtaagcataagatacatatatcttcccctaccatgtgatgaaaggacttagttgaaattatgtgggcattgccagttaccacaaaaagcttggttaaggcccattttcattcactaaggaacatcttgggatgaacttgagtttttattaggttattgtgggtagctatgactcattactaagctacaagagccaaattaattctggtttcagttagaactctattcacagttctaaagcatgcaaatccactcagccacctttatgaatttctcacaaagtctaaagtacaactgcttgccagttaacacttccttacggtttgaaggtttcagaaagatgtaacaataatatgttacaaaagtctcgtttgtcaggttataattgactgtaaacaggtttgggggagggagaggcacacatcataagacattacataacaatgttttgtgccagattttttagtccatttgtgcaggtaaaaagctaactcttaaagggccaaagaacagagacatttgtcttccaccttattccactccaaactcaggctgtcttggcagtggaggatactgttctatgtcagataatacagaaatatttggcatcacttccattaaattctttcctgcagcacactgcaaaataaaaaatcacatctgaaaatcagaacaatttgaggttaggaaataaaattttacaatatgtaaaaacactccaggttgggcgcagtggctcaagtctgtaatcccagcactttgggaggccgaggtgggcagatcacttgaggccaggagttcaagaccaccctggccaacatggcgaaaccctgtctctacaaaataccagaaattagccaggcatggtggcacgcacctgcaatcccagctgcacgggaggctgaggcaggagaatcgcttggacctgggaggcagatgttgcagtgagcagagattgcaccactgcacttgagcctgagtgacaaagtgagactccgtctaaaaaagccaagtgaaagtgactatatatttttactcttgatcttttttccagggtttattctacttaaagtcttaaaatataaaaaacaatgcacaaaaaaggccatggtattacatgagaaaactaaaatccaaatgtttgcaatcaaatacaaaagatacctgactacaaatcacaaaattccatttcaagccatcttgatggcactctaaatggctgttgaataaagtttaaatacctttataaaactagcaaagatgttaaaagctctagggtgaacgtgcattgaattgaagaactctaatgggcttttttccttcacagaaaactcttctgcctcacaagtagcataatggatttaaagcaagttacatacacttgacaaacagctatttctagatatggttgttgtacaagatgatgtggtttaaaagcccatcctccattaaaaggaagtcctggacaacctcttttagacactaaacatgcaaactcgtgcttgaggggcaaatgagccagtcactgggctggggcccagctcagccatcattaagcattagaatatagagaaactgccattattcatgtcctcttcactgtcacttgctcttgccagactgtcgaaagggtggttgaagtgttcttgctggtcagaagaaactgctccaaagaacatgcaagaaaactttctgagacacagagaccctggcacttcctctgtgttgctgacactgctttctgatacttcactgacatctccatccactcttttcattgcagggctgccacagttttccaatgcagatatgtttgtgagagtctccttaggataaagccttcttggtgctgctttttttgaaatacattccagggcctggccagttacatttttgccagcctttttttcaatcagatctgacctttttcgtttctgtgaaagacacagtgactgtggtgaagatgctctactttgttcatcagctaatgtggccaaaataaagttagcttccactaacatatcatcaatactcaaagccagaggtttcccagggaaatcaaaataaatggatataggagcatgtgtagcttctgaaaatgtcagtattcccttcaattctttgaaacaaaatgttatctcagtgtccattccaatttgaaagaagtcaaactcatctgagccaacaaacatctcactgtgtacagcattgctcaaatccattgattcctcattagaactcttgaggcaaaaattcagtggagtaacagcaagagtaacttcctcttgacttgatgtaaaaagaacaatggcatcagcaagcaatcatgtctgtagaagaattgaataactactttgcatttatcagatctggtgaatattctgcacttctctatatttctttcaagggaattcagacatctaaagatgggcaaaattgacttcattcccaatttgcattttaaatgcagtgttgtgtcaagttcattttcactcattttcactaaagctgaccattgataatgctgaaaaaacacaggagagaacaggacacatccatatgctgaccgagaagaattcacacatcttagagcaagaccttttttagatgggtctagccagaactcgtcactaattcgtgatagagcttgaactgctttcccaaatactcgaatgttccggggataggggcacggtcctccgtttccagacggttcctactcgtttcccgcaaaaagcacctc

SEQ ID NO: 14871 - RNA, 3121 nt, Homo sapiens
  source 1..3121: mol_type = other RNA
gctgggattacaggcatgagccactacaccccgccagtattaactataataatagtccaatgctgcatccaggctattactgatgatgatgcctttaagacctaaacccctctgcctacttcaatgaatgaaccagaaatgttatcctcagcaaagagacctacagagttacttttgtgtataaaagctccctgtgtaggcatctgcatttgttagaaataccagaaattcagtgttaatcatcagtgtaagcataagatacatatatcttcccctaccatgtgatgaaaggacttagttgaaattatgtgggcattgccagttaccacaaaaagcttggttaaggcccattttcattcactaaggaacatcttgggatgaacttgagtttttattaggttattgtgggtagctatgactcattactaagctacaagagccaaattaattctggtttcagttagaactctattcacagttctaaagcatgcaaatccactcagccacctttatgaatttctcacaaagtctaaagtacaactgcttgccagttaacacttccttacggtttgaaggtttcagaaagatgtaacaataatatgttacaaaagtctcgtttgtcaggttataattgactgtaaacaggtttgggggagggagaggcacacatcataagacattacataacaatgttttgtgccagattttttagtccatttgtgcaggtaaaaagctaactcttaaagggccaaagaacagagacatttgtcttccaccttattccactccaaactcaggctgtcttggcagtggaggatactgttctatgtcagataatacagaaatatttggcatcacttccattaaattctttcctgcagcacactgcaaaataaaaaatcacatctgaaaatcagaacaatttgaggttaggaaataaaattttacaatatgtaaaaacactccaggttgggcgcagtggctcaagtctgtaatcccagcactttgggaggccgaggtgggcagatcacttgaggccaggagttcaagaccaccctggccaacatggcgaaaccctgtctctacaaaataccagaaattagccaggcatggtggcacgcacctgcaatcccagctgcacgggaggctgaggcaggagaatcgcttggacctgggaggcagatgttgcagtgagcagagattgcaccactgcacttgagcctgagtgacaaagtgagactccgtctaaaaaagccaagtgaaagtgactatatatttttactcttgatcttttttccagggtttattctacttaaagtcttaaaatataaaaaacaatgcacaaaaaaggccatggtattacatgagaaaactaaaatccaaatgtttgcaatcaaatacaaaagatacctgactacaaatcacaaaattccatttcaagccatcttgatggcactctaaatggctgttgaataaagtttaaatacctttataaaactagcaaagatgttaaaagctctagggtgaacgtgcattgaattgaagaactctaatgggcttttttccttcacagaaaactcttctgcctcacaagtagcataatggatttaaagcaagttacatacacttgacaaacagctatttctagatatggttgttgtacaagatgatgtggtttaaaagcccatcctccattaaaaggaagtcctggacaacctcttttagacactaaacatgcaaactcgtgcttgaggggcaaatgagccagtcactgggctggggcccagctcagccatcattaagcattagaatatagagaaactgccattattcatgtcctcttcactgtcacttgctcttgccagactgtcgaaagggtggttgaagtgttcttgctggtcagaagaaactgctccaaagaacatgcaagaaaactttctgagacacagagaccctggcacttcctctgtgttgctgacactgctttctgatacttcactgacatctccatccactcttttcattgcagggctgccacagttttccaatgcagatatgtttgtgagagtctccttaggataaagccttcttggtgctgctttttttgaaatacattccagggcctggccagttacatttttgccagcctttttttcaatcagatctgacctttttcgtttctgtgaaagacacagtgactgtggtgaagatgctctactttgttcatcagctaatgtggccaaaataaagttagcttccactaacatatcatcaatactcaaagccagaggtttcccagggaaatcaaaataaatggatataggagcatgtgtagcttctgaaaatgtcagtattcccttcaattctttgaaacaaaatgttatctcagtgtccattccaatttgaaagaagtcaaactcatctgagccaacaaacatctcactgtgtacagcattgctcaaatccattgattcctcattagaactcttgaggcaaaaattcagtggagtaacagcaagagtaacttcctcttgacttgatgtaaaaagaacaatggcatcagcaagcaatcatgtctgtagaagaattgaataactactttgcatttatcagatctggtgaatattctgcacttctctatatttctttcaagggaattcagacatctaaagatgggcaaaattgacttcattcccaatttgcattttaaatgcagtgttgtgtcaagttcattttcactcattttcactaaagctgaccattgataatgctgaaaaaacacaggagagaacaggacacatccatatgctgaccgagaagaattcacacatcttagagcaagaccttttttagatgggtctagccagaactcgtcactaattcgtgatagagcttgaactgctttcccaaatactgactgccgctcatcacgcacttcagcatggctgccatccgccctaaaaagcaggctcggaaggcgcgcctcagctcgacggcccaggtgcccggatgttgcccgcgcttttcaaagcttcgcgatctcgtctctgcactctaccaccccgcctccacaagttcccaaacggctttacggcggagaagggtccgtgcgggcctccgt

SEQ ID NO: 14872 - RNA, 2937 nt, Homo sapiens
  source 1..2937: mol_type = other RNA
gctgggattacaggcatgagccactacaccccgccagtattaactataataatagtccaatgctgcatccaggctattactgatgatgatgcctttaagacctaaacccctctgcctacttcaatgaatgaaccagaaatgttatcctcagcaaagagacctacagagttacttttgtgtataaaagctccctgtgtaggcatctgcatttgttagaaataccagaaattcagtgttaatcatcagtgtaagcataagatacatatatcttcccctaccatgtgatgaaaggacttagttgaaattatgtgggcattgccagttaccacaaaaagcttggttaaggcccattttcattcactaaggaacatcttgggatgaacttgagtttttattaggttattgtgggtagctatgactcattactaagctacaagagccaaattaattctggtttcagttagaactctattcacagttctaaagcatgcaaatccactcagccacctttatgaatttctcacaaagtctaaagtacaactgcttgccagttaacacttccttacggtttgaaggtttcagaaagatgtaacaataatatgttacaaaagtctcgtttgtcaggttataattgactgtaaacaggtttgggggagggagaggcacacatcataagacattacataacaatgttttgtgccagattttttagtccatttgtgcaggtaaaaagctaactcttaaagggccaaagaacagagacatttgtcttccaccttattccactccaaactcaggctgtcttggcagtggaggatactgttctatgtcagataatacagaaatatttggcatcacttccattaaattctttcctgcagcacactgcaaaataaaaaatcacatctgaaaatcagaacaatttgaggttaggaaataaaattttacaatatgtaaaaacactccaggttgggcgcagtggctcaagtctgtaatcccagcactttgggaggccgaggtgggcagatcacttgaggccaggagttcaagaccaccctggccaacatggcgaaaccctgtctctacaaaataccagaaattagccaggcatggtggcacgcacctgcaatcccagctgcacgggaggctgaggcaggagaatcgcttggacctgggaggcagatgttgcagtgagcagagattgcaccactgcacttgagcctgagtgacaaagtgagactccgtctaaaaaagccaagtgaaagtgactatatatttttactcttgatcttttttccagggtttattctacttaaagtcttaaaatataaaaaacaatgcacaaaaaaggccatggtattacatgagaaaactaaaatccaaatgtttgcaatcaaatacaaaagatacctgactacaaatcacaaaattccatttcaagccatcttgatggcactctaaatggctgttgaataaagtttaaatacctttataaaactagcaaagatgttaaaagctctagggtgaacgtgcattgaattgaagaactctaatgggcttttttccttcacagaaaactcttctgcctcacaagtagcataatggatttaaagcaagttacatacacttgacaaacagctatttctagatatggttgttgtacaagatgatgtggtttaaaagcccatcctccattaaaaggaagtcctggacaacctcttttagacactaaacatgcaaactcgtgcttgaggggcaaatgagccagtcactgggctggggcccagctcagccatcattaagcattagaatatagagaaactgccattattcatgtcctcttcactgtcacttgctcttgccagactgtcgaaagggtggttgaagtgttcttgctggtcagaagaaactgctccaaagaacatgcaagaaaactttctgagacacagagaccctggcacttcctctgtgttgctgacactgctttctgatacttcactgacatctccatccactcttttcattgcagggctgccacagttttccaatgcagatatgtttgtgagagtctccttaggataaagccttcttggtgctgctttttttgaaatacattccagggcctggccagttacatttttgccagcctttttttcaatcagatctgacctttttcgtttctgtgaaagacacagtgactgtggtgaagatgctctactttgttcatcagctaatgtggccaaaataaagttagcttccactaacatatcatcaatactcaaagccagaggtttcccagggaaatcaaaataaatggatataggagcatgtgtagcttctgaaaatgtcagtattcccttcaattctttgaaacaaaatgttatctcagtgtccattccaatttgaaagaagtcaaactcatctgagccaacaaacatctcactgtgtacagcattgctcaaatccattgattcctcattagaactcttgaggcaaaaattcagtggagtaacagcaagagtaacttcctcttgacttgatgtaaaaagaacaatggcatcagcaagcaatcatgtctgtagaagaattgaataactactttgcatttatcagatctggtgaatattctgcacttctctatatttctttcaagggaattcagacatctaaagatgggcaaaattgacttcattcccaatttgcattttaaatgcagtgttgtgtcaagttcattttcactcattttcactaaagctgaccattgataatgctgaaaaaacacaggagagaacaggacacatccatatgctgaccgagaagaattcacacatcttagagcaagaccttttttagatgggtctagccagaactcgtcactaattcgtgatagagcttgaactgctttcccaaatattcagcatggctgccatccgccct

SEQ ID NO: 14873 - RNA, 2933 nt, Homo sapiens
  source 1..2933: mol_type = other RNA
gctgggattacaggcatgagccactacaccccgccagtattaactataataatagtccaatgctgcatccaggctattactgatgatgatgcctttaagacctaaacccctctgcctacttcaatgaatgaaccagaaatgttatcctcagcaaagagacctacagagttacttttgtgtataaaagctccctgtgtaggcatctgcatttgttagaaataccagaaattcagtgttaatcatcagtgtaagcataagatacatatatcttcccctaccatgtgatgaaaggacttagttgaaattatgtgggcattgccagttaccacaaaaagcttggttaaggcccattttcattcactaaggaacatcttgggatgaacttgagtttttattaggttattgtgggtagctatgactcattactaagctacaagagccaaattaattctggtttcagttagaactctattcacagttctaaagcatgcaaatccactcagccacctttatgaatttctcacaaagtctaaagtacaactgcttgccagttaacacttccttacggtttgaaggtttcagaaagatgtaacaataatatgttacaaaagtctcgtttgtcaggttataattgactgtaaacaggtttgggggagggagaggcacacatcataagacattacataacaatgttttgtgccagattttttagtccatttgtgcaggtaaaaagctaactcttaaagggccaaagaacagagacatttgtcttccaccttattccactccaaactcaggctgtcttggcagtggaggatactgttctatgtcagataatacagaaatatttggcatcacttccattaaattctttcctgcagcacactgcaaaataaaaaatcacatctgaaaatcagaacaatttgaggttaggaaataaaattttacaatatgtaaaaacactccaggttgggcgcagtggctcaagtctgtaatcccagcactttgggaggccgaggtgggcagatcacttgaggccaggagttcaagaccaccctggccaacatggcgaaaccctgtctctacaaaataccagaaattagccaggcatggtggcacgcacctgcaatcccagctgcacgggaggctgaggcaggagaatcgcttggacctgggaggcagatgttgcagtgagcagagattgcaccactgcacttgagcctgagtgacaaagtgagactccgtctaaaaaagccaagtgaaagtgactatatatttttactcttgatcttttttccagggtttattctacttaaagtcttaaaatataaaaaacaatgcacaaaaaaggccatggtattacatgagaaaactaaaatccaaatgtttgcaatcaaatacaaaagatacctgactacaaatcacaaaattccatttcaagccatcttgatggcactctaaatggctgttgaataaagtttaaatacctttataaaactagcaaagatgttaaaagctctagggtgaacgtgcattgaattgaagaactctaatgggcttttttccttcacagaaaactcttctgcctcacaagtagcataatggatttaaagcaagttacatacacttgacaaacagctatttctagatatggttgttgtacaagatgatgtggtttaaaagcccatcctccattaaaaggaagtcctggacaacctcttttagacactaaacatgcaaactcgtgcttgaggggcaaatgagccagtcactgggctggggcccagctcagccatcattaagcattagaatatagagaaactgccattattcatgtcctcttcactgtcacttgctcttgccagactgtcgaaagggtggttgaagtgttcttgctggtcagaagaaactgctccaaagaacatgcaagaaaactttctgagacacagagaccctggcacttcctctgtgttgctgacactgctttctgatacttcactgacatctccatccactcttttcattgcagggctgccacagttttccaatgcagatatgtttgtgagagtctccttaggataaagccttcttggtgctgctttttttgaaatacattccagggcctggccagttacatttttgccagcctttttttcaatcagatctgacctttttcgtttctgtgaaagacacagtgactgtggtgaagatgctctactttgttcatcagctaatgtggccaaaataaagttagcttccactaacatatcatcaatactcaaagccagaggtttcccagggaaatcaaaataaatggatataggagcatgtgtagcttctgaaaatgtcagtattcccttcaattctttgaaacaaaatgttatctcagtgtccattccaatttgaaagaagtcaaactcatctgagccaacaaacatctcactgtgtacagcattgctcaaatccattgattcctcattagaactcttgaggcaaaaattcagtggagtaacagcaagagtaacttcctcttgacttgatgtaaaaagaacaatggcatcagcaagcaatcttggttgaatcattagcgtattagtacaaacattcttgtcaaaaataacttgcaaaggctgactttcttgaaaacatatattatgagttcttttaataccatgtctgtagaagaattgaataactactttgcatttatcagatctggtgaatattctgcacttctctatatttctttcaagggaattcagacatctaaagatgggcaaaattgaaccttttttagatgggtctagccagaactcgtcactaattcgtgatagagcttgaactgctttcccaaatactgactgccgctcatcacgcacttcagcatggctgccatccgccctaaaaagcaggctcggaaggcgcgcctcagc

SEQ ID NO: 14874 - RNA, 2990 nt, Homo sapiens
  source 1..2990: mol_type = other RNA
gctgggattacaggcatgagccactacaccccgccagtattaactataataatagtccaatgctgcatccaggctattactgatgatgatgcctttaagacctaaacccctctgcctacttcaatgaatgaaccagaaatgttatcctcagcaaagagacctacagagttacttttgtgtataaaagctccctgtgtaggcatctgcatttgttagaaataccagaaattcagtgttaatcatcagtgtaagcataagatacatatatcttcccctaccatgtgatgaaaggacttagttgaaattatgtgggcattgccagttaccacaaaaagcttggttaaggcccattttcattcactaaggaacatcttgggatgaacttgagtttttattaggttattgtgggtagctatgactcattactaagctacaagagccaaattaattctggtttcagttagaactctattcacagttctaaagcatgcaaatccactcagccacctttatgaatttctcacaaagtctaaagtacaactgcttgccagttaacacttccttacggtttgaaggtttcagaaagatgtaacaataatatgttacaaaagtctcgtttgtcaggttataattgactgtaaacaggtttgggggagggagaggcacacatcataagacattacataacaatgttttgtgccagattttttagtccatttgtgcaggtaaaaagctaactcttaaagggccaaagaacagagacatttgtcttccaccttattccactccaaactcaggctgtcttggcagtggaggatactgttctatgtcagataatacagaaatatttggcatcacttccattaaattctttcctgcagcacactgcaaaataaaaaatcacatctgaaaatcagaacaatttgaggttaggaaataaaattttacaatatgtaaaaacactccaggttgggcgcagtggctcaagtctgtaatcccagcactttgggaggccgaggtgggcagatcacttgaggccaggagttcaagaccaccctggccaacatggcgaaaccctgtctctacaaaataccagaaattagccaggcatggtggcacgcacctgcaatcccagctgcacgggaggctgaggcaggagaatcgcttggacctgggaggcagatgttgcagtgagcagagattgcaccactgcacttgagcctgagtgacaaagtgagactccgtctaaaaaagccaagtgaaagtgactatatatttttactcttgatcttttttccagggtttattctacttaaagtcttaaaatataaaaaacaatgcacaaaaaaggccatggtattacatgagaaaactaaaatccaaatgtttgcaatcaaatacaaaagatacctgactacaaatcacaaaattccatttcaagccatcttgatggcactctaaatggctgttgaataaagtttaaatacctttataaaactagcaaagatgttaaaagctctagggtgaacgtgcattgaattgaagaactctaatgggcttttttccttcacagaaaactcttctgcctcacaagtagcataatggatttaaagcaagttacatacacttgacaaacagctatttctagatatggttgttgtacaagatgatgtggtttaaaagcccatcctccattaaaaggaagtcctggacaacctcttttagacactaaacatgcaaactcgtgcttgaggggcaaatgagccagtcactgggctggggcccagctcagccatcattaagcattagaatatagagaaactgccattattcatgtcctcttcactgtcacttgctcttgccagactgtcgaaagggtggttgaagtgttcttgctggtcagaagaaactgctccaaagaacatgcaagaaaactttctgagacacagagaccctggcacttcctctgtgttgctgacactgctttctgatacttcactgacatctccatccactcttttcattgcagggctgccacagttttccaatgcagatatgtttgtgagagtctccttaggataaagccttcttggtgctgctttttttgaaatacattccagggcctggccagttacatttttgccagcctttttttcaatcagatctgacctttttcgtttctgtgaaagacacagtgactgtggtgaagatgctctactttgttcatcagctaatgtggccaaaataaagttagcttccactaacatatcatcaatactcaaagccagaggtttcccagggaaatcaaaataaatggatataggagcatgtgtagcttctgaaaatgtcagtattcccttcaattctttgaaacaaaatgttatctcagtgtccattccaatttgaaagaagtcaaactcatctgagccaacaaacatctcactgtgtacagcattgctcaaatccattgattcctcattagaactcttgaggcaaaaattcagtggagtaacagcaagagtaacttcctcttgacttgatgtaaaaagaacaatggcatcagcaagcaatcttggttgaatcattagcgtattagtacaaacattcttgtcaaaaataacttgcaaaggctgactttcttgaaaacatatattatgagttcttttaataccatgtctgtagaagaattgaataactactttgcatttatcagatctggtgaatattctgcacttctctatatttctttcaagggaattcagacatctaaagatgggcaaaattgaaccttttttagatgggtctagccagaactcgtcactaattcgtgatagagcttgaactgctttcccaaatactttcacctgactgccgctcatcacgcacttcagcatggctgccatccgccctaaaaagcaggctcggaaggcgcgcctcagctcgacggcccaggtgcccggatgttgcccgcgcttttcaaagcttcgcga

SEQ ID NO: 14875 - RNA, 3074 nt, Homo sapiens
  source 1..3074: mol_type = other RNA
gctgggattacaggcatgagccactacaccccgccagtattaactataataatagtccaatgctgcatccaggctattactgatgatgatgcctttaagacctaaacccctctgcctacttcaatgaatgaaccagaaatgttatcctcagcaaagagacctacagagttacttttgtgtataaaagctccctgtgtaggcatctgcatttgttagaaataccagaaattcagtgttaatcatcagtgtaagcataagatacatatatcttcccctaccatgtgatgaaaggacttagttgaaattatgtgggcattgccagttaccacaaaaagcttggttaaggcccattttcattcactaaggaacatcttgggatgaacttgagtttttattaggttattgtgggtagctatgactcattactaagctacaagagccaaattaattctggtttcagttagaactctattcacagttctaaagcatgcaaatccactcagccacctttatgaatttctcacaaagtctaaagtacaactgcttgccagttaacacttccttacggtttgaaggtttcagaaagatgtaacaataatatgttacaaaagtctcgtttgtcaggttataattgactgtaaacaggtttgggggagggagaggcacacatcataagacattacataacaatgttttgtgccagattttttagtccatttgtgcaggtaaaaagctaactcttaaagggccaaagaacagagacatttgtcttccaccttattccactccaaactcaggctgtcttggcagtggaggatactgttctatgtcagataatacagaaatatttggcatcacttccattaaattctttcctgcagcacactgcaaaataaaaaatcacatctgaaaatcagaacaatttgaggttaggaaataaaattttacaatatgtaaaaacactccaggttgggcgcagtggctcaagtctgtaatcccagcactttgggaggccgaggtgggcagatcacttgaggccaggagttcaagaccaccctggccaacatggcgaaaccctgtctctacaaaataccagaaattagccaggcatggtggcacgcacctgcaatcccagctgcacgggaggctgaggcaggagaatcgcttggacctgggaggcagatgttgcagtgagcagagattgcaccactgcacttgagcctgagtgacaaagtgagactccgtctaaaaaagccaagtgaaagtgactatatatttttactcttgatcttttttccagggtttattctacttaaagtcttaaaatataaaaaacaatgcacaaaaaaggccatggtattacatgagaaaactaaaatccaaatgtttgcaatcaaatacaaaagatacctgactacaaatcacaaaattccatttcaagccatcttgatggcactctaaatggctgttgaataaagtttaaatacctttataaaactagcaaagatgttaaaagctctagggtgaacgtgcattgaattgaagaactctaatgggcttttttccttcacagaaaactcttctgcctcacaagtagcataatggatttaaagcaagttacatacacttgacaaacagctatttctagatatggttgttgtacaagatgatgtggtttaaaagcccatcctccattaaaaggaagtcctggacaacctcttttagacactaaacatgcaaactcgtgcttgaggggcaaatgagccagtcactgggctggggcccagctcagccatcattaagcattagaatatagagaaactgccattattcatgtcctcttcactgtcacttgctcttgccagactgtcgaaagggtggttgaagtgttcttgctggtcagaagaaactgctccaaagaacatgcaagaaaactttctgagacacagagaccctggcacttcctctgtgttgctgacactgctttctgatacttcactgacatctccatccactcttttcattgcagggctgccacagttttccaatgcagatatgtttgtgagagtctccttaggataaagccttcttggtgctgctttttttgaaatacattccagggcctggccagttacatttttgccagcctttttttcaatcagatctgacctttttcgtttctgtgaaagacacagtgactgtggtgaagatgctctactttgttcatcagctaatgtggccaaaataaagttagcttccactaacatatcatcaatactcaaagccagaggtttcccagggaaatcaaaataaatggatataggagcatgtgtagcttctgaaaatgtcagtattcccttcaattctttgaaacaaaatgttatctcagtgtccattccaatttgaaagaagtcaaactcatctgagccaacaaacatctcactgtgtacagcattgctcaaatccattgattcctcattagaactcttgaggcaaaaattcagtggagtaacagcaagagtaacttcctcttgacttgatgtaaaaagaacaatggcatcagcaagcaatcttggttgaatcattagcgtattagtacaaacattcttgtcaaaaataacttgcaaaggctgactttcttgaaaacatatattatgagttcttttaataccatgtctgtagaagaattgaataactactttgcatttatcagatctggtgaatattctgcacttctctatatttctttcaagggaattcagacatctaaagatgggcaaaattgacttcattcccaatttgcattttaaatgcagtgttgtgtcaagttcattttcactcattttcactaaagctgaccattgataatgaccttttttagatgggtctagccagaactcgtcactaattcgtgatagagcttgaactgctttcccaaatactttcacctgactgccgctcatcacgcacttcagcatggctgccatccgccctaaaaagcaggctcggaaggcgcgcctcagctcgacggcccaggtgcccggatgttgcccgcgcttttcaaagcttcgcga

SEQ ID NO: 14876 - RNA, 3202 nt, Homo sapiens
  source 1..3202: mol_type = other RNA
gctgggattacaggcatgagccactacaccccgccagtattaactataataatagtccaatgctgcatccaggctattactgatgatgatgcctttaagacctaaacccctctgcctacttcaatgaatgaaccagaaatgttatcctcagcaaagagacctacagagttacttttgtgtataaaagctccctgtgtaggcatctgcatttgttagaaataccagaaattcagtgttaatcatcagtgtaagcataagatacatatatcttcccctaccatgtgatgaaaggacttagttgaaattatgtgggcattgccagttaccacaaaaagcttggttaaggcccattttcattcactaaggaacatcttgggatgaacttgagtttttattaggttattgtgggtagctatgactcattactaagctacaagagccaaattaattctggtttcagttagaactctattcacagttctaaagcatgcaaatccactcagccacctttatgaatttctcacaaagtctaaagtacaactgcttgccagttaacacttccttacggtttgaaggtttcagaaagatgtaacaataatatgttacaaaagtctcgtttgtcaggttataattgactgtaaacaggtttgggggagggagaggcacacatcataagacattacataacaatgttttgtgccagattttttagtccatttgtgcaggtaaaaagctaactcttaaagggccaaagaacagagacatttgtcttccaccttattccactccaaactcaggctgtcttggcagtggaggatactgttctatgtcagataatacagaaatatttggcatcacttccattaaattctttcctgcagcacactgcaaaataaaaaatcacatctgaaaatcagaacaatttgaggttaggaaataaaattttacaatatgtaaaaacactccaggttgggcgcagtggctcaagtctgtaatcccagcactttgggaggccgaggtgggcagatcacttgaggccaggagttcaagaccaccctggccaacatggcgaaaccctgtctctacaaaataccagaaattagccaggcatggtggcacgcacctgcaatcccagctgcacgggaggctgaggcaggagaatcgcttggacctgggaggcagatgttgcagtgagcagagattgcaccactgcacttgagcctgagtgacaaagtgagactccgtctaaaaaagccaagtgaaagtgactatatatttttactcttgatcttttttccagggtttattctacttaaagtcttaaaatataaaaaacaatgcacaaaaaaggccatggtattacatgagaaaactaaaatccaaatgtttgcaatcaaatacaaaagatacctgactacaaatcacaaaattccatttcaagccatcttgatggcactctaaatggctgttgaataaagtttaaatacctttataaaactagcaaagatgttaaaagctctagggtgaacgtgcattgaattgaagaactctaatgggcttttttccttcacagaaaactcttctgcctcacaagtagcataatggatttaaagcaagttacatacacttgacaaacagctatttctagatatggttgttgtacaagatgatgtggtttaaaagcccatcctccattaaaaggaagtcctggacaacctcttttagacactaaacatgcaaactcgtgcttgaggggcaaatgagccagtcactgggctggggcccagctcagccatcattaagcattagaatatagagaaactgccattattcatgtcctcttcactgtcacttgctcttgccagactgtcgaaagggtggttgaagtgttcttgctggtcagaagaaactgctccaaagaacatgcaagaaaactttctgagacacagagaccctggcacttcctctgtgttgctgacactgctttctgatacttcactgacatctccatccactcttttcattgcagggctgccacagttttccaatgcagatatgtttgtgagagtctccttaggataaagccttcttggtgctgctttttttgaaatacattccagggcctggccagttacatttttgccagcctttttttcaatcagatctgacctttttcgtttctgtgaaagacacagtgactgtggtgaagatgctctactttgttcatcagctaatgtggccaaaataaagttagcttccactaacatatcatcaatactcaaagccagaggtttcccagggaaatcaaaataaatggatataggagcatgtgtagcttctgaaaatgtcagtattcccttcaattctttgaaacaaaatgttatctcagtgtccattccaatttgaaagaagtcaaactcatctgagccaacaaacatctcactgtgtacagcattgctcaaatccattgattcctcattagaactcttgaggcaaaaattcagtggagtaacagcaagagtaacttcctcttgacttgatgtaaaaagaacaatggcatcagcaagcaatcttggttgaatcattagcgtattagtacaaacattcttgtcaaaaataacttgcaaaggctgactttcttgaaaacatatattatgagttcttttaataccatgtctgtagaagaattgaataactactttgcatttatcagatctggtgaatattctgcacttctctatatttctttcaagggaattcagacatctaaagatgggcaaaattgacttcattcccaatttgcattttaaatgcagtgttgtgtcaagttcattttcactcattttcactaaagctgaccattgataatgctgaaaaaacacaggagagaacaggacacatccatatgctgaccgagaagaattcacacatcttagagcaagaccttttttagatgggtctagccagaactcgtcactaattcgtgatagagcttgaactgctttcccaaatactattaacgtctgcttttctctctgctaaatgggaagacaacaaaggccgctccacctttcacctgactgccgctcatcacgcacttcagcatggctgccatccgccctaaaaagcaggctcggaaggcgcgcctcagctcgacggcccaggtgcccggatgttgcccgcgcttttcaaagcttcgcga

SEQ ID NO: 14877 - RNA, 3093 nt, Homo sapiens
  source 1..3093: mol_type = other RNA
gctgggattacaggcatgagccactacaccccgccagtattaactataataatagtccaatgctgcatccaggctattactgatgatgatgcctttaagacctaaacccctctgcctacttcaatgaatgaaccagaaatgttatcctcagcaaagagacctacagagttacttttgtgtataaaagctccctgtgtaggcatctgcatttgttagaaataccagaaattcagtgttaatcatcagtgtaagcataagatacatatatcttcccctaccatgtgatgaaaggacttagttgaaattatgtgggcattgccagttaccacaaaaagcttggttaaggcccattttcattcactaaggaacatcttgggatgaacttgagtttttattaggttattgtgggtagctatgactcattactaagctacaagagccaaattaattctggtttcagttagaactctattcacagttctaaagcatgcaaatccactcagccacctttatgaatttctcacaaagtctaaagtacaactgcttgccagttaacacttccttacggtttgaaggtttcagaaagatgtaacaataatatgttacaaaagtctcgtttgtcaggttataattgactgtaaacaggtttgggggagggagaggcacacatcataagacattacataacaatgttttgtgccagattttttagtccatttgtgcaggtaaaaagctaactcttaaagggccaaagaacagagacatttgtcttccaccttattccactccaaactcaggctgtcttggcagtggaggatactgttctatgtcagataatacagaaatatttggcatcacttccattaaattctttcctgcagcacactgcaaaataaaaaatcacatctgaaaatcagaacaatttgaggttaggaaataaaattttacaatatgtaaaaacactccaggttgggcgcagtggctcaagtctgtaatcccagcactttgggaggccgaggtgggcagatcacttgaggccaggagttcaagaccaccctggccaacatggcgaaaccctgtctctacaaaataccagaaattagccaggcatggtggcacgcacctgcaatcccagctgcacgggaggctgaggcaggagaatcgcttggacctgggaggcagatgttgcagtgagcagagattgcaccactgcacttgagcctgagtgacaaagtgagactccgtctaaaaaagccaagtgaaagtgactatatatttttactcttgatcttttttccagggtttattctacttaaagtcttaaaatataaaaaacaatgcacaaaaaaggccatggtattacatgagaaaactaaaatccaaatgtttgcaatcaaatacaaaagatacctgactacaaatcacaaaattccatttcaagccatcttgatggcactctaaatggctgttgaataaagtttaaatacctttataaaactagcaaagatgttaaaagctctagggtgaacgtgcattgaattgaagaactctaatgggcttttttccttcacagaaaactcttctgcctcacaagtagcataatggatttaaagcaagttacatacacttgacaaacagctatttctagatatggttgttgtacaagatgatgtggtttaaaagcccatcctccattaaaaggaagtcctggacaacctcttttagacactaaacatgcaaactcgtgcttgaggggcaaatgagccagtcactgggctggggcccagctcagccatcattaagcattagaatatagagaaactgccattattcatgtcctcttcactgtcacttgctcttgccagactgtcgaaagggtggttgaagtgttcttgctggtcagaagaaactgctccaaagaacatgcaagaaaactttctgagacacagagaccctggcacttcctctgtgttgctgacactgctttctgatacttcactgacatctccatccactcttttcattgcagggctgccacagttttccaatgcagatatgtttgtgagagtctccttaggataaagccttcttggtgctgctttttttgaaatacattccagggcctggccagttacatttttgccagcctttttttcaatcagatctgacctttttcgtttctgtgaaagacacagtgactgtggtgaagatgctctactttgttcatcagctaatgtggccaaaataaagttagcttccactaacatatcatcaatactcaaagccagaggtttcccagggaaatcaaaataaatggatataggagcatgtgtagcttctgaaaatgtcagtattcccttcaattctttgaaacaaaatgttatctcagtgtccattccaatttgaaagaagtcaaactcatctgagccaacaaacatctcactgtgtacagcattgctcaaatccattgattcctcattagaactcttgaggcaaaaattcagtggagtaacagcaagagtaacttcctcttgacttgatgtaaaaagaacaatggcatcagcaagcaatcttggttgaatcattagcgtattagtacaaacattcttgtcaaaaataacttgcaaaggctgactttcttgaaaacatatattatgagttcttttaataccatgtctgtagaagaattgaataactactttgcatttatcagatctggtgaatattctgcacttctctatatttctttcaagggaattcagacatctaaagatgggcaaaattgacttcattcccaatttgcattttaaatgcagtgttgtgtcaagttcattttcactcattttcactaaagctgaccattgataatgctgaaaaaacacaggagagaacaggacacatccatatgctgaccgagaagaattcacacatcttagagcaagaccttttttagatgggtctagccagaactcgtcactaattcgtgatagagcttgaactgctttcccaaatactcgaatgttccggggataggggcacggtcctccgtttccagacggttcctactcgtttcccgcaaaaagcacctcccgc

SEQ ID NO: 14878 - RNA, 3059 nt, Homo sapiens
  source 1..3059: mol_type = other RNA
gctgggattacaggcatgagccactacaccccgccagtattaactataataatagtccaatgctgcatccaggctattactgatgatgatgcctttaagacctaaacccctctgcctacttcaatgaatgaaccagaaatgttatcctcagcaaagagacctacagagttacttttgtgtataaaagctccctgtgtaggcatctgcatttgttagaaataccagaaattcagtgttaatcatcagtgtaagcataagatacatatatcttcccctaccatgtgatgaaaggacttagttgaaattatgtgggcattgccagttaccacaaaaagcttggttaaggcccattttcattcactaaggaacatcttgggatgaacttgagtttttattaggttattgtgggtagctatgactcattactaagctacaagagccaaattaattctggtttcagttagaactctattcacagttctaaagcatgcaaatccactcagccacctttatgaatttctcacaaagtctaaagtacaactgcttgccagttaacacttccttacggtttgaaggtttcagaaagatgtaacaataatatgttacaaaagtctcgtttgtcaggttataattgactgtaaacaggtttgggggagggagaggcacacatcataagacattacataacaatgttttgtgccagattttttagtccatttgtgcaggtaaaaagctaactcttaaagggccaaagaacagagacatttgtcttccaccttattccactccaaactcaggctgtcttggcagtggaggatactgttctatgtcagataatacagaaatatttggcatcacttccattaaattctttcctgcagcacactgcaaaataaaaaatcacatctgaaaatcagaacaatttgaggttaggaaataaaattttacaatatgtaaaaacactccaggttgggcgcagtggctcaagtctgtaatcccagcactttgggaggccgaggtgggcagatcacttgaggccaggagttcaagaccaccctggccaacatggcgaaaccctgtctctacaaaataccagaaattagccaggcatggtggcacgcacctgcaatcccagctgcacgggaggctgaggcaggagaatcgcttggacctgggaggcagatgttgcagtgagcagagattgcaccactgcacttgagcctgagtgacaaagtgagactccgtctaaaaaagccaagtgaaagtgactatatatttttactcttgatcttttttccagggtttattctacttaaagtcttaaaatataaaaaacaatgcacaaaaaaggccatggtattacatgagaaaactaaaatccaaatgtttgcaatcaaatacaaaagatacctgactacaaatcacaaaattccatttcaagccatcttgatggcactctaaatggctgttgaataaagtttaaatacctttataaaactagcaaagatgttaaaagctctagggtgaacgtgcattgaattgaagaactctaatgggcttttttccttcacagaaaactcttctgcctcacaagtagcataatggatttaaagcaagttacatacacttgacaaacagctatttctagatatggttgttgtacaagatgatgtggtttaaaagcccatcctccattaaaaggaagtcctggacaacctcttttagacactaaacatgcaaactcgtgcttgaggggcaaatgagccagtcactgggctggggcccagctcagccatcattaagcattagaatatagagaaactgccattattcatgtcctcttcactgtcacttgctcttgccagactgtcgaaagggtggttgaagtgttcttgctggtcagaagaaactgctccaaagaacatgcaagaaaactttctgagacacagagaccctggcacttcctctgtgttgctgacactgctttctgatacttcactgacatctccatccactcttttcattgcagggctgccacagttttccaatgcagatatgtttgtgagagtctccttaggataaagccttcttggtgctgctttttttgaaatacattccagggcctggccagttacatttttgccagcctttttttcaatcagatctgacctttttcgtttctgtgaaagacacagtgactgtggtgaagatgctctactttgttcatcagctaatgtggccaaaataaagttagcttccactaacatatcatcaatactcaaagccagaggtttcccagggaaatcaaaataaatggatataggagcatgtgtagcttctgaaaatgtcagtattcccttcaattctttgaaacaaaatgttatctcagtgtccattccaatttgaaagaagtcaaactcatctgagccaacaaacatctcactgtgtacagcattgctcaaatccattgattcctcattagaactcttgaggcaaaaattcagtggagtaacagcaagagtaacttcctcttgacttgatgtaaaaagaacaatggcatcagcaagcaatcttggttgaatcattagcgtattagtacaaacattcttgtcaaaaataacttgcaaaggctgactttcttgaaaacatatattatgagttcttttaataccatgtctgtagaagaattgaataactactttgcatttatcagatctggtgaatattctgcacttctctatatttctttcaagggaattcagacatctaaagatgggcaaaattgacttcattcccaatttgcattttaaatgcagtgttgtgtcaagttcattttcactcattttcactaaagctgaccattgataatgctgaaaaaacacaggagagaacaggacacatccatatgctgaccgagaagaattcacacatcttagagcaagaccttttttagatgggtctagccagaactcgtcactaattcgtgatagagcttgaactgctttcccaaatactgactgccgctcatcacgcacttcagcatggctgccatccgccct

SEQ ID NO: 14879 - RNA, 3066 nt, Homo sapiens
  source 1..3066: mol_type = other RNA
gctgggattacaggcatgagccactacaccccgccagtattaactataataatagtccaatgctgcatccaggctattactgatgatgatgcctttaagacctaaacccctctgcctacttcaatgaatgaaccagaaatgttatcctcagcaaagagacctacagagttacttttgtgtataaaagctccctgtgtaggcatctgcatttgttagaaataccagaaattcagtgttaatcatcagtgtaagcataagatacatatatcttcccctaccatgtgatgaaaggacttagttgaaattatgtgggcattgccagttaccacaaaaagcttggttaaggcccattttcattcactaaggaacatcttgggatgaacttgagtttttattaggttattgtgggtagctatgactcattactaagctacaagagccaaattaattctggtttcagttagaactctattcacagttctaaagcatgcaaatccactcagccacctttatgaatttctcacaaagtctaaagtacaactgcttgccagttaacacttccttacggtttgaaggtttcagaaagatgtaacaataatatgttacaaaagtctcgtttgtcaggttataattgactgtaaacaggtttgggggagggagaggcacacatcataagacattacataacaatgttttgtgccagattttttagtccatttgtgcaggtaaaaagctaactcttaaagggccaaagaacagagacatttgtcttccaccttattccactccaaactcaggctgtcttggcagtggaggatactgttctatgtcagataatacagaaatatttggcatcacttccattaaattctttcctgcagcacactgcaaaataaaaaatcacatctgaaaatcagaacaatttgaggttaggaaataaaattttacaatatgtaaaaacactccaggttgggcgcagtggctcaagtctgtaatcccagcactttgggaggccgaggtgggcagatcacttgaggccaggagttcaagaccaccctggccaacatggcgaaaccctgtctctacaaaataccagaaattagccaggcatggtggcacgcacctgcaatcccagctgcacgggaggctgaggcaggagaatcgcttggacctgggaggcagatgttgcagtgagcagagattgcaccactgcacttgagcctgagtgacaaagtgagactccgtctaaaaaagccaagtgaaagtgactatatatttttactcttgatcttttttccagggtttattctacttaaagtcttaaaatataaaaaacaatgcacaaaaaaggccatggtattacatgagaaaactaaaatccaaatgtttgcaatcaaatacaaaagatacctgactacaaatcacaaaattccatttcaagccatcttgatggcactctaaatggctgttgaataaagtttaaatacctttataaaactagcaaagatgttaaaagctctagggtgaacgtgcattgaattgaagaactctaatgggcttttttccttcacagaaaactcttctgcctcacaagtagcataatggatttaaagcaagttacatacacttgacaaacagctatttctagatatggttgttgtacaagatgatgtggtttaaaagcccatcctccattaaaaggaagtcctggacaacctcttttagacactaaacatgcaaactcgtgcttgaggggcaaatgagccagtcactgggctggggcccagctcagccatcattaagcattagaatatagagaaactgccattattcatgtcctcttcactgtcacttgctcttgccagactgtcgaaagggtggttgaagtgttcttgctggtcagaagaaactgctccaaagaacatgcaagaaaactttctgagacacagagaccctggcacttcctctgtgttgctgacactgctttctgatacttcactgacatctccatccactcttttcattgcagggctgccacagttttccaatgcagatatgtttgtgagagtctccttaggataaagccttcttggtgctgctttttttgaaatacattccagggcctggccagttacatttttgccagcctttttttcaatcagatctgacctttttcgtttctgtgaaagacacagtgactgtggtgaagatgctctactttgttcatcagctaatgtggccaaaataaagttagcttccactaacatatcatcaatactcaaagccagaggtttcccagggaaatcaaaataaatggatataggagcatgtgtagcttctgaaaatgtcagtattcccttcaattctttgaaacaaaatgttatctcagtgtccattccaatttgaaagaagtcaaactcatctgagccaacaaacatctcactgtgtacagcattgctcaaatccattgattcctcattagaactcttgaggcaaaaattcagtggagtaacagcaagagtaacttcctcttgacttgatgtaaaaagaacaatggcatcagcaagcaatcttggttgaatcattagcgtattagtacaaacattcttgtcaaaaataacttgcaaaggctgactttcttgaaaacatatattatgagttcttttaataccatgtctgtagaagaattgaataactactttgcatttatcagatctggtgaatattctgcacttctctatatttctttcaagggaattcagacatctaaagatgggcaaaattgacttcattcccaatttgcattttaaatgcagtgttgtgtcaagttcattttcactcattttcactaaagctgaccattgataatgctgaaaaaacacaggagagaacaggacacatccatatgctgaccgagaagaattcacacatcttagagcaagaccttttttagatgggtctagccagaactcgtcactaattcgtgatagagcttgaactgctttcccaaatactttcacctgactgccgctcatcacgcacttcagcatggctgccatccgccct

SEQ ID NO: 14880 - RNA, 3037 nt, Homo sapiens
  source 1..3037: mol_type = other RNA
gctgggattacaggcatgagccactacaccccgccagtattaactataataatagtccaatgctgcatccaggctattactgatgatgatgcctttaagacctaaacccctctgcctacttcaatgaatgaaccagaaatgttatcctcagcaaagagacctacagagttacttttgtgtataaaagctccctgtgtaggcatctgcatttgttagaaataccagaaattcagtgttaatcatcagtgtaagcataagatacatatatcttcccctaccatgtgatgaaaggacttagttgaaattatgtgggcattgccagttaccacaaaaagcttggttaaggcccattttcattcactaaggaacatcttgggatgaacttgagtttttattaggttattgtgggtagctatgactcattactaagctacaagagccaaattaattctggtttcagttagaactctattcacagttctaaagcatgcaaatccactcagccacctttatgaatttctcacaaagtctaaagtacaactgcttgccagttaacacttccttacggtttgaaggtttcagaaagatgtaacaataatatgttacaaaagtctcgtttgtcaggttataattgactgtaaacaggtttgggggagggagaggcacacatcataagacattacataacaatgttttgtgccagattttttagtccatttgtgcaggtaaaaagctaactcttaaagggccaaagaacagagacatttgtcttccaccttattccactccaaactcaggctgtcttggcagtggaggatactgttctatgtcagataatacagaaatatttggcatcacttccattaaattctttcctgcagcacactgcaaaataaaaaatcacatctgaaaatcagaacaatttgaggttaggaaataaaattttacaatatgtaaaaacactccaggttgggcgcagtggctcaagtctgtaatcccagcactttgggaggccgaggtgggcagatcacttgaggccaggagttcaagaccaccctggccaacatggcgaaaccctgtctctacaaaataccagaaattagccaggcatggtggcacgcacctgcaatcccagctgcacgggaggctgaggcaggagaatcgcttggacctgggaggcagatgttgcagtgagcagagattgcaccactgcacttgagcctgagtgacaaagtgagactccgtctaaaaaagccaagtgaaagtgactatatatttttactcttgatcttttttccagggtttattctacttaaagtcttaaaatataaaaaacaatgcacaaaaaaggccatggtattacatgagaaaactaaaatccaaatgtttgcaatcaaatacaaaagatacctgactacaaatcacaaaattccatttcaagccatcttgatggcactctaaatggctgttgaataaagtttaaatacctttataaaactagcaaagatgttaaaagctctagggtgaacgtgcattgaattgaagaactctaatgggcttttttccttcacagaaaactcttctgcctcacaagtagcataatggatttaaagcaagttacatacacttgacaaacagctatttctagatatggttgttgtacaagatgatgtggtttaaaagcccatcctccattaaaaggaagtcctggacaacctcttttagacactaaacatgcaaactcgtgcttgaggggcaaatgagccagtcactgggctggggcccagctcagccatcattaagcattagaatatagagaaactgccattattcatgtcctcttcactgtcacttgctcttgccagactgtcgaaagggtggttgaagtgttcttgctggtcagaagaaactgctccaaagaacatgcaagaaaactttctgagacacagagaccctggcacttcctctgtgttgctgacactgctttctgatacttcactgacatctccatccactcttttcattgcagggctgccacagttttccaatgcagatatgtttgtgagagtctccttaggataaagccttcttggtgctgctttttttgaaatacattccagggcctggccagttacatttttgccagcctttttttcaatcagatctgacctttttcgtttctgtgaaagacacagtgactgtggtgaagatgctctactttgttcatcagctaatgtggccaaaataaagttagcttccactaacatatcatcaatactcaaagccagaggtttcccagggaaatcaaaataaatggatataggagcatgtgtagcttctgaaaatgtcagtattcccttcaattctttgaaacaaaatgttatctcagtgtccattccaatttgaaagaagtcaaactcatctgagccaacaaacatctcactgtgtacagcattgctcaaatccattgattcctcattagaactcttgaggcaaaaattcagtggagtaacagcaagagtaacttcctcttgacttgatgtaaaaagaacaatggcatcagcaagcaatcttggttgaatcattagcgtattagtacaaacattcttgtcaaaaataacttgcaaaggctgactttcttgaaaacatatattatgagttcttttaataccatgtctgtagaagaattgaataactactttgcatttatcagatctggtgaatattctgcacttctctatatttctttcaagggaattcagacatctaaagatgggcaaaattgacttcattcccaatttgcattttaaatgcagtgttgtgtcaagttcattttcactcattttcactaaagctgaccattgataatgctgaaaaaacacaggagagaacaggacacatccatatgctgaccgagaagaattcacacatcttagagcaagaccttttttagatgggtctagccagaactcgtcactaattcgtgatagagcttgaactgctttcccaaatattcagcatggctgccatccgccct

SEQ ID NO: 14881 - RNA, 2995 nt, Homo sapiens
  source 1..2995: mol_type = other RNA
gctgggattacaggcatgagccactacaccccgccagtattaactataataatagtccaatgctgcatccaggctattactgatgatgatgcctttaagacctaaacccctctgcctacttcaatgaatgaaccagaaatgttatcctcagcaaagagacctacagagttacttttgtgtataaaagctccctgtgtaggcatctgcatttgttagaaataccagaaattcagtgttaatcatcagtgtaagcataagatacatatatcttcccctaccatgtgatgaaaggacttagttgaaattatgtgggcattgccagttaccacaaaaagcttggttaaggcccattttcattcactaaggaacatcttgggatgaacttgagtttttattaggttattgtgggtagctatgactcattactaagctacaagagccaaattaattctggtttcagttagaactctattcacagttctaaagcatgcaaatccactcagccacctttatgaatttctcacaaagtctaaagtacaactgcttgccagttaacacttccttacggtttgaaggtttcagaaagatgtaacaataatatgttacaaaagtctcgtttgtcaggttataattgactgtaaacaggtttgggggagggagaggcacacatcataagacattacataacaatgttttgtgccagattttttagtccatttgtgcaggtaaaaagctaactcttaaagggccaaagaacagagacatttgtcttccaccttattccactccaaactcaggctgtcttggcagtggaggatactgttctatgtcagataatacagaaatatttggcatcacttccattaaattctttcctgcagcacactgcaaaataaaaaatcacatctgaaaatcagaacaatttgaggttaggaaataaaattttacaatatgtaaaaacactccaggttgggcgcagtggctcaagtctgtaatcccagcactttgggaggccgaggtgggcagatcacttgaggccaggagttcaagaccaccctggccaacatggcgaaaccctgtctctacaaaataccagaaattagccaggcatggtggcacgcacctgcaatcccagctgcacgggaggctgaggcaggagaatcgcttggacctgggaggcagatgttgcagtgagcagagattgcaccactgcacttgagcctgagtgacaaagtgagactccgtctaaaaaagccaagtgaaagtgactatatatttttactcttgatcttttttccagggtttattctacttaaagtcttaaaatataaaaaacaatgcacaaaaaaggccatggtattacatgagaaaactaaaatccaaatgtttgcaatcaaatacaaaagatacctgactacaaatcacaaaattccatttcaagccatcttgatggcactctaaatggctgttgaataaagtttaaatacctttataaaactagcaaagatgttaaaagctctagggtgaacgtgcattgaattgaagaactctaatgggcttttttccttcacagaaaactcttctgcctcacaagtagcataatggatttaaagcaagttacatacacttgacaaacagctatttctagatatggttgttgtacaagatgatgtggtttaaaagcccatcctccattaaaaggaagtcctggacaacctcttttagacactaaacatgcaaactcgtgcttgaggggcaaatgagccagtcactgggctggggcccagctcagccatcattaagcattagaatatagagaaactgccattattcatgtcctcttcactgtcacttgctcttgccagactgtcgaaagggtggttgaagtgttcttgctggtcagaagaaactgctccaaagaacatgcaagaaaactttctgagacacagagaccctggcacttcctctgtgttgctgacactgctttctgatacttcactgacatctccatccactcttttcattgcagggctgccacagttttccaatgcagatatgtttgtgagagtctccttaggataaagccttcttggtgctgctttttttgaaatacattccagggcctggccagttacatttttgccagcctttttttcaatcagatctgacctttttcgtttctgtgaaagacacagtgactgtggtgaagatgctctactttgttcatcagctaatgtggccaaaataaagttagcttccactaacatatcatcaatactcaaagccagaggtttcccagggaaatcaaaataaatggatataggagcatgtgtagcttctgaaaatgtcagtattcccttcaattctttgaaacaaaatgttatctcagtgtccattccaatttgaaagaagtcaaactcatctgagccaacaaacatctcactgtgtacagcattgctcaaatccattgattcctcattagaactcttgaggcaaaaattcagtggagtaacagcaagagtaacttcctcttgacttgatgtaaaaagaacaatggcatcagcaagcaatcttggttgaatcattagcgtattagtacaaacattcttgtcaaaaataacttgcaaaggctgactttcttgaaaacatatattatgagttcttttaataccatgtctgtagaagaattgaataactactttgcatttatcagatctggtgaatattctgcacttctctatatttctttcaagggaattcagacatctaaagatgggcaaaattgacttcattcccaatttgcattttaaatgcagtgttgtgtcaagttcattttcactcattttcactaaagctgaccattgataatgctgaaaaaacacaggagagaacaggacacatccatatgctgaccgagaagaattcacacatcttagagcaagctttcacctgactgccgctcatcacgcacttcagcatggctgccatccgccct

SEQ ID NO: 14882 - RNA, 3278 nt, Homo sapiens
  source 1..3278: mol_type = other RNA
gctgggattacaggcatgagccactacaccccgccagtattaactataataatagtccaatgctgcatccaggctattactgatgatgatgcctttaagacctaaacccctctgcctacttcaatgaatgaaccagaaatgttatcctcagcaaagagacctacagagttacttttgtgtataaaagctccctgtgtaggcatctgcatttgttagaaataccagaaattcagtgttaatcatcagtgtaagcataagatacatatatcttcccctaccatgtgatgaaaggacttagttgaaattatgtgggcattgccagttaccacaaaaagcttggttaaggcccattttcattcactaaggaacatcttgggatgaacttgagtttttattaggttattgtgggtagctatgactcattactaagctacaagagccaaattaattctggtttcagttagaactctattcacagttctaaagcatgcaaatccactcagccacctttatgaatttctcacaaagtctaaagtacaactgcttgccagttaacacttccttacggtttgaaggtttcagaaagatgtaacaataatatgttacaaaagtctcgtttgtcaggttataattgactgtaaacaggtttgggggagggagaggcacacatcataagacattacataacaatgttttgtgccagattttttagtccatttgtgcaggtaaaaagctaactcttaaagggccaaagaacagagacatttgtcttccaccttattccactccaaactcaggctgtcttggcagtggaggatactgttctatgtcagataatacagaaatatttggcatcacttccattaaattctttcctgcagcacactgcaaaataaaaaatcacatctgaaaatcagaacaatttgaggttaggaaataaaattttacaatatgtaaaaacactccaggttgggcgcagtggctcaagtctgtaatcccagcactttgggaggccgaggtgggcagatcacttgaggccaggagttcaagaccaccctggccaacatggcgaaaccctgtctctacaaaataccagaaattagccaggcatggtggcacgcacctgcaatcccagctgcacgggaggctgaggcaggagaatcgcttggacctgggaggcagatgttgcagtgagcagagattgcaccactgcacttgagcctgagtgacaaagtgagactccgtctaaaaaagccaagtgaaagtgactatatatttttactcttgatcttttttccagggtttattctacttaaagtcttaaaatataaaaaacaatgcacaaaaaaggccatggtattacatgagaaaactaaaatccaaatgtttgcaatcaaatacaaaagatacctgactacaaatcacaaaattccatttcaagccatcttgatggcactctaaatggctgttgaataaagtttaaatacctttataaaactagcaaagatgttaaaagctctagggtgaacgtgcattgaattgaagaactctaatgggcttttttccttcacagaaaactcttctgcctcacaagtagcataatggatttaaagcaagttacatacacttgacaaacagctatttctagatatggttgttgtacaagatgatgtggtttaaaagcccatcctccattaaaaggaagtcctggacaacctcttttagacactaaacatgcaaactcgtgcttgaggggcaaatgagccagtcactgggctggggcccagctcagccatcattaagcattagaatatagagaaactgccattattcatgtcctcttcactgtcacttgctcttgccagactgtcgaaagggtggttgaagtgttcttgctggtcagaagaaactgctccaaagaacatgcaagaaaactttctgagacacagagaccctggcacttcctctgtgttgctgacactgctttctgatacttcactgacatctccatccactcttttcattgcagggctgccacagttttccaatgcagatatgtttgtgagagtctccttaggataaagccttcttggtgctgctttttttgaaatacattccagggcctggccagttacatttttgccagcctttttttcaatcagatctgacctttttcgtttctgtgaaagacacagtgactgtggtgaagatgctctactttgttcatcagctaatgtggccaaaataaagttagcttccactaacatatcatcaatactcaaagccagaggtttcccagggaaatcaaaataaatggatataggagcatgtgtagcttctgaaaatgtcagtattcccttcaattctttgaaacaaaatgttatctcagtgtccattccaatttgaaagaagtcaaactcatctgagccaacaaacatctcactgtgtacagcattgctcaaatccattgattcctcattagaactcttgaggcaaaaattcagtggagtaacagcaagagtaacttcctcttgacttgatgtaaaaagaacaatggcatcagcaagcaatcttggttgaatcattagcgtattagtacaaacattcttgtcaaaaataacttgcaaaggctgactttcttgaaaacatatattatgagttcttttaatacccacacaccattaccagcctctggtatctaccattctactctctacctccatgagatcaactttttagcgtccacattgtgagaacatgcaatacttgactttccatgcctggcttatttcacttaacatagtgacctctagttccatccacgttgcatgtctgtagaagaattgaataactactttgcatttatcagatctggtgaatattctgcacttctctatatttctttcaagggaattcagacatctaaagatgggcaaaattgacttcattcccaatttgcattttaaatgcagtgttgtgtcaagttcattttcactcattttcactaaagctgaccattgataatgctgaaaaaacacaggagagaacaggacacatccatatgctgaccgagaagaattcacacatcttagagcaagaccttttttagatgggtctagccagaactcgtcactaattcgtgatagagcttgaactgctttcccaaatactattaacgtctgcttttctctctgctaaatgggaagacaacaaaggccgctccacctttcacctgactgccgctcatcacgcacttcagcatggctgccatccgccct

SEQ ID NO: 14883 - RNA, 3215 nt, Homo sapiens
  source 1..3215: mol_type = other RNA
gctgggattacaggcatgagccactacaccccgccagtattaactataataatagtccaatgctgcatccaggctattactgatgatgatgcctttaagacctaaacccctctgcctacttcaatgaatgaaccagaaatgttatcctcagcaaagagacctacagagttacttttgtgtataaaagctccctgtgtaggcatctgcatttgttagaaataccagaaattcagtgttaatcatcagtgtaagcataagatacatatatcttcccctaccatgtgatgaaaggacttagttgaaattatgtgggcattgccagttaccacaaaaagcttggttaaggcccattttcattcactaaggaacatcttgggatgaacttgagtttttattaggttattgtgggtagctatgactcattactaagctacaagagccaaattaattctggtttcagttagaactctattcacagttctaaagcatgcaaatccactcagccacctttatgaatttctcacaaagtctaaagtacaactgcttgccagttaacacttccttacggtttgaaggtttcagaaagatgtaacaataatatgttacaaaagtctcgtttgtcaggttataattgactgtaaacaggtttgggggagggagaggcacacatcataagacattacataacaatgttttgtgccagattttttagtccatttgtgcaggtaaaaagctaactcttaaagggccaaagaacagagacatttgtcttccaccttattccactccaaactcaggctgtcttggcagtggaggatactgttctatgtcagataatacagaaatatttggcatcacttccattaaattctttcctgcagcacactgcaaaataaaaaatcacatctgaaaatcagaacaatttgaggttaggaaataaaattttacaatatgtaaaaacactccaggttgggcgcagtggctcaagtctgtaatcccagcactttgggaggccgaggtgggcagatcacttgaggccaggagttcaagaccaccctggccaacatggcgaaaccctgtctctacaaaataccagaaattagccaggcatggtggcacgcacctgcaatcccagctgcacgggaggctgaggcaggagaatcgcttggacctgggaggcagatgttgcagtgagcagagattgcaccactgcacttgagcctgagtgacaaagtgagactccgtctaaaaaagccaagtgaaagtgactatatatttttactcttgatcttttttccagggtttattctacttaaagtcttaaaatataaaaaacaatgcacaaaaaaggccatggtattacatgagaaaactaaaatccaaatgtttgcaatcaaatacaaaagatacctgactacaaatcacaaaattccatttcaagccatcttgatggcactctaaatggctgttgaataaagtttaaatacctttataaaactagcaaagatgttaaaagctctagggtgaacgtgcattgaattgaagaactctaatgggcttttttccttcacagaaaactcttctgcctcacaagtagcataatggatttaaagcaagttacatacacttgacaaacagctatttctagatatggttgttgtacaagatgatgtggtttaaaagcccatcctccattaaaaggaagtcctggacaacctcttttagacactaaacatgcaaactcgtgcttgaggggcaaatgagccagtcactgggctggggcccagctcagccatcattaagcattagaatatagagaaactgccattattcatgtcctcttcactgtcacttgctcttgccagactgtcgaaagggtggttgaagtgttcttgctggtcagaagaaactgctccaaagaacatgcaagaaaactttctgagacacagagaccctggcacttcctctgtgttgctgacactgctttctgatacttcactgacatctccatccactcttttcattgcagggctgccacagttttccaatgcagatatgtttgtgagagtctccttaggataaagccttcttggtgctgctttttttgaaatacattccagggcctggccagttacatttttgccagcctttttttcaatcagatctgacctttttcgtttctgtgaaagacacagtgactgtggtgaagatgctctactttgttcatcagctaatgtggccaaaataaagttagcttccactaacatatcatcaatactcaaagccagaggtttcccagggaaatcaaaataaatggatataggagcatgtgtagcttctgaaaatgtcagtattcccttcaattctttgaaacaaaatgttatctcagtgtccattccaatttgaaagaagtcaaactcatctgagccaacaaacatctcactgtgtacagcattgctcaaatccattgattcctcattagaactcttgaggcaaaaattcagtggagtaacagcaagagtaacttcctcttgacttgatgtaaaaagaacaatggcatcagcaagcaatcttggttgaatcattagcgtattagtacaaacattcttgtcaaaaataacttgcaaaggctgactttcttgaaaacatatattatgagttcttttaatacccacacaccattaccagcctctggtatctaccattctactctctacctccatgagatcaactttttagcgtccacattgtgagaacatgcaatacttgactttccatgcctggcttatttcacttaacatagtgacctctagttccatccacgttgcatgtctgtagaagaattgaataactactttgcatttatcagatctggtgaatattctgcacttctctatatttctttcaagggaattcagacatctaaagatgggcaaaattgacttcattcccaatttgcattttaaatgcagtgttgtgtcaagttcattttcactcattttcactaaagctgaccattgataatgctgaaaaaacacaggagagaacaggacacatccatatgctgaccgagaagaattcacacatcttagagcaagaccttttttagatgggtctagccagaactcgtcactaattcgtgatagagcttgaactgctttcccaaatactgactgccgctcatcacgcacttcagcatggctgccatccgccct

SEQ ID NO: 14884 - RNA, 2624 nt, Homo sapiens
  source 1..2624: mol_type = other RNA
gctgggattacaggcatgagccactacaccccgccagtattaactataataatagtccaatgctgcatccaggctattactgatgatgatgcctttaagacctaaacccctctgcctacttcaatgaatgaaccagaaatgttatcctcagcaaagagacctacagagttacttttgtgtataaaagctccctgtgtaggcatctgcatttgttagaaataccagaaattcagtgttaatcatcagtgtaagcataagatacatatatcttcccctaccatgtgatgaaaggacttagttgaaattatgtgggcattgccagttaccacaaaaagcttggttaaggcccattttcattcactaaggaacatcttgggatgaacttgagtttttattaggttattgtgggtagctatgactcattactaagctacaagagccaaattaattctggtttcagttagaactctattcacagttctaaagcatgcaaatccactcagccacctttatgaatttctcacaaagtctaaagtacaactgcttgccagttaacacttccttacggtttgaaggtttcagaaagatgtaacaataatatgttacaaaagtctcgtttgtcaggttataattgactgtaaacaggtttgggggagggagaggcacacatcataagacattacataacaatgttttgtgccagattttttagtccatttgtgcaggtaaaaagctaactcttaaagggccaaagaacagagacatttgtcttccaccttattccactccaaactcaggctgtcttggcagtggaggatactgttctatgtcagataatacagaaatatttggcatcacttccattaaattctttcctgcagcacactgcaaaataaaaaatcacatctgaaaatcagaacaatttgaggttaggaaataaaattttacaatatgtaaaaacactccaggttgggcgcagtggctcaagtctgtaatcccagcactttgggaggccgaggtgggcagatcacttgaggccaggagttcaagaccaccctggccaacatggcgaaaccctgtctctacaaaataccagaaattagccaggcatggtggcacgcacctgcaatcccagctgcacgggaggctgaggcaggagaatcgcttggacctgggaggcagatgttgcagtgagcagagattgcaccactgcacttgagcctgagtgacaaagtgagactccgtctaaaaaagccaagtgaaagtgactatatatttttactcttgatcttttttccagggtttattctacttaaagtcttaaaatataaaaaacaatgcacaaaaaaggccatggtattacatgagaaaactaaaatccaaatgtttgcaatcaaatacaaaagatacctgactacaaatcacaaaattccatttcaagccatcttgatggcactctaaatggctgttgaataaagtttaaatacctttataaaactagcaaagatgttaaaagctctagggtgaacgtgcattgaattgaagaactctaatgggcttttttccttcacagaaaactcttctgcctcacaagtagcataatggatttaaagcaagttacatacacttgacaaacagctatttctagatatggttgttgtacaagatgatgtggtttaaaagcccatcctccattaaaaggaagtcctggacaacctcttttagacactaaacatgcaaactcgtgcttgaggggcaaatgagccagtcactgggctggggcccagctcagccatcattaagcattagaatatagagaaactgccattattcatgtcctcttcactgtcacttgctcttgccagactgtcgaaagggtggttgaagtgttcttgctggtcagaagaaactgctccaaagaacatgcaagaaaactttctgagacacagagaccctggcacttcctctgtgttgctgacactgctttctgatacttcactgacatctccatccactcttttcattgcagggctgccacagttttccaatgcagatatgtttgtgagagtctccttaggataaagccttcttggtgctgctttttttgaaatacattccagggcctggccagttacatttttgccagcctttttttcaatcagatctgacctttttcgtttctgtgaaagacacagtgactgtggtgaagatgctctactttgttcatcagctaatgtggccaaaataaagttagcttccactaacatatcatcaatactcaaagccagaggtttcccagggaaatcaaaataaatggatataggagcatgtgtagcttctgaaaatgtcagtattcccttcaattctttgaaacaaaatgttatctcagtgtccattccaatttgaaagaagtcaaactcatctgagccaacaaacatctcactgtgtacagcattgctcaaatccattgattcctcattagaactcttgaggcaaaaattcagtggagtaacagcaagagtaacttcctcttgacttgatgtaaaaagaacaatggcatcagcaagcaatctttcacctgactgccgctcatcacgcacttcagcatggctgccatccgccct

SEQ ID NO: 14885 - RNA, 1810 nt, Homo sapiens
  source 1..1810: mol_type = other RNA
gctgggattacaggcatgagccactacaccccgccagtattaactataataatagtccaatgctgcatccaggctattactgatgatgatgcctttaagacctaaacccctctgcctacttcaatgaatgaaccagaaatgttatcctcagcaaagagacctacagagttacttttgtgtataaaagctccctgtgtaggcatctgcatttgttagaaataccagaaattcagtgttaatcatcagtgtaagcataagatacatatatcttcccctaccatgtgatgaaaggacttagttgaaattatgtgggcattgccagttaccacaaaaagcttggttaaggcccattttcattcactaaggaacatcttgggatgaacttgagtttttattaggttattgtgggtagctatgactcattactaagctacaagagccaaattaattctggtttcagttagaactctattcacagttctaaagcatgcaaatccactcagccacctttatgaatttctcacaaagtctaaagtacaactgcttgccagttaacacttccttacggtttgaaggtttcagaaagatgtaacaataatatgttacaaaagtctcgtttgtcaggttataattgactgtaaacaggtttgggggagggagaggcacacatcataagacattacataacaatgttttgtgccagattttttagtccatttgtgcaggtaaaaagctaactcttaaagggccaaagaacagagacatttgtcttccaccttattccactccaaactcaggctgtcttggcagtggaggatactgttctatgtcagataatacagaaatatttggcatcacttccattaaattctttcctgcagcacactttctgagacacagagaccctggcacttcctctgtgttgctgacactgctttctgatacttcactgacatctccatccactcttttcattgcagggctgccacagttttccaatgcagatatgtttgtgagagtctccttaggataaagccttcttggtgctgctttttttgaaatacattccagggcctggccagttacatttttgccagcctttttttcaatcagatctgacctttttcgtttctgtgaaagacacagtgactgtggtgaagatgctctactttgttcatcagctaatgtggccaaaataaagttagcttccactaacatatcatcaatactcaaagccagaggtttcccagggaaatcaaaataaatggatataggagcatgtgtagcttctgaaaatgtcagtattcccttcaattctttgaaacaaaatgttatctcagtgtccattccaatttgaaagaagtcaaactcatctgagccaacaaacatctcactgtgtacagcattgctcaaatcatgtctgtagaagaattgaataactactttgcatttatcagatctggtgaatattctgcacttctctatatttctttcaagggaattcagacatctaaagatgggcaaaattgacttcattcccaatttgcattttaaatgcagtgttgtgtcaagttcattttcactcattttcactaaagctgaccattgataatgctgaaaaaacacaggagagaacaggacacatccatatgctgaccgagaagaattcacacatcttagagcaagaccttttttagatgggtctagccagaactcgtcactaattcgtgatagagcttgaactgctttcccaaatactttcacctgactgccgctcatcacgcacttcagcatggctgccatccgccct

SEQ ID NO: 14886 - RNA, 2072 nt, Homo sapiens
  source 1..2072: mol_type = other RNA
gctgggattacaggcatgagccactacaccccgccagtattaactataataatagtccaatgctgcatccaggctattactgatgatgatgcctttaagacctaaacccctctgcctacttcaatgaatgaaccagaaatgttatcctcagcaaagagacctacagagttacttttgtgtataaaagctccctgtgtaggcatctgcatttgttagaaataccagaaattcagtgttaatcatcagtgtaagcataagatacatatatcttcccctaccatgtgatgaaaggacttagttgaaattatgtgggcattgccagttaccacaaaaagcttggttaaggcccattttcattcactaaggaacatcttgggatgaacttgagtttttattaggttattgtgggtagctatgactcattactaagctacaagagccaaattaattctggtttcagttagaactctattcacagttctaaagcatgcaaatccactcagccacctttatgaatttctcacaaagtctaaagtacaactgcttgccagttaacacttccttacggtttgaaggtttcagaaagatgtaacaataatatgttacaaaagtctcgtttgtcaggttataattgactgtaaacaggtttgggggagggagaggcacacatcataagacattacataacaatgttttgtgccagattttttagtccatttgtgcaggtaaaaagctaactcttaaagggccaaagaacagagacatttgtcttccaccttattccactccaaactcaggctgtcttggcagtggaggatactgttctatgtcagataatacagaaatatttggcatcacttccattaaattctttcctgcagcacactttctgagacacagagaccctggcacttcctctgtgttgctgacactgctttctgatacttcactgacatctccatccactcttttcattgcagggctgccacagttttccaatgcagatatgtttgtgagagtctccttaggataaagccttcttggtgctgctttttttgaaatacattccagggcctggccagttacatttttgccagcctttttttcaatcagatctgacctttttcgtttctgtgaaagacacagtgactgtggtgaagatgctctactttgttcatcagctaatgtggccaaaataaagttagcttccactaacatatcatcaatactcaaagccagaggtttcccagggaaatcaaaataaatggatataggagcatgtgtagcttctgaaaatgtcagtattcccttcaattctttgaaacaaaatgttatctcagtgtccattccaatttgaaagaagtcaaactcatctgagccaacaaacatctcactgtgtacagcattgctcaaatccattgattcctcattagaactcttgaggcaaaaattcagtggagtaacagcaagagtaacttcctcttgacttgatgtaaaaagaacaatggcatcagcaagcaatcatgtctgtagaagaattgaataactactttgcatttatcagatctggtgaatattctgcacttctctatatttctttcaagggaattcagacatctaaagatgggcaaaattgacttcattcccaatttgcattttaaatgcagtgttgtgtcaagttcattttcactcattttcactaaagctgaccattgataatgctgaaaaaacacaggagagaacaggacacatccatatgctgaccgagaagaattcacacatcttagagcaagaccttttttagatgggtctagccagaactcgtcactaattcgtgatagagcttgaactgctttcccaaatactgactgccgctcatcacgcacttcagcatggctgccatccgccctaaaaagcaggctcggaaggcgcgcctcagctcgacggcccaggtgcccggatgttgcccgcgcttttcaaagcttcgcgatctcgtctctgcactctaccaccccgcctccacaagttcccaaacggctttacggcggagaagggtccgtgcgggcctccgt

SEQ ID NO: 14887 - RNA, 1888 nt, Homo sapiens
  source 1..1888: mol_type = other RNA
gctgggattacaggcatgagccactacaccccgccagtattaactataataatagtccaatgctgcatccaggctattactgatgatgatgcctttaagacctaaacccctctgcctacttcaatgaatgaaccagaaatgttatcctcagcaaagagacctacagagttacttttgtgtataaaagctccctgtgtaggcatctgcatttgttagaaataccagaaattcagtgttaatcatcagtgtaagcataagatacatatatcttcccctaccatgtgatgaaaggacttagttgaaattatgtgggcattgccagttaccacaaaaagcttggttaaggcccattttcattcactaaggaacatcttgggatgaacttgagtttttattaggttattgtgggtagctatgactcattactaagctacaagagccaaattaattctggtttcagttagaactctattcacagttctaaagcatgcaaatccactcagccacctttatgaatttctcacaaagtctaaagtacaactgcttgccagttaacacttccttacggtttgaaggtttcagaaagatgtaacaataatatgttacaaaagtctcgtttgtcaggttataattgactgtaaacaggtttgggggagggagaggcacacatcataagacattacataacaatgttttgtgccagattttttagtccatttgtgcaggtaaaaagctaactcttaaagggccaaagaacagagacatttgtcttccaccttattccactccaaactcaggctgtcttggcagtggaggatactgttctatgtcagataatacagaaatatttggcatcacttccattaaattctttcctgcagcacactttctgagacacagagaccctggcacttcctctgtgttgctgacactgctttctgatacttcactgacatctccatccactcttttcattgcagggctgccacagttttccaatgcagatatgtttgtgagagtctccttaggataaagccttcttggtgctgctttttttgaaatacattccagggcctggccagttacatttttgccagcctttttttcaatcagatctgacctttttcgtttctgtgaaagacacagtgactgtggtgaagatgctctactttgttcatcagctaatgtggccaaaataaagttagcttccactaacatatcatcaatactcaaagccagaggtttcccagggaaatcaaaataaatggatataggagcatgtgtagcttctgaaaatgtcagtattcccttcaattctttgaaacaaaatgttatctcagtgtccattccaatttgaaagaagtcaaactcatctgagccaacaaacatctcactgtgtacagcattgctcaaatccattgattcctcattagaactcttgaggcaaaaattcagtggagtaacagcaagagtaacttcctcttgacttgatgtaaaaagaacaatggcatcagcaagcaatcatgtctgtagaagaattgaataactactttgcatttatcagatctggtgaatattctgcacttctctatatttctttcaagggaattcagacatctaaagatgggcaaaattgacttcattcccaatttgcattttaaatgcagtgttgtgtcaagttcattttcactcattttcactaaagctgaccattgataatgctgaaaaaacacaggagagaacaggacacatccatatgctgaccgagaagaattcacacatcttagagcaagaccttttttagatgggtctagccagaactcgtcactaattcgtgatagagcttgaactgctttcccaaatattcagcatggctgccatccgccct

SEQ ID NO: 14888 - RNA, 2017 nt, Homo sapiens
  source 1..2017: mol_type = other RNA
gctgggattacaggcatgagccactacaccccgccagtattaactataataatagtccaatgctgcatccaggctattactgatgatgatgcctttaagacctaaacccctctgcctacttcaatgaatgaaccagaaatgttatcctcagcaaagagacctacagagttacttttgtgtataaaagctccctgtgtaggcatctgcatttgttagaaataccagaaattcagtgttaatcatcagtgtaagcataagatacatatatcttcccctaccatgtgatgaaaggacttagttgaaattatgtgggcattgccagttaccacaaaaagcttggttaaggcccattttcattcactaaggaacatcttgggatgaacttgagtttttattaggttattgtgggtagctatgactcattactaagctacaagagccaaattaattctggtttcagttagaactctattcacagttctaaagcatgcaaatccactcagccacctttatgaatttctcacaaagtctaaagtacaactgcttgccagttaacacttccttacggtttgaaggtttcagaaagatgtaacaataatatgttacaaaagtctcgtttgtcaggttataattgactgtaaacaggtttgggggagggagaggcacacatcataagacattacataacaatgttttgtgccagattttttagtccatttgtgcaggtaaaaagctaactcttaaagggccaaagaacagagacatttgtcttccaccttattccactccaaactcaggctgtcttggcagtggaggatactgttctatgtcagataatacagaaatatttggcatcacttccattaaattctttcctgcagcacactttctgagacacagagaccctggcacttcctctgtgttgctgacactgctttctgatacttcactgacatctccatccactcttttcattgcagggctgccacagttttccaatgcagatatgtttgtgagagtctccttaggataaagccttcttggtgctgctttttttgaaatacattccagggcctggccagttacatttttgccagcctttttttcaatcagatctgacctttttcgtttctgtgaaagacacagtgactgtggtgaagatgctctactttgttcatcagctaatgtggccaaaataaagttagcttccactaacatatcatcaatactcaaagccagaggtttcccagggaaatcaaaataaatggatataggagcatgtgtagcttctgaaaatgtcagtattcccttcaattctttgaaacaaaatgttatctcagtgtccattccaatttgaaagaagtcaaactcatctgagccaacaaacatctcactgtgtacagcattgctcaaatccattgattcctcattagaactcttgaggcaaaaattcagtggagtaacagcaagagtaacttcctcttgacttgatgtaaaaagaacaatggcatcagcaagcaatcttggttgaatcattagcgtattagtacaaacattcttgtcaaaaataacttgcaaaggctgactttcttgaaaacatatattatgagttcttttaataccatgtctgtagaagaattgaataactactttgcatttatcagatctggtgaatattctgcacttctctatatttctttcaagggaattcagacatctaaagatgggcaaaattgacttcattcccaatttgcattttaaatgcagtgttgtgtcaagttcattttcactcattttcactaaagctgaccattgataatgctgaaaaaacacaggagagaacaggacacatccatatgctgaccgagaagaattcacacatcttagagcaagaccttttttagatgggtctagccagaactcgtcactaattcgtgatagagcttgaactgctttcccaaatactttcacctgactgccgctcatcacgcacttcagcatggctgccatccgccct

SEQ ID NO: 14889 - RNA, 2015 nt, Homo sapiens
  source 1..2015: mol_type = other RNA
gctgggattacaggcatgagccactacaccccgccagtattaactataataatagtccaatgctgcatccaggctattactgatgatgatgcctttaagacctaaacccctctgcctacttcaatgaatgaaccagaaatgttatcctcagcaaagagacctacagagttacttttgtgtataaaagctccctgtgtaggcatctgcatttgttagaaataccagaaattcagtgttaatcatcagtgtaagcataagatacatatatcttcccctaccatgtgatgaaaggacttagttgaaattatgtgggcattgccagttaccacaaaaagcttggttaaggcccattttcattcactaaggaacatcttgggatgaacttgagtttttattaggttattgtgggtagctatgactcattactaagctacaagagccaaattaattctggtttcagttagaactctattcacagttctaaagcatgcaaatccactcagccacctttatgaatttctcacaaagtctaaagtacaactgcttgccagttaacacttccttacggtttgaaggtttcagaaagatgtaacaataatatgttacaaaagtctcgtttgtcaggttataattgactgtaaacaggtttgggggagggagaggcacacatcataagacattacataacaatgttttgtgccagattttttagtccatttgtgcaggtaaaaagctaactcttaaagggccaaagaacagagacatttgtcttccaccttattccactccaaactcaggctgtcttggcagtggaggatactgttctatgtcagataatacagaaatatttggcatcacttccattaaattctttcctgcagcacactttctgagacacagagaccctggcacttcctctgtgttgctgacactgctttctgatacttcactgacatctccatccactcttttcattgcagggctgccacagttttccaatgcagatatgtttgtgagagtctccttaggataaagccttcttggtgctgctttttttgaaatacattccagggcctggccagttacatttttgccagcctttttttcaatcagatctgacctttttcgtttctgtgaaagacacagtgactgtggtgaagatgctctactttgttcatcagctaatgtggccaaaataaagttagcttccactaacatatcatcaatactcaaagccagaggtttcccagggaaatcaaaataaatggatataggagcatgtgtagcttctgaaaatgtcagtattcccttcaattctttgaaacaaaatgttatctcagtgtccattccaatttgaaagaagtcaaactcatctgagccaacaaacatctcactgtgtacagcattgctcaaatccattgattcctcattagaactcttgaggcaaaaattcagtggagtaacagcaagagtaacttcctcttgacttgatgtaaaaagaacaatggcatcagcaagcaatcttggttgaatcattagcgtattagtacaaacattcttgtcaaaaataacttgcaaaggctgactttcttgaaaacatatattatgagttcttttaataccatgtctgtagaagaattgaataactactttgcatttatcagatctggtgaatattctgcacttctctatatttctttcaagggaattcagacatctaaagatgggcaaaattgacttcattcccaatttgcattttaaatgcagtgttgtgtcaagttcattttcactcattttcactaaagctgaccattgataatgctgaaaaaacacaggagagaacaggacacatccatatgctgaccgagaagaattcacacatcttagagcaagcttttttagatgggtctagccagaactcgtcactaattcgtgatagagcttgaactgctttcccaaatactttcacctgactgccgctcatcacgcacttcagcatggctgccatccgccct

SEQ ID NO: 14890 - RNA, 2062 nt, Homo sapiens
  source 1..2062: mol_type = other RNA
gctgggattacaggcatgagccactacacccggccccccaatatattctttagtctaaagtaaactgcttcttcccattccccacactctccagttcccatttttcccttattgcaggctccaatgttcctgccttctccttgctgcactgccatctgcattaacccctcccctgctgtgctcagctatggaaatgccaaagtccctaacactcagttccataaactttacctcaccctctttatccccctaataaaatgtttgcatttgggtcaaaagcgatggctcacgcctgtaatcccagcactttgggaggccaaggtgggcagatcaagaggtcaggagatcgagaccatcctggccaacatggtgaaaccccatctctattaaaaatacaaaaattagctgggcatggtggtaggcgcctgtagtcccagctacttgggaggccaaggcaggagaatcgcttgaacacgggaggcagagcttgcagtgagctgagatcgcaccattgcactccaacttggcgacagagcaagactctgtctcagaaaaaaaaaaaagtttgcattttgtcctggcccctgccaggcatatctctcctggtggctgccctgccctgtggtcacagttcttggtccgcctgcagaatcttataattattgttgagaatgtttagcttctcctccagctcctgagccaccttcttcagctcctcagctgtctctgactttgccccctcatgtaagtgctttgattcgtacacgaggtagactacatccagcacaagaaagaagcttacaggggccacatccgtgagcttgactcctctgctcatttccaggatgctgggttcattaaccctctccacctgttcaccgctttcagctgagattggctcagtgacccgggggcgtgaggctgaggcatgcggtactgactgaagattggctctggctcgtctgagggcacggatgtccttcccaatgcctcgtgtgagttggtaagtattgccagctaaggaaagaaagttggatatgttctcacccaaaaactccctcacctccttcaatttgtcaaggcttttgatgaccaggtcgtgggcttgggcttgtgtccaccacttctttccgtagtccatggtactgctggtaatcccggtcaaagcggctgtgattcccaactccatcccaggttccaagagtacaaggctgcctccctctgtgaagggtgccagacccatgccgacgagggtcaggatgccagaggaaatgctgagagagccagacaccacattggcgatggtggtgcctttgtggaccttctgaaccccatctgcaagggcacggagccttcttatgttatcctcaagctcacttttcaaccgaggaaactctttcagaaaccagtttctgtactgctggcctttatcgtgccagtttttgtctttcatgatcatttgtcttgcaaggttgtccagagctttacggagctcatctgcctcattcctgggcagttcagcagcagccacgaatccgttccaggcctcattatcagtcagcaggagtagcagattctgtgtgctcactttttccttgaaatacttaatggcatcctcaataaagatactgctctcatgcaaaggagattcctcctgctggtcttgggcactctcagatgggcagtggagggggttcttcgacggggcatgggggcgggaccctcagcactgatccttgaggcacctccatgttgcctctgtcctctgcaggctggtctcagggtacacggctctccactgtcacctctggacccagctgggcctgggtccatggtgccagcagcccagtcaccgaggggcttactttgaggatctccagtatctgtcccacttggaacgttttgttgcacccagatgcagaggacagagactctcagcaaagcagctccctccatgtcgctgcagggcctcctccaaggaatcttcccctggcagagactgagcaagatccagctgttctgagctgtgtggatcccacctccagttatgcgtctgtataat

SEQ ID NO: 14891 - RNA, 1874 nt, Homo sapiens
  source 1..1874: mol_type = other RNA
gctgggattacaggcatgagccactacacccggccccccaatatattctttagtctaaagtaaactgcttcttcccattccccacactctccagttcccatttttcccttattgcaggctccaatgttcctgccttctccttgctgcactgccatctgcattaacccctcccctgctgtgctcagctatggaaatgccaaagtccctaacactcagttccataaactttacctcaccctctttatccccctaataaaatgtttgcatttgggtcaaaagcgatggctcacgcctgtaatcccagcactttgggaggccaaggtgggcagatcaagaggtcaggagatcgagaccatcctggccaacatggtgaaaccccatctctattaaaaatacaaaaattagctgggcatggtggtaggcgcctgtagtcccagctacttgggaggccaaggcaggagaatcgcttgaacacgggaggcagagcttgcagtgagctgagatcgcaccattgcactccaacttggcgacagagcaagactctgtctcagaaaaaaaaaaaagtttgcattttgtcctggcccctgccaggcatatctctcctggtggctgccctgccctgtggtcacagttcttggtccgcctgcagaatcttataattattgttgagaatgtttagcttctcctccagctcctgagccaccttcttcagctcctcagctgtctctgactttgccccctcatgtaagtgctttgattcgtacacgaggtagactacatccagcacaagaaagaagcttacaggggccacatccgtgagcttgactcctctgctcatttccaggatgctgggttcattaaccctctccacctgttcaccgctttcagctgagattggctcagtgacccgggggcgtgaggctgaggcatgcggtactgactgaagattggctctggctcgtctgagggcacggatgtccttcccaatgcctcgtgtgagttggtaagtattgccagctaaggaaagaaagttggatatgttctcacccaaaaactccctcacctccttcaatttgtcaaggcttttgatgaccaggtcgtgggcttgggcttgtgtccaccacttctttccgtagtccatggtactgctggtaatcccggtcaaagcggctgtgattcccaactccatcccaggttccaagagtacaaggctgcctccctctgtgaagggtgccagacccatgccgacgagggtcaggatgccagaggaaatgctgagagagccagacaccacattggcgatggtggtgcctttgtggaccttctgaaccccatctgcaagggcacggagccttcttatgttatcctcaagctcacttttcaaccgaggaaactctttcagaaaccagtttctgtactgctggcctttatcgtgccagtttttgtctttcatgatcatttgtcttgcaaggttgtccagagctttacggagctcatctgcctcattcctgggcagttcagcagcagccacgaatccgttccaggcctcattatcagtcagcaggagtagcagattctgtgtgctcactttttccttgaaatacttaatggcatcctcaataaagatactgctctctgggtccatggtgccagcagcccagtcaccgaggggcttactttgaggatctccagtatctgtcccacttggaacgttttgttgcacccagatgcagaggacagagactctcagcaaagcagctccctccatgtcgctgcagggcctcctccaaggaatcttcccctggcagagactgagcaagatccagctgttctgagctgtgtggatcccacctccagttatgcgtctgtataat

SEQ ID NO: 14892 - RNA, 1913 nt, Homo sapiens
  source 1..1913: mol_type = other RNA
gctgggattacaggcatgagccactacacccggccccccaatatattctttagtctaaagtaaactgcttcttcccattccccacactctccagttcccatttttcccttattgcaggctccaatgttcctgccttctccttgctgcactgccatctgcattaacccctcccctgctgtgctcagctatggaaatgccaaagtccctaacactcagttccataaactttacctcaccctctttatccccctaataaaatgtttgcatttgggtcaaaagcgatggctcacgcctgtaatcccagcactttgggaggccaaggtgggcagatcaagaggtcaggagatcgagaccatcctggccaacatggtgaaaccccatctctattaaaaatacaaaaattagctgggcatggtggtaggcgcctgtagtcccagctacttgggaggccaaggcaggagaatcgcttgaacacgggaggcagagcttgcagtgagctgagatcgcaccattgcactccaacttggcgacagagcaagactctgtctcagaaaaaaaaaaaagtttgcattttgtcctggcccctgccaggcatatctctcctggtggctgccctgccctgtggtcacagttcttggtccgcctgcagaatcttataattattgttgagaatgtttagcttctcctccagctcctgagccaccttcttcagctcctcagctgtctctgactttgccccctcatgtaagtgctttgattcgtacacgaggtagactacatccagcacaagaaagaagcttacaggggccacatccgtgagcttgactcctctgctcatttccaggatgctgggttcattaaccctctccacctgttcaccgctttcagctgagattggctcagtgacccgggggcgtgaggctgaggcatgcggtactgactgaagattggctctggctcgtctgagggcacggatgtccttcccaatgcctcgtgtgagttggtaagtattgccagctaaggaaagaaagttggatatgttctcacccaaaaactccctcacctccttcaatttgtcaaggcttttgatgaccaggtcgtgggcttgggcttgtgtccaccacttctttccgtagtccatggtactgctggtaatcccggtcaaagcggctgtgattcccaactccatcccaggttccaagagtacaaggctgcctccctctgtgaagggtgccagacccatgccgacgagggtcaggatgccagaggaaatgctgagagagccagacaccacattggcgatggtggtgcctttgtggaccttctgaaccccatctgcaagggcacggagccttcttatgttatcctcaagctcacttttcaaccgaggaaactctttcagaaaccagtttctgtactgctggcctttatcgtgccagtttttgtctttcatgatcatttgtcttgcaaggttgtccagagctttacggagctcatctgcctcattcctgggcagttcagcagcagccacgaatccgttccaggcctcattatcagtcagcaggagtagcagattctgtgtgctcactttttccttgaaatacttaatggcatcctcaataaagatactgctctctgggtccatggtgccagcagcccagtcaccgaggggcttactttgaggatctccagtatctgtcccacttggaacgttttgttgcacccagatgcagaggacagagactctcagcaaagcagctccctccatgtcgctgcagggcctcctccttgagcaggaaaagaggggttgagacagtgtgctcctccaaggaatcttcccctggcagagactgagcaagatccagctgttctgagctgtgtggatcccacctccagttatgcgtctgtataat

SEQ ID NO: 14893 - RNA, 2144 nt, Homo sapiens
  source 1..2144: mol_type = other RNA
gctgggattacaggcatgagccactacacccggccccccaatatattctttagtctaaagtaaactgcttcttcccattccccacactctccagttcccatttttcccttattgcaggctccaatgttcctgccttctccttgctgcactgccatctgcattaacccctcccctgctgtgctcagctatggaaatgccaaagtccctaacactcagttccataaactttacctcaccctctttatccccctaataaaatgtttgcatttgggtcaaaagcgatggctcacgcctgtaatcccagcactttgggaggccaaggtgggcagatcaagaggtcaggagatcgagaccatcctggccaacatggtgaaaccccatctctattaaaaatacaaaaattagctgggcatggtggtaggcgcctgtagtcccagctacttgggaggccaaggcaggagaatcgcttgaacacgggaggcagagcttgcagtgagctgagatcgcaccattgcactccaacttggcgacagagcaagactctgtctcagaaaaaaaaaaaagtttgcattttgtcctggcccctgccaggcatatctctcctggtggctgccctgccctgtggtcacagttcttggtccgcctgcagaatcttataattattgttgagaatgtttagcttctcctccagctcctgagccaccttcttcagctcctcagctgtctctgactttgccccctcatgtaagtgctttgattcgtacacgaggtagactacatccagcacaagaaagaagcttacaggggccacatccgtgagcttgactcctctgctcatttccaggatgctgggttcattaaccctctccacctgttcaccgctttcagctgagattggctcagtgacccgggggcgtgaggctgaggcatgcggtactgactgaagattggctctggctcgtctgagggcacggatgtccttcccaatgcctcgtgtgagttggtaagtattgccagctaaggaaagaaagttggatatgttctcacccaaaaactccctcacctccttcaatttgtcaaggcttttgatgaccaggtcgtgggcttgggcttgtgtccaccacttctttccgtagtccatggtactgctggtaatcccggtcaaagcggctgtgattcccaactccatcccaggttccaagagtacaaggctgcctccctctgtgaagggtgccagacccatgccgacgagggtcaggatgccagaggaaatgctgagagagccagacaccacattggcgatggtggtgcctttgtggaccttctgaaccccatctgcaagggcacggagccttcttatgttatcctcaagctcacttttcaaccgaggaaactctttcagaaaccagtttctgtactgctggcctttatcgtgccagtttttgtctttcatgatcatttgtcttgcaaggttgtccagagctttacggagctcatctgcctcattcctgggcagttcagcagcagccacgaatccgttccaggcctcattatcagtcagcaggagtagcagattctgtgtgctcactttttccttgaaatacttaatggcatcctcaataaagatactgctctctgggtccatggtgccagcagcccagtcaccgaggggcttactttgaggatctccagtatctgtcccacttggaacgttttgttgcaccctcgctccagcttcctctgccctcactcccacaccaaggaaaagtgcactcatccagatgcagaggacagagactctcagcaaagcagctccctccatgtcgctgcagggcctcctcaattccacagtgtggcttttgaatctcatgattgcaaagctggcatcatgccacaggcaccattctgcaacgcacccttctcactcccctgtctcagccacgtttcccattagggacacagcacagcctgtttcttctccatcaccccagaagtcaaggaatcttcccctggcagagactgagcaagatccagctgttctgagctgtgtggatcccacctccagttatgcgtctgtataataaccagacaggtcctccagtccccaagatataccgaggaattcgaaagggaaagtgaaagtc

SEQ ID NO: 14894 - RNA, 1928 nt, Homo sapiens
  source 1..1928: mol_type = other RNA
gctgggattacaggcatgagccactacacccggccccccaatatattctttagtctaaagtaaactgcttcttcccattccccacactctccagttcccatttttcccttattgcaggctccaatgttcctgccttctccttgctgcactgccatctgcattaacccctcccctgctgtgctcagctatggaaatgccaaagtccctaacactcagttccataaactttacctcaccctctttatccccctaataaaatgtttgcatttgggtcaaaagcgatggctcacgcctgtaatcccagcactttgggaggccaaggtgggcagatcaagaggtcaggagatcgagaccatcctggccaacatggtgaaaccccatctctattaaaaatacaaaaattagctgggcatggtggtaggcgcctgtagtcccagctacttgggaggccaaggcaggagaatcgcttgaacacgggaggcagagcttgcagtgagctgagatcgcaccattgcactccaacttggcgacagagcaagactctgtctcagaaaaaaaaaaaagtttgcattttgtcctggcccctgccaggcatatctctcctggtggctgccctgccctgtggtcacagttcttggtccgcctgcagaatcttataattattgttgagaatgtttagcttctcctccagctcctgagccaccttcttcagctcctcagctgtctctgactttgccccctcatgtaagtgctttgattcgtacacgaggtagactacatccagcacaagaaagaagcttacaggggccacatccgtgagcttgactcctctgctcatttccaggatgctgggttcattaaccctctccacctgttcaccgctttcagctgagattggctcagtgacccgggggcgtgaggctgaggcatgcggtactgactgaagattggctctggctcgtctgagggcacggatgtccttcccaatgcctcgtgtgagttggtaagtattgccagctaaggaaagaaagttggatatgttctcacccaaaaactccctcacctccttcaatttgtcaaggcttttgatgaccaggtcgtgggcttgggcttgtgtccaccacttctttccgtagtccatggtactgctggtaatcccggtcaaagcggctgtgattcccaactccatcccaggttccaagagtacaaggctgcctccctctgtgaagggtgccagacccatgccgacgagggtcaggatgccagaggaaatgctgagagagccagacaccacattggcgatggtggtgcctttgtggaccttctgaaccccatctgcaagggcacggagccttcttatgttatcctcaagctcacttttcaaccgaggaaactctttcagaaaccagtttctgtactgctggcctttatcgtgccagtttttgtctttcatgatcatttgtcttgcaaggttgtccagagctttacggagctcatctgcctcattcctgggcagttcagcagcagccacgaatccgttccaggcctcattatcagtcagcaggagtagcagattctgtgtgctcactttttccttgaaatacttaatggcatcctcaataaagatactgctctctgggtccatggtgccagcagcccagtcaccgaggggcttactttgaggatctccagtatctgtcccacttggaacgttttgttgcaccctcgctccagcttcctctgccctcactcccacaccaaggaaaagtgcactcatccagatgcagaggacagagactctcagcaaagcagctccctccatgtcgctgcagggcctcctccaaggaatcttcccctggcagagactgagcaagatccagctgttctgagctgtgtggatcccacctccagttatgcgtctgtataat

SEQ ID NO: 14895 - RNA, 1967 nt, Homo sapiens
  source 1..1967: mol_type = other RNA
gctgggattacaggcatgagccactacacccggccccccaatatattctttagtctaaagtaaactgcttcttcccattccccacactctccagttcccatttttcccttattgcaggctccaatgttcctgccttctccttgctgcactgccatctgcattaacccctcccctgctgtgctcagctatggaaatgccaaagtccctaacactcagttccataaactttacctcaccctctttatccccctaataaaatgtttgcatttgggtcaaaagcgatggctcacgcctgtaatcccagcactttgggaggccaaggtgggcagatcaagaggtcaggagatcgagaccatcctggccaacatggtgaaaccccatctctattaaaaatacaaaaattagctgggcatggtggtaggcgcctgtagtcccagctacttgggaggccaaggcaggagaatcgcttgaacacgggaggcagagcttgcagtgagctgagatcgcaccattgcactccaacttggcgacagagcaagactctgtctcagaaaaaaaaaaaagtttgcattttgtcctggcccctgccaggcatatctctcctggtggctgccctgccctgtggtcacagttcttggtccgcctgcagaatcttataattattgttgagaatgtttagcttctcctccagctcctgagccaccttcttcagctcctcagctgtctctgactttgccccctcatgtaagtgctttgattcgtacacgaggtagactacatccagcacaagaaagaagcttacaggggccacatccgtgagcttgactcctctgctcatttccaggatgctgggttcattaaccctctccacctgttcaccgctttcagctgagattggctcagtgacccgggggcgtgaggctgaggcatgcggtactgactgaagattggctctggctcgtctgagggcacggatgtccttcccaatgcctcgtgtgagttggtaagtattgccagctaaggaaagaaagttggatatgttctcacccaaaaactccctcacctccttcaatttgtcaaggcttttgatgaccaggtcgtgggcttgggcttgtgtccaccacttctttccgtagtccatggtactgctggtaatcccggtcaaagcggctgtgattcccaactccatcccaggttccaagagtacaaggctgcctccctctgtgaagggtgccagacccatgccgacgagggtcaggatgccagaggaaatgctgagagagccagacaccacattggcgatggtggtgcctttgtggaccttctgaaccccatctgcaagggcacggagccttcttatgttatcctcaagctcacttttcaaccgaggaaactctttcagaaaccagtttctgtactgctggcctttatcgtgccagtttttgtctttcatgatcatttgtcttgcaaggttgtccagagctttacggagctcatctgcctcattcctgggcagttcagcagcagccacgaatccgttccaggcctcattatcagtcagcaggagtagcagattctgtgtgctcactttttccttgaaatacttaatggcatcctcaataaagatactgctctctgggtccatggtgccagcagcccagtcaccgaggggcttactttgaggatctccagtatctgtcccacttggaacgttttgttgcaccctcgctccagcttcctctgccctcactcccacaccaaggaaaagtgcactcatccagatgcagaggacagagactctcagcaaagcagctccctccatgtcgctgcagggcctcctccttgagcaggaaaagaggggttgagacagtgtgctcctccaaggaatcttcccctggcagagactgagcaagatccagctgttctgagctgtgtggatcccacctccagttatgcgtctgtataat

SEQ ID NO: 14896 - RNA, 8343 nt, Homo sapiens
  source 1..8343: mol_type = other RNA
gctgggattacaggcatgagccactacacctggccatcatgacaattttcaaagcccctctgaaattctatttttattcccattttacagataaggacattgagacccagaaagcaactgctcaaaagtctagggaaagactctagcaatttcagtgattttataacaatagattgccttggagatgtattttttttttcggaaagtaggtcaggttctaaatggatcatttagaacggacaggagatagggaaatactgggtagaaaagggtggttccctggcaagtgccccactatcaagccaggatactcatgcccctaaatggagacaggcattcctgttttcatgcccaaaagctgccttttggctcaccacagcccctatcctgtacccatgtaaaccccagactgcaggctccagaagcagacaaggagaagagtagacaagtggcagaatggcgtgggagagagaagagaagggccatccgaatgctgagagaagtttggctggggatggtcagagaggagattggctactggatggccaaactccaggggaagaacatcttcccactccatcccccttccagctccccattcgtctcattgagagcaatttccaccactcaataatacccccacattcatccttcaagtctgtatgtgacctgactcttctgggatgttggacgagagcttgggtacagaaagctgtcacactggccctctgccattgtgaaaaggcagagaattcactgagctggttaacagataagctgcccgcgaatggcaaggctgaaagagtacactgtaacacagcccatttgggctttgggagttgcaggctctcaaccctgaatgctgccctggggctggagcccaggggtgcttactctggctcctgaacctacctgtctgcatgctcccctcacataaggggtttgaggagcagtggttactgaacagatgagtcacatccctgtctcacgttcagcaaggggtgtcagggaattctcccatttcaatttctcagtgttttctcctacgcagtctgttgtggtggtggtcattagtgccatccagcaaatattttggcatgagctccctgcagacttccttctcactggctctccatgacctccccactgggctgcctgagggcattgacttcatttggaaaatgcatttagaaatgtcactggctggaaagtattgagctctaaagcctccttggaactgtggatgcaaagaatgtgaagagccagtctcctgtaagcaccgaatcccaagtcatcatcttgaaaatggagaaaataagggttagaaaggggaatgagatgaccaagattatactgttggggatatagcagtgaaataaagaagttaggtaaggtccctgctcttatgaagctaaagattcagtgagggagattgacaacatgcaagaaaacaaataattccaaaagtaaaacagagtacaatggcaaagaataatgagcttaggggatatttgatatatggtagtcaaaggatgtctcttggaagaggtgatatttaaactgagacttgaaagatgtaaaggcaccagcaaagatctggggcaggagtgttccgggagtgaaaaggagtagcaagttcaaagttcataaggcagaaatacgtttggtgtgtttgaagtttggtgtggcacaaatcccagtgagctagggtgttagtggtaagcgatgcggtgacagaggttggtgaggcaaaatgtgtagggtttaggccacattcagggttcaaattttatttaattacgaaggaagggaagcctcctggaaagtttcaagcagtgaagtgacaaaactggattagtgatttgaaagatccttctgccatggtatatagaataggctattggaggatgagaatagaaacagagagacagttaagagtttaaattccaggtaggattttatttcaatagtctaattgagagatagtgatggagtaaaccaaggttatagactggagaaaagggagggaagtggacaaactggagctatatttggagcgagattttgcaggatgctgggaaagagtgaggtaaagggaatgggtagttgaggatggttttctccattgtgtttttccttgaatgactggatatgtgctagtgacatttattgagacgaagaaggctgggagaagagacgacatgggggcataagattaaaagtgggaagagttgtggaggaatttatgggttaggccagtggaaacttccatctttatcccactggctaaaactcaacctcacagccagatctaactgcaagggagactggggcaggtaatctaggtgtgtgacctcaaagagaagaaaagtttggtgatcatctctcccatggtgcaccactggccacttgattcttaggtacgaaagcttctcaacctaagagtcattcaactcacgacttgggccaggggtcctttcttctcagtcatgacctcactcagccacttgggagctgagccagcccacatttaggtaagacctgagctagaatttggagtaggttcccctcctttctccccctgagttcagttaacttatttttatcctgtagctctaactctggactcaatctttttttttcttttttaagagacaagctcttgctgtgtcccccaggttggacagtagtggtgcaatcatagctcaatagagcctcagactcttggcctcaagcaatcctcttgcctcagccttctgagtcactggaattataggcataagccagtgtgcccagctcgggaatcattctttatctcagtcatgtccaggctcctgtttgaacatagacctcatatactttagacttgacttctgatacctatccctgcagactctgtctcaagttcattattagtttcttgtgaagaacaccatatttggatgtttgtggctttgggtatgattctctcagtcttccaaactgtaaagctgggtttggtagtgttgtgaagtggccttagaatgtaacagatatgcagaatcactgtggaaggaggctctagataagagtcgaagttgtagagggatccagtcattgtcagagccacagtgctgaggcagggggagagccagggaacgaatgctcaactctgctctcctgccaccttttggtctttctattagccagtccaacctgaagtcagaggagacaggagctcctgtgatgtggagaagggcagtgaatgattctgggaaaacagcagagagaataagcagcactggtggagggtctaggaggtgatgggatgcaagggcactggacttgccttgggagccaacttgctgagggactttaagcaaatagcctgatccttttctgtttctcccccgcaacccatcaataaatagggataataacttacccatttcctggggttgttattgtcagcctaaataacaaacagagagaggctttctaaaagaaaaaaatatttatttgggaatagtgcatgagaatacactgcaatgagactgctgtgcccatatgagtactcagggaggtaaaagaaagaaatggtttttaaaggaaaaaatgaggagaattacataattgttttgaaataattatccttggttacaaagataaataacaagagtgacaccagtctgagattggacaggcaattgctgggcagatgtccttgcaaaggtattcttttgtgtaagtttgtaatggtctttgtacaaggttgtgttttttgcagtcattgtgatagtgtttcttgtcaggtatacgaatatgagaatcctctcttcatggacttctgtggctctatttatcagggtttttttaaaaacaaacaagcaaacaagcaaacaaaaaaaaactttagtgactccattttgatttggacaattgtcacgttataaagatcaggtgacataatagatgtacctcattaatttgtatttatgttgaattttataatttctaaatctttctcatgtctcttacctcatttgcttctcaatactagtctttagagtagtcaagataggttttattattcccattttatagggaagatgactgagttgcagaaattaagtggtttcctaaaagttaccaggttaagagatctgttgactcaaacttgactgtaattttctcctagtatactttgaatgctatttaattcagcattgtaggtgattttgagggactattatcatctttgtaaagcataaaagttccagatgaggagcctgagacagtacctttcatgtggtctggaagaacagcacccgggattcaggcctgctttcttatctgggaagacaccacagggagggaaaaagctgtgctgccggttttcataaccagccacttctgtttctcttggcactgaaggttaaactgtagaaatgtgtgaattgtctgctcccttctgaggtttgtgtatttctctttccgccagtctttccctcctaaatgacttgatagagatcttggagaataaggatgtgtcctccagagcattagagccatgcttactccagagtccagaggttcatataattatatgtcaggcactgctgagactcctctaaggtcacacatataaatagcagaggaggctttgagtaaagatgtggctcattctgaagttcatgggaacggaagaaagcatgctctcctaagaggcaagaaacaaaatgtaggcactctactacttaccttgtcaccttgggaaaatacatttatcctctttcagggaaaggactacctttctgattcccaggccaatgccctttctgttgaccttcttgggtttcatttttcacatgtacaaagatgttggcatagcctgaccctgtcctgcattttcacacctacatggtgatatacatgccccaggcccttattagtgacctgattctgtaaagtgagctttctattgagagatccatgtgattattcctaggcaccgatcgccaccagtacttgatagagtcactcaatattgcaaagcagtaaatagaacaactttgtgtgtgtagttcagcagaggagataaccttacatttcagattctttgcttttgttctcccagtccttctctaaacacccttcccccagccttgctttttctctttcatcaggtgccttctgcttttagtcccatctgttcctccttttcctcattttctctccaattgggacctggaagatatgaaaacatacatctgaaatacaagatttgttgcctgggagagatcagaggattgtttttttcttttctttttttttctttaacagcatgatcaaatcttagttctttgctgaaaacttttccagacagggtagtttctttgctaattaaaaggttggataatgagcatttagtgttctggtgattaagacctcctcagcctcacaggtcagtgccacctgaattaattggcaccttctcagttggggttcagttctcacattttatcctaccaagaatggcattcagagctctctgtaatccaccctcatgcagttttcccagcccttcctccctttactacaccactctctgttgatgtagtgatttaacctctgtcaccctcttgctatgtgatttgcttccttgccactatattccctatttccctctgactgaaatggtttagttatgattgtagacttaggagacagtatgtattggaatcattggaactagccctgtcacactagttgtttaacacctcagcctttttttttttttttttttttttttttttgtgacaaagttttgctcttgttgcgcaggctggagtacaatggtgtgatctcagctcatcgtaatccttgcctcacgggttcaagcaattctcctgcctcatcctcccaagtagctgggattacaggcatgcgccaccatgccaggctaattttgtatttttagtagagacggggtttctccatgttggtcaggctggtctcgaattcccaacctcaggagatccgctcatctcggcctcccaaaatgctgggattacaggcatgagccaccacgcctggcctaatctcatcgatctaacctataaaaaagagaataataacttactcacctcattggatagttatgaagataagatagagtataaagggtttggcagagcgtctgtcctatggtaaatgctcgctaactggttagctactataattttctatttgtatctattcaaatctcactgcttctgcaagtctcctaacaaaaagttttgccaaaatttattttgccattgaaagtaatggcaaaagccacaattttgcacaaaccaagaagccttctctgcttatcttccagtccaagattatctcctcttcctagtattcttattttgtgacttttatagaatcacttggttggtctgggtttatgtttaaagttcctgactacaggtgaaatactcttggagaaagagacctaaacttctagcgtaacgctgagacacatcttcatagaatagaattgttattttatgtccccaattaaagggattttatttttgtggatgttttcttgggttgagtgttctactgatttattgaatggtctactgatttctcattatgtgaaaactccagagtcctaggtgtgtttcttccaagagcctaattaattcaggctgctaaggctgccacatggactctggtttaaagactaggctatttggtgagcaattctaagtcctattttggaacactaaggtcatatacctttggaatgccaaattacaagatgctttgaaggaacttttagggtaaatcacaatctcatccgtgtgcatctgcagttaaggtttataaagagaagtttggttcctgattttcagtagcagtatcattagttttttaaaaactacaggaaattttacatgtattttgcctcacaaataccaacaattaggtcagaattcagaaaagtggattctgtttgcatagaattacattaattctgcattctctcatagcaaagttgaaagagaggattaatcacttattcatgcaaaaccaattcacatgaatcatttatttatcttgttctggtaattttgcagagctcatttttacatgcctcaggttgcagataaagtgaaaactcagagggtgatttaccctccacaataaagacctgatggccgtgtaaacagcatgcttcctataggaaatcaataggtaaccatggaaatgactccacaatgggaaattctatttctttatgaacaaatcatcaaaaagatcaattgtaagatgaaaaggctttgcctgtgccctatctttcgcaaaggcttttggtctatgtaaagaagaaaatatgtgccttggtgacagtaaagaattatcttaaagctgtattgagaatgaacatcacttgttactttataaagtttgggctgaaatgtcttgtcctccattcctggaggcctagctaagaaacttatatctaatggcaagaagaatgttccagaatacaggatgcttgaattcttgatccagcttaatttctttcttttttttaggaaaaaaacaagacaaaacaaaaaaacaagggtaataatatccaacgccaaagagcctttgataattaaataagataatagttggtaaagaatatagtacagtgcccagcacagagcaagtggaaaatgctattaacagccacttgtacagtgatgataattgcccaaacaatattaatcccactagtaaagggttttcacattacaggtattttttttaaaactttcatcttaggttcggggtacatgtgaaggtttgttacataggtaaagtcatgttatgggggtttattatacagattatttcatcacccaggaattaaacccagtacccaataattatcttttctgctcctctccctcctcccacctttcccactcaactagaccccagtgtctgatgtttccttctttgtgttcataagttcttatcatttagctcccacttataagtgagaatatgcagtatttggttttttgttcctgcattcatttgctgaggataatagcctccagctccatccatgttcctgcaaaagacaagatttcattttttatggctgtatagtattccatggtgtatatgtaccacaatttctttatccaatctgtcactgatgggcatttagattgatttcatgtctttgctattgtgaacagtgccacagtgaacatttgtgtgcatgtgtctatatggtagagtgctttatatccctctgggtatatacccagtaataggattgacccaggctaatttccagca

SEQ ID NO: 14897 - RNA, 1820 nt, Homo sapiens
  source 1..1820: mol_type = other RNA
gctgggattacaggcatgagccactacacctggccgaccacttatatttaaatacctgtttccgattctcttaggtcgagatctaggagtggaattgctggcttagatgtaattctatgtttaactttttgaggaactgccaaacttttccacagtggcttcactattttacattcccaccagcaatttatgagtttggtaatctttttgttttcctttgaagaaccagcctcatctttgagcccatgtgttgacgggaatatttaagatgtattcttggctaggcgcagtggctcatgcctgtaatcccagtactttgggaggctgaggtgggtggatcccttgagcccaggagttcgaaaccagcttggatgacatgatgaaacctcgtctctatttaaaaaaaaaaatacaaaagttagctagatgtggtggcatgcgcctgtagcgtcctgtagtcccacctactctggggactggaggtggaaggatcacctgagcccaggaggttgaggctgcagtgagctgtgattgcatcattgcacttcagcctgggcaacagagtgagactctgtctcaaaaaaaaaaattactctcgtagcaaatttcaggaatacaatacattattattaactatagtcatcacgctgtacattaagcctcccaaacttattaatcttatttccaaaagtttgtatgctttgaccaacacccccccgcattttcccccactcccagcgcctctgataatgtgacttccaccccattttgtccaaagatgtacagctaagcaggagctagccacttagcatatgccaaagtgattgcttcagggatgggcacgtgacccgagccaggccagtgagattcaactctgaatcagaacaacccctggatttttgttacttgggtcaatttaaaaaaaaaaacactttaaaaaattaagccaatttgagctggctttcctgacacttggccaagtgaccaccctgtataattaagatctgcttgtttaaaatctctgtccaagagatttacttcctatgtatgttttacatgtattcaatgtcaattctacactggttacagctacaagatgatactagagttgagctcacaccagtaggacaagacaggatcaatgaatggtcagagatgggattttgcagacaaaggggaacttccggctgcaggtgttatcattccatgacctcagagcactggtaggcctgtaccatatctgcacgcagtcctcttcttctgggtccgcgtggacgccatcatctggctggctgccatcccagtagctgtagtcataggatgagccatcagtccattcaaactgcccttcctgtctgtgatcatgaaggcctgtccagacgtcagctgggatgccgggaacacagctgttcacgaggtcatatacaaagacattctcctcccagctgtggatggaggccagcttggcggacttcctgcccacagagaactcagaacagtagaggtcggcctcagcccaggtcttattgagagggaagaatcgatagcagtggcctttgaactccatccagaacagggggcacagggaaggcaggggcagctctggcagggctggactgatactgatgtctgtttgtggaaaggcctgtgcagagtggagggtcaggaaggctgcagcccacagtgtccacctttgcatcctgagctcctagaaagcaacctcccagcctgagtggaggagagaggctttttggctggagcttgggtccaggattgctctcctagggtcagatggagcctggcaggagctgggacagact

SEQ ID NO: 14898 - RNA, 1626 nt, Homo sapiens
  source 1..1626: mol_type = other RNA
gctgggattacaggcatgagccactacacctggcctcttcctatctcttacattaatttaaaagattaataaatgcatggacagtgttttagatataataaaatattaataaagacatttatatttttatatataataaaatgattagtttaccaacaatcaaaataaaaagatcccaaagccacagataaggatagcctacagtggtctttatgttcctttgtataattccttttttttcagagtccagtcttggatgtaatccaattgcgataagaagtcactcgagtatagacacctggcttattctttttaccacatccatcaccccagcttactattccaacaagatgccagatatttctggaatcagggtaagctagtggtccaccagaatcattctgacatgcatcagcttctcctgacataaatccagcacataacattgtatcagtcacaaagccagagtatgcatatgaggcattgcaaattttgttgtcaataatcttcaaaaagtcttcttgaagtatcactggaaatgaaccattcatataaagtgttccccaacctgtaactacaacattgtcattttctgagagcttcattttggcttcaggaagacaaatcttacgaatgtactctgtaaaagaaacttcttcagcaagctgcacaagggcaatatcatcatgaagcccaggactgctataattttcatgaaaaataatgttttggactttccgtgtcatatatggtttatttactacaattccaaagttgacagtccaatcttttgaattatttttcttagcaaagcagtgagctgcagataatagccacctgctgctgatcagagaggctccacagtagtgacggcctttccattgcatgctggcctgccatggccatgccccctccagggagctttttccattcacaattttgttgccagttatgatactgttggctacttgtctcccacaacagttgttggtaagcatttcagaagcagccttgctgatttccatgagtttaatggaagcaggaactgcattccaggatgccatgttgtttttcaacatctgatgtaatttagccttgattttagtcctcatgctaactccttctgctggaggaaacttgaatttcagctgtaactgcacatttgaaccattggcattaggcagaagtttgatgacctcagatttgacatattccttatatatactggaattttgaaatgcatttaacatcttagtctcaatatctttgcttagatttgtgctggcttgtgaagctgcgttttcacaattatcattgtatgtgactccagaaatatgaaaatcaccttgataatagtaagtcttctcaactgccagaaaatgaacaagaagaccaatggttactcccaagattgccgccactccaagaaaaataaagatcgtagtccatagtggccaagatctttgggaagatatgccgtgcctgtacataatgttctgattgttatggcagtatcaggtataacggtggtaatgatgatgacgaagataacgataacgatgacaatgctggtaatagtgatgacaaaagttagaaccttctgacgcagcttttgacttatgtgct

SEQ ID NO: 14899 - RNA, 1577 nt, Homo sapiens
  source 1..1577: mol_type = other RNA
gctgggattacaggcatgagccactacacctggctaagaatttactttgtatacatgttaaaaaaaaaaaaaacctaatatgtattaactcctaacacctaagaggaaacctctggtaaaaagagtctttcactccaaggacacggcagagcctgtgccatcttctaagtagatgaactttccagagtccaccaagaggtcctgaatcttctctcttgcatgtctctcttccatcctctccaaggcatccagcagggtgtggatcgaggcgttccgtccagttttgttgacccatttcatcagcattgcatacaaggcatcccctgggcctgctgtaccagctctgaccacatcgatctcatttttcgtgaggtccagctgcctcatgagctggtcccaggagtcaaagggcacgatgtttgcaaacttgtcaaagaacagcatcagagtctcagtggggtcagcaccatttgctggaaccagcagcctcctcctctgagacccttcagcttctgccggtcccagcagacactgtgcctcccctggggactgtacagtgacacctgtcaaatctgccggctcctggctttccatttgctgctcagagacgaaagtggacagcgagtctgcgttgctcagaatctcgttgtgagcattgtcctcagccccaggccctcgtaggagacccaagcgccagaaacacaccctgtccatgcacttggggtcccctccacaacctgagccgatgcaacaacagacaatcagcacagccaccaacagcaacggaacaaccaaagtcacaaccaaaatcacccatatattatgtccattgcctgattctttgtggacacactcgatgtcactccagggcgtacaatccttgaccttgaccatccctctggggcaccctctgctgcacttccggcacatctcagcagaattgtcattccggaaagttcctggtttgcactgacatgctgtgttcctggtcgtggtgcagggacttctctcttcttcatctgatttacaagctgtacatgggaggcaagcaaacaaattgttggaagcattggtgtaacccacaccctctgtgcaccggttacaggctccaggatgttctgatctatgagatcctggtggacacaactctcccaaagggctatgttcccattgctgtgtgccaattgattgatcatgaagtttgatggttgcagctgagctaggtacgacctgcagcaggaccccgacgacgacaaacttgaaggtcttgtggacccggagccgagggctggcttcccgcgccggcctgggtcctggggcgcgccctgcccgggcccgggcactgggtccgtgctgtcccatggaggtagggagcgctcctcggcccccgcctcgtggttcaatcctccccgcggaagagccccacactttgctgggtgtggccgcggctgcctctgtcccactcgctgcgctcccgggattcggagtcactgccaggaacgcacctagatgtactctagctggtggtggcgccatcctgccaggtcaatccaagaagcagcgtgcttggctatgac

SEQ ID NO: 14900 - RNA, 1418 nt, Homo sapiens
  source 1..1418: mol_type = other RNA
gctgggattacaggcatgagccactacacctggctagcctgttcttaagaggggtataaagaggagttgtgtgtcagctcagagtaagttcaggtcaaagtttgggagcctgaggaaggaaagaaacttagacaaagtttggttaacaagtattttgttctgaccactgaagacaaacttattatttaattgtttatgagacccccaaaaaagggaatttagagtctgtggctttgtgatatcaaaaacaggaaagatgtttctttgcagtaaatgctcttggaaaacacaaaggatgggggatttctttaatcacagctgttgctgttacctacccaccccattcccccccaccgctttttcttgccatttacatttcttccatttggctgttcctgacttgtatctttataataaactggtaaatgcatgtatagtgttttgttgagttctgtgagtagttatattaagttattaaacttgaggagcaggttatgggagcccccaatttataggcagtagctcagaaggatagatgggcccctaataatcgcagctgggatctgcagtgggggcagtgttgtgggactgagccctgaacttttggcgtctgcgttgactcaggatggtatcagaattgagttattattggacaaccaattggtgttggagaattggttgctgttaaaactctatacatttggtgtcaggaaaaaatatcccaggggtttaggcaggagggaaactctgttcccctgcacacagtctgtcacaatgcacattgtcctgtgattccagatctcctctcagggtaaaaggggactgaggacttagaagaaaggagttctgagaacagaccccctgcccccaacctgctaccacacgattctcacctacttatgaacatacccactaggaatagatgtggccacaccctccacaaaacaagacttgactatcaggaattatgtttatagggcctttgcacctagaattgctcaccaaaaaattcacacaagttcctagaggactcctggctctttcctacccttgatcctcaaacagcagcagcaacctttccctccatccacctagacctgtggaccaccagtcataatctcatctgcatcatctaggtattgaatgcagtgatatgtcacaatctccttttttcggcatggcccaggcagaagtggtcagtcacatcaccttgatgttggactcagccatgtgtcataatacacagtatatccagggctcaggcagaagagaagagtcacatcatctagttgctggtccaattatatgttgcaatcacttgttttggcagaacctggagcgcagtccgtttgcagccggcggcaggtgaggtttcagcgcgggtagccagcggggttgaggcctggggggagcggagc

SEQ ID NO: 14901 - RNA, 1798 nt, Homo sapiens
  source 1..1798: mol_type = other RNA
gctgggattacaggcatgagccactacacgtggcgttttgaatcctcttctgtacaaagatacaatctgagtccttaggacatttatagcctaatattttcttccatcaaagttgctaaaccccatcaccagaataccacaattaatattctcaggatagattattaatagttgcctaggaataagaatggtatgtggcaatgatagaaatttgaaatggcagatttattaagtatttttaagccatcaagttacaaaaggctattaggggtcttaaaaagacaaagagtatacaataaaacaataagcaattacagattgttttaggttgaacaatttttgtacagttatatctatagtacattactaatttacttagcaaactttatcctgagatttgcaaatttaaaaaaatgaagaatcaaactatattttcttttctgtttttttgaaacagagtctccactctgtcatccaggctggagtacagtggtgtgatctcagctcaacatagcctcaacctcttgggttcaaggaatctcgtgcctcagcctcccaagtagctgggattacaggcatgcaccaccgtgctcggctaattttttgtatttttagtagagatggggtttcaccatgttagccaggctgctctttaactcctggcctcaagttgatatgcctgccttggcctcccaagtactgggattacaggcgtgagccaccgtgcccggcctcaaactatattttctaattagtacagtaaatacacattaatcatgacacaattatttcttctggatacagcaggaaaaattaagttaagagaaagtgcttcatatttcttgatttgttataaaaaggagagatcctctagatttctgggtaagagggaaagctagcaatcccacaatgatttcctttatttcttgccatccgaatatatccttcttcaccaaagttgtggccccagctgtttttcacaagccagtattctttcccattaagatcaccatagccaaccacaagtacaccatgattcacattctgagtacaggatggttcatagtagacaccacttctgtagaggaagaaagaaggatgacgcgcatctacaccaacagacactgggcctttattggccacagcttctttcaggacatcttctctgccataaggaagttcagtgtactttgaacatgtggcagcacgatattttgagtcatattgacatttctgatccatggctttgtagggataggaagcgtctgagtcgatgcccttgttatcaatgatgtactggaaagccgttgtcatgaagccaccattgcagcctttgtttccatatttttcagttgagcaatccaccaggttctgggcactgagagacaccagctttcctgttttcagcttcagctgtgcttccagggcccccacagcactgaaagcccagcaagcaccacaagaacccatgtctcccaggtggttcatgcccagatcgtatgagtgcattcccattgaatgctccaggttgtgaagcatcacaaactttagattcttttcccagatgagacgtcgtactgcttcttcattcttttccttgtattgtttgccataggttttcttccagagatgccagtggtgatccagggtaggatctttatgcaactgtgccactgcagaggagcacaccaagagcacacaaaccagccgtttcattgtgatagaaccagcagttgctcccacagtaagagtccttgaattagtgggctctcttctaagatttcaaagcaacaaggag

SEQ ID NO: 14902 - RNA, 1948 nt, Homo sapiens
  source 1..1948: mol_type = other RNA
gctgggattacaggcatgagccactacacgtggcgttttgaatcctcttctgtacaaagatacaatctgagtccttaggacatttatagcctaatattttcttccatcaaagttgctaaaccccatcaccagaataccacaattaatattctcaggatagattattaatagttgcctaggaataagaatggtatgtggcaatgatagaaatttgaaatggcagatttattaagtatttttaagccatcaagttacaaaaggctattaggggtcttaaaaagacaaagagtatacaataaaacaataagcaattacagattgttttaggttgaacaatttttgtacagttatatctatagtacattactaatttacttagcaaactttatcctgagatttgcaaatttaaaaaaatgaagaatcaaactatattttcttttctgtttttttgaaacagagtctccactctgtcatccaggctggagtacagtggtgtgatctcagctcaacatagcctcaacctcttgggttcaaggaatctcgtgcctcagcctcccaagtagctgggattacaggcatgcaccaccgtgctcggctaattttttgtatttttagtagagatggggtttcaccatgttagccaggctgctctttaactcctggcctcaagttgatatgcctgccttggcctcccaagtactgggattacaggcgtgagccaccgtgcccggcctcaaactatattttctaattagtacagtaaatacacattaatcatgacacaattatttcttctggatacagcaggaaaaattaagttaagagaaagtgcttcatatttcttgatttgttataaaaaggagagatcctctagatttctgggtaagagggaaagctagcaatcccacaatgatttcctttatttcttgccatccgaatatatccttcttcaccaaagttgtggccccagctgtttttcacaagccagtattctttcccattaagatcaccatagccaaccacaagtacaccatgattcacattctgagtacaggatggttcatagtagacaccacttctgtagaggaagaaagaaggatgacgcgcatctacaccaacagacactgggcctttattggccacagcttctttcaggacatcttctctgccataaggaagttcagtgtactttgaacatgtggcagcacgatattttgagtcatattgacatttctgatccatggctttgtagggataggaagcgtctgagtcgatgcccttgttatcaatgatgtactggaaagccgttgtcatgaagccaccattgcagcctttgtttccatatttttcagttgagcaatccaccaggttctgggcactgagagacaccagctttcctgttttcagcttcagctgtgcttccagggcccccacagcactgaaagcccagcaagcaccacaagaaccttgatatttcacttcagtaacacaccctttctctctccagtccacagaatcaggcaatatccgattagggtttgacttatatgtgatatttctctgccactggctgggaactctcagggaactcatcaaagacatcacttcttcactggtcatgtctcccaggtggttcatgcccagatcgtatgagtgcattcccattgaatgctccaggttgtgaagcatcacaaactttagattcttttcccagatgagacgtcgtactgcttcttcattcttttccttgtattgtttgccataggttttcttccagagatgccagtggtgatccagggtaggatctttatgcaactgtgccactgcagaggagcacaccaagagcacacaaaccagccgtttcattgtgatagaaccagcagttgctcccacagtaagagtccttgaattagtgggctctcttctaagatttcaaagcaacaaggag

SEQ ID NO: 14903 - RNA, 7965 nt, Homo sapiens
  source 1..7965: mol_type = other RNA
gctgggattacaggcatgagccactacacttggcctttgaaacttacttttacaaaagatagttcatttctctcctgggaagaccagcgaacatcctctggtttggagggcctccagctctctccatattctgagccaaggaaaagctggctaaagaattgaagtctgttgtgtccccacagggtcctcttgttaaaacctgcagtggtcaattgtgactgcacagactagaacttcacagatgggttaatcccactttcacattgtggatctttgactgtcacatgaaagaccaggtgacacaagacacatctgaagctctatttccttgctattttgaacattattttaagggagaacgaaagtcctttcattgtcagtccaggtttatttagatggtgtcttggtcagctttcagagcctaggtcacattgttcatattcttgactttttgctctcttagctagcatgacaggttgggatgaatttccctctttcctcaaagtctggtgactgcatccagtctctaaggatgtgatgctacccatggcccttttctgacttcgagattggacaggccagtcacacttctatttattgggtatatataaaacccactccagtgaacagaactgagccccatgaaggcaggaactacactgtgtgtagtgtctcatagttgtggttagttaatatttttgacaaattgacctgcaggctcacctactctaaaacaaaagacatactttacctttgcctaccaaagtttgacttgaaagcttttaagtttgtctggtctgtcaggtgaaaagccactcagtaaagtcaaacagatacacctcttagatcttggaatatggcccacagaaatggattcttctggagccagagtacctcaagatgttggctttcctgagggttttagtattatatatacttgtatttttaaaaatccatctctgtattcatggaattctttaatatctttggctgttgttaaaagcaagaattggccaccctgagggtttgtagactagttttggcctgtgacaggaatcctttttaattctagctttgtttatgaactagatgtagtttgtctcaaattaattctcgatgttgaaaacactgaggacagattcttgagcagaattaccagttataagcctggaaggtgaggtggtggacacccaaatccgagctactagcttggttcagtcttcttaaagcacaaaccattttcaacatcctattctttatttctaatgaggtaaaatatggacatgttctagcccttcttctaagcttgatattttaaaggtttggtaccactttggttaagctagaaaaacaaaactttttttccttcgtaagtgtagagttctgtgagttctgtcaaacatgtaatcaatcaatcatcagcagtcaagatattgaagtcacaccacccctaaaaattccctcatgtccctttgtaattaactcccattcccagctcaggaggccattgatgtgtttgccttccctgtagtttttcctattcctgaatgctatataaatggagactgtttttttaagagacagggtcttgctatgttgcccaagtgcagtggctgttcagacattatagcatactacagccttgaactcctgggctcaggcaatcctctcacctcagcctcctgagtagctgggactacaagtgcatgccactatgcccagctaatggaggcttttgagtctggctttttatttagcatgatgcttgagacttatccatattatcagtagttcattattttattcccaagaagtattgcattgccatggatgtacaaatttattcattcaccaggtggaaggctacttcactgaattcagtttttggtgattatgaataaagttgctatattcacatacaggtttgtgtgaatatgttccttcacttgggtaaatacctacgaatgggattgctttgtcacagattattagaaaatggatggattgttttttaaactgcctgtgcacctttgcagttcctccagcaatgtatgagagttcaagttgctctgcatcgtaagcagaatttggtatattcagtttcaataggtgtatgccattttggttttaatttacattttcttaatgatttatgatagtattttcctgtgttcttatggcatcaacttcttttgcaaagtgtcttcaaatattttacccatttaaaaatcgttttaacagatctcatcttattaccttgctggacatttcatctcagtagtttcattactccaagttaggtctttctgtgtgccttttttttctggctaaaattatgttacttcctttggtcatcctgagcaagtgtgtggcctctattcagatatatgcctctgttaaaggcattccacacagatccagcataatgattgagttttgcttctcacctttgttctctccacccagtaaggtgtggagctgttaataaagttcattattttattggccaagattattgatgctcataggttgaagaacccatgacattcacatgagtttgtatgttcctgtttataaactctacttgttcaaagtgtcattaatattcttgagaaactggcagttttattatgaaggatatctgcaattcatagcaattactcctttttaacctagagacactgatttaacttaataaaacctgtttataggatgaaacttgtagctcagtcttaccaaggatttaaggattcatatatgagtgtttttctttctcctttacacctagttaattaaccttgtatcttatgtctcacttgctgactcttcagaccttttttttttggaacaaaaagcagctgcgtgtaaattacgacagcaactgaattttccatgaatcatattcacttttctgaaggcaactctgcatgcagttacagaaatgtcctactggggctcctcctttgcctacttcaattttaagaattctgaggtcaggagaggtaatagggcacacacctaatttgttaattaagcaaggattctaatgatatatcacatactcaaatcctggattttccctaaaatatgattattatattgggaatttgaaaacatgttgagcagtggtaaagtacatgacacactagaagccaaaaatcagaaccctacatttaaagttcataataaaagatccacccgagtataaccaataatatttggtttagatattttatagcttttctacctttttaggaaatttagagtgttttattaagttgaccagaagtgtggtattatcaatattattttgaaactattcaaaaattcctactggttaaaaagcttttttttttttttaaattgtgctgaggctatgccattttctccctctctgaagaaagtatgtaccttttagatacagattaacagtaacaaatggccactgagcactgctttttttcctttatggaaacttctcatgttcatgcagactagctacaacagcttcttaaaaaaagatactttttggccaccaaactacctctttggcatccaaggtaatgcaggaaaactttgacccaaagtattcccatatattatttgcattaagcatgtcacttatgaaatgagaagtgatctcaaggattttagtgctgaatcctcaactaaaattttatttccttgtgctgaatagaacacatacagatccatattaaaaacagtcatcatattaggcaaattcaatctgtcaatgtagttttagtccagaaccaaaccagtgatagttaggaattacagagttaccaaccaaactgatttgctttcctggtggttctttgtgtaacagatgagagaaataaagtggcagagtaccagtgaacatttggagaaaatacctaattattttcttcctaacccaagttagccactgaatagtcatctcagaatagtcacctcatcccagttggcccattaggttcctgtgtgcttcatcttctgtgagaaaaaaaaaccttatatcattccttatttcagatgtaagatgccaggtgagttattttccacaaatttcttaagctcattactggaaaaaaaaatttctcaaaacttttagtaatgaatgagtgtacaagcagcaattggatattaatcccatggtgcaaggatttcctgcaaagtacctttaatgtgtttaaatcagcagcaagcattaggacatgctattttggccccataagttaggtgtgtagcactacacattagacaccaagtcatcccaaccaatatttatccatatgaacagataaactgaacaaaaacatagttctgataaaacctgcattcacaacctaatgtagtttaaagtaaattttttcacaattgagggctgctatttaggactgttttgttaataataaaaacaggaattatatagaagataaaacaccattttttactgctatataatgtcttgctatataaaacataccctcaacaagtcaaaatatttaaaaccagtgtttcaaataccaaaaatcacagctatgttactgttcagtaactccactcaaataaatgttagtactgcattcttgaaggaaaaaaactgcagccaaggcaagaactctgaagtttgcactcagagtttaaaagacagacccctactctgcaaactgaagactgccactctgcttcaataactccagcctgccacattttacttcaattggtaaagcactctgctgagaatataaaaagttataaaaaggcaatcataaaagattaaatattggtaggcatgtaagcttccttttaataaaaacaaaaatagtcaatgtcatctatttaaataagtatcctttgttatagagtgttccagttattgaaaaagggcccttaaaaaacccaactgtctacatctttaaaccctaccccttttaccccatagtacacatttgagggaagagtcatttaatgtgcaaattggcaaaacaaatgtggaggagaggggacttcttgaaatgatgtgcccaatcaattcttggtttattcttttccaaaaagtaaaataaccaaagtcttaaaagtacacaaaacagaccttcatctttgcattcctttccaaataaacccaaaaagtatgtacagcatgtttaatagtatgcaatatgcaaaagctttgtgttgctgttagcaacatctatacccacccaccctctttattcacaagtgtacctctactaaccataattacatcactaagcctgttagtttgagagggtcttaaatttgttaaaactggaaaatctttgtataggggctccattcatttgactcaaggttatagacttccaccgtattcagaaattcattgccatcgaatcctcccactgcataaatggtgttccctacagttgcaatcccagcattgctccttggtgaagtcatatttcccatcatcttccattcatttctagttggatcatacatttccacacaactgatggcatgagaaccatcaaagccaccacatacaaacagttttccattaagaacagccactccagctcctcgcctagccacattcatgggtgcaattaaagtccaggtattattttcaggattgtatcgttctactgtgttcagacaattccaagattctgcacctccgattatgtacaaataaccaccaagctcacagactgcagactggtgtctccgaatgttaagaggggcacagcttgtccacaactttgttacaggatcaaatacatcacaatttttcagtcctttttgaccatatggatcagagccaccaacgatgtataactttccattcagagcacacactcctgcattacaacggttagttctcaattctggaacaggaatccagtcatctatgtttgaatcatacatctctccacaactcaggtcatctgagtggccatttgatccacctaccacatagagctggcccatgagtacagccatttgaaatcgggctcttggtgttctcatgggagcaagaaaggaccagtgatctgtatgtggattatagcattcgactgttcgaagacattcctctctgttatagccacctgcagctatgagtttgccattcatctctgctgttcccagaccagatcgtgcgtactgcataggagacatgggcttttcgattagctcatcttgttgcatctcaaagcttaaactcttacttagttttggagtacttgttggtgagctctgtgggctgtttctcccatgaagaaaaatgacacagaatataccatccagcacagccaggcacaagtaagtgttatttgaagtcttttctgaagcaacgattttccactcatgcttagggctttgtactgtagcatttggagaagagagacatccagttgaactgctacttatctgcttatggccattctcacgtggtggctttttctcagactgtgcaatgtgtacctgcacaaactgaatgtggtcatcatcactgccaaacacctcagcctgtccatctagtaggttcccatcaagcagcttgtgatcagctgagtagtacaaggtttgaaccattaaatcatcatcgttctctgcccacagcggatttttcttaggagaactggggcaggactgctgcttctttacgtgtcaatacacttgaggtttcttcttgtttcttcagtcttgggtatcctagttttgttaataaacctcttccatcagctcttccagactgtctccattctcccagatgctacgctgcacccagttgattacctttgtatataatttgccattgctgggcaagcaaacattatcttcaagcattacctccaactttagccttggaagcttaagaaactcctcctcttcagaaatttgtaacaaatgctcctgaatataagcatcaaccttattcaacaaacgggagtctcccatacaacttgcaaaatttcggtaagagatgcagctggtaacatccattctagacagtaaataatcaccacaaacctgctttactcgatccatcttcagcttttttgctgcagaataaacatcttttaccaattccttatctgctttcaactgagcagtgtaggcataattcaacaagacttcaacagcttctggattgagatcatcaaatttaacgtgagaaattccatgaggatcactatcactattaaagatttcaaataaatagggactgcagcaagctagcactgctctgtgtgctaacatttcatggccacagacctgaagtcgaacatcacagaactggccacttttcctcagggcatttaatttggcaacagaagactcaataaaattttcatcctcaaacatcaaatatccattgggaatcatttttccttataaatttggctactctgttggtggcaaatgtatttctgggaactcttaagtaatccaaggacaaaggagtgttaaaaggtgcacttcgtcagggtatgaagacaggtggttgaaatgaaggcaggtgtgtcttaagctctaatggtgattccaaaactatcaggcttgaaaatgatgtaatcaagtccttaaaagctatagacacgaatttcttctgtgataatgatgcatcataatctggttcatctctgaagagatggaaacattcatttctagagcttcgatgggaagcaggaggaagcgggcgggaatcggcccaacggaaagcgccagaaggcggcggaagacgggagcggtcaagtagaaggacgaggggccagtccgtggagactgaaaggaagggggagcgccaccgagaactcgcgggaactcgctcgctcgccgatacagccgcgccgaagcagcaggcggagaaactgcgcccagcagctctgagcgaccgacctccacgcgcgaccgggagacactgcctccgccgccgccgaccgctcgcgccgcaccccctcgcac

SEQ ID NO: 14904 - RNA, 7661 nt, Homo sapiens
  source 1..7661: mol_type = other RNA
gctgggattacaggcatgagccactacacttggcctttgaaacttacttttacaaaagatagttcatttctctcctgggaagaccagcgaacatcctctggtttggagggcctccagctctctccatattctgagccaaggaaaagctggctaaagaattgaagtctgttgtgtccccacagggtcctcttgttaaaacctgcagtggtcaattgtgactgcacagactagaacttcacagatgggttaatcccactttcacattgtggatctttgactgtcacatgaaagaccaggtgacacaagacacatctgaagctctatttccttgctattttgaacattattttaagggagaacgaaagtcctttcattgtcagtccaggtttatttagatggtgtcttggtcagctttcagagcctaggtcacattgttcatattcttgactttttgctctcttagctagcatgacaggttgggatgaatttccctctttcctcaaagtctggtgactgcatccagtctctaaggatgtgatgctacccatggcccttttctgacttcgagattggacaggccagtcacacttctatttattgggtatatataaaacccactccagtgaacagaactgagccccatgaaggcaggaactacactgtgtgtagtgtctcatagttgtggttagttaatatttttgacaaattgacctgcaggctcacctactctaaaacaaaagacatactttacctttgcctaccaaagtttgacttgaaagcttttaagtttgtctggtctgtcaggtgaaaagccactcagtaaagtcaaacagatacacctcttagatcttggaatatggcccacagaaatggattcttctggagccagagtacctcaagatgttggctttcctgagggttttagtattatatatacttgtatttttaaaaatccatctctgtattcatggaattctttaatatctttggctgttgttaaaagcaagaattggccaccctgagggtttgtagactagttttggcctgtgacaggaatcctttttaattctagctttgtttatgaactagatgtagtttgtctcaaattaattctcgatgttgaaaacactgaggacagattcttgagcagaattaccagttataagcctggaaggtgaggtggtggacacccaaatccgagctactagcttggttcagtcttcttaaagcacaaaccattttcaacatcctattctttatttctaatgaggtaaaatatggacatgttctagcccttcttctaagcttgatattttaaaggtttggtaccactttggttaagctagaaaaacaaaactttttttccttcgtaagtgtagagttctgtgagttctgtcaaacatgtaatcaatcaatcatcagcagtcaagatattgaagtcacaccacccctaaaaattccctcatgtccctttgtaattaactcccattcccagctcaggaggccattgatgtgtttgccttccctgtagtttttcctattcctgaatgctatataaatggagactgtttttttaagagacagggtcttgctatgttgcccaagtgcagtggctgttcagacattatagcatactacagccttgaactcctgggctcaggcaatcctctcacctcagcctcctgagtagctgggactacaagtgcatgccactatgcccagctaatggaggcttttgagtctggctttttatttagcatgatgcttgagacttatccatattatcagtagttcattattttattcccaagaagtattgcattgccatggatgtacaaatttattcattcaccaggtggaaggctacttcactgaattcagtttttggtgattatgaataaagttgctatattcacatacaggtttgtgtgaatatgttccttcacttgggtaaatacctacgaatgggattgctttgtcacagattattagaaaatggatggattgttttttaaactgcctgtgcacctttgcagttcctccagcaatgtatgagagttcaagttgctctgcatcgtaagcagaatttggtatattcagtttcaataggtgtatgccattttggttttaatttacattttcttaatgatttatgatagtattttcctgtgttcttatggcatcaacttcttttgcaaagtgtcttcaaatattttacccatttaaaaatcgttttaacagatctcatcttattaccttgctggacatttcatctcagtagtttcattactccaagttaggtctttctgtgtgccttttttttctggctaaaattatgttacttcctttggtcatcctgagcaagtgtgtggcctctattcagatatatgcctctgttaaaggcattccacacagatccagcataatgattgagttttgcttctcacctttgttctctccacccagtaaggtgtggagctgttaataaagttcattattttattggccaagattattgatgctcataggttgaagaacccatgacattcacatgagtttgtatgttcctgtttataaactctacttgttcaaagtgtcattaatattcttgagaaactggcagttttattatgaaggatatctgcaattcatagcaattactcctttttaacctagagacactgatttaacttaataaaacctgtttataggatgaaacttgtagctcagtcttaccaaggatttaaggattcatatatgagtgtttttctttctcctttacacctagttaattaaccttgtatcttatgtctcacttgctgactcttcagaccttttttttttggaacaaaaagcagctgcgtgtaaattacgacagcaactgaattttccatgaatcatattcacttttctgaaggcaactctgcatgcagttacagaaatgtcctactggggctcctcctttgcctacttcaattttaagaattctgaggtcaggagaggtaatagggcacacacctaatttgttaattaagcaaggattctaatgatatatcacatactcaaatcctggattttccctaaaatatgattattatattgggaatttgaaaacatgttgagcagtggtaaagtacatgacacactagaagccaaaaatcagaaccctacatttaaagttcataataaaagatccacccgagtataaccaataatatttggtttagatattttatagcttttctacctttttaggaaatttagagtgttttattaagttgaccagaagtgtggtattatcaatattattttgaaactattcaaaaattcctactggttaaaaagcttttttttttttttaaattgtgctgaggctatgccattttctccctctctgaagaaagtatgtaccttttagatacagattaacagtaacaaatggccactgagcactgctttttttcctttatggaaacttctcatgttcatgcagactagctacaacagcttcttaaaaaaagatactttttggccaccaaactacctctttggcatccaaggtaatgcaggaaaactttgacccaaagtattcccatatattatttgcattaagcatgtcacttatgaaatgagaagtgatctcaaggattttagtgctgaatcctcaactaaaattttatttccttgtgctgaatagaacacatacagatccatattaaaaacagtcatcatattaggcaaattcaatctgtcaatgtagttttagtccagaaccaaaccagtgatagttaggaattacagagttaccaaccaaactgatttgctttcctggtggttctttgtgtaacagatgagagaaataaagtggcagagtaccagtgaacatttggagaaaatacctaattattttcttcctaacccaagttagccactgaatagtcatctcagaatagtcacctcatcccagttggcccattaggttcctgtgtgcttcatcttctgtgagaaaaaaaaaccttatatcattccttatttcagatgtaagatgccaggtgagttattttccacaaatttcttaagctcattactggaaaaaaaaatttctcaaaacttttagtaatgaatgagtgtacaagcagcaattggatattaatcccatggtgcaaggatttcctgcaaagtacctttaatgtgtttaaatcagcagcaagcattaggacatgctattttggccccataagttaggtgtgtagcactacacattagacaccaagtcatcccaaccaatatttatccatatgaacagataaactgaacaaaaacatagttctgataaaacctgcattcacaacctaatgtagtttaaagtaaattttttcacaattgagggctgctatttaggactgttttgttaataataaaaacaggaattatatagaagataaaacaccattttttactgctatataatgtcttgctatataaaacataccctcaacaagtcaaaatatttaaaaccagtgtttcaaataccaaaaatcacagctatgttactgttcagtaactccactcaaataaatgttagtactgcattcttgaaggaaaaaaactgcagccaaggcaagaactctgaagtttgcactcagagtttaaaagacagacccctactctgcaaactgaagactgccactctgcttcaataactccagcctgccacattttacttcaattggtaaagcactctgctgagaatataaaaagttataaaaaggcaatcataaaagattaaatattggtaggcatgtaagcttccttttaataaaaacaaaaatagtcaatgtcatctatttaaataagtatcctttgttatagagtgttccagttattgaaaaagggcccttaaaaaacccaactgtctacatctttaaaccctaccccttttaccccatagtacacatttgagggaagagtcatttaatgtgcaaattggcaaaacaaatgtggaggagaggggacttcttgaaatgatgtgcccaatcaattcttggtttattcttttccaaaaagtaaaataaccaaagtcttaaaagtacacaaaacagaccttcatctttgcattcctttccaaataaacccaaaaagtatgtacagcatgtttaatagtatgcaatatgcaaaagctttgtgttgctgttagcaacatctatacccacccaccctctttattcacaagtgtacctctactaaccataattacatcactaagcctgttagtttgagagggtcttaaatttgttaaaactggaaaatctttgtataggggctccattcatttgactcaaggttatagacttccaccgtattcagaaattcattgccatcgaatcctcccactgcataaatggtgttccctacagttgcaatcccagcattgctccttggtgaagtcatatttcccatcatcttccattcatttctagttggatcatacatttccacacaactgatggcatgagaaccatcaaagccaccacatacaaacagttttccattaagaacagccactccagctcctcgcctagccacattcatgggtgcaattaaagtccaggtattattttcaggattgtatcgttctactgtgttcagacaattccaagattctgcacctccgattatgtacaaataaccaccaagctcacagactgcagactggtgtctccgaatgttaagaggggcacagcttgtccacaactttgttacaggatcaaatacatcacaatttttcagtcctttttgaccatatggatcagagccaccaacgatgtataactttccattcagagcacacactcctgcattacaacggttagttctcaattctggaacaggaatccagtcatctatgtttgaatcatacatctctccacaactcaggtcatctgagtggccatttgatccacctaccacatagagctggcccatgagtacagccatttgaaatcgggctcttggtgttctcatgggagcaagaaaggaccagtgatctgtatgtggattatagcattcgactgttcgaagacattcctctctgttatagccacctgcagctatgagtttgccattcatctctgctgttcccagaccagatcgtgcgtactgcataggagacatgggcttttcgattagctcatcttgttgcatctcaaagcttaaactcttacttagttttggagtacttgttggtgagctctgtgggctgtttctcccatgaagaaaaatgacacagaatataccatccagcacagccaggcacaagtaagtgttatttgaagtcttttctgaagcaacgattttccactcatgcttagggctttgtactgtagcatttggagaagagagacatccagttgaactgctacttatctgcttatggccattctcacgtggtggctttttctcagactgtgcaatgtgtacctgcacaaactgaatgtggtcatcatcactgccaaacacctcagcctgtccatctagtaggttcccatcaagcagcttgtgatcagctgagtagtacaaggtttgaacctcttccatcagctcttccagactgtctccattctcccagatgctacgctgcacccagttgattacctttgtatataatttgccattgctgggcaagcaaacattatcttcaagcattacctccaactttagccttggaagcttaagaaactcctcctcttcagaaatttgtaacaaatgctcctgaatataagcatcaaccttattcaacaaacgggagtctcccatacaacttgcaaaatttcggtaagagatgcagctggtaacatccattctagacagtaaataatcaccacaaacctgctttactcgatccatcttcagcttttttgctgcagaataaacatcttttaccaattccttatctgctttcaacctgaagtcgaacatcacagaactggccacttttcctcagggcatttaatttggcaacagaagactcaataaaattttcatcctcaaacatcaaatatccattgggaatcatttttccttataaatttggctactctgttggtggcaaatgtatttctgggaactcttaagtaatccaaggacaaaggagtgttaaaaggtgcacttcgtcagggtatgaagacaggtggttgaaatgaaggcaggtgtgtcttaagctctaatggtgattccaaaactatcaggcttgaaaatgatgtaatcaagtccttaaaagctatagacacgaatttcttctgtgataatgatgcatcataatctggttcatctctgaagagatggaaacattcatttctagagcttcgatgggaagcaggaggaagcgggcgggaatcggcccaacggaaagcgccagaaggcggcggaagacgggagcggtcaagtagaaggacgaggggccagtccgtggagactgaaaggaagggggagcgccaccgagaactcgcgggaactcgctcgctcgccgatacagccgcgccgaagcagcaggcggagaaactgcgcccagcagctctgagcgaccgacctccacgcgcgaccgggagacactgcctccgccgccgccgaccgctcgcgccgcaccccctcgcacgtcacca

SEQ ID NO: 14905 - RNA, 7824 nt, Homo sapiens
  source 1..7824: mol_type = other RNA
gctgggattacaggcatgagccactacacttggcctttgaaacttacttttacaaaagatagttcatttctctcctgggaagaccagcgaacatcctctggtttggagggcctccagctctctccatattctgagccaaggaaaagctggctaaagaattgaagtctgttgtgtccccacagggtcctcttgttaaaacctgcagtggtcaattgtgactgcacagactagaacttcacagatgggttaatcccactttcacattgtggatctttgactgtcacatgaaagaccaggtgacacaagacacatctgaagctctatttccttgctattttgaacattattttaagggagaacgaaagtcctttcattgtcagtccaggtttatttagatggtgtcttggtcagctttcagagcctaggtcacattgttcatattcttgactttttgctctcttagctagcatgacaggttgggatgaatttccctctttcctcaaagtctggtgactgcatccagtctctaaggatgtgatgctacccatggcccttttctgacttcgagattggacaggccagtcacacttctatttattgggtatatataaaacccactccagtgaacagaactgagccccatgaaggcaggaactacactgtgtgtagtgtctcatagttgtggttagttaatatttttgacaaattgacctgcaggctcacctactctaaaacaaaagacatactttacctttgcctaccaaagtttgacttgaaagcttttaagtttgtctggtctgtcaggtgaaaagccactcagtaaagtcaaacagatacacctcttagatcttggaatatggcccacagaaatggattcttctggagccagagtacctcaagatgttggctttcctgagggttttagtattatatatacttgtatttttaaaaatccatctctgtattcatggaattctttaatatctttggctgttgttaaaagcaagaattggccaccctgagggtttgtagactagttttggcctgtgacaggaatcctttttaattctagctttgtttatgaactagatgtagtttgtctcaaattaattctcgatgttgaaaacactgaggacagattcttgagcagaattaccagttataagcctggaaggtgaggtggtggacacccaaatccgagctactagcttggttcagtcttcttaaagcacaaaccattttcaacatcctattctttatttctaatgaggtaaaatatggacatgttctagcccttcttctaagcttgatattttaaaggtttggtaccactttggttaagctagaaaaacaaaactttttttccttcgtaagtgtagagttctgtgagttctgtcaaacatgtaatcaatcaatcatcagcagtcaagatattgaagtcacaccacccctaaaaattccctcatgtccctttgtaattaactcccattcccagctcaggaggccattgatgtgtttgccttccctgtagtttttcctattcctgaatgctatataaatggagactgtttttttaagagacagggtcttgctatgttgcccaagtgcagtggctgttcagacattatagcatactacagccttgaactcctgggctcaggcaatcctctcacctcagcctcctgagtagctgggactacaagtgcatgccactatgcccagctaatggaggcttttgagtctggctttttatttagcatgatgcttgagacttatccatattatcagtagttcattattttattcccaagaagtattgcattgccatggatgtacaaatttattcattcaccaggtggaaggctacttcactgaattcagtttttggtgattatgaataaagttgctatattcacatacaggtttgtgtgaatatgttccttcacttgggtaaatacctacgaatgggattgctttgtcacagattattagaaaatggatggattgttttttaaactgcctgtgcacctttgcagttcctccagcaatgtatgagagttcaagttgctctgcatcgtaagcagaatttggtatattcagtttcaataggtgtatgccattttggttttaatttacattttcttaatgatttatgatagtattttcctgtgttcttatggcatcaacttcttttgcaaagtgtcttcaaatattttacccatttaaaaatcgttttaacagatctcatcttattaccttgctggacatttcatctcagtagtttcattactccaagttaggtctttctgtgtgccttttttttctggctaaaattatgttacttcctttggtcatcctgagcaagtgtgtggcctctattcagatatatgcctctgttaaaggcattccacacagatccagcataatgattgagttttgcttctcacctttgttctctccacccagtaaggtgtggagctgttaataaagttcattattttattggccaagattattgatgctcataggttgaagaacccatgacattcacatgagtttgtatgttcctgtttataaactctacttgttcaaagtgtcattaatattcttgagaaactggcagttttattatgaaggatatctgcaattcatagcaattactcctttttaacctagagacactgatttaacttaataaaacctgtttataggatgaaacttgtagctcagtcttaccaaggatttaaggattcatatatgagtgtttttctttctcctttacacctagttaattaaccttgtatcttatgtctcacttgctgactcttcagaccttttttttttggaacaaaaagcagctgcgtgtaaattacgacagcaactgaattttccatgaatcatattcacttttctgaaggcaactctgcatgcagttacagaaatgtcctactggggctcctcctttgcctacttcaattttaagaattctgaggtcaggagaggtaatagggcacacacctaatttgttaattaagcaaggattctaatgatatatcacatactcaaatcctggattttccctaaaatatgattattatattgggaatttgaaaacatgttgagcagtggtaaagtacatgacacactagaagccaaaaatcagaaccctacatttaaagttcataataaaagatccacccgagtataaccaataatatttggtttagatattttatagcttttctacctttttaggaaatttagagtgttttattaagttgaccagaagtgtggtattatcaatattattttgaaactattcaaaaattcctactggttaaaaagcttttttttttttttaaattgtgctgaggctatgccattttctccctctctgaagaaagtatgtaccttttagatacagattaacagtaacaaatggccactgagcactgctttttttcctttatggaaacttctcatgttcatgcagactagctacaacagcttcttaaaaaaagatactttttggccaccaaactacctctttggcatccaaggtaatgcaggaaaactttgacccaaagtattcccatatattatttgcattaagcatgtcacttatgaaatgagaagtgatctcaaggattttagtgctgaatcctcaactaaaattttatttccttgtgctgaatagaacacatacagatccatattaaaaacagtcatcatattaggcaaattcaatctgtcaatgtagttttagtccagaaccaaaccagtgatagttaggaattacagagttaccaaccaaactgatttgctttcctggtggttctttgtgtaacagatgagagaaataaagtggcagagtaccagtgaacatttggagaaaatacctaattattttcttcctaacccaagttagccactgaatagtcatctcagaatagtcacctcatcccagttggcccattaggttcctgtgtgcttcatcttctgtgagaaaaaaaaaccttatatcattccttatttcagatgtaagatgccaggtgagttattttccacaaatttcttaagctcattactggaaaaaaaaatttctcaaaacttttagtaatgaatgagtgtacaagcagcaattggatattaatcccatggtgcaaggatttcctgcaaagtacctttaatgtgtttaaatcagcagcaagcattaggacatgctattttggccccataagttaggtgtgtagcactacacattagacaccaagtcatcccaaccaatatttatccatatgaacagataaactgaacaaaaacatagttctgataaaacctgcattcacaacctaatgtagtttaaagtaaattttttcacaattgagggctgctatttaggactgttttgttaataataaaaacaggaattatatagaagataaaacaccattttttactgctatataatgtcttgctatataaaacataccctcaacaagtcaaaatatttaaaaccagtgtttcaaataccaaaaatcacagctatgttactgttcagtaactccactcaaataaatgttagtactgcattcttgaaggaaaaaaactgcagccaaggcaagaactctgaagtttgcactcagagtttaaaagacagacccctactctgcaaactgaagactgccactctgcttcaataactccagcctgccacattttacttcaattggtaaagcactctgctgagaatataaaaagttataaaaaggcaatcataaaagattaaatattggtaggcatgtaagcttccttttaataaaaacaaaaatagtcaatgtcatctatttaaataagtatcctttgttatagagtgttccagttattgaaaaagggcccttaaaaaacccaactgtctacatctttaaaccctaccccttttaccccatagtacacatttgagggaagagtcatttaatgtgcaaattggcaaaacaaatgtggaggagaggggacttcttgaaatgatgtgcccaatcaattcttggtttattcttttccaaaaagtaaaataaccaaagtcttaaaagtacacaaaacagaccttcatctttgcattcctttccaaataaacccaaaaagtatgtacagcatgtttaatagtatgcaatatgcaaaagctttgtgttgctgttagcaacatctatacccacccaccctctttattcacaagtgtacctctactaaccataattacatcactaagcctgttagtttgagagggtcttaaatttgttaaaactggaaaatctttgtataggggctccattcatttgactcaaggttatagacttccaccgtattcagaaattcattgccatcgaatcctcccactgcataaatggtgttccctacagttgcaatcccagcattgctccttggtgaagtcatatttcccatcatcttccattcatttctagttggatcatacatttccacacaactgatggcatgagaaccatcaaagccaccacatacaaacagttttccattaagaacagccactccagctcctcgcctagccacattcatgggtgcaattaaagtccaggtattattttcaggattgtatcgttctactgtgttcagacaattccaagattctgcacctccgattatgtacaaataaccaccaagctcacagactgcagactggtgtctccgaatgttaagaggggcacagcttgtccacaactttgttacaggatcaaatacatcacaatttttcagtcctttttgaccatatggatcagagccaccaacgatgtataactttccattcagagcacacactcctgcattacaacggttagttctcaattctggaacaggaatccagtcatctatgtttgaatcatacatctctccacaactcaggtcatctgagtggccatttgatccacctaccacatagagctggcccatgagtacagccatttgaaatcgggctcttggtgttctcatgggagcaagaaaggaccagtgatctgtatgtggattatagcattcgactgttcgaagacattcctctctgttatagccacctgcagctatgagtttgccattcatctctgctgttcccagaccagatcgtgcgtactgcataggagacatgggcttttcgattagctcatcttgttgcatctcaaagcttaaactcttacttagttttggagtacttgttggtgagctctgtgggctgtttctcccatgaagaaaaatgacacagaatataccatccagcacagccaggcacaagtaagtgttatttgaagtcttttctgaagcaacgattttccactcatgcttagggctttgtactgtagcatttggagaagagagacatccagttgaactgctacttatctgcttatggccattctcacgtggtggctttttctcagactgtgcaatgtgtacctgcacaaactgaatgtggtcatcatcactgccaaacacctcagcctgtccatctagtaggttcccatcaagcagcttgtgatcagctgagtagtacaaggtttgaacctcttccatcagctcttccagactgtctccattctcccagatgctacgctgcacccagttgattacctttgtatataatttgccattgctgggcaagcaaacattatcttcaagcattacctccaactttagccttggaagcttaagaaactcctcctcttcagaaatttgtaacaaatgctcctgaatataagcatcaaccttattcaacaaacgggagtctcccatacaacttgcaaaatttcggtaagagatgcagctggtaacatccattctagacagtaaataatcaccacaaacctgctttactcgatccatcttcagcttttttgctgcagaataaacatcttttaccaattccttatctgctttcaactgagcagtgtaggcataattcaacaagacttcaacagcttctggattgagatcatcaaatttaacgtgagaaattccatgaggatcactatcactattaaagatttcaaataaatagggactgcagcaagctagcactgctctgtgtgctaacatttcatggccacagacctgaagtcgaacatcacagaactggccacttttcctcagggcatttaatttggcaacagaagactcaataaaattttcatcctcaaacatcaaatatccattgggaatcatttttccttataaatttggctactctgttggtggcaaatgtatttctgggaactcttaagtaatccaaggacaaaggagtgttaaaaggtgcacttcgtcagggtatgaagacaggtggttgaaatgaaggcaggtgtgtcttaagctctaatggtgattccaaaactatcaggcttgaaaatgatgtaatcaagtccttaaaagctatagacacgaatttcttctgtgataatgatgcatcataatctggttcatctctgaagagatggaaacattcatttctagagcttcgatgggaagcaggaggaagcgggcgggaatcggcccaacggaaagcgccagaaggcggcggaagacgggagcggtcaagtagaaggacgaggggccagtccgtggagactgaaaggaagggggagcgccaccgagaactcgcgggaactcgctcgctcgccgatacagccgcgccgaagcagcaggcggagaaactgcgcccagcagctctgagcgaccgacctccacgcgcgaccgggagacactgcctccgccgccgccgaccgctcgcgccgcaccccctcgcac

SEQ ID NO: 14906 - RNA, 7944 nt, Homo sapiens
  source 1..7944: mol_type = other RNA
gctgggattacaggcatgagccactacacttggcctttgaaacttacttttacaaaagatagttcatttctctcctgggaagaccagcgaacatcctctggtttggagggcctccagctctctccatattctgagccaaggaaaagctggctaaagaattgaagtctgttgtgtccccacagggtcctcttgttaaaacctgcagtggtcaattgtgactgcacagactagaacttcacagatgggttaatcccactttcacattgtggatctttgactgtcacatgaaagaccaggtgacacaagacacatctgaagctctatttccttgctattttgaacattattttaagggagaacgaaagtcctttcattgtcagtccaggtttatttagatggtgtcttggtcagctttcagagcctaggtcacattgttcatattcttgactttttgctctcttagctagcatgacaggttgggatgaatttccctctttcctcaaagtctggtgactgcatccagtctctaaggatgtgatgctacccatggcccttttctgacttcgagattggacaggccagtcacacttctatttattgggtatatataaaacccactccagtgaacagaactgagccccatgaaggcaggaactacactgtgtgtagtgtctcatagttgtggttagttaatatttttgacaaattgacctgcaggctcacctactctaaaacaaaagacatactttacctttgcctaccaaagtttgacttgaaagcttttaagtttgtctggtctgtcaggtgaaaagccactcagtaaagtcaaacagatacacctcttagatcttggaatatggcccacagaaatggattcttctggagccagagtacctcaagatgttggctttcctgagggttttagtattatatatacttgtatttttaaaaatccatctctgtattcatggaattctttaatatctttggctgttgttaaaagcaagaattggccaccctgagggtttgtagactagttttggcctgtgacaggaatcctttttaattctagctttgtttatgaactagatgtagtttgtctcaaattaattctcgatgttgaaaacactgaggacagattcttgagcagaattaccagttataagcctggaaggtgaggtggtggacacccaaatccgagctactagcttggttcagtcttcttaaagcacaaaccattttcaacatcctattctttatttctaatgaggtaaaatatggacatgttctagcccttcttctaagcttgatattttaaaggtttggtaccactttggttaagctagaaaaacaaaactttttttccttcgtaagtgtagagttctgtgagttctgtcaaacatgtaatcaatcaatcatcagcagtcaagatattgaagtcacaccacccctaaaaattccctcatgtccctttgtaattaactcccattcccagctcaggaggccattgatgtgtttgccttccctgtagtttttcctattcctgaatgctatataaatggagactgtttttttaagagacagggtcttgctatgttgcccaagtgcagtggctgttcagacattatagcatactacagccttgaactcctgggctcaggcaatcctctcacctcagcctcctgagtagctgggactacaagtgcatgccactatgcccagctaatggaggcttttgagtctggctttttatttagcatgatgcttgagacttatccatattatcagtagttcattattttattcccaagaagtattgcattgccatggatgtacaaatttattcattcaccaggtggaaggctacttcactgaattcagtttttggtgattatgaataaagttgctatattcacatacaggtttgtgtgaatatgttccttcacttgggtaaatacctacgaatgggattgctttgtcacagattattagaaaatggatggattgttttttaaactgcctgtgcacctttgcagttcctccagcaatgtatgagagttcaagttgctctgcatcgtaagcagaatttggtatattcagtttcaataggtgtatgccattttggttttaatttacattttcttaatgatttatgatagtattttcctgtgttcttatggcatcaacttcttttgcaaagtgtcttcaaatattttacccatttaaaaatcgttttaacagatctcatcttattaccttgctggacatttcatctcagtagtttcattactccaagttaggtctttctgtgtgccttttttttctggctaaaattatgttacttcctttggtcatcctgagcaagtgtgtggcctctattcagatatatgcctctgttaaaggcattccacacagatccagcataatgattgagttttgcttctcacctttgttctctccacccagtaaggtgtggagctgttaataaagttcattattttattggccaagattattgatgctcataggttgaagaacccatgacattcacatgagtttgtatgttcctgtttataaactctacttgttcaaagtgtcattaatattcttgagaaactggcagttttattatgaaggatatctgcaattcatagcaattactcctttttaacctagagacactgatttaacttaataaaacctgtttataggatgaaacttgtagctcagtcttaccaaggatttaaggattcatatatgagtgtttttctttctcctttacacctagttaattaaccttgtatcttatgtctcacttgctgactcttcagaccttttttttttggaacaaaaagcagctgcgtgtaaattacgacagcaactgaattttccatgaatcatattcacttttctgaaggcaactctgcatgcagttacagaaatgtcctactggggctcctcctttgcctacttcaattttaagaattctgaggtcaggagaggtaatagggcacacacctaatttgttaattaagcaaggattctaatgatatatcacatactcaaatcctggattttccctaaaatatgattattatattgggaatttgaaaacatgttgagcagtggtaaagtacatgacacactagaagccaaaaatcagaaccctacatttaaagttcataataaaagatccacccgagtataaccaataatatttggtttagatattttatagcttttctacctttttaggaaatttagagtgttttattaagttgaccagaagtgtggtattatcaatattattttgaaactattcaaaaattcctactggttaaaaagcttttttttttttttaaattgtgctgaggctatgccattttctccctctctgaagaaagtatgtaccttttagatacagattaacagtaacaaatggccactgagcactgctttttttcctttatggaaacttctcatgttcatgcagactagctacaacagcttcttaaaaaaagatactttttggccaccaaactacctctttggcatccaaggtaatgcaggaaaactttgacccaaagtattcccatatattatttgcattaagcatgtcacttatgaaatgagaagtgatctcaaggattttagtgctgaatcctcaactaaaattttatttccttgtgctgaatagaacacatacagatccatattaaaaacagtcatcatattaggcaaattcaatctgtcaatgtagttttagtccagaaccaaaccagtgatagttaggaattacagagttaccaaccaaactgatttgctttcctggtggttctttgtgtaacagatgagagaaataaagtggcagagtaccagtgaacatttggagaaaatacctaattattttcttcctaacccaagttagccactgaatagtcatctcagaatagtcacctcatcccagttggcccattaggttcctgtgtgcttcatcttctgtgagaaaaaaaaaccttatatcattccttatttcagatgtaagatgccaggtgagttattttccacaaatttcttaagctcattactggaaaaaaaaatttctcaaaacttttagtaatgaatgagtgtacaagcagcaattggatattaatcccatggtgcaaggatttcctgcaaagtacctttaatgtgtttaaatcagcagcaagcattaggacatgctattttggccccataagttaggtgtgtagcactacacattagacaccaagtcatcccaaccaatatttatccatatgaacagataaactgaacaaaaacatagttctgataaaacctgcattcacaacctaatgtagtttaaagtaaattttttcacaattgagggctgctatttaggactgttttgttaataataaaaacaggaattatatagaagataaaacaccattttttactgctatataatgtcttgctatataaaacataccctcaacaagtcaaaatatttaaaaccagtgtttcaaataccaaaaatcacagctatgttactgttcagtaactccactcaaataaatgttagtactgcattcttgaaggaaaaaaactgcagccaaggcaagaactctgaagtttgcactcagagtttaaaagacagacccctactctgcaaactgaagactgccactctgcttcaataactccagcctgccacattttacttcaattggtaaagcactctgctgagaatataaaaagttataaaaaggcaatcataaaagattaaatattggtaggcatgtaagcttccttttaataaaaacaaaaatagtcaatgtcatctatttaaataagtatcctttgttatagagtgttccagttattgaaaaagggcccttaaaaaacccaactgtctacatctttaaaccctaccccttttaccccatagtacacatttgagggaagagtcatttaatgtgcaaattggcaaaacaaatgtggaggagaggggacttcttgaaatgatgtgcccaatcaattcttggtttattcttttccaaaaagtaaaataaccaaagtcttaaaagtacacaaaacagaccttcatctttgcattcctttccaaataaacccaaaaagtatgtacagcatgtttaatagtatgcaatatgcaaaagctttgtgttgctgttagcaacatctatacccacccaccctctttattcacaagtgtacctctactaaccataattacatcactaagcctgttagtttgagagggtcttaaatttgttaaaactggaaaatctttgtataggggctccattcatttgactcaaggttatagacttccaccgtattcagaaattcattgccatcgaatcctcccactgcataaatggtgttccctacagttgcaatcccagcattgctccttggtgaagtcatatttcccatcatcttccattcatttctagttggatcatacatttccacacaactgatggcatgagaaccatcaaagccaccacatacaaacagttttccattaagaacagccactccagctcctcgcctagccacattcatgggtgcaattaaagtccaggtattattttcaggattgtatcgttctactgtgttcagacaattccaagattctgcacctccgattatgtacaaataaccaccaagctcacagactgcagactggtgtctccgaatgttaagaggggcacagcttgtccacaactttgttacaggatcaaatacatcacaatttttcagtcctttttgaccatatggatcagagccaccaacgatgtataactttccattcagagcacacactcctgcattacaacggttagttctcaattctggaacaggaatccagtcatctatgtttgaatcatacatctctccacaactcaggtcatctgagtggccatttgatccacctaccacatagagctggcccatgagtacagccatttgaaatcgggctcttggtgttctcatgggagcaagaaaggaccagtgatctgtatgtggattatagcattcgactgttcgaagacattcctctctgttatagccacctgcagctatgagtttgccattcatctctgctgttcccagaccagatcgtgcgtactgcataggagacatgggcttttcgattagctcatcttgttgcatctcaaagcttaaactcttacttagttttggagtacttgttggtgagctctgtgggctgtttctcccatgaagaaaaatgacacagaatataccatccagcacagccaggcacaagtaagtgttatttgaagtcttttctgaagcaacgattttccactcatgcttagggctttgtactgtagcatttggagaagagagacatccagttgaactgctacttatctgcttatggccattctcacgtggtggctttttctgcacaaactgaatgtggtcatcatcactgccaaacacctcagcctgtccatctagtaggttcccatcaagcagcttgtgatcagctgagtagtacaaggtttgaaccattaaatcatcatcgttctctgcccacagcggatttttcttaggagaactggggcaggactgctgcttctttacgtgtcaatacacttgaggtttcttcttgtttcttcagtcttgggtatcctagttttgttaataaacctcttccatcagctcttccagactgtctccattctcccagatgctacgctgcacccagttgattacctttgtatataatttgccattgctgggcaagcaaacattatcttcaagcattacctccaactttagccttggaagcttaagaaactcctcctcttcagaaatttgtaacaaatgctcctgaatataagcatcaaccttattcaacaaacgggagtctcccatacaacttgcaaaatttcggtaagagatgcagctggtaacatccattctagacagtaaataatcaccacaaacctgctttactcgatccatcttcagcttttttgctgcagaataaacatcttttaccaattccttatctgctttcaactgagcagtgtaggcataattcaacaagacttcaacagcttctggattgagatcatcaaatttaacgtgagaaattccatgaggatcactatcactattaaagatttcaaataaatagggactgcagcaagctagcactgctctgtgtgctaacatttcatggccacagacctgaagtcgaacatcacagaactggccacttttcctcagggcatttaatttggcaacagaagactcaataaaattttcatcctcaaacatcaaatatccattgggaatcatttttccttataaatttggctactctgttggtggcaaatgtatttctgggaactcttaagtaatccaaggacaaaggagtgttaaaaggtgcacttcgtcagggtatgaagacaggtggttgaaatgaaggcaggtgtgtcttaagctctaatggtgattccaaaactatcaggcttgaaaatgatgtaatcaagtccttaaaagctatagacacgaatttcttctgtgataatgatgcatcataatctggttcatctctgaagagatggaaacattcatttctagagcttcgatgggaagcaggaggaagcgggcgggaatcggcccaacggaaagcgccagaaggcggcggaagacgggagcggtcaagtagaaggacgaggggccagtccgtggagactgaaaggaagggggagcgccaccgagaactcgcgggaactcgctcgctcgccgatacagccgcgccgaagcagcaggcggagaaactgcgcccagcagctctgagcgaccgacctccacgcgcgaccgggagacactgcctccgccgccgccgaccgctcgcgccgcaccccctcgcac

SEQ ID NO: 14907 - RNA, 3793 nt, Homo sapiens
  source 1..3793: mol_type = other RNA
gctgggattacaggcatgagccactacgcctggccaagaaaaatattttcaataaatttagtataggttaagtgtgcagtgtttatacaagtctacatgttccaactgtctatagcatgcaggacagtaacatgctatacgggtttgtagcctaggagcaacagactataccatatagcctaggtgtactggtaggctataccatctaggtttgtggaagtaaacaacatgatgtttacacaatgacaatatcacctaacgatgcatttctcagaacatatctctgtcattaagtgatgcgtgactctatttgctcctttatctctaacattacattgtaagggtaaggactgtgttatcaagcctgtattcctaacaaaatctatgtttaagaaatatttattgtgagtttactatgtatcaggtacagtgctaggtactcacaattggagacataattttatagatgagaacactgaaactctgagaaattaagaacttactcaaagtcacacagctggcaaatgggttgcaccagtatacctacctccagaatatatattgggtaaaggatctgtttgcatgaacaaacaaaaaaatcatattcttgtaagtatttttacaccctgtaccagtagatctttctttaaataaattccgaagatgaacaatttttgtcccatctaaaatattcaaagcaaagtccacctgttctgactctagaacaaaaagctacaaatagaggaaataaataagttgaattcaaatgctgctgagaaaaggcaatgtatattatagttctgtggtagtactgataacattcaagtcattcttaggcaccagtcttacgtatatgaagtcactttttcattccattgtacaaaactcatattttgagaaaaatctaatagctaatagtctccaacaccatatgatcataatcctttagcttaagtagagatctacttattaaatgaggcaccatcaacctaaggaaagataagctgtaagagaatgaagacagaggtatatcaagtaacaagaacattcttccttatcaggataaaatgtttatcagtattcaaataaaatatcttaaatggaaagagacaggaaagaacatggttaaatcacagaaaatgaagaaagggagaagctgatcatgatcttgtacaacattatgacagcactaaggtattacgtatccaatacaaggatacttaatagaccaaagaatttaaaatcccagggaactggaataaccagccacaaaagaggcctctctttgttgtggttcacaacacaaaaggccatcaacaaattaggaaatattaaaattaagagagcagcaggtttcttcttggtagacagctcatgctaccatccacaaagtgagcagtggaaggggtatttaatgtcaaggctttattttgaatttctgttccagatgcctctccacagcattcatcacaccttccttcacacttgaagggaaaagtccttaagagttcaccacattttggtgttatttttagcataaacatttgtttttctataagaagtatctctctggattcaaaccacagaaatgtcaatgaatgttatttccattgtataatcatttaaaagtcacctacagagctgggtgcagcagcttgtgcctgtaatctcagttactcaggaggctaaggcaggaggattgtgtgaggtcaggagttcaagaccagcctggacaacatggcaagaccctcatctctacaggaaaaaaaaaaggcacctacaaattgaaactgacttgatagtttaggatcatttatcaccagtcccatgtacttgtagttgatttcaaatgtttggtacaggtgactgtaagacttcaagtattccatgaaaataacattcatgctgggatcataaaattacatttctgggacagtatttttaaagtctgtttttaacttttgtcttcaagagctactttcttcttgctgttctgaccagtgacctttttccacatacttactgtttatccttagctttttctaagaaacattttggagttgtactaatgctctccctttccaatggtttcttaatcatctttttcttttgtttgcttagtagtttctgaaaaccttttatgtattctggtacaggacacccagcctgctgtataacattagcaacgcttcttaataatggcttatcatcctcagtgaaaaatgtaattgcttttcccttattccctgctcttccagttcgacctatcctgtggatatattccactgagctagttggaaagtcatagttgatcaccaagttcacacctttaaaatcaatccctcttgctagcaaggctgtacaaatcagaacccagatttttcctgctctgaaactgtggactgtgttatctctctgttgttgtgttctctctgcatgaataacatccacattaataccttcatatatgagctcatgaaaaagttctttagccctttcaatggactgaacaaaaacaagaacaggtggattgaaaccctttttaacaagttctctcacggccagaagttttccggtctcagatccaacaaagagaagctcttgttctacagtttctactgcagaattccttgctccaatggacacactgatgacattgtccaggttgagtttgcaccactgttcaacatcatatgcaaaagttgcactgaacatagctcttcggaccttgtgggatgtgcaggccaggaaaatggaagccagctggtctctgaacccagttttgccatcttcaaacagtttatctgattcgtctactacaagccactcaacacttgctaggtcgattccggggggatcttgctttaataaatagattagtcgatttggagtagtcacaagaatatcaaactttttagatgatttaggtccaaatttcttggctgccactgctgctttgtggatcatgtgtattctgaatcctgttccctcagaaatttttattaactctctgtgaatctggctggcaagttctcgtgttggtgatataatcagggctctgaagcctttatttgcgggttgtttcagctgcattaaaataggaatgctaaaagctaatgtttttccagatccagttggagcagaagccagaagttcccgaccatgcagcataactgggatggcttgcatttggattggcgtaggcatttggaaacctgcatctagaatgttctgaagtagtcgagaattgattttatattcctggtcaagttgctgaaatgtagcaattgggtcaggaagatcggttccttggacgtgaattttgtgtttattccgcaagaagtttatcttttcttttctgagattctccaactttccggaagttagtttactttctctctgaacttttttgtcttcaatctttgcttctacagatgacatccactgtatagtagcaccttcttcttgggaagcaatttctgaagtcatcgtcttcctttttttcttgctctgctccctcttcctttcagttaggctctcttcttttttctctccattttggggcttctgatgtgtttgtgatgctccacacacacctgggacagacttcttgtttccaaaaaagtccagtccctgaagcacctccgaagaatcaaagtcatatttcctttttcctatctggaatcgagctgcgtctgccgagaagcgtctcgtgtcgaatttggcccccgcgccgagccggcgaaagagatcgtggacgtccatctttacccagaaagcgccacagttctac

SEQ ID NO: 14908 - RNA, 3950 nt, Homo sapiens
  source 1..3950: mol_type = other RNA
gctgggattacaggcatgagccactacgcctggccaagaaaaatattttcaataaatttagtataggttaagtgtgcagtgtttatacaagtctacatgttccaactgtctatagcatgcaggacagtaacatgctatacgggtttgtagcctaggagcaacagactataccatatagcctaggtgtactggtaggctataccatctaggtttgtggaagtaaacaacatgatgtttacacaatgacaatatcacctaacgatgcatttctcagaacatatctctgtcattaagtgatgcgtgactctatttgctcctttatctctaacattacattgtaagggtaaggactgtgttatcaagcctgtattcctaacaaaatctatgtttaagaaatatttattgtgagtttactatgtatcaggtacagtgctaggtactcacaattggagacataattttatagatgagaacactgaaactctgagaaattaagaacttactcaaagtcacacagctggcaaatgggttgcaccagtatacctacctccagaatatatattgggtaaaggatctgtttgcatgaacaaacaaaaaaatcatattcttgtaagtatttttacaccctgtaccagtagatctttctttaaataaattccgaagatgaacaatttttgtcccatctaaaatattcaaagcaaagtccacctgttctgactctagaacaaaaagctacaaatagaggaaataaataagttgaattcaaatgctgctgagaaaaggcaatgtatattatagttctgtggtagtactgataacattcaagtcattcttaggcaccagtcttacgtatatgaagtcactttttcattccattgtacaaaactcatattttgagaaaaatctaatagctaatagtctccaacaccatatgatcataatcctttagcttaagtagagatctacttattaaatgaggcaccatcaacctaaggaaagataagctgtaagagaatgaagacagaggtatatcaagtaacaagaacattcttccttatcaggataaaatgtttatcagtattcaaataaaatatcttaaatggaaagagacaggaaagaacatggttaaatcacagaaaatgaagaaagggagaagctgatcatgatcttgtacaacattatgacagcactaaggtattacgtatccaatacaaggatacttaatagaccaaagaatttaaaatcccagggaactggaataaccagccacaaaagaggcctctctttgttgtggttcacaacacaaaaggccatcaacaaattaggaaatattaaaattaagagagcagcaggtttcttcttggtagacagctcatgctaccatccacaaagtgagcagtggaaggggtatttaatgtcaaggctttattttgaatttctgttccagatgcctctccacagcattcatcacaccttccttcacacttgaagggaaaagtccttaagagttcaccacattttggtgttatttttagcataaacatttgtttttctataagaagtatctctctggattcaaaccacagaaatgtcaatgaatgttatttccattgtataatcatttaaaagtcacctacagagctgggtgcagcagcttgtgcctgtaatctcagttactcaggaggctaaggcaggaggattgtgtgaggtcaggagttcaagaccagcctggacaacatggcaagaccctcatctctacaggaaaaaaaaaaggcacctacaaattgaaactgacttgatagtttaggatcatttatcaccagtcccatgtacttgtagttgatttcaaatgtttggtacaggtgactgtaagacttcaagtattccatgaaaataacattcatgctgggatcataaaattacatttctgggacagtatttttaaagtctgtttttaacttttgtcttcaagagctactttcttcttgctgttctgaccagtgacctttttctgtttatccttagctttttctaagaaacattttggagttgtactaatgctctccctttccaatggtttcttaatcatctttttcttttgtttgcttagtagtttctgaaaaccttttatgtattctggtacaggacacccagcctgctgtataacattagcaacgcttcttaataatggcttatcatcctcagtgaaaaatgtaattgcttttcccttattccctgctcttccagttcgacctatcctgtggatatattccactgagctagttggaaagtcatagttgatcaccaagttcacacctttaaaatcaatccctcttgctagcaaggctgtacaaatcagaacccagatttttcctgctctgaaactgtggactgtgttatctctctgttgttgtgttctctctgcatgaataacatccacattaataccttcatatatgagctcatgaaaaagttctttagccctttcaatggactgaacaaaaacaagaacaggtggattgaaaccctttttaacaagttctctcacggccagaagttttccggtctcagatccaacaaagagaagctcttgttctacagtttctactgcagaattccttgctccaatggacacactgatgacattgtccaggttgagtttgcaccactgttcaacatcatatgcaaaagttgcactgaacatagctcttcggaccttgtgggatgtgcaggccaggaaaatggaagccagctggtctctgaacccagttttgccatcttcaaacagtttatctgattcgtctactacaagccactcaacacttgctaggtcgattccggggggatcttgctttaataaatagattagtcgatttggagtagtcacaagaatatcaaactttttagatgatttaggtccaaatttcttggctgccactgctgctttgtggatcatgtgtattctgaatcctgttccctcagaaatttttattaactctctgtgaatagaaagacttaaaagacttgcccacatggagtaagatccggagcactgtgctgtgtagaggatacttgaccatgacagaagacgtgggccttgctttttaagatctttttattaccttcaaataagaaagatcactgaagtaaaaaccaatcgcatactcttcaaaagctacaagtcatacctggctggcaagttctcgtgttggtgatataatcagggctctgaagcctttatttgcgggttgtttcagctgcattaaaataggaatgctaaaagctaatgtttttccagatccagttggagcagaagccagaagttcccgaccatgcagcataactgggatggcttgcatttggattggcgtaggcatttggaaacctgcatctagaatgttctgaagtagtcgagaattgattttatattcctggtcaagttgctgaaatgtagcaattgggtcaggaagatcggttccttggacgtgaattttgtgtttattccgcaagaagtttatcttttcttttctgagattctccaactttccggaagttagtttactttctctctgaacttttttgtcttcaatctttgcttctacagatgacatccactgtatagtagcaccttcttcttgggaagcaatttctgaagtcatcgtcttcctttttttcttgctctgctccctcttcctttcagttaggctctcttcttttttctctccattttggggcttctgatgtgtttgtgatgctccacacacacctgggacagacttcttgtttccaaaaaagtccagtccctgaagcacctccgaagaatcaaagtcatatttcctttttcctatctggaatcgagctgcgtctgccgagaagcgtctcgtgtcgaatttggcccccgcgccgagccggcgaaagagatcgtggacgtccatctttacccagaaagc

SEQ ID NO: 14909 - RNA, 3780 nt, Homo sapiens
  source 1..3780: mol_type = other RNA
gctgggattacaggcatgagccactacgcctggccaagaaaaatattttcaataaatttagtataggttaagtgtgcagtgtttatacaagtctacatgttccaactgtctatagcatgcaggacagtaacatgctatacgggtttgtagcctaggagcaacagactataccatatagcctaggtgtactggtaggctataccatctaggtttgtggaagtaaacaacatgatgtttacacaatgacaatatcacctaacgatgcatttctcagaacatatctctgtcattaagtgatgcgtgactctatttgctcctttatctctaacattacattgtaagggtaaggactgtgttatcaagcctgtattcctaacaaaatctatgtttaagaaatatttattgtgagtttactatgtatcaggtacagtgctaggtactcacaattggagacataattttatagatgagaacactgaaactctgagaaattaagaacttactcaaagtcacacagctggcaaatgggttgcaccagtatacctacctccagaatatatattgggtaaaggatctgtttgcatgaacaaacaaaaaaatcatattcttgtaagtatttttacaccctgtaccagtagatctttctttaaataaattccgaagatgaacaatttttgtcccatctaaaatattcaaagcaaagtccacctgttctgactctagaacaaaaagctacaaatagaggaaataaataagttgaattcaaatgctgctgagaaaaggcaatgtatattatagttctgtggtagtactgataacattcaagtcattcttaggcaccagtcttacgtatatgaagtcactttttcattccattgtacaaaactcatattttgagaaaaatctaatagctaatagtctccaacaccatatgatcataatcctttagcttaagtagagatctacttattaaatgaggcaccatcaacctaaggaaagataagctgtaagagaatgaagacagaggtatatcaagtaacaagaacattcttccttatcaggataaaatgtttatcagtattcaaataaaatatcttaaatggaaagagacaggaaagaacatggttaaatcacagaaaatgaagaaagggagaagctgatcatgatcttgtacaacattatgacagcactaaggtattacgtatccaatacaaggatacttaatagaccaaagaatttaaaatcccagggaactggaataaccagccacaaaagaggcctctctttgttgtggttcacaacacaaaaggccatcaacaaattaggaaatattaaaattaagagagcagcaggtttcttcttggtagacagctcatgctaccatccacaaagtgagcagtggaaggggtatttaatgtcaaggctttattttgaatttctgttccagatgcctctccacagcattcatcacaccttccttcacacttgaagggaaaagtccttaagagttcaccacattttggtgttatttttagcataaacatttgtttttctataagaagtatctctctggattcaaaccacagaaatgtcaatgaatgttatttccattgtataatcatttaaaagtcacctacagagctgggtgcagcagcttgtgcctgtaatctcagttactcaggaggctaaggcaggaggattgtgtgaggtcaggagttcaagaccagcctggacaacatggcaagaccctcatctctacaggaaaaaaaaaaggcacctacaaattgaaactgacttgatagtttaggatcatttatcaccagtcccatgtacttgtagttgatttcaaatgtttggtacaggtgactgtaagacttcaagtattccatgaaaataacattcatgctgggatcataaaattacatttctgggacagtatttttaaagtctgtttttaacttttgtcttcaagagctactttcttcttgctgttctgaccagtgacctttttctgtttatccttagctttttctaagaaacattttggagttgtactaatgctctccctttccaatggtttcttaatcatctttttcttttgtttgcttagtagtttctgaaaaccttttatgtattctggtacaggacacccagcctgctgtataacattagcaacgcttcttaataatggcttatcatcctcagtgaaaaatgtaattgcttttcccttattccctgctcttccagttcgacctatcctgtggatatattccactgagctagttggaaagtcatagttgatcaccaagttcacacctttaaaatcaatccctcttgctagcaaggctgtacaaatcagaacccagatttttcctgctctgaaactgtggactgtgttatctctctgttgttgtgttctctctgcatgaataacatccacattaataccttcatatatgagctcatgaaaaagttctttagccctttcaatggactgaacaaaaacaagaacaggtggattgaaaccctttttaacaagttctctcacggccagaagttttccggtctcagatccaacaaagagaagctcttgttctacagtttctactgcagaattccttgctccaatggacacactgatgacattgtccaggttgagtttgcaccactgttcaacatcatatgcaaaagttgcactgaacatagctcttcggaccttgtgggatgtgcaggccaggaaaatggaagccagctggtctctgaacccagttttgccatcttcaaacagtttatctgattcgtctactacaagccactcaacacttgctaggtcgattccggggggatcttgctttaataaatagattagtcgatttggagtagtcacaagaatatcaaactttttagatgatttaggtccaaatttcttggctgccactgctgctttgtggatcatgtgtattctgaatcctgttccctcagaaatttttattaactctctgtgaatctggctggcaagttctcgtgttggtgatataatcagggctctgaagcctttatttgcgggttgtttcagctgcattaaaataggaatgctaaaagctaatgtttttccagatccagttggagcagaagccagaagttcccgaccatgcagcataactgggatggcttgcatttggattggcgtaggcatttggaaacctgcatctagaatgttctgaagtagtcgagaattgattttatattcctggtcaagttgctgaaatgtagcaattgggtcaggaagatcggttccttggacgtgaattttgtgtttattccgcaagaagtttatcttttcttttctgagattctccaactttccggaagttagtttactttctctctgaacttttttgtcttcaatctttgcttctacagatgacatccactgtatagtagcaccttcttcttgggaagcaatttctgaagtcatcgtcttcctttttttcttgctctgctccctcttcctttcagttaggctctcttcttttttctctccattttggggcttctgatgtgtttgtgatgctccacacacacctgggacagacttcttgtttccaaaaaagtccagtccctgaagcacctccgaagaatcaaagtcatatttcctttttcctatctggaatcgagctgcgtctgccgagaagcgtctcgtgtcgaatttggcccccgcgccgagccggcgaaagagatcgtggacgtccatctttacccagaaagcgccacagttct

SEQ ID NO: 14910 - RNA, 3895 nt, Homo sapiens
  source 1..3895: mol_type = other RNA
gctgggattacaggcatgagccactacgcctggccaagaaaaatattttcaataaatttagtataggttaagtgtgcagtgtttatacaagtctacatgttccaactgtctatagcatgcaggacagtaacatgctatacgggtttgtagcctaggagcaacagactataccatatagcctaggtgtactggtaggctataccatctaggtttgtggaagtaaacaacatgatgtttacacaatgacaatatcacctaacgatgcatttctcagaacatatctctgtcattaagtgatgcgtgactctatttgctcctttatctctaacattacattgtaagggtaaggactgtgttatcaagcctgtattcctaacaaaatctatgtttaagaaatatttattgtgagtttactatgtatcaggtacagtgctaggtactcacaattggagacataattttatagatgagaacactgaaactctgagaaattaagaacttactcaaagtcacacagctggcaaatgggttgcaccagtatacctacctccagaatatatattgggtaaaggatctgtttgcatgaacaaacaaaaaaatcatattcttgtaagtatttttacaccctgtaccagtagatctttctttaaataaattccgaagatgaacaatttttgtcccatctaaaatattcaaagcaaagtccacctgttctgactctagaacaaaaagctacaaatagaggaaataaataagttgaattcaaatgctgctgagaaaaggcaatgtatattatagttctgtggtagtactgataacattcaagtcattcttaggcaccagtcttacgtatatgaagtcactttttcattccattgtacaaaactcatattttgagaaaaatctaatagctaatagtctccaacaccatatgatcataatcctttagcttaagtagagatctacttattaaatgaggcaccatcaacctaaggaaagataagctgtaagagaatgaagacagaggtatatcaagtaacaagaacattcttccttatcaggataaaatgtttatcagtattcaaataaaatatcttaaatggaaagagacaggaaagaacatggttaaatcacagaaaatgaagaaagggagaagctgatcatgatcttgtacaacattatgacagcactaaggtattacgtatccaatacaaggatacttaatagaccaaagaatttaaaatcccagggaactggaataaccagccacaaaagaggcctctctttgttgtggttcacaacacaaaaggccatcaacaaattaggaaatattaaaattaagagagcagcaggtttcttcttggtagacagctcatgctaccatccacaaagtgagcagtggaaggggtatttaatgtcaaggctttattttgaatttctgttccagatgcctctccacagcattcatcacaccttccttcacacttgaagggaaaagtccttaagagttcaccacattttggtgttatttttagcataaacatttgtttttctataagaagtatctctctggattcaaaccacagaaatgtcaatgaatgttatttccattgtataatcatttaaaagtcacctacagagctgggtgcagcagcttgtgcctgtaatctcagttactcaggaggctaaggcaggaggattgtgtgaggtcaggagttcaagaccagcctggacaacatggcaagaccctcatctctacaggaaaaaaaaaaggcacctacaaattgaaactgacttgatagtttaggatcatttatcaccagtcccatgtacttgtagttgatttcaaatgtttggtacaggtgactgtaagacttcaagtattccatgaaaataacattcatgctgggatcataaaattacatttctgggacagtatttttaaagtctgtttttaacttttgtcttcaagagctactttcttcttgctgttctgaccagtgacctttttctgtttatccttagctttttctaagaaacattttggagttgtactaatgctctccctttccaatggtttcttaatcatctttttcttttgtttgcttagtagtttctgaaaaccttttatgtattctggtacaggacacccagcctgctgtataacattagcaacgcttcttaataatggcttatcatcctcagtgaaaaatgtaattgcttttcccttattccctgctcttccagttcgacctatcctgtggatatattccactgagctagttggaaagtcatagttgatcaccaagttcacacctttaaaatcaatccctcttgctagcaaggctgtacaaatcagaacccagatttttcctgctctgaaactgtggactgtgttatctctctgttgttgtgttctctctgcatgaataacatccacattaataccttcatatatgagctcatgaaaaagttctttagccctttcaatggactgaacaaaaacaagaacaggtggattgaaaccctttttaacaagttctctcacggccagaagttttccggtctcagatccaacaaagagaagctcttgttctacagtttctactgcagaattccttgctccaatggacacactgatgacattgtccaggttgagtttgcaccactgttcaacatcatatgcaaaagttgcactgaacatagctcttcggaccttgtgggatgtgcaggccaggaaaatggaagccagctggtctctgaacccagttttgccatcttcaaacagtttatctgattcgtctactacaagccactcaacacttgctaggtcgattccggggggatcttgctttaataaatagattagtcgatttggagtagtcacaagaatatcaaactttttagatgatttaggtccaaatttcttggctgccactgctgctttgtggatcatgtgtattctgaatcctgttccctcagaaatttttattaactctctgtgaatctggctggcaagttctcgtgttggtgatataatcagggctctgaagcctttatttgcgggttgtttcagctgcattaaaataggaatgctaaaagctaatgtttttccagatccagttggagcagaagccagaagttcccgaccatgcagcataactgggatggcttgcatttggattggcgtaggcatttggaaacctgcatctagaatgttctgaagtagtcgagaattgattttatattcctggtcaagttgctgaaatgtagcaattgggtcaggaagatcggttccttggacgtgaattttgtgtttattccgcaagaagtttatcttttcttttctgagattctccaactttccggaagttagtttactttctctctgaacttttttgtcttcaatctttgcttctacagatgacatccactgtatagtagcaccttcttcttgggaagcaatttctggctgggcgtggtggctcacatctgtaatcccagcactttgggagcccaaggtgggtgaatcacgaggtcaggagatcgagaccatactggctaacatggtgaaaccctgtctctgaagtcatcgtcttcctttttttcttgctctgctccctcttcctttcagttaggctctcttcttttttctctccattttggggcttctgatgtgtttgtgatgctccacacacacctgggacagacttcttgtttccaaaaaagtccagtccctgaagcacctccgaagaatcaaagtcatatttcctttttcctatctggaatcgagctgcgtctgccgagaagcgtctcgtgtcgaatttggcccccgcgccgagccggcgaaagagatcgtggacgtccatctttacccagaaagcgccacagttct

SEQ ID NO: 14911 - RNA, 7370 nt, Homo sapiens
  source 1..7370: mol_type = other RNA
gctgggattacaggcatgagccactacgttcagcctaatttttttatttttagtatagacctgatttcaccatttttggcccggctggtctcaaactcctgacctcaagtgatctgcctgccttggcctcccaaagggctgggattacaggcgtgagccaccaatcctggccaagtggaacccactttaaataaaactgacaactaccggtatggttaggagggtatcccatactcttgtcttttacctagagtttaacaatgacttggattttccctcagccatgcacccattaaaacgcactaaggaaagacccttgagtcagagatttttgaatccaatgaaattagaatcgtctaccaataaggagactactgggtgctagacttaactgtcgaaacaccgttccacatgacagaaatcaacacttgtctgtttacattaaccgagcagagcttagtcacccatcactggattcgacctcgagcagacagctctacctgactcagggtcggaagagtgatacaaggtgtgcaacatatgaagctcctaatgcccatcactaacaagtgacacggaggcaggggaaacagagagtgccgctaccgattcaggtcacgcaaaggagggaggctctttcaaggtcttgctccaacttcacgttttcacattatttcagagtaagaaaagaagtggtgcagacaactcaagaaataaaatgggcaaaaattatacacatctctatttactaggagaagtaaaaaaataaaacaacccctgtgttgaaaccaggcagtattggaatcaggaggtgaagatctgtttcataatctagtgatttcaagagagtgtgtcagatcaacggagatgaataattgtgcacaaatacacgagcaacagcattggcttgactctaaaggaggaccagaatgtgtctctacttccactgctaacgcccctctgcagaaaatgttcagtgtgcgtggcatcgtgctagtcccacctggatatactaatttatggacggccttttctagccaatgggtagagaacaaactcccaggtttggaagccaagcctctctgaggaggcacagaaaagaactatccgatgtccacgttcagtgtgtacacacaacacacagagacaaaaacagaggccaggctccgtcagaggacacactctagctgagcaaaggctgcattcggcaactagggtggtgtaaacacctcggatctcactgcagccggaaggaagtcacggcatagtcccttttcaggagtctgagggataccacttgtgttgcaaaccacagatcccaagtattagacgtattcccttcttggtggaggcctactctagaagaatcaaaaaccgatgaccctctcagcgaatccgatgttaaagctcctaactaggtgaccctttagcactacagacgtaaaaatgactctaatgcactccctagaaaaggcagtgaagcaaagggggctgctgagagtttacatggttttcatataaagaggcttttaactttggaaaaagcgggcctggaaagaacactacccccattccagttgacggctttttaagtactttgtggccttcctgccgcggtgcaaaatgaggtctattttaggaactggcttctttactgcggggttagatgccaacatttcaccagggttggacgatctcacacatgagtttctggcacttttaggagggatttcctcaagtgatacactagggaatgagcctttcagcaaaaagcggttccccggagtcagttgccagctccaggagattaattggccattttttcatatgttttatgtgcaagatatttaatatgggatgaaaaatggaacacgaggaaaagcaggtattagtttggtctgaaagaggtggtaatccacagatttgcttttgtttcgacagtttctaagcagtggaacaattacctaacagtgcaccaagtaatttgttaaagttgaaaacagtaagggcgttcatgtgcgccaaggtattctgggctgaaaacagcaattttgaattttcatggcagacccaactcctaagctggctccactctgtcctatcagattttggtggtggtggcagagaatgtcataggcctgtggctggcaccgaccaagctgtcagggtggtacgaaaaggagaggaaacaggagtgctggacatggacccagctctgggtagctgatggtgataacacatcgattttttgtttcccttttgaaaataagcagaaaatgatgtgggtggaaagtcctccttaggagttcacagggactgctcgtatttagcagggccctctaaatggggactggtgaaaacaaagatgttttgaacggggatccagaatttcgcccttgactctcggcaggtatgaccctgggtgcctgtgagctaggagaggaaattctgtatgcagggcaaacatgttacaaggggaggagatggcactgcacttcaggtctccaaatgcagtgtgctaggaatggcctcgctgacagttggaatcacggatacattaattacagcgaaggcaaaagtaagctacagtgacagggagctgggggcggagggagaaggcactttgccatgggagcacatctgttttataataagcaggtctataattctcttgtgaaagatcatgttctgctatcttctctgaggctggaaaatataaatactgtattttaccaagaggaggaggaaaggagatgatcaaatttgtttgcctgttgccaagtgtttgagattttccaccctttttcttttgtgtgcaacattctctttaactagagtgggggaaaagtcaacctgcttttctaagggtaaaaggcaccgtcaggcgtctcatgaatagggccctggccttttaacaagttttcaagccttggttgcggctactgtatagtcagaaaataaatgcatgtatggtgttgagctattaaggtgaaatgtgtggcctggggccaaaggaactggtgtgggttgagaggtaaaatgcttacatctaactgcacaaaagtcagtctgaaatgtcacatctctagatggatggaagtatcatgagttggggtcttggggaagcggcgtgtgggggaaaggagcaatggggttgaatgtaccaagtatgttgtgagccactgatcctaatagcagcaaaactactaaaccatgaagacatagaaggcatctgctcagcgcgaaagctacagaatcttctcataaagtctactgagaactgttccattataaacatatttttcttgctctagggagagttaaggggaaggaatgggagctgtcagggtcccagggctgtcctacctgccgttttggtcacagtgactgccacgtgctcttccaagggcactgcagctggagaacactacctgccaaatagcaaagcagatctctttcttactcctattatttattttagcactctttgttttacttcaaggtggcaattatatatgtgtgtgtatatatatatatttatttaaataatattagatctaattcattaattatacttgtaagtttgtattttcttaatagtccaaagttggtattttgaagttccacattactctgattttttaaacaaaaaaatgagaaagcaagaatggtcacattgacaaaggtcgaaatgaaagtgcaggaagaacaacgagaaataaagcacttaaaatgaataggtaggaactgcctccacaggattctgagaaaagaaactaaaacgaccctctttgggaatatacttactagatagccttatctaccagtctacacgacgatgtctttaacaaccaccccaggacatttcctccggccagcatcatgaaaaaaatcataaatatcaaccatgggcacccgttgaaaactgttaagaaagccatgtgtacagcctggaaaacacggtggagcgtcacatcattaggtgggtgatgggattagtaccgaaaaacagaccgacaacacgcagttattggtcgcagaggtttcttctcttctcaggaaaaaaacttctgagattaacttcaaaaccagaaccagccctcctcataaatgaggggtgtatgctttctgtcagagggggcttggctcctgtttccagccatcggctctgcttacgtgattccccgcctccacaggaggaactgaggcgggagcgccacggacaccaggtcctggaaggacccagcagtctcttgtgttttgaaggttttcttatgaaacagatgatgatgggtgcctgcctcagttacctcagcctctgtgaaggctaaaaataaataacacaaaaataacctaaagcactgttttgtgcaggaaatgcttccttttgtgtcttgggtaataaaatgtaccgagagacagagagaaaaaaaaagtctgaactataaagcattgtgtataccacgttttgtctgggagcaagcagctgaaattcttggctaagtgtaatccagctattggtagtttctcgagccacagaggttctgtggatcgtctggacaatgatgtacacagagcatacgtacaggacgtataggtatttgcgtatatataaataaatatatatatctatatctagttgaagaggatacatactcttcttccaaaggggtctaactggctagttaggaggccgctctggggctgatggattgttgattggtgaatccctggccttcgggtcggctggagtcaggtgttctggtaggacagctcgaacatggtgcaagcctcctctagactctcgtccatgttcagtctctgccagaaagacttctgcttcttctgcagctctcggcgaacacacctcgggcaggggacagacttttctttgcattcagaatggaaaacggctccacagctttcacacctgctgcaggtcggcaagtgaatacaggtggatctgttgaaggaggtattctctggggaaaattctgcggcggagatcctctgccaccgctgcccggcagctgaacaaataggctcggagcgacttcagccgctgccgcagccgcagcacggcggccagcggctctgcgtggtggtacagcatggcgttctcctgctggatgtcgatgagcggctcttcgtacacgtactccagaaactccttggcctgcttcgacaccttatactttgaagtatcccagttgtggactatgcgtgctggaatgagaaagctgtcatccacgtggcagctactgcagtaataccacccactgtagttgcacaccttggctttcccattggaaagacctatggatcgctggcagcctgcacatttgaaactctgagcagtgagtcctcgttccaaagacaaagtcgtcaaaatgctcaggaagctggtagtcacagattggcgtttgttcttcctgagttcatgcccacccatttgatccttgggtttgttcctcagtgtgacttgcaggttttgctctgaactcctcgccacattggcagctatcttcagagcctccatccattcctgagccctctgtcgggtctcagctcggaggcgaaggacatcctgggggaaaatgacttgaaagcaagagtcgcagccatccaggttgtccatctggacagccagacacacgtccacgttgtagctcaacagtggatcctcgtctagcttgccaggctgaaaagccataaggtaagccctgctcagcacaaatgtaaatgccttccagttgttttggacagtcagcctgtagagagtccctgatttgaggatgttttggtactgtttggagctgtccaggacaggggacggtggcagcagcccactggttttcttctggaaactatgattctgtgtatagtcatcatgatggccaagccctggtgagattgtcagctcattctgccgccccatgtaaccgggcacagcagcatgcactacttcccaaagcttctgtccccagtccaaagcctcccatggtgactctgcctttagctgtagctgagtgttgtcatacaaaacagtatccaccatcctggcctccaggttgcctaaaacagatatgctctggaagtgtgaaagctggtacgtggcataaaggttttgattcccactgctgtcgaggctgtagaagtataagttgtaaggtgaaagttctgcataacagctttgccagtaactgtcatggtcctttctaatctccaggtaacccttctttagaatgtttgggaatgtctgcttgtgttcagtatttccttgagcatcttctatcttatttggtgagggcaacagaaaagatggcctggtgacatgcgggccttgaagcaatggctgctgctgttgctgctgctgcaaaggcgtggttttgaggactaccctccagtccacttgggtaatatctgatcgtgatcgagcatgccctggcttgaaagttgaggtctcatccagtaagtcatttacagaacgaggccggtccctccgacgctgacagatattgaagaaattaaaggttgatgcttccttttgttccatccaggaaagattatctggggttgtccctctctggaccataaactgttctttggcagggaagacattttgagctttggtttctaagagcctgctcttacagtggtcccaaatcatgccccccttgcccagggaggtgacatttctcatagcaccattgtctgttatgttactgagtacctcatgccccaccagttcagggacttcctggatcccataaacctctgcctgctgcacagccttttctagattactatccaaagtactaaagaattcctccgtaacttctaaggctgggctgatatcatccacttccaaagcttccatgtcacaggctccaggaggccttagcctcctaagctggttccagaaatggcttcatgaacattcacccaaccaagaggggtgcttcagcaatagagctatggaaacaactggaagaaaccttcattgggctccctggagcaggccaaacccaaagtggttgatgttttcctggtaattaaaagcatttgctagtggctaatgggcattaacagatgtatagggagaccaaatgttcctttgagattattcttcagtgagacctctgtgaagacaacagcaagtacttgtcaaagcaatgccacgccaatccttgatttcctgggccccggctgctactctccattcacctgcggggccttcagtccgctcctggaggggcttgactcccgcagcctgccgcccgcctcacggtgacagcccgcccgggcgctgaccatcccggcccggctctgtttacaagcggcttctcgcggtcccactctgaaatgct

SEQ ID NO: 14912 - RNA, 6592 nt, Homo sapiens
  source 1..6592: mol_type = other RNA
gctgggattacaggcatgagccactacgttcagcctaatttttttatttttagtatagacctgatttcaccatttttggcccggctggtctcaaactcctgacctcaagtgatctgcctgccttggcctcccaaagggctgggattacaggcgtgagccaccaatcctggccaagtggaacccactttaaataaaactgacaactaccggtatggttaggagggtatcccatactcttgtcttttacctagagtttaacaatgacttggattttccctcagccatgcacccattaaaacgcactaaggaaagacccttgagtcagagatttttgaatccaatgaaattagaatcgtctaccaataaggagactactgggtgctagacttaactgtcgaaacaccgttccacatgacagaaatcaacacttgtctgtttacattaaccgagcagagcttagtcacccatcactggattcgacctcgagcagacagctctacctgactcagggtcggaagagtgatacaaggtgtgcaacatatgaagctcctaatgcccatcactaacaagtgacacggaggcaggggaaacagagagtgccgctaccgattcaggtcacgcaaaggagggaggctctttcaaggtcttgctccaacttcacgttttcacattatttcagagtaagaaaagaagtggtgcagacaactcaagaaataaaatgggcaaaaattatacacatctctatttactaggagaagtaaaaaaataaaacaacccctgtgttgaaaccaggcagtattggaatcaggaggtgaagatctgtttcataatctagtgatttcaagagagtgtgtcagatcaacggagatgaataattgtgcacaaatacacgagcaacagcattggcttgactctaaaggaggaccagaatgtgtctctacttccactgctaacgcccctctgcagaaaatgttcagtgtgcgtggcatcgtgctagtcccacctggatatactaatttatggacggccttttctagccaatgggtagagaacaaactcccaggtttggaagccaagcctctctgaggaggcacagaaaagaactatccgatgtccacgttcagtgtgtacacacaacacacagagacaaaaacagaggccaggctccgtcagaggacacactctagctgagcaaaggctgcattcggcaactagggtggtgtaaacacctcggatctcactgcagccggaaggaagtcacggcatagtcccttttcaggagtctgagggataccacttgtgttgcaaaccacagatcccaagtattagacgtattcccttcttggtggaggcctactctagaagaatcaaaaaccgatgaccctctcagcgaatccgatgttaaagctcctaactaggtgaccctttagcactacagacgtaaaaatgactctaatgcactccctagaaaaggcagtgaagcaaagggggctgctgagagtttacatggttttcatataaagaggcttttaactttggaaaaagcgggcctggaaagaacactacccccattccagttgacggctttttaagtactttgtggccttcctgccgcggtgcaaaatgaggtctattttaggaactggcttctttactgcggggttagatgccaacatttcaccagggttggacgatctcacacatgagtttctggcacttttaggagggatttcctcaagtgatacactagggaatgagcctttcagcaaaaagcggttccccggagtcagttgccagctccaggagattaattggccattttttcatatgttttatgtgcaagatatttaatatgggatgaaaaatggaacacgaggaaaagcaggtattagtttggtctgaaagaggtggtaatccacagatttgcttttgtttcgacagtttctaagcagtggaacaattacctaacagtgcaccaagtaatttgttaaagttgaaaacagtaagggcgttcatgtgcgccaaggtattctgggctgaaaacagcaattttgaattttcatggcagacccaactcctaagctggctccactctgtcctatcagattttggtggtggtggcagagaatgtcataggcctgtggctggcaccgaccaagctgtcagggtggtacgaaaaggagaggaaacaggagtgctggacatggacccagctctgggtagctgatggtgataacacatcgattttttgtttcccttttgaaaataagcagaaaatgatgtgggtggaaagtcctccttaggagttcacagggactgctcgtatttagcagggccctctaaatggggactggtgaaaacaaagatgttttgaacggggatccagaatttcgcccttgactctcggcaggtatgaccctgggtgcctgtgagctaggagaggaaattctgtatgcagggcaaacatgttacaaggggaggagatggcactgcacttcaggtctccaaatgcagtgtgctaggaatggcctcgctgacagttggaatcacggatacattaattacagcgaaggcaaaagtaagctacagtgacagggagctgggggcggagggagaaggcactttgccatgggagcacatctgttttataataagcaggtctataattctcttgtgaaagatcatgttctgctatcttctctgaggctggaaaatataaatactgtattttaccaagaggaggaggaaaggagatgatcaaatttgtttgcctgttgccaagtgtttgagattttccaccctttttcttttgtgtgcaacattctctttaactagagtgggggaaaagtcaacctgcttttctaagggtaaaaggcaccgtcaggcgtctcatgaatagggccctggccttttaacaagttttcaagccttggttgcggctactgtatagtcagaaaataaatgcatgtatggtgttgagctattaaggtgaaatgtgtggcctggggccaaaggaactggtgtgggttgagaggtaaaatgcttacatctaactgcacaaaagtcagtctgaaatgtcacatctctagatggatggaagtatcatgagttggggtcttggggaagcggcgtgtgggggaaaggagcaatggggttgaatgtaccaagtatgttgtgagccactgatcctaatagcagcaaaactactaaaccatgaagacatagaaggcatctgctcagcgcgaaagctacagaatcttctcataaagtctactgagaactgttccattataaacatatttttcttgctctagggagagttaaggggaaggaatgggagctgtcagggtcccagggctgtcctacctgccgttttggtcacagtgactgccacgtgctcttccaagggcactgcagctggagaacactacctgccaaatagcaaagcagatctctttcttactcctattatttattttagcactctttgttttacttcaaggtggcaattatatatgtgtgtgtatatatatatatttatttaaataatattagatctaattcattaattatacttgtaagtttgtattttcttaatagtccaaagttggtattttgaagttccacattactctgattttttaaacaaaaaaatgagaaagcaagaatggtcacattgacaaaggtcgaaatgaaagtgcaggaagaacaacgagaaataaagcacttaaaatgaataggtaggaactgcctccacaggattctgagaaaagaaactaaaacgaccctctttgggaatatacttactagatagccttatctaccagtctacacgacgatgtctttaacaaccaccccaggacatttcctccggccagcatcatgaaaaaaatcataaatatcaaccatgggcacccgttgaaaactgttaagaaagccatgtgtacagcctggaaaacacggtggagcgtcacatcattaggtgggtgatgggattagtaccgaaaaacagaccgacaacacgcagttattggtcgcagaggtttcttctcttctcaggaaaaaaacttctgagattaacttcaaaaccagaaccagccctcctcataaatgaggggtgtatgctttctgtcagagggggcttggctcctgtttccagccatcggctctgcttacgtgattccccgcctccacaggaggaactgaggcgggagcgccacggacaccaggtcctggaaggacccagcagtctcttgtgttttgaaggttttcttatgaaacagatgatgatgggtgcctgcctcagttacctcagcctctgtgaaggctaaaaataaataacacaaaaataacctaaagcactgttttgtgcaggaaatgcttccttttgtgtcttgggtaataaaatgtaccgagagacagagagaaaaaaaaagtctgaactataaagcattgtgtataccacgttttgtctgggagcaagcagctgaaattcttggctaagtgtaatccagctattggtagtttctcgagccacagaggttctgtggatcgtctggacaatgatgtacacagagcatacgtacaggacgtataggtatttgcgtatatataaataaatatatatatctatatctagttgaagaggatacatactcttcttccaaaggggtctaactggctagttaggaggccgctctggggctgatggattgttgattggtgaatccctggccttcgggtcggctggagtcaggtgttctggtaggacagctcgaacatggtgcaagcctcctctagactctcgtccatgttcagtctctgccagaaagacttctgcttcttctgcagctctcggcgaacacacctcgggcaggggacagacttttctttgcattcagaatggaaaacggctccacagctttcacacctgcttgttgaaatatcctcaaaagggtagaggatctctccattgttacagatttcacagatgaaccccttctggctacaaagactgcagctgtacacgtgtgaggtggcaaatttaatgaccttgcccaagaatggagccagctttccctctattacctgctgcaggtcggcaagtgaatacaggtggatctgttgaaggaggtattctctggggaaaattctgcggcggagatcctctgccaccgctgcccggcagctgaacaaataggctcggagcgacttcagccgctgccgcagccgcagcacggcggccagcggctctgcgtggtggtacagcatggcgttctcctgctggatgtcgatgagcggctcttcgtacacgtactccagaaactccttggcctgcttcgacaccttatactttgaagtatcccagttgtggactatgcgtgctggaatgagaaagctgtcatccacgtggcagctactgcagtaataccacccactgtagttgcacaccttggctttcccattggaaagacctatggatcgctggcagccagtatttccttgagcatcttctatcttatttggtgagggcaacagaaaagatggcctggtgacatgcgggccttgaagcaatggctgctgctgttgctgctgctgcaaaggcgtggttttgaggactaccctccagtccacttgggtaatatctgatcgtgatcgagcatgccctggcttgaaagttgaggtctcatccagtaagtcatttacagaacgaggccggtccctccgacgctgacagatattgaagaaattaaaggttgatgcttccttttgttccatccaggaaagattatctggggttgtccctctctggaccataaactgttctttggcagggaagacattttgagctttggtttctaagagcctgctcttacagtggtcccaaatcatgccccccttgcccagggaggtgacatttctcatagcaccattgtctgttatgttactgagtacctcatgccccaccagttcagggacttcctggatcccataaacctctgcctgctgcacagccttttctagattactatccaaagtactaaagaattcctccgtaacttctaaggctgggctgatatcatccacttccaaagcttccatgtcacaggctccaggaggccttagcctcctaagctggttccagaaatggcttcatgaacattcacccaaccaagaggggtgcttcagcaatagagctatggaaacaactggaagaaaccttcattgggctccctggagcaggccaaacccaaagtggttgatgttttcctggtaattaaaagcatttgctagtggctaatgggcattaacagatgtatagggagaccaaatgttcctttgagattattcttcagtgagacctctgtgaagacaacagcaagtacttgtcaaagcaatgccacgccaatccttgatttcctgggccccggctgctactctccattcacctgcggggccttcagtccgctcctggaggggcttgactcccgcagcctgccgcccgcctcacggtgacagcccgcccgggcgctgaccatcccggcccggctctgtttacaagcggcttctcgcggtcccactctgaaatgct

SEQ ID NO: 14913 - RNA, 6953 nt, Homo sapiens
  source 1..6953: mol_type = other RNA
gctgggattacaggcatgagccactacgttcagcctaatttttttatttttagtatagacctgatttcaccatttttggcccggctggtctcaaactcctgacctcaagtgatctgcctgccttggcctcccaaagggctgggattacaggcgtgagccaccaatcctggccaagtggaacccactttaaataaaactgacaactaccggtatggttaggagggtatcccatactcttgtcttttacctagagtttaacaatgacttggattttccctcagccatgcacccattaaaacgcactaaggaaagacccttgagtcagagatttttgaatccaatgaaattagaatcgtctaccaataaggagactactgggtgctagacttaactgtcgaaacaccgttccacatgacagaaatcaacacttgtctgtttacattaaccgagcagagcttagtcacccatcactggattcgacctcgagcagacagctctacctgactcagggtcggaagagtgatacaaggtgtgcaacatatgaagctcctaatgcccatcactaacaagtgacacggaggcaggggaaacagagagtgccgctaccgattcaggtcacgcaaaggagggaggctctttcaaggtcttgctccaacttcacgttttcacattatttcagagtaagaaaagaagtggtgcagacaactcaagaaataaaatgggcaaaaattatacacatctctatttactaggagaagtaaaaaaataaaacaacccctgtgttgaaaccaggcagtattggaatcaggaggtgaagatctgtttcataatctagtgatttcaagagagtgtgtcagatcaacggagatgaataattgtgcacaaatacacgagcaacagcattggcttgactctaaaggaggaccagaatgtgtctctacttccactgctaacgcccctctgcagaaaatgttcagtgtgcgtggcatcgtgctagtcccacctggatatactaatttatggacggccttttctagccaatgggtagagaacaaactcccaggtttggaagccaagcctctctgaggaggcacagaaaagaactatccgatgtccacgttcagtgtgtacacacaacacacagagacaaaaacagaggccaggctccgtcagaggacacactctagctgagcaaaggctgcattcggcaactagggtggtgtaaacacctcggatctcactgcagccggaaggaagtcacggcatagtcccttttcaggagtctgagggataccacttgtgttgcaaaccacagatcccaagtattagacgtattcccttcttggtggaggcctactctagaagaatcaaaaaccgatgaccctctcagcgaatccgatgttaaagctcctaactaggtgaccctttagcactacagacgtaaaaatgactctaatgcactccctagaaaaggcagtgaagcaaagggggctgctgagagtttacatggttttcatataaagaggcttttaactttggaaaaagcgggcctggaaagaacactacccccattccagttgacggctttttaagtactttgtggccttcctgccgcggtgcaaaatgaggtctattttaggaactggcttctttactgcggggttagatgccaacatttcaccagggttggacgatctcacacatgagtttctggcacttttaggagggatttcctcaagtgatacactagggaatgagcctttcagcaaaaagcggttccccggagtcagttgccagctccaggagattaattggccattttttcatatgttttatgtgcaagatatttaatatgggatgaaaaatggaacacgaggaaaagcaggtattagtttggtctgaaagaggtggtaatccacagatttgcttttgtttcgacagtttctaagcagtggaacaattacctaacagtgcaccaagtaatttgttaaagttgaaaacagtaagggcgttcatgtgcgccaaggtattctgggctgaaaacagcaattttgaattttcatggcagacccaactcctaagctggctccactctgtcctatcagattttggtggtggtggcagagaatgtcataggcctgtggctggcaccgaccaagctgtcagggtggtacgaaaaggagaggaaacaggagtgctggacatggacccagctctgggtagctgatggtgataacacatcgattttttgtttcccttttgaaaataagcagaaaatgatgtgggtggaaagtcctccttaggagttcacagggactgctcgtatttagcagggccctctaaatggggactggtgaaaacaaagatgttttgaacggggatccagaatttcgcccttgactctcggcaggtatgaccctgggtgcctgtgagctaggagaggaaattctgtatgcagggcaaacatgttacaaggggaggagatggcactgcacttcaggtctccaaatgcagtgtgctaggaatggcctcgctgacagttggaatcacggatacattaattacagcgaaggcaaaagtaagctacagtgacagggagctgggggcggagggagaaggcactttgccatgggagcacatctgttttataataagcaggtctataattctcttgtgaaagatcatgttctgctatcttctctgaggctggaaaatataaatactgtattttaccaagaggaggaggaaaggagatgatcaaatttgtttgcctgttgccaagtgtttgagattttccaccctttttcttttgtgtgcaacattctctttaactagagtgggggaaaagtcaacctgcttttctaagggtaaaaggcaccgtcaggcgtctcatgaatagggccctggccttttaacaagttttcaagccttggttgcggctactgtatagtcagaaaataaatgcatgtatggtgttgagctattaaggtgaaatgtgtggcctggggccaaaggaactggtgtgggttgagaggtaaaatgcttacatctaactgcacaaaagtcagtctgaaatgtcacatctctagatggatggaagtatcatgagttggggtcttggggaagcggcgtgtgggggaaaggagcaatggggttgaatgtaccaagtatgttgtgagccactgatcctaatagcagcaaaactactaaaccatgaagacatagaaggcatctgctcagcgcgaaagctacagaatcttctcataaagtctactgagaactgttccattataaacatatttttcttgctctagggagagttaaggggaaggaatgggagctgtcagggtcccagggctgtcctacctgccgttttggtcacagtgactgccacgtgctcttccaagggcactgcagctggagaacactacctgccaaatagcaaagcagatctctttcttactcctattatttattttagcactctttgttttacttcaaggtggcaattatatatgtgtgtgtatatatatatatttatttaaataatattagatctaattcattaattatacttgtaagtttgtattttcttaatagtccaaagttggtattttgaagttccacattactctgattttttaaacaaaaaaatgagaaagcaagaatggtcacattgacaaaggtcgaaatgaaagtgcaggaagaacaacgagaaataaagcacttaaaatgaataggtaggaactgcctccacaggattctgagaaaagaaactaaaacgaccctctttgggaatatacttactagatagccttatctaccagtctacacgacgatgtctttaacaaccaccccaggacatttcctccggccagcatcatgaaaaaaatcataaatatcaaccatgggcacccgttgaaaactgttaagaaagccatgtgtacagcctggaaaacacggtggagcgtcacatcattaggtgggtgatgggattagtaccgaaaaacagaccgacaacacgcagttattggtcgcagaggtttcttctcttctcaggaaaaaaacttctgagattaacttcaaaaccagaaccagccctcctcataaatgaggggtgtatgctttctgtcagagggggcttggctcctgtttccagccatcggctctgcttacgtgattccccgcctccacaggaggaactgaggcgggagcgccacggacaccaggtcctggaaggacccagcagtctcttgtgttttgaaggttttcttatgaaacagatgatgatgggtgcctgcctcagttacctcagcctctgtgaaggctaaaaataaataacacaaaaataacctaaagcactgttttgtgcaggaaatgcttccttttgtgtcttgggtaataaaatgtaccgagagacagagagaaaaaaaaagtctgaactataaagcattgtgtataccacgttttgtctgggagcaagcagctgaaattcttggctaagtgtaatccagctattggtagtttctcgagccacagaggttctgtggatcgtctggacaatgatgtacacagagcatacgtacaggacgtataggtatttgcgtatatataaataaatatatatatctatatctagttgaagaggatacatactcttcttccaaaggggtctaactggctagttaggaggccgctctggggctgatggattgttgattggtgaatccctggccttcgggtcggctggagtcaggtgttctggtaggacagctcgaacatggtgcaagcctcctctagactctcgtccatgttcagtctctgccagaaagacttctgcttcttctgcagctctcggcgaacacacctcgggcaggggacagacttttctttgcattcagaatggaaaacggctccacagctttcacacctgcttgttgaaatatcctcaaaagggtagaggatctctccattgttacagatttcacagatgaaccccttctggctacaaagactgcagctgtacacgtgtgaggtggcaaatttaatgaccttgcccaagaatggagccagctttccctctattacctgctgcaggtcggcaagtgaatacaggtggatctgttgaaggaggtattctctggggaaaattctgcggcggagatcctctgccaccgctgcccggcagctgaacaaataggctcggagcgacttcagccgctgccgcagccgcagcacggcggccagcggctctgcgtggtggtacagcatggcgttctcctgctggatgtcgatgagcggctcttcgtacacgtactccagaaactccttggcctgcttcgacaccttatactttgaagtatcccagttgtggactatgcgtgctggaatgagaaagctgtcatccacgtggcagctactgcagtaataccacccactgtagttgcacaccttggctttcccattggaaagacctatggatcgctggcagcctgcacatttgaaactctgagcagtgagtcctcgttccaaagacaaagtcgtcaaaatgctcaggaagctggtagtcacagattggcgtttgttcttcctgagttcatgcccacccatttgatccttgggtttgttcctcagtgtgacttgcaggttttgctctgaactcctcgccacattggcagctatcttcagagcctccatccattcctgagccctctgtcgggtctcagctcggaggcgaaggacatcctgggggaaaatgacttgaaagcaagagtcgcagccatccaggttgtccatctggacagccagacacacgtccacgttgtagctcaacagtggatcctcgtctagcttgccaggctgaaaagccataaggtaagccctgctcagcacaaatgtaaatgccttccagttgttttggacagtcagcctgtagagagtccctgatttgaggatgttttggtactgtttggagctgtccaggacaggggacggtggcagcagcccactggttttcttctggaaactatgattctgtgtatagtcatcatgatggccaagccctggtgagattgtcagctcattctgccgccccatgtaaccgggcacagcagcatgcactacttcccaaagcttctgtccccagtccaaagcctcccatggtgactctgcctttagctgtagctgagtgttgtcatacaaaacagtatccaccatcctggcctccaggttgcctaaaacagatatgctctggaagtgtgaaagctggtacgtggcataaaggttttgattcccactgctgtcgaggctgtagaagtataagttgtaaggtgaaagttctgcataacagctttgccagtaactgtcatggtcctttctaatctccaggtaacccttctttagaatgtttgggaatgtctgcttgtgttcaggcagttggagatgcgagtctgcagctcaaggaagaggtcttgcctgaccccagatctcctgggtcctcatctccagctctagccaaggtactacactgcctccctctgcttttggcatattcctcaggagaaacaacgagtctttcttcagtttggattactaacttcaaaggttttaaaataaattttactcagagatcttggctgattttgactagttggcacctggatattggcacacccctccacaaatgcttatgagaataccggcctcagaataggtgatcagccatgcaatctagaactccagcctgagaatgggtggccactgcttgcccctgcccttcaactgatgggcaataggaatatgatttatcttgcctgctctccagagaatgccgaaagaaaaggtgtcaaaaacttggcatgccatttactcacattcgctatctcctggatgactaaaaggtggcagtggctgggagcagtggctcacgcctgtaaccccaacagtttgagagg

SEQ ID NO: 14914 - RNA, 7495 nt, Homo sapiens
  source 1..7495: mol_type = other RNA
gctgggattacaggcatgagccactacgttcagcctaatttttttatttttagtatagacctgatttcaccatttttggcccggctggtctcaaactcctgacctcaagtgatctgcctgccttggcctcccaaagggctgggattacaggcgtgagccaccaatcctggccaagtggaacccactttaaataaaactgacaactaccggtatggttaggagggtatcccatactcttgtcttttacctagagtttaacaatgacttggattttccctcagccatgcacccattaaaacgcactaaggaaagacccttgagtcagagatttttgaatccaatgaaattagaatcgtctaccaataaggagactactgggtgctagacttaactgtcgaaacaccgttccacatgacagaaatcaacacttgtctgtttacattaaccgagcagagcttagtcacccatcactggattcgacctcgagcagacagctctacctgactcagggtcggaagagtgatacaaggtgtgcaacatatgaagctcctaatgcccatcactaacaagtgacacggaggcaggggaaacagagagtgccgctaccgattcaggtcacgcaaaggagggaggctctttcaaggtcttgctccaacttcacgttttcacattatttcagagtaagaaaagaagtggtgcagacaactcaagaaataaaatgggcaaaaattatacacatctctatttactaggagaagtaaaaaaataaaacaacccctgtgttgaaaccaggcagtattggaatcaggaggtgaagatctgtttcataatctagtgatttcaagagagtgtgtcagatcaacggagatgaataattgtgcacaaatacacgagcaacagcattggcttgactctaaaggaggaccagaatgtgtctctacttccactgctaacgcccctctgcagaaaatgttcagtgtgcgtggcatcgtgctagtcccacctggatatactaatttatggacggccttttctagccaatgggtagagaacaaactcccaggtttggaagccaagcctctctgaggaggcacagaaaagaactatccgatgtccacgttcagtgtgtacacacaacacacagagacaaaaacagaggccaggctccgtcagaggacacactctagctgagcaaaggctgcattcggcaactagggtggtgtaaacacctcggatctcactgcagccggaaggaagtcacggcatagtcccttttcaggagtctgagggataccacttgtgttgcaaaccacagatcccaagtattagacgtattcccttcttggtggaggcctactctagaagaatcaaaaaccgatgaccctctcagcgaatccgatgttaaagctcctaactaggtgaccctttagcactacagacgtaaaaatgactctaatgcactccctagaaaaggcagtgaagcaaagggggctgctgagagtttacatggttttcatataaagaggcttttaactttggaaaaagcgggcctggaaagaacactacccccattccagttgacggctttttaagtactttgtggccttcctgccgcggtgcaaaatgaggtctattttaggaactggcttctttactgcggggttagatgccaacatttcaccagggttggacgatctcacacatgagtttctggcacttttaggagggatttcctcaagtgatacactagggaatgagcctttcagcaaaaagcggttccccggagtcagttgccagctccaggagattaattggccattttttcatatgttttatgtgcaagatatttaatatgggatgaaaaatggaacacgaggaaaagcaggtattagtttggtctgaaagaggtggtaatccacagatttgcttttgtttcgacagtttctaagcagtggaacaattacctaacagtgcaccaagtaatttgttaaagttgaaaacagtaagggcgttcatgtgcgccaaggtattctgggctgaaaacagcaattttgaattttcatggcagacccaactcctaagctggctccactctgtcctatcagattttggtggtggtggcagagaatgtcataggcctgtggctggcaccgaccaagctgtcagggtggtacgaaaaggagaggaaacaggagtgctggacatggacccagctctgggtagctgatggtgataacacatcgattttttgtttcccttttgaaaataagcagaaaatgatgtgggtggaaagtcctccttaggagttcacagggactgctcgtatttagcagggccctctaaatggggactggtgaaaacaaagatgttttgaacggggatccagaatttcgcccttgactctcggcaggtatgaccctgggtgcctgtgagctaggagaggaaattctgtatgcagggcaaacatgttacaaggggaggagatggcactgcacttcaggtctccaaatgcagtgtgctaggaatggcctcgctgacagttggaatcacggatacattaattacagcgaaggcaaaagtaagctacagtgacagggagctgggggcggagggagaaggcactttgccatgggagcacatctgttttataataagcaggtctataattctcttgtgaaagatcatgttctgctatcttctctgaggctggaaaatataaatactgtattttaccaagaggaggaggaaaggagatgatcaaatttgtttgcctgttgccaagtgtttgagattttccaccctttttcttttgtgtgcaacattctctttaactagagtgggggaaaagtcaacctgcttttctaagggtaaaaggcaccgtcaggcgtctcatgaatagggccctggccttttaacaagttttcaagccttggttgcggctactgtatagtcagaaaataaatgcatgtatggtgttgagctattaaggtgaaatgtgtggcctggggccaaaggaactggtgtgggttgagaggtaaaatgcttacatctaactgcacaaaagtcagtctgaaatgtcacatctctagatggatggaagtatcatgagttggggtcttggggaagcggcgtgtgggggaaaggagcaatggggttgaatgtaccaagtatgttgtgagccactgatcctaatagcagcaaaactactaaaccatgaagacatagaaggcatctgctcagcgcgaaagctacagaatcttctcataaagtctactgagaactgttccattataaacatatttttcttgctctagggagagttaaggggaaggaatgggagctgtcagggtcccagggctgtcctacctgccgttttggtcacagtgactgccacgtgctcttccaagggcactgcagctggagaacactacctgccaaatagcaaagcagatctctttcttactcctattatttattttagcactctttgttttacttcaaggtggcaattatatatgtgtgtgtatatatatatatttatttaaataatattagatctaattcattaattatacttgtaagtttgtattttcttaatagtccaaagttggtattttgaagttccacattactctgattttttaaacaaaaaaatgagaaagcaagaatggtcacattgacaaaggtcgaaatgaaagtgcaggaagaacaacgagaaataaagcacttaaaatgaataggtaggaactgcctccacaggattctgagaaaagaaactaaaacgaccctctttgggaatatacttactagatagccttatctaccagtctacacgacgatgtctttaacaaccaccccaggacatttcctccggccagcatcatgaaaaaaatcataaatatcaaccatgggcacccgttgaaaactgttaagaaagccatgtgtacagcctggaaaacacggtggagcgtcacatcattaggtgggtgatgggattagtaccgaaaaacagaccgacaacacgcagttattggtcgcagaggtttcttctcttctcaggaaaaaaacttctgagattaacttcaaaaccagaaccagccctcctcataaatgaggggtgtatgctttctgtcagagggggcttggctcctgtttccagccatcggctctgcttacgtgattccccgcctccacaggaggaactgaggcgggagcgccacggacaccaggtcctggaaggacccagcagtctcttgtgttttgaaggttttcttatgaaacagatgatgatgggtgcctgcctcagttacctcagcctctgtgaaggctaaaaataaataacacaaaaataacctaaagcactgttttgtgcaggaaatgcttccttttgtgtcttgggtaataaaatgtaccgagagacagagagaaaaaaaaagtctgaactataaagcattgtgtataccacgttttgtctgggagcaagcagctgaaattcttggctaagtgtaatccagctattggtagtttctcgagccacagaggttctgtggatcgtctggacaatgatgtacacagagcatacgtacaggacgtataggtatttgcgtatatataaataaatatatatatctatatctagttgaagaggatacatactcttcttccaaaggggtctaactggctagttaggaggccgctctggggctgatggattgttgattggtgaatccctggccttcgggtcggctggagtcaggtgttctggtaggacagctcgaacatggtgcaagcctcctctagactctcgtccatgttcagtctctgccagaaagacttctgcttcttctgcagctctcggcgaacacacctcgggcaggggacagacttttctttgcattcagaatggaaaacggctccacagctttcacacctgcttgttgaaatatcctcaaaagggtagaggatctctccattgttacagatttcacagatgaaccccttctggctacaaagactgcagctgtacacgtgtgaggtggcaaatttaatgaccttgcccaagaatggagccagctttccctctattacctgctgcaggtcggcaagtgaatacaggtggatctgttgaaggaggtattctctggggaaaattctgcggcggagatcctctgccaccgctgcccggcagctgaacaaataggctcggagcgacttcagccgctgccgcagccgcagcacggcggccagcggctctgcgtggtggtacagcatggcgttctcctgctggatgtcgatgagcggctcttcgtacacgtactccagaaactccttggcctgcttcgacaccttatactttgaagtatcccagttgtggactatgcgtgctggaatgagaaagctgtcatccacgtggcagctactgcagtaataccacccactgtagttgcacaccttggctttcccattggaaagacctatggatcgctggcagcctgcacatttgaaactctgagcagtgagtcctcgttccaaagacaaagtcgtcaaaatgctcaggaagctggtagtcacagattggcgtttgttcttcctgagttcatgcccacccatttgatccttgggtttgttcctcagtgtgacttgcaggttttgctctgaactcctcgccacattggcagctatcttcagagcctccatccattcctgagccctctgtcgggtctcagctcggaggcgaaggacatcctgggggaaaatgacttgaaagcaagagtcgcagccatccaggttgtccatctggacagccagacacacgtccacgttgtagctcaacagtggatcctcgtctagcttgccaggctgaaaagccataaggtaagccctgctcagcacaaatgtaaatgccttccagttgttttggacagtcagcctgtagagagtccctgatttgaggatgttttggtactgtttggagctgtccaggacaggggacggtggcagcagcccactggttttcttctggaaactatgattctgtgtatagtcatcatgatggccaagccctggtgagattgtcagctcattctgccgccccatgtaaccgggcacagcagcatgcactacttcccaaagcttctgtccccagtccaaagcctcccatggtgactctgcctttagctgtagctgagtgttgtcatacaaaacagtatccaccatcctggcctccaggttgcctaaaacagatatgctctggaagtgtgaaagctggtacgtggcataaaggttttgattcccactgctgtcgaggctgtagaagtataagttgtaaggtgaaagttctgcataacagctttgccagtaactgtcatggtcctttctaatctccaggtaacccttctttagaatgtttgggaatgtctgcttgtgttcagtatttccttgagcatcttctatcttatttggtgagggcaacagaaaagatggcctggtgacatgcgggccttgaagcaatggctgctgctgttgctgctgctgcaaaggcgtggttttgaggactaccctccagtccacttgggtaatatctgatcgtgatcgagcatgccctggcttgaaagttgaggtctcatccagtaagtcatttacagaacgaggccggtccctccgacgctgacagatattgaagaaattaaaggttgatgcttccttttgttccatccaggaaagattatctggggttgtccctctctggaccataaactgttctttggcagggaagacattttgagctttggtttctaagagcctgctcttacagtggtcccaaatcatgccccccttgcccagggaggtgacatttctcatagcaccattgtctgttatgttactgagtacctcatgccccaccagttcagggacttcctggatcccataaacctctgcctgctgcacagccttttctagattactatccaaagtactaaagaattcctccgtaacttctaaggctgggctgatatcatccacttccaaagcttccatgtcacaggctccaggaggccttagcctcctaagctggttccagaaatggcttcatgaacattcacccaaccaagaggggtgcttcagcaatagagctatggaaacaactggaagaaaccttcattgggctccctggagcaggccaaacccaaagtggttgatgttttcctggtaattaaaagcatttgctagtggctaatgggcattaacagatgtatagggagaccaaatgttcctttgagattattcttcagtgagacctctgtgaagacaacagcaagtacttgtcaaagcaatgccacgccaatccttgatttcctgggccccggctgctactctccattcacctgcggggccttcagtccgctcctggaggggcttgactcccgcagcctgccgcccgcctcacggtgacagcccgcccgggcgctgaccatcccggcccggctctgtttac

SEQ ID NO: 14915 - RNA, 7863 nt, Homo sapiens
  source 1..7863: mol_type = other RNA
gctgggattacaggcatgagccactacgttcagcctaatttttttatttttagtatagacctgatttcaccatttttggcccggctggtctcaaactcctgacctcaagtgatctgcctgccttggcctcccaaagggctgggattacaggcgtgagccaccaatcctggccaagtggaacccactttaaataaaactgacaactaccggtatggttaggagggtatcccatactcttgtcttttacctagagtttaacaatgacttggattttccctcagccatgcacccattaaaacgcactaaggaaagacccttgagtcagagatttttgaatccaatgaaattagaatcgtctaccaataaggagactactgggtgctagacttaactgtcgaaacaccgttccacatgacagaaatcaacacttgtctgtttacattaaccgagcagagcttagtcacccatcactggattcgacctcgagcagacagctctacctgactcagggtcggaagagtgatacaaggtgtgcaacatatgaagctcctaatgcccatcactaacaagtgacacggaggcaggggaaacagagagtgccgctaccgattcaggtcacgcaaaggagggaggctctttcaaggtcttgctccaacttcacgttttcacattatttcagagtaagaaaagaagtggtgcagacaactcaagaaataaaatgggcaaaaattatacacatctctatttactaggagaagtaaaaaaataaaacaacccctgtgttgaaaccaggcagtattggaatcaggaggtgaagatctgtttcataatctagtgatttcaagagagtgtgtcagatcaacggagatgaataattgtgcacaaatacacgagcaacagcattggcttgactctaaaggaggaccagaatgtgtctctacttccactgctaacgcccctctgcagaaaatgttcagtgtgcgtggcatcgtgctagtcccacctggatatactaatttatggacggccttttctagccaatgggtagagaacaaactcccaggtttggaagccaagcctctctgaggaggcacagaaaagaactatccgatgtccacgttcagtgtgtacacacaacacacagagacaaaaacagaggccaggctccgtcagaggacacactctagctgagcaaaggctgcattcggcaactagggtggtgtaaacacctcggatctcactgcagccggaaggaagtcacggcatagtcccttttcaggagtctgagggataccacttgtgttgcaaaccacagatcccaagtattagacgtattcccttcttggtggaggcctactctagaagaatcaaaaaccgatgaccctctcagcgaatccgatgttaaagctcctaactaggtgaccctttagcactacagacgtaaaaatgactctaatgcactccctagaaaaggcagtgaagcaaagggggctgctgagagtttacatggttttcatataaagaggcttttaactttggaaaaagcgggcctggaaagaacactacccccattccagttgacggctttttaagtactttgtggccttcctgccgcggtgcaaaatgaggtctattttaggaactggcttctttactgcggggttagatgccaacatttcaccagggttggacgatctcacacatgagtttctggcacttttaggagggatttcctcaagtgatacactagggaatgagcctttcagcaaaaagcggttccccggagtcagttgccagctccaggagattaattggccattttttcatatgttttatgtgcaagatatttaatatgggatgaaaaatggaacacgaggaaaagcaggtattagtttggtctgaaagaggtggtaatccacagatttgcttttgtttcgacagtttctaagcagtggaacaattacctaacagtgcaccaagtaatttgttaaagttgaaaacagtaagggcgttcatgtgcgccaaggtattctgggctgaaaacagcaattttgaattttcatggcagacccaactcctaagctggctccactctgtcctatcagattttggtggtggtggcagagaatgtcataggcctgtggctggcaccgaccaagctgtcagggtggtacgaaaaggagaggaaacaggagtgctggacatggacccagctctgggtagctgatggtgataacacatcgattttttgtttcccttttgaaaataagcagaaaatgatgtgggtggaaagtcctccttaggagttcacagggactgctcgtatttagcagggccctctaaatggggactggtgaaaacaaagatgttttgaacggggatccagaatttcgcccttgactctcggcaggtatgaccctgggtgcctgtgagctaggagaggaaattctgtatgcagggcaaacatgttacaaggggaggagatggcactgcacttcaggtctccaaatgcagtgtgctaggaatggcctcgctgacagttggaatcacggatacattaattacagcgaaggcaaaagtaagctacagtgacagggagctgggggcggagggagaaggcactttgccatgggagcacatctgttttataataagcaggtctataattctcttgtgaaagatcatgttctgctatcttctctgaggctggaaaatataaatactgtattttaccaagaggaggaggaaaggagatgatcaaatttgtttgcctgttgccaagtgtttgagattttccaccctttttcttttgtgtgcaacattctctttaactagagtgggggaaaagtcaacctgcttttctaagggtaaaaggcaccgtcaggcgtctcatgaatagggccctggccttttaacaagttttcaagccttggttgcggctactgtatagtcagaaaataaatgcatgtatggtgttgagctattaaggtgaaatgtgtggcctggggccaaaggaactggtgtgggttgagaggtaaaatgcttacatctaactgcacaaaagtcagtctgaaatgtcacatctctagatggatggaagtatcatgagttggggtcttggggaagcggcgtgtgggggaaaggagcaatggggttgaatgtaccaagtatgttgtgagccactgatcctaatagcagcaaaactactaaaccatgaagacatagaaggcatctgctcagcgcgaaagctacagaatcttctcataaagtctactgagaactgttccattataaacatatttttcttgctctagggagagttaaggggaaggaatgggagctgtcagggtcccagggctgtcctacctgccgttttggtcacagtgactgccacgtgctcttccaagggcactgcagctggagaacactacctgccaaatagcaaagcagatctctttcttactcctattatttattttagcactctttgttttacttcaaggtggcaattatatatgtgtgtgtatatatatatatttatttaaataatattagatctaattcattaattatacttgtaagtttgtattttcttaatagtccaaagttggtattttgaagttccacattactctgattttttaaacaaaaaaatgagaaagcaagaatggtcacattgacaaaggtcgaaatgaaagtgcaggaagaacaacgagaaataaagcacttaaaatgaataggtaggaactgcctccacaggattctgagaaaagaaactaaaacgaccctctttgggaatatacttactagatagccttatctaccagtctacacgacgatgtctttaacaaccaccccaggacatttcctccggccagcatcatgaaaaaaatcataaatatcaaccatgggcacccgttgaaaactgttaagaaagccatgtgtacagcctggaaaacacggtggagcgtcacatcattaggtgggtgatgggattagtaccgaaaaacagaccgacaacacgcagttattggtcgcagaggtttcttctcttctcaggaaaaaaacttctgagattaacttcaaaaccagaaccagccctcctcataaatgaggggtgtatgctttctgtcagagggggcttggctcctgtttccagccatcggctctgcttacgtgattccccgcctccacaggaggaactgaggcgggagcgccacggacaccaggtcctggaaggacccagcagtctcttgtgttttgaaggttttcttatgaaacagatgatgatgggtgcctgcctcagttacctcagcctctgtgaaggctaaaaataaataacacaaaaataacctaaagcactgttttgtgcaggaaatgcttccttttgtgtcttgggtaataaaatgtaccgagagacagagagaaaaaaaaagtctgaactataaagcattgtgtataccacgttttgtctgggagcaagcagctgaaattcttggctaagtgtaatccagctattggtagtttctcgagccacagaggttctgtggatcgtctggacaatgatgtacacagagcatacgtacaggacgtataggtatttgcgtatatataaataaatatatatatctatatctagttgaagaggatacatactcttcttccaaaggggtctaactggctagttaggaggccgctctggggctgatggattgttgattggtgaatccctggccttcgggtcggctggagtcaggtgttctggtaggacagctcgaacatggtgcaagcctcctctagactctcgtccatgttcagtctctgccagaaagacttctgcttcttctgcagctctcggcgaacacacctcgggcaggggacagacttttctttgcattcagaatggaaaacggctccacagctttcacacctgcttgttgaaatatcctcaaaagggtagaggatctctccattgttacagatttcacagatgaaccccttctggctacaaagactgcagctgtacacgtgtgaggtggcaaatttaatgaccttgcccaagaatggagccagctttccctctattacctgctgcaggtcggcaagtgaatacaggtggatctgttgaaggaggtattctctggggaaaattctgcggcggagatcctctgccaccgctgcccggcagctgaacaaataggctcggagcgacttcagccgctgccgcagccgcagcacggcggccagcggctctgcgtggtggtacagcatggcgttctcctgctggatgtcgatgagcggctcttcgtacacgtactccagaaactccttggcctgcttcgacaccttatactttgaagtatcccagttgtggactatgcgtgctggaatgagaaagctgtcatccacgtggcagctactgcagtaataccacccactgtagttgcacaccttggctttcccattggaaagacctatggatcgctggcagcctgcacatttgaaactctgagcagtgagtcctcgttccaaagacaaagtcgtcaaaatgctcaggaagctggtagtcacagattggcgtttgttcttcctgagttcatgcccacccatttgatccttgggtttgttcctcagtgtgacttgcaggttttgctctgaactcctcgccacattggcagctatcttcagagcctccatccattcctgagccctctgtcgggtctcagctcggaggcgaaggacatcctgggggaaaatgacttgaaagcaagagtcgcagccatccaggttgtccatctggacagccagacacacgtccacgttgtagctcaacagtggatcctcgtctagcttgccaggctgaaaagccataaggtaagccctgctcagcacaaatgtaaatgccttccagttgttttggacagtcagcctgtagagagtccctgatttgaggatgttttggtactgtttggagctgtccaggacaggggacggtggcagcagcccactggttttcttctggaaactatgattctgtgtatagtcatcatgatggccaagccctggtgagattgtcagctcattctgccgccccatgtaaccgggcacagcagcatgcactacttcccaaagcttctgtccccagtccaaagcctcccatggtgactctgcctttagctgtagctgagtgttgtcatacaaaacagtatccaccatcctggcctccaggttgcctaaaacagatatgctctggaagtgtgaaagctggtacgtggcataaaggttttgattcccactgctgtcgaggctgtagaagtataagttgtaaggtgaaagttctgcataacagctttgccagtaactgtcatggtcctttctaatctccaggtaacccttctttagaatgtttgggaatgtctgcttgtgttcagtatttccttgagcatcttctatcttatttggtgagggcaacagaaaagatggcctggtgacatgcgggccttgaagcaatggctgctgctgttgctgctgctgcaaaggcgtggttttgaggactaccctccagtccacttgggtaatatctgatcgtgatcgagcatgccctggcttgaaagttgaggtctcatccagtaagtcatttacagaacgaggccggtccctccgacgctgacagatattgaagaaattaaaggttgatgcttccttttgttccatccaggaaagattatctggggttgtccctctctggaccataaactgttctttggcagggaagacattttgagctttggtttctaagagcctgctcttacagtggtcccaaatcatgccccccttgcccagggaggtgacatttctcatagcaccattgtctgttatgttactgagtacctcatgccccaccagttcagggacttcctggatcccataaacctctgcctgctgcacagccttttctagattactatccaaagtactaaagaattcctccgtaacttctaaggctgggctgatatcatccacttccaaagcttccatgtcacaggctccaggaggccttagcctcctaagctggttccagaaatggcttcatgaacattcacccaaccaagaggggtgcttcagcaatagagctatggaaacaactggaagaaaccttcattgggctccctggagcaggccaaacccaaagtggttgatgttttcctggtaattaaaagcatttgctagtggctaatgggcattaacagatgtatagggagaccaaatgttcctttgagattattcttcagtgagacctctgtgaagacaacagcaagtacttgtcaaagcaatgccacgccaatccttgatttccttgtcagcaggaaggcaaattatgcatgtttttcaatgtctggtatgatcccacagtagccaatgaaacagagcaaacataatgcatggaatttattgctggtggtcatttttatcacgctctcactcagcactgagttctctgaattaattggcttgcatcagaaactccaagctaggatgtagttcagttccttatgaaccaaatgccaaatgtactctgggccccggctgctactctccattcacctgcggggccttcagtccgctcctggaggggcttgactcccgcagcctgccgcccgcctcacggtgacagcccgcccgggcgctgaccatcccggcccggctctgtttacaagcggcttctcgcggtcccactctgaaatgcttccgccggcggcccgggcagccagagccggacacacaaggttccaggccgcgaggacgagtctttcctgcccgagggacccggcagctaggcaaggcctgaccgcacccgccagg

SEQ ID NO: 14916 - RNA, 859 nt, Homo sapiens
  source 1..859: mol_type = other RNA
gctgggattacaggcatgagccactatgccatgtcagttaatccttccttttactccaaaactagtattaaggtaagaggtggaagctgggttgggagaagcacatggcacacctggcccccatgaatactgttatttattatgatactatgggtctcttccggtaccaggatagacggggataatctggcctccatgccggggacatgtcctgcagcgggtggtatagtggccctcactggaagtagaagagggtgttaaaacacaataatgtaaggaggaggcaactggcagtggtatacaccccacgtgtggggacaaagtcagggaaagactgagatccagtgaatataatgagtgttcacctgggaggtgggagactcgggctacggctggctgcatcacccactcactgtgtgaccttcaaccgttactgagtccttgtggcttaagtcgcccaagtgccaagtacacaggaacttaaggacatactatgctgccattaaaaagtgatatttactattcatttactatttaatgttaaatctaaaaccagtgcacaaaattgtatatacattacagttacagccatgtaaaaggctttcctctggtaggaaagaaatcctattggagaacataccaaaccgttaacaggaatcattgtgtttagatggtagaatcataggtaatttttttcccttctttccttttgtaagttttctaaagcttctcccatgcaagtactaactaggcctgaccgtgcttagcttctgagatcagatgagatcagacatattcaaggtagtatggctgtaggctaatttttcttttcttttctcttttcttttttttttttttt

SEQ ID NO: 14917 - RNA, 4496 nt, Homo sapiens
  source 1..4496: mol_type = other RNA
gctgggattacaggcatgagccactatgcccaacctgagcaggatgacttaaacctgatcaattctactccaaaacagcaactatcattaagtcaggggtgtcaaggaggactctgtgaaggcaaagactagactgggatgtgtgcgagagtgggataagaaggcccatccctagcagactgcaggagtgactctggcatagaattcatggccagccctaactagtgtgatgggtggcagggaggaggcatctgctcagtgttcaaacaaaatccttacaagttctggggctggacctctgtgtcactcctgaatcccaatgtatccgttacctttacaagaaactggtgtggttcttgtctgctaagggcaagacctgttttctgaatttactttctgataataaagtaacaccatggaaaagaagaacctcagaaaaatatggggtcaccacatgggctttcccagtgctagctgcctgttttggaaagctgcaatgtaggctacagagggcagtctgaaaagagtccttctgctttcgcttcctggagcttaagaagaaaagaggaattaccaaggttgtggtgggttatttactctggaaatatcttggtcacactgtccgtggcaaaagcggaaagcctagcttatgtggatagttgaaggtgactgtgtgggccatcattatctacaatagaaatgactcaagccctagcatgtaatctcttagggacttaacaagttaaaaagaaacaaaaaatcatattggaaatggcctcttggtttaatataaacttggttacaacattcaaatttatctttacggaaatttcacactgctcctaggagcccttatagcatctgattctaagttattctgaaggaaaaaaaaattattctgaaatataccttattaggatgatcactggaattctaccagatataagtaaaaggctaaatgggttttaaataaatacaagctaaattaccttcttctggggttaacaattagaatcccaaataccccaacatctcaactagaaaggccttcacagtaattctatgaaattgtaaatgatgccaaattttttttttttttttgagatggagtcttgcactgtcacccggggtggaatacaatggtgcaatctcggctcactgcaacctccactcccaggttcaagcgattctcctgcctgagcctctcaagtagctgggattacaggcgcccaccaccatgcccagctaattttttgtatttttagtagagacggggtttcactatgttggccaggctggtcttgaacccctgacctcgtgatccgcccgcctcggcctcccaaagtgctgggattacaggtgtgggtcaccgtgcctggccaatgccaatttttgaaaacagatttgatctttagggtaaatgcctgagtcagctgacaaactccatatacatgaatatgtccaagtgaaattacctaaagaataattttttttctttctttttttttttttaagagacagggtctcactgtgtcacccagactggagtgcagtggcatgatcacagctcactgttgccttgacctcctgggctcaagtgatccttccacctcagcctcctaagtatttgggactacatgcatgcatcaccacacctgacaaattaaaaaaaaattttttttttgccaggtgcagtggctcacatctgtaatcccagcactctgagaggctgaggtgggcggatcacctgaggttgggagtttgagaccagcctgaccaacacagagaaaccctgtctctattaaaaatacaaaattcgcccggcatggtggcgcatgcctgtaatcccagctactcaggaggttgaggcaggagaatcactttaatctgggaggcggaggttgcggtgagccaagaccgcaccattgcactccagcctgggcaacaagagcgaaactccgtctcaaaaagaaaacaaaaaaaaaatttttgtttttgtagagacaggatctcactctgttgcctaggctggtcttaagcgatcctcccagctcagcctcccaaagcactacaattataggcatgagccattgagcctggcctgagaattttctttaatttcaaaaaaatagctgctgcttctttaaagagtttaaaaattgatcggttcaatggcaaagctacacaacaactctggagtagaaggaaagaactctctttatagtacaacctctttccagcatactgccatcagctagtagaggcaactgcaaacaaatggtaggagttgcccaggaaggtatttgggctggacaaagtgatagcaaccctccagaccctggctccttataaatgtatagcaattcattcatacaaactgcacagaggttaaacaaaacctactaaaaaaattaaaaaatcccacaaaatccccaacccagaaaacgtttcctggctctctactaacagtaaaatgtgctgagcccaaattttctgctctaacatgggtcccacggacctatcagtctgctctggggtgctgacctgctgggtcctgagcagggtctttccctaagcatcactgtgggtttggagacagctgtaatgtgtgcagctgtcagcagaaagtacaatgccactgggctacatatgtccatatcatccaccaccatttcccactgtaaaaccaaaggctgcaactgtgaacaaatgtggacttcctcaaaggacaaatgaggagactgaaggctacatttcctcctttgagaaccattagagagtgtctacagttatacaacaggtttctgcagaccctgtggtaacttccaaaagcaagagtagcagcaagagaggaaaggagcatgtttatactttggactttgtatcaggcacttaaattgttggagagacatgccgttttgaaccaaagatataaaaactgggttggagtaatctttacaagtggtctaatgaatgggccttcagaagcaaagtggaggtgtgggttgaacctctgcccatcctttagtgctgactttcaagttttctaaatgcccataaccacagcaatggcagcagtggcggcaacggcaggaacagttctgtcatgtctgttttctgtatgtgttctgtggctgaccagaaggttttggtgtcacactaagaaggctctggggtgtggcacacctactgcccgaggttgcccagatccacgctggagccaaacatcttcaccagctgttcctcatagtgtgagatgttcctcttcatgatgtccatgcagggccccagaagcctctcgaatgcttgtacatccataacctgcttctaatcaagatgctcacttcgccagactctatgatgtaaaagctatcagccttttcaccctgagtgattatgcgttctccatccttatagatcttctctcctattacatccacaatcttcattcgttctgacacctctagtgatttaaggaggggcacagactcaataaatgattcaaacatcttcctcttctttgcattatttttcactatgattcttctaaaagtcacccggtccagtccccaaagggagccttctgaggtagcaacaatggtagcagctctcggggtgttgtacatcagagctagttctccaaaactgccacggttgtcatattgaccaacagagcgggtttgattatcttttgttactaaaatgtcataagttccccgttctatgacataaaagttgtctccatcatctccttggtcaatgacatgctcatcagctttgactatcctttcaaacatggcatcgagaacttgagaaagctgttcctgatcaagatttttgaaaaggagaatatctttgcaagcttcctgaagtctgcatctctgttcatcagttttaggatgaatcacccttggatctgtatcttcctcttcctcatcagggttataggtctcagcacagactgatactcgtctattaaatctgctaggaactggaacttccaagtcctcgtcctcctccgactcgctgtcccctttggcgtcggcgacacggtccgggccgggttctggcggggggtggcccaggctctggcgtggggtggcggcgggcaggactgaggctggggcgcgggcctcgcgcaggcgggtgaagtactccactgcgaattcgacgaggtcaggcggctgctgtcgcagcacctccaccgtgtagccctgcagcagctccgtgagccccggcgggatctggatgtggctcatgccggcggcggccgaagggatagacgggttgggccgccggcggccactgtctccgcgctcactcacgccggcctttcgctccgcgcccgcgaggtctcttcgcgcacggccccggctcacgtcgcgccgctctttggccggctctgcgtttccgggccgcgcaaccctacgctaccacggccgacctggcaccgccgccgctgtcactgggcagccgccgccgccgcggggaccgac

SEQ ID NO: 14918 - RNA, 4595 nt, Homo sapiens
  source 1..4595: mol_type = other RNA
gctgggattacaggcatgagccactatgcccaacctgagcaggatgacttaaacctgatcaattctactccaaaacagcaactatcattaagtcaggggtgtcaaggaggactctgtgaaggcaaagactagactgggatgtgtgcgagagtgggataagaaggcccatccctagcagactgcaggagtgactctggcatagaattcatggccagccctaactagtgtgatgggtggcagggaggaggcatctgctcagtgttcaaacaaaatccttacaagttctggggctggacctctgtgtcactcctgaatcccaatgtatccgttacctttacaagaaactggtgtggttcttgtctgctaagggcaagacctgttttctgaatttactttctgataataaagtaacaccatggaaaagaagaacctcagaaaaatatggggtcaccacatgggctttcccagtgctagctgcctgttttggaaagctgcaatgtaggctacagagggcagtctgaaaagagtccttctgctttcgcttcctggagcttaagaagaaaagaggaattaccaaggttgtggtgggttatttactctggaaatatcttggtcacactgtccgtggcaaaagcggaaagcctagcttatgtggatagttgaaggtgactgtgtgggccatcattatctacaatagaaatgactcaagccctagcatgtaatctcttagggacttaacaagttaaaaagaaacaaaaaatcatattggaaatggcctcttggtttaatataaacttggttacaacattcaaatttatctttacggaaatttcacactgctcctaggagcccttatagcatctgattctaagttattctgaaggaaaaaaaaattattctgaaatataccttattaggatgatcactggaattctaccagatataagtaaaaggctaaatgggttttaaataaatacaagctaaattaccttcttctggggttaacaattagaatcccaaataccccaacatctcaactagaaaggccttcacagtaattctatgaaattgtaaatgatgccaaattttttttttttttttgagatggagtcttgcactgtcacccggggtggaatacaatggtgcaatctcggctcactgcaacctccactcccaggttcaagcgattctcctgcctgagcctctcaagtagctgggattacaggcgcccaccaccatgcccagctaattttttgtatttttagtagagacggggtttcactatgttggccaggctggtcttgaacccctgacctcgtgatccgcccgcctcggcctcccaaagtgctgggattacaggtgtgggtcaccgtgcctggccaatgccaatttttgaaaacagatttgatctttagggtaaatgcctgagtcagctgacaaactccatatacatgaatatgtccaagtgaaattacctaaagaataattttttttctttctttttttttttttaagagacagggtctcactgtgtcacccagactggagtgcagtggcatgatcacagctcactgttgccttgacctcctgggctcaagtgatccttccacctcagcctcctaagtatttgggactacatgcatgcatcaccacacctgacaaattaaaaaaaaattttttttttgccaggtgcagtggctcacatctgtaatcccagcactctgagaggctgaggtgggcggatcacctgaggttgggagtttgagaccagcctgaccaacacagagaaaccctgtctctattaaaaatacaaaattcgcccggcatggtggcgcatgcctgtaatcccagctactcaggaggttgaggcaggagaatcactttaatctgggaggcggaggttgcggtgagccaagaccgcaccattgcactccagcctgggcaacaagagcgaaactccgtctcaaaaagaaaacaaaaaaaaaatttttgtttttgtagagacaggatctcactctgttgcctaggctggtcttaagcgatcctcccagctcagcctcccaaagcactacaattataggcatgagccattgagcctggcctgagaattttctttaatttcaaaaaaatagctgctgcttctttaaagagtttaaaaattgatcggttcaatggcaaagctacacaacaactctggagtagaaggaaagaactctctttatagtacaacctctttccagcatactgccatcagctagtagaggcaactgcaaacaaatggtaggagttgcccaggaaggtatttgggctggacaaagtgatagcaaccctccagaccctggctccttataaatgtatagcaattcattcatacaaactgcacagaggttaaacaaaacctactaaaaaaattaaaaaatcccacaaaatccccaacccagaaaacgtttcctggctctctactaacagtaaaatgtgctgagcccaaattttctgctctaacatgggtcccacggacctatcagtctgctctggggtgctgacctgctgggtcctgagcagggtctttccctaagcatcactgtgggtttggagacagctgtaatgtgtgcagctgtcagcagaaagtacaatgccactgggctacatatgtccatatcatccaccaccatttcccactgtaaaaccaaaggctgcaactgtgaacaaatgtggacttcctcaaaggacaaatgaggagactgaaggctacatttcctcctttgagaaccattagagagtgtctacagttatacaacaggtttctgcagaccctgtggtaacttccaaaagcaagagtagcagcaagagaggaaaggagcatgtttatactttggactttgtatcaggcacttaaattgttggagagacatgccgttttgaaccaaagatataaaaactgggttggagtaatctttacaagtggtctaatgaatgggccttcagaagcaaagtggaggtgtgggttgaacctctgcccatcctttagtgctgactttcaagttttctaaatgcccataaccacagcaatggcagcagtggcggcaacggcaggaacagttctgtcatgtctgttttctgtatgtgttctgtggctgaccagaaggttttggtgtcacactaagaaggctctggggtgtggcacacctactgcccgaggttgcccagatccacgctggagccaaacatcttcaccagctgttcctcatagtgtgagatgttcctcttcatgatgtccatgcagggccccagaagcctctcgaatgcttgtacatccataactaagcatttgacatctccaactgcataagctgaggcagctctgggtttgttggtgaccagggcaagctctccaaagtactgccccttatggcagcgggcaatctcgacctcctggttcccaccatccttgtttgatttagtcctgcttctaatcaagatgctcacttcgccagactctatgatgtaaaagctatcagccttttcaccctgagtgattatgcgttctccatccttatagatcttctctcctattacatccacaatcttcattcgttctgacacctctagtgatttaaggaggggcacagactcaataaatgattcaaacatcttcctcttctttgcattatttttcactatgattcttctaaaagtcacccggtccagtccccaaagggagccttctgaggtagcaacaatggtagcagctctcggggtgttgtacatcagagctagttctccaaaactgccacggttgtcatattgaccaacagagcgggtttgattatcttttgttactaaaatgtcataagttccccgttctatgacataaaagttgtctccatcatctccttggtcaatgacatgctcatcagctttgactatcctttcaaacatggcatcgagaacttgagaaagctgttcccttggatctgtatcttcctcttcctcatcagggttataggtctcagcacagactgatactcgtctattaaatctgctaggaactggaacttccaagtcctcgtcctcctccgactcgctgtcccctttggcgtcggcgacacggtccgggccgggttctggcggggggtggcccaggctctggcgtggggtggcggcgggcaggactgaggctggggcgcgggcctcgcgcaggcgggtgaagtactccactgcgaattcgacgaggtcaggcggctgctgtcgcagcacctccaccgtgtagccctgcagcagctccgtgagccccggcgggatctggatgtggctcatgccggcggcggccgaagggatagacgggttgggccgccggcggccactgtctccgcgctcactcacgccggcctttcgctccgcgcccgcgaggtctcttcgcgcacggccccggctcacgtcgcgccgctctttggccggctctgcgtttccgggccgcgcaaccctacgctaccacggccgacctggcaccgccgccgctgtcactgggcagccgccgccgccgcggggaccgacgggcaggcgagctggacgggcggggcaggcgtcctggttgt

SEQ ID NO: 14919 - RNA, 4679 nt, Homo sapiens
  source 1..4679: mol_type = other RNA
gctgggattacaggcatgagccactatgcccaacctgagcaggatgacttaaacctgatcaattctactccaaaacagcaactatcattaagtcaggggtgtcaaggaggactctgtgaaggcaaagactagactgggatgtgtgcgagagtgggataagaaggcccatccctagcagactgcaggagtgactctggcatagaattcatggccagccctaactagtgtgatgggtggcagggaggaggcatctgctcagtgttcaaacaaaatccttacaagttctggggctggacctctgtgtcactcctgaatcccaatgtatccgttacctttacaagaaactggtgtggttcttgtctgctaagggcaagacctgttttctgaatttactttctgataataaagtaacaccatggaaaagaagaacctcagaaaaatatggggtcaccacatgggctttcccagtgctagctgcctgttttggaaagctgcaatgtaggctacagagggcagtctgaaaagagtccttctgctttcgcttcctggagcttaagaagaaaagaggaattaccaaggttgtggtgggttatttactctggaaatatcttggtcacactgtccgtggcaaaagcggaaagcctagcttatgtggatagttgaaggtgactgtgtgggccatcattatctacaatagaaatgactcaagccctagcatgtaatctcttagggacttaacaagttaaaaagaaacaaaaaatcatattggaaatggcctcttggtttaatataaacttggttacaacattcaaatttatctttacggaaatttcacactgctcctaggagcccttatagcatctgattctaagttattctgaaggaaaaaaaaattattctgaaatataccttattaggatgatcactggaattctaccagatataagtaaaaggctaaatgggttttaaataaatacaagctaaattaccttcttctggggttaacaattagaatcccaaataccccaacatctcaactagaaaggccttcacagtaattctatgaaattgtaaatgatgccaaattttttttttttttttgagatggagtcttgcactgtcacccggggtggaatacaatggtgcaatctcggctcactgcaacctccactcccaggttcaagcgattctcctgcctgagcctctcaagtagctgggattacaggcgcccaccaccatgcccagctaattttttgtatttttagtagagacggggtttcactatgttggccaggctggtcttgaacccctgacctcgtgatccgcccgcctcggcctcccaaagtgctgggattacaggtgtgggtcaccgtgcctggccaatgccaatttttgaaaacagatttgatctttagggtaaatgcctgagtcagctgacaaactccatatacatgaatatgtccaagtgaaattacctaaagaataattttttttctttctttttttttttttaagagacagggtctcactgtgtcacccagactggagtgcagtggcatgatcacagctcactgttgccttgacctcctgggctcaagtgatccttccacctcagcctcctaagtatttgggactacatgcatgcatcaccacacctgacaaattaaaaaaaaattttttttttgccaggtgcagtggctcacatctgtaatcccagcactctgagaggctgaggtgggcggatcacctgaggttgggagtttgagaccagcctgaccaacacagagaaaccctgtctctattaaaaatacaaaattcgcccggcatggtggcgcatgcctgtaatcccagctactcaggaggttgaggcaggagaatcactttaatctgggaggcggaggttgcggtgagccaagaccgcaccattgcactccagcctgggcaacaagagcgaaactccgtctcaaaaagaaaacaaaaaaaaaatttttgtttttgtagagacaggatctcactctgttgcctaggctggtcttaagcgatcctcccagctcagcctcccaaagcactacaattataggcatgagccattgagcctggcctgagaattttctttaatttcaaaaaaatagctgctgcttctttaaagagtttaaaaattgatcggttcaatggcaaagctacacaacaactctggagtagaaggaaagaactctctttatagtacaacctctttccagcatactgccatcagctagtagaggcaactgcaaacaaatggtaggagttgcccaggaaggtatttgggctggacaaagtgatagcaaccctccagaccctggctccttataaatgtatagcaattcattcatacaaactgcacagaggttaaacaaaacctactaaaaaaattaaaaaatcccacaaaatccccaacccagaaaacgtttcctggctctctactaacagtaaaatgtgctgagcccaaattttctgctctaacatgggtcccacggacctatcagtctgctctggggtgctgacctgctgggtcctgagcagggtctttccctaagcatcactgtgggtttggagacagctgtaatgtgtgcagctgtcagcagaaagtacaatgccactgggctacatatgtccatatcatccaccaccatttcccactgtaaaaccaaaggctgcaactgtgaacaaatgtggacttcctcaaaggacaaatgaggagactgaaggctacatttcctcctttgagaaccattagagagtgtctacagttatacaacaggtttctgcagaccctgtggtaacttccaaaagcaagagtagcagcaagagaggaaaggagcatgtttatactttggactttgtatcaggcacttaaattgttggagagacatgccgttttgaaccaaagatataaaaactgggttggagtaatctttacaagtggtctaatgaatgggccttcagaagcaaagtggaggtgtgggttgaacctctgcccatcctttagtgctgactttcaagttttctaaatgcccataaccacagcaatggcagcagtggcggcaacggcaggaacagttctgtcatgtctgttttctgtatgtgttctgtggctgaccagaaggttttggtgtcacactaagaaggctctggggtgtggcacacctactgcccgaggttgcccagatccacgctggagccaaacatcttcaccagctgttcctcatagtgtgagatgttcctcttcatgatgtccatgcagggccccagaagcctctcgaatgcttgtacatccataactaagcatttgacatctccaactgcataagctgaggcagctctgggtttgttggtgaccagggcaagctctccaaagtactgccccttatggcagcgggcaatctcgacctcctggttcccaccatccttgtttgatttagtcctgcttctaatcaagatgctcacttcgccagactctatgatgtaaaagctatcagccttttcaccctgagtgattatgcgttctccatccttatagatcttctctcctattacatccacaatcttcattcgttctgacacctctagtgatttaaggaggggcacagactcaataaatgattcaaacatcttcctcttctttgcattatttttcactatgattcttctaaaagtcacccggtccagtccccaaagggagccttctgaggtagcaacaatggtagcagctctcggggtgttgtacatcagagctagttctccaaaactgccacggttgtcatattgaccaacagagcgggtttgattatcttttgttactaaaatgtcataagttccccgttctatgacataaaagttgtctccatcatctccttggtcaatgacatgctcatcagctttgactatcctttcaaacatggcatcgagaacttgagaaagctgttcctgatcaagatttttgaaaaggagaatatctttgcaagcttcctgaagtctgcatctctgttcatcagttttaggatgaatcacccttggatctgtatcttcctcttcctcatcagggttataggtctcagcacagactgatactcgtctattaaatctgctaggaactggaacttccaagtcctcgtcctcctccgactcgctgtcccctttggcgtcggcgacacggtccgggccgggttctggcggggggtggcccaggctctggcgtggggtggcggcgggcaggactgaggctggggcgcgggcctcgcgcaggcgggtgaagtactccactgcgaattcgacgaggtcaggcggctgctgtcgcagcacctccaccgtgtagccctgcagcagctccgtgagccccggcgggatctggatgtggctcatgccggcggcggccgaagggatagacgggttgggccgccggcggccactgtctccgcgctcactcacgccggcctttcgctccgcgcccgcgaggtctcttcgcgcacggccccggctcacgtcgcgccgctctttggccggctctgcgtttccgggccgcgcaaccctacgctaccacggccgacctggcaccgccgccgctgtcactgggcagccgccgccgccgcggggaccgacgggcaggcgagctggacgggcggggcaggcgtcctggttgt

SEQ ID NO: 14920 - RNA, 4613 nt, Homo sapiens
  source 1..4613: mol_type = other RNA
gctgggattacaggcatgagccactatgcccaacctgagcaggatgacttaaacctgatcaattctactccaaaacagcaactatcattaagtcaggggtgtcaaggaggactctgtgaaggcaaagactagactgggatgtgtgcgagagtgggataagaaggcccatccctagcagactgcaggagtgactctggcatagaattcatggccagccctaactagtgtgatgggtggcagggaggaggcatctgctcagtgttcaaacaaaatccttacaagttctggggctggacctctgtgtcactcctgaatcccaatgtatccgttacctttacaagaaactggtgtggttcttgtctgctaagggcaagacctgttttctgaatttactttctgataataaagtaacaccatggaaaagaagaacctcagaaaaatatggggtcaccacatgggctttcccagtgctagctgcctgttttggaaagctgcaatgtaggctacagagggcagtctgaaaagagtccttctgctttcgcttcctggagcttaagaagaaaagaggaattaccaaggttgtggtgggttatttactctggaaatatcttggtcacactgtccgtggcaaaagcggaaagcctagcttatgtggatagttgaaggtgactgtgtgggccatcattatctacaatagaaatgactcaagccctagcatgtaatctcttagggacttaacaagttaaaaagaaacaaaaaatcatattggaaatggcctcttggtttaatataaacttggttacaacattcaaatttatctttacggaaatttcacactgctcctaggagcccttatagcatctgattctaagttattctgaaggaaaaaaaaattattctgaaatataccttattaggatgatcactggaattctaccagatataagtaaaaggctaaatgggttttaaataaatacaagctaaattaccttcttctggggttaacaattagaatcccaaataccccaacatctcaactagaaaggccttcacagtaattctatgaaattgtaaatgatgccaaattttttttttttttttgagatggagtcttgcactgtcacccggggtggaatacaatggtgcaatctcggctcactgcaacctccactcccaggttcaagcgattctcctgcctgagcctctcaagtagctgggattacaggcgcccaccaccatgcccagctaattttttgtatttttagtagagacggggtttcactatgttggccaggctggtcttgaacccctgacctcgtgatccgcccgcctcggcctcccaaagtgctgggattacaggtgtgggtcaccgtgcctggccaatgccaatttttgaaaacagatttgatctttagggtaaatgcctgagtcagctgacaaactccatatacatgaatatgtccaagtgaaattacctaaagaataattttttttctttctttttttttttttaagagacagggtctcactgtgtcacccagactggagtgcagtggcatgatcacagctcactgttgccttgacctcctgggctcaagtgatccttccacctcagcctcctaagtatttgggactacatgcatgcatcaccacacctgacaaattaaaaaaaaattttttttttgccaggtgcagtggctcacatctgtaatcccagcactctgagaggctgaggtgggcggatcacctgaggttgggagtttgagaccagcctgaccaacacagagaaaccctgtctctattaaaaatacaaaattcgcccggcatggtggcgcatgcctgtaatcccagctactcaggaggttgaggcaggagaatcactttaatctgggaggcggaggttgcggtgagccaagaccgcaccattgcactccagcctgggcaacaagagcgaaactccgtctcaaaaagaaaacaaaaaaaaaatttttgtttttgtagagacaggatctcactctgttgcctaggctggtcttaagcgatcctcccagctcagcctcccaaagcactacaattataggcatgagccattgagcctggcctgagaattttctttaatttcaaaaaaatagctgctgcttctttaaagagtttaaaaattgatcggttcaatggcaaagctacacaacaactctggagtagaaggaaagaactctctttatagtacaacctctttccagcatactgccatcagctagtagaggcaactgcaaacaaatggtaggagttgcccaggaaggtatttgggctggacaaagtgatagcaaccctccagaccctggctccttataaatgtatagcaattcattcatacaaactgcacagaggttaaacaaaacctactaaaaaaattaaaaaatcccacaaaatccccaacccagaaaacgtttcctggctctctactaacagtaaaatgtgctgagcccaaattttctgctctaacatgggtcccacggacctatcagtctgctctggggtgctgacctgctgggtcctgagcagggtctttccctaagcatcactgtgggtttggagacagctgtaatgtgtgcagctgtcagcagaaagtacaatgccactgggctacatatgtccatatcatccaccaccatttcccactgtaaaaccaaaggctgcaactgtgaacaaatgtggacttcctcaaaggacaaatgaggagactgaaggctacatttcctcctttgagaaccattagagagtgtctacagttatacaacaggtttctgcagaccctgtggtaacttccaaaagcaagagtagcagcaagagaggaaaggagcatgtttatactttggactttgtatcaggcacttaaattgttggagagacatgccgttttgaaccaaagatataaaaactgggttggagtaatctttacaagtggtctaatgaatgggccttcagaagcaaagtggaggtgtgggttgaacctctgcccatcctttagtgctgactttcaagttttctaaatgcccataaccacagcaatggcagcagtggcggcaacggcaggaacagttctgtcatgtctgttttctgtatgtgttctgtggctgaccagaaggttttggtgtcacactaagaaggctctggggtgtggcacacctactgcccgaggttgcccagatccacgctggagccaaacatcttcaccagctgttcctcatagtgtgagatgttcctcttcatgatgtccatgcagggccccagaagcctctcgaatgcttgtacatccataactaagcatttgacatctccaactgcataagctgaggcagctctgggtttgttggtgaccagggcaagctctccaaagtactgccccttatggcagcgggcaatctcgacctcctggttcccaccatccttgtttgatttagtctgagtgattatgcgttctccatccttatagatcttctctcctattacatccacaatcttcattcgttctgacacctctagtgatttaaggaggggcacagactcaataaatgattcaaacatcttcctcttctttgcattatttttcactatgattcttctaaaagtcacccggtccagtccccaaagggagccttctgaggtagcaacaatggtagcagctctcggggtgttgtacatcagagctagttctccaaaactgccacggttgtcatattgaccaacagagcgggtttgattatcttttgttactaaaatgtcataagttccccgttctatgacataaaagttgtctccatcatctccttggtcaatgacatgctcatcagctttgactatcctttcaaacatggcatcgagaacttgagaaagctgttcctgatcaagatttttgaaaaggagaatatctttgcaagcttcctgaagtctgcatctctgttcatcagttttaggatgaatcacccttggatctgtatcttcctcttcctcatcagggttataggtctcagcacagactgatactcgtctattaaatctgctaggaactggaacttccaagtcctcgtcctcctccgactcgctgtcccctttggcgtcggcgacacggtccgggccgggttctggcggggggtggcccaggctctggcgtggggtggcggcgggcaggactgaggctggggcgcgggcctcgcgcaggcgggtgaagtactccactgcgaattcgacgaggtcaggcggctgctgtcgcagcacctccaccgtgtagccctgcagcagctccgtgagccccggcgggatctggatgtggctcatgccggcggcggccgaagggatagacgggttgggccgccggcggccactgtctccgcgctcactcacgccggcctttcgctccgcgcccgcgaggtctcttcgcgcacggccccggctcacgtcgcgccgctctttggccggctctgcgtttccgggccgcgcaaccctacgctaccacggccgacctggcaccgccgccgctgtcactgggcagccgccgccgccgcggggaccgacgggcaggcgagctggacgggcggggcaggcgtcctggttgt

SEQ ID NO: 14921 - RNA, 3289 nt, Homo sapiens
  source 1..3289: mol_type = other RNA
gctgggattacaggcatgagccactatgccccactttgcccggctaattttgtatttttagtagagatggggtttccccgtgttggtcagcctggtctcaaactcctgacctcaggtgatccacccgacttgacctgccaaagtgctgggattacaggcgtgagccactgcacccgccagccatgtcttttcatgtctccagctctggtgcggctgaagggtgtgggcaggtggacctcagccggcccatctgcccagcgaggatgtgaattcctgcctgagtgcctgtgagtaccccacgagaaggatgggctacctcttgggtgagacaggtggatgcatctataacccccgaggccggaaggtccccactcaaagcccagtgcctccccgtcccctgggcccacatcccagagtagacggccctgccagacagaggggtgagggccacagagatgagtgccggagtccaaatcggtgcaactttaccacgagtgagatctggttggccgatgccactgaatccgggttagaggacgaggaagaggaagacgaggaggaagaggagacggaatttccttccgagacccgctttctcttgcgcttgggaatgctgctgtctttggctggcaccttggcatcattgcagatttctgcaaagggttggagctggttaatgatgaccatgcggacatgctctcgggccttcaggatcttctccagccggtggatgtcgtacgtgttggggttccggaaggggatgtcatcaggcagacccgtgacctccacggcgtctgggctgtcccggattagtttataagggaccagcaccggccggttcaggcccagggcctcaccgtatttctcgttgaagagttccttcacctgctcccgcaggatcaccttctccccgagtctgttggcgtcatcttcatcaggctttgggatgagtccttggaaaggcctggtgactgtgaacttgatcttgtcagccacagcaagaatcctctccaggttctgggagccgaaggtacagggctttcggaacgggattcctgggggcagcccctcgatgatcacggagccggggttactcttgatccgcttgtaggggacctggaccgggtacttgatgcccaaggcttccccgtatttcttattgaaaaggtcctggacctgctcccttagtgtgttggcgatgtcgatccgtgagagcctcgcgtcataattttcttgaaagccctgtctcttcaggctctcgtccaccagagggtccccggaatccctctcttgactatccatgatgggctctttgactccctcagtgagcagctcgggcctcttgatgacaaactggatgctgttgctggcctccagaatcttccggagcttggcgatcccgaagcagttgggcctgcggagggagatgccttcaggcagtcccaccacaaacagctcctccgggtgcatcagaaacttggagtacggcaccttgacgggctccgagatgccaatggccttggcgtatcgtgtgttgaagagcagctccacctgcttccgcaggggccggatcacgtcaccgtggctgtcctccacgggcctctcctcgggccgcgcgtcctcactcagacctttgtctgtcagcatctccatcccataaccagaatcctccgatggcaggtgcccaggcatcgagtctgtcatttcctcagaggttggcgaggggtctgggacggtgacctgaatgatgtccagatcctctggctcaattttgatcggcctcagcccgcccagctccccggaggttcctggcccacagtcttcagacatgctgcccttgtctgaccgagcattcccagcaaggtcaaggacggtggccctagagacctctgcagaggtgtcctctggcgggctggctggctccagcttcgtggtgtctttggtaaacttgttccctgtgaaaattcgctcatcaaacatcctcttaatgatgaagtggatactatggcgctcctccaggatccgcttcagcttggggactccataagtgcaggggcgcttgaaggggatcttgtccgggatgcccacgatctccacagcctccgggtcacaggcaatcttccggtagggcacggggaccatgtggtccaggcccagggcttccgcatatctgctgttaaacaggatctgcacacactcccggagcgtgttgatgtcctcggtttcctttatgaaggcgtcccacttctctgacttgtcatggacgatggagaagagaatgcgcttggaggcatggacgttctggatgagaggcccaccaggcccagtgggcttctgtccacaacagtcggagaagtcttgggcaccggtggccttgggctctggcatgggccgactcaggcccaggtcgctgggggcaagggggcaggaaggtgcttcctgcttgagctctcggatggcgtggttggggagcgccgtgctgtacaggaagctggccatggaggaggaggtggcggttgggggcaggtcctggggtggcaccttgggggcctggccatgcaggccacagtcccgtgaccccttgggaatcagggagacaccgttcagctccaccagggccttcgagtcccgcccgccatcctcaagtggcctcttgagcttgaagcggatgcggtggctgtgttccaggatggccatgagggccttggggtcatactcggctggccttcggaaggccaggccttcgggcagcccctgcacggccagcagccctggctccctgagcagcctctcatagggcagtggcaccacactggcccttcccagggcctcgctataaagaacatcaaacacctcctctaccatcttccgcagaaggtacacatctgagccatgttccagggaggaccgagggaggctacggcctccaccctcgccccgctgcaccttcttggggtgctctgcctccggatccttccacgggggccctcggcagaacctgaggaagtctgactgtagctccttccgggcattcaggaacattctccccttctctgtgcccaccacaaaggcgctctcatcgtgcacggcgacacaggccacctcggcgttcagtttggacagcgctgagcacatggagtctaaggcagacacgaggctggtgatgatctcgtctttgcgggtgaacgcggagttccagcggtcgggtccgcagccgttggtggggacgtcacagcgcttacccagcaaggccatggtcgcctcattcgccaactgcagcagcctgcgg

SEQ ID NO: 14922 - RNA, 3444 nt, Homo sapiens
  source 1..3444: mol_type = other RNA
gctgggattacaggcatgagccactatgccccactttgcccggctaattttgtatttttagtagagatggggtttccccgtgttggtcagcctggtctcaaactcctgacctcaggtgatccacccgacttgacctgccaaagtgctgggattacaggcgtgagccactgcacccgccagccatgtcttttcatgtctccagctctggtgcggctgaagggtgtgggcaggtggacctcagccggcccatctgcccagcgaggatgtgaattcctgcctgagtgcctgtgagtaccccacgagaaggatgggctacctcttgggtgagacaggtggatgcatctataacccccgaggccggaaggtccccactcaaagcccagtgcctccccgtcccctgggcccacatcccagagtagacggccctgccagacagaggggtgagggccacagagatgagtgccggagtccaaatcggtgcaactttaccacgagtgagatctggttggccgatgccactgaatccgggttagaggacgaggaagaggaagacgaggaggaagaggagacggaatttccttccgagacccgctttctcttgcgcttgggaatgctgctgtctttggctggcaccttggcatcattgcagatttctgcaaagggttggagctggttaatgatgaccatgcggacatgctctcgggccttcaggatcttctccagccggtggatgtcgtacgtgttggggttccggaaggggatgtcatcaggcagacccgtgacctccacggcgtctgggctgtcccggattagtttataagggaccagcaccggccggttcaggcccagggcctcaccgtatttctcgttgaagagttccttcacctgctcccgcaggatcaccttctccccgagtctgttggcgtcatcttcatcaggctttgggatgagtccttggaaaggcctggtgactgtgaacttgatcttgtcagccacagcaagaatcctctccaggttctgggagccgaaggtacagggctttcggaacgggattcctgggggcagcccctcgatgatcacggagccggggttactcttgatccgcttgtaggggacctggaccgggtacttgatgcccaaggcttccccgtatttcttattgaaaaggtcctggacctgctcccttagtgtgttggcgatgtcgatccgtgagagcctcgcgtcataattttcttgaaagccctgtctcttcaggctctcgtccaccagagggtccccggaatccctctcttgactatccatgatgggctctttgactccctcagtgagcagctcgggcctcttgatgacaaactggatgctgttgctggcctccagaatcttccggagcttggcgatcccgaagcagttgggcctgcggagggagatgccttcaggcagtcccaccacaaacagctcctccgggtgcatcagaaacttggagtacggcaccttgacgggctccgagatgccaatggccttggcgtatcgtgtgttgaagagcagctccacctgcttccgcaggggccggatcacgtcaccgtggctgtcctccacgggcctctcctcgggccgcgcgtcctcactcagacctttgtctgtcagcatctccatcccataaccagaatcctccgatggcaggtgcccaggcatcgagtctgtcatttcctcagaggttggcgaggggtctgggacggtgacctgaatgatgtccagatcctctggctcaattttgatcggcctcagcccgcccagctccccggaggttcctggcccacagtcttcagacatgctgcccttgtctgaccgagcattcccagcaaggtcaaggacggtggccctagagacctctgcagaggtgtcctctggcgggctggctggctccagcttcgtggtgtctttggtaaacttgttccctgtgaaaattcgctcatcaaacatcctcttaatgatgaagtggatactatggcgctcctccaggatccgcttcagcttggggactccataagtgcaggggcgcttgaaggggatcttgtccgggatgcccacgatctccacagcctccgggtcacaggcaatcttccggtagggcacggggaccatgtggtccaggcccagggcttccgcatatctgctgttaaacaggatctgcacacactcccggagcgtgttgatgtcctcggtttcctttatgaaggcgtcccacttctctgacttgtcatggacgatggagaagagaatgcgcttggaggcatggacgttctggatgagaggcccaccaggcccagtgggcttctgtccacaacagtcggagaagtcttgggcaccggtggccttgggctctggcatgggccgactcaggcccaggtcgctgggggcaagggggcaggaaggtgcttcctgcttgagctctcggatggcgtggttggggagcgccgtgctgtacaggaagctggccatggaggaggaggtggcggttgggggcaggtcctggggtggcaccttgggggcctggccatgcaggccacagtcccgtgaccccttgggaatcagggagacaccgttcagctccaccagggccttcgagtcccgcccgccatcctcaagtggcctcttgagcttgaagcggatgcggtggctgtgttccaggatggccatgagggccttggggtcatactcggctggccttcggaaggccaggccttcgggcagcccctgcacggccagcagccctggctccctgagcagcctctcatagggcagtggcaccacactggcccttcccagggcctcgctataaagaacatcaaacacctcctctaccatcttccgcagaaggtacacatctgagccatgttccagggaggaccgagggaggctacggcctccaccctcgccccgctgcaccttcttggggtgctctgcctccggatccttccacgggggccctcggcagaacctgaggaagtctgactgtagctccttccgggcattcaggaacattctccccttctctgtgcccaccacaaaggcgctctcatcgtgcacggcgacacaggccacctcggcgttcagtttggacagcgctgagcacatggagtctaaggcagacacgaggctggtgatgatctcgtctttgcgggtgaacgcggagttccagcggtcgggtccgcagccgttggtggggacgtcacagcgcttacccagcaaggccatggtcgccttggaggatccccaagcgctcctgccagcggcgccccggccccggcccgcggccaggactcagcctcctgccgctgcctccttaattaatccgggagaatgggggaaggagaggcagagggaggcgaggacggcggcgcggcgagggcggggagggaggcgcggggagggggcgcggggggg

SEQ ID NO: 14923 - RNA, 7049 nt, Homo sapiens
  source 1..7049: mol_type = other RNA
gctgggattacaggcatgagccactatgcccggcccacatttttttaaaaagttaaaatgtaaaagcacttttaagagacaagttagacagaaggtggtggagtacattttctgctctcctagcttctgtgtcctttaaactcctgccctcaaccatcctcttatcgtccaccacctccattcccctaggattcccaggtccccttagcactcaggggctgtggtctcaccttcaaatgaaaaacaacaacttcaaaattttatttattgcacactgaggtgtcaagaatcctaagtacactaatactacattgtagacataaaccaggtagaataatgcttaacacaagaaaataaatacacttgaagtggaatttctggcattagtgactagctgatgttaaaaagctgaatttacccagaatccacagagataatgctgagcagttttttagaaagttggggaggcttatttctgttgtttcccttgggtgtttatttccctgtacctctctcagtcatcactatttccttgaacagggtccagaaacagactcatttctggcatgtaacacatgaatatataaaggcgtaccatatttattcttgtcaagtaccctgatttaccaatctgcaaactaagttttcagattgataaatgtgaaactggattcagttattaaactggatcaagtttcaatctgaaacttaataactgaatccaggaagtgtcagttaaatggtcttaattaaaatgatagttgttcagaatggcaaaatgaatcatactggaacaccaaaggtctgttttgcattcgctgaagaaaggttacttttagtaggataattctataaaatgtaacttgcatagaaaggctttattatgggttctgtctgtcacaaatagcatcaaatcaatcatctcagttctggaatatgagattcactacattaaattaatactttcattccaaaatagaaattcatattttaaaccactgaaattgatataaaccactgctttaatattgtaaacctaaatgtccaactataatgaccaacttatctaataatgaaaactgcagtagcagaactattaagcagatctttataattaacttatgaagactatttaacatagaaaaatatttatatgtaaaaaacacagacccaaattacatattctctataagtatatggttaaaaaacctgcaagaaaatatacctaaatgctaatgttcattgcattcagatgatagaattatggattttatccatagatttttcttctagattttatagtttttaaaaattatgatgccccttatatttatattgggaaatatacatttaaacaaactattatttggctaccatgctaatattcacaaccatgtggcactagcctaaaataaacttttcagaagaaactaaattattctatctaaatattctgggaaacgtttaagtgatattggaatctctatcaaaatttccacaccagagtgaagaaagacaaattagatgtgggatgaaagttgttctcactgataagtgagagctaaatgatgagaacacatggacacataaagggcaacaacacacactggggtctattggagggtggagggtaggaggagggagaggatcaggaaaaattactaatgggtactaggcttaacacctgggtgatgaaatcatctatacaacaaacccccatgacgtaagtttacctatgaaacaaactggcacatgtacccctgaacttaaaagttgttaaaaaaaaaatttttttaagagagatgaaagtgactcaagaagctgtgtcaccaaatctttgagagctatgtcaccaaatcaaaaaataacagaaaaccagacaagatcataagaaatcatttgcacaatcaagtggcatcattccaaaccactggaggagcaatgcccgctttctttttaaaattctcctgggaaaattactcctcagcctcctttataaatccttgaggaaatgtcaagttctttcacgacaagaaaaactctcagctgggcacagtggctcacacctgtaatcccagcactttgggaagctgaggtgggcagatgcttgagctcaggagtttaagaccagcctggacaacatggcaaaatgtagtctctacaaaaagatacaaaaattagctgggcatggtggtacatacctgtagtcccagctactcaggaggctgaggcagaaggatcccttgagcccaggaagtcaaggctgcagtgagccatatcatgccactgcactccagcctgggcaaaagagcaagaccctgtctcaaaaacaaataaataaatacaaacgcttctttacgaaagtctcacaagtttagctgaaaagagatatggactctcacataccttatttcagatctaaacatgagttcctcatctataaaatggagctaatatcaccaatactattggatcatgaacagaattaaaccagttattggtaaatcccccaaaataataaacaagccatgtttattccctcattctatcttacctcttctcttagtgtttctcacagtgtggaataccaccattgcatcagaatcactgagcactcgccacaaaggttggtttcataaatcccagaggcatcatggtccctcttttttttttttttttttttttagagacagggtcttgccctgttgcccagactggagtacagtggcacaatcaaggctcactgcaacctctgcaaccttctgcctcctgggctcaagcaatcctcccacctcagcctcctaagtagcggggactacaggtggtgccaccacacccagctagtttttgtatttttttgtagagatggggtttcaccatggcacccaggctggtcttgaccttccgggctcaagcaatccgcccacctcagcctcccgagactataatccctgctgggattacagatgtgagccaacatccctggccttaattcttttattatttaacaaaaattttttagagataagatctcttgtctgttgcccaagtgggagtgtagtggcgcaatcataactcactgcagcctcaaactactgggctcaatcaatcaccctgccttagcctccctagtagctgggactgtcggcccacacctggataattttttattttttgtagagatgaggtcttactatgttgcccaggctggtctcaaactcctggcctcaagcaatcctcctgcctggcctcccaaagtgctgggattacaggcttgagctaccacaccctgccatgactctttaattctgcatttttgtcagatactacaagtgatccttaggtactgtaaagcgtaaggaccattaaaattaaactattttaatatattttattacctcattaggctcagaaacaattaaaaatcttctttccccctaaaatactttaaaaacttgaaggtgttcctcaaggacaggaaagtaagatctggggccctcctattttaaattaaaaacccaaattatttgacccattcttctaagggtatatattgttcatacttcaagcatctgtcttcctctctaaagcctccctagtttcttcatctgtctacttaggagcaacttaaactagactataatctatcacagctcaaaaagaaaagagtacttactaaatgatcccaaattaaactcgtttaaaattaataagtcaaataaaattaataattccattcttcttagatagccagtaggaatagcagcttcttccaagcatgagagaatgggtgtgccttttatgcccaaatcaagaaataccaaaaaacaaacaaacaaacaaacaaaaaactgtcatgaattttagtatcttattaatttctaattagattttaacttctaattttggtaagtagttcaaaataacaacaacaacaacaaaaaaaaaaacacctgaaactagtggaaaaaacttccacagctttataatatcgtagcattctttacacaaaagtcaattcctaaaccctcaaatttcagaacataaaaataaatttccatttacagatttcccccttccagttccaaaagtagttattctagagtaagtattcaacacataaaatttagctgaatcaaataaaaaacaatcaccaaatgcaaatatcaattccaaagcacagattttatatatactgctttcatatttcccttttgcttcttttctagataaaagcaggaaattgtaaatattcactaaaaaactcgaaccaagcacattggccttttcaagtaattcagaaaaggtagatcatcaagagaaactcctgagacacagcagtcttcagtgcattcacaagagcctctgactataagctttctctagttaaccgccagaagatggattacttgtgctatgcatgcagatgcactcaatttcctttaccagataagctacaaacactctactaccaaccaaacttgtcccttccatcaaaacatttttcatactctttagcaaagtagtcacccctcctaggagaagctaattcaaatacactcattagcatctttggttacaagagcaatatagtgtgtagatgcagttaagagttctaccatggctaagtcaacattggataaaatcctataggtagatataaatgtaacctgcattttctaagctccttataagtcatcatattaagtccagatctttttgaaattttatacttattaagggcagtcatctctcactggggccactttctgtaactcaggtcaattgagaaggtcattgaatatgattcctccagtcccttccaagacaggctaggtttccaaggggcacacaaaggacaagaacatgtccagctggttcttcacaataacttcatctggatgcagcttgtgcggtagataatgggccagggtcatctcccaggcatcgacgagatatactccaacccctgagaacatcctccgaaggatggtgtccagctgaaagttgtaccagtcgctgttgaaaaggctcacctcaggtcccagctcttgggcgttggccgtccggatgaccaccacggtctttgggcttcgatcgaggagccgaaccactgctcgacggatgttcctgagccgccggatgtacacttccaaagggaaggtgctgaagtgagaccatacagctatggcaaccactgtgttcttccctcccacaatgccattcagctcattcgccacataatggagctcattgctaaagacagtcgtgaagcggatgggtggaccatggcagcggtatttgagcaggatgttgtgcttctggtccactgcaaggaagggacccacattcttgggactacccaagttaaactccactaaatctggaacaaatgtagtaaggtattcaaaccattgcctgattgttgagtcaccaaataaatgcaccacttttctttgtaagcactctgtaatgttgtcagggtcattaaactgacgcatcttaaactttctgggcctccactggtctttataataatacccagaaggaaaagttcctgagccttgagatagttctagactgttagtttctctggaagaaagcactctctgcagcggttaggagacctttcaggtatccacctttgaaatgggtaattctgctgctgcaagggagcttctttggtttgaagcagaaccagggctccccagtgtagaggtctgtaaagttacacaggggcagattcccaggaagacacacgttgcactcagtagtttcagaaattcttcctgaacggaagagactcttgaaatagaccctgtctggtttatcttcctgtaagcgctgaagaactctgatcccttcactggggtggaccagagatacggatactttaactttgcctggccatagcaaagtaaagaaaaccttgtaaaacccattctggtaatccaccaccctgcccacagccccagcctgcagcttgagggagtgaattctggcctgcaggtagtctccaccatacttcttgggctttctttgaaaatcctgcacatgaaccagcacctcaagctggcttcccaccttaaagaaggcagcagagttcaagatgacaaagtagctggaagaagggtcagtgctcttcacaaaggggactgggcccacatcaggaacctgccggtgcaaggcagccagcaaggagtcctcctccatgcgctcctggctggacagggtctgctgatcatagccacagtagggatttcggctaattcctgtcacctgggaggaaacaaactgtccactgctgtcgatgaaagtggctgaaacagtctcatggtccaagtactctacctgagtaacattgatgaccagcaccaccaccatcaacactgcaagcagacagcagaaaagccgtagtttgaagaaattggtccacattgtctggctgtgtcttgttcacccatggccgacaccatgctaccttcactctttaaaattccatgtctttgcttttctgagctgcagatgagctttcagtttcatttgcttctatcctgctagtacccttaagagctcttatgcagaggagagactgcagttgattcaagaagcacatttttcttcaaagaaatcctatagtcccagttactcaggaggctgaggtaggagaattgcttgagcctgggaggtcgaggctgcagtgaaccatgatcatcacaccaatgtactccagcctgggcaacagagcaggactcttttttggaaattttccaagaagagatgcttactggaactagaaattagaagttacgtctaactttccttccagcatgaaattctgaactcaggcaattttgaccagaggtcctcatttttttcatgccacatgtgaagcacacataaatgttttttacatttctatacaattcttcttgctccgggacccgcccgcccttcgctctccgggggccagggatcctgacgccccggtcggtcgccgcagcgccaggccgctagccccccgcttcctcacccggcgacgtctcctc

SEQ ID NO: 14924 - RNA, 7127 nt, Homo sapiens
  source 1..7127: mol_type = other RNA
gctgggattacaggcatgagccactatgcccggcccacatttttttaaaaagttaaaatgtaaaagcacttttaagagacaagttagacagaaggtggtggagtacattttctgctctcctagcttctgtgtcctttaaactcctgccctcaaccatcctcttatcgtccaccacctccattcccctaggattcccaggtccccttagcactcaggggctgtggtctcaccttcaaatgaaaaacaacaacttcaaaattttatttattgcacactgaggtgtcaagaatcctaagtacactaatactacattgtagacataaaccaggtagaataatgcttaacacaagaaaataaatacacttgaagtggaatttctggcattagtgactagctgatgttaaaaagctgaatttacccagaatccacagagataatgctgagcagttttttagaaagttggggaggcttatttctgttgtttcccttgggtgtttatttccctgtacctctctcagtcatcactatttccttgaacagggtccagaaacagactcatttctggcatgtaacacatgaatatataaaggcgtaccatatttattcttgtcaagtaccctgatttaccaatctgcaaactaagttttcagattgataaatgtgaaactggattcagttattaaactggatcaagtttcaatctgaaacttaataactgaatccaggaagtgtcagttaaatggtcttaattaaaatgatagttgttcagaatggcaaaatgaatcatactggaacaccaaaggtctgttttgcattcgctgaagaaaggttacttttagtaggataattctataaaatgtaacttgcatagaaaggctttattatgggttctgtctgtcacaaatagcatcaaatcaatcatctcagttctggaatatgagattcactacattaaattaatactttcattccaaaatagaaattcatattttaaaccactgaaattgatataaaccactgctttaatattgtaaacctaaatgtccaactataatgaccaacttatctaataatgaaaactgcagtagcagaactattaagcagatctttataattaacttatgaagactatttaacatagaaaaatatttatatgtaaaaaacacagacccaaattacatattctctataagtatatggttaaaaaacctgcaagaaaatatacctaaatgctaatgttcattgcattcagatgatagaattatggattttatccatagatttttcttctagattttatagtttttaaaaattatgatgccccttatatttatattgggaaatatacatttaaacaaactattatttggctaccatgctaatattcacaaccatgtggcactagcctaaaataaacttttcagaagaaactaaattattctatctaaatattctgggaaacgtttaagtgatattggaatctctatcaaaatttccacaccagagtgaagaaagacaaattagatgtgggatgaaagttgttctcactgataagtgagagctaaatgatgagaacacatggacacataaagggcaacaacacacactggggtctattggagggtggagggtaggaggagggagaggatcaggaaaaattactaatgggtactaggcttaacacctgggtgatgaaatcatctatacaacaaacccccatgacgtaagtttacctatgaaacaaactggcacatgtacccctgaacttaaaagttgttaaaaaaaaaatttttttaagagagatgaaagtgactcaagaagctgtgtcaccaaatctttgagagctatgtcaccaaatcaaaaaataacagaaaaccagacaagatcataagaaatcatttgcacaatcaagtggcatcattccaaaccactggaggagcaatgcccgctttctttttaaaattctcctgggaaaattactcctcagcctcctttataaatccttgaggaaatgtcaagttctttcacgacaagaaaaactctcagctgggcacagtggctcacacctgtaatcccagcactttgggaagctgaggtgggcagatgcttgagctcaggagtttaagaccagcctggacaacatggcaaaatgtagtctctacaaaaagatacaaaaattagctgggcatggtggtacatacctgtagtcccagctactcaggaggctgaggcagaaggatcccttgagcccaggaagtcaaggctgcagtgagccatatcatgccactgcactccagcctgggcaaaagagcaagaccctgtctcaaaaacaaataaataaatacaaacgcttctttacgaaagtctcacaagtttagctgaaaagagatatggactctcacataccttatttcagatctaaacatgagttcctcatctataaaatggagctaatatcaccaatactattggatcatgaacagaattaaaccagttattggtaaatcccccaaaataataaacaagccatgtttattccctcattctatcttacctcttctcttagtgtttctcacagtgtggaataccaccattgcatcagaatcactgagcactcgccacaaaggttggtttcataaatcccagaggcatcatggtccctcttttttttttttttttttttttagagacagggtcttgccctgttgcccagactggagtacagtggcacaatcaaggctcactgcaacctctgcaaccttctgcctcctgggctcaagcaatcctcccacctcagcctcctaagtagcggggactacaggtggtgccaccacacccagctagtttttgtatttttttgtagagatggggtttcaccatggcacccaggctggtcttgaccttccgggctcaagcaatccgcccacctcagcctcccgagactataatccctgctgggattacagatgtgagccaacatccctggccttaattcttttattatttaacaaaaattttttagagataagatctcttgtctgttgcccaagtgggagtgtagtggcgcaatcataactcactgcagcctcaaactactgggctcaatcaatcaccctgccttagcctccctagtagctgggactgtcggcccacacctggataattttttattttttgtagagatgaggtcttactatgttgcccaggctggtctcaaactcctggcctcaagcaatcctcctgcctggcctcccaaagtgctgggattacaggcttgagctaccacaccctgccatgactctttaattctgcatttttgtcagatactacaagtgatccttaggtactgtaaagcgtaaggaccattaaaattaaactattttaatatattttattacctcattaggctcagaaacaattaaaaatcttctttccccctaaaatactttaaaaacttgaaggtgttcctcaaggacaggaaagtaagatctggggccctcctattttaaattaaaaacccaaattatttgacccattcttctaagggtatatattgttcatacttcaagcatctgtcttcctctctaaagcctccctagtttcttcatctgtctacttaggagcaacttaaactagactataatctatcacagctcaaaaagaaaagagtacttactaaatgatcccaaattaaactcgtttaaaattaataagtcaaataaaattaataattccattcttcttagatagccagtaggaatagcagcttcttccaagcatgagagaatgggtgtgccttttatgcccaaatcaagaaataccaaaaaacaaacaaacaaacaaacaaaaaactgtcatgaattttagtatcttattaatttctaattagattttaacttctaattttggtaagtagttcaaaataacaacaacaacaacaaaaaaaaaaacacctgaaactagtggaaaaaacttccacagctttataatatcgtagcattctttacacaaaagtcaattcctaaaccctcaaatttcagaacataaaaataaatttccatttacagatttcccccttccagttccaaaagtagttattctagagtaagtattcaacacataaaatttagctgaatcaaataaaaaacaatcaccaaatgcaaatatcaattccaaagcacagattttatatatactgctttcatatttcccttttgcttcttttctagataaaagcaggaaattgtaaatattcactaaaaaactcgaaccaagcacattggccttttcaagtaattcagaaaaggtagatcatcaagagaaactcctgagacacagcagtcttcagtgcattcacaagagcctctgactataagctttctctagttaaccgccagaagatggattacttgtgctatgcatgcagatgcactcaatttcctttaccagataagctacaaacactctactaccaaccaaacttgtcccttccatcaaaacatttttcatactctttagcaaagtagtcacccctcctaggagaagctaattcaaatacactcattagcatctttggttacaagagcaatatagtgtgtagatgcagttaagagttctaccatggctaagtcaacattggataaaatcctataggtagatataaatgtaacctgcattttctaagctccttataagtcatcatattaagtccagatctttttgaaattttatacttattaagggcagtcatctctcactggggccactttctgtaactcaggtcaattgagaaggtcattgaatatgattcctccagtcccttccaagacaggctaggtttccaaggggcacacaaaggacaagaacatgtccagctggttcttcacaataacttcatctggatgcagcttgtgcggtagataatgggccagggtcatctcccaggcatcgacgagatatactccaacccctgagaacatcctccgaaggatggtgtccagctgaaagttgtaccagtcgctgttgaaaaggctcacctcaggtcccagctcttgggcgttggccgtccggatgaccaccacggtctttgggcttcgatcgaggagccgaaccactgctcgacggatgttcctgagccgccggatgtacacttccaaagggaaggtgctgaagtgagaccatacagctatggcaaccactgtgttcttccctcccacaatgccattcagctcattcgccacataatggagctcattgctaaagacagtcgtgaagcggatgggtggaccatggcagcggtatttgagcaggatgttgtgcttctggtccactgcaaggaagggacccacattcttgggactacccaagttaaactccactaaatctggaacaaatgtagtaaggtattcaaaccattgcctgattgttgagtcaccaaataaatgcaccacttttctttgtaagcactctgtaatgttgtcagggtcattaaactgacgcatcttaaactttctgggcctccactggtctttataataatacccagaaggaaaagttcctgagccttgagatagttctagactgttagtttcttttattctcctgggaatcacagttacccaatcaggtccactggagttgactggcattttgatattgacaccactctggaagaaagcactctctgcagcggttaggagacctttcaggtatccacctttgaaatgggtaattctgctgctgcaagggagcttctttggtttgaagcagaaccagggctccccagtgtagaggtctgtaaagttacacaggggcagattcccaggaagacacacgttgcactcagtagtttcagaaattcttcctgaacggaagagactcttgaaatagaccctgtctggtttatcttcctgtaagcgctgaagaactctgatcccttcactggggtggaccagagatacggatactttaactttgcctggccatagcaaagtaaagaaaaccttgtaaaacccattctggtaatccaccaccctgcccacagccccagcctgcagcttgagggagtgaattctggcctgcaggtagtctccaccatacttcttgggctttctttgaaaatcctgcacatgaaccagcacctcaagctggcttcccaccttaaagaaggcagcagagttcaagatgacaaagtagctggaagaagggtcagtgctcttcacaaaggggactgggcccacatcaggaacctgccggtgcaaggcagccagcaaggagtcctcctccatgcgctcctggctggacagggtctgctgatcatagccacagtagggatttcggctaattcctgtcacctgggaggaaacaaactgtccactgctgtcgatgaaagtggctgaaacagtctcatggtccaagtactctacctgagtaacattgatgaccagcaccaccaccatcaacactgcaagcagacagcagaaaagccgtagtttgaagaaattggtccacattgtctggctgtgtcttgttcacccatggccgacaccatgctaccttcactctttaaaattccatgtctttgcttttctgagctgcagatgagctttcagtttcatttgcttctatcctgctagtacccttaagagctcttatgcagaggagagactgcagttgattcaagaagcacatttttcttcaaagaaatcctatagtcccagttactcaggaggctgaggtaggagaattgcttgagcctgggaggtcgaggctgcagtgaaccatgatcatcacaccaatgtactccagcctgggcaacagagcaggactctgtcttttttggaaattttccaagaagagatgcttactggaactagaaattagaagttacgtctaactttccttccagcatgaaattctgaactcaggcaattttgaccagaggtcctcatttttttcatgccacatgtgaagcacacataaatgttttttacatttctatacaattcttcttgctccgggacccgcccgcccttcgctctccgggggccagggatcctgacgccccggtcggtcgccgcagcgccaggccgctagccccccgcttcctcacccggcgacgtctcctc

SEQ ID NO: 14925 - RNA, 7284 nt, Homo sapiens
  source 1..7284: mol_type = other RNA
gctgggattacaggcatgagccactatgcccggcccacatttttttaaaaagttaaaatgtaaaagcacttttaagagacaagttagacagaaggtggtggagtacattttctgctctcctagcttctgtgtcctttaaactcctgccctcaaccatcctcttatcgtccaccacctccattcccctaggattcccaggtccccttagcactcaggggctgtggtctcaccttcaaatgaaaaacaacaacttcaaaattttatttattgcacactgaggtgtcaagaatcctaagtacactaatactacattgtagacataaaccaggtagaataatgcttaacacaagaaaataaatacacttgaagtggaatttctggcattagtgactagctgatgttaaaaagctgaatttacccagaatccacagagataatgctgagcagttttttagaaagttggggaggcttatttctgttgtttcccttgggtgtttatttccctgtacctctctcagtcatcactatttccttgaacagggtccagaaacagactcatttctggcatgtaacacatgaatatataaaggcgtaccatatttattcttgtcaagtaccctgatttaccaatctgcaaactaagttttcagattgataaatgtgaaactggattcagttattaaactggatcaagtttcaatctgaaacttaataactgaatccaggaagtgtcagttaaatggtcttaattaaaatgatagttgttcagaatggcaaaatgaatcatactggaacaccaaaggtctgttttgcattcgctgaagaaaggttacttttagtaggataattctataaaatgtaacttgcatagaaaggctttattatgggttctgtctgtcacaaatagcatcaaatcaatcatctcagttctggaatatgagattcactacattaaattaatactttcattccaaaatagaaattcatattttaaaccactgaaattgatataaaccactgctttaatattgtaaacctaaatgtccaactataatgaccaacttatctaataatgaaaactgcagtagcagaactattaagcagatctttataattaacttatgaagactatttaacatagaaaaatatttatatgtaaaaaacacagacccaaattacatattctctataagtatatggttaaaaaacctgcaagaaaatatacctaaatgctaatgttcattgcattcagatgatagaattatggattttatccatagatttttcttctagattttatagtttttaaaaattatgatgccccttatatttatattgggaaatatacatttaaacaaactattatttggctaccatgctaatattcacaaccatgtggcactagcctaaaataaacttttcagaagaaactaaattattctatctaaatattctgggaaacgtttaagtgatattggaatctctatcaaaatttccacaccagagtgaagaaagacaaattagatgtgggatgaaagttgttctcactgataagtgagagctaaatgatgagaacacatggacacataaagggcaacaacacacactggggtctattggagggtggagggtaggaggagggagaggatcaggaaaaattactaatgggtactaggcttaacacctgggtgatgaaatcatctatacaacaaacccccatgacgtaagtttacctatgaaacaaactggcacatgtacccctgaacttaaaagttgttaaaaaaaaaatttttttaagagagatgaaagtgactcaagaagctgtgtcaccaaatctttgagagctatgtcaccaaatcaaaaaataacagaaaaccagacaagatcataagaaatcatttgcacaatcaagtggcatcattccaaaccactggaggagcaatgcccgctttctttttaaaattctcctgggaaaattactcctcagcctcctttataaatccttgaggaaatgtcaagttctttcacgacaagaaaaactctcagctgggcacagtggctcacacctgtaatcccagcactttgggaagctgaggtgggcagatgcttgagctcaggagtttaagaccagcctggacaacatggcaaaatgtagtctctacaaaaagatacaaaaattagctgggcatggtggtacatacctgtagtcccagctactcaggaggctgaggcagaaggatcccttgagcccaggaagtcaaggctgcagtgagccatatcatgccactgcactccagcctgggcaaaagagcaagaccctgtctcaaaaacaaataaataaatacaaacgcttctttacgaaagtctcacaagtttagctgaaaagagatatggactctcacataccttatttcagatctaaacatgagttcctcatctataaaatggagctaatatcaccaatactattggatcatgaacagaattaaaccagttattggtaaatcccccaaaataataaacaagccatgtttattccctcattctatcttacctcttctcttagtgtttctcacagtgtggaataccaccattgcatcagaatcactgagcactcgccacaaaggttggtttcataaatcccagaggcatcatggtccctcttttttttttttttttttttttagagacagggtcttgccctgttgcccagactggagtacagtggcacaatcaaggctcactgcaacctctgcaaccttctgcctcctgggctcaagcaatcctcccacctcagcctcctaagtagcggggactacaggtggtgccaccacacccagctagtttttgtatttttttgtagagatggggtttcaccatggcacccaggctggtcttgaccttccgggctcaagcaatccgcccacctcagcctcccgagactataatccctgctgggattacagatgtgagccaacatccctggccttaattcttttattatttaacaaaaattttttagagataagatctcttgtctgttgcccaagtgggagtgtagtggcgcaatcataactcactgcagcctcaaactactgggctcaatcaatcaccctgccttagcctccctagtagctgggactgtcggcccacacctggataattttttattttttgtagagatgaggtcttactatgttgcccaggctggtctcaaactcctggcctcaagcaatcctcctgcctggcctcccaaagtgctgggattacaggcttgagctaccacaccctgccatgactctttaattctgcatttttgtcagatactacaagtgatccttaggtactgtaaagcgtaaggaccattaaaattaaactattttaatatattttattacctcattaggctcagaaacaattaaaaatcttctttccccctaaaatactttaaaaacttgaaggtgttcctcaaggacaggaaagtaagatctggggccctcctattttaaattaaaaacccaaattatttgacccattcttctaagggtatatattgttcatacttcaagcatctgtcttcctctctaaagcctccctagtttcttcatctgtctacttaggagcaacttaaactagactataatctatcacagctcaaaaagaaaagagtacttactaaatgatcccaaattaaactcgtttaaaattaataagtcaaataaaattaataattccattcttcttagatagccagtaggaatagcagcttcttccaagcatgagagaatgggtgtgccttttatgcccaaatcaagaaataccaaaaaacaaacaaacaaacaaacaaaaaactgtcatgaattttagtatcttattaatttctaattagattttaacttctaattttggtaagtagttcaaaataacaacaacaacaacaaaaaaaaaaacacctgaaactagtggaaaaaacttccacagctttataatatcgtagcattctttacacaaaagtcaattcctaaaccctcaaatttcagaacataaaaataaatttccatttacagatttcccccttccagttccaaaagtagttattctagagtaagtattcaacacataaaatttagctgaatcaaataaaaaacaatcaccaaatgcaaatatcaattccaaagcacagattttatatatactgctttcatatttcccttttgcttcttttctagataaaagcaggaaattgtaaatattcactaaaaaactcgaaccaagcacattggccttttcaagtaattcagaaaaggtagatcatcaagagaaactcctgagacacagcagtcttcagtgcattcacaagagcctctgactataagctttctctagttaaccgccagaagatggattacttgtgctatgcatgcagatgcactcaatttcctttaccagataagctacaaacactctactaccaaccaaacttgtcccttccatcaaaacatttttcatactctttagcaaagtagtcacccctcctaggagaagctaattcaaatacactcattagcatctttggttacaagagcaatatagtgtgtagatgcagttaagagttctaccatggctaagtcaacattggataaaatcctataggtagatataaatgtaacctgcattttctaagctccttataagtcatcatattaagtccagatctttttgaaattttatacttattaagggcagtcatctctcactggggccactttctgtaactcaggtcaattgagaaggtcattgaatatgattcctccagtcccttccaagacaggctaggtttccaaggggcacacaaaggacaagaacatgtccagctggttcttcacaataacttcatctggatgcagcttgtgcggtagataatgggccagggtcatctcccaggcatcgacgagatatactccaacccctgagaacatcctccgaaggatggtgtccagctgaaagttgtaccagtcgctgttgaaaaggctcacctcaggtcccagctcttgggcgttggccgtccggatgaccaccacggtctttgggcttcgatcgaggagccgaaccactgctcgacggatgttcctgagccgccggatgtacacttccaaagggaaggtgctgaagtgagaccatacagctatggcaaccactgtgttcttccctcccacaatgccattcagctcattcgccacataatggagctcattgctaaagacagtcgtgaagcggatgggtggaccatggcagcggtatttgagcaggatgttgtgcttctggtccactgcaaggaagggacccacattcttgggactacccaagttaaactccactaaatctggaacaaatgtagtaaggtattcaaaccattgcctgattgttgagtcaccaaataaatgcaccacttttctttgtaagcactctgtaatgttgtcagggtcattaaactgacgcatcttaaactttctgggcctccactggtctttataataatacccagaaggaaaagttcctgagccttgagatagttctagactgttagtttcttttattctcctgggaatcacagttacccaatcaggtccactggagttgactggcattttgatattgacaccactctggaagaaagcactctctgcagcggttaggagacctttcaggtatccacctttgaaatgggtaattctgctgctgcaagggagcttctttggtttgaagcagaaccagggctccccagtgtagaggtctgtaaagttacacaggggcagattcccaggaagacacacgttgcactcagtagtttcagaaattcttcctgaacggaagagactcttgaaatagaccctgtctggtttatcttcctgtaagcgctgaagaactctgatcccttcactggggtggaccagagatacggatactttaactttgcctggccatagcaaagtaaagaaaaccttgtaaaacccattctggtaatccaccaccctgcccacagccccagcctgcagcttgagggagtgaattctggcctgcaggtagtctccaccatacttcttgggctttctttgaaaatcctgcacatgaaccagcacctcaagctggcttcccaccttaaagaaggcagcagagttcaagatgacaaagtagctggaagaagggtcagtgctcttcacaaaggggactgggcccacatcaggaacctgccggtgcaaggcagccagcaaggagtcctcctccatgcgctcctggctggacagggtctgctgatcatagccacagtagggatttcggctaattcctgtcacctgggaggaaacaaactgtccactgctgtcgatgaaagtggctgaaacagtctcatggtccaagtactctacctgagtaacattgatgaccagcaccaccaccatcaacactgcaagcagacagcagaaaagccgtagtttgaagaaattggtccacattgtctggctgtgtcttgttcacccatggccgacaccatgctaccttcactctttaaaattccatgtctttgcttttctgagctgcagatgagctttcagtttcatttgcttctatcctgctagtacccttaagagctcttatgcagaggagagactgcagttgattcaagaagcacatttttcttcaaagaaatcctatagtcccagttactcaggaggctgaggtaggagaattgcttgagcctgggaggtcgaggctgcagtgaaccatgatcatcacaccaatgtactccagcctgggcaacagagcaggactctgtcttttttggaaattttccaagaagagatgcttactggaactagaaattagaagttacgtctaactttccttccagcatgaaattctgaactcaggcaattttgaccagaggtcctcatttttttcatgccacatgtgaagcacacataaatgttttttacatttctatacaattcttcttgcttgtaaagttacactcgtttctccccatacgacctgaatctgatgtccccaaacggcagctcagtaaggccagaacagtccaccgtgtgacagcagcgccagccaagaggcagctggtgcccagagcagcgatgagccgagagatatgagatgggcagggaggcgtcgccaagtgctccgcaccgggttagtgaaggtgcctggaggacagaagtctttcgctgcggcgtggaggtccgaactgtaccgagctgtggcgttgccgcaagt

SEQ ID NO: 14926 - RNA, 7123 nt, Homo sapiens
  source 1..7123: mol_type = other RNA
gctgggattacaggcatgagccactatgcccggcccacatttttttaaaaagttaaaatgtaaaagcacttttaagagacaagttagacagaaggtggtggagtacattttctgctctcctagcttctgtgtcctttaaactcctgccctcaaccatcctcttatcgtccaccacctccattcccctaggattcccaggtccccttagcactcaggggctgtggtctcaccttcaaatgaaaaacaacaacttcaaaattttatttattgcacactgaggtgtcaagaatcctaagtacactaatactacattgtagacataaaccaggtagaataatgcttaacacaagaaaataaatacacttgaagtggaatttctggcattagtgactagctgatgttaaaaagctgaatttacccagaatccacagagataatgctgagcagttttttagaaagttggggaggcttatttctgttgtttcccttgggtgtttatttccctgtacctctctcagtcatcactatttccttgaacagggtccagaaacagactcatttctggcatgtaacacatgaatatataaaggcgtaccatatttattcttgtcaagtaccctgatttaccaatctgcaaactaagttttcagattgataaatgtgaaactggattcagttattaaactggatcaagtttcaatctgaaacttaataactgaatccaggaagtgtcagttaaatggtcttaattaaaatgatagttgttcagaatggcaaaatgaatcatactggaacaccaaaggtctgttttgcattcgctgaagaaaggttacttttagtaggataattctataaaatgtaacttgcatagaaaggctttattatgggttctgtctgtcacaaatagcatcaaatcaatcatctcagttctggaatatgagattcactacattaaattaatactttcattccaaaatagaaattcatattttaaaccactgaaattgatataaaccactgctttaatattgtaaacctaaatgtccaactataatgaccaacttatctaataatgaaaactgcagtagcagaactattaagcagatctttataattaacttatgaagactatttaacatagaaaaatatttatatgtaaaaaacacagacccaaattacatattctctataagtatatggttaaaaaacctgcaagaaaatatacctaaatgctaatgttcattgcattcagatgatagaattatggattttatccatagatttttcttctagattttatagtttttaaaaattatgatgccccttatatttatattgggaaatatacatttaaacaaactattatttggctaccatgctaatattcacaaccatgtggcactagcctaaaataaacttttcagaagaaactaaattattctatctaaatattctgggaaacgtttaagtgatattggaatctctatcaaaatttccacaccagagtgaagaaagacaaattagatgtgggatgaaagttgttctcactgataagtgagagctaaatgatgagaacacatggacacataaagggcaacaacacacactggggtctattggagggtggagggtaggaggagggagaggatcaggaaaaattactaatgggtactaggcttaacacctgggtgatgaaatcatctatacaacaaacccccatgacgtaagtttacctatgaaacaaactggcacatgtacccctgaacttaaaagttgttaaaaaaaaaatttttttaagagagatgaaagtgactcaagaagctgtgtcaccaaatctttgagagctatgtcaccaaatcaaaaaataacagaaaaccagacaagatcataagaaatcatttgcacaatcaagtggcatcattccaaaccactggaggagcaatgcccgctttctttttaaaattctcctgggaaaattactcctcagcctcctttataaatccttgaggaaatgtcaagttctttcacgacaagaaaaactctcagctgggcacagtggctcacacctgtaatcccagcactttgggaagctgaggtgggcagatgcttgagctcaggagtttaagaccagcctggacaacatggcaaaatgtagtctctacaaaaagatacaaaaattagctgggcatggtggtacatacctgtagtcccagctactcaggaggctgaggcagaaggatcccttgagcccaggaagtcaaggctgcagtgagccatatcatgccactgcactccagcctgggcaaaagagcaagaccctgtctcaaaaacaaataaataaatacaaacgcttctttacgaaagtctcacaagtttagctgaaaagagatatggactctcacataccttatttcagatctaaacatgagttcctcatctataaaatggagctaatatcaccaatactattggatcatgaacagaattaaaccagttattggtaaatcccccaaaataataaacaagccatgtttattccctcattctatcttacctcttctcttagtgtttctcacagtgtggaataccaccattgcatcagaatcactgagcactcgccacaaaggttggtttcataaatcccagaggcatcatggtccctcttttttttttttttttttttttagagacagggtcttgccctgttgcccagactggagtacagtggcacaatcaaggctcactgcaacctctgcaaccttctgcctcctgggctcaagcaatcctcccacctcagcctcctaagtagcggggactacaggtggtgccaccacacccagctagtttttgtatttttttgtagagatggggtttcaccatggcacccaggctggtcttgaccttccgggctcaagcaatccgcccacctcagcctcccgagactataatccctgctgggattacagatgtgagccaacatccctggccttaattcttttattatttaacaaaaattttttagagataagatctcttgtctgttgcccaagtgggagtgtagtggcgcaatcataactcactgcagcctcaaactactgggctcaatcaatcaccctgccttagcctccctagtagctgggactgtcggcccacacctggataattttttattttttgtagagatgaggtcttactatgttgcccaggctggtctcaaactcctggcctcaagcaatcctcctgcctggcctcccaaagtgctgggattacaggcttgagctaccacaccctgccatgactctttaattctgcatttttgtcagatactacaagtgatccttaggtactgtaaagcgtaaggaccattaaaattaaactattttaatatattttattacctcattaggctcagaaacaattaaaaatcttctttccccctaaaatactttaaaaacttgaaggtgttcctcaaggacaggaaagtaagatctggggccctcctattttaaattaaaaacccaaattatttgacccattcttctaagggtatatattgttcatacttcaagcatctgtcttcctctctaaagcctccctagtttcttcatctgtctacttaggagcaacttaaactagactataatctatcacagctcaaaaagaaaagagtacttactaaatgatcccaaattaaactcgtttaaaattaataagtcaaataaaattaataattccattcttcttagatagccagtaggaatagcagcttcttccaagcatgagagaatgggtgtgccttttatgcccaaatcaagaaataccaaaaaacaaacaaacaaacaaacaaaaaactgtcatgaattttagtatcttattaatttctaattagattttaacttctaattttggtaagtagttcaaaataacaacaacaacaacaaaaaaaaaaacacctgaaactagtggaaaaaacttccacagctttataatatcgtagcattctttacacaaaagtcaattcctaaaccctcaaatttcagaacataaaaataaatttccatttacagatttcccccttccagttccaaaagtagttattctagagtaagtattcaacacataaaatttagctgaatcaaataaaaaacaatcaccaaatgcaaatatcaattccaaagcacagattttatatatactgctttcatatttcccttttgcttcttttctagataaaagcaggaaattgtaaatattcactaaaaaactcgaaccaagcacattggccttttcaagtaattcagaaaaggtagatcatcaagagaaactcctgagacacagcagtcttcagtgcattcacaagagcctctgactataagctttctctagttaaccgccagaagatggattacttgtgctatgcatgcagatgcactcaatttcctttaccagataagctacaaacactctactaccaaccaaacttgtcccttccatcaaaacatttttcatactctttagcaaagtagtcacccctcctaggagaagctaattcaaatacactcattagcatctttggttacaagagcaatatagtgtgtagatgcagttaagagttctaccatggctaagtcaacattggataaaatcctataggtagatataaatgtaacctgcattttctaagctccttataagtcatcatattaagtccagatctttttgaaattttatacttattaagggcagtcatctctcactggggccactttctgtaactcaggtcaattgagaaggtcattgaatatgattcctccagtcccttccaagacaggctaggtttccaaggggcacacaaaggacaagaacatgtccagctggttcttcacaataacttcatctggatgcagcttgtgcggtagataatgggccagggtcatctcccaggcatcgacgagatatactccaacccctgagaacatcctccgaaggatggtgtccagctgaaagttgtaccagtcgctgttgaaaaggctcacctcaggtcccagctcttgggcgttggccgtccggatgaccaccacggtctttgggcttcgatcgaggagccgaaccactgctcgacggatgttcctgagccgccggatgtacacttccaaagggaaggtgctgaagtgagaccatacagctatggcaaccactgtgttcttccctcccacaatgccattcagctcattcgccacataatggagctcattgctaaagacagtcgtgaagcggatgggtggaccatggcagcggtatttgagcaggatgttgtgcttctggtccactgcaaggaagggacccacattcttgggactacccaagttaaactccactaaatctggaacaaatgtagtaaggtattcaaaccattgcctgattgttgagtcaccaaataaatgcaccacttttctttgtaagcactctgtaatgttgtcagggtcattaaactgacgcatcttaaactttctgggcctccactggtctttataataatacccagaaggaaaagttcctgagccttgagatagttctagactgttagtttcttttattctcctgggaatcacagttacccaatcaggtccactggagttgactggcattttgatattgacaccactctggaagaaagcactctctgcagcggttaggagacctttcaggtatccacctttgaaatgggtaattctgctgctgcaagggagcttctttggtttgaagcagaaccagggctccccagtgtagaggtctgtaaagttacacaggggcagattcccaggaagacacacgttgcactcagtagtttcagaaattcttcctgaacggaagagactcttgaaatagaccctgtctggtttatcttcctgtaagcgctgaagaactctgatcccttcactggggtggaccagagatacggatactttaactttgcctggccatagcaaagtaaagaaaaccttgtaaaacccattctggtaatccaccaccctgcccacagccccagcctgcagcttgagggagtgaattctggcctgcaggtagtctccaccatacttcttgggctttctttgaaaatcctgcacatgaaccagcacctcaagctggcttcccaccttaaagaaggcagcagagttcaagatgacaaagtagctggaagaagggtcagtgctcttcacaaaggggactgggcccacatcaggaacctgccggtgcaaggcagccagcaaggagtcctcctccatgcgctcctggctggacagggtctgctgatcatagccacagtagggatttcggctaattcctgtcacctgggaggaaacaaactgtccactgctgtcgatgaaagtggctgaaacagtctcatggtccaagtactctacctgagtaacattgatgaccagcaccaccaccatcaacactgcaagcagacagcagaaaagccgtagtttgaagaaattggtccacattgtctggctgtgtcttgttcacccatggccgacaccatgctaccttcactctttaaaattccatgtctttgcttttctgagctgcagatgagctttcagtttcatttgcttctatcctgctagtacccttaagagctcttatgcagaggagagactgcagttgattcaagaagcacatttttcttcaaagaaatcctatagtcccagttactcaggaggctgaggtaggagaattgcttgagcctgggaggtcgaggctgcagtgaaccatgatcatcacaccaatgtactccagcctgggcaacagagcaggactcttttttggaaattttccaagaagagatgcttactggaactagaaattagaagttacgtctaactttccttccagcatgaaattctgaactcaggcaattttgaccagaggtcctcatttttttcatgccacatgtgaagcacacataaatgttttttacatttctatacaattcttcttgctccgggacccgcccgcccttcgctctccgggggccagggatcctgacgccccggtcggtcgccgcagcgccaggccgctagccccccgcttcctcacccggcgacgtctcctc

SEQ ID NO: 14927 - RNA, 7290 nt, Homo sapiens
  source 1..7290: mol_type = other RNA
gctgggattacaggcatgagccactatgcccggcccacatttttttaaaaagttaaaatgtaaaagcacttttaagagacaagttagacagaaggtggtggagtacattttctgctctcctagcttctgtgtcctttaaactcctgccctcaaccatcctcttatcgtccaccacctccattcccctaggattcccaggtccccttagcactcaggggctgtggtctcaccttcaaatgaaaaacaacaacttcaaaattttatttattgcacactgaggtgtcaagaatcctaagtacactaatactacattgtagacataaaccaggtagaataatgcttaacacaagaaaataaatacacttgaagtggaatttctggcattagtgactagctgatgttaaaaagctgaatttacccagaatccacagagataatgctgagcagttttttagaaagttggggaggcttatttctgttgtttcccttgggtgtttatttccctgtacctctctcagtcatcactatttccttgaacagggtccagaaacagactcatttctggcatgtaacacatgaatatataaaggcgtaccatatttattcttgtcaagtaccctgatttaccaatctgcaaactaagttttcagattgataaatgtgaaactggattcagttattaaactggatcaagtttcaatctgaaacttaataactgaatccaggaagtgtcagttaaatggtcttaattaaaatgatagttgttcagaatggcaaaatgaatcatactggaacaccaaaggtctgttttgcattcgctgaagaaaggttacttttagtaggataattctataaaatgtaacttgcatagaaaggctttattatgggttctgtctgtcacaaatagcatcaaatcaatcatctcagttctggaatatgagattcactacattaaattaatactttcattccaaaatagaaattcatattttaaaccactgaaattgatataaaccactgctttaatattgtaaacctaaatgtccaactataatgaccaacttatctaataatgaaaactgcagtagcagaactattaagcagatctttataattaacttatgaagactatttaacatagaaaaatatttatatgtaaaaaacacagacccaaattacatattctctataagtatatggttaaaaaacctgcaagaaaatatacctaaatgctaatgttcattgcattcagatgatagaattatggattttatccatagatttttcttctagattttatagtttttaaaaattatgatgccccttatatttatattgggaaatatacatttaaacaaactattatttggctaccatgctaatattcacaaccatgtggcactagcctaaaataaacttttcagaagaaactaaattattctatctaaatattctgggaaacgtttaagtgatattggaatctctatcaaaatttccacaccagagtgaagaaagacaaattagatgtgggatgaaagttgttctcactgataagtgagagctaaatgatgagaacacatggacacataaagggcaacaacacacactggggtctattggagggtggagggtaggaggagggagaggatcaggaaaaattactaatgggtactaggcttaacacctgggtgatgaaatcatctatacaacaaacccccatgacgtaagtttacctatgaaacaaactggcacatgtacccctgaacttaaaagttgttaaaaaaaaaatttttttaagagagatgaaagtgactcaagaagctgtgtcaccaaatctttgagagctatgtcaccaaatcaaaaaataacagaaaaccagacaagatcataagaaatcatttgcacaatcaagtggcatcattccaaaccactggaggagcaatgcccgctttctttttaaaattctcctgggaaaattactcctcagcctcctttataaatccttgaggaaatgtcaagttctttcacgacaagaaaaactctcagctgggcacagtggctcacacctgtaatcccagcactttgggaagctgaggtgggcagatgcttgagctcaggagtttaagaccagcctggacaacatggcaaaatgtagtctctacaaaaagatacaaaaattagctgggcatggtggtacatacctgtagtcccagctactcaggaggctgaggcagaaggatcccttgagcccaggaagtcaaggctgcagtgagccatatcatgccactgcactccagcctgggcaaaagagcaagaccctgtctcaaaaacaaataaataaatacaaacgcttctttacgaaagtctcacaagtttagctgaaaagagatatggactctcacataccttatttcagatctaaacatgagttcctcatctataaaatggagctaatatcaccaatactattggatcatgaacagaattaaaccagttattggtaaatcccccaaaataataaacaagccatgtttattccctcattctatcttacctcttctcttagtgtttctcacagtgtggaataccaccattgcatcagaatcactgagcactcgccacaaaggttggtttcataaatcccagaggcatcatggtccctcttttttttttttttttttttttagagacagggtcttgccctgttgcccagactggagtacagtggcacaatcaaggctcactgcaacctctgcaaccttctgcctcctgggctcaagcaatcctcccacctcagcctcctaagtagcggggactacaggtggtgccaccacacccagctagtttttgtatttttttgtagagatggggtttcaccatggcacccaggctggtcttgaccttccgggctcaagcaatccgcccacctcagcctcccgagactataatccctgctgggattacagatgtgagccaacatccctggccttaattcttttattatttaacaaaaattttttagagataagatctcttgtctgttgcccaagtgggagtgtagtggcgcaatcataactcactgcagcctcaaactactgggctcaatcaatcaccctgccttagcctccctagtagctgggactgtcggcccacacctggataattttttattttttgtagagatgaggtcttactatgttgcccaggctggtctcaaactcctggcctcaagcaatcctcctgcctggcctcccaaagtgctgggattacaggcttgagctaccacaccctgccatgactctttaattctgcatttttgtcagatactacaagtgatccttaggtactgtaaagcgtaaggaccattaaaattaaactattttaatatattttattacctcattaggctcagaaacaattaaaaatcttctttccccctaaaatactttaaaaacttgaaggtgttcctcaaggacaggaaagtaagatctggggccctcctattttaaattaaaaacccaaattatttgacccattcttctaagggtatatattgttcatacttcaagcatctgtcttcctctctaaagcctccctagtttcttcatctgtctacttaggagcaacttaaactagactataatctatcacagctcaaaaagaaaagagtacttactaaatgatcccaaattaaactcgtttaaaattaataagtcaaataaaattaataattccattcttcttagatagccagtaggaatagcagcttcttccaagcatgagagaatgggtgtgccttttatgcccaaatcaagaaataccaaaaaacaaacaaacaaacaaacaaaaaactgtcatgaattttagtatcttattaatttctaattagattttaacttctaattttggtaagtagttcaaaataacaacaacaacaacaaaaaaaaaaacacctgaaactagtggaaaaaacttccacagctttataatatcgtagcattctttacacaaaagtcaattcctaaaccctcaaatttcagaacataaaaataaatttccatttacagatttcccccttccagttccaaaagtagttattctagagtaagtattcaacacataaaatttagctgaatcaaataaaaaacaatcaccaaatgcaaatatcaattccaaagcacagattttatatatactgctttcatatttcccttttgcttcttttctagataaaagcaggaaattgtaaatattcactaaaaaactcgaaccaagcacattggccttttcaagtaattcagaaaaggtagatcatcaagagaaactcctgagacacagcagtcttcagtgcattcacaagagcctctgactataagctttctctagttaaccgccagaagatggattacttgtgctatgcatgcagatgcactcaatttcctttaccagataagctacaaacactctactaccaaccaaacttgtcccttccatcaaaacatttttcatactctttagcaaagtagtcacccctcctaggagaagctaattcaaatacactcattagcatctttggttacaagagcaatatagtgtgtagatgcagttaagagttctaccatggctaagtcaacattggataaaatcctataggtagatataaatgtaacctgcattttctaagctccttataagtcatcatattaagtccagatctttttgaaattttatacttattaagggcagtcatctctcactggggccactttctgtaactcaggtcaattgagaaggtcattgaatatgattcctccagtcccttccaagacaggctaggtttccaaggggcacacaaaggacaagaacatgtccagctggttcttcacaataacttcatctggatgcagcttgtgcggtagataatgggccagggtcatctcccaggcatcgacgagatatactccaacccctgagaacatcctccgaaggatggtgtccagctgaaagttgtaccagtcgctgttgaaaaggctcacctcaggtcccagctcttgggcgttggccgtccggatgaccaccacggtctttgggcttcgatcgaggagccgaaccactgctcgacggatgttcctgagccgccggatgtacacttccaaagggaaggtgctgaagtgagaccatacagctatggcaaccactgtgttcttccctcccacaatgccattcagctcattcgccacataatggagctcattgctaaagacagtcgtgaagcggatgggtggaccatggcagcggtatttgagcaggatgttgtgcttctggtccactgcaaggaagggacccacattcttgggactacccaagttaaactccactaaatctggaacaaatgtagtaaggtattcaaaccattgcctgattgttgagtcaccaaataaatgcaccacttttctttgtaagcactctgtaatgttgtcagggtcattaaactgacgcatcttaaactttctgggcctccactggtctttataataatacccagaaggaaaagttcctgagccttgagatagttctagactgttagtttcttttattctcctgggaatcacagttacccaatcaggtccactggagttgactggcattttgatattgacaccactctggaagaaagcactctctgcagcggttaggagacctttcaggtatccacctttgaaatgggtaattctgctgctgcaagggagcttctttggtttgaagcagaaccagggctccccagtgtagaggtctgtaaagttacacaggggcagattcccaggaagacacacgttgcactcagtagtttcagaaattcttcctgaacggaagagactcttgaaatagaccctgtctggtttatcttcctgtaagcgctgaagaactctgatcccttcactggggtggaccagagatacggatactttaactttgcctggccatagcaaagtaaagaaaaccttgtaaaacccattctggtaatccaccaccctgcccacagccccagcctgcagcttgagggagtgaattctggcctgcaggtagtctccaccatacttcttgggctttctttgaaaatcctgcacatgaaccagcacctcaagctggcttcccaccttaaagaaggcagcagagttcaagatgacaaagtagctggaagaagggtcagtgctcttcacaaaggggactgggcccacatcaggaacctgccggtgcaaggcagccagcaaggagtcctcctccatgcgctcctggctggacagggtctgctgatcatagccacagtagggatttcggctaattcctgtcacctgggaggaaacaaactgtccactgctgtcgatgaaagtggctgaaacagtctcatggtccaagtactctacctgagtaacattgatgaccagcaccaccaccatcaacactgcaagcagacagcagaaaagccgtagtttgaagaaattggtccacattgtctggctgtgtcttgttcacccatggccgacaccatgctaccttcactctttaaaattccatgtctttgcttttctgagctgcagatgagctttcagtttcatttgcttctatcctgctagtacccttaagagctcttatgcagaggagagactgcagttgattcaagaagcacatttttcttcaaagaaatcctatagtcccagttactcaggaggctgaggtaggagaattgcttgagcctgggaggtcgaggctgcagtgaaccatgatcatcacaccaatgtactccagcctgggcaacagagcaggactcttttttggaaattttccaagaagagatgcttactggaactagaaattagaagttacgtctaactttccttccagcatgaaattctgaactcaggcaattttgaccagaggtcctcatttttttcatgccacatgtgaagcacacataaatgttttttacatttctatacaattcttcttgctgaatctgatgtccccaaacggcagctcagtaaggccagaacagtccaccgtgtgacagcagcgccagccaagaggcagctggtgcccagagcagcgatgagccgagagatatgagatgggcagggaggcgtcgccaagtgctccgcaccgggttagtgaaggtgcctccgggacccgcccgcccttcgctctccgggggccagggatcctgacgccccggtcggtcgccgcagcgccaggccgctagccccccgcttcctcacccggcgacgtctcctc

SEQ ID NO: 14928 - RNA, 7341 nt, Homo sapiens
  source 1..7341: mol_type = other RNA
gctgggattacaggcatgagccactatgcccggcccacatttttttaaaaagttaaaatgtaaaagcacttttaagagacaagttagacagaaggtggtggagtacattttctgctctcctagcttctgtgtcctttaaactcctgccctcaaccatcctcttatcgtccaccacctccattcccctaggattcccaggtccccttagcactcaggggctgtggtctcaccttcaaatgaaaaacaacaacttcaaaattttatttattgcacactgaggtgtcaagaatcctaagtacactaatactacattgtagacataaaccaggtagaataatgcttaacacaagaaaataaatacacttgaagtggaatttctggcattagtgactagctgatgttaaaaagctgaatttacccagaatccacagagataatgctgagcagttttttagaaagttggggaggcttatttctgttgtttcccttgggtgtttatttccctgtacctctctcagtcatcactatttccttgaacagggtccagaaacagactcatttctggcatgtaacacatgaatatataaaggcgtaccatatttattcttgtcaagtaccctgatttaccaatctgcaaactaagttttcagattgataaatgtgaaactggattcagttattaaactggatcaagtttcaatctgaaacttaataactgaatccaggaagtgtcagttaaatggtcttaattaaaatgatagttgttcagaatggcaaaatgaatcatactggaacaccaaaggtctgttttgcattcgctgaagaaaggttacttttagtaggataattctataaaatgtaacttgcatagaaaggctttattatgggttctgtctgtcacaaatagcatcaaatcaatcatctcagttctggaatatgagattcactacattaaattaatactttcattccaaaatagaaattcatattttaaaccactgaaattgatataaaccactgctttaatattgtaaacctaaatgtccaactataatgaccaacttatctaataatgaaaactgcagtagcagaactattaagcagatctttataattaacttatgaagactatttaacatagaaaaatatttatatgtaaaaaacacagacccaaattacatattctctataagtatatggttaaaaaacctgcaagaaaatatacctaaatgctaatgttcattgcattcagatgatagaattatggattttatccatagatttttcttctagattttatagtttttaaaaattatgatgccccttatatttatattgggaaatatacatttaaacaaactattatttggctaccatgctaatattcacaaccatgtggcactagcctaaaataaacttttcagaagaaactaaattattctatctaaatattctgggaaacgtttaagtgatattggaatctctatcaaaatttccacaccagagtgaagaaagacaaattagatgtgggatgaaagttgttctcactgataagtgagagctaaatgatgagaacacatggacacataaagggcaacaacacacactggggtctattggagggtggagggtaggaggagggagaggatcaggaaaaattactaatgggtactaggcttaacacctgggtgatgaaatcatctatacaacaaacccccatgacgtaagtttacctatgaaacaaactggcacatgtacccctgaacttaaaagttgttaaaaaaaaaatttttttaagagagatgaaagtgactcaagaagctgtgtcaccaaatctttgagagctatgtcaccaaatcaaaaaataacagaaaaccagacaagatcataagaaatcatttgcacaatcaagtggcatcattccaaaccactggaggagcaatgcccgctttctttttaaaattctcctgggaaaattactcctcagcctcctttataaatccttgaggaaatgtcaagttctttcacgacaagaaaaactctcagctgggcacagtggctcacacctgtaatcccagcactttgggaagctgaggtgggcagatgcttgagctcaggagtttaagaccagcctggacaacatggcaaaatgtagtctctacaaaaagatacaaaaattagctgggcatggtggtacatacctgtagtcccagctactcaggaggctgaggcagaaggatcccttgagcccaggaagtcaaggctgcagtgagccatatcatgccactgcactccagcctgggcaaaagagcaagaccctgtctcaaaaacaaataaataaatacaaacgcttctttacgaaagtctcacaagtttagctgaaaagagatatggactctcacataccttatttcagatctaaacatgagttcctcatctataaaatggagctaatatcaccaatactattggatcatgaacagaattaaaccagttattggtaaatcccccaaaataataaacaagccatgtttattccctcattctatcttacctcttctcttagtgtttctcacagtgtggaataccaccattgcatcagaatcactgagcactcgccacaaaggttggtttcataaatcccagaggcatcatggtccctcttttttttttttttttttttttagagacagggtcttgccctgttgcccagactggagtacagtggcacaatcaaggctcactgcaacctctgcaaccttctgcctcctgggctcaagcaatcctcccacctcagcctcctaagtagcggggactacaggtggtgccaccacacccagctagtttttgtatttttttgtagagatggggtttcaccatggcacccaggctggtcttgaccttccgggctcaagcaatccgcccacctcagcctcccgagactataatccctgctgggattacagatgtgagccaacatccctggccttaattcttttattatttaacaaaaattttttagagataagatctcttgtctgttgcccaagtgggagtgtagtggcgcaatcataactcactgcagcctcaaactactgggctcaatcaatcaccctgccttagcctccctagtagctgggactgtcggcccacacctggataattttttattttttgtagagatgaggtcttactatgttgcccaggctggtctcaaactcctggcctcaagcaatcctcctgcctggcctcccaaagtgctgggattacaggcttgagctaccacaccctgccatgactctttaattctgcatttttgtcagatactacaagtgatccttaggtactgtaaagcgtaaggaccattaaaattaaactattttaatatattttattacctcattaggctcagaaacaattaaaaatcttctttccccctaaaatactttaaaaacttgaaggtgttcctcaaggacaggaaagtaagatctggggccctcctattttaaattaaaaacccaaattatttgacccattcttctaagggtatatattgttcatacttcaagcatctgtcttcctctctaaagcctccctagtttcttcatctgtctacttaggagcaacttaaactagactataatctatcacagctcaaaaagaaaagagtacttactaaatgatcccaaattaaactcgtttaaaattaataagtcaaataaaattaataattccattcttcttagatagccagtaggaatagcagcttcttccaagcatgagagaatgggtgtgccttttatgcccaaatcaagaaataccaaaaaacaaacaaacaaacaaacaaaaaactgtcatgaattttagtatcttattaatttctaattagattttaacttctaattttggtaagtagttcaaaataacaacaacaacaacaaaaaaaaaaacacctgaaactagtggaaaaaacttccacagctttataatatcgtagcattctttacacaaaagtcaattcctaaaccctcaaatttcagaacataaaaataaatttccatttacagatttcccccttccagttccaaaagtagttattctagagtaagtattcaacacataaaatttagctgaatcaaataaaaaacaatcaccaaatgcaaatatcaattccaaagcacagattttatatatactgctttcatatttcccttttgcttcttttctagataaaagcaggaaattgtaaatattcactaaaaaactcgaaccaagcacattggccttttcaagtaattcagaaaaggtagatcatcaagagaaactcctgagacacagcagtcttcagtgcattcacaagagcctctgactataagctttctctagttaaccgccagaagatggattacttgtgctatgcatgcagatgcactcaatttcctttaccagataagctacaaacactctactaccaaccaaacttgtcccttccatcaaaacatttttcatactctttagcaaagtagtcacccctcctaggagaagctaattcaaatacactcattagcatctttggttacaagagcaatatagtgtgtagatgcagttaagagttctaccatggctaagtcaacattggataaaatcctataggtagatataaatgtaacctgcattttctaagctccttataagtcatcatattaagtccagatctttttgaaattttatacttattaagggcagtcatctctcactggggccactttctgtaactcaggtcaattgagaaggtcattgaatatgattcctccagtcccttccaagacaggctaggtttccaaggggcacacaaaggacaagaacatgtccagctggttcttcacaataacttcatctggatgcagcttgtgcggtagataatgggccagggtcatctcccaggcatcgacgagatatactccaacccctgagaacatcctccgaaggatggtgtccagctgaaagttgtaccagtcgctgttgaaaaggctcacctcaggtcccagctcttgggcgttggccgtccggatgaccaccacggtctttgggcttcgatcgaggagccgaaccactgctcgacggatgttcctgagccgccggatgtacacttccaaagggaaggtgctgaagtgagaccatacagctatggcaaccactgtgttcttccctcccacaatgccattcagctcattcgccacataatggagctcattgctaaagacagtcgtgaagcggatgggtggaccatggcagcggtatttgagcaggatgttgtgcttctggtccactgcaaggaagggacccacattcttgggactacccaagttaaactccactaaatctggaacaaatgtagtaaggtattcaaaccattgcctgattgttgagtcaccaaataaatgcaccacttttctttgtaagcactctgtaatgttgtcagggtcattaaactgacgcatcttaaactttctgggcctccactggtctttataataatacccagaaggaaaagttcctgagccttgagatagttctagactgttagtttcttttattctcctgggaatcacagttacccaatcaggtccactggagttgactggcattttgatattgacaccactctggaagaaagcactctctgcagcggttaggagacctttcaggtatccacctttgaaatgggtaattctgctgctgcaagggagcttctttggtttgaagcagaaccagggctccccagtgtagaggtctgtaaagttacacaggggcagattcccaggaagacacacgttgcactcagtagtttcagaaattcttcctgaacggaagagactcttgaaatagaccctgtctggtttatcttcctgtaagcgctgaagaactctgatcccttcactggggtggaccagagatacggatactttaactttgcctggccatagcaaagtaaagaaaaccttgtaaaacccattctggtaatccaccaccctgcccacagccccagcctgcagcttgagggagtgaattctggcctgcaggtagtctccaccatacttcttgggctttctttgaaaatcctgcacatgaaccagcacctcaagctggcttcccaccttaaagaaggcagcagagttcaagatgacaaagtagctggaagaagggtcagtgctcttcacaaaggggactgggcccacatcaggaacctgccggtgcaaggcagccagcaaggagtcctcctccatgcgctcctggctggacagggtctgctgatcatagccacagtagggatttcggctaattcctgtcacctgggaggaaacaaactgtccactgctgtcgatgaaagtggctgaaacagtctcatggtccaagtactctacctgagtaacattgatgaccagcaccaccaccatcaacactgcaagcagacagcagaaaagccgtagtttgaagaaattggtccacattgtctggctgtgtcttgttcacccatggccgacaccatgctaccttcactctttaaaattccatgtctttgcttttctgagctgcagatgagctttcagtttcatttgcttctatcctgctagtacccttaagagctcttatgcagaggagagactgcagttgattcaagaagcacatttttcttcaaagaaatcctatagtcccagttactcaggaggctgaggtaggagaattgcttgagcctgggaggtcgaggctgcagtgaaccatgatcatcacaccaatgtactccagcctgggcaacagagcaggactcttttttggaaattttccaagaagagatgcttactggaactagaaattagaagttacgtctaactttccttccagcatgaaattctgaactcaggcaattttgaccagaggtcctcatttttttcatgccacatgtgaagcacacataaatgttttttacatttctatacaattcttcttgctgaatctgatgtccccaaacggcagctcagtaaggccagaacagtccaccgtgtgacagcagcgccagccaagaggcagctggtgcccagagcagcgatgagccgagagatatgagatgggcagggaggcgtcgccaagtgctccgcaccgggttagtgaaggtgcctggaggacagaagtctttcgctgcggcgtggaggtccgaactgtaccgagctccgggacccgcccgcccttcgctctccgggggccagggatcctgacgccccggtcggtcgccgcagcgccaggccgctagccccccgcttcctcacccggcgacgtctcctc

SEQ ID NO: 14929 - RNA, 7246 nt, Homo sapiens
  source 1..7246: mol_type = other RNA
gctgggattacaggcatgagccactatgcccggcccacatttttttaaaaagttaaaatgtaaaagcacttttaagagacaagttagacagaaggtggtggagtacattttctgctctcctagcttctgtgtcctttaaactcctgccctcaaccatcctcttatcgtccaccacctccattcccctaggattcccaggtccccttagcactcaggggctgtggtctcaccttcaaatgaaaaacaacaacttcaaaattttatttattgcacactgaggtgtcaagaatcctaagtacactaatactacattgtagacataaaccaggtagaataatgcttaacacaagaaaataaatacacttgaagtggaatttctggcattagtgactagctgatgttaaaaagctgaatttacccagaatccacagagataatgctgagcagttttttagaaagttggggaggcttatttctgttgtttcccttgggtgtttatttccctgtacctctctcagtcatcactatttccttgaacagggtccagaaacagactcatttctggcatgtaacacatgaatatataaaggcgtaccatatttattcttgtcaagtaccctgatttaccaatctgcaaactaagttttcagattgataaatgtgaaactggattcagttattaaactggatcaagtttcaatctgaaacttaataactgaatccaggaagtgtcagttaaatggtcttaattaaaatgatagttgttcagaatggcaaaatgaatcatactggaacaccaaaggtctgttttgcattcgctgaagaaaggttacttttagtaggataattctataaaatgtaacttgcatagaaaggctttattatgggttctgtctgtcacaaatagcatcaaatcaatcatctcagttctggaatatgagattcactacattaaattaatactttcattccaaaatagaaattcatattttaaaccactgaaattgatataaaccactgctttaatattgtaaacctaaatgtccaactataatgaccaacttatctaataatgaaaactgcagtagcagaactattaagcagatctttataattaacttatgaagactatttaacatagaaaaatatttatatgtaaaaaacacagacccaaattacatattctctataagtatatggttaaaaaacctgcaagaaaatatacctaaatgctaatgttcattgcattcagatgatagaattatggattttatccatagatttttcttctagattttatagtttttaaaaattatgatgccccttatatttatattgggaaatatacatttaaacaaactattatttggctaccatgctaatattcacaaccatgtggcactagcctaaaataaacttttcagaagaaactaaattattctatctaaatattctgggaaacgtttaagtgatattggaatctctatcaaaatttccacaccagagtgaagaaagacaaattagatgtgggatgaaagttgttctcactgataagtgagagctaaatgatgagaacacatggacacataaagggcaacaacacacactggggtctattggagggtggagggtaggaggagggagaggatcaggaaaaattactaatgggtactaggcttaacacctgggtgatgaaatcatctatacaacaaacccccatgacgtaagtttacctatgaaacaaactggcacatgtacccctgaacttaaaagttgttaaaaaaaaaatttttttaagagagatgaaagtgactcaagaagctgtgtcaccaaatctttgagagctatgtcaccaaatcaaaaaataacagaaaaccagacaagatcataagaaatcatttgcacaatcaagtggcatcattccaaaccactggaggagcaatgcccgctttctttttaaaattctcctgggaaaattactcctcagcctcctttataaatccttgaggaaatgtcaagttctttcacgacaagaaaaactctcagctgggcacagtggctcacacctgtaatcccagcactttgggaagctgaggtgggcagatgcttgagctcaggagtttaagaccagcctggacaacatggcaaaatgtagtctctacaaaaagatacaaaaattagctgggcatggtggtacatacctgtagtcccagctactcaggaggctgaggcagaaggatcccttgagcccaggaagtcaaggctgcagtgagccatatcatgccactgcactccagcctgggcaaaagagcaagaccctgtctcaaaaacaaataaataaatacaaacgcttctttacgaaagtctcacaagtttagctgaaaagagatatggactctcacataccttatttcagatctaaacatgagttcctcatctataaaatggagctaatatcaccaatactattggatcatgaacagaattaaaccagttattggtaaatcccccaaaataataaacaagccatgtttattccctcattctatcttacctcttctcttagtgtttctcacagtgtggaataccaccattgcatcagaatcactgagcactcgccacaaaggttggtttcataaatcccagaggcatcatggtccctcttttttttttttttttttttttagagacagggtcttgccctgttgcccagactggagtacagtggcacaatcaaggctcactgcaacctctgcaaccttctgcctcctgggctcaagcaatcctcccacctcagcctcctaagtagcggggactacaggtggtgccaccacacccagctagtttttgtatttttttgtagagatggggtttcaccatggcacccaggctggtcttgaccttccgggctcaagcaatccgcccacctcagcctcccgagactataatccctgctgggattacagatgtgagccaacatccctggccttaattcttttattatttaacaaaaattttttagagataagatctcttgtctgttgcccaagtgggagtgtagtggcgcaatcataactcactgcagcctcaaactactgggctcaatcaatcaccctgccttagcctccctagtagctgggactgtcggcccacacctggataattttttattttttgtagagatgaggtcttactatgttgcccaggctggtctcaaactcctggcctcaagcaatcctcctgcctggcctcccaaagtgctgggattacaggcttgagctaccacaccctgccatgactctttaattctgcatttttgtcagatactacaagtgatccttaggtactgtaaagcgtaaggaccattaaaattaaactattttaatatattttattacctcattaggctcagaaacaattaaaaatcttctttccccctaaaatactttaaaaacttgaaggtgttcctcaaggacaggaaagtaagatctggggccctcctattttaaattaaaaacccaaattatttgacccattcttctaagggtatatattgttcatacttcaagcatctgtcttcctctctaaagcctccctagtttcttcatctgtctacttaggagcaacttaaactagactataatctatcacagctcaaaaagaaaagagtacttactaaatgatcccaaattaaactcgtttaaaattaataagtcaaataaaattaataattccattcttcttagatagccagtaggaatagcagcttcttccaagcatgagagaatgggtgtgccttttatgcccaaatcaagaaataccaaaaaacaaacaaacaaacaaacaaaaaactgtcatgaattttagtatcttattaatttctaattagattttaacttctaattttggtaagtagttcaaaataacaacaacaacaacaaaaaaaaaaacacctgaaactagtggaaaaaacttccacagctttataatatcgtagcattctttacacaaaagtcaattcctaaaccctcaaatttcagaacataaaaataaatttccatttacagatttcccccttccagttccaaaagtagttattctagagtaagtattcaacacataaaatttagctgaatcaaataaaaaacaatcaccaaatgcaaatatcaattccaaagcacagattttatatatactgctttcatatttcccttttgcttcttttctagataaaagcaggaaattgtaaatattcactaaaaaactcgaaccaagcacattggccttttcaagtaattcagaaaaggtagatcatcaagagaaactcctgagacacagcagtcttcagtgcattcacaagagcctctgactataagctttctctagttaaccgccagaagatggattacttgtgctatgcatgcagatgcactcaatttcctttaccagataagctacaaacactctactaccaaccaaacttgtcccttccatcaaaacatttttcatactctttagcaaagtagtcacccctcctaggagaagctaattcaaatacactcattagcatctttggttacaagagcaatatagtgtgtagatgcagttaagagttctaccatggctaagtcaacattggataaaatcctataggtagatataaatgtaacctgcattttctaagctccttataagtcatcatattaagtccagatctttttgaaattttatacttattaagggcagtcatctctcactggggccactttctgtaactcaggtcaattgagaaggtcattgaatatgattcctccagtcccttccaagacaggctaggtttccaaggggcacacaaaggacaagaacatgtccagctggttcttcacaataacttcatctggatgcagcttgtgcggtagataatgggccagggtcatctcccaggcatcgacgagatatactccaacccctgagaacatcctccgaaggatggtgtccagctgaaagttgtaccagtcgctgttgaaaaggctcacctcaggtcccagctcttgggcgttggccgtccggatgaccaccacggtctttgggcttcgatcgaggagccgaaccactgctcgacggatgttcctgagccgccggatgtacacttccaaagggaaggtgctgaagtgagaccatacagctatggcaaccactgtgttcttccctcccacaatgccattcagctcattcgccacataatggagctcattgctaaagacagtcgtgaagcggatgggtggaccatggcagcggtatttgagcaggatgttgtgcttctggtccactgcaaggaagggacccacattcttgggactacccaagttaaactccactaaatctggaacaaatgtagtaaggtattcaaaccattgcctgattgttgagtcaccaaataaatgcaccacttttctttgtaagcactctgtaatgttgtcagggtcattaaactgacgcatcttaaactttctgggcctccactggtctttataataatacccagaaggaaaagttcctgagccttgagatagttctagactgttagtttcttttattctcctgggaatcacagttacccaatcaggtccactggagttgactggcattttgatattgacaccactctggaagaaagcactctctgcagcggttaggagacctttcaggtatccacctttgaaatgggtaattctgctgctgcaagggagcttctttggtttgaagcagaaccagggctccccagtgtagaggtctgtaaagttacacaggggcagattcccaggaagacacacgttgcactcagtagtttcagaaattcttcctgaacggaagagactcttgaaatagaccctgtctggtttatcttcctgtaagcgctgaagaactctgatcccttcactggggtggaccagagatacggatactttaactttgcctggccatagcaaagtaaagaaaaccttgtaaaacccattctggtaatccaccaccctgcccacagccccagcctgcagcttgagggagtgaattctggcctgcaggtagtctccaccatacttcttgggctttctttgaaaatcctgcacatgaaccagcacctcaagctggcttcccaccttaaagaaggcagcagagttcaagatgacaaagtagctggaagaagggtcagtgctcttcacaaaggggactgggcccacatcaggaacctgccggtgcaaggcagccagcaaggagtcctcctccatgcgctcctggctggacagggtctgctgatcatagccacagtagggatttcggctaattcctgtcacctgggaggaaacaaactgtccactgctgtcgatgaaagtggctgaaacagtctcatggtccaagtactctacctgagtaacattgatgaccagcaccaccaccatcaacactgcaagcagacagcagaaaagccgtagtttgaagaaattggtccacattgtctggctgtgtcttgttcacccatggccgacaccatgctaccttcactctttaaaattccatgtctttgcttttctgagctgcagatgagctttcagtttcatttgcttctatcctgctagtacccttaagagctcttatgcagaggagagactgcagttgattcaagaagcacatttttcttcaaagaaatcctatagtcccagttactcaggaggctgaggtaggagaattgcttgagcctgggaggtcgaggctgcagtgaaccatgatcatcacaccaatgtactccagcctgggcaacagagcaggactcttttttggaaattttccaagaagagatgcttactggaactagaaattagaagttacgtctaactttccttccagcatgaaattctgaactcaggcaattttgaccagaggtcctcatttttttcatgccacatgtgaagcacacataaatgttttttacatttctatacaattcttcttgctgaatctgatgtccccaaacggcagctcagtaaggccagaacagtccaccgtgtgacagcagcgccagccaagaggcagctggtgcccagagcagcgatgagccgagagatatgagatgggcagggaggcgtcgccaagtgctccgcaccgggttagtgaaggtgcctggaggacagaagtctttcgctgcggcgtggaggtccgaactgtaccgagctgtggcgttgccgcaagt

SEQ ID NO: 14930 - RNA, 7375 nt, Homo sapiens
  source 1..7375: mol_type = other RNA
gctgggattacaggcatgagccactatgcccggcccacatttttttaaaaagttaaaatgtaaaagcacttttaagagacaagttagacagaaggtggtggagtacattttctgctctcctagcttctgtgtcctttaaactcctgccctcaaccatcctcttatcgtccaccacctccattcccctaggattcccaggtccccttagcactcaggggctgtggtctcaccttcaaatgaaaaacaacaacttcaaaattttatttattgcacactgaggtgtcaagaatcctaagtacactaatactacattgtagacataaaccaggtagaataatgcttaacacaagaaaataaatacacttgaagtggaatttctggcattagtgactagctgatgttaaaaagctgaatttacccagaatccacagagataatgctgagcagttttttagaaagttggggaggcttatttctgttgtttcccttgggtgtttatttccctgtacctctctcagtcatcactatttccttgaacagggtccagaaacagactcatttctggcatgtaacacatgaatatataaaggcgtaccatatttattcttgtcaagtaccctgatttaccaatctgcaaactaagttttcagattgataaatgtgaaactggattcagttattaaactggatcaagtttcaatctgaaacttaataactgaatccaggaagtgtcagttaaatggtcttaattaaaatgatagttgttcagaatggcaaaatgaatcatactggaacaccaaaggtctgttttgcattcgctgaagaaaggttacttttagtaggataattctataaaatgtaacttgcatagaaaggctttattatgggttctgtctgtcacaaatagcatcaaatcaatcatctcagttctggaatatgagattcactacattaaattaatactttcattccaaaatagaaattcatattttaaaccactgaaattgatataaaccactgctttaatattgtaaacctaaatgtccaactataatgaccaacttatctaataatgaaaactgcagtagcagaactattaagcagatctttataattaacttatgaagactatttaacatagaaaaatatttatatgtaaaaaacacagacccaaattacatattctctataagtatatggttaaaaaacctgcaagaaaatatacctaaatgctaatgttcattgcattcagatgatagaattatggattttatccatagatttttcttctagattttatagtttttaaaaattatgatgccccttatatttatattgggaaatatacatttaaacaaactattatttggctaccatgctaatattcacaaccatgtggcactagcctaaaataaacttttcagaagaaactaaattattctatctaaatattctgggaaacgtttaagtgatattggaatctctatcaaaatttccacaccagagtgaagaaagacaaattagatgtgggatgaaagttgttctcactgataagtgagagctaaatgatgagaacacatggacacataaagggcaacaacacacactggggtctattggagggtggagggtaggaggagggagaggatcaggaaaaattactaatgggtactaggcttaacacctgggtgatgaaatcatctatacaacaaacccccatgacgtaagtttacctatgaaacaaactggcacatgtacccctgaacttaaaagttgttaaaaaaaaaatttttttaagagagatgaaagtgactcaagaagctgtgtcaccaaatctttgagagctatgtcaccaaatcaaaaaataacagaaaaccagacaagatcataagaaatcatttgcacaatcaagtggcatcattccaaaccactggaggagcaatgcccgctttctttttaaaattctcctgggaaaattactcctcagcctcctttataaatccttgaggaaatgtcaagttctttcacgacaagaaaaactctcagctgggcacagtggctcacacctgtaatcccagcactttgggaagctgaggtgggcagatgcttgagctcaggagtttaagaccagcctggacaacatggcaaaatgtagtctctacaaaaagatacaaaaattagctgggcatggtggtacatacctgtagtcccagctactcaggaggctgaggcagaaggatcccttgagcccaggaagtcaaggctgcagtgagccatatcatgccactgcactccagcctgggcaaaagagcaagaccctgtctcaaaaacaaataaataaatacaaacgcttctttacgaaagtctcacaagtttagctgaaaagagatatggactctcacataccttatttcagatctaaacatgagttcctcatctataaaatggagctaatatcaccaatactattggatcatgaacagaattaaaccagttattggtaaatcccccaaaataataaacaagccatgtttattccctcattctatcttacctcttctcttagtgtttctcacagtgtggaataccaccattgcatcagaatcactgagcactcgccacaaaggttggtttcataaatcccagaggcatcatggtccctcttttttttttttttttttttttagagacagggtcttgccctgttgcccagactggagtacagtggcacaatcaaggctcactgcaacctctgcaaccttctgcctcctgggctcaagcaatcctcccacctcagcctcctaagtagcggggactacaggtggtgccaccacacccagctagtttttgtatttttttgtagagatggggtttcaccatggcacccaggctggtcttgaccttccgggctcaagcaatccgcccacctcagcctcccgagactataatccctgctgggattacagatgtgagccaacatccctggccttaattcttttattatttaacaaaaattttttagagataagatctcttgtctgttgcccaagtgggagtgtagtggcgcaatcataactcactgcagcctcaaactactgggctcaatcaatcaccctgccttagcctccctagtagctgggactgtcggcccacacctggataattttttattttttgtagagatgaggtcttactatgttgcccaggctggtctcaaactcctggcctcaagcaatcctcctgcctggcctcccaaagtgctgggattacaggcttgagctaccacaccctgccatgactctttaattctgcatttttgtcagatactacaagtgatccttaggtactgtaaagcgtaaggaccattaaaattaaactattttaatatattttattacctcattaggctcagaaacaattaaaaatcttctttccccctaaaatactttaaaaacttgaaggtgttcctcaaggacaggaaagtaagatctggggccctcctattttaaattaaaaacccaaattatttgacccattcttctaagggtatatattgttcatacttcaagcatctgtcttcctctctaaagcctccctagtttcttcatctgtctacttaggagcaacttaaactagactataatctatcacagctcaaaaagaaaagagtacttactaaatgatcccaaattaaactcgtttaaaattaataagtcaaataaaattaataattccattcttcttagatagccagtaggaatagcagcttcttccaagcatgagagaatgggtgtgccttttatgcccaaatcaagaaataccaaaaaacaaacaaacaaacaaacaaaaaactgtcatgaattttagtatcttattaatttctaattagattttaacttctaattttggtaagtagttcaaaataacaacaacaacaacaaaaaaaaaaacacctgaaactagtggaaaaaacttccacagctttataatatcgtagcattctttacacaaaagtcaattcctaaaccctcaaatttcagaacataaaaataaatttccatttacagatttcccccttccagttccaaaagtagttattctagagtaagtattcaacacataaaatttagctgaatcaaataaaaaacaatcaccaaatgcaaatatcaattccaaagcacagattttatatatactgctttcatatttcccttttgcttcttttctagataaaagcaggaaattgtaaatattcactaaaaaactcgaaccaagcacattggccttttcaagtaattcagaaaaggtagatcatcaagagaaactcctgagacacagcagtcttcagtgcattcacaagagcctctgactataagctttctctagttaaccgccagaagatggattacttgtgctatgcatgcagatgcactcaatttcctttaccagataagctacaaacactctactaccaaccaaacttgtcccttccatcaaaacatttttcatactctttagcaaagtagtcacccctcctaggagaagctaattcaaatacactcattagcatctttggttacaagagcaatatagtgtgtagatgcagttaagagttctaccatggctaagtcaacattggataaaatcctataggtagatataaatgtaacctgcattttctaagctccttataagtcatcatattaagtccagatctttttgaaattttatacttattaagggcagtcatctctcactggggccactttctgtaactcaggtcaattgagaaggtcattgaatatgattcctccagtcccttccaagacaggctaggtttccaaggggcacacaaaggacaagaacatgtccagctggttcttcacaataacttcatctggatgcagcttgtgcggtagataatgggccagggtcatctcccaggcatcgacgagatatactccaacccctgagaacatcctccgaaggatggtgtccagctgaaagttgtaccagtcgctgttgaaaaggctcacctcaggtcccagctcttgggcgttggccgtccggatgaccaccacggtctttgggcttcgatcgaggagccgaaccactgctcgacggatgttcctgagccgccggatgtacacttccaaagggaaggtgctgaagtgagaccatacagctatggcaaccactgtgttcttccctcccacaatgccattcagctcattcgccacataatggagctcattgctaaagacagtcgtgaagcggatgggtggaccatggcagcggtatttgagcaggatgttgtgcttctggtccactgcaaggaagggacccacattcttgggactacccaagttaaactccactaaatctggaacaaatgtagtaaggtattcaaaccattgcctgattgttgagtcaccaaataaatgcaccacttttctttgtaagcactctgtaatgttgtcagggtcattaaactgacgcatcttaaactttctgggcctccactggtctttataataatacccagaaggaaaagttcctgagccttgagatagttctagactgttagtttcttttattctcctgggaatcacagttacccaatcaggtccactggagttgactggcattttgatattgacaccactctggaagaaagcactctctgcagcggttaggagacctttcaggtatccacctttgaaatgggtaattctgctgctgcaagggagcttctttggtttgaagcagaaccagggctccccagtgtagaggtctgtaaagttacacaggggcagattcccaggaagacacacgttgcactcagtagtttcagaaattcttcctgaacggaagagactcttgaaatagaccctgtctggtttatcttcctgtaagcgctgaagaactctgatcccttcactggggtggaccagagatacggatactttaactttgcctggccatagcaaagtaaagaaaaccttgtaaaacccattctggtaatccaccaccctgcccacagccccagcctgcagcttgagggagtgaattctggcctgcaggtagtctccaccatacttcttgggctttctttgaaaatcctgcacatgaaccagcacctcaagctggcttcccaccttaaagaaggcagcagagttcaagatgacaaagtagctggaagaagggtcagtgctcttcacaaaggggactgggcccacatcaggaacctgccggtgcaaggcagccagcaaggagtcctcctccatgcgctcctggctggacagggtctgctgatcatagccacagtagggatttcggctaattcctgtcacctgggaggaaacaaactgtccactgctgtcgatgaaagtggctgaaacagtctcatggtccaagtactctacctgagtaacattgatgaccagcaccaccaccatcaacactgcaagcagacagcagaaaagccgtagtttgaagaaattggtccacattgtctggctgtgtcttgttcacccatggccgacaccatgctaccttcactctttaaaattccatgtctttgcttttctgagctgcagatgagctttcagtttcatttgcttctatcctgctagtacccttaagagctcttatgcagaggagagactgcagttgattcaagaagcacatttttcttcaaagaaatcctatagtcccagttactcaggaggctgaggtaggagaattgcttgagcctgggaggtcgaggctgcagtgaaccatgatcatcacaccaatgtactccagcctgggcaacagagcaggactcttttttggaaattttccaagaagagatgcttactggaactagaaattagaagttacgtctaactttccttccagcatgaaattctgaactcaggcaattttgaccagaggtcctcatttttttcatgccacatgtgaagcacacataaatgttttttacatttctatacaattcttcttgcttgtaaagttacactcgtttctccccatacgacctgaatctgatgtccccaaacggcagctcagtaaggccagaacagtccaccgtgtgacagcagcgccagccaagaggcagctggtgcccagagcagcgatgagccgagagatatgagatgggcagggaggcgtcgccaagtgctccgcaccgggttagtgaaggtgcctggaggacagaagtctttcgctgcggcgtggaggtccgaactgtaccgagctccgggacccgcccgcccttcgctctccgggggccagggatcctgacgccccggtcggtcgccgcagcgccaggccgctagccccccgcttcctcacccggcgacgtctcctc

SEQ ID NO: 14931 - RNA, 7280 nt, Homo sapiens
  source 1..7280: mol_type = other RNA
gctgggattacaggcatgagccactatgcccggcccacatttttttaaaaagttaaaatgtaaaagcacttttaagagacaagttagacagaaggtggtggagtacattttctgctctcctagcttctgtgtcctttaaactcctgccctcaaccatcctcttatcgtccaccacctccattcccctaggattcccaggtccccttagcactcaggggctgtggtctcaccttcaaatgaaaaacaacaacttcaaaattttatttattgcacactgaggtgtcaagaatcctaagtacactaatactacattgtagacataaaccaggtagaataatgcttaacacaagaaaataaatacacttgaagtggaatttctggcattagtgactagctgatgttaaaaagctgaatttacccagaatccacagagataatgctgagcagttttttagaaagttggggaggcttatttctgttgtttcccttgggtgtttatttccctgtacctctctcagtcatcactatttccttgaacagggtccagaaacagactcatttctggcatgtaacacatgaatatataaaggcgtaccatatttattcttgtcaagtaccctgatttaccaatctgcaaactaagttttcagattgataaatgtgaaactggattcagttattaaactggatcaagtttcaatctgaaacttaataactgaatccaggaagtgtcagttaaatggtcttaattaaaatgatagttgttcagaatggcaaaatgaatcatactggaacaccaaaggtctgttttgcattcgctgaagaaaggttacttttagtaggataattctataaaatgtaacttgcatagaaaggctttattatgggttctgtctgtcacaaatagcatcaaatcaatcatctcagttctggaatatgagattcactacattaaattaatactttcattccaaaatagaaattcatattttaaaccactgaaattgatataaaccactgctttaatattgtaaacctaaatgtccaactataatgaccaacttatctaataatgaaaactgcagtagcagaactattaagcagatctttataattaacttatgaagactatttaacatagaaaaatatttatatgtaaaaaacacagacccaaattacatattctctataagtatatggttaaaaaacctgcaagaaaatatacctaaatgctaatgttcattgcattcagatgatagaattatggattttatccatagatttttcttctagattttatagtttttaaaaattatgatgccccttatatttatattgggaaatatacatttaaacaaactattatttggctaccatgctaatattcacaaccatgtggcactagcctaaaataaacttttcagaagaaactaaattattctatctaaatattctgggaaacgtttaagtgatattggaatctctatcaaaatttccacaccagagtgaagaaagacaaattagatgtgggatgaaagttgttctcactgataagtgagagctaaatgatgagaacacatggacacataaagggcaacaacacacactggggtctattggagggtggagggtaggaggagggagaggatcaggaaaaattactaatgggtactaggcttaacacctgggtgatgaaatcatctatacaacaaacccccatgacgtaagtttacctatgaaacaaactggcacatgtacccctgaacttaaaagttgttaaaaaaaaaatttttttaagagagatgaaagtgactcaagaagctgtgtcaccaaatctttgagagctatgtcaccaaatcaaaaaataacagaaaaccagacaagatcataagaaatcatttgcacaatcaagtggcatcattccaaaccactggaggagcaatgcccgctttctttttaaaattctcctgggaaaattactcctcagcctcctttataaatccttgaggaaatgtcaagttctttcacgacaagaaaaactctcagctgggcacagtggctcacacctgtaatcccagcactttgggaagctgaggtgggcagatgcttgagctcaggagtttaagaccagcctggacaacatggcaaaatgtagtctctacaaaaagatacaaaaattagctgggcatggtggtacatacctgtagtcccagctactcaggaggctgaggcagaaggatcccttgagcccaggaagtcaaggctgcagtgagccatatcatgccactgcactccagcctgggcaaaagagcaagaccctgtctcaaaaacaaataaataaatacaaacgcttctttacgaaagtctcacaagtttagctgaaaagagatatggactctcacataccttatttcagatctaaacatgagttcctcatctataaaatggagctaatatcaccaatactattggatcatgaacagaattaaaccagttattggtaaatcccccaaaataataaacaagccatgtttattccctcattctatcttacctcttctcttagtgtttctcacagtgtggaataccaccattgcatcagaatcactgagcactcgccacaaaggttggtttcataaatcccagaggcatcatggtccctcttttttttttttttttttttttagagacagggtcttgccctgttgcccagactggagtacagtggcacaatcaaggctcactgcaacctctgcaaccttctgcctcctgggctcaagcaatcctcccacctcagcctcctaagtagcggggactacaggtggtgccaccacacccagctagtttttgtatttttttgtagagatggggtttcaccatggcacccaggctggtcttgaccttccgggctcaagcaatccgcccacctcagcctcccgagactataatccctgctgggattacagatgtgagccaacatccctggccttaattcttttattatttaacaaaaattttttagagataagatctcttgtctgttgcccaagtgggagtgtagtggcgcaatcataactcactgcagcctcaaactactgggctcaatcaatcaccctgccttagcctccctagtagctgggactgtcggcccacacctggataattttttattttttgtagagatgaggtcttactatgttgcccaggctggtctcaaactcctggcctcaagcaatcctcctgcctggcctcccaaagtgctgggattacaggcttgagctaccacaccctgccatgactctttaattctgcatttttgtcagatactacaagtgatccttaggtactgtaaagcgtaaggaccattaaaattaaactattttaatatattttattacctcattaggctcagaaacaattaaaaatcttctttccccctaaaatactttaaaaacttgaaggtgttcctcaaggacaggaaagtaagatctggggccctcctattttaaattaaaaacccaaattatttgacccattcttctaagggtatatattgttcatacttcaagcatctgtcttcctctctaaagcctccctagtttcttcatctgtctacttaggagcaacttaaactagactataatctatcacagctcaaaaagaaaagagtacttactaaatgatcccaaattaaactcgtttaaaattaataagtcaaataaaattaataattccattcttcttagatagccagtaggaatagcagcttcttccaagcatgagagaatgggtgtgccttttatgcccaaatcaagaaataccaaaaaacaaacaaacaaacaaacaaaaaactgtcatgaattttagtatcttattaatttctaattagattttaacttctaattttggtaagtagttcaaaataacaacaacaacaacaaaaaaaaaaacacctgaaactagtggaaaaaacttccacagctttataatatcgtagcattctttacacaaaagtcaattcctaaaccctcaaatttcagaacataaaaataaatttccatttacagatttcccccttccagttccaaaagtagttattctagagtaagtattcaacacataaaatttagctgaatcaaataaaaaacaatcaccaaatgcaaatatcaattccaaagcacagattttatatatactgctttcatatttcccttttgcttcttttctagataaaagcaggaaattgtaaatattcactaaaaaactcgaaccaagcacattggccttttcaagtaattcagaaaaggtagatcatcaagagaaactcctgagacacagcagtcttcagtgcattcacaagagcctctgactataagctttctctagttaaccgccagaagatggattacttgtgctatgcatgcagatgcactcaatttcctttaccagataagctacaaacactctactaccaaccaaacttgtcccttccatcaaaacatttttcatactctttagcaaagtagtcacccctcctaggagaagctaattcaaatacactcattagcatctttggttacaagagcaatatagtgtgtagatgcagttaagagttctaccatggctaagtcaacattggataaaatcctataggtagatataaatgtaacctgcattttctaagctccttataagtcatcatattaagtccagatctttttgaaattttatacttattaagggcagtcatctctcactggggccactttctgtaactcaggtcaattgagaaggtcattgaatatgattcctccagtcccttccaagacaggctaggtttccaaggggcacacaaaggacaagaacatgtccagctggttcttcacaataacttcatctggatgcagcttgtgcggtagataatgggccagggtcatctcccaggcatcgacgagatatactccaacccctgagaacatcctccgaaggatggtgtccagctgaaagttgtaccagtcgctgttgaaaaggctcacctcaggtcccagctcttgggcgttggccgtccggatgaccaccacggtctttgggcttcgatcgaggagccgaaccactgctcgacggatgttcctgagccgccggatgtacacttccaaagggaaggtgctgaagtgagaccatacagctatggcaaccactgtgttcttccctcccacaatgccattcagctcattcgccacataatggagctcattgctaaagacagtcgtgaagcggatgggtggaccatggcagcggtatttgagcaggatgttgtgcttctggtccactgcaaggaagggacccacattcttgggactacccaagttaaactccactaaatctggaacaaatgtagtaaggtattcaaaccattgcctgattgttgagtcaccaaataaatgcaccacttttctttgtaagcactctgtaatgttgtcagggtcattaaactgacgcatcttaaactttctgggcctccactggtctttataataatacccagaaggaaaagttcctgagccttgagatagttctagactgttagtttcttttattctcctgggaatcacagttacccaatcaggtccactggagttgactggcattttgatattgacaccactctggaagaaagcactctctgcagcggttaggagacctttcaggtatccacctttgaaatgggtaattctgctgctgcaagggagcttctttggtttgaagcagaaccagggctccccagtgtagaggtctgtaaagttacacaggggcagattcccaggaagacacacgttgcactcagtagtttcagaaattcttcctgaacggaagagactcttgaaatagaccctgtctggtttatcttcctgtaagcgctgaagaactctgatcccttcactggggtggaccagagatacggatactttaactttgcctggccatagcaaagtaaagaaaaccttgtaaaacccattctggtaatccaccaccctgcccacagccccagcctgcagcttgagggagtgaattctggcctgcaggtagtctccaccatacttcttgggctttctttgaaaatcctgcacatgaaccagcacctcaagctggcttcccaccttaaagaaggcagcagagttcaagatgacaaagtagctggaagaagggtcagtgctcttcacaaaggggactgggcccacatcaggaacctgccggtgcaaggcagccagcaaggagtcctcctccatgcgctcctggctggacagggtctgctgatcatagccacagtagggatttcggctaattcctgtcacctgggaggaaacaaactgtccactgctgtcgatgaaagtggctgaaacagtctcatggtccaagtactctacctgagtaacattgatgaccagcaccaccaccatcaacactgcaagcagacagcagaaaagccgtagtttgaagaaattggtccacattgtctggctgtgtcttgttcacccatggccgacaccatgctaccttcactctttaaaattccatgtctttgcttttctgagctgcagatgagctttcagtttcatttgcttctatcctgctagtacccttaagagctcttatgcagaggagagactgcagttgattcaagaagcacatttttcttcaaagaaatcctatagtcccagttactcaggaggctgaggtaggagaattgcttgagcctgggaggtcgaggctgcagtgaaccatgatcatcacaccaatgtactccagcctgggcaacagagcaggactcttttttggaaattttccaagaagagatgcttactggaactagaaattagaagttacgtctaactttccttccagcatgaaattctgaactcaggcaattttgaccagaggtcctcatttttttcatgccacatgtgaagcacacataaatgttttttacatttctatacaattcttcttgcttgtaaagttacactcgtttctccccatacgacctgaatctgatgtccccaaacggcagctcagtaaggccagaacagtccaccgtgtgacagcagcgccagccaagaggcagctggtgcccagagcagcgatgagccgagagatatgagatgggcagggaggcgtcgccaagtgctccgcaccgggttagtgaaggtgcctggaggacagaagtctttcgctgcggcgtggaggtccgaactgtaccgagctgtggcgttgccgcaagt

SEQ ID NO: 14932 - RNA, 6916 nt, Homo sapiens
  source 1..6916: mol_type = other RNA
gctgggattacaggcatgagccactatgcccggcccacatttttttaaaaagttaaaatgtaaaagcacttttaagagacaagttagacagaaggtggtggagtacattttctgctctcctagcttctgtgtcctttaaactcctgccctcaaccatcctcttatcgtccaccacctccattcccctaggattcccaggtccccttagcactcaggggctgtggtctcaccttcaaatgaaaaacaacaacttcaaaattttatttattgcacactgaggtgtcaagaatcctaagtacactaatactacattgtagacataaaccaggtagaataatgcttaacacaagaaaataaatacacttgaagtggaatttctggcattagtgactagctgatgttaaaaagctgaatttacccagaatccacagagataatgctgagcagttttttagaaagttggggaggcttatttctgttgtttcccttgggtgtttatttccctgtacctctctcagtcatcactatttccttgaacagggtccagaaacagactcatttctggcatgtaacacatgaatatataaaggcgtaccatatttattcttgtcaagtaccctgatttaccaatctgcaaactaagttttcagattgataaatgtgaaactggattcagttattaaactggatcaagtttcaatctgaaacttaataactgaatccaggaagtgtcagttaaatggtcttaattaaaatgatagttgttcagaatggcaaaatgaatcatactggaacaccaaaggtctgttttgcattcgctgaagaaaggttacttttagtaggataattctataaaatgtaacttgcatagaaaggctttattatgggttctgtctgtcacaaatagcatcaaatcaatcatctcagttctggaatatgagattcactacattaaattaatactttcattccaaaatagaaattcatattttaaaccactgaaattgatataaaccactgctttaatattgtaaacctaaatgtccaactataatgaccaacttatctaataatgaaaactgcagtagcagaactattaagcagatctttataattaacttatgaagactatttaacatagaaaaatatttatatgtaaaaaacacagacccaaattacatattctctataagtatatggttaaaaaacctgcaagaaaatatacctaaatgctaatgttcattgcattcagatgatagaattatggattttatccatagatttttcttctagattttatagtttttaaaaattatgatgccccttatatttatattgggaaatatacatttaaacaaactattatttggctaccatgctaatattcacaaccatgtggcactagcctaaaataaacttttcagaagaaactaaattattctatctaaatattctgggaaacgtttaagtgatattggaatctctatcaaaatttccacaccagagtgaagaaagacaaattagatgtgggatgaaagttgttctcactgataagtgagagctaaatgatgagaacacatggacacataaagggcaacaacacacactggggtctattggagggtggagggtaggaggagggagaggatcaggaaaaattactaatgggtactaggcttaacacctgggtgatgaaatcatctatacaacaaacccccatgacgtaagtttacctatgaaacaaactggcacatgtacccctgaacttaaaagttgttaaaaaaaaaatttttttaagagagatgaaagtgactcaagaagctgtgtcaccaaatctttgagagctatgtcaccaaatcaaaaaataacagaaaaccagacaagatcataagaaatcatttgcacaatcaagtggcatcattccaaaccactggaggagcaatgcccgctttctttttaaaattctcctgggaaaattactcctcagcctcctttataaatccttgaggaaatgtcaagttctttcacgacaagaaaaactctcagctgggcacagtggctcacacctgtaatcccagcactttgggaagctgaggtgggcagatgcttgagctcaggagtttaagaccagcctggacaacatggcaaaatgtagtctctacaaaaagatacaaaaattagctgggcatggtggtacatacctgtagtcccagctactcaggaggctgaggcagaaggatcccttgagcccaggaagtcaaggctgcagtgagccatatcatgccactgcactccagcctgggcaaaagagcaagaccctgtctcaaaaacaaataaataaatacaaacgcttctttacgaaagtctcacaagtttagctgaaaagagatatggactctcacataccttatttcagatctaaacatgagttcctcatctataaaatggagctaatatcaccaatactattggatcatgaacagaattaaaccagttattggtaaatcccccaaaataataaacaagccatgtttattccctcattctatcttacctcttctcttagtgtttctcacagtgtggaataccaccattgcatcagaatcactgagcactcgccacaaaggttggtttcataaatcccagaggcatcatggtccctcttttttttttttttttttttttagagacagggtcttgccctgttgcccagactggagtacagtggcacaatcaaggctcactgcaacctctgcaaccttctgcctcctgggctcaagcaatcctcccacctcagcctcctaagtagcggggactacaggtggtgccaccacacccagctagtttttgtatttttttgtagagatggggtttcaccatggcacccaggctggtcttgaccttccgggctcaagcaatccgcccacctcagcctcccgagactataatccctgctgggattacagatgtgagccaacatccctggccttaattcttttattatttaacaaaaattttttagagataagatctcttgtctgttgcccaagtgggagtgtagtggcgcaatcataactcactgcagcctcaaactactgggctcaatcaatcaccctgccttagcctccctagtagctgggactgtcggcccacacctggataattttttattttttgtagagatgaggtcttactatgttgcccaggctggtctcaaactcctggcctcaagcaatcctcctgcctggcctcccaaagtgctgggattacaggcttgagctaccacaccctgccatgactctttaattctgcatttttgtcagatactacaagtgatccttaggtactgtaaagcgtaaggaccattaaaattaaactattttaatatattttattacctcattaggctcagaaacaattaaaaatcttctttccccctaaaatactttaaaaacttgaaggtgttcctcaaggacaggaaagtaagatctggggccctcctattttaaattaaaaacccaaattatttgacccattcttctaagggtatatattgttcatacttcaagcatctgtcttcctctctaaagcctccctagtttcttcatctgtctacttaggagcaacttaaactagactataatctatcacagctcaaaaagaaaagagtacttactaaatgatcccaaattaaactcgtttaaaattaataagtcaaataaaattaataattccattcttcttagatagccagtaggaatagcagcttcttccaagcatgagagaatgggtgtgccttttatgcccaaatcaagaaataccaaaaaacaaacaaacaaacaaacaaaaaactgtcatgaattttagtatcttattaatttctaattagattttaacttctaattttggtaagtagttcaaaataacaacaacaacaacaaaaaaaaaaacacctgaaactagtggaaaaaacttccacagctttataatatcgtagcattctttacacaaaagtcaattcctaaaccctcaaatttcagaacataaaaataaatttccatttacagatttcccccttccagttccaaaagtagttattctagagtaagtattcaacacataaaatttagctgaatcaaataaaaaacaatcaccaaatgcaaatatcaattccaaagcacagattttatatatactgctttcatatttcccttttgcttcttttctagataaaagcaggaaattgtaaatattcactaaaaaactcgaaccaagcacattggccttttcaagtaattcagaaaaggtagatcatcaagagaaactcctgagacacagcagtcttcagtgcattcacaagagcctctgactataagctttctctagttaaccgccagaagatggattacttgtgctatgcatgcagatgcactcaatttcctttaccagataagctacaaacactctactaccaaccaaacttgtcccttccatcaaaacatttttcatactctttagcaaagtagtcacccctcctaggagaagctaattcaaatacactcattagcatctttggttacaagagcaatatagtgtgtagatgcagttaagagttctaccatggctaagtcaacattggataaaatcctataggtagatataaatgtaacctgcattttctaagctccttataagtcatcatattaagtccagatctttttgaaattttatacttattaagggcagtcatctctcactggggccactttctgtaactcaggtcaattgagaaggtcattgaatatgattcctccagtcccttccaagacaggctaggtttccaaggggcacacaaaggacaagaacatgtccagctggttcttcacaataacttcatctggatgcagcttgtgcggtagataatgggccagggtcatctcccaggcatcgacgagatatactccaacccctgagaacatcctccgaaggatggtgtccagctgaaagttgtaccagtcgctgttgaaaaggctcacctcaggtcccagctcttgggcgttggccgtccggatgaccaccacggtctttgggcttcgatcgaggagccgaaccactgctcgacggatgttcctgagccgccggatgtacacttccaaagggaaggtgctgaagtgagaccatacagctatggcaaccactgtgttcttccctcccacaatgccattcagctcattcgccacataatggagctcattgctaaagacagtcgtgaagcggatgggtggaccatggcagcggtatttgagcaggatgttgtgcttctggtccactgcaaggaagggacccacattcttgggactacccaagttaaactccactaaatcttttattctcctgggaatcacagttacccaatcaggtccactggagttgactggcattttgatattgacaccactctggaagaaagcactctctgcagcggttaggagacctttcaggtatccacctttgaaatgggtaattctgctgctgcaagggagcttctttggtttgaagcagaaccagggctccccagtgtagaggtctgtaaagttacacaggggcagattcccaggaagacacacgttgcactcagtagtttcagaaattcttcctgaacggaagagactcttgaaatagaccctgtctggtttatcttcctgtaagcgctgaagaactctgatcccttcactggggtggaccagagatacggatactttaactttgcctggccatagcaaagtaaagaaaaccttgtaaaacccattctggtaatccaccaccctgcccacagccccagcctgcagcttgagggagtgaattctggcctgcaggtagtctccaccatacttcttgggctttctttgaaaatcctgcacatgaaccagcacctcaagctggcttcccaccttaaagaaggcagcagagttcaagatgacaaagtagctggaagaagggtcagtgctcttcacaaaggggactgggcccacatcaggaacctgccggtgcaaggcagccagcaaggagtcctcctccatgcgctcctggctggacagggtctgctgatcatagccacagtagggatttcggctaattcctgtcacctgggaggaaacaaactgtccactgctgtcgatgaaagtggctgaaacagtctcatggtccaagtactctacctgagtaacattgatgaccagcaccaccaccatcaacactgcaagcagacagcagaaaagccgtagtttgaagaaattggtccacattgtctggctgtgtcttgttcacccatggccgacaccatgctaccttcactctttaaaattccatgtctttgcttttctgagctgcagatgagctttcagtttcatttgcttctatcctgctagtacccttaagagctcttatgcagaggagagactgcagttgattcaagaagcacatttttcttcaaagaaatcctatagtcccagttactcaggaggctgaggtaggagaattgcttgagcctgggaggtcgaggctgcagtgaaccatgatcatcacaccaatgtactccagcctgggcaacagagcaggactcttttttggaaattttccaagaagagatgcttactggaactagaaattagaagttacgtctaactttccttccagcatgaaattctgaactcaggcaattttgaccagaggtcctcatttttttcatgccacatgtgaagcacacataaatgttttttacatttctatacaattcttcttgctccgggacccgcccgcccttcgctctccgggggccagggatcctgacgccccggtcggtcgccgcagcgccaggccgctagccccccgcttcctcacccggcgacgtctcctc

SEQ ID NO: 14933 - RNA, 7039 nt, Homo sapiens
  source 1..7039: mol_type = other RNA
gctgggattacaggcatgagccactatgcccggcccacatttttttaaaaagttaaaatgtaaaagcacttttaagagacaagttagacagaaggtggtggagtacattttctgctctcctagcttctgtgtcctttaaactcctgccctcaaccatcctcttatcgtccaccacctccattcccctaggattcccaggtccccttagcactcaggggctgtggtctcaccttcaaatgaaaaacaacaacttcaaaattttatttattgcacactgaggtgtcaagaatcctaagtacactaatactacattgtagacataaaccaggtagaataatgcttaacacaagaaaataaatacacttgaagtggaatttctggcattagtgactagctgatgttaaaaagctgaatttacccagaatccacagagataatgctgagcagttttttagaaagttggggaggcttatttctgttgtttcccttgggtgtttatttccctgtacctctctcagtcatcactatttccttgaacagggtccagaaacagactcatttctggcatgtaacacatgaatatataaaggcgtaccatatttattcttgtcaagtaccctgatttaccaatctgcaaactaagttttcagattgataaatgtgaaactggattcagttattaaactggatcaagtttcaatctgaaacttaataactgaatccaggaagtgtcagttaaatggtcttaattaaaatgatagttgttcagaatggcaaaatgaatcatactggaacaccaaaggtctgttttgcattcgctgaagaaaggttacttttagtaggataattctataaaatgtaacttgcatagaaaggctttattatgggttctgtctgtcacaaatagcatcaaatcaatcatctcagttctggaatatgagattcactacattaaattaatactttcattccaaaatagaaattcatattttaaaccactgaaattgatataaaccactgctttaatattgtaaacctaaatgtccaactataatgaccaacttatctaataatgaaaactgcagtagcagaactattaagcagatctttataattaacttatgaagactatttaacatagaaaaatatttatatgtaaaaaacacagacccaaattacatattctctataagtatatggttaaaaaacctgcaagaaaatatacctaaatgctaatgttcattgcattcagatgatagaattatggattttatccatagatttttcttctagattttatagtttttaaaaattatgatgccccttatatttatattgggaaatatacatttaaacaaactattatttggctaccatgctaatattcacaaccatgtggcactagcctaaaataaacttttcagaagaaactaaattattctatctaaatattctgggaaacgtttaagtgatattggaatctctatcaaaatttccacaccagagtgaagaaagacaaattagatgtgggatgaaagttgttctcactgataagtgagagctaaatgatgagaacacatggacacataaagggcaacaacacacactggggtctattggagggtggagggtaggaggagggagaggatcaggaaaaattactaatgggtactaggcttaacacctgggtgatgaaatcatctatacaacaaacccccatgacgtaagtttacctatgaaacaaactggcacatgtacccctgaacttaaaagttgttaaaaaaaaaatttttttaagagagatgaaagtgactcaagaagctgtgtcaccaaatctttgagagctatgtcaccaaatcaaaaaataacagaaaaccagacaagatcataagaaatcatttgcacaatcaagtggcatcattccaaaccactggaggagcaatgcccgctttctttttaaaattctcctgggaaaattactcctcagcctcctttataaatccttgaggaaatgtcaagttctttcacgacaagaaaaactctcagctgggcacagtggctcacacctgtaatcccagcactttgggaagctgaggtgggcagatgcttgagctcaggagtttaagaccagcctggacaacatggcaaaatgtagtctctacaaaaagatacaaaaattagctgggcatggtggtacatacctgtagtcccagctactcaggaggctgaggcagaaggatcccttgagcccaggaagtcaaggctgcagtgagccatatcatgccactgcactccagcctgggcaaaagagcaagaccctgtctcaaaaacaaataaataaatacaaacgcttctttacgaaagtctcacaagtttagctgaaaagagatatggactctcacataccttatttcagatctaaacatgagttcctcatctataaaatggagctaatatcaccaatactattggatcatgaacagaattaaaccagttattggtaaatcccccaaaataataaacaagccatgtttattccctcattctatcttacctcttctcttagtgtttctcacagtgtggaataccaccattgcatcagaatcactgagcactcgccacaaaggttggtttcataaatcccagaggcatcatggtccctcttttttttttttttttttttttagagacagggtcttgccctgttgcccagactggagtacagtggcacaatcaaggctcactgcaacctctgcaaccttctgcctcctgggctcaagcaatcctcccacctcagcctcctaagtagcggggactacaggtggtgccaccacacccagctagtttttgtatttttttgtagagatggggtttcaccatggcacccaggctggtcttgaccttccgggctcaagcaatccgcccacctcagcctcccgagactataatccctgctgggattacagatgtgagccaacatccctggccttaattcttttattatttaacaaaaattttttagagataagatctcttgtctgttgcccaagtgggagtgtagtggcgcaatcataactcactgcagcctcaaactactgggctcaatcaatcaccctgccttagcctccctagtagctgggactgtcggcccacacctggataattttttattttttgtagagatgaggtcttactatgttgcccaggctggtctcaaactcctggcctcaagcaatcctcctgcctggcctcccaaagtgctgggattacaggcttgagctaccacaccctgccatgactctttaattctgcatttttgtcagatactacaagtgatccttaggtactgtaaagcgtaaggaccattaaaattaaactattttaatatattttattacctcattaggctcagaaacaattaaaaatcttctttccccctaaaatactttaaaaacttgaaggtgttcctcaaggacaggaaagtaagatctggggccctcctattttaaattaaaaacccaaattatttgacccattcttctaagggtatatattgttcatacttcaagcatctgtcttcctctctaaagcctccctagtttcttcatctgtctacttaggagcaacttaaactagactataatctatcacagctcaaaaagaaaagagtacttactaaatgatcccaaattaaactcgtttaaaattaataagtcaaataaaattaataattccattcttcttagatagccagtaggaatagcagcttcttccaagcatgagagaatgggtgtgccttttatgcccaaatcaagaaataccaaaaaacaaacaaacaaacaaacaaaaaactgtcatgaattttagtatcttattaatttctaattagattttaacttctaattttggtaagtagttcaaaataacaacaacaacaacaaaaaaaaaaacacctgaaactagtggaaaaaacttccacagctttataatatcgtagcattctttacacaaaagtcaattcctaaaccctcaaatttcagaacataaaaataaatttccatttacagatttcccccttccagttccaaaagtagttattctagagtaagtattcaacacataaaatttagctgaatcaaataaaaaacaatcaccaaatgcaaatatcaattccaaagcacagattttatatatactgctttcatatttcccttttgcttcttttctagataaaagcaggaaattgtaaatattcactaaaaaactcgaaccaagcacattggccttttcaagtaattcagaaaaggtagatcatcaagagaaactcctgagacacagcagtcttcagtgcattcacaagagcctctgactataagctttctctagttaaccgccagaagatggattacttgtgctatgcatgcagatgcactcaatttcctttaccagataagctacaaacactctactaccaaccaaacttgtcccttccatcaaaacatttttcatactctttagcaaagtagtcacccctcctaggagaagctaattcaaatacactcattagcatctttggttacaagagcaatatagtgtgtagatgcagttaagagttctaccatggctaagtcaacattggataaaatcctataggtagatataaatgtaacctgcattttctaagctccttataagtcatcatattaagtccagatctttttgaaattttatacttattaagggcagtcatctctcactggggccactttctgtaactcaggtcaattgagaaggtcattgaatatgattcctccagtcccttccaagacaggctaggtttccaaggggcacacaaaggacaagaacatgtccagctggttcttcacaataacttcatctggatgcagcttgtgcggtagataatgggccagggtcatctcccaggcatcgacgagatatactccaacccctgagaacatcctccgaaggatggtgtccagctgaaagttgtaccagtcgctgttgaaaaggctcacctcaggtcccagctcttgggcgttggccgtccggatgaccaccacggtctttgggcttcgatcgaggagccgaaccactgctcgacggatgttcctgagccgccggatgtacacttccaaagggaaggtgctgaagtgagaccatacagctatggcaaccactgtgttcttccctcccacaatgccattcagctcattcgccacataatggagctcattgctaaagacagtcgtgaagcggatgggtggaccatggcagcggtatttgagcaggatgttgtgcttctggtccactgcaaggaagggacccacattcttgggactacccaagttaaactccactaaatcttttattctcctgggaatcacagttacccaatcaggtccactggagttgactggcattttgatattgacaccactctggaagaaagcactctctgcagcggttaggagacctttcaggtatccacctttgaaatgggtaattctgctgctgcaagggagcttctttggtttgaagcagaaccagggctccccagtgtagaggtctgtaaagttacacaggggcagattcccaggaagacacacgttgcactcagtagtttcagaaattcttcctgaacggaagagactcttgaaatagaccctgtctggtttatcttcctgtaagcgctgaagaactctgatcccttcactggggtggaccagagatacggatactttaactttgcctggccatagcaaagtaaagaaaaccttgtaaaacccattctggtaatccaccaccctgcccacagccccagcctgcagcttgagggagtgaattctggcctgcaggtagtctccaccatacttcttgggctttctttgaaaatcctgcacatgaaccagcacctcaagctggcttcccaccttaaagaaggcagcagagttcaagatgacaaagtagctggaagaagggtcagtgctcttcacaaaggggactgggcccacatcaggaacctgccggtgcaaggcagccagcaaggagtcctcctccatgcgctcctggctggacagggtctgctgatcatagccacagtagggatttcggctaattcctgtcacctgggaggaaacaaactgtccactgctgtcgatgaaagtggctgaaacagtctcatggtccaagtactctacctgagtaacattgatgaccagcaccaccaccatcaacactgcaagcagacagcagaaaagccgtagtttgaagaaattggtccacattgtctggctgtgtcttgttcacccatggccgacaccatgctaccttcactctttaaaattccatgtctttgcttttctgagctgcagatgagctttcagtttcatttgcttctatcctgctagtacccttaagagctcttatgcagaggagagactgcagttgattcaagaagcacatttttcttcaaagaaatcctatagtcccagttactcaggaggctgaggtaggagaattgcttgagcctgggaggtcgaggctgcagtgaaccatgatcatcacaccaatgtactccagcctgggcaacagagcaggactcttttttggaaattttccaagaagagatgcttactggaactagaaattagaagttacgtctaactttccttccagcatgaaattctgaactcaggcaattttgaccagaggtcctcatttttttcatgccacatgtgaagcacacataaatgttttttacatttctatacaattcttcttgctgaatctgatgtccccaaacggcagctcagtaaggccagaacagtccaccgtgtgacagcagcgccagccaagaggcagctggtgcccagagcagcgatgagccgagagatatgagatgggcagggaggcgtcgccaagtgctccgcaccgggttagtgaaggtgcctggaggacagaagtctttcgctgcggcgtggaggtccgaactgtaccgagctgtggcgttgccgcaagt

SEQ ID NO: 14934 - RNA, 7073 nt, Homo sapiens
  source 1..7073: mol_type = other RNA
gctgggattacaggcatgagccactatgcccggcccacatttttttaaaaagttaaaatgtaaaagcacttttaagagacaagttagacagaaggtggtggagtacattttctgctctcctagcttctgtgtcctttaaactcctgccctcaaccatcctcttatcgtccaccacctccattcccctaggattcccaggtccccttagcactcaggggctgtggtctcaccttcaaatgaaaaacaacaacttcaaaattttatttattgcacactgaggtgtcaagaatcctaagtacactaatactacattgtagacataaaccaggtagaataatgcttaacacaagaaaataaatacacttgaagtggaatttctggcattagtgactagctgatgttaaaaagctgaatttacccagaatccacagagataatgctgagcagttttttagaaagttggggaggcttatttctgttgtttcccttgggtgtttatttccctgtacctctctcagtcatcactatttccttgaacagggtccagaaacagactcatttctggcatgtaacacatgaatatataaaggcgtaccatatttattcttgtcaagtaccctgatttaccaatctgcaaactaagttttcagattgataaatgtgaaactggattcagttattaaactggatcaagtttcaatctgaaacttaataactgaatccaggaagtgtcagttaaatggtcttaattaaaatgatagttgttcagaatggcaaaatgaatcatactggaacaccaaaggtctgttttgcattcgctgaagaaaggttacttttagtaggataattctataaaatgtaacttgcatagaaaggctttattatgggttctgtctgtcacaaatagcatcaaatcaatcatctcagttctggaatatgagattcactacattaaattaatactttcattccaaaatagaaattcatattttaaaccactgaaattgatataaaccactgctttaatattgtaaacctaaatgtccaactataatgaccaacttatctaataatgaaaactgcagtagcagaactattaagcagatctttataattaacttatgaagactatttaacatagaaaaatatttatatgtaaaaaacacagacccaaattacatattctctataagtatatggttaaaaaacctgcaagaaaatatacctaaatgctaatgttcattgcattcagatgatagaattatggattttatccatagatttttcttctagattttatagtttttaaaaattatgatgccccttatatttatattgggaaatatacatttaaacaaactattatttggctaccatgctaatattcacaaccatgtggcactagcctaaaataaacttttcagaagaaactaaattattctatctaaatattctgggaaacgtttaagtgatattggaatctctatcaaaatttccacaccagagtgaagaaagacaaattagatgtgggatgaaagttgttctcactgataagtgagagctaaatgatgagaacacatggacacataaagggcaacaacacacactggggtctattggagggtggagggtaggaggagggagaggatcaggaaaaattactaatgggtactaggcttaacacctgggtgatgaaatcatctatacaacaaacccccatgacgtaagtttacctatgaaacaaactggcacatgtacccctgaacttaaaagttgttaaaaaaaaaatttttttaagagagatgaaagtgactcaagaagctgtgtcaccaaatctttgagagctatgtcaccaaatcaaaaaataacagaaaaccagacaagatcataagaaatcatttgcacaatcaagtggcatcattccaaaccactggaggagcaatgcccgctttctttttaaaattctcctgggaaaattactcctcagcctcctttataaatccttgaggaaatgtcaagttctttcacgacaagaaaaactctcagctgggcacagtggctcacacctgtaatcccagcactttgggaagctgaggtgggcagatgcttgagctcaggagtttaagaccagcctggacaacatggcaaaatgtagtctctacaaaaagatacaaaaattagctgggcatggtggtacatacctgtagtcccagctactcaggaggctgaggcagaaggatcccttgagcccaggaagtcaaggctgcagtgagccatatcatgccactgcactccagcctgggcaaaagagcaagaccctgtctcaaaaacaaataaataaatacaaacgcttctttacgaaagtctcacaagtttagctgaaaagagatatggactctcacataccttatttcagatctaaacatgagttcctcatctataaaatggagctaatatcaccaatactattggatcatgaacagaattaaaccagttattggtaaatcccccaaaataataaacaagccatgtttattccctcattctatcttacctcttctcttagtgtttctcacagtgtggaataccaccattgcatcagaatcactgagcactcgccacaaaggttggtttcataaatcccagaggcatcatggtccctcttttttttttttttttttttttagagacagggtcttgccctgttgcccagactggagtacagtggcacaatcaaggctcactgcaacctctgcaaccttctgcctcctgggctcaagcaatcctcccacctcagcctcctaagtagcggggactacaggtggtgccaccacacccagctagtttttgtatttttttgtagagatggggtttcaccatggcacccaggctggtcttgaccttccgggctcaagcaatccgcccacctcagcctcccgagactataatccctgctgggattacagatgtgagccaacatccctggccttaattcttttattatttaacaaaaattttttagagataagatctcttgtctgttgcccaagtgggagtgtagtggcgcaatcataactcactgcagcctcaaactactgggctcaatcaatcaccctgccttagcctccctagtagctgggactgtcggcccacacctggataattttttattttttgtagagatgaggtcttactatgttgcccaggctggtctcaaactcctggcctcaagcaatcctcctgcctggcctcccaaagtgctgggattacaggcttgagctaccacaccctgccatgactctttaattctgcatttttgtcagatactacaagtgatccttaggtactgtaaagcgtaaggaccattaaaattaaactattttaatatattttattacctcattaggctcagaaacaattaaaaatcttctttccccctaaaatactttaaaaacttgaaggtgttcctcaaggacaggaaagtaagatctggggccctcctattttaaattaaaaacccaaattatttgacccattcttctaagggtatatattgttcatacttcaagcatctgtcttcctctctaaagcctccctagtttcttcatctgtctacttaggagcaacttaaactagactataatctatcacagctcaaaaagaaaagagtacttactaaatgatcccaaattaaactcgtttaaaattaataagtcaaataaaattaataattccattcttcttagatagccagtaggaatagcagcttcttccaagcatgagagaatgggtgtgccttttatgcccaaatcaagaaataccaaaaaacaaacaaacaaacaaacaaaaaactgtcatgaattttagtatcttattaatttctaattagattttaacttctaattttggtaagtagttcaaaataacaacaacaacaacaaaaaaaaaaacacctgaaactagtggaaaaaacttccacagctttataatatcgtagcattctttacacaaaagtcaattcctaaaccctcaaatttcagaacataaaaataaatttccatttacagatttcccccttccagttccaaaagtagttattctagagtaagtattcaacacataaaatttagctgaatcaaataaaaaacaatcaccaaatgcaaatatcaattccaaagcacagattttatatatactgctttcatatttcccttttgcttcttttctagataaaagcaggaaattgtaaatattcactaaaaaactcgaaccaagcacattggccttttcaagtaattcagaaaaggtagatcatcaagagaaactcctgagacacagcagtcttcagtgcattcacaagagcctctgactataagctttctctagttaaccgccagaagatggattacttgtgctatgcatgcagatgcactcaatttcctttaccagataagctacaaacactctactaccaaccaaacttgtcccttccatcaaaacatttttcatactctttagcaaagtagtcacccctcctaggagaagctaattcaaatacactcattagcatctttggttacaagagcaatatagtgtgtagatgcagttaagagttctaccatggctaagtcaacattggataaaatcctataggtagatataaatgtaacctgcattttctaagctccttataagtcatcatattaagtccagatctttttgaaattttatacttattaagggcagtcatctctcactggggccactttctgtaactcaggtcaattgagaaggtcattgaatatgattcctccagtcccttccaagacaggctaggtttccaaggggcacacaaaggacaagaacatgtccagctggttcttcacaataacttcatctggatgcagcttgtgcggtagataatgggccagggtcatctcccaggcatcgacgagatatactccaacccctgagaacatcctccgaaggatggtgtccagctgaaagttgtaccagtcgctgttgaaaaggctcacctcaggtcccagctcttgggcgttggccgtccggatgaccaccacggtctttgggcttcgatcgaggagccgaaccactgctcgacggatgttcctgagccgccggatgtacacttccaaagggaaggtgctgaagtgagaccatacagctatggcaaccactgtgttcttccctcccacaatgccattcagctcattcgccacataatggagctcattgctaaagacagtcgtgaagcggatgggtggaccatggcagcggtatttgagcaggatgttgtgcttctggtccactgcaaggaagggacccacattcttgggactacccaagttaaactccactaaatcttttattctcctgggaatcacagttacccaatcaggtccactggagttgactggcattttgatattgacaccactctggaagaaagcactctctgcagcggttaggagacctttcaggtatccacctttgaaatgggtaattctgctgctgcaagggagcttctttggtttgaagcagaaccagggctccccagtgtagaggtctgtaaagttacacaggggcagattcccaggaagacacacgttgcactcagtagtttcagaaattcttcctgaacggaagagactcttgaaatagaccctgtctggtttatcttcctgtaagcgctgaagaactctgatcccttcactggggtggaccagagatacggatactttaactttgcctggccatagcaaagtaaagaaaaccttgtaaaacccattctggtaatccaccaccctgcccacagccccagcctgcagcttgagggagtgaattctggcctgcaggtagtctccaccatacttcttgggctttctttgaaaatcctgcacatgaaccagcacctcaagctggcttcccaccttaaagaaggcagcagagttcaagatgacaaagtagctggaagaagggtcagtgctcttcacaaaggggactgggcccacatcaggaacctgccggtgcaaggcagccagcaaggagtcctcctccatgcgctcctggctggacagggtctgctgatcatagccacagtagggatttcggctaattcctgtcacctgggaggaaacaaactgtccactgctgtcgatgaaagtggctgaaacagtctcatggtccaagtactctacctgagtaacattgatgaccagcaccaccaccatcaacactgcaagcagacagcagaaaagccgtagtttgaagaaattggtccacattgtctggctgtgtcttgttcacccatggccgacaccatgctaccttcactctttaaaattccatgtctttgcttttctgagctgcagatgagctttcagtttcatttgcttctatcctgctagtacccttaagagctcttatgcagaggagagactgcagttgattcaagaagcacatttttcttcaaagaaatcctatagtcccagttactcaggaggctgaggtaggagaattgcttgagcctgggaggtcgaggctgcagtgaaccatgatcatcacaccaatgtactccagcctgggcaacagagcaggactcttttttggaaattttccaagaagagatgcttactggaactagaaattagaagttacgtctaactttccttccagcatgaaattctgaactcaggcaattttgaccagaggtcctcatttttttcatgccacatgtgaagcacacataaatgttttttacatttctatacaattcttcttgcttgtaaagttacactcgtttctccccatacgacctgaatctgatgtccccaaacggcagctcagtaaggccagaacagtccaccgtgtgacagcagcgccagccaagaggcagctggtgcccagagcagcgatgagccgagagatatgagatgggcagggaggcgtcgccaagtgctccgcaccgggttagtgaaggtgcctggaggacagaagtctttcgctgcggcgtggaggtccgaactgtaccgagctgtggcgttgccgcaagt

SEQ ID NO: 14935 - RNA, 6482 nt, Homo sapiens
  source 1..6482: mol_type = other RNA
gctgggattacaggcatgagccactatgcccggcctatgcttattttaaaatgtcaattgtcactcacaaaatgaaatgctagtttggttaaaaaaaaaaaagtcttatatacagacagacatgactgttttgctaatgaagagaaccccccacaagtgatacattccaatatccatatactgtgtaatatataatgtgattctcttataatggtccccacagactagtttcttcccaaacctatatgtcactatgtatttggtatttatttattaaagtatgatatgagatttcttgatttacgttttccactaaaactaccacaatgaattttgggaaaaggggttgaccatcatataactcccggtgaccccaacaagttaaaactatcttgtagaagccatgtgctatttcatgtcaaaatacaggaaaagatactgcattctgccaaatgctcagtccagaaagtagaagaccatgattgacttcagattttttttttttttgcctcagtaaacagtacagaaaatgatctgagaatgaaattattttttaaaagcccaaaggagaaaaagaataacaagatatcatagtctagcatttacaggccaaggtcaaaaacctgggtgcaatggatcccatcagcatgtaattacatagattttatatcccttctgcagttaaaatatttcatcttatcttaaaacacattgctgtggtctggagaccagcagtctctcccccacatctctcttcattcttgcttgtttcagtttcttatcttattcctctctgccctttctgtaaagaaagcaaagttatcttctcatgactacgtgattaaggggtatatataaggatgaattatacataaagatccatgtaaataatttatgttaaaatatttaagttaaacaatttcgatagaaaaagttcatttctatggaaagacagaattgcaaatcaacagtgtttttacatatatacatacatgtataaattcacagaaagggttttttaagttgacctagtggtctttatgtatcatagtcattttctaaagctgagaatctatagtagataatagtatgcaaataacaagaagtttgattctaataaaattggtaagaatgaagaagcaacatgatccactacagatgtcaatacagtctgaagaataggaactggttggccacagttcatatactaatacattcttggagaatacaaaatttaagaatgaaaacattaagacattcttgacttttgagttaattttagcttataaatatcatgtgcttaatcttagacccactaacacaaatatcatatgatataggaaatcttcattaatctattctgcattatagcaaagatacctataaaacccaagacgcttgttccctagaagtttacttgctccggttggtgcttgctactcaggttgtatctagtccagaaagatcatcagaaatttatcacagacaatatgctcagattaagaacttaaggctttgaatataaccagaaaacaaataaaagcaaccaccctgtttccaaaaagtaaggacaaggaaaagtaaaacagaattgtgaactcaaaagtatttttgacaaaagtttttagaaggcatcaaagaatctttaacaaccctgcagtaccacaaactttatcgttttctttatatatttataactagaacaagtgttcttaaaaaaaaaaaatccaaacgtgtgcgtatatatatatggggaaagggtacatttaaaaggttagtttctgtaaaaagtttaataatttttaaaaaaattggggtaagttaagtcacctagtgaagataagtacacaaacctgatgtcaaattaaacttcagggaaaacaaaatgtgctttttctatccattttctttgttaaagtaaaaatgttcttgatagttatttaaaatccaaggaatgatgccccttcccatttcccttccttatactctgcaattcgaattaccgtatcacatctagaaagttaataattatctatattcttgtgggaaggggccttcatattaaattttcagtataaaaccataccctaaagagttttattgcttgcatacatgatgacactgtgatgccattattacaaaagtggctggtgttttttattgagccccacttaaaaccaagataaaagtctgcactatatttcatacttaacacgccaaatggtaggctttcagcaaaagcaaaatttaagcttaaaatattgaaatgttttataatgaatagaaattttgtcaaggaagtactttttaaagtttggaggaagggcactttaaagaaaagatgacttggaaagcaccaaatgagtgaaaataaagaattaagacccacagggaacgttggttttaatgggaaagcaaccaatgatatttttaggttgtcatgactgctcaagtatgttggaagggaaaaggcattgattattcttatcatcaatcacactttgaggtctcttggttgaattgtttaataaatggctaagggtattactttacctttcattgagtaaaaacatcagtgattctttaataagagagaagcgggtaaggctgtttcactgcttctctttgcgtttagctgaagaatgtggggtggaaagtgaatatggtgaccggataaccagaaattctcttctagtattaatgcttctcatttaaaaaattaaagataatgactgttaagagcatgataataaacattatctttacatgagtattctttcaatgatctaagttaaataacattgatatttattgagccaaaacttaagtgtgtccatgttacttctgttttggtagggaaagtgtagtcttcttgcttttaaaaatagttttcaaaaataatctgacttataaatcttcccattggcccatacattaccattgttctagtcacacttacaaaagtcctcttccccagttaatcattctgtatttccattgcttctcttttcttgagattaagaaaaccaaagcatcatctatagctacagtttaattttccaaaaaaccactctgagtatacatcacacacataccccgctggccattaaaaaagagaagcaatgtaaattttcttctagtctttccctgatttaatagggcctaagaagctacttttatctctttttggctccatctatttggtttaatgttaatgatcatggctgataatccttttatggaggaagggaacctattatgtcagcaataattggttcacttgctcctttggggtggaaaaaataagatatttcttaaagtaacaaggcctgaataaatgtgtggcagtctcaaattctattctatatctaaggtgtaatccttacatactaaagatagtgggatcattcttgtagatttctagcagactggtacattaaaaagtgacaatgtttggggtatgacagtataaaaaaaggtttaatttgagaaaaaggattaagttaaatagtaaacttagtgtgagattttaatcacaagtacaaaagagtgaagagcagccttcatgacaaggaatcatgtgaccagcccccaccccaaacataggttatcacatgtggattttgtttcattccgacaaaggaaaaggcccatacagttatcttaagtgttcattatatagagaccttatttaaccatgctcgattatcttacggaaaagaaaaacattacgataaatgtggtttccacatatcctagttctgtaaaaggtcaggtgtctcataaagtttgggttttggtgaaaatgtttgtacatgctgatgttaactactgcaataattataggattgtaaacggtaaaataacctgtatgactttgactgtcccagtgaccaaaatgcactttaatcttagaataatcaagactgaagcattaactgaaccctcatcttatattaatagcaccttctaagagaggcactgttttaaataggcacagaaacaaaaaatggtactttaaaagtactgttggaattcacaaatatatcccatgccacataaattaccgcttattataaaaatatcaataccctcaaatgccaatcagcaaaacataaatcaccaaaacatttcttcagtttagaacattgctcaattccacgataaaccatgctttatatttaaaaaataaattagagatgaatgtgaacctaaaagcatgtataatatatatatttaatactatatatacataattgctatatacttaagacattcttaggagtatttctacaaaaacaagttatcttttctttataaatcggaaatctgaacaccaacaatttgtcctttttcttttgttttaaaagaacagacatcatttatgcagctagagatttataaactaaattaaataagttaatacaatagcctcaactgtccctgtatttttcaccatggatctattttggcaacatggaggtatatctttcaaactgttccaggtcctacatgtgaaagagaagaagacatgaaaggatttcttaaatggaagtgctcattctaacctgacggtgacagaatcaattgatacaccatttcttcaagacaaaaaagcacatattcaaggaatagctcaaaaaatgctccagttttcacattatttcaaaactttatcggtagaatgactctgcacactaatttcactaagagtacataaacataggaaaatagtcctcaaaagatgcatttatgggcctatatttttcaacataaagtgctagcagatgtgtaagaagagctgggaatgtcttgagctgtaagtcctgagacctccacaccatggctggtcctggaggagttcagcattctgattttttcttaggttcaggatgatcatccaaggtggctggatgctcatttggaccacctggtgtctcacctgtgacagctaaaaggatgactttcagccacttctgcttcagttcctcactgtctgcagcaaagctgtgcacggacttagactgggtcagtttgaaactgtgtggcaggtctgcgctccttggcatttcatccaccacatagcccagaagtggaatggtggcctgggctctgacgtcctggggggcaccatacatgtacagcacaagagggtcttgcttggggatcacacaccaagctttctgccaaggttttgacttctccatatactgaagaaagctgcacaccacactgtttccagatacttctgctgattcaatctctaaaattccttttcttttcttttcttcactgtctgtgaatccacttatgatttgataacagtctttacaaactttgctcaatttaccaccatcatattcaagttgagctttgtagtcggagcatttccaacaaaccacatatccacatgctcgacaatgatgcctccttcgtgtcagtgcattgaaaggttctttacatttcatacacattgtcacttcattatctcggatccatcttggggctcttttccctagctcagcagtagaaacctctgagtgaatgtcattatcctttgcaattgcatttctgaaggtttcatgcctttgatgaaaagcatcgatggtttcttgaagggccttgatccattcttctttgtcttgcgcagaactggcctgcagttccagtgttctctctttcccagacacctggaaagtatgtggatattcttcattttgagtctctacaattttcattccatcaatgccaaccctggttcgaactgtgaatttagagcctaccaagctgaatttgggcacacagtacagcaacatgttgttgaataagaaaaggtagcgttcttgtgctgaagtgttccgagcagctagtttgaggatctgtccttcttttattagttcatttgaagggtttacaatgtcttcttcttctcccaacatttcataaatctctaagagtttctttaggttctccattttccttattgcactattagaatggcttgctgctgtagatataatttcaagtgattttttagcatcattccagtccagggaatcaggaggcaatttccttagatagtccttaaggagcatctcataccggggaatccgctgaacaggttctagcatgtgatgctgcaaagttaagctcccacagattttctgtttctgaatttcttcaaccactgatttgaactggggaatacgttctgtcatgtttttaaccaattccattgcattatcaaatcctttcacatattctccatacatcttaaggaatggtgccaatttctgaaggatgtctccaattctaggagtagtttcccatctctgctggaaacgagcctcggtttgcttcttccaacagtttgcaataaaatacctcttaattgccattctgttacatgtaggcagaaggaggtctattccttcataatgtccagatggttgttaattttctaaattcacctccactctatt

SEQ ID NO: 14936 - RNA, 6725 nt, Homo sapiens
  source 1..6725: mol_type = other RNA
gctgggattacaggcatgagccactatgcccggcctatgcttattttaaaatgtcaattgtcactcacaaaatgaaatgctagtttggttaaaaaaaaaaaagtcttatatacagacagacatgactgttttgctaatgaagagaaccccccacaagtgatacattccaatatccatatactgtgtaatatataatgtgattctcttataatggtccccacagactagtttcttcccaaacctatatgtcactatgtatttggtatttatttattaaagtatgatatgagatttcttgatttacgttttccactaaaactaccacaatgaattttgggaaaaggggttgaccatcatataactcccggtgaccccaacaagttaaaactatcttgtagaagccatgtgctatttcatgtcaaaatacaggaaaagatactgcattctgccaaatgctcagtccagaaagtagaagaccatgattgacttcagattttttttttttttgcctcagtaaacagtacagaaaatgatctgagaatgaaattattttttaaaagcccaaaggagaaaaagaataacaagatatcatagtctagcatttacaggccaaggtcaaaaacctgggtgcaatggatcccatcagcatgtaattacatagattttatatcccttctgcagttaaaatatttcatcttatcttaaaacacattgctgtggtctggagaccagcagtctctcccccacatctctcttcattcttgcttgtttcagtttcttatcttattcctctctgccctttctgtaaagaaagcaaagttatcttctcatgactacgtgattaaggggtatatataaggatgaattatacataaagatccatgtaaataatttatgttaaaatatttaagttaaacaatttcgatagaaaaagttcatttctatggaaagacagaattgcaaatcaacagtgtttttacatatatacatacatgtataaattcacagaaagggttttttaagttgacctagtggtctttatgtatcatagtcattttctaaagctgagaatctatagtagataatagtatgcaaataacaagaagtttgattctaataaaattggtaagaatgaagaagcaacatgatccactacagatgtcaatacagtctgaagaataggaactggttggccacagttcatatactaatacattcttggagaatacaaaatttaagaatgaaaacattaagacattcttgacttttgagttaattttagcttataaatatcatgtgcttaatcttagacccactaacacaaatatcatatgatataggaaatcttcattaatctattctgcattatagcaaagatacctataaaacccaagacgcttgttccctagaagtttacttgctccggttggtgcttgctactcaggttgtatctagtccagaaagatcatcagaaatttatcacagacaatatgctcagattaagaacttaaggctttgaatataaccagaaaacaaataaaagcaaccaccctgtttccaaaaagtaaggacaaggaaaagtaaaacagaattgtgaactcaaaagtatttttgacaaaagtttttagaaggcatcaaagaatctttaacaaccctgcagtaccacaaactttatcgttttctttatatatttataactagaacaagtgttcttaaaaaaaaaaaatccaaacgtgtgcgtatatatatatggggaaagggtacatttaaaaggttagtttctgtaaaaagtttaataatttttaaaaaaattggggtaagttaagtcacctagtgaagataagtacacaaacctgatgtcaaattaaacttcagggaaaacaaaatgtgctttttctatccattttctttgttaaagtaaaaatgttcttgatagttatttaaaatccaaggaatgatgccccttcccatttcccttccttatactctgcaattcgaattaccgtatcacatctagaaagttaataattatctatattcttgtgggaaggggccttcatattaaattttcagtataaaaccataccctaaagagttttattgcttgcatacatgatgacactgtgatgccattattacaaaagtggctggtgttttttattgagccccacttaaaaccaagataaaagtctgcactatatttcatacttaacacgccaaatggtaggctttcagcaaaagcaaaatttaagcttaaaatattgaaatgttttataatgaatagaaattttgtcaaggaagtactttttaaagtttggaggaagggcactttaaagaaaagatgacttggaaagcaccaaatgagtgaaaataaagaattaagacccacagggaacgttggttttaatgggaaagcaaccaatgatatttttaggttgtcatgactgctcaagtatgttggaagggaaaaggcattgattattcttatcatcaatcacactttgaggtctcttggttgaattgtttaataaatggctaagggtattactttacctttcattgagtaaaaacatcagtgattctttaataagagagaagcgggtaaggctgtttcactgcttctctttgcgtttagctgaagaatgtggggtggaaagtgaatatggtgaccggataaccagaaattctcttctagtattaatgcttctcatttaaaaaattaaagataatgactgttaagagcatgataataaacattatctttacatgagtattctttcaatgatctaagttaaataacattgatatttattgagccaaaacttaagtgtgtccatgttacttctgttttggtagggaaagtgtagtcttcttgcttttaaaaatagttttcaaaaataatctgacttataaatcttcccattggcccatacattaccattgttctagtcacacttacaaaagtcctcttccccagttaatcattctgtatttccattgcttctcttttcttgagattaagaaaaccaaagcatcatctatagctacagtttaattttccaaaaaaccactctgagtatacatcacacacataccccgctggccattaaaaaagagaagcaatgtaaattttcttctagtctttccctgatttaatagggcctaagaagctacttttatctctttttggctccatctatttggtttaatgttaatgatcatggctgataatccttttatggaggaagggaacctattatgtcagcaataattggttcacttgctcctttggggtggaaaaaataagatatttcttaaagtaacaaggcctgaataaatgtgtggcagtctcaaattctattctatatctaaggtgtaatccttacatactaaagatagtgggatcattcttgtagatttctagcagactggtacattaaaaagtgacaatgtttggggtatgacagtataaaaaaaggtttaatttgagaaaaaggattaagttaaatagtaaacttagtgtgagattttaatcacaagtacaaaagagtgaagagcagccttcatgacaaggaatcatgtgaccagcccccaccccaaacataggttatcacatgtggattttgtttcattccgacaaaggaaaaggcccatacagttatcttaagtgttcattatatagagaccttatttaaccatgctcgattatcttacggaaaagaaaaacattacgataaatgtggtttccacatatcctagttctgtaaaaggtcaggtgtctcataaagtttgggttttggtgaaaatgtttgtacatgctgatgttaactactgcaataattataggattgtaaacggtaaaataacctgtatgactttgactgtcccagtgaccaaaatgcactttaatcttagaataatcaagactgaagcattaactgaaccctcatcttatattaatagcaccttctaagagaggcactgttttaaataggcacagaaacaaaaaatggtactttaaaagtactgttggaattcacaaatatatcccatgccacataaattaccgcttattataaaaatatcaataccctcaaatgccaatcagcaaaacataaatcaccaaaacatttcttcagtttagaacattgctcaattccacgataaaccatgctttatatttaaaaaataaattagagatgaatgtgaacctaaaagcatgtataatatatatatttaatactatatatacataattgctatatacttaagacattcttaggagtatttctacaaaaacaagttatcttttctttataaatcggaaatctgaacaccaacaatttgtcctttttcttttgttttaaaagaacagacatcatttatgcagctagagatttataaactaaattaaataagttaatacaatagcctcaactgtccctgtatttttcaccatggatctattttggcaacatggaggtatatctttcaaactgttccaggtcctacatgtgaaagagaagaagacatgaaaggatttcttaaatggaagtgctcattctaacctgacggtgacagaatcaattgatacaccatttcttcaagacaaaaaagcacatattcaaggaatagctcaaaaaatgctccagttttcacattatttcaaaactttatcggtagaatgactctgcacactaatttcactaagagtacataaacataggaaaatagtcctcaaaagatgcatttatgggcctatatttttcaacataaagtgctagcagatgtgtaagaagagctgggaatgtcttgagctgtaagtcctgagacctccacaccatggctggtcctggaggagttcagcattctgattttttcttaggttcaggatgatcatccaaggtggctggatgctcatttggaccacctggtgtctcacctgtgacagctaaaaggatgactttcagccacttctgcttcagttcctcactgtctgcagcaaagctgtgcacggacttagactgggtcagtttgaaactgtgtggcaggtctgcgctccttggcatttcatccaccacatagcccagaagtggaatggtggcctgggctctgacgtcctggggggcaccatacatgtacagcacaagagggtcttgcttggggatcacacaccaagctttctgccaaggttttgacttctccatatactgaagaaagctgcacaccacactgtttccagatacttctgctgattcaatctctaaaattccttttcttttcttttcttcactgtctgtgaatccacttatgatttgataacagtctttacaaactttgctcaatttaccaccatcatattcaagttgagctttgtagtcggagcatttccaacaaaccacatatccacatgctcgacaatgatgcctccttcgtgtcagtgcattgaaaggttctttacatttcatacacattgtcacttcattatctcggatccatcttggggctcttttccctagctcagcagtagaaacctctgagtgaatgtcattatcctttgcaattgcatttctgaaggtttcatgcctttgatgaaaagcatcgatggtttcttgaagggccttgatccattcttctttgtcttgcgcagaactggcctgcagttccagtgttctctctttcccagacacctggaaagtatgtggatattcttcattttgagtctctacaattttcattccatcaatgccaaccctggttcgaactgtgaatttagagcctaccaagctgaatttgggcacacagtacagcaacatgttgttgaataagaaaaggtagcgttcttgtgctgaagtgttccgagcagctagtttgaggatctgtccttcttttattagttcatttgaagggtttacaatgtcttcttcttctcccaacatttcataaatctctaagagtttctttaggttctccattttccttattgcactattagaatggcttgctgctgtagatataatttcaagtgattttttagcatcattccagtccagggaatcaggaggcaatttccttagatagtccttaaggagcatctcataccggggaatccgctgaacaggttctagcatgtgatgctgcaaagttaagctcccacagattttctgtttctgaatttcttcaaccactgatttgaactggggaatacgttctgtcatgtttttaaccaattccattgcattatcaaatcctttcacatattctccatacatcttaaggaatggtgccaatttctgaaggatgtctccaattctaggagtagtttcccatctctgctggaaacgagcctcggtttgcttcttccaacagtttgcaataaaatacctgatctaagaggtcaagtcggttgacataagctctttcagtaagcaaaagttcattggctattttgtgaagtttttgctcattagtctccttgtggctttggacttgcagctgagtgttttgctggcctgttcccatttattccctgagcctcttcttcagatacattctcaccaaccagtgtggttgtgctgcttgtggagcaaggtggaactaaagcgatctttggacaggtactgctgcctgtggctcctgagggcacctggcccttgaaggcagcggtccctacacgtcccaggtgcgacgcgggcctgctccagggccggggcaccccgggcggc

SEQ ID NO: 14937 - RNA, 7020 nt, Homo sapiens
  source 1..7020: mol_type = other RNA
gctgggattacaggcatgagccactatgcccggcctatgcttattttaaaatgtcaattgtcactcacaaaatgaaatgctagtttggttaaaaaaaaaaaagtcttatatacagacagacatgactgttttgctaatgaagagaaccccccacaagtgatacattccaatatccatatactgtgtaatatataatgtgattctcttataatggtccccacagactagtttcttcccaaacctatatgtcactatgtatttggtatttatttattaaagtatgatatgagatttcttgatttacgttttccactaaaactaccacaatgaattttgggaaaaggggttgaccatcatataactcccggtgaccccaacaagttaaaactatcttgtagaagccatgtgctatttcatgtcaaaatacaggaaaagatactgcattctgccaaatgctcagtccagaaagtagaagaccatgattgacttcagattttttttttttttgcctcagtaaacagtacagaaaatgatctgagaatgaaattattttttaaaagcccaaaggagaaaaagaataacaagatatcatagtctagcatttacaggccaaggtcaaaaacctgggtgcaatggatcccatcagcatgtaattacatagattttatatcccttctgcagttaaaatatttcatcttatcttaaaacacattgctgtggtctggagaccagcagtctctcccccacatctctcttcattcttgcttgtttcagtttcttatcttattcctctctgccctttctgtaaagaaagcaaagttatcttctcatgactacgtgattaaggggtatatataaggatgaattatacataaagatccatgtaaataatttatgttaaaatatttaagttaaacaatttcgatagaaaaagttcatttctatggaaagacagaattgcaaatcaacagtgtttttacatatatacatacatgtataaattcacagaaagggttttttaagttgacctagtggtctttatgtatcatagtcattttctaaagctgagaatctatagtagataatagtatgcaaataacaagaagtttgattctaataaaattggtaagaatgaagaagcaacatgatccactacagatgtcaatacagtctgaagaataggaactggttggccacagttcatatactaatacattcttggagaatacaaaatttaagaatgaaaacattaagacattcttgacttttgagttaattttagcttataaatatcatgtgcttaatcttagacccactaacacaaatatcatatgatataggaaatcttcattaatctattctgcattatagcaaagatacctataaaacccaagacgcttgttccctagaagtttacttgctccggttggtgcttgctactcaggttgtatctagtccagaaagatcatcagaaatttatcacagacaatatgctcagattaagaacttaaggctttgaatataaccagaaaacaaataaaagcaaccaccctgtttccaaaaagtaaggacaaggaaaagtaaaacagaattgtgaactcaaaagtatttttgacaaaagtttttagaaggcatcaaagaatctttaacaaccctgcagtaccacaaactttatcgttttctttatatatttataactagaacaagtgttcttaaaaaaaaaaaatccaaacgtgtgcgtatatatatatggggaaagggtacatttaaaaggttagtttctgtaaaaagtttaataatttttaaaaaaattggggtaagttaagtcacctagtgaagataagtacacaaacctgatgtcaaattaaacttcagggaaaacaaaatgtgctttttctatccattttctttgttaaagtaaaaatgttcttgatagttatttaaaatccaaggaatgatgccccttcccatttcccttccttatactctgcaattcgaattaccgtatcacatctagaaagttaataattatctatattcttgtgggaaggggccttcatattaaattttcagtataaaaccataccctaaagagttttattgcttgcatacatgatgacactgtgatgccattattacaaaagtggctggtgttttttattgagccccacttaaaaccaagataaaagtctgcactatatttcatacttaacacgccaaatggtaggctttcagcaaaagcaaaatttaagcttaaaatattgaaatgttttataatgaatagaaattttgtcaaggaagtactttttaaagtttggaggaagggcactttaaagaaaagatgacttggaaagcaccaaatgagtgaaaataaagaattaagacccacagggaacgttggttttaatgggaaagcaaccaatgatatttttaggttgtcatgactgctcaagtatgttggaagggaaaaggcattgattattcttatcatcaatcacactttgaggtctcttggttgaattgtttaataaatggctaagggtattactttacctttcattgagtaaaaacatcagtgattctttaataagagagaagcgggtaaggctgtttcactgcttctctttgcgtttagctgaagaatgtggggtggaaagtgaatatggtgaccggataaccagaaattctcttctagtattaatgcttctcatttaaaaaattaaagataatgactgttaagagcatgataataaacattatctttacatgagtattctttcaatgatctaagttaaataacattgatatttattgagccaaaacttaagtgtgtccatgttacttctgttttggtagggaaagtgtagtcttcttgcttttaaaaatagttttcaaaaataatctgacttataaatcttcccattggcccatacattaccattgttctagtcacacttacaaaagtcctcttccccagttaatcattctgtatttccattgcttctcttttcttgagattaagaaaaccaaagcatcatctatagctacagtttaattttccaaaaaaccactctgagtatacatcacacacataccccgctggccattaaaaaagagaagcaatgtaaattttcttctagtctttccctgatttaatagggcctaagaagctacttttatctctttttggctccatctatttggtttaatgttaatgatcatggctgataatccttttatggaggaagggaacctattatgtcagcaataattggttcacttgctcctttggggtggaaaaaataagatatttcttaaagtaacaaggcctgaataaatgtgtggcagtctcaaattctattctatatctaaggtgtaatccttacatactaaagatagtgggatcattcttgtagatttctagcagactggtacattaaaaagtgacaatgtttggggtatgacagtataaaaaaaggtttaatttgagaaaaaggattaagttaaatagtaaacttagtgtgagattttaatcacaagtacaaaagagtgaagagcagccttcatgacaaggaatcatgtgaccagcccccaccccaaacataggttatcacatgtggattttgtttcattccgacaaaggaaaaggcccatacagttatcttaagtgttcattatatagagaccttatttaaccatgctcgattatcttacggaaaagaaaaacattacgataaatgtggtttccacatatcctagttctgtaaaaggtcaggtgtctcataaagtttgggttttggtgaaaatgtttgtacatgctgatgttaactactgcaataattataggattgtaaacggtaaaataacctgtatgactttgactgtcccagtgaccaaaatgcactttaatcttagaataatcaagactgaagcattaactgaaccctcatcttatattaatagcaccttctaagagaggcactgttttaaataggcacagaaacaaaaaatggtactttaaaagtactgttggaattcacaaatatatcccatgccacataaattaccgcttattataaaaatatcaataccctcaaatgccaatcagcaaaacataaatcaccaaaacatttcttcagtttagaacattgctcaattccacgataaaccatgctttatatttaaaaaataaattagagatgaatgtgaacctaaaagcatgtataatatatatatttaatactatatatacataattgctatatacttaagacattcttaggagtatttctacaaaaacaagttatcttttctttataaatcggaaatctgaacaccaacaatttgtcctttttcttttgttttaaaagaacagacatcatttatgcagctagagatttataaactaaattaaataagttaatacaatagcctcaactgtccctgtatttttcaccatggatctattttggcaacatggaggtatatctttcaaactgttccaggtcctacatgtgaaagagaagaagacatgaaaggatttcttaaatggaagtgctcattctaacctgacggtgacagaatcaattgatacaccatttcttcaagacaaaaaagcacatattcaaggaatagctcaaaaaatgctccagttttcacattatttcaaaactttatcggtagaatgactctgcacactaatttcactaagagtacataaacataggaaaatagtcctcaaaagatgcatttatgggcctatatttttcaacataaagtgctagcagatgtgtaagaagagctgggaatgtcttgagctgtaagtcctgagacctccacaccatggctggtcctggaggagttcagcattctgattttttcttaggttcaggatgatcatccaaggtggctggatgctcatttggaccacctggtgtctcacctgtgacagctaaaaggatgactttcagccacttctgcttcagttcctcactgtctgcagcaaagctgtgcacggacttagactgggtcagtttgaaactgtgtggcaggtctgcgctccttggcatttcatccaccacatagcccagaagtggaatggtggcctgggctctgacgtcctggggggcaccatacatgtacagcacaagagggtcttgcttggggatcacacaccaagctttctgccaaggttttgacttctccatatactgaagaaagctgcacaccacactgtttccagatacttctgctgattcaatctctaaaattccttttcttttcttttcttcactgtctgtgaatccacttatgatttgataacagtctttacaaactttgctcaatttaccaccatcatattcaagttgagctttgtagtcggagcatttccaacaaaccacatatccacatgctcgacaatgatgcctccttcgtgtcagtgcattgaaaggttctttacatttcatacacattgtcacttcattatctcggatccatcttggggctcttttccctagctcagcagtagaaacctctgagtgaatgtcattatcctttgcaattgcatttctgaaggtttcatgcctttgatgaaaagcatcgatggtttcttgaagggccttgatccattcttctttgtcttgcgcagaactggcctgcagttccagtgttctctctttcccagacacctggaaagtatgtggatattcttcattttgagtctctacaattttcattccatcaatgccaaccctggttcgaactgtgaatttagagcctaccaagctgaatttgggcacacagtacagcaacatgttgttgaataagaaaaggtagcgttcttgtgctgaagtgttccgagcagctagtttgaggatctgtccttcttttattagttcatttgaagggtttacaatgtcttcttcttctcccaacatttcataaatctctaagagtttctttaggttctccattttccttattgcactattagaatggcttgctgctgtagatataatttcaagtgattttttagcatcattccagtccagggaatcaggaggcaatttccttagatagtccttaaggagcatctcataccggggaatccgctgaacaggttctagcatgtgatgctgcaaagttaagctcccacagattttctgtttctgaatttcttcaaccactgatttgaactggggaatacgttctgtcatgtttttaaccaattccattgcattatcaaatcctttcacatattctccatacatcttaaggaatggtgccaatttctgaaggatgtctccaattctaggagtagtttcccattcttgcattcgtttctccagctctggcaagaggaatttactatggaaggcatttattgatgaaatattagaaaagattttattcaccatctctgctggaaacgagcctcggtttgcttcttccaacagtttgcaataaaatacctcttaattgccattctgttacatgtaggcagaaggaggtctattccttcataatgtccagatggttgttaattttctaaattcacctccactctattttctgatctaagaggtcaagtcggttgacataagctctttcagtaagcaaaagttcattggctattttgtgaagtttttgctcattagtctccttcatctcatggtgctggtccagctgctccagttccagagggctttccccattttccctctcttgtaccttggtttctgtttctgcccctctttcttctagggggagcactgggcctatgcctggagtcctgtagctactgtcagaagcatttccatcacagctgtctgttgtgggtgatgcaggagctgtggcagtttcatctctttctccattcactatgtgcgtatcaagcaagggttcagaagcttgaatagaagtatctgagctaagagtggcagctttctcctcctcacattccatctggttttgtgctgccattacaccgttggccacacaagtctgtgcaccctgagt

SEQ ID NO: 14938 - RNA, 6642 nt, Homo sapiens
  source 1..6642: mol_type = other RNA
gctgggattacaggcatgagccactatgcccggcctatgcttattttaaaatgtcaattgtcactcacaaaatgaaatgctagtttggttaaaaaaaaaaaagtcttatatacagacagacatgactgttttgctaatgaagagaaccccccacaagtgatacattccaatatccatatactgtgtaatatataatgtgattctcttataatggtccccacagactagtttcttcccaaacctatatgtcactatgtatttggtatttatttattaaagtatgatatgagatttcttgatttacgttttccactaaaactaccacaatgaattttgggaaaaggggttgaccatcatataactcccggtgaccccaacaagttaaaactatcttgtagaagccatgtgctatttcatgtcaaaatacaggaaaagatactgcattctgccaaatgctcagtccagaaagtagaagaccatgattgacttcagattttttttttttttgcctcagtaaacagtacagaaaatgatctgagaatgaaattattttttaaaagcccaaaggagaaaaagaataacaagatatcatagtctagcatttacaggccaaggtcaaaaacctgggtgcaatggatcccatcagcatgtaattacatagattttatatcccttctgcagttaaaatatttcatcttatcttaaaacacattgctgtggtctggagaccagcagtctctcccccacatctctcttcattcttgcttgtttcagtttcttatcttattcctctctgccctttctgtaaagaaagcaaagttatcttctcatgactacgtgattaaggggtatatataaggatgaattatacataaagatccatgtaaataatttatgttaaaatatttaagttaaacaatttcgatagaaaaagttcatttctatggaaagacagaattgcaaatcaacagtgtttttacatatatacatacatgtataaattcacagaaagggttttttaagttgacctagtggtctttatgtatcatagtcattttctaaagctgagaatctatagtagataatagtatgcaaataacaagaagtttgattctaataaaattggtaagaatgaagaagcaacatgatccactacagatgtcaatacagtctgaagaataggaactggttggccacagttcatatactaatacattcttggagaatacaaaatttaagaatgaaaacattaagacattcttgacttttgagttaattttagcttataaatatcatgtgcttaatcttagacccactaacacaaatatcatatgatataggaaatcttcattaatctattctgcattatagcaaagatacctataaaacccaagacgcttgttccctagaagtttacttgctccggttggtgcttgctactcaggttgtatctagtccagaaagatcatcagaaatttatcacagacaatatgctcagattaagaacttaaggctttgaatataaccagaaaacaaataaaagcaaccaccctgtttccaaaaagtaaggacaaggaaaagtaaaacagaattgtgaactcaaaagtatttttgacaaaagtttttagaaggcatcaaagaatctttaacaaccctgcagtaccacaaactttatcgttttctttatatatttataactagaacaagtgttcttaaaaaaaaaaaatccaaacgtgtgcgtatatatatatggggaaagggtacatttaaaaggttagtttctgtaaaaagtttaataatttttaaaaaaattggggtaagttaagtcacctagtgaagataagtacacaaacctgatgtcaaattaaacttcagggaaaacaaaatgtgctttttctatccattttctttgttaaagtaaaaatgttcttgatagttatttaaaatccaaggaatgatgccccttcccatttcccttccttatactctgcaattcgaattaccgtatcacatctagaaagttaataattatctatattcttgtgggaaggggccttcatattaaattttcagtataaaaccataccctaaagagttttattgcttgcatacatgatgacactgtgatgccattattacaaaagtggctggtgttttttattgagccccacttaaaaccaagataaaagtctgcactatatttcatacttaacacgccaaatggtaggctttcagcaaaagcaaaatttaagcttaaaatattgaaatgttttataatgaatagaaattttgtcaaggaagtactttttaaagtttggaggaagggcactttaaagaaaagatgacttggaaagcaccaaatgagtgaaaataaagaattaagacccacagggaacgttggttttaatgggaaagcaaccaatgatatttttaggttgtcatgactgctcaagtatgttggaagggaaaaggcattgattattcttatcatcaatcacactttgaggtctcttggttgaattgtttaataaatggctaagggtattactttacctttcattgagtaaaaacatcagtgattctttaataagagagaagcgggtaaggctgtttcactgcttctctttgcgtttagctgaagaatgtggggtggaaagtgaatatggtgaccggataaccagaaattctcttctagtattaatgcttctcatttaaaaaattaaagataatgactgttaagagcatgataataaacattatctttacatgagtattctttcaatgatctaagttaaataacattgatatttattgagccaaaacttaagtgtgtccatgttacttctgttttggtagggaaagtgtagtcttcttgcttttaaaaatagttttcaaaaataatctgacttataaatcttcccattggcccatacattaccattgttctagtcacacttacaaaagtcctcttccccagttaatcattctgtatttccattgcttctcttttcttgagattaagaaaaccaaagcatcatctatagctacagtttaattttccaaaaaaccactctgagtatacatcacacacataccccgctggccattaaaaaagagaagcaatgtaaattttcttctagtctttccctgatttaatagggcctaagaagctacttttatctctttttggctccatctatttggtttaatgttaatgatcatggctgataatccttttatggaggaagggaacctattatgtcagcaataattggttcacttgctcctttggggtggaaaaaataagatatttcttaaagtaacaaggcctgaataaatgtgtggcagtctcaaattctattctatatctaaggtgtaatccttacatactaaagatagtgggatcattcttgtagatttctagcagactggtacattaaaaagtgacaatgtttggggtatgacagtataaaaaaaggtttaatttgagaaaaaggattaagttaaatagtaaacttagtgtgagattttaatcacaagtacaaaagagtgaagagcagccttcatgacaaggaatcatgtgaccagcccccaccccaaacataggttatcacatgtggattttgtttcattccgacaaaggaaaaggcccatacagttatcttaagtgttcattatatagagaccttatttaaccatgctcgattatcttacggaaaagaaaaacattacgataaatgtggtttccacatatcctagttctgtaaaaggtcaggtgtctcataaagtttgggttttggtgaaaatgtttgtacatgctgatgttaactactgcaataattataggattgtaaacggtaaaataacctgtatgactttgactgtcccagtgaccaaaatgcactttaatcttagaataatcaagactgaagcattaactgaaccctcatcttatattaatagcaccttctaagagaggcactgttttaaataggcacagaaacaaaaaatggtactttaaaagtactgttggaattcacaaatatatcccatgccacataaattaccgcttattataaaaatatcaataccctcaaatgccaatcagcaaaacataaatcaccaaaacatttcttcagtttagaacattgctcaattccacgataaaccatgctttatatttaaaaaataaattagagatgaatgtgaacctaaaagcatgtataatatatatatttaatactatatatacataattgctatatacttaagacattcttaggagtatttctacaaaaacaagttatcttttctttataaatcggaaatctgaacaccaacaatttgtcctttttcttttgttttaaaagaacagacatcatttatgcagctagagatttataaactaaattaaataagttaatacaatagcctcaactgtccctgtatttttcaccatggatctattttggcaacatggaggtatatctttcaaactgttccaggtcctacatgtgaaagagaagaagacatgaaaggatttcttaaatggaagtgctcattctaacctgacggtgacagaatcaattgatacaccatttcttcaagacaaaaaagcacatattcaaggaatagctcaaaaaatgctccagttttcacattatttcaaaactttatcggtagaatgactctgcacactaatttcactaagagtacataaacataggaaaatagtcctcaaaagatgcatttatgggcctatatttttcaacataaagtgctagcagatgtgtaagaagagctgggaatgtcttgagctgtaagtcctgagacctccacaccatggctggtcctggaggagttcagcattctgattttttcttaggttcaggatgatcatccaaggtggctggatgctcatttggaccacctggtgtctcacctgtgacagctaaaaggatgactttcagccacttctgcttcagttcctcactgtctgcagcaaagctgtgcacggacttagactgggtcagtttgaaactgtgtggcaggtctgcgctccttggcatttcatccaccacatagcccagaagtggaatggtggcctgggctctgacgtcctggggggcaccatacatgtacagcacaagagggtcttgcttggggatcacacaccaagctttctgccaaggttttgacttctccatatactgaagaaagctgcacaccacactgtttccagatacttctgctgattcaatctctaaaattccttttcttttcttttcttcactgtctgtgaatccacttatgatttgataacagtctttacaaactttgctcaatttaccaccatcatattcaagttgagctttgtagtcggagcatttccaacaaaccacatatccacatgctcgacaatgatgcctccttcgtgtcagtgcattgaaaggttctttacatttcatacacattgtcacttcattatctcggatccatcttggggctcttttccctagctcagcagtagaaacctctgagtgaatgtcattatcctttgcaattgcatttctgaaggtttcatgcctttgatgaaaagcatcgatggtttcttgaagggccttgatccattcttctttgtcttgcgcagaactggcctgcagttccagtgttctctctttcccagacacctggaaagtatgtggatattcttcattttgagtctctacaattttcattccatcaatgccaaccctggttcgaactgtgaatttagagcctaccaagctgaatttgggcacacagtacagcaacatgttgttgaataagaaaaggtagcgttcttgtgctgaagtgttccgagcagctagtttgaggatctgtccttcttttattagttcatttgaagggtttacaatgtcttcttcttctcccaacatttcataaatctctaagagtttctttaggttctccattttccttattgcactattagaatggcttgctgctgtagatataatttcaagtgattttttagcatcattccagtccagggaatcaggaggcaatttccttagatagtccttaaggagcatctcataccggggaatccgctgaacaggttctagcatgtgatgctgcaaagttaagctcccacagattttctgtttctgaatttcttcaaccactgatttgaactggggaatacgttctgtcatgtttttaaccaattccattgcattatcaaatcctttcacatattctccatacatcttaaggaatggtgccaatttctgaaggatgtctccaattctaggagtagtttcccattcttgcattcgtttctccagctctggcaagaggaatttactatggaaggcatttattgatgaaatattagaaaagattttattcaccatctctgctggaaacgagcctcggtttgcttcttccaacagtttgcaataaaatacctgatctaagaggtcaagtcggttgacataagctctttcagtaagcaaaagttcattggctattttgtgaagtttttgctcattagtctccataatgttgaatcagtgggagacctgatcttgttttcctgcaactagacagtcccatctgggagtgatgggagacagc

SEQ ID NO: 14939 - RNA, 7759 nt, Homo sapiens
  source 1..7759: mol_type = other RNA
gctgggattacaggcatgagccactatgcccggcctatgcttattttaaaatgtcaattgtcactcacaaaatgaaatgctagtttggttaaaaaaaaaaaagtcttatatacagacagacatgactgttttgctaatgaagagaaccccccacaagtgatacattccaatatccatatactgtgtaatatataatgtgattctcttataatggtccccacagactagtttcttcccaaacctatatgtcactatgtatttggtatttatttattaaagtatgatatgagatttcttgatttacgttttccactaaaactaccacaatgaattttgggaaaaggggttgaccatcatataactcccggtgaccccaacaagttaaaactatcttgtagaagccatgtgctatttcatgtcaaaatacaggaaaagatactgcattctgccaaatgctcagtccagaaagtagaagaccatgattgacttcagattttttttttttttgcctcagtaaacagtacagaaaatgatctgagaatgaaattattttttaaaagcccaaaggagaaaaagaataacaagatatcatagtctagcatttacaggccaaggtcaaaaacctgggtgcaatggatcccatcagcatgtaattacatagattttatatcccttctgcagttaaaatatttcatcttatcttaaaacacattgctgtggtctggagaccagcagtctctcccccacatctctcttcattcttgcttgtttcagtttcttatcttattcctctctgccctttctgtaaagaaagcaaagttatcttctcatgactacgtgattaaggggtatatataaggatgaattatacataaagatccatgtaaataatttatgttaaaatatttaagttaaacaatttcgatagaaaaagttcatttctatggaaagacagaattgcaaatcaacagtgtttttacatatatacatacatgtataaattcacagaaagggttttttaagttgacctagtggtctttatgtatcatagtcattttctaaagctgagaatctatagtagataatagtatgcaaataacaagaagtttgattctaataaaattggtaagaatgaagaagcaacatgatccactacagatgtcaatacagtctgaagaataggaactggttggccacagttcatatactaatacattcttggagaatacaaaatttaagaatgaaaacattaagacattcttgacttttgagttaattttagcttataaatatcatgtgcttaatcttagacccactaacacaaatatcatatgatataggaaatcttcattaatctattctgcattatagcaaagatacctataaaacccaagacgcttgttccctagaagtttacttgctccggttggtgcttgctactcaggttgtatctagtccagaaagatcatcagaaatttatcacagacaatatgctcagattaagaacttaaggctttgaatataaccagaaaacaaataaaagcaaccaccctgtttccaaaaagtaaggacaaggaaaagtaaaacagaattgtgaactcaaaagtatttttgacaaaagtttttagaaggcatcaaagaatctttaacaaccctgcagtaccacaaactttatcgttttctttatatatttataactagaacaagtgttcttaaaaaaaaaaaatccaaacgtgtgcgtatatatatatggggaaagggtacatttaaaaggttagtttctgtaaaaagtttaataatttttaaaaaaattggggtaagttaagtcacctagtgaagataagtacacaaacctgatgtcaaattaaacttcagggaaaacaaaatgtgctttttctatccattttctttgttaaagtaaaaatgttcttgatagttatttaaaatccaaggaatgatgccccttcccatttcccttccttatactctgcaattcgaattaccgtatcacatctagaaagttaataattatctatattcttgtgggaaggggccttcatattaaattttcagtataaaaccataccctaaagagttttattgcttgcatacatgatgacactgtgatgccattattacaaaagtggctggtgttttttattgagccccacttaaaaccaagataaaagtctgcactatatttcatacttaacacgccaaatggtaggctttcagcaaaagcaaaatttaagcttaaaatattgaaatgttttataatgaatagaaattttgtcaaggaagtactttttaaagtttggaggaagggcactttaaagaaaagatgacttggaaagcaccaaatgagtgaaaataaagaattaagacccacagggaacgttggttttaatgggaaagcaaccaatgatatttttaggttgtcatgactgctcaagtatgttggaagggaaaaggcattgattattcttatcatcaatcacactttgaggtctcttggttgaattgtttaataaatggctaagggtattactttacctttcattgagtaaaaacatcagtgattctttaataagagagaagcgggtaaggctgtttcactgcttctctttgcgtttagctgaagaatgtggggtggaaagtgaatatggtgaccggataaccagaaattctcttctagtattaatgcttctcatttaaaaaattaaagataatgactgttaagagcatgataataaacattatctttacatgagtattctttcaatgatctaagttaaataacattgatatttattgagccaaaacttaagtgtgtccatgttacttctgttttggtagggaaagtgtagtcttcttgcttttaaaaatagttttcaaaaataatctgacttataaatcttcccattggcccatacattaccattgttctagtcacacttacaaaagtcctcttccccagttaatcattctgtatttccattgcttctcttttcttgagattaagaaaaccaaagcatcatctatagctacagtttaattttccaaaaaaccactctgagtatacatcacacacataccccgctggccattaaaaaagagaagcaatgtaaattttcttctagtctttccctgatttaatagggcctaagaagctacttttatctctttttggctccatctatttggtttaatgttaatgatcatggctgataatccttttatggaggaagggaacctattatgtcagcaataattggttcacttgctcctttggggtggaaaaaataagatatttcttaaagtaacaaggcctgaataaatgtgtggcagtctcaaattctattctatatctaaggtgtaatccttacatactaaagatagtgggatcattcttgtagatttctagcagactggtacattaaaaagtgacaatgtttggggtatgacagtataaaaaaaggtttaatttgagaaaaaggattaagttaaatagtaaacttagtgtgagattttaatcacaagtacaaaagagtgaagagcagccttcatgacaaggaatcatgtgaccagcccccaccccaaacataggttatcacatgtggattttgtttcattccgacaaaggaaaaggcccatacagttatcttaagtgttcattatatagagaccttatttaaccatgctcgattatcttacggaaaagaaaaacattacgataaatgtggtttccacatatcctagttctgtaaaaggtcaggtgtctcataaagtttgggttttggtgaaaatgtttgtacatgctgatgttaactactgcaataattataggattgtaaacggtaaaataacctgtatgactttgactgtcccagtgaccaaaatgcactttaatcttagaataatcaagactgaagcattaactgaaccctcatcttatattaatagcaccttctaagagaggcactgttttaaataggcacagaaacaaaaaatggtactttaaaagtactgttggaattcacaaatatatcccatgccacataaattaccgcttattataaaaatatcaataccctcaaatgccaatcagcaaaacataaatcaccaaaacatttcttcagtttagaacattgctcaattccacgataaaccatgctttatatttaaaaaataaattagagatgaatgtgaacctaaaagcatgtataatatatatatttaatactatatatacataattgctatatacttaagacattcttaggagtatttctacaaaaacaagttatcttttctttataaatcggaaatctgaacaccaacaatttgtcctttttcttttgttttaaaagaacagacatcatttatgcagctagagatttataaactaaattaaataagttaatacaatagcctcaactgtccctgtatttttcaccatggatctattttggcaacatggaggtatatctttcaaactgttccaggtcctacatgtgaaagagaagaagacatgaaaggatttcttaaatggaagtgctcattctaacctgacggtgacagaatcaattgatacaccatttcttcaagacaaaaaagcacatattcaaggaatagctcaaaaaatgctccagttttcacattatttcaaaactttatcggtagaatgactctgcacactaatttcactaagagtacataaacataggaaaatagtcctcaaaagatgcatttatgggcctatatttttcaacataaagtgctagcagatgtgtaagaagagctgggaatgtcttgagctgtaagtcctgagacctccacaccatggctggtcctggaggagttcagcattctgattttttcttaggttcaggatgatcatccaaggtggctggatgctcatttggaccacctggtgtctcacctgtgacagctaaaaggatgactttcagccacttctgcttcagttcctcactgtctgcagcaaagctgtgcacggacttagactgggtcagtttgaaactgtgtggcaggtctgcgctccttggcatttcatccaccacatagcccagaagtggaatggtggcctgggctctgacgtcctggggggcaccatacatgtacagcacaagagggtcttgcttggggatcacacaccaagctttctgccaaggttttgacttctccatatactgaagaaagctgcacaccacactgtttccagatacttctgctgattcaatctctaaaattccttttcttttcttttcttcactgtctgtgaatccacttatgatttgataacagtctttacaaactttgctcaatttaccaccatcatattcaagttgagctttgtagtcggagcatttccaacaaaccacatatccacatgctcgacaatgatgcctccttcgtgtcagtgcattgaaaggttctttacatttcatacacattgtcacttcattatctcggatccatcttggggctcttttccctagctcagcagtagaaacctctgagtgaatgtcattatcctttgcaattgcatttctgaaggtttcatgcctttgatgaaaagcatcgatggtttcttgaagggccttgatccattcttctttgtcttgcgcagaactggcctgcagttccagtgttctctctttcccagacacctggaaagtatgtggatattcttcattttgagtctctacaattttcattccatcaatgccaaccctggttcgaactgtgaatttagagcctaccaagctgaatttgggcacacagtacagcaacatgttgttgaataagaaaaggtagcgttcttgtgctgaagtgttccgagcagctagtttgaggatctgtccttcttttattagttcatttgaagggtttacaatgtcttcttcttctcccaacatttcataaatctctaagagtttctttaggttctccattttccttattgcactattagaatggcttgctgctgtagatataatttcaagtgattttttagcatcattccagtccagggaatcaggaggcaatttccttagatagtccttaaggagcatctcataccggggaatccgctgaacaggttctagcatgtgatgctgcaaagttaagctcccacagattttctgtttctgaatttcttcaaccactgatttgaactggggaatacgttctgtcatgtttttaaccaattccattgcattatcaaatcctttcacatattctccatacatcttaaggaatggtgccaatttctgaaggatgtctccaattctaggagtagtttcccattcttgcattcgtttctccagctctggcaagaggaatttactatggaaggcatttattgatgaaatattagaaaagattttattcaccatctctgctggaaacgagcctcggtttgcttcttccaacagtttgcaataaaatacctgatctaagaggtcaagtcggttgacataagctctttcagtaagcaaaagttcattggctattttgtgaagtttttgctcattagtctccttcatctcatggtgctggtccagctgctccagttccagagggctttccccattttccctctcttgtaccttggtttctgtttctgcccctctttcttctagggggagcactgggcctatgcctggagtcctgtagctactgtcagaagcatttccatcacagctgtctgttgtgggtgatgcaggagctgtggcagtttcatctctttctccattcactatgtgcgtatcaagcaagggttcagaagcttgaatagaagtatctgagctaagagtggcagctttctcctcctcacattccatctggttttgtgctgccattacaccgttggccacacaagtctgtgcaccctgagtcttatctgtatcatttccctgcctctgtggcaagtgctgggagaggagtttttgttgaggtgtggttgtcaatccatgccttcctggggttctaggagcatttaggttcacagcagactctttcttcaaatcactataatttgataatgagctgcctccttcaaagcgactgatgagatctgataccttactgggtttttcttttgagacacaagaagcagaggcaggtttaatttcctccatccttggttttgcactaggtaaagctttatgcctgggggtttggtgtatattggacgaaggtgaattctgcaggtgtaatggctttggaggcacttctggaagaagggtgaggagtcatgtcgcctcctaattacatgcctcattttcccccagctggttcccctggtttttagtgatctcatctcttttataaactcagttagctgacagttggctcatgctcactggcctagatcttgtggctttggacttgcagctgagtgttttgctggcctgttcccatttattccctgagcctcttcttcagatacattctcaccaaccagtgtggttgtgctgcttgtggagcaaggtggaactaaagcgatctttggacaggtactgctgccttataaaagctgaatttattcctcttggccagaagtcacaaatggttgaagtaaaactcccttcatttgttcttccagcgagccaaagcaagcctcccattaacccggtccattgcagataatctcacccagcacaggctcccctgctttccccacttcccagcccagcaaggataatcacattccggtggggagtgaacagatggt

SEQ ID NO: 14940 - RNA, 7580 nt, Homo sapiens
  source 1..7580: mol_type = other RNA
gctgggattacaggcatgagccactatgcccggcctatgcttattttaaaatgtcaattgtcactcacaaaatgaaatgctagtttggttaaaaaaaaaaaagtcttatatacagacagacatgactgttttgctaatgaagagaaccccccacaagtgatacattccaatatccatatactgtgtaatatataatgtgattctcttataatggtccccacagactagtttcttcccaaacctatatgtcactatgtatttggtatttatttattaaagtatgatatgagatttcttgatttacgttttccactaaaactaccacaatgaattttgggaaaaggggttgaccatcatataactcccggtgaccccaacaagttaaaactatcttgtagaagccatgtgctatttcatgtcaaaatacaggaaaagatactgcattctgccaaatgctcagtccagaaagtagaagaccatgattgacttcagattttttttttttttgcctcagtaaacagtacagaaaatgatctgagaatgaaattattttttaaaagcccaaaggagaaaaagaataacaagatatcatagtctagcatttacaggccaaggtcaaaaacctgggtgcaatggatcccatcagcatgtaattacatagattttatatcccttctgcagttaaaatatttcatcttatcttaaaacacattgctgtggtctggagaccagcagtctctcccccacatctctcttcattcttgcttgtttcagtttcttatcttattcctctctgccctttctgtaaagaaagcaaagttatcttctcatgactacgtgattaaggggtatatataaggatgaattatacataaagatccatgtaaataatttatgttaaaatatttaagttaaacaatttcgatagaaaaagttcatttctatggaaagacagaattgcaaatcaacagtgtttttacatatatacatacatgtataaattcacagaaagggttttttaagttgacctagtggtctttatgtatcatagtcattttctaaagctgagaatctatagtagataatagtatgcaaataacaagaagtttgattctaataaaattggtaagaatgaagaagcaacatgatccactacagatgtcaatacagtctgaagaataggaactggttggccacagttcatatactaatacattcttggagaatacaaaatttaagaatgaaaacattaagacattcttgacttttgagttaattttagcttataaatatcatgtgcttaatcttagacccactaacacaaatatcatatgatataggaaatcttcattaatctattctgcattatagcaaagatacctataaaacccaagacgcttgttccctagaagtttacttgctccggttggtgcttgctactcaggttgtatctagtccagaaagatcatcagaaatttatcacagacaatatgctcagattaagaacttaaggctttgaatataaccagaaaacaaataaaagcaaccaccctgtttccaaaaagtaaggacaaggaaaagtaaaacagaattgtgaactcaaaagtatttttgacaaaagtttttagaaggcatcaaagaatctttaacaaccctgcagtaccacaaactttatcgttttctttatatatttataactagaacaagtgttcttaaaaaaaaaaaatccaaacgtgtgcgtatatatatatggggaaagggtacatttaaaaggttagtttctgtaaaaagtttaataatttttaaaaaaattggggtaagttaagtcacctagtgaagataagtacacaaacctgatgtcaaattaaacttcagggaaaacaaaatgtgctttttctatccattttctttgttaaagtaaaaatgttcttgatagttatttaaaatccaaggaatgatgccccttcccatttcccttccttatactctgcaattcgaattaccgtatcacatctagaaagttaataattatctatattcttgtgggaaggggccttcatattaaattttcagtataaaaccataccctaaagagttttattgcttgcatacatgatgacactgtgatgccattattacaaaagtggctggtgttttttattgagccccacttaaaaccaagataaaagtctgcactatatttcatacttaacacgccaaatggtaggctttcagcaaaagcaaaatttaagcttaaaatattgaaatgttttataatgaatagaaattttgtcaaggaagtactttttaaagtttggaggaagggcactttaaagaaaagatgacttggaaagcaccaaatgagtgaaaataaagaattaagacccacagggaacgttggttttaatgggaaagcaaccaatgatatttttaggttgtcatgactgctcaagtatgttggaagggaaaaggcattgattattcttatcatcaatcacactttgaggtctcttggttgaattgtttaataaatggctaagggtattactttacctttcattgagtaaaaacatcagtgattctttaataagagagaagcgggtaaggctgtttcactgcttctctttgcgtttagctgaagaatgtggggtggaaagtgaatatggtgaccggataaccagaaattctcttctagtattaatgcttctcatttaaaaaattaaagataatgactgttaagagcatgataataaacattatctttacatgagtattctttcaatgatctaagttaaataacattgatatttattgagccaaaacttaagtgtgtccatgttacttctgttttggtagggaaagtgtagtcttcttgcttttaaaaatagttttcaaaaataatctgacttataaatcttcccattggcccatacattaccattgttctagtcacacttacaaaagtcctcttccccagttaatcattctgtatttccattgcttctcttttcttgagattaagaaaaccaaagcatcatctatagctacagtttaattttccaaaaaaccactctgagtatacatcacacacataccccgctggccattaaaaaagagaagcaatgtaaattttcttctagtctttccctgatttaatagggcctaagaagctacttttatctctttttggctccatctatttggtttaatgttaatgatcatggctgataatccttttatggaggaagggaacctattatgtcagcaataattggttcacttgctcctttggggtggaaaaaataagatatttcttaaagtaacaaggcctgaataaatgtgtggcagtctcaaattctattctatatctaaggtgtaatccttacatactaaagatagtgggatcattcttgtagatttctagcagactggtacattaaaaagtgacaatgtttggggtatgacagtataaaaaaaggtttaatttgagaaaaaggattaagttaaatagtaaacttagtgtgagattttaatcacaagtacaaaagagtgaagagcagccttcatgacaaggaatcatgtgaccagcccccaccccaaacataggttatcacatgtggattttgtttcattccgacaaaggaaaaggcccatacagttatcttaagtgttcattatatagagaccttatttaaccatgctcgattatcttacggaaaagaaaaacattacgataaatgtggtttccacatatcctagttctgtaaaaggtcaggtgtctcataaagtttgggttttggtgaaaatgtttgtacatgctgatgttaactactgcaataattataggattgtaaacggtaaaataacctgtatgactttgactgtcccagtgaccaaaatgcactttaatcttagaataatcaagactgaagcattaactgaaccctcatcttatattaatagcaccttctaagagaggcactgttttaaataggcacagaaacaaaaaatggtactttaaaagtactgttggaattcacaaatatatcccatgccacataaattaccgcttattataaaaatatcaataccctcaaatgccaatcagcaaaacataaatcaccaaaacatttcttcagtttagaacattgctcaattccacgataaaccatgctttatatttaaaaaataaattagagatgaatgtgaacctaaaagcatgtataatatatatatttaatactatatatacataattgctatatacttaagacattcttaggagtatttctacaaaaacaagttatcttttctttataaatcggaaatctgaacaccaacaatttgtcctttttcttttgttttaaaagaacagacatcatttatgcagctagagatttataaactaaattaaataagttaatacaatagcctcaactgtccctgtatttttcaccatggatctattttggcaacatggaggtatatctttcaaactgttccaggtcctacatgtgaaagagaagaagacatgaaaggatttcttaaatggaagtgctcattctaacctgacggtgacagaatcaattgatacaccatttcttcaagacaaaaaagcacatattcaaggaatagctcaaaaaatgctccagttttcacattatttcaaaactttatcggtagaatgactctgcacactaatttcactaagagtacataaacataggaaaatagtcctcaaaagatgcatttatgggcctatatttttcaacataaagtgctagcagatgtgtaagaagagctgggaatgtcttgagctgtaagtcctgagacctccacaccatggctggtcctggaggagttcagcattctgattttttcttaggttcaggatgatcatccaaggtggctggatgctcatttggaccacctggtgtctcacctgtgacagctaaaaggatgactttcagccacttctgcttcagttcctcactgtctgcagcaaagctgtgcacggacttagactgggtcagtttgaaactgtgtggcaggtctgcgctccttggcatttcatccaccacatagcccagaagtggaatggtggcctgggctctgacgtcctggggggcaccatacatgtacagcacaagagggtcttgcttggggatcacacaccaagctttctgccaaggttttgacttctccatatactgaagaaagctgcacaccacactgtttccagatacttctgctgattcaatctctaaaattccttttcttttcttttcttcactgtctgtgaatccacttatgatttgataacagtctttacaaactttgctcaatttaccaccatcatattcaagttgagctttgtagtcggagcatttccaacaaaccacatatccacatgctcgacaatgatgcctccttcgtgtcagtgcattgaaaggttctttacatttcatacacattgtcacttcattatctcggatccatcttggggctcttttccctagctcagcagtagaaacctctgagtgaatgtcattatcctttgcaattgcatttctgaaggtttcatgcctttgatgaaaagcatcgatggtttcttgaagggccttgatccattcttctttgtcttgcgcagaactggcctgcagttccagtgttctctctttcccagacacctggaaagtatgtggatattcttcattttgagtctctacaattttcattccatcaatgccaaccctggttcgaactgtgaatttagagcctaccaagctgaatttgggcacacagtacagcaacatgttgttgaataagaaaaggtagcgttcttgtgctgaagtgttccgagcagctagtttgaggatctgtccttcttttattagttcatttgaagggtttacaatgtcttcttcttctcccaacatttcataaatctctaagagtttctttaggttctccattttccttattgcactattagaatggcttgctgctgtagatataatttcaagtgattttttagcatcattccagtccagggaatcaggaggcaatttccttagatagtccttaaggagcatctcataccggggaatccgctgaacaggttctagcatgtgatgctgcaaagttaagctcccacagattttctgtttctgaatttcttcaaccactgatttgaactggggaatacgttctgtcatgtttttaaccaattccattgcattatcaaatcctttcacatattctccatacatcttaaggaatggtgccaatttctgaaggatgtctccaattctaggagtagtttcccattcttgcattcgtttctccagctctggcaagaggaatttactatggaaggcatttattgatgaaatattagaaaagattttattcaccatctctgctggaaacgagcctcggtttgcttcttccaacagtttgcaataaaatacctgatctaagaggtcaagtcggttgacataagctctttcagtaagcaaaagttcattggctattttgtgaagtttttgctcattagtctccttcatctcatggtgctggtccagctgctccagttccagagggctttccccattttccctctcttgtaccttggtttctgtttctgcccctctttcttctagggggagcactgggcctatgcctggagtcctgtagctactgtcagaagcatttccatcacagctgtctgttgtgggtgatgcaggagctgtggcagtttcatctctttctccattcactatgtgcgtatcaagcaagggttcagaagcttgaatagaagtatctgagctaagagtggcagctttctcctcctcacattccatctggttttgtgctgccattacaccgttggccacacaagtctgtgcaccctgagtcttatctgtatcatttccctgcctctgtggcaagtgctgggagaggagtttttgttgaggtgtggttgtcaatccatgccttcctggggttctaggagcatttaggttcacagcagactctttcttcaaatcactataatttgataatgagctgcctccttcaaagcgactgatgagatctgataccttactgggtttttcttttgagacacaagaagcagaggcaggtttaatttcctccatccttggttttgcactaggtaaagctttatgcctgggggtttggtgtatattggacgaaggtgaattctgcaggtgtaatggctttggaggcacttgtggctttggacttgcagctgagtgttttgctggcctgttcccatttattccctgagcctcttcttcagatacattctcaccaaccagtgtggttgtgctgcttgtggagcaaggtggaactaaagcgatctttggacaggtactgctgcagccccccataaaagattcttttcataacatccagcaatcttctgattaacctatttcctgcttctggagcaaggatttggatccataatttgttggtagaaactataggcattctgtatttagacactagacacatacacatctagtgttcaacatgataaagaactaact

SEQ ID NO: 14941 - RNA, 7530 nt, Homo sapiens
  source 1..7530: mol_type = other RNA
gctgggattacaggcatgagccactatgcccggcctatgcttattttaaaatgtcaattgtcactcacaaaatgaaatgctagtttggttaaaaaaaaaaaagtcttatatacagacagacatgactgttttgctaatgaagagaaccccccacaagtgatacattccaatatccatatactgtgtaatatataatgtgattctcttataatggtccccacagactagtttcttcccaaacctatatgtcactatgtatttggtatttatttattaaagtatgatatgagatttcttgatttacgttttccactaaaactaccacaatgaattttgggaaaaggggttgaccatcatataactcccggtgaccccaacaagttaaaactatcttgtagaagccatgtgctatttcatgtcaaaatacaggaaaagatactgcattctgccaaatgctcagtccagaaagtagaagaccatgattgacttcagattttttttttttttgcctcagtaaacagtacagaaaatgatctgagaatgaaattattttttaaaagcccaaaggagaaaaagaataacaagatatcatagtctagcatttacaggccaaggtcaaaaacctgggtgcaatggatcccatcagcatgtaattacatagattttatatcccttctgcagttaaaatatttcatcttatcttaaaacacattgctgtggtctggagaccagcagtctctcccccacatctctcttcattcttgcttgtttcagtttcttatcttattcctctctgccctttctgtaaagaaagcaaagttatcttctcatgactacgtgattaaggggtatatataaggatgaattatacataaagatccatgtaaataatttatgttaaaatatttaagttaaacaatttcgatagaaaaagttcatttctatggaaagacagaattgcaaatcaacagtgtttttacatatatacatacatgtataaattcacagaaagggttttttaagttgacctagtggtctttatgtatcatagtcattttctaaagctgagaatctatagtagataatagtatgcaaataacaagaagtttgattctaataaaattggtaagaatgaagaagcaacatgatccactacagatgtcaatacagtctgaagaataggaactggttggccacagttcatatactaatacattcttggagaatacaaaatttaagaatgaaaacattaagacattcttgacttttgagttaattttagcttataaatatcatgtgcttaatcttagacccactaacacaaatatcatatgatataggaaatcttcattaatctattctgcattatagcaaagatacctataaaacccaagacgcttgttccctagaagtttacttgctccggttggtgcttgctactcaggttgtatctagtccagaaagatcatcagaaatttatcacagacaatatgctcagattaagaacttaaggctttgaatataaccagaaaacaaataaaagcaaccaccctgtttccaaaaagtaaggacaaggaaaagtaaaacagaattgtgaactcaaaagtatttttgacaaaagtttttagaaggcatcaaagaatctttaacaaccctgcagtaccacaaactttatcgttttctttatatatttataactagaacaagtgttcttaaaaaaaaaaaatccaaacgtgtgcgtatatatatatggggaaagggtacatttaaaaggttagtttctgtaaaaagtttaataatttttaaaaaaattggggtaagttaagtcacctagtgaagataagtacacaaacctgatgtcaaattaaacttcagggaaaacaaaatgtgctttttctatccattttctttgttaaagtaaaaatgttcttgatagttatttaaaatccaaggaatgatgccccttcccatttcccttccttatactctgcaattcgaattaccgtatcacatctagaaagttaataattatctatattcttgtgggaaggggccttcatattaaattttcagtataaaaccataccctaaagagttttattgcttgcatacatgatgacactgtgatgccattattacaaaagtggctggtgttttttattgagccccacttaaaaccaagataaaagtctgcactatatttcatacttaacacgccaaatggtaggctttcagcaaaagcaaaatttaagcttaaaatattgaaatgttttataatgaatagaaattttgtcaaggaagtactttttaaagtttggaggaagggcactttaaagaaaagatgacttggaaagcaccaaatgagtgaaaataaagaattaagacccacagggaacgttggttttaatgggaaagcaaccaatgatatttttaggttgtcatgactgctcaagtatgttggaagggaaaaggcattgattattcttatcatcaatcacactttgaggtctcttggttgaattgtttaataaatggctaagggtattactttacctttcattgagtaaaaacatcagtgattctttaataagagagaagcgggtaaggctgtttcactgcttctctttgcgtttagctgaagaatgtggggtggaaagtgaatatggtgaccggataaccagaaattctcttctagtattaatgcttctcatttaaaaaattaaagataatgactgttaagagcatgataataaacattatctttacatgagtattctttcaatgatctaagttaaataacattgatatttattgagccaaaacttaagtgtgtccatgttacttctgttttggtagggaaagtgtagtcttcttgcttttaaaaatagttttcaaaaataatctgacttataaatcttcccattggcccatacattaccattgttctagtcacacttacaaaagtcctcttccccagttaatcattctgtatttccattgcttctcttttcttgagattaagaaaaccaaagcatcatctatagctacagtttaattttccaaaaaaccactctgagtatacatcacacacataccccgctggccattaaaaaagagaagcaatgtaaattttcttctagtctttccctgatttaatagggcctaagaagctacttttatctctttttggctccatctatttggtttaatgttaatgatcatggctgataatccttttatggaggaagggaacctattatgtcagcaataattggttcacttgctcctttggggtggaaaaaataagatatttcttaaagtaacaaggcctgaataaatgtgtggcagtctcaaattctattctatatctaaggtgtaatccttacatactaaagatagtgggatcattcttgtagatttctagcagactggtacattaaaaagtgacaatgtttggggtatgacagtataaaaaaaggtttaatttgagaaaaaggattaagttaaatagtaaacttagtgtgagattttaatcacaagtacaaaagagtgaagagcagccttcatgacaaggaatcatgtgaccagcccccaccccaaacataggttatcacatgtggattttgtttcattccgacaaaggaaaaggcccatacagttatcttaagtgttcattatatagagaccttatttaaccatgctcgattatcttacggaaaagaaaaacattacgataaatgtggtttccacatatcctagttctgtaaaaggtcaggtgtctcataaagtttgggttttggtgaaaatgtttgtacatgctgatgttaactactgcaataattataggattgtaaacggtaaaataacctgtatgactttgactgtcccagtgaccaaaatgcactttaatcttagaataatcaagactgaagcattaactgaaccctcatcttatattaatagcaccttctaagagaggcactgttttaaataggcacagaaacaaaaaatggtactttaaaagtactgttggaattcacaaatatatcccatgccacataaattaccgcttattataaaaatatcaataccctcaaatgccaatcagcaaaacataaatcaccaaaacatttcttcagtttagaacattgctcaattccacgataaaccatgctttatatttaaaaaataaattagagatgaatgtgaacctaaaagcatgtataatatatatatttaatactatatatacataattgctatatacttaagacattcttaggagtatttctacaaaaacaagttatcttttctttataaatcggaaatctgaacaccaacaatttgtcctttttcttttgttttaaaagaacagacatcatttatgcagctagagatttataaactaaattaaataagttaatacaatagcctcaactgtccctgtatttttcaccatggatctattttggcaacatggaggtatatctttcaaactgttccaggtcctacatgtgaaagagaagaagacatgaaaggatttcttaaatggaagtgctcattctaacctgacggtgacagaatcaattgatacaccatttcttcaagacaaaaaagcacatattcaaggaatagctcaaaaaatgctccagttttcacattatttcaaaactttatcggtagaatgactctgcacactaatttcactaagagtacataaacataggaaaatagtcctcaaaagatgcatttatgggcctatatttttcaacataaagtgctagcagatgtgtaagaagagctgggaatgtcttgagctgtaagtcctgagacctccacaccatggctggtcctggaggagttcagcattctgattttttcttaggttcaggatgatcatccaaggtggctggatgctcatttggaccacctggtgtctcacctgtgacagctaaaaggatgactttcagccacttctgcttcagttcctcactgtctgcagcaaagctgtgcacggacttagactgggtcagtttgaaactgtgtggcaggtctgcgctccttggcatttcatccaccacatagcccagaagtggaatggtggcctgggctctgacgtcctggggggcaccatacatgtacagcacaagagggtcttgcttggggatcacacaccaagctttctgccaaggttttgacttctccatatactgaagaaagctgcacaccacactgtttccagatacttctgctgattcaatctctaaaattccttttcttttcttttcttcactgtctgtgaatccacttatgatttgataacagtctttacaaactttgctcaatttaccaccatcatattcaagttgagctttgtagtcggagcatttccaacaaaccacatatccacatgctcgacaatgatgcctccttcgtgtcagtgcattgaaaggttctttacatttcatacacattgtcacttcattatctcggatccatcttggggctcttttccctagctcagcagtagaaacctctgagtgaatgtcattatcctttgcaattgcatttctgaaggtttcatgcctttgatgaaaagcatcgatggtttcttgaagggccttgatccattcttctttgtcttgcgcagaactggcctgcagttccagtgttctctctttcccagacacctggaaagtatgtggatattcttcattttgagtctctacaattttcattccatcaatgccaaccctggttcgaactgtgaatttagagcctaccaagctgaatttgggcacacagtacagcaacatgttgttgaataagaaaaggtagcgttcttgtgctgaagtgttccgagcagctagtttgaggatctgtccttcttttattagttcatttgaagggtttacaatgtcttcttcttctcccaacatttcataaatctctaagagtttctttaggttctccattttccttattgcactattagaatggcttgctgctgtagatataatttcaagtgattttttagcatcattccagtccagggaatcaggaggcaatttccttagatagtccttaaggagcatctcataccggggaatccgctgaacaggttctagcatgtgatgctgcaaagttaagctcccacagattttctgtttctgaatttcttcaaccactgatttgaactggggaatacgttctgtcatgtttttaaccaattccattgcattatcaaatcctttcacatattctccatacatcttaaggaatggtgccaatttctgaaggatgtctccaattctaggagtagtttcccattcttgcattcgtttctccagctctggcaagaggaatttactatggaaggcatttattgatgaaatattagaaaagattttattcaccatctctgctggaaacgagcctcggtttgcttcttccaacagtttgcaataaaatacctgatctaagaggtcaagtcggttgacataagctctttcagtaagcaaaagttcattggctattttgtgaagtttttgctcattagtctccttcatctcatggtgctggtccagctgctccagttccagagggctttccccattttccctctcttgtaccttggtttctgtttctgcccctctttcttctagggggagcactgggcctatgcctggagtcctgtagctactgtcagaagcatttccatcacagctgtctgttgtgggtgatgcaggagctgtggcagtttcatctctttctccattcactatgtgcgtatcaagcaagggttcagaagcttgaatagaagtatctgagctaagagtggcagctttctcctcctcacattccatctggttttgtgctgccattacaccgttggccacacaagtctgtgcaccctgagtcttatctgtatcatttccctgcctctgtggcaagtgctgggagaggagtttttgttgaggtgtggttgtcaatccatgccttcctggggttctaggagcatttaggttcacagcagactctttcttcaaatcactataatttgataatgagctgcctccttcaaagcgactgatgagatctgataccttactgggtttttcttttgagacacaagaagcagaggcaggtttaatttcctccatccttggttttgcactaggtaaagctttatgcctgggggtttggtgtatattggacgaaggtgaattctgcaggtgtaatggctttggaggcacttgtggctttggacttgcagctgagtgttttgctggcctgttcccatttattccctgagcctcttcttcagatacattctcaccaaccagtgtggttgtgctgcttgtggagcaaggtggaactaaagcgatctttggacaggtactgctgcctgtaatctcagctactcaggagactgaggtgggagaattgcttgaatccgggaggcggaggttgcagtgagccaagactgtgccactgcacaccagcctaggtgacagagtgagactccat

SEQ ID NO: 14942 - RNA, 7810 nt, Homo sapiens
  source 1..7810: mol_type = other RNA
gctgggattacaggcatgagccactatgcccggcctatgcttattttaaaatgtcaattgtcactcacaaaatgaaatgctagtttggttaaaaaaaaaaaagtcttatatacagacagacatgactgttttgctaatgaagagaaccccccacaagtgatacattccaatatccatatactgtgtaatatataatgtgattctcttataatggtccccacagactagtttcttcccaaacctatatgtcactatgtatttggtatttatttattaaagtatgatatgagatttcttgatttacgttttccactaaaactaccacaatgaattttgggaaaaggggttgaccatcatataactcccggtgaccccaacaagttaaaactatcttgtagaagccatgtgctatttcatgtcaaaatacaggaaaagatactgcattctgccaaatgctcagtccagaaagtagaagaccatgattgacttcagattttttttttttttgcctcagtaaacagtacagaaaatgatctgagaatgaaattattttttaaaagcccaaaggagaaaaagaataacaagatatcatagtctagcatttacaggccaaggtcaaaaacctgggtgcaatggatcccatcagcatgtaattacatagattttatatcccttctgcagttaaaatatttcatcttatcttaaaacacattgctgtggtctggagaccagcagtctctcccccacatctctcttcattcttgcttgtttcagtttcttatcttattcctctctgccctttctgtaaagaaagcaaagttatcttctcatgactacgtgattaaggggtatatataaggatgaattatacataaagatccatgtaaataatttatgttaaaatatttaagttaaacaatttcgatagaaaaagttcatttctatggaaagacagaattgcaaatcaacagtgtttttacatatatacatacatgtataaattcacagaaagggttttttaagttgacctagtggtctttatgtatcatagtcattttctaaagctgagaatctatagtagataatagtatgcaaataacaagaagtttgattctaataaaattggtaagaatgaagaagcaacatgatccactacagatgtcaatacagtctgaagaataggaactggttggccacagttcatatactaatacattcttggagaatacaaaatttaagaatgaaaacattaagacattcttgacttttgagttaattttagcttataaatatcatgtgcttaatcttagacccactaacacaaatatcatatgatataggaaatcttcattaatctattctgcattatagcaaagatacctataaaacccaagacgcttgttccctagaagtttacttgctccggttggtgcttgctactcaggttgtatctagtccagaaagatcatcagaaatttatcacagacaatatgctcagattaagaacttaaggctttgaatataaccagaaaacaaataaaagcaaccaccctgtttccaaaaagtaaggacaaggaaaagtaaaacagaattgtgaactcaaaagtatttttgacaaaagtttttagaaggcatcaaagaatctttaacaaccctgcagtaccacaaactttatcgttttctttatatatttataactagaacaagtgttcttaaaaaaaaaaaatccaaacgtgtgcgtatatatatatggggaaagggtacatttaaaaggttagtttctgtaaaaagtttaataatttttaaaaaaattggggtaagttaagtcacctagtgaagataagtacacaaacctgatgtcaaattaaacttcagggaaaacaaaatgtgctttttctatccattttctttgttaaagtaaaaatgttcttgatagttatttaaaatccaaggaatgatgccccttcccatttcccttccttatactctgcaattcgaattaccgtatcacatctagaaagttaataattatctatattcttgtgggaaggggccttcatattaaattttcagtataaaaccataccctaaagagttttattgcttgcatacatgatgacactgtgatgccattattacaaaagtggctggtgttttttattgagccccacttaaaaccaagataaaagtctgcactatatttcatacttaacacgccaaatggtaggctttcagcaaaagcaaaatttaagcttaaaatattgaaatgttttataatgaatagaaattttgtcaaggaagtactttttaaagtttggaggaagggcactttaaagaaaagatgacttggaaagcaccaaatgagtgaaaataaagaattaagacccacagggaacgttggttttaatgggaaagcaaccaatgatatttttaggttgtcatgactgctcaagtatgttggaagggaaaaggcattgattattcttatcatcaatcacactttgaggtctcttggttgaattgtttaataaatggctaagggtattactttacctttcattgagtaaaaacatcagtgattctttaataagagagaagcgggtaaggctgtttcactgcttctctttgcgtttagctgaagaatgtggggtggaaagtgaatatggtgaccggataaccagaaattctcttctagtattaatgcttctcatttaaaaaattaaagataatgactgttaagagcatgataataaacattatctttacatgagtattctttcaatgatctaagttaaataacattgatatttattgagccaaaacttaagtgtgtccatgttacttctgttttggtagggaaagtgtagtcttcttgcttttaaaaatagttttcaaaaataatctgacttataaatcttcccattggcccatacattaccattgttctagtcacacttacaaaagtcctcttccccagttaatcattctgtatttccattgcttctcttttcttgagattaagaaaaccaaagcatcatctatagctacagtttaattttccaaaaaaccactctgagtatacatcacacacataccccgctggccattaaaaaagagaagcaatgtaaattttcttctagtctttccctgatttaatagggcctaagaagctacttttatctctttttggctccatctatttggtttaatgttaatgatcatggctgataatccttttatggaggaagggaacctattatgtcagcaataattggttcacttgctcctttggggtggaaaaaataagatatttcttaaagtaacaaggcctgaataaatgtgtggcagtctcaaattctattctatatctaaggtgtaatccttacatactaaagatagtgggatcattcttgtagatttctagcagactggtacattaaaaagtgacaatgtttggggtatgacagtataaaaaaaggtttaatttgagaaaaaggattaagttaaatagtaaacttagtgtgagattttaatcacaagtacaaaagagtgaagagcagccttcatgacaaggaatcatgtgaccagcccccaccccaaacataggttatcacatgtggattttgtttcattccgacaaaggaaaaggcccatacagttatcttaagtgttcattatatagagaccttatttaaccatgctcgattatcttacggaaaagaaaaacattacgataaatgtggtttccacatatcctagttctgtaaaaggtcaggtgtctcataaagtttgggttttggtgaaaatgtttgtacatgctgatgttaactactgcaataattataggattgtaaacggtaaaataacctgtatgactttgactgtcccagtgaccaaaatgcactttaatcttagaataatcaagactgaagcattaactgaaccctcatcttatattaatagcaccttctaagagaggcactgttttaaataggcacagaaacaaaaaatggtactttaaaagtactgttggaattcacaaatatatcccatgccacataaattaccgcttattataaaaatatcaataccctcaaatgccaatcagcaaaacataaatcaccaaaacatttcttcagtttagaacattgctcaattccacgataaaccatgctttatatttaaaaaataaattagagatgaatgtgaacctaaaagcatgtataatatatatatttaatactatatatacataattgctatatacttaagacattcttaggagtatttctacaaaaacaagttatcttttctttataaatcggaaatctgaacaccaacaatttgtcctttttcttttgttttaaaagaacagacatcatttatgcagctagagatttataaactaaattaaataagttaatacaatagcctcaactgtccctgtatttttcaccatggatctattttggcaacatggaggtatatctttcaaactgttccaggtcctacatgtgaaagagaagaagacatgaaaggatttcttaaatggaagtgctcattctaacctgacggtgacagaatcaattgatacaccatttcttcaagacaaaaaagcacatattcaaggaatagctcaaaaaatgctccagttttcacattatttcaaaactttatcggtagaatgactctgcacactaatttcactaagagtacataaacataggaaaatagtcctcaaaagatgcatttatgggcctatatttttcaacataaagtgctagcagatgtgtaagaagagctgggaatgtcttgagctgtaagtcctgagacctccacaccatggctggtcctggaggagttcagcattctgattttttcttaggttcaggatgatcatccaaggtggctggatgctcatttggaccacctggtgtctcacctgtgacagctaaaaggatgactttcagccacttctgcttcagttcctcactgtctgcagcaaagctgtgcacggacttagactgggtcagtttgaaactgtgtggcaggtctgcgctccttggcatttcatccaccacatagcccagaagtggaatggtggcctgggctctgacgtcctggggggcaccatacatgtacagcacaagagggtcttgcttggggatcacacaccaagctttctgccaaggttttgacttctccatatactgaagaaagctgcacaccacactgtttccagatacttctgctgattcaatctctaaaattccttttcttttcttttcttcactgtctgtgaatccacttatgatttgataacagtctttacaaactttgctcaatttaccaccatcatattcaagttgagctttgtagtcggagcatttccaacaaaccacatatccacatgctcgacaatgatgcctccttcgtgtcagtgcattgaaaggttctttacatttcatacacattgtcacttcattatctcggatccatcttggggctcttttccctagctcagcagtagaaacctctgagtgaatgtcattatcctttgcaattgcatttctgaaggtttcatgcctttgatgaaaagcatcgatggtttcttgaagggccttgatccattcttctttgtcttgcgcagaactggcctgcagttccagtgttctctctttcccagacacctggaaagtatgtggatattcttcattttgagtctctacaattttcattccatcaatgccaaccctggttcgaactgtgaatttagagcctaccaagctgaatttgggcacacagtacagcaacatgttgttgaataagaaaaggtagcgttcttgtgctgaagtgttccgagcagctagtttgaggatctgtccttcttttattagttcatttgaagggtttacaatgtcttcttcttctcccaacatttcataaatctctaagagtttctttaggttctccattttccttattgcactattagaatggcttgctgctgtagatataatttcaagtgattttttagcatcattccagtccagggaatcaggaggcaatttccttagatagtccttaaggagcatctcataccggggaatccgctgaacaggttctagcatgtgatgctgcaaagttaagctcccacagattttctgtttctgaatttcttcaaccactgatttgaactggggaatacgttctgtcatgtttttaaccaattccattgcattatcaaatcctttcacatattctccatacatcttaaggaatggtgccaatttctgaaggatgtctccaattctaggagtagtttcccattcttgcattcgtttctccagctctggcaagaggaatttactatggaaggcatttattgatgaaatattagaaaagattttattcaccatctctgctggaaacgagcctcggtttgcttcttccaacagtttgcaataaaatacctgatctaagaggtcaagtcggttgacataagctctttcagtaagcaaaagttcattggctattttgtgaagtttttgctcattagtctccttcatctcatggtgctggtccagctgctccagttccagagggctttccccattttccctctcttgtaccttggtttctgtttctgcccctctttcttctagggggagcactgggcctatgcctggagtcctgtagctactgtcagaagcatttccatcacagctgtctgttgtgggtgatgcaggagctgtggcagtttcatctctttctccattcactatgtgcgtatcaagcaagggttcagaagcttgaatagaagtatctgagctaagagtggcagctttctcctcctcacattccatctggttttgtgctgccattacaccgttggccacacaagtctgtgcaccctgagtcttatctgtatcatttccctgcctctgtggcaagtgctgggagaggagtttttgttgaggtgtggttgtcaatccatgccttcctggggttctaggagcatttaggttcacagcagactctttcttcaaatcactataatttgataatgagctgcctccttcaaagcgactgatgagatctgataccttactgggtttttcttttgagacacaagaagcagaggcaggtttaatttcctccatccttggttttgcactaggtaaagctttatgcctgggggtttggtgtatattggacgaaggtgaattctgcaggtgtaatggctttggaggcacttgtggctttggacttgcagctgagtgttttgctggcctgttcccatttattccctgagcctcttcttcagatacattctcaccaaccagtgtggttgtgctgcttgtggagcaaggtggaactaaagcgatctttggacaggtactgctgcctgtggctcctgagggcacctggcccttgaaggcagcggtccctacacgtcccaggtgcgacgcgggcctgctccagggccggggcaccccgggcggcaggtaggaggggttggacttccgccggatcgccacccgcctgaagttggagccgccctcgtcgctcatcctgccgggctcgaccgccgctccccgactcctcccgctcccgtccagccgcgagcggcccctggggggcgtcgcctgcatgcccaggttcggcgcgactccgggggcgccctctactgcggcgtctcctcagcgagtgcctcctctccctctccttcccggtacgctccctcccggcgtcgcggcgagtttggctgcggcgactcctgcggcagtcgcagcgtctcggtatctgc

SEQ ID NO: 14943 - RNA, 7704 nt, Homo sapiens
  source 1..7704: mol_type = other RNA
gctgggattacaggcatgagccactatgcccggcctatgcttattttaaaatgtcaattgtcactcacaaaatgaaatgctagtttggttaaaaaaaaaaaagtcttatatacagacagacatgactgttttgctaatgaagagaaccccccacaagtgatacattccaatatccatatactgtgtaatatataatgtgattctcttataatggtccccacagactagtttcttcccaaacctatatgtcactatgtatttggtatttatttattaaagtatgatatgagatttcttgatttacgttttccactaaaactaccacaatgaattttgggaaaaggggttgaccatcatataactcccggtgaccccaacaagttaaaactatcttgtagaagccatgtgctatttcatgtcaaaatacaggaaaagatactgcattctgccaaatgctcagtccagaaagtagaagaccatgattgacttcagattttttttttttttgcctcagtaaacagtacagaaaatgatctgagaatgaaattattttttaaaagcccaaaggagaaaaagaataacaagatatcatagtctagcatttacaggccaaggtcaaaaacctgggtgcaatggatcccatcagcatgtaattacatagattttatatcccttctgcagttaaaatatttcatcttatcttaaaacacattgctgtggtctggagaccagcagtctctcccccacatctctcttcattcttgcttgtttcagtttcttatcttattcctctctgccctttctgtaaagaaagcaaagttatcttctcatgactacgtgattaaggggtatatataaggatgaattatacataaagatccatgtaaataatttatgttaaaatatttaagttaaacaatttcgatagaaaaagttcatttctatggaaagacagaattgcaaatcaacagtgtttttacatatatacatacatgtataaattcacagaaagggttttttaagttgacctagtggtctttatgtatcatagtcattttctaaagctgagaatctatagtagataatagtatgcaaataacaagaagtttgattctaataaaattggtaagaatgaagaagcaacatgatccactacagatgtcaatacagtctgaagaataggaactggttggccacagttcatatactaatacattcttggagaatacaaaatttaagaatgaaaacattaagacattcttgacttttgagttaattttagcttataaatatcatgtgcttaatcttagacccactaacacaaatatcatatgatataggaaatcttcattaatctattctgcattatagcaaagatacctataaaacccaagacgcttgttccctagaagtttacttgctccggttggtgcttgctactcaggttgtatctagtccagaaagatcatcagaaatttatcacagacaatatgctcagattaagaacttaaggctttgaatataaccagaaaacaaataaaagcaaccaccctgtttccaaaaagtaaggacaaggaaaagtaaaacagaattgtgaactcaaaagtatttttgacaaaagtttttagaaggcatcaaagaatctttaacaaccctgcagtaccacaaactttatcgttttctttatatatttataactagaacaagtgttcttaaaaaaaaaaaatccaaacgtgtgcgtatatatatatggggaaagggtacatttaaaaggttagtttctgtaaaaagtttaataatttttaaaaaaattggggtaagttaagtcacctagtgaagataagtacacaaacctgatgtcaaattaaacttcagggaaaacaaaatgtgctttttctatccattttctttgttaaagtaaaaatgttcttgatagttatttaaaatccaaggaatgatgccccttcccatttcccttccttatactctgcaattcgaattaccgtatcacatctagaaagttaataattatctatattcttgtgggaaggggccttcatattaaattttcagtataaaaccataccctaaagagttttattgcttgcatacatgatgacactgtgatgccattattacaaaagtggctggtgttttttattgagccccacttaaaaccaagataaaagtctgcactatatttcatacttaacacgccaaatggtaggctttcagcaaaagcaaaatttaagcttaaaatattgaaatgttttataatgaatagaaattttgtcaaggaagtactttttaaagtttggaggaagggcactttaaagaaaagatgacttggaaagcaccaaatgagtgaaaataaagaattaagacccacagggaacgttggttttaatgggaaagcaaccaatgatatttttaggttgtcatgactgctcaagtatgttggaagggaaaaggcattgattattcttatcatcaatcacactttgaggtctcttggttgaattgtttaataaatggctaagggtattactttacctttcattgagtaaaaacatcagtgattctttaataagagagaagcgggtaaggctgtttcactgcttctctttgcgtttagctgaagaatgtggggtggaaagtgaatatggtgaccggataaccagaaattctcttctagtattaatgcttctcatttaaaaaattaaagataatgactgttaagagcatgataataaacattatctttacatgagtattctttcaatgatctaagttaaataacattgatatttattgagccaaaacttaagtgtgtccatgttacttctgttttggtagggaaagtgtagtcttcttgcttttaaaaatagttttcaaaaataatctgacttataaatcttcccattggcccatacattaccattgttctagtcacacttacaaaagtcctcttccccagttaatcattctgtatttccattgcttctcttttcttgagattaagaaaaccaaagcatcatctatagctacagtttaattttccaaaaaaccactctgagtatacatcacacacataccccgctggccattaaaaaagagaagcaatgtaaattttcttctagtctttccctgatttaatagggcctaagaagctacttttatctctttttggctccatctatttggtttaatgttaatgatcatggctgataatccttttatggaggaagggaacctattatgtcagcaataattggttcacttgctcctttggggtggaaaaaataagatatttcttaaagtaacaaggcctgaataaatgtgtggcagtctcaaattctattctatatctaaggtgtaatccttacatactaaagatagtgggatcattcttgtagatttctagcagactggtacattaaaaagtgacaatgtttggggtatgacagtataaaaaaaggtttaatttgagaaaaaggattaagttaaatagtaaacttagtgtgagattttaatcacaagtacaaaagagtgaagagcagccttcatgacaaggaatcatgtgaccagcccccaccccaaacataggttatcacatgtggattttgtttcattccgacaaaggaaaaggcccatacagttatcttaagtgttcattatatagagaccttatttaaccatgctcgattatcttacggaaaagaaaaacattacgataaatgtggtttccacatatcctagttctgtaaaaggtcaggtgtctcataaagtttgggttttggtgaaaatgtttgtacatgctgatgttaactactgcaataattataggattgtaaacggtaaaataacctgtatgactttgactgtcccagtgaccaaaatgcactttaatcttagaataatcaagactgaagcattaactgaaccctcatcttatattaatagcaccttctaagagaggcactgttttaaataggcacagaaacaaaaaatggtactttaaaagtactgttggaattcacaaatatatcccatgccacataaattaccgcttattataaaaatatcaataccctcaaatgccaatcagcaaaacataaatcaccaaaacatttcttcagtttagaacattgctcaattccacgataaaccatgctttatatttaaaaaataaattagagatgaatgtgaacctaaaagcatgtataatatatatatttaatactatatatacataattgctatatacttaagacattcttaggagtatttctacaaaaacaagttatcttttctttataaatcggaaatctgaacaccaacaatttgtcctttttcttttgttttaaaagaacagacatcatttatgcagctagagatttataaactaaattaaataagttaatacaatagcctcaactgtccctgtatttttcaccatggatctattttggcaacatggaggtatatctttcaaactgttccaggtcctacatgtgaaagagaagaagacatgaaaggatttcttaaatggaagtgctcattctaacctgacggtgacagaatcaattgatacaccatttcttcaagacaaaaaagcacatattcaaggaatagctcaaaaaatgctccagttttcacattatttcaaaactttatcggtagaatgactctgcacactaatttcactaagagtacataaacataggaaaatagtcctcaaaagatgcatttatgggcctatatttttcaacataaagtgctagcagatgtgtaagaagagctgggaatgtcttgagctgtaagtcctgagacctccacaccatggctggtcctggaggagttcagcattctgattttttcttaggttcaggatgatcatccaaggtggctggatgctcatttggaccacctggtgtctcacctgtgacagctaaaaggatgactttcagccacttctgcttcagttcctcactgtctgcagcaaagctgtgcacggacttagactgggtcagtttgaaactgtgtggcaggtctgcgctccttggcatttcatccaccacatagcccagaagtggaatggtggcctgggctctgacgtcctggggggcaccatacatgtacagcacaagagggtcttgcttggggatcacacaccaagctttctgccaaggttttgacttctccatatactgaagaaagctgcacaccacactgtttccagatacttctgctgattcaatctctaaaattccttttcttttcttttcttcactgtctgtgaatccacttatgatttgataacagtctttacaaactttgctcaatttaccaccatcatattcaagttgagctttgtagtcggagcatttccaacaaaccacatatccacatgctcgacaatgatgcctccttcgtgtcagtgcattgaaaggttctttacatttcatacacattgtcacttcattatctcggatccatcttggggctcttttccctagctcagcagtagaaacctctgagtgaatgtcattatcctttgcaattgcatttctgaaggtttcatgcctttgatgaaaagcatcgatggtttcttgaagggccttgatccattcttctttgtcttgcgcagaactggcctgcagttccagtgttctctctttcccagacacctggaaagtatgtggatattcttcattttgagtctctacaattttcattccatcaatgccaaccctggttcgaactgtgaatttagagcctaccaagctgaatttgggcacacagtacagcaacatgttgttgaataagaaaaggtagcgttcttgtgctgaagtgttccgagcagctagtttgaggatctgtccttcttttattagttcatttgaagggtttacaatgtcttcttcttctcccaacatttcataaatctctaagagtttctttaggttctccattttccttattgcactattagaatggcttgctgctgtagatataatttcaagtgattttttagcatcattccagtccagggaatcaggaggcaatttccttagatagtccttaaggagcatctcataccggggaatccgctgaacaggttctagcatgtgatgctgcaaagttaagctcccacagattttctgtttctgaatttcttcaaccactgatttgaactggggaatacgttctgtcatgtttttaaccaattccattgcattatcaaatcctttcacatattctccatacatcttaaggaatggtgccaatttctgaaggatgtctccaattctaggagtagtttcccattcttgcattcgtttctccagctctggcaagaggaatttactatggaaggcatttattgatgaaatattagaaaagattttattcaccatctctgctggaaacgagcctcggtttgcttcttccaacagtttgcaataaaatacctgatctaagaggtcaagtcggttgacataagctctttcagtaagcaaaagttcattggctattttgtgaagtttttgctcattagtctccttcatctcatggtgctggtccagctgctccagttccagagggctttccccattttccctctcttgtaccttggtttctgtttctgcccctctttcttctagggggagcactgggcctatgcctggagtcctgtagctactgtcagaagcatttccatcacagctgtctgttgtgggtgatgcaggagctgtggcagtttcatctctttctccattcactatgtgcgtatcaagcaagggttcagaagcttgaatagaagtatctgagctaagagtggcagctttctcctcctcacattccatctggttttgtgctgccattacaccgttggccacacaagtctgtgcaccctgagtcttatctgtatcatttccctgcctctgtggcaagtgctgggagaggagtttttgttgaggtgtggttgtcaatccatgccttcctggggttctaggagcatttaggttcacagcagactctttcttcaaatcactataatttgataatgagctgcctccttcaaagcgactgatgagatctgataccttactgggtttttcttttgagacacaagaagcagaggcaggtttaatttcctccatccttggttttgcactaggtaaagctttatgcctgggggtttggtgtatattggacgaaggtgaattctgcaggtgtaatggctttggaggcacttgtggctttggacttgcagctgagtgttttgctggcctgttcccatttattccctgagcctcttcttcagatacattctcaccaaccagtgtggttgtgctgcttgtggagcaaggtggaactaaagcgatctttggacaggtactgctgccttataaaagctgaatttattcctcttggccagaagtcacaaatggttgaagtaaaactcccttcatttgttcttccagcgagccaaagcaagcctcccattaacccggtccattgcagataatctcacccagcacaggctcccctgctttccccacttcccagcccagcaaggataatcacattccggtggggagtgaacagatggtggattccatggtaaccagccctcctaaggcgattggtagaagtgtgtgactactgcttattgggtaacaatcgctgtctttgtgctcc

SEQ ID NO: 14944 - RNA, 7585 nt, Homo sapiens
  source 1..7585: mol_type = other RNA
gctgggattacaggcatgagccactatgcccggcctatgcttattttaaaatgtcaattgtcactcacaaaatgaaatgctagtttggttaaaaaaaaaaaagtcttatatacagacagacatgactgttttgctaatgaagagaaccccccacaagtgatacattccaatatccatatactgtgtaatatataatgtgattctcttataatggtccccacagactagtttcttcccaaacctatatgtcactatgtatttggtatttatttattaaagtatgatatgagatttcttgatttacgttttccactaaaactaccacaatgaattttgggaaaaggggttgaccatcatataactcccggtgaccccaacaagttaaaactatcttgtagaagccatgtgctatttcatgtcaaaatacaggaaaagatactgcattctgccaaatgctcagtccagaaagtagaagaccatgattgacttcagattttttttttttttgcctcagtaaacagtacagaaaatgatctgagaatgaaattattttttaaaagcccaaaggagaaaaagaataacaagatatcatagtctagcatttacaggccaaggtcaaaaacctgggtgcaatggatcccatcagcatgtaattacatagattttatatcccttctgcagttaaaatatttcatcttatcttaaaacacattgctgtggtctggagaccagcagtctctcccccacatctctcttcattcttgcttgtttcagtttcttatcttattcctctctgccctttctgtaaagaaagcaaagttatcttctcatgactacgtgattaaggggtatatataaggatgaattatacataaagatccatgtaaataatttatgttaaaatatttaagttaaacaatttcgatagaaaaagttcatttctatggaaagacagaattgcaaatcaacagtgtttttacatatatacatacatgtataaattcacagaaagggttttttaagttgacctagtggtctttatgtatcatagtcattttctaaagctgagaatctatagtagataatagtatgcaaataacaagaagtttgattctaataaaattggtaagaatgaagaagcaacatgatccactacagatgtcaatacagtctgaagaataggaactggttggccacagttcatatactaatacattcttggagaatacaaaatttaagaatgaaaacattaagacattcttgacttttgagttaattttagcttataaatatcatgtgcttaatcttagacccactaacacaaatatcatatgatataggaaatcttcattaatctattctgcattatagcaaagatacctataaaacccaagacgcttgttccctagaagtttacttgctccggttggtgcttgctactcaggttgtatctagtccagaaagatcatcagaaatttatcacagacaatatgctcagattaagaacttaaggctttgaatataaccagaaaacaaataaaagcaaccaccctgtttccaaaaagtaaggacaaggaaaagtaaaacagaattgtgaactcaaaagtatttttgacaaaagtttttagaaggcatcaaagaatctttaacaaccctgcagtaccacaaactttatcgttttctttatatatttataactagaacaagtgttcttaaaaaaaaaaaatccaaacgtgtgcgtatatatatatggggaaagggtacatttaaaaggttagtttctgtaaaaagtttaataatttttaaaaaaattggggtaagttaagtcacctagtgaagataagtacacaaacctgatgtcaaattaaacttcagggaaaacaaaatgtgctttttctatccattttctttgttaaagtaaaaatgttcttgatagttatttaaaatccaaggaatgatgccccttcccatttcccttccttatactctgcaattcgaattaccgtatcacatctagaaagttaataattatctatattcttgtgggaaggggccttcatattaaattttcagtataaaaccataccctaaagagttttattgcttgcatacatgatgacactgtgatgccattattacaaaagtggctggtgttttttattgagccccacttaaaaccaagataaaagtctgcactatatttcatacttaacacgccaaatggtaggctttcagcaaaagcaaaatttaagcttaaaatattgaaatgttttataatgaatagaaattttgtcaaggaagtactttttaaagtttggaggaagggcactttaaagaaaagatgacttggaaagcaccaaatgagtgaaaataaagaattaagacccacagggaacgttggttttaatgggaaagcaaccaatgatatttttaggttgtcatgactgctcaagtatgttggaagggaaaaggcattgattattcttatcatcaatcacactttgaggtctcttggttgaattgtttaataaatggctaagggtattactttacctttcattgagtaaaaacatcagtgattctttaataagagagaagcgggtaaggctgtttcactgcttctctttgcgtttagctgaagaatgtggggtggaaagtgaatatggtgaccggataaccagaaattctcttctagtattaatgcttctcatttaaaaaattaaagataatgactgttaagagcatgataataaacattatctttacatgagtattctttcaatgatctaagttaaataacattgatatttattgagccaaaacttaagtgtgtccatgttacttctgttttggtagggaaagtgtagtcttcttgcttttaaaaatagttttcaaaaataatctgacttataaatcttcccattggcccatacattaccattgttctagtcacacttacaaaagtcctcttccccagttaatcattctgtatttccattgcttctcttttcttgagattaagaaaaccaaagcatcatctatagctacagtttaattttccaaaaaaccactctgagtatacatcacacacataccccgctggccattaaaaaagagaagcaatgtaaattttcttctagtctttccctgatttaatagggcctaagaagctacttttatctctttttggctccatctatttggtttaatgttaatgatcatggctgataatccttttatggaggaagggaacctattatgtcagcaataattggttcacttgctcctttggggtggaaaaaataagatatttcttaaagtaacaaggcctgaataaatgtgtggcagtctcaaattctattctatatctaaggtgtaatccttacatactaaagatagtgggatcattcttgtagatttctagcagactggtacattaaaaagtgacaatgtttggggtatgacagtataaaaaaaggtttaatttgagaaaaaggattaagttaaatagtaaacttagtgtgagattttaatcacaagtacaaaagagtgaagagcagccttcatgacaaggaatcatgtgaccagcccccaccccaaacataggttatcacatgtggattttgtttcattccgacaaaggaaaaggcccatacagttatcttaagtgttcattatatagagaccttatttaaccatgctcgattatcttacggaaaagaaaaacattacgataaatgtggtttccacatatcctagttctgtaaaaggtcaggtgtctcataaagtttgggttttggtgaaaatgtttgtacatgctgatgttaactactgcaataattataggattgtaaacggtaaaataacctgtatgactttgactgtcccagtgaccaaaatgcactttaatcttagaataatcaagactgaagcattaactgaaccctcatcttatattaatagcaccttctaagagaggcactgttttaaataggcacagaaacaaaaaatggtactttaaaagtactgttggaattcacaaatatatcccatgccacataaattaccgcttattataaaaatatcaataccctcaaatgccaatcagcaaaacataaatcaccaaaacatttcttcagtttagaacattgctcaattccacgataaaccatgctttatatttaaaaaataaattagagatgaatgtgaacctaaaagcatgtataatatatatatttaatactatatatacataattgctatatacttaagacattcttaggagtatttctacaaaaacaagttatcttttctttataaatcggaaatctgaacaccaacaatttgtcctttttcttttgttttaaaagaacagacatcatttatgcagctagagatttataaactaaattaaataagttaatacaatagcctcaactgtccctgtatttttcaccatggatctattttggcaacatggaggtatatctttcaaactgttccaggtcctacatgtgaaagagaagaagacatgaaaggatttcttaaatggaagtgctcattctaacctgacggtgacagaatcaattgatacaccatttcttcaagacaaaaaagcacatattcaaggaatagctcaaaaaatgctccagttttcacattatttcaaaactttatcggtagaatgactctgcacactaatttcactaagagtacataaacataggaaaatagtcctcaaaagatgcatttatgggcctatatttttcaacataaagtgctagcagatgtgtaagaagagctgggaatgtcttgagctgtaagtcctgagacctccacaccatggctggtcctggaggagttcagcattctgattttttcttaggttcaggatgatcatccaaggtggctggatgctcatttggaccacctggtgtctcacctgtgacagctaaaaggatgactttcagccacttctgcttcagttcctcactgtctgcagcaaagctgtgcacggacttagactgggtcagtttgaaactgtgtggcaggtctgcgctccttggcatttcatccaccacatagcccagaagtggaatggtggcctgggctctgacgtcctggggggcaccatacatgtacagcacaagagggtcttgcttggggatcacacaccaagctttctgccaaggttttgacttctccatatactgaagaaagctgcacaccacactgtttccagatacttctgctgattcaatctctaaaattccttttcttttcttttcttcactgtctgtgaatccacttatgatttgataacagtctttacaaactttgctcaatttaccaccatcatattcaagttgagctttgtagtcggagcatttccaacaaaccacatatccacatgctcgacaatgatgcctccttcgtgtcagtgcattgaaaggttctttacatttcatacacattgtcacttcattatctcggatccatcttggggctcttttccctagctcagcagtagaaacctctgagtgaatgtcattatcctttgcaattgcatttctgaaggtttcatgcctttgatgaaaagcatcgatggtttcttgaagggccttgatccattcttctttgtcttgcgcagaactggcctgcagttccagtgttctctctttcccagacacctggaaagtatgtggatattcttcattttgagtctctacaattttcattccatcaatgccaaccctggttcgaactgtgaatttagagcctaccaagctgaatttgggcacacagtacagcaacatgttgttgaataagaaaaggtagcgttcttgtgctgaagtgttccgagcagctagtttgaggatctgtccttcttttattagttcatttgaagggtttacaatgtcttcttcttctcccaacatttcataaatctctaagagtttctttaggttctccattttccttattgcactattagaatggcttgctgctgtagatataatttcaagtgattttttagcatcattccagtccagggaatcaggaggcaatttccttagatagtccttaaggagcatctcataccggggaatccgctgaacaggttctagcatgtgatgctgcaaagttaagctcccacagattttctgtttctgaatttcttcaaccactgatttgaactggggaatacgttctgtcatgtttttaaccaattccattgcattatcaaatcctttcacatattctccatacatcttaaggaatggtgccaatttctgaaggatgtctccaattctaggagtagtttcccattcttgcattcgtttctccagctctggcaagaggaatttactatggaaggcatttattgatgaaatattagaaaagattttattcaccatctctgctggaaacgagcctcggtttgcttcttccaacagtttgcaataaaatacctgatctaagaggtcaagtcggttgacataagctctttcagtaagcaaaagttcattggctattttgtgaagtttttgctcattagtctccttcatctcatggtgctggtccagctgctccagttccagagggctttccccattttccctctcttgtaccttggtttctgtttctgcccctctttcttctagggggagcactgggcctatgcctggagtcctgtagctactgtcagaagcatttccatcacagctgtctgttgtgggtgatgcaggagctgtggcagtttcatctctttctccattcactatgtgcgtatcaagcaagggttcagaagcttgaatagaagtatctgagctaagagtggcagctttctcctcctcacattccatctggttttgtgctgccattacaccgttggccacacaagtctgtgcaccctgagtcttatctgtatcatttccctgcctctgtggcaagtgctgggagaggagtttttgttgaggtgtggttgtcaatccatgccttcctggggttctaggagcatttaggttcacagcagactctttcttcaaatcactataatttgataatgagctgcctccttcaaagcgactgatgagatctgataccttactgggtttttcttttgagacacaagaagcagaggcaggtttaatttcctccatccttggttttgcactaggtaaagctttatgcctgggggtttggtgtatattggacgaaggtgaattctgcaggtgtaatggctttggaggcacttgtggctttggacttgcagctgagtgttttgctggcctgttcccatttattccctgagcctcttcttcagatacattctcaccaaccagtgtggttgtgctgcttgtggagcaaggtggaactaaagcgatctttggacaggtactgctgccttgatcagtggacatgatttcacatatactgataattaatctactctggtttaataaaaagatatttggctttactcttttaaagttcatgtgataaaatctcactcctggctgtaaagcttcagggaggctgaagattacacaggatctgccaggagctcagaccaatgcactat

SEQ ID NO: 14945 - RNA, 7488 nt, Homo sapiens
  source 1..7488: mol_type = other RNA
gctgggattacaggcatgagccactatgcccggcctatgcttattttaaaatgtcaattgtcactcacaaaatgaaatgctagtttggttaaaaaaaaaaaagtcttatatacagacagacatgactgttttgctaatgaagagaaccccccacaagtgatacattccaatatccatatactgtgtaatatataatgtgattctcttataatggtccccacagactagtttcttcccaaacctatatgtcactatgtatttggtatttatttattaaagtatgatatgagatttcttgatttacgttttccactaaaactaccacaatgaattttgggaaaaggggttgaccatcatataactcccggtgaccccaacaagttaaaactatcttgtagaagccatgtgctatttcatgtcaaaatacaggaaaagatactgcattctgccaaatgctcagtccagaaagtagaagaccatgattgacttcagattttttttttttttgcctcagtaaacagtacagaaaatgatctgagaatgaaattattttttaaaagcccaaaggagaaaaagaataacaagatatcatagtctagcatttacaggccaaggtcaaaaacctgggtgcaatggatcccatcagcatgtaattacatagattttatatcccttctgcagttaaaatatttcatcttatcttaaaacacattgctgtggtctggagaccagcagtctctcccccacatctctcttcattcttgcttgtttcagtttcttatcttattcctctctgccctttctgtaaagaaagcaaagttatcttctcatgactacgtgattaaggggtatatataaggatgaattatacataaagatccatgtaaataatttatgttaaaatatttaagttaaacaatttcgatagaaaaagttcatttctatggaaagacagaattgcaaatcaacagtgtttttacatatatacatacatgtataaattcacagaaagggttttttaagttgacctagtggtctttatgtatcatagtcattttctaaagctgagaatctatagtagataatagtatgcaaataacaagaagtttgattctaataaaattggtaagaatgaagaagcaacatgatccactacagatgtcaatacagtctgaagaataggaactggttggccacagttcatatactaatacattcttggagaatacaaaatttaagaatgaaaacattaagacattcttgacttttgagttaattttagcttataaatatcatgtgcttaatcttagacccactaacacaaatatcatatgatataggaaatcttcattaatctattctgcattatagcaaagatacctataaaacccaagacgcttgttccctagaagtttacttgctccggttggtgcttgctactcaggttgtatctagtccagaaagatcatcagaaatttatcacagacaatatgctcagattaagaacttaaggctttgaatataaccagaaaacaaataaaagcaaccaccctgtttccaaaaagtaaggacaaggaaaagtaaaacagaattgtgaactcaaaagtatttttgacaaaagtttttagaaggcatcaaagaatctttaacaaccctgcagtaccacaaactttatcgttttctttatatatttataactagaacaagtgttcttaaaaaaaaaaaatccaaacgtgtgcgtatatatatatggggaaagggtacatttaaaaggttagtttctgtaaaaagtttaataatttttaaaaaaattggggtaagttaagtcacctagtgaagataagtacacaaacctgatgtcaaattaaacttcagggaaaacaaaatgtgctttttctatccattttctttgttaaagtaaaaatgttcttgatagttatttaaaatccaaggaatgatgccccttcccatttcccttccttatactctgcaattcgaattaccgtatcacatctagaaagttaataattatctatattcttgtgggaaggggccttcatattaaattttcagtataaaaccataccctaaagagttttattgcttgcatacatgatgacactgtgatgccattattacaaaagtggctggtgttttttattgagccccacttaaaaccaagataaaagtctgcactatatttcatacttaacacgccaaatggtaggctttcagcaaaagcaaaatttaagcttaaaatattgaaatgttttataatgaatagaaattttgtcaaggaagtactttttaaagtttggaggaagggcactttaaagaaaagatgacttggaaagcaccaaatgagtgaaaataaagaattaagacccacagggaacgttggttttaatgggaaagcaaccaatgatatttttaggttgtcatgactgctcaagtatgttggaagggaaaaggcattgattattcttatcatcaatcacactttgaggtctcttggttgaattgtttaataaatggctaagggtattactttacctttcattgagtaaaaacatcagtgattctttaataagagagaagcgggtaaggctgtttcactgcttctctttgcgtttagctgaagaatgtggggtggaaagtgaatatggtgaccggataaccagaaattctcttctagtattaatgcttctcatttaaaaaattaaagataatgactgttaagagcatgataataaacattatctttacatgagtattctttcaatgatctaagttaaataacattgatatttattgagccaaaacttaagtgtgtccatgttacttctgttttggtagggaaagtgtagtcttcttgcttttaaaaatagttttcaaaaataatctgacttataaatcttcccattggcccatacattaccattgttctagtcacacttacaaaagtcctcttccccagttaatcattctgtatttccattgcttctcttttcttgagattaagaaaaccaaagcatcatctatagctacagtttaattttccaaaaaaccactctgagtatacatcacacacataccccgctggccattaaaaaagagaagcaatgtaaattttcttctagtctttccctgatttaatagggcctaagaagctacttttatctctttttggctccatctatttggtttaatgttaatgatcatggctgataatccttttatggaggaagggaacctattatgtcagcaataattggttcacttgctcctttggggtggaaaaaataagatatttcttaaagtaacaaggcctgaataaatgtgtggcagtctcaaattctattctatatctaaggtgtaatccttacatactaaagatagtgggatcattcttgtagatttctagcagactggtacattaaaaagtgacaatgtttggggtatgacagtataaaaaaaggtttaatttgagaaaaaggattaagttaaatagtaaacttagtgtgagattttaatcacaagtacaaaagagtgaagagcagccttcatgacaaggaatcatgtgaccagcccccaccccaaacataggttatcacatgtggattttgtttcattccgacaaaggaaaaggcccatacagttatcttaagtgttcattatatagagaccttatttaaccatgctcgattatcttacggaaaagaaaaacattacgataaatgtggtttccacatatcctagttctgtaaaaggtcaggtgtctcataaagtttgggttttggtgaaaatgtttgtacatgctgatgttaactactgcaataattataggattgtaaacggtaaaataacctgtatgactttgactgtcccagtgaccaaaatgcactttaatcttagaataatcaagactgaagcattaactgaaccctcatcttatattaatagcaccttctaagagaggcactgttttaaataggcacagaaacaaaaaatggtactttaaaagtactgttggaattcacaaatatatcccatgccacataaattaccgcttattataaaaatatcaataccctcaaatgccaatcagcaaaacataaatcaccaaaacatttcttcagtttagaacattgctcaattccacgataaaccatgctttatatttaaaaaataaattagagatgaatgtgaacctaaaagcatgtataatatatatatttaatactatatatacataattgctatatacttaagacattcttaggagtatttctacaaaaacaagttatcttttctttataaatcggaaatctgaacaccaacaatttgtcctttttcttttgttttaaaagaacagacatcatttatgcagctagagatttataaactaaattaaataagttaatacaatagcctcaactgtccctgtatttttcaccatggatctattttggcaacatggaggtatatctttcaaactgttccaggtcctacatgtgaaagagaagaagacatgaaaggatttcttaaatggaagtgctcattctaacctgacggtgacagaatcaattgatacaccatttcttcaagacaaaaaagcacatattcaaggaatagctcaaaaaatgctccagttttcacattatttcaaaactttatcggtagaatgactctgcacactaatttcactaagagtacataaacataggaaaatagtcctcaaaagatgcatttatgggcctatatttttcaacataaagtgctagcagatgtgtaagaagagctgggaatgtcttgagctgtaagtcctgagacctccacaccatggctggtcctggaggagttcagcattctgattttttcttaggttcaggatgatcatccaaggtggctggatgctcatttggaccacctggtgtctcacctgtgacagctaaaaggatgactttcagccacttctgcttcagttcctcactgtctgcagcaaagctgtgcacggacttagactgggtcagtttgaaactgtgtggcaggtctgcgctccttggcatttcatccaccacatagcccagaagtggaatggtggcctgggctctgacgtcctggggggcaccatacatgtacagcacaagagggtcttgcttggggatcacacaccaagctttctgccaaggttttgacttctccatatactgaagaaagctgcacaccacactgtttccagatacttctgctgattcaatctctaaaattccttttcttttcttttcttcactgtctgtgaatccacttatgatttgataacagtctttacaaactttgctcaatttaccaccatcatattcaagttgagctttgtagtcggagcatttccaacaaaccacatatccacatgctcgacaatgatgcctccttcgtgtcagtgcattgaaaggttctttacatttcatacacattgtcacttcattatctcggatccatcttggggctcttttccctagctcagcagtagaaacctctgagtgaatgtcattatcctttgcaattgcatttctgaaggtttcatgcctttgatgaaaagcatcgatggtttcttgaagggccttgatccattcttctttgtcttgcgcagaactggcctgcagttccagtgttctctctttcccagacacctggaaagtatgtggatattcttcattttgagtctctacaattttcattccatcaatgccaaccctggttcgaactgtgaatttagagcctaccaagctgaatttgggcacacagtacagcaacatgttgttgaataagaaaaggtagcgttcttgtgctgaagtgttccgagcagctagtttgaggatctgtccttcttttattagttcatttgaagggtttacaatgtcttcttcttctcccaacatttcataaatctctaagagtttctttaggttctccattttccttattgcactattagaatggcttgctgctgtagatataatttcaagtgattttttagcatcattccagtccagggaatcaggaggcaatttccttagatagtccttaaggagcatctcataccggggaatccgctgaacaggttctagcatgtgatgctgcaaagttaagctcccacagattttctgtttctgaatttcttcaaccactgatttgaactggggaatacgttctgtcatgtttttaaccaattccattgcattatcaaatcctttcacatattctccatacatcttaaggaatggtgccaatttctgaaggatgtctccaattctaggagtagtttcccattcttgcattcgtttctccagctctggcaagaggaatttactatggaaggcatttattgatgaaatattagaaaagattttattcaccatctctgctggaaacgagcctcggtttgcttcttccaacagtttgcaataaaatacctgatctaagaggtcaagtcggttgacataagctctttcagtaagcaaaagttcattggctattttgtgaagtttttgctcattagtctccttcatctcatggtgctggtccagctgctccagttccagagggctttccccattttccctctcttgtaccttggtttctgtttctgcccctctttcttctagggggagcactgggcctatgcctggagtcctgtagctactgtcagaagcatttccatcacagctgtctgttgtgggtgatgcaggagctgtggcagtttcatctctttctccattcactatgtgcgtatcaagcaagggttcagaagcttgaatagaagtatctgagctaagagtggcagctttctcctcctcacattccatctggttttgtgctgccattacaccgttggccacacaagtctgtgcaccctgagtcttatctgtatcatttccctgcctctgtggcaagtgctgggagaggagtttttgttgaggtgtggttgtcaatccatgccttcctggggttctaggagcatttaggttcacagcagactctttcttcaaatcactataatttgataatgagctgcctccttcaaagcgactgatgagatctgataccttactgggtttttcttttgagacacaagaagcagaggcaggtttaatttcctccatccttggttttgcactaggtaaagctttatgcctgggggtttggtgtatattggacgaaggtgaattctgcaggtgtaatggctttggaggcacttgtggctttggacttgcagctgagtgttttgctggcctgttcccatttattccctgagcctcttcttcagatacattctcaccaaccagtgtggttgtgctgcttgtggagcaaggtggaactaaagcgatctttggacaggtactgctgctcttcgtggaaatttgtctttttctgagattagatgagattgagcacattccgggtggtatggctgtagactgtcttttt

SEQ ID NO: 14946 - RNA, 7396 nt, Homo sapiens
  source 1..7396: mol_type = other RNA
gctgggattacaggcatgagccactatgcccggcctatgcttattttaaaatgtcaattgtcactcacaaaatgaaatgctagtttggttaaaaaaaaaaaagtcttatatacagacagacatgactgttttgctaatgaagagaaccccccacaagtgatacattccaatatccatatactgtgtaatatataatgtgattctcttataatggtccccacagactagtttcttcccaaacctatatgtcactatgtatttggtatttatttattaaagtatgatatgagatttcttgatttacgttttccactaaaactaccacaatgaattttgggaaaaggggttgaccatcatataactcccggtgaccccaacaagttaaaactatcttgtagaagccatgtgctatttcatgtcaaaatacaggaaaagatactgcattctgccaaatgctcagtccagaaagtagaagaccatgattgacttcagattttttttttttttgcctcagtaaacagtacagaaaatgatctgagaatgaaattattttttaaaagcccaaaggagaaaaagaataacaagatatcatagtctagcatttacaggccaaggtcaaaaacctgggtgcaatggatcccatcagcatgtaattacatagattttatatcccttctgcagttaaaatatttcatcttatcttaaaacacattgctgtggtctggagaccagcagtctctcccccacatctctcttcattcttgcttgtttcagtttcttatcttattcctctctgccctttctgtaaagaaagcaaagttatcttctcatgactacgtgattaaggggtatatataaggatgaattatacataaagatccatgtaaataatttatgttaaaatatttaagttaaacaatttcgatagaaaaagttcatttctatggaaagacagaattgcaaatcaacagtgtttttacatatatacatacatgtataaattcacagaaagggttttttaagttgacctagtggtctttatgtatcatagtcattttctaaagctgagaatctatagtagataatagtatgcaaataacaagaagtttgattctaataaaattggtaagaatgaagaagcaacatgatccactacagatgtcaatacagtctgaagaataggaactggttggccacagttcatatactaatacattcttggagaatacaaaatttaagaatgaaaacattaagacattcttgacttttgagttaattttagcttataaatatcatgtgcttaatcttagacccactaacacaaatatcatatgatataggaaatcttcattaatctattctgcattatagcaaagatacctataaaacccaagacgcttgttccctagaagtttacttgctccggttggtgcttgctactcaggttgtatctagtccagaaagatcatcagaaatttatcacagacaatatgctcagattaagaacttaaggctttgaatataaccagaaaacaaataaaagcaaccaccctgtttccaaaaagtaaggacaaggaaaagtaaaacagaattgtgaactcaaaagtatttttgacaaaagtttttagaaggcatcaaagaatctttaacaaccctgcagtaccacaaactttatcgttttctttatatatttataactagaacaagtgttcttaaaaaaaaaaaatccaaacgtgtgcgtatatatatatggggaaagggtacatttaaaaggttagtttctgtaaaaagtttaataatttttaaaaaaattggggtaagttaagtcacctagtgaagataagtacacaaacctgatgtcaaattaaacttcagggaaaacaaaatgtgctttttctatccattttctttgttaaagtaaaaatgttcttgatagttatttaaaatccaaggaatgatgccccttcccatttcccttccttatactctgcaattcgaattaccgtatcacatctagaaagttaataattatctatattcttgtgggaaggggccttcatattaaattttcagtataaaaccataccctaaagagttttattgcttgcatacatgatgacactgtgatgccattattacaaaagtggctggtgttttttattgagccccacttaaaaccaagataaaagtctgcactatatttcatacttaacacgccaaatggtaggctttcagcaaaagcaaaatttaagcttaaaatattgaaatgttttataatgaatagaaattttgtcaaggaagtactttttaaagtttggaggaagggcactttaaagaaaagatgacttggaaagcaccaaatgagtgaaaataaagaattaagacccacagggaacgttggttttaatgggaaagcaaccaatgatatttttaggttgtcatgactgctcaagtatgttggaagggaaaaggcattgattattcttatcatcaatcacactttgaggtctcttggttgaattgtttaataaatggctaagggtattactttacctttcattgagtaaaaacatcagtgattctttaataagagagaagcgggtaaggctgtttcactgcttctctttgcgtttagctgaagaatgtggggtggaaagtgaatatggtgaccggataaccagaaattctcttctagtattaatgcttctcatttaaaaaattaaagataatgactgttaagagcatgataataaacattatctttacatgagtattctttcaatgatctaagttaaataacattgatatttattgagccaaaacttaagtgtgtccatgttacttctgttttggtagggaaagtgtagtcttcttgcttttaaaaatagttttcaaaaataatctgacttataaatcttcccattggcccatacattaccattgttctagtcacacttacaaaagtcctcttccccagttaatcattctgtatttccattgcttctcttttcttgagattaagaaaaccaaagcatcatctatagctacagtttaattttccaaaaaaccactctgagtatacatcacacacataccccgctggccattaaaaaagagaagcaatgtaaattttcttctagtctttccctgatttaatagggcctaagaagctacttttatctctttttggctccatctatttggtttaatgttaatgatcatggctgataatccttttatggaggaagggaacctattatgtcagcaataattggttcacttgctcctttggggtggaaaaaataagatatttcttaaagtaacaaggcctgaataaatgtgtggcagtctcaaattctattctatatctaaggtgtaatccttacatactaaagatagtgggatcattcttgtagatttctagcagactggtacattaaaaagtgacaatgtttggggtatgacagtataaaaaaaggtttaatttgagaaaaaggattaagttaaatagtaaacttagtgtgagattttaatcacaagtacaaaagagtgaagagcagccttcatgacaaggaatcatgtgaccagcccccaccccaaacataggttatcacatgtggattttgtttcattccgacaaaggaaaaggcccatacagttatcttaagtgttcattatatagagaccttatttaaccatgctcgattatcttacggaaaagaaaaacattacgataaatgtggtttccacatatcctagttctgtaaaaggtcaggtgtctcataaagtttgggttttggtgaaaatgtttgtacatgctgatgttaactactgcaataattataggattgtaaacggtaaaataacctgtatgactttgactgtcccagtgaccaaaatgcactttaatcttagaataatcaagactgaagcattaactgaaccctcatcttatattaatagcaccttctaagagaggcactgttttaaataggcacagaaacaaaaaatggtactttaaaagtactgttggaattcacaaatatatcccatgccacataaattaccgcttattataaaaatatcaataccctcaaatgccaatcagcaaaacataaatcaccaaaacatttcttcagtttagaacattgctcaattccacgataaaccatgctttatatttaaaaaataaattagagatgaatgtgaacctaaaagcatgtataatatatatatttaatactatatatacataattgctatatacttaagacattcttaggagtatttctacaaaaacaagttatcttttctttataaatcggaaatctgaacaccaacaatttgtcctttttcttttgttttaaaagaacagacatcatttatgcagctagagatttataaactaaattaaataagttaatacaatagcctcaactgtccctgtatttttcaccatggatctattttggcaacatggaggtatatctttcaaactgttccaggtcctacatgtgaaagagaagaagacatgaaaggatttcttaaatggaagtgctcattctaacctgacggtgacagaatcaattgatacaccatttcttcaagacaaaaaagcacatattcaaggaatagctcaaaaaatgctccagttttcacattatttcaaaactttatcggtagaatgactctgcacactaatttcactaagagtacataaacataggaaaatagtcctcaaaagatgcatttatgggcctatatttttcaacataaagtgctagcagatgtgtaagaagagctgggaatgtcttgagctgtaagtcctgagacctccacaccatggctggtcctggaggagttcagcattctgattttttcttaggttcaggatgatcatccaaggtggctggatgctcatttggaccacctggtgtctcacctgtgacagctaaaaggatgactttcagccacttctgcttcagttcctcactgtctgcagcaaagctgtgcacggacttagactgggtcagtttgaaactgtgtggcaggtctgcgctccttggcatttcatccaccacatagcccagaagtggaatggtggcctgggctctgacgtcctggggggcaccatacatgtacagcacaagagggtcttgcttggggatcacacaccaagctttctgccaaggttttgacttctccatatactgaagaaagctgcacaccacactgtttccagatacttctgctgattcaatctctaaaattccttttcttttcttttcttcactgtctgtgaatccacttatgatttgataacagtctttacaaactttgctcaatttaccaccatcatattcaagttgagctttgtagtcggagcatttccaacaaaccacatatccacatgctcgacaatgatgcctccttcgtgtcagtgcattgaaaggttctttacatttcatacacattgtcacttcattatctcggatccatcttggggctcttttccctagctcagcagtagaaacctctgagtgaatgtcattatcctttgcaattgcatttctgaaggtttcatgcctttgatgaaaagcatcgatggtttcttgaagggccttgatccattcttctttgtcttgcgcagaactggcctgcagttccagtgttctctctttcccagacacctggaaagtatgtggatattcttcattttgagtctctacaattttcattccatcaatgccaaccctggttcgaactgtgaatttagagcctaccaagctgaatttgggcacacagtacagcaacatgttgttgaataagaaaaggtagcgttcttgtgctgaagtgttccgagcagctagtttgaggatctgtccttcttttattagttcatttgaagggtttacaatgtcttcttcttctcccaacatttcataaatctctaagagtttctttaggttctccattttccttattgcactattagaatggcttgctgctgtagatataatttcaagtgattttttagcatcattccagtccagggaatcaggaggcaatttccttagatagtccttaaggagcatctcataccggggaatccgctgaacaggttctagcatgtgatgctgcaaagttaagctcccacagattttctgtttctgaatttcttcaaccactgatttgaactggggaatacgttctgtcatgtttttaaccaattccattgcattatcaaatcctttcacatattctccatacatcttaaggaatggtgccaatttctgaaggatgtctccaattctaggagtagtttcccattcttgcattcgtttctccagctctggcaagaggaatttactatggaaggcatttattgatgaaatattagaaaagattttattcaccatctctgctggaaacgagcctcggtttgcttcttccaacagtttgcaataaaatacctgatctaagaggtcaagtcggttgacataagctctttcagtaagcaaaagttcattggctattttgtgaagtttttgctcattagtctccttcatctcatggtgctggtccagctgctccagttccagagggctttccccattttccctctcttgtaccttggtttctgtttctgcccctctttcttctagggggagcactgggcctatgcctggagtcctgtagctactgtcagaagcatttccatcacagctgtctgttgtgggtgatgcaggagctgtggcagtttcatctctttctccattcactatgtgcgtatcaagcaagggttcagaagcttgaatagaagtatctgagctaagagtggcagctttctcctcctcacattccatctggttttgtgctgccattacaccgttggccacacaagtctgtgcaccctgagtcttatctgtatcatttccctgcctctgtggcaagtgctgggagaggagtttttgttgaggtgtggttgtcaatccatgccttcctggggttctaggagcatttaggttcacagcagactctttcttcaaatcactataatttgataatgagcttgtggctttggacttgcagctgagtgttttgctggcctgttcccatttattccctgagcctcttcttcagatacattctcaccaaccagtgtggttgtgctgcttgtggagcaaggtggaactaaagcgatctttggacaggtactgctgcagccccccataaaagattcttttcataacatccagcaatcttctgattaacctatttcctgcttctggagcaaggatttggatccataatttgttggtagaaactataggcattctgtatttagacactagacacatacacatctagtgttcaacatgataaagaactaact

SEQ ID NO: 14947 - RNA, 7328 nt, Homo sapiens
  source 1..7328: mol_type = other RNA
gctgggattacaggcatgagccactatgcccggcctatgcttattttaaaatgtcaattgtcactcacaaaatgaaatgctagtttggttaaaaaaaaaaaagtcttatatacagacagacatgactgttttgctaatgaagagaaccccccacaagtgatacattccaatatccatatactgtgtaatatataatgtgattctcttataatggtccccacagactagtttcttcccaaacctatatgtcactatgtatttggtatttatttattaaagtatgatatgagatttcttgatttacgttttccactaaaactaccacaatgaattttgggaaaaggggttgaccatcatataactcccggtgaccccaacaagttaaaactatcttgtagaagccatgtgctatttcatgtcaaaatacaggaaaagatactgcattctgccaaatgctcagtccagaaagtagaagaccatgattgacttcagattttttttttttttgcctcagtaaacagtacagaaaatgatctgagaatgaaattattttttaaaagcccaaaggagaaaaagaataacaagatatcatagtctagcatttacaggccaaggtcaaaaacctgggtgcaatggatcccatcagcatgtaattacatagattttatatcccttctgcagttaaaatatttcatcttatcttaaaacacattgctgtggtctggagaccagcagtctctcccccacatctctcttcattcttgcttgtttcagtttcttatcttattcctctctgccctttctgtaaagaaagcaaagttatcttctcatgactacgtgattaaggggtatatataaggatgaattatacataaagatccatgtaaataatttatgttaaaatatttaagttaaacaatttcgatagaaaaagttcatttctatggaaagacagaattgcaaatcaacagtgtttttacatatatacatacatgtataaattcacagaaagggttttttaagttgacctagtggtctttatgtatcatagtcattttctaaagctgagaatctatagtagataatagtatgcaaataacaagaagtttgattctaataaaattggtaagaatgaagaagcaacatgatccactacagatgtcaatacagtctgaagaataggaactggttggccacagttcatatactaatacattcttggagaatacaaaatttaagaatgaaaacattaagacattcttgacttttgagttaattttagcttataaatatcatgtgcttaatcttagacccactaacacaaatatcatatgatataggaaatcttcattaatctattctgcattatagcaaagatacctataaaacccaagacgcttgttccctagaagtttacttgctccggttggtgcttgctactcaggttgtatctagtccagaaagatcatcagaaatttatcacagacaatatgctcagattaagaacttaaggctttgaatataaccagaaaacaaataaaagcaaccaccctgtttccaaaaagtaaggacaaggaaaagtaaaacagaattgtgaactcaaaagtatttttgacaaaagtttttagaaggcatcaaagaatctttaacaaccctgcagtaccacaaactttatcgttttctttatatatttataactagaacaagtgttcttaaaaaaaaaaaatccaaacgtgtgcgtatatatatatggggaaagggtacatttaaaaggttagtttctgtaaaaagtttaataatttttaaaaaaattggggtaagttaagtcacctagtgaagataagtacacaaacctgatgtcaaattaaacttcagggaaaacaaaatgtgctttttctatccattttctttgttaaagtaaaaatgttcttgatagttatttaaaatccaaggaatgatgccccttcccatttcccttccttatactctgcaattcgaattaccgtatcacatctagaaagttaataattatctatattcttgtgggaaggggccttcatattaaattttcagtataaaaccataccctaaagagttttattgcttgcatacatgatgacactgtgatgccattattacaaaagtggctggtgttttttattgagccccacttaaaaccaagataaaagtctgcactatatttcatacttaacacgccaaatggtaggctttcagcaaaagcaaaatttaagcttaaaatattgaaatgttttataatgaatagaaattttgtcaaggaagtactttttaaagtttggaggaagggcactttaaagaaaagatgacttggaaagcaccaaatgagtgaaaataaagaattaagacccacagggaacgttggttttaatgggaaagcaaccaatgatatttttaggttgtcatgactgctcaagtatgttggaagggaaaaggcattgattattcttatcatcaatcacactttgaggtctcttggttgaattgtttaataaatggctaagggtattactttacctttcattgagtaaaaacatcagtgattctttaataagagagaagcgggtaaggctgtttcactgcttctctttgcgtttagctgaagaatgtggggtggaaagtgaatatggtgaccggataaccagaaattctcttctagtattaatgcttctcatttaaaaaattaaagataatgactgttaagagcatgataataaacattatctttacatgagtattctttcaatgatctaagttaaataacattgatatttattgagccaaaacttaagtgtgtccatgttacttctgttttggtagggaaagtgtagtcttcttgcttttaaaaatagttttcaaaaataatctgacttataaatcttcccattggcccatacattaccattgttctagtcacacttacaaaagtcctcttccccagttaatcattctgtatttccattgcttctcttttcttgagattaagaaaaccaaagcatcatctatagctacagtttaattttccaaaaaaccactctgagtatacatcacacacataccccgctggccattaaaaaagagaagcaatgtaaattttcttctagtctttccctgatttaatagggcctaagaagctacttttatctctttttggctccatctatttggtttaatgttaatgatcatggctgataatccttttatggaggaagggaacctattatgtcagcaataattggttcacttgctcctttggggtggaaaaaataagatatttcttaaagtaacaaggcctgaataaatgtgtggcagtctcaaattctattctatatctaaggtgtaatccttacatactaaagatagtgggatcattcttgtagatttctagcagactggtacattaaaaagtgacaatgtttggggtatgacagtataaaaaaaggtttaatttgagaaaaaggattaagttaaatagtaaacttagtgtgagattttaatcacaagtacaaaagagtgaagagcagccttcatgacaaggaatcatgtgaccagcccccaccccaaacataggttatcacatgtggattttgtttcattccgacaaaggaaaaggcccatacagttatcttaagtgttcattatatagagaccttatttaaccatgctcgattatcttacggaaaagaaaaacattacgataaatgtggtttccacatatcctagttctgtaaaaggtcaggtgtctcataaagtttgggttttggtgaaaatgtttgtacatgctgatgttaactactgcaataattataggattgtaaacggtaaaataacctgtatgactttgactgtcccagtgaccaaaatgcactttaatcttagaataatcaagactgaagcattaactgaaccctcatcttatattaatagcaccttctaagagaggcactgttttaaataggcacagaaacaaaaaatggtactttaaaagtactgttggaattcacaaatatatcccatgccacataaattaccgcttattataaaaatatcaataccctcaaatgccaatcagcaaaacataaatcaccaaaacatttcttcagtttagaacattgctcaattccacgataaaccatgctttatatttaaaaaataaattagagatgaatgtgaacctaaaagcatgtataatatatatatttaatactatatatacataattgctatatacttaagacattcttaggagtatttctacaaaaacaagttatcttttctttataaatcggaaatctgaacaccaacaatttgtcctttttcttttgttttaaaagaacagacatcatttatgcagctagagatttataaactaaattaaataagttaatacaatagcctcaactgtccctgtatttttcaccatggatctattttggcaacatggaggtatatctttcaaactgttccaggtcctacatgtgaaagagaagaagacatgaaaggatttcttaaatggaagtgctcattctaacctgacggtgacagaatcaattgatacaccatttcttcaagacaaaaaagcacatattcaaggaatagctcaaaaaatgctccagttttcacattatttcaaaactttatcggtagaatgactctgcacactaatttcactaagagtacataaacataggaaaatagtcctcaaaagatgcatttatgggcctatatttttcaacataaagtgctagcagatgtgtaagaagagctgggaatgtcttgagctgtaagtcctgagacctccacaccatggctggtcctggaggagttcagcattctgattttttcttaggttcaggatgatcatccaaggtggctggatgctcatttggaccacctggtgtctcacctgtgacagctaaaaggatgactttcagccacttctgcttcagttcctcactgtctgcagcaaagctgtgcacggacttagactgggtcagtttgaaactgtgtggcaggtctgcgctccttggcatttcatccaccacatagcccagaagtggaatggtggcctgggctctgacgtcctggggggcaccatacatgtacagcacaagagggtcttgcttggggatcacacaccaagctttctgccaaggttttgacttctccatatactgaagaaagctgcacaccacactgtttccagatacttctgctgattcaatctctaaaattccttttcttttcttttcttcactgtctgtgaatccacttatgatttgataacagtctttacaaactttgctcaatttaccaccatcatattcaagttgagctttgtagtcggagcatttccaacaaaccacatatccacatgctcgacaatgatgcctccttcgtgtcagtgcattgaaaggttctttacatttcatacacattgtcacttcattatctcggatccatcttggggctcttttccctagctcagcagtagaaacctctgagtgaatgtcattatcctttgcaattgcatttctgaaggtttcatgcctttgatgaaaagcatcgatggtttcttgaagggccttgatccattcttctttgtcttgcgcagaactggcctgcagttccagtgttctctctttcccagacacctggaaagtatgtggatattcttcattttgagtctctacaattttcattccatcaatgccaaccctggttcgaactgtgaatttagagcctaccaagctgaatttgggcacacagtacagcaacatgttgttgaataagaaaaggtagcgttcttgtgctgaagtgttccgagcagctagtttgaggatctgtccttcttttattagttcatttgaagggtttacaatgtcttcttcttctcccaacatttcataaatctctaagagtttctttaggttctccattttccttattgcactattagaatggcttgctgctgtagatataatttcaagtgattttttagcatcattccagtccagggaatcaggaggcaatttccttagatagtccttaaggagcatctcataccggggaatccgctgaacaggttctagcatgtgatgctgcaaagttaagctcccacagattttctgtttctgaatttcttcaaccactgatttgaactggggaatacgttctgtcatgtttttaaccaattccattgcattatcaaatcctttcacatattctccatacatcttaaggaatggtgccaatttctgaaggatgtctccaattctaggagtagtttcccattcttgcattcgtttctccagctctggcaagaggaatttactatggaaggcatttattgatgaaatattagaaaagattttattcaccatctctgctggaaacgagcctcggtttgcttcttccaacagtttgcaataaaatacctgatctaagaggtcaagtcggttgacataagctctttcagtaagcaaaagttcattggctattttgtgaagtttttgctcattagtctccttcatctcatggtgctggtccagctgctccagttccagagggctttccccattttccctctcttgtaccttggtttctgtttctgcccctctttcttctagggggagcactgggcctatgcctggagtcctgtagctactgtcagaagcatttccatcacagctgtctgttgtgggtgatgcaggagctgtggcagtttcatctctttctccattcactatgtgcgtatcaagcaagggttcagaagcttgaatagaagtatctgagctaagagtggcagctttctcctcctcacattccatctggttttgtgctgccattacaccgttggccacacaagtctgtgcaccctgagtcttatctgtatcatttccctgcctctgtggcaagtgctgggagaggagtttttgttgaggtgtggttgtcaatccatgccttcctggggttctaggagcatttaggttcacagcagactctttcttcaaatcactataatttgataatgagcttgtggctttggacttgcagctgagtgttttgctggcctgttcccatttattccctgagcctcttcttcagatacattctcaccaaccagtgtggttgtgctgcttgtggagcaaggtggaactaaagcgatctttggacaggtactgctgcctgtggctcctgagggcacctggcccttgaaggcagcggtccctacacgtcccaggtgcgacgcgggcctgctccagggccggggcaccccgggcggcaggtag

SEQ ID NO: 14948 - RNA, 7400 nt, Homo sapiens
  source 1..7400: mol_type = other RNA
gctgggattacaggcatgagccactatgcccggcctatgcttattttaaaatgtcaattgtcactcacaaaatgaaatgctagtttggttaaaaaaaaaaaagtcttatatacagacagacatgactgttttgctaatgaagagaaccccccacaagtgatacattccaatatccatatactgtgtaatatataatgtgattctcttataatggtccccacagactagtttcttcccaaacctatatgtcactatgtatttggtatttatttattaaagtatgatatgagatttcttgatttacgttttccactaaaactaccacaatgaattttgggaaaaggggttgaccatcatataactcccggtgaccccaacaagttaaaactatcttgtagaagccatgtgctatttcatgtcaaaatacaggaaaagatactgcattctgccaaatgctcagtccagaaagtagaagaccatgattgacttcagattttttttttttttgcctcagtaaacagtacagaaaatgatctgagaatgaaattattttttaaaagcccaaaggagaaaaagaataacaagatatcatagtctagcatttacaggccaaggtcaaaaacctgggtgcaatggatcccatcagcatgtaattacatagattttatatcccttctgcagttaaaatatttcatcttatcttaaaacacattgctgtggtctggagaccagcagtctctcccccacatctctcttcattcttgcttgtttcagtttcttatcttattcctctctgccctttctgtaaagaaagcaaagttatcttctcatgactacgtgattaaggggtatatataaggatgaattatacataaagatccatgtaaataatttatgttaaaatatttaagttaaacaatttcgatagaaaaagttcatttctatggaaagacagaattgcaaatcaacagtgtttttacatatatacatacatgtataaattcacagaaagggttttttaagttgacctagtggtctttatgtatcatagtcattttctaaagctgagaatctatagtagataatagtatgcaaataacaagaagtttgattctaataaaattggtaagaatgaagaagcaacatgatccactacagatgtcaatacagtctgaagaataggaactggttggccacagttcatatactaatacattcttggagaatacaaaatttaagaatgaaaacattaagacattcttgacttttgagttaattttagcttataaatatcatgtgcttaatcttagacccactaacacaaatatcatatgatataggaaatcttcattaatctattctgcattatagcaaagatacctataaaacccaagacgcttgttccctagaagtttacttgctccggttggtgcttgctactcaggttgtatctagtccagaaagatcatcagaaatttatcacagacaatatgctcagattaagaacttaaggctttgaatataaccagaaaacaaataaaagcaaccaccctgtttccaaaaagtaaggacaaggaaaagtaaaacagaattgtgaactcaaaagtatttttgacaaaagtttttagaaggcatcaaagaatctttaacaaccctgcagtaccacaaactttatcgttttctttatatatttataactagaacaagtgttcttaaaaaaaaaaaatccaaacgtgtgcgtatatatatatggggaaagggtacatttaaaaggttagtttctgtaaaaagtttaataatttttaaaaaaattggggtaagttaagtcacctagtgaagataagtacacaaacctgatgtcaaattaaacttcagggaaaacaaaatgtgctttttctatccattttctttgttaaagtaaaaatgttcttgatagttatttaaaatccaaggaatgatgccccttcccatttcccttccttatactctgcaattcgaattaccgtatcacatctagaaagttaataattatctatattcttgtgggaaggggccttcatattaaattttcagtataaaaccataccctaaagagttttattgcttgcatacatgatgacactgtgatgccattattacaaaagtggctggtgttttttattgagccccacttaaaaccaagataaaagtctgcactatatttcatacttaacacgccaaatggtaggctttcagcaaaagcaaaatttaagcttaaaatattgaaatgttttataatgaatagaaattttgtcaaggaagtactttttaaagtttggaggaagggcactttaaagaaaagatgacttggaaagcaccaaatgagtgaaaataaagaattaagacccacagggaacgttggttttaatgggaaagcaaccaatgatatttttaggttgtcatgactgctcaagtatgttggaagggaaaaggcattgattattcttatcatcaatcacactttgaggtctcttggttgaattgtttaataaatggctaagggtattactttacctttcattgagtaaaaacatcagtgattctttaataagagagaagcgggtaaggctgtttcactgcttctctttgcgtttagctgaagaatgtggggtggaaagtgaatatggtgaccggataaccagaaattctcttctagtattaatgcttctcatttaaaaaattaaagataatgactgttaagagcatgataataaacattatctttacatgagtattctttcaatgatctaagttaaataacattgatatttattgagccaaaacttaagtgtgtccatgttacttctgttttggtagggaaagtgtagtcttcttgcttttaaaaatagttttcaaaaataatctgacttataaatcttcccattggcccatacattaccattgttctagtcacacttacaaaagtcctcttccccagttaatcattctgtatttccattgcttctcttttcttgagattaagaaaaccaaagcatcatctatagctacagtttaattttccaaaaaaccactctgagtatacatcacacacataccccgctggccattaaaaaagagaagcaatgtaaattttcttctagtctttccctgatttaatagggcctaagaagctacttttatctctttttggctccatctatttggtttaatgttaatgatcatggctgataatccttttatggaggaagggaacctattatgtcagcaataattggttcacttgctcctttggggtggaaaaaataagatatttcttaaagtaacaaggcctgaataaatgtgtggcagtctcaaattctattctatatctaaggtgtaatccttacatactaaagatagtgggatcattcttgtagatttctagcagactggtacattaaaaagtgacaatgtttggggtatgacagtataaaaaaaggtttaatttgagaaaaaggattaagttaaatagtaaacttagtgtgagattttaatcacaagtacaaaagagtgaagagcagccttcatgacaaggaatcatgtgaccagcccccaccccaaacataggttatcacatgtggattttgtttcattccgacaaaggaaaaggcccatacagttatcttaagtgttcattatatagagaccttatttaaccatgctcgattatcttacggaaaagaaaaacattacgataaatgtggtttccacatatcctagttctgtaaaaggtcaggtgtctcataaagtttgggttttggtgaaaatgtttgtacatgctgatgttaactactgcaataattataggattgtaaacggtaaaataacctgtatgactttgactgtcccagtgaccaaaatgcactttaatcttagaataatcaagactgaagcattaactgaaccctcatcttatattaatagcaccttctaagagaggcactgttttaaataggcacagaaacaaaaaatggtactttaaaagtactgttggaattcacaaatatatcccatgccacataaattaccgcttattataaaaatatcaataccctcaaatgccaatcagcaaaacataaatcaccaaaacatttcttcagtttagaacattgctcaattccacgataaaccatgctttatatttaaaaaataaattagagatgaatgtgaacctaaaagcatgtataatatatatatttaatactatatatacataattgctatatacttaagacattcttaggagtatttctacaaaaacaagttatcttttctttataaatcggaaatctgaacaccaacaatttgtcctttttcttttgttttaaaagaacagacatcatttatgcagctagagatttataaactaaattaaataagttaatacaatagcctcaactgtccctgtatttttcaccatggatctattttggcaacatggaggtatatctttcaaactgttccaggtcctacatgtgaaagagaagaagacatgaaaggatttcttaaatggaagtgctcattctaacctgacggtgacagaatcaattgatacaccatttcttcaagacaaaaaagcacatattcaaggaatagctcaaaaaatgctccagttttcacattatttcaaaactttatcggtagaatgactctgcacactaatttcactaagagtacataaacataggaaaatagtcctcaaaagatgcatttatgggcctatatttttcaacataaagtgctagcagatgtgtaagaagagctgggaatgtcttgagctgtaagtcctgagacctccacaccatggctggtcctggaggagttcagcattctgattttttcttaggttcaggatgatcatccaaggtggctggatgctcatttggaccacctggtgtctcacctgtgacagctaaaaggatgactttcagccacttctgcttcagttcctcactgtctgcagcaaagctgtgcacggacttagactgggtcagtttgaaactgtgtggcaggtctgcgctccttggcatttcatccaccacatagcccagaagtggaatggtggcctgggctctgacgtcctggggggcaccatacatgtacagcacaagagggtcttgcttggggatcacacaccaagctttctgccaaggttttgacttctccatatactgaagaaagctgcacaccacactgtttccagatacttctgctgattcaatctctaaaattccttttcttttcttttcttcactgtctgtgaatccacttatgatttgataacagtctttacaaactttgctcaatttaccaccatcatattcaagttgagctttgtagtcggagcatttccaacaaaccacatatccacatgctcgacaatgatgcctccttcgtgtcagtgcattgaaaggttctttacatttcatacacattgtcacttcattatctcggatccatcttggggctcttttccctagctcagcagtagaaacctctgagtgaatgtcattatcctttgcaattgcatttctgaaggtttcatgcctttgatgaaaagcatcgatggtttcttgaagggccttgatccattcttctttgtcttgcgcagaactggcctgcagttccagtgttctctctttcccagacacctggaaagtatgtggatattcttcattttgagtctctacaattttcattccatcaatgccaaccctggttcgaactgtgaatttagagcctaccaagctgaatttgggcacacagtacagcaacatgttgttgaataagaaaaggtagcgttcttgtgctgaagtgttccgagcagctagtttgaggatctgtccttcttttattagttcatttgaagggtttacaatgtcttcttcttctcccaacatttcataaatctctaagagtttctttaggttctccattttccttattgcactattagaatggcttgctgctgtagatataatttcaagtgattttttagcatcattccagtccagggaatcaggaggcaatttccttagatagtccttaaggagcatctcataccggggaatccgctgaacaggttctagcatgtgatgctgcaaagttaagctcccacagattttctgtttctgaatttcttcaaccactgatttgaactggggaatacgttctgtcatgtttttaaccaattccattgcattatcaaatcctttcacatattctccatacatcttaaggaatggtgccaatttctgaaggatgtctccaattctaggagtagtttcccattcttgcattcgtttctccagctctggcaagaggaatttactatggaaggcatttattgatgaaatattagaaaagattttattcaccatctctgctggaaacgagcctcggtttgcttcttccaacagtttgcaataaaatacctgatctaagaggtcaagtcggttgacataagctctttcagtaagcaaaagttcattggctattttgtgaagtttttgctcattagtctccttcatctcatggtgctggtccagctgctccagttccagagggctttccccattttccctctcttgtaccttggtttctgtttctgcccctctttcttctagggggagcactgggcctatgcctggagtcctgtagctactgtcagaagcatttccatcacagctgtctgttgtgggtgatgcaggagctgtggcagtttcatctctttctccattcactatgtgcgtatcaagcaagggttcagaagcttgaatagaagtatctgagctaagagtggcagctttctcctcctcacattccatctggttttgtgctgccattacaccgttggccacacaagtctgtgcaccctgagtcttatctgtatcatttccctgcctctgtggcaagtgctgggagaggagtttttgttgaggtgtggttgtcaatccatgccttcctggggttctaggagcatttaggttcacagcagactctttcttcaaatcactataatttgataatgagcttgtggctttggacttgcagctgagtgttttgctggcctgttcccatttattccctgagcctcttcttcagatacattctcaccaaccagtgtggttgtgctgcttgtggagcaaggtggaactaaagcgatctttggacaggtactgctgccttataaaagctgaatttattcctcttggccagaagtcacaaatggttgaagtaaaactcccttcatttgttcttccagcgagccaaagcaagcctcccattaacccggtccattgcagataatctcacccagcacaggctcccctgctttccccacttcccagcccagcaaggat

SEQ ID NO: 14949 - RNA, 7401 nt, Homo sapiens
  source 1..7401: mol_type = other RNA
gctgggattacaggcatgagccactatgcccggcctatgcttattttaaaatgtcaattgtcactcacaaaatgaaatgctagtttggttaaaaaaaaaaaagtcttatatacagacagacatgactgttttgctaatgaagagaaccccccacaagtgatacattccaatatccatatactgtgtaatatataatgtgattctcttataatggtccccacagactagtttcttcccaaacctatatgtcactatgtatttggtatttatttattaaagtatgatatgagatttcttgatttacgttttccactaaaactaccacaatgaattttgggaaaaggggttgaccatcatataactcccggtgaccccaacaagttaaaactatcttgtagaagccatgtgctatttcatgtcaaaatacaggaaaagatactgcattctgccaaatgctcagtccagaaagtagaagaccatgattgacttcagattttttttttttttgcctcagtaaacagtacagaaaatgatctgagaatgaaattattttttaaaagcccaaaggagaaaaagaataacaagatatcatagtctagcatttacaggccaaggtcaaaaacctgggtgcaatggatcccatcagcatgtaattacatagattttatatcccttctgcagttaaaatatttcatcttatcttaaaacacattgctgtggtctggagaccagcagtctctcccccacatctctcttcattcttgcttgtttcagtttcttatcttattcctctctgccctttctgtaaagaaagcaaagttatcttctcatgactacgtgattaaggggtatatataaggatgaattatacataaagatccatgtaaataatttatgttaaaatatttaagttaaacaatttcgatagaaaaagttcatttctatggaaagacagaattgcaaatcaacagtgtttttacatatatacatacatgtataaattcacagaaagggttttttaagttgacctagtggtctttatgtatcatagtcattttctaaagctgagaatctatagtagataatagtatgcaaataacaagaagtttgattctaataaaattggtaagaatgaagaagcaacatgatccactacagatgtcaatacagtctgaagaataggaactggttggccacagttcatatactaatacattcttggagaatacaaaatttaagaatgaaaacattaagacattcttgacttttgagttaattttagcttataaatatcatgtgcttaatcttagacccactaacacaaatatcatatgatataggaaatcttcattaatctattctgcattatagcaaagatacctataaaacccaagacgcttgttccctagaagtttacttgctccggttggtgcttgctactcaggttgtatctagtccagaaagatcatcagaaatttatcacagacaatatgctcagattaagaacttaaggctttgaatataaccagaaaacaaataaaagcaaccaccctgtttccaaaaagtaaggacaaggaaaagtaaaacagaattgtgaactcaaaagtatttttgacaaaagtttttagaaggcatcaaagaatctttaacaaccctgcagtaccacaaactttatcgttttctttatatatttataactagaacaagtgttcttaaaaaaaaaaaatccaaacgtgtgcgtatatatatatggggaaagggtacatttaaaaggttagtttctgtaaaaagtttaataatttttaaaaaaattggggtaagttaagtcacctagtgaagataagtacacaaacctgatgtcaaattaaacttcagggaaaacaaaatgtgctttttctatccattttctttgttaaagtaaaaatgttcttgatagttatttaaaatccaaggaatgatgccccttcccatttcccttccttatactctgcaattcgaattaccgtatcacatctagaaagttaataattatctatattcttgtgggaaggggccttcatattaaattttcagtataaaaccataccctaaagagttttattgcttgcatacatgatgacactgtgatgccattattacaaaagtggctggtgttttttattgagccccacttaaaaccaagataaaagtctgcactatatttcatacttaacacgccaaatggtaggctttcagcaaaagcaaaatttaagcttaaaatattgaaatgttttataatgaatagaaattttgtcaaggaagtactttttaaagtttggaggaagggcactttaaagaaaagatgacttggaaagcaccaaatgagtgaaaataaagaattaagacccacagggaacgttggttttaatgggaaagcaaccaatgatatttttaggttgtcatgactgctcaagtatgttggaagggaaaaggcattgattattcttatcatcaatcacactttgaggtctcttggttgaattgtttaataaatggctaagggtattactttacctttcattgagtaaaaacatcagtgattctttaataagagagaagcgggtaaggctgtttcactgcttctctttgcgtttagctgaagaatgtggggtggaaagtgaatatggtgaccggataaccagaaattctcttctagtattaatgcttctcatttaaaaaattaaagataatgactgttaagagcatgataataaacattatctttacatgagtattctttcaatgatctaagttaaataacattgatatttattgagccaaaacttaagtgtgtccatgttacttctgttttggtagggaaagtgtagtcttcttgcttttaaaaatagttttcaaaaataatctgacttataaatcttcccattggcccatacattaccattgttctagtcacacttacaaaagtcctcttccccagttaatcattctgtatttccattgcttctcttttcttgagattaagaaaaccaaagcatcatctatagctacagtttaattttccaaaaaaccactctgagtatacatcacacacataccccgctggccattaaaaaagagaagcaatgtaaattttcttctagtctttccctgatttaatagggcctaagaagctacttttatctctttttggctccatctatttggtttaatgttaatgatcatggctgataatccttttatggaggaagggaacctattatgtcagcaataattggttcacttgctcctttggggtggaaaaaataagatatttcttaaagtaacaaggcctgaataaatgtgtggcagtctcaaattctattctatatctaaggtgtaatccttacatactaaagatagtgggatcattcttgtagatttctagcagactggtacattaaaaagtgacaatgtttggggtatgacagtataaaaaaaggtttaatttgagaaaaaggattaagttaaatagtaaacttagtgtgagattttaatcacaagtacaaaagagtgaagagcagccttcatgacaaggaatcatgtgaccagcccccaccccaaacataggttatcacatgtggattttgtttcattccgacaaaggaaaaggcccatacagttatcttaagtgttcattatatagagaccttatttaaccatgctcgattatcttacggaaaagaaaaacattacgataaatgtggtttccacatatcctagttctgtaaaaggtcaggtgtctcataaagtttgggttttggtgaaaatgtttgtacatgctgatgttaactactgcaataattataggattgtaaacggtaaaataacctgtatgactttgactgtcccagtgaccaaaatgcactttaatcttagaataatcaagactgaagcattaactgaaccctcatcttatattaatagcaccttctaagagaggcactgttttaaataggcacagaaacaaaaaatggtactttaaaagtactgttggaattcacaaatatatcccatgccacataaattaccgcttattataaaaatatcaataccctcaaatgccaatcagcaaaacataaatcaccaaaacatttcttcagtttagaacattgctcaattccacgataaaccatgctttatatttaaaaaataaattagagatgaatgtgaacctaaaagcatgtataatatatatatttaatactatatatacataattgctatatacttaagacattcttaggagtatttctacaaaaacaagttatcttttctttataaatcggaaatctgaacaccaacaatttgtcctttttcttttgttttaaaagaacagacatcatttatgcagctagagatttataaactaaattaaataagttaatacaatagcctcaactgtccctgtatttttcaccatggatctattttggcaacatggaggtatatctttcaaactgttccaggtcctacatgtgaaagagaagaagacatgaaaggatttcttaaatggaagtgctcattctaacctgacggtgacagaatcaattgatacaccatttcttcaagacaaaaaagcacatattcaaggaatagctcaaaaaatgctccagttttcacattatttcaaaactttatcggtagaatgactctgcacactaatttcactaagagtacataaacataggaaaatagtcctcaaaagatgcatttatgggcctatatttttcaacataaagtgctagcagatgtgtaagaagagctgggaatgtcttgagctgtaagtcctgagacctccacaccatggctggtcctggaggagttcagcattctgattttttcttaggttcaggatgatcatccaaggtggctggatgctcatttggaccacctggtgtctcacctgtgacagctaaaaggatgactttcagccacttctgcttcagttcctcactgtctgcagcaaagctgtgcacggacttagactgggtcagtttgaaactgtgtggcaggtctgcgctccttggcatttcatccaccacatagcccagaagtggaatggtggcctgggctctgacgtcctggggggcaccatacatgtacagcacaagagggtcttgcttggggatcacacaccaagctttctgccaaggttttgacttctccatatactgaagaaagctgcacaccacactgtttccagatacttctgctgattcaatctctaaaattccttttcttttcttttcttcactgtctgtgaatccacttatgatttgataacagtctttacaaactttgctcaatttaccaccatcatattcaagttgagctttgtagtcggagcatttccaacaaaccacatatccacatgctcgacaatgatgcctccttcgtgtcagtgcattgaaaggttctttacatttcatacacattgtcacttcattatctcggatccatcttggggctcttttccctagctcagcagtagaaacctctgagtgaatgtcattatcctttgcaattgcatttctgaaggtttcatgcctttgatgaaaagcatcgatggtttcttgaagggccttgatccattcttctttgtcttgcgcagaactggcctgcagttccagtgttctctctttcccagacacctggaaagtatgtggatattcttcattttgagtctctacaattttcattccatcaatgccaaccctggttcgaactgtgaatttagagcctaccaagctgaatttgggcacacagtacagcaacatgttgttgaataagaaaaggtagcgttcttgtgctgaagtgttccgagcagctagtttgaggatctgtccttcttttattagttcatttgaagggtttacaatgtcttcttcttctcccaacatttcataaatctctaagagtttctttaggttctccattttccttattgcactattagaatggcttgctgctgtagatataatttcaagtgattttttagcatcattccagtccagggaatcaggaggcaatttccttagatagtccttaaggagcatctcataccggggaatccgctgaacaggttctagcatgtgatgctgcaaagttaagctcccacagattttctgtttctgaatttcttcaaccactgatttgaactggggaatacgttctgtcatgtttttaaccaattccattgcattatcaaatcctttcacatattctccatacatcttaaggaatggtgccaatttctgaaggatgtctccaattctaggagtagtttcccattcttgcattcgtttctccagctctggcaagaggaatttactatggaaggcatttattgatgaaatattagaaaagattttattcaccatctctgctggaaacgagcctcggtttgcttcttccaacagtttgcaataaaatacctgatctaagaggtcaagtcggttgacataagctctttcagtaagcaaaagttcattggctattttgtgaagtttttgctcattagtctccttcatctcatggtgctggtccagctgctccagttccagagggctttccccattttccctctcttgtaccttggtttctgtttctgcccctctttcttctagggggagcactgggcctatgcctggagtcctgtagctactgtcagaagcatttccatcacagctgtctgttgtgggtgatgcaggagctgtggcagtttcatctctttctccattcactatgtgcgtatcaagcaagggttcagaagcttgaatagaagtatctgagctaagagtggcagctttctcctcctcacattccatctggttttgtgctgccattacaccgttggccacacaagtctgtgcaccctgagtcttatctgtatcatttccctgcctctgtggcaagtgctgggagaggagtttttgttgaggtgtggttgtcaatccatgccttcctggggttctaggagcatttaggttcacagcagactctttcttcaaatcactataatttgataatgagcttgtggctttggacttgcagctgagtgttttgctggcctgttcccatttattccctgagcctcttcttcagatacattctcaccaaccagtgtggttgtgctgcttgtggagcaaggtggaactaaagcgatctttggacaggtactgctgccttgatcagtggacatgatttcacatatactgataattaatctactctggtttaataaaaagatatttggctttactcttttaaagttcatgtgataaaatctcactcctggctgtaaagcttcagggaggctgaagattacacaggatctgccaggagctcagaccaatgcactat

SEQ ID NO: 14950 - RNA, 8109 nt, Homo sapiens
  source 1..8109: mol_type = other RNA
gctgggattacaggcatgagccactatgcccggcctatgcttattttaaaatgtcaattgtcactcacaaaatgaaatgctagtttggttaaaaaaaaaaaagtcttatatacagacagacatgactgttttgctaatgaagagaaccccccacaagtgatacattccaatatccatatactgtgtaatatataatgtgattctcttataatggtccccacagactagtttcttcccaaacctatatgtcactatgtatttggtatttatttattaaagtatgatatgagatttcttgatttacgttttccactaaaactaccacaatgaattttgggaaaaggggttgaccatcatataactcccggtgaccccaacaagttaaaactatcttgtagaagccatgtgctatttcatgtcaaaatacaggaaaagatactgcattctgccaaatgctcagtccagaaagtagaagaccatgattgacttcagattttttttttttttgcctcagtaaacagtacagaaaatgatctgagaatgaaattattttttaaaagcccaaaggagaaaaagaataacaagatatcatagtctagcatttacaggccaaggtcaaaaacctgggtgcaatggatcccatcagcatgtaattacatagattttatatcccttctgcagttaaaatatttcatcttatcttaaaacacattgctgtggtctggagaccagcagtctctcccccacatctctcttcattcttgcttgtttcagtttcttatcttattcctctctgccctttctgtaaagaaagcaaagttatcttctcatgactacgtgattaaggggtatatataaggatgaattatacataaagatccatgtaaataatttatgttaaaatatttaagttaaacaatttcgatagaaaaagttcatttctatggaaagacagaattgcaaatcaacagtgtttttacatatatacatacatgtataaattcacagaaagggttttttaagttgacctagtggtctttatgtatcatagtcattttctaaagctgagaatctatagtagataatagtatgcaaataacaagaagtttgattctaataaaattggtaagaatgaagaagcaacatgatccactacagatgtcaatacagtctgaagaataggaactggttggccacagttcatatactaatacattcttggagaatacaaaatttaagaatgaaaacattaagacattcttgacttttgagttaattttagcttataaatatcatgtgcttaatcttagacccactaacacaaatatcatatgatataggaaatcttcattaatctattctgcattatagcaaagatacctataaaacccaagacgcttgttccctagaagtttacttgctccggttggtgcttgctactcaggttgtatctagtccagaaagatcatcagaaatttatcacagacaatatgctcagattaagaacttaaggctttgaatataaccagaaaacaaataaaagcaaccaccctgtttccaaaaagtaaggacaaggaaaagtaaaacagaattgtgaactcaaaagtatttttgacaaaagtttttagaaggcatcaaagaatctttaacaaccctgcagtaccacaaactttatcgttttctttatatatttataactagaacaagtgttcttaaaaaaaaaaaatccaaacgtgtgcgtatatatatatggggaaagggtacatttaaaaggttagtttctgtaaaaagtttaataatttttaaaaaaattggggtaagttaagtcacctagtgaagataagtacacaaacctgatgtcaaattaaacttcagggaaaacaaaatgtgctttttctatccattttctttgttaaagtaaaaatgttcttgatagttatttaaaatccaaggaatgatgccccttcccatttcccttccttatactctgcaattcgaattaccgtatcacatctagaaagttaataattatctatattcttgtgggaaggggccttcatattaaattttcagtataaaaccataccctaaagagttttattgcttgcatacatgatgacactgtgatgccattattacaaaagtggctggtgttttttattgagccccacttaaaaccaagataaaagtctgcactatatttcatacttaacacgccaaatggtaggctttcagcaaaagcaaaatttaagcttaaaatattgaaatgttttataatgaatagaaattttgtcaaggaagtactttttaaagtttggaggaagggcactttaaagaaaagatgacttggaaagcaccaaatgagtgaaaataaagaattaagacccacagggaacgttggttttaatgggaaagcaaccaatgatatttttaggttgtcatgactgctcaagtatgttggaagggaaaaggcattgattattcttatcatcaatcacactttgaggtctcttggttgaattgtttaataaatggctaagggtattactttacctttcattgagtaaaaacatcagtgattctttaataagagagaagcgggtaaggctgtttcactgcttctctttgcgtttagctgaagaatgtggggtggaaagtgaatatggtgaccggataaccagaaattctcttctagtattaatgcttctcatttaaaaaattaaagataatgactgttaagagcatgataataaacattatctttacatgagtattctttcaatgatctaagttaaataacattgatatttattgagccaaaacttaagtgtgtccatgttacttctgttttggtagggaaagtgtagtcttcttgcttttaaaaatagttttcaaaaataatctgacttataaatcttcccattggcccatacattaccattgttctagtcacacttacaaaagtcctcttccccagttaatcattctgtatttccattgcttctcttttcttgagattaagaaaaccaaagcatcatctatagctacagtttaattttccaaaaaaccactctgagtatacatcacacacataccccgctggccattaaaaaagagaagcaatgtaaattttcttctagtctttccctgatttaatagggcctaagaagctacttttatctctttttggctccatctatttggtttaatgttaatgatcatggctgataatccttttatggaggaagggaacctattatgtcagcaataattggttcacttgctcctttggggtggaaaaaataagatatttcttaaagtaacaaggcctgaataaatgtgtggcagtctcaaattctattctatatctaaggtgtaatccttacatactaaagatagtgggatcattcttgtagatttctagcagactggtacattaaaaagtgacaatgtttggggtatgacagtataaaaaaaggtttaatttgagaaaaaggattaagttaaatagtaaacttagtgtgagattttaatcacaagtacaaaagagtgaagagcagccttcatgacaaggaatcatgtgaccagcccccaccccaaacataggttatcacatgtggattttgtttcattccgacaaaggaaaaggcccatacagttatcttaagtgttcattatatagagaccttatttaaccatgctcgattatcttacggaaaagaaaaacattacgataaatgtggtttccacatatcctagttctgtaaaaggtcaggtgtctcataaagtttgggttttggtgaaaatgtttgtacatgctgatgttaactactgcaataattataggattgtaaacggtaaaataacctgtatgactttgactgtcccagtgaccaaaatgcactttaatcttagaataatcaagactgaagcattaactgaaccctcatcttatattaatagcaccttctaagagaggcactgttttaaataggcacagaaacaaaaaatggtactttaaaagtactgttggaattcacaaatatatcccatgccacataaattaccgcttattataaaaatatcaataccctcaaatgccaatcagcaaaacataaatcaccaaaacatttcttcagtttagaacattgctcaattccacgataaaccatgctttatatttaaaaaataaattagagatgaatgtgaacctaaaagcatgtataatatatatatttaatactatatatacataattgctatatacttaagacattcttaggagtatttctacaaaaacaagttatcttttctttataaatcggaaatctgaacaccaacaatttgtcctttttcttttgttttaaaagaacagacatcatttatgcagctagagatttataaactaaattaaataagttaatacaatagcctcaactgtccctgtatttttcaccatggatctattttggcaacatggaggtatatctttcaaactgttccaggtcctacatgtgaaagagaagaagacatgaaaggatttcttaaatggaagtgctcattctaacctgacggtgacagaatcaattgatacaccatttcttcaagacaaaaaagcacatattcaaggaatagctcaaaaaatgctccagttttcacattatttcaaaactttatcggtagaatgactctgcacactaatttcactaagagtacataaacataggaaaatagtcctcaaaagatgcatttatgggcctatatttttcaacataaagtgctagcagatgtgtaagaagagctgggaatgtcttgagctgtaagtcctgagacctccacaccatggctggtcctggaggagttcagcattctgattttttcttaggttcaggatgatcatccaaggtggctggatgctcatttggaccacctggtgtctcacctgtgacagctaaaaggatgactttcagccacttctgcttcagttcctcactgtctgcagcaaagctgtgcacggacttagactgggtcagtttgaaactgtgtggcaggtctgcgctccttggcatttcatccaccacatagcccagaagtggaatggtggcctgggctctgacgtcctggggggcaccatacatgtacagcacaagagggtcttgcttggggatcacacaccaagctttctgccaaggttttgacttctccatatactgaagaaagctgcacaccacactgtttccagatacttctgctgattcaatctctaaaattccttttcttttcttttcttcactgtctgtgaatccacttatgatttgataacagtctttacaaactttgctcaatttaccaccatcatattcaagttgagctttgtagtcggagcatttccaacaaaccacatatccacatgctcgacaatgatgcctccttcgtgtcagtgcattgaaaggttctttacatttcatacacattgtcacttcattatctcggatccatcttggggctcttttccctagctcagcagtagaaacctctgagtgaatgtcattatcctttgcaattgcatttctgaaggtttcatgcctttgatgaaaagcatcgatggtttcttgaagggccttgatccattcttctttgtcttgcgcagaactggcctgcagttccagtgttctctctttcccagacacctggaaagtatgtggatattcttcattttgagtctctacaattttcattccatcaatgccaaccctggttcgaactgtgaatttagagcctaccaagctgaatttgggcacacagtacagcaacatgttgttgaataagaaaaggtagcgttcttgtgctgaagtgttccgagcagctagtttgaggatctgtccttcttttattagttcatttgaagggtttacaatgtcttcttcttctcccaacatttcataaatctctaagagtttctttaggttctccattttccttattgcactattagaatggcttgctgctgtagatataatttcaagtgattttttagcatcattccagtccagggaatcaggaggcaatttccttagatagtccttaaggagcatctcataccggggaatccgctgaacaggttctagcatgtgatgctgcaaagttaagctcccacagattttctgtttctgaatttcttcaaccactgatttgaactggggaatacgttctgtcatgtttttaaccaattccattgcattatcaaatcctttcacatattctccatacatcttaaggaatggtgccaatttctgaaggatgtctccaattctaggagtagtttcccattcttgcattcgtttctccagctctggcaagaggaatttactatggaaggcatttattgatgaaatattagaaaagattttattcaccatctctgctggaaacgagcctcggtttgcttcttccaacagtttgcaataaaatacctgatctaagaggtcaagtcggttgacataagctctttcagtaagcaaaagttcattggctattttgtgaagtttttgctcattagtctccttcatctcatggtgctggtccagctgctccagttccagagggctttccccattttccctctcttgtaccttggtttctgtttctgcccctctttcttctagggggagcactgggcctatgcctggagtcctgtagctactgtcagaagcatttccatcacagctgtctgttgtgggtgatgcaggagctgtggcagtttcatctctttctccattcactatgtgcgtatcaagcaagggttcagaagcttgaatagaagtatctgagctaagagtggcagctttctcctcctcacattccatctggttttgtgctgccattacaccgttggccacacaagtctgtgcaccctgagtcttatctgtatcatttccctgcctctgtggcaagtgctgggagaggagtttttgttgaggtgtggttgtcaatccatgccttcctggggttctaggagcatttaggttcacagcagactctttcttcaaatcactataatttgataatgagcttgtttcatcctcacaataattccaaagacagggatcccatagagaaatctaggcttagaaattaaggtggccaatgtcacaatgtaacaagcagaaaagccagaggtcaaaccatgaatccaactctaaatcccatggtcttcaccccaagttatgatgtactggagcagaaggacagaatgagcatcagatgaataggtcttcagttgagatttgcccccttgaggaggacaactttggcctggataatttcccaagtagtctttagagatttgaatcaaactgtcctccttctcctgcccacatcagtctctggattccctggtggaaagatcctcaacagatcctctgcctccttcaaagcgactgatgagatctgataccttactgggtttttcttttgagacacaagaagcagaggcaggtttaatttcctccatccttggttttgcactaggtaaagctttatgcctgggggtttggtgtatattggacgaaggtgaattctgcaggtgtaatggctttggaggcacttctggaagaagggtgaggagtcatgtcgcctcctaattacatgcctcattttcccccagctggttcccctggtttttagtgatctcatctcttttataaactcagttagctgacagttggctcatgctcactggcctagatcttgtggctttggacttgcagctgagtgttttgctggcctgttcccatttattccctgagcctcttcttcagatacattctcaccaaccagtgtggttgtgctgcttgtggagcaaggtggaactaaagcgatctttggacaggtactgctgccttataaaagctgaatttattcctcttggccagaagtcacaaatggttgaagtaaaactcccttcatttgttcttccagcgagccaaagcaagcctcccattaacccggtccattgcagataatctcacccagcacaggctcccctgctttccccacttcccagcccagcaaggataatcacattccggtggggagtgaacagatggt

SEQ ID NO: 14951 - RNA, 7976 nt, Homo sapiens
  source 1..7976: mol_type = other RNA
gctgggattacaggcatgagccactatgcccggcctatgcttattttaaaatgtcaattgtcactcacaaaatgaaatgctagtttggttaaaaaaaaaaaagtcttatatacagacagacatgactgttttgctaatgaagagaaccccccacaagtgatacattccaatatccatatactgtgtaatatataatgtgattctcttataatggtccccacagactagtttcttcccaaacctatatgtcactatgtatttggtatttatttattaaagtatgatatgagatttcttgatttacgttttccactaaaactaccacaatgaattttgggaaaaggggttgaccatcatataactcccggtgaccccaacaagttaaaactatcttgtagaagccatgtgctatttcatgtcaaaatacaggaaaagatactgcattctgccaaatgctcagtccagaaagtagaagaccatgattgacttcagattttttttttttttgcctcagtaaacagtacagaaaatgatctgagaatgaaattattttttaaaagcccaaaggagaaaaagaataacaagatatcatagtctagcatttacaggccaaggtcaaaaacctgggtgcaatggatcccatcagcatgtaattacatagattttatatcccttctgcagttaaaatatttcatcttatcttaaaacacattgctgtggtctggagaccagcagtctctcccccacatctctcttcattcttgcttgtttcagtttcttatcttattcctctctgccctttctgtaaagaaagcaaagttatcttctcatgactacgtgattaaggggtatatataaggatgaattatacataaagatccatgtaaataatttatgttaaaatatttaagttaaacaatttcgatagaaaaagttcatttctatggaaagacagaattgcaaatcaacagtgtttttacatatatacatacatgtataaattcacagaaagggttttttaagttgacctagtggtctttatgtatcatagtcattttctaaagctgagaatctatagtagataatagtatgcaaataacaagaagtttgattctaataaaattggtaagaatgaagaagcaacatgatccactacagatgtcaatacagtctgaagaataggaactggttggccacagttcatatactaatacattcttggagaatacaaaatttaagaatgaaaacattaagacattcttgacttttgagttaattttagcttataaatatcatgtgcttaatcttagacccactaacacaaatatcatatgatataggaaatcttcattaatctattctgcattatagcaaagatacctataaaacccaagacgcttgttccctagaagtttacttgctccggttggtgcttgctactcaggttgtatctagtccagaaagatcatcagaaatttatcacagacaatatgctcagattaagaacttaaggctttgaatataaccagaaaacaaataaaagcaaccaccctgtttccaaaaagtaaggacaaggaaaagtaaaacagaattgtgaactcaaaagtatttttgacaaaagtttttagaaggcatcaaagaatctttaacaaccctgcagtaccacaaactttatcgttttctttatatatttataactagaacaagtgttcttaaaaaaaaaaaatccaaacgtgtgcgtatatatatatggggaaagggtacatttaaaaggttagtttctgtaaaaagtttaataatttttaaaaaaattggggtaagttaagtcacctagtgaagataagtacacaaacctgatgtcaaattaaacttcagggaaaacaaaatgtgctttttctatccattttctttgttaaagtaaaaatgttcttgatagttatttaaaatccaaggaatgatgccccttcccatttcccttccttatactctgcaattcgaattaccgtatcacatctagaaagttaataattatctatattcttgtgggaaggggccttcatattaaattttcagtataaaaccataccctaaagagttttattgcttgcatacatgatgacactgtgatgccattattacaaaagtggctggtgttttttattgagccccacttaaaaccaagataaaagtctgcactatatttcatacttaacacgccaaatggtaggctttcagcaaaagcaaaatttaagcttaaaatattgaaatgttttataatgaatagaaattttgtcaaggaagtactttttaaagtttggaggaagggcactttaaagaaaagatgacttggaaagcaccaaatgagtgaaaataaagaattaagacccacagggaacgttggttttaatgggaaagcaaccaatgatatttttaggttgtcatgactgctcaagtatgttggaagggaaaaggcattgattattcttatcatcaatcacactttgaggtctcttggttgaattgtttaataaatggctaagggtattactttacctttcattgagtaaaaacatcagtgattctttaataagagagaagcgggtaaggctgtttcactgcttctctttgcgtttagctgaagaatgtggggtggaaagtgaatatggtgaccggataaccagaaattctcttctagtattaatgcttctcatttaaaaaattaaagataatgactgttaagagcatgataataaacattatctttacatgagtattctttcaatgatctaagttaaataacattgatatttattgagccaaaacttaagtgtgtccatgttacttctgttttggtagggaaagtgtagtcttcttgcttttaaaaatagttttcaaaaataatctgacttataaatcttcccattggcccatacattaccattgttctagtcacacttacaaaagtcctcttccccagttaatcattctgtatttccattgcttctcttttcttgagattaagaaaaccaaagcatcatctatagctacagtttaattttccaaaaaaccactctgagtatacatcacacacataccccgctggccattaaaaaagagaagcaatgtaaattttcttctagtctttccctgatttaatagggcctaagaagctacttttatctctttttggctccatctatttggtttaatgttaatgatcatggctgataatccttttatggaggaagggaacctattatgtcagcaataattggttcacttgctcctttggggtggaaaaaataagatatttcttaaagtaacaaggcctgaataaatgtgtggcagtctcaaattctattctatatctaaggtgtaatccttacatactaaagatagtgggatcattcttgtagatttctagcagactggtacattaaaaagtgacaatgtttggggtatgacagtataaaaaaaggtttaatttgagaaaaaggattaagttaaatagtaaacttagtgtgagattttaatcacaagtacaaaagagtgaagagcagccttcatgacaaggaatcatgtgaccagcccccaccccaaacataggttatcacatgtggattttgtttcattccgacaaaggaaaaggcccatacagttatcttaagtgttcattatatagagaccttatttaaccatgctcgattatcttacggaaaagaaaaacattacgataaatgtggtttccacatatcctagttctgtaaaaggtcaggtgtctcataaagtttgggttttggtgaaaatgtttgtacatgctgatgttaactactgcaataattataggattgtaaacggtaaaataacctgtatgactttgactgtcccagtgaccaaaatgcactttaatcttagaataatcaagactgaagcattaactgaaccctcatcttatattaatagcaccttctaagagaggcactgttttaaataggcacagaaacaaaaaatggtactttaaaagtactgttggaattcacaaatatatcccatgccacataaattaccgcttattataaaaatatcaataccctcaaatgccaatcagcaaaacataaatcaccaaaacatttcttcagtttagaacattgctcaattccacgataaaccatgctttatatttaaaaaataaattagagatgaatgtgaacctaaaagcatgtataatatatatatttaatactatatatacataattgctatatacttaagacattcttaggagtatttctacaaaaacaagttatcttttctttataaatcggaaatctgaacaccaacaatttgtcctttttcttttgttttaaaagaacagacatcatttatgcagctagagatttataaactaaattaaataagttaatacaatagcctcaactgtccctgtatttttcaccatggatctattttggcaacatggaggtatatctttcaaactgttccaggtcctacatgtgaaagagaagaagacatgaaaggatttcttaaatggaagtgctcattctaacctgacggtgacagaatcaattgatacaccatttcttcaagacaaaaaagcacatattcaaggaatagctcaaaaaatgctccagttttcacattatttcaaaactttatcggtagaatgactctgcacactaatttcactaagagtacataaacataggaaaatagtcctcaaaagatgcatttatgggcctatatttttcaacataaagtgctagcagatgtgtaagaagagctgggaatgtcttgagctgtaagtcctgagacctccacaccatggctggtcctggaggagttcagcattctgattttttcttaggttcaggatgatcatccaaggtggctggatgctcatttggaccacctggtgtctcacctgtgacagctaaaaggatgactttcagccacttctgcttcagttcctcactgtctgcagcaaagctgtgcacggacttagactgggtcagtttgaaactgtgtggcaggtctgcgctccttggcatttcatccaccacatagcccagaagtggaatggtggcctgggctctgacgtcctggggggcaccatacatgtacagcacaagagggtcttgcttggggatcacacaccaagctttctgccaaggttttgacttctccatatactgaagaaagctgcacaccacactgtttccagatacttctgctgattcaatctctaaaattccttttcttttcttttcttcactgtctgtgaatccacttatgatttgataacagtctttacaaactttgctcaatttaccaccatcatattcaagttgagctttgtagtcggagcatttccaacaaaccacatatccacatgctcgacaatgatgcctccttcgtgtcagtgcattgaaaggttctttacatttcatacacattgtcacttcattatctcggatccatcttggggctcttttccctagctcagcagtagaaacctctgagtgaatgtcattatcctttgcaattgcatttctgaaggtttcatgcctttgatgaaaagcatcgatggtttcttgaagggccttgatccattcttctttgtcttgcgcagaactggcctgcagttccagtgttctctctttcccagacacctggaaagtatgtggatattcttcattttgagtctctacaattttcattccatcaatgccaaccctggttcgaactgtgaatttagagcctaccaagctgaatttgggcacacagtacagcaacatgttgttgaataagaaaaggtagcgttcttgtgctgaagtgttccgagcagctagtttgaggatctgtccttcttttattagttcatttgaagggtttacaatgtcttcttcttctcccaacatttcataaatctctaagagtttctttaggttctccattttccttattgcactattagaatggcttgctgctgtagatataatttcaagtgattttttagcatcattccagtccagggaatcaggaggcaatttccttagatagtccttaaggagcatctcataccggggaatccgctgaacaggttctagcatgtgatgctgcaaagttaagctcccacagattttctgtttctgaatttcttcaaccactgatttgaactggggaatacgttctgtcatgtttttaaccaattccattgcattatcaaatcctttcacatattctccatacatcttaaggaatggtgccaatttctgaaggatgtctccaattctaggagtagtttcccattcttgcattcgtttctccagctctggcaagaggaatttactatggaaggcatttattgatgaaatattagaaaagattttattcaccatctctgctggaaacgagcctcggtttgcttcttccaacagtttgcaataaaatacctgatctaagaggtcaagtcggttgacataagctctttcagtaagcaaaagttcattggctattttgtgaagtttttgctcattagtctccttcatctcatggtgctggtccagctgctccagttccagagggctttccccattttccctctcttgtaccttggtttctgtttctgcccctctttcttctagggggagcactgggcctatgcctggagtcctgtagctactgtcagaagcatttccatcacagctgtctgttgtgggtgatgcaggagctgtggcagtttcatctctttctccattcactatgtgcgtatcaagcaagggttcagaagcttgaatagaagtatctgagctaagagtggcagctttctcctcctcacattccatctggttttgtgctgccattacaccgttggccacacaagtctgtgcaccctgagtcttatctgtatcatttccctgcctctgtggcaagtgctgggagaggagtttttgttgaggtgtggttgtcaatccatgccttcctggggttctaggagcatttaggttcacagcagactctttcttcaaatcactataatttgataatgagcttgtttcatcctcacaataattccaaagacagggatcccatagagaaatctaggcttagaaattaaggtggccaatgtcacaatgtaacaagcagaaaagccagaggtcaaaccatgaatccaactctaaatcccatggtcttcaccccaagttatgatgtactggagcagaaggacagaatgagcatcagatgaataggtcttcagttgagatttgcccccttgaggaggacaactttggcctggataatttcccaagtagtctttagagatttgaatcaaactgtcctccttctcctgcccacatcagtctctggattccctggtggaaagatcctcaacagatcctctgcctccttcaaagcgactgatgagatctgataccttactgggtttttcttttgagacacaagaagcagaggcaggtttaatttcctccatccttggttttgcactaggtaaagctttatgcctgggggtttggtgtatattggacgaaggtgaattctgcaggtgtaatggctttggaggcacttgtggctttggacttgcagctgagtgttttgctggcctgttcccatttattccctgagcctcttcttcagatacattctcaccaaccagtgtggttgtgctgcttgtggagcaaggtggaactaaagcgatctttggacaggtactgctgccttataaaagctgaatttattcctcttggccagaagtcacaaatggttgaagtaaaactcccttcatttgttcttccagcgagccaaagcaagcctcccattaacccggtccattgcagataatctcacccagcacaggctcccctgctttccccacttcccagcccagcaaggataatcacattccggtggggagtgaacagatggtggattccatg

SEQ ID NO: 14952 - RNA, 7775 nt, Homo sapiens
  source 1..7775: mol_type = other RNA
gctgggattacaggcatgagccactatgcccggcctatgcttattttaaaatgtcaattgtcactcacaaaatgaaatgctagtttggttaaaaaaaaaaaagtcttatatacagacagacatgactgttttgctaatgaagagaaccccccacaagtgatacattccaatatccatatactgtgtaatatataatgtgattctcttataatggtccccacagactagtttcttcccaaacctatatgtcactatgtatttggtatttatttattaaagtatgatatgagatttcttgatttacgttttccactaaaactaccacaatgaattttgggaaaaggggttgaccatcatataactcccggtgaccccaacaagttaaaactatcttgtagaagccatgtgctatttcatgtcaaaatacaggaaaagatactgcattctgccaaatgctcagtccagaaagtagaagaccatgattgacttcagattttttttttttttgcctcagtaaacagtacagaaaatgatctgagaatgaaattattttttaaaagcccaaaggagaaaaagaataacaagatatcatagtctagcatttacaggccaaggtcaaaaacctgggtgcaatggatcccatcagcatgtaattacatagattttatatcccttctgcagttaaaatatttcatcttatcttaaaacacattgctgtggtctggagaccagcagtctctcccccacatctctcttcattcttgcttgtttcagtttcttatcttattcctctctgccctttctgtaaagaaagcaaagttatcttctcatgactacgtgattaaggggtatatataaggatgaattatacataaagatccatgtaaataatttatgttaaaatatttaagttaaacaatttcgatagaaaaagttcatttctatggaaagacagaattgcaaatcaacagtgtttttacatatatacatacatgtataaattcacagaaagggttttttaagttgacctagtggtctttatgtatcatagtcattttctaaagctgagaatctatagtagataatagtatgcaaataacaagaagtttgattctaataaaattggtaagaatgaagaagcaacatgatccactacagatgtcaatacagtctgaagaataggaactggttggccacagttcatatactaatacattcttggagaatacaaaatttaagaatgaaaacattaagacattcttgacttttgagttaattttagcttataaatatcatgtgcttaatcttagacccactaacacaaatatcatatgatataggaaatcttcattaatctattctgcattatagcaaagatacctataaaacccaagacgcttgttccctagaagtttacttgctccggttggtgcttgctactcaggttgtatctagtccagaaagatcatcagaaatttatcacagacaatatgctcagattaagaacttaaggctttgaatataaccagaaaacaaataaaagcaaccaccctgtttccaaaaagtaaggacaaggaaaagtaaaacagaattgtgaactcaaaagtatttttgacaaaagtttttagaaggcatcaaagaatctttaacaaccctgcagtaccacaaactttatcgttttctttatatatttataactagaacaagtgttcttaaaaaaaaaaaatccaaacgtgtgcgtatatatatatggggaaagggtacatttaaaaggttagtttctgtaaaaagtttaataatttttaaaaaaattggggtaagttaagtcacctagtgaagataagtacacaaacctgatgtcaaattaaacttcagggaaaacaaaatgtgctttttctatccattttctttgttaaagtaaaaatgttcttgatagttatttaaaatccaaggaatgatgccccttcccatttcccttccttatactctgcaattcgaattaccgtatcacatctagaaagttaataattatctatattcttgtgggaaggggccttcatattaaattttcagtataaaaccataccctaaagagttttattgcttgcatacatgatgacactgtgatgccattattacaaaagtggctggtgttttttattgagccccacttaaaaccaagataaaagtctgcactatatttcatacttaacacgccaaatggtaggctttcagcaaaagcaaaatttaagcttaaaatattgaaatgttttataatgaatagaaattttgtcaaggaagtactttttaaagtttggaggaagggcactttaaagaaaagatgacttggaaagcaccaaatgagtgaaaataaagaattaagacccacagggaacgttggttttaatgggaaagcaaccaatgatatttttaggttgtcatgactgctcaagtatgttggaagggaaaaggcattgattattcttatcatcaatcacactttgaggtctcttggttgaattgtttaataaatggctaagggtattactttacctttcattgagtaaaaacatcagtgattctttaataagagagaagcgggtaaggctgtttcactgcttctctttgcgtttagctgaagaatgtggggtggaaagtgaatatggtgaccggataaccagaaattctcttctagtattaatgcttctcatttaaaaaattaaagataatgactgttaagagcatgataataaacattatctttacatgagtattctttcaatgatctaagttaaataacattgatatttattgagccaaaacttaagtgtgtccatgttacttctgttttggtagggaaagtgtagtcttcttgcttttaaaaatagttttcaaaaataatctgacttataaatcttcccattggcccatacattaccattgttctagtcacacttacaaaagtcctcttccccagttaatcattctgtatttccattgcttctcttttcttgagattaagaaaaccaaagcatcatctatagctacagtttaattttccaaaaaaccactctgagtatacatcacacacataccccgctggccattaaaaaagagaagcaatgtaaattttcttctagtctttccctgatttaatagggcctaagaagctacttttatctctttttggctccatctatttggtttaatgttaatgatcatggctgataatccttttatggaggaagggaacctattatgtcagcaataattggttcacttgctcctttggggtggaaaaaataagatatttcttaaagtaacaaggcctgaataaatgtgtggcagtctcaaattctattctatatctaaggtgtaatccttacatactaaagatagtgggatcattcttgtagatttctagcagactggtacattaaaaagtgacaatgtttggggtatgacagtataaaaaaaggtttaatttgagaaaaaggattaagttaaatagtaaacttagtgtgagattttaatcacaagtacaaaagagtgaagagcagccttcatgacaaggaatcatgtgaccagcccccaccccaaacataggttatcacatgtggattttgtttcattccgacaaaggaaaaggcccatacagttatcttaagtgttcattatatagagaccttatttaaccatgctcgattatcttacggaaaagaaaaacattacgataaatgtggtttccacatatcctagttctgtaaaaggtcaggtgtctcataaagtttgggttttggtgaaaatgtttgtacatgctgatgttaactactgcaataattataggattgtaaacggtaaaataacctgtatgactttgactgtcccagtgaccaaaatgcactttaatcttagaataatcaagactgaagcattaactgaaccctcatcttatattaatagcaccttctaagagaggcactgttttaaataggcacagaaacaaaaaatggtactttaaaagtactgttggaattcacaaatatatcccatgccacataaattaccgcttattataaaaatatcaataccctcaaatgccaatcagcaaaacataaatcaccaaaacatttcttcagtttagaacattgctcaattccacgataaaccatgctttatatttaaaaaataaattagagatgaatgtgaacctaaaagcatgtataatatatatatttaatactatatatacataattgctatatacttaagacattcttaggagtatttctacaaaaacaagttatcttttctttataaatcggaaatctgaacaccaacaatttgtcctttttcttttgttttaaaagaacagacatcatttatgcagctagagatttataaactaaattaaataagttaatacaatagcctcaactgtccctgtatttttcaccatggatctattttggcaacatggaggtatatctttcaaactgttccaggtcctacatgtgaaagagaagaagacatgaaaggatttcttaaatggaagtgctcattctaacctgacggtgacagaatcaattgatacaccatttcttcaagacaaaaaagcacatattcaaggaatagctcaaaaaatgctccagttttcacattatttcaaaactttatcggtagaatgactctgcacactaatttcactaagagtacataaacataggaaaatagtcctcaaaagatgcatttatgggcctatatttttcaacataaagtgctagcagatgtgtaagaagagctgggaatgtcttgagctgtaagtcctgagacctccacaccatggctggtcctggaggagttcagcattctgattttttcttaggttcaggatgatcatccaaggtggctggatgctcatttggaccacctggtgtctcacctgtgacagctaaaaggatgactttcagccacttctgcttcagttcctcactgtctgcagcaaagctgtgcacggacttagactgggtcagtttgaaactgtgtggcaggtctgcgctccttggcatttcatccaccacatagcccagaagtggaatggtggcctgggctctgacgtcctggggggcaccatacatgtacagcacaagagggtcttgcttggggatcacacaccaagctttctgccaaggttttgacttctccatatactgaagaaagctgcacaccacactgtttccagatacttctgctgattcaatctctaaaattccttttcttttcttttcttcactgtctgtgaatccacttatgatttgataacagtctttacaaactttgctcaatttaccaccatcatattcaagttgagctttgtagtcggagcatttccaacaaaccacatatccacatgctcgacaatgatgcctccttcgtgtcagtgcattgaaaggttctttacatttcatacacattgtcacttcattatctcggatccatcttggggctcttttccctagctcagcagtagaaacctctgagtgaatgtcattatcctttgcaattgcatttctgaaggtttcatgcctttgatgaaaagcatcgatggtttcttgaagggccttgatccattcttctttgtcttgcgcagaactggcctgcagttccagtgttctctctttcccagacacctggaaagtatgtggatattcttcattttgagtctctacaattttcattccatcaatgccaaccctggttcgaactgtgaatttagagcctaccaagctgaatttgggcacacagtacagcaacatgttgttgaataagaaaaggtagcgttcttgtgctgaagtgttccgagcagctagtttgaggatctgtccttcttttattagttcatttgaagggtttacaatgtcttcttcttctcccaacatttcataaatctctaagagtttctttaggttctccattttccttattgcactattagaatggcttgctgctgtagatataatttcaagtgattttttagcatcattccagtccagggaatcaggaggcaatttccttagatagtccttaaggagcatctcataccggggaatccgctgaacaggttctagcatgtgatgctgcaaagttaagctcccacagattttctgtttctgaatttcttcaaccactgatttgaactggggaatacgttctgtcatgtttttaaccaattccattgcattatcaaatcctttcacatattctccatacatcttaaggaatggtgccaatttctgaaggatgtctccaattctaggagtagtttcccattcttgcattcgtttctccagctctggcaagaggaatttactatggaaggcatttattgatgaaatattagaaaagattttattcaccatctctgctggaaacgagcctcggtttgcttcttccaacagtttgcaataaaatacctgatctaagaggtcaagtcggttgacataagctctttcagtaagcaaaagttcattggctattttgtgaagtttttgctcattagtctccttcatctcatggtgctggtccagctgctccagttccagagggctttccccattttccctctcttgtaccttggtttctgtttctgcccctctttcttctagggggagcactgggcctatgcctggagtcctgtagctactgtcagaagcatttccatcacagctgtctgttgtgggtgatgcaggagctgtggcagtttcatctctttctccattcactatgtgcgtatcaagcaagggttcagaagcttgaatagaagtatctgagctaagagtggcagctttctcctcctcacattccatctggttttgtgctgccattacaccgttggccacacaagtctgtgcaccctgagtcttatctgtatcatttccctgcctctgtggcaagtgctgggagaggagtttttgttgaggtgtggttgtcaatccatgccttcctggggttctaggagcatttaggttcacagcagactctttcttcaaatcactataatttgataatgagtcttcagttgagatttgcccccttgaggaggacaactttggcctggataatttcccaagtagtctttagagatttgaatcaaactgtcctccttctcctgcccacatcagtctctggattccctggtggaaagatcctcaacagatcctctgcctccttcaaagcgactgatgagatctgataccttactgggtttttcttttgagacacaagaagcagaggcaggtttaatttcctccatccttggttttgcactaggtaaagctttatgcctgggggtttggtgtatattggacgaaggtgaattctgcaggtgtaatggctttggaggcacttgtggctttggacttgcagctgagtgttttgctggcctgttcccatttattccctgagcctcttcttcagatacattctcaccaaccagtgtggttgtgctgcttgtggagcaaggtggaactaaagcgatctttggacaggtactgctgccttataaaagctgaatttattcctcttggccagaagtcacaaatggttgaagtaaaactcccttcatttgttcttccagcgagccaaagcaagcctcccattaacccggtccattgcagataatctcacccagcacaggctcccctgctttccccacttcccagcccagcaaggataatcacattccggtggggagtgaacagatggtggattccatg

SEQ ID NO: 14953 - RNA, 6892 nt, Homo sapiens
  source 1..6892: mol_type = other RNA
gctgggattacaggcatgagccactatgcccggcctatgcttattttaaaatgtcaattgtcactcacaaaatgaaatgctagtttggttaaaaaaaaaaaagtcttatatacagacagacatgactgttttgctaatgaagagaaccccccacaagtgatacattccaatatccatatactgtgtaatatataatgtgattctcttataatggtccccacagactagtttcttcccaaacctatatgtcactatgtatttggtatttatttattaaagtatgatatgagatttcttgatttacgttttccactaaaactaccacaatgaattttgggaaaaggggttgaccatcatataactcccggtgaccccaacaagttaaaactatcttgtagaagccatgtgctatttcatgtcaaaatacaggaaaagatactgcattctgccaaatgctcagtccagaaagtagaagaccatgattgacttcagattttttttttttttgcctcagtaaacagtacagaaaatgatctgagaatgaaattattttttaaaagcccaaaggagaaaaagaataacaagatatcatagtctagcatttacaggccaaggtcaaaaacctgggtgcaatggatcccatcagcatgtaattacatagattttatatcccttctgcagttaaaatatttcatcttatcttaaaacacattgctgtggtctggagaccagcagtctctcccccacatctctcttcattcttgcttgtttcagtttcttatcttattcctctctgccctttctgtaaagaaagcaaagttatcttctcatgactacgtgattaaggggtatatataaggatgaattatacataaagatccatgtaaataatttatgttaaaatatttaagttaaacaatttcgatagaaaaagttcatttctatggaaagacagaattgcaaatcaacagtgtttttacatatatacatacatgtataaattcacagaaagggttttttaagttgacctagtggtctttatgtatcatagtcattttctaaagctgagaatctatagtagataatagtatgcaaataacaagaagtttgattctaataaaattggtaagaatgaagaagcaacatgatccactacagatgtcaatacagtctgaagaataggaactggttggccacagttcatatactaatacattcttggagaatacaaaatttaagaatgaaaacattaagacattcttgacttttgagttaattttagcttataaatatcatgtgcttaatcttagacccactaacacaaatatcatatgatataggaaatcttcattaatctattctgcattatagcaaagatacctataaaacccaagacgcttgttccctagaagtttacttgctccggttggtgcttgctactcaggttgtatctagtccagaaagatcatcagaaatttatcacagacaatatgctcagattaagaacttaaggctttgaatataaccagaaaacaaataaaagcaaccaccctgtttccaaaaagtaaggacaaggaaaagtaaaacagaattgtgaactcaaaagtatttttgacaaaagtttttagaaggcatcaaagaatctttaacaaccctgcagtaccacaaactttatcgttttctttatatatttataactagaacaagtgttcttaaaaaaaaaaaatccaaacgtgtgcgtatatatatatggggaaagggtacatttaaaaggttagtttctgtaaaaagtttaataatttttaaaaaaattggggtaagttaagtcacctagtgaagataagtacacaaacctgatgtcaaattaaacttcagggaaaacaaaatgtgctttttctatccattttctttgttaaagtaaaaatgttcttgatagttatttaaaatccaaggaatgatgccccttcccatttcccttccttatactctgcaattcgaattaccgtatcacatctagaaagttaataattatctatattcttgtgggaaggggccttcatattaaattttcagtataaaaccataccctaaagagttttattgcttgcatacatgatgacactgtgatgccattattacaaaagtggctggtgttttttattgagccccacttaaaaccaagataaaagtctgcactatatttcatacttaacacgccaaatggtaggctttcagcaaaagcaaaatttaagcttaaaatattgaaatgttttataatgaatagaaattttgtcaaggaagtactttttaaagtttggaggaagggcactttaaagaaaagatgacttggaaagcaccaaatgagtgaaaataaagaattaagacccacagggaacgttggttttaatgggaaagcaaccaatgatatttttaggttgtcatgactgctcaagtatgttggaagggaaaaggcattgattattcttatcatcaatcacactttgaggtctcttggttgaattgtttaataaatggctaagggtattactttacctttcattgagtaaaaacatcagtgattctttaataagagagaagcgggtaaggctgtttcactgcttctctttgcgtttagctgaagaatgtggggtggaaagtgaatatggtgaccggataaccagaaattctcttctagtattaatgcttctcatttaaaaaattaaagataatgactgttaagagcatgataataaacattatctttacatgagtattctttcaatgatctaagttaaataacattgatatttattgagccaaaacttaagtgtgtccatgttacttctgttttggtagggaaagtgtagtcttcttgcttttaaaaatagttttcaaaaataatctgacttataaatcttcccattggcccatacattaccattgttctagtcacacttacaaaagtcctcttccccagttaatcattctgtatttccattgcttctcttttcttgagattaagaaaaccaaagcatcatctatagctacagtttaattttccaaaaaaccactctgagtatacatcacacacataccccgctggccattaaaaaagagaagcaatgtaaattttcttctagtctttccctgatttaatagggcctaagaagctacttttatctctttttggctccatctatttggtttaatgttaatgatcatggctgataatccttttatggaggaagggaacctattatgtcagcaataattggttcacttgctcctttggggtggaaaaaataagatatttcttaaagtaacaaggcctgaataaatgtgtggcagtctcaaattctattctatatctaaggtgtaatccttacatactaaagatagtgggatcattcttgtagatttctagcagactggtacattaaaaagtgacaatgtttggggtatgacagtataaaaaaaggtttaatttgagaaaaaggattaagttaaatagtaaacttagtgtgagattttaatcacaagtacaaaagagtgaagagcagccttcatgacaaggaatcatgtgaccagcccccaccccaaacataggttatcacatgtggattttgtttcattccgacaaaggaaaaggcccatacagttatcttaagtgttcattatatagagaccttatttaaccatgctcgattatcttacggaaaagaaaaacattacgataaatgtggtttccacatatcctagttctgtaaaaggtcaggtgtctcataaagtttgggttttggtgaaaatgtttgtacatgctgatgttaactactgcaataattataggattgtaaacggtaaaataacctgtatgactttgactgtcccagtgaccaaaatgcactttaatcttagaataatcaagactgaagcattaactgaaccctcatcttatattaatagcaccttctaagagaggcactgttttaaataggcacagaaacaaaaaatggtactttaaaagtactgttggaattcacaaatatatcccatgccacataaattaccgcttattataaaaatatcaataccctcaaatgccaatcagcaaaacataaatcaccaaaacatttcttcagtttagaacattgctcaattccacgataaaccatgctttatatttaaaaaataaattagagatgaatgtgaacctaaaagcatgtataatatatatatttaatactatatatacataattgctatatacttaagacattcttaggagtatttctacaaaaacaagttatcttttctttataaatcggaaatctgaacaccaacaatttgtcctttttcttttgttttaaaagaacagacatcatttatgcagctagagatttataaactaaattaaataagttaatacaatagcctcaactgtccctgtatttttcaccatggatctattttggcaacatggaggtatatctttcaaactgttccaggtcctacatgtgaaagagaagaagacatgaaaggatttcttaaatggaagtgctcattctaacctgacggtgacagaatcaattgatacaccatttcttcaagacaaaaaagcacatattcaaggaatagctcaaaaaatgctccagttttcacattatttcaaaactttatcggtagaatgactctgcacactaatttcactaagagtacataaacataggaaaatagtcctcaaaagatgcatttatgggcctatatttttcaacataaagtgctagcagatgtgtaagaagagctgggaatgtcttgagctgtaagtcctgagacctccacaccatggctggtcctggaggagttcagcattctgattttttcttaggttcaggatgatcatccaaggtggctggatgctcatttggaccacctggtgtctcacctgtgacagctaaaaggatgactttcagccacttctgcttcagttcctcactgtctgcagcaaagctgtgcacggacttagactgggtcagtttgaaactgtgtggcaggtctgcgctccttggcatttcatccaccacatagcccagaagtggaatggtggcctgggctctgacgtcctggggggcaccatacatgtacagcacaagagggtcttgcttggggatcacacaccaagctttctgccaaggttttgacttctccatatactgaagaaagctgcacaccacactgtttccagatacttctgctgattcaatctctaaaattccttttcttttcttttcttcactgtctgtgaatccacttatgatttgataacagtctttacaaactttgctcaatttaccaccatcatattcaagttgagctttgtagtcggagcatttccaacaaaccacatatccacatgctcgacaatgatgcctccttcgtgtcagtgcattgaaaggttctttacatttcatacacattgtcacttcattatctcggatccatcttggggctcttttccctagctcagcagtagaaacctctgagtgaatgtcattatcctttgcaattgcatttctgaaggtttcatgcctttgatgaaaagcatcgatggtttcttgaagggccttgatccattcttctttgtcttgcgcagaactggcctgcagttccagtgttctctctttcccagacacctggaaagtatgtggatattcttcattttgagtctctacaattttcattccatcaatgccaaccctggttcgaactgtgaatttagagcctaccaagctgaatttgggcacacagtacagcaacatgttgttgaataagaaaaggtagcgttcttgtgctgaagtgttccgagcagctagtttgaggatctgtccttcttttattagttcatttgaagggtttacaatgtcttcttcttctcccaacatttcataaatctctaagagtttctttaggttctccattttccttattgcactattagaatggcttgctgctgtagatataatttcaagtgattttttagcatcattccagtccagggaatcaggaggcaatttccttagatagtccttaaggagcatctcataccggggaatccgctgaacaggttctagcatgtgatgctgcaaagttaagctcccacagattttctgtttctgaatttcttcaaccactgatttgaactggggaatacgttctgtcatgtttttaaccaattccattgcattatcaaatcctttcacatattctccatacatcttaaggaatggtgccaatttctgaaggatgtctccaattctaggagtagtttcccattcttgcattcgtttctccagctctggcaagaggaatttactatggaaggcatttattgatgaaatattagaaaagattttattcaccatctctgctggaaacgagcctcggtttgcttcttccaacagtttgcaataaaatacctgatctaagaggtcaagtcggttgacataagctctttcagtaagcaaaagttcattggctattttgtgaagtttttgctcattagtctccttgtggctttggacttgcagctgagtgttttgctggcctgttcccatttattccctgagcctcttcttcagatacattctcaccaaccagtgtggttgtgctgcttgtggagcaaggtggaactaaagcgatctttggacaggtactgctgccttataaaagctgaatttattcctcttggccagaagtcacaaatggttgaagtaaaactcccttcatttgttcttccagcgagccaaagcaagcctcccattaacccggtccattgcagataatctcacccagcacaggctcccctgctttccccacttcccagcccagcaaggat

SEQ ID NO: 14954 - RNA, 6922 nt, Homo sapiens
  source 1..6922: mol_type = other RNA
gctgggattacaggcatgagccactatgcccggcctatgcttattttaaaatgtcaattgtcactcacaaaatgaaatgctagtttggttaaaaaaaaaaaagtcttatatacagacagacatgactgttttgctaatgaagagaaccccccacaagtgatacattccaatatccatatactgtgtaatatataatgtgattctcttataatggtccccacagactagtttcttcccaaacctatatgtcactatgtatttggtatttatttattaaagtatgatatgagatttcttgatttacgttttccactaaaactaccacaatgaattttgggaaaaggggttgaccatcatataactcccggtgaccccaacaagttaaaactatcttgtagaagccatgtgctatttcatgtcaaaatacaggaaaagatactgcattctgccaaatgctcagtccagaaagtagaagaccatgattgacttcagattttttttttttttgcctcagtaaacagtacagaaaatgatctgagaatgaaattattttttaaaagcccaaaggagaaaaagaataacaagatatcatagtctagcatttacaggccaaggtcaaaaacctgggtgcaatggatcccatcagcatgtaattacatagattttatatcccttctgcagttaaaatatttcatcttatcttaaaacacattgctgtggtctggagaccagcagtctctcccccacatctctcttcattcttgcttgtttcagtttcttatcttattcctctctgccctttctgtaaagaaagcaaagttatcttctcatgactacgtgattaaggggtatatataaggatgaattatacataaagatccatgtaaataatttatgttaaaatatttaagttaaacaatttcgatagaaaaagttcatttctatggaaagacagaattgcaaatcaacagtgtttttacatatatacatacatgtataaattcacagaaagggttttttaagttgacctagtggtctttatgtatcatagtcattttctaaagctgagaatctatagtagataatagtatgcaaataacaagaagtttgattctaataaaattggtaagaatgaagaagcaacatgatccactacagatgtcaatacagtctgaagaataggaactggttggccacagttcatatactaatacattcttggagaatacaaaatttaagaatgaaaacattaagacattcttgacttttgagttaattttagcttataaatatcatgtgcttaatcttagacccactaacacaaatatcatatgatataggaaatcttcattaatctattctgcattatagcaaagatacctataaaacccaagacgcttgttccctagaagtttacttgctccggttggtgcttgctactcaggttgtatctagtccagaaagatcatcagaaatttatcacagacaatatgctcagattaagaacttaaggctttgaatataaccagaaaacaaataaaagcaaccaccctgtttccaaaaagtaaggacaaggaaaagtaaaacagaattgtgaactcaaaagtatttttgacaaaagtttttagaaggcatcaaagaatctttaacaaccctgcagtaccacaaactttatcgttttctttatatatttataactagaacaagtgttcttaaaaaaaaaaaatccaaacgtgtgcgtatatatatatggggaaagggtacatttaaaaggttagtttctgtaaaaagtttaataatttttaaaaaaattggggtaagttaagtcacctagtgaagataagtacacaaacctgatgtcaaattaaacttcagggaaaacaaaatgtgctttttctatccattttctttgttaaagtaaaaatgttcttgatagttatttaaaatccaaggaatgatgccccttcccatttcccttccttatactctgcaattcgaattaccgtatcacatctagaaagttaataattatctatattcttgtgggaaggggccttcatattaaattttcagtataaaaccataccctaaagagttttattgcttgcatacatgatgacactgtgatgccattattacaaaagtggctggtgttttttattgagccccacttaaaaccaagataaaagtctgcactatatttcatacttaacacgccaaatggtaggctttcagcaaaagcaaaatttaagcttaaaatattgaaatgttttataatgaatagaaattttgtcaaggaagtactttttaaagtttggaggaagggcactttaaagaaaagatgacttggaaagcaccaaatgagtgaaaataaagaattaagacccacagggaacgttggttttaatgggaaagcaaccaatgatatttttaggttgtcatgactgctcaagtatgttggaagggaaaaggcattgattattcttatcatcaatcacactttgaggtctcttggttgaattgtttaataaatggctaagggtattactttacctttcattgagtaaaaacatcagtgattctttaataagagagaagcgggtaaggctgtttcactgcttctctttgcgtttagctgaagaatgtggggtggaaagtgaatatggtgaccggataaccagaaattctcttctagtattaatgcttctcatttaaaaaattaaagataatgactgttaagagcatgataataaacattatctttacatgagtattctttcaatgatctaagttaaataacattgatatttattgagccaaaacttaagtgtgtccatgttacttctgttttggtagggaaagtgtagtcttcttgcttttaaaaatagttttcaaaaataatctgacttataaatcttcccattggcccatacattaccattgttctagtcacacttacaaaagtcctcttccccagttaatcattctgtatttccattgcttctcttttcttgagattaagaaaaccaaagcatcatctatagctacagtttaattttccaaaaaaccactctgagtatacatcacacacataccccgctggccattaaaaaagagaagcaatgtaaattttcttctagtctttccctgatttaatagggcctaagaagctacttttatctctttttggctccatctatttggtttaatgttaatgatcatggctgataatccttttatggaggaagggaacctattatgtcagcaataattggttcacttgctcctttggggtggaaaaaataagatatttcttaaagtaacaaggcctgaataaatgtgtggcagtctcaaattctattctatatctaaggtgtaatccttacatactaaagatagtgggatcattcttgtagatttctagcagactggtacattaaaaagtgacaatgtttggggtatgacagtataaaaaaaggtttaatttgagaaaaaggattaagttaaatagtaaacttagtgtgagattttaatcacaagtacaaaagagtgaagagcagccttcatgacaaggaatcatgtgaccagcccccaccccaaacataggttatcacatgtggattttgtttcattccgacaaaggaaaaggcccatacagttatcttaagtgttcattatatagagaccttatttaaccatgctcgattatcttacggaaaagaaaaacattacgataaatgtggtttccacatatcctagttctgtaaaaggtcaggtgtctcataaagtttgggttttggtgaaaatgtttgtacatgctgatgttaactactgcaataattataggattgtaaacggtaaaataacctgtatgactttgactgtcccagtgaccaaaatgcactttaatcttagaataatcaagactgaagcattaactgaaccctcatcttatattaatagcaccttctaagagaggcactgttttaaataggcacagaaacaaaaaatggtactttaaaagtactgttggaattcacaaatatatcccatgccacataaattaccgcttattataaaaatatcaataccctcaaatgccaatcagcaaaacataaatcaccaaaacatttcttcagtttagaacattgctcaattccacgataaaccatgctttatatttaaaaaataaattagagatgaatgtgaacctaaaagcatgtataatatatatatttaatactatatatacataattgctatatacttaagacattcttaggagtatttctacaaaaacaagttatcttttctttataaatcggaaatctgaacaccaacaatttgtcctttttcttttgttttaaaagaacagacatcatttatgcagctagagatttataaactaaattaaataagttaatacaatagcctcaactgtccctgtatttttcaccatggatctattttggcaacatggaggtatatctttcaaactgttccaggtcctacatgtgaaagagaagaagacatgaaaggatttcttaaatggaagtgctcattctaacctgacggtgacagaatcaattgatacaccatttcttcaagacaaaaaagcacatattcaaggaatagctcaaaaaatgctccagttttcacattatttcaaaactttatcggtagaatgactctgcacactaatttcactaagagtacataaacataggaaaatagtcctcaaaagatgcatttatgggcctatatttttcaacataaagtgctagcagatgtgtaagaagagctgggaatgtcttgagctgtaagtcctgagacctccacaccatggctggtcctggaggagttcagcattctgattttttcttaggttcaggatgatcatccaaggtggctggatgctcatttggaccacctggtgtctcacctgtgacagctaaaaggatgactttcagccacttctgcttcagttcctcactgtctgcagcaaagctgtgcacggacttagactgggtcagtttgaaactgtgtggcaggtctgcgctccttggcatttcatccaccacatagcccagaagtggaatggtggcctgggctctgacgtcctggggggcaccatacatgtacagcacaagagggtcttgcttggggatcacacaccaagctttctgccaaggttttgacttctccatatactgaagaaagctgcacaccacactgtttccagatacttctgctgattcaatctctaaaattccttttcttttcttttcttcactgtctgtgaatccacttatgatttgataacagtctttacaaactttgctcaatttaccaccatcatattcaagttgagctttgtagtcggagcatttccaacaaaccacatatccacatgctcgacaatgatgcctccttcgtgtcagtgcattgaaaggttctttacatttcatacacattgtcacttcattatctcggatccatcttggggctcttttccctagctcagcagtagaaacctctgagtgaatgtcattatcctttgcaattgcatttctgaaggtttcatgcctttgatgaaaagcatcgatggtttcttgaagggccttgatccattcttctttgtcttgcgcagaactggcctgcagttccagtgttctctctttcccagacacctggaaagtatgtggatattcttcattttgagtctctacaattttcattccatcaatgccaaccctggttcgaactgtgaatttagagcctaccaagctgaatttgggcacacagtacagcaacatgttgttgaataagaaaaggtagcgttcttgtgctgaagtgttccgagcagctagtttgaggatctgtccttcttttattagttcatttgaagggtttacaatgtcttcttcttctcccaacatttcataaatctctaagagtttctttaggttctccattttccttattgcactattagaatggcttgctgctgtagatataatttcaagtgattttttagcatcattccagtccagggaatcaggaggcaatttccttagatagtccttaaggagcatctcataccggggaatccgctgaacaggttctagcatgtgatgctgcaaagttaagctcccacagattttctgtttctgaatttcttcaaccactgatttgaactggggaatacgttctgtcatgtttttaaccaattccattgcattatcaaatcctttcacatattctccatacatcttaaggaatggtgccaatttctgaaggatgtctccaattctaggagtagtttcccattcttgcattcgtttctccagctctggcaagaggaatttactatggaaggcatttattgatgaaatattagaaaagattttattcaccatctctgctggaaacgagcctcggtttgcttcttccaacagtttgcaataaaatacctgatctaagaggtcaagtcggttgacataagctctttcagtaagcaaaagttcattggctattttgtgaagtttttgctcattagtctccttgtggctttggacttgcagctgagtgttttgctggcctgttcccatttattccctgagcctcttcttcagatacattctcaccaaccagtgtggttgtgctgcttgtggagcaaggtggaactaaagcgatctttggacaggtactgctgccttgatcagtggacatgatttcacatatactgataattaatctactctggtttaataaaaagatatttggctttactcttttaaagttcatgtgataaaatctcactcctggctgtaaagcttcagggaggctgaagattacacaggatctgccaggagctcagaccaatgcactatgacttcagtgcattcttcgaacttactgc

SEQ ID NO: 14955 - RNA, 7703 nt, Homo sapiens
  source 1..7703: mol_type = other RNA
gctgggattacaggcatgagccactatgcccggcctatgcttattttaaaatgtcaattgtcactcacaaaatgaaatgctagtttggttaaaaaaaaaaaagtcttatatacagacagacatgactgttttgctaatgaagagaaccccccacaagtgatacattccaatatccatatactgtgtaatatataatgtgattctcttataatggtccccacagactagtttcttcccaaacctatatgtcactatgtatttggtatttatttattaaagtatgatatgagatttcttgatttacgttttccactaaaactaccacaatgaattttgggaaaaggggttgaccatcatataactcccggtgaccccaacaagttaaaactatcttgtagaagccatgtgctatttcatgtcaaaatacaggaaaagatactgcattctgccaaatgctcagtccagaaagtagaagaccatgattgacttcagattttttttttttttgcctcagtaaacagtacagaaaatgatctgagaatgaaattattttttaaaagcccaaaggagaaaaagaataacaagatatcatagtctagcatttacaggccaaggtcaaaaacctgggtgcaatggatcccatcagcatgtaattacatagattttatatcccttctgcagttaaaatatttcatcttatcttaaaacacattgctgtggtctggagaccagcagtctctcccccacatctctcttcattcttgcttgtttcagtttcttatcttattcctctctgccctttctgtaaagaaagcaaagttatcttctcatgactacgtgattaaggggtatatataaggatgaattatacataaagatccatgtaaataatttatgttaaaatatttaagttaaacaatttcgatagaaaaagttcatttctatggaaagacagaattgcaaatcaacagtgtttttacatatatacatacatgtataaattcacagaaagggttttttaagttgacctagtggtctttatgtatcatagtcattttctaaagctgagaatctatagtagataatagtatgcaaataacaagaagtttgattctaataaaattggtaagaatgaagaagcaacatgatccactacagatgtcaatacagtctgaagaataggaactggttggccacagttcatatactaatacattcttggagaatacaaaatttaagaatgaaaacattaagacattcttgacttttgagttaattttagcttataaatatcatgtgcttaatcttagacccactaacacaaatatcatatgatataggaaatcttcattaatctattctgcattatagcaaagatacctataaaacccaagacgcttgttccctagaagtttacttgctccggttggtgcttgctactcaggttgtatctagtccagaaagatcatcagaaatttatcacagacaatatgctcagattaagaacttaaggctttgaatataaccagaaaacaaataaaagcaaccaccctgtttccaaaaagtaaggacaaggaaaagtaaaacagaattgtgaactcaaaagtatttttgacaaaagtttttagaaggcatcaaagaatctttaacaaccctgcagtaccacaaactttatcgttttctttatatatttataactagaacaagtgttcttaaaaaaaaaaaatccaaacgtgtgcgtatatatatatggggaaagggtacatttaaaaggttagtttctgtaaaaagtttaataatttttaaaaaaattggggtaagttaagtcacctagtgaagataagtacacaaacctgatgtcaaattaaacttcagggaaaacaaaatgtgctttttctatccattttctttgttaaagtaaaaatgttcttgatagttatttaaaatccaaggaatgatgccccttcccatttcccttccttatactctgcaattcgaattaccgtatcacatctagaaagttaataattatctatattcttgtgggaaggggccttcatattaaattttcagtataaaaccataccctaaagagttttattgcttgcatacatgatgacactgtgatgccattattacaaaagtggctggtgttttttattgagccccacttaaaaccaagataaaagtctgcactatatttcatacttaacacgccaaatggtaggctttcagcaaaagcaaaatttaagcttaaaatattgaaatgttttataatgaatagaaattttgtcaaggaagtactttttaaagtttggaggaagggcactttaaagaaaagatgacttggaaagcaccaaatgagtgaaaataaagaattaagacccacagggaacgttggttttaatgggaaagcaaccaatgatatttttaggttgtcatgactgctcaagtatgttggaagggaaaaggcattgattattcttatcatcaatcacactttgaggtctcttggttgaattgtttaataaatggctaagggtattactttacctttcattgagtaaaaacatcagtgattctttaataagagagaagcgggtaaggctgtttcactgcttctctttgcgtttagctgaagaatgtggggtggaaagtgaatatggtgaccggataaccagaaattctcttctagtattaatgcttctcatttaaaaaattaaagataatgactgttaagagcatgataataaacattatctttacatgagtattctttcaatgatctaagttaaataacattgatatttattgagccaaaacttaagtgtgtccatgttacttctgttttggtagggaaagtgtagtcttcttgcttttaaaaatagttttcaaaaataatctgacttataaatcttcccattggcccatacattaccattgttctagtcacacttacaaaagtcctcttccccagttaatcattctgtatttccattgcttctcttttcttgagattaagaaaaccaaagcatcatctatagctacagtttaattttccaaaaaaccactctgagtatacatcacacacataccccgctggccattaaaaaagagaagcaatgtaaattttcttctagtctttccctgatttaatagggcctaagaagctacttttatctctttttggctccatctatttggtttaatgttaatgatcatggctgataatccttttatggaggaagggaacctattatgtcagcaataattggttcacttgctcctttggggtggaaaaaataagatatttcttaaagtaacaaggcctgaataaatgtgtggcagtctcaaattctattctatatctaaggtgtaatccttacatactaaagatagtgggatcattcttgtagatttctagcagactggtacattaaaaagtgacaatgtttggggtatgacagtataaaaaaaggtttaatttgagaaaaaggattaagttaaatagtaaacttagtgtgagattttaatcacaagtacaaaagagtgaagagcagccttcatgacaaggaatcatgtgaccagcccccaccccaaacataggttatcacatgtggattttgtttcattccgacaaaggaaaaggcccatacagttatcttaagtgttcattatatagagaccttatttaaccatgctcgattatcttacggaaaagaaaaacattacgataaatgtggtttccacatatcctagttctgtaaaaggtcaggtgtctcataaagtttgggttttggtgaaaatgtttgtacatgctgatgttaactactgcaataattataggattgtaaacggtaaaataacctgtatgactttgactgtcccagtgaccaaaatgcactttaatcttagaataatcaagactgaagcattaactgaaccctcatcttatattaatagcaccttctaagagaggcactgttttaaataggcacagaaacaaaaaatggtactttaaaagtactgttggaattcacaaatatatcccatgccacataaattaccgcttattataaaaatatcaataccctcaaatgccaatcagcaaaacataaatcaccaaaacatttcttcagtttagaacattgctcaattccacgataaaccatgctttatatttaaaaaataaattagagatgaatgtgaacctaaaagcatgtataatatatatatttaatactatatatacataattgctatatacttaagacattcttaggagtatttctacaaaaacaagttatcttttctttataaatcggaaatctgaacaccaacaatttgtcctttttcttttgttttaaaagaacagacatcatttatgcagctagagatttataaactaaattaaataagttaatacaatagcctcaactgtccctgtatttttcaccatggatctattttggcaacatggaggtatatctttcaaactgttccaggtcctacatgtgaaagagaagaagacatgaaaggatttcttaaatggaagtgctcattctaacctgacggtgacagaatcaattgatacaccatttcttcaagacaaaaaagcacatattcaaggaatagctcaaaaaatgctccagttttcacattatttcaaaactttatcggtagaatgactctgcacactaatttcactaagagtacataaacataggaaaatagtcctcaaaagatgcatttatgggcctatatttttcaacataaagtgctagcagatgtgtaagaagagctgggaatgtcttgagctgtaagtcctgagacctccacaccatggctggtcctggaggagttcagcattctgattttttcttaggttcaggatgatcatccaaggtggctggatgctcatttggaccacctggtgtctcacctgtgacagctaaaaggatgactttcagccacttctgcttcagttcctcactgtctgcagcaaagctgtgcacggacttagactgggtcagtttgaaactgtgtggcaggtctgcgctccttggcatttcatccaccacatagcccagaagtggaatggtggcctgggctctgacgtcctggggggcaccatacatgtacagcacaagagggtcttgcttggggatcacacaccaagctttctgccaaggttttgacttctccatatactgaagaaagctgcacaccacactgtttccagatacttctgctgattcaatctctaaaattccttttcttttcttttcttcactgtctgtgaatccacttatgatttgataacagtctttacaaactttgctcaatttaccaccatcatattcaagttgagctttgtagtcggagcatttccaacaaaccacatatccacatgctcgacaatgatgcctccttcgtgtcagtgcattgaaaggttctttacatttcatacacattgtcacttcattatctcggatccatcttggggctcttttccctagctcagcagtagaaacctctgagtgaatgtcattatcctttgcaattgcatttctgaaggtttcatgcctttgatgaaaagcatcgatggtttcttgaagggccttgatccattcttctttgtcttgcgcagaactggcctgcagttccagtgttctctctttcccagacacctggaaagtatgtggatattcttcattttgagtctctacaattttcattccatcaatgccaaccctggttcgaactgtgaatttagagcctaccaagctgaatttgggcacacagtacagcaacatgttgttgaataagaaaaggtagcgttcttgtgctgaagtgttccgagcagctagtttgaggatctgtccttcttttattagttcatttgaagggtttacaatgtcttcttcttctcccaacatttcataaatctctaagagtttctttaggttctccattttccttattgcactattagaatggcttgctgctgtagatataatttcaagtgattttttagcatcattccagtccagggaatcaggaggcaatttccttagatagtccttaaggagcatctcataccggggaatccgctgaacaggttctagcatgtgatgctgcaaagttaagctcccacagattttctgtttctgtaatgagaaaggttttctgaatttcttcaaccactgatttgaactggggaatacgttctgtcatgtttttaaccaattccattgcattatcaaatcctttcacatattctccatacatcttaaggaatggtgccaatttctgaaggatgtctccaattctaggagtagtttcccattcttgcattcgtttctccagctctggcaagaggaatttactatggaaggcatttattgatgaaatattagaaaagattttattcaccatctctgctggaaacgagcctcggtttgcttcttccaacagtttgcaataaaatacctcttaattgccattctgttacatgtaggcagaaggaggtctattccttcataatgtccagatggttgttaattttctaaattcacctccactctattttctgatctaagaggtcaagtcggttgacataagctctttcagtaagcaaaagttcattggctattttgtgaagtttttgctcattagtctccttcatctcatggtgctggtccagctgctccagttccagagggctttccccattttccctctcttgtaccttggtttctgtttctgcccctctttcttctagggggagcactgggcctatgcctggagtcctgtagctactgtcagaagcatttccatcacagctgtctgttgtgggtgatgcaggagctgtggcagtttcatctctttctccattcactatgtgcgtatcaagcaagggttcagaagcttgaatagaagtatctgagctaagagtggcagctttctcctcctcacattccatctggttttgtgctgccattacaccgttggccacacaagtctgtgcaccctgagtcttatctgtatcatttccctgcctctgtggcaagtgctgggagaggagtttttgttgaggtgtggttgtcaatccatgccttcctggggttctaggagcatttaggttcacagcagactctttcttcaaatcactataatttgataatgagctgcctccttcaaagcgactgatgagatctgataccttactgggtttttcttttgagacacaagaagcagaggcaggtttaatttcctccatccttggttttgcactaggtaaagctttatgcctgggggtttggtgtatattggacgaaggtgaattctgcaggtgtaatggctttggaggcacttgtggctttggacttgcagctgagtgttttgctggcctgttcccatttattccctgagcctcttcttcagatacattctcaccaaccagtgtggttgtgctgcttgtggagcaaggtggaactaaagcgatctttggacaggtactgctgccttataaaagctgaatttattcctcttggccagaagtcacaaatggttgaagtaaaactcccttcatttgttcttccagcgagccaaagcaagcctcccattaacccggtccattgcagataatctcacccagcacaggctcccctgctttccccacttcccagcccagcaaggat

SEQ ID NO: 14956 - RNA, 3670 nt, Homo sapiens
  source 1..3670: mol_type = other RNA
gctgggattacaggcatgagccactatgcccggcctatgcttattttaaaatgtcaattgtcactcacaaaatgaaatgctagtttggttaaaaaaaaaaaagtcttatatacagacagacatgactgttttgctaatgaagagaaccccccacaagtgatacattccaatatccatatactgtgtaatatataatgtgattctcttataatggtccccacagactagtttcttcccaaacctatatgtcactatgtatttggtatttatttattaaagtatgatatgagatttcttgatttacgttttccactaaaactaccacaatgaattttgggaaaaggggttgaccatcatataactcccggtgaccccaacaagttaaaactatcttgtagaagccatgtgctatttcatgtcaaaatacaggaaaagatactgcattctgccaaatgctcagtccagaaagtagaagaccatgattgacttcagattttttttttttttgcctcagtaaacagtacagaaaatgatctgagaatgaaattattttttaaaagcccaaaggagaaaaagaataacaagatatcatagtctagcatttacaggccaaggtcaaaaacctgggtgcaatggatcccatcagcatgtaattacatagattttatatcccttctgcagttaaaatatttcatcttatcttaaaacacattgctgtggtctggagaccagcagtctctcccccacatctctcttcattcttgcttgtttcagtttcttatcttattcctctctgccctttctgtgacagctaaaaggatgactttcagccacttctgcttcagttcctcactgtctgcagcaaagctgtgcacggacttagactgggtcagtttgaaactgtgtggcaggtctgcgctccttggcatttcatccaccacatagcccagaagtggaatggtggcctgggctctgacgtcctggggggcaccatacatgtacagcacaagagggtcttgcttggggatcacacaccaagctttctgccaaggttttgacttctccatatactgaagaaagctgcacaccacactgtttccagatacttctgctgattcaatctctaaaattccttttcttttcttttcttcactgtctgtgaatccacttatgatttgataacagtctttacaaactttgctcaatttaccaccatcatattcaagttgagctttgtagtcggagcatttccaacaaaccacatatccacatgctcgacaatgatgcctccttcgtgtcagtgcattgaaaggttctttacatttcatacacattgtcacttcattatctcggatccatcttggggctcttttccctagctcagcagtagaaacctctgagtgaatgtcattatcctttgcaattgcatttctgaaggtttcatgcctttgatgaaaagcatcgatggtttcttgaagggccttgatccattcttctttgtcttgcgcagaactggcctgcagttccagtgttctctctttcccagacacctggaaagtatgtggatattcttcattttgagtctctacaattttcattccatcaatgccaaccctggttcgaactgtgaatttagagcctaccaagctgaatttgggcacacagtacagcaacatgttgttgaataagaaaaggtagcgttcttgtgctgaagtgttccgagcagctagtttgaggatctgtccttcttttattagttcatttgaagggtttacaatgtcttcttcttctcccaacatttcataaatctctaagagtttctttaggttctccattttccttattgcactattagaatggcttgctgctgtagatataatttcaagtgattttttagcatcattccagtccagggaatcaggaggcaatttccttagatagtccttaaggagcatctcataccggggaatccgctgaacaggttctagcatgtgatgctgcaaagttaagctcccacagattttctgtttctgaatttcttcaaccactgatttgaactggggaatacgttctgtcatgtttttaaccaattccattgcattatcaaatcctttcacatattctccatacatcttaaggaatggtgccaatttctgaaggatgtctccaattctaggagtagtttcccattcttgcattcgtttctccagctctggcaagaggaatttactatggaaggcatttattgatgaaatattagaaaagattttattcaccatctctgctggaaacgagcctcggtttgcttcttccaacagtttgcaataaaatacctgatctaagaggtcaagtcggttgacataagctctttcagtaagcaaaagttcattggctattttgtgaagtttttgctcattagtctccttcatctcatggtgctggtccagctgctccagttccagagggctttccccattttccctctcttgtaccttggtttctgtttctgcccctctttcttctagggggagcactgggcctatgcctggagtcctgtagctactgtcagaagcatttccatcacagctgtctgttgtgggtgatgcaggagctgtggcagtttcatctctttctccattcactatgtgcgtatcaagcaagggttcagaagcttgaatagaagtatctgagctaagagtggcagctttctcctcctcacattccatctggttttgtgctgccattacaccgttggccacacaagtctgtgcaccctgagtcttatctgtatcatttccctgcctctgtggcaagtgctgggagaggagtttttgttgaggtgtggttgtcaatccatgccttcctggggttctaggagcatttaggttcacagcagactctttcttcaaatcactataatttgataatgagctgcctccttcaaagcgactgatgagatctgataccttactgggtttttcttttgagacacaagaagcagaggcaggtttaatttcctccatccttggttttgcactaggtaaagctttatgcctgggggtttggtgtatattggacgaaggtgaattctgcaggtgtaatggctttggaggcacttgtggctttggacttgcagctgagtgttttgctggcctgttcccatttattccctgagcctcttcttcagatacattctcaccaaccagtgtggttgtgctgcttgtggagcaaggtggaactaaagcgatctttggacaggtactgctgcctgtggctcctgagggcacctggcccttgaaggcagcggtccctacacgtcccaggtgcgacgcgggcctgctccagggccggggcaccccgggcggcaggtaggaggggttggacttccgccggatcgccacccgcctgaagttggagccgccctcgtcgctcatcctgccgggctcgaccgccgctccccgactcctcccgctcccgtccagccgcgagcggcccctggggggcgtcgcctgcatgcccaggttcggcgcgactccgggggcgccctctactgcggcgtctcctcagcgagtgcctcctctccctctccttcccggtacgctccctcccggcgtcgcggcgagtttggctgcggcgactcctgcggcagtcgcagcgtctcggtatctgc

SEQ ID NO: 14957 - RNA, 3444 nt, Homo sapiens
  source 1..3444: mol_type = other RNA
gctgggattacaggcatgagccactatgcccggcctatgcttattttaaaatgtcaattgtcactcacaaaatgaaatgctagtttggttaaaaaaaaaaaagtcttatatacagacagacatgactgttttgctaatgaagagaaccccccacaagtgatacattccaatatccatatactgtgtaatatataatgtgattctcttataatggtccccacagactagtttcttcccaaacctatatgtcactatgtatttggtatttatttattaaagtatgatatgagatttcttgatttacgttttccactaaaactaccacaatgaattttgggaaaaggggttgaccatcatataactcccggtgaccccaacaagttaaaactatcttgtagaagccatgtgctatttcatgtcaaaatacaggaaaagatactgcattctgccaaatgctcagtccagaaagtagaagaccatgattgacttcagattttttttttttttgcctcagtaaacagtacagaaaatgatctgagaatgaaattattttttaaaagcccaaaggagaaaaagaataacaagatatcatagtctagcatttacaggccaaggtcaaaaacctgggtgcaatggatcccatcagcatgtaattacatagattttatatcccttctgcagttaaaatatttcatcttatcttaaaacacattgctgtggtctggagaccagcagtctctcccccacatctctcttcattcttgcttgtttcagtttcttatcttattcctctctgccctttctgtgacagctaaaaggatgactttcagccacttctgcttcagttcctcactgtctgcagcaaagctgtgcacggacttagactgggtcagtttgaaactgtgtggcaggtctgcgctccttggcatttcatccaccacatagcccagaagtggaatggtggcctgggctctgacgtcctggggggcaccatacatgtacagcacaagagggtcttgcttggggatcacacaccaagctttctgccaaggttttgacttctccatatactgaagaaagctgcacaccacactgtttccagatacttctgctgattcaatctctaaaattccttttcttttcttttcttcactgtctgtgaatccacttatgatttgataacagtctttacaaactttgctcaatttaccaccatcatattcaagttgagctttgtagtcggagcatttccaacaaaccacatatccacatgctcgacaatgatgcctccttcgtgtcagtgcattgaaaggttctttacatttcatacacattgtcacttcattatctcggatccatcttggggctcttttccctagctcagcagtagaaacctctgagtgaatgtcattatcctttgcaattgcatttctgaaggtttcatgcctttgatgaaaagcatcgatggtttcttgaagggccttgatccattcttctttgtcttgcgcagaactggcctgcagttccagtgttctctctttcccagacacctggaaagtatgtggatattcttcattttgagtctctacaattttcattccatcaatgccaaccctggttcgaactgtgaatttagagcctaccaagctgaatttgggcacacagtacagcaacatgttgttgaataagaaaaggtagcgttcttgtgctgaagtgttccgagcagctagtttgaggatctgtccttcttttattagttcatttgaagggtttacaatgtcttcttcttctcccaacatttcataaatctctaagagtttctttaggttctccattttccttattgcactattagaatggcttgctgctgtagatataatttcaagtgattttttagcatcattccagtccagggaatcaggaggcaatttccttagatagtccttaaggagcatctcataccggggaatccgctgaacaggttctagcatgtgatgctgcaaagttaagctcccacagattttctgtttctgaatttcttcaaccactgatttgaactggggaatacgttctgtcatgtttttaaccaattccattgcattatcaaatcctttcacatattctccatacatcttaaggaatggtgccaatttctgaaggatgtctccaattctaggagtagtttcccattcttgcattcgtttctccagctctggcaagaggaatttactatggaaggcatttattgatgaaatattagaaaagattttattcaccatctctgctggaaacgagcctcggtttgcttcttccaacagtttgcaataaaatacctgatctaagaggtcaagtcggttgacataagctctttcagtaagcaaaagttcattggctattttgtgaagtttttgctcattagtctccttcatctcatggtgctggtccagctgctccagttccagagggctttccccattttccctctcttgtaccttggtttctgtttctgcccctctttcttctagggggagcactgggcctatgcctggagtcctgtagctactgtcagaagcatttccatcacagctgtctgttgtgggtgatgcaggagctgtggcagtttcatctctttctccattcactatgtgcgtatcaagcaagggttcagaagcttgaatagaagtatctgagctaagagtggcagctttctcctcctcacattccatctggttttgtgctgccattacaccgttggccacacaagtctgtgcaccctgagtcttatctgtatcatttccctgcctctgtggcaagtgctgggagaggagtttttgttgaggtgtggttgtcaatccatgccttcctggggttctaggagcatttaggttcacagcagactctttcttcaaatcactataatttgataatgagctgcctccttcaaagcgactgatgagatctgataccttactgggtttttcttttgagacacaagaagcagaggcaggtttaatttcctccatccttggttttgcactaggtaaagctttatgcctgggggtttggtgtatattggacgaaggtgaattctgcaggtgtaatggctttggaggcacttgtggctttggacttgcagctgagtgttttgctggcctgttcccatttattccctgagcctcttcttcagatacattctcaccaaccagtgtggttgtgctgcttgtggagcaaggtggaactaaagcgatctttggacaggtactgctgccttataaaagctgaatttattcctcttggccagaagtcacaaatggttgaagtaaaactcccttcatttgttcttccagcgagccaaagcaagcctcccattaacccggtccattgcagataatctcacccagcacaggctcccctgctttccccacttcccagcccagcaaggat

SEQ ID NO: 14958 - RNA, 3445 nt, Homo sapiens
  source 1..3445: mol_type = other RNA
gctgggattacaggcatgagccactatgcccggcctatgcttattttaaaatgtcaattgtcactcacaaaatgaaatgctagtttggttaaaaaaaaaaaagtcttatatacagacagacatgactgttttgctaatgaagagaaccccccacaagtgatacattccaatatccatatactgtgtaatatataatgtgattctcttataatggtccccacagactagtttcttcccaaacctatatgtcactatgtatttggtatttatttattaaagtatgatatgagatttcttgatttacgttttccactaaaactaccacaatgaattttgggaaaaggggttgaccatcatataactcccggtgaccccaacaagttaaaactatcttgtagaagccatgtgctatttcatgtcaaaatacaggaaaagatactgcattctgccaaatgctcagtccagaaagtagaagaccatgattgacttcagattttttttttttttgcctcagtaaacagtacagaaaatgatctgagaatgaaattattttttaaaagcccaaaggagaaaaagaataacaagatatcatagtctagcatttacaggccaaggtcaaaaacctgggtgcaatggatcccatcagcatgtaattacatagattttatatcccttctgcagttaaaatatttcatcttatcttaaaacacattgctgtggtctggagaccagcagtctctcccccacatctctcttcattcttgcttgtttcagtttcttatcttattcctctctgccctttctgtgacagctaaaaggatgactttcagccacttctgcttcagttcctcactgtctgcagcaaagctgtgcacggacttagactgggtcagtttgaaactgtgtggcaggtctgcgctccttggcatttcatccaccacatagcccagaagtggaatggtggcctgggctctgacgtcctggggggcaccatacatgtacagcacaagagggtcttgcttggggatcacacaccaagctttctgccaaggttttgacttctccatatactgaagaaagctgcacaccacactgtttccagatacttctgctgattcaatctctaaaattccttttcttttcttttcttcactgtctgtgaatccacttatgatttgataacagtctttacaaactttgctcaatttaccaccatcatattcaagttgagctttgtagtcggagcatttccaacaaaccacatatccacatgctcgacaatgatgcctccttcgtgtcagtgcattgaaaggttctttacatttcatacacattgtcacttcattatctcggatccatcttggggctcttttccctagctcagcagtagaaacctctgagtgaatgtcattatcctttgcaattgcatttctgaaggtttcatgcctttgatgaaaagcatcgatggtttcttgaagggccttgatccattcttctttgtcttgcgcagaactggcctgcagttccagtgttctctctttcccagacacctggaaagtatgtggatattcttcattttgagtctctacaattttcattccatcaatgccaaccctggttcgaactgtgaatttagagcctaccaagctgaatttgggcacacagtacagcaacatgttgttgaataagaaaaggtagcgttcttgtgctgaagtgttccgagcagctagtttgaggatctgtccttcttttattagttcatttgaagggtttacaatgtcttcttcttctcccaacatttcataaatctctaagagtttctttaggttctccattttccttattgcactattagaatggcttgctgctgtagatataatttcaagtgattttttagcatcattccagtccagggaatcaggaggcaatttccttagatagtccttaaggagcatctcataccggggaatccgctgaacaggttctagcatgtgatgctgcaaagttaagctcccacagattttctgtttctgaatttcttcaaccactgatttgaactggggaatacgttctgtcatgtttttaaccaattccattgcattatcaaatcctttcacatattctccatacatcttaaggaatggtgccaatttctgaaggatgtctccaattctaggagtagtttcccattcttgcattcgtttctccagctctggcaagaggaatttactatggaaggcatttattgatgaaatattagaaaagattttattcaccatctctgctggaaacgagcctcggtttgcttcttccaacagtttgcaataaaatacctgatctaagaggtcaagtcggttgacataagctctttcagtaagcaaaagttcattggctattttgtgaagtttttgctcattagtctccttcatctcatggtgctggtccagctgctccagttccagagggctttccccattttccctctcttgtaccttggtttctgtttctgcccctctttcttctagggggagcactgggcctatgcctggagtcctgtagctactgtcagaagcatttccatcacagctgtctgttgtgggtgatgcaggagctgtggcagtttcatctctttctccattcactatgtgcgtatcaagcaagggttcagaagcttgaatagaagtatctgagctaagagtggcagctttctcctcctcacattccatctggttttgtgctgccattacaccgttggccacacaagtctgtgcaccctgagtcttatctgtatcatttccctgcctctgtggcaagtgctgggagaggagtttttgttgaggtgtggttgtcaatccatgccttcctggggttctaggagcatttaggttcacagcagactctttcttcaaatcactataatttgataatgagctgcctccttcaaagcgactgatgagatctgataccttactgggtttttcttttgagacacaagaagcagaggcaggtttaatttcctccatccttggttttgcactaggtaaagctttatgcctgggggtttggtgtatattggacgaaggtgaattctgcaggtgtaatggctttggaggcacttgtggctttggacttgcagctgagtgttttgctggcctgttcccatttattccctgagcctcttcttcagatacattctcaccaaccagtgtggttgtgctgcttgtggagcaaggtggaactaaagcgatctttggacaggtactgctgccttgatcagtggacatgatttcacatatactgataattaatctactctggtttaataaaaagatatttggctttactcttttaaagttcatgtgataaaatctcactcctggctgtaaagcttcagggaggctgaagattacacaggatctgccaggagctcagaccaatgcactat

SEQ ID NO: 14959 - RNA, 5675 nt, Homo sapiens
  source 1..5675: mol_type = other RNA
gctgggattacaggcatgagccactatgcctcgcccagaaactgagtttctactctggcaagttaaacataaaaaattagtacatatcaggctgggtggctctaggccacatgcaagcaagctgcaaactgaattgcctctgcagctgcagaaggctaatttctacattgatatttggaaacactaacagctagaaaacaccactctactcatttttaaaaataagatcatattaaatgatgttacatgcatcatttatatattgctcacagtgccagcatcctcaaatatggttttaattttggtagatatcttgctagggggagcacatttccaagttatccagatatagggccctctttccttctctttctgtccacatgcaaccagatgctttgtggagttaaagttgacatttatttaaatgccacttggtgtctggtttttcacctttaatttagggttttctagctgggatgtaaaagaatcacttggagggatttttcaaaataccaatggccaggccactagccagtcaatcagaagcaaaatctccttggatgggacctggaaatctttagagttttccagcattttaatgaacatccctgattaagaaccaccgggtcttaagagtgtggcatatgtatttttcaagttcctagaggctctccaaaacaaaacaaaaaaaatctgctttattctctgcctggtgttgatgcatcagtctctttagccgttagtctgatcctggaaatttatggtcataatttgatgagcaatgttgggaatgacttcttctttttttttttttttttttgttttgagacagagtctcactctgttgaccaggctggagtgtagtggggcgatctccgctcactgcaacctccaccccaatactttcatttttaaatattatttatggcatccagatttgcataagatggactgggtcaatggccatgccctttataaatcaatattcttaagttctgcaaattcagtttcctaaagagccaaatcacatcctactcatcagcaaggcgggtagacatcattttcacaatcacttctaattttccaccattgtaaaaaaaaataaaatatgtaatcactttcttattgtaaaataaagaatttacttttccaggacctactgcctccctgtcccccccccccctttttttttttcaaacaatcttgaaccctttgtcacgagtcagttgccaagagaagcctatttgttggtttgagagcagttcatgcagacacagaccacttcctctgagaattcatttgcttcctcaggatggaatctggctgggcctctgaccttgctggtcacgtgggccggggcctccatcagtcataccctggactcctatctgtgtctaaacaccacgccccacccccaactgcacggcagccactcgcatagcactctgggagggctgtgggcatgagcagcgaggactccatcagcagctcccccacatgagccctgctgatgagggggcttgcgaagcagctttgatgtgctggtaaatccaggtgcaaaacagaactcaagttaaggcctccgcacagcactgcgttctaactgtgaaggattcttactctagtgtcctgtgtggaggtattggaattgtccattgctaagactcagaggagaaaagcacttagcatcgcaggacttggagcaccggtgctgaggcaacccttcattcattcgtcggatgtgtgttaaggcccagggcaggggtcacggattctcctctcacacagcacgtgggtggcaggaccaacaccgggtctgacctcccagccgggggcacaggctgctcaccccaggcctggaatctgtcagatgcccttcccgtgctgacttgacttagacaggcctcctgaccttcccacaaaggtcatgtgtgatttgcaggggttctggccgcttgaaaggttcctgagaaagcacatgcaatgaggacagagcttgcagagggaggacaggcatgcagaaggctctgtgtgcagccccagacctgggtaccttcatcaccgtcctcaccccacctccgggtgtgcacatagggagcaggtctcctgtgttatggcccaagcagggctgttaggacactgagaacattccctcctcccgcaggagagagaggtccaaggtgccctacatcgtgcgccagtgcgtggaggagatcgagcgccgaggcatggaggaggtgggcatctaccgcatgtctggggtggccgcagacatccaggcactgaaggcagccttcaacgtcagtgagtgtcggcctgcgcaggacgggatggaggtgtgggcagtggtgtccgcgatgagatctcagagtgctccacggcccaggcatgtcacatccttctctgtgtcttttcttcatttatcaggatcttcaaggaggccgctgcatttccgtgctctttccagataacaaggacgtgtcggtgatgatgagcgagatggacgtgaacgccatcgcaggcacgctgaagctgtatttccgtgagctgcccgagcccctcttcactgacgagttctaccccaacttcgcagagggcatcggtgagcactggaggccttggcctcatgggagacgtctcctccacgtgcactgctgccctcagaggctgtgaaaagtgaggtgtgggaacctgagctgtgcttcctctgccatggtcggaattttaacccaacctcaaaaagcaggggaccaaaactgagcctatcctggaaggccttgcccatccccagaggggtccccatccatatttctcaaggaggccaagtgggtgaaatggtcagcactgccgtgctgtggggtcctaaagtctgctgtcctccttcctgcagaccagggctaaacactggtgcccaggtgctcttgccatgggtcctggtccagccaagcatggtttcaaacatgacctgacccttagtcaacctggaggctgatgtctagagtgggcgctggagcgtgcagcacctgtagcctgtgcatcacccttagggcaggtctgcctcccgggcccatgcacagaggacctggtctcccagcctgcaggtgcccctgtggtgtccaggacaacgaggggttctctgcgtacttggtggggctgggaccctcccacttcccacctccttgtgtccctcactcccctgtttcattccatgctgagcctcccctgccttgggctccctggggagggggtggtggcaggagttgcccgagggcagctctgcccatgagcagctgctctagcggctcctcctgctgctgtttgccgggtgctgctgaccccaaggctggagtcagcttgcagcacagccagggtcgaggtcactccctccctgaggactctagcacggcacagcccctctgcctctctcctggtggtggcgttgaaacagcaccctctgcttcggtcctctaataagatgctggaatgtaatcctggacaatccgtgtcctggcagcatttggtcttcctctaagcgcctggctccgctgttctcaggagtgggttctgaagtctccgcctcctgcctcaacagcctgtgtggtggcaaagccggtgtggggctggggaacgcagcgttctccaggagggggacccggctctccttctgcaatgcaggcgaaggcctagatgccagtgtgacctcccacaaggcgtggcttccagactccccggccggaagtgatgcttttttgccgtgggccctgggtttgaagcagcctggctttctcttggtaagtggctggtgtcttagcagctgcaatctgagctcagccacctacacaccaccgtggccgacactttcattaagaagtttcctgagacgacttgcgtgcatgttgacttcatgatcagcgccgctgggaagaacccctgagccggtggggtggggctgtggccaccgctctggcacgagcccctcagtcttgggtggtttttgcctggtccaggatttggtgttgctgctgagttcagcctttccaccacctccgcatgggctgtgggtgttgtcagctgcctcccgccttggcttcagtagctcacccagcttacaggggagctgccctgggctggagatgggcacgcaccctgggtcctacttgaatgaatgcagcttgaggagacccggccatatacactgggccacgggttaccttcggcaatgcccacatcagctgtcagcctgagcctccccaggagagcaaggctcacatgacaaaggctgcccgtggccaatgaggtggctgagcccagccaggacctttctcggactcccgggatgtggctctgctcgtgagctgcctggtcagctctctcggggtgagaggggcttgtcacacgggcccctgcctgcagtgtgacccttctcagcttctctcagcagccctgcctgcggagtgtcaccgccaccatgatcatttccctgacactgcgagggtgtggggacgtcctgggtagagacagggcccatggcagcagcaggctcaggggcgccctgcactggtgggctggggacctggtggagaccacgccaagggctggacaaggggacgagcctccaccctggcctctccgcaggcctcagcagcccctcccacaggcagaagggttgacactgggttctgccctcactgcaagagctgcaagtgccatgtgctgttctgcccaatctggtgtctgcaggtgagggaagggctgccgctggcccgtttctgagtgttcagcacctaagggtgacagcactgtctgtccctaccctccaggtcctgtttgaaaatcaaacccatgctcacaggccaatttttttttcttttagagacagggtctcactttgtcacccaagctggagtgcagtggtgcgattatagctcaatgcagcctccaattcccggactcaagggaccttcctgcctcagcctgccaagtagcttggactatagctgtgtgttttattattattttgtagacatggggtctggctatgttgtccaggctattctcaaaattcccggcctcgagcaatcctcctgccttggcctctcaaaggttgggattacaggtgtgaggcaaggcacccagctcagccacagagccctgttgcatctctcttactaggagcaagagctgactgccccctcatccccattccagagtgttggggctgtgttgagccgaggccaggccactggcatgggcccagggagcgggatcattcactgctgccccaaatctgagatcattccaccttgacaagacttcctcatccaatccctttacttgacagctggggaaaccaatgcgcacagagcacccccagctcactcggggtctcagagctgatccatgagcagaggctgagatcctgggatcttgtcccccagcctccctgcaagcttactccctttctgctggaagagatggggccggacctcgaccagcagccctggcctggacgtgactgtgctcatgcaggtattgaggccgagatgccccagcatcatatgtttttctttttttttttctttcttttttgagattggctcactgcaacctctgcctcccgcttaaagtgattctcctgcctcagtcttccaagtagctgggcctacaggcttgta

SEQ ID NO: 14960 - RNA, 6197 nt, Homo sapiens
  source 1..6197: mol_type = other RNA
gctgggattacaggcatgagccactatgcctcgcccagaaactgagtttctactctggcaagttaaacataaaaaattagtacatatcaggctgggtggctctaggccacatgcaagcaagctgcaaactgaattgcctctgcagctgcagaaggctaatttctacattgatatttggaaacactaacagctagaaaacaccactctactcatttttaaaaataagatcatattaaatgatgttacatgcatcatttatatattgctcacagtgccagcatcctcaaatatggttttaattttggtagatatcttgctagggggagcacatttccaagttatccagatatagggccctctttccttctctttctgtccacatgcaaccagatgctttgtggagttaaagttgacatttatttaaatgccacttggtgtctggtttttcacctttaatttagggttttctagctgggatgtaaaagaatcacttggagggatttttcaaaataccaatggccaggccactagccagtcaatcagaagcaaaatctccttggatgggacctggaaatctttagagttttccagcattttaatgaacatccctgattaagaaccaccgggtcttaagagtgtggcatatgtatttttcaagttcctagaggctctccaaaacaaaacaaaaaaaatctgctttattctctgcctggtgttgatgcatcagtctctttagccgttagtctgatcctggaaatttatggtcataatttgatgagcaatgttgggaatgacttcttctttttttttttttttttttgttttgagacagagtctcactctgttgaccaggctggagtgtagtggggcgatctccgctcactgcaacctccaccccaatactttcatttttaaatattatttatggcatccagatttgcataagatggactgggtcaatggccatgccctttataaatcaatattcttaagttctgcaaattcagtttcctaaagagccaaatcacatcctactcatcagcaaggcgggtagacatcattttcacaatcacttctaattttccaccattgtaaaaaaaaataaaatatgtaatcactttcttattgtaaaataaagaatttacttttccaggacctactgcctccctgtcccccccccccctttttttttttcaaacaatcttgaaccctttgtcacgagtcagttgccaagagaagcctatttgttggtttgagagcagttcatgcagacacagaccacttcctctgagaattcatttgcttcctcaggatggaatctggctgggcctctgaccttgctggtcacgtgggccggggcctccatcagtcataccctggactcctatctgtgtctaaacaccacgccccacccccaactgcacggcagccactcgcatagcactctgggagggctgtgggcatgagcagcgaggactccatcagcagctcccccacatgagccctgctgatgagggggcttgcgaagcagctttgatgtgctggtaaatccaggtgcaaaacagaactcaagttaaggcctccgcacagcactgcgttctaactgtgaaggattcttactctagtgtcctgtgtggaggtattggaattgtccattgctaagactcagaggagaaaagcacttagcatcgcaggacttggagcaccggtgctgaggcaacccttcattcattcgtcggatgtgtgttaaggcccagggcaggggtcacggattctcctctcacacagcacgtgggtggcaggaccaacaccgggtctgacctcccagccgggggcacaggctgctcaccccaggcctggaatctgtcagatgcccttcccgtgctgacttgacttagacaggcctcctgaccttcccacaaaggtcatgtgtgatttgcaggggttctggccgcttgaaaggttcctgagaaagcacatgcaatgaggacagagcttgcagagggaggacaggcatgcagaaggctctgtgtgcagccccagacctgggtaccttcatcaccgtcctcaccccacctccgggtgtgcacatagggagcaggtctcctgtgttatggcccaagcagggctgttaggacactgagaacattccctcctcccgcaggagagagaggtccaaggtgccctacatcgtgcgccagtgcgtggaggagatcgagcgccgaggcatggaggaggtgggcatctaccgcatgtctggggtggccgcagacatccaggcactgaaggcagccttcaacgtcagtgagtgtcggcctgcgcaggacgggatggaggtgtgggcagtggtgtccgcgatgagatctcagagtgctccacggcccaggcatgtcacatccttctctgtgtcttttcttcatttatcaggatcttcaaggaggccgctgcatttccgtgctctttccagataacaaggacgtgtcggtgatgatgagcgagatggacgtgaacgccatcgcaggcacgctgaagctgtatttccgtgagctgcccgagcccctcttcactgacgagttctaccccaacttcgcagagggcatcggtgagcactggaggccttggcctcatgggagacgtctcctccacgtgcactgctgccctcagaggctgtgaaaagtgaggtgtgggaacctgagctgtgcttcctctgccatggtcggaattttaacccaacctcaaaaagcaggggaccaaaactgagcctatcctggaaggccttgcccatccccagaggggtccccatccatatttctcaaggaggccaagtgggtgaaatggtcagcactgccgtgctgtggggtcctaaagtctgctgtcctccttcctgcagaccagggctaaacactggtgcccaggtgctcttgccatgggtcctggtccagccaagcatggtttcaaacatgacctgacccttagtcaacctggaggctgatgtctagagtgggcgctggagcgtgcagcacctgtagcctgtgcatcacccttagggcaggtctgcctcccgggcccatgcacagaggacctggtctcccagcctgcaggtgcccctgtggtgtccaggacaacgaggggttctctgcgtacttggtggggctgggaccctcccacttcccacctccttgtgtccctcactcccctgtttcattccatgctgagcctcccctgccttgggctccctggggagggggtggtggcaggagttgcccgagggcagctctgcccatgagcagctgctctagcggctcctcctgctgctgtttgccgggtgctgctgaccccaaggctggagtcagcttgcagcacagccagggtcgaggtcactccctccctgaggactctagcacggcacagcccctctgcctctctcctggtggtggcgttgaaacagcaccctctgcttcggtcctctaataagatgctggaatgtaatcctggacaatccgtgtcctggcagcatttggtcttcctctaagcgcctggctccgctgttctcaggagtgggttctgaagtctccgcctcctgcctcaacagcctgtgtggtggcaaagccggtgtggggctggggaacgcagcgttctccaggagggggacccggctctccttctgcaatgcaggcgaaggcctagatgccagtgtgacctcccacaaggcgtggcttccagactccccggccggaagtgatgcttttttgccgtgggccctgggtttgaagcagcctggctttctcttggtaagtggctggtgtcttagcagctgcaatctgagctcagccacctacacaccaccgtggccgacactttcattaagaagtttcctgagacgacttgcgtgcatgttgacttcatgatcagcgccgctgggaagaacccctgagccggtggggtggggctgtggccaccgctctggcacgagcccctcagtcttgggtggtttttgcctggtccaggatttggtgttgctgctgagttcagcctttccaccacctccgcatgggctgtgggtgttgtcagctgcctcccgccttggcttcagtagctcacccagcttacaggggagctgccctgggctggagatgggcacgcaccctgggtcctatgtgtttcaggaactgaggttcagctggcagtgggatgaggctggcccccttctccgctttcgttccgggaggcctcccgtagagcggtaggggctcgagatggcatttcgtttggggcacgagctggtccgggaggtctgggatctctggttctgacctctgggcacctgctgcagctgtggctgaggcccagaaatgtgaagggcctccatccactccagtagtgaccccaacgtggggttcaatgtggaggggggaggggctgctgcggcagctgcaggagcagaagtgccacaccttgttcttctcatgcccacatccatgcttgcagctgggaagggggcaggaatcagcgaggtgacctgggctgagtcctgggaatgggaagaggtggcaggaaggggatctgaggaggagaacagggggcctggtggtttgtgcttcttcccagacatgggagctgtagaggggacacctgcagcagatgctaagggggccagtaggcccaggcagtcttgggacttgtgtgtctcctgctgtacatccatactgggtgctttagaaatggcaggcagaccagaagtccctgttgcaagtgaggacaaagtgtgggaaggtcgtgagggtctgcagtccgagatggccttgtcctcaacctgcagtgcactgttgatgcgctggaatgccgcctccttctcccggtccaggtcttcaacagtgacccggtaccccagctctaagggaggtggcagcatcaaaggctcccctcgcctgcgtggcagcaggggaaacttgtgtgtactgggcctagaggcctcggatgtggaggagtcattcctgagggcgagtgtctgccctggtgctatatctgctgccttttcacactgggtgtgacctgaagagacagcctgaggcctgtcctcactcactgtctttgaggaactgagggtcagctggcagtgggatgaggctggccccctcctccgctttagccccggcaagcctcccgtggagctgtaggagctggagatggcatttcggttggtgcaggagctcgtccaggaggtctgggatgtctggttatatctgatttctgacctctgggcatggaggtctgtctgcagaggcccgggcccgggcacaaagggagagaggcctctattgtcccgcaggggccgaaatgcagacggtgcatccccggtgacctcggggacccttctctgatcaccaggattctcttggactctagggtccttgtcctgctcaggcatccctgccccgctctccttgagggccctcaacactatcttccctggacacaagtctggggacagccgggtgttgtggaccccaaaggggtgactcccggctcctgggccccacagagagtccatgttctcagtgcagtggctgagctggaggacgccctggaactcggagcacacagcactggcttgctgtggtacctgtgcaatcaaattgaaggcaggatcccaggaaggaaggcagggcttgcaggatcacggaaaaccttcttagagttgtcttgacaccactgatgtcaagtgtccgggtgcttgtaggatggcctgccactcagtccacgggcaggagcaacggggagatcccacaggcaaagtgaactgggggatgggctgaacgggctccaggcaactgagccctactggcaggtcctcggcctgggcccgaacaggaaggaggggcacagagtgcccaggtaaccgctcctgggagcagtggggaaccgtcggttgcttgaactctcgagagctgggctctgagcgtcctcgtccagccgccaactcggccaacggctaagccagcagtttcttctgttgccgggcaacgcgccttttaaacctgagggagcgggcgcgtgagcacatcacggcgcccgtgacagagcgagcttaacggattaataagcgcagccaggtacccgcgcgaggcgcttgctggcaatggcgggaggcggacgtggggggtcatgcaataggtactggaaggagagaggcgagc

SEQ ID NO: 14961 - RNA, 6733 nt, Homo sapiens
  source 1..6733: mol_type = other RNA
gctgggattacaggcatgagccactatgcctggcccagaaactgagtttctactctggcaagttaaacaaaaaattagtacatatcaggctgggtggctctaggccacatgcaagcaagctgcaaactgaattgcctctgcagctgcagaaggctaatttctacattgatatttggaaacactaacagctagaaaacaccactctactcatttttaaaaataagatcatattaaatgatgttacatgcatcatttatatattgctcgcagtgccagcatcctcaaatatggttttaattttggtagatatcttgctagggggagcacatttccaagttatccagatatagggccctctttccttctctttctgtccacgtgcaaccagatgctttgtggagttaaagttgacatttatttaaatgccacttggtgtctggtttttcacctttaatttagggttttctagctgggatgtaaaagaatcacttggagggatttttcaaaataccaatggccaggccactagccagtcaatcagaagcaaaatctccttggatgggacctggaagtctttacagttttccagcattttaatgaacatccctgattaagaaccaccgggtcttaagagtgtgccatatgtatttttcaagttcctagaggctctccaaaacaaaacaaaaaaaatctgctttattctctgcctggtgttgatgcatcagtctctttagccgttagtctgatcctggaaatttatggtcataatttgatgagcaatgttgggaatgacttcttcttctttttttttttttttttgttttgagacagagtctcactctgttgaccaggctggagtgtagtggggcgatctccgctcactgcaacctccaccccaatactttcatttttaaatattatttatggcatccagatttgcataagatggactgggtcaatggccatgccctttataaatcaatattcttaagttctgcaaattcagtttcctaaagagccaaatcacatcctactcatcagcaaggcgggtagacatcattttcacaatcacttctaattttccaccattgtaaaaaaaataaaatatgtaatcactttcttattgtaaaataaagaatttacttttccaggacctactgcctccctgttccccccccccttttttttttttcaaacaatcttgaaccctttgtcacgagtcagttgccaagagaagcctatttgttggtttgagagcagttcatgcagacacagaccacttcctctgagaattcatttgcttccccaggatggaatctggctgggcctctgaccttgctggtcacgtgggccggggcctccatcagtcataccctggactcctatctgtgtctaaacacacgccccacccccaactgcacggcagccactcgcatagcactctgggagggctgtgggcatgagcagcgaggactccatcagcagctcccccacataagccctgctgatgagggggcttgcgaagcagctttgatgtgctggtaaatccaggtgcaaaacagaactcaagttaaggcctccgcacagcactgcgttctaactgtgaaggattcttactctagtgtcctgtgtggaggtattggaattgtccattgctaagactcagaggagaaaagcacttagcatcgcaggacttggagcaccggtgctgaggcaacccttcattcattcgtcggatgtgtgttaaggcccagggcaggggtcagggtttctcctctcacacagcacgtgggtggcaggaccaacaccgggtctgacctcccagccgggggcacaggctgctaaccccaggcctggaatctgtcagatgcccttcccgtgctgacttgacttagacaggcctcctgaccttcccgcaaaggtcatgtgtgattcgcaggggttctggccgcttgaaaggttcctgagaaagtacatgcaatgaggacagagcttgcagagggaggacaggcatgcagaaggctctgtgtgcagccccagacctgggtaccttcgtcaccgtcctcaccccacctccgggtgcgcagatagggagcaggtctcctgtgttatggcccaagcagggctgttaggacactgagaacattccctcctcccgcaggagagagaggtccaaggtgccctacatcgtgcgccagtgcatggaggagatcgagcgccgaggcatggaggaggtgggcatctaccgcatgtctggggtggccgcagacatccaggcactgaaggcaggcttcaacgtcagtgagtgtcggcctgcgcaggacgggatggaggtgtgggcagtggtgtccccgatgagatctcagagtgctccatggcccaggcatgtcacatccttctctgtgtcttttcttcatttatcaggatcttcaaggaggccgctgcatttccgtgctctttccagataacaaggacgtgtcagtgatgatgagcgagatggacgtgaacgccatcgcaggcatgctgaagctgtacttccgtgagctgcccgagcccctcttcactgacgagttctaccccaacttcgcagagggcatcggtgagcactggaggccttggcctcatgggagacgtctcctccacgtgcactgctgccctcagaggctgtgaaaagtgaggtgtgggaacccgagctgtgcttcctctgccatggtcggaattttaacccaacctcaaaaagcaggggaccaaaactgagcctatcctggaaggccttgcccatccccagagggctccccatccatatttctcaaggaggccaagtgggtgaaatggtcagcactgccgtgctgtggggtcctaaagtctgctgtcctccttcctgcagaccagggctaaacactggtgcccaggtgctcttgccatgggtcctggtccagccaagcatggtttcaaacatgacctgacccttagtcaacctggaggctgatgtctagagtgggcgctggagcgtgcagcacctgtagcctgtgcatcacccttagggcaggtctgcctcccgggcccatgcacagaggacctggtctcccagcctgcaggtgcccctgtggtgtccaggatgtcgagggggtctctgcgtacttggtggggctgggaccctcccacttcccacctccttgtgtccctcactcccctgtttcattccatgctgagcctcccctgccttgggctccctggggagggggtggtggcaggagttgcccgagggcagctctgcccatgagcagctgctctagcggctcctcctgctgctgttcgccgggtgctgctgaccccaaggctggagtcagcttgcagcacagccagggtcgaggtcactccctccctgaggactctagcacggcacagcccctctgcctctctcctggtggtggcgttgaaacagcaccctctgcttcggtcctctacaggatggcagagaaggaggcagtcaataagatgtccctgcacaaccttggcacggtgtttggccccacgctgctccggccctccgagaaggagagcaagctccctgccaaccccagccagcccatcaccatgactgacagctggtccttggaggtcatgtcccaggtatgggaagacagcctccagcccatgcaaccccagcctgacagaggtggcctctgcctgccccacccccagtcctgcccatcttccgacttgcattgtatgtggtggtggctgagattcagagacagggacttgcctaggtttgcatggatgggagtgatagggggtgcctaggccacctcctggtcctgctggtgcaccttgctgggggcttaaaaccaccccaagtgttcgagtgtggtggctcatgcctgtaatcccagcactttgggaggccgaggcaggacaactgaacccaggtgtttgagaccagtctgggcaatgtagcaaaccccatctccagaaaaaatacaaagaaaaattaggcaggcattggggcacatatctgtaatcctaggtatctgggaggctgacacaggaggattgcttgagcccaggagttagaggctgcagtgatccatgatggagccactgtactccagcctgggggacagagcaaggccctgtgcatctctaaaataaataaccaccccccacccaacaagtcatgccttgtcaggaccccaccccacccccgtctcactgtaaggggttcatgacaccagcaggggtttctagcacctgaggtggacttgggatcttgggccccaaagacctcccaccagcagctgtgcgcccccttccgagccactctcctcttccccactccgcgagggcaggtcgaggtgctgctgtacttcttgcggctggaggccatccctgccctggacagcaagggacagagcatcctgttctccaccgatgtctaaaggtcccagtccatctcctggaggcggacagacggcctggaaacctctggctaatcaggccatctaataagatgctggaatgtaatccctggacaatccgtgtcctggcagcatttggtcttcctctaagcgcctggctccgctgttctcaggagtgggttctgaagtctctatctgggcccggtgggctcccttgtcctggcttccatctctgtctcagcgaccattcagccctgtggccaccgctctggcatgagcccctcagtcttgggtggtttctgcctggtccaggatttggtgttgctgctgagtccagcctttccaccacctccgcatgggctgtgggtgttgtcagctgcctcccgccttggcttcagtagctcacccagcttacaggggagctgccctgggctggagatgggcacgcaccctgggtcctatgtgtttcaggaactgagggtcagctggcagtgggatgaggctggcccccttctccgctttcgttccgggaggcctcccgtagagcggtaggggctcgagatggcatttcgtttggggcacgagctggtccgggaggtctgggatctctggttctgacctctgggcacctgctgcagctgtggctgaggcccagaaatgtgaagggcctccatccactccagtagtgaccccaacgtggggttcaatgtggaggggggaggggctgctgcggcagctgcaggagcagaagtgccacaccttgttcttctcatgcccgcatccatgcttgcagctgggaagggggcaggaatcagcgaggtgacctgggctgagtcctgggaatgggaagaggtggcaggaaggggatctgaggaggagaacagggggcctggtggtctgtgcttcttcccagacatgggagctgtagaggggacccctgcagcagatgctaagggggccagtaggcccaggcagtcttgggacttgtgtgtctcctgctgtgcatccatactgggtgctttagaaacggcaggcagaccagaagcccctgttgcaagtgaggacaaagtgtgggaaggccgtgagggtctgcagtccgagatggccttgtcctcaacctgcagtgcactgttgatgcgctggaatgccgcctccttctcccggtccaggtcttcaacagtgacccggtaccccagctctaagggaggtggcagcatcaaaggctcccctcgcctgcgtggcagcaggggaaacttgtgtgtactgggcctagaggcctcggatgtggaggagtcattcctgagggcgagtgtctaccctggtgctatatctgctgccttttcacactgggtgtgacctgaagagacagcctgaggcctgtcctcactcactgtctttgaggaactgagggtcagctggcagtgggatgaggctggccccctcctccgctttagccccggcaagcctcccgtggagctgtaggagctggagatggcatttcggttggtgcaggagctcgtccaggaggtctgggatgtctggttatatctgatttctgacctctgggcatggaggtctgtctgcagaggcccgggcccgggcacaaagggagagaggcctctattgtcccgcaggggccgaaatgcagacggtgcatccccggtgacctcggggacccttctctgatcaccaggattctcttggactctagggtccttgtcctgctcaggcatccctgccccgctctccttgagggccctcaacactatcttccctggacacaagtctggggacagccggctgttgtggaccccaaaggggtgactcccggctcctgggccccacagagagtccatgttctcagtgcagtggctgagctggaggacgccctggaactcggagcacgcagcactggcttgctgtggtacctgtgcaatcaaattgaaggcaggatcccaggaaggaaggcagggcttgcaggatcacggaaaaccttcttagagttgtcttgacaccactgatgtcaagtgtccgggtgcttgtaggatggcctgccactcagtccacgggcaggagcaacggggagatcccacaagcaaagtgaactgggggatgggctgaacgggctccaggcaactgagccctactggcaggtcctcggcctgggcccgaacaggaaggaggggcacagagtgcccaggtaaccgctcctgggagcagtggggaaccgtcggttgcttgaactctcgagagctgggctctgagcgtcctcgtccagccgccaactcggccaacggctaagccagcagttt

SEQ ID NO: 14962 - RNA, 3586 nt, Homo sapiens
  source 1..3586: mol_type = other RNA
gctgggattacaggcatgagccactatgcttggcctaatttttttttttatttttagtagagacaggatcttgctatgttgcccaggctggtctcaaactcctgggctcaagcaatcttccctcctcagcctcccaaagtgctgggattataggcgcaagccaccttacccagccaaaattaacatttataatagtgggtttgatgattggtcttagtagtatgttttgttgaacttctcaaaaatgagaaagtaacgttttatataactggacatgactgaatgaaatcattttctaaaagcttataataaggacatgaaagggtagtatggtcaaaatgtagattttttttcctgcaaaagaaccatccacaggcaaattatctaagtcccctgaatatgaaatatgacactattagaagtggtaaggtgcaactgcatgtatgacaaagtaagttgctgaatgtcttcacaatcaaaagcactaacttttaaaggcctcaagtactaaagcataattttagggatagaggaaagtgttcttgtttttgtaaatgagtatgggtcatggcatgactttggttttattttgggtcctcaaactgagagctttcttatgataatctgtatataaatagcaaaaaaaaacaatgggaatgttcataggataaataatatgagtgcaaatttttgccagaaagttctggaaatgtaggacttggttctttttataagtgcttttaaccttttcagactcattaatttcataaaccaatttaagcaattatttctatcagctacagatattttcttcacaaatataaagggttttgctcccctccccatcctccagcctccaccaatttgtgcctgtaactgccacttgatagctgctcagtaagactttaaatatcaggttctagtgccaacaaatccagaagtcagaaaaattctaagttacaatcgccagaatatctttcatgcattctattttactttattgttacagtttaaacaaattcagaaacgtggggtgtttctggctacttgagtaaaacgcactgcaaacgcaaagggaacaacgctgtaaacttaaatgatttctgaacagctcaggatcctcctggaggggatccttttcatctcacatattgattctgaacactatgttagcacctgctcccagaaggtcccttgacactggagcaagtcagaatatcttaatatcatagcttatttaacagcaggaaagcaactttaacatagacttgaggtttaggtagatctggtattatctagaacccaggcttaaattttgcaaaaagtttccaaagagcataagaaagtaaaacagaggtaccagaactgaagacatcattaacaaacaaaatatttccactcctaaccaaactgcaaccctttcagtatagcctgaggtatttttaaacatttgtacaagctaaagatcattcacagtttccaaagctgctttttactgagatagcttcaaattttcacaatatgtgactttcagacgttttcatataccagagtctctgccctcagactcatggaaacatcagagatatttagtggcagaaaatggttcttctagtgataagggttctatttcccaattattgtgctattcctaggatgtgattaaaaaaatatgaaatttgcaatttgtataaaaggaaaggaaacttgcttaaaattcaaaaagcaagtccagtctggtggaggtatgtaagatattaaataatagagtcagattctttcttgaacattccagatgaacttgacagcagagagttctggttttccaacattttctccatcttttcttttccagtggttttactgatctctctttgcttcttactatggatccacgggataaaacaaagcacagcacctccaataaggggagggactccagcgaggtagaatgccacatcataggagcccagtttgtcacgaagtaaccctgcaatgggtgggccaacagtcatgggtatagacatgaatccgagcagaaatccaattgcttgggagacatcctgggcaccaactaactcaaaggctatgggagccataatggaaatgaagcatccatcgaagagacccatgatgaggcacacagcaatgagggccccaaagatgctacacagaggaatcatcatggacatcagaccaatgaagaaaaaggagagtacctgtagataaaccttcttcacaccaggcacataatctgcaatccggccaaagagcagtcgtccaactcctgaagtgacgccaatgcacatgagaacaacctctttatttttttcatcttgaaatctttcatttacatgtttcatcaagtgaacataaggcacaaagtatccaaaaagtgcaagtggtattccaactgcccacactgcataagctgtcaccttgaagatggcaaaattgaaaattttttttggaggactgaactttttcctggaaaagagggaggatccgctacctccactctctttatctttggtactggtagcaagaggtcggtaagtaaagccagccagaaagagaacaaacatgaagatgcagagcaccctcaatgtgtaaaagaggcccacgctgtcaatcagaacccttaagagcaaaggcagcaggattgtgaagacactgctgccagcagtgacaatgccattcaccagtccaaggcgcttcttgaaatagtgtcccaaaatgaccaatgaaggctggtatgcaaaggagcagccgcaggcaaatatgattccataggtaaggtacagaggctcgatggaacaaacaaggtagtaaaagaaaaggccgcattttatattttttccccaaggttatgtcaggaacatttgcacagaggtgcagttgtgcctgtttttgctggcctaagggctgtagaccaaccttcgccctgtactgcactgttctcagtattgtgcaagacaacaagaaatcatattctgactacagaaagacttaaattaagtgtattcctttagtgatcccagtttgtaagctgtaaggccatgcatgtgtcaaaagaataatggattaaataatcttacagtttaaccaaataattgcacatttcttaggaagataaaggatcatatcattatgttctttgaaacaattatggtaaggaataaaactagttaaagttttttgaaaaggctatcagtagtaaaagcaaacaatttgttagaaagtaagattaaagttggttaataattaaaattttggataataatgctagtctagcaacatgctgaggtaatcataaggaactctagaatctgataaaattaaggcatgttggcaatcctctctctgagatgcccttctccctctactaatccacagctagcaccaccttcaaatcaggctcaagaatcacttctaggctttcccaaattaatctcacctcactctgatcaccctttactgaatctccactctttgtttagccaacatattaagcaactactgtgtaccagatacattgtggaaaagaatattaaaaatctggtccttggccagacgtggtggctca

SEQ ID NO: 14963 - RNA, 3555 nt, Homo sapiens
  source 1..3555: mol_type = other RNA
gctgggattacaggcatgagccactatgcttggcctaatttttttttttatttttagtagagacaggatcttgctatgttgcccaggctggtctcaaactcctgggctcaagcaatcttccctcctcagcctcccaaagtgctgggattataggcgcaagccaccttacccagccaaaattaacatttataatagtgggtttgatgattggtcttagtagtatgttttgttgaacttctcaaaaatgagaaagtaacgttttatataactggacatgactgaatgaaatcattttctaaaagcttataataaggacatgaaagggtagtatggtcaaaatgtagattttttttcctgcaaaagaaccatccacaggcaaattatctaagtcccctgaatatgaaatatgacactattagaagtggtaaggtgcaactgcatgtatgacaaagtaagttgctgaatgtcttcacaatcaaaagcactaacttttaaaggcctcaagtactaaagcataattttagggatagaggaaagtgttcttgtttttgtaaatgagtatgggtcatggcatgactttggttttattttgggtcctcaaactgagagctttcttatgataatctgtatataaatagcaaaaaaaaacaatgggaatgttcataggataaataatatgagtgcaaatttttgccagaaagttctggaaatgtaggacttggttctttttataagtgcttttaaccttttcagactcattaatttcataaaccaatttaagcaattatttctatcagctacagatattttcttcacaaatataaagggttttgctcccctccccatcctccagcctccaccaatttgtgcctgtaactgccacttgatagctgctcagtaagactttaaatatcaggttctagtgccaacaaatccagaagtcagaaaaattctaagttacaatcgccagaatatctttcatgcattctattttactttattgttacagtttaaacaaattcagaaacgtggggtgtttctggctacttgagtaaaacgcactgcaaacgcaaagggaacaacgctgtaaacttaaatgatttctgaacagctcaggatcctcctggaggggatccttttcatctcacatattgattctgaacactatgttagcacctgctcccagaaggtcccttgacactggagcaagtcagaatatcttaatatcatagcttatttaacagcaggaaagcaactttaacatagacttgaggtttaggtagatctggtattatctagaacccaggcttaaattttgcaaaaagtttccaaagagcataagaaagtaaaacagaggtaccagaactgaagacatcattaacaaacaaaatatttccactcctaaccaaactgcaaccctttcagtatagcctgaggtatttttaaacatttgtacaagctaaagatcattcacagtttccaaagctgctttttactgagatagcttcaaattttcacaatatgtgactttcagacgttttcatataccagagtctctgccctcagactcatggaaacatcagagatatttagtggcagaaaatggttcttctagtgataagggttctatttcccaattattgtgctattcctaggatgtgattaaaaaaatatgaaatttgcaatttgtataaaaggaaaggaaacttgcttaaaattcaaaaagcaagtccagtctggtggaggtatgtaagatattaaataatagagtcagattctttcttgaacattccagatgaacttgacagcagagagttctggttttccaacattttctccatcttttcttttccagtggttttactgatctctctttgcttcttactatggatccacgggataaaacaaagcacagcacctccaataaggggagggactccagcgaggtagaatgccacatcataggagcccagtttgtcacgaagtaaccctgcaatgggtgggccaacagtcatgggtatagacatgaatccgagcagaaatccaattgcttgggagacatcctgggcaccaactaactcaaaggctatgggagccataatggaaatgaagcatccatcgaagagacccatgatgaggcacacagcaatgagggccccaaagatgctacacagaggaatcatcatggacatcagaccaatgaagaaaaaggagagtacctgtagataaaccttcttcacaccaggcacataatctgcaatccggccaaagagcagtcgtccaactcctgaagtgacgccaatgcacatgagaacaacctctttatttttttcatcttgaaatctttcatttacatgtttcatcaagtgaacataaggcacaaagtatccaaaaagtgcaagtggtattccaactgcccacactgcataagctgtcaccttgaagatggcaaaattgaaaattttttttggaggactgaactttttcctggaaaagagggaggatccgctacctccactctctttatctttggtactggtagcaagaggtcggtaagtaaagccagccagaaagagaacaaacatgaagatgcagagcaccctcaatgtgtaaaagaggcccacgctgtcaatcagaacccttaagagcaaaggcagcaggattgtgaagacactgctgccagcagtgacaatgccattcaccagtccaaggcgcttcttgaaatagtgtcccaaaatgaccaatgaaggctggtatgcaaaggagcagccgcaggcaaatatgattccataggtaaggtacagaggctcgatggaacttacaaaagaactggacatgagcccaacaaatccaacagcagcacccacgacagctgttttccgacaaccaaataggtctgtgaagacgctgactattgggcagcaaaagaaaatcatccccatggagagagaacctacccatgctgtcttaaagaccatcttgtcatcgtctttggagccgaaggtttccagcatggacacgaagagcaccccgcaagcgttctggatgccgaacaccgacccgttgcaccacatggccgccagcatcaccagccagccccagccgccctcggggggttcggggggctcatggggctccgcggtcgccggccccgccagctccacctccaccttctcgacagccgcctcggggctgtccgagggtcccgggccgggcggcggagcggcccccgtgggcgcggggccgagcggctgcgcctcgctcgtgccccgcgcggagtccggctcctcctgggagagcaccatggcccgaggcgggcccctcaggcgccggagaagcgcgagggacgcgagttaccagcgggctcccggaggagctgcggggctcctggcgggctaacgaggccgaggcgagggcggcggagcccctggcgggcgggcgggctggcagcgcgcaggcggccagcgcgcaggcggccgcgaggacagctggcgcgcgcgaacacctcggggatcgacactgaagcctctaggtcacagccccgcacccccgact

SEQ ID NO: 14964 - RNA, 3587 nt, Homo sapiens
  source 1..3587: mol_type = other RNA
gctgggattacaggcatgagccactatgcttggcctaatttttttttttatttttagtagagacaggatcttgctatgttgcccaggctggtctcaaactcctgggctcaagcaatcttccctcctcagcctcccaaagtgctgggattataggcgcaagccaccttacccagccaaaattaacatttataatagtgggtttgatgattggtcttagtagtatgttttgttgaacttctcaaaaatgagaaagtaacgttttatataactggacatgactgaatgaaatcattttctaaaagcttataataaggacatgaaagggtagtatggtcaaaatgtagattttttttcctgcaaaagaaccatccacaggcaaattatctaagtcccctgaatatgaaatatgacactattagaagtggtaaggtgcaactgcatgtatgacaaagtaagttgctgaatgtcttcacaatcaaaagcactaacttttaaaggcctcaagtactaaagcataattttagggatagaggaaagtgttcttgtttttgtaaatgagtatgggtcatggcatgactttggttttattttgggtcctcaaactgagagctttcttatgataatctgtatataaatagcaaaaaaaaacaatgggaatgttcataggataaataatatgagtgcaaatttttgccagaaagttctggaaatgtaggacttggttctttttataagtgcttttaaccttttcagactcattaatttcataaaccaatttaagcaattatttctatcagctacagatattttcttcacaaatataaagggttttgctcccctccccatcctccagcctccaccaatttgtgcctgtaactgccacttgatagctgctcagtaagactttaaatatcaggttctagtgccaacaaatccagaagtcagaaaaattctaagttacaatcgccagaatatctttcatgcattctattttactttattgttacagtttaaacaaattcagaaacgtggggtgtttctggctacttgagtaaaacgcactgcaaacgcaaagggaacaacgctgtaaacttaaatgatttctgaacagctcaggatcctcctggaggggatccttttcatctcacatattgattctgaacactatgttagcacctgctcccagaaggtcccttgacactggagcaagtcagaatatcttaatatcatagcttatttaacagcaggaaagcaactttaacatagacttgaggtttaggtagatctggtattatctagaacccaggcttaaattttgcaaaaagtttccaaagagcataagaaagtaaaacagaggtaccagaactgaagacatcattaacaaacaaaatatttccactcctaaccaaactgcaaccctttcagtatagcctgaggtatttttaaacatttgtacaagctaaagatcattcacagtttccaaagctgctttttactgagatagcttcaaattttcacaatatgtgactttcagacgttttcatataccagagtctctgccctcagactcatggaaacatcagagatatttagtggcagaaaatggttcttctagtgataagggttctatttcccaattattgtgctattcctaggatgtgattaaaaaaatatgaaatttgcaatttgtataaaaggaaaggaaacttgcttaaaattcaaaaagcaagtccagtctggtggaggtatgtaagatattaaataatagagtcagattctttcttgaacattccagatgaacttgacagcagagagttctggttttccaacattttctccatcttttcttttccagtggttttactgatctctctttgcttcttactatggatccacgggataaaacaaagcacagcacctccaataaggggagggactccagcgaggtagaatgccacatcataggagcccagtttgtcacgaagtaaccctgcaatgggtgggccaacagtcatgggtatagacatgaatccgagcagaaatccaattgcttgggagacatcctgggcaccaactaactcaaaggctatgggagccataatggaaatgaagcatccatcgaagagacccatgatgaggcacacagcaatgagggccccaaagatgctacacagaggaatcatcatggacatcagaccaatgaagaaaaaggagagtacctgtagataaaccttcttcacaccaggcacataatctgcaatccggccaaagagcagtcgtccaactcctgaagtgacgccaatgcacatgagaacaacctctttatttttttcatcttgaaatctttcatttacatgtttcatctgaacagtcaaattgcagcagatgttgagatcaagtgaacataaggcacaaagtatccaaaaagtgcaagtggtattccaactgcccacactgcataagctgtcaccttgaagatggcaaaattgaaaattttttttggaggactgaactttttcctggaaaagagggaggatccgctacctccactctctttatctttggtactggtagcaagaggtcggtaagtaaagccagccagaaagagaacaaacatgaagatgcagagcaccctcaatgtgtaaaagaggcccacgctgtcaatcagaacccttaagagcaaaggcagcaggattgtgaagacactgctgccagcagtgacaatgccattcaccagtccaaggcgcttcttgaaatagtgtcccaaaatgaccaatgaaggctggtatgcaaaggagcagccgcaggcaaatatgattccataggtaaggtacagaggctcgatggaacttacaaaagaactggacatgagcccaacaaatccaacagcagcacccacgacagctgttttccgacaaccaaataggtctgtgaagacgctgactattgggcagcaaaagaaaatcatccccatggagagagaacctacccatgctgtcttaaagaccatcttgtcatcgtctttggagccgaaggtttccagcatggacacgaagagcaccccgcaagcgttctggatgccgaacaccgacccgttgcaccacatggccgccagcatcaccagccagccccagccgccctcggggggttcggggggctcatggggctccgcggtcgccggccccgccagctccacctccaccttctcgacagccgcctcggggctgtccgagggtcccgggccgggcggcggagcggcccccgtgggcgcggggccgagcggctgcgcctcgctcgtgccccgcgcggagtccggctcctcctgggagagcaccatggcccgaggcgggcccctcaggcgccggagaagcgcgagggacgcgagttaccagcgggctcccggaggagctgcggggctcctggcgggctaacgaggccgaggcgagggcggcggagcccctggcgggcgggcgggctggcagcgcgcaggcggccagcgcgcaggcggccgcgaggacagctggcgcgcgcgaacacctcggggatcgacactgaagcctctaggtcacagccccgcacccccgact

SEQ ID NO: 14965 - RNA, 2926 nt, Homo sapiens
  source 1..2926: mol_type = other RNA
gctgggattacaggcatgagccactccgcctggccaagcaggtcttctaatatccattttatagacagacacactgaggcttagagtggctgggtgactggccacaagtcctgcagtgctggtatttgaactcaggtgtgcctgacccaaagctttgctcttcatcacatttgtacctcctgatacctccgggccttctcttcccactggaagtgctgccacccaccaacatacaccttgttttttgctcatcctaatcctccctgacttcagggcccataccaactcctacctcctggaagagccctcccagcccaccttggcccacaaagatctgagcaactcctcccaaataattaagaggagggaaactggaccccagaagtgggaatagagggaaggatggataaaaaaggatggaatcatgccaagatcaaaatgaatccttagatgcttgggacttatgtctcagagctgagggcggtgctgagaaacctatctgtacctctgtttcctcctcaacaagatggaagctcgagtgtttgtgttgctgtctcatccctgcccaggggaggaggaaggaagtccttaggttcagaaatcaacaaatacattagccaccctgtgctgggtgcctactatgtgccatgtgcttttacacacagcaaccccatgatggcgggccgggggggcctcatcctcattgtatagatgaagaaacgaaggcacaggcagtgatgcagctggcccagggacagggtttgtgagtggtagagacaccatttgacccagttctgtctcactctggaatctgagctgctttctctttacactgctctcctccaccctcatcccacctgggctagagccttggagctcctcttagcctcttagaactccatccccaagaggtggggtctttgagaaaaatggagagacttcagcttctgtgtctaacttctcaagccttggggatggtctgatttcccctggagacctggatgtgacgggggtattaaggtggtttttcaaagacccctctacaggaggacttttgtgcttggtttgtgctaaataaacatgcagtccacctggacaattgtcacatgacccccatggtgaccacacactctgacctcttccatgtgaacctagcttctgacatcttgtctcatcgcctgtcaccccaggtgtgtcacaccaggtaggctgtgtgtcatgtccttatggacctgccccggcacacccagtctcacctacgacacgcttgcccaaatcagagggctcccacttcatgagacgcctgatgattcccactccccgagcccggagcataaaggaagagaggtactgaacagccacagacgagggtggaccctggggcagggatgtctgttgaacctgggaggagacagtgaacatcagcctgggaagggctgggcagaggggagccattggtccctgtacctgccatgacagttccgacccctttagactaatactgctcatgggcccactgccctagggccatccagggcagtgtcacacctgaaggcatcagatccccttccagctccaaatttcctgcctccaatgggcaggcgagtgctagggagtgtggatctgcctaggggagtactgcccagcactgaaacccttcctttttccacctggtttgggggttggaggggctgtgggctcagatccccgttcctgcctcttcagctggccacacctcacactttgctgaagtaggtggccacctccttacgcggaggccggggcccacccccagcccagccgttgcccatcagcggtggctcctcctggcccagccgcagaggcggtttgcatttgtgccagctcgtgagcagcctgttcatggtgccttgatccgtgatgccacgcagcttctccctttcctcctccgcaccatcgggggtcgtgggggcagctgcggaagcaggggccgtggccagtgtcccgtgggtgtgacccagctccaggtcatggttcatggcctcgaagaactgctggatgcagaccttggcaaaggctttggcgtgctccgtgcacgtctcgtcgaagagcttgcgctcgatgtcgatatagtgggaccagtacttgctcttgaggaaggcggcctgcgtgaagcagggccgcacagagcgcaccacgaatgccagcagagtggtcagcagcacgaaggaccagcccagcgcctgggagatgcagcggaggtaacgcacggccacctctcgggccaacagccagtcgccatcgtagatctcagggcagggcacccgggccagcaggcgggcgagctcgggggcaggaaggccgggtgccaggctgccgttgcccagtgcgctcacgggcacggcagtgcagaaggcacagaggaagcatttgccgtcgagtagcgtgacggccacccagacgacaggcgcgatgagggcgcgctgggccatggagcagaacatgtagcgcaacacagcggggtccttggcccggcggcccagcggccgcttccactcttcggccagcatggacacgttgttgttcatgaccaggccaagcagaaagagcaccaggggtggcgccagcaggatgcccgcgctgtaggctgcattgtagcccggcaggcaggggcagttgaagtcgaaggccgagtacatctgggcactggccagggccatgatgccacagatgccattcatgaaggactcctggttggactgcaggaactggaagatcatccggaacttgtccatcatgcccgctgtggggcccggcctcctcttcccaactcactgctgcctccaagagggcccctgctgcccaccctgcccactgggtgcccacctcatgactcgggctctcctggctgggaccaacagagctcagagcagaggctgaggtcact

SEQ ID NO: 14966 - RNA, 10243 nt, Homo sapiens
  source 1..10243: mol_type = other RNA
gctgggattacaggcatgagccactctgcctggccgagaccagttttcaatttagaacatgaggttatatgagacactataaaagtattaatgaacagtataaaagatgagaaattctaagatcataagtactgctctgagccttgaaacatttaaaagatagcactgaatgaggttatctgaatctgtagaatttacacctgcaagccatattctgaagggatcctggatactggttgctaacttttaaagccatcaggctcagaataaaaatgctttagagtagctggtaaagatcctgaagtaactaaataaaaaagggaagcccagcatcacttactaatgaagatgtgcaattgcagttgatcagttgttcaagaactgtaaattatgtggacatcataaatgaagagagaagaatataaaaatgtcagcaatatgttataactaacttagtccatagaatagtgtgtataccggaatagtgtgtatccaggaaatagaagtaggaaaccaaagtatcagggaaaaggagaaggactttataaatatacttaaaattgtcaaatgaggctaatgtaacacttcacactgggtaccagtattggaagtggtagcaggagcagcagtagtaatagcaggagcaaaacacatagcacttcccacatgtgagatgctattctcagtatttcacacctactaactcttttaagcctcctaacatgagcattaaacactatgagacagtgttgcatgatgaaataaactggggaaaactctagataaactgtcactttcctagaagggaatacatcatactagcagcatttcttatatatctgtttgacaaaagaaatcttttcatggtacttctcacagggctagagattcctggaatactccattggagatattgatctgatatttgtaaaaggggtttgaaaagtaagagtgtcctgttaatcatcaaattattgaatttcagaattcttaggttctcttattccatataaaatatttaatacaatgtttcagacaaatggtcattcaagtattgtttaggagcctgcattggctagaagtgcagtctctcagaaagataaggcatttcaccatggaaaggcaatacaattcattgaaaacactttttttttgtattaaagtagtgtttttcttgtataaatctcattcactgactgcctgactgctgtaataatgtaaagtcctcttataactccaagttacaaaatgacaaaaagaaaaattagaataaggatggaaaattttagagaaaagtttaaaattaatacagtggaactgcagtgggtcgaatggtggcccttcaaaaagatatgcccacccaggacctgtgaacctgtgaatgtgactttatttgaaacaggggtctttgcagatgtaattcagttaaggatctcataatgagatcaagctgtatttgggtgggccctaaatccaatgacaggtgtccataagagaaaagaagggacaatgatacacacagaaggtgacgtgaagaccagcagagactggagcggtgcatctataaaccaagccatgccaaggattgccagtagaaactgggagaggggcatgggagggattctccctcagagcctccaggaagaattagccctgctaacactttggttttcaacttctggcctccagaagggtgagagagtaaacttctgttgttttaagccacttggttcgtgataattttatagcagtactaggaaaccaatataatgagattaaaacaaatatttaaattaccagaataaaattagatcatatcaaacccaattgcaaaatgaccgaggaaaagatgacaaaaaaactgaggatacaataaaatcagaaaataaaggcaggtgaatatgggaatgctgaattaaaagggcaagggagaaactaagttaagtggatggttaggaacctgtacgaaggagataataaatattgtctctattctattgtaatataactaataaatagtagttaaggaattattaggatgtttaaggaattatcaggaataagaatgctactttatgttctactgagttaaataaatacgacacaaattatccaagtttctgtttctacccaaaatactgactaaaaatgaaggataagcatgttgttggatggtgaatagaataatggggacagtgggtgacaggaaagagaccacacccagggagagacagcctaggctctgttctggcttctacttcttcctgcaaggtcaaacttatggctccaatgacaaaagtagcctttgtcaatctttgaagaattgctacactatttgtcaccacactgaaaggaacatgctgatctacactttgttttcaaactcacccatattcccatgcttttccagtttcaacttagcactctaatatctgctgtgtctcctgtgaaccttagactctgacttctcttatttagccccttctgaggctatttcatgcaaggcatgtgcaaaagtacaattgagaatgacaagcaaagggtcctggcttctagggctccagcaaacaatgcaccagaagaaattaagcctatatacaaatgcctataattctcacatcactatattctatgtgaactatgaaatggagtattaatgattcataaaattctaccttcaatccagaccactctcctcagtgccagctgcatcctgaaccattgaatatccgcaggtacctaaacactgtgcaaaactgaatatattctcttttctcttaaatctgttctatctcttctgtttcctggattgttaatggttttatcacttgccagttgtccaaagcaaatacttatgtaccatacttgtactaatttgatttcaaatcctttatccaatcaactcaacctctaagatatacgcaaacctgccactatccttctctgctgtcactatgcaactcatgttcaaagcatgcttatccctctcacggacatctgcaatagcctcctaactcatcttccctctgtgcatgcctccctctaggccactcctcaggaacagtcagtggtcttttaagacaatgtaaattagttcatgccattttctgtctgtaaaacttcaatactttcctagtgcaaatatcagaatccacttactatactcacaacacattggtcctttttcagttccttaaaaatatgaagttctctaatgcttatgaaccttcacacaaacgacctctttgctatgcaggttccctattggccaccaccccacaccctgtcagctcttgtagatcctttaagtttagcctgactgtcacttcttcaaaaagcccttctctgaccctgaaggctaaatggccctgctcccatttccttgcacttatgcttcagcttcataaggattatcaaaatttgtgattattgaaggtgtttgtttttgtctgttcttgttcaccagattgtgtatcttattcactattataattcaagtatctagcacaaggcctagcacatactaagtactgaaaatattttcaggataaagggatgaatgaatgaatgaatgaataaatgaatgaatgaatgaatgaagcaaatccaatgaggtcacaggtaaggaacggatggcttcaaatatgatctgttcagtacatgctagtgttccacacgtcctgaaatcaatggaccagacgcttctatgtctgaagcaggcaaaagaaggacactgtcactacctcccaattcttcagatatagccagcaaatgggatcatctccacaactgaaaacttctattctgaaatatttcagacttaaagtagcaaggagagcaaaaggaattcccacatatttttcattcagactccccaaatgttaacattttatgatgtttgctttatcaatctatgtatttttcctgagccacttgagaataaattgcagacataatgccccttattgctaaatactcagcacacgttcctgaaaaacaaaggtattctcttctcttatataaccacagtacaattatcaaaagcagaaaattgcattgatgcggtactattttttaatcaagagaatttattcaaaatttgccaattgtatcacatcttttatagcaacatatatacacacatattttataacatatacaaaatatgttactatacacacacacatatatatacatacgtgtgtgtgtgtgtgtgtgtgtatgtatcttcccaacccctgttctaggattcaatccaagaccacatgttatatgtagttgtcacatctcttggtctcctttaatctgaaacagttcctcagactttttctttaatgacactgaaggttttagagtatagaccaattattttgcagaatgtcttttagtttgggattgtctgatgtttcctcatgattagattccacttatgctttttggggacaataataccaccaaagtgttggtttgtcctgcttggagcattatattaggaggtacatgatatttatttgtcccattattagggatgttaacttcaatcacttggttattactattacccttttgtaattaataagttcttacagaagatacttggatattatataaatatagtgatagccatttaaaaaaattacccaactctactctgtggcccaactaattctctacaaataaaaacttggcaaaatatttaaggtctgcttatgggtcacaaaatagctaaacatacaacttttcctaatgcaccaatctgttaacattaccttacctgcttctctcatgcaaacaaaggaaaaaacctaagatgctatttttaaaagaacattataaaatctctaatttcattcctcattcatcagatgagaaagctaaggtccagacaggctaagtgactcgcctaaggtcagacagctactctggcagacctcaaaataattatgtgttcattgtagagcaagaaatgcaaaagtcaatttaatgcccttcaaatatacaagccctacaggtaaacctaaagcaatctaaggcaggtttgagatgaccattttggaaaataatgggatttttacaaagatccatagaacatctttcatggagtcactgaagtttctagaggaagcccaagagctccctgctatgcctgagttctctctttgttctttttctttctctcttttcttctcccttagaaatgctcttaagtcattccaaagacaaagataaaatcccatcactctgggagagaggctgagagacagcctacaatgggcccctaactttaaaatgttatgctccttgcccaatactttggacacttgcttaattctaatcaatatctttttagatgttactttgaatttgcataagatagtcctgtcataatcttatcacattgtacatacttgaaaaaataattggtaaacattctacgaacattctaacctagagtagcccaaaagtaagtggccactacagtgccctggggctttcttttccaaggtgactagattatttaaaaataataacaataataaacagcaggtttcaggagttgaagttctattctcaacctctactcagaacacagaatggttccaagctttaccttgcctgctctgtatcctccaaggacttttagaagtaatggagatgccatttctgtccaacccagtatcccaaggtaataatgcttggcaaatgttatttttagatgatagcagcatacctaaagctatgaaccaaaggtaagcaatatgaagacatcttgcacaatctttctatacaaacatgcagcatttcctccttaccacttcctgggatgtataaaatgcataaaaatagaagcagtctttctttaagggtgagcttttatcaagacttggtataaaaataagcaagttatatttaaaaaatcataaaggcaaagatgtacattgctatgagtcataattagtaaatgtattcaagccttagaaatataggaaagtactgtgttagaataagagttagaagtagcagcagtagtagaggaagtagaagttgtagagtcagcagtaacttttactgtttaccatgtaagagcactatgctaagtgctttatatagaacacctcatttagtcctcagaaccatcttagtcttcctctaactttatacaaagttagtataaagtaaataaaacactggaatggtatcacaaatttgatctaagattgtaatccttctttgcagtaacgaatgactaatcttggagtgttaaccactgtgcaatcattaccaacctacaccccttctctccttttgagttgctttacgagggagatcttacctgaccactctatataaaaatatgaaactcctccaaaccagacttgcctgagtttccccattgaaatgtaaactccataaaggcaggaactttgtcttcttaattgctatatcccagaaccagaacagtgccttgtatgtgttaggtgtttaatatatatctgtttaacgaatgaatgaataattgatgaacaaaaccaaacgataacaaatataaaattttcaatgaattgtttgctttcccttcacaattacaaaaaaaaagttttagtggcttgattcaagttgtcagaatctcttaaaaagactggatagggaagtttgaactcatgagtttatttgctgaaaaatttatctggggctagcatggatattcaaagacattctactggctatgcttttttttaagaaaaagtcctgtaattcccttcttagttgtcaaacaagttgagcattaaatacttcattaaacatgagacataattttaagttagacaacttcattcattgccgggctacattctctgagtacctccatgtactaaacactaaggaattggctgggagtgaaccacagagtgaaatatgagggttagtgaccttcctacctaatatgggacatctgttctccctgtctgccccacttctccctcctaggctctctagagctaagtgaacaactcaaacaggatttttcatctaactgacctccctggcaacttttattatctcttgctgctgggaaggcaaagaaacagagcttcgaaaattacatgtttcatgctgggggaaatgtcatagcttcaacagagttttaagatattggtaggaaaattgtttttttggagaaaacttccatttttgaatgagcaaaaattatgcctatttgagaatctaaaataatcaggtaatcttgggctaaaaaataacaccataaaatctaataggtgtttaaagttttaacataaagttcgctctactttcattgcacgagcttaggcatacatcattgatcactgtgaggaaaacatatattaagttacttaaataaaaaatatgtcagttgatgtgacagattgtttgtttacttgaattgaaatgtataaaacttcactgatgttgttgaaacccagagcattacctgttcccctttcagtttctgctttcaaggaaaaatataaagttatattaaaccgacgcaaattctgttttcaaatacctctagatatcccagtgttgcttaggctaaagattctaagagtaatgaaattgtattcacttcttccccaaaacacttatttaaaaaaaataaagtgatatcagattaagaaaataaaatcacaccttcttgatgacatttttcaatttttttgttacatgctctatctccaggaagattatgtaacattaaacgatgagagaaaaggttttcgacttagactcacagtccaaccataacatgcttttgtttgcatgctaatcttttgtgattagttgtagcacacagctcattagctgttgcctgctctattacccctctgtccagctgaatgttctggctccttgtatggaaactgcagagttgtatctaaggttctgaacccttccttgagagaatgatgcttgtagtactccacaagttccattaaacttttaaattttctattttctgcaatgtgaaaaaagccatctcttgttaaaatcttgatgtgctttgcttcattattgtacttaatgctaattgcatattctcctgactctttggtcctgtgcctcacaaggtaagtactatttaccctattaataagttcggtctctgcttgcaatctttccattgctccagcataccagggttggcaagaataatctactggtttgggcacacatgggcaaggcttgactgcatcacttggaaaaaatccaacctctccagatgctaaatttctgccctgccaaaacagactgtgtgcatctcctttcagaagttcaacggtatccccggcctggagctgtaaagggggtccttcatgcagagctgggggtggtgttccagaatagttcctaatgacctgcatctttggtaaacctggatccacctgtttaggagttcttcgcagtccattggtccgtttctctggtagtttgagtgtcccttgttcaccagaattaactctgccacaattgtctactcttcccaaacattctttgtgtgctctcgctccacacttaaaacataaatagccttgataaaatgttcccctcaggagcatctggcagactttgcaggatgtgactcgagtgaaggtatgcatcttgaagtcgtggaaattggagtctgcatagtctggtcttatgttagacaaagccatttcaaactgttctagccatttcttctttaaatcttttgttttgcaataaaattctaacccattttgtccttgggtatggatgaggtagaagccataagaccactttttgttttctttatcggttgtaggattattggctatcttgtactgctgaagatctattatttccttcatttcatagttatcaccttttctcttacatacgatcactgccaaatcaaataagaagatatgcctttcttgtttggtatgcttgtctagagtggttattcgaatttcaccatctccctgaggtcgtccaaaaagcaaaactggttggttcaaattctctatagatagctgaaactgtttaatttcacgaagggtctcattatctcttttcacttcattcacatattgtgccaagtccttcatggcatcaagagccagtttcagatttgccttctcagtcggatcagtggtatgtttgaccagttcctggaggagaaggtggtactttaaaacacgttgcataggaaccacaagcaagtctcgaagagtaaatttcccattatttgctcttttggaacattcctctaatttcagtttgacatcttcttttgtcttagaaatgtagtctaaactagagatggctgactccactccactgcagtactgcccgtaaataaccaatctttccttgtagttaataaaaacttggtacaagttctggtcatttttatttacaatggaatcatgaatctcttgcattaggttccgatgaagttttacaagttcaggaatgttgatgaatactgaatcaaattctgctgctgtcagaaatctttttagtggtgccatgaaatacttttctattgactccaaagtttctgtatatttttcttctgtctgcttaatttctgctagacaacaacttcgtatatcattttctggacatttgggctgatgtgcttcctctgccttcattaagtcctcatagacttctccaccttcatcttccccataaacacagtcatagagatcttcttcatcttccacaagggtttcatctattaaatcaggaaggcctttgtagatgtcttcatcattaatgctttcttctgttgggaagggcctgattcctgtggccaatgctataggtgttcgagaaagtcgtgataatgtttctataacctttccaaagtcacgaacatcaaacaagtcaaatgcctcgaaaagttcacttttcctcattccaaacgtctcacaacaggccgtgagaaatgtccttatgttcttcaaacagagaaactgggacatctgcggcctcaggttgatctccttcaggttgatggagtgcgcccggaggttgttaagcagctggcagagcaggactccatcgcggagggtctgcgcaaggtcgaacacctgagccgagtcccaggtcacccggtggttggtgggcagcaccttgcaatggatgagccactgcgcgcactgcttccacggctccatgcccgacggctccgggacgcggctgggccggggcgggcggcaaggat

SEQ ID NO: 14967 - RNA, 2872 nt, Homo sapiens
  source 1..2872: mol_type = other RNA
gctgggattacaggcatgagccactgaacccggccctgagttttaagttcttacctgcctaattgtcctggctagaacctccagtacaatgctgaatagaagtggtgagcttggagatcattttcttgttccatatcttaggataagagctttcagtctttcatcattatgtatgatgttagctgtgggtcttcatagatatcctttctcaggttgaagaagttcctgtttacttctagtctgttcactgcttttatcatgaaaggctactggaggttgtcaaatgctttgtgtctatggaaatgattatgtatttatcttttgtgaattatcccattaatatactggatttactgattttcgtatgttaaaccaatcttgctttcctgggataaatcccaatggatcacagtgtataattcttttgatatcttgctggatttcatttgctagtactttttttttttgcctctgtattcaaaagggatattggtattagttttctttcctagtaatgtctttggttatggtatccatgtcttctttaactcatgtgtctggttatggtatccatgtcttctttaactcgtgtgtgtgtgtatgtatgtaaccttaggcactctaaaatgcagggctcagggcaggaacctctcttgctcagctctaacccttctggtcacctcttagtgactttttccccctttaagtctgccatttgaaggacattatatcctaattacacctgaatagaagggagaactttgggtcacatcctacagacagttctcaagactaataatttacatttattgaatactttctatatactcaggcattgctctaacccctttgcatgtgttaactcaatcttcccaactaaggaaactttgacttggaaaggttcagtgatttgttcaatggtaacacactggagagtgactacattttaattagggcaaaattttccatttggccaagaacaaaatctaacagccactgctattttgtgaatagtaatttgaaaattaaaggaaaatttttttaaagaaaagctttgttcttcaagtgtgatcgttattattcttgggccaaaatgcttttcaaggtacatgttttaatctttttttaaaaaattattttattagagtcagggtctcactatgttgcccaggctggtcctgaacaattggactcaagtgatctgcccgcctgggcctcccaaagtgctgggattacagttgtaagccaccatgccaggccacatttctacattcttaataaagtccgtggaatctacttcaaatgcaattttaatttatatttcaatctatgaagatattgggttggtgcaaaactaactgcggttttggactgtgaattttaaatcattataactaggctcaacgcatttttattaatcaaaataggaaccattacaatcaacacatttttgccaacgagaaataagttggtttattcctgtagcgtaaaaatccgtgctttgggattcgacgaactcttggaaagcattttctgcatcctgctggttgtggaagcgttttccctgcaaaaagttgttgagatgcttaaagacgtggtagttggttggcaagaggtcaggtgaatacggtggatgaggcaaaacttcatagcccaattcattcaacttttgaagtgtgggttgtgcaacatgcggtcgggcattgtcgtggagaagaattgggccctttctgttgaccaatgccagctgcaggcgttgcagtttttggttcatctcatcgatttcctgagcatacttctcagatgtaatggtttcaccgggattcagaaagctgtagtggatcagaccagcagcagaccaccaaatagtgaccatgaccttttttgggtgcaagattggctttgggaagtgctttggagcttcttcttgatccaaccactgagctgatcgtcgccggttgtcatataaaatccacttttcatcacacgtcacaatccgatcgagaaatggttcgttgtggttgcgtagaataagagaagatgacacttcaaaacgacgatttttttgattttcagtcagctcatgaggcacccacttatcgagctttttcacctttccaatttgcttcaaatgtcgaacgaccgtagaatggttgacattgagttcttcagcaacttctcgtgtagttgtaaggggatcagcttcgatgattgctctcaactggtcgttgtcaacttctgatggccggccactacgctcctcatcttcaaggctctcatctcctttgcaaaacttcttgaaccaccactgcactgtacgttcgttagcagttcctgggccaaatgcattgttgatgttgcgagttgtttctgctgctttacgacccattttgaactcgaataagaaaattgctcgaatttgctttttgtctaacatcattttcatagtctcaagggtcaatcgcttgcaggaggggaacacagaaggggctgagccacacatgctgggttccttctcatttccacaactgatgttcgacttttctacggggcagtacagagaactgtgagagacacctgagaccagggaggtaaatgactccccccgtgatgcctccttgagttctgaggacaggactggacaaaaagccaggttctcacaaggcctccggttctgcgcttcagggaatggactgaaaaggacaacacccttgctaaggtgatgccgtgggtcaacagaaaaaggcccaggccggggcatgcacacctattcccgcgcaccaacgggtgcgctgtaagagaagacaaaaggtcgcgactgggaggccgtcccagcgaggcggcttgaggagaccacgtgggggagccgcgc

SEQ ID NO: 14968 - RNA, 3162 nt, Homo sapiens
  source 1..3162: mol_type = other RNA
gctgggattacaggcatgagccactgaacccggccctgagttttaagttcttacctgcctaattgtcctggctagaacctccagtacaatgctgaatagaagtggtgagcttggagatcattttcttgttccatatcttaggataagagctttcagtctttcatcattatgtatgatgttagctgtgggtcttcatagatatcctttctcaggttgaagaagttcctgtttacttctagtctgttcactgcttttatcatgaaaggctactggaggttgtcaaatgctttgtgtctatggaaatgattatgtatttatcttttgtgaattatcccattaatatactggatttactgattttcgtatgttaaaccaatcttgctttcctgggataaatcccaatggatcacagtgtataattcttttgatatcttgctggatttcatttgctagtactttttttttttgcctctgtattcaaaagggatattggtattagttttctttcctagtaatgtctttggttatggtatccatgtcttctttaactcatgtgtctggttatggtatccatgtcttctttaactcgtgtgtgtgtgtatgtatgtaaccttaggcactctaaaatgcagggctcagggcaggaacctctcttgctcagctctaacccttctggtcacctcttagtgactttttccccctttaagtctgccatttgaaggacattatatcctaattacacctgaatagaagggagaactttgggtcacatcctacagacagttctcaagactaataatttacatttattgaatactttctatatactcaggcattgctctaacccctttgcatgtgttaactcaatcttcccaactaaggaaactttgacttggaaaggttcagtgatttgttcaatggtaacacactggagagtgactacattttaattagggcaaaattttccatttggccaagaacaaaatctaacagccactgctattttgtgaatagtaatttgaaaattaaaggaaaatttttttaaagaaaagctttgttcttcaagtgtgatcgttattattcttgggccaaaatgcttttcaaggtacatgttttaatctttttttaaaaaattattttattagagtcagggtctcactatgttgcccaggctggtcctgaacaattggactcaagtgatctgcccgcctgggcctcccaaagtgctgggattacagttgtaagccaccatgccaggccacatttctacattcttaataaagtccgtggaatctacttcaaatgcaattttaatttatatttcaatctatgaagatattgggttggtgcaaaactaactgcggttttggactgtgaattttaaatcattataactaggctcaacgcatttttattaatcaaaataggaaccattacaatcaacacatttttgccaacgagaaataagttggtttattcctgtagcgtaaaaatccgtgctttgggattcgacgaactcttggaaagcattttctgcatcctgctggttgtggaagcgttttccctgcaaaaagttgttgagatgcttaaagacgtggtagttggttggcaagaggtcaggtgaatacggtggatgaggcaaaacttcatagcccaattcattcaacttttgaagtgtgggttgtgcaacatgcggtcgggcattgtcgtggagaagaattgggccctttctgttgaccaatgccagctgcaggcgttgcagtttttggttcatctcatcgatttcctgagcatacttctcagatgtaatggtttcaccgggattcagaaagctgtagtggatcagaccagcagcagaccaccaaatagtgaccatgaccttttttgggtgcaagattggctttgggaagtgctttggagcttcttcttgatccaaccactgagctgatcgtcgccggttgtcatataaaatccacttttcatcacacgtcacaatccgatcgagaaatggttcgttgtggttgcgtagaataagagaagatgacacttcaaaacgacgatttttttgattttcagtcagctcatgaggcacccacttatcgagctttttcacctttccaatttgcttcaaatgtcgaacgaccgtagaatggttgacattgagttcttcagcaacttctcgtgtagttgtaaggggatcagcttcgatgattgctctcaactggtcgttgtcaacttctgatggccggccactacgctcctcatcttcaaggctctcatctcctttgcaaaacttcttgaaccaccactgcactgtacgttcgttagcagttcctgggccaaatgcattgttgatgttgcgagttgtttctgctgctttacgacccattttgaactcgaataagaaaattgctcgaatttgctttttgtctaacatcattttcatagtctcaagggtcaatcgcttgcaggaggggaacacagaaggggctgagccacacatgctgggttccttctcatttccacaactgatgttcgacttttcttcctttcggtataaattccaaggtacgaagtccccagccttttttatgcgtcttgaacacttggaagtggaactgtagacctttctggaccactctgtttctgcagtggtcactgcatcggcacaggacattgcattcaaaaacaggctctgcatactttcctccagatcctatatctctaaggcatgagttatcatcatagttctctccatggcggagacaggagcaagtgccagggaggcagggagttttgacacaaatgcatccgggaaaggttatttgagtgggatcaatgtctgctccaggtccaactacatgatcaggagtgtactgtgagagacacctgagaccagggaggtaaatgactccccccgtgatgcctccttgagttctgaggacaggactggacaaaaagccaggttctcacaaggcctccggttctgcgcttcagggaatggactgaaaaggacaacacccttgctaaggtgatgccgtgggtcaacagaaaaaggcccaggccggggcatgcacacctattcccgcgcaccaacgggtgcgctgtaagagaagacaaaaggtcgcgactgggaggccgtcccagcgaggcggcttgagg

SEQ ID NO: 14969 - RNA, 9018 nt, Homo sapiens
  source 1..9018: mol_type = other RNA
gctgggattacaggcatgagccactgaacctggcctcctgattgttctttttctttttctttctttttttttttgagatggagtttcgctcattgcccaggctggagtgcaatggcgcgatctcagctcaccacaacctctgcctcccaggttcaagcgattctcctgcctcaccctcccgagtagctgggattataggcatgcaccaccacacccggctaattttatatttttagtagagacggggtttctcatgttagtcaggctgatctcgaactcccaacctcaggtgatccgcctgcctcagcctcccaaagtgctgggattacaggcgtgagccaccgcgcccagtgcctcctgatttttctacgcctccttctcttttccttcttcctattaatctgttaaaagttttctttcaacccttttccaaccactggtctagaaattatatataaatacgtggccctcgtggactttagccgaatctcctcccaaatagcatagtgaccttgaaaggcatgaacaccaggatgttgtctagtacttcagttgcgccttttgtcgctactctatacgttagtcactgttattattgctttacacagtcaatgacagtttagacagatccaatggtttctaaggttttccggcattccttctcacatctttcttcctttccttatgtacacaagttccttttttcggggaatctgttattgataaattgtttttatcttgtctttttttttttttgagacagaatctcactttgcccaagctggagtacagtggcgcgatctcggctcactgcaacctctgtctccctggttcaagcaattctgtctgcctcagtctcccaagtagctgggaacacaggtgcccgccaccacacctggctaattttgtatttctagtagagatggggtttctccttgttggtccggctggtctcaaactcctgacctctgcccgcctcggcctcccagagtgctgggattacaggcgggagccaccatgcccggcttgtcctaccttttacagatgaggtgggctcagaattctagactgcacttctctcagtaatttgaagccatgctctatcttcggacttttgttgttccagttgtgaaaccagttctctgtccaattgctctttggagagacattttaatctcttagtgttgctgttaggatcttccctgagtctgatatgttctgtggttcgactatgattattttagttacgaatttaggtttgtgtatcatgctttggactcaacggtttcctggatcttaaaatttcaagattttcaggctgggcgcagtggctcatgcctgtaatcccagcactttgggaggccgaagcaggcagatcacctgaggtcaggagttcgagaccatcttgaccaacatagtgaaaccccatctctacaaaaaatacaaaaattagccgggcgtggtggtgtgcacctgtaatcccagctgcttgggaggctgagatatgagaattgcttgaacctgggaggcagaggttgtaatgagccgagatttcgccattgcactccagcctgggcaacaaacgcgaaactccgtcaaaatgaaaaacaaaaaacacttcaagattttcattaattttggaaaattctggccacgatctctttgcatgtggctgctccccagttctcattttttggtttgtgttagatacttgctggcatgttgggccttcttattgtcttgtgctaaccacacacgcacatcacacacacacacacacacacacacacatacacacacacacacacacacacacacacacagagtcgtccctccatatcctcaagggattgcttccaggactccccttggataccaaaatctgaggatgctcaagtcttttatataaaatggcacaatatttgcatatatcctatgcacatcatctttaaatcatctctagattacctaatacaatgtagatgctacataatcattatactgtattatttaaggaataatgacaataaaaaagaaaacctgtacatgtccagcacagacacaattgtttttcaaatattttcaactcactcttggttgaatccatggatgcagaacccatggatgtggagggttgactgtaaatatatatatgtctcattagctgtgctatgtcccgggtaactgcctcagacagctctcttctagtgcactaattctcttcatctatgtctcacttgtattttaacaccctccaaccaagttgttaatttttttttttgagacagtgtctcactgtgtcgctcaggcaagagtacaacggtgccatcttgactcactgcgagcgccatctcccgggttcaagcgaatctcctgccccagccacctgagtagctgggattacaggtatgagccactacgcccagctaattcttttgtatttttagtagcaatcaggttttaccatgttggccaggctggtctcaaactcctgacctaaaatgatctggccgcctcagcctcccaaagtgctgggattataggcgtgagccaccatgcccggccccaagttgttaattcctatgactacatttttaatctatttttttcttccaaatctgcattgtcatttttggggggtgttttgttggtttgttttagagacagggtctcactatgttgcccaggctgtccttaaactcctgggctcaagtaatcctctagcctcagcctcccaagtagttgggactacaggtgcatactaccatgcccagctttgcagtcttaaaaaaaaaaaaaaaaaaaaaaaaaaaaaaaaaaaaaaaagagaactggccgggcgcggtggctcatgcctgtaatcccagcactttgggaaggtgaggggggcggatcacctgaagccgggagttcgagaccagcctgaccaacatggagaaatcccgtctctaccaaaaatacaaaattagccaggcatggtggcgcatgcctgtaatctcagctactcaggaggatgaggcaggagaattgcttgaacccagaaggcggaggttgcagtgagccgagatcacaccattgcactccagcctgggcaacaagagcaaaactctgtctcaaaaaaaacaaaaacaaaaacaaaaaacaaaaaaactacaaaaagtatattaagaactacaaaaagggctgggcactgtggctcatgcctgtaatcccagcactttgggaggccaaggtgggaggatcacttgagcccaggagtttgaagctgcagtgagccgtgaccatgccactgcactttggcctgggcaacagagtgacaccctgtcaaaaaaaaaaaaaaaaagcataaagaaagaatacagaacaagccactaagcaataccaagcttaaggaaattgccaacacagcagaggccccagtcatacccccttcctgtttttgcctttcagagataaccagggatgtgaattttttcaaattctcaagcatctcgttagacttttgctggatatatatagatccctaagcacgcaaaatattatttccgtattttatactagattactgcattttcttttgtaaacatttttcccgctcaatgttgtttaagttgtattctgagccatatcactgctctagttgaattcattttcactgctgtaatctcttgcatgaatggactacagtggtcccttttcctattgaaggacttttggttgctttccaatttcctgctatcatgaactatgctgctgtaagtgtaactgtacacctgatatttctctatatattggtgcatggacttctcagggcttttctcaactagagttctgcaagagaattctggcataaagatgacttcagggaggatgttctcaactttcccacagtcagtacatagctagcacgttctagatgttcaggaggcgtggcgaggtggctcacgcctgtaatcccagcactttgggaggccaaggcaggatgatggctcaagcccaggagttggagaccagtgtggacaaaatgacgagaccccatctctataaaaaatatgaaaaattggcccagcatggtggcatgtgcttgtagtcccagctcctcaagaggctgaggcaggattggctgagcctggcagctcgaggctgcagtgagccgtgatcacgccactgcactccagcctgggtaacatagcaagaccctgtctcaaaaaaaaaaatttttttggggggggccgacatgatgcaaatagcatctaactgtggtcttggtttatgtgtacatatttcctgaatagctacatggttgaacgtttgccttttttttttcttttgagatgaagtcttgctctgttgcccaggctggagtgcaggtggtatgatctcggctcactgcaacctctgcctcctggggttcaaatgattctgatgcctcagcctcccaagtagctgggattacaggcgcccgccaccatgcctggctaattttggtatttttagtagagatggggtctcgccatgttggccaggttggtctcggactcctgacctcaggtgatccacccgtctcagcctcccaaagtgctgggattacaggcataagccactgcgctaggccggtttttgttgtgttttgagacggagtctcgctctgttgcccaggctggagtgcagtaacactatcttggctcactgcaacctccacctcctgggttcaagccattctcctgcctcagcatactgagtagctgggattacaggcacgcaccaccacacccggctaattcttgtatttttagtatagatggggcttcaccatgctggccatgctggtctcgaactcctgacctccagtgatcggtctgcctcggcttcccaaagtattgggctcacgggcgtgagccaccacgcctggccgaacggtcgccatttgtatttcatcttcttcatactgtctgttcacacacagcccattttgttaggttctctttttctgatttgtagacgttataacccgcatgcaaattatttgccttgttggatgttgtaacagctctgtcttaacagcattttgctcttttctattcagagtctctgtgcctttaggcacttgcaacagattgactgcatagtgtatttgtttacatgccgataatctttgaagttcgtgaggatctgatcctgctgtttcaagtttgctttcatgcacgtgttttgtaattttcaggatgtgccctcatgttgagggtctattgtgtgcgaggatcttaggtaacaaggcatgaagttaggtccctccagggaggttttctgtcataaacatcttggcctggttgtctgcaaaccagattgatattacaagcgtggggtctaaatgagtggtgactttttctcctgtggatctcaggcagagagaggacacagtgcttattctcaggggtggagggcaaatgttttttctagtccatctttttactgttaagtatcatgaccctcgaggatcccagcttcacgcaggagtcatctccactgcatttcaccatcttcccgatgcccaaagtcctatctgccacctggcccccaaacctaaacccggtggtttccaagagcaactccggtgtgagcccccacggtgtcttccgcgtctacttccttcgtcttgggctcctgtgggtctccttgcttttttatgggcacggctaggtgcgtctgcttcatttcctgcatttctacagtctgtagtggagggtttgcaggtcttatctgataagttgctggaaactgaagtctctcttctgtcctgtggaccagccctctcctgtccctgcggtgtcccagcatgggggctccacagggtggggacagtgacagcccacactggagctaggccccgggggtggcagcgaggatggcaaatggggtcagccccagggttttctggaggggccatgagggctggctgctgatatgggtgtggacagtgaggggaggggccccagggatgccttcagggctttggtctgaggcctgggctggggcagcgtcattgactgagatggggaagacctacgtgggcggaaggttctactcaggctgttaggtcggatgcccactagacacctgaggacgagctcggcaagacaggagagggagggggagaatgaaggcaagagggtgctggccaggcagggccatcagcactggtcggggagggggccaagagcaggcagcacttcctgcatatgtgctatttcccccatggaccaagtagcagttcacagaagaagcatctgggggccttgttaatgttttccgggaccctggccccagagcctccactttggcaggtcagggctggcccacgaacctgcatttctagctaggacacaggggatgctgctgtggacacaaggaccatgctctgagtgggccatcagtttggggagaggtggggacaagctgttggccatctgagggtgcagcagattggatgagagaagactctgcctctgtggcctcctctgtgtggcccaggagtggtggcccatggtccagcactgcagctgcctcttcccgcagctgcttttcctgtgtttcagctggggaagcagagggagctggtgacacctcgtggggccacagggaaggtcggcgacaaaaccaggcaagccctgtggtcacgcaggaggagttgggaccacgctgcatcagaggaaggctgtggagtattcaatgaatggaatttaatgtaactatgacataaacacacacagggtggggaggacgggtgaccaagcgcagacgtgggtgacacgtggccccgctctctggaccctcagtgggaaaaagtctgaggctggcgtctctcaccaaaccccacctcccctggtgggtcaatactgatctggctgagtgacagcatctcgtgacccaggctggccctgggaaggcgccacaggcgaggcctgcgagtccagggagcaggcagacgctacagtggcccccgagcgcgccaggtgccagcctcgacgtgtaaatggcccgctgcgggcgctgccgggaaggaagacaagaagggtgagggctcgtcctcaccaagtgcttcctgagtgccgtaggacgtgggtgggacatggggacagtgagggtaacacaaacagcaacgaatgcacaaagacaagttccaggaacacccataaacccataacgttcaacaaaatggcaacaaaacgacgcccctgctggcctggcgaggctggcgcttccttcgtggcagatgccacctgcagctggctggctggcaagcgttggccaagctttttggtacctgggagctcaacagcataaaaggctgtaacctctacacggaaaaatttcacatccttcccctgaaactgacttcaggggcaaagaaacgagacttcttgaagaccagcctcttctgggaaaggggcttctgagacgagtgtcgacggcagagcagatggcctggggaaggcaggggtccctgggcagaggctgggagggtggccagagaccagggagggcccctccatctggtgggtttggcaggtgtgtcccctggtgctgccaccaggagccccgaggccggggtgttggctgcgacagcccctcactgggtccggagctggtaatctccattctgcgtgatataacgcacccagggcagggcctggtacccactcttctcaatgatcttcaggtagcgcacctggatgccggaggtagtgaagtaagggatctcgaacttgacactgatcgggggcttgccctccttgtcttcggcctccacactaggcaggccgaagtgggcccgcatcaggtactccttgccgcccgggaaggacttgatggaccacacgatctcgctgttctcggggacccacttaacgctccccaccgtcgtcttgaacttgggtgagtcggcatcattgggcacgggaatgtggatctccacgttgttggctgttgaccgccgcttgaactggcttttggccttgatcatgtactcgatgcggctgtgggagtgcttctcgatcaccgactcgatccatatcaaaggcttgacgtgggtgttgagacggtaggacatgagctcgaactcgccgtcgggtgggatgaaggagatggtgcggtcattctcgaagcgtgatagccgcacacactggtggaacttcacatcctccagctccacggatttgcttttgccgcggcccgtgttgtcaaagaggaccttgtcgttgaggcccaggcgcagctcgggcatgcccgagaggaagactcgcatcttgatggagcccacgatctcgctgcgcaggacattgccgttggcgctgaccaagaggttgacagactcgatgacgtccaagaacacctcattcttccgatacttgatgccttcggaccgccaggacaccgcgttggtgacggtggctggtggccgcggggcccctgtttccagcttgtggccttcctgagtgatgtactcctgcaggatcttgctgtcggtggtctgggggtagccgaagtccatgagctcgtccagcagctcgtagatgataacaaagttgtcccggatgctctcctcctccagctccttgaagtactcggaaaacacctgcaccaccttatagaggaaagaaaagaccagcgacacgcacgcgttcttcttggatgtggcaaccagatacaggttgttgtgtttgatccacatgaaacggacccccccgtgggccaggatgggcgacagcatcccctcctcctccttctccatcaggatgggcatgaagtgctccacctctgacatgtccacgtcgccacggtagttccggcagatgagcaccttgcccttcaggtccagcacgtagacggcgctggcggacatgatggctgcaggaggcctcggcagcggccgagggcggtggcggcggcagcgacggtggggactgctgggcgttgagcaaggccgggcgccgcccgcgacagctcacctccacttcc

SEQ ID NO: 14970 - RNA, 9054 nt, Homo sapiens
  source 1..9054: mol_type = other RNA
gctgggattacaggcatgagccactgaacctggcctcctgattgttctttttctttttctttctttttttttttgagatggagtttcgctcattgcccaggctggagtgcaatggcgcgatctcagctcaccacaacctctgcctcccaggttcaagcgattctcctgcctcaccctcccgagtagctgggattataggcatgcaccaccacacccggctaattttatatttttagtagagacggggtttctcatgttagtcaggctgatctcgaactcccaacctcaggtgatccgcctgcctcagcctcccaaagtgctgggattacaggcgtgagccaccgcgcccagtgcctcctgatttttctacgcctccttctcttttccttcttcctattaatctgttaaaagttttctttcaacccttttccaaccactggtctagaaattatatataaatacgtggccctcgtggactttagccgaatctcctcccaaatagcatagtgaccttgaaaggcatgaacaccaggatgttgtctagtacttcagttgcgccttttgtcgctactctatacgttagtcactgttattattgctttacacagtcaatgacagtttagacagatccaatggtttctaaggttttccggcattccttctcacatctttcttcctttccttatgtacacaagttccttttttcggggaatctgttattgataaattgtttttatcttgtctttttttttttttgagacagaatctcactttgcccaagctggagtacagtggcgcgatctcggctcactgcaacctctgtctccctggttcaagcaattctgtctgcctcagtctcccaagtagctgggaacacaggtgcccgccaccacacctggctaattttgtatttctagtagagatggggtttctccttgttggtccggctggtctcaaactcctgacctctgcccgcctcggcctcccagagtgctgggattacaggcgggagccaccatgcccggcttgtcctaccttttacagatgaggtgggctcagaattctagactgcacttctctcagtaatttgaagccatgctctatcttcggacttttgttgttccagttgtgaaaccagttctctgtccaattgctctttggagagacattttaatctcttagtgttgctgttaggatcttccctgagtctgatatgttctgtggttcgactatgattattttagttacgaatttaggtttgtgtatcatgctttggactcaacggtttcctggatcttaaaatttcaagattttcaggctgggcgcagtggctcatgcctgtaatcccagcactttgggaggccgaagcaggcagatcacctgaggtcaggagttcgagaccatcttgaccaacatagtgaaaccccatctctacaaaaaatacaaaaattagccgggcgtggtggtgtgcacctgtaatcccagctgcttgggaggctgagatatgagaattgcttgaacctgggaggcagaggttgtaatgagccgagatttcgccattgcactccagcctgggcaacaaacgcgaaactccgtcaaaatgaaaaacaaaaaacacttcaagattttcattaattttggaaaattctggccacgatctctttgcatgtggctgctccccagttctcattttttggtttgtgttagatacttgctggcatgttgggccttcttattgtcttgtgctaaccacacacgcacatcacacacacacacacacacacacacacatacacacacacacacacacacacacacacacagagtcgtccctccatatcctcaagggattgcttccaggactccccttggataccaaaatctgaggatgctcaagtcttttatataaaatggcacaatatttgcatatatcctatgcacatcatctttaaatcatctctagattacctaatacaatgtagatgctacataatcattatactgtattatttaaggaataatgacaataaaaaagaaaacctgtacatgtccagcacagacacaattgtttttcaaatattttcaactcactcttggttgaatccatggatgcagaacccatggatgtggagggttgactgtaaatatatatatgtctcattagctgtgctatgtcccgggtaactgcctcagacagctctcttctagtgcactaattctcttcatctatgtctcacttgtattttaacaccctccaaccaagttgttaatttttttttttgagacagtgtctcactgtgtcgctcaggcaagagtacaacggtgccatcttgactcactgcgagcgccatctcccgggttcaagcgaatctcctgccccagccacctgagtagctgggattacaggtatgagccactacgcccagctaattcttttgtatttttagtagcaatcaggttttaccatgttggccaggctggtctcaaactcctgacctaaaatgatctggccgcctcagcctcccaaagtgctgggattataggcgtgagccaccatgcccggccccaagttgttaattcctatgactacatttttaatctatttttttcttccaaatctgcattgtcatttttggggggtgttttgttggtttgttttagagacagggtctcactatgttgcccaggctgtccttaaactcctgggctcaagtaatcctctagcctcagcctcccaagtagttgggactacaggtgcatactaccatgcccagctttgcagtcttaaaaaaaaaaaaaaaaaaaaaaaaaaaaaaaaaaaaaaaagagaactggccgggcgcggtggctcatgcctgtaatcccagcactttgggaaggtgaggggggcggatcacctgaagccgggagttcgagaccagcctgaccaacatggagaaatcccgtctctaccaaaaatacaaaattagccaggcatggtggcgcatgcctgtaatctcagctactcaggaggatgaggcaggagaattgcttgaacccagaaggcggaggttgcagtgagccgagatcacaccattgcactccagcctgggcaacaagagcaaaactctgtctcaaaaaaaacaaaaacaaaaacaaaaaacaaaaaaactacaaaaagtatattaagaactacaaaaagggctgggcactgtggctcatgcctgtaatcccagcactttgggaggccaaggtgggaggatcacttgagcccaggagtttgaagctgcagtgagccgtgaccatgccactgcactttggcctgggcaacagagtgacaccctgtcaaaaaaaaaaaaaaaaagcataaagaaagaatacagaacaagccactaagcaataccaagcttaaggaaattgccaacacagcagaggccccagtcatacccccttcctgtttttgcctttcagagataaccagggatgtgaattttttcaaattctcaagcatctcgttagacttttgctggatatatatagatccctaagcacgcaaaatattatttccgtattttatactagattactgcattttcttttgtaaacatttttcccgctcaatgttgtttaagttgtattctgagccatatcactgctctagttgaattcattttcactgctgtaatctcttgcatgaatggactacagtggtcccttttcctattgaaggacttttggttgctttccaatttcctgctatcatgaactatgctgctgtaagtgtaactgtacacctgatatttctctatatattggtgcatggacttctcagggcttttctcaactagagttctgcaagagaattctggcataaagatgacttcagggaggatgttctcaactttcccacagtcagtacatagctagcacgttctagatgttcaggaggcgtggcgaggtggctcacgcctgtaatcccagcactttgggaggccaaggcaggatgatggctcaagcccaggagttggagaccagtgtggacaaaatgacgagaccccatctctataaaaaatatgaaaaattggcccagcatggtggcatgtgcttgtagtcccagctcctcaagaggctgaggcaggattggctgagcctggcagctcgaggctgcagtgagccgtgatcacgccactgcactccagcctgggtaacatagcaagaccctgtctcaaaaaaaaaaatttttttggggggggccgacatgatgcaaatagcatctaactgtggtcttggtttatgtgtacatatttcctgaatagctacatggttgaacgtttgccttttttttttcttttgagatgaagtcttgctctgttgcccaggctggagtgcaggtggtatgatctcggctcactgcaacctctgcctcctggggttcaaatgattctgatgcctcagcctcccaagtagctgggattacaggcgcccgccaccatgcctggctaattttggtatttttagtagagatggggtctcgccatgttggccaggttggtctcggactcctgacctcaggtgatccacccgtctcagcctcccaaagtgctgggattacaggcataagccactgcgctaggccggtttttgttgtgttttgagacggagtctcgctctgttgcccaggctggagtgcagtaacactatcttggctcactgcaacctccacctcctgggttcaagccattctcctgcctcagcatactgagtagctgggattacaggcacgcaccaccacacccggctaattcttgtatttttagtatagatggggcttcaccatgctggccatgctggtctcgaactcctgacctccagtgatcggtctgcctcggcttcccaaagtattgggctcacgggcgtgagccaccacgcctggccgaacggtcgccatttgtatttcatcttcttcatactgtctgttcacacacagcccattttgttaggttctctttttctgatttgtagacgttataacccgcatgcaaattatttgccttgttggatgttgtaacagctctgtcttaacagcattttgctcttttctattcagagtctctgtgcctttaggcacttgcaacagattgactgcatagtgtatttgtttacatgccgataatctttgaagttcgtgaggatctgatcctgctgtttcaagtttgctttcatgcacgtgttttgtaattttcaggatgtgccctcatgttgagggtctattgtgtgcgaggatcttaggtaacaaggcatgaagttaggtccctccagggaggttttctgtcataaacatcttggcctggttgtctgcaaaccagattgatattacaagcgtggggtctaaatgagtggtgactttttctcctgtggatctcaggcagagagaggacacagtgcttattctcaggggtggagggcaaatgttttttctagtccatctttttactgttaagtatcatgaccctcgaggatcccagcttcacgcaggagtcatctccactgcatttcaccatcttcccgatgcccaaagtcctatctgccacctggcccccaaacctaaacccggtggtttccaagagcaactccggtgtgagcccccacggtgtcttccgcgtctacttccttcgtcttgggctcctgtgggtctccttgcttttttatgggcacggctaggtgcgtctgcttcatttcctgcatttctacagtctgtagtggagggtttgcaggtcttatctgataagttgctggaaactgaagtctctcttctgtcctgtggaccagccctctcctgtccctgcggtgtcccagcatgggggctccacagggtggggacagtgacagcccacactggagctaggccccgggggtggcagcgaggatggcaaatggggtcagccccagggttttctggaggggccatgagggctggctgctgatatgggtgtggacagtgaggggaggggccccagggatgccttcagggctttggtctgaggcctgggctggggcagcgtcattgactgagatggggaagacctacgtgggcggaaggttctactcaggctgttaggtcggatgcccactagacacctgaggacgagctcggcaagacaggagagggagggggagaatgaaggcaagagggtgctggccaggcagggccatcagcactggtcggggagggggccaagagcaggcagcacttcctgcatatgtgctatttcccccatggaccaagtagcagttcacagaagaagcatctgggggccttgttaatgttttccgggaccctggccccagagcctccactttggcaggtcagggctggcccacgaacctgcatttctagctaggacacaggggatgctgctgtggacacaaggaccatgctctgagtgggccatcagtttggggagaggtggggacaagctgttggccatctgagggtgcagcagattggatgagagaagactctgcctctgtggcctcctctgtgtggcccaggagtggtggcccatggtccagcactgcagctgcctcttcccgcagctgcttttcctgtgtttcagctggggaagcagagggagctggtgacacctcgtggggccacagggaaggtcggcgacaaaaccaggcaagccctgtggtcacgcaggaggagttgggaccacgctgcatcagaggaaggctgtggagtattcaatgaatggaatttaatgtaactatgacataaacacacacagggtggggaggacgggtgaccaagcgcagacgtgggtgacacgtggccccgctctctggaccctcagtgggaaaaagtctgaggctggcgtctctcaccaaaccccacctcccctggtgggtcaatactgatctggctgagtgacagcatctcgtgacccaggctggccctgggaaggcgccacaggcgaggcctgcgagtccagggagcaggcagacgctacagtggcccccgagcgcgccaggtgccagcctcgacgtgtaaatggcccgctgcgggcgctgccgggaaggaagacaagaagggtgagggctcgtcctcaccaagtgcttcctgagtgccgtaggacgtgggtgggacatggggacagtgagggtaacacaaacagcaacgaatgcacaaagacaagttccaggaacacccataaacccataacgttcaacaaaatggcaacaaaacgacgcccctgctggcctggcgaggctggcgcttccttcgtggcagatgccacctgcagctggctggctggcaagcgttggccaagctttttggtacctgggagctcaacagcataaaaggctgtaacctctacacggaaaaatttcacatccttcccctgaaactgacttcaggggcaaagaaacgagacttcttgaagaccagcctcttctgggaaaggggcttctgagacgagtgtcgacggcagagcagatggcctggggaaggcaggggtccctgggcagaggctgggagggtggccagagaccagggagggcccctccatctggtgggtttggcaggtgtgtcccctggtgctgccaccaggagccccgaggccggggtgttggctgcgacagcccctcactgggtccggagctggtaatctccattctgcgtgatataacgcacccagggcagggcctggtacccactcttctcaatgatcttcaggtagcgcacctggatgccggaggtagtgaagtaagggatctcgaacttgacactgatcgggggcttgccctccttgtcttcggcctccacactaggcaggccgaagtgggcccgcatcaggtactccttgccgcccgggaaggacttgatggaccacacgatctcgctgttctcggggacccacttaacgctccccaccgtcgtcttgaacttgggtgagtcggcatcattgggcacgggaatgtggatctccacgttgttggctgttgaccgccgcttgaactggcttttggccttgatcatgtactcgatgcggctgtgggagtgcttctcgatcaccgactcgatccatatcaaaggcttgacgtgggtgttgagacggtaggacatgagctcgaactcgccgtcgggtgggatgaaggagatggtgcggtcattctcgaagcgtgatagccgcacacactggtggaacttcacatcctccagctccacggatttgcttttgccgcggcccgtgttgtcaaagaggaccttgtcgttgaggcccaggcgcagctcgggcatgcccgagaggaagactcgcatcttgatggagcccacgatctcgctgcgcaggacattgccgttggcgctgaccgtgtgacccagccatcccactcctgggtatttacccaagaggttgacagactcgatgacgtccaagaacacctcattcttccgatacttgatgccttcggaccgccaggacaccgcgttggtgacggtggctggtggccgcggggcccctgtttccagcttgtggccttcctgagtgatgtactcctgcaggatcttgctgtcggtggtctgggggtagccgaagtccatgagctcgtccagcagctcgtagatgataacaaagttgtcccggatgctctcctcctccagctccttgaagtactcggaaaacacctgcaccaccttatagaggaaagaaaagaccagcgacacgcacgcgttcttcttggatgtggcaaccagatacaggttgttgtgtttgatccacatgaaacggacccccccgtgggccaggatgggcgacagcatcccctcctcctccttctccatcaggatgggcatgaagtgctccacctctgacatgtccacgtcgccacggtagttccggcagatgagcaccttgcccttcaggtccagcacgtagacggcgctggcggacatgatggctgcaggaggcctcggcagcggccgagggcggtggcggcggcagcgacggtggggactgctgggcgttgagcaaggccgggcgccgcccgcgacagctcacctccacttcc

SEQ ID NO: 14971 - RNA, 854 nt, Homo sapiens
  source 1..854: mol_type = other RNA
gctgggattacaggcatgagccactgagcccagccagaaacatattaatactataaacaacactcagccctgggctggttaagaggctggagactgaaaggtggtgttgattgaccatggacccagggaaatatctgcagtgggttaaggatactctgtgtgtcttacaaaacagagacacagatgctgcctaagaacgaggtcctcctggaaccggtgccagggaaggattttgttgctcacactagtcttgatcttctgggctcgagtgatcctcctgcctaagtgttgggattacaggcatgtaccaccgcgtccagatgcctggtatcctggagtcccaggagcactttttctggaagtaggagcttgtttcctgcaggtgccaagacagagaccgacattgtttgttggctgggtcggtctcccagttttcagctggctccagtctcacctgttgctcacacaccctccatgtctcccatagtcccctcggtggggacagaggcactggatgaagccctgctcgtcaccacagagacactgtgcaacctcagtttccccaggtggagaccggaccaacagtgatggcctctgcctcttcaggtcatagtacagatgaatacaggctggcacggcctaggcactcagtaacacacagcagaggcacagggacttaagatggagtgtcccaggcagccacagttggctggcacccagctgggaagggcccaagggcttttaaagcagggtgaaaaaaaagcccacctcctttctgggaaactgaaactgaaaacctaattaatcctctgcctgtaggtgcctcatgcaagagctgctggtcagagcacttc

SEQ ID NO: 14972 - RNA, 746 nt, Homo sapiens
  source 1..746: mol_type = other RNA
gctgggattacaggcatgagccactgagcccagccagaaacatattaatactataaacaacactcagccctgggctggttaagaggctggagactgaaaggtggtgttgattgaccatggacccagggaaatatctgcagtgggttaaggatactctgtgtgtcttacaaaacagagacacagatgctgcctaagaacgaggtcctcctggaaccggtgccagggaaggattttgttgctcacactagtcttgatcttctgggctcgagtgatcctcctgcctaagtgttgggattacaggcatgtaccaccgcgtctgtaccaaagggaaagttaggtctggagactgagccacacaacactgaagttcctttcccgaatgcatggctgttgcttcctgattgtgttaagtggttaagcattgtagcttacccagatgcctggtatcctggagtcccaggagcactttttctggaagtaggagcttgtttcctgcaggtgccaagacagagaccgacattgtttgttggctgggtcggtctcccagttttcagctggctccagtctcacctgttgctcacacaccctccatgtctcccatagtcccctcggtggggacagaggcactggatgaagccctgctcgtcaccacagagacacctcctttctgggaaactgaaactgaaaacctaattaatcctctgcctgtaggtgcctcatgcaagagctgctggtcagagcacttc

SEQ ID NO: 14973 - RNA, 2213 nt, Homo sapiens
  source 1..2213: mol_type = other RNA
gctgggattacaggcatgagccactgagcccggcccaaaatgaatcttttacatttactgttacttactgttaaacatcttggtgagtgagttgtgggcaccctgagtacataaacacctttgcaatcacaaagcttttaagatcaaaactgttatagaaatagatcaagcagccttaggcacagacggtattgttgtagaatccacagcagttagtaagggccatagcactgaactccttatcttcccagggaccagaaaaagaaggagggttggtgccattcagagaagtactctgaaagagccctctgcagcacatgtaggtctcataggttctattggtgaaacttgtgtttgggaaggagacacagtcagcttcagctcccctggggacatagaggattcctgccatacaggcactgataagggatacacaggcccctgtgaagagggccctgaccacaaccttggacaagtcactcttccggtgaggtactattgatgtcaagcctccaagtgtgattcctatggaactaagattggcaaatccacagagtgaaaatgttgtaatgatttcagctctcacagaaatccactgtttctctccctcaatccactcctccattccagagagacgtttgttcttgtattgagacagttgctgataagccacaaactcatttatgaagaacttgattcccaccatctcagccaccattggacagtctgtccactctacacccatcatgaaaaccatgggccttaggagataggagcagatgacctggaaagtgagcccctgtatgtccaccaattcccccagccaggagagggcagcattgatgaaggccaacacagccaaaaaggcaatcaggttggctgctacattagtagcaaggcctatggcatctacggctccgttgctggcagcttccaggacattcctctccttcccacggggcagctttaccccctcctcactcttgaacttggactcctccacttccggatacgctagctttgatgaggcgagagcacaaggggcggccatcacagaggcagaaatcagggatgatgcatcaaccccaaaggctatgaaggctcccagcacagtgccagaaatggtggcaaaccctccagtcatcaccgcatggatttcagagagtgtcatgtccccaaggtagggacggatgagcagaggtgcctctgtcatacccacaaagatgtttcctgccacagccagggtctctgtagcagtggtgcccatagtgatttgtaaaaaccaggcgaccttctgaactacccattgcacaaggcccaggtagtagagaatggacaccacacatccaaagaaaatgatgattggtaaggcctgaaaagcaaagacatccttgaccagtgtatccccaaagacaaaactggagccggccacagtgtagttcaggaaaatctggacctgctctcccagccactgaaatacagtatatccaagatcagttctgatgaccaagatcccaaagacaaattgaagacctaggcccgaaaacactgtcctccaggacactgcgctgtggtgtttggagcaggcaaagaggataaggatgaacatgcagattcctgcaaaggggatcagctgctctggcctttgggctgtgtctaaagccaaccacagtataaggccaaccaaggagactcctgcaaacacccatttcgtccaaagcctcaggcgggagttttcaaagggcttcagacatcttgttaattttttgcccaggagctttttcaaaaacgagtgaaccaggacaaagatcaccaagcaggtgatgacaaacaaggccagtgccctctggaaattcaagatgcaagctgccaggagataggcagcataggccaaacacaacaggcccaacaggatcttcttgaacaagctggcgtgtgttttgcagaaacttcttgctttgctgaaaggccaccgactcctcctctggtaagtggaagggcccagtccatcccccaggctgtgtccttgtgcgtcagtcctcttgcttccctcaggctctacttctttttccatgagctccagccccgggttcactgtgccagtctccactgtggacagagcaatggactgtcttccacttgctttctccatctcctgttctcctcaacccagcttgtggaattgattccctctggctcctcagtgaaggact

SEQ ID NO: 14974 - RNA, 12029 nt, Homo sapiens
  source 1..12029: mol_type = other RNA
gctgggattacaggcatgagccactgagcctgaccccaccccctttacatttttaaaaatgtctgaggtcctcaaataacttttacttatgaggattacattgatcgaagaaattggaactgaaagtttcggaatatacaagcacacattctattacccatcagtgatgtcatgacattatatagcttctgtaaaactccactgttcacttgtgaatatgaggaaaaggcaaataacatcatagtgccagtataaaaattttgatctcacatattccctgaaaaggatcttgaaggttcaataccacatcttgatagtgatcaagagatacattaacttccttttttctgtctgtgactcttggttagggcaaatttcaaatccattataatacatacattgcagcaacactgagtttcttataataggtactatccaaagctttcttttttttacatgtatcacttaatcctcacaaccacctgaggattaataccatttacctgtcttacagataaggaaaacaatcatttttcaattatgactatgcccccaaacactggtttggatggagccttcactggtatagagaatgaccttcttcccttagactagactctggctataataaaggatggtttaatcatcccctgaagcaatgcataagataatctgcaatgtatcttcacatactgtaccttatttgataggcaagagacccataaaggaagctgagcatggattatcagcttcatcacaaatctgaagaaactgacatttatgttatgttgccttacccaagttgggacatcagagcagcaactaaaatccaggtcttcttcctattacatgccgtaaaaggtattgtttctttccctcccctcaaaattttcagtcaaatgtcagcttttaggaagagccaatcactctgaactagaattgttctcttcacttaaaatttctcaagcctaacttctttttgggtcctacaaaccgggaaaatacctcagaattggaaccacatgtttacagtataagaaatgacacaagtgtgacttgggcaaaaagaggataactttccccttcagagaaataatccctttatccaaggcctggagattagtgtttgaggtagaataaaagcacagtaaaatgattctatggtttgaattttggctcttctgctcaagtactttctttggtagtatactaattaccactgaattactaattattaattattattaattactaataaaagtaaaatgtagtagtggtggtggtctctttgagttattgaacattaagtagcaaacattacattaagtactttatgtacactctttcacttaccatgtccttgagatgattatgactaaatttaataaatgtccttttgtgcactaacccatttaaaccccacatccttgagataggaataactattacttcccgcacttgcagaacagtttataactgctacagccaggccttagctactatgcaatattataaaactaagagtacaaaaacgaagaaatcatgaaagtcccttcagtacagccagaaaagaacacttctaattactcagagaaatacatgttgtgccagtcgctttatctcctttagcgagggaaatcttctaaggtcttcaatgacataatgtcactgaaactattccctcacacttaaataatgtacatgaagataaaattctaggctgtaattttcttccttcgacacactggaaattttactttttatcttactattaaaacatctgttatcggccaggtgcagtggctcacaccctgtaatcacagcactttgtgaggccgaggcaggcagatcacctgagttcaggagttcgaggctagcctggccaacatggcgaaaccccgtctctactaattaaaatacaaaaattctgggaatggtagtgggagcctgtaatcccagctacttgggaggctaaggctggagaactgcttgaacctgggaagcggagattgcagtgagccaacatcgtgccattgcactccagtctgggcgacaagagcagaactccatctgagaaaaaaaaaaaaatctattatctgatcaatgttcctttgtaggtgacctttctctgaaagatttctaagattgtttttgatgctcttatttgctctataatgcatacaggtatagggaatttcttgttttctgtttaacagttaacaaatgaggtctttttttttttttaagtaagaaacaaggtatcgctctgttgctagactggagtgcagtgacgcgatctcggccacatgatccactagcctcagcctcccaaactgctgggattacaggcaccactgcgcccggcctcatttatttctttaattctaggaaacagtattttttttaatccagtgtattcgcttggtttttctagctttattactgctttgtttccaacatgctgttatatagtggtgacaaaacaaacaagatgctcaatctcatggaaattatgaggcagacagattagcaacagtgggatattttgcaggggagagggagaccatacattctaggtgaaatgtgagctaagaccaaattagcaagcagctatcatgcacgtatctgagtgaggaacacagctaaacgtcaattccaaacaataacgaattgatcaatgatgaatttaatctcagagttgctggatgcctctcttcaggtctgctcagacctcaattttccaatcttgtcccccaagaaaaagattaaacctgtcttgtgctgagtagtgtaatattccagtacggcttctcttgcgccctagtgctcaggccacgcagtggctcacgcttgtaatcccagcactttgggaggccgaggtgggcagatcacctgagatcagttcgggaccagtcaggccaagatggtgaaaccctgtctctactaaaaatacaaaaatcagttgggtgtggtggcatgcacctgtaatcccaactacccaggaggctgatgcaggagaatcgctggaccccgctcggaggcagaggctgcagtgagccgagatcacgccactacactgtagcctaggcgacagagcaagactccgtctcaaaaaaacaagacaaaaaaaaaacttatctaaaattgctaagactaaaaaaatcatataccattgctaagacattgatgaaagatttcatcacacgtttgcttggaaatgttcaagtaccacctttaccatacctcttaacaccttcaaaatatggaatagtgactcactaaagaaataaagccaaaaagtattttttatactttgatcaggttctcaaagataaggcctagtttaagaataatttttcatgtaagacaagacagggagtatttgtttctacatcatgaaatgagtccatctattcccctctgtcccttactaaaatctggaaactaaatgactgtaaaaaatgaaacaggtgttaaacacccccagacaataaaatagaagcaatggcaaagcaagattttgggaactgaaaaataaatggatcagtgttaactgactcaatagacaacagaaatgaaagtatcagtgttagatagaggttttcactaaaaaacccagaagtggttgaaagaagagtcaaacaccatggccccatacctccctgtaaagtaattaccactccccctcacagtgtaagaaatgtcacgactaactcactgaaaagggtgaatcagtctggaataggggaatccacatatagacagggtagagtattttactgaaaactgaggaagtctacattttgaacagtaaaatctctaatacactgtccctcctcctcaccccaaaagaaaactggcaaagtacatatactcacacaggacaagtgattagagaatttctctcagatatatatgtacatattctctctcatatacatatactgacaattgggtgaccctcaaataaatggtctagtgaaatcacactggagtaaaatccacctgttgagaaccctcatgcatggagcttagagagatttcttctagctcttaaatttgaggaacagtaaatgatcccaaggcatttgaagaagcatcaaaataaaagacagactaaactttaaaaagggaagaatcatttaatgaaacaagactatgcagatgggggaaagaaattttgttacgagttctaggcagaagtgctagtggtggtggctcatacatataataccaatgctttgggaagcaaacataggaggaccctctgagaacaggaattcaagacgagcctgggcaacatagcaagaccctgtctcaagaaattttttttttttttttaaattatctgggcatagtgtcacatgcctgtagccaagatattctgaaagctgagatgggaagatggcttgagcccagaaattcaagaatgtagtgagctatagttgcaccactgctctccaacctggacaacagcaagaccatgtctcattcaaacaaaaaaattctaggcagagaagggaccacacattcaaaagacaaaaccctccaagaaatcattctaaaaaatccccatgaattaaaagacagattttcagactgagctgattcaagagtaaaacaaaacaaaaataagatacacaacataaagatgggcatggtgtcacatgagtgtagtccacattacttgagtgacatagggggaaagataacttgaaaccaggaattcacaagtctgtgcaacatagcaggagtctctttaaaaatgaaaaaaaaaaagaaaaaaaaaaaagacccataccaagacacatcactgtgttattaatttagaatacaaaagacaaagaaacactggaagctcacattaacaaaaggctggttccccccaccttcaacagactggaaatcaaagcagcattcgggccaggtgcaggagctcacacctgtaatcccagccctttgggaggccaagccggggggaattgctggagcccaggagttcaggaccagcctgggcaacatggtgagaccctgtctccacaaaaaattaaaaatttagcagggcatttggtgcatggctgtggtccaaactaaattggtggctgaggcaggaggatcacttgagcccgggaggtcaaggctgcagtgagctgtattcatgcctaggtgacagaatgagaccctgtctcaaaaaaaaaaaaaaaaaaaaggaaccattaattttctctcccacaacactggaagttctgagacaacacaacaactttcgaaattctgagaagataataattcctactctaaaatcccaaaccagaactatccatcaaatataagaatccaacaaaaatacagccagatatgcgagttctcaaaaaattcatttcccttgaattcttttcttgggaaaacacaagacaacataatccatcaaagtgagcgagtaaaccaaggaggaaaaaaagttagatccagccaggcgcagtggctcacacctgtagtaccaacactttgggaggccgaggagggtggatcacctgaggtcaggagttcgagaccagcgtggccaacatggtgaaaccctgtccctactaaaaatacaaaaattagctgggcatggtggtgggcgcttgtaattctagctactcaggaggctgaggcaggagaatagtttaaacctgggagacagaggttgcagtgagccgagatcaagccattgcactccagcctgggcaacaagagtgaaactctgtcttaaaggaaaaaaaaagggggggggggggagacacaagacacagtaaacagtaattccaaaacatgaaacagccaacaggaatacccaggagtatggtaaaggaaggttccagatggaatcagttctacagtccaaactagaagaatgttccagggagtagaggtgatgggatatatttggagggggaggtttattactgaatcatgagatctgttttaatatactgaggggcttatatttccagagtgattagatataaattactggtaggtaaaaaacagttaagtattaacttcagggagaaaaaaaaagctgcacaagaatgaaaataaaatcacagcatattccatggcttatctaaagctttaataatacttacacagccataataaaagtaattattgagccaatcaaaagttatataactacactaaaaagatgtaagggatcattatttcatgttgaagtggtgagaggtggtaggaatgcaggcttttcaagaaggtatttctaagaatttttaagcatttgctcttaaatatgaggaacagtaaatgatcccaaggcatctgaagaaacatcaaaataaaacactaaactaaggggaaaatcaaatgaaacagactatgtggggggtggcggggggtgggggcagagacatgacgacttttatagaaagtaggctgggcgcattggctcaggcctgtaatcccagcacttagtccgaggcagatgatcagttgaggtgaggagttcgagaccagcctggccaacatggtgaaaccacgtttctactaaaaataagaaaattagccaggtgtggtggcgcacacttctagtcccagctactcgggaggccaaggaatgagaatcacttaaacccggggggcagatgttgcagtgagccaagatcacaccactgtacttcagcccaggtgacgaagtgaaactgtttataaaaaaaaaaaaaaaaaaagccagatgtggtggctcacgcctgcaatcccagcactttgggaggccaaggcgggcagatcacaaggtcaggagttggagaccagccttaccaacatggtgaaacccagtctctactaaaaatataaaaattagccaggcatggtggcatgcacctgtaaccccagctgctcaggaggctgaggtaggagaatcgcttgaacccgggacacagagattgcagtcagctgagattgcactactgcactccagcctgggcgacagtgcgagactcaaaaaaaggggaaaaaaaggaaagaaagaaaaagtacaggcaacaagatttcctttagaatcagacatgaaatatgagggaaggaagagaagaatgactctaagatttttggtttaaataactggaagaataaagttgtcatttattgaactaaggaaaatgcaaaagaagtaaatttggattaaacaagatgaaaagtacagatatagttatcaagcacctagtaaacagtcggatatgtgaatctggaattcaggagaaaggttctggctggagatataaatttgagtcaccagcacagttcccattaaagaaatgaagaccatcaagggaatcccaaactaggcttaggatatttcaatgtttagaggatagaaaaggaaacagcaaaggaaactgagaaaagagtcagagaaataggaagaaaaagcaggaaaatatgtttcctagaagccaaataaagtaaatgttttaatggagaagagtcaacaactgtatgaaatgctgctaatagatcaagtaaaatgaggtcactgacgtcacgagaccttaaaaataccagctccaatggaaatgaatatctgattggaatgggttcagaaaaaacagaacaaactaaaaacaatgaatacaggcaaggagttttgctataatagaactctttttcaaggagctttgttataaaagaaatgagacattgcaattggctcaagctacgacaaacaatatatccgcagtatataataaagggcagatggggacagatgggcacagatgctaggtttacagatgcaacggtgacaacttttaaagattcttttctgactgcgtctattttctcagggcaatagggagcaaagtgagagggaggagatatgagacgtgcaatgacagagtaaaactatgaaaccagtcatttaggacaatgtaacaggaaagactgggtcactaaggacaagatcacgagtttcaagcaagcctaggtcagcatgcttatgtaatgggttaacattttgacttaaaaaacaaataaacctgctctatagtcttttatttaaccaaatgttctatctgaagtttttcttcaccaccaaagaacttatccatgtaaccaaaacccacctgtacctcaaaacgattaaaataaaaatttaaaagaaaagacctgtgccaataggacacagggaaaaaaaattaagtttttcttaagtgacggttccattatccttaacagatcatctgatctgcatttgaatatacatggcaacagcaatatttttccatgaaataaacactaacacagaaatgtatggcttatggagtatgtcccctctccagggtacattcaggatttctcttcctcattgtctgatatcctttcacacagggtctaaattgtgcctcttttggcctttatgctgttctattacagattgtgcattacttacatattcctaaggcctattctcttatatttggttctagttaacccactactataaattttcagggtctgtcttgttttgcatgatacactaccatttccaatttctagtcgtttctcaagaccctaaagtttcattcagaaacttctcttgtgctaacacaatgtccacttgaaatctctatatgacacactcctatagtactagtgaatgaaaccaagaaaacaaaataaccaaatcctaccgacagccaagtcttttgctattattgcacctaagctattcctgaagaaataatttaatgagatcatcttataaggaacatttatttggtaaactatctcatagaaatagactctaaaatcaaacagtttcttaaacaacagagagcataatcccaatctctccccatgaaaagcctacttcataactgaagtacctaaagcccatgaactgcattactagaagaaaggagggaaaaagacatttactaaacttccacaggaagactgtataaatctggaagtggttaagtacacatcagcctgtatccaagaatactactcagtctcaaaaattaactgaaaatctaaacttaatatggatacttctttgttcttggtaaggctcagaaaattaccatctatttaagtacgcatggtactagttacatgtcaactgatataataaaaaaggtgaagtggacaatcagtatttcaaacccaatacagggaaatcactagatgtaaataagaacttttaaaagctattcttgagctccactttaaaacaaacattcaggactggaatcttcagaattttctaatatcttgaatatccccatcttctctttaattggtcctgaagcattcatttgatcaataagatcacttcgatctaacaacaactctagatctttatcactaatgaccttctctcttgatccttttatttccctttcataatctctagattttaataattccattaattccttaggatctaagaaattcttagacagatttaatccagactgaccacctttgaaatgatttttatggatgatcaacttttccagtttccttttagcagctgctctttccacaattttctgatcgatagtatttgctgtaacaaggcgataaacaacaactggctttgtctgaccaattctatgacatctatcctgggcctgaagatccgactgggggttccaatcactatcataaatgataactgtatctgctgcagtcagattaatgcccaggccaccagctcgtgtactcactaagaagataaacacctctggatccgtgttgaagctgtgcatgtttttttctctctctgagtaagacatggacccatcaagcctgctgaagttgaaatctctgagatggcagtaatccatcaaaatgtccaacatgcttgtcatttgtgaaaaaagcagcaccttgtgacctcttttttttagttctggcagcattcgatccaaaatcaagaacttcccagaatttgttaccaattcttcatcgatcttaaattcttgtgtaacagggtctataggatattcaatcaaatatggatgattacaacatttacgaagtagcatcattatattctgcagcttcagattaacttcagattctacagggatattcacttccacaacagctctttctcggtccacctctggctgtatttgactgatcagtttttccaattcattagggaaatcatctattttgctgtaatttattgattttctagttcgtcgttttggtcgaccagtaggacttaactcaattgtttctttctcactggatccaaacatgtttgcaattgtacggttcacaatggctgtataaaagatctcctgcttctttgaaagtggagcataaacgactacttctcgtttaggaggaacttcaagagcaacatcagacttcagtcttctcaataagaaaggtgttaaaatctcaaaattggtatgaagcttgagtaaataagtattttcatatggacgtatatcatataaatcttttctggagggcaatttgccttcaaagaagccctcatctgtaaactctgacacatacattctaggaattctttcctggtgcagcatatgcaatacattctgttctctttctttagcaataatatcttcagcagtttcagaaagactagtgatgtcaaaccaagactcaaagcttttcaagtcatcaaatacatctggcaacaaaaagtttagcaatgaccaaagttctgataaattgttttgcaagggagtaccagtcaaaagaagtttgttatcagcattgaatcgttttaactccctgattagacggcacttcatattcttaatcctgtgtccttcatctactattaagtatttccaatagcaatgctgtaacgcatttcggtctctcatggctatttcaaatgacgtgattaccacaggatgaatctgcaaagtccctttccgtttgtaaatatttcttaccaatttttgacgttcctcctgggttccatgatataacattgtagggatatctggtgtaaatcttttgaattcagccatccagttaggaagtgtagacaaagggccacagacaagaaaaggtcctggtactcctctctgaatcatcaatgcaatagtagcaatgcactgaactgtcttacccaatcccatttcatctgctaaaatgccattaattccattttcccaaagcatcctaagccattccatgccttctacttggtaccatcgcatcactcctccagtgaagtgctttggttgttgaaaaggtactggctgaccattacacttccggactgggtcaaaaaagaatttagtattctgcctaaccgtttcagacaatctatctttaattatactattcgaatctttatttttctgaagatcttccacacagagattagtagaggaggagttttcatcctcattctcctttttattttttttagccacagacaaaatttcctcttttgacatgacctctgaaatattgtatgattcatcttctcttcctctttttttcctcataactggcttctcttcacttgcatcaattgaatttttaccctttttaacttttaaagactccttttttctctccaatttttctttcttcttctgttcctctaattgttgctgttccattttcgtcaataaaaatttggagtatatattgcttttttcaagcaaatgttgaagtctacggtaccgaatttctgtcgactctctatcccaagacatgcgagccttttccagcatcttccgctctctctctagtccagcagcttcaagctgttcttcctcttctagcatggccggggtaatcacagcagtgtccagttgttcaaccattgctggagcctccgagccgccgctgcccgcgggccgttccgctggcatgcctggacactcacccgggaaccgggtcccctcctctcagagcctgcaatgccgcgagctaactcctcacaaccgctgccggcccagccttctagccaaatcccccgccagggaaaaaagcgcgcttctccttcgcgggaaaat

SEQ ID NO: 14975 - RNA, 3774 nt, Homo sapiens
  source 1..3774: mol_type = other RNA
gctgggattacaggcatgagccactgagcctggccgagaatcttatttcttaacaaacaactatatacattagcttgattgcctataaagggatatgaacctgacctcatatatgagagtactgtcctaaatggaatttgcatgatgacaggatttattctgttttaggatcatgtgatatttgaataaacagaaatataaaaacaaagaatgacagatgcagctgaatactcaagagtgaaggatgagagacagggactctgaaatgagatctttttccccaagtgttttattgttactgggcattgaaggaagaatctgataatgctattctggtagagctttacaatggcatttatatgacaccatatttggaaaggttcctcagacaatctaagtgccagcaagttgaatggcattattactggataataacaaggctggaaaacttagaatagcttaccttcccattgcgttacctaatttatctaatatatcctaaatgtaagtactttgggaatttcagaagaaaaagtattgaatgtcaacacaaataatcttttttgtctttataatttctaagatctctattattttagaagatattctaaatattattttagaagattactgaaattgctcaaaaatccccaaagagctattaaaggtctgtgatttttttaaatctttttggcattctttccctataaacataggtatattaaaatataattgatgggaagattatagagtatgaagcttgagaaatctgtatttccacatagataacaattgcattggcagaatctgtctgttgtagctattttggaactctggagtccactgaaggcctgaatattccagggaaaggggcacaaattgtgattaatttcaatcaatttcagttcttagcacagtaataactacccattccccatctttcagccccatggcaggcagctgtgcatgtactcctggtttgcacatggcttgtgggagccacggtgggcaaaaaggactctatcctgcaaatattgggatctgtattctgattactgattgccgttttcaatcacagaggtacaaaaaagaggtggtagccattattgttgtaccttcctctctagctgaagtgactcctagggaatttaaagggctgatgccttttttcgcttcccttaatttttcttctttccctttttgggacccagatattgaaaactaggacattcaaaagcaactacatatgtgggagactttagatagctactgtgcatgttccaggcaaggcactggctcagaaaagactttaagtttatacctcagagtgatccttgctatagagttggcctacaacaatcaaaaacatgaaaacaaataccagcaaccctagcaaagggggagaatctgatttcaagaattatcatattattcgattcatatgtccagttttcaacaaaaataaaattacaaggcatatagagcaacaggaacgtattaagcattaaagggaaaataaataaataaaccaatggacactgagctgaaaagacctaatgatggatccattagccagatacttaaactacctatcatagagatgatcaaaaaaactaaaggaataattggggaaagtcaagaaaataatgtctgatcaaaagggcaacatcaataaagagagagtgatgcaaagaaaccaaaaataaattgtaaagctgaaaaatataatgactgacatgagaaattcactagaactcaaaggcagattttgacaggcagaagaaagaattaatgaatttaaagataggtcaatgaaaattaagtctgaggaacagagagaaaaaaaaagttgaagaaagatgaacagagcctaagggacctgtggtacaccatcaagtgaaccaacgtatgcattgtgagagccccagaaggaaaagagggagacagaaaggggcagagagattatttgaagaaataatgaataaaaacttcccaaatttgttgaatgacatgaatatgaacatcaaaaagctcaccaaaatacaaatagggtgagcctgaaagactcacaccaaaacacattataaatactactattgaaagtcagagacaaagagagaattttgaaagcagcagaagagaagagatttgtcatgcactagggatcctcactaagattatcagcagattttttcattagaagctttacaggccagaaggctcagatattcaaagtggtaaaagaaaaaaaactgtcagccaataatcacgtatccaacaaaactgtactgcaaaagaagtaaaggagtgaagaagaaattaaggcattcccagataaaacctgagaaaatttattagaactagatctgcccttcaagaaatgctaaagggagtccagaaggttaaaatgaggtgatgctagacagtaacttgaagctatataaagaaataaaggtctttgtattggtaaatatatttgtaagtagaaaagctagtgttattttaacatggtatgtaattccactttttgtttctatatgaattaagagaataacggatttttaaaatatattggtctaaaaatcaatattattataactttggtttataactccatgttttgttttctatataatttaagagactaatggataaaaattattagttgatgttttgaggaagtcaagatatatagatgtaattttatgacatcaacaacagaaaggggagggtataatgttgttaaagtagcacagtttttatatgttatagaagttaagctggcataaattcaaattacagtgtaataacttcaggatgttaaatataatttccatggtaaccacaaagacaacagctaaagaatatacagaaaaaatcgaaaaggaatttaatcatttcattatcaaaacaagaaatcaaccaaacacaaaagaagacaggaatacaggaaatgagggacaaaataaacctataaggcatatagaaaacaagtcacaaaatgacagaatcaaacctctccttaacagtaattactttaaatgtaaatggattaaacagcctagtcaatagacagaggttgacaaaatggttttaaaaaatcataatccaactatatactgtcttcacagacttactttagaaccagtgatgcaaataggttaaaagtaaaaggacagaaaaggatattccatgtaaatagtaaaccaaaacagagcagagttggctatactaatatcagaaaaaatagactttaaataaaaaatgctagcaaagagacaaaagacagaagttaagtaagaaaacagaggacttgaacaaaacagtaaaccagctggatctaacagatacatgccaaacactctacctaacaacagcatacacattcttctcaagtacacgtgagacattttccaggatagaccatatgcaaggccacaaatgaagtctcagtaaattttaaaagacagacattgtacagagtgtcttctctgatcacaataggatggcattagaaatcagtaacagaaggaaaactgaaaaattcaaaaatttgtgaaaattgaataacacaatcttaagcaacaactggattaaataagaaaacacaaggggaattagataatacttaaaagacaaatgaaaacaaaaacacaacatatccaaacatatggaagtaatgaaaacagtactaaggggaaattttatagctacaaatacttatatttaaaaataagacaaatgtctaagcttacaacttagaaactagaaaaa

SEQ ID NO: 14976 - RNA, 4545 nt, Homo sapiens
  source 1..4545: mol_type = other RNA
gctgggattacaggcatgagccactgagcctggcctactctaatattctttagtggcatcctttctcacttaaaaaaaaaaatcactgcaattgtcctacaaggctctatatcagtgatggcctggagaagggttatactagctcacaagagctgactgttatattttccattgctagcttgaaattggccatggtgagagtgtttacaccagaaaaactgcaaacactacagatcaggaccttttattattgatttttttccctagagagccagctgctaaacatttaccagaataccagtaccctatatgatctatcccacctcacctccatgttagctcaatgttctcacctcatcttttgccactttcccatttgcccaacctactccactggcatattccttcctgcttcaggtcttgcatatactgtttagtttgcctggactatgtaaattactgtgtaacacagtctacctaaaacaacaaaccaaaattctccacctccacagcacacatgacatagaatattttatcagtttatctatctgtctgtctgcctgtctgtctgcctgtctatctatctatctatcatcctgcattcatctcttcgtgataggctgtaaactccacaaaggaaactgatgtcaattttgtcctgctgtatccccagtaccttaaaaaagccatggcaaacagcaggtgctcaataaatatttttctgaacaaatgaatggatagaagttgcccttagtggtctaaatctaaatatttacatttctatctctttttaatagaaattacttgccatgttgagtatgaagaattattgatttttaaatgcacaaatagctgttttgaatgacacccatgcttttggtttaaatctcttatgctcatctgagtatacctagccatgagtccatctagtctgcctgttatggttcatttgatgacaaatacagggagagatgaaagcaacatccatctacaagggataaaggccagagcttgacaaatgactgtcaaaatggagagaggggtcaacttacatgctaaaggtttacacccggtatctagaagaaaagtagtaccctgacacaagcaataagctaagagaagtagctggtttaacagatgctggtgaatttgttttagataaaccaaaattgaaatggctgatggttgtattaggaaaagcacctcatgtctggatgtgggaatcatcaacacatgtactctttttgaactcaaaactgagttgtctcatgaacagaagtagaaagggggaaggagcatggaaaagacagatattaagctgatcattgaataaagaaaattaggtagaaccccagataatccccactgctgtagaacatggaaaagaatcagaaaagatgacatcgagaaaggaacaatgggaaaggtctactttgggctggaagagatcaaaagctcagtgtggaacatgttcagtttgagatgtctctgaagtatctgtgaacgaacgtcagataggtgtttagatgcataagtgtgaaattcagctaaagtttgagctcatataaatggagttaacagctaatagatggtatataaagccttgggcatgtataaggtcacccagggagagaatcttatgagcagcagagagtcgagaataaagctatattccacatttgatggcttggtaagaaaaagcctgtaaagtgagcagccaaagatgtaggcgaaaaaatacaagagaatatttgtctcagggaaaccatggaaaaaggagattcaagaaagggcaacacatattgctgaggtcaattaaaagttcactggatacagagcaagaattcactggatggagatgcacacatacatacatcccttttagactaaactgtatttttgaagttataagaaggaaaaccagattaaaatggattgcaaactaagaaaatgtaggcaatatgaacagaaaacacttaaaaaatgtgtaaagagtagaaagagagggtgcaagatgaggatgtgaggtatatgaatgattttttttttttaagagatacttgaccatatttataaaacaatgagatggaatttctgcttctggtatggctgacaatcttacagtagataacaactataagctttgaacaaacttataaaaagcaactgctggaggaggaggtgaagcaagatggccagatagcacctcctagagattatccccctcccccaccgcaggaacaccaaattagtacccacacaagaaagcacctttgtaagaacaagaaatcagatgagtgatcacagtacctgattttaacactgtattaaagaaaaaggcactgtagaaggtaggaaagacagtattgaattgcctacacacccctctctcatcccccatcagctgcagcatggtgcagagagaatctgtgtaggccaggcatggtggctcacgcctgtaatcccagcactttgggaggctgaggcaggtggatcacctgaggtcaggagttcaagagaagcctggccaacatggtgaaaccccgtctctactaaaaatacaaaaattagccgggtgtggtggcaggtgtctgtaatcccagctactcgggagagggaggtaggagaatcgcttgaacctaggaggcggaggctgcagtgagcgaagatcgcaccactgcacttcagtgcctggtcaacagggtgagactccaccaaaaaaaaagaaaaagagagaatctgtgtgcactggacagtgcttccccgtcacagtggagagcaacacatgacagaacccacagagagagtatttagaccagccctaaccacaggggaattgtctatcccagtgggcagaaactgagttccagctagcaccatcatcatgggctaaagcactctggggtcctaaataaacttgaatagcagtctacgccacaagactgcaattcctgggcaagctctggtgctgtaccgtgcttgagtcagccaacttgggatacacaagacccagtgagacaccagccagggcagccaagggagtgcctgcatcacccctcctccaatcccaggcagtacaaattgcagctgcagaagagattccttccctccacttgaggagaggggagggaagagtaaagaggactttgtcttgcaacttggagacctgctcagccacagtaggacagcacacttggtagagtcctgagggcctcattccaggacctagctcccggatgacctttgtagacacaccctgggccagaagggaacccgctgccttgaagggaagaacccagctctggcagaattcataatatgctgactaaagagcccttgggccttgaaaaacatcagttgtacccaggcagtatttgctgtatgtcttgggtgagactcagagatgttctggcttcagtcctgacatagcacagtcccagtggtagtggtcataggcatgcttgtatcacctctcccctagctccaggcaactcagcatggagagacagaaactccatttgtacgtaagtattcacagcaactttattcataataaccaaaccttcattattatctcaggaggaatacaatgagttagaagctcatacagccttccacgaacttcaaggagcctttgtggagtttgctgactgacaatagcatttgcagtctccctcagatacacctcccaatctgtctcagggatttcttgatctgcagtaaaaggatattgttgcactctgcaggcttcacacataagcagggcttttctgagatttctacaagacttctctgcaagtctatgagccagttgtgaaggaagattcagaccttccttcttacacacagtagataacacgtggcaaatatcttcaatgctgggagcaggcacacgaaccgccaagcacctactacgaataggtgggatcactttagatgtagaattgcagcacaagatcaatctgcaggtagacatatatttttccatggttcttcgcaaggcatgctgagcatctttggtgagtttgtcaacttctgtcaataataccactttaaaatccctttgagagtttgtttcaagttgttgtgattgtgccactgttttcaacatctcctgaatgactactcggtcactatttccagcatcactaggattaacttcaaggtggtagttacttgcaatggtgctaatttcaattttttttttagatggagttgtgatggtctgatgttcaattctcaatttttccactccaacaccataaagttcacgtagaatacacataattcttgtcttttttccagcacctgatggtccgtacactaacagatgaggaaagtcaccacactgcaccaggttccgcagctgggccgcctgctccttgtgatagtccagccgtcccaaggagcagggccgatacttgtccacccagaggctcatggcagctcgagttcccgggggcctacgcttgaaaatcccgcgcgagcgcgcgtcctccccacaacgcagagacaagttttcccgcgagctccaaatctcgtgac

SEQ ID NO: 14977 - RNA, 3400 nt, Homo sapiens
  source 1..3400: mol_type = other RNA
gctgggattacaggcatgagccactgagcctggctgtgtttttctttctcattgcagagacaaagcgggttacttctggttcattcacgcatccaagtcctgacatgtctcaagggcattactgtgcttgtcagggagggagggcccagtccatcctctggttattcccatccatcccctaggccttcccttggctcaccctgccccctgccaggcccctttgcttgctggcctgacggggctgggtctctgtggctggaggagatggcctctgccccacccccctcgactgtcctgggcacaaaggagaacagctttgcctggaaagggcccaagacaccctgagaaacttgtagcgatgggacctgcctcctgcagccctccacctgcgtcatccttcctgtgccctccttgtctacaccagggccatgcggtcacccctgagggctctaatgttactaggcaaaggcctgagtctgagcaggacagggtggggcaagctccaacccaaagtctactctattatcaggagaagctccatgctatccagaggaccccgacacacaccccaagccaatttcccttcatccccaggaaagtgtgccaccaactgaggaggaaatgtatctgcttctcttcctagcactcccgtgaactcaaccaggaagatactgctgtttggctttaaaaatagtacattctagctggacttttatggtcttgtgaagaacactgtgctcatgccctcccacacctggcctctgcccctgcctggccctgtccagctgcccacatcagctctgcacaagctcttcagggtccctctgcagagacgtggttcaaggcagatttacgagttcagccttggccgaggccttctccccatggctcccatccacattccagctgttctcccacatcccaggcagctcggggctgggatgttctgtgtctctttttctacctctaccacaactggctcagtcgcacccccagccctatttcagctctgccctggccagccctgtggaggtacagggtcctgtcatgccagaacccagaccccaaccattcccagcctgcccagagctcacttacattcatgataacaacaatggtgtgtgtctaaggataaccttgttgggactctagttggtcatgcccgtcccctcccactctgaagggctgaaatttaaccgaaaggtaatttgttccatctggacttcaggtgccaggtttgaggctacatccgatctggaaagttattttcagtgtgtgtagattctatgattagtcctcaagttatttctttagggccagagatgagtttcaccgaagctatatcacatttctggcaccccatggtaggacttagagaaagcccccaaggacgatctccatgaggcggagccggccctagggagctaatagactatagaaataactccagagccagggaagcctcgaacacaaattttacaaggagccaattgagtggttgagcagttgaaggcaggcctatcttgtttttgcttgagggcaggtttctaacataatggaaagagaagactgtaatgatcaccccctatatacctgatcttctcttaaggtccttcaaggatgtaattgattctgtcaatatccttcatatttaaggccataagttgctgcttggttcaattaaggtagaattgcttctggttaagatctcaaactaggcatctgggactatctaaaagtttctctggaaactggaatgtaagcaatgcaagatgtatggcttaacctgtagatataactcatgtcaagaaaacagtggggttgggcatggtggctcatgcctgtaatcccagcactttaggaggctgaggtgggaggatcacttgaggccaggggttcgaggccagcctgggcaacatatcaagacccccatctctacataaaaagaagaagaaacgaaaagaaaagaaaagaaaagaaaagagtggaagagtgcaggagccgagagggagagaaaatgtagtggtgaggggcagcttctggaaaggcccatactacagagggaggaatcctgaattcctcactatctctctaacatcaggtaagcatctcatgatgcagttagaaagcacatttccttcttcagtttcccctctggctgtgtgacccagcccagatctgtttacacttggagctaccaggagcctatccggccacctggctttcccatcagcacctggggctggtgccatcccaggcccctccctctgcacctgcctttttgctatctgcagagggtttgtagaaaccttaggggaagaaagctagggtggttccctacctcaactttgagcccaattatacctctttctctcccacttcccagtagctgtcacagaagagccatggggaagtcccctcctggggaccaaggaggaggctctccaacctgtgcccctctaggtactgtccatcacagaagtgctactgcttctcttggtctgcatgctggaacttgggagctgagtctgagtcaagtctgatggctgagaatctgggggctggtagaaaatccaggcccataagcatgagtcacagtctaggagaaaagggcgagtgtgataattatttgtcaccaagagctggtgagagtggtgtggtggaaaggagagcatctgcctctccagggacttgggaccccacctctgcatctcttgttctttggctgggggtgctggctgtggtggagtcaagatcggagtaccccaggcctccagcatagagacgagatcgcatcggccacttcttgagagggtgcaagtagcggagtccacgcaggaagggcggccaggcagggccaggcaactcgtggccgagtgtgcgggtgaggtgggctatgtagctggcggcgagcaccagcacgtccaacttggagagcttggtgtcgggcggcacggcaggcagagcagcctgcaaggccaagaaggcctggcgcagcgtcctgacccggctccgctcccgcgcggcattctcaggactggcctcgctcctgccaagagccaggcccccagccctggtccctcgagggccaggggtagctctgctccatctctggttgctccagcttctttcttcccacgggtcctgccttgtcctgctgaggcggctcctcttcctgtcagcgcctggcagcaaccgtgctttggcctgagtctggctatgccccacccctggcatggctggtggccctctggccttcctctgtgacatgccaccccactggggctgcagcccacagagcagaaacacagtgcctgaggaggccttggactcaagctagctggctgtggctggtcatccagccagcaatatctacatccgaggaagctggcgccaactc

SEQ ID NO: 14978 - RNA, 358 nt, Homo sapiens
  source 1..358: mol_type = other RNA
gctgggattacaggcatgagccactgattccagcccaggcaataattttaaaacagtagttataaatataatcaatatcctccaaattaaatatgaatataatgaaaagccaaatggaactgagaatattgccccagaatgaccaacatcaagagatgttctgtgaataactagtgaaataactggaaaaaatatcctttggatatctcaggtccaatacccctttatttggagtgtgttcatgcatgagtggtctctcaaattctctgccaatctggagagtctctgtgttcttctgatttcacagcatgagaatgccttatgtcttccacatagagcaatgccagtgaaactgcaa

SEQ ID NO: 14979 - RNA, 5629 nt, Homo sapiens
  source 1..5629: mol_type = other RNA
gctgggattacaggcatgagccactgcaaccagccttaagtttttaaattgagatcaaattcacacagcataatattcacccttttaaagtgtatagttgagtgacctgtagtatataaacaaaattgtacaacctttacccatgccacattttcattaccccaaatgacacagttcttttaagtttacatatatagccatttcaatttctcatatacaatattgtttatttgtcatccttatttcacctctggaatcactaaactttgtctcattttttttctcttccatcaaatatcaattttggattcagatccagtttttttctttcaattatttctgccttttaaaataatactacctccttcctcccacaattcatttcagcttgttttagttccttgggttctatattttttcttcctagtattacaatatatgcacaaatattaggttataaaacttccaatacaacttttactgccactcacaggtttttcaattgttttcattttcatgtacatttaaataatgtatatattagggatttattccttaacccatgttaattaagagggaatattgaattaataatcagatatttgatggttatcctattgtactgcttcttctggtcaaataatgttgccagtatgttttctgcattttggggggaaatattagaaaaaattttataatctcttcctgcttttttgacagctgtgctttctactactcatcatattttcagggtttcagattggtaaccgtttattttttattttgtaagacagagtctcgctctgtcacccagtctggagtgtgcagtggtgcaatctcagctcactataacctccaactcccaggttcaagcaatcctcccacctcagcctcttgagtagctaggattacaggcatgcaacaccatgcctggctatttgtttttgtttttgttttttttgtatttttagtagagacggggtttcaccatgttggccaggctggtctcgagctcctgacctcaagtgatccacccaccttggcctcccaaagtgctaggattacaggtgtgagccaccgcgcccagcctcagactggtattctttatgtagcataaaagataaagtctgaacaaagactatgcacacatactttttctcttccttttaaaattccacactgaataataatgatagggaaaggcttcgttatactcattacaagtgtttctctttttccaccatgaattacaaatttgccaaaggtaaacaacatggttaaaatcctttccataaatcctaatgaagatacttatgataatgagtatatcactgataatagtggaaaacttttactaaacctgtattatgtgataacagtttgaggtactttgcatttattaattcattgactcttcacagcaatccaatacatacagccttattatagatgcctagacataattttttaaaataccactaacagccaggggcggtggctcacacctataatcccagcactttgggaagccaaggcaggaggatcacgaggtcaggagtttgagagcagcctggccaatatggtgaaaccccatctctactaataatacaaaaattagctaggcatggtggcgcgcgcctgtagtcccagctactcgggaggctgaggcggaagactcacttgaactcgggaggcagaggttgcagtgagccgagattgcaccactgccctccagcctgggcaacagagcgagactgtgtctcaaaaaacaaaaacaccactaatagctataagaaaaaataattgaccgggcacagtggctcacacctgtaatccccgaactttgggaggccgaggtgggtggatcacaaggtcaagagttcaagaccagcctggccaacatagtgaaaccctgtctctactaaaaatacaaaaattagccaggcatggtgtcgtgcgcctgtagtctcagatactaggaaggctgaggcaggagaatcgcttgaacccgggaggcagcagttgtggtgaactgagattgtgccactgcacttcagcctgggcaacagagtgaactccatctcaaaaaaaaaaaaaaacaaacaaacaaaaaattaatatctggattgataaataacactttcataacagtgttactttctagtatggcattgggattaggattgatgtaagggaacaaaacagctcacaaggagaaaatgtagataattttagcaattaaaataaatgttttaaaagtaaaaataagcatccaatgaggtcagcagtttttgtgtttttttgagacggaatctcactctgtcccccaggctggagtgcagtggcaccatctcagctcactgcaacctccgcctcccaggttcaagcaattctcctgtctcagcctcccgagtagctgggattacaggtacatgccaccacgcccagctaagtagagacggggtttcactgttagccaggatggccttaatcttcagaccttgtgatccgcccacctcggcctcccaaagtgctgggattacaggcatgagccactgtgcccagccgaggtcagcttttatagctgcaaaaatttagtggcaaccataatgggaatagtcattttaaagtcattaaatatgtcatgaaaataataaaaatctatatttactgaaatggcactcatgaaatctttggcatgataaaagcagttaagggtacagcatgcatatcataattacactttcttaaaaaagcaaagtatagcacgattttctctaccaaattgagagcagccatctataagtatgattacaattaattttggctttttagtttgtaattttttgctttgtgattttggcttaacaattaaaaatgtacatttgtaaaataaaaagaccggccgcagtggctcacgcctgtaatcccagcactttcggaggccgaggcgggtggatcacctgaagtcgggagattgagaccatcctggctaacatggtgaaaccccgtctctactaaaaatacaaaaaattagccgggtgttgtggcacatgcctgtaatcccaactactcaaaaggctgaggcagaagaaccacttgaacctgggaggcgaaggttgtgacgagccgagattgcaccattgcactccagcctaggcaacaagagcgaaactccgtctcaacaaaaaataaagccaggtgcaatcgctcatgcctgtaatcccagcactttgggaggctgaggcaggtggatcacctgaggtcaggagttcaagactatcctgaccaacatggagaaaccctgtctctactaaaaatagaaaattagcagggtgtggtggcacacgcctgtgatcccagctactcaggagtctgaggcaggagaattgcttgaagccgggaggtggaggttgcagcgagccgagattgcgccactgcactccagcctgggcaacagagtgaaactccgtctcaaaaaacatataataataataataaaataaaacaaaaagactaacactaacttcaaaaacaaagttaaacctccacaaggaatttaaaaatattaaaggtcacacaattcaaacagtgtgatactggtgcaaacacaaatacacagatcagaaaagatagctctaaaaacacaagcaaatataaacatgagtataatgtgtcaccaagaaagtagaacaaaacaatgaatgaaagaattatagaacagctggcatcggtatatgactgggggagagagggaatgtcactttagactccgaatttataacctggaatgaaatacatttggatacaaaatttaaatacaaagttttaaaaaaaactacggaagagggtaactattagacatgatttttggtttaaaatatgaggaaggtgacaggggctttaatttttattatttattagtatgaattccctgatgacgaatgagatccgagccactactaaaagccttcccacattccttacagttatagggcttttcaccagtgtgaattctcagatgtcgagtaaggtttgagcatttattaaaggcctttccacattcattacattcatatggtttttcatctgtatgaattctctgatgctggaaaagttgtgagttctgagtaaaggccttcccacattcaagacattcaaagggtttctcaccagcgtgaattctctgatgttgacgaagctgtgagctctgagtaaaagcctttccacattccttacaatcatagggtttctcaccagtgtgaattctctgatgattagtaagtgctgagccactactaaaggctttgccacattccttgcactcatagggtttctcaccagtatgaattctctgatgttgaacaagctttgagctctgggtaaaggctttgccacattccttacattcatagggtttctcacctgtatgaattcgtgcatgctgaaaaagttgtgagctcttagtaaaggctttcccacatactttacattcataaggtttttcaccagtgtgaattcgctgatggtcaataagatttgagcaataactaaaggccttcccacattccttacattcatagggtttcttaccggtatggattctctgatgttgagaaaggtatgagctacaactgaaggcctttccacattccttacattcaaagggtttttcgccagtatgaattttcagatgccgagtaacatgtgaaccacaactaaagaatttcccacactctttacattcataagatttttcaccaatatgaattctctgatgttgaataaattgtgagttctgactaaaggcctttccacatttcttacattcatagggtctgtcttcattattaattatttgatggagagtaaggaatgtctgttgaataaatgtgggcatgtattcaggagtgaatatttcttgactaaaatgcccatttggatatcccagttgttttgcaaggtggcttctatattccaaaacatctccaaaactggagtactcaaggccatgctttgtaagtcccattatctccctctggcataattctatttcataaacttccttctttagagataataacttggtttcacacatcgattccagatctgaacacaggcctcttgtaagctctctgccaaccatccagggctctttcccttgttccaataaggagatcacttgaggcttaggagtgtaaagtcccattgaaaccagattgccgtagttctccaacatcacatctctgtataagtccctctgaacagggtccaggcagtcccactcctcctgagagaagtctatggacacatcactgaacatcactgatccctcagccatggcttctagtattgcagatggttagtcttccttgaggccgttctcagaggtatctaaggtagtcaaactcatagaaacagaaagtagaacagtggctgccaggggctgtaatcccagctactcaggaggctgaggcaagagaatcgcttgaacccggaaagcagaggctgcagtgagctgagatcatgccactgcactccagcttgggcaacagagtgagactccgtctgcgggccccagccgagcctgcaagacccaggccgctcaccgcgcacttcccctaccctt

SEQ ID NO: 14980 - RNA, 5599 nt, Homo sapiens
  source 1..5599: mol_type = other RNA
gctgggattacaggcatgagccactgcaaccagccttaagtttttaaattgagatcaaattcacacagcataatattcacccttttaaagtgtatagttgagtgacctgtagtatataaacaaaattgtacaacctttacccatgccacattttcattaccccaaatgacacagttcttttaagtttacatatatagccatttcaatttctcatatacaatattgtttatttgtcatccttatttcacctctggaatcactaaactttgtctcattttttttctcttccatcaaatatcaattttggattcagatccagtttttttctttcaattatttctgccttttaaaataatactacctccttcctcccacaattcatttcagcttgttttagttccttgggttctatattttttcttcctagtattacaatatatgcacaaatattaggttataaaacttccaatacaacttttactgccactcacaggtttttcaattgttttcattttcatgtacatttaaataatgtatatattagggatttattccttaacccatgttaattaagagggaatattgaattaataatcagatatttgatggttatcctattgtactgcttcttctggtcaaataatgttgccagtatgttttctgcattttggggggaaatattagaaaaaattttataatctcttcctgcttttttgacagctgtgctttctactactcatcatattttcagggtttcagattggtaaccgtttattttttattttgtaagacagagtctcgctctgtcacccagtctggagtgtgcagtggtgcaatctcagctcactataacctccaactcccaggttcaagcaatcctcccacctcagcctcttgagtagctaggattacaggcatgcaacaccatgcctggctatttgtttttgtttttgttttttttgtatttttagtagagacggggtttcaccatgttggccaggctggtctcgagctcctgacctcaagtgatccacccaccttggcctcccaaagtgctaggattacaggtgtgagccaccgcgcccagcctcagactggtattctttatgtagcataaaagataaagtctgaacaaagactatgcacacatactttttctcttccttttaaaattccacactgaataataatgatagggaaaggcttcgttatactcattacaagtgtttctctttttccaccatgaattacaaatttgccaaaggtaaacaacatggttaaaatcctttccataaatcctaatgaagatacttatgataatgagtatatcactgataatagtggaaaacttttactaaacctgtattatgtgataacagtttgaggtactttgcatttattaattcattgactcttcacagcaatccaatacatacagccttattatagatgcctagacataattttttaaaataccactaacagccaggggcggtggctcacacctataatcccagcactttgggaagccaaggcaggaggatcacgaggtcaggagtttgagagcagcctggccaatatggtgaaaccccatctctactaataatacaaaaattagctaggcatggtggcgcgcgcctgtagtcccagctactcgggaggctgaggcggaagactcacttgaactcgggaggcagaggttgcagtgagccgagattgcaccactgccctccagcctgggcaacagagcgagactgtgtctcaaaaaacaaaaacaccactaatagctataagaaaaaataattgaccgggcacagtggctcacacctgtaatccccgaactttgggaggccgaggtgggtggatcacaaggtcaagagttcaagaccagcctggccaacatagtgaaaccctgtctctactaaaaatacaaaaattagccaggcatggtgtcgtgcgcctgtagtctcagatactaggaaggctgaggcaggagaatcgcttgaacccgggaggcagcagttgtggtgaactgagattgtgccactgcacttcagcctgggcaacagagtgaactccatctcaaaaaaaaaaaaaaacaaacaaacaaaaaattaatatctggattgataaataacactttcataacagtgttactttctagtatggcattgggattaggattgatgtaagggaacaaaacagctcacaaggagaaaatgtagataattttagcaattaaaataaatgttttaaaagtaaaaataagcatccaatgaggtcagcagtttttgtgtttttttgagacggaatctcactctgtcccccaggctggagtgcagtggcaccatctcagctcactgcaacctccgcctcccaggttcaagcaattctcctgtctcagcctcccgagtagctgggattacaggtacatgccaccacgcccagctaagtagagacggggtttcactgttagccaggatggccttaatcttcagaccttgtgatccgcccacctcggcctcccaaagtgctgggattacaggcatgagccactgtgcccagccgaggtcagcttttatagctgcaaaaatttagtggcaaccataatgggaatagtcattttaaagtcattaaatatgtcatgaaaataataaaaatctatatttactgaaatggcactcatgaaatctttggcatgataaaagcagttaagggtacagcatgcatatcataattacactttcttaaaaaagcaaagtatagcacgattttctctaccaaattgagagcagccatctataagtatgattacaattaattttggctttttagtttgtaattttttgctttgtgattttggcttaacaattaaaaatgtacatttgtaaaataaaaagaccggccgcagtggctcacgcctgtaatcccagcactttcggaggccgaggcgggtggatcacctgaagtcgggagattgagaccatcctggctaacatggtgaaaccccgtctctactaaaaatacaaaaaattagccgggtgttgtggcacatgcctgtaatcccaactactcaaaaggctgaggcagaagaaccacttgaacctgggaggcgaaggttgtgacgagccgagattgcaccattgcactccagcctaggcaacaagagcgaaactccgtctcaacaaaaaataaagccaggtgcaatcgctcatgcctgtaatcccagcactttgggaggctgaggcaggtggatcacctgaggtcaggagttcaagactatcctgaccaacatggagaaaccctgtctctactaaaaatagaaaattagcagggtgtggtggcacacgcctgtgatcccagctactcaggagtctgaggcaggagaattgcttgaagccgggaggtggaggttgcagcgagccgagattgcgccactgcactccagcctgggcaacagagtgaaactccgtctcaaaaaacatataataataataataaaataaaacaaaaagactaacactaacttcaaaaacaaagttaaacctccacaaggaatttaaaaatattaaaggtcacacaattcaaacagtgtgatactggtgcaaacacaaatacacagatcagaaaagatagctctaaaaacacaagcaaatataaacatgagtataatgtgtcaccaagaaagtagaacaaaacaatgaatgaaagaattatagaacagctggcatcggtatatgactgggggagagagggaatgtcactttagactccgaatttataacctggaatgaaatacatttggatacaaaatttaaatacaaagttttaaaaaaaactacggaagagggtaactattagacatgatttttggtttaaaatatgaggaaggtgacaggggctttaatttttattatttattagtatgaattccctgatgacgaatgagatccgagccactactaaaagccttcccacattccttacagttatagggcttttcaccagtgtgaattctcagatgtcgagtaaggtttgagcatttattaaaggcctttccacattcattacattcatatggtttttcatctgtatgaattctctgatgctggaaaagttgtgagttctgagtaaaggccttcccacattcaagacattcaaagggtttctcaccagcgtgaattctctgatgttgacgaagctgtgagctctgagtaaaagcctttccacattccttacaatcatagggtttctcaccagtgtgaattctctgatgattagtaagtgctgagccactactaaaggctttgccacattccttgcactcatagggtttctcaccagtatgaattctctgatgttgaacaagctttgagctctgggtaaaggctttgccacattccttacattcatagggtttctcacctgtatgaattcgtgcatgctgaaaaagttgtgagctcttagtaaaggctttcccacatactttacattcataaggtttttcaccagtgtgaattcgctgatggtcaataagatttgagcaataactaaaggccttcccacattccttacattcatagggtttcttaccggtatggattctctgatgttgagaaaggtatgagctacaactgaaggcctttccacattccttacattcaaagggtttttcgccagtatgaattttcagatgccgagtaacatgtgaaccacaactaaagaatttcccacactctttacattcataagatttttcaccaatatgaattctctgatgttgaataaattgtgagttctgactaaaggcctttccacatttcttacattcatagggtctgtcttcattattaattatttgatggagagtaaggaatgtctgttgaataaatgtgggcatgtattcaggagtgaatatttcttgactaaaatgcccatttggatatcccagttgttttgcaaggtggcttctatattccaaaacatctccaaaactggagtactcaaggccatgctttgtaagtcccattatctccctctggcataattctatttcataaacttccttctttagagataataacttggtttcacacatcgattccagatctgaacacaggcctcttgtaagctctctgccaaccatccagggctctttcccttgttccaataaggagatcacttgaggcttaggagtgtaaagtcccattgaaaccagattgccgtagttctccaacatcacatctctgtataagtccctctgaacagggtccaggcagtcccactcctcctgagagaagtctatggacacatcactgaacatcactgatccctcagccatggcttctagtattgcagatggttagtcttccttgaggccgttctcatgtctgttgaagtataaaaagggactcagtctcatgatcaacagcttaggaaacttaaatgcacattgctaagtgaaagaagccaattcaaaaagactacatactgtatgattacaacattctggaaaaggcaaaactatggagacaataaaaagattaggagttgacagggagggaggatcagtcagggcacagaggccttttagagcaat

SEQ ID NO: 14981 - RNA, 5799 nt, Homo sapiens
  source 1..5799: mol_type = other RNA
gctgggattacaggcatgagccactgcaaccagccttaagtttttaaattgagatcaaattcacacagcataatattcacccttttaaagtgtatagttgagtgacctgtagtatataaacaaaattgtacaacctttacccatgccacattttcattaccccaaatgacacagttcttttaagtttacatatatagccatttcaatttctcatatacaatattgtttatttgtcatccttatttcacctctggaatcactaaactttgtctcattttttttctcttccatcaaatatcaattttggattcagatccagtttttttctttcaattatttctgccttttaaaataatactacctccttcctcccacaattcatttcagcttgttttagttccttgggttctatattttttcttcctagtattacaatatatgcacaaatattaggttataaaacttccaatacaacttttactgccactcacaggtttttcaattgttttcattttcatgtacatttaaataatgtatatattagggatttattccttaacccatgttaattaagagggaatattgaattaataatcagatatttgatggttatcctattgtactgcttcttctggtcaaataatgttgccagtatgttttctgcattttggggggaaatattagaaaaaattttataatctcttcctgcttttttgacagctgtgctttctactactcatcatattttcagggtttcagattggtaaccgtttattttttattttgtaagacagagtctcgctctgtcacccagtctggagtgtgcagtggtgcaatctcagctcactataacctccaactcccaggttcaagcaatcctcccacctcagcctcttgagtagctaggattacaggcatgcaacaccatgcctggctatttgtttttgtttttgttttttttgtatttttagtagagacggggtttcaccatgttggccaggctggtctcgagctcctgacctcaagtgatccacccaccttggcctcccaaagtgctaggattacaggtgtgagccaccgcgcccagcctcagactggtattctttatgtagcataaaagataaagtctgaacaaagactatgcacacatactttttctcttccttttaaaattccacactgaataataatgatagggaaaggcttcgttatactcattacaagtgtttctctttttccaccatgaattacaaatttgccaaaggtaaacaacatggttaaaatcctttccataaatcctaatgaagatacttatgataatgagtatatcactgataatagtggaaaacttttactaaacctgtattatgtgataacagtttgaggtactttgcatttattaattcattgactcttcacagcaatccaatacatacagccttattatagatgcctagacataattttttaaaataccactaacagccaggggcggtggctcacacctataatcccagcactttgggaagccaaggcaggaggatcacgaggtcaggagtttgagagcagcctggccaatatggtgaaaccccatctctactaataatacaaaaattagctaggcatggtggcgcgcgcctgtagtcccagctactcgggaggctgaggcggaagactcacttgaactcgggaggcagaggttgcagtgagccgagattgcaccactgccctccagcctgggcaacagagcgagactgtgtctcaaaaaacaaaaacaccactaatagctataagaaaaaataattgaccgggcacagtggctcacacctgtaatccccgaactttgggaggccgaggtgggtggatcacaaggtcaagagttcaagaccagcctggccaacatagtgaaaccctgtctctactaaaaatacaaaaattagccaggcatggtgtcgtgcgcctgtagtctcagatactaggaaggctgaggcaggagaatcgcttgaacccgggaggcagcagttgtggtgaactgagattgtgccactgcacttcagcctgggcaacagagtgaactccatctcaaaaaaaaaaaaaaacaaacaaacaaaaaattaatatctggattgataaataacactttcataacagtgttactttctagtatggcattgggattaggattgatgtaagggaacaaaacagctcacaaggagaaaatgtagataattttagcaattaaaataaatgttttaaaagtaaaaataagcatccaatgaggtcagcagtttttgtgtttttttgagacggaatctcactctgtcccccaggctggagtgcagtggcaccatctcagctcactgcaacctccgcctcccaggttcaagcaattctcctgtctcagcctcccgagtagctgggattacaggtacatgccaccacgcccagctaagtagagacggggtttcactgttagccaggatggccttaatcttcagaccttgtgatccgcccacctcggcctcccaaagtgctgggattacaggcatgagccactgtgcccagccgaggtcagcttttatagctgcaaaaatttagtggcaaccataatgggaatagtcattttaaagtcattaaatatgtcatgaaaataataaaaatctatatttactgaaatggcactcatgaaatctttggcatgataaaagcagttaagggtacagcatgcatatcataattacactttcttaaaaaagcaaagtatagcacgattttctctaccaaattgagagcagccatctataagtatgattacaattaattttggctttttagtttgtaattttttgctttgtgattttggcttaacaattaaaaatgtacatttgtaaaataaaaagaccggccgcagtggctcacgcctgtaatcccagcactttcggaggccgaggcgggtggatcacctgaagtcgggagattgagaccatcctggctaacatggtgaaaccccgtctctactaaaaatacaaaaaattagccgggtgttgtggcacatgcctgtaatcccaactactcaaaaggctgaggcagaagaaccacttgaacctgggaggcgaaggttgtgacgagccgagattgcaccattgcactccagcctaggcaacaagagcgaaactccgtctcaacaaaaaataaagccaggtgcaatcgctcatgcctgtaatcccagcactttgggaggctgaggcaggtggatcacctgaggtcaggagttcaagactatcctgaccaacatggagaaaccctgtctctactaaaaatagaaaattagcagggtgtggtggcacacgcctgtgatcccagctactcaggagtctgaggcaggagaattgcttgaagccgggaggtggaggttgcagcgagccgagattgcgccactgcactccagcctgggcaacagagtgaaactccgtctcaaaaaacatataataataataataaaataaaacaaaaagactaacactaacttcaaaaacaaagttaaacctccacaaggaatttaaaaatattaaaggtcacacaattcaaacagtgtgatactggtgcaaacacaaatacacagatcagaaaagatagctctaaaaacacaagcaaatataaacatgagtataatgtgtcaccaagaaagtagaacaaaacaatgaatgaaagaattatagaacagctggcatcggtatatgactgggggagagagggaatgtcactttagactccgaatttataacctggaatgaaatacatttggatacaaaatttaaatacaaagttttaaaaaaaactacggaagagggtaactattagacatgatttttggtttaaaatatgaggaaggtgacaggggctttaatttttattatttattagtatgaattccctgatgacgaatgagatccgagccactactaaaagccttcccacattccttacagttatagggcttttcaccagtgtgaattctcagatgtcgagtaaggtttgagcatttattaaaggcctttccacattcattacattcatatggtttttcatctgtatgaattctctgatgctggaaaagttgtgagttctgagtaaaggccttcccacattcaagacattcaaagggtttctcaccagcgtgaattctctgatgttgacgaagctgtgagctctgagtaaaagcctttccacattccttacaatcatagggtttctcaccagtgtgaattctctgatgattagtaagtgctgagccactactaaaggctttgccacattccttgcactcatagggtttctcaccagtatgaattctctgatgttgaacaagctttgagctctgggtaaaggctttgccacattccttacattcatagggtttctcacctgtatgaattcgtgcatgctgaaaaagttgtgagctcttagtaaaggctttcccacatactttacattcataaggtttttcaccagtgtgaattcgctgatggtcaataagatttgagcaataactaaaggccttcccacattccttacattcatagggtttcttaccggtatggattctctgatgttgagaaaggtatgagctacaactgaaggcctttccacattccttacattcaaagggtttttcgccagtatgaattttcagatgccgagtaacatgtgaaccacaactaaagaatttcccacactctttacattcataagatttttcaccaatatgaattctctgatgttgaataaattgtgagttctgactaaaggcctttccacatttcttacattcatagggtctgtcttcattattaattatttgatggagagtaaggaatgtctgttgaataaatgtgggcatgtattcaggagtgaatatttcttgactaaaatgcccatttggatatcccagttgttttgcaaggtggcttctatattccaaaacatctccaaaactggagtactcaaggccatgctttgtaagtcccattatctccctctggcataattctatttcataaacttccttctttagagataataacttggtttcacacatcgattccagatctgaacacaggcctcttgtaagctctctgccaaccatccagggctctttcccttgttccaataaggagatcacttgaggcttaggagtgtaaagtcccattgaaaccagattgccgtagttctccaacatcacatctctgtataagtccctctgaacagggtccaggcagtcccactcctcctgagagaagtctatggacacatcactgaacatcactgatccctcagccatggcttctagtattgcagatggttagtcttccttgaggccgttctccgatcactggagatgactctcactccataccctgcccctttgccttatacacaataaataacagcgcgaccaggcattcggggccaataccggtctctgtgtcttggtgatagtggtccctcaggcccagctgtcttttcttctatctctgtcttgggtctttatttctacaatctctcgtctccacacacaaagagaaaatcccacaggccctgcagggctggtatcgcctgtaatcccagctactcaggaggctgaggcaagagaatcgcttgaacccggaaagcagaggctgcagtgagctgagatcatgccactgcactccagcttgggcaacagagtgagactccgtctgcgggccccagccgagcctgcaagacccaggccgctcaccgcgcacttcccctaccctt

SEQ ID NO: 14982 - RNA, 5587 nt, Homo sapiens
  source 1..5587: mol_type = other RNA
gctgggattacaggcatgagccactgcaaccagccttaagtttttaaattgagatcaaattcacacagcataatattcacccttttaaagtgtatagttgagtgacctgtagtatataaacaaaattgtacaacctttacccatgccacattttcattaccccaaatgacacagttcttttaagtttacatatatagccatttcaatttctcatatacaatattgtttatttgtcatccttatttcacctctggaatcactaaactttgtctcattttttttctcttccatcaaatatcaattttggattcagatccagtttttttctttcaattatttctgccttttaaaataatactacctccttcctcccacaattcatttcagcttgttttagttccttgggttctatattttttcttcctagtattacaatatatgcacaaatattaggttataaaacttccaatacaacttttactgccactcacaggtttttcaattgttttcattttcatgtacatttaaataatgtatatattagggatttattccttaacccatgttaattaagagggaatattgaattaataatcagatatttgatggttatcctattgtactgcttcttctggtcaaataatgttgccagtatgttttctgcattttggggggaaatattagaaaaaattttataatctcttcctgcttttttgacagctgtgctttctactactcatcatattttcagggtttcagattggtaaccgtttattttttattttgtaagacagagtctcgctctgtcacccagtctggagtgtgcagtggtgcaatctcagctcactataacctccaactcccaggttcaagcaatcctcccacctcagcctcttgagtagctaggattacaggcatgcaacaccatgcctggctatttgtttttgtttttgttttttttgtatttttagtagagacggggtttcaccatgttggccaggctggtctcgagctcctgacctcaagtgatccacccaccttggcctcccaaagtgctaggattacaggtgtgagccaccgcgcccagcctcagactggtattctttatgtagcataaaagataaagtctgaacaaagactatgcacacatactttttctcttccttttaaaattccacactgaataataatgatagggaaaggcttcgttatactcattacaagtgtttctctttttccaccatgaattacaaatttgccaaaggtaaacaacatggttaaaatcctttccataaatcctaatgaagatacttatgataatgagtatatcactgataatagtggaaaacttttactaaacctgtattatgtgataacagtttgaggtactttgcatttattaattcattgactcttcacagcaatccaatacatacagccttattatagatgcctagacataattttttaaaataccactaacagccaggggcggtggctcacacctataatcccagcactttgggaagccaaggcaggaggatcacgaggtcaggagtttgagagcagcctggccaatatggtgaaaccccatctctactaataatacaaaaattagctaggcatggtggcgcgcgcctgtagtcccagctactcgggaggctgaggcggaagactcacttgaactcgggaggcagaggttgcagtgagccgagattgcaccactgccctccagcctgggcaacagagcgagactgtgtctcaaaaaacaaaaacaccactaatagctataagaaaaaataattgaccgggcacagtggctcacacctgtaatccccgaactttgggaggccgaggtgggtggatcacaaggtcaagagttcaagaccagcctggccaacatagtgaaaccctgtctctactaaaaatacaaaaattagccaggcatggtgtcgtgcgcctgtagtctcagatactaggaaggctgaggcaggagaatcgcttgaacccgggaggcagcagttgtggtgaactgagattgtgccactgcacttcagcctgggcaacagagtgaactccatctcaaaaaaaaaaaaaaacaaacaaacaaaaaattaatatctggattgataaataacactttcataacagtgttactttctagtatggcattgggattaggattgatgtaagggaacaaaacagctcacaaggagaaaatgtagataattttagcaattaaaataaatgttttaaaagtaaaaataagcatccaatgaggtcagcagtttttgtgtttttttgagacggaatctcactctgtcccccaggctggagtgcagtggcaccatctcagctcactgcaacctccgcctcccaggttcaagcaattctcctgtctcagcctcccgagtagctgggattacaggtacatgccaccacgcccagctaagtagagacggggtttcactgttagccaggatggccttaatcttcagaccttgtgatccgcccacctcggcctcccaaagtgctgggattacaggcatgagccactgtgcccagccgaggtcagcttttatagctgcaaaaatttagtggcaaccataatgggaatagtcattttaaagtcattaaatatgtcatgaaaataataaaaatctatatttactgaaatggcactcatgaaatctttggcatgataaaagcagttaagggtacagcatgcatatcataattacactttcttaaaaaagcaaagtatagcacgattttctctaccaaattgagagcagccatctataagtatgattacaattaattttggctttttagtttgtaattttttgctttgtgattttggcttaacaattaaaaatgtacatttgtaaaataaaaagaccggccgcagtggctcacgcctgtaatcccagcactttcggaggccgaggcgggtggatcacctgaagtcgggagattgagaccatcctggctaacatggtgaaaccccgtctctactaaaaatacaaaaaattagccgggtgttgtggcacatgcctgtaatcccaactactcaaaaggctgaggcagaagaaccacttgaacctgggaggcgaaggttgtgacgagccgagattgcaccattgcactccagcctaggcaacaagagcgaaactccgtctcaacaaaaaataaagccaggtgcaatcgctcatgcctgtaatcccagcactttgggaggctgaggcaggtggatcacctgaggtcaggagttcaagactatcctgaccaacatggagaaaccctgtctctactaaaaatagaaaattagcagggtgtggtggcacacgcctgtgatcccagctactcaggagtctgaggcaggagaattgcttgaagccgggaggtggaggttgcagcgagccgagattgcgccactgcactccagcctgggcaacagagtgaaactccgtctcaaaaaacatataataataataataaaataaaacaaaaagactaacactaacttcaaaaacaaagttaaacctccacaaggaatttaaaaatattaaaggtcacacaattcaaacagtgtgatactggtgcaaacacaaatacacagatcagaaaagatagctctaaaaacacaagcaaatataaacatgagtataatgtgtcaccaagaaagtagaacaaaacaatgaatgaaagaattatagaacagctggcatcggtatatgactgggggagagagggaatgtcactttagactccgaatttataacctggaatgaaatacatttggatacaaaatttaaatacaaagttttaaaaaaaactacggaagagggtaactattagacatgatttttggtttaaaatatgaggaaggtgacaggggctttaatttttattatttattagtatgaattccctgatgacgaatgagatccgagccactactaaaagccttcccacattccttacagttatagggcttttcaccagtgtgaattctcagatgtcgagtaaggtttgagcatttattaaaggcctttccacattcattacattcatatggtttttcatctgtatgaattctctgatgctggaaaagttgtgagttctgagtaaaggccttcccacattcaagacattcaaagggtttctcaccagcgtgaattctctgatgttgacgaagctgtgagctctgagtaaaagcctttccacattccttacaatcatagggtttctcaccagtgtgaattctctgatgattagtaagtgctgagccactactaaaggctttgccacattccttgcactcatagggtttctcaccagtatgaattctctgatgttgaacaagctttgagctctgggtaaaggctttgccacattccttacattcatagggtttctcacctgtatgaattcgtgcatgctgaaaaagttgtgagctcttagtaaaggctttcccacatactttacattcataaggtttttcaccagtgtgaattcgctgatggtcaataagatttgagcaataactaaaggccttcccacattccttacattcatagggtttcttaccggtatggattctctgatgttgagaaaggtatgagctacaactgaaggcctttccacattccttacattcaaagggtttttcgccagtatgaattttcagatgccgagtaacatgtgaaccacaactaaagaatttcccacactctttacattcataagatttttcaccaatatgaattctctgatgttgaataaattgtgagttctgactaaaggcctttccacatttcttacattcatagggtctgtcttcattattaattatttgatggagagtaaggaatgtctgttgaataaatgtgggcatgtattcaggagtgaatatttcttgactaaaatgcccatttggatatcccagttgttttgcaaggtggcttctatattccaaaacatctccaaaactggagtactcaaggccatgctttgtaagtcccattatctccctctggcataattctatttcataaacttccttctttagagataataacttggtttcacacatcgattccagatctgaacacaggcctcttgtaagctctctgccaaccatccagggctctttcccttgttccaataaggagatcacttgaggcttaggagtgtaaagtcccattgaaaccagattgccgtagttctccaacatcacatctctgtataagtccctctgaacagggtccaggcagtcccactcctcctgagagaagtctatggacacatcactgaacatcactgatccctcagccatggcttctagtattgcagatggttagtcttccttgaggccgttctcctgaaaaaggacagtgttctgtaatcccagctactcaggaggctgaggcaagagaatcgcttgaacccggaaagcagaggctgcagtgagctgagatcatgccactgcactccagcttgggcaacagagtgagactccgtctgcgggccccagccgagcctgcaagacccaggccgctcaccgcgcacttcccctaccctt

SEQ ID NO: 14983 - RNA, 5447 nt, Homo sapiens
  source 1..5447: mol_type = other RNA
gctgggattacaggcatgagccactgcaaccagccttaagtttttaaattgagatcaaattcacacagcataatattcacccttttaaagtgtatagttgagtgacctgtagtatataaacaaaattgtacaacctttacccatgccacattttcattaccccaaatgacacagttcttttaagtttacatatatagccatttcaatttctcatatacaatattgtttatttgtcatccttatttcacctctggaatcactaaactttgtctcattttttttctcttccatcaaatatcaattttggattcagatccagtttttttctttcaattatttctgccttttaaaataatactacctccttcctcccacaattcatttcagcttgttttagttccttgggttctatattttttcttcctagtattacaatatatgcacaaatattaggttataaaacttccaatacaacttttactgccactcacaggtttttcaattgttttcattttcatgtacatttaaataatgtatatattagggatttattccttaacccatgttaattaagagggaatattgaattaataatcagatatttgatggttatcctattgtactgcttcttctggtcaaataatgttgccagtatgttttctgcattttggggggaaatattagaaaaaattttataatctcttcctgcttttttgacagctgtgctttctactactcatcatattttcagggtttcagattggtaaccgtttattttttattttgtaagacagagtctcgctctgtcacccagtctggagtgtgcagtggtgcaatctcagctcactataacctccaactcccaggttcaagcaatcctcccacctcagcctcttgagtagctaggattacaggcatgcaacaccatgcctggctatttgtttttgtttttgttttttttgtatttttagtagagacggggtttcaccatgttggccaggctggtctcgagctcctgacctcaagtgatccacccaccttggcctcccaaagtgctaggattacaggtgtgagccaccgcgcccagcctcagactggtattctttatgtagcataaaagataaagtctgaacaaagactatgcacacatactttttctcttccttttaaaattccacactgaataataatgatagggaaaggcttcgttatactcattacaagtgtttctctttttccaccatgaattacaaatttgccaaaggtaaacaacatggttaaaatcctttccataaatcctaatgaagatacttatgataatgagtatatcactgataatagtggaaaacttttactaaacctgtattatgtgataacagtttgaggtactttgcatttattaattcattgactcttcacagcaatccaatacatacagccttattatagatgcctagacataattttttaaaataccactaacagccaggggcggtggctcacacctataatcccagcactttgggaagccaaggcaggaggatcacgaggtcaggagtttgagagcagcctggccaatatggtgaaaccccatctctactaataatacaaaaattagctaggcatggtggcgcgcgcctgtagtcccagctactcgggaggctgaggcggaagactcacttgaactcgggaggcagaggttgcagtgagccgagattgcaccactgccctccagcctgggcaacagagcgagactgtgtctcaaaaaacaaaaacaccactaatagctataagaaaaaataattgaccgggcacagtggctcacacctgtaatccccgaactttgggaggccgaggtgggtggatcacaaggtcaagagttcaagaccagcctggccaacatagtgaaaccctgtctctactaaaaatacaaaaattagccaggcatggtgtcgtgcgcctgtagtctcagatactaggaaggctgaggcaggagaatcgcttgaacccgggaggcagcagttgtggtgaactgagattgtgccactgcacttcagcctgggcaacagagtgaactccatctcaaaaaaaaaaaaaaacaaacaaacaaaaaattaatatctggattgataaataacactttcataacagtgttactttctagtatggcattgggattaggattgatgtaagggaacaaaacagctcacaaggagaaaatgtagataattttagcaattaaaataaatgttttaaaagtaaaaataagcatccaatgaggtcagcagtttttgtgtttttttgagacggaatctcactctgtcccccaggctggagtgcagtggcaccatctcagctcactgcaacctccgcctcccaggttcaagcaattctcctgtctcagcctcccgagtagctgggattacaggtacatgccaccacgcccagctaagtagagacggggtttcactgttagccaggatggccttaatcttcagaccttgtgatccgcccacctcggcctcccaaagtgctgggattacaggcatgagccactgtgcccagccgaggtcagcttttatagctgcaaaaatttagtggcaaccataatgggaatagtcattttaaagtcattaaatatgtcatgaaaataataaaaatctatatttactgaaatggcactcatgaaatctttggcatgataaaagcagttaagggtacagcatgcatatcataattacactttcttaaaaaagcaaagtatagcacgattttctctaccaaattgagagcagccatctataagtatgattacaattaattttggctttttagtttgtaattttttgctttgtgattttggcttaacaattaaaaatgtacatttgtaaaataaaaagaccggccgcagtggctcacgcctgtaatcccagcactttcggaggccgaggcgggtggatcacctgaagtcgggagattgagaccatcctggctaacatggtgaaaccccgtctctactaaaaatacaaaaaattagccgggtgttgtggcacatgcctgtaatcccaactactcaaaaggctgaggcagaagaaccacttgaacctgggaggcgaaggttgtgacgagccgagattgcaccattgcactccagcctaggcaacaagagcgaaactccgtctcaacaaaaaataaagccaggtgcaatcgctcatgcctgtaatcccagcactttgggaggctgaggcaggtggatcacctgaggtcaggagttcaagactatcctgaccaacatggagaaaccctgtctctactaaaaatagaaaattagcagggtgtggtggcacacgcctgtgatcccagctactcaggagtctgaggcaggagaattgcttgaagccgggaggtggaggttgcagcgagccgagattgcgccactgcactccagcctgggcaacagagtgaaactccgtctcaaaaaacatataataataataataaaataaaacaaaaagactaacactaacttcaaaaacaaagttaaacctccacaaggaatttaaaaatattaaaggtcacacaattcaaacagtgtgatactggtgcaaacacaaatacacagatcagaaaagatagctctaaaaacacaagcaaatataaacatgagtataatgtgtcaccaagaaagtagaacaaaacaatgaatgaaagaattatagaacagctggcatcggtatatgactgggggagagagggaatgtcactttagactccgaatttataacctggaatgaaatacatttggatacaaaatttaaatacaaagttttaaaaaaaactacggaagagggtaactattagacatgatttttggtttaaaatatgaggaaggtgacaggggctttaatttttattatttattagtatgaattccctgatgacgaatgagatccgagccactactaaaagccttcccacattccttacagttatagggcttttcaccagtgtgaattctcagatgtcgagtaaggtttgagcatttattaaaggcctttccacattcattacattcatatggtttttcatctgtatgaattctctgatgctggaaaagttgtgagttctgagtaaaggccttcccacattcaagacattcaaagggtttctcaccagcgtgaattctctgatgttgacgaagctgtgagctctgagtaaaagcctttccacattccttacaatcatagggtttctcaccagtgtgaattctctgatgattagtaagtgctgagccactactaaaggctttgccacattccttgcactcatagggtttctcaccagtatgaattctctgatgttgaacaagctttgagctctgggtaaaggctttgccacattccttacattcatagggtttctcacctgtatgaattcgtgcatgctgaaaaagttgtgagctcttagtaaaggctttcccacatactttacattcataaggtttttcaccagtgtgaattcgctgatggtcaataagatttgagcaataactaaaggccttcccacattccttacattcatagggtttcttaccggtatggattctctgatgttgagaaaggtatgagctacaactgaaggcctttccacattccttacattcaaagggtttttcgccagtatgaattttcagatgccgagtaacatgtgaaccacaactaaagaatttcccacactctttacattcataagatttttcaccaatatgaattctctgatgttgaataaattgtgagttctgactaaaggcctttccacatttcttacattcatagggtctgtcttcattattaattatttgatggagagtaaggaatgtctgttgaataaatgtgggcatgtattcaggagtgaatatttcttgactaaaatgcccatttggatatcccagttgttttgcaaggtggcttctatattccaaaacatctccaaaactggagtactcaaggccatgctttgtaagtcccattatctccctctggcataattctatttcataaacttccttctttagagataataacttggtttcacacatcgattccagatctgaacacaggcctcttgtaagctctctgccaaccatccagggctctttcccttgttccaataaggagatcacttgaggcttaggagtgtaaagtcccattgaaaccagattgccgtagttctccaacatcacatctctgtataagtccctctgaacagggtccaggcagtcccactcctcctgagagaagtctatggacacatcactgaacatcactgatccctcagccatggcttctagtattgcagatggttagtcttccttgaggccgttctcctgcgggccccagccgagcctgcaagacccaggccgctcaccgcgcacttcccctaccctt

SEQ ID NO: 14984 - RNA, 5569 nt, Homo sapiens
  source 1..5569: mol_type = other RNA
gctgggattacaggcatgagccactgcaaccagccttaagtttttaaattgagatcaaattcacacagcataatattcacccttttaaagtgtatagttgagtgacctgtagtatataaacaaaattgtacaacctttacccatgccacattttcattaccccaaatgacacagttcttttaagtttacatatatagccatttcaatttctcatatacaatattgtttatttgtcatccttatttcacctctggaatcactaaactttgtctcattttttttctcttccatcaaatatcaattttggattcagatccagtttttttctttcaattatttctgccttttaaaataatactacctccttcctcccacaattcatttcagcttgttttagttccttgggttctatattttttcttcctagtattacaatatatgcacaaatattaggttataaaacttccaatacaacttttactgccactcacaggtttttcaattgttttcattttcatgtacatttaaataatgtatatattagggatttattccttaacccatgttaattaagagggaatattgaattaataatcagatatttgatggttatcctattgtactgcttcttctggtcaaataatgttgccagtatgttttctgcattttggggggaaatattagaaaaaattttataatctcttcctgcttttttgacagctgtgctttctactactcatcatattttcagggtttcagattggtaaccgtttattttttattttgtaagacagagtctcgctctgtcacccagtctggagtgtgcagtggtgcaatctcagctcactataacctccaactcccaggttcaagcaatcctcccacctcagcctcttgagtagctaggattacaggcatgcaacaccatgcctggctatttgtttttgtttttgttttttttgtatttttagtagagacggggtttcaccatgttggccaggctggtctcgagctcctgacctcaagtgatccacccaccttggcctcccaaagtgctaggattacaggtgtgagccaccgcgcccagcctcagactggtattctttatgtagcataaaagataaagtctgaacaaagactatgcacacatactttttctcttccttttaaaattccacactgaataataatgatagggaaaggcttcgttatactcattacaagtgtttctctttttccaccatgaattacaaatttgccaaaggtaaacaacatggttaaaatcctttccataaatcctaatgaagatacttatgataatgagtatatcactgataatagtggaaaacttttactaaacctgtattatgtgataacagtttgaggtactttgcatttattaattcattgactcttcacagcaatccaatacatacagccttattatagatgcctagacataattttttaaaataccactaacagccaggggcggtggctcacacctataatcccagcactttgggaagccaaggcaggaggatcacgaggtcaggagtttgagagcagcctggccaatatggtgaaaccccatctctactaataatacaaaaattagctaggcatggtggcgcgcgcctgtagtcccagctactcgggaggctgaggcggaagactcacttgaactcgggaggcagaggttgcagtgagccgagattgcaccactgccctccagcctgggcaacagagcgagactgtgtctcaaaaaacaaaaacaccactaatagctataagaaaaaataattgaccgggcacagtggctcacacctgtaatccccgaactttgggaggccgaggtgggtggatcacaaggtcaagagttcaagaccagcctggccaacatagtgaaaccctgtctctactaaaaatacaaaaattagccaggcatggtgtcgtgcgcctgtagtctcagatactaggaaggctgaggcaggagaatcgcttgaacccgggaggcagcagttgtggtgaactgagattgtgccactgcacttcagcctgggcaacagagtgaactccatctcaaaaaaaaaaaaaaacaaacaaacaaaaaattaatatctggattgataaataacactttcataacagtgttactttctagtatggcattgggattaggattgatgtaagggaacaaaacagctcacaaggagaaaatgtagataattttagcaattaaaataaatgttttaaaagtaaaaataagcatccaatgaggtcagcagtttttgtgtttttttgagacggaatctcactctgtcccccaggctggagtgcagtggcaccatctcagctcactgcaacctccgcctcccaggttcaagcaattctcctgtctcagcctcccgagtagctgggattacaggtacatgccaccacgcccagctaagtagagacggggtttcactgttagccaggatggccttaatcttcagaccttgtgatccgcccacctcggcctcccaaagtgctgggattacaggcatgagccactgtgcccagccgaggtcagcttttatagctgcaaaaatttagtggcaaccataatgggaatagtcattttaaagtcattaaatatgtcatgaaaataataaaaatctatatttactgaaatggcactcatgaaatctttggcatgataaaagcagttaagggtacagcatgcatatcataattacactttcttaaaaaagcaaagtatagcacgattttctctaccaaattgagagcagccatctataagtatgattacaattaattttggctttttagtttgtaattttttgctttgtgattttggcttaacaattaaaaatgtacatttgtaaaataaaaagaccggccgcagtggctcacgcctgtaatcccagcactttcggaggccgaggcgggtggatcacctgaagtcgggagattgagaccatcctggctaacatggtgaaaccccgtctctactaaaaatacaaaaaattagccgggtgttgtggcacatgcctgtaatcccaactactcaaaaggctgaggcagaagaaccacttgaacctgggaggcgaaggttgtgacgagccgagattgcaccattgcactccagcctaggcaacaagagcgaaactccgtctcaacaaaaaataaagccaggtgcaatcgctcatgcctgtaatcccagcactttgggaggctgaggcaggtggatcacctgaggtcaggagttcaagactatcctgaccaacatggagaaaccctgtctctactaaaaatagaaaattagcagggtgtggtggcacacgcctgtgatcccagctactcaggagtctgaggcaggagaattgcttgaagccgggaggtggaggttgcagcgagccgagattgcgccactgcactccagcctgggcaacagagtgaaactccgtctcaaaaaacatataataataataataaaataaaacaaaaagactaacactaacttcaaaaacaaagttaaacctccacaaggaatttaaaaatattaaaggtcacacaattcaaacagtgtgatactggtgcaaacacaaatacacagatcagaaaagatagctctaaaaacacaagcaaatataaacatgagtataatgtgtcaccaagaaagtagaacaaaacaatgaatgaaagaattatagaacagctggcatcggtatatgactgggggagagagggaatgtcactttagactccgaatttataacctggaatgaaatacatttggatacaaaatttaaatacaaagttttaaaaaaaactacggaagagggtaactattagacatgatttttggtttaaaatatgaggaaggtgacaggggctttaatttttattatttattagtatgaattccctgatgacgaatgagatccgagccactactaaaagccttcccacattccttacagttatagggcttttcaccagtgtgaattctcagatgtcgagtaaggtttgagcatttattaaaggcctttccacattcattacattcatatggtttttcatctgtatgaattctctgatgctggaaaagttgtgagttctgagtaaaggccttcccacattcaagacattcaaagggtttctcaccagcgtgaattctctgatgttgacgaagctgtgagctctgagtaaaagcctttccacattccttacaatcatagggtttctcaccagtgtgaattctctgatgattagtaagtgctgagccactactaaaggctttgccacattccttgcactcatagggtttctcaccagtatgaattctctgatgttgaacaagctttgagctctgggtaaaggctttgccacattccttacattcatagggtttctcacctgtatgaattcgtgcatgctgaaaaagttgtgagctcttagtaaaggctttcccacatactttacattcataaggtttttcaccagtgtgaattcgctgatggtcaataagatttgagcaataactaaaggccttcccacattccttacattcatagggtttcttaccggtatggattctctgatgttgagaaaggtatgagctacaactgaaggcctttccacattccttacattcaaagggtttttcgccagtatgaattttcagatgccgagtaacatgtgaaccacaactaaagaatttcccacactctttacattcataagatttttcaccaatatgaattctctgatgttgaataaattgtgagttctgactaaaggcctttccacatttcttacattcatagggtctgtcttcattattaattatttgatggagagtaaggaatgtctgttgaataaatgtgggcatgtattcaggagtgaatatttcttgactaaaatgcccatttggatatcccagttgttttgcaaggtggcttctatattccaaaacatctccaaaactggagtactcaaggccatgctttgtaagtcccattatctccctctggcataattctatttcataaacttccttctttagagataataacttggtttcacacatcgattccagatctgaacacaggcctcttgtaagctctctgccaaccatccagggctctttcccttgttccaataaggagatcacttgaggcttaggagtgtaaagtcccattgaaaccagattgccgtagttctccaacatcacatctctgtataagtccctctgaacagggtccaggcagtcccactcctcctgagagaagtctatggacacatcactgaacatcactgatccctcagccatggcttctagtattgcagatggttagtcttccttgaggccgttctcctgtaatcccagctactcaggaggctgaggcaagagaatcgcttgaacccggaaagcagaggctgcagtgagctgagatcatgccactgcactccagcttgggcaacagagtgagactccgtctgcgggccccagccgagcctgcaagacccaggccgctcaccgcgcacttcccctaccctt

SEQ ID NO: 14985 - RNA, 5794 nt, Homo sapiens
  source 1..5794: mol_type = other RNA
gctgggattacaggcatgagccactgcaaccagccttaagtttttaaattgagatcaaattcacacagcataatattcacccttttaaagtgtatagttgagtgacctgtagtatataaacaaaattgtacaacctttacccatgccacattttcattaccccaaatgacacagttcttttaagtttacatatatagccatttcaatttctcatatacaatattgtttatttgtcatccttatttcacctctggaatcactaaactttgtctcattttttttctcttccatcaaatatcaattttggattcagatccagtttttttctttcaattatttctgccttttaaaataatactacctccttcctcccacaattcatttcagcttgttttagttccttgggttctatattttttcttcctagtattacaatatatgcacaaatattaggttataaaacttccaatacaacttttactgccactcacaggtttttcaattgttttcattttcatgtacatttaaataatgtatatattagggatttattccttaacccatgttaattaagagggaatattgaattaataatcagatatttgatggttatcctattgtactgcttcttctggtcaaataatgttgccagtatgttttctgcattttggggggaaatattagaaaaaattttataatctcttcctgcttttttgacagctgtgctttctactactcatcatattttcagggtttcagattggtaaccgtttattttttattttgtaagacagagtctcgctctgtcacccagtctggagtgtgcagtggtgcaatctcagctcactataacctccaactcccaggttcaagcaatcctcccacctcagcctcttgagtagctaggattacaggcatgcaacaccatgcctggctatttgtttttgtttttgttttttttgtatttttagtagagacggggtttcaccatgttggccaggctggtctcgagctcctgacctcaagtgatccacccaccttggcctcccaaagtgctaggattacaggtgtgagccaccgcgcccagcctcagactggtattctttatgtagcataaaagataaagtctgaacaaagactatgcacacatactttttctcttccttttaaaattccacactgaataataatgatagggaaaggcttcgttatactcattacaagtgtttctctttttccaccatgaattacaaatttgccaaaggtaaacaacatggttaaaatcctttccataaatcctaatgaagatacttatgataatgagtatatcactgataatagtggaaaacttttactaaacctgtattatgtgataacagtttgaggtactttgcatttattaattcattgactcttcacagcaatccaatacatacagccttattatagatgcctagacataattttttaaaataccactaacagccaggggcggtggctcacacctataatcccagcactttgggaagccaaggcaggaggatcacgaggtcaggagtttgagagcagcctggccaatatggtgaaaccccatctctactaataatacaaaaattagctaggcatggtggcgcgcgcctgtagtcccagctactcgggaggctgaggcggaagactcacttgaactcgggaggcagaggttgcagtgagccgagattgcaccactgccctccagcctgggcaacagagcgagactgtgtctcaaaaaacaaaaacaccactaatagctataagaaaaaataattgaccgggcacagtggctcacacctgtaatccccgaactttgggaggccgaggtgggtggatcacaaggtcaagagttcaagaccagcctggccaacatagtgaaaccctgtctctactaaaaatacaaaaattagccaggcatggtgtcgtgcgcctgtagtctcagatactaggaaggctgaggcaggagaatcgcttgaacccgggaggcagcagttgtggtgaactgagattgtgccactgcacttcagcctgggcaacagagtgaactccatctcaaaaaaaaaaaaaaacaaacaaacaaaaaattaatatctggattgataaataacactttcataacagtgttactttctagtatggcattgggattaggattgatgtaagggaacaaaacagctcacaaggagaaaatgtagataattttagcaattaaaataaatgttttaaaagtaaaaataagcatccaatgaggtcagcagtttttgtgtttttttgagacggaatctcactctgtcccccaggctggagtgcagtggcaccatctcagctcactgcaacctccgcctcccaggttcaagcaattctcctgtctcagcctcccgagtagctgggattacaggtacatgccaccacgcccagctaagtagagacggggtttcactgttagccaggatggccttaatcttcagaccttgtgatccgcccacctcggcctcccaaagtgctgggattacaggcatgagccactgtgcccagccgaggtcagcttttatagctgcaaaaatttagtggcaaccataatgggaatagtcattttaaagtcattaaatatgtcatgaaaataataaaaatctatatttactgaaatggcactcatgaaatctttggcatgataaaagcagttaagggtacagcatgcatatcataattacactttcttaaaaaagcaaagtatagcacgattttctctaccaaattgagagcagccatctataagtatgattacaattaattttggctttttagtttgtaattttttgctttgtgattttggcttaacaattaaaaatgtacatttgtaaaataaaaagaccggccgcagtggctcacgcctgtaatcccagcactttcggaggccgaggcgggtggatcacctgaagtcgggagattgagaccatcctggctaacatggtgaaaccccgtctctactaaaaatacaaaaaattagccgggtgttgtggcacatgcctgtaatcccaactactcaaaaggctgaggcagaagaaccacttgaacctgggaggcgaaggttgtgacgagccgagattgcaccattgcactccagcctaggcaacaagagcgaaactccgtctcaacaaaaaataaagccaggtgcaatcgctcatgcctgtaatcccagcactttgggaggctgaggcaggtggatcacctgaggtcaggagttcaagactatcctgaccaacatggagaaaccctgtctctactaaaaatagaaaattagcagggtgtggtggcacacgcctgtgatcccagctactcaggagtctgaggcaggagaattgcttgaagccgggaggtggaggttgcagcgagccgagattgcgccactgcactccagcctgggcaacagagtgaaactccgtctcaaaaaacatataataataataataaaataaaacaaaaagactaacactaacttcaaaaacaaagttaaacctccacaaggaatttaaaaatattaaaggtcacacaattcaaacagtgtgatactggtgcaaacacaaatacacagatcagaaaagatagctctaaaaacacaagcaaatataaacatgagtataatgtgtcaccaagaaagtagaacaaaacaatgaatgaaagaattatagaacagctggcatcggtatatgactgggggagagagggaatgtcactttagactccgaatttataacctggaatgaaatacatttggatacaaaatttaaatacaaagttttaaaaaaaactacggaagagggtaactattagacatgatttttggtttaaaatatgaggaaggtgacaggggctttaatttttattatttattagtatgaattccctgatgacgaatgagatccgagccactactaaaagccttcccacattccttacagttatagggcttttcaccagtgtgaattctcagatgtcgagtaaggtttgagcatttattaaaggcctttccacattcattacattcatatggtttttcatctgtatgaattctctgatgctggaaaagttgtgagttctgagtaaaggccttcccacattcaagacattcaaagggtttctcaccagcgtgaattctctgatgttgacgaagctgtgagctctgagtaaaagcctttccacattccttacaatcatagggtttctcaccagtgtgaattctctgatgattagtaagtgctgagccactactaaaggctttgccacattccttgcactcatagggtttctcaccagtatgaattctctgatgttgaacaagctttgagctctgggtaaaggctttgccacattccttacattcatagggtttctcacctgtatgaattcgtgcatgctgaaaaagttgtgagctcttagtaaaggctttcccacatactttacattcataaggtttttcaccagtgtgaattcgctgatggtcaataagatttgagcaataactaaaggccttcccacattccttacattcatagggtttcttaccggtatggattctctgatgttgagaaaggtatgagctacaactgaaggcctttccacattccttacattcaaagggtttttcgccagtatgaattttcagatgccgagtaacatgtgaaccacaactaaagaatttcccacactctttacattcataagatttttcaccaatatgaattctctgatgttgaataaattgtgagttctgactaaaggcctttccacatttcttacattcatagggtctgtcttcattattaattatttgatggagagtaaggaatgtctgttgaataaatgtgggcatgtattcaggagtgaatatttcttgactaaaatgcccatttggatatcccagttgttttgcaaggtggcttctatattccaaaacatctccaaaactggagtactcaaggccatgctttgtaagtcccattatctccctctggcataattctatttcataaacttccttctttagagataataacttggtttcacacatcgattccagatctgaacacaggcctcttgtaagctctctgccaaccatccagggctctttcccttgttccaataaggagatcacttgaggcttaggagtgtaaagtcccattgaaaccagattgccgtagttctccaacatcacatctctgtataagtccctctgaacagggtccaggcagtcccactcctcctgagagaagtctatggacacatcactgaacatcactgatccctcagccatggcttctagtattgcagatggttagtcttccttgaggccgttctcctgtaatcccagctactcaggaggctgaggcaagagaatcgcttgaacccggaaagcagaggctgcagtgagctgagatcatgccactgcactccagcttgggcaacagagtgagactccgtcttgtatttggtttggtcaacagccattcttcctctgggtaactctcttgacgagagcagagctgaagaagaaaggaatgatgagatgccaggcctttcttgtggcccagactgagcagatcagaggtcattttggatctacagctactatatgcccgacacactcatacatgcccaacactccagaccagcctggtcagtcccttcaaactcccatgcacgtacctgcgggccccagccgagcctgcaagacccaggccgctcaccgcgcacttcccctaccctt

SEQ ID NO: 14986 - RNA, 5990 nt, Homo sapiens
  source 1..5990: mol_type = other RNA
gctgggattacaggcatgagccactgcaaccagccttaagtttttaaattgagatcaaattcacacagcataatattcacccttttaaagtgtatagttgagtgacctgtagtatataaacaaaattgtacaacctttacccatgccacattttcattaccccaaatgacacagttcttttaagtttacatatatagccatttcaatttctcatatacaatattgtttatttgtcatccttatttcacctctggaatcactaaactttgtctcattttttttctcttccatcaaatatcaattttggattcagatccagtttttttctttcaattatttctgccttttaaaataatactacctccttcctcccacaattcatttcagcttgttttagttccttgggttctatattttttcttcctagtattacaatatatgcacaaatattaggttataaaacttccaatacaacttttactgccactcacaggtttttcaattgttttcattttcatgtacatttaaataatgtatatattagggatttattccttaacccatgttaattaagagggaatattgaattaataatcagatatttgatggttatcctattgtactgcttcttctggtcaaataatgttgccagtatgttttctgcattttggggggaaatattagaaaaaattttataatctcttcctgcttttttgacagctgtgctttctactactcatcatattttcagggtttcagattggtaaccgtttattttttattttgtaagacagagtctcgctctgtcacccagtctggagtgtgcagtggtgcaatctcagctcactataacctccaactcccaggttcaagcaatcctcccacctcagcctcttgagtagctaggattacaggcatgcaacaccatgcctggctatttgtttttgtttttgttttttttgtatttttagtagagacggggtttcaccatgttggccaggctggtctcgagctcctgacctcaagtgatccacccaccttggcctcccaaagtgctaggattacaggtgtgagccaccgcgcccagcctcagactggtattctttatgtagcataaaagataaagtctgaacaaagactatgcacacatactttttctcttccttttaaaattccacactgaataataatgatagggaaaggcttcgttatactcattacaagtgtttctctttttccaccatgaattacaaatttgccaaaggtaaacaacatggttaaaatcctttccataaatcctaatgaagatacttatgataatgagtatatcactgataatagtggaaaacttttactaaacctgtattatgtgataacagtttgaggtactttgcatttattaattcattgactcttcacagcaatccaatacatacagccttattatagatgcctagacataattttttaaaataccactaacagccaggggcggtggctcacacctataatcccagcactttgggaagccaaggcaggaggatcacgaggtcaggagtttgagagcagcctggccaatatggtgaaaccccatctctactaataatacaaaaattagctaggcatggtggcgcgcgcctgtagtcccagctactcgggaggctgaggcggaagactcacttgaactcgggaggcagaggttgcagtgagccgagattgcaccactgccctccagcctgggcaacagagcgagactgtgtctcaaaaaacaaaaacaccactaatagctataagaaaaaataattgaccgggcacagtggctcacacctgtaatccccgaactttgggaggccgaggtgggtggatcacaaggtcaagagttcaagaccagcctggccaacatagtgaaaccctgtctctactaaaaatacaaaaattagccaggcatggtgtcgtgcgcctgtagtctcagatactaggaaggctgaggcaggagaatcgcttgaacccgggaggcagcagttgtggtgaactgagattgtgccactgcacttcagcctgggcaacagagtgaactccatctcaaaaaaaaaaaaaaacaaacaaacaaaaaattaatatctggattgataaataacactttcataacagtgttactttctagtatggcattgggattaggattgatgtaagggaacaaaacagctcacaaggagaaaatgtagataattttagcaattaaaataaatgttttaaaagtaaaaataagcatccaatgaggtcagcagtttttgtgtttttttgagacggaatctcactctgtcccccaggctggagtgcagtggcaccatctcagctcactgcaacctccgcctcccaggttcaagcaattctcctgtctcagcctcccgagtagctgggattacaggtacatgccaccacgcccagctaagtagagacggggtttcactgttagccaggatggccttaatcttcagaccttgtgatccgcccacctcggcctcccaaagtgctgggattacaggcatgagccactgtgcccagccgaggtcagcttttatagctgcaaaaatttagtggcaaccataatgggaatagtcattttaaagtcattaaatatgtcatgaaaataataaaaatctatatttactgaaatggcactcatgaaatctttggcatgataaaagcagttaagggtacagcatgcatatcataattacactttcttaaaaaagcaaagtatagcacgattttctctaccaaattgagagcagccatctataagtatgattacaattaattttggctttttagtttgtaattttttgctttgtgattttggcttaacaattaaaaatgtacatttgtaaaataaaaagaccggccgcagtggctcacgcctgtaatcccagcactttcggaggccgaggcgggtggatcacctgaagtcgggagattgagaccatcctggctaacatggtgaaaccccgtctctactaaaaatacaaaaaattagccgggtgttgtggcacatgcctgtaatcccaactactcaaaaggctgaggcagaagaaccacttgaacctgggaggcgaaggttgtgacgagccgagattgcaccattgcactccagcctaggcaacaagagcgaaactccgtctcaacaaaaaataaagccaggtgcaatcgctcatgcctgtaatcccagcactttgggaggctgaggcaggtggatcacctgaggtcaggagttcaagactatcctgaccaacatggagaaaccctgtctctactaaaaatagaaaattagcagggtgtggtggcacacgcctgtgatcccagctactcaggagtctgaggcaggagaattgcttgaagccgggaggtggaggttgcagcgagccgagattgcgccactgcactccagcctgggcaacagagtgaaactccgtctcaaaaaacatataataataataataaaataaaacaaaaagactaacactaacttcaaaaacaaagttaaacctccacaaggaatttaaaaatattaaaggtcacacaattcaaacagtgtgatactggtgcaaacacaaatacacagatcagaaaagatagctctaaaaacacaagcaaatataaacatgagtataatgtgtcaccaagaaagtagaacaaaacaatgaatgaaagaattatagaacagctggcatcggtatatgactgggggagagagggaatgtcactttagactccgaatttataacctggaatgaaatacatttggatacaaaatttaaatacaaagttttaaaaaaaactacggaagagggtaactattagacatgatttttggtttaaaatatgaggaaggtgacaggggctttaatttttattatttattagtatgaattccctgatgacgaatgagatccgagccactactaaaagccttcccacattccttacagttatagggcttttcaccagtgtgaattctcagatgtcgagtaaggtttgagcatttattaaaggcctttccacattcattacattcatatggtttttcatctgtatgaattctctgatgctggaaaagttgtgagttctgagtaaaggccttcccacattcaagacattcaaagggtttctcaccagcgtgaattctctgatgttgacgaagctgtgagctctgagtaaaagcctttccacattccttacaatcatagggtttctcaccagtgtgaattctctgatgattagtaagtgctgagccactactaaaggctttgccacattccttgcactcatagggtttctcaccagtatgaattctctgatgttgaacaagctttgagctctgggtaaaggctttgccacattccttacattcatagggtttctcacctgtatgaattcgtgcatgctgaaaaagttgtgagctcttagtaaaggctttcccacatactttacattcataaggtttttcaccagtgtgaattcgctgatggtcaataagatttgagcaataactaaaggccttcccacattccttacattcatagggtttcttaccggtatggattctctgatgttgagaaaggtatgagctacaactgaaggcctttccacattccttacattcaaagggtttttcgccagtatgaattttcagatgccgagtaacatgtgaaccacaactaaagaatttcccacactctttacattcataagatttttcaccaatatgaattctctgatgttgaataaattgtgagttctgactaaaggcctttccacatttcttacattcatagggtctgtcttcattattaattatttgatggagagtaaggaatgtctgttgaataaatgtgggcatgtattcaggagtgaatatttcttgactaaaatgcccatttggatatcccagttgttttgcaaggtggcttctatattccaaaacatctccaaaactggagtactcaaggccatgctttgtaagtcccattatctccctctggcataattctatttcataaacttccttctttagagataataacttggtttcacacatcgattccagatctgaacacaggcctcttgtaagctctctgccaaccatccagggctctttcccttgttccaataaggagatcacttgaggcttaggagtgtaaagtcccattgaaaccagattgccgtagttctccaacatcacatctctgtataagtccctctgaacagggtccaggcagtcccactcctcctgagagaagtctatggacacatcactgaacatcactgatccctcagccatggcttctagtattgcagatggttagtcttccttgaggccgttctcctgtaatcccagctactcaggaggctgaggcaagagaatcgcttgaacccggaaagcagaggctgcagtgagctgagatcatgccactgcactccagcttgggcaacagagtgagactccgtcttgtatttggtttggtcaacagccattcttcctctgggtaactctcttgacgagagcagagctgaagaagaaaggaatgatgagatgccaggcctttcttgtggcccagactgagcagatcagaggtcattttggatctacagctactatctgaggtggggaggtcgagaccagcctgaccaacacggagaaaccccgtctctactgaaaatacaaaattagcagggcgtggtgacacacgcctgtaatcccagctactaggaaggctgaggcaggagaattgcttgaaccggggaggcggaggttgcggtgagccgagattgcgccattgcactccagcctgggcaacaacagcgaaactccgcatgcccaacactccagaccagcctggtcagtcccttcaaactcccatgcacgtacctgcgggccccagccgagcctgcaagacccaggccgctcaccgcgcacttcccctaccctt

SEQ ID NO: 14987 - RNA, 5986 nt, Homo sapiens
  source 1..5986: mol_type = other RNA
gctgggattacaggcatgagccactgcaaccagccttaagtttttaaattgagatcaaattcacacagcataatattcacccttttaaagtgtatagttgagtgacctgtagtatataaacaaaattgtacaacctttacccatgccacattttcattaccccaaatgacacagttcttttaagtttacatatatagccatttcaatttctcatatacaatattgtttatttgtcatccttatttcacctctggaatcactaaactttgtctcattttttttctcttccatcaaatatcaattttggattcagatccagtttttttctttcaattatttctgccttttaaaataatactacctccttcctcccacaattcatttcagcttgttttagttccttgggttctatattttttcttcctagtattacaatatatgcacaaatattaggttataaaacttccaatacaacttttactgccactcacaggtttttcaattgttttcattttcatgtacatttaaataatgtatatattagggatttattccttaacccatgttaattaagagggaatattgaattaataatcagatatttgatggttatcctattgtactgcttcttctggtcaaataatgttgccagtatgttttctgcattttggggggaaatattagaaaaaattttataatctcttcctgcttttttgacagctgtgctttctactactcatcatattttcagggtttcagattggtaaccgtttattttttattttgtaagacagagtctcgctctgtcacccagtctggagtgtgcagtggtgcaatctcagctcactataacctccaactcccaggttcaagcaatcctcccacctcagcctcttgagtagctaggattacaggcatgcaacaccatgcctggctatttgtttttgtttttgttttttttgtatttttagtagagacggggtttcaccatgttggccaggctggtctcgagctcctgacctcaagtgatccacccaccttggcctcccaaagtgctaggattacaggtgtgagccaccgcgcccagcctcagactggtattctttatgtagcataaaagataaagtctgaacaaagactatgcacacatactttttctcttccttttaaaattccacactgaataataatgatagggaaaggcttcgttatactcattacaagtgtttctctttttccaccatgaattacaaatttgccaaaggtaaacaacatggttaaaatcctttccataaatcctaatgaagatacttatgataatgagtatatcactgataatagtggaaaacttttactaaacctgtattatgtgataacagtttgaggtactttgcatttattaattcattgactcttcacagcaatccaatacatacagccttattatagatgcctagacataattttttaaaataccactaacagccaggggcggtggctcacacctataatcccagcactttgggaagccaaggcaggaggatcacgaggtcaggagtttgagagcagcctggccaatatggtgaaaccccatctctactaataatacaaaaattagctaggcatggtggcgcgcgcctgtagtcccagctactcgggaggctgaggcggaagactcacttgaactcgggaggcagaggttgcagtgagccgagattgcaccactgccctccagcctgggcaacagagcgagactgtgtctcaaaaaacaaaaacaccactaatagctataagaaaaaataattgaccgggcacagtggctcacacctgtaatccccgaactttgggaggccgaggtgggtggatcacaaggtcaagagttcaagaccagcctggccaacatagtgaaaccctgtctctactaaaaatacaaaaattagccaggcatggtgtcgtgcgcctgtagtctcagatactaggaaggctgaggcaggagaatcgcttgaacccgggaggcagcagttgtggtgaactgagattgtgccactgcacttcagcctgggcaacagagtgaactccatctcaaaaaaaaaaaaaaacaaacaaacaaaaaattaatatctggattgataaataacactttcataacagtgttactttctagtatggcattgggattaggattgatgtaagggaacaaaacagctcacaaggagaaaatgtagataattttagcaattaaaataaatgttttaaaagtaaaaataagcatccaatgaggtcagcagtttttgtgtttttttgagacggaatctcactctgtcccccaggctggagtgcagtggcaccatctcagctcactgcaacctccgcctcccaggttcaagcaattctcctgtctcagcctcccgagtagctgggattacaggtacatgccaccacgcccagctaagtagagacggggtttcactgttagccaggatggccttaatcttcagaccttgtgatccgcccacctcggcctcccaaagtgctgggattacaggcatgagccactgtgcccagccgaggtcagcttttatagctgcaaaaatttagtggcaaccataatgggaatagtcattttaaagtcattaaatatgtcatgaaaataataaaaatctatatttactgaaatggcactcatgaaatctttggcatgataaaagcagttaagggtacagcatgcatatcataattacactttcttaaaaaagcaaagtatagcacgattttctctaccaaattgagagcagccatctataagtatgattacaattaattttggctttttagtttgtaattttttgctttgtgattttggcttaacaattaaaaatgtacatttgtaaaataaaaagaccggccgcagtggctcacgcctgtaatcccagcactttcggaggccgaggcgggtggatcacctgaagtcgggagattgagaccatcctggctaacatggtgaaaccccgtctctactaaaaatacaaaaaattagccgggtgttgtggcacatgcctgtaatcccaactactcaaaaggctgaggcagaagaaccacttgaacctgggaggcgaaggttgtgacgagccgagattgcaccattgcactccagcctaggcaacaagagcgaaactccgtctcaacaaaaaataaagccaggtgcaatcgctcatgcctgtaatcccagcactttgggaggctgaggcaggtggatcacctgaggtcaggagttcaagactatcctgaccaacatggagaaaccctgtctctactaaaaatagaaaattagcagggtgtggtggcacacgcctgtgatcccagctactcaggagtctgaggcaggagaattgcttgaagccgggaggtggaggttgcagcgagccgagattgcgccactgcactccagcctgggcaacagagtgaaactccgtctcaaaaaacatataataataataataaaataaaacaaaaagactaacactaacttcaaaaacaaagttaaacctccacaaggaatttaaaaatattaaaggtcacacaattcaaacagtgtgatactggtgcaaacacaaatacacagatcagaaaagatagctctaaaaacacaagcaaatataaacatgagtataatgtgtcaccaagaaagtagaacaaaacaatgaatgaaagaattatagaacagctggcatcggtatatgactgggggagagagggaatgtcactttagactccgaatttataacctggaatgaaatacatttggatacaaaatttaaatacaaagttttaaaaaaaactacggaagagggtaactattagacatgatttttggtttaaaatatgaggaaggtgacaggggctttaatttttattatttattagtatgaattccctgatgacgaatgagatccgagccactactaaaagccttcccacattccttacagttatagggcttttcaccagtgtgaattctcagatgtcgagtaaggtttgagcatttattaaaggcctttccacattcattacattcatatggtttttcatctgtatgaattctctgatgctggaaaagttgtgagttctgagtaaaggccttcccacattcaagacattcaaagggtttctcaccagcgtgaattctctgatgttgacgaagctgtgagctctgagtaaaagcctttccacattccttacaatcatagggtttctcaccagtgtgaattctctgatgattagtaagtgctgagccactactaaaggctttgccacattccttgcactcatagggtttctcaccagtatgaattctctgatgttgaacaagctttgagctctgggtaaaggctttgccacattccttacattcatagggtttctcacctgtatgaattcgtgcatgctgaaaaagttgtgagctcttagtaaaggctttcccacatactttacattcataaggtttttcaccagtgtgaattcgctgatggtcaataagatttgagcaataactaaaggccttcccacattccttacattcatagggtttcttaccggtatggattctctgatgttgagaaaggtatgagctacaactgaaggcctttccacattccttacattcaaagggtttttcgccagtatgaattttcagatgccgagtaacatgtgaaccacaactaaagaatttcccacactctttacattcataagatttttcaccaatatgaattctctgatgttgaataaattgtgagttctgactaaaggcctttccacatttcttacattcatagggtctgtcttcattattaattatttgatggagagtaaggaatgtctgttgaataaatgtgggcatgtattcaggagtgaatatttcttgactaaaatgcccatttggatatcccagttgttttgcaaggtggcttctatattccaaaacatctccaaaactggagtactcaaggccatgctttgtaagtcccattatctccctctggcataattctatttcataaacttccttctttagagataataacttggtttcacacatcgattccagatctgaacacaggcctcttgtaagctctctgccaaccatccagggctctttcccttgttccaataaggagatcacttgaggcttaggagtgtaaagtcccattgaaaccagattgccgtagttctccaacatcacatctctgtataagtccctctgaacagggtccaggcagtcccactcctcctgagagaagtctatggacacatcactgaacatcactgatccctcagccatggcttctagtattgcagatggttagtcttccttgaggccgttctcctgtaatcccagctactcaggaggctgaggcaagagaatcgcttgaacccggaaagcagaggctgcagtgagctgagatcatgccactgcactccagcttgggcaacagagtgagactccgtcttgtatttggtttggtcaacagccattcttcctctgggtaactctcttgacgagagcagagctgaagaagaaaggaatgatgagatgccaggcctttcttgtggcccagactgagcagatcagaggtcattttggatctacagctactatctgaggtggggaggtcgagaccagcctgaccaacacggagaaaccccgtctctactgaaaatacaaaattagcagggcgtggtgacacacgcctgtaatcccagctactaggaaggctgaggcaggagaattgcttgaaccggggaggcggaggttgcggtgagccgagattgcgccattgcactccagcctgggcaacaacagcgaaactccgcccaacactccagaccagcctggtcagtcccttcaaactcccatgcacgtacctgcgggccccagccgagcctgcaagacccaggccgctcaccgcgcacttcccctaccctt

SEQ ID NO: 14988 - RNA, 6936 nt, Homo sapiens
  source 1..6936: mol_type = other RNA
gctgggattacaggcatgagccactgcaaccagccttaagtttttaaattgagatcaaattcacacagcataatattcacccttttaaagtgtatagttgagtgacctgtagtatataaacaaaattgtacaacctttacccatgccacattttcattaccccaaatgacacagttcttttaagtttacatatatagccatttcaatttctcatatacaatattgtttatttgtcatccttatttcacctctggaatcactaaactttgtctcattttttttctcttccatcaaatatcaattttggattcagatccagtttttttctttcaattatttctgccttttaaaataatactacctccttcctcccacaattcatttcagcttgttttagttccttgggttctatattttttcttcctagtattacaatatatgcacaaatattaggttataaaacttccaatacaacttttactgccactcacaggtttttcaattgttttcattttcatgtacatttaaataatgtatatattagggatttattccttaacccatgttaattaagagggaatattgaattaataatcagatatttgatggttatcctattgtactgcttcttctggtcaaataatgttgccagtatgttttctgcattttggggggaaatattagaaaaaattttataatctcttcctgcttttttgacagctgtgctttctactactcatcatattttcagggtttcagattggtaaccgtttattttttattttgtaagacagagtctcgctctgtcacccagtctggagtgtgcagtggtgcaatctcagctcactataacctccaactcccaggttcaagcaatcctcccacctcagcctcttgagtagctaggattacaggcatgcaacaccatgcctggctatttgtttttgtttttgttttttttgtatttttagtagagacggggtttcaccatgttggccaggctggtctcgagctcctgacctcaagtgatccacccaccttggcctcccaaagtgctaggattacaggtgtgagccaccgcgcccagcctcagactggtattctttatgtagcataaaagataaagtctgaacaaagactatgcacacatactttttctcttccttttaaaattccacactgaataataatgatagggaaaggcttcgttatactcattacaagtgtttctctttttccaccatgaattacaaatttgccaaaggtaaacaacatggttaaaatcctttccataaatcctaatgaagatacttatgataatgagtatatcactgataatagtggaaaacttttactaaacctgtattatgtgataacagtttgaggtactttgcatttattaattcattgactcttcacagcaatccaatacatacagccttattatagatgcctagacataattttttaaaataccactaacagccaggggcggtggctcacacctataatcccagcactttgggaagccaaggcaggaggatcacgaggtcaggagtttgagagcagcctggccaatatggtgaaaccccatctctactaataatacaaaaattagctaggcatggtggcgcgcgcctgtagtcccagctactcgggaggctgaggcggaagactcacttgaactcgggaggcagaggttgcagtgagccgagattgcaccactgccctccagcctgggcaacagagcgagactgtgtctcaaaaaacaaaaacaccactaatagctataagaaaaaataattgaccgggcacagtggctcacacctgtaatccccgaactttgggaggccgaggtgggtggatcacaaggtcaagagttcaagaccagcctggccaacatagtgaaaccctgtctctactaaaaatacaaaaattagccaggcatggtgtcgtgcgcctgtagtctcagatactaggaaggctgaggcaggagaatcgcttgaacccgggaggcagcagttgtggtgaactgagattgtgccactgcacttcagcctgggcaacagagtgaactccatctcaaaaaaaaaaaaaaacaaacaaacaaaaaattaatatctggattgataaataacactttcataacagtgttactttctagtatggcattgggattaggattgatgtaagggaacaaaacagctcacaaggagaaaatgtagataattttagcaattaaaataaatgttttaaaagtaaaaataagcatccaatgaggtcagcagtttttgtgtttttttgagacggaatctcactctgtcccccaggctggagtgcagtggcaccatctcagctcactgcaacctccgcctcccaggttcaagcaattctcctgtctcagcctcccgagtagctgggattacaggtacatgccaccacgcccagctaagtagagacggggtttcactgttagccaggatggccttaatcttcagaccttgtgatccgcccacctcggcctcccaaagtgctgggattacaggcatgagccactgtgcccagccgaggtcagcttttatagctgcaaaaatttagtggcaaccataatgggaatagtcattttaaagtcattaaatatgtcatgaaaataataaaaatctatatttactgaaatggcactcatgaaatctttggcatgataaaagcagttaagggtacagcatgcatatcataattacactttcttaaaaaagcaaagtatagcacgattttctctaccaaattgagagcagccatctataagtatgattacaattaattttggctttttagtttgtaattttttgctttgtgattttggcttaacaattaaaaatgtacatttgtaaaataaaaagaccggccgcagtggctcacgcctgtaatcccagcactttcggaggccgaggcgggtggatcacctgaagtcgggagattgagaccatcctggctaacatggtgaaaccccgtctctactaaaaatacaaaaaattagccgggtgttgtggcacatgcctgtaatcccaactactcaaaaggctgaggcagaagaaccacttgaacctgggaggcgaaggttgtgacgagccgagattgcaccattgcactccagcctaggcaacaagagcgaaactccgtctcaacaaaaaataaagccaggtgcaatcgctcatgcctgtaatcccagcactttgggaggctgaggcaggtggatcacctgaggtcaggagttcaagactatcctgaccaacatggagaaaccctgtctctactaaaaatagaaaattagcagggtgtggtggcacacgcctgtgatcccagctactcaggagtctgaggcaggagaattgcttgaagccgggaggtggaggttgcagcgagccgagattgcgccactgcactccagcctgggcaacagagtgaaactccgtctcaaaaaacatataataataataataaaataaaacaaaaagactaacactaacttcaaaaacaaagttaaacctccacaaggaatttaaaaatattaaaggtcacacaattcaaacagtgtgatactggtgcaaacacaaatacacagatcagaaaagatagctctaaaaacacaagcaaatataaacatgagtataatgtgtcaccaagaaagtagaacaaaacaatgaatgaaagaattatagaacagctggcatcggtatatgactgggggagagagggaatgtcactttagactccgaatttataacctggaatgaaatacatttggatacaaaatttaaatacaaagttttaaaaaaaactacggaagagggtaactattagacatgatttttggtttaaaatatgaggaaggtgacaggggctttaatttttattatttattagtatgaattccctgatgacgaatgagatccgagccactactaaaagccttcccacattccttacagttatagggcttttcaccagtgtgaattctcagatgtcgagtaaggtttgagcatttattaaaggcctttccacattcattacattcatatggtttttcatctgtatgaattctctgatgctggaaaagttgtgagttctgagtaaaggccttcccacattcaagacattcaaagggtttctcaccagcgtgaattctctgatgttgacgaagctgtgagctctgagtaaaagcctttccacattccttacaatcatagggtttctcaccagtgtgaattctctgatgattagtaagtgctgagccactactaaaggctttgccacattccttgcactcatagggtttctcaccagtatgaattctctgatgttgaacaagctttgagctctgggtaaaggctttgccacattccttacattcatagggtttctcacctgtatgaattcgtgcatgctgaaaaagttgtgagctcttagtaaaggctttcccacatactttacattcataaggtttttcaccagtgtgaattcgctgatggtcaataagatttgagcaataactaaaggccttcccacattccttacattcatagggtttcttaccggtatggattctctgatgttgagaaaggtatgagctacaactgaaggcctttccacattccttacattcaaagggtttttcgccagtatgaattttcagatgccgagtaacatgtgaaccacaactaaagaatttcccacactctttacattcataagatttttcaccaatatgaattctctgatgttgaataaattgtgagttctgactaaaggcctttccacatttcttacattcatagggtctgtcttcattattaattatttgatggagagtaaggaatgtctgttgaataaatgtgggcatgtattcaggagtgaatatttcttgactaaaatgcccatttggatatcccagttgttttgcaaggtggcttctatattccaaaacatctccaaaactggagtactcaaggccatgctttgtaagtcccattatctccctctggcataattctatttcataaacttccttctttagagataataacttggtttcacacatcgattccagatctgaacacaggcctcttgtaagctctctgccaaccatccagggctctttcccttgttccaataaggagatcacttgaggcttaggagtgtaaagtcccattgaaaccagattgccgtagttctccaacatcacatctctgtataagtccctctgaacagggtccaggcagtcccactcctcctgagagaagtctatggacacatcactgaacatcactgatccctcagccatggcttctagtattgcagatggttagtcttccttgaggccgttctcctgtaatcccagctactcaggaggctgaggcaagagaatcgcttgaacccggaaagcagaggctgcagtgagctgagatcatgccactgcactccagcttgggcaacagagtgagactccgtcttgtatttggtttggtcaacagccattcttcctctgggtaactctcttgacgagagcagagctgaagaagaaaggaatgatgagatgccaggcctttcttgtggcccagactgagcagatcagaggtcattttggatctacagctactatctgaggtggggaggtcgagaccagcctgaccaacacggagaaaccccgtctctactgaaaatacaaaattagcagggcgtggtgacacacgcctgtaatcccagctactaggaaggctgaggcaggagaattgcttgaaccggggaggcggaggttgcggtgagccgagattgcgccattgcactccagcctgggcaacaacagcgaaactccgccttaaaacaaaacaaaacaaaaacagagaagtgtaggctgtcatgagcattcttggtatcagaggggtgaggtctctcctctcgagaatctgtcctgacctcacagggagagctggagtcacaaagacagtcacaagcaccccctacccaatgctgcagtcacccagccaccatggggacccacatagacctccacaggcacgcctcacccaaacaataacactatatatggtcacacaatcattgtcccacatctaccttgaggataagttacactagcatatttacagacccctcaaacatagcaccattcagaaccagagtgctacagatagtcacaataccacacgcactactgagccacacaaagttacagttcccccctccccaggacccctattgagcactacacacaatcacacattcaaaataacacaatgaccactaggacacacatatcaccccggcacgattacacgcactttccaaccgcagacacagtgctacataaagttacatggtcacactctcacattctcacgttactgggttatttctgggtagtagatttactcagtaaggcatccagtacacttaagtgctgctaacagtcatacaaacacaattacacacacccctcagactaacacacagtcacagcctcatcagattctctccacacaaacaccctccacaaatgtcacgcaaagttacacagccacacacaatcacagtcccaacacgggacacagtcatacctacacatacagccttacattgttacaattacacaactacaacgaggatatacaatcacacccgcgcacacagagaggcacagtcacataaggtcacactcacacacggaagcccacgcctcgcgcccgcctccccaccaccccctctatcagcccgaccaactcatacatgcccgacacactcatacatgcccaacactccagaccagcctggtcagtcccttcaaactcccatgcacgtacctgcgggccccagccgagcctgcaagacccaggccgctcaccgcgcacttcccctaccctt

SEQ ID NO: 14989 - RNA, 5720 nt, Homo sapiens
  source 1..5720: mol_type = other RNA
gctgggattacaggcatgagccactgcaaccagccttaagtttttaaattgagatcaaattcacacagcataatattcacccttttaaagtgtatagttgagtgacctgtagtatataaacaaaattgtacaacctttacccatgccacattttcattaccccaaatgacacagttcttttaagtttacatatatagccatttcaatttctcatatacaatattgtttatttgtcatccttatttcacctctggaatcactaaactttgtctcattttttttctcttccatcaaatatcaattttggattcagatccagtttttttctttcaattatttctgccttttaaaataatactacctccttcctcccacaattcatttcagcttgttttagttccttgggttctatattttttcttcctagtattacaatatatgcacaaatattaggttataaaacttccaatacaacttttactgccactcacaggtttttcaattgttttcattttcatgtacatttaaataatgtatatattagggatttattccttaacccatgttaattaagagggaatattgaattaataatcagatatttgatggttatcctattgtactgcttcttctggtcaaataatgttgccagtatgttttctgcattttggggggaaatattagaaaaaattttataatctcttcctgcttttttgacagctgtgctttctactactcatcatattttcagggtttcagattggtaaccgtttattttttattttgtaagacagagtctcgctctgtcacccagtctggagtgtgcagtggtgcaatctcagctcactataacctccaactcccaggttcaagcaatcctcccacctcagcctcttgagtagctaggattacaggcatgcaacaccatgcctggctatttgtttttgtttttgttttttttgtatttttagtagagacggggtttcaccatgttggccaggctggtctcgagctcctgacctcaagtgatccacccaccttggcctcccaaagtgctaggattacaggtgtgagccaccgcgcccagcctcagactggtattctttatgtagcataaaagataaagtctgaacaaagactatgcacacatactttttctcttccttttaaaattccacactgaataataatgatagggaaaggcttcgttatactcattacaagtgtttctctttttccaccatgaattacaaatttgccaaaggtaaacaacatggttaaaatcctttccataaatcctaatgaagatacttatgataatgagtatatcactgataatagtggaaaacttttactaaacctgtattatgtgataacagtttgaggtactttgcatttattaattcattgactcttcacagcaatccaatacatacagccttattatagatgcctagacataattttttaaaataccactaacagccaggggcggtggctcacacctataatcccagcactttgggaagccaaggcaggaggatcacgaggtcaggagtttgagagcagcctggccaatatggtgaaaccccatctctactaataatacaaaaattagctaggcatggtggcgcgcgcctgtagtcccagctactcgggaggctgaggcggaagactcacttgaactcgggaggcagaggttgcagtgagccgagattgcaccactgccctccagcctgggcaacagagcgagactgtgtctcaaaaaacaaaaacaccactaatagctataagaaaaaataattgaccgggcacagtggctcacacctgtaatccccgaactttgggaggccgaggtgggtggatcacaaggtcaagagttcaagaccagcctggccaacatagtgaaaccctgtctctactaaaaatacaaaaattagccaggcatggtgtcgtgcgcctgtagtctcagatactaggaaggctgaggcaggagaatcgcttgaacccgggaggcagcagttgtggtgaactgagattgtgccactgcacttcagcctgggcaacagagtgaactccatctcaaaaaaaaaaaaaaacaaacaaacaaaaaattaatatctggattgataaataacactttcataacagtgttactttctagtatggcattgggattaggattgatgtaagggaacaaaacagctcacaaggagaaaatgtagataattttagcaattaaaataaatgttttaaaagtaaaaataagcatccaatgaggtcagcagtttttgtgtttttttgagacggaatctcactctgtcccccaggctggagtgcagtggcaccatctcagctcactgcaacctccgcctcccaggttcaagcaattctcctgtctcagcctcccgagtagctgggattacaggtacatgccaccacgcccagctaagtagagacggggtttcactgttagccaggatggccttaatcttcagaccttgtgatccgcccacctcggcctcccaaagtgctgggattacaggcatgagccactgtgcccagccgaggtcagcttttatagctgcaaaaatttagtggcaaccataatgggaatagtcattttaaagtcattaaatatgtcatgaaaataataaaaatctatatttactgaaatggcactcatgaaatctttggcatgataaaagcagttaagggtacagcatgcatatcataattacactttcttaaaaaagcaaagtatagcacgattttctctaccaaattgagagcagccatctataagtatgattacaattaattttggctttttagtttgtaattttttgctttgtgattttggcttaacaattaaaaatgtacatttgtaaaataaaaagaccggccgcagtggctcacgcctgtaatcccagcactttcggaggccgaggcgggtggatcacctgaagtcgggagattgagaccatcctggctaacatggtgaaaccccgtctctactaaaaatacaaaaaattagccgggtgttgtggcacatgcctgtaatcccaactactcaaaaggctgaggcagaagaaccacttgaacctgggaggcgaaggttgtgacgagccgagattgcaccattgcactccagcctaggcaacaagagcgaaactccgtctcaacaaaaaataaagccaggtgcaatcgctcatgcctgtaatcccagcactttgggaggctgaggcaggtggatcacctgaggtcaggagttcaagactatcctgaccaacatggagaaaccctgtctctactaaaaatagaaaattagcagggtgtggtggcacacgcctgtgatcccagctactcaggagtctgaggcaggagaattgcttgaagccgggaggtggaggttgcagcgagccgagattgcgccactgcactccagcctgggcaacagagtgaaactccgtctcaaaaaacatataataataataataaaataaaacaaaaagactaacactaacttcaaaaacaaagttaaacctccacaaggaatttaaaaatattaaaggtcacacaattcaaacagtgtgatactggtgcaaacacaaatacacagatcagaaaagatagctctaaaaacacaagcaaatataaacatgagtataatgtgtcaccaagaaagtagaacaaaacaatgaatgaaagaattatagaacagctggcatcggtatatgactgggggagagagggaatgtcactttagactccgaatttataacctggaatgaaatacatttggatacaaaatttaaatacaaagttttaaaaaaaactacggaagagggtaactattagacatgatttttggtttaaaatatgaggaaggtgacaggggctttaatttttattatttattagtatgaattccctgatgacgaatgagatccgagccactactaaaagccttcccacattccttacagttatagggcttttcaccagtgtgaattctcagatgtcgagtaaggtttgagcatttattaaaggcctttccacattcattacattcatatggtttttcatctgtatgaattctctgatgctggaaaagttgtgagttctgagtaaaggccttcccacattcaagacattcaaagggtttctcaccagcgtgaattctctgatgttgacgaagctgtgagctctgagtaaaagcctttccacattccttacaatcatagggtttctcaccagtgtgaattctctgatgattagtaagtgctgagccactactaaaggctttgccacattccttgcactcatagggtttctcaccagtatgaattctctgatgttgaacaagctttgagctctgggtaaaggctttgccacattccttacattcatagggtttctcacctgtatgaattcgtgcatgctgaaaaagttgtgagctcttagtaaaggctttcccacatactttacattcataaggtttttcaccagtgtgaattcgctgatggtcaataagatttgagcaataactaaaggccttcccacattccttacattcatagggtttcttaccggtatggattctctgatgttgagaaaggtatgagctacaactgaaggcctttccacattccttacattcaaagggtttttcgccagtatgaattttcagatgccgagtaacatgtgaaccacaactaaagaatttcccacactctttacattcataagatttttcaccaatatgaattctctgatgttgaataaattgtgagttctgactaaaggcctttccacatttcttacattcatagggtctgtcttcattattaattatttgatggagagtaaggaatgtctgttgaataaatgtgggcatgtattcaggagtgaatatttcttgactaaaatgcccatttggatatcccagttgttttgcaaggtggcttctatattccaaaacatctccaaaactggagtactcaaggccatgctttgtaagtcccattatctccctctggcataattctatttcataaacttccttctttagagataataacttggtttcacacatcgattccagatctgaacacaggcctcttgtaagctctctgccaaccatccagggctctttcccttgttccaataaggagatcacttgaggcttaggagtgtaaagtcccattgaaaccagattgccgtagttctccaacatcacatctctgtataagtccctctgaacagggtccaggcagtcccactcctcctgagagaagtctatggacacatcactgaacatcactgatccctcagccatggcttctagtattgcagatggttagtcttccttgaggccgttctcctgtaatcccagctactcaggaggctgaggcaagagaatcgcttgaacccggaaagcagaggctgcagtgagctgagatcatgccactgcactccagcttgggcaacagagtgagactccgtcttgtatttggtttggtcaacagccattcttcctctgggtaactctcttgacgagagcagagctgaagaagaaaggaatgatgagatgccaggcctttcttgtggcccagactgagcagatcagaggtcattttggatctacagctactatctgcgggccccagccgagcctgcaagacccaggccgctcaccgcgcacttcccctaccctt

SEQ ID NO: 14990 - RNA, 5631 nt, Homo sapiens
  source 1..5631: mol_type = other RNA
gctgggattacaggcatgagccactgcaaccagccttaagtttttaaattgagatcaaattcacacagcataatattcacccttttaaagtgtatagttgagtgacctgtagtatataaacaaaattgtacaacctttacccatgccacattttcattaccccaaatgacacagttcttttaagtttacatatatagccatttcaatttctcatatacaatattgtttatttgtcatccttatttcacctctggaatcactaaactttgtctcattttttttctcttccatcaaatatcaattttggattcagatccagtttttttctttcaattatttctgccttttaaaataatactacctccttcctcccacaattcatttcagcttgttttagttccttgggttctatattttttcttcctagtattacaatatatgcacaaatattaggttataaaacttccaatacaacttttactgccactcacaggtttttcaattgttttcattttcatgtacatttaaataatgtatatattagggatttattccttaacccatgttaattaagagggaatattgaattaataatcagatatttgatggttatcctattgtactgcttcttctggtcaaataatgttgccagtatgttttctgcattttggggggaaatattagaaaaaattttataatctcttcctgcttttttgacagctgtgctttctactactcatcatattttcagggtttcagattggtaaccgtttattttttattttgtaagacagagtctcgctctgtcacccagtctggagtgtgcagtggtgcaatctcagctcactataacctccaactcccaggttcaagcaatcctcccacctcagcctcttgagtagctaggattacaggcatgcaacaccatgcctggctatttgtttttgtttttgttttttttgtatttttagtagagacggggtttcaccatgttggccaggctggtctcgagctcctgacctcaagtgatccacccaccttggcctcccaaagtgctaggattacaggtgtgagccaccgcgcccagcctcagactggtattctttatgtagcataaaagataaagtctgaacaaagactatgcacacatactttttctcttccttttaaaattccacactgaataataatgatagggaaaggcttcgttatactcattacaagtgtttctctttttccaccatgaattacaaatttgccaaaggtaaacaacatggttaaaatcctttccataaatcctaatgaagatacttatgataatgagtatatcactgataatagtggaaaacttttactaaacctgtattatgtgataacagtttgaggtactttgcatttattaattcattgactcttcacagcaatccaatacatacagccttattatagatgcctagacataattttttaaaataccactaacagccaggggcggtggctcacacctataatcccagcactttgggaagccaaggcaggaggatcacgaggtcaggagtttgagagcagcctggccaatatggtgaaaccccatctctactaataatacaaaaattagctaggcatggtggcgcgcgcctgtagtcccagctactcgggaggctgaggcggaagactcacttgaactcgggaggcagaggttgcagtgagccgagattgcaccactgccctccagcctgggcaacagagcgagactgtgtctcaaaaaacaaaaacaccactaatagctataagaaaaaataattgaccgggcacagtggctcacacctgtaatccccgaactttgggaggccgaggtgggtggatcacaaggtcaagagttcaagaccagcctggccaacatagtgaaaccctgtctctactaaaaatacaaaaattagccaggcatggtgtcgtgcgcctgtagtctcagatactaggaaggctgaggcaggagaatcgcttgaacccgggaggcagcagttgtggtgaactgagattgtgccactgcacttcagcctgggcaacagagtgaactccatctcaaaaaaaaaaaaaaacaaacaaacaaaaaattaatatctggattgataaataacactttcataacagtgttactttctagtatggcattgggattaggattgatgtaagggaacaaaacagctcacaaggagaaaatgtagataattttagcaattaaaataaatgttttaaaagtaaaaataagcatccaatgaggtcagcagtttttgtgtttttttgagacggaatctcactctgtcccccaggctggagtgcagtggcaccatctcagctcactgcaacctccgcctcccaggttcaagcaattctcctgtctcagcctcccgagtagctgggattacaggtacatgccaccacgcccagctaagtagagacggggtttcactgttagccaggatggccttaatcttcagaccttgtgatccgcccacctcggcctcccaaagtgctgggattacaggcatgagccactgtgcccagccgaggtcagcttttatagctgcaaaaatttagtggcaaccataatgggaatagtcattttaaagtcattaaatatgtcatgaaaataataaaaatctatatttactgaaatggcactcatgaaatctttggcatgataaaagcagttaagggtacagcatgcatatcataattacactttcttaaaaaagcaaagtatagcacgattttctctaccaaattgagagcagccatctataagtatgattacaattaattttggctttttagtttgtaattttttgctttgtgattttggcttaacaattaaaaatgtacatttgtaaaataaaaagaccggccgcagtggctcacgcctgtaatcccagcactttcggaggccgaggcgggtggatcacctgaagtcgggagattgagaccatcctggctaacatggtgaaaccccgtctctactaaaaatacaaaaaattagccgggtgttgtggcacatgcctgtaatcccaactactcaaaaggctgaggcagaagaaccacttgaacctgggaggcgaaggttgtgacgagccgagattgcaccattgcactccagcctaggcaacaagagcgaaactccgtctcaacaaaaaataaagccaggtgcaatcgctcatgcctgtaatcccagcactttgggaggctgaggcaggtggatcacctgaggtcaggagttcaagactatcctgaccaacatggagaaaccctgtctctactaaaaatagaaaattagcagggtgtggtggcacacgcctgtgatcccagctactcaggagtctgaggcaggagaattgcttgaagccgggaggtggaggttgcagcgagccgagattgcgccactgcactccagcctgggcaacagagtgaaactccgtctcaaaaaacatataataataataataaaataaaacaaaaagactaacactaacttcaaaaacaaagttaaacctccacaaggaatttaaaaatattaaaggtcacacaattcaaacagtgtgatactggtgcaaacacaaatacacagatcagaaaagatagctctaaaaacacaagcaaatataaacatgagtataatgtgtcaccaagaaagtagaacaaaacaatgaatgaaagaattatagaacagctggcatcggtatatgactgggggagagagggaatgtcactttagactccgaatttataacctggaatgaaatacatttggatacaaaatttaaatacaaagttttaaaaaaaactacggaagagggtaactattagacatgatttttggtttaaaatatgaggaaggtgacaggggctttaatttttattatttattagtatgaattccctgatgacgaatgagatccgagccactactaaaagccttcccacattccttacagttatagggcttttcaccagtgtgaattctcagatgtcgagtaaggtttgagcatttattaaaggcctttccacattcattacattcatatggtttttcatctgtatgaattctctgatgctggaaaagttgtgagttctgagtaaaggccttcccacattcaagacattcaaagggtttctcaccagcgtgaattctctgatgttgacgaagctgtgagctctgagtaaaagcctttccacattccttacaatcatagggtttctcaccagtgtgaattctctgatgattagtaagtgctgagccactactaaaggctttgccacattccttgcactcatagggtttctcaccagtatgaattctctgatgttgaacaagctttgagctctgggtaaaggctttgccacattccttacattcatagggtttctcacctgtatgaattcgtgcatgctgaaaaagttgtgagctcttagtaaaggctttcccacatactttacattcataaggtttttcaccagtgtgaattcgctgatggtcaataagatttgagcaataactaaaggccttcccacattccttacattcatagggtttcttaccggtatggattctctgatgttgagaaaggtatgagctacaactgaaggcctttccacattccttacattcaaagggtttttcgccagtatgaattttcagatgccgagtaacatgtgaaccacaactaaagaatttcccacactctttacattcataagatttttcaccaatatgaattctctgatgttgaataaattgtgagttctgactaaaggcctttccacatttcttacattcatagggtctgtcttcattattaattatttgatggagagtaaggaatgtctgttgaataaatgtgggcatgtattcaggagtgaatatttcttgactaaaatgcccatttggatatcccagttgttttgcaaggtggcttctatattccaaaacatctccaaaactggagtactcaaggccatgctttgtaagtcccattatctccctctggcataattctatttcataaacttccttctttagagataataacttggtttcacacatcgattccagatctgaacacaggcctcttgtaagctctctgccaaccatccagggctctttcccttgttccaataaggagatcacttgaggcttaggagtgtaaagtcccattgaaaccagattgccgtagttctccaacatcacatctctgtataagtccctctgaacagggtccaggcagtcccactcctcctgagagaagtctatggacacatcactgaacatcactgatccctcagccatggcttctagtattgcagatggttagtcttccttgaggccgttctcctgtaatcccagctactcaggaggctgaggcaagagaatcgcttgaacccggaaagcagaggctgcagtgagctgagatcatgccactgcactccagcttgggcaacagagtgagactccgtcttgtatttggtttggtcaacagccattcttcctctgggtaactctcttgacgagagcagagctgcgggccccagccgagcctgcaagacccaggccgctcaccgcgcacttcccctaccctt

SEQ ID NO: 14991 - RNA, 6814 nt, Homo sapiens
  source 1..6814: mol_type = other RNA
gctgggattacaggcatgagccactgcaaccagccttaagtttttaaattgagatcaaattcacacagcataatattcacccttttaaagtgtatagttgagtgacctgtagtatataaacaaaattgtacaacctttacccatgccacattttcattaccccaaatgacacagttcttttaagtttacatatatagccatttcaatttctcatatacaatattgtttatttgtcatccttatttcacctctggaatcactaaactttgtctcattttttttctcttccatcaaatatcaattttggattcagatccagtttttttctttcaattatttctgccttttaaaataatactacctccttcctcccacaattcatttcagcttgttttagttccttgggttctatattttttcttcctagtattacaatatatgcacaaatattaggttataaaacttccaatacaacttttactgccactcacaggtttttcaattgttttcattttcatgtacatttaaataatgtatatattagggatttattccttaacccatgttaattaagagggaatattgaattaataatcagatatttgatggttatcctattgtactgcttcttctggtcaaataatgttgccagtatgttttctgcattttggggggaaatattagaaaaaattttataatctcttcctgcttttttgacagctgtgctttctactactcatcatattttcagggtttcagattggtaaccgtttattttttattttgtaagacagagtctcgctctgtcacccagtctggagtgtgcagtggtgcaatctcagctcactataacctccaactcccaggttcaagcaatcctcccacctcagcctcttgagtagctaggattacaggcatgcaacaccatgcctggctatttgtttttgtttttgttttttttgtatttttagtagagacggggtttcaccatgttggccaggctggtctcgagctcctgacctcaagtgatccacccaccttggcctcccaaagtgctaggattacaggtgtgagccaccgcgcccagcctcagactggtattctttatgtagcataaaagataaagtctgaacaaagactatgcacacatactttttctcttccttttaaaattccacactgaataataatgatagggaaaggcttcgttatactcattacaagtgtttctctttttccaccatgaattacaaatttgccaaaggtaaacaacatggttaaaatcctttccataaatcctaatgaagatacttatgataatgagtatatcactgataatagtggaaaacttttactaaacctgtattatgtgataacagtttgaggtactttgcatttattaattcattgactcttcacagcaatccaatacatacagccttattatagatgcctagacataattttttaaaataccactaacagccaggggcggtggctcacacctataatcccagcactttgggaagccaaggcaggaggatcacgaggtcaggagtttgagagcagcctggccaatatggtgaaaccccatctctactaataatacaaaaattagctaggcatggtggcgcgcgcctgtagtcccagctactcgggaggctgaggcggaagactcacttgaactcgggaggcagaggttgcagtgagccgagattgcaccactgccctccagcctgggcaacagagcgagactgtgtctcaaaaaacaaaaacaccactaatagctataagaaaaaataattgaccgggcacagtggctcacacctgtaatccccgaactttgggaggccgaggtgggtggatcacaaggtcaagagttcaagaccagcctggccaacatagtgaaaccctgtctctactaaaaatacaaaaattagccaggcatggtgtcgtgcgcctgtagtctcagatactaggaaggctgaggcaggagaatcgcttgaacccgggaggcagcagttgtggtgaactgagattgtgccactgcacttcagcctgggcaacagagtgaactccatctcaaaaaaaaaaaaaaacaaacaaacaaaaaattaatatctggattgataaataacactttcataacagtgttactttctagtatggcattgggattaggattgatgtaagggaacaaaacagctcacaaggagaaaatgtagataattttagcaattaaaataaatgttttaaaagtaaaaataagcatccaatgaggtcagcagtttttgtgtttttttgagacggaatctcactctgtcccccaggctggagtgcagtggcaccatctcagctcactgcaacctccgcctcccaggttcaagcaattctcctgtctcagcctcccgagtagctgggattacaggtacatgccaccacgcccagctaagtagagacggggtttcactgttagccaggatggccttaatcttcagaccttgtgatccgcccacctcggcctcccaaagtgctgggattacaggcatgagccactgtgcccagccgaggtcagcttttatagctgcaaaaatttagtggcaaccataatgggaatagtcattttaaagtcattaaatatgtcatgaaaataataaaaatctatatttactgaaatggcactcatgaaatctttggcatgataaaagcagttaagggtacagcatgcatatcataattacactttcttaaaaaagcaaagtatagcacgattttctctaccaaattgagagcagccatctataagtatgattacaattaattttggctttttagtttgtaattttttgctttgtgattttggcttaacaattaaaaatgtacatttgtaaaataaaaagaccggccgcagtggctcacgcctgtaatcccagcactttcggaggccgaggcgggtggatcacctgaagtcgggagattgagaccatcctggctaacatggtgaaaccccgtctctactaaaaatacaaaaaattagccgggtgttgtggcacatgcctgtaatcccaactactcaaaaggctgaggcagaagaaccacttgaacctgggaggcgaaggttgtgacgagccgagattgcaccattgcactccagcctaggcaacaagagcgaaactccgtctcaacaaaaaataaagccaggtgcaatcgctcatgcctgtaatcccagcactttgggaggctgaggcaggtggatcacctgaggtcaggagttcaagactatcctgaccaacatggagaaaccctgtctctactaaaaatagaaaattagcagggtgtggtggcacacgcctgtgatcccagctactcaggagtctgaggcaggagaattgcttgaagccgggaggtggaggttgcagcgagccgagattgcgccactgcactccagcctgggcaacagagtgaaactccgtctcaaaaaacatataataataataataaaataaaacaaaaagactaacactaacttcaaaaacaaagttaaacctccacaaggaatttaaaaatattaaaggtcacacaattcaaacagtgtgatactggtgcaaacacaaatacacagatcagaaaagatagctctaaaaacacaagcaaatataaacatgagtataatgtgtcaccaagaaagtagaacaaaacaatgaatgaaagaattatagaacagctggcatcggtatatgactgggggagagagggaatgtcactttagactccgaatttataacctggaatgaaatacatttggatacaaaatttaaatacaaagttttaaaaaaaactacggaagagggtaactattagacatgatttttggtttaaaatatgaggaaggtgacaggggctttaatttttattatttattagtatgaattccctgatgacgaatgagatccgagccactactaaaagccttcccacattccttacagttatagggcttttcaccagtgtgaattctcagatgtcgagtaaggtttgagcatttattaaaggcctttccacattcattacattcatatggtttttcatctgtatgaattctctgatgctggaaaagttgtgagttctgagtaaaggccttcccacattcaagacattcaaagggtttctcaccagcgtgaattctctgatgttgacgaagctgtgagctctgagtaaaagcctttccacattccttacaatcatagggtttctcaccagtgtgaattctctgatgattagtaagtgctgagccactactaaaggctttgccacattccttgcactcatagggtttctcaccagtatgaattctctgatgttgaacaagctttgagctctgggtaaaggctttgccacattccttacattcatagggtttctcacctgtatgaattcgtgcatgctgaaaaagttgtgagctcttagtaaaggctttcccacatactttacattcataaggtttttcaccagtgtgaattcgctgatggtcaataagatttgagcaataactaaaggccttcccacattccttacattcatagggtttcttaccggtatggattctctgatgttgagaaaggtatgagctacaactgaaggcctttccacattccttacattcaaagggtttttcgccagtatgaattttcagatgccgagtaacatgtgaaccacaactaaagaatttcccacactctttacattcataagatttttcaccaatatgaattctctgatgttgaataaattgtgagttctgactaaaggcctttccacatttcttacattcatagggtctgtcttcattattaattatttgatggagagtaaggaatgtctgttgaataaatgtgggcatgtattcaggagtgaatatttcttgactaaaatgcccatttggatatcccagttgttttgcaaggtggcttctatattccaaaacatctccaaaactggagtactcaaggccatgctttgtaagtcccattatctccctctggcataattctatttcataaacttccttctttagagataataacttggtttcacacatcgattccagatctgaacacaggcctcttgtaagctctctgccaaccatccagggctctttcccttgttccaataaggagatcacttgaggcttaggagtgtaaagtcccattgaaaccagattgccgtagttctccaacatcacatctctgtataagtccctctgaacagggtccaggcagtcccactcctcctgagagaagtctatggacacatcactgaacatcactgatccctcagccatggcttctagtattgcagatggttagtcttccttgaggccgttctccttgtatttggtttggtcaacagccattcttcctctgggtaactctcttgacgagagcagagctgaagaagaaaggaatgatgagatgccaggcctttcttgtggcccagactgagcagatcagaggtcattttggatctacagctactatctgaggtggggaggtcgagaccagcctgaccaacacggagaaaccccgtctctactgaaaatacaaaattagcagggcgtggtgacacacgcctgtaatcccagctactaggaaggctgaggcaggagaattgcttgaaccggggaggcggaggttgcggtgagccgagattgcgccattgcactccagcctgggcaacaacagcgaaactccgccttaaaacaaaacaaaacaaaaacagagaagtgtaggctgtcatgagcattcttggtatcagaggggtgaggtctctcctctcgagaatctgtcctgacctcacagggagagctggagtcacaaagacagtcacaagcaccccctacccaatgctgcagtcacccagccaccatggggacccacatagacctccacaggcacgcctcacccaaacaataacactatatatggtcacacaatcattgtcccacatctaccttgaggataagttacactagcatatttacagacccctcaaacatagcaccattcagaaccagagtgctacagatagtcacaataccacacgcactactgagccacacaaagttacagttcccccctccccaggacccctattgagcactacacacaatcacacattcaaaataacacaatgaccactaggacacacatatcaccccggcacgattacacgcactttccaaccgcagacacagtgctacataaagttacatggtcacactctcacattctcacgttactgggttatttctgggtagtagatttactcagtaaggcatccagtacacttaagtgctgctaacagtcatacaaacacaattacacacacccctcagactaacacacagtcacagcctcatcagattctctccacacaaacaccctccacaaatgtcacgcaaagttacacagccacacacaatcacagtcccaacacgggacacagtcatacctacacatacagccttacattgttacaattacacaactacaacgaggatatacaatcacacccgcgcacacagagaggcacagtcacataaggtcacactcacacacggaagcccacgcctcgcgcccgcctccccaccaccccctctatcagcccgaccaactcatacatgcccgacacactcatacatgcccaacactccagaccagcctggtcagtcccttcaaactcccatgcacgtacctgcgggccccagccgagcctgcaagacccaggccgctcaccgcgcacttcccctaccctt

SEQ ID NO: 14992 - RNA, 5509 nt, Homo sapiens
  source 1..5509: mol_type = other RNA
gctgggattacaggcatgagccactgcaaccagccttaagtttttaaattgagatcaaattcacacagcataatattcacccttttaaagtgtatagttgagtgacctgtagtatataaacaaaattgtacaacctttacccatgccacattttcattaccccaaatgacacagttcttttaagtttacatatatagccatttcaatttctcatatacaatattgtttatttgtcatccttatttcacctctggaatcactaaactttgtctcattttttttctcttccatcaaatatcaattttggattcagatccagtttttttctttcaattatttctgccttttaaaataatactacctccttcctcccacaattcatttcagcttgttttagttccttgggttctatattttttcttcctagtattacaatatatgcacaaatattaggttataaaacttccaatacaacttttactgccactcacaggtttttcaattgttttcattttcatgtacatttaaataatgtatatattagggatttattccttaacccatgttaattaagagggaatattgaattaataatcagatatttgatggttatcctattgtactgcttcttctggtcaaataatgttgccagtatgttttctgcattttggggggaaatattagaaaaaattttataatctcttcctgcttttttgacagctgtgctttctactactcatcatattttcagggtttcagattggtaaccgtttattttttattttgtaagacagagtctcgctctgtcacccagtctggagtgtgcagtggtgcaatctcagctcactataacctccaactcccaggttcaagcaatcctcccacctcagcctcttgagtagctaggattacaggcatgcaacaccatgcctggctatttgtttttgtttttgttttttttgtatttttagtagagacggggtttcaccatgttggccaggctggtctcgagctcctgacctcaagtgatccacccaccttggcctcccaaagtgctaggattacaggtgtgagccaccgcgcccagcctcagactggtattctttatgtagcataaaagataaagtctgaacaaagactatgcacacatactttttctcttccttttaaaattccacactgaataataatgatagggaaaggcttcgttatactcattacaagtgtttctctttttccaccatgaattacaaatttgccaaaggtaaacaacatggttaaaatcctttccataaatcctaatgaagatacttatgataatgagtatatcactgataatagtggaaaacttttactaaacctgtattatgtgataacagtttgaggtactttgcatttattaattcattgactcttcacagcaatccaatacatacagccttattatagatgcctagacataattttttaaaataccactaacagccaggggcggtggctcacacctataatcccagcactttgggaagccaaggcaggaggatcacgaggtcaggagtttgagagcagcctggccaatatggtgaaaccccatctctactaataatacaaaaattagctaggcatggtggcgcgcgcctgtagtcccagctactcgggaggctgaggcggaagactcacttgaactcgggaggcagaggttgcagtgagccgagattgcaccactgccctccagcctgggcaacagagcgagactgtgtctcaaaaaacaaaaacaccactaatagctataagaaaaaataattgaccgggcacagtggctcacacctgtaatccccgaactttgggaggccgaggtgggtggatcacaaggtcaagagttcaagaccagcctggccaacatagtgaaaccctgtctctactaaaaatacaaaaattagccaggcatggtgtcgtgcgcctgtagtctcagatactaggaaggctgaggcaggagaatcgcttgaacccgggaggcagcagttgtggtgaactgagattgtgccactgcacttcagcctgggcaacagagtgaactccatctcaaaaaaaaaaaaaaacaaacaaacaaaaaattaatatctggattgataaataacactttcataacagtgttactttctagtatggcattgggattaggattgatgtaagggaacaaaacagctcacaaggagaaaatgtagataattttagcaattaaaataaatgttttaaaagtaaaaataagcatccaatgaggtcagcagtttttgtgtttttttgagacggaatctcactctgtcccccaggctggagtgcagtggcaccatctcagctcactgcaacctccgcctcccaggttcaagcaattctcctgtctcagcctcccgagtagctgggattacaggtacatgccaccacgcccagctaagtagagacggggtttcactgttagccaggatggccttaatcttcagaccttgtgatccgcccacctcggcctcccaaagtgctgggattacaggcatgagccactgtgcccagccgaggtcagcttttatagctgcaaaaatttagtggcaaccataatgggaatagtcattttaaagtcattaaatatgtcatgaaaataataaaaatctatatttactgaaatggcactcatgaaatctttggcatgataaaagcagttaagggtacagcatgcatatcataattacactttcttaaaaaagcaaagtatagcacgattttctctaccaaattgagagcagccatctataagtatgattacaattaattttggctttttagtttgtaattttttgctttgtgattttggcttaacaattaaaaatgtacatttgtaaaataaaaagaccggccgcagtggctcacgcctgtaatcccagcactttcggaggccgaggcgggtggatcacctgaagtcgggagattgagaccatcctggctaacatggtgaaaccccgtctctactaaaaatacaaaaaattagccgggtgttgtggcacatgcctgtaatcccaactactcaaaaggctgaggcagaagaaccacttgaacctgggaggcgaaggttgtgacgagccgagattgcaccattgcactccagcctaggcaacaagagcgaaactccgtctcaacaaaaaataaagccaggtgcaatcgctcatgcctgtaatcccagcactttgggaggctgaggcaggtggatcacctgaggtcaggagttcaagactatcctgaccaacatggagaaaccctgtctctactaaaaatagaaaattagcagggtgtggtggcacacgcctgtgatcccagctactcaggagtctgaggcaggagaattgcttgaagccgggaggtggaggttgcagcgagccgagattgcgccactgcactccagcctgggcaacagagtgaaactccgtctcaaaaaacatataataataataataaaataaaacaaaaagactaacactaacttcaaaaacaaagttaaacctccacaaggaatttaaaaatattaaaggtcacacaattcaaacagtgtgatactggtgcaaacacaaatacacagatcagaaaagatagctctaaaaacacaagcaaatataaacatgagtataatgtgtcaccaagaaagtagaacaaaacaatgaatgaaagaattatagaacagctggcatcggtatatgactgggggagagagggaatgtcactttagactccgaatttataacctggaatgaaatacatttggatacaaaatttaaatacaaagttttaaaaaaaactacggaagagggtaactattagacatgatttttggtttaaaatatgaggaaggtgacaggggctttaatttttattatttattagtatgaattccctgatgacgaatgagatccgagccactactaaaagccttcccacattccttacagttatagggcttttcaccagtgtgaattctcagatgtcgagtaaggtttgagcatttattaaaggcctttccacattcattacattcatatggtttttcatctgtatgaattctctgatgctggaaaagttgtgagttctgagtaaaggccttcccacattcaagacattcaaagggtttctcaccagcgtgaattctctgatgttgacgaagctgtgagctctgagtaaaagcctttccacattccttacaatcatagggtttctcaccagtgtgaattctctgatgattagtaagtgctgagccactactaaaggctttgccacattccttgcactcatagggtttctcaccagtatgaattctctgatgttgaacaagctttgagctctgggtaaaggctttgccacattccttacattcatagggtttctcacctgtatgaattcgtgcatgctgaaaaagttgtgagctcttagtaaaggctttcccacatactttacattcataaggtttttcaccagtgtgaattcgctgatggtcaataagatttgagcaataactaaaggccttcccacattccttacattcatagggtttcttaccggtatggattctctgatgttgagaaaggtatgagctacaactgaaggcctttccacattccttacattcaaagggtttttcgccagtatgaattttcagatgccgagtaacatgtgaaccacaactaaagaatttcccacactctttacattcataagatttttcaccaatatgaattctctgatgttgaataaattgtgagttctgactaaaggcctttccacatttcttacattcatagggtctgtcttcattattaattatttgatggagagtaaggaatgtctgttgaataaatgtgggcatgtattcaggagtgaatatttcttgactaaaatgcccatttggatatcccagttgttttgcaaggtggcttctatattccaaaacatctccaaaactggagtactcaaggccatgctttgtaagtcccattatctccctctggcataattctatttcataaacttccttctttagagataataacttggtttcacacatcgattccagatctgaacacaggcctcttgtaagctctctgccaaccatccagggctctttcccttgttccaataaggagatcacttgaggcttaggagtgtaaagtcccattgaaaccagattgccgtagttctccaacatcacatctctgtataagtccctctgaacagggtccaggcagtcccactcctcctgagagaagtctatggacacatcactgaacatcactgatccctcagccatggcttctagtattgcagatggttagtcttccttgaggccgttctccttgtatttggtttggtcaacagccattcttcctctgggtaactctcttgacgagagcagagctgcgggccccagccgagcctgcaagacccaggccgctcaccgcgcacttcccctaccctt

SEQ ID NO: 14993 - RNA, 2564 nt, Homo sapiens
  source 1..2564: mol_type = other RNA
gctgggattacaggcatgagccactgcaagtggcccatttaaatgttctataacaatattcagtgattacaatttctttgattcaaatacataagcaaatgcacaagcaataatgtatgcagtacatattaaacatcattactgcctaaacttgattaaacaaatgaataactttataattaaaaatatgtttctaggcaaagttaaatatattgacattagaagtaatatattcttgcatgtgtgggccacaaagaccttggctaaagtgtacattttaaaggtgcaaagcataaaaacagagcttttgagaatgacagcttcaagaagacaaaccaattaactcccaaatattggcttcaattcaagcgatatttctgtaaaatatacatttcatgacttcaattattacctaatgaatgcaaaaagccactatgactacactacacaggaattcaatgacagaacttctgtataaatacagtacagttgctcattttttagtagatttttttttcctccctgaatccacatgcatcaattctgttaactttgtaatatatgttacaaaatcaatagttaccttaaaatatttcatagcacactcaaattgtatgattcttatggtacttattgtactttggcttccagtagcccagtggacataacatgaccatgactgcttagacaactacttgtatgcctcagggcatctgcttcaagataggccattaaaagctcagtgcggcgaatgagtaactgcatgaggtcttcagctaaagtctctgtacttgaatagcgcaccttctcaaagtcaaaaatgtctttgagaaataaaagaacttgattcttaaaaaagcaacataaatcatacagagaatttctaggacccaaaaagccccaggctaggacaggactgatgtgttcacaaatggcataaaaatgggcaaaaaatccatctgggatctgcttcatctgttgtcttttctgtttcagcaccgaccaacaacttgaagccacagctgtttctttgaaggatgagtttagccatcgattatttactacattctgtatggatgtgggtgggttttccaaatcttcaaaggagtccattaatataaaatccagaacaacatcataaaaatttagatttttcacccctctagcagcaagttccatttcagtactaccccagtgatcggtctgctctaaaaaatagatcatttcatcaaaaacatcttcaaacttctttggattctttcgtgctttcacaattaaagctgataaaattttccttccgctctcagcgaggaatatcctgttagctgattctgaaagaattacctgaaaagcctgtcgaatacagtgaagtttggcaagaaaatcactgtctcctaggcactccaacatttcagttctcagtactctggagtaaatttttccttcttcaactaaatgcatggcttcctcgtaaaatgggcagtgacaaagggactccaggctgtaggtatgccgtacttctctgtgttctgcaagctctgctgcggaagcaaaggaatccgtggatgcgatgctcaaggtgtctcgcaggccaaagtcttccacattacccttcatggtgatatctgtatctttatcaatatcatcagcaagggaattaggatcagatgccccaagggtagcttcaaactcctcttggagacgataggctctttgcagcagagcttcgagtttatggataaattcagtactaataatatcatctacattttcttcagcaatggcatctcctgcacccagtttaatggaaccacaggcttcatcttcagcctgtctattgcgaaaggtcagagcttgttcccatcgacgcaatgcctcttcaaacaattccatacccattaagtataagttctctggagtagtcacaggaatattaacaagtttaatatcatcttcatctgctttgtcccaggaattagaattgccacaagcgcagctatgacaagaattgacactctggacagaggccaaactctgtgcagaacctgaatatttactgaaaagtcctccattagcatagttacaaacttgagatcctttgtctttggtagaacttaaagataatgtcaaattctgtctgctactggaacaacttgaacctttgtctgatgctgctcttttagtgtattcaagtatgaggtgctctggttcccatggtaatatttttcctttcttctttccacgttttcttttaaagtgatgagccagaaaaattacagatatagcactcactgcagttaccacaaacaactttttagccaccggagaaaatttgatctgggagagagaatagtaccaagtcagaggaagatcaaacactcttagcgctgctgtcttcaaggaaaactgtgattcacttactgtttcttctgacatggctcctcttctaatctggagctccaggccaggtacagctggcctgcccacgccagcttcccagctgatgcctggcgctgagcagcagtctgacatggagaaggcggagtccttccggggtcaggagt

SEQ ID NO: 14994 - RNA, 2606 nt, Homo sapiens
  source 1..2606: mol_type = other RNA
gctgggattacaggcatgagccactgcaagtggcccatttaaatgttctataacaatattcagtgattacaatttctttgattcaaatacataagcaaatgcacaagcaataatgtatgcagtacatattaaacatcattactgcctaaacttgattaaacaaatgaataactttataattaaaaatatgtttctaggcaaagttaaatatattgacattagaagtaatatattcttgcatgtgtgggccacaaagaccttggctaaagtgtacattttaaaggtgcaaagcataaaaacagagcttttgagaatgacagcttcaagaagacaaaccaattaactcccaaatattggcttcaattcaagcgatatttctgtaaaatatacatttcatgacttcaattattacctaatgaatgcaaaaagccactatgactacactacacaggaattcaatgacagaacttctgtataaatacagtacagttgctcattttttagtagatttttttttcctccctgaatccacatgcatcaattctgttaactttgtaatatatgttacaaaatcaatagttaccttaaaatatttcatagcacactcaaattgtatgattcttatggtacttattgtactttggcttccagtagcccagtggacataacatgaccatgactgcttagacaactacttgtatgcctcagggcatctgcttcaagataggccattaaaagctcagtgcggcgaatgagtaactgcatgaggtcttcagctaaagtctctgtacttgaatagcgcaccttctcaaagtcaaaaatgtctttgagaaataaaagaacttgattcttaaaaaagcaacataaatcatacagagaatttctaggacccaaaaagccccaggctaggacaggactgatgtgttcacaaatggcataaaaatgggcaaaaaatccatctgggatcttcatctgttgtcttttctgtttcagcaccgaccaacaacttgaagccacagctgtttctttgaaggatgagtttagccatcgattatttactacattctgtatggatgtgggtgggttttccaaatcttcaaaggagtccattaatataaaatccagaacaacatcataaaaatttagatttttcacccctctagcagcaagttccatttcagtactaccccagtgatcggtctgctctaaaaaatagatcatttcatcaaaaacatcttcaaacttctttggattctttcgtgctttcacaattaaagctgataaaattttccttccgctctcagcgaggaatatcctgttagctgattctgaaagaattacctgaaaagcctgtcgaatacagtgaagtttggcaagaaaatcactgtctcctaggcactccaacatttcagttctcagtactctggagtaaatttttccttcttcaactaaatgcatggcttcctcgtaaaatgggcagtgacaaagggactccaggctgtaggtatgccgtacttctctgtgttctgcaagctctgctgcggaagcaaaggaatccgtggatgcgatgctcaaggtgtctcgcaggccaaagtcttccacattacccttcatggtgatatctgtatctttatcaatatcatcagcaagggaattaggatcagatgccccaagggtagcttcaaactcctcttggagacgataggctctttgcagcagagcttcgagtttatggataaattcagtactaataatatcatctacattttcttcagcaatggcatctcctgcacccagtttaatggaaccacaggcttcatcttcagcctgtctattgcgaaaggtcagagcttgttcccatcgacgcaatgcctcttcaaacaattccatacccattaagtataagttctctggagtagtcacaggaatattaacaagtttaatatcatcttcatctgctttgtcccaggaattagaattgccacaagcgcagctatgacaagaattgacactctggacagaggccaaactctgtgcagaacctgaatatttactgaaaagtcctccattagcatagttacaaacttgagatcctttgtctttggtagaacttaaagataatgtcaaattctgtctgctactggaacaacttgaacctttgtctgatgctgctcttttagtgtattcaagtatgaggtgctctggttcccatggtaatatttttcctttcttctttccacgttttcttttaaagtgatgagccagaaaaattacagatatagcactcactgcagttaccacaaacaactttttagccaccggagaaaatttgatctgggagagagaatagtaccaagtcagaggaagatcaaacactcttagcgctgctgtcttcaaggaaaactgtgattcacttactgtttcttctgacatggctcctcttcaggcccgaccctgcttagcttctgagatgagacgaggtcgggggtgttcagggtggcacggccgtagaccctctggctttccgccgctccacctggcactccgagagctaacgccagcgatggagtccgcgccacccctgccccgaggcctctgccccaact

SEQ ID NO: 14995 - RNA, 2611 nt, Homo sapiens
  source 1..2611: mol_type = other RNA
gctgggattacaggcatgagccactgcaagtggcccatttaaatgttctataacaatattcagtgattacaatttctttgattcaaatacataagcaaatgcacaagcaataatgtatgcagtacatattaaacatcattactgcctaaacttgattaaacaaatgaataactttataattaaaaatatgtttctaggcaaagttaaatatattgacattagaagtaatatattcttgcatgtgtgggccacaaagaccttggctaaagtgtacattttaaaggtgcaaagcataaaaacagagcttttgagaatgacagcttcaagaagacaaaccaattaactcccaaatattggcttcaattcaagcgatatttctgtaaaatatacatttcatgacttcaattattacctaatgaatgcaaaaagccactatgactacactacacaggaattcaatgacagaacttctgtataaatacagtacagttgctcattttttagtagatttttttttcctccctgaatccacatgcatcaattctgttaactttgtaatatatgttacaaaatcaatagttaccttaaaatatttcatagcacactcaaattgtatgattcttatggtacttattgtactttggcttccagtagcccagtggacataacatgaccatgactgcttagacaactacttgtatgcctcagggcatctgcttcaagataggccattaaaagctcagtgcggcgaatgagtaactgcatgaggtcttcagctaaagtctctgtacttgaatagcgcaccttctcaaagtcaaaaatgtctttgagaaataaaagaacttgattcttaaaaaagcaacataaatcatacagagaatttctaggacccaaaaagccccaggctaggacaggactgatgtgttcacaaatggcataaaaatgggcaaaaaatccatctgggatcttcatctgttgtcttttctgtttcagcaccgaccaacaacttgaagccacagctgtttctttgaaggatgagtttagccatcgattatttactacattctgtatggatgtgggtgggttttccaaatcttcaaaggagtccattaatataaaatccagaacaacatcataaaaatttagatttttcacccctctagcagcaagttccatttcagtactaccccagtgatcggtctgctctaaaaaatagatcatttcatcaaaaacatcttcaaacttctttggattctttcgtgctttcacaattaaagctgataaaattttccttccgctctcagcgaggaatatcctgttagctgattctgaaagaattacctgaaaagcctgtcgaatacagtgaagtttggcaagaaaatcactgtctcctaggcactccaacatttcagttctcagtactctggagtaaatttttccttcttcaactaaatgcatggcttcctcgtaaaatgggcagtgacaaagggactccaggctgtaggtatgccgtacttctctgtgttctgcaagctctgctgcggaagcaaaggaatccgtggatgcgatgctcaaggtgtctcgcaggccaaagtcttccacattacccttcatggtgatatctgtatctttatcaatatcatcagcaagggaattaggatcagatgccccaagggtagcttcaaactcctcttggagacgataggctctttgcagcagagcttcgagtttatggataaattcagtactaataatatcatctacattttcttcagcaatggcatctcctgcacccagtttaatggaaccacaggcttcatcttcagcctgtctattgcgaaaggtcagagcttgttcccatcgacgcaatgcctcttcaaacaattccatacccattaagtataagttctctggagtagtcacaggaatattaacaagtttaatatcatcttcatctgctttgtcccaggaattagaattgccacaagcgcagctatgacaagaattgacactctggacagaggccaaactctgtgcagaacctgaatatttactgaaaagtcctccattagcatagttacaaacttgagatcctttgtctttggtagaacttaaagataatgtcaaattctgtctgctactggaacaacttgaacctttgtctgatgctgctcttttagtgtattcaagtatgaggtgctctggttcccatggtaatatttttcctttcttctttccacgttttcttttaaagtgatgagccagaaaaattacagatatagcactcactgcagttaccacaaacaactttttagccaccggagaaaatttgatctgggagagagaatagtaccaagtcagaggaagatcaaacactcttagcgctgctgtcttcaaggaaaactgtgattcacttactgtttcttctgacatggctcctcttctaatcaggcccgaccctgcttagcttctgagatgagacgaggtcgggggtgttcagggtggcacggccgtagaccctctggctttccgccgctccacctggcactccgagagctaacgccagcgatggagtccgcgccacccctgccccgaggcctctgccccaact

SEQ ID NO: 14996 - RNA, 2836 nt, Homo sapiens
  source 1..2836: mol_type = other RNA
gctgggattacaggcatgagccactgcaagtggcccatttaaatgttctataacaatattcagtgattacaatttctttgattcaaatacataagcaaatgcacaagcaataatgtatgcagtacatattaaacatcattactgcctaaacttgattaaacaaatgaataactttataattaaaaatatgtttctaggcaaagttaaatatattgacattagaagtaatatattcttgcatgtgtgggccacaaagaccttggctaaagtgtacattttaaaggtgcaaagcataaaaacagagcttttgagaatgacagcttcaagaagacaaaccaattaactcccaaatattggcttcaattcaagcgatatttctgtaaaatatacatttcatgacttcaattattacctaatgaatgcaaaaagccactatgactacactacacaggaattcaatgacagaacttctgtataaatacagtacagttgctcattttttagtagatttttttttcctccctgaatccacatgcatcaattctgttaactttgtaatatatgttacaaaatcaatagttaccttaaaatatttcatagcacactcaaattgtatgattcttatggtacttattgtactttggcttccagtagcccagtggacataacatgaccatgactgcttagacaactacttgtatgcctcagggcatctgcttcaagataggccattaaaagctcagtgcggcgaatgagtaactgcatgaggtcttcagctaaagtctctgtacttgaatagcgcaccttctcaaagtcaaaaatgtctttgagaaataaaagaacttgattcttaaaaaagcaacataaatcatacagagaatttctaggacccaaaaagccccaggctaggacaggactgatgtgttcacaaatggcataaaaatgggcaaaaaatccatctgggatcttcatctgttgtcttttctgtttcagcaccgaccaacaacttgaagccacagctgtttctttgaaggatgagtttagccatcgattatttactacattctgtatggatgtgggtgggttttccaaatcttcaaaggagtccattaatataaaatccagaacaacatcataaaaatttagatttttcacccctctagcagcaagttccatttcagtactaccccagtgatcggtctgctctaaaaaatagatcatttcatcaaaaacatcttcaaacttctttggattctttcgtgctttcacaattaaagctgataaaattttccttccgctctcagcgaggaatatcctgttagctgattctgaaagaattacctgaaaagcctgtcgaatacagtgaagtttggcaagaaaatcactgtctcctaggcactccaacatttcagttctcagtactctggagtaaatttttccttcttcaactaaatgcatggcttcctcgtaaaatgggcagtgacaaagggactccaggctgtaggtatgccgtacttctctgtgttctgcaagctctgctgcggaagcaaaggaatccgtggatgcgatgctcaaggtgtctcgcaggccaaagtcttccacattacccttcatggtgatatctgtatctttatcaatatcatcagcaagggaattaggatcagatgccccaagggtagcttcaaactcctcttggagacgataggctctttgcagcagagcttcgagtttatggataaattcagtactaataatatcatctacattttcttcagcaatggcatctcctgcacccagtttaatggaaccacaggcttcatcttcagcctgtctattgcgaaaggtcagagcttgttcccatcgacgcaatgcctcttcaaacaattccatacccattaagtataagttctctggagtagtcacaggaatattaacaagtttaatatcatcttcatctgctttgtcccaggaattagaattgccacaagcgcagctatgacaagaattgacactctggacagaggccaaactctgtgcagaacctgaatatttactgaaaagtcctccattagcatagttacaaacttgagatcctttgtctttggtagaacttaaagataatgtcaaattctgtctgctactggaacaacttgaacctttgtctgatgctgctcttttagtgtattcaagtatgaggtgctctggttcccatggtaatatttttcctttcttctttccacgttttcttttaaagtgatgagccagaaaaattacagatatagcactcactgcagttaccacaaacaactttttagccaccggagaaaatttgatctgggagagagaatagtaccaagtcagaggaagatcaaacactcttagcgctgctgtcttcaaggaaaactgtgattcacttactgtttcttctgacatggctcctcttctaatctccagcgcgctctcccccgaccccacagcagcccctcgcggagctctcctctgctgtcttcctttttctttgccaagaacaccagaaaagggggtccctccagctcggccgtccagacccttcctctggctcagagcagtggcgagcccatcccaattccgcgcttcctttgcaggcctccctctggcgtggggaccctcctgctttcctatgcaagtactaaccaggcccgaccctgcttagcttctgagatgagacgaggtcgggggtgttcagggtggcacggccgtagaccctctggctttccgccgctccacctggcactccgagagctaacgccagcgatggagtccgcgccacccctgccccgaggcctctgccccaact

SEQ ID NO: 14997 - RNA, 2561 nt, Homo sapiens
  source 1..2561: mol_type = other RNA
gctgggattacaggcatgagccactgcaagtggcccatttaaatgttctataacaatattcagtgattacaatttctttgattcaaatacataagcaaatgcacaagcaataatgtatgcagtacatattaaacatcattactgcctaaacttgattaaacaaatgaataactttataattaaaaatatgtttctaggcaaagttaaatatattgacattagaagtaatatattcttgcatgtgtgggccacaaagaccttggctaaagtgtacattttaaaggtgcaaagcataaaaacagagcttttgagaatgacagcttcaagaagacaaaccaattaactcccaaatattggcttcaattcaagcgatatttctgtaaaatatacatttcatgacttcaattattacctaatgaatgcaaaaagccactatgactacactacacaggaattcaatgacagaacttctgtataaatacagtacagttgctcattttttagtagatttttttttcctccctgaatccacatgcatcaattctgttaactttgtaatatatgttacaaaatcaatagttaccttaaaatatttcatagcacactcaaattgtatgattcttatggtacttattgtactttggcttccagtagcccagtggacataacatgaccatgactgcttagacaactacttgtatgcctcagggcatctgcttcaagataggccattaaaagctcagtgcggcgaatgagtaactgcatgaggtcttcagctaaagtctctgtacttgaatagcgcaccttctcaaagtcaaaaatgtctttgagaaataaaagaacttgattcttaaaaaagcaacataaatcatacagagaatttctaggacccaaaaagccccaggctaggacaggactgatgtgttcacaaatggcataaaaatgggcaaaaaatccatctgggatcttcatctgttgtcttttctgtttcagcaccgaccaacaacttgaagccacagctgtttctttgaaggatgagtttagccatcgattatttactacattctgtatggatgtgggtgggttttccaaatcttcaaaggagtccattaatataaaatccagaacaacatcataaaaatttagatttttcacccctctagcagcaagttccatttcagtactaccccagtgatcggtctgctctaaaaaatagatcatttcatcaaaaacatcttcaaacttctttggattctttcgtgctttcacaattaaagctgataaaattttccttccgctctcagcgaggaatatcctgttagctgattctgaaagaattacctgaaaagcctgtcgaatacagtgaagtttggcaagaaaatcactgtctcctaggcactccaacatttcagttctcagtactctggagtaaatttttccttcttcaactaaatgcatggcttcctcgtaaaatgggcagtgacaaagggactccaggctgtaggtatgccgtacttctctgtgttctgcaagctctgctgcggaagcaaaggaatccgtggatgcgatgctcaaggtgtctcgcaggccaaagtcttccacattacccttcatggtgatatctgtatctttatcaatatcatcagcaagggaattaggatcagatgccccaagggtagcttcaaactcctcttggagacgataggctctttgcagcagagcttcgagtttatggataaattcagtactaataatatcatctacattttcttcagcaatggcatctcctgcacccagtttaatggaaccacaggcttcatcttcagcctgtctattgcgaaaggtcagagcttgttcccatcgacgcaatgcctcttcaaacaattccatacccattaagtataagttctctggagtagtcacaggaatattaacaagtttaatatcatcttcatctgctttgtcccaggaattagaattgccacaagcgcagctatgacaagaattgacactctggacagaggccaaactctgtgcagaacctgaatatttactgaaaagtcctccattagcatagttacaaacttgagatcctttgtctttggtagaacttaaagataatgtcaaattctgtctgctactggaacaacttgaacctttgtctgatgctgctcttttagtgtattcaagtatgaggtgctctggttcccatggtaatatttttcctttcttctttccacgttttcttttaaagtgatgagccagaaaaattacagatatagcactcactgcagttaccacaaacaactttttagccaccggagaaaatttgatctgggagagagaatagtaccaagtcagaggaagatcaaacactcttagcgctgctgtcttcaaggaaaactgtgattcacttactgtttcttctgacatggctcctcttctaatctggagctccaggccaggtacagctggcctgcccacgccagcttcccagctgatgcctggcgctgagcagcagtctgacatggagaaggcggagtccttccggggtcaggagt

SEQ ID NO: 14998 - RNA, 1741 nt, Homo sapiens
  source 1..1741: mol_type = other RNA
gctgggattacaggcatgagccactgcacaatgacagcaacaccatagcaattaaagtccattccgcaggtttgtgtataatatttctatttgttaacctgaaagttcgaacaagatttttaagttgtgtgtaaatatctcccaatgtaatctgaagaggaaccagaagcccaggcaacactttactcaacttttcaagtacgatgcgttttctaatctggttctgggaacttgagtctatcagtggaaaggtggaatcatgctcttctgagtcttgtgatttggtggtttcttcacccaaaacataccgtcctctgtaaaactccctgatcctcagatttaacttttcagtttcttttttcaaattctcgtaacttggcagtggtttaatggctgtacctgagcccctaaaaggtaaagactcatccaagctgttctgagattccctccaggcagggaaatgactatctggatctgagattatgtcatcttcatcaagttcttctttaaccagagaggcttcgggtttcagacacacagaagcataattctggccatacaaaaacctcaatgtttcttctgtcttccactcaatcaaagtctccttcaaaactttaagtaagtttctctttccaacttcaggacacacctgcactgaactagacactgacctagacacttggtttgatttggcaaattttctcttaaaatgctctgcacttttcttacttatgcctactagagttatttctgacctactgtattcactttcagaattttctgacgcttttaatctttcaggcaaagtgctatttgaagaactctgagtatttactttctgtaaaggaagttcacatgtagcatctttctcctgactatctaatttgcaatcgcctaactgctcagtgacatctactactgtctgttctttgtctttgtgtttggagttagctttgtgaccagctttctttttcattatgcttttttggtgcagctgtggtctaatatttgttgaatttggtctgtttcctggtagaatggaggaaacaaagtcttgctcattgtcactgctactatcactgtgagtgctagaagaactagattcatattgcttttcaaagtggctaggattgtcgatatctgatgttttaatggctttactgcataactgtacttcttctccagaatggccactttgttcttcctttagcagttgaaaatcaggatgcctctcttcttctcgaacccatactggagttttgggaatttgtgcttcaaaaaacttagatgcttgataacaaaaattgctgcaaaaagactttctttcagtaatatcatagactttattggttttggtagaaattttatatttctgttttggtacaattcccagcttcttctgacataaaggataaccacagagtttgacaatagaacgttcatccacgacatcactgtagtgagcaggtgtaatgaacctcccacactccattaggaactcttctgtaatattctcctctaaaagctgttcaacaatatgtagagcttttctctcaaattcaatcttctttctcacagctgcttctagttcagctttccttttagaagcatcttcttgtttcaaagtacttgtctgtttagtacctgcggcttttcgagagcagcggggagccccggccttgcggccggcagaagacggcccagcgaagtccgccatgggggagagtagtctgccggacgg

SEQ ID NO: 14999 - RNA, 3807 nt, Homo sapiens
  source 1..3807: mol_type = other RNA
gctgggattacaggcatgagccactgcacacagcccaaagtatttatcctttattttgtggttatatgttgggaaagaagaacgtggaaaagaagtgaactaacaaattttcaggtattaatattacaattcagtacattctgacaaaaagaattatttcctatgaaattacacccattggctgggtgcagtggttcacggctgcaatcccagcactttgggaggccaaggtgggaggatcacttgaggccaggaattaaagactaccctgggcaacacagcaagaccctgtctctacaaaaaaagaaaaagaaaaaaaaattacacccactgagaaacagaatgtgtaacagtaaaacaacagagcagcttccatgtgattttgataggaaagctttaattggtgactaagctttgtaaaaaggatgtaaacaggggaaagaatgaaaagaataagatttatctacataatgaagtttgactttttacagtaaataaaatacctatttattaatatttccaaatattaattagatttaataatactatatatttgttacaatgccttcatcagaaaatttaataattaagaagatacttgaagttcattcaaatggcacttgcagaaatgcaacttaatttctagttctatcatatctgtctccaaaatggacatatatgacagcaaaaacaaaattctctataaatctctccattagttacattactatgtaactaaaatagctagttctataataaaaggattttatgtgccaaatcctgaccaagagagaaataaagtcattattgctgcaaatccaaatggaacctaacccaaatgtagggaggggcaaataaagtgaaaacatgttggaaggtggggtcaactgccttaggacaattctacatccagcttgacactactcacgacttactcctcctcactgtttcttccaagaaagtctaagcatgtgaaactgtccttgttgctccctgtggatctctggctgagtggctaaagggcaatcctgagcatagacacactctcctcccttctatcagctgtcccccacacatactcacagggatgagtagactgaacaaacatcaaaaagacgcaggaacaaataaaataccccaataaaggcaattcttaagtggtcaataaattagggcacttcttcaaattaagctctgtcaattaggcacttaataaaaacaaaagacatttatacaagcatctaaataacaaagaaagataaagaacaagagaaagacaagatttatgttaactaccagcatgttatacttcagccagaagtttttgaaagaaacgttatttgagaaggaaaataagtagtatttttctgtttcttaaaaatcaatattctttctagttcattaactaaaattagtttttcagtgttttcaacatagaaagaatgctcagattttggttgaacaaggaaaaattaaggcagtgtctttaagaccagtaaaggaaagcattaactatctcataagcttatctgagagggacatattaagctcatatttggatataatattaggaaattatggctttaaacataaaatattaatgtttcaaaattccacattttctcagttattctttctttttagctatatgtacttcaaatagcccacttaaagaattaaagaaatacgtttcacataattttggaacaatatgtgcatggtacttgacccagaactattagcttggatggtaaatcattatgttcctatgtaccactgacccagtataaaaaggaagaggacccataactgtcaaaatgtggttggaaatgactaatgtcctttggaatttgctacaaaatagaagatataaagttttgaggtattgctgccttaccatggtttaggggaaaaaaataagagttttttgttccgttttgtttttttaaaagcaatgcttcttaagttatgaagcttatttaaaattttctcctcttagtcattgtcatatgggttatccctgagcttcatctcatctgcacgtcacataaaccagctacctatggttttgatcatttcatttagtgttatgtcttgttataccaattcatggagcgtttcactgctttggcccagttttccagactcatttcatattcttgacatttcttctgtggcttgaaaaccacttcactttgtctcagtttctttagttcctccttgtcagtccaaaacccaacagcaaggccagctagagaagctgcacccaggcatgacatgtcaatgtcggcaggtctgtctatattctcattaatcaggtctgaagtcatctgcatgacaaaaccattcttacaaactcctccatctgcccggatttttcttacaggaatatgaatctctttcttcatcatctcatataactgtttgtttctgaaagctattgactccaatattgctcgtacaagatggtatttactggtagaaggcttcaaacccataaaagaggcacatgcccaggggtcatttaatggagcctgtaatccactaaaagatggaacaaaacaaactccttcagaatcctccaaacttttggccattttttcagtctcagcagcatctgtgaaaaggtctaactgctgagcccattttatggcagtaccagtgtctcctgcattgctttcagctaagcatacgacttcttgcccaatcttccacccaattaatggataaaagcctccagtagtctgttgaaggctatttccagtgttaatatccaaaaatgtcccagttcccatggttaatttcacatcacctgtctggaagcagcactctccaaacatggctgattgctggtcagcaaccaaggcaactattggtataggcacaccaaatatctcttcatccactgatccaaaattgtggcttgtgtccctcacaggaggtaggagagaaagtggtatcgaaattagagaggtaatcatcccactccaacacatcttatatgggtcaaaaagtccagttgtactagcatttgaaaaatctgtggcatatacagaaccttttgtgagcttatataacaaccaggtatcaatagtcccaaagcagcaattttcttcttcaactgccttttgcacctcagtcaagttctgtaaaatccagaccaatctcaaagaagtctgctgggttgtgaaagtgaacaaactggctgtaaaaagtcgtttacttctagtgaaaaagtgaagcactcggcaagaactgtgaaatatcttcataagaagagaattattccaagattttacaagttcaacagctcttaagtcttgccaacttataaagttgtgaaaatgatttcctgttttcttgttccacgtaataaaagttgctctctgtgttgaaatgccaagaccaacaatttgattcatctgtattcctgcagctttgactgcttcttttattacggcaacaaattgaatccaaagaacatcaggatcaatttctacccagccaatttgaggataaagattttctaccttctgcacgctggagccgcagacccgcgccgcccggtcatagacgtggcagcggatcacagaactgcccacatccagccccagcacgaagccggggtaccgcggctcctgcgctctctgctccgggtccgtgagcagccccgacatcccgatcccgcacgcctctccgctacagccgcctacccagagggcgcgctacaaatcccaatgctccagagtccccgggcggcccaacccgggccccaacccggctcagccggagagcctagagaggcct

SEQ ID NO: 15000 - RNA, 4890 nt, Homo sapiens
  source 1..4890: mol_type = other RNA
gctgggattacaggcatgagccactgcacacagcccaaagtatttatcctttattttgtggttatatgttgggaaagaagaacgtggaaaagaagtgaactaacaaattttcaggtattaatattacaattcagtacattctgacaaaaagaattatttcctatgaaattacacccattggctgggtgcagtggttcacggctgcaatcccagcactttgggaggccaaggtgggaggatcacttgaggccaggaattaaagactaccctgggcaacacagcaagaccctgtctctacaaaaaaagaaaaagaaaaaaaaattacacccactgagaaacagaatgtgtaacagtaaaacaacagagcagcttccatgtgattttgataggaaagctttaattggtgactaagctttgtaaaaaggatgtaaacaggggaaagaatgaaaagaataagatttatctacataatgaagtttgactttttacagtaaataaaatacctatttattaatatttccaaatattaattagatttaataatactatatatttgttacaatgccttcatcagaaaatttaataattaagaagatacttgaagttcattcaaatggcacttgcagaaatgcaacttaatttctagttctatcatatctgtctccaaaatggacatatatgacagcaaaaacaaaattctctataaatctctccattagttacattactatgtaactaaaatagctagttctataataaaaggattttatgtgccaaatcctgaccaagagagaaataaagtcattattgctgcaaatccaaatggaacctaacccaaatgtagggaggggcaaataaagtgaaaacatgttggaaggtggggtcaactgccttaggacaattctacatccagcttgacactactcacgacttactcctcctcactgtttcttccaagaaagtctaagcatgtgaaactgtccttgttgctccctgtggatctctggctgagtggctaaagggcaatcctgagcatagacacactctcctcccttctatcagctgtcccccacacatactcacagggatgagtagactgaacaaacatcaaaaagacgcaggaacaaataaaataccccaataaaggcaattcttaagtggtcaataaattagggcacttcttcaaattaagctctgtcaattaggcacttaataaaaacaaaagacatttatacaagcatctaaataacaaagaaagataaagaacaagagaaagacaagatttatgttaactaccagcatgttatacttcagccagaagtttttgaaagaaacgttatttgagaaggaaaataagtagtatttttctgtttcttaaaaatcaatattctttctagttcattaactaaaattagtttttcagtgttttcaacatagaaagaatgctcagattttggttgaacaaggaaaaattaaggcagtgtctttaagaccagtaaaggaaagcattaactatctcataagcttatctgagagggacatattaagctcatatttggatataatattaggaaattatggctttaaacataaaatattaatgtttcaaaattccacattttctcagttattctttctttttagctatatgtacttcaaatagcccacttaaagaattaaagaaatacgtttcacataattttggaacaatatgtgcatggtacttgacccagaactattagcttggatggtaaatcattatgttcctatgtaccactgacccagtataaaaaggaagaggacccataactgtcaaaatgtggttggaaatgactaatgtcctttggaatttgctacaaaatagaagatataaagttttgaggtattgctgccttaccatggtttaggggaaaaaaataagagttttttgttccgttttgtttttttaaaagcaatgcttcttaagttatgaagcttatttaaaattttctcctcttagtcattgtcatatgggttatccctgagcttcatctcatctgcacgtcacataaaccagctacctatggttttgatcatttcatttagtgttatgtcttgttataccaattcatggagcgtttcactgctttggcccagttttccagactcatttcatattcttgacatttcttctgtggcttgaaaaccacttcactttgtctcagtttctttagttcctccttgtcagtccaaaacccaacagcaaggccagctagagaagctgcacccaggcatgacatgtcaatgtcggcaggtctgtctatattctcattaatcaggtctgaagtcatctgcatgacaaaaccattcttacaaactcctccatctgcccggatttttcttacaggaatatgaatctctttcttcatcatctcatataactgtttgtttctgaaagctattgactccaatattgctcgtacaagatggtatttactggtagaaggcttcaaacccataaaagaggcacatgcccaggggtcatttaatggagcctgtaatccactaaaagatggaacaaaacaaactccttcagaatcctccaaacttttggccattttttcagtctcagcagcatctgtgaaaaggtctaactgctgagcccattttatggcagtaccagtgtctcctgcattgctttcagctaagcatacgacttcttgcccaatcttccacccaattaatggataaaagcctccagtagtctgttgaaggctatttccagtgttaatatccaaaaatgtcccagttcccatggttaatttcacatcacctgtctggaagcagcactctccaaacatggctgattgctggtcagcaacctatagtcctagctactcaggaggctgaggcagaagagtcacttgaacccgagaggcggaggtcacagtgagccatcggtgagatcatgccattgcactccagtctgggagacaagagtgaaactccatctcaaaaacaacaacaacaacaacaactcatttaaagaaccctctgtcactaattggtaactcttccagccataccttaatctaaccctgcacctatgcctagattgaataagaccgatcctctctaaatgataatgattttgtaacttggaaattaaattccctttccctcagctgctcccccagctactgtggagactgcacatcttgcaacaggtggtctctacctcctgcttaagctgccacaggaaatcaaaggcaatgtgaaaggactcttaaaaatcaaaaacaggcttggcacagtgactcatgcctgtagtcccagcactttgggaggcaaaggtggcagaaggccccagtctaggagttcgagatcagccaggggaacacagcaaaatcctatgtctaccaaaaatacaaaaaattagccaggtgtcgtggcacacacctgtggtcttggctacttgggaggctggggtggaagaatcacctgagcccaggaagccgaggctgcagtgaggcatgattataccactgcactccagcctgagtgacagagtgagaccctgtctcaaaaaaaaaaaaaaaaatcaaaaatggcaaatatttcattattctacaaacttatttactggtagatgatggctaaggactttattaaatgtacatacaactttctctgctagtttaagttgccctaacactgtttgtggttacacattatcaaacagaacataaatattcgccccatcactgtgttttgtctcagagtaccaaatgtaaactaaataccactcagaattaaaaaaaattttttttaatttaagttttctgataaacaatatacaagcaagtcagaaaaggttataaagtacttccatgatagaatactggctcaatggtccccttcccaaaaatatagcagatattctggtcatatccagggacctttaacaaggcaactattggtataggcacaccaaatatctcttcatccactgatccaaaattgtggcttgtgtccctcacaggaggtaggagagaaagtggtatcgaaattagagaggtaatcatcccactccaacacatcttatatgggtcaaaaagtccagttgtactagcatttgaaaaatctgtggcatatacagaaccttttgtgagcttatataacaaccaggtatcaatagtcccaaagcagcaattttcttcttcaactgccttttgcacctcagtcaagttctgtaaaatccagaccaatctcaaagaagtctgctgggttgtgaaagtgaacaaactggctgtaaaaagtcgtttacttctagtgaaaaagtgaagcactcggcaagaactgtgaaatatcttcataagaagagaattattccaagattttacaagttcaacagctcttaagtcttgccaacttataaagttgtgaaaatgatttcctgttttcttgttccacgtaataaaagttgctctctgtgttgaaatgccaagaccaacaatttgattcatctgtattcctgcagctttgactgcttcttttattacggcaacaaattgaatccaaagaacatcaggatcaatttctacccagccaatttgaggataaagattttctaccttctgcacgctggagccgcagacccgcgccgcccggtcatagacgtggcagcggatcacagaactgcccacatccagccccagcacgaagccggggtaccgcggctcctgcgctctctgctccgggtccgtgagcagccccgacatcccgatcccgcacgcctctccgctacagccgcctacccagagggcgcgctacaaatcccaatgctccagagtccccgggcggcccaacccgggccccaacccggctcagccggagagcctagagaggcct

SEQ ID NO: 15001 - RNA, 3215 nt, Homo sapiens
  source 1..3215: mol_type = other RNA
gctgggattacaggcatgagccactgcacacagccccttttatactctttaagcaagtttagaattagtgattatcagtcacttatagcaggggcacagcttgaagaaacagacaaaatgcagaagaagaggtcaagcattactggaattaaatcaccactgttaattcctaatgcagttggtccaaataaatcacaagttttattatccagctctctcctactggcaaagcaaaggcagggaagacagttattgatgagcacatcttccttcatgcctcaagaaactcaaaattccatgcctcctaacacaagtgcaagaatgacatgtgcacaactgggggaggtgtgtgctctgaggagagacaccaggagacacagggctccatctagtaccaagagatgcatgcctgcagtctcagtggtgagatgtcgtctttttaaacatttcaatctcagtgatgagaggttgtcttttcaaccagtgaaaggtaatctagcagaacagaaaacatgccacagaaagggcattgcaggcaggcagcgtgagtcagaccccaggtggagctgggaaatttgcccagacccaaaggcctatccacctgtgccatccaaatgtggcaaaatgccaaccttgcatctgaggcaaccatttttgtccaccactccttgccacacaatagggtttggggagctcttggctttcccatactcaactatgagagccgggaatattttcatgataattgagatttcttcgtacagtattcagaaagagaaagttgaattgactgaggtcaagatggcattcttctgagcattctactgttgtccttagctttgttcacattaattgtagcctgggcacagacttcactgcggtttctagcatgggaggtgactatatgacatgtattgctggctgtgaatgagccaggatctctgaaccctgcctgtgccctgaggcacacaagaccttcccaagcctttagctcacattgacccaaccctcttctacaaacacctgtactctagtactctagtctttgattaaatgtaatctcatcttactccattctttttttaaaagtgtgattattctttcacagctagaatataggttccttaaggggcaaggactacattttatgattctttgtttgtgcccacagaactacacaccactgtctgacctagccttgtattttttttcttttagacagagtcttgctctgtcacccaggctgaagtgcagtggcacagtattagcccactgctgccttgacctccagtgctcaaggaatcctcctgcctcggccttctgagtagctggaactacaggcgcatgccatcatgcccagctaattttgtaaattatttgtggaggccaggtcttgctatgcttcccaggctgagcttgaactcctgagcacaagcgattctcccacctcggccttccaaagtgctgggattacaggcacaagccaccgtgcctgaccatagccctgtctctttaagtaatcccagaaattcaagaacagagagctctggacatcccagttctttttaccacaaaactcttggatccactaactacctaactcttaatctccagcttctcctacaacaacaagcttcatccttgtccaatatcacctctaaacttagaaatttgcccctcactattcatcccattggatctgaaatggacttggcttttttggtttggcctcctgttgccccctggctctatccattctgggtacctactccaggagatcaagcctacactcacaagacccaacctgtgattagcaagatgcacaaggccaccactgagatcatctgtggttcctgttggagagaactgaagaaactgggcatgctacaatcatcatgagtgcagtcagaaggaggacataattctgccaagccacctgctgcttctcctaccaccagcagcagcagccccttcccctggatgttcattcacctctcaggtaagcaagaaggaatagtccgacttggctcaccaccacctgaagcaacatttgatttatcagggaaagcaaaaatgaattgaggaatcaagacatgaaagtagaaaagactgaaagctccctgaaggcaagcattatgtgtgtcttattcataattgcatcttcaggtcatgccagtgtctaacctgttagtaggttctcaataaatttgtggaaataattagaaatagaatgtctgtcttttatctccatcatactgttttttgagggaattaagtcaataaacgtgttattgacataggcagacacattttagatacttgtgtgttaagtttcactattgatgtagataaaatgctagtttcactattgatgtagataaaattctatggcacttgcactccagcctgggcaacaagagtgaaactccatatcaaaataaaaaaaaatgctatggcacacagacagcactttatggagtcaattattctgttcaaattgggagcctacaggggaaaaagtagcatttgagctgggtcttgaaataggaaacagccatttcaaaggaaagtataatgatgagaataaaattggcctcacaattaagactctttgagggacagcctcctcctcagaaaagagctgctggtgcccctctggcagacagagctgattgctgacaacagtcctctatcacagatgctccacaacacaccggagatgcccgagaggaaccccgggacataagtggggagcacatggcttatgataattttagctctcacccaaggtctgctaatggctcatgtagctcagcctggaagatgcctcagaacactggtcagttctagggctccctcaaggagttctgggctattcttggtgggccctggggatttaagtctgactatgtgagtcagaatgcagatggaaaagtctggtgccttagagagggcctggaaccagctgggtgtggtttttcgcacatgtaatcccagcactttgtgcgaatcacttgaggccaggagttccagaccagcctgggcaacagggcaaaaccccatctctactaaaaatacccaaagtagccaagtgtggtggcacgtgcctgtagttccagctactcaggaggctgaggcatgagaatcgcttgaacctgagaggtggaggttgtggtgagctgagataccaccactgcactccagcctgggcaaca

SEQ ID NO: 15002 - RNA, 442 nt, Homo sapiens
  source 1..442: mol_type = other RNA
gctgggattacaggcatgagccactgcacactgcttacgcttgatctcagcacaaccaggctaggagctcttcctgtcccattggtgtctatgcagcacactcctcagcacactgcagatacctgataaatgctgataaccacttgccaggtagtcctccaccatcctttctacctttgtcttttcttcaaaagggcagattggttccctggaaaaaaacccacgggacaaataaatggctgccattctctgaagctgatggtgtgatgatgtgcatcccttccttgatgccaagatcacctcaggccagcttatgaatctaggtggatagaggcaatctccattcctctttgtacagggttatttgcggtccacagcctgggcagactccaccaccataaaggcgaaaccgcactgacggagaggagccagcgccggaaaa

SEQ ID NO: 15003 - RNA, 437 nt, Homo sapiens
  source 1..437: mol_type = other RNA
gctgggattacaggcatgagccactgcacactgcttacgcttgatctcagcacaaccaggctaggagctcttcctgtcccattggtgtctatgcagcacactcctcagcacactgcagatacctgataaccacttgccaggtagtcctccaccatcctttctacctttgtcttttcttcaaaagggcagattggttcccacgggacaaataaatggctgccattctctgaagctgatggtgtgatgatgtgcatcccttccttgatgccaagatcacctcaggccagcttatgaatctaggtggatagaggcaatctccattcctctttgtacagggttatttgcggtccacagcctgggcagactccaccaccataaaggcgaaaccgcactgacggagaggagccagcgccggaaaagatggcggtggtgcgctg

SEQ ID NO: 15004 - RNA, 433 nt, Homo sapiens
  source 1..433: mol_type = other RNA
gctgggattacaggcatgagccactgcacactgcttacgcttgatctcagcacaaccaggctaggagctcttcctgtcccattggtgtctatgcagcacactcctcagcacactgcagatacctgataaccacttgccaggtagtcctccaccatcctttctacctttgtcttttcttcaaaagggcagattggttccctggaaaaaaacccacgggacaaataaatggctgccattctctgaagctgatggtgtgatgatgtgcatcccttccttgatgccaagatcacctcaggccagcttatgaatctaggtggatagaggcaatctccattcctctttgtacagggttatttgcggtccacagcctgggcagactccaccaccataaaggcgaaaccgcactgacggagaggagccagcgccggaaaag

SEQ ID NO: 15005 - RNA, 450 nt, Homo sapiens
  source 1..450: mol_type = other RNA
gctgggattacaggcatgagccactgcacactgcttacgcttgatctcagcacaaccaggctaggagctcttcctgtcccattggtgtctatgcagcacactcctcagcacactgcagatacctgataaccacttgccaggtagtcctccaccatcctttctacctttgtcttttcttcaaaagggcagattggttccctggaaaaaaacccacgggacaaataaatggctgccattctctgaagctgatggtgtgatgatgtgcatcccttccttgatgccaagatcacctcaggccagcttatgaatctaggtggatagaggcaatctccattcctctttgtacagggttatttgcggtccacagcctgggcagactccaccaccataaaggcgaaaccgcactgacggagaggagccagcgccggaaaagatggcggtggtgcgctg

SEQ ID NO: 15006 - RNA, 2306 nt, Homo sapiens
  source 1..2306: mol_type = other RNA
gctgggattacaggcatgagccactgcaccaagccaagaattagaagatacttctaaaagatattttaaaagaaccaatggaaacttagagatgataaaacccaagcaggataaacaaagaaaaccacccaaggcacatcttaaattgcagaaaactagtgacaaatcttagaagcagtcagattaaacaaggcgtatgacatacaggcacaaagaagccaaggatttcttgtcccctcctccccctccacccaaaaaaaaaagccagaagaaaatggaacatctttaaggtggtaaaagaaaaaatactgtcaatctagaactgtatatgcagcaatatagcctttaaaaactgaggtgatgtaaaagcattttcagacaaaagctgcatgaattatgaccagcagatttgcagtccaggaactgttataggatgctcttcagatgaaaggaaaatgataccagaggcaaactttataaaaggaatgaaaagttctataaatactttttttttttgagacggagtttcactcttgtcacccaggctggagtgcaatggtgcgatcttggctcactgcaacctctgccctctgggttcaagcgattttcctgcctcagcctcccgagtagctgggattacaggcacgtgccaccacgcctggctaatttgtgtatttttagtggagacagggtttcaccatgttggtcaggctggtctcgaattcctgacctcatgatctgcctcctggaggtggcaataccttagatgcgagaaggatctaaatctgcaggaagatataccatattcatgggttgaggactcaatattgttatgatttataagtccttgttatggactgaattgtggcccctgcctaccaaattcctatgtcgaagccctaacctccaatgtgactttatttggagatgaggcctttaaagaggggaacgttaaatgagattctagggatagagccctcatctgataggactgatgtcctcgtaagatgaagagactcctgagatgtgtgtgcacaggaggaagtccaccacgagaggtacacagtgagaagggggccgtctgcaagccgggaagagaggcctcaccgggagccaaccctgccagcatctcctctagaaccgtgaagaaataaatgtccattgtttaaacccgctagtccgtggtcttctgttacggcagccgagcaaactaataccgtccccaaatagggatgataggttcactgcagttccagtgacaatcccagcacactttttacagtgttcagcagacactgatgagttgattttacaacgtgcgtggaaatgcaacagacctaggaccaccaagaccattctgaaaaagcagaactggaggactcatcataccccctggtttcaagatttgccttaaaacggcaatagttaagataatgtggtgttaggacaaggatagacctaaaggccagtctaacagaaggtagtgtccagaaataaaccccaacttaacacagccaggaattttttctaatggagccaacgttattcaacgggataagaaaggtctttttaacaaatggtgttagaacaatagagtaaacatatgggatggtggggaatcatcctcaggctcttcctcacacaacacacacaagttaagagatgtgttacagacttaaaagccgaaactgaatcttctggaagatatattattgcaaccctggaataggcagattttttttttagaacatagaaaagcattagccacaaaagaaagaataaattgaactgcactaaaacttaaaaaatctgctgatcaaatgacagtcaataaagtataaatacacatatccctcaaaggatttgtatgtgaggaatccctacaaatcagtaagataatgcaatttaaaatgagcaatagacaaatatgtaaattacaatcagcgcatcaggtcaaaatcagacatcaaagaaaagcaagggaaaatcacactgtggccccagtgcacacccacctgaatgactaacctgacactaccaagtgttgacaacaatgtggggccactggaatcctcacactgctgctggagtgtaaaacactaccaccaactttggataaatctttggcagttgtggtacagttaaacataaacacaccatgactcagttccttctacttccagagaattacttcccaaagaaatgaaaataatgtctgcaagaagactggcacacaaatgttcataagaggtttacttattatagccccaaatagggaacaacccagatgtctatcaagagaatgg

SEQ ID NO: 15007 - RNA, 1764 nt, Homo sapiens
  source 1..1764: mol_type = other RNA
gctgggattacaggcatgagccactgcaccaggccacatctaccttttggagagtagcttctacctgtctggaacattgggatgtctgattggctataaaatccaagaccccaaatatggattagcttcagattccatacaactagtatcccaccaccaccaagagtgagtccccaggaaccccactggaatctttcctcagtggaaactagcttatctttgtctatttcaaagctagtgctaatttcagttattgtctattttggcctccaatcataagagctgttaggagaatttttaggtgaaactatttgaaaggcagaagtgagccagaccaaacagcaaggtctgagtcaacgaggaggcagaatgaaatgcgcagattatccacagacccagtataggcccttgggagttgaaaaacagggccacatagttgcatttgagcaggggtcagttagatttgttcattaataaacctacacagctcctgaacaaaatccactgggaaattgacctttttgtgctcgccctgtagtatgttgtaagggtgtataacacatttagtaaaaagagaccctgttgaatttaatctggtgatattatacaagcaattacttgtactcacataggtaattcccgtaacttgagtgcatgatgcctgaaagcacaatatatcttttgcaggcatcacttggactggttttctatattttggtattgatcaggttattaattgaaacagttaaggccaggcatggtggctcacgcctgtaatcccagaactttgggagaccgaggctggtggatcacttgaggcaaggaggttcgagaccagcctggccaacatagcaaaatctagtctctactaaaaattcaaaaatcagctggatgcggtggtgcatgcctagagtcccagctacttgggtggctgaggcaggagaattgcttgaaccttggaggtggaggctgtagtgagccaagataaggccactgcactccaacctaggcaacagagtgagactgcctcagaaaaaaaaaaaaaaaggaaaagttaaagtgttgcttttagtgagtgcaggaaaacaagtagcaatggtgttcagaatatcaaggatagctttctatccttcccttggaattttggggtgactctcattggcaacatggagaggcattggcattagcggaattgtttccttatttttttggcaataaaaacaaacccaataagccacaaactctggttctgtgctagagcatatgctcaagctaaagccatccactgattatcgtcccatggatttttctgtagggaaaaagaaagaattagggcaacaggaaatgcggagaaaagaaaaaatgtaaggctttcatgatgatacagaagtcttgatctgtgatcttgggaaagctgtccacagctagaatgcccgctgctctggagagatatttccttagacagctttaccttaaagtctccagcaggtgtacagttccaggagtctgaagaggcccttctgagttgtgaggtgtggacccaagtttcaaggccctgaagcttcactgcagtgtaggtgttgagaagatctcagcacggtcccttccaaagagttgtcaagagcagcctttctctgatgtcatttccagaagacacaatctccaggttctagactgtggaaggtttgattatcctcagttggtggatcttgaaaagcttcctttatctgtagtcccagctactcgggaggctgatgcaggaga

SEQ ID NO: 15008 - RNA, 3615 nt, Homo sapiens
  source 1..3615: mol_type = other RNA
gctgggattacaggcatgagccactgcacccagcagacccaggacaatatttcaaggaaatattactatgttaataaaaagagtgtcactgggagcgatggcacttatgacccttgcatgaaaggacctccatatttcagctacgtcagtgatgatctccagtgcggatggagacagtggcacacagagcgcccctaacatcagtgcaaaggaagaggcacaattacattgcaaatggtgagattcctactccagtgttccttctcttgacctactctagctctcaaaaactcgacacaatgagactccttgagttccacctgatgttctcaaattcttctttcccagtgacgaactgtgctgcactaaattcatagtcactggactccccaggaaaccaaaaatctcaggatgatgacatttgagtaaaaaggttccaggtgacaactcgtgtatgaaaagtggtgactgcaccttcctttgcaacaagaggcttttagcaattcttcaagcaccaaaccatgcactgaacatctgcataagttctgggttatcatggttatgacttcctctgttctcaaagacattcatccatgtttacatgggttgttaggctatttctttactcaaatgactcttcttttcctgggatgctccaagtattcaaagaagatcacggcactttgaggatggacacagagaatcaaacatgatagatctccctcgctctgcatccagaaaggcccatcctttgtctggctcaggactcaggggaagtgcgagatggaagctgttcgaagatcatcatcagacttttctgctctctcttgacacaacagcctcaagcccccacacgtcactggctgctactgaaacatgctcacaagaaatcctgaaccatgctttgagccagagttaccaaaatggacgaggtatttctcaggagaaactgtcgccttcatagattcatgaacagggacaggaccgccatgaacgatctgtctgaaaatgccctcccactttcctctaagggaaactgttcttggacaatcacttacgatgtctttccttaaaggttattctgtgctgaaagtattgcaagcatcccatcatgattaatggaaggcagagaagccacttttaaagagataaaatagaaccacagtgtaagtcagcaaaacggtcaagtaaatcgtgatgcctctgcttatcatggagctgcattaaagagaaattaactccagaggtcaagacaatactatagtgtagggagagaattattgttccttcctgaagacttttctccctgaggcaagacagcacataccatagattaaactttcatcagcagatcttggaattccatcagtctttcattactgactggctcagagaatcccctactagatgtcatcaggaaactctacttcttccagactgagaccccacctaatcactccggccattgtcgcggcccacgccccacacgcggatgctgacgatgggctgcgagtgcagcacgctgcggtccatggggtccaccaggctgagcatgtcattctccaggatcaggtacatgtctttcccctctccccaaatcccgactgtgtctcggatgtcatttttgcagtaggaaagttgcctgatgcagttgttgaccgcaacactacttttaccgggggcgaggtcctcttctgccatctctacccatcccagagaacgcacagcaaaacacttggcttctgggtcactgttgatactacaagaatcatcatcatcagggtgtggggcatttctgagtttcaaagatgcatagcgtagggttgctccttcaaactcttttaaactggggtccgggttaacagtggctgcatgcaaatccttccaaatgtcactattaatctttcccccattcagaacagcaaaatcactccatggctgtttctcgttctctggggtgggagatggcgttacagaactaagtgaccctttcctagaaccctggagatctgctgggatggagacgggccgttcccactgagtcgttcctgttgggatgtgccaataataggtcccggcaatgtcactgactcttttccagccaggcggcaaatctggatcagtctgaaatgagtgatcactccatatatctgctgtttcatccggggagctgggtgaggcactgtcttgggacaacgttgtccagctggactcctcatcgctcggtgccaggttctggatccggtgcagtgcacagtcggttttggcccctgttttcggatgatccttcttggtttctgggctggatgacactgtggctacttggccgtcttcagggctggactggggtctgtttggtttctgcagcagcaaatcgccattcccaatgatggtggaggcctggccctggactggctgggatttctcttccgcagtcccatggtgattgcctcggttctgctctagttctctggctgaggtttccagatctgcatagtaatttaggaagctcttagttctcctgggctgggagggtaaaatctcacagctcgaggaatcctgtgggtggggctctttaccctctaacttctcagaagttatgttgatgactgcagtggggctcaggtttttgttggggtcctgctgcccttgctctgcagccttacggagctggttctccccatttttcaccagcttgatgttggcagagccatttcccagcaggggctgtgcagctggatccgagaggcccatggccgcctggatgttagttagtgcatattttttcctgcatttgggaggtgtgctgttcttggtttctgtgtgttttatttcagcgttcaacagttcattgtgggaggatcggaggttaagggtgtttggtggtgtggctgggctgttccgatttgtgacgtctgtagttccgctgctggccataaacactgccaaggtgtcaacacctgagtcagctggaagtacttctgacatggatcaccaggcgtcagcaatggtgcaggaaataggttataatttgaaatatgagctgcctggacaacagtgagcccatagcgacagtcaacacattggcagaggcctcggcagttcccaagtcctcaggaaagactgagatggttagttttcccaggtctttggtacaaagctcagaaggcaagctcctttttttccccacaaagtctgttaattaatagcaagcacccaaggaggtcaggcagcccaaagagatcgatctgattttgcttaaattattgtcagcctcagcttttcacaggagctttcttttatggattttccatccagcaaatgtttctgttccacggctgggcagatccgaccacagcatgcttggctacagaccacagcagctcacccacagcaactccaaccagtggtgcgcgcggcgctcgcctcggctccggcgcccagcggctctgctccagtctcgcccttcccggagcgcccagatcagatgcggttacagcgcactagcttcctacttgagaccagaacgggctccggcaactgagcatgctcagtgccgttccgcgagtcccgcgcagggagcggcgctgacgagattccacttctccaggcttt

SEQ ID NO: 15009 - RNA, 862 nt, Homo sapiens
  source 1..862: mol_type = other RNA
gctgggattacaggcatgagccactgcacccagccaaaatgtcacttctcttaatttcaagagaatgcccaattaaaaagcaaatacaataatgggatcctaagacataaaatggacattaggtaaaaattgaaatctaaataaatagggattttagttaatactaatgtatccatattggtccattaattgttaacatacgtatcatattaatgtaaaatgttaataggaggaaaactgtgtggggagtatatggaaagtctctgtactatcttcacaatttttctgtaaatataaaactgttctcaaaaataaagtttatttttgtaatcccagcactttgggaggctgaggcaggaaagtcatttgaagccaagagtcctataccagcctgagcaacatagtgagacactatctctacaaagcaacaacaacaacaacaacaacaacaacaacaaaatatacacacacacacacacacacacacacacaaattagccagcatgtgcactcaggaggttgacgtgggaagatcacttgagcccagaaggtcaaggctgcagtgagtctagatcagaccactgcactccagcatggaattgactttgtcttctggcccctgcacttggcctgtcacggtgcctttgctggtattcttcacccagccaaccactcctattttcctagcttcatcttctgtatacattctgaagcaaacaccctgcactcttccgaacacctcgtagtccacggatttgagtgactgggcggtagacatggcggcggcgagccctctgttgaggagccggagaggggctcggggcgcagcgactgcggcggctgcgagagggaggggacacat

SEQ ID NO: 15010 - RNA, 6027 nt, Homo sapiens
  source 1..6027: mol_type = other RNA
gctgggattacaggcatgagccactgcacccagccaaacatgacttttccatccagagtaaatccaactaacaagaatccacccttggagttcatgtaaaaatacatgacacagggtgatgaaagtgctttgaaactagatacaggcagtggttctatagcatggtgaatgtactcaaggcaacttctttactttaaaatcgttaattttatgccatgtgaattgcatctcaataaaaattgttttcattttaaaaattgtaaatgactgcagtgtgtgtatagagatgatcactgtggcgagtagtggaggcactggaggcagcctgcaggcctgccctttatacaccttggttaatcatggtactaatgtacccacacagctaacacaatggaatgacaaatcctacagttagacatggaaggagcatcagactatgttgtgaagacagaaagaggatcttgtaggataaaattcctattagcaaaaagcaaaaaccaaaacccaataccaagtctgtttctgtgtatgtagtctgcaaagacacatgccattgctgaactgctgaacttgcttccctgtgggtacttctttacagatgtctgtattgttcacattttttaaagcaccaattacttttgtttaaaaaaatacacttaaaaaaggcagtaagacaagctctgtcaatcatctataggacaagaagcaaagacaccccagctgcaataagcacacctagtgccagggaccagggctcctgggacaaacactgatccatggctggtgcccaggggcctggaacatcttgttagatcagaaattaggggagtgcttccaaaaatgctgggatataggaggcactcgaaggggctctcgctggccaagtcgggaactatctgaggaactcttcccccatccccaaaggtcaatgatgaagtcgacttttgaaaaaatgggaatccatagtggatatatgaaaataaatgaaggagaagggagggatgactggcaaatgaggaaggagtgctgggctgcagaaacgtcgcttggcagtcatcataaagattgaatcaggccagaatcagcaacatttgctgaacctggtcggggaatggggaagagtctcatgaggaacagggtatgtacatggagacagtgtgtctccagagatttcttattagttgaaaagaaaaaaacagtaaccatgctatggagaaagtggacacacctcgactaggtgtgccaggtactcatttattgcctcttaactccaaatttccctgaccttgcccttccttgtcacactgaagagggggctctgaaaactcctttaccctttgccagcctgacccacagtgggctctgaaggggctaacaaggctagaggaggaagatggcctttttcttctgtctcctttcgtcctgcacgggtcccagcagcattccccaccgtgacagctctctgctcctgtggcttggcgggggggcacctccagtaagttgattctccagcatgggacaggcagcatatcccaggcaaccacagccacccctcggaggtctctccaccttggggaacctcctctgagtttccacgttccttctctgttttctcttcccttagccctaggggtgatggctgttctctgctaagctgctttagagctcttttttatcccttttagtagttaactaccttctacacagttaacaattacttatattaaaaccttcctgttcacatttcctcctccttggactagatgatcaaaacgaacatccccactgtggggcagatgggcattgtgtgcctcgagatgcgatgccctgagaggccgcgtgacgcaggtagtggttcagccacctggaatgcaaaaccaaatctaatcacgaggaaatcgcagacaaacacagataagcagcaccacctaaaacgaactgtatccttacaaactgttcctatcatcacagacaaagctatggaaatgatccagattaaagaagaccaaggagacatgacaactcaactgattacctgatccagaccagatccagcaccgcagagggaaaggtgctatagaggacacgatgcggccaatgggaatatgagtggtgaggtattctatcagtgttagatggacggaatttgacaactgtactgcagtcgtcagagagtatcttcttcttggtaagtacccactgaggtattaggggtaaaaggccatgacaggtgtggaggcagcaggagggagggagagggagagacagggggttggcgcaagggagagagaacgcacacacatttgagaacacacatgacagatagaatgggacgaaatgttaataggtgtatctgggcaaaggatatttgagcctcatttgtacagtttttattcttgcaacttttctgtagctttgaaatcatttccaagtaaaattaacttttttaaaagaggccatacaatatagcagtggtcctcaaccagggctgtgtcctggacacaccctagagcaccttagatgctctgggacccaggcatctgtagttctcaaagtgccccggtgcttccaatgtgcagccacgggcaggaaacaccagcctagtgggtgagctcactcactaaatttcagacatgacgagcagtgcttttgctctctgaagaacaagcactgggtaatgccaacacctagcctcagctacacgggggaagggcagaaacaagatgttgaatttgcatggccctggccaacacagacaacatccccttctagtggttcccaggcaagagaaaaaggcatttccaggacaactgtgccaggaattaaacacaagttaaaactggcaggagctggaatggtttcccagacctcagagctacctccccacctccatctttttggtctcactggtaatatggccagtctgggtccagctggcagagcacacgggaggaggctgctctctcaccaggcaaactgaggactgagtacaggaagggtgtggagaattatcctcttgggcaagttgaagaacaaggctactgcttggcatatttcccaaagccatttcccactctagaggccctgttctgtcctgtagaaagagtggagaacaaccaacatcacagtccaaatattgctcacctcagggccagcctgtgacagggtacccacaggatggttcatattgaaaactggggggaccatgctcgggggaggtggtggtagtgaaaggtcacaaacattcttgcccactgtgcaacaggcaggggcaagaggtgggatgggtcagtagtcacatgataaatcccccggggcctctgaaatcacattctggtaacttccactttgtgaaaaggagttagtttttactcctctcctttcccgtgtcttctccattttcaggtgggacagatctgcatgatatttgggcatctcaaaactgacgagcccaaaactgaccatgagtcacacccccagatgtgttctctaactactccctagctctgtgactttgtttccccagttgactgagccagaaacctgggactcatcctagatgagtcttctcttctcccttctctgtcccacgtccaatcaatgatcgaattccaccactgtcctgcctccaaacagccagaatccaccgctcaccaccgcccccaacagtgccctgctgcccactgctaagctctctcaactgctatgccagcctaactgaagcccagtcacaccaattcatcctggcttcagcacggccggcttgcatcaccaccttcttctcagttcaccttccaaatcaaacctccaaagagctgcttccacctacaagtcagctctcacctccacaggatgttccgtaagacactagagggcctgggctttcctgcttctccaacttctttccccagccttgtattttaagctccctgcacacacaattttgtttcacactcttgtgtaccatctttcaacaaagcctatccagcctccaagcttgggcatctcctccaggaagtcacccctgacctctccggaactcccctttggactcccattctattactacaaccactgcagtgtgaaaattatcttctcctatgtatgtctcctatactaggactccgaactccttgaagacaaggacagtatcgccactgtatccccagtgcattgcacaaagtagagctctatatttctaggatatactggactgaaagcatctgtggttttttgaatatcaagccctttagaatctggcaacagctataacgaaaacacacgtaaaccatgatgaactatagacagcaccaacaaagaaaacatgatactgctgctctggaactgaaatatcccccaaataatgaaaaataatatgttgggggctgatacagagtttattgaattagatttttctatttacaactgagatcacatctacatactattttgctagtctacatgggtacattatttccaacaagcttaagacttaccatgaatgggctcattcatacaaaaacacactcacactaattcttttaaaacagtagtgcatacattatactcctcctataaagccaactttgattaaaaaccactagtttcaaagctcagtctctgattttgaagatgaaccaagatatacgccatatgatcctacaatctattttagtcattttgtacagctgctatcttattggactacagtaaatattttttaaaaggacaccaatgaggggcaccatctggtgttaaccttaaccagaaagctggtttcctcctcctccccgcaaaaacctttggccaagagttctccactgtgaagactgaaaggacctggtgacatttcggcatcagtcctgttaccacttggaggtaacagaagcaggctcgtgtcctcctttaattctaccacactacatgactcgcaattggttctgaaattagaacgttcaccatcgtacttaaaatcttaggggcatgaagagtcagctagaacaaggaaaaagaaagtcgcaggtagtaggtaagtaggtgggcacatgaaaagccaagctgctctgtccaacaccagtgtacatgtgctttaactaaatgaactccagaggccaacagcagcagacctgctcaattcaccttccaaatcagaacaagaccaaaaagctcaggcttgagttgtcaactatgcataggttccgccagtgatgaggagctcgtaagcaggatctctactccttctgcacaacacgatgcaagcacacagcatgcccagcagctgaatagctgcaaatgccagtgcggcccagatcacatgcatcatgatttcttgtagcttcttcactactagagcctcacacccctcagcatagaggtcggaagggtgggccaggctgccattacaattgctggcagtctctctgcagcagctaagagggacactctggtttttggtttctttgaaccaatctgtattttcccagtctgagtagttgtgaattccacaacaatgcagctgtctctgtacataatcaatagcccggctagcagcatcagggttggttccattgtaggtcttatacactttctgaatgctgcgatcaacctcattttccaccgtggcaagtccacagcgactttcccggattgtggcacagcagccaattagcccaatgatgaaaagcagggctcctacagctatgatcactacagcagggatgagcgtgtacacatcttcaaagaagtggtcatagtcatcataagtgatgaagacataggctcccacatagcataaaatgccagctgccccccagaagatgaggttgagaaagaccagcacggtcttggaggaggtgatgccgcactggcccatggcgccggtggcccgcgaaggcccggcccggagagcggggctgcgctcaccgagagagcggcaatggcggcggcgcctcctcgctaggaactgcacggcctgcgcggcgctccccgcagcccctgcgccgtcgcgcagccccgaccccagcaagt

SEQ ID NO: 15011 - RNA, 5910 nt, Homo sapiens
  source 1..5910: mol_type = other RNA
gctgggattacaggcatgagccactgcacccagccaaacatgacttttccatccagagtaaatccaactaacaagaatccacccttggagttcatgtaaaaatacatgacacagggtgatgaaagtgctttgaaactagatacaggcagtggttctatagcatggtgaatgtactcaaggcaacttctttactttaaaatcgttaattttatgccatgtgaattgcatctcaataaaaattgttttcattttaaaaattgtaaatgactgcagtgtgtgtatagagatgatcactgtggcgagtagtggaggcactggaggcagcctgcaggcctgccctttatacaccttggttaatcatggtactaatgtacccacacagctaacacaatggaatgacaaatcctacagttagacatggaaggagcatcagactatgttgtgaagacagaaagaggatcttgtaggataaaattcctattagcaaaaagcaaaaaccaaaacccaataccaagtctgtttctgtgtatgtagtctgcaaagacacatgccattgctgaactgctgaacttgcttccctgtgggtacttctttacagatgtctgtattgttcacattttttaaagcaccaattacttttgtttaaaaaaatacacttaaaaaaggcagtaagacaagctctgtcaatcatctataggacaagaagcaaagacaccccagctgcaataagcacacctagtgccagggaccagggctcctgggacaaacactgatccatggctggtgcccaggggcctggaacatcttgttagatcagaaattaggggagtgcttccaaaaatgctgggatataggaggcactcgaaggggctctcgctggccaagtcgggaactatctgaggaactcttcccccatccccaaaggtcaatgatgaagtcgacttttgaaaaaatgggaatccatagtggatatatgaaaataaatgaaggagaagggagggatgactggcaaatgaggaaggagtgctgggctgcagaaacgtcgcttggcagtcatcataaagattgaatcaggccagaatcagcaacatttgctgaacctggtcggggaatggggaagagtctcatgaggaacagggtatgtacatggagacagtgtgtctccagagatttcttattagttgaaaagaaaaaaacagtaaccatgctatggagaaagtggacacacctcgactaggtgtgccaggtactcatttattgcctcttaactccaaatttccctgaccttgcccttccttgtcacactgaagagggggctctgaaaactcctttaccctttgccagcctgacccacagtgggctctgaaggggctaacaaggctagaggaggaagatggcctttttcttctgtctcctttcgtcctgcacgggtcccagcagcattccccaccgtgacagctctctgctcctgtggcttggcgggggggcacctccagtaagttgattctccagcatgggacaggcagcatatcccaggcaaccacagccacccctcggaggtctctccaccttggggaacctcctctgagtttccacgttccttctctgttttctcttcccttagccctaggggtgatggctgttctctgctaagctgctttagagctcttttttatcccttttagtagttaactaccttctacacagttaacaattacttatattaaaaccttcctgttcacatttcctcctccttggactagatgatcaaaacgaacatccccactgtggggcagatgggcattgtgtgcctcgagatgcgatgccctgagaggccgcgtgacgcaggtagtggttcagccacctggaatgcaaaaccaaatctaatcacgaggaaatcgcagacaaacacagataagcagcaccacctaaaacgaactgtatccttacaaactgttcctatcatcacagacaaagctatggaaatgatccagattaaagaagaccaaggagacatgacaactcaactgattacctgatccagaccagatccagcaccgcagagggaaaggtgctatagaggacacgatgcggccaatgggaatatgagtggtgaggtattctatcagtgttagatggacggaatttgacaactgtactgcagtcgtcagagagtatcttcttcttggtaagtacccactgaggtattaggggtaaaaggccatgacaggtgtggaggcagcaggagggagggagagggagagacagggggttggcgcaagggagagagaacgcacacacatttgagaacacacatgacagatagaatgggacgaaatgttaataggtgtatctgggcaaaggatatttgagcctcatttgtacagtttttattcttgcaacttttctgtagctttgaaatcatttccaagtaaaattaacttttttaaaagaggccatacaatatagcagtggtcctcaaccagggctgtgtcctggacacaccctagagcaccttagatgctctgggacccaggcatctgtagttctcaaagtgccccggtgcttccaatgtgcagccacgggcaggaaacaccagcctagtgggtgagctcactcactaaatttcagacatgacgagcagtgcttttgctctctgaagaacaagcactgggtaatgccaacacctagcctcagctacacgggggaagggcagaaacaagatgttgaatttgcatggccctggccaacacagacaacatccccttctagtggttcccaggcaagagaaaaaggcatttccaggacaactgtgccaggaattaaacacaagttaaaactggcaggagctggaatggtttcccagacctcagagctacctccccacctccatctttttggtctcactggtaatatggccagtctgggtccagctggcagagcacacgggaggaggctgctctctcaccaggcaaactgaggactgagtacaggaagggtgtggagaattatcctcttgggcaagttgaagaacaaggctactgcttggcatatttcccaaagccatttcccactctagaggccctgttctgtcctgtagaaagagtggagaacaaccaacatcacagtccaaatattgctcacctcagggccagcctgtgacagggtacccacaggatggttcatattgaaaactggggggaccatgctcgggggaggtggtggtagtgaaaggtcacaaacattcttgcccactgtgcaacaggcaggggcaagaggtgggatgggtcagtagtcacatgataaatcccccggggcctctgaaatcacattctggtaacttccactttgtgaaaaggagttagtttttactcctctcctttcccgtgtcttctccattttcaggtgggacagatctgcatgatatttgggcatctcaaaactgacgagcccaaaactgaccatgagtcacacccccagatgtgttctctaactactccctagctctgtgactttgtttccccagttgactgagccagaaacctgggactcatcctagatgagtcttctcttctcccttctctgtcccacgtccaatcaatgatcgaattccaccactgtcctgcctccaaacagccagaatccaccgctcaccaccgcccccaacagtgccctgctgcccactgctaagctctctcaactgctatgccagcctaactgaagcccagtcacaccaattcatcctggcttcagcacggccggcttgcatcaccaccttcttctcagttcaccttccaaatcaaacctccaaagagctgcttccacctacaagtcagctctcacctccacaggatgttccgtaagacactagagggcctgggctttcctgcttctccaacttctttccccagccttgtattttaagctccctgcacacacaattttgtttcacactcttgtgtaccatctttcaacaaagcctatccagcctccaagcttgggcatctcctccaggaagtcacccctgacctctccggaactcccctttggactcccattctattactacaaccactgcagtgtgaaaattatcttctcctatgtatgtctcctatactaggactccgaactccttgaagacaaggacagtatcgccactgtatccccagtgcattgcacaaagtagagctctatatttctaggatatactggactgaaagcatctgtggttttttgaatatcaagccctttagaatctggcaacagctataacgaaaacacacgtaaaccatgatgaactatagacagcaccaacaaagaaaacatgatactgctgctctggaactgaaatatcccccaaataatgaaaaataatatgttgggggctgatacagagtttattgaattagatttttctatttacaactgagatcacatctacatactattttgctagtctacatgggtacattatttccaacaagcttaagacttaccatgaatgggctcattcatacaaaaacacactcacactaattcttttaaaacagtagtgcatacattatactcctcctataaagccaactttgattaaaaaccactagtttcaaagctcagtctctgattttgaagatgaaccaagatatacgccatatgatcctacaatctattttagtcattttgtacagctgctatcttattggactacagtaaatattttttaaaaggacaccaatgaggggcaccatctggtgttaaccttaaccagaaagctggtttcctcctcctccccgcaaaaacctttggccaagagttctccactgtgaagactgaaaggacctggtgacatttcggcatcagtcctgttaccacttggaggtaacagaagcaggctcgtgtcctcctttaattctaccacactacatgactcgcaattggttctgaaattagaacgttcaccatcgtacttaaaatcttaggggcatgaagagtcagctagaacaaggaaaaagaaagtcgcaggtagtaggtaagtaggtgggcacatgaaaagccaagctgctctgtccaacaccagtgtacatgtgctttaactaaatgaactccagaggccaacagcagcagacctgctcaattcaccttccaaatcagaacaagaccaaaaagctcaggcttgagttgtcaactatgcataggttccgccagtgatgaggagctcgtaagcaggatctctactccttctgcacaacacgatgcaagcacacagcatgcccagcagctgaatagctgcaaatgccagtgcggcccagatcacatgcatcatgatttcttgtagcttcttcactactagagcctcacacccctcagcatagaggtcggaagggtgggccaggctgccattacaattgctggcagtctctctgcagcagctaagagggacactctggtttttggtttctttgaaccaatctgtattttcccagtctgagtagttgtgaattccacaacaatgcagctgtctctgtacataatcaatagcccggctagcagcatcagggttggttccattgtaggtcttatacactttctgaatgctgcgatcaacctcattttccacctttgctctgtaaacatatcccaaaaccactacaacaacttctgtgacaaaaaccaagagcaggatgatgacaaaccagaagatgaggttgagaaagaccagcacggtcttggaggaggtgatgccgcactggcccatggcgccggtggcccgcgaaggcccggcccggagagcggggctgcgctcaccgagagagcggcaatggcggcggcgcctcctcgctaggaactgcacggcctgcgcggcgctccccgcagcccctgcgccgtcgcgcagccccgaccccagcaagt

SEQ ID NO: 15012 - RNA, 6102 nt, Homo sapiens
  source 1..6102: mol_type = other RNA
gctgggattacaggcatgagccactgcacccagccaaacatgacttttccatccagagtaaatccaactaacaagaatccacccttggagttcatgtaaaaatacatgacacagggtgatgaaagtgctttgaaactagatacaggcagtggttctatagcatggtgaatgtactcaaggcaacttctttactttaaaatcgttaattttatgccatgtgaattgcatctcaataaaaattgttttcattttaaaaattgtaaatgactgcagtgtgtgtatagagatgatcactgtggcgagtagtggaggcactggaggcagcctgcaggcctgccctttatacaccttggttaatcatggtactaatgtacccacacagctaacacaatggaatgacaaatcctacagttagacatggaaggagcatcagactatgttgtgaagacagaaagaggatcttgtaggataaaattcctattagcaaaaagcaaaaaccaaaacccaataccaagtctgtttctgtgtatgtagtctgcaaagacacatgccattgctgaactgctgaacttgcttccctgtgggtacttctttacagatgtctgtattgttcacattttttaaagcaccaattacttttgtttaaaaaaatacacttaaaaaaggcagtaagacaagctctgtcaatcatctataggacaagaagcaaagacaccccagctgcaataagcacacctagtgccagggaccagggctcctgggacaaacactgatccatggctggtgcccaggggcctggaacatcttgttagatcagaaattaggggagtgcttccaaaaatgctgggatataggaggcactcgaaggggctctcgctggccaagtcgggaactatctgaggaactcttcccccatccccaaaggtcaatgatgaagtcgacttttgaaaaaatgggaatccatagtggatatatgaaaataaatgaaggagaagggagggatgactggcaaatgaggaaggagtgctgggctgcagaaacgtcgcttggcagtcatcataaagattgaatcaggccagaatcagcaacatttgctgaacctggtcggggaatggggaagagtctcatgaggaacagggtatgtacatggagacagtgtgtctccagagatttcttattagttgaaaagaaaaaaacagtaaccatgctatggagaaagtggacacacctcgactaggtgtgccaggtactcatttattgcctcttaactccaaatttccctgaccttgcccttccttgtcacactgaagagggggctctgaaaactcctttaccctttgccagcctgacccacagtgggctctgaaggggctaacaaggctagaggaggaagatggcctttttcttctgtctcctttcgtcctgcacgggtcccagcagcattccccaccgtgacagctctctgctcctgtggcttggcgggggggcacctccagtaagttgattctccagcatgggacaggcagcatatcccaggcaaccacagccacccctcggaggtctctccaccttggggaacctcctctgagtttccacgttccttctctgttttctcttcccttagccctaggggtgatggctgttctctgctaagctgctttagagctcttttttatcccttttagtagttaactaccttctacacagttaacaattacttatattaaaaccttcctgttcacatttcctcctccttggactagatgatcaaaacgaacatccccactgtggggcagatgggcattgtgtgcctcgagatgcgatgccctgagaggccgcgtgacgcaggtagtggttcagccacctggaatgcaaaaccaaatctaatcacgaggaaatcgcagacaaacacagataagcagcaccacctaaaacgaactgtatccttacaaactgttcctatcatcacagacaaagctatggaaatgatccagattaaagaagaccaaggagacatgacaactcaactgattacctgatccagaccagatccagcaccgcagagggaaaggtgctatagaggacacgatgcggccaatgggaatatgagtggtgaggtattctatcagtgttagatggacggaatttgacaactgtactgcagtcgtcagagagtatcttcttcttggtaagtacccactgaggtattaggggtaaaaggccatgacaggtgtggaggcagcaggagggagggagagggagagacagggggttggcgcaagggagagagaacgcacacacatttgagaacacacatgacagatagaatgggacgaaatgttaataggtgtatctgggcaaaggatatttgagcctcatttgtacagtttttattcttgcaacttttctgtagctttgaaatcatttccaagtaaaattaacttttttaaaagaggccatacaatatagcagtggtcctcaaccagggctgtgtcctggacacaccctagagcaccttagatgctctgggacccaggcatctgtagttctcaaagtgccccggtgcttccaatgtgcagccacgggcaggaaacaccagcctagtgggtgagctcactcactaaatttcagacatgacgagcagtgcttttgctctctgaagaacaagcactgggtaatgccaacacctagcctcagctacacgggggaagggcagaaacaagatgttgaatttgcatggccctggccaacacagacaacatccccttctagtggttcccaggcaagagaaaaaggcatttccaggacaactgtgccaggaattaaacacaagttaaaactggcaggagctggaatggtttcccagacctcagagctacctccccacctccatctttttggtctcactggtaatatggccagtctgggtccagctggcagagcacacgggaggaggctgctctctcaccaggcaaactgaggactgagtacaggaagggtgtggagaattatcctcttgggcaagttgaagaacaaggctactgcttggcatatttcccaaagccatttcccactctagaggccctgttctgtcctgtagaaagagtggagaacaaccaacatcacagtccaaatattgctcacctcagggccagcctgtgacagggtacccacaggatggttcatattgaaaactggggggaccatgctcgggggaggtggtggtagtgaaaggtcacaaacattcttgcccactgtgcaacaggcaggggcaagaggtgggatgggtcagtagtcacatgataaatcccccggggcctctgaaatcacattctggtaacttccactttgtgaaaaggagttagtttttactcctctcctttcccgtgtcttctccattttcaggtgggacagatctgcatgatatttgggcatctcaaaactgacgagcccaaaactgaccatgagtcacacccccagatgtgttctctaactactccctagctctgtgactttgtttccccagttgactgagccagaaacctgggactcatcctagatgagtcttctcttctcccttctctgtcccacgtccaatcaatgatcgaattccaccactgtcctgcctccaaacagccagaatccaccgctcaccaccgcccccaacagtgccctgctgcccactgctaagctctctcaactgctatgccagcctaactgaagcccagtcacaccaattcatcctggcttcagcacggccggcttgcatcaccaccttcttctcagttcaccttccaaatcaaacctccaaagagctgcttccacctacaagtcagctctcacctccacaggatgttccgtaagacactagagggcctgggctttcctgcttctccaacttctttccccagccttgtattttaagctccctgcacacacaattttgtttcacactcttgtgtaccatctttcaacaaagcctatccagcctccaagcttgggcatctcctccaggaagtcacccctgacctctccggaactcccctttggactcccattctattactacaaccactgcagtgtgaaaattatcttctcctatgtatgtctcctatactaggactccgaactccttgaagacaaggacagtatcgccactgtatccccagtgcattgcacaaagtagagctctatatttctaggatatactggactgaaagcatctgtggttttttgaatatcaagccctttagaatctggcaacagctataacgaaaacacacgtaaaccatgatgaactatagacagcaccaacaaagaaaacatgatactgctgctctggaactgaaatatcccccaaataatgaaaaataatatgttgggggctgatacagagtttattgaattagatttttctatttacaactgagatcacatctacatactattttgctagtctacatgggtacattatttccaacaagcttaagacttaccatgaatgggctcattcatacaaaaacacactcacactaattcttttaaaacagtagtgcatacattatactcctcctataaagccaactttgattaaaaaccactagtttcaaagctcagtctctgattttgaagatgaaccaagatatacgccatatgatcctacaatctattttagtcattttgtacagctgctatcttattggactacagtaaatattttttaaaaggacaccaatgaggggcaccatctggtgttaaccttaaccagaaagctggtttcctcctcctccccgcaaaaacctttggccaagagttctccactgtgaagactgaaaggacctggtgacatttcggcatcagtcctgttaccacttggaggtaacagaagcaggctcgtgtcctcctttaattctaccacactacatgactcgcaattggttctgaaattagaacgttcaccatcgtacttaaaatcttaggggcatgaagagtcagctagaacaaggaaaaagaaagtcgcaggtagtaggtaagtaggtgggcacatgaaaagccaagctgctctgtccaacaccagtgtacatgtgctttaactaaatgaactccagaggccaacagcagcagacctgctcaattcaccttccaaatcagaacaagaccaaaaagctcaggcttgagttgtcaactatgcataggttccgccagtgatgaggagctcgtaagcaggatctctactccttctgcacaacacgatgcaagcacacagcatgcccagcagctgaatagctgcaaatgccagtgcggcccagatcacatgcatcatgatttcttgtagcttcttcactactagagcctcacacccctcagcatagaggtcggaagggtgggccaggctgccattacaattgctggcagtctctctgcagcagctaagagggacactctggtttttggtttctttgaaccaatctgtattttcccagtctgagtagttgtgaattccacaacaatgcagctgtctctgtacataatcaatagcccggctagcagcatcagggttggttccattgtaggtcttatacactttctgaatgctgcgatcaacctcattttccacctttgctctgtaaacatatcccaaaaccactacaacaacttctgtgacaaaaaccaagagcaggatgatgacaaacgtggcaagtccacagcgactttcccggattgtggcacagcagccaattagcccaatgatgaaaagcagggctcctacagctatgatcactacagcagggatgagcgtgtacacatcttcaaagaagtggtcatagtcatcataagtgatgaagacataggctcccacatagcataaaatgccagctgccccccagaagatgaggttgagaaagaccagcacggtcttggaggaggtgatgccgcactggcccatggcgccggtggcccgcgaaggcccggcccggagagcggggctgcgctcaccgagagagcggcaatggcggcggcgcctcctcgctaggaactgcacggcctgcgcggcgctccccgcagcccctgcgccgtcgcgcagccccgaccccagcaagt

SEQ ID NO: 15013 - RNA, 3360 nt, Homo sapiens
  source 1..3360: mol_type = other RNA
gctgggattacaggcatgagccactgcacccagccaacgatgcccctctttaaagtcatcgcaggagaaaaggaagtgcaatggagaagcaggagggcaggtggatacccccctccacctcaacaaagctctttggaacggcctcagccccccacaggagcatggggaggatggaggaagccacatgtttgcagggccttttccatgtcagatgctgtgtgtgcccccagactgggtggctgggcctgcaaccctggagctggttgacaatggcttggtgtgctggcagagtgggcagcaggttcccgaaccagctgggccaggtggctgtccgccaggatgcacattgacaggtgtgggtgctgcttttgggggacagcagtctggagaaaccgggtgaaggactaggagagacccagtcctctgtgaaaggcccagccacaaggttccttctgtcccagcccactgggcttctagtggggatgccaatggctaagagaccttctgtggctgtgcgggtgggagtgaggcctggaggccagcctcaatttccactgagaacccagtgtggcccatggcaggtttgagccccagaagagcaagcgatcgccatactgagcccctggagggtgggaagggaggacccactggcccagctcctgagcacgctgaggagctgggcctcaggtggtcctggcacgcaggatgttcagggcctctcacggcaccaggctctgcactcccacacagaagggacaaagtggcggctgctgaattagcagagtgcaggagtttgcagcccagctcctgcccagcccagtgggcacgttacttcctcttattttcccttctgcaaaatgacgattcccgtgagcccaggaagcccaggagatgcactgcaaagcaagcaaagcctccctggcctggagtctgcacctgggaacatggcagtgggctggcctccagcttcacagagcctcaggccctgagcgggtggggagggcatgcaagcatgcccatggggcctgcacttctgctccatgcagcctggagatgctggttactaccccaaactccttctcgccatgcgtcttggtcatgtggggctgagacagggtggaaaacccacctcagcccagttctccagaggggactctagctatagattcctcctccaaaggcctctccttccactgactccctgaaagtcgtccaggcaaggagagctcatcatgagtactgatgcctctgtctgtttcatgtcagaagcatcagcaaccagtatgaaggggcaaccttcttcatttcttacagatccaaaggtcaggaaaaggaggagagagaagggaaagagaaggtggctgctttgacacttgaatggcgtgaaagtgaaaagccggggccgtgggaggaagaggagaaagcgcgccgccaaggctgacctgatgatgaaagggcctctgacctccaggagcttccgttcgctgctgaatctcttgagaaggttgatcatgaacttataaaagtaagaattcatggtgggagttgaaggagaacattctaagcctttggtaccagaggtgttcagtaggccggctctgccaggggtgggcacctggagctctgagtggctggcctggaggtcagggccatcgagggggcctgggtcatccgtctggcctgcgggggaggaagcgatttctgccagcacctccaggtccttcaggatcacctcatccgattcatccgataacgtctgcagtaggatgggaaagaggctgtccgtgtgccggaacatcttccgaggagttttgatgtagaggtggtagagccacttgagaactgcaatcctggtcatcatcccaatggccgtgtcactgaggtggcagtttaggacctgcacgatcccgtcgaggtgaagggtcactggggctctttcagtgctggctgcagtgaagacactgatgccgctactgaagctggagtcacaggaaccatctggacctccactggctgtgccctcctgctttggcagggcatcgtcaggggtgggctctgcctgcctctgcccaggtctcagctcatccagctcgtcgtcctcgggggtgaccagcttcatcaggctctggttgcacacgttggccacttctttgatgcttttcttgcggtcatcgtaggccaagcagggcaagacagcagtcaggatcccggaggagtaaggcagcatgacgcggcccgccagctggatgaactcccgcatccagcacatggctgtcagctggatgaggtcatctgttgtctggcagtggatcaccaggatgttggccatctcagcaaacttcacactggaggggttcttcttaatttcttttaagaattctccaagaacaacctcacacattttgcgaatctctttgccattgtcacccaggatctggaagagtccatccaggatctccggcaggtaatccagcaggttaatgtctggcaccgactccagaaccaggatccaggagatgatgaactgccgggcatactggttgttggagtaaatcctctctcgcaacaaggggatgaagctcaccaggtcaaacttgttgctctcagtcacaatgtcctttaaaaggcggtctaggagctcagatccgcttttcacattggggtctgggtcggctgccagcttgctcagcccgtcaaagagcacgttgaagtggggcagcacagcgccccgggccaccttgacgatgttgtagagggcctcgcaggcatagtagcgcagcctgctgtctgcatcattgaagcaggtcagcactggctcgatcagctccttcaggtagagccctgagtccttgcccagtgcgatggagcaggcggccaggccgatgaggccccctttccggctgtgggggtgctgagacagggcaaactcctgggacagggtctggatcacatgcttgatttgcacggtattgttctgggccacgaactcccggaccagcttctcgatctccagcgctgccaccttccgcttttcgtacagcttgtcattgagggcgcgcacgatgttaggcgtgagcggcgcgaaatccttctcggggttcatggtggcagctgggggaacctcgcgactccttagcccgcggctgccggggccgcgccggggccaggggagtctgcggctccgctctgcccccggcgccggcgcatggaccacgccgctctaggcttgcctgccacgctccgccgcctcgccctggaacccgggcccggaccccgctccagcacacctgaccctggccgcttaacaactcccgcccggcactagcgggactcacgagacagcggccatgttactcgagt

SEQ ID NO: 15014 - RNA, 2754 nt, Homo sapiens
  source 1..2754: mol_type = other RNA
gctgggattacaggcatgagccactgcacccagccagtcattgcattttcaaggaatctctcaggcataaattctctgacgttgtcaaaggaatgaattctaactgcaaaagttaccaccttcatttgtaaggtttctctccactatgaattctgtgatggcttgcaaggtttgaactctgactttagaactttccacacgttacatttgtaaggtttcccaccagtatggattgtctgatgggtagttaggcttgaacagatactaaagggtttcccacactcatatggtttctctccggtatgaattctctgatgccttgcaagttttgaagtttgactaaaggctttgccacactcattacacttgtaaggtttctctccagtatgaattccccgatgtcttgcaaggtgtgaattctgagtgaagaccttcccacactcattgcatttgtaaggtttttttccagtatggattgcctgatgggtagttaggcttgaacggacactaaaggctttcccacactgattacactcatatggtttctctccagtatgaactctctgatgccttgcaagctttgatgtttgactaaaggctttgccacattcattacactggtaaggtttacctccagtatgaactctccgatgtcttgcaaggtgtgaattctgagtgaagaccttgccacactcattacatttgtaaggtttttcaccagtatggatgacctgatgggtagttaggtttgaatgttcactaaaggctttgccatactcattatacttgtaaggtttctctccagtatgaattcgctgatgccttgaaaggtatgaattatgcctaaagaccttgccacattcattacatttataaggtttctctccagtatgaattccccgatgtcttgcaaggtgtgaattctgagtgaagaccttgccacactcattacatttgtaaggtttttctccagtatggatgacctgatgggtagttaggcttgaatacacactgaaggctttgccgcactcattacacatataaggcttcactccagtatgaattctttgatgatttgcaaggtgtgaattttgagtgaagaccttgccacattcattacatttgtaaggcttttctccagtatggatgacctgatgggtagttaggtttgaatgtgctctaaaggctttgccacactcattacacttataaggtttctctccagtatgaattagctgatgccttgcaaggtgtgaattacgcctaaagaccttgccgcattcatgacatttgtaaggcttttctccggtgtgaattaccagatgaatagctaggcttgaacgaacaccaaaggctttgccgcactcattacacttgtaaggtttctctccagtgtgaattctccagtgatttgtaaggtgtgaattttgagtgaagaccttgccacattcattacatttgtaaggtttttctccactgtgggttgcctgatggatagctaagcttgaacgagctctaaaggctttcccacactcattacacttgtaaggtttctctccagtatgaattcctcgatgtcttacaaggtgtgaattctgagtgaagaccttgccacattcgttacatttataaggtttctctccagtgtgaattttctgatgttgtgagagttgtgaatttcgactaaagaccttaccacactcattacatttgtaacgtttttcgccagtatggatcacctgatgggtagttaggtttgaacgtgttctaaaggctttgccacactcataacatttgtaaggtttctctttagtatgacttctctgatgacttgcaaggtgtgaattttgaggaaagaccatgccacatccattagatttgtaagggcttccccaattatttgctttttgcccctgtgtgagtaataaagaagagataaaatctttgagatatttcttagaaatgtgggttttgacattataaggcatttgttgaggtggtgaaactgaggaattattgttgaaagacttctcaacctgattacattcataaattttcccttcatattgaaaaagctgcagttcaggcagatgtgactgaaggcttaatccaagctgatttttaataagcttgtttcttgcatctcttttatcatgttcatctcttccatgagtgagattgccttcttgggtcaaaagcactcctttgtaatttccttcagcatctctgcattgatactcaaggccatgtgtatttttctggacttccctgaaggaacatccttcaatgtcttggctttcctgtctttccaacatcactgtttggaatacttctcctgtattactcttccctttgtgtagtaaatctttcattacaaattcggaagagagagctgtgatcacagctttgatccattcccatccatctgggtttcctgctatttgtacttggctctccaaagtgaaaggctccttcccttgctccaacatagagataatactgaggtcaaaacaagagattcccagggaggccaggttcctataattctccaacatcacgtccctgtacaaagtcctctgagcggggtccaggcatgtccactcctcctgagagaattctatagccacatccctgaatgtcacctgtccctgggtgagagccatgcctgacttgtctttctttcctcttcctcttcttcaagggttcttcgctcggcggcgtcacccgcacccaacacgatccgcttccggaact

SEQ ID NO: 15015 - RNA, 3086 nt, Homo sapiens
  source 1..3086: mol_type = other RNA
gctgggattacaggcatgagccactgcacccagccagtcattgcattttcaaggaatctctcaggcataaattctctgacgttgtcaaaggaatgaattctaactgcaaaagttaccaccttcatttgtaaggtttctctccactatgaattctgtgatggcttgcaaggtttgaactctgactttagaactttccacacgttacatttgtaaggtttcccaccagtatggattgtctgatgggtagttaggcttgaacagatactaaagggtttcccacactcatatggtttctctccggtatgaattctctgatgccttgcaagttttgaagtttgactaaaggctttgccacactcattacacttgtaaggtttctctccagtatgaattccccgatgtcttgcaaggtgtgaattctgagtgaagaccttcccacactcattgcatttgtaaggtttttttccagtatggattgcctgatgggtagttaggcttgaacggacactaaaggctttcccacactgattacactcatatggtttctctccagtatgaactctctgatgccttgcaagctttgatgtttgactaaaggctttgccacattcattacactggtaaggtttacctccagtatgaactctccgatgtcttgcaaggtgtgaattctgagtgaagaccttgccacactcattacatttgtaaggtttttcaccagtatggatgacctgatgggtagttaggtttgaatgttcactaaaggctttgccatactcattatacttgtaaggtttctctccagtatgaattcgctgatgccttgaaaggtatgaattatgcctaaagaccttgccacattcattacatttataaggtttctctccagtatgaattccccgatgtcttgcaaggtgtgaattctgagtgaagaccttgccacactcattacatttgtaaggtttttctccagtatggatgacctgatgggtagttaggcttgaatacacactgaaggctttgccgcactcattacacatataaggcttcactccagtatgaattctttgatgatttgcaaggtgtgaattttgagtgaagaccttgccacattcattacatttgtaaggcttttctccagtatggatgacctgatgggtagttaggtttgaatgtgctctaaaggctttgccacactcattacacttataaggtttctctccagtatgaattagctgatgccttgcaaggtgtgaattacgcctaaagaccttgccgcattcatgacatttgtaaggcttttctccggtgtgaattaccagatgaatagctaggcttgaacgaacaccaaaggctttgccgcactcattacacttgtaaggtttctctccagtgtgaattctccagtgatttgtaaggtgtgaattttgagtgaagaccttgccacattcattacatttgtaaggtttttctccactgtgggttgcctgatggatagctaagcttgaacgagctctaaaggctttcccacactcattacacttgtaaggtttctctccagtatgaattcctcgatgtcttacaaggtgtgaattctgagtgaagaccttgccacattcgttacatttataaggtttctctccagtgtgaattttctgatgttgtgagagttgtgaatttcgactaaagaccttaccacactcattacatttgtaacgtttttcgccagtatggatcacctgatgggtagttaggtttgaacgtgttctaaaggctttgccacactcataacatttgtaaggtttctctttagtatgacttctctgatgacttgcaaggtgtgaattttgaggaaagaccatgccacatccattagatttgtaagggcttccccaattatttgctttttgcccctgtgtgagtaataaagaagagataaaatctttgagatatttcttagaaatgtgggttttgacattataaggcatttgttgaggtggtgaaactgaggaattattgttgaaagacttctcaacctgattacattcataaattttcccttcatattgaaaaagctgcagttcaggcagatgtgactgaaggcttaatccaagctgatttttaataagcttgtttcttgcatctcttttatcatgttcatctcttccatgagtgagattgccttcttgggtcaaaagcactcctttgtaatttccttcagcatctctgcattgatactcaaggccatgtgtatttttctggacttccctgaaggaacatccttcaatgtcttggctttcctgtctttccaacatcactgtttggaatacttctcctgtattactcttccctttgtgtagtaaatctttcattacaaattcggaagagagagctgtgatcacagctttgatccattcccatccatctgggtttcctgctatttgtacttggctctccaaagtgaaaggctccttcccttgctccaacatagagataatactgaggtcaaaacaagagattcctgccagggaggccaggttcctataattctccaacatcacgtccctgtacaaagtcctctgagcggggtccaggcatgtccactcctcctgagagaattctatagccacatccctgaatgtcacctgtccctgggtgagagccatgcctgacttgtctttctttcctcttcctcttcttcaagggttcttcctgaggtcaggagttcgagatcagcctgggcaacacggtgaaaccccgtctctactaaaaatacaaaattagccgggcgtggtggcacatgcctgtaatcccagctactcgggaggctgaggcaggagaatcgcttgaacctgggaggcggaggatgcggtgagccgaaatcgcgccattgcactccagcctggacaacaagagtaaatctccgtctcaccaaaaaaaaaaaaaaagaaaaaaaaaaaggtctgtagcgagcccgggaactggctgcggaaacggggcacggcggttcgcaagtttaatccatactgagggacactcacgctcggcggcgtcacccgcacccaacacgatccgcttccggaact

SEQ ID NO: 15016 - RNA, 2757 nt, Homo sapiens
  source 1..2757: mol_type = other RNA
gctgggattacaggcatgagccactgcacccagccagtcattgcattttcaaggaatctctcaggcataaattctctgacgttgtcaaaggaatgaattctaactgcaaaagttaccaccttcatttgtaaggtttctctccactatgaattctgtgatggcttgcaaggtttgaactctgactttagaactttccacacgttacatttgtaaggtttcccaccagtatggattgtctgatgggtagttaggcttgaacagatactaaagggtttcccacactcatatggtttctctccggtatgaattctctgatgccttgcaagttttgaagtttgactaaaggctttgccacactcattacacttgtaaggtttctctccagtatgaattccccgatgtcttgcaaggtgtgaattctgagtgaagaccttcccacactcattgcatttgtaaggtttttttccagtatggattgcctgatgggtagttaggcttgaacggacactaaaggctttcccacactgattacactcatatggtttctctccagtatgaactctctgatgccttgcaagctttgatgtttgactaaaggctttgccacattcattacactggtaaggtttacctccagtatgaactctccgatgtcttgcaaggtgtgaattctgagtgaagaccttgccacactcattacatttgtaaggtttttcaccagtatggatgacctgatgggtagttaggtttgaatgttcactaaaggctttgccatactcattatacttgtaaggtttctctccagtatgaattcgctgatgccttgaaaggtatgaattatgcctaaagaccttgccacattcattacatttataaggtttctctccagtatgaattccccgatgtcttgcaaggtgtgaattctgagtgaagaccttgccacactcattacatttgtaaggtttttctccagtatggatgacctgatgggtagttaggcttgaatacacactgaaggctttgccgcactcattacacatataaggcttcactccagtatgaattctttgatgatttgcaaggtgtgaattttgagtgaagaccttgccacattcattacatttgtaaggcttttctccagtatggatgacctgatgggtagttaggtttgaatgtgctctaaaggctttgccacactcattacacttataaggtttctctccagtatgaattagctgatgccttgcaaggtgtgaattacgcctaaagaccttgccgcattcatgacatttgtaaggcttttctccggtgtgaattaccagatgaatagctaggcttgaacgaacaccaaaggctttgccgcactcattacacttgtaaggtttctctccagtgtgaattctccagtgatttgtaaggtgtgaattttgagtgaagaccttgccacattcattacatttgtaaggtttttctccactgtgggttgcctgatggatagctaagcttgaacgagctctaaaggctttcccacactcattacacttgtaaggtttctctccagtatgaattcctcgatgtcttacaaggtgtgaattctgagtgaagaccttgccacattcgttacatttataaggtttctctccagtgtgaattttctgatgttgtgagagttgtgaatttcgactaaagaccttaccacactcattacatttgtaacgtttttcgccagtatggatcacctgatgggtagttaggtttgaacgtgttctaaaggctttgccacactcataacatttgtaaggtttctctttagtatgacttctctgatgacttgcaaggtgtgaattttgaggaaagaccatgccacatccattagatttgtaagggcttccccaattatttgctttttgcccctgtgtgagtaataaagaagagataaaatctttgagatatttcttagaaatgtgggttttgacattataaggcatttgttgaggtggtgaaactgaggaattattgttgaaagacttctcaacctgattacattcataaattttcccttcatattgaaaaagctgcagttcaggcagatgtgactgaaggcttaatccaagctgatttttaataagcttgtttcttgcatctcttttatcatgttcatctcttccatgagtgagattgccttcttgggtcaaaagcactcctttgtaatttccttcagcatctctgcattgatactcaaggccatgtgtatttttctggacttccctgaaggaacatccttcaatgtcttggctttcctgtctttccaacatcactgtttggaatacttctcctgtattactcttccctttgtgtagtaaatctttcattacaaattcggaagagagagctgtgatcacagctttgatccattcccatccatctgggtttcctgctatttgtacttggctctccaaagtgaaaggctccttcccttgctccaacatagagataatactgaggtcaaaacaagagattcctgccagggaggccaggttcctataattctccaacatcacgtccctgtacaaagtcctctgagcggggtccaggcatgtccactcctcctgagagaattctatagccacatccctgaatgtcacctgtccctgggtgagagccatgcctgacttgtctttctttcctcttcctcttcttcaagggttcttcgctcggcggcgtcacccgcacccaacacgatccgcttccggaact

SEQ ID NO: 15017 - RNA, 4756 nt, Homo sapiens
  source 1..4756: mol_type = other RNA
gctgggattacaggcatgagccactgcacccagccccatttttttcttaagtattcattcttttcataattgacttttctaatcttcagaacaagactgtgagctccgtgaatgaatacctagctccggttccttatacctagaatgaactttataatcaccagacacactgcagtttgttttcctctctcctgtggacctctgctgggaagctgcatacatctctttttcctgcctagtgaaggcttttgaatttgcaactcctggttctgtacccgtcaagaataagttggctggccctctttagtctgctgatactgataggaaggacaagtacactacttaaaacattatttaactgccccatagaagttaatagaaccagtgctggggaatacccccatctggatttaaccagcccatgtaataggtagatcttttttgtttttccaaaagtactaggcctaatcataggattaactaatattccatcaaactgggaaaagtttaagaacaacatgtgaagacagtagcaggtttgcttggtaatgaagaaagctaattgaagaagctcataagagatgttttttgatgttaaccagtgttatctcagacctcctgaggcagtgtgttctgtagacctcttctatcagaatcactttgctagtttggtagtatagagacaagaaatagaactaggatggtacaagtctttccatttggttcgtgtctgggtctagccttttgttaccaatatttcaaatgtaccattatatagggctgtagttagtatgtagttattggttgccttggttttgcaattgatcattctccaaataagtgaataaaatatatataccaagaactcaccatgtacactaaaacaccctgaaacctatttgttaaaagtgtaaacttttggtagttaagctaccacctcaatgtgaccatatatagaggcaaggcagtgcctttccagaccaagtcagggactagagtgctctctagcattggagcggggtggggaggatcagagagtctgtttcattcatcttcaaataataatagttaatacttagcacttatgtgctaagcactgttctaagcccttaacatatgtcagcaacttcatgaggaaactgaggcataatataatttagtaactgacccagtatcacacagctagtaggtggcagaaccagacttcagcccaggcagtcaggttccagagtatatactttaacctgtactctatactgccttataaaggcaatgaaaatttgacagatacacttaaatcagtaaacatttatgattcattttacatgttagctaaaagtccacgtccttgagaagcaaaaattcctcaaccctgtatttctatgggttgaactgccttctaggcagtcacaagtttggggtactctgtgcacccaaattcatgtatcttgttttgtcttttcccttagcaattgatctgataaacaatctgcttcaagtgaagatgagaaaacgttacagtgttgacaaatctcttagtcatccctggctacaggtaaaaaaaaatgtaatctctctttggcaatcctcatttgagtagttcactctgatttgtcccacctaatgagaccactctaagatcagcagaataataaaagtgctcttaagtgattaatttgtactatggctgaatctctggaaaccatacagcattcagatcggtaatgacaggcaattaaactcccatgaactgaaagcaatgacttagcctttcatagacctatgtgttcatttcacctttttgtaagattagtatgacatattaatttatcaaatttattttaaatgtctactgaaggatttatttttgcattgaagagattttttaaaaatgtttggcttaattctcccaaagttactttatagatttatcaaaagataccctccaaacttcagagtaaggagggaagctttagaactattttatagggagtgagaggcagaattagctttaaaacaaatgtaatctcatctaccagttactaaattatcctaataagcatccaagcactttcccccactttgagtaaggtttaggcctcacgttgtatagaacaaaatgttttagtgattattattagccacctaagaagcctgaagcaaattttttttaatttcagaaattagttacgttcattcattggagactctgagtttgaaaaatttctttaaattgctcatttaaaatatcacaagtagaacttagtacatagtagatacttatgagtagcgcctgtcaattatttgactagggcactaaacaacaacaaaaaaaaacacaaaacaaaaaccaggttgacagtattttgtttcttttgtttcatcattacaatttcattttctcctaggactatcagacttggcttgaccttagagaatttgaaactcgcattggagaacgttacattacacatgaaagtgatgatgctcgctgggaaatacatgcatacacacataaccttgtatacccaaagcacttcattatggctcctaatccagatgatatggaagaagatccttaatcactgagctaacctaaataaggaaggatttcattttatggactgatattttgctgtgtaacttgttctttgtagattgtcatctgcagtgctgcagtatatgaaatgtgtttcctttattttgatttcttgggccgactgaagggtaaaatgtccaagctgaaatatcactgccaagcaagttcactaaacccagctacaacggatgcaaagggttttgactgacgtgcattcctctgatatcttccaccttgaagtctctgatgaggtagcaaggcaaaaaagttaaatctctctcccatcttctttggattcattaacatatcatatccttgaagtaactgctgcctcactgatggctcatttgatttatctaaaagaaccttcagccggacatcaatacccatattttttaaaaatgtgtgttgttttattgggcccagagaggctacttttccctgtgccattcttcgcaaataactgaagtccacatcagctgttagatctgctgttcctggggcaattaagacatcatgaagcttgtggtcgcaaaaccctctgaaggtatctgtctttgttccatcatgaccataatcagcaaccagtgcagcacctccagttaatgcaatgcgttgagaaagttcctcgatgataacaccagcatcaggacacacttcaacatgatcccttgtttcgtcatgttgtatgaaggcttctgctggggtggcagaaggtgccaaaacaaacctcagtttatcagaaacctgtggatcaatgtcaacaaatacttctcgccatccctgtggtgttttctgaaatttatgcacaggaagaacatcaaaaaattcatgtgcaagataaaagctgtaccctgaaatagcagttaaagcttttattcatcacaaggcttgaaagaaattagaagtcagagttgttagctggaagggaatttgatttcataaaatcgggcttctcagcctgagaaggctgaggcaggaatggcttgagatcccttacccaagatcgtacccccactttggctttgagtcaagactcaaactagtcaatactagtcagtattcctgactagtacagggattttcccccacaccttgcttgtctttaggcaagtaaggattttttaaaagactctataactgaactaaacccacctactaacactgcttccatcagccccagctgccttgggctgctccgtcatcggtacaaccctagctatagggaaatactcaaaagtacaaaggagatttacattttgtttgggattttacaaagcttcatgaaataaactactacttaatgtcaggcaactttattttctattaagatgctcttttctagaaaaaagtaggctactctctatggataagggacttggcagcagtaactcaatctattatattgctgtaaaaagttacagtcccatcaatactgtgagggttgtgatcaaaattctttcattaatccacataaaggtaattaccttttggaacatcgtgcagatctcggtaccaggaaattggaatcccagacttagtgacacctttcatatacactggggatccagcatttcgctctaacgggaccttctctttagtcagtgtcaatgcttgaatctcacttaatttttggcttacctctaccagatgtactgaaatgtcacaatttttcagcacagatccaagttgagtgaacaccctcaaaatatctcccacgagggttcccctacctgggcccagttccaccagctggaaagctgtgctttttccagtggccatccattcactaatgaaccatatacctagtagctccccaaagatttgacttatttcaggtgaagtaatgaaatctcctttttcgcctagcatgtcacggtacacataataacccttggctggattagtcaacacctccttcatgtactcggccacagtgatgggaccagtagactttattttgtacataagatgccgcagcatcggcgtcaccgggttttctgcaggctcattcccggagctgaagtatttccctctccaaataaaaggaatggctgcgcgcgccacggcacacaacggccccaaacctgacctcagcagtacactcatgctgaaattcgcaggctagctcgctccgccaggagctggggcttagac

SEQ ID NO: 15018 - RNA, 4123 nt, Homo sapiens
  source 1..4123: mol_type = other RNA
gctgggattacaggcatgagccactgcacccagccccatttttttcttaagtattcattcttttcataattgacttttctaatcttcagaacaagactgtgagctccgtgaatgaatacctagctccggttccttatacctagaatgaactttataatcaccagacacactgcagtttgttttcctctctcctgtggacctctgctgggaagctgcatacatctctttttcctgcctagtgaaggcttttgaatttgcaactcctggttctgtacccgtcaagaataagttggctggccctctttagtctgctgatactgataggaaggacaagtacactacttaaaacattatttaactgccccatagaagttaatagaaccagtgctggggaatacccccatctggatttaaccagcccatgtaataggtagatcttttttgtttttccaaaagtactaggcctaatcataggattaactaatattccatcaaactgggaaaagtttaagaacaacatgtgaagacagtagcaggtttgcttggtaatgaagaaagctaattgaagaagctcataagagatgttttttgatgttaaccagtgttatctcagacctcctgaggcagtgtgttctgtagacctcttctatcagaatcactttgctagtttggtagtatagagacaagaaatagaactaggatggtacaagtctttccatttggttcgtgtctgggtctagccttttgttaccaatatttcaaatgtaccattatatagggctgtagttagtatgtagttattggttgccttggttttgcaattgatcattctccaaataagtgaataaaatatatataccaagaactcaccatgtacactaaaacaccctgaaacctatttgttaaaagtgtaaacttttggtagttaagctaccacctcaatgtgaccatatatagaggcaaggcagtgcctttccagaccaagtcagggactagagtgctctctagcattggagcggggtggggaggatcagagagtctgtttcattcatcttcaaataataatagttaatacttagcacttatgtgctaagcactgttctaagcccttaacatatgtcagcaacttcatgaggaaactgaggcataatataatttagtaactgacccagtatcacacagctagtaggtggcagaaccagacttcagcccaggcagtcaggttccagagtatatactttaacctgtactctatactgccttataaaggcaatgaaaatttgacagatacacttaaatcagtaaacatttatgattcattttacatgttagctaaaagtccacgtccttgagaagcaaaaattcctcaaccctgtatttctatgggttgaactgccttctaggcagtcacaagtttggggtactctgtgcacccaaattcatgtatcttgttttgtcttttcccttagcaattgatctgataaacaatctgcttcaagtgaagatgagaaaacgttacagtgttgacaaatctcttagtcatccctggctacaggtaaaaaaaaatgtaatctctctttggcaatcctcatttgagtagttcactctgatttgtcccacctaatgagaccactctaagatcagcagaataataaaagtgctcttaagtgattaatttgtactatggctgaatctctggaaaccatacagcattcagatcggtaatgacaggcaattaaactcccatgaactgaaagcaatgacttagcctttcatagacctatgtgttcatttcacctttttgtaagattagtatgacatattaatttatcaaatttattttaaatgtctactgaaggatttatttttgcattgaagagattttttaaaaatgtttggcttaattctcccaaagttactttatagatttatcaaaagataccctccaaacttcagagtaaggagggaagctttagaactattttatagggagtgagaggcagaattagctttaaaacaaatgtaatctcatctaccagttactaaattatcctaataagcatccaagcactttcccccactttgagtaaggtttaggcctcacgttgtatagaacaaaatgttttagtgattattattagccacctaagaagcctgaagcaaattttttttaatttcagaaattagttacgttcattcattggagactctgagtttgaaaaatttctttaaattgctcatttaaaatatcacaagtagaacttagtacatagtagatacttatgagtagcgcctgtcaattatttgactagggcactaaacaacaacaaaaaaaaacacaaaacaaaaaccaggttgacagtattttgtttcttttgtttcatcattacaatttcattttctcctaggactatcagacttggcttgaccttagagaatttgaaactcgcattggagaacgttacattacacatgaaagtgatgatgctcgctgggaaatacatgcatacacacataaccttgtatacccaaagcacttcattatggctcctaatccagatgatatggaagaagatccttaatcactgagctaacctaaataaggaaggatttcattttatggactgatattttgctgtgtaacttgttctttgtagattgtcatctgcagtgctgcagtatatgaaatgtgtttcctttattttgatttcttgggccgactgaagggtaaaatgtccaagctgaaatatcactgccaagcaagttcactaaacccagctacaacggatgcaaagggttttgactgacgtgcattcctctgatatcttccaccttgaagtctctgatgaggtagcaaggcaaaaaagttaaatctctctcccatcttctttggattcattaacatatcatatccttgaagtaactgctgcctcactgatggctcatttgatttatctaaaagaaccttcagccggacatcaatacccatattttttaaaaatgtgtgttgttttattgggcccagagaggctacttttccctgtgccattcttcgcaaataactgaagtccacatcagctgttagatctgctgttcctggggcaattaagacatcatgaagcttgtggtcgcaaaaccctctgaaggtatctgtctttgttccatcatgaccataatcagcaaccagtgcagcacctccagttaatgcaatgcgttgagaaagttcctcgatgataacaccagcatcaggacacacttcaacatgatcccttgtttcgtcatgttgtatgaaggcttctgctggggtggcagaaggtgccaaaacaaacctcagtttatcagaaacctgtggatcaatgtcaacaaatacttctcgccatccctgtggtgttttctgaaatttatgcacaggaagaacatcaaaaaattcatgtgcaagataaaagctgtacccttttggaacatcgtgcagatctcggtaccaggaaattggaatcccagacttagtgacacctttcatatacactggggatccagcatttcgctctaacgggaccttctctttagtcagtgtcaatgcttgaatctcacttaatttttggcttacctctaccagatgtactgaaatgtcacaatttttcagcacagatccaagttgagtgaacaccctcaaaatatctcccacgagggttcccctacctgggcccagttccaccagctggaaagctgtgctttttccagtggccatccattcactaatgaaccatatacctagtagctccccaaagatttgacttatttcaggtgaagtaatgaaatctcctttttcgcctagcatgtcacggtacacataataacccttggctggattagtcaacacctccttcatgtactcggccacagtgatgggaccagtagactttattttgtacataagatgccgcagcatcggcgtcaccgggttttctgcaggctcattcccggagctgaagtatttccctctccaaataaaaggaatggctgcgcgcgccacggcacacaacggccccaaacctgacctcagcagtacactcatgctgaaattcgcaggctagctcgctccgccaggagctggggcttagac

SEQ ID NO: 15019 - RNA, 1054 nt, Homo sapiens
  source 1..1054: mol_type = other RNA
gctgggattacaggcatgagccactgcacccagccctgtttcattcttcacctcagttaaattctgcataaccttcagctctcatcccatattccagaactgtaaggaaagcttcaggtttcctcatatgctctctcatagtgaccctaaatttatcttctgtaattataaagttgtatgattatttgattcatgtgcatcttcccatgagatggtaagctcccagggggctgggttcatgtctgttttgctcaccctcgtacccccaatgctgcacacaatattttcagagtctttgtataattctggtataaagaatgctgataccttgttgtcttcagaaaccagtgacagacttgcactgtctgtccccttgaagacagattgtcatgtggcttgttttggtcactagggcttaaggggcctcaggctggcactcgaaaccaggcgttctcatttccctttggcatcaccctgaacggctgtgcctggagctggcgcggggctgaagaggggaggaaatacatgtgaggaaaatcagaggagagggtcgggaacagatgtgggcataaagggaaggcctctgacttgaaataaacaaataggagtcccgcagctggaaggacaaatcctttcacgtcgcgggtgatgtgggattggggcgattttgctctccctttgttctttcccctgccttccacgtttccagggtatttgattgatgtctgtcttctctgttaagttattccaccgtgaggagagagccggtggcagtacctggcacgcagcgggcgcccagtatagacagcaaatgatttgcaagttttcggcgctgagcacgtggagctttggaaaccaggacagcaaatgagtgtctcggagaccacaaaagcggttccggcgcgtgcgaaaggcggtggctgggcgacggcggagggaacggcgcagagcggggcgccccgccgggagcgctgcctgcgtggcgcccgaggcgggggcgcggggggccgcgcatagcacgtgctcgtctgggagccggccgggccgaggcggg

SEQ ID NO: 15020 - RNA, 1059 nt, Homo sapiens
  source 1..1059: mol_type = other RNA
gctgggattacaggcatgagccactgcacccagccctgtttcattcttcacctcagttaaattctgcataaccttcagctctcatcccatattccagaactgtaaggaaagcttcaggtttcctcatatgctctctcatagtgaccctaaatttatcttctgtaattataaagttgtatgattatttgattcatgtgcatcttcccatgagatggtaagctcccagggggctgggttcatgtctgttttgctcaccctcgtacccccaatgctgcacacaatattttcagagtctttgtataattctggtataaagaatgctgtactgataccttgttgtcttcagaaaccagtgacagacttgcactgtctgtccccttgaagacagattgtcatgtggcttgttttggtcactagggcttaaggggcctcaggctggcactcgaaaccaggcgttctcatttccctttggcatcaccctgaacggctgtgcctggagctggcgcggggctgaagaggggaggaaatacatgtgaggaaaatcagaggagagggtcgggaacagatgtgggcataaagggaaggcctctgacttgaaataaacaaataggagtcccgcagctggaaggacaaatcctttcacgtcgcgggtgatgtgggattggggcgattttgctctccctttgttctttcccctgccttccacgtttccagggtatttgattgatgtctgtcttctctgttaagttattccaccgtgaggagagagccggtggcagtacctggcacgcagcgggcgcccagtatagacagcaaatgatttgcaagttttcggcgctgagcacgtggagctttggaaaccaggacagcaaatgagtgtctcggagaccacaaaagcggttccggcgcgtgcgaaaggcggtggctgggcgacggcggagggaacggcgcagagcggggcgccccgccgggagcgctgcctgcgtggcgcccgaggcgggggcgcggggggccgcgcatagcacgtgctcgtctgggagccggccgggccgaggcggg

SEQ ID NO: 15021 - RNA, 1062 nt, Homo sapiens
  source 1..1062: mol_type = other RNA
gctgggattacaggcatgagccactgcacccagccctgtttcattcttcacctcagttaaattctgcataaccttcagctctcatcccatattccagaactgtaaggaaagcttcaggtttcctcatatgctctctcatagtgaccctaaatttatcttctgtaattataaagttgtatgattatttgattcatgtgcatcttcccatgagatggtaagctcccagggggctgggttcatgtctgttttgctcaccctcgtacccccaatgctgcacacaatattttcagagtctttgtataattctggtataaagaatgctgtactgataccttgttgtcttcagaaaccagtgacagacttgcactgtctgtccccttgaagacagattgtcatgtggcttgttttggtcactagggcttaaggggcctcaggctggcactcgaaaccaggcgttctcatttccctttggcatcaccctgaacggctgtgcctggagctggcgcggggctgaagaggggaggaaatacatgtgaggaaaatcagaggagagggtcgggaacagatgtgggcataaagggaaggcctctgacttgaaataaacaaataggagtcccgcagctggaaggacaaatcctttcacgtcgcgggtgatgtgggattggggcgattttgctctccctttgttctttcccctgccttccacgtttccagggtatttgattgatgtctgtcttctctgttaagttattccaccgtgaggagagagccggtggcagtacctggcacgcagcgggcgcccagtatagacctgagcaaatgatttgcaagttttcggcgctgagcacgtggagctttggaaaccaggacagcaaatgagtgtctcggagaccacaaaagcggttccggcgcgtgcgaaaggcggtggctgggcgacggcggagggaacggcgcagagcggggcgccccgccgggagcgctgcctgcgtggcgcccgaggcgggggcgcggggggccgcgcatagcacgtgctcgtctgggagccggccgggccgaggcggg

SEQ ID NO: 15022 - RNA, 1087 nt, Homo sapiens
  source 1..1087: mol_type = other RNA
gctgggattacaggcatgagccactgcacccagccctgtttcattcttcacctcagttaaattctgcataaccttcagctctcatcccatattccagaactgtaaggaaagcttcaggtttcctcatatgctctctcatagtgaccctaaatttatcttctgtaattataaagttgtatgattatttgattcatgtgcatcttcccatgagatggtaagctcccagggggctgggttcatgtctgttttgctcaccctcgtacccccaatgctgcacacaatattttcagagtctttgtataattctggtataaagaatgctgtactgataccttgttgtcttcagaaaccagtgacagacttgcactgtctgtccccttgaagacagattgtcatgtggcttgttttggtcactagggcttaaggggcctcaggctggcactcgaaaccaggcgttctcatttccctttggcatcaccctgaacggctgtgcctggagctggcgcggggctgaagaggggaggaaatacatgtgaggaaaatcagaggagagggtcgggaacagatgtgggcataaagggaaggcctctgacttgaaataaacaaataggagtcccgcagctggaaggacaaatcctttcacgtcgcgggtgatgtgggattggggcgattttgctctccctttgttctttcccctgccttccacgtttccagggtatttgattgatgtctgtcttctctgttaagttattccaccgtgaggagagagccggtggcagtacctggcacgcagcgggcgcccagtatagacgtagtaggcgacccctaaacatctgtacagcaaatgatttgcaagttttcggcgctgagcacgtggagctttggaaaccaggacagcaaatgagtgtctcggagaccacaaaagcggttccggcgcgtgcgaaaggcggtggctgggcgacggcggagggaacggcgcagagcggggcgccccgccgggagcgctgcctgcgtggcgcccgaggcgggggcgcggggggccgcgcatagcacgtgctcgtctgggagccggccgggccgaggcggg

SEQ ID NO: 15023 - RNA, 976 nt, Homo sapiens
  source 1..976: mol_type = other RNA
gctgggattacaggcatgagccactgcacccagccctgtttcattcttcacctcagttaaattctgcataaccttcagctctcatcccatattccagaactgtaaggaaagcttcaggtttcctcatatgctctctcatagtgaccctaaatttatcttctgtaattataaagttgtatgattatttgattcatgtgcatcttcccatgagatggtaagctcccagggggctgggttcatgtctgttttgctcaccctcgtacccccaatgctgcacacaatattttcagagtctttgtataattctggtataaagaatgctgtactgataccttgttgtcttcagaaaccagtgacagacttgcactgtctgtccccttgaagacagattgtcatgtggcttgttttggtcactagggcttaaggggcctcaggctggcactcgaaaccaggcgttctcatttccctttggcatcaccctgaacggctgtgcctggagctggcgcggggttgaaataaacaaataggagtcccgcagctggaaggacaaatcctttcacgtcgcgggtgatgtgggattggggcgattttgctctccctttgttctttcccctgccttccacgtttccagggtatttgattgatgtctgtcttctctgttaagttattccaccgtgaggagagagccggtggcagtacctggcacgcagcgggcgcccagtatagacagcaaatgatttgcaagttttcggcgctgagcacgtggagctttggaaaccaggacagcaaatgagtgtctcggagaccacaaaagcggttccggcgcgtgcgaaaggcggtggctgggcgacggcggagggaacggcgcagagcggggcgccccgccgggagcgctgcctgcgtggcgcccgaggcgggggcgcggggggccgcgcatagcacgtgctcgtctgggagccggccgggccgaggcggg

SEQ ID NO: 15024 - RNA, 4308 nt, Homo sapiens
  source 1..4308: mol_type = other RNA
gctgggattacaggcatgagccactgcacccagccgacatcaccatccttcctgactctgaatttatatactactaaccagcaatcattttcctccacctattcaacacagaagtacctaacagtaaaagatgagagatacctatctggcatgtgagaaaatgatatatagctactgacggggatttcctttgaggatgctgagtaaacttcgtggtgtgtgcctgcatttccactgcaatctatcacatgtgatgagttgtggaatttcccacttgtggcatcacactggggctcaaagagtttcagattttggagcatgtttttttgttttttgagatgggagccttgctctgtcacccaggctggagtgcagtggtgtgatctcagctcactgcaacctcaacctccagggttcctgcctcagcctcccgagtagctggggttacaggtgccccccaccacacccaggtaattttttgtatttttagtagagatggggtttcgccatgttggccaggctggtctggagctcctgacctcaggttatccgtccactttgacctcccaaagtgctgggattacaggtatgagccaccacgcccggcctagattttggagcattttgaatttgggatggtgaatctgtactgttgttcctctccccccacaaccatcttgccgatggggaaactgaagcattgagaggtgatggaaattgctggaggtcatatagctggtgagtggcagagtggactcagaacccaggatcatctgattgcaaaatctgtttccttcatctctgtactgtgcaacaatgacaagaatactattggcgataacaacaataacccacaaattttgacttgtcattcacaacaacaacaaaacaataataacaatacattcacctctggggtcgaaacccatatcctagaatcctaggaactaaggattccctccagccacactgcagcaatgctcatttgcatagaccctctaatttgtatgcatatcattatctgcccccacccaacccaccagctccctgtgttttatgcttccagctggcttggcggattgtcattctgtcctggatgtgtctaataagggcgtcttgcgggatgtagcctctacttcctcaggaattgtggattggagaggaagccagatccagacgtgaggtctctggtttcccccacatttcctgcatggacttgagccaactgggtccaggttcctcatctgtagaatgacctccatgggtcattacctccatccctctgcctctaggagccaccacttgttgctgatggttgccccccatccgactcctccctttccctgtggggctctttaggcctgacaattcctctccacccttcttcagtttgttcccctaagaactagacagatccaggtacaactatttgccatttatttcaaagatcagtggttaagaggcccagggttatgaacaaggtctggtcctcaccccgagatgtgttagtctgggctggggagggccctcaggctgtgtgtatatgtgtgtaatgttgtgtgtttgtcattgtgatgtgtgtgtgatgtgtgtgtcattgtgatgttgtgtgtgtgtaatgttgtgtttgtcattgtgatgtgtgtgtaatgtgtgtttgtcatcgtgatgttgtgtgtgtaatgtgtgtttgtcatcgtgatgttgtgtgtgtaatgtgtgtttgtcattgtgatgttgtgtgtgtgtaatgtgtatttgtcatggtgatattgtgtgtgtgtatgtgtgtaaccaggtctgactataacttggtctgtctgtgtctaatgtaatgagtattaattaccaagtgtgacggtgacacctctgggagtggctgtgtagctgggatgctgtctgagttttgtgtgcttgtgttataacatacacacagtgctgtgactgtctgtgatgccgtctgtgacttccatgtgattgtgtggttgtgcatgaatctggcacttcgcgtgtatgagtctatagttgtgaaagagtggctgagattatgcagccatgtgacagattttgtgggatgccataggtgtgactgtagagtcattcttccttcctttcaatcagcaagcatttccctagagcatgctttgtgccaggccctgggccggatgccggggacagatccgtggtgtcctattagggatgtctatgcttggcagtgatgaaatcagccatggtggtagcatttacaccatggaaattggcaaacattacaaagctgtccccctcccaggacagctggttgttaaacagttatgagcacgctgccgtgctcatgtatctgagtgtaactctttgtgaccaggctgaggtgtggccaccagtctgtgggtgggatctgagtatgtggggtggggctgggctcttcatgatgagtcccgatgatcagtctcccgcccaccctgtccgtactcatgatgagagtagggaagtggatgaagtttcccacccccagccaagtccctggaatcccaagccccactttcttctgaatcaaaagcataaatacccacccctcaccccttcttcctgaatatcaggcaaatcaactttaccccatgtttgggggcccacagaccccaagtctctgggtttttgtccttagtattgtccgtggcagggtctgcagtctacgtgggtcttctgaaggtgcctgctggggcttcatctcgccttggtggtgcccactgagctctccgcctttgagttttgggttccctggagtgtcccccaagatctgtttcctgagttttcttttttcttcctttcttttttttgaggcacagtctcactgcgtttcccaggttggagtgcagtggtgtgatctcggctcactgcaacctccgcctcccgggtttaagcaaaattatcctgcctcagcctcctgagtagctggattacaggcaggcaccaccacgtccggctaatttttgtatttttagtagagatggggttttgccatgttagccaggctggtctcgaactcctgacctcaggtgatccgcctgccttggcctcccaaagtgctgggattacaggcgagagccaccacgcccagcctctgcttcgtgagttttctttcccctgaggcaccctctgagttctccacgtgtcagacccatgtccaatgcaccacgctccttccttcacaccatgaaagccccgaagtaagaccgggtaccatcacgcagtcgaaccaggcgttcatccagcacacggacgaccaccttctccccagcctccaggtgtaccacaccacccaggaagctgctgtcccaccagacccgggagctgctggtggcccgtccgcagggtgactgctggctgaccaacagctccagctcctcggggtagcggggtgtgcgcttgtagaggccgtgggtgatggtgctggccaggcccagcgggcagcccacaccgcccagctgcaccttggagtagatgtagtagtagccagctttggtgaccacaagggccccatcgtggtagctgaggcccctcaggaaggccaggcccagctgagtctcccataacagcggccccccgctgccggtcaagctggagttggcccctgtgagatgcgctgctgggttgacctcgtgagaccttcgctcttgtatcagctgctcccaggagcctgcaggtccgtcaggcaggcgggtgaccatctctcctagacgccagtgcagctgcaggaggaaccagccttggacggccagcccggcccccatcagcaacagcaagagacccagacccacccgggccacactgcacgactgtctccggtggcttcgtcccagcctcgtgaatgggatgtcggtctgtccatccaccacaaacactgagggccgtacgacactctcctccatgcccaaggtgtctggagcagggctgacacgcctgggtccttcaacctcagaggaaaccgaaattgctcaacactcctgggctgtgcacgactttccagaggcttctgaaaatgtgactcaggtggcaagtgcagtggggagcccccagctttcccttcttggatgcttcattcgcttggggccaccaaatatcgactgaggactttctgcccatgccaggctctgctctcggtgtgggggatgcagcaatgaacaacagcaagaagggtccctgctcctcttctggtggagccagagagacaagaaacctcgtaaacaagaaaataatacgttgtgggtttttttgttcgtttatttgttttgtttttgagatggagtctcg

SEQ ID NO: 15025 - RNA, 4017 nt, Homo sapiens
  source 1..4017: mol_type = other RNA
gctgggattacaggcatgagccactgcacccagccgacatcaccatccttcctgactctgaatttatatactactaaccagcaatcattttcctccacctattcaacacagaagtacctaacagtaaaagatgagagatacctatctggcatgtgagaaaatgatatatagctactgacggggatttcctttgaggatgctgagtaaacttcgtggtgtgtgcctgcatttccactgcaatctatcacatgtgatgagttgtggaatttcccacttgtggcatcacactggggctcaaagagtttcagattttggagcatgtttttttgttttttgagatgggagccttgctctgtcacccaggctggagtgcagtggtgtgatctcagctcactgcaacctcaacctccagggttcctgcctcagcctcccgagtagctggggttacaggtgccccccaccacacccaggtaattttttgtatttttagtagagatggggtttcgccatgttggccaggctggtctggagctcctgacctcaggttatccgtccactttgacctcccaaagtgctgggattacaggtatgagccaccacgcccggcctagattttggagcattttgaatttgggatggtgaatctgtactgttgttcctctccccccacaaccatcttgccgatggggaaactgaagcattgagaggtgatggaaattgctggaggtcatatagctggtgagtggcagagtggactcagaacccaggatcatctgattgcaaaatctgtttccttcatctctgtactgtgcaacaatgacaagaatactattggcgataacaacaataacccacaaattttgacttgtcattcacaacaacaacaaaacaataataacaatacattcacctctggggtcgaaacccatatcctagaatcctaggaactaaggattccctccagccacactgcagcaatgctcatttgcatagaccctctaatttgtatgcatatcattatctgcccccacccaacccaccagctccctgtgttttatgcttccagctggcttggcggattgtcattctgtcctggatgtgtctaataagggcgtcttgcgggatgtagcctctacttcctcaggaattgtggattggagaggaagccagatccagacgtgaggtctctggtttcccccacatttcctgcatggacttgagccaactgggtccaggttcctcatctgtagaatgacctccatgggtcattacctccatccctctgcctctaggagccaccacttgttgctgatggttgccccccatccgactcctccctttccctgtggggctctttaggcctgacaattcctctccacccttcttcagtttgttcccctaagaactagacagatccaggtacaactatttgccatttatttcaaagatcagtggttaagaggcccagggttatgaacaaggtctggtcctcaccccgagatgtgttagtctgggctggggagggccctcaggctgtgtgtatatgtgtgtaatgttgtgtgtttgtcattgtgatgtgtgtgtgatgtgtgtgtcattgtgatgttgtgtgtgtgtaatgttgtgtttgtcattgtgatgtgtgtgtaatgtgtgtttgtcatcgtgatgttgtgtgtgtaatgtgtgtttgtcatcgtgatgttgtgtgtgtaatgtgtgtttgtcattgtgatgttgtgtgtgtgtaatgtgtatttgtcatggtgatattgtgtgtgtgtatgtgtgtaaccaggtctgactataacttggtctgtctgtgtctaatgtaatgagtattaattaccaagtgtgacggtgacacctctgggagtggctgtgtagctgggatgctgtctgagttttgtgtgcttgtgttataacatacacacagtgctgtgactgtctgtgatgccgtctgtgacttccatgtgattgtgtggttgtgcatgaatctggcacttcgcgtgtatgagtctatagttgtgaaagagtggctgagattatgcagccatgtgacagattttgtgggatgccataggtgtgactgtagagtcattcttccttcctttcaatcagcaagcatttccctagagcatgctttgtgccaggccctgggccggatgccggggacagatccgtggtgtcctattagggatgtctatgcttggcagtgatgaaatcagccatggtggtagcatttacaccatggaaattggcaaacattacaaagctgtccccctcccaggacagctggttgttaaacagttatgagcacgctgccgtgctcatgtatctgagtgtaactctttgtgaccaggctgaggtgtggccaccagtctgtgggtgggatctgagtatgtggggtggggctgggctcttcatgatgagtcccgatgatcagtctcccgcccaccctgtccgtactcatgatgagagtagggaagtggatgaagtttcccacccccagccaagtccctggaatcccaagccccactttcttctgaatcaaaagcataaatacccacccctcaccccttcttcctgaatatcaggcaaatcaactttaccccatgtttgggggcccacagaccccaagtctctgggtttttgtccttagtattgtccgtggcagggtctgcagtctacgtgggtcttctgaaggtgcctgctggggcttcatctcgccttggtggtgcccactgagctctccgcctttgagttttgggttccctggagtgtcccccaagatctgtttcctgagttttcttttttcttcctttcttttttttgaggcacagtctcactgcgtttcccaggttggagtgcagtggtgtgatctcggctcactgcaacctccgcctcccgggtttaagcaaaattatcctgcctcagcctcctgagtagctggattacaggcaggcaccaccacgtccggctaatttttgtatttttagtagagatggggttttgccatgttagccaggctggtctcgaactcctgacctcaggtgatccgcctgccttggcctcccaaagtgctgggattacaggcgagagccaccacgcccagcctctgcttcgtgagttttctttcccctgaggcaccctctgagttctccacgtgtcagacccatgtccaatgcaccacgctccttccttcacaccatgaaagccccgaagtaagaccgggtaccatcacgcagtcgaaccaggcgttcatccagcacacggacgaccaccttctccccagcctccaggtgtaccacaccacccaggaagctgctgtcccaccagacccgggagctgctggtggcccgtccgcagggtgactgctggctgaccaacagctccagctcctcggggtagcggggtgtgcgcttgtagaggccgtgggtgatggtgctggccaggcccagcgggcagcccacaccgcccagctgcaccttggagtagatgtagtagtagccagctttggtgaccacaagggccccatcgtggtagctgaggcccctcaggaaggccaggcccagctgagtctcccataacagcggccccccgctgccggtcaagctggagttggcccctgtgagatgcgctgctgggttgacctcgtgagaccttcgctcttgtatcagctgctcccaggagcctgcaggtccgtcaggcaggcgggtgaccatctctcctagacgccagtgcagctgcaggaggaaccagccttggacggccagcccggcccccatcagcaacagcaagagacccagacccacccgggccacactgcacgactgtctccggtggcttcgtcccagcctcgtgaatgggatgtcggtctgtccatccaccacaaacactgagggccgtacgacactctcctccatgcccaaggtgtctggagcagggctgacacgcctgggtccttcaacctcagaggaaaccgaaattgctcaacactcctgggctgtgcacgct

SEQ ID NO: 15026 - RNA, 3907 nt, Homo sapiens
  source 1..3907: mol_type = other RNA
gctgggattacaggcatgagccactgcacccagccgacatcaccatccttcctgactctgaatttatatactactaaccagcaatcattttcctccacctattcaacacagaagtacctaacagtaaaagatgagagatacctatctggcatgtgagaaaatgatatatagctactgacggggatttcctttgaggatgctgagtaaacttcgtggtgtgtgcctgcatttccactgcaatctatcacatgtgatgagttgtggaatttcccacttgtggcatcacactggggctcaaagagtttcagattttggagcatgtttttttgttttttgagatgggagccttgctctgtcacccaggctggagtgcagtggtgtgatctcagctcactgcaacctcaacctccagggttcctgcctcagcctcccgagtagctggggttacaggtgccccccaccacacccaggtaattttttgtatttttagtagagatggggtttcgccatgttggccaggctggtctggagctcctgacctcaggttatccgtccactttgacctcccaaagtgctgggattacaggtatgagccaccacgcccggcctagattttggagcattttgaatttgggatggtgaatctgtactgttgttcctctccccccacaaccatcttgccgatggggaaactgaagcattgagaggtgatggaaattgctggaggtcatatagctggtgagtggcagagtggactcagaacccaggatcatctgattgcaaaatctgtttccttcatctctgtactgtgcaacaatgacaagaatactattggcgataacaacaataacccacaaattttgacttgtcattcacaacaacaacaaaacaataataacaatacattcacctctggggtcgaaacccatatcctagaatcctaggaactaaggattccctccagccacactgcagcaatgctcatttgcatagaccctctaatttgtatgcatatcattatctgcccccacccaacccaccagctccctgtgttttatgcttccagctggcttggcggattgtcattctgtcctggatgtgtctaataagggcgtcttgcgggatgtagcctctacttcctcaggaattgtggattggagaggaagccagatccagacgtgaggtctctggtttcccccacatttcctgcatggacttgagccaactgggtccaggttcctcatctgtagaatgacctccatgggtcattacctccatccctctgcctctaggagccaccacttgttgctgatggttgccccccatccgactcctccctttccctgtggggctctttaggcctgacaattcctctccacccttcttcagtttgttcccctaagaactagacagatccaggtacaactatttgccatttatttcaaagatcagtggttaagaggcccagggttatgaacaaggtctggtcctcaccccgagatgtgttagtctgggctggggagggccctcaggctgtgtgtatatgtgtgtaatgttgtgtgtttgtcattgtgatgtgtgtgtgatgtgtgtgtcattgtgatgttgtgtgtgtgtaatgttgtgtttgtcattgtgatgtgtgtgtaatgtgtgtttgtcatcgtgatgttgtgtgtgtaatgtgtgtttgtcatcgtgatgttgtgtgtgtaatgtgtgtttgtcattgtgatgttgtgtgtgtgtaatgtgtatttgtcatggtgatattgtgtgtgtgtatgtgtgtaaccaggtctgactataacttggtctgtctgtgtctaatgtaatgagtattaattaccaagtgtgacggtgacacctctgggagtggctgtgtagctgggatgctgtctgagttttgtgtgcttgtgttataacatacacacagtgctgtgactgtctgtgatgccgtctgtgacttccatgtgattgtgtggttgtgcatgaatctggcacttcgcgtgtatgagtctatagttgtgaaagagtggctgagattatgcagccatgtgacagattttgtgggatgccataggtgtgactgtagagtcattcttccttcctttcaatcagcaagcatttccctagagcatgctttgtgccaggccctgggccggatgccggggacagatccgtggtgtcctattagggatgtctatgcttggcagtgatgaaatcagccatggtggtagcatttacaccatggaaattggcaaacattacaaagctgtccccctcccaggacagctggttgttaaacagttatgagcacgctgccgtgctcatgtatctgagtgtaactctttgtgaccaggctgaggtgtggccaccagtctgtgggtgggatctgagtatgtggggtggggctgggctcttcatgatgagtcccgatgatcagtctcccgcccaccctgtccgtactcatgatgagagtagggaagtggatgaagtttcccacccccagccaagtccctggaatcccaagccccactttcttctgaatcaaaagcataaatacccacccctcaccccttcttcctgaatatcaggcaaatcaactttaccccatgtttgggggcccacagaccccaagtctctgggtttttgtccttagtattgtccgtggcagggtctgcagtctacgtgggtcttctgaaggtgcctgctggggcttcatctcgccttggtggtgcccactgagctctccgcctttgagttttgggttccctggagtgtcccccaagatctgtttcctgagttttcttttttcttcctttcttttttttgaggcacagtctcactgcgtttcccaggttggagtgcagtggtgtgatctcggctcactgcaacctccgcctcccgggtttaagcaaaattatcctgcctcagcctcctgagtagctggattacaggcaggcaccaccacgtccggctaatttttgtatttttagtagagatggggttttgccatgttagccaggctggtctcgaactcctgacctcaggtgatccgcctgccttggcctcccaaagtgctgggattacaggcgagagccaccacgcccagcctctgcttcgtgagttttctttcccctgaggcaccctctgagttctccacgtgtcagacccatgtccaatgcaccacgctccttccttcacaccatgaaagccccgaagtaagaccgggtaccatcacgcagtcgaaccaggcgttcatccagcacacggacgaccaccttctccccagcctccaggtgtaccacaccacccaggaagctgctgtcccaccagacccgggagctgctggtggcccgtccgcagggtgactgctggctgaccaacagctccagctcctcggggtagcggggtgtgcgcttgtagaggccgtgggtgatggtgctggccaggcccagcgggcagcccacaccgcccagctgcaccttggagtagatgtagtagtagccagctttggtgaccacaagggccccatcgtggtagctgaggcccctcaggaaggccaggcccagctgagtctcccataacagcggccccccgctgccggtcaagctggagttggcccctgtgagatgcgctgctgggttgacctcgtgagaccttcgctcttgtatcagctgctcccaggagcctgcaggtccgtcccgggccacactgcacgactgtctccggtggcttcgtcccagcctcgtgaatgggatgtcggtctgtccatccaccacaaacactgagggccgtacgacactctcctccatgcccaaggtgtctggagcagggctgacacgcctgggtccttcaacctcagaggaaaccgaaattgctcaacactcctgggctgtgcacg

SEQ ID NO: 15027 - RNA, 3337 nt, Homo sapiens
  source 1..3337: mol_type = other RNA
gctgggattacaggcatgagccactgcacccagcctaataactgatataatttttttaagtgaaatgaaatgttcctttatttacatatgaattaaatagaaaattcaaagtaattcttttaataaaaacccatatactaatatattttaaggttggatactaacagcattttcacaagatccaaagtgtggatgacgaactaggcaataaggacatgtgtgccacataactaagggtaactaaaggaagatgagtacctcacaaccaaaagcagttaactatgcctggcataccaccctgtcatgtgggcagatcactgttcccatgctgggtaagagtctccaagaagggaagcccttatgcagtaattctgtaactatattaaatttggtaatctaacattaaactttttcgtgagcagtgaatatacacatggtcatatgaaaactgccctggagaccgggttaattattaaataaactaaaaggggagaaatgctgatagataaaattatgtcaattccagggtgttcaatggaataaagaaacagcagcagctgcttcaaaagtagactatgatcagaaacctcagatggtaacctttaaaaattgtggaatccagagtctcaacctaaacctacataggagctacagccagggagttctttctaagttcctcaagtgattctgatgattggccaagctggaaacttctgaactgggggagaaagccaacctaggtaaatgtagagacttttagaattcaacatttgattatcatttactccacattttcccccagctgtctcaccttctctatttttctaacagtgaacaataaaagggcttggcaagtgaaggaaaaagtcagtagagtacctaaaatggatttgactatattcaagccactttcatatattaactagataaaaggataccatactgctatttgaaattcaatcacaaagcaaaaatgtcataattttaatgtattttaagggaagacggggttcttaacatgaatatgtaatacaaaaacaattctaaataataatatttaatagaagaaaaaatctgtataattatttagaagtaactctgtttttaaaatttcaatgttaggaagaaaatcccttaaatttgaaatagcggaatattctctcatatgaaaaaactgtgtcccagtgttattcttcaacttagaaattaggcaaagtattttagtactatttctgcttacatattgttttgtatgaatgttttaagtatgaataatattttggtttttagtgtgcatgctaatataaaaatatggatttttttctcctacactgactttgtacactttccaggcccgaagaataaaaaacttttaaaatatcctgtgttcactagcaaaccttggaacgataaaaaaaggtagtacctacataagaaattttacattgaaattacaattgtatgtttttcaggagttaaagtgattcaatttttcaatattcaaacacaaaatagtaaatttttatttactatagcacaattcaagtattctcttaaatttatatttagtcaactaaaacatgacagtgactttataagagctttccttttaaaaggttgctgttataaaaaagtatgactctattactctaaatgcttagaataagtggaaagaacaaatgacagtagacaaaaacctttatgagtgagtcatcaacacataaaaggttgcacacatcagtaataggacatgtgaaggtaacatcccaaaagtatttgaactcatgtaaacaaagactatgtatattcctaagggagaaaatgtactaccaagataaaatatattcaaacggctgtgactttaaaccatgtattagttgaataccacacaaaaccaaaaaggcattatctatcatttaataactgaaagatattacttatttgtgagataaaaggataatgcttttttaaaaccaataatgaaaaagaagtattttgaaaacaaacatctgtttgctagaaataaatatacttgcttagttattttaatgtattgcagcataggaatattgtgctagcattgaccattaacattcaatcagtagtttaaaatattttttccacattgagtcttgaatcctctacctggtcagctgacccacaactttcaaaagagttttattttcctgctttagctgttcattttcatcttctatgtcatctaggtctctatttaataaatcaatttcttctttgagttttccaatcatttcctctttatcttgcatcagtctcacaagtcttaggttttcttgtctttctcttactacttccttttcaagatcttcaattttcttttccagtgtgctacttgaaaccagagtacctgaaacatttgcatccctgttatatctagggaacccacttctatctgttcgagaatatctacttgagacatcttcttcagagacactggttgtgcttttatatctgcctgaaactgttctaggtggctcctgtagcagataggaactgcctggatctagtaagtttacagcttcattctgaatagtgttctgttgtgtaattgcatcttctcgtttccgctctttctgccctgcttcatcatcttcgtactcatctaagcactctgcggcagggatgttgaccacgccggtggagcgccgcttctcccgcagcttcctcttctcgatctgccccttgcctttcctggcactggggcccgagctcttgcccttctctgggacgccgtccggctcctcctcgtcacgctggggcggcggtgcagccgaggcagaggcggctgggggctcgtcctccgaccgccgcgggccgggggccgcccgcgtcagcatggcggagccgaccgcgcagttcacgcccccgggaccggggacggcaggtgcggccggcgcgccgcccgggaggttgttgttgagctcgttggcagcggcggccgccggggtgcccagagcccccgcggggggcttcccagcggcgtcgctgctgccccctcccgggggggccgggcccggggggttctgcttggcgcgcatcttctcgcgtttcgccttccactcctccaggaagtctgtggtgctgccgccgaggccgctgctggtccggtagccaccggtcgccatattcccaaaggggccggtcgggctctcacctcaggccgcccaccagggctccggccgctgcctcctcttccttcctgcggccccgaggatgccaggagacgacctccaggagagggacggccgccgctcccacagcagccggcggggctacagtacggaccccgacgatcgcc

SEQ ID NO: 15028 - RNA, 3426 nt, Homo sapiens
  source 1..3426: mol_type = other RNA
gctgggattacaggcatgagccactgcacccagcctaataactgatataatttttttaagtgaaatgaaatgttcctttatttacatatgaattaaatagaaaattcaaagtaattcttttaataaaaacccatatactaatatattttaaggttggatactaacagcattttcacaagatccaaagtgtggatgacgaactaggcaataaggacatgtgtgccacataactaagggtaactaaaggaagatgagtacctcacaaccaaaagcagttaactatgcctggcataccaccctgtcatgtgggcagatcactgttcccatgctgggtaagagtctccaagaagggaagcccttatgcagtaattctgtaactatattaaatttggtaatctaacattaaactttttcgtgagcagtgaatatacacatggtcatatgaaaactgccctggagaccgggttaattattaaataaactaaaaggggagaaatgctgatagataaaattatgtcaattccagggtgttcaatggaataaagaaacagcagcagctgcttcaaaagtagactatgatcagaaacctcagatggtaacctttaaaaattgtggaatccagagtctcaacctaaacctacataggagctacagccagggagttctttctaagttcctcaagtgattctgatgattggccaagctggaaacttctgaactgggggagaaagccaacctaggtaaatgtagagacttttagaattcaacatttgattatcatttactccacattttcccccagctgtctcaccttctctatttttctaacagtgaacaataaaagggcttggcaagtgaaggaaaaagtcagtagagtacctaaaatggatttgactatattcaagccactttcatatattaactagataaaaggataccatactgctatttgaaattcaatcacaaagcaaaaatgtcataattttaatgtattttaagggaagacggggttcttaacatgaatatgtaatacaaaaacaattctaaataataatatttaatagaagaaaaaatctgtataattatttagaagtaactctgtttttaaaatttcaatgttaggaagaaaatcccttaaatttgaaatagcggaatattctctcatatgaaaaaactgtgtcccagtgttattcttcaacttagaaattaggcaaagtattttagtactatttctgcttacatattgttttgtatgaatgttttaagtatgaataatattttggtttttagtgtgcatgctaatataaaaatatggatttttttctcctacactgactttgtacactttccaggcccgaagaataaaaaacttttaaaatatcctgtgttcactagcaaaccttggaacgataaaaaaaggtagtacctacataagaaattttacattgaaattacaattgtatgtttttcaggagttaaagtgattcaatttttcaatattcaaacacaaaatagtaaatttttatttactatagcacaattcaagtattctcttaaatttatatttagtcaactaaaacatgacagtgactttataagagctttccttttaaaaggttgctgttataaaaaagtatgactctattactctaaatgcttagaataagtggaaagaacaaatgacagtagacaaaaacctttatgagtgagtcatcaacacataaaaggttgcacacatcagtaataggacatgtgaaggtaacatcccaaaagtatttgaactcatgtaaacaaagactatgtatattcctaagggagaaaatgtactaccaagataaaatatattcaaacggctgtgactttaaaccatgtattagttgaataccacacaaaaccaaaaaggcattatctatcatttaataactgaaagatattacttatttgtgagataaaaggataatgcttttttaaaaccaataatgaaaaagaagtattttgaaaacaaacatctgtttgctagaaataaatatacttgcttagttattttaatgtattgcagcataggaatattgtgctagcattgaccattaacattcaatcagtagtttaaaatattttttccacattgagtcttgaatcctctacctggtcagctgacccacaactttcaaaagagttttattttcctgctttagctgttcattttcatcttctatgtcatctaggtctctatttaataaatcaatttcttctttgagttttccaatcatttcctctttatcttgcatcagtctcacaagtcttaggttttcttgtctttctcttactacttccttttcaagatcttcaattttcttttccagtgtgctacttgaaaccagagtacctgaaacatttgcatccctgttatatctagggaacccacttctatctgttcgagaatatctacttgagacatcttcttcagagacactggttgtgcttttatatctgcctgaaactgttctaggtggctcctgtagcagataggaactgcctggatctagtaagtttacagcttcattctgaatagtgttctgttgtgtaattgcatcttctcgtttccgctctttctgccctgcttcatcatcttcgtactcatctaagcactctgcggcagggatgttgaccacgccggtggagcgccgcttctcccgcagcttcctcttctcgatctgccccttgcctttcctggcactggggcccgagctcttgcccttctctgggacgccgtccggctcctcctcgtcacgctggggcggcggtgcagccgaggcagaggcggctgggggctcgtcctccgaccgccgcgggccgggggccgcccgcgtcagcatggcggagccgaccgcgcagttcacgcccccgggaccggggacggcaggtgcggccggcgcgccgcccgggaggttgttgttgagctcgttggcagcggcggccgccggggtgcccagagcccccgcggggggcttcccagcggcgtcgctgctgccccctcccgggggggccgggcccggggggttctgcttggcgcgcatcttctcgcgtttcgccttccactcctccaggaagtctgtggtgctgccgccgaggccgctgctggtccggtagccaccggtcgccatattcccaaaggggccggtcgggctctcacctcaggccgcccaccagggctccggccgctgcctcctcttccttcctgcggccccgaggatgccaggagacgacctccaggagagggacggccgccgctcccacagcagccggcggggctgtcggctcgtcgtatcgcctgctccgcgctctagccaccgccggtccgaggtccccgtcagctacaaccccactcccaaggcgaggcgcggagctcctagccggttcgcagag

SEQ ID NO: 15029 - RNA, 3404 nt, Homo sapiens
  source 1..3404: mol_type = other RNA
gctgggattacaggcatgagccactgcacccagcctaataactgatataatttttttaagtgaaatgaaatgttcctttatttacatatgaattaaatagaaaattcaaagtaattcttttaataaaaacccatatactaatatattttaaggttggatactaacagcattttcacaagatccaaagtgtggatgacgaactaggcaataaggacatgtgtgccacataactaagggtaactaaaggaagatgagtacctcacaaccaaaagcagttaactatgcctggcataccaccctgtcatgtgggcagatcactgttcccatgctgggtaagagtctccaagaagggaagcccttatgcagtaattctgtaactatattaaatttggtaatctaacattaaactttttcgtgagcagtgaatatacacatggtcatatgaaaactgccctggagaccgggttaattattaaataaactaaaaggggagaaatgctgatagataaaattatgtcaattccagggtgttcaatggaataaagaaacagcagcagctgcttcaaaagtagactatgatcagaaacctcagatggtaacctttaaaaattgtggaatccagagtctcaacctaaacctacataggagctacagccagggagttctttctaagttcctcaagtgattctgatgattggccaagctggaaacttctgaactgggggagaaagccaacctaggtaaatgtagagacttttagaattcaacatttgattatcatttactccacattttcccccagctgtctcaccttctctatttttctaacagtgaacaataaaagggcttggcaagtgaaggaaaaagtcagtagagtacctaaaatggatttgactatattcaagccactttcatatattaactagataaaaggataccatactgctatttgaaattcaatcacaaagcaaaaatgtcataattttaatgtattttaagggaagacggggttcttaacatgaatatgtaatacaaaaacaattctaaataataatatttaatagaagaaaaaatctgtataattatttagaagtaactctgtttttaaaatttcaatgttaggaagaaaatcccttaaatttgaaatagcggaatattctctcatatgaaaaaactgtgtcccagtgttattcttcaacttagaaattaggcaaagtattttagtactatttctgcttacatattgttttgtatgaatgttttaagtatgaataatattttggtttttagtgtgcatgctaatataaaaatatggatttttttctcctacactgactttgtacactttccaggcccgaagaataaaaaacttttaaaatatcctgtgttcactagcaaaccttggaacgataaaaaaaggtagtacctacataagaaattttacattgaaattacaattgtatgtttttcaggagttaaagtgattcaatttttcaatattcaaacacaaaatagtaaatttttatttactatagcacaattcaagtattctcttaaatttatatttagtcaactaaaacatgacagtgactttataagagctttccttttaaaaggttgctgttataaaaaagtatgactctattactctaaatgcttagaataagtggaaagaacaaatgacagtagacaaaaacctttatgagtgagtcatcaacacataaaaggttgcacacatcagtaataggacatgtgaaggtaacatcccaaaagtatttgaactcatgtaaacaaagactatgtatattcctaagggagaaaatgtactaccaagataaaatatattcaaacggctgtgactttaaaccatgtattagttgaataccacacaaaaccaaaaaggcattatctatcatttaataactgaaagatattacttatttgtgagataaaaggataatgcttttttaaaaccaataatgaaaaagaagtattttgaaaacaaacatctgtttgctagaaataaatatacttgcttagttattttaatgtattgcagcataggaatattgtgctagcattgaccattaacattcaatcagtagtttaaaatattttttccacattgagtcttgaatcctctacctggtcagctgacccacaactttcaaaagagttttattttcctgctttagctgttcattttcatcttctatgtcatctaggtctctatttaataaatcaatttcttctttgagttttccaatcatttcctctttatcttgcatcagtctcacaagtcttaggttttcttgtctttctcttactacttccttttcaagatcttcaattttcttttccagtgtgctacttgaaaccagagtacctgaaacatttgcatccctgttatatctagggaacccacttctatctgttcgagaatatctacttgagacatcttcttcagagacactggttgtgcttttatatctgcctgaaactgttctaggtggctcctgtagcagataggaactgcctggatctagtaagtttacagcttcattctgaatagtgttctgttgtgtaattgcatcttctcgtttccgctctttctgccctgcttcatcatcttcgtactcatctaagcactctgcggcagggatgttgaccacgccggtggagcgccgcttctcccgcagcttcctcttctcgatctgccccttgcctttcctggcactggggcccgagctcttgcccttctctgggacgccgtccggctcctcctcgtcacgctggggcggcggtgcagccgaggcagaggcggctgggggctcgtcctccgaccgccgcgggccgggggccgcccgcgtcagcatggcggagccgaccgcgcagttcacgcccccgggaccggggacggcaggtgcggccggcgcgccgcccgggaggttgttgttgagctcgttggcagcggcggccgccggggtgcccagagcccccgcggggggcttcccagcggcgtcgctgctgccccctcccgggggggccgggcccggggggttctgcttggcgcgcatcttctcgcgtttcgccttccactcctccaggaagtctgtggtgctgccgccgaggccgctgctggtccggtagccaccggtcgccatattcccaaaggggccggtcgggctctcacctcaggccgcccaccagggctccggccgctgcctcctcttccttcctgcggccccgaggatgccaggagacgacctccaggagagggacggccgccgctcccacagcagccggcggggcttggaggagcttgtaggggacgaggcgtagggctgggatccggctcccaggtgtgccgaagctggcgcgcgctcttccgccgcgcggaaagt

SEQ ID NO: 15030 - RNA, 4312 nt, Homo sapiens
  source 1..4312: mol_type = other RNA
gctgggattacaggcatgagccactgcacccagcctcaattgtttaaaattcagttttctttacctgaagatatgaatgtatgaattattagagtggttatttaggaggaaaagcgtgtaaagttaagtttttagaatttagactgtttgaaactctgaattcatgtcagtcagtagccattttaaaaccctacaatgacttcatgttccttgctttaatatttccattgtagtgactaaatattggagccaaaattccattagttcaatttattttaaaagtttctgatttgtatatctgtacagataagaatcttaattgaatgacagtaactacaagttttatacctgtggcaaatactgtattagcatctatagatttagggcaatctttaagaaaaaatggaatggtcagagtctaagttatttcatcactgtactttggttaatgtgaactatgattcatatattttatcctttcaaactgaaattacctgctagagtgagcaaccatctcaccactgtggctctttagcttttcccatatgtaatctagaggtactggaataataagaacacaaaatcataatgaaggctgccaaagattataattttttattaagatctcgagtaactccctgtaagctcactgtggtaaatagatttggttctaataccacaattcctcaaagctctatgttcttaacggtgctgtcttaatagaaataaaatgtaaaccatgtgtgattttatcttttctagtaagcacatttaaaaataattggaaacagatgattcttttttttgagacagagtctcactctgtcgcccaggctggagtgcagtggcacaatctcagctcactgcagcctcctcctcctgggttcaagcaattctcctgcctcagcctcccaagtagctgggactacaggtgcgcaccaccatgcctggctaatttttgtatttttagtaggcagggttttgccacactggccaggctggtctcgaactcctgacctcaggtgacctgcccaccctggcctctcaaagtgctgggattagaggcgtgagccactgcgcctggccaagattcattttaattgtgtatttttctttaacccaatatttccaatgttaacatttcaacatgtaatcaatacaaaaaattaggagatatttaaccttttattgtcctttagagcacatctcaatttggactaaccatatttcaaatgctcaacagctacatatgggtagtggctactgcactggacatcgaagttctagaactctctcttacaaatgaacactatcactgtcgttgaaaactttcttgagatagtttattttatacaaacaaactgtatttcttattattcctgaaatatctcatattggcatcctgccatttcattgtagtgcctatcatttttccattgatactgataaagttgcctaagacacaacttcctacatagaggaaataagaggaacaaaccccttttggacagaatctattaaaactcattccactatccctatgtacataaataacattgcctctgctgagtggaatttgcattcgttacttcaaaattcagactcatctacctttccaagttagacagttggggaaagaacttcctaaatcttaaggttgaaggcagagggctcaaccccactccagattcaggcaaggggaataggaaagaaagtgcgagataagagcatggtggcctcttggggtcccttgatgggggctgttgggaagtggaaggcattcttttaaggggataagaagcaaatggaagacttgctccaactctagagttttcagagagttagaggaggtggagagatttactcctgccatggatcatatgcatttctaccatcaactcctggttttgcagtatttttataaatggagtttggaccttggtgacactcagcctctcttccccttttcctatgttgctcaatcttcctttccctcctaggttcttacacatttcaaacccttgccaataacagtattttagttatcaggtctcaccattccctctggttgttgagcctttggataaaaatccacatggctatggagtgggttttgttggaaaaagtgaccgtcctctaactgcacctctatttctggctcctcaaacagcaaagggtaataataaggcatggtagaggttttcccatttttcagtgactagactgtgaatatttacagatgaattttctattattaatgttattgtggttgttttaaaataaaagttctgaatgtatatatgaccaaaacaaacaaacaaaaagagcacagtgaactcaaatcatattccattacaatagtcccaggacttcattagacagactcccagtaattaagcctccaatcttaaaatgttaaacatttcaacatgtattgactaattcctgtaaaatacagaaagtgcaacatcaccaaacgtgcatttcccaggattcattttagaattctcatgaaaatttaataatagtatttcagttaattatggcatttgagaaaaagatactaatggggaaagatcacatacatgctttgggtgatacgttaaaaaaacctacaataattagtagtattgccttaacatttctaaaatcacataaaaatgatcatctttgattgccatttcagtaattttgaatacagggtatgttattttctgctcactagtaatcaaaacacataaaacagacttgtaacaaatattcagagtcgattattttcataagctaaacagttccgatactttaagatttgtgtttgagcatacagtactgcaatgttggctacataaaataaaaaaatctttttaagaggaagctcaataatcagaggctgtattgcatttaaggatttaacactggctatatacaaaagggaaagcatttcaatgagaaatacttcacgttaccaagttctctcctttaatatggcaacattcagcagcttatgctactcttttatcctttggttcccagtgacaaacaatgcagtaataatgcctctggttttagttcctcttggatgacatttattagcagagagagagacctgatgctttagctgaaatttggcagcccaagaagtgcaccaactgctccaaagtaaccctcatgttctagaaacaatgcttttagttgaccttttgaccagtaatccagtgcatatgccaaaagtttcattgagagggtattgacacgtaaaaagtttccaacaaagacaactctgtttattttctcattaacagcacacattcgtgccacagaaccaatgttattggtgatagtaactaaagtagctcttgccagatcttctttactaacagattctcgcttctccttataaatcatattcccaaaactagatgctacagcccaacctggcaaaccaaatctttcataatctcctccataaatatcacggaccagcttgtcagcttgtgtgctatcacctttggatgccatttcaagagcctcttcaaaactttcacagccagtcaataaactgcataaacccagaaaggtaccccctccaaggcttgtcccagtcactcgtttatagttgtctttggaatggactgctaaaatactgactcctgagccaatgttcactacaagcagtggatagggatcatccaggttaaaaggcatcttttggcatcgctcaggttctgaggcattagcaaaataatagcactcggcttgtccattgaaactgacagagtctatatacagcaagccctttacaaggcagtcaagttcatccagtttgtgcaggtggaggtttccaattgtgcgaaaatctttttcaaacttgtaagcaccacctcctgtagcacatagcaccgtctgcaatgttgagaagtttttatctcttcccatttggataaaagtaggcaggtcctgggttggaaacctgataaagtgcaagttccctcttcggccaaaaagtgttaaatctttcagttcaaggtgtacatcccgaatgccggtggatccatatgccacgttagaagtcaaatatttccgaatactttttaaactctcaacttcttcttgctcttcctctgctgtgatatcaataggttcaaagtacgagagctttactagagttcccccaatgtccatgccaaaccatgggaaagagggtttcttggcatctttgatcttcatggcgtcggcccgaggggcgatggacggcctccgatccggggcactgagagcagaggcggcgactccggaggtggctgggccgcgc

SEQ ID NO: 15031 - RNA, 157 nt, Homo sapiens
  source 1..157: mol_type = other RNA
gctgggattacaggcatgagccactgcacccagcctgaacttgcatactttcttgtcatctttttgcttccctgtaattcagtttgtttcgttcacatgtcgtacacctagcagcaaaacacctttccaaatctctgcctctagtgtaaagagccca

SEQ ID NO: 15032 - RNA, 1409 nt, Homo sapiens
  source 1..1409: mol_type = other RNA
gctgggattacaggcatgagccactgcacccagcctgacaaatttcttttcaaaggcttattccagtttcctaaggctagcatgagatgtatacattttccagggacaaatttgtacttctgaattgactcaggcagcacaggctacgtatctcatcacagtccatttagaagcatttgcggtgaacagtggaggggcctgactggtggcactcccgcttgctgatccacattggctggaaggtggacagtgaggccaggatggagctgctgatccacatggaatacttgtgctcagagacagccatgatcttgatcttcatggtcctgggtgctggggcagtgatctccttctacatcctgtgtgtgatacttgggtgcatggcaatgctgccagacagcaccacattggtgtacaggtccttgcagatatccacatcacacttcatgatggaggtcaagatggtctcctggatgcagcaagattccatgcccaggaaggagggctgggacagcgcctctggacaccagaaccactcattgctgatggtgaccaccaggctgtgggagagcttgtagctcttctccaggaaggaagaggacacggcagtggccatctcctgctgcaagtccaaggcaacacagcatagcttttcctggatgtcacgcacaatcccccacttcactgtggtgatgaagctgtagcgggcccctcgaggatcttcaccacgtagtcggccaggtcccggccagccagggccaaacacaggatgactgggagagggtggctgtatccttggagatgggcaagtgtgggtgaccccatcgcctgagtcccccatggtgccaatggcactgacagaggcatgcagggacagggtgacctgaatggccctgtacttgactggggtgttgaaggccccaaacatgatctgaatcatcttctctctgttggccttggggctcgggggcctcggtcagcagcaccagttgctccttaggggccacgtgcagcccattgcggaaggtatggtgctagatcttccccatgtggtcccagttggtgatgaggcctgctccatggggtgcttcaggatcaggatgctgcttgctctgggcctcatcgcccacataggagtcctagcccctgcccaccatcatgccctggtgccaggggtgcctgacaatggagaggaacatgacttgagggcattgtccccagcaaaggcagacttgcacatggcaaagctattgtcaacaatgagcaaggtgatttctgcttccattgtgatcgttctggaggctgagaagttcaagatcaaggtgctggcagatgtggttcctggtgagggtcctcttcccagtttgctgatggcctccttcttgctgtgtgctagttattgatgctca

SEQ ID NO: 15033 - RNA, 1311 nt, Homo sapiens
  source 1..1311: mol_type = other RNA
gctgggattacaggcatgagccactgcacccagcctgcatttctgctttttaactttctagttacttgtatgtcctcgctttcgtacgtgcagtttggttgagagatgttagtggacagatgatggacatgaaagacgggttagaatgggagggaaatacacctgctatttttgtaccctagtatgtcctagtggtaaaaatgtgtcatatgcaactgcaaaagaaaggggaacatgttaaatgtcctagttttttctgttatctcaatgtgttgctctattcctattaagttttcctctcacatttactacaattagttctatattatcttgacaccattttctacgcttaaaacaacctcttccccctaactttaaaatcaggtacagtaaaagcctcttgttgaggatgtggttatcttggtagatgagagtgtgtcagaaacaggtagaaacttacctagcaaaagaactagtactgtatcttgacttgttatatggcaacaatcaattagatgataatttctatttaaaagcattctatatggggaaagacatgttcattttgataagtaaagacaaaatctaggtttttagttgatgtgtgttgtacatgtggtctttggaaagcaaaccaaactatgtattattgacattaaaaatgatgacttaatgctgggtaaatcctgtactcagaagatactcactgatgatccatccctgggtaaaccttctttgtctacactcattatctgtgatctcatccagtcttgtggctttaaatactatatggtgacaactacagccgagacctctcccctgaacttcagactcttctgtccagaagattatacaaattctctgtttggttatagaatttagaatgccccaaatcaagataattctccctcaattctgttcctcctataagcttccccaatcggtaaatgaaaactgtgtccttctagttaatcataccaaaatcctaaaaatcatccttaactcctctcatctctgatatccatatccaacccatgagcaaatactgtcaatctgccagaatccaaacatctctccagccccattgccaccaccctggtccaagccaccaccaggccttgcctagaatattgcaatacttttttttttttttttttttttttttttttttttgagacagagatggcatctcactctgttgcccaggatggagtacagtagctcaatcatagcttattacaacctccaactcctggatcaagcaatcctcccaactctgcgtcccgagtacctgggactataggcatgtgc

SEQ ID NO: 15034 - RNA, 5327 nt, Homo sapiens
  source 1..5327: mol_type = other RNA
gctgggattacaggcatgagccactgcacccagccttcaactgcttatttctaaatagcttctgagtgtcctgtgttggtaaagttaatatctcccaactcctagattgtacacataggctcctttgattttcttttaagaattctgttgctttaaaattttacgtcttaaagccacccagaatttatttttgtgctgttaatccaaattttcttcctttaagattaaaaggttctgttccagaattctttttaagtaaactactcttttcccctgtggtttcagatttcacctttttcacatatgaaaaagttcatatatatcgaagtctatttctgaattttctactgtgttctaatgatgtatttacctgttcctttgccaatacaatattaatttcattagaatggcttcatgttatcttctggtatctagcatggcattttaaaaatttttaattattatagatatataattgttgtatatatttattgggtacatgtgatgtttttatacatggtatgatttttttcatatatttttttcaatgattgtcaaaaaatcattgagatttagtgtaattccaaaagaagtacatataaattatgttttcttgtcagtatggagaacagctcttgattttggtaccctgtcttcttagaaaagttaactcaaaaaatagtcttttcatttattggtgtacaaccatatcatcagtaaaaatggatagttttaccttttctgctgtttataccaattcatttctttttattgccttcactggaatctctaagccaatattgaattcctgattttaaaaaatggctttggcataatatatgctttggggtttgggttaaaaaaaattttttttaagaaaaaccgctttaagtggttcccatctattacaatgtaaattaacacattctatgaaatgccttctcagtatctgttgagagttcatatgattcttctcctttaaactgttaatttgattgatgcatttcctattaactgaactggtttggcattcttgggatgactcttactatgtcactctttgggtatatggctgaattctatttgctagtattttaactataatttttgtttctatattcatgagtaagactggtctgaagttttctttttttttttttttttttgacggagtttcgctcttgtcacccaggctggatggcacgatcttggctcaccgcaacctctacctcctgggtacaagcaattctcctgcctcatgcctcaacctcccaagtagctgggactacaggtgtgtgccaccacacccggctaatttttgtatttttagtagagatggggtttcaccatctcgaacttctgacctcatgatccacctgcctcggcctcccaaagtgttgggattacaggcgtgagccaccgcacccagcagaagttttcttttttcaactatctgtatttgattttggtgttaaaatttattctgacttaataaaataaatgagtacagttcatggattgtattacatccatataataaataacactggtattactctttctttaaaagatagaactaagcatgaactcttctgagcctggagcattttcccattatagatctttaatagcttttttgagtttttcaatgttaactatcctaccaagttttctacttcttattgcagttttcataacttaagtttattagaaaagcatccacctcctctttttaaaaaatatgttgattagagttgtatgaggtatctttttatcacttaaaaaatcatattgatatctgtggttatgtctcctttctcattctggatcaggcagtcttacatggagggaaatcttgaaaaatgtagattccacatggccatttattttctaatatggatgacatagcaactcagggaagcagacttctttccaaacattgaaataattaaaaccttgggatttagtgtctaggacacttgcaaggaaatttatatgaaaaaaatgaatattcttgaattaatttgcagagggatagagagaaaagaaattctccttcagtggtctacgcatgaaacatttctgagttatacaacctgtatatagaatagtgtatctagaatagtgtagcaatgctactaatttgctacaagatattttaagcaagactaagaaaatatgaacagtgtactgtacaccagggtgacactacattttgtcaaatagtttacagtgtttcatttacccagtatcaggttcttaaactattccttagcttgcatttttaatataaataactacattttagtaaaatttttggccaaattatccaaatacatttaaaaacactgctttattatttctgcagaggacagtaacaacctctatagccatttacatgtattacaaaaaggtggaaaaatgtagctggtataataaagttcttttaacaatagtgggccatgttgttgttatttttttgtattgttaagacatcaaaagacaatgatgatatttaaagtggaaaagttttctgaatggcattctatatgttgtgtgacatgtgtctgatattcacattttatgttaatttcacatttacaactccaaaatacaaataatgctgattgtatggctcactgtggaatataccagagtatgcctttaagtctcttcacagatattttgtattctgctgttattccatttaatacatttttaaacgtttacatgccagggtgtccatgcttatgtttgagaaagtattttctagaaaagtttgtatcacaattagatcatgatttccattatgatacaacactgtcggttgggcgcgttggctcatgcctgtaatcccaacactttgggaggccaagggcggggggttggggggtatcacgaggtcaggagttcgagaccagcctagccaaagagaccagcctgaccaacatggtgaaaccccatctctactaaaaatacaaaaattagccaggcgtggtggcaggtgcctgtaatcccagctacttgggaggctgaggcaggagaactgcttgaacctgggaggctgaggttacagtgagccgagatagtgccattgcactccagcctgggaaacagagaatacaactcaaaataaataaataaataaaataaaaacacactgttcaaattcattaaaatgataagatttctcctaaggataaattccctacataccggccaggcgcggtggctcacgcctgtaatcccagcactttgggaggacaaggcgggcagatcacaaggtcaggagatcgagaccatcctggctaacacggtgaaaccccgtctctactaaaaatacaaaaaaaaaattagccgggcatggtggtgggcacctgtagtcccagctactcgggaggctgaggcaggagaatggcgtgaacccgggaggcagagcttgcagtaagccgagatcgcgccactgcactccagcctgggtgacaaagtgagattccaactcaaaaaaaaaaaaaaaaaattccctacataccatgaaaccagatattttgctcaagtatttcccacaattattaagttttcattcctgtaggcattcttccgagcatgaattttctgatgtctgctgaggtttggcttctggtagaaagctttcccacattcattgcacccatagggcttctctcctgtgtgagttctccaatgtttattgaggcatgacttctggctgaaggattttccacattctctgcaacgatacggtctttctcctgtgtgcatttttcgatgtacattgaggtatgacttctcaccaaacgatttcccgcattcactgcagacaaagggtctctctcctgtgtgtgttctctgatgttctgtgcggtgtgacttctgggtaaaggctttcccacaaaaaaaacattcaaagggtcttaccccagtgtgaattctctggtgtttgatgagggttgacttatgtgaaaaggctttcccacagtcagtgcagccataaggcttctccccagtgtgacttctctgatgcctaatgaattcagacttgtagcagaaggctttcccacactcactacagacgtggggtttttctgtaggtggaaccctcttccgtttgtacaagagagaatcacttactgctggtttatacataagtgccgggttctgggtgaaagctttctcacagtgactgcaaccccggggcttttctccattaggtcgtctaccatgatttatacgctgaagcaatttcccataagcataacactcatcttgcttttttgcacagtttctcttaaaaccaatcaagtctaaattatggttcaaattctttccacaagggttccagttactagggctctggattgaagaaaaaagatcagtgctcagaagtgatattttcccaaacttattatattcacagcttttctccttgggcaatgttttcttgcttatggctgcgcctggcctcaaaagcatgtcttgccgtcttttcctctggatattaactcgccagatgtcttcccaacagtggcagcccgggcatgctgcctcaccaatccatggtgcttcttcctgctccagtctgaggatcacatctggtttggtgccttcataacccactgagacgaggttgctataggtttccagcatcacatcccggtacagggccctctgagcaggactcagccggtgccactcctcttgggtgaagcccacaaccacatctttgaatgacacaggtatctggtattcgatcattttctgctgttcttgaaaaagatctgacacctatactcttcaaaaatgtcgacttcatggaagatgaacactgagaaactgctcctgattaaaggagactaaagggatgtgtcacctaaaggcagcatatgatcctggattagatcacttagctgcagggccttctgtagatgttgtgaccaaggtcctgtggctctaagggctggcaggagctagagagccctcccgtccagcaaggtggcaggatccaaaggtctgcagggcacccagagaactcagtaaatttgttttctaaccacgggcaaggtcacatccatccccgctgtcacagagtcagaatggatttccagaaaccagcctcactcttgggatgctggcacagatgcgtatgtcattacctttgccagaaagagccccatgcaccctgaaaatcaagacatttcacagaactcgcatttattgattcccacacactcccaatccatcttcttcagagaccgtgccactgactcccgcaaacctctgtccgccaccactgaggccccgcgaggctc

SEQ ID NO: 15035 - RNA, 5215 nt, Homo sapiens
  source 1..5215: mol_type = other RNA
gctgggattacaggcatgagccactgcacccagccttcaactgcttatttctaaatagcttctgagtgtcctgtgttggtaaagttaatatctcccaactcctagattgtacacataggctcctttgattttcttttaagaattctgttgctttaaaattttacgtcttaaagccacccagaatttatttttgtgctgttaatccaaattttcttcctttaagattaaaaggttctgttccagaattctttttaagtaaactactcttttcccctgtggtttcagatttcacctttttcacatatgaaaaagttcatatatatcgaagtctatttctgaattttctactgtgttctaatgatgtatttacctgttcctttgccaatacaatattaatttcattagaatggcttcatgttatcttctggtatctagcatggcattttaaaaatttttaattattatagatatataattgttgtatatatttattgggtacatgtgatgtttttatacatggtatgatttttttcatatatttttttcaatgattgtcaaaaaatcattgagatttagtgtaattccaaaagaagtacatataaattatgttttcttgtcagtatggagaacagctcttgattttggtaccctgtcttcttagaaaagttaactcaaaaaatagtcttttcatttattggtgtacaaccatatcatcagtaaaaatggatagttttaccttttctgctgtttataccaattcatttctttttattgccttcactggaatctctaagccaatattgaattcctgattttaaaaaatggctttggcataatatatgctttggggtttgggttaaaaaaaattttttttaagaaaaaccgctttaagtggttcccatctattacaatgtaaattaacacattctatgaaatgccttctcagtatctgttgagagttcatatgattcttctcctttaaactgttaatttgattgatgcatttcctattaactgaactggtttggcattcttgggatgactcttactatgtcactctttgggtatatggctgaattctatttgctagtattttaactataatttttgtttctatattcatgagtaagactggtctgaagttttctttttttttttttttttttgacggagtttcgctcttgtcacccaggctggatggcacgatcttggctcaccgcaacctctacctcctgggtacaagcaattctcctgcctcatgcctcaacctcccaagtagctgggactacaggtgtgtgccaccacacccggctaatttttgtatttttagtagagatggggtttcaccatctcgaacttctgacctcatgatccacctgcctcggcctcccaaagtgttgggattacaggcgtgagccaccgcacccagcagaagttttcttttttcaactatctgtatttgattttggtgttaaaatttattctgacttaataaaataaatgagtacagttcatggattgtattacatccatataataaataacactggtattactctttctttaaaagatagaactaagcatgaactcttctgagcctggagcattttcccattatagatctttaatagcttttttgagtttttcaatgttaactatcctaccaagttttctacttcttattgcagttttcataacttaagtttattagaaaagcatccacctcctctttttaaaaaatatgttgattagagttgtatgaggtatctttttatcacttaaaaaatcatattgatatctgtggttatgtctcctttctcattctggatcaggcagtcttacatggagggaaatcttgaaaaatgtagattccacatggccatttattttctaatatggatgacatagcaactcagggaagcagacttctttccaaacattgaaataattaaaaccttgggatttagtgtctaggacacttgcaaggaaatttatatgaaaaaaatgaatattcttgaattaatttgcagagggatagagagaaaagaaattctccttcagtggtctacgcatgaaacatttctgagttatacaacctgtatatagaatagtgtatctagaatagtgtagcaatgctactaatttgctacaagatattttaagcaagactaagaaaatatgaacagtgtactgtacaccagggtgacactacattttgtcaaatagtttacagtgtttcatttacccagtatcaggttcttaaactattccttagcttgcatttttaatataaataactacattttagtaaaatttttggccaaattatccaaatacatttaaaaacactgctttattatttctgcagaggacagtaacaacctctatagccatttacatgtattacaaaaaggtggaaaaatgtagctggtataataaagttcttttaacaatagtgggccatgttgttgttatttttttgtattgttaagacatcaaaagacaatgatgatatttaaagtggaaaagttttctgaatggcattctatatgttgtgtgacatgtgtctgatattcacattttatgttaatttcacatttacaactccaaaatacaaataatgctgattgtatggctcactgtggaatataccagagtatgcctttaagtctcttcacagatattttgtattctgctgttattccatttaatacatttttaaacgtttacatgccagggtgtccatgcttatgtttgagaaagtattttctagaaaagtttgtatcacaattagatcatgatttccattatgatacaacactgtcggttgggcgcgttggctcatgcctgtaatcccaacactttgggaggccaagggcggggggttggggggtatcacgaggtcaggagttcgagaccagcctagccaaagagaccagcctgaccaacatggtgaaaccccatctctactaaaaatacaaaaattagccaggcgtggtggcaggtgcctgtaatcccagctacttgggaggctgaggcaggagaactgcttgaacctgggaggctgaggttacagtgagccgagatagtgccattgcactccagcctgggaaacagagaatacaactcaaaataaataaataaataaaataaaaacacactgttcaaattcattaaaatgataagatttctcctaaggataaattccctacataccggccaggcgcggtggctcacgcctgtaatcccagcactttgggaggacaaggcgggcagatcacaaggtcaggagatcgagaccatcctggctaacacggtgaaaccccgtctctactaaaaatacaaaaaaaaaattagccgggcatggtggtgggcacctgtagtcccagctactcgggaggctgaggcaggagaatggcgtgaacccgggaggcagagcttgcagtaagccgagatcgcgccactgcactccagcctgggtgacaaagtgagattccaactcaaaaaaaaaaaaaaaaaattccctacataccatgaaaccagatattttgctcaagtatttcccacaattattaagttttcattcctgtaggcattcttccgagcatgaattttctgatgtctgctgaggtttggcttctggtagaaagctttcccacattcattgcacccatagggcttctctcctgtgtgagttctccaatgtttattgaggcatgacttctggctgaaggattttccacattctctgcaacgatacggtctttctcctgtgtgcatttttcgatgtacattgaggtatgacttctcaccaaacgatttcccgcattcactgcagacaaagggtctctctcctgtgtgtgttctctgatgttctgtgcggtgtgacttctgggtaaaggctttcccacaaaaaaaacattcaaagggtcttaccccagtgtgaattctctggtgtttgatgagggttgacttatgtgaaaaggctttcccacagtcagtgcagccataaggcttctccccagtgtgacttctctgatgcctaatgaattcagacttgtagcagaaggctttcccacactcactacagacgtggggtttttctgtaggtggaaccctcttccgtttgtacaagagagaatcacttactgctggtttatacataagtgccgggttctgggtgaaagctttctcacagtgactgcaaccccggggcttttctccattaggtcgtctaccatgatttatacgctgaagcaatttcccataagcataacactcatcttgcttttttgcacagtttctcttaaaaccaatcaagtctaaattatggttcaaattctttccacaagggttccagttactagggctctggattgaagaaaaaagatcagtgctcagaagtgatattttcccaaacttattatattcacagcttttctccttgggcaatgttttcttgcttatggctgcgcctggcctcaaaagcatgtcttgccgtcttttcctctggatattaactcgccagatgtcttcccaacagtggcagcccgggcatgctgcctcaccaatccatggtgcttcttcctgctccagtctgaggatcacatctggtttggtgccttcataacccactgagacgaggttgctataggtttccagcatcacatcccggtacagggccctctgagcaggactcagccggtgccactcctcttgggtgaagcccacaaccacatctttgaatgacacaggtatctggtattcgatcattttctgctgttcttgaaaaagatctgacacctatactcttcaaaaatgtcgacttcatggaagatgaacactgagaaactgctcctgattaaaggagactaaagggatgtgtcacctaaaggcagcatatgatcctggattagatcacttagctgcagggccttctgtagatgttgtgaccaaggtcctgtggctctaagggctggcaggagctagagagccctcccgtccagcaaggtggcaggatccaaaggtctgcagggcacccagagaactcagtaaatttgttttctaaccacgggcaaggtcacatccatccccgctgtcacagagtcagaatggatttccagaaaccagcctcactcttgggatgctggcacagatgcgtatgtcattacctttgccagaaagagccgcggtataaggtcgtcccatcctgaat

SEQ ID NO: 15036 - RNA, 5614 nt, Homo sapiens
  source 1..5614: mol_type = other RNA
gctgggattacaggcatgagccactgcacccagccttcaactgcttatttctaaatagcttctgagtgtcctgtgttggtaaagttaatatctcccaactcctagattgtacacataggctcctttgattttcttttaagaattctgttgctttaaaattttacgtcttaaagccacccagaatttatttttgtgctgttaatccaaattttcttcctttaagattaaaaggttctgttccagaattctttttaagtaaactactcttttcccctgtggtttcagatttcacctttttcacatatgaaaaagttcatatatatcgaagtctatttctgaattttctactgtgttctaatgatgtatttacctgttcctttgccaatacaatattaatttcattagaatggcttcatgttatcttctggtatctagcatggcattttaaaaatttttaattattatagatatataattgttgtatatatttattgggtacatgtgatgtttttatacatggtatgatttttttcatatatttttttcaatgattgtcaaaaaatcattgagatttagtgtaattccaaaagaagtacatataaattatgttttcttgtcagtatggagaacagctcttgattttggtaccctgtcttcttagaaaagttaactcaaaaaatagtcttttcatttattggtgtacaaccatatcatcagtaaaaatggatagttttaccttttctgctgtttataccaattcatttctttttattgccttcactggaatctctaagccaatattgaattcctgattttaaaaaatggctttggcataatatatgctttggggtttgggttaaaaaaaattttttttaagaaaaaccgctttaagtggttcccatctattacaatgtaaattaacacattctatgaaatgccttctcagtatctgttgagagttcatatgattcttctcctttaaactgttaatttgattgatgcatttcctattaactgaactggtttggcattcttgggatgactcttactatgtcactctttgggtatatggctgaattctatttgctagtattttaactataatttttgtttctatattcatgagtaagactggtctgaagttttctttttttttttttttttttgacggagtttcgctcttgtcacccaggctggatggcacgatcttggctcaccgcaacctctacctcctgggtacaagcaattctcctgcctcatgcctcaacctcccaagtagctgggactacaggtgtgtgccaccacacccggctaatttttgtatttttagtagagatggggtttcaccatctcgaacttctgacctcatgatccacctgcctcggcctcccaaagtgttgggattacaggcgtgagccaccgcacccagcagaagttttcttttttcaactatctgtatttgattttggtgttaaaatttattctgacttaataaaataaatgagtacagttcatggattgtattacatccatataataaataacactggtattactctttctttaaaagatagaactaagcatgaactcttctgagcctggagcattttcccattatagatctttaatagcttttttgagtttttcaatgttaactatcctaccaagttttctacttcttattgcagttttcataacttaagtttattagaaaagcatccacctcctctttttaaaaaatatgttgattagagttgtatgaggtatctttttatcacttaaaaaatcatattgatatctgtggttatgtctcctttctcattctggatcaggcagtcttacatggagggaaatcttgaaaaatgtagattccacatggccatttattttctaatatggatgacatagcaactcagggaagcagacttctttccaaacattgaaataattaaaaccttgggatttagtgtctaggacacttgcaaggaaatttatatgaaaaaaatgaatattcttgaattaatttgcagagggatagagagaaaagaaattctccttcagtggtctacgcatgaaacatttctgagttatacaacctgtatatagaatagtgtatctagaatagtgtagcaatgctactaatttgctacaagatattttaagcaagactaagaaaatatgaacagtgtactgtacaccagggtgacactacattttgtcaaatagtttacagtgtttcatttacccagtatcaggttcttaaactattccttagcttgcatttttaatataaataactacattttagtaaaatttttggccaaattatccaaatacatttaaaaacactgctttattatttctgcagaggacagtaacaacctctatagccatttacatgtattacaaaaaggtggaaaaatgtagctggtataataaagttcttttaacaatagtgggccatgttgttgttatttttttgtattgttaagacatcaaaagacaatgatgatatttaaagtggaaaagttttctgaatggcattctatatgttgtgtgacatgtgtctgatattcacattttatgttaatttcacatttacaactccaaaatacaaataatgctgattgtatggctcactgtggaatataccagagtatgcctttaagtctcttcacagatattttgtattctgctgttattccatttaatacatttttaaacgtttacatgccagggtgtccatgcttatgtttgagaaagtattttctagaaaagtttgtatcacaattagatcatgatttccattatgatacaacactgtcggttgggcgcgttggctcatgcctgtaatcccaacactttgggaggccaagggcggggggttggggggtatcacgaggtcaggagttcgagaccagcctagccaaagagaccagcctgaccaacatggtgaaaccccatctctactaaaaatacaaaaattagccaggcgtggtggcaggtgcctgtaatcccagctacttgggaggctgaggcaggagaactgcttgaacctgggaggctgaggttacagtgagccgagatagtgccattgcactccagcctgggaaacagagaatacaactcaaaataaataaataaataaaataaaaacacactgttcaaattcattaaaatgataagatttctcctaaggataaattccctacataccggccaggcgcggtggctcacgcctgtaatcccagcactttgggaggacaaggcgggcagatcacaaggtcaggagatcgagaccatcctggctaacacggtgaaaccccgtctctactaaaaatacaaaaaaaaaattagccgggcatggtggtgggcacctgtagtcccagctactcgggaggctgaggcaggagaatggcgtgaacccgggaggcagagcttgcagtaagccgagatcgcgccactgcactccagcctgggtgacaaagtgagattccaactcaaaaaaaaaaaaaaaaaattccctacataccatgaaaccagatattttgctcaagtatttcccacaattattaagttttcattcctgtaggcattcttccgagcatgaattttctgatgtctgctgaggtttggcttctggtagaaagctttcccacattcattgcacccatagggcttctctcctgtgtgagttctccaatgtttattgaggcatgacttctggctgaaggattttccacattctctgcaacgatacggtctttctcctgtgtgcatttttcgatgtacattgaggtatgacttctcaccaaacgatttcccgcattcactgcagacaaagggtctctctcctgtgtgtgttctctgatgttctgtgcggtgtgacttctgggtaaaggctttcccacaaaaaaaacattcaaagggtcttaccccagtgtgaattctctggtgtttgatgagggttgacttatgtgaaaaggctttcccacagtcagtgcagccataaggcttctccccagtgtgacttctctgatgcctaatgaattcagacttgtagcagaaggctttcccacactcactacagacgtggggtttttctgtaggtggaaccctcttccgtttgtacaagagagaatcacttactgctggtttatacataagtgccgggttctgggtgaaagctttctcacagtgactgcaaccccggggcttttctccattaggtcgtctaccatgatttatacgctgaagcaatttcccataagcataacactcatcttgcttttttgcacagtttctcttaaaaccaatcaagtctaaattatggttcaaattctttccacaagggttccagttactagggctctggattgaagaaaaaagatcagtgctcagaagtgatattttcccaaacttattatattcacagcttttctccttgggcaatgttttcttgcttatggctgcgcctggcctcaaaagcatgtcttgccgtcttttcctctggatattaactcgccagatgtcttcccaacagtggcagcccgggcatgctgcctcaccaatccatggtgcttcttcctgctccagtctgaggatcacatctggtttggtgccttcataacccactgagacgaggttgctataggtttccagcatcacatcccggtacagggccctctgagcaggactcagccggtgccactcctcttgggtgaagcccacaaccacatctttgaatgacacaggtatctggtattcgatcattttctgctgttcttgaaaaagatctgacacctatactcttcaaaaatgtcgacttcatggaagatgaacactgagaaactgctcctgattaaaggagactaaagggatgtgtcacctaaaggcagcatatgatcctggattagatcctctcccttcactctgtcttcctggatcttgggccaaccatcctcccttcatttagccatggagagtccctggaaagagtaacgtcttcaggtttggtcttgctcagcttctggctcagggatgaagctatttccttttatgtgggagtctttgctctgacaagaggtatggggtctgagtgattccttcagaagggaattttcatcccaagttcccttctcctggacagtgtctttaacctggcctgcccaggcactcacagctccatctctcaacagtaactcacacttagctgcagggccttctgtagatgttgtgaccaaggtcctgtggctctaagggctggcaggagctagagagccctcccgtccagcaaggtggcaggatccaaaggtctgcagggcacccagagaactcagtaaatttgttttctaaccacgggcaaggtcacatccatccccgctgtcacagagtcagaatggatttccagaaaccagcctcactcttgggatgctggcacagatgcgtatgtcattacctttgccagaaagagccccatgcaccctgaaaatcaagacatttcacagaactcgcatttattgattcccacacactcccaatccatcttcttcagagaccgtgccactgactcccgcaaacctctgtccgccaccactgaggccccgcgaggctc

SEQ ID NO: 15037 - RNA, 5237 nt, Homo sapiens
  source 1..5237: mol_type = other RNA
gctgggattacaggcatgagccactgcacccagccttcaactgcttatttctaaatagcttctgagtgtcctgtgttggtaaagttaatatctcccaactcctagattgtacacataggctcctttgattttcttttaagaattctgttgctttaaaattttacgtcttaaagccacccagaatttatttttgtgctgttaatccaaattttcttcctttaagattaaaaggttctgttccagaattctttttaagtaaactactcttttcccctgtggtttcagatttcacctttttcacatatgaaaaagttcatatatatcgaagtctatttctgaattttctactgtgttctaatgatgtatttacctgttcctttgccaatacaatattaatttcattagaatggcttcatgttatcttctggtatctagcatggcattttaaaaatttttaattattatagatatataattgttgtatatatttattgggtacatgtgatgtttttatacatggtatgatttttttcatatatttttttcaatgattgtcaaaaaatcattgagatttagtgtaattccaaaagaagtacatataaattatgttttcttgtcagtatggagaacagctcttgattttggtaccctgtcttcttagaaaagttaactcaaaaaatagtcttttcatttattggtgtacaaccatatcatcagtaaaaatggatagttttaccttttctgctgtttataccaattcatttctttttattgccttcactggaatctctaagccaatattgaattcctgattttaaaaaatggctttggcataatatatgctttggggtttgggttaaaaaaaattttttttaagaaaaaccgctttaagtggttcccatctattacaatgtaaattaacacattctatgaaatgccttctcagtatctgttgagagttcatatgattcttctcctttaaactgttaatttgattgatgcatttcctattaactgaactggtttggcattcttgggatgactcttactatgtcactctttgggtatatggctgaattctatttgctagtattttaactataatttttgtttctatattcatgagtaagactggtctgaagttttctttttttttttttttttttgacggagtttcgctcttgtcacccaggctggatggcacgatcttggctcaccgcaacctctacctcctgggtacaagcaattctcctgcctcatgcctcaacctcccaagtagctgggactacaggtgtgtgccaccacacccggctaatttttgtatttttagtagagatggggtttcaccatctcgaacttctgacctcatgatccacctgcctcggcctcccaaagtgttgggattacaggcgtgagccaccgcacccagcagaagttttcttttttcaactatctgtatttgattttggtgttaaaatttattctgacttaataaaataaatgagtacagttcatggattgtattacatccatataataaataacactggtattactctttctttaaaagatagaactaagcatgaactcttctgagcctggagcattttcccattatagatctttaatagcttttttgagtttttcaatgttaactatcctaccaagttttctacttcttattgcagttttcataacttaagtttattagaaaagcatccacctcctctttttaaaaaatatgttgattagagttgtatgaggtatctttttatcacttaaaaaatcatattgatatctgtggttatgtctcctttctcattctggatcaggcagtcttacatggagggaaatcttgaaaaatgtagattccacatggccatttattttctaatatggatgacatagcaactcagggaagcagacttctttccaaacattgaaataattaaaaccttgggatttagtgtctaggacacttgcaaggaaatttatatgaaaaaaatgaatattcttgaattaatttgcagagggatagagagaaaagaaattctccttcagtggtctacgcatgaaacatttctgagttatacaacctgtatatagaatagtgtatctagaatagtgtagcaatgctactaatttgctacaagatattttaagcaagactaagaaaatatgaacagtgtactgtacaccagggtgacactacattttgtcaaatagtttacagtgtttcatttacccagtatcaggttcttaaactattccttagcttgcatttttaatataaataactacattttagtaaaatttttggccaaattatccaaatacatttaaaaacactgctttattatttctgcagaggacagtaacaacctctatagccatttacatgtattacaaaaaggtggaaaaatgtagctggtataataaagttcttttaacaatagtgggccatgttgttgttatttttttgtattgttaagacatcaaaagacaatgatgatatttaaagtggaaaagttttctgaatggcattctatatgttgtgtgacatgtgtctgatattcacattttatgttaatttcacatttacaactccaaaatacaaataatgctgattgtatggctcactgtggaatataccagagtatgcctttaagtctcttcacagatattttgtattctgctgttattccatttaatacatttttaaacgtttacatgccagggtgtccatgcttatgtttgagaaagtattttctagaaaagtttgtatcacaattagatcatgatttccattatgatacaacactgtcggttgggcgcgttggctcatgcctgtaatcccaacactttgggaggccaagggcggggggttggggggtatcacgaggtcaggagttcgagaccagcctagccaaagagaccagcctgaccaacatggtgaaaccccatctctactaaaaatacaaaaattagccaggcgtggtggcaggtgcctgtaatcccagctacttgggaggctgaggcaggagaactgcttgaacctgggaggctgaggttacagtgagccgagatagtgccattgcactccagcctgggaaacagagaatacaactcaaaataaataaataaataaaataaaaacacactgttcaaattcattaaaatgataagatttctcctaaggataaattccctacataccggccaggcgcggtggctcacgcctgtaatcccagcactttgggaggacaaggcgggcagatcacaaggtcaggagatcgagaccatcctggctaacacggtgaaaccccgtctctactaaaaatacaaaaaaaaaattagccgggcatggtggtgggcacctgtagtcccagctactcgggaggctgaggcaggagaatggcgtgaacccgggaggcagagcttgcagtaagccgagatcgcgccactgcactccagcctgggtgacaaagtgagattccaactcaaaaaaaaaaaaaaaaaattccctacataccatgaaaccagatattttgctcaagtatttcccacaattattaagttttcattcctgtaggcattcttccgagcatgaattttctgatgtctgctgaggtttggcttctggtagaaagctttcccacattcattgcacccatagggcttctctcctgtgtgagttctccaatgtttattgaggcatgacttctggctgaaggattttccacattctctgcaacgatacggtctttctcctgtgtgcatttttcgatgtacattgaggtatgacttctcaccaaacgatttcccgcattcactgcagacaaagggtctctctcctgtgtgtgttctctgatgttctgtgcggtgtgacttctgggtaaaggctttcccacaaaaaaaacattcaaagggtcttaccccagtgtgaattctctggtgtttgatgagggttgacttatgtgaaaaggctttcccacagtcagtgcagccataaggcttctccccagtgtgacttctctgatgcctaatgaattcagacttgtagcagaaggctttcccacactcactacagacgtggggtttttctgtaggtggaaccctcttccgtttgtacaagagagaatcacttactgctggtttatacataagtgccgggttctgggtgaaagctttctcacagtgactgcaaccccggggcttttctccattaggtcgtctaccatgatttatacgctgaagcaatttcccataagcataacactcatcttgcttttttgcacagtttctcttaaaaccaatcaagtctaaattatggttcaaattctttccacaagggttccagttactagggctctggattgaagaaaaaagatcagtgctcagaagtgatattttcccaaacttattatattcacagcttttctccttgggcaatgttttcttgcttatggctgcgcctggcctcaaaagcatgtcttgccgtcttttcctctggatattaactcgccagatgtcttcccaacagtggcagcccgggcatgctgcctcaccaatccatggtgcttcttcctgctccagtctgaggatcacatctggtttggtgccttcataacccactgagacgaggttgctataggtttccagcatcacatcccggtacagggccctctgagcaggactcagccggtgccactcctcttgggtgaagcccacaaccacatctttgaatgacacaggtatctggtattcgatcattttctgctgttcttgaaaaagatctgacacctatactcttcaaaaatgtcgacttcatggaagatgaacactgagaaactgctcctgattaaaggagactaaagggatgtgtcacctaaaggcagcatatgatcctggattagatctcagtaaatttgttttctaaccacgggcaaggtcacatccatccccgctgtcacagagtcagaatggatttccagaaaccagcctcactcttgggatgctggcacagatgcgtatgtcattacctttgccagaaagagccccatgcaccctgaaaatcaagacatttcacagaactcgcatttattgattcccacacactcccaatccatcttcttcagagaccgtgccactgactcccgcaaacctctgtccgccaccactgaggccccgcgaggctcagacgccgaatctcttaacccttcagttcccttgtcatt

SEQ ID NO: 15038 - RNA, 596 nt, Homo sapiens
  source 1..596: mol_type = other RNA
gctgggattacaggcatgagccactgcacccagcctttttttaattattatttgaagaatttaagattggaattaattgctccttgaatgtttggtagactcatctgtaataccatttgagcctagaatattctggtttttttgagacggagtcttgccctattgcccaggccggagtgcagtgggattacacgcgtgagccaccatgcctggccagaatattctttattgtaaaatttaaagctgtaatttcaatgtcttgaagagttatagatctaattagattttccatttctcctggagtcaatttggtacaaacagtcaataaagactacaagaccagtttaagtagatttttcagtttgagtgtcctggatcatgtacacaatcatgaatgtgaagtctgtctgcatgaagaatcatctgtggttataaattcttaggaggttttttccttcttccctctggaacaacggttgaagcaggcaagtttcctaatcaccttctctcctttagtagggcagcatttttcttttttataaatagttggcctggccaggcatggtggctcacgcctataatcctagcactttggg

SEQ ID NO: 15039 - RNA, 2342 nt, Homo sapiens
  source 1..2342: mol_type = other RNA
gctgggattacaggcatgagccactgcacccagctgaataaactatttttaagaaatatgtacagaaatctttgctccctcaaaaatacacattgtcaatcacatataatcaaagataactgaaaatgaactgaggcattacattctcctgtggataacaggaaacactggacatttcctgaccagagcaaggtgttccttctcacatgagagtcctggatgagaccagtcactgcacagggcagcagagctctcatcaagttggttctgatggcagcatagtagctgtcaggctgaatcaagaacaaggtcactaccagcaggaacaaaggtgcatgtaaacaaatcacacctcctaccaactcaatctgcagactaggggagttgagcatcagagaacattccccacccatgacagtctgcattatctctctggtatgtacattacaatacttaaagaaaaaccaaactgtagatagaacttgaatgtggagcttctggggacatctttggaaacctacacctctgaaaaaaggaaagtcaagagatttggaggatactcttgattgacaagccagagaatcaggaaaatgggctagaatcagggggccacacagcccatgtgaatttggctggctctaaaatgtgactaaggccttcctcatgtctgccttcgaaatcatatgtaagataggccaccagtgaatcccagcgtggcatcacctaactccatctctacattttattgccttcctttattgacacttcaagctgggagggatgcttgaggccaggagttcaagaccaacctggacaagatagtgagaccctgtctctattaaaataaaaattaaaaaatagcatttctctcatatattaatagtgtgagttctttcatgttttcgacagtaactggaacgaatgaaggctttcccacattccttacattggtaaggtttctctccagtgtgaattctttcatgtattctaatatatatggaacaagtgaaggctttcccacaatgcttacattcataaggtttttctccagcgtgagtcctttcatgtctatgaaaggagctgacacaatgaaatgctttcccacattgcttacattcatagggtttctcaccagtgtgagtccttccatgtattcgaatgtacttggcagatctgaaggctttcccacattgcttacacccatcgggtttctctccagtgtgagtcctttcatgatattgaaacgaagtggaacaagtgaaggctttcccacattgcttgcatttgtagggtttctctccagtgtgacttctttcatgcctttgaaatgaactgggagagtaaaaggctttcccacatatcttacatttatgaggcctctctccagtgtgcattctcatgtgtcttcgaaagcttataaggcgagataatgctttcccatatagtttacattcatagggtttttctcctgtgtgagtcctttcatgcctgtgaaaagaactgggacaattgaaggctttcccacattccttacatttgtacggcttctctcctgtgtgtgtcctttcatgtctgcgaaaggaactggaaaaattgaatgatttcccacactccttacattcatatggcttctccccagtgtgagttctttcatggattcgaacagaactgtgccaactgaaggctttaccacattgtttacattcatatcgtttctctccagtgtgagttcgttcatgggtaaggtataaactgagacaatccaaggctttcccacaaaacttacatttataaggtccatctccactgtgcgttaccatatatcttcgaatgcttgcaggagaaatgaaagatttttcacattccttacaatcaaaaggtttctctctagtgtgaggcctttcatgtgttcgaaagcagtggctatggctcaaggctttcctacgttgtttatgtttatatggcttctctaaaaatttctgacacttatgtggttggtgtccagtgtcagttctgatgttcctattaaaggatgaatatcccatgaagatttctccacatgtaccactttcacatgattttactccaggaagagttttcttgttcagcatgtcttccggaacctgggtgaaagtttctccacactgactaccttctgcactctcaaagagtctctctcccataaaatttcatttccctgcttcttggtgtcccggcgtcctctttatgactccggagcaggtcacagcgcaggtgacagcgtcacaggagccgtggcggaggcacctggggcctctcggagcagcaaggactggatgcagaacgcaacggaccccagcaac

SEQ ID NO: 15040 - RNA, 2521 nt, Homo sapiens
  source 1..2521: mol_type = other RNA
gctgggattacaggcatgagccactgcacccagctgaataaactatttttaagaaatatgtacagaaatctttgctccctcaaaaatacacattgtcaatcacatataatcaaagataactgaaaatgaactgaggcattacattctcctgtggataacaggaaacactggacatttcctgaccagagcaaggtgttccttctcacatgagagtcctggatgagaccagtcactgcacagggcagcagagctctcatcaagttggttctgatggcagcatagtagctgtcaggctgaatcaagaacaaggtcactaccagcaggaacaaaggtgcatgtaaacaaatcacacctcctaccaactcaatctgcagactaggggagttgagcatcagagaacattccccacccatgacagtctgcattatctctctggtatgtacattacaatacttaaagaaaaaccaaactgtagatagaacttgaatgtggagcttctggggacatctttggaaacctacacctctgaaaaaaggaaagtcaagagatttggaggatactcttgattgacaagccagagaatcaggaaaatgggctagaatcagggggccacacagcccatgtgaatttggctggctctaaaatgtgactaaggccttcctcatgtctgccttcgaaatcatatgtaagataggccaccagtgaatcccagcgtggcatcacctaactccatctctacattttattgccttcctttattgacacttcaagctgggagggatgcttgaggccaggagttcaagaccaacctggacaagatagtgagaccctgtctctattaaaataaaaattaaaaaatagcatttctctcatatattaatagtgtgagttctttcatgttttcgacagtaactggaacgaatgaaggctttcccacattccttacattggtaaggtttctctccagtgtgaattctttcatgtattctaatatatatggaacaagtgaaggctttcccacaatgcttacattcataaggtttttctccagcgtgagtcctttcatgtctatgaaaggagctgacacaatgaaatgctttcccacattgcttacattcatagggtttctcaccagtgtgagtccttccatgtattcgaatgtacttggcagatctgaaggctttcccacattgcttacacccatcgggtttctctccagtgtgagtcctttcatgatattgaaacgaagtggaacaagtgaaggctttcccacattgcttgcatttgtagggtttctctccagtgtgacttctttcatgcctttgaaatgaactgggagagtaaaaggctttcccacatatcttacatttatgaggcctctctccagtgtgcattctcatgtgtcttcgaaagcttataaggcgagataatgctttcccatatagtttacattcatagggtttttctcctgtgtgagtcctttcatgcctgtgaaaagaactgggacaattgaaggctttcccacattccttacatttgtacggcttctctcctgtgtgtgtcctttcatgtctgcgaaaggaactggaaaaattgaatgatttcccacactccttacattcatatggcttctccccagtgtgagttctttcatggattcgaacagaactgtgccaactgaaggctttaccacattgtttacattcatatcgtttctctccagtgtgagttcgttcatgggtaaggtataaactgagacaatccaaggctttcccacaaaacttacatttataaggtccatctccactgtgcgttaccatatatcttcgaatgcttgcaggagaaatgaaagatttttcacattccttacaatcaaaaggtttctctctagtgtgaggcctttcatgtgttcgaaagcagtggctatggctcaaggctttcctacgttgtttatgtttatatggcttctctaaaaatttctgacacttatgtggttggtgtccagtgtcagttctgatgttcctattaaaggatgaatatcccatgaagatttctccacatgtaccactttcacatgattttactccaggaagagttttcttgttcagcatgtcttccggaacctgggtgaaagtttctccacactgactaccttctgcactctcaaagagtctctctcccataaaatttctatacagatgaggttcgtgaaggtttcctgcatcacatctctgtagagatcttctggaaaggattcaacaaggcccactcctcctgggtgaagttcacagccacatcctcaaaggccactgggtccatttccctgcttcttggtgtcccggcgtcctctttatgactccggagcaggtcacagcgcaggtgacagcgtcacaggagccgtggcggaggcacctggggcctctcggagcagcaaggactggatgcagaacgcaacggaccccagcaacaaaggagtgcagagactctgagtgcggccttctgcttccccggattgacagtt

SEQ ID NO: 15041 - RNA, 4985 nt, Homo sapiens
  source 1..4985: mol_type = other RNA
gctgggattacaggcatgagccactgcacccagttctaaagttttttttttttttttttttttttttttaaagagatgggggtcttactatgttggctaagctggtctcaaactccttgcctcaggtaatccttctgcctcagcctcccaaagtgctgagattacaggcatgagccaccatgcccgacttccctttgtgtaaaatgagataatatgtatgtcacagaattgttttaaggatgataaaggactaagtgagataatgtaggtgaagtttagtatgatgcctggctcatagttaagtgctgaattatgatagtaatcaatatctactcctaacctctttcttcacagattttaagcttctgtctttctagggggttaagagtcataaaccaaaattacactttcctctgctaggtttcctccctttcctcttcttgacagtctgatgggaaacaaaggcacacataagagcctagttccaagtagtcaagagcctgagaggaagggatatggagagtaatccttcatatctccaggagtgcctgtgaagaagctgaggaatgggactgggaaagcacacaaaataaggaaaacctttcctggggttgggaaagagaagaaagtgcacagctggctacataccataagaattttgtgtcaaaatgtttaaaagcctccaaagattgaatggaattgtctgggactggggaaaaggggctgggacctgggagagagagggaatagggagaagacggtaccctctaaaggcactagctgccattaaatgctccctgagtgccacagggagcaggagttacgttctctgggcattagccttggggaaaagcctgctatgccagtaatcagggttatcaaaggcagagtctgtagcctctaagctacgtagagtttttaggcgggcataatggacatggggggcctgatgtccaggcccctgaaaagctctcatctcttcatacccttgctcagatgctgggcaggcccccatggctgcataatcacccccaggaccacctccatctcgttgccgattcatatattcatagtcttcatctggagttgtgcctgcagtgggcatgatgggtacagggtggagtgggcaactctgtgtgctgcccagagaggcactgaggtctgaccccacatccatgtactcataacccagctcctcaagggaacttggcctagggggatgaggtggactgtgccttctcctccggttcatgtattcatactcctcatcttcatcttcttcttcagtacccaggacagaactgagacccactgaagaaagggtgccttcccgggaggagggagtacctttgaggtgtgtatctggcatgacataaccgttgacatcctcttcctctaacccgggtggggagagtggggtaacaggagtcagcagactgtggcgctgggaatggtaggcgctatctccgcgtggccgtgggctccggctcctgctccggctcctacacattgacactttctcctggagctcagcctcagagcctgttacatgcccctctgatgactctgatgccaggcatccccgtggcattgggtgtagagagactggacgggggcaccgttcactgctcccagaaactgcagactcctggcaagactccccaagattaccctggttcatgggcatgtatccagatgatggacttaaaaggctctggctcccacgtggccgattaagtgttccaactggtaggctgagggcggagcccagtgtggtggttgccaggttgtcctcctctgcttccaagtctaggtctaggtctagttctggctccagctctacttcctctagcttcttgtttgtcagaccatggggctctggcccaggggctattccaggcccactctctctctttatgaccagataccgtggtgggtctcgggccatcctggtgaactcattggctagttctttaaaggttgggcgaatgttctcatcaatcatccaacacttgaccatcaccatgtagacatcaattgtgcagatctggggctgtgccaaccgctcccccttctctagcaggtctggtacttcagccaatcgtagccctgcatagggctctgccccgaaggtcatcaactcccaaactgtcacaccatagctccagacatcactctggtgtgtgtatttcccaaagtggatactctcaagggccatccacttaattggagtcttggcctcactgtatagcagctgcttatcatcaggaggcagcaggtcagccacaccaaaatctgccacctgaacctgactgggtgacttgagtagcacgtttcgggcagccaggtttctatgcaccataccatgttcctcaaggtagtacattcccttggcaatttgtactccccagttgagcagcagctgtggccccagtgccccccggtgttgtctcacatgatccagcagagaacccagaggcaaatattgagtgacaagctgcagagatgaccctgggcatagtcccagcagccttacaatgtgggcatggtccaggctgccaatggccagcatatgatctgtcacagcttgaaaactctgccgtccactcttgtcctcaatgactttaatgcagactggaatcttgattgattcaccctcagggatccacactcctttgtgcacagttccaaagacacccgagccaagcactttaagcttccttagctctgtctctttgaagattctggccaagactttgttagccttctcactggggtccagaggctctatgctctcaccccgttccaagtatcgcctcatagcccttttattctgaatccggcgcccacgccagtagagaaaagtgccgcccagcatcatgaaaatcactaccaatcctgctatcactgtcaaagccattgtcagatgggttttgccgatcagcaccagtgtttgtcctaaacagtcttgaagctctggtcctttacacccctgggtgcagttctcatggcagggccgacattcattctgaacatctgggtacttgtagattgggcccttggcacctaggactccatgggggcagctgctcacacagtggggcccatctcgaaaatgggcacattgagcacaagtatcagagcccgagccattgcatgtggcagtgccctccatgggttggcattccgggtggcaggagaagcattcggcctcatgggcaaattctcgaggctccccattcagaaagttgcagtgggtcacacagacacctcctcggctataatttcgacaggacaagcactgaccagggcctgggccccagcatcccccagaggagcacagtgggtcacacactttgccctctgccacgcagtctctgcgcggccgattatgcttgatgtctagtcgctcttccgtaggcccccgaagcaccttggtccagttcaaagagtggtggtagcagagctgcctattggcacttatatagatacgcccagcactaatttccttcagggatcggaagcccagagatgtgacattcaagttcttcatgatcaacaatgagaagccccggttgtagaggcttctgcctccaatggttgtcaaattggaaaaaacactgaagttgtgcatgtggggcggccaggactggatgttcaggtaacctgtgatctcccgtactgtccggaagacattgagcttctctgggtccagggcagggatcttgtgccaggggtctccattgaggccggtgatcagaaagtccaggttgcccaggatcttggtgcagttcacaaatccatcaatgttgctcgagtccacagtctggaagcggctcccagagcctgttccctcacaggctttgggacatagtcccccacaaggctcacacatcttgagcccatttttatctacttccatcttgtcaggaggacaggccctgacacaggatgtttgatccaccacaaagttatggggacagctggctacacaaactcctccatactgatacttggtgtggggattgggttccagctggaaagttagcttgttgtagacaagaggctgtggacagcgaggtacacaggctccactgtcattgaagtgccggcaggcaaagcagtctgtgtcctgagggcctgagcagcccccggcacactcatcatggcagcactggttggggttgggcccaaagcagtgaccattacactgaggagcacagatggtcttggtcaatgtctggcagtcttctgatccaggaccccagcatcgccccttgcaaacctcatgacaggggggacagcttctgccattgtccttcaccactatctcagcatctcggtccctcacgatgtccctccagtcaattgtgtccatgtgacaaagcttatcgttcttctcaatataaacaccccctgacagaatctcggtgagctgagtcaagcggagctggcgcagagcgtggctggagttggtgttatagttcaacatgacgaagatggcaaacttcccatcgtagacctgggtccctcgcaccacgcggaggttgggcaatggtagagtagagaattcattcatggccacgaggacatagcctgtcacttctcgaatccactgcaggaaggagaggtcggcattgtgtcccgtgagcacaatctcaaggttccccatcaccacctcacacctctcgtagagcttgtacagtgtctggtattggttctcagcatcgccggtcacactcaggccattcagagtcccaggacacactgcctgagagttgcccacctcggagccccgggccaggctgaaaagcaagcccagcacctgcagagcgtcgttcgccctcatgactccgcagagggtgaagggagcccagccaagtccggcccgggggcccctaggctaggacatcgaggcaagagccacctgaaccgctggcgaattggtggctgctgcggcgacggcagcggaggttgcaaattgc

SEQ ID NO: 15042 - RNA, 1548 nt, Homo sapiens
  source 1..1548: mol_type = other RNA
gctgggattacaggcatgagccactgcacccgaccggatattttctattctatttcattttgttaaaattcccaatcagaacccactaaattaattctgtgggccatcagtaggtcacaactggcaattcgaaaaattgaaactttccaaactccgttgccctgtgggggcccctgtgcatggcagatgctctgctttgtgcgaggggaaaagaccatatggctacagggcaggtggatgaggggagtgggcggcaggcacaggcaatgaatgcaggaaggactgggagggcacccaccccccaactggggatccaagaggccaaggtggcctgaatggactgaccccttcctgggtctcagctcctgtcccagtcccagtccagcccgcactcacagcattgtctggatggaagacataggaggcaggtgaattgtccaggatgagcacccgccgcaggtctcgacccaaccggctcaggtccttcacgtagttcccccggtggaagacgcaggactctcgaaacagccgggcccggaaggccccccatttgtccagcaggtcagctactgggtctgcgtacttggcgaggctagcagtgaacagcacacattcaaagagctcgcccattcgctgcaggaactcatccacgtgaggacgcttcaacacgtagacctggtggaccaccccatcaatctccacagggatgatgaagtccgcgttgttcactggcttgaaggagctgtgcaccagggtctcgtccaggtcgatgaccacgcagatcttgtctgagtcctgggccttggcctcagggagcaggtattggactggggtctgcttagggatggcgccattctcctccacaagcaggggcgccccgctgtgagcaggcagggcctccccatcatcccggcagacacagcagaagagtgagtggaggatgccccggcttcggggcttctgggaagctgctgacttctggtcacctttccaccttgccctcagttccggggcagccagacccaggcgagggtgggcagacctgggggcagcgtccagatcctgaggtccacacggggaaaaggagaagacagacccccccaccccggcccagccacgctgggggacgcagcctcgtcggggcggcgaggctttgcggggtggtgcgtgcccactaggcgcacgactctccccgcgggcgccaagcgactcttggaagtgccggccgtcctctctgtgcctccgagggggtcggcgcctccacgcgtgacgcgaagtttgtggggaacgtagctgtgtgttggcgggagatccctccaagcctccccagcctgctgtcacctcggcgccccctcccaagaccctaccggaccgcagcccgggggggtgggggtggggggtggggcggagtctcagcgggtggcccataggcgccctcctcagctcccccatctcccagccccattggcgccaatggtgggggggcgcccatgcaccacgcaatgcctgccaggaaacccccgaagagttccctctctattcctgcct

SEQ ID NO: 15043 - RNA, 1973 nt, Homo sapiens
  source 1..1973: mol_type = other RNA
gctgggattacaggcatgagccactgcacccgaccggatattttctattctatttcattttgttaaaattcccaatcagaacccactaaattaattctgtgggccatcagtaggtcacaactggcaattcgaaaaattgaaactttccaaactccgttgccctgtgggggcccctgtgcatggcagatgctctgctttgtgcgaggggaaaagaccatatggctacagggcaggtggatgaggggagtgggcggcaggcacaggcaatgaatgcaggaaggactgggagggcacccaccccccaactggggatccaagaggccaaggtggcctgaatggactgaccccttcctgggtctcagctcctgtcccagtcccagtccagcccgcactcacagcattgtctggatggaagacataggaggcaggtgaattgtccaggatgagcacccgccgcaggtctcgacccaaccggctcaggtccttcacgtagttcccccggtggaagacgcaggactctcgaaacagccgggcccggaaggccccccatttgtccagcaggtcagctactgggtctgcgtacttggcgaggctagcagtgaacagcacacattcaaagagctcgcccattcgctgcaggaactcatccacgtgaggacgcttcaacacgtagacctggtggaccaccccatcaatctccacagggatgatgaagtccgcgttgttcactggcttgaaggagctgtgcaccagggtctcgtccaggtcgatgaccacgcagatcttgtctgagtcctgggccttggcctcagggagcaggtattggactggggtctgcttagggatggcgccattctcctccacaagcaggggcgccccgctgtgagcaggcagggcctccccatcatcccggcagacacagcagaagagtgagtggaggatgccccggcttcggggcttctgggaagctgctgacttctggtcacctttgccccgcagcgggccccgagcctcctccttgctgatctgagtaatgacggccgagctgtccatggggccgggcgcgctccgctccggccggactctggcccgggcgcccggcctcccccccggctggggccggaatcggggcgcgggggggaggggaggggtgggagggagggatccccgcgagctccggaggggaggggagccaggttctaggggggagggggagggagggggcgcggaggaaactttgttacaacatggagtttccttcccgcgaggcggatgcaaacatggaacccaggcgccgtttcaaggctcccccttaaaagggcaacggcttcggcgtgacctggactcggctgcggctttcgccacttctgggaccggcgcggctaggcggactgggaggcgggccgggccgggttcctgccgcgctccagggggcgtcgcctcccttcctgccgcccgccggcggggctgagtctctgcggctgcgtggcaggcccggcacccggctcaccgttccaggccgccgagcgccctcggccaaggcccgcccgccgggagcgcccacgccggggagtgcccgagtgcggcgcggctccacctctgcgttttctgaagacccgggactagaggcttctcggtttcctcgttgaggacttggagatagcactacctcatctgtaaaatgggtcttctctcctgtctggtggtcgcagagatcacctcgcaaggacgtcaagagccagcgaaggctctgctggcccgaaacagctgtgcaaacctcagaatcacgctcttgaatgggacggtcgccgccccccgcagccccagggcgaggtgcccccggtctgtaggacgtgaaattctaactctctgccctgggaaagccccctgccgacctctccccacggccccacccggggccccgcacgtctacccgccgcgcacgggccaccgcgcgttcccgcctgaagttt

SEQ ID NO: 15044 - RNA, 1543 nt, Homo sapiens
  source 1..1543: mol_type = other RNA
gctgggattacaggcatgagccactgcacccgaccggatattttctattctatttcattttgttaaaattcccaatcagaacccactaaattaattctgtgggccatcagtaggtcacaactggcaattcgaaaaattgaaactttccaaactccgttgccctgtgggggcccctgtgcatggcagatgctctgctttgtgcgaggggaaaagaccatatggctacagggcaggtggatgaggggagtgggcggcaggcacaggcaatgaatgcaggaaggactgggagggcacccaccccccaactggggatccaagaggccaaggtggcctgaatggactgaccccttcctgggtctcagctcctgtcccagtcccagtccagcccgcactcacagcattgtctggatggaagacataggaggcaggtgaattgtccaggatgagcacccgccgcaggtctcgacccaaccggctcaggtccttcacgtagttcccccggtggaagacgcaggactctcgaaacagccgggcccggaaggccccccatttgtccagcaggtcagctactgggtctgcgtacttggcgaggctagcagtgaacagcacacattcaaagagctcgcccattcgctgcaggaactcatccacgtgaggacgcttcaacacgtagacctggtggaccaccccatcaatctccacagggatgatgaagtccgcgttgttcactggcttgaaggagctgtgcaccagggtctcgtccaggtcgatgaccacgcagatcttgtctgagtcctgggccttggcctcagggagcaggtattggactggggtcttagggatggcgccattctcctccacaagcaggggcgccccgctgtgagcaggcagggcctccccatcatcccggcagacacagcagaagagtgagtggaggatgccccggcttcggggcttctgggaagctgctgacttctggtcacctttccaccttgccctcagttccggggcagccagacccaggcgagggtgggcagacctgggggcagcgtccagatcctgaggtccacacggggaaaaggagaagacagacccccccaccccggcccagccacgctgggggacgcagcctcgtcggggcggcgaggctttgcggggtggtgcgtgcccactaggcgcacgactctccccgcgggcgccaagcgactcttggaagtgccggccgtcctctctgtgcctccgagggggtcggcgcctccacgcgtgacgcgaagtttgtggggaacgtagctgtgtgttggcgggagatccctccaagcctccccagcctgctgtcacctcggcgccccctcccaagaccctaccggaccgcagcccgggggggtgggggtggggggtggggcggagtctcagcgggtggcccataggcgccctcctcagctcccccatctcccagccccattggcgccaatggtgggggggcgcccatgcaccacgcaatgcctgccaggaaacccccgaagagttccctctctattcctgc

SEQ ID NO: 15045 - RNA, 1965 nt, Homo sapiens
  source 1..1965: mol_type = other RNA
gctgggattacaggcatgagccactgcacccgaccggatattttctattctatttcattttgttaaaattcccaatcagaacccactaaattaattctgtgggccatcagtaggtcacaactggcaattcgaaaaattgaaactttccaaactccgttgccctgtgggggcccctgtgcatggcagatgctctgctttgtgcgaggggaaaagaccatatggctacagggcaggtggatgaggggagtgggcggcaggcacaggcaatgaatgcaggaaggactgggagggcacccaccccccaactggggatccaagaggccaaggtggcctgaatggactgaccccttcctgggtctcagctcctgtcccagtcccagtccagcccgcactcacagcattgtctggatggaagacataggaggcaggtgaattgtccaggatgagcacccgccgcaggtctcgacccaaccggctcaggtccttcacgtagttcccccggtggaagacgcaggactctcgaaacagccgggcccggaaggccccccatttgtccagcaggtcagctactgggtctgcgtacttggcgaggctagcagtgaacagcacacattcaaagagctcgcccattcgctgcaggaactcatccacgtgaggacgcttcaacacgtagacctggtggaccaccccatcaatctccacagggatgatgaagtccgcgttgttcactggcttgaaggagctgtgcaccagggtctcgtccaggtcgatgaccacgcagatcttgtctgagtcctgggccttggcctcagggagcaggtattggactggggtcttagggatggcgccattctcctccacaagcaggggcgccccgctgtgagcaggcagggcctccccatcatcccggcagacacagcagaagagtgagtggaggatgccccggcttcggggcttctgggaagctgctgacttctggtcacctttgccccgcagcgggccccgagcctcctccttgctgatctgagtaatgacggccgagctgtccatggggccgggcgcgctccgctccggccggactctggcccgggcgcccggcctcccccccggctggggccggaatcggggcgcgggggggaggggaggggtgggagggagggatccccgcgagctccggaggggaggggagccaggttctaggggggagggggagggagggggcgcggaggaaactttgttacaacatggagtttccttcccgcgaggcggatgcaaacatggaacccaggcgccgtttcaaggctcccccttaaaagggcaacggcttcggcgtgacctggactcggctgcggctttcgccacttctgggaccggcgcggctaggcggactgggaggcgggccgggccgggttcctgccgcgctccagggggcgtcgcctcccttcctgccgcccgccggcggggctgagtctctgcggctgcgtggcaggcccggcacccggctcaccgttccaggccgccgagcgccctcggccaaggcccgcccgccgggagcgcccacgccggggagtgcccgagtgcggcgcggctccacctctgcgttttctgaagacccgggactagaggcttctcggtttcctcgttgaggacttggagatagcactacctcatctgtaaaatgggtcttctctcctgtctggtggtcgcagagatcacctcgcaaggacgtcaagagccagcgaaggctctgctggcccgaaacagctgtgcaaacctcagaatcacgctcttgaatgggacggtcgccgccccccgcagccccagggcgaggtgcccccggtctgtaggacgtgaaattctaactctctgccctgggaaagccccctgccgacctctccccacggccccacccggggccccgcacgtctacccgccgcgcacgggccaccgcgcgttcccgcctga

SEQ ID NO: 15046 - RNA, 4891 nt, Homo sapiens
  source 1..4891: mol_type = other RNA
gctgggattacaggcatgagccactgcacccggccaagaagagtacactttataacagcaataacaacaataacagcttgtggcaattacaaagtgaaaagtactgtgccaagaactttgcacaaattatctcatctaatcctcacaacaaccctcctaggcaggcattccctttctgcagtcaagaaagcacgttcagaaaggtcaagatgcacagctactatgctgagtcacacatccatatggtgaagcagggcagggattcaaaggcccaaattttctcatgccaaagcctaagctccttctctcttacctttccttcatccccttttacatgagtaatagcctccaagggggtcacctagagttctactcaggattcaagtaaagatgtgtgtctgagggatgagctacatttcccaagatctgcttatctgctgcttggtttgggcaaacagccatctgcaccatttctttcctcttggctgtgacaggtgaactgttctagcacagaccaggtcactgccttgtgccttgaagctcaaatgataaaacctatgcccttcagcccagctgctggtcctttggcaaaccaacccctgtgcctgtgcccctcagtgaaatatcttctgtcccaaagggctgctggcacactggcttcatctgccttggtttttctcagattccacgcagctttctatcggagcattaatgcatttattggtttacacatccttctcttttttccagattgtgagccccataaggtcagggactgtgtctttatttatctctgtattcacagggcctagtgcagggatggtacagaatagacatctagcaaatacctaatcatcccccccaagtccgtttcttcctaggagaaaatggaggtaacaatatccatcttgggggacaccaggaaggttaactgagataatgtctaaaccagacttagcagagcactcagcacatactaagtactcaataaatgacatcacctatgattactattattatgttatacaatattagatactccaggccaggtgtggtggctcacacttagaatcccagtgctttggaaggacaaggcaggaggattacttgaagccaggagttcgagaccagcctgggcaacacagtgagatcccatctctacaaaaaaatttctttaaaaattagccagacatggtggcatacctgtagtcctagctacttgggaggctgaggtgggaggattgcttcagcccaggaatttgaggttgcagtgagctatgactgcgccactgcattccagcctggacaacagactgagagtctgcctctaaaaaatttaatttagttaaaattaattaaaaaaaatttttttttgagacagagtttcgctcttgttgcccaggctggagtgcaatagcatggtcttggctcactgcaacctccgccacctgggttccaacgattcttctgcctcagcctcccgagtagctgggattacaggtgcccgccacaacatccagctaatttttgtatttttagtagagatggggtttcaccatgttggccaggatggtctcgaactcctgacctcgtgatctgcccacttcagcctcccaaagtgctgggattacaggtgtgagccaccacgcctggcctaatttaaaattttttaattaaaaaaattaatttacatttaaatcctgacttttgctatggtaggaatgaactttactattccttgtctcatgaactgggagtgactaaatgtgtccctagttgcagtattattttttgttttcttatttctattttagattaaatcagacaacatgtgcatgctttacctataaagtttctctcaattcttggacaaagattcactcaaatgagctggaaggtgagaggttaagaaggcagaagcctgggagtcacacagaaacacattacagatgtcatgtccctgggctgagtttagaaaagacaagatgtttgccaggcagaaagagggcatattggaaataggctggcaatcccagtggttagaggagcaggaggcaaaggttcagaggcagcataatagaagcgcctatcaaattatcaaattaatagttccacaaagcttgttacaaaaaattgcactcctctaggcccattttccttttccctcacaacacttttctctttttcctctgtccaatacttacagcatttaatgtgttgatacatctgtcttccctctaccagatggtgactcccttgagaacagggactgtgtcttatctactgttaattacccagtgtctacagcagagaacttcggaaacctttctaaacctgggcttgctgctgcgtaaaatgcagtggataatccctacttcatacggctggtatgaaagttttacctttgtatgaggtcatatttgtaacatacttaccagcatgcacgtaataaaatactgaaagagtaaatctatgaataaatgtagtgacccaagcaccaactctctactcctgcttttcactcagcctaggaaaaactacaacggaatccttcccctatggagaaatcatgattcctatttctgtctttggccacaattttcttattttcttgttccactccacctcgtagcagaaatatcacggattctgtaggcgcttcctggttctaggttgtggagctcctcagggcttggaagtgagtggaaagaaatgttcaacttctgtttctcttctctttccctctcctcctttcccctcatgttcacacttctacctttcccatggtttttgttcgaacaacccttaaactcaatttctctttggagacttcccttagttttcttgtcaggtgattcctcattgacggctgaaggtgggatgaacatgtggtttgccttttttgtatctgctgcttttggatcaatattcttcatttccctggagaagttgtcttgcagctcctttagatgcttgtcaaaataattccattcagtccaatgatgctggtacaactgattgaggttgtctttccgcttcttcatgctgcacagggtctcgctgatgacatcagtatacgttggggtgcagtcaggggtgctcgtggtcttttcccttctgactatcaacacattcttgccgtgctgctgcagactggcatagttctggagaaagtacacaatcagagggctcttcccataaatgttgaagaggtttgaagtcagctcagggcttttgcaggcagcacacgactttttaggaaacatattctcacattctcttgcttctgatatcctcttgacttcttgcgtaggtttcttcaagaccagggtctgacaatgatgctcttttgcagtattctgcattcgtaagcttttttctgagttctgcttggccgaagaggttttttcactgggtgaatttgcactagaagactgagggtggtagaatttcctgctctgggctggcttctgggagaaggctctcttaccagcaaacaaagaaaactctctccctgctatcttaccctttgtcagtcttcttctgtacaacattaattcttctctgcggaatcgctctgggtctagttccgagtagtcccagctgtcatagctctgtgggctaggataggtgcctgaaatccacaggctcattgtgttacagatgtcagacttgaattcgtgcgtgtcgaaccaggactgtggaaagcagcaacagaagctggtgtacacggctttgctgagaagtgatggcagcctttttaagagcgcctcttcagagtgggacttgggtacacgaaacaaaagtaaggcatagtgctgggctatccggtcaaacagattattctggagctccttgtttggctggtacctctcatgaaatatccaccaaaagctatccagccagatggctcttggagaagaagaagagagaaacttctctaattctctacctgaacagaaatgcttgccactaaggcagtctctctcagcccggaccacgttgcccaccatgtcacagaagtccacgccattcggaagcttgtttggcttggagctgttgaagttggaatactggtacagctctgccagcagatttttatctgctgttttcctttttataacagaagatctggcatgtctgagttcggagcctttgcaggaatactgagatttcctttgtctcttgacccatgaaaagagcatcaaggctgagggaaaggtttttgcctttgtcttctggactgctgcgagttttctctcttaaagccttcttctccaactcaaatctctcaattgccaggctgttggccgacggctcggtacgcagatttatgtcagcaatcttttggttcacctggtgcatggagccaataaggcatgagggtggattgttctctaactccttcctcacagtcttcaccattgtattccgtgcgacaagcgagacagccaggtgctcatccactggtatcataggtagggtggtgaggttgatgacctccatcttcctgaagtgattcattgtccaatttcttgtaaatggacaaacaaaaagcttccacttttaagagcctctcatttcccactccaatcttgtcgtttgtttaatcagcctcctgaaagcatcggcggaatttgacgaacccggggccggtcccgccacgggtccctcaggggaccccgcaaagttctgggtcggcccccgacagccggtgcccccaaactcacagcaaggggtgccctttgccttgtgctgggggatgaggaggggagttggggagaggcccattttgctactctgagtccaggcgttctctaggcaacgccggcgcggtctccactttcccgtttagcataacaatggaaccttcgtgagccgccgcgttgtc

SEQ ID NO: 15047 - RNA, 4805 nt, Homo sapiens
  source 1..4805: mol_type = other RNA
gctgggattacaggcatgagccactgcacccggccaagaagagtacactttataacagcaataacaacaataacagcttgtggcaattacaaagtgaaaagtactgtgccaagaactttgcacaaattatctcatctaatcctcacaacaaccctcctaggcaggcattccctttctgcagtcaagaaagcacgttcagaaaggtcaagatgcacagctactatgctgagtcacacatccatatggtgaagcagggcagggattcaaaggcccaaattttctcatgccaaagcctaagctccttctctcttacctttccttcatccccttttacatgagtaatagcctccaagggggtcacctagagttctactcaggattcaagtaaagatgtgtgtctgagggatgagctacatttcccaagatctgcttatctgctgcttggtttgggcaaacagccatctgcaccatttctttcctcttggctgtgacaggtgaactgttctagcacagaccaggtcactgccttgtgccttgaagctcaaatgataaaacctatgcccttcagcccagctgctggtcctttggcaaaccaacccctgtgcctgtgcccctcagtgaaatatcttctgtcccaaagggctgctggcacactggcttcatctgccttggtttttctcagattccacgcagctttctatcggagcattaatgcatttattggtttacacatccttctcttttttccagattgtgagccccataaggtcagggactgtgtctttatttatctctgtattcacagggcctagtgcagggatggtacagaatagacatctagcaaatacctaatcatcccccccaagtccgtttcttcctaggagaaaatggaggtaacaatatccatcttgggggacaccaggaaggttaactgagataatgtctaaaccagacttagcagagcactcagcacatactaagtactcaataaatgacatcacctatgattactattattatgttatacaatattagatactccaggccaggtgtggtggctcacacttagaatcccagtgctttggaaggacaaggcaggaggattacttgaagccaggagttcgagaccagcctgggcaacacagtgagatcccatctctacaaaaaaatttctttaaaaattagccagacatggtggcatacctgtagtcctagctacttgggaggctgaggtgggaggattgcttcagcccaggaatttgaggttgcagtgagctatgactgcgccactgcattccagcctggacaacagactgagagtctgcctctaaaaaatttaatttagttaaaattaattaaaaaaaatttttttttgagacagagtttcgctcttgttgcccaggctggagtgcaatagcatggtcttggctcactgcaacctccgccacctgggttccaacgattcttctgcctcagcctcccgagtagctgggattacaggtgcccgccacaacatccagctaatttttgtatttttagtagagatggggtttcaccatgttggccaggatggtctcgaactcctgacctcgtgatctgcccacttcagcctcccaaagtgctgggattacaggtgtgagccaccacgcctggcctaatttaaaattttttaattaaaaaaattaatttacatttaaatcctgacttttgctatggtaggaatgaactttactattccttgtctcatgaactgggagtgactaaatgtgtccctagttgcagtattattttttgttttcttatttctattttagattaaatcagacaacatgtgcatgctttacctataaagtttctctcaattcttggacaaagattcactcaaatgagctggaaggtgagaggttaagaaggcagaagcctgggagtcacacagaaacacattacagatgtcatgtccctgggctgagtttagaaaagacaagatgtttgccaggcagaaagagggcatattggaaataggctggcaatcccagtggttagaggagcaggaggcaaaggttcagaggcagcataatagaagcgcctatcaaattatcaaattaatagttccacaaagcttgttacaaaaaattgcactcctctaggcccattttccttttccctcacaacacttttctctttttcctctgtccaatacttacagcatttaatgtgttgatacatctgtcttccctctaccagatggtgactcccttgagaacagggactgtgtcttatctactgttaattacccagtgtctacagcagagaacttcggaaacctttctaaacctgggcttgctgctgcgtaaaatgcagtggataatccctacttcatacggctggtatgaaagttttacctttgtatgaggtcatatttgtaacatacttaccagcatgcacgtaataaaatactgaaagagtaaatctatgaataaatgtagtgacccaagcaccaactctctactcctgcttttcactcagcctaggaaaaactacaacggaatccttcccctatggagaaatcatgattcctatttctgtctttggccacaattttcttattttcttgttccactccacctcgtagcagaaatatcacggattctgtaggcgcttcctggttctaggttgtggagctcctcagggcttggaagtgagtggaaagaaatgttcaacttctgtttctcttctctttccctctcctcctttcccctccttagttttcttgtcaggtgattcctcattgacggctgaaggtgggatgaacatgtggtttgccttttttgtatctgctgcttttggatcaatattcttcatttccctggagaagttgtcttgcagctcctttagatgcttgtcaaaataattccattcagtccaatgatgctggtacaactgattgaggttgtctttccgcttcttcatgctgcacagggtctcgctgatgacatcagtatacgttggggtgcagtcaggggtgctcgtggtcttttcccttctgactatcaacacattcttgccgtgctgctgcagactggcatagttctggagaaagtacacaatcagagggctcttcccataaatgttgaagaggtttgaagtcagctcagggcttttgcaggcagcacacgactttttaggaaacatattctcacattctcttgcttctgatatcctcttgacttcttgcgtaggtttcttcaagaccagggtctgacaatgatgctcttttgcagtattctgcattcgtaagcttttttctgagttctgcttggccgaagaggttttttcactgggtgaatttgcactagaagactgagggtggtagaatttcctgctctgggctggcttctgggagaaggctctcttaccagcaaacaaagaaaactctctcccctttgtcagtcttcttctgtacaacattaattcttctctgcggaatcgctctgggtctagttccgagtagtcccagctgtcatagctctgtgggctaggataggtgcctgaaatccacaggctcattgtgttacagatgtcagacttgaattcgtgcgtgtcgaaccaggactgtggaaagcagcaacagaagctggtgtacacggctttgctgagaagtgatggcagcctttttaagagcgcctcttcagagtgggacttgggtacacgaaacaaaagtaaggcatagtgctgggctatccggtcaaacagattattctggagctccttgtttggctggtacctctcatgaaatatccaccaaaagctatccagccagatggctcttggagaagaagaagagagaaacttctctaattctctacctgaacagaaatgcttgccactaaggcagtctctctcagcccggaccacgttgcccaccatgtcacagaagtccacgccattcggaagcttgtttggcttggagctgttgaagttggaatactggtacagctctgccagcagatttttatctgctgttttcctttttataacagaagatctggcatgtctgagttcggagcctttgcaggaatactgagatttcctttgtctcttgacccatgaaaagagcatcaaggctgagggaaaggtttttgcctttgtcttctggactgctgcgagttttctctcttaaagccttcttctccaactcaaatctctcaattgccaggctgttggccgacggctcggtacgcagatttatgtcagcaatcttttggttcacctggtgcatggagccaataaggcatgagggtggattgttctctaactccttcctcacagtcttcaccattgtattccgtgcgacaagcgagacagccaggtgctcatccactggtatcataggtagggtggtgaggttgatgacctccatcttcctgaagtgattcattgtccaatttcttgtaaatggacaaacaaaaagcttccacttttaagagcctctcatttcccactccaatcttgtcgtttgtttaatcagcctcctgaaagcatcggcggaatttgacgaacccggggccggtcccgccacgggtccctcaggggaccccgcaaagttctgggtcggcccccgacagccggtgcccccaaactcacagcaaggggtgccctttgccttgtgctgggggatgaggaggggagttggggagaggcccattttgctactctgagtccaggcgttctctaggcaacgccggcgcggtctccactttcccgtttagcataacaatggaaccttcgtgagccgccgcgttgtc

SEQ ID NO: 15048 - RNA, 4765 nt, Homo sapiens
  source 1..4765: mol_type = other RNA
gctgggattacaggcatgagccactgcacccggccaagaagagtacactttataacagcaataacaacaataacagcttgtggcaattacaaagtgaaaagtactgtgccaagaactttgcacaaattatctcatctaatcctcacaacaaccctcctaggcaggcattccctttctgcagtcaagaaagcacgttcagaaaggtcaagatgcacagctactatgctgagtcacacatccatatggtgaagcagggcagggattcaaaggcccaaattttctcatgccaaagcctaagctccttctctcttacctttccttcatccccttttacatgagtaatagcctccaagggggtcacctagagttctactcaggattcaagtaaagatgtgtgtctgagggatgagctacatttcccaagatctgcttatctgctgcttggtttgggcaaacagccatctgcaccatttctttcctcttggctgtgacaggtgaactgttctagcacagaccaggtcactgccttgtgccttgaagctcaaatgataaaacctatgcccttcagcccagctgctggtcctttggcaaaccaacccctgtgcctgtgcccctcagtgaaatatcttctgtcccaaagggctgctggcacactggcttcatctgccttggtttttctcagattccacgcagctttctatcggagcattaatgcatttattggtttacacatccttctcttttttccagattgtgagccccataaggtcagggactgtgtctttatttatctctgtattcacagggcctagtgcagggatggtacagaatagacatctagcaaatacctaatcatcccccccaagtccgtttcttcctaggagaaaatggaggtaacaatatccatcttgggggacaccaggaaggttaactgagataatgtctaaaccagacttagcagagcactcagcacatactaagtactcaataaatgacatcacctatgattactattattatgttatacaatattagatactccaggccaggtgtggtggctcacacttagaatcccagtgctttggaaggacaaggcaggaggattacttgaagccaggagttcgagaccagcctgggcaacacagtgagatcccatctctacaaaaaaatttctttaaaaattagccagacatggtggcatacctgtagtcctagctacttgggaggctgaggtgggaggattgcttcagcccaggaatttgaggttgcagtgagctatgactgcgccactgcattccagcctggacaacagactgagagtctgcctctaaaaaatttaatttagttaaaattaattaaaaaaaatttttttttgagacagagtttcgctcttgttgcccaggctggagtgcaatagcatggtcttggctcactgcaacctccgccacctgggttccaacgattcttctgcctcagcctcccgagtagctgggattacaggtgcccgccacaacatccagctaatttttgtatttttagtagagatggggtttcaccatgttggccaggatggtctcgaactcctgacctcgtgatctgcccacttcagcctcccaaagtgctgggattacaggtgtgagccaccacgcctggcctaatttaaaattttttaattaaaaaaattaatttacatttaaatcctgacttttgctatggtaggaatgaactttactattccttgtctcatgaactgggagtgactaaatgtgtccctagttgcagtattattttttgttttcttatttctattttagattaaatcagacaacatgtgcatgctttacctataaagtttctctcaattcttggacaaagattcactcaaatgagctggaaggtgagaggttaagaaggcagaagcctgggagtcacacagaaacacattacagatgtcatgtccctgggctgagtttagaaaagacaagatgtttgccaggcagaaagagggcatattggaaataggctggcaatcccagtggttagaggagcaggaggcaaaggttcagaggcagcataatagaagcgcctatcaaattatcaaattaatagttccacaaagcttgttacaaaaaattgcactcctctaggcccattttccttttccctcacaacacttttctctttttcctctgtccaatacttacagcatttaatgtgttgatacatctgtcttccctctaccagatggtgactcccttgagaacagggactgtgtcttatctactgttaattacccagtgtctacagcagagaacttcggaaacctttctaaacctgggcttgctgctgcgtaaaatgcagtggataatccctacttcatacggctggtatgaaagttttacctttgtatgaggtcatatttgtaacatacttaccagcatgcacgtaataaaatactgaaagagtaaatctatgaataaatgtagtgacccaagcaccaactctctactcctgcttttcactcagcctaggaaaaactacaacggaatccttcccctatggagaaatcatgattcctatttctgtctttggccacaattttcttattttcttgttccactccacctcgtagcagaaatatcacggattctgtaggcgcttcctggttctaggttgtggagctcctcagggcttggaagtgagtggaaagaaatgttcaacttctgtttctcttctctttccctctcctcctttcccctccttagttttcttgtcaggtgattcctcattgacggctgaaggtgggatgaacatgtggtttgccttttttgtatctgctgcttttggatcaatattcttcatttccctggagaagttgtcttgcagctcctttagatgcttgtcaaaataattccattcagtccaatgatgctggtacaactgattgaggttgtctttccgcttcttcatgctgcacagggtctcgctgatgacatcagtatacgttggggtgcagtcaggggtgctcgtggtcttttcccttctgactatcaacacattcttgccgtgctgctgcagactggcatagttctggagaaagtacacaatcagagggctcttcccataaatgttgaagaggtttgaagtcagctcagggcttttgcaggcagcacacgactttttaggaaacatattctcacattctcttgcttctgatatcctcttgacttcttgcgtaggtttcttcaagaccagggtctgacaatgatgctcttttgcagtattctgcattcgtaagcttttttctgagttctgcttggccgaagaggttttttcactgggtgaatttgcactagaagactgagggtggtagaatttcctgctctgggctggcttctgggagaaggctctcttaccagcaaacaaagaaaactctctcccctttgtcagtcttcttctgtacaacattaattcttctctgcggaatcgctctgggtctagttccgagtagtcccagctgtcatagctctgtgggctaggataggtgcctgaaatccacaggctcattgtgttacagatgtcagacttgaattcgtgcgtgtcgaaccaggactgtggaaagcagcaacagaagctggtgtacacggctttgctgagaagtgatggcagcctttttaagagcgcctcttcagagtgggacttgggtacacgaaacaaaagtaaggcatagtgctgggctatccggtcaaacagattattctggagctccttgtttggctggtacctctcatgaaatatccaccaaaagctatccagccagatggctcttggagaagaagaagagagaaacttctctaattctctacctgaacagaaatgcttgccactaaggcagtctctctcagcccggaccacgttgcccaccatgtcacagaagtccacgccattcggaagcttgtttggcttggagctgttgaagttggaatactggtacagctctgccagcagatttttatctgctgttttcctttttataacagaagatctggcatgtctgagttcggagcctttgcaggaatactgagatttcctttgtctcttgactttgtcttctggactgctgcgagttttctctcttaaagccttcttctccaactcaaatctctcaattgccaggctgttggccgacggctcggtacgcagatttatgtcagcaatcttttggttcacctggtgcatggagccaataaggcatgagggtggattgttctctaactccttcctcacagtcttcaccattgtattccgtgcgacaagcgagacagccaggtgctcatccactggtatcataggtagggtggtgaggttgatgacctccatcttcctgaagtgattcattgtccaatttcttgtaaatggacaaacaaaaagcttccacttttaagagcctctcatttcccactccaatcttgtcgtttgtttaatcagcctcctgaaagcatcggcggaatttgacgaacccggggccggtcccgccacgggtccctcaggggaccccgcaaagttctgggtcggcccccgacagccggtgcccccaaactcacagcaaggggtgccctttgccttgtgctgggggatgaggaggggagttggggagaggcccattttgctactctgagtccaggcgttctctaggcaacgccggcgcggtctccactttcccgtttagcataacaatggaaccttcgtgagccgccgcgttgtc

SEQ ID NO: 15049 - RNA, 4602 nt, Homo sapiens
  source 1..4602: mol_type = other RNA
gctgggattacaggcatgagccactgcacccggccaagaagagtacactttataacagcaataacaacaataacagcttgtggcaattacaaagtgaaaagtactgtgccaagaactttgcacaaattatctcatctaatcctcacaacaaccctcctaggcaggcattccctttctgcagtcaagaaagcacgttcagaaaggtcaagatgcacagctactatgctgagtcacacatccatatggtgaagcagggcagggattcaaaggcccaaattttctcatgccaaagcctaagctccttctctcttacctttccttcatccccttttacatgagtaatagcctccaagggggtcacctagagttctactcaggattcaagtaaagatgtgtgtctgagggatgagctacatttcccaagatctgcttatctgctgcttggtttgggcaaacagccatctgcaccatttctttcctcttggctgtgacaggtgaactgttctagcacagaccaggtcactgccttgtgccttgaagctcaaatgataaaacctatgcccttcagcccagctgctggtcctttggcaaaccaacccctgtgcctgtgcccctcagtgaaatatcttctgtcccaaagggctgctggcacactggcttcatctgccttggtttttctcagattccacgcagctttctatcggagcattaatgcatttattggtttacacatccttctcttttttccagattgtgagccccataaggtcagggactgtgtctttatttatctctgtattcacagggcctagtgcagggatggtacagaatagacatctagcaaatacctaatcatcccccccaagtccgtttcttcctaggagaaaatggaggtaacaatatccatcttgggggacaccaggaaggttaactgagataatgtctaaaccagacttagcagagcactcagcacatactaagtactcaataaatgacatcacctatgattactattattatgttatacaatattagatactccaggccaggtgtggtggctcacacttagaatcccagtgctttggaaggacaaggcaggaggattacttgaagccaggagttcgagaccagcctgggcaacacagtgagatcccatctctacaaaaaaatttctttaaaaattagccagacatggtggcatacctgtagtcctagctacttgggaggctgaggtgggaggattgcttcagcccaggaatttgaggttgcagtgagctatgactgcgccactgcattccagcctggacaacagactgagagtctgcctctaaaaaatttaatttagttaaaattaattaaaaaaaatttttttttgagacagagtttcgctcttgttgcccaggctggagtgcaatagcatggtcttggctcactgcaacctccgccacctgggttccaacgattcttctgcctcagcctcccgagtagctgggattacaggtgcccgccacaacatccagctaatttttgtatttttagtagagatggggtttcaccatgttggccaggatggtctcgaactcctgacctcgtgatctgcccacttcagcctcccaaagtgctgggattacaggtgtgagccaccacgcctggcctaatttaaaattttttaattaaaaaaattaatttacatttaaatcctgacttttgctatggtaggaatgaactttactattccttgtctcatgaactgggagtgactaaatgtgtccctagttgcagtattattttttgttttcttatttctattttagattaaatcagacaacatgtgcatgctttacctataaagtttctctcaattcttggacaaagattcactcaaatgagctggaaggtgagaggttaagaaggcagaagcctgggagtcacacagaaacacattacagatgtcatgtccctgggctgagtttagaaaagacaagatgtttgccaggcagaaagagggcatattggaaataggctggcaatcccagtggttagaggagcaggaggcaaaggttcagaggcagcataatagaagcgcctatcaaattatcaaattaatagttccacaaagcttgttacaaaaaattgcactcctctaggcccattttccttttccctcacaacacttttctctttttcctctgtccaatacttacagcatttaatgtgttgatacatctgtcttccctctaccagatggtgactcccttgagaacagggactgtgtcttatctactgttaattacccagtgtctacagcagagaacttcggaaacctttctaaacctgggcttgctgctgcgtaaaatgcagtggataatccctacttcatacggctggtatgaaagttttacctttgtatgaggtcatatttgtaacatacttaccagcatgcacgtaataaaatactgaaagagtaaatctatgaataaatgtagtgacccaagcaccaactctctactcctgcttttcactcagcctaggaaaaactacaacggaatccttcccctatggagaaatcatgattcctatttctgtctttggccacaattttcttattttcttgttccactccacctcgtagcagaaatatcacggattctgtaggcgcttcctggttctaggttgtggagctcctcagggcttggaagtgagtggaaagaaatgttcaacttctgtttctcttctctttccctctcctcctttcccctccttagttttcttgtcaggtgattcctcattgacggctgaaggtgggatgaacatgtggtttgccttttttgtatctgctgcttttggatcaatattcttcatttccctggagaagttgtcttgcagctcctttagatgcttgtcaaaataattccattcagtccaatgatgctggtacaactgattgaggttgtctttccgcttcttcatgctgcacagggtctcgctgatgacatcagtatacgttggggtgcagtcaggggtgctcgtggtcttttcccttctgactatcaacacattcttgccgtgctgctgcagactggcatagttctggagaaagtacacaatcagagggctcttcccataaatgttgaagaggtttgaagtcagctcagggcttttgcaggcagcacacgactttttaggaaacatattctcacattctcttgcttctgatatcctcttgacttcttgcgtaggtttcttcaagaccagggtctgacaatgatgctcttttgcagtattctgcattcgtaagcttttttctgagttctgcttggccgaagaggttttttcactgggtgaatttgcactagaagactgagggtggtagaatttcctgctctgggctggcttctgggagaaggctctcttaccagcaaacaaagaaaactctctccctgctatcttaccctttgtcagtcttcttctgtacaacattaattcttctctgcggaatcgctctgggtctagttccgagtagtcccagctgtcatagctctgtgggctaggataggtgcctgaaatccacaggctcattgtgttacagatgtcagacttgaattcgtgcgtgtcgaaccaggactgtggaaagcagcaacagaagctggtgtacacggctttgctgagaagtgatggcagcctctggtacctctcatgaaatatccaccaaaagctatccagccagatggctcttggagaagaagaagagagaaacttctctaattctctacctgaacagaaatgcttgccactaaggcagtctctctcagcccggaccacgttgcccaccatgtcacagaagtccacgccattcggaagcttgtttggcttggagctgttgaagttggaatactggtacagctctgccagcagatttttatctgctgttttcctttttataacagaagatctggcatgtctgagttcggagcctttgcaggaatactgagatttcctttgtctcttgacaggctgttggccgacggctcggtacgcagatttatgtcagcaatcttttggttcacctggtgcatggagccaataaggcatgagggtggattgttctctaactccttcctcacagtcttcaccattgtattccgtgcgacaagcgagacagccaggtgctcatccactggtatcataggtagggtggtgaggttgatgacctccatcttcctgaagtgattcattgtccaatttcttgtaaatggacaaacaaaaagcttccacttttaagagcctctcatttcccactccaatcttgtcgtttgtttaatcagcctcctgaaagcatcggcggaatttgacgaacccggggccggtcccgccacgggtccctcaggggaccccgcaaagttctgggtcggcccccgacagccggtgcccccaaactcacagcaaggggtgccctttgccttgtgctgggggatgaggaggggagttggggagaggcccattttgctactctgagtccaggcgttctctaggcaacgccggcgcggtctccactttcccgtttagcataacaatggaaccttcgtgagccgccgcgttgtc

SEQ ID NO: 15050 - RNA, 2346 nt, Homo sapiens
  source 1..2346: mol_type = other RNA
gctgggattacaggcatgagccactgcacccggccaagacatctttgtaaatacctgattgtggagaattagggggaattgaggctaactggtcactggcttcagtaattgagagtatgtggcactactcactgagacagaaaatacaaaacgtggaacagataactatggtgagtgtggaagaactcagtttgaacactgcatatgagatgtttgtgacataaaagtagcagtggttaacaggatttgtaaacccatgagtgcaaacctttactgtgtcacacatcaaatgaataaccaagttaggaagttaaagcttaaagtgccttctaaaaaaatcaataaaaatagtccctaagtgtaggagtagtagtactgagaatgaagtatgaatacaggtgactgagtacactttattcctttatgtttttagtgcatttaaagtattacagcaaatgatttagaagttttctaaagaggattgctgtggtttggaagttaggcatcttgcattcatagtttgactaaaggctaagcatttaaccaaatatgagatgcgttggtggtatagtggtgaggatagctgccttctaaatatgtactataaacacacatactccagagagtcacaaagtcaagtgaaagaaattccaaaaagaaagacatggctgacagtgtcaaacattactgagtagtcaaaggagctaaaaaccaggaaggcagcattagatgttggccacttgttcataagtgattttttttttctactgtaaaccttgaactcctaggctcaggcgatcctctctcctcagactctcttgtgttgctaggactacactacagatacacacaaccacgtttggctatttttaaaattttttttatagagatgaagtctcactatgttgctcaggctggtgtcaaactcctggcctcaagtgatgttcctgtcttggcctcccaaagtgttgggattacaggcatgagccaccatgtcagcccataaatgatcttcggagaggtgtttcagtagaactggaataccatacggggcagaagattttgtaagcagaatatagtagtcctcccatatccgcaggggatacagtccaaaactcccagtggatgcctgaaactgacgttttagagagatcaactccatgtccagttgcctcaggatggtgttggctgcattgggactacaggaaactgctaccacatcttcctgggttaaatacatgcccttaggtggacggcacttagaacgctgagaatgatggcgatgttgtaaactctgatactctcttcttccaagtccaatcttgctagtttggacaggttgttcagtattaccctcttttttggcttcttttttgggatcataatcactatcattcccatccattggatgtgtttcttctacatcatcatcactgtcaccctgattatgtctattagctagtttacgagcctggcgatccatcaaacttgtcctagagcgagtttttttccaagaatagtaatattttacaaggcttgcaattgtcttatctggaagcatttgctgaatcctgtgaaagctctttccatgaaaactaaaggcttgttcaaataggactttatcttccactgtccactcatccggaaagggagtgaaattagggagatcagcaagggacttctcaatgttatgtttatgccagaacaacatgccaagtgcctgttccacattgtagccatgcttttcctttgcaattgcaatgtattcatccaatttggcatctgggatactgtgatatggagaccatacaagcatccctccattgtctttatctgtgtactttgtagcacctataatcccagcactttgggaggccaaggagggcggatggcttgagccccggagtttgagaccagcctgggaaacatagcaagaccttgtctctactggatcaaattcagggatccgagcttggtattcggctccgactctcatcccaacatcaccgtgctcgtcgtcgctgctgcagccgctctcgggctctgagtagtgcagcccgccgttggtggacgaggcgccgctgccgccgccgcctgccgggctcttggcgctgccgttggccgatcggttcttccccagtaactcgggccctttctccatcatgccgggcatggtagaacaggggagggggaaaggtgaggggaagaggcaggcgtcagggtgaaggcggagatggcttagagcgcgggcgggagggaaaggaggaggaggaggagacggcggcggcggcggaggaggaggaggctgttaatatggagccgccataaccgccccgctccggcagt

SEQ ID NO: 15051 - RNA, 2362 nt, Homo sapiens
  source 1..2362: mol_type = other RNA
gctgggattacaggcatgagccactgcacccggccaagacatctttgtaaatacctgattgtggagaattagggggaattgaggctaactggtcactggcttcagtaattgagagtatgtggcactactcactgagacagaaaatacaaaacgtggaacagataactatggtgagtgtggaagaactcagtttgaacactgcatatgagatgtttgtgacataaaagtagcagtggttaacaggatttgtaaacccatgagtgcaaacctttactgtgtcacacatcaaatgaataaccaagttaggaagttaaagcttaaagtgccttctaaaaaaatcaataaaaatagtccctaagtgtaggagtagtagtactgagaatgaagtatgaatacaggtgactgagtacactttattcctttatgtttttagtgcatttaaagtattacagcaaatgatttagaagttttctaaagaggattgctgtggtttggaagttaggcatcttgcattcatagtttgactaaaggctaagcatttaaccaaatatgagatgcgttggtggtatagtggtgaggatagctgccttctaaatatgtactataaacacacatactccagagagtcacaaagtcaagtgaaagaaattccaaaaagaaagacatggctgacagtgtcaaacattactgagtagtcaaaggagctaaaaaccaggaaggcagcattagatgttggccacttgttcataagtgattttttttttctactgtaaaccttgaactcctaggctcaggcgatcctctctcctcagactctcttgtgttgctaggactacactacagatacacacaaccacgtttggctatttttaaaattttttttatagagatgaagtctcactatgttgctcaggctggtgtcaaactcctggcctcaagtgatgttcctgtcttggcctcccaaagtgttgggattacaggcatgagccaccatgtcagcccataaatgatcttcggagaggtgtttcagtagaactggaataccatacggggcagaagattttgtaagcagaatatagtagtcctcccatatccgcaggggatacagtccaaaactcccagtggatgcctgaaactgacgttttagagagatcaactccatgtccagttgcctcaggatggtgttggctgcattgggactacaggaaactgctaccacatcttcctgggttaaatacatgcccttaggtggacggcacttagaacgctgagaatgatggcgatgttgtaaactctgatactctcttcttccaagtccaatcttgctagtttggacaggttgttcagtattaccctcttttttggcttcttttttgggatcataatcactatcattcccatccattggatgtgtttcttctacatcatcatcactgtcaccctgattatgtctattagctagtttacgagcctggcgatccatcaaacttgtcctagagcgagtttttttccaagaatagtaatattttacaaggcttgcaattgtcttatctggaagcatttgctgaatcctgtgaaagctctttccatgaaaactaaaggcttgttcaaataggactttatcttccactgtccactcatccggaaagggagtgaaattagggagatcagcaagggacttctcaatgttatgtttatgccagaacaacatgccaagtgcctgttccacattgtagccatgcttttcctttgcaattgcaatgtattcatccaatttggcatctgggatactgtgatatggagaccatacaagcatccctccattgtctttatctgtgtactttgtagcacctataatcccagcactttgggaggccaaggagggcggatggcttgagccccggagtttgagaccagcctgggaaacatagcaagaccttgtctctactggatcaaattcagggatccgagcttggtattcggctccgactctcatcccaacatcgtgctcgtcgtcgctgctgcagccgctctcgggctctgagtagtgcagcccgccgttggtggacgaggcgccgctgccgccgccgcctgccgggctcttggcgctgccgttggccgatcggttcttccccagtaactcgggccctttctccatcatgccgggcatggtagaacaggggagggggaaaggtgaggggaagaggcaggcgtcagggtgaaggcggagatggcttagagcgcgggcgggagggaaaggaggaggaggaggagacggcggcggcggcggaggaggaggaggctgttaatatggagccgccataaccgccccgctccggcagtagcgcagtcgcctcacaac

SEQ ID NO: 15052 - RNA, 1634 nt, Homo sapiens
  source 1..1634: mol_type = other RNA
gctgggattacaggcatgagccactgcacccggccacaagcttctacttcttgcagaatgcctttgtcccatgaaacctagtccacgagtgctatgacacttcctgaagtcttgggtggggtgaacgcacaaatcctgggggtgtagagaggaggaggatgtttacttaaaatgtcttaaggttcagcattgacagagaggcaatatccaaatcactctaagttttgttttgggtcctctgacaattgagtttccataatctggtcggctcagagacaccatcatgtgtggtatattcacaaatgcagacaaagaaaattctagaaagccaggggtgaaaaagctctcctttctcagacgattctgtgaagtctatgtgggctaaggagagaagaacaaaagtttctctgggccttggcctcttggggatcccttctctcattttctaaaaactgtttctcacaccaggctaaggaggtggtggggaaggtctcccttcccctgcccacctcagacagttctagggagatggaggtttcaccacttggccactagtctcaaataactggaaggttccttttttcctgaggtcatgaaatgttctggaaccacagcgcccccgccagccctccgtgggagcacagaggggcaggccttgattggtcttctcaccctacagccacttttttggcccaactctcgagcaagccttcatcaccatcagggtctcatgggcagtctgggtttgccagcccagtccttgaacttggagagggaggtggggcttggaaatgccttgtccccagggtgggggggacaccttgtccttggagctggctgagccctgtgcccatggctgggttcagtttgcaggtatagctgtagcactctttgctggtgggaatggagaggtctcgctggccttctttgcctttttcttctttttggtcccaagcgacacctggtccccgttgagctcacctgacttctgcttctggactgtggccatgctggtgggggtggtggcagcgacagccgagtcgacactggccaccttcttggctttctttttcaacttccttttcttctttgcctccttctccactgttccagggctgtggatggctgactcctgtaggatgtcggacgccgacacagctgcctcccggcaccgccgccactcctcgtcactgtcctcactgctggagctggagggctgtcgctttcggcggggttggggagactcttccttctcacggccatcatcctccaaagcgactttctgtaccttagcttttgctggctcctttgctgcttctgagatggtaatgaagctgtccagcagggctcccagcttcttggctacgtgggctcggaattcaggggtggtctgaagctcgttgccatcttgttcatgctcattcaccttatgcctgaggctcggttgggaggttgacaactggctatttgcagcaccggctcttggcttccctgccacgtgcgggcgttgctccaagccccaagccggcattgccgcctcgcggcaccgctccagctcctccgcatcgctactgctgttactactttccgaatcgctcactgtgccactgggcgccgccatcttgaaccaccgc

SEQ ID NO: 15053 - RNA, 1568 nt, Homo sapiens
  source 1..1568: mol_type = other RNA
gctgggattacaggcatgagccactgcacccggccacaagcttctacttcttgcagaatgcctttgtcccatgaaacctagtccacgagtgctatgacacttcctgaagtcttgggtggggtgaacgcacaaatcctgggggtgtagagaggaggaggatgtttacttaaaatgtcttaaggttcagcattgacagagaggcaatatccaaatcactctaagttttgttttgggtcctctgacaattgagtttccataatctggtcggctcagagacaccatcatgtgtggtatattcacaaatgcagacaaagaaaattctagaaagccaggggtgaaaaagctctcctttctcagacgattctgtgaagtctatgtgggctaaggagagaagaacaaaagtttctctgggccttggcctcttggggatcccttctctcattttctaaaaactgtttctcacaccaggctaaggaggtggtggggaaggtctcccttcccctgcccacctcagacagttctagggagatggaggtttcaccacttggccactagtctcaaataactggaaggttccttttttcctgaggtcatgaaatgttctggaaccacagcgcccccgccagccctccgtgggagcacagaggggcaggccttgattggtcttctcaccctacagccacttttttggcccaactctcgagcaagccttcatcaccatcagggtctcatgggcagtctgggtttgccagcccagtccttgaacttggagagggaggtggggcttggaaatgccttgtccccagggtgggggggacaccttgtccttggagctggctgagccctgtgcccatggctgggttcagtttgcaggtatagctgtagcactctttgctggtgggaatggagaggtctcgctggccttctttgcctttttcttctttttggtcccaagcgacacctggtccccgttgagctcacctgacttctgcttctggactgtggccatgctggtgggggtggtggcagcgacagccgagtcgacactggccaccttcttggctttctttttcaacttccttttcttctttgcctccttctccactgttccagggctgtggatggctgactcctgtaggatgtcggacgccgacacagctgcctcccggcaccgccgccactcctcgtcactgtcctcactgctggagctggagggctgtcgctttcggcggggttggggagactcttccttctcacggcctccagggacagatgtgaagaaaaggcggaaaccatcatcctccaaagcgactttctgtaccttagcttttgctggctcctttgctgcttctgagatggtaatgaagctgaggctcggttgggaggttgacaactggctatttgcagcaccggctcttggcttccctgccacgtgcgggcgttgctccaagccccaagccggcattgccgcctcgcggcaccgctccagctcctccgcatcgctactgctgttactactttccgaatcgctcactgtgccactgggcgccgccatcttgaaccaccgc

SEQ ID NO: 15054 - RNA, 1667 nt, Homo sapiens
  source 1..1667: mol_type = other RNA
gctgggattacaggcatgagccactgcacccggccacaagcttctacttcttgcagaatgcctttgtcccatgaaacctagtccacgagtgctatgacacttcctgaagtcttgggtggggtgaacgcacaaatcctgggggtgtagagaggaggaggatgtttacttaaaatgtcttaaggttcagcattgacagagaggcaatatccaaatcactctaagttttgttttgggtcctctgacaattgagtttccataatctggtcggctcagagacaccatcatgtgtggtatattcacaaatgcagacaaagaaaattctagaaagccaggggtgaaaaagctctcctttctcagacgattctgtgaagtctatgtgggctaaggagagaagaacaaaagtttctctgggccttggcctcttggggatcccttctctcattttctaaaaactgtttctcacaccaggctaaggaggtggtggggaaggtctcccttcccctgcccacctcagacagttctagggagatggaggtttcaccacttggccactagtctcaaataactggaaggttccttttttcctgaggtcatgaaatgttctggaaccacagcgcccccgccagccctccgtgggagcacagaggggcaggccttgattggtcttctcaccctacagccacttttttggcccaactctcgagcaagccttcatcaccatcagggtctcatgggcagtctgggtttgccagcccagtccttgaacttggagagggaggtggggcttggaaatgccttgtccccagggtgggggggacaccttgtccttggagctggctgagccctgtgcccatggctgggttcagtttgcaggtatagctgtagcactctttgctggtgggaatggagaggtctcgctggccttctttgcctttttcttctttttggtcccaagcgacacctggtccccgttgagctcacctgacttctgcttctggactgtggccatgctggtgggggtggtggcagcgacagccgagtcgacactggccaccttcttggctttctttttcaacttccttttcttctttgcctccttctccactgttccagggctgtggatggctgactcctgtaggatgtcggacgccgacacagctgcctcccggcaccgccgccactcctcgtcactgtcctcactgctggagctggagggctgtcgctttcggcggggttggggagactcttccttctcacggcctccagggacagatgtgaagaaaaggcggaaaccatcatcctccaaagcgactttctgtaccttagcttttgctggctcctttgctgcttctgagatggtaatgaagctgtccagcagggctcccagcttcttggctacgtgggctcggaattcaggggtggtctgaagctcgttgccatcttgttcatgctcattcaccttatgcctgaggctcggttgggaggttgacaactggctatttgcagcaccggctcttggcttccctgccacgtgcgggcgttgctccaagccccaagccggcattgccgcctcgcggcaccgctccagctcctccgcatcgctactgctgttactactttccgaatcgctcactgtgccactgggcgccgccatcttgaaccaccgc

SEQ ID NO: 15055 - RNA, 1924 nt, Homo sapiens
  source 1..1924: mol_type = other RNA
gctgggattacaggcatgagccactgcacccggccacaagcttctacttcttgcagaatgcctttgtcccatgaaacctagtccacgagtgctatgacacttcctgaagtcttgggtggggtgaacgcacaaatcctgggggtgtagagaggaggaggatgtttacttaaaatgtcttaaggttcagcattgacagagaggcaatatccaaatcactctaagttttgttttgggtcctctgacaattgagtttccataatctggtcggctcagagacaccatcatgtgtggtatattcacaaatgcagacaaagaaaattctagaaagccaggggtgaaaaagctctcctttctcagacgattctgtgaagtctatgtgggctaaggagagaagaacaaaagtttctctgggccttggcctcttggggatcccttctctcattttctaaaaactgtttctcacaccaggctaaggaggtggtggggaaggtctcccttcccctgcccacctcagacagttctagggagatggaggtttcaccacttggccactagtctcaaataactggaaggttccttttttcctgaggtcatgaaatgttctggaaccacagcgcccccgccagccctccgtgggagcacagaggggcaggccttgattggtcttctcaccctacagccacttttttggcccaactctcgagcaagccttcatcaccatcagggtctcatgggcagtctgggtttgccagcccagtccttgaacttggagagggaggtggggcttggaaatgccttgtccccagggtgggggggacaccttgtccttggagctggctgagccctgtgcccatggctgggttcagtttgcaggtatagctgtagcactctttgctggtgggaatggagaggtctcgctggccttctttgcctttttcttctttttggtcccaagcgacacctggtccccgttgagctcacctgacttctgcttctggactgtggccatgctggtgggggtggtggcagcgacagccgagtcgacactggccaccttcttggctttctttttcaacttccttttcttctttgcctccttctccactgttccagggctgtggatggctgactcctgtaggatgtcggacgccgacacagctgcctcccggcaccgccgccactcctcgtcactgtcctcactgctggagctggagggctgtcgctttcggcggggttggggagactcttccttctcacggcctccagggacagatgtgaagaaaaggcggaaaccatcatcctccaaagcgactttctgtaccttagcttttgctggctcctttgctgcttctgagatggtaatgaagctgtccagcagggctcccagcttcttggctacgtgggctcggaattcaggggtggtctgaagctcgttgccatcttgttcatgctcattcaccttatgcctgaggctcggttgggaggttgacaactggctatttgcagcacctgggttttgacagaacatctttggctgctgtgcagcgtgagactgttggggcaaaggcaggaacacggagtctgctgcagtaattgatgtggtgagaagtgggtgaactccagatagatgcacttttaagatggagtcaaggccgggcgcggtggctcacgcctgtaatcccagcactttgggaggctgaggcaggcggatcacgaggtcaagagatcgagaccatcctggtcaacatggtgaaaccccatctctacggctcttggcttccctgccacgtgcgggcgttgctccaagccccaagccggcattgccgcctcgcggcaccgctccagctcctccgcatcgctactgctgttactactttccgaatcgctcactgtgccactgggcgccgccatcttgaaccaccgc

SEQ ID NO: 15056 - RNA, 1677 nt, Homo sapiens
  source 1..1677: mol_type = other RNA
gctgggattacaggcatgagccactgcacccggccacaagcttctacttcttgcagaatgcctttgtcccatgaaacctagtccacgagtgctatgacacttcctgaagtcttgggtggggtgaacgcacaaatcctgggggtgtagagaggaggaggatgtttacttaaaatgtcttaaggttcagcattgacagagaggcaatatccaaatcactctaagttttgttttgggtcctctgacaattgagtttccataatctggtcggctcagagacaccatcatgtgtggtatattcacaaatgcagacaaagaaaattctagaaagccaggggtgaaaaagctctcctttctcagacgattctgtgaagtctatgtgggctaaggagagaagaacaaaagtttctctgggccttggcctcttggggatcccttctctcattttctaaaaactgtttctcacaccaggctaaggaggtggtggggaaggtctcccttcccctgcccacctcagacagttctagggagatggaggtttcaccacttggccactagtctcaaataactggaaggttccttttttcctgaggtcatgaaatgttctggaaccacagcgcccccgccagccctccgtgggagcacagaggggcaggccttgattggtcttctcaccctacagccacttttttggcccaactctcgagcaagccttcatcaccatcagggtctcatgggcagtctgggtttgccagcccagtccttgaacttggagagggaggtggggcttggaaatgccttgtccccagggtgggggggacaccttgtccttggagctggctgagccctgtgcccatggctgggttcagtttgcaggtatagctgtagcactctttgctggtgggaatggagaggtctcgctggccttctttgcctttttcttctttttggtcccaagcgacacctggtccccgttgagctcacctgacttctgcttctggactgtggccatgctggtgggggtggtggcagcgacagccgagtcgacactggccaccttcttggctttctttttcaacttccttttcttctttgcctccttctccactgttccagggctgtggatggctgactcctgtaggatgtcggacgccgacacagctgcctcccggcaccgccgccactcctcgtcactgtcctcactgctggagctggagggctgtcgctttcggcggggttggggagactcttccttctcacggcctccagggacagatgtgaagaaaaggcggaaaccatcatcctccaaagcgactttctgtaccttagcttttgctggctcctttgctgcttctgagatggtaatgaagctttgtttacctgtccagcagggctcccagcttcttggctacgtgggctcggaattcaggggtggtctgaagctcgttgccatcttgttcatgctcattcaccttatgcctgaggctcggttgggaggttgacaactggctatttgcagcaccggctcttggcttccctgccacgtgcgggcgttgctccaagccccaagccggcattgccgcctcgcggcaccgctccagctcctccgcatcgctactgctgttactactttccgaatcgctcactgtgccactgggcgccgccatcttgaaccaccgc

SEQ ID NO: 15057 - RNA, 1631 nt, Homo sapiens
  source 1..1631: mol_type = other RNA
gctgggattacaggcatgagccactgcacccggccacaagcttctacttcttgcagaatgcctttgtcccatgaaacctagtccacgagtgctatgacacttcctgaagtcttgggtggggtgaacgcacaaatcctgggggtgtagagaggaggaggatgtttacttaaaatgtcttaaggttcagcattgacagagaggcaatatccaaatcactctaagttttgttttgggtcctctgacaattgagtttccataatctggtcggctcagagacaccatcatgtgtggtatattcacaaatgcagacaaagaaaattctagaaagccaggggtgaaaaagctctcctttctcagacgattctgtgaagtctatgtgggctaaggagagaagaacaaaagtttctctgggccttggcctcttggggatcccttctctcattttctaaaaactgtttctcacaccaggctaaggaggtggtggggaaggtctcccttcccctgcccacctcagacagttctagggagatggaggtttcaccacttggccactagtctcaaataactggaaggttccttttttcctgaggtcatgaaatgttctggaaccacagcgcccccgccagccctccgtgggagcacagaggggcaggccttgattggtcttctcaccctacagccacttttttggcccaactctcgagcaagccttcatcaccatcagggtctcatgggcagtctgggtttgccagcccagtccttgaacttggagagggaggtggggcttggaaatgccttgtccccagggtgggggggacaccttgtccttggagctggctgagccctgtgcccatggctgggttcagtttgcaggtatagctgtagcactctttgctggtgggaatggagaggtctcgctggccttctttgcctttttcttctttttggtcccaagcgacacctggtccccgttgagctcacctgacttctgcttctggactgtggccatgctggtgggggtggtggcagcgacagccgagtcgacactggccaccttcttggctttctttttcaacttccttttcttctttgcctccttctccactgttccagggctgtggatggctgactcctgtaggatgtcggacgccgacacagctgcctcccggcaccgccgccactcctcgtcactgtcctcactggagctggagggctgtcgctttcggcggggttggggagactcttccttctcacggccatcatcctccaaagcgactttctgtaccttagcttttgctggctcctttgctgcttctgagatggtaatgaagctgtccagcagggctcccagcttcttggctacgtgggctcggaattcaggggtggtctgaagctcgttgccatcttgttcatgctcattcaccttatgcctgaggctcggttgggaggttgacaactggctatttgcagcaccggctcttggcttccctgccacgtgcgggcgttgctccaagccccaagccggcattgccgcctcgcggcaccgctccagctcctccgcatcgctactgctgttactactttccgaatcgctcactgtgccactgggcgccgccatcttgaaccaccgc

SEQ ID NO: 15058 - RNA, 1664 nt, Homo sapiens
  source 1..1664: mol_type = other RNA
gctgggattacaggcatgagccactgcacccggccacaagcttctacttcttgcagaatgcctttgtcccatgaaacctagtccacgagtgctatgacacttcctgaagtcttgggtggggtgaacgcacaaatcctgggggtgtagagaggaggaggatgtttacttaaaatgtcttaaggttcagcattgacagagaggcaatatccaaatcactctaagttttgttttgggtcctctgacaattgagtttccataatctggtcggctcagagacaccatcatgtgtggtatattcacaaatgcagacaaagaaaattctagaaagccaggggtgaaaaagctctcctttctcagacgattctgtgaagtctatgtgggctaaggagagaagaacaaaagtttctctgggccttggcctcttggggatcccttctctcattttctaaaaactgtttctcacaccaggctaaggaggtggtggggaaggtctcccttcccctgcccacctcagacagttctagggagatggaggtttcaccacttggccactagtctcaaataactggaaggttccttttttcctgaggtcatgaaatgttctggaaccacagcgcccccgccagccctccgtgggagcacagaggggcaggccttgattggtcttctcaccctacagccacttttttggcccaactctcgagcaagccttcatcaccatcagggtctcatgggcagtctgggtttgccagcccagtccttgaacttggagagggaggtggggcttggaaatgccttgtccccagggtgggggggacaccttgtccttggagctggctgagccctgtgcccatggctgggttcagtttgcaggtatagctgtagcactctttgctggtgggaatggagaggtctcgctggccttctttgcctttttcttctttttggtcccaagcgacacctggtccccgttgagctcacctgacttctgcttctggactgtggccatgctggtgggggtggtggcagcgacagccgagtcgacactggccaccttcttggctttctttttcaacttccttttcttctttgcctccttctccactgttccagggctgtggatggctgactcctgtaggatgtcggacgccgacacagctgcctcccggcaccgccgccactcctcgtcactgtcctcactggagctggagggctgtcgctttcggcggggttggggagactcttccttctcacggcctccagggacagatgtgaagaaaaggcggaaaccatcatcctccaaagcgactttctgtaccttagcttttgctggctcctttgctgcttctgagatggtaatgaagctgtccagcagggctcccagcttcttggctacgtgggctcggaattcaggggtggtctgaagctcgttgccatcttgttcatgctcattcaccttatgcctgaggctcggttgggaggttgacaactggctatttgcagcaccggctcttggcttccctgccacgtgcgggcgttgctccaagccccaagccggcattgccgcctcgcggcaccgctccagctcctccgcatcgctactgctgttactactttccgaatcgctcactgtgccactgggcgccgccatcttgaaccaccgc

SEQ ID NO: 15059 - RNA, 1757 nt, Homo sapiens
  source 1..1757: mol_type = other RNA
gctgggattacaggcatgagccactgcacccggccacaagcttctacttcttgcagaatgcctttgtcccatgaaacctagtccacgagtgctatgacacttcctgaagtcttgggtggggtgaacgcacaaatcctgggggtgtagagaggaggaggatgtttacttaaaatgtcttaaggttcagcattgacagagaggcaatatccaaatcactctaagttttgttttgggtcctctgacaattgagtttccataatctggtcggctcagagacaccatcatgtgtggtatattcacaaatgcagacaaagaaaattctagaaagccaggggtgaaaaagctctcctttctcagacgattctgtgaagtctatgtgggctaaggagagaagaacaaaagtttctctgggccttggcctcttggggatcccttctctcattttctaaaaactgtttctcacaccaggctaaggaggtggtggggaaggtctcccttcccctgcccacctcagacagttctagggagatggaggtttcaccacttggccactagtctcaaataactggaaggttccttttttcctgaggtcatgaaatgttctggaaccacagcgcccccgccagccctccgtgggagcacagaggggcaggccttgattggtcttctcaccctacagccacttttttggcccaactctcgagcaagccttcatcaccatcagggtctcatgggcagtctgggtttgccagcccagtccttgaacttggagagggaggtggggcttggaaatgccttgtccccagggtgggggggacaccttgtccttggagctggctgagccctgtgcccatggctgggttcagtttgcaggtatagctgtagcactctttgctggtgggaatggagaggtctcgctggccttctttgcctttttcttctttttggtcccaagcgacacctggtccccgttgagctcacctgacttctgcttctggactgtggccatgctggtgggggtggtggcagcgacagccgagtcgacactggccaccttcttggctttctttttcaacttccttttcttctttgcctccttctccactgttccagggctgtggatggctgactcctgtaggatgtcggacgccgacacagctgcctcccggcaccgccgccactcctcgtcactgtcctcactggagctggagggctgtcgctttcggcggggttggggagactcttccttctcacggcctccagggacagatgtgaagaaaaggcggaaaccatcatcctccaaagcgactttctgtaccttagcttttgctggctcctttgctgcttctgagatggtaatgaagctgtccagcagggctcccagcttcttggctacgtgggctcggaattcaggggtggtctgaagctcgttgccatcttgttcatgctcattcaccttatgcctggaaatgccaggcgtgaagcctagcatctggcacacgcaggggatcagtatttgttgaataagtgaaacttgaacccaaagtgcatagtacctgaggctcggttgggaggttgacaactggctatttgcagcaccggctcttggcttccctgccacgtgcgggcgttgctccaagccccaagccggcattgccgcctcgcggcaccgctccagctcctccgcatcgctactgctgttactactttccgaatcgctcactgtgccactgggcgccgccatcttgaaccaccgc

SEQ ID NO: 15060 - RNA, 2287 nt, Homo sapiens
  source 1..2287: mol_type = other RNA
gctgggattacaggcatgagccactgcacccggccaggaatgtttcctaattatgcttaaagtccagaagtaaagtattattattaaagtgcagatgccagtttctacagttagcaggtgtgagaacaaagataatccaaaatgatgcttaaaacatcaactcatttctatcagactttagttctcctcttgtagggctacaggagaaagcaaaagaaactccaagttactgggttctccagtatgataagtaaaggttgtcaaggtcgtgcagtagaaaagaaacaggcagagctgaatgttagctcagctcttagatagctgttgcagcattaggcctatcatttctcctttctgagccttagcaaacaaaggtaataatacttatttcacaggtttgttacatgtaatcttacacattgcatgtgtgcaataaatggtaacttattctaaaaggtggggcttagttgttgagggtattagtattggaccatataaaactgacattttttatagataaaaaatagccaaattttagacttcactctaaggtgataccctcctaggaaccttgaggaaactgttacagtgaggccacagtgtggagggcaaggtcaggttccttggtgagttttgagtcaatggtcatggatggccattttcattagtgactagtttataatatgctgaaataatatacaccatcatgaagcctgggtatctcagactatcccattccctacccacaatatagatcaacattttacatcttgctaaagttagcatattaagctcattgtatttgcatggttacacttctcttccatgctgctaagagtcacaagtacacaagaagaatgggcataaacatatcggtacacctgccctttctgataataccagtaagatagacaatcatgtctagactcatggtgatccatgtactttcctaaaagtgtgatttcagagtgtttcccatattgttgatttccttctcagtcgctcttctttggatttgaggcagacgtttctggaaatttccactcagcaggatgtagagaaaagggttaatgctgctgctggcatagctgagacagatggagaggtaataacccacatagaaggccagtgtgggctgttccatctgtaagttcaccagttgtatcacatgataaggggcagcactcaggataaagactaccaccagcaccagcaccatctttgtcaacttcatcactctctgttttggtacactgggattgcagcatctggcatccttattctgttgatacatctcccaagtatagcataaaattaaaatatagcacaccaaaatcaagggtagagggaaaaaaaaagttgttatcgtcaaataaagtgtataccagagtacatcgtcaggggatgtcaaatcaaaagcacaactctcaacaccgtctttaaatttgatgaccttcgagtagacccagacaggcaatgccaggataaaggaagctgcccaaaggcccaaattgatccggatggtcttgtaccttgttctccaacgtgtcagtcgaaatggttggacgagggcaaagtacctgtccacactcattacagtcatgatggcactacaggcaaattggttacaagtatccagggatgtgatgatggtgcagagaggccccccaaacacccactctccccctcgggcccattggtgaataagaaaaggcattccaactatgtggaccaaatcagccacagccaggttgcagatatagatgtcagggactgtttttttcctggatcttattatagtgaatacaatgaggatgttgccaaccagccctgttgaacagataatcccaatcatggaagggaggatgactgtatctaccacactggcagtttgataagcaaactctttattccaggatttgtttaaaagttcggcagaggtgttccaacaagatgcatgaaatggattcattgttcgtggactttccagggattaaagctgggtgctcgcgtcctccccgcgcggcggacagcccgggcgcccttcctctctgcgggactgcaggtctatccgctaagcgcgcgtgaccaaaaacggctctcagcgggtcccagctgacggaaggtgggggaggagtgcgagggtctctgagacaggttgggagccagccccacctccatttccaaagcgggggtccaggcacaggaacagccaaacgcccgaaccagcggggttacctttgccacttcatccaatccgagcatcgggtgcgtcgtgctcttttct

SEQ ID NO: 15061 - RNA, 2048 nt, Homo sapiens
  source 1..2048: mol_type = other RNA
gctgggattacaggcatgagccactgcacccggccaggaatgtttcctaattatgcttaaagtccagaagtaaagtattattattaaagtgcagatgccagtttctacagttagcaggtgtgagaacaaagataatccaaaatgatgcttaaaacatcaactcatttctatcagactttagttctcctcttgtagggctacaggagaaagcaaaagaaactccaagttactgggttctccagtatgataagtaaaggttgtcaaggtcgtgcagtagaaaagaaacaggcagagctgaatgttagctcagctcttagatagctgttgcagcattaggcctatcatttctcctttctgagccttagcaaacaaaggtaataatacttatttcacaggtttgttacatgtaatcttacacattgcatgtgtgcaataaatggtaacttattctaaaaggtggggcttagttgttgagggtattagtattggaccatataaaactgacattttttatagataaaaaatagccaaattttagacttcactctaaggtgataccctcctaggaaccttgaggaaactgttacagtgaggccacagtgtggagggcaaggtcaggttccttggtgagttttgagtcaatggtcatggatggccattttcattagtgactagtttataatatgctgaaataatatacaccatcatgaagcctgggtatctcagactatcccattccctacccacaatatagatcaacattttacatcttgctaaagttagcatattaagctcattgtatttgcatggttacacttctcttccatgctgctaagagtcacaagtacacaagaagaatgggcataaacatatcggtacacctgccctttctgataataccagtaagatagacaatcatgtctagactcatggtgatccatgtactttcctaaaagtgtgatttcagagtgtttcccatattgttgatttccttctcagtcgctcttctttggatttgaggcagacgtttctggaaatttccactcagcaggatgtagagaaaagggttaatgctgctgctggcatagctgagacagatggagaggtaataacccacatagaaggccagtgtgggctgttccatctgtaagttcaccagttgtatcacatgataaggggcagcactcaggataaagactaccaccagcaccagcaccatctttgtcaacttcatcactctctgttttggtacactgggattgcagcatctggcatccttattctgttgatacatctcccaagtatagcataaaattaaaatatagcacaccaaaatcaagggtagagggaaaaaaaaagttgttatcgtcaaataaagtgtataccagagtacatcgtcaggggatgtcaaatcaaaagcacaactctcaacaccgtctttaaatttgatgaccttcgagtagacccagacaggcaatgccaggataaaggaagctgcccaaaggcccaaattgatccggatggtcttgtaccttgttctccaacgtgtcagtcgaaatggttggacgagggcaaagtacctgtccacactcattacagtcatgatggcactacaggcaaattggttacaagtatccagggatgtgatgatggtgcagagaggccccccaaacacccactctccccctcgggcccattggtgaataagaaaaggcattccaactatgtggaccaaatcagccacagccaggttgcagatatagatgtcagggactgtttttttcctggatcttattatagtgaatacaatgaggatgttgccaaccagccctgttgaacagataatcccaatcatggaagggaggatgactgtatctaccacactggcagtttgataagcaaactctttattccaggatttgtttaaaagttcggcagaggtgttccaacaagatgcatgaaatggattcattgttcgtggactttccagggattaaagctttgccacttcatccaatccgagcatcgggtgcgtcgtgctcttttct

SEQ ID NO: 15062 - RNA, 5456 nt, Homo sapiens
  source 1..5456: mol_type = other RNA
gctgggattacaggcatgagccactgcacccggcccacattgggaatttttttttttttaaacagtgtcactctgttgcccagactggagtgcagtggcacaatctcagctcactacaacctctgcctcccagattcaagtgattctcctgcctcagcctcctaagtagctgggattacacgcatgcgtcaccacacacacctaatttttgttattttttgtagagatgggttttccccatgttggccagcctggtctcaaactcccagcctcaagtgatccgcccaccttggcctcccaaagtgtgggattacaggcatgagccaccacacctgacccacattgggaaatcttgttaatatcagattacaattaagtgggaatagtggtgaggctgagactatttctaataagttccctggtgatactgaggctgctgttcctcaaatcatacttgggagtagcaatgttctagagatgatctagtgggtttttttgagacagagttactctatcgcccaggctggaatgcagtggaaatctcggctcactgcaacctctgcctcccaggttcaagtgattctcctgcctcagcctcccaactagctgggattacacgcacccaccaccatgcccggctaatttttgtatttttagtagatacagggtttcgccatgttggccatgcttgtcttgaactcctgacttcacgtggtccacctgccttggcctcccaaagtgctgggataacaggcataaaccaccacgcctggcaagatttgattatgacttatcagatctaaacagagttcctgaactagtcaagtagcaatctaattctacattagaacaaaacgcaagagataggccaatggttagaactgagggtataatagggtttacctgtatgaaattcactgtttattaagtcacttttatgtacagaaagacctgccctagttaccatatcacttttagggtttcaaggcttcatctcacattcttcagctgaaaacaggtaaatctggtgaaggtattatctgaactgcccgtcacagagctagagagaagtttttcttttgttttttttttttttgagacagtctctcactctcaccctggctggagtgcattggtgtgatctcaactcactgcaacctccaccttccaggttcaagcaattctcctgcctcagtctcccgagtacctgggattacaggcgcctgccaccaagcccagctaattttttttagtagagacggggttttgccaccttgcccaggctggtctcgaactcctgagctcctgcaatccactcacctcagcctccctaaatgctgggattataggcatgaggaaccgcacccagcctaaagagaagtttttcttttttttttttttttgagacggagtctcgctctgtcacccaggctggagtgcagtggcgcgctctcggctcactgcaagctccgcctcccgggttcacaccattctcctgcctcagcctcccgagtagctgggactacaggcgcctgccaccgcacccggctaatttttttttgtattttttagtagagacggggtttcaccgtggtctcgatctcctgaccttgtgatccgcccgcctcggcctcccaaagtgctgggattgcaggcgtgagccactgcgcccggccaagagaagtttttcttaaaatcctttttttgggggggccaggatcggtggctaacatctgtaatcccagcaactttgggaggtcgaggcaggcggatcatgaggtcaagcaatcgagaccatcctggccaacatggtgaaacctcatctctattaaaaatacaaaaattagctgagtgtggtagcacgtgcctgtagtcccagctacttgggaggctgaggcaggagaattgcttgaacccaggagacggaggttgcggtgagctgagaacgcaccactgcattctagcctgacgacagagggagactccgtctcaaaaataaaaaataaaaataaaaataatcccttttttttttttaactatgcaagtctcattacatttaaaacccttttttaaacttggtcccttttctgtgccaactttatgtttgtttttgttcttgtttttgtttgagatggagtctcgctctgttgcccaggctggagtgcggtggcgcgatctcagctcactccaacctctgcctcctgggttcaagtgattctcctgccttagcctcctgagtagctgggattacaggcgtgcaccaccacgcctggataattttttttgtaattttagtagagatggggtttcaccatattggtctgaaactcctgacctcgtgatctgcccgccttggcctcccaaagtgctggcattacaggtatgagccactgtgcctggcccctattttttattttctgagatgaagtctcgctctgttgcccaggctggagcgcactagcatgatctcagctcaatgcaacctccgcctccaaggttaaagcaattcttctgcctcagcctctaagtagctgggatcacaggtgcctggaacgtgcctggctaatttttctatttttagtagagatggttttgccatgttggccaggctggtctcaaactcctgacctcaggtgatctgtctgcctcggcctcccaaagtgttaggattacaggcgtgagccattgtacccggccgagttacataatttgaatacattgttattaatctgcaataatctgtaaggtattatctccattttacagatgagaatgtgaagaaaatgacttgttcaaggccctcattgcaataaccagagctaagtttgcaaccacgtctcttagactccaaggcccacacactttttactttatgacactgcctccctaaatgctaaagattaaaaactctggtaggatgaatttttacatctctgtcagcagtgggattagaatccatgcctgtgaagagatgggaccgtaactcagcacctaaatggattattttttgtattaaaaatttcataattccctttctcagggaaatctgtaaagataaaatattaaagataaagatctgtaaagataaaaaatattaaatcctacaggcaagcctgagggcagcactaatgtgttaatggcttaaaaaatgattccaatgtttgcatgccctcaggcctggggcgtttattagtgcaggccaaagggctcttgggatttcttttgccttgatgagatacggcagaaacaacctgggggtttgaagagtggggctgcaaaaaggatttctgcaactccaatgcaaaatgatagtccatgtgttctggcatatcccataccggtaccagggagccacacttctcacagggcacttggtcctcagcagctagaagacttggatttggggttgctttctgagtcacctccagcacagatttggaagctgaagaggcgtgcatgctttggctgttgtgggccaaatccatctctgcaggagttgctttagaggattcttctagcttcgacaccccttcacaaacagggacacaccctggatactctgttggtaaagagtttggtaatgctttacagttggaccatgggttttgttggggggaagaaactgaagaattattaagctgtttctgctttagaagcagacttttctgcttaaagaagggctcagttcctgtactttgactggtttgaaaaggtaatgagggcttggatggtgaattgctcatgggagcctgagtgggagcagtaagagatgaaagcgaagcttctttaactttctgcctttctgcagctttttggaagaatgattccagagacgtggttgctttcttagtggctgtcaccgctgggccacttccctgggtcttagcttctgagctggtaactggcacctttggcagagaacttgggtcactgctcaagaagctggtgatgtcattctgtctggattccagaagtattacagttcttgatgacagtaaatgcatcatggctcatcttgtgagcatcatagcgggtaagggcacagcagcggcgcaggctgctgaggcgtttgtctccttgtacacgaatgctcacaaccagctgggtggctaccctgtcattatcatttcggtctttagtcagtctctcctctagttcctgggctaattgcaacagccaccattgtacctgttcccgagtagcaagagctgtttttcctgggaagttcttactacagccaatggttttgggtagttgcctgggtttaactggatcatgttcaatccctcggcacatggcatatagccaagacccattcttctccccaaaatgactctggagctgggattcagtgaactgggtcagttcacccatgtattctatccctaggatctcaatgacagaggcccctagctttcctccaagactacggattttgcgaatgggcatttggctgaagagctgtgggactgacccatgtgaaaccagggtttggcggttgggcttgtttagtccacaggccagttttgccaggaccttattgtgtgaaattccagctgaacactgaaaaccagtctccctctctatggctgctctcatttcctccacaatcactgctcccacggtgagctgcaggtctggagaggtgaggttatcaatctgaagagaatcgagccattgaaataagccttgttttcgcatcccctctttctgaacagtctcttctgccgttgtagggccttggggcaacccttcaatgtaagtgcttggcaacaagtctgccgagataggctgaccttgtagcttttgtagtctctcttgtacagcactggtcagatctacgtaagcctcatcaatgctggcacgttcaatcacagcaaaacgagacattatctccatcacttcaacactggcttcccggtacttggtgaggttagctttcccacgggactcacgaacttgtgccagtagaagatctggacataacttcttagcatcatctgcccacatacttctagtgactccaaatgcacgagcttcataactcactgcaattattccaccacccttccatgatttgtactgtacaactgcacaaggtttattcctcaaatgaggattttgccgctgctccacttgaacaaaaaaacagtccatgtccacgagagcaaccactcgatcctgtccagtagccatttttcaaggtaacaaacacctggcaaaactgccagcagcggttgccgaaaatgctgggttcggtgcctactggaaggaaaatggaagggctcctgaatatcttttcgcctttctaggagcggtccagtgagtttcgagcgagatttattccctgtgacgacggagaaaccgagaagggatcgtaaaggatcctgcccgggcaaccgtccccagcagggatcagacgagagcggcgcgcccagcaatgcagccgccagact

SEQ ID NO: 15063 - RNA, 5527 nt, Homo sapiens
  source 1..5527: mol_type = other RNA
gctgggattacaggcatgagccactgcacccggcccacattgggaatttttttttttttaaacagtgtcactctgttgcccagactggagtgcagtggcacaatctcagctcactacaacctctgcctcccagattcaagtgattctcctgcctcagcctcctaagtagctgggattacacgcatgcgtcaccacacacacctaatttttgttattttttgtagagatgggttttccccatgttggccagcctggtctcaaactcccagcctcaagtgatccgcccaccttggcctcccaaagtgtgggattacaggcatgagccaccacacctgacccacattgggaaatcttgttaatatcagattacaattaagtgggaatagtggtgaggctgagactatttctaataagttccctggtgatactgaggctgctgttcctcaaatcatacttgggagtagcaatgttctagagatgatctagtgggtttttttgagacagagttactctatcgcccaggctggaatgcagtggaaatctcggctcactgcaacctctgcctcccaggttcaagtgattctcctgcctcagcctcccaactagctgggattacacgcacccaccaccatgcccggctaatttttgtatttttagtagatacagggtttcgccatgttggccatgcttgtcttgaactcctgacttcacgtggtccacctgccttggcctcccaaagtgctgggataacaggcataaaccaccacgcctggcaagatttgattatgacttatcagatctaaacagagttcctgaactagtcaagtagcaatctaattctacattagaacaaaacgcaagagataggccaatggttagaactgagggtataatagggtttacctgtatgaaattcactgtttattaagtcacttttatgtacagaaagacctgccctagttaccatatcacttttagggtttcaaggcttcatctcacattcttcagctgaaaacaggtaaatctggtgaaggtattatctgaactgcccgtcacagagctagagagaagtttttcttttgttttttttttttttgagacagtctctcactctcaccctggctggagtgcattggtgtgatctcaactcactgcaacctccaccttccaggttcaagcaattctcctgcctcagtctcccgagtacctgggattacaggcgcctgccaccaagcccagctaattttttttagtagagacggggttttgccaccttgcccaggctggtctcgaactcctgagctcctgcaatccactcacctcagcctccctaaatgctgggattataggcatgaggaaccgcacccagcctaaagagaagtttttcttttttttttttttttgagacggagtctcgctctgtcacccaggctggagtgcagtggcgcgctctcggctcactgcaagctccgcctcccgggttcacaccattctcctgcctcagcctcccgagtagctgggactacaggcgcctgccaccgcacccggctaatttttttttgtattttttagtagagacggggtttcaccgtggtctcgatctcctgaccttgtgatccgcccgcctcggcctcccaaagtgctgggattgcaggcgtgagccactgcgcccggccaagagaagtttttcttaaaatcctttttttgggggggccaggatcggtggctaacatctgtaatcccagcaactttgggaggtcgaggcaggcggatcatgaggtcaagcaatcgagaccatcctggccaacatggtgaaacctcatctctattaaaaatacaaaaattagctgagtgtggtagcacgtgcctgtagtcccagctacttgggaggctgaggcaggagaattgcttgaacccaggagacggaggttgcggtgagctgagaacgcaccactgcattctagcctgacgacagagggagactccgtctcaaaaataaaaaataaaaataaaaataatcccttttttttttttaactatgcaagtctcattacatttaaaacccttttttaaacttggtcccttttctgtgccaactttatgtttgtttttgttcttgtttttgtttgagatggagtctcgctctgttgcccaggctggagtgcggtggcgcgatctcagctcactccaacctctgcctcctgggttcaagtgattctcctgccttagcctcctgagtagctgggattacaggcgtgcaccaccacgcctggataattttttttgtaattttagtagagatggggtttcaccatattggtctgaaactcctgacctcgtgatctgcccgccttggcctcccaaagtgctggcattacaggtatgagccactgtgcctggcccctattttttattttctgagatgaagtctcgctctgttgcccaggctggagcgcactagcatgatctcagctcaatgcaacctccgcctccaaggttaaagcaattcttctgcctcagcctctaagtagctgggatcacaggtgcctggaacgtgcctggctaatttttctatttttagtagagatggttttgccatgttggccaggctggtctcaaactcctgacctcaggtgatctgtctgcctcggcctcccaaagtgttaggattacaggcgtgagccattgtacccggccgagttacataatttgaatacattgttattaatctgcaataatctgtaaggtattatctccattttacagatgagaatgtgaagaaaatgacttgttcaaggccctcattgcaataaccagagctaagtttgcaaccacgtctcttagactccaaggcccacacactttttactttatgacactgcctccctaaatgctaaagattaaaaactctggtaggatgaatttttacatctctgtcagcagtgggattagaatccatgcctgtgaagagatgggaccgtaactcagcacctaaatggattattttttgtattaaaaatttcataattccctttctcagggaaatctgtaaagataaaatattaaagataaagatctgtaaagataaaaaatattaaatcctacaggcaagcctgagggcagcactaatgtgttaatggcttaaaaaatgattccaatgtttgcatgccctcaggcctggggcgtttattagtgcaggccaaagggctcttgggatttcttttgccttgatgagatacggcagaaacaacctgggggtttgaagagtggggctgcaaaaaggatttctgcaactccaatgcaaaatgatagtccatgtgttctggcatatcccataccggtaccagggagccacacttctcacagggcacttggtcctcagcagctagaagacttggatttggggttgctttctgagtcacctccagcacagatttggaagctgaagaggcgtgcatgctttggctgttgtgggccaaatccatctctgcaggagttgctttagaggattcttctagcttcgacaccccttcacaaacagggacacaccctggatactctgttggtaaagagtttggtaatgctttacagttggaccatgggttttgttggggggaagaaactgaagaattattaagctgtttctgctttagaagcagacttttctgcttaaagaagggctcagttcctgtactttgactggtttgaaaaggtaatgagggcttggatggtgaattgctcatgggagcctgagtgggagcagtaagagatgaaagcgaagcttctttaactttctgcctttctgcagctttttggaagaatgattccagagacgtggttgctttcttagtggctgtcaccgctgggccacttccctgggtcttagcttctgagctggtaactggcacctttggcagagaacttgggtcactgctcaagaagctggtgatgtctgtagaagatgaaggggcagaggcagaaaattttgtagcacagaggaaaagcattgtgagaggaggagaccattctgtctggattccagaagtattacagttcttgatgacagtaaatgcatcatggctcatcttgtgagcatcatagcgggtaagggcacagcagcggcgcaggctgctgaggcgtttgtctccttgtacacgaatgctcacaaccagctgggtggctaccctgtcattatcatttcggtctttagtcagtctctcctctagttcctgggctaattgcaacagccaccattgtacctgttcccgagtagcaagagctgtttttcctgggaagttcttactacagccaatggttttgggtagttgcctgggtttaactggatcatgttcaatccctcggcacatggcatatagccaagacccattcttctccccaaaatgactctggagctgggattcagtgaactgggtcagttcacccatgtattctatccctaggatctcaatgacagaggcccctagctttcctccaagactacggattttgcgaatgggcatttggctgaagagctgtgggactgacccatgtgaaaccagggtttggcggttgggcttgtttagtccacaggccagttttgccaggaccttattgtgtgaaattccagctgaacactgaaaaccagtctccctctctatggctgctctcatttcctccacaatcactgctcccacggtgagctgcaggtctggagaggtgaggttatcaatctgaagagaatcgagccattgaaataagccttgttttcgcatcccctctttctgaacagtctcttctgccgttgtagggccttggggcaacccttcaatgtaagtgcttggcaacaagtctgccgagataggctgaccttgtagcttttgtagtctctcttgtacagcactggtcagatctacgtaagcctcatcaatgctggcacgttcaatcacagcaaaacgagacattatctccatcacttcaacactggcttcccggtacttggtgaggttagctttcccacgggactcacgaacttgtgccagtagaagatctggacataacttcttagcatcatctgcccacatacttctagtgactccaaatgcacgagcttcataactcactgcaattattccaccacccttccatgatttgtactgtacaactgcacaaggtttattcctcaaatgaggattttgccgctgctccacttgaacaaaaaaacagtccatgtccacgagagcaaccactcgatcctgtccagtagccatttttcaaggtaacaaacacctggcaaaactgccagcagcggttgccgaaaatgctgggttcggtgcctactggaaggaaaatggaagggctcctgaatatcttttcgcctttctaggagcggtccagtgagtttcgagcgagatttattccctgtgacgacggagaaaccgagaagggatcgtaaaggatcctgcccgggcaaccgtccccagcagggatcagacgagagcggcgcgcccagcaatgcagccgccagact

SEQ ID NO: 15064 - RNA, 5168 nt, Homo sapiens
  source 1..5168: mol_type = other RNA
gctgggattacaggcatgagccactgcacccggcccacattgggaatttttttttttttaaacagtgtcactctgttgcccagactggagtgcagtggcacaatctcagctcactacaacctctgcctcccagattcaagtgattctcctgcctcagcctcctaagtagctgggattacacgcatgcgtcaccacacacacctaatttttgttattttttgtagagatgggttttccccatgttggccagcctggtctcaaactcccagcctcaagtgatccgcccaccttggcctcccaaagtgtgggattacaggcatgagccaccacacctgacccacattgggaaatcttgttaatatcagattacaattaagtgggaatagtggtgaggctgagactatttctaataagttccctggtgatactgaggctgctgttcctcaaatcatacttgggagtagcaatgttctagagatgatctagtgggtttttttgagacagagttactctatcgcccaggctggaatgcagtggaaatctcggctcactgcaacctctgcctcccaggttcaagtgattctcctgcctcagcctcccaactagctgggattacacgcacccaccaccatgcccggctaatttttgtatttttagtagatacagggtttcgccatgttggccatgcttgtcttgaactcctgacttcacgtggtccacctgccttggcctcccaaagtgctgggataacaggcataaaccaccacgcctggcaagatttgattatgacttatcagatctaaacagagttcctgaactagtcaagtagcaatctaattctacattagaacaaaacgcaagagataggccaatggttagaactgagggtataatagggtttacctgtatgaaattcactgtttattaagtcacttttatgtacagaaagacctgccctagttaccatatcacttttagggtttcaaggcttcatctcacattcttcagctgaaaacaggtaaatctggtgaaggtattatctgaactgcccgtcacagagctagagagaagtttttcttttgttttttttttttttgagacagtctctcactctcaccctggctggagtgcattggtgtgatctcaactcactgcaacctccaccttccaggttcaagcaattctcctgcctcagtctcccgagtacctgggattacaggcgcctgccaccaagcccagctaattttttttagtagagacggggttttgccaccttgcccaggctggtctcgaactcctgagctcctgcaatccactcacctcagcctccctaaatgctgggattataggcatgaggaaccgcacccagcctaaagagaagtttttcttttttttttttttttgagacggagtctcgctctgtcacccaggctggagtgcagtggcgcgctctcggctcactgcaagctccgcctcccgggttcacaccattctcctgcctcagcctcccgagtagctgggactacaggcgcctgccaccgcacccggctaatttttttttgtattttttagtagagacggggtttcaccgtggtctcgatctcctgaccttgtgatccgcccgcctcggcctcccaaagtgctgggattgcaggcgtgagccactgcgcccggccaagagaagtttttcttaaaatcctttttttgggggggccaggatcggtggctaacatctgtaatcccagcaactttgggaggtcgaggcaggcggatcatgaggtcaagcaatcgagaccatcctggccaacatggtgaaacctcatctctattaaaaatacaaaaattagctgagtgtggtagcacgtgcctgtagtcccagctacttgggaggctgaggcaggagaattgcttgaacccaggagacggaggttgcggtgagctgagaacgcaccactgcattctagcctgacgacagagggagactccgtctcaaaaataaaaaataaaaataaaaataatcccttttttttttttaactatgcaagtctcattacatttaaaacccttttttaaacttggtcccttttctgtgccaactttatgtttgtttttgttcttgtttttgtttgagatggagtctcgctctgttgcccaggctggagtgcggtggcgcgatctcagctcactccaacctctgcctcctgggttcaagtgattctcctgccttagcctcctgagtagctgggattacaggcgtgcaccaccacgcctggataattttttttgtaattttagtagagatggggtttcaccatattggtctgaaactcctgacctcgtgatctgcccgccttggcctcccaaagtgctggcattacaggtatgagccactgtgcctggcccctattttttattttctgagatgaagtctcgctctgttgcccaggctggagcgcactagcatgatctcagctcaatgcaacctccgcctccaaggttaaagcaattcttctgcctcagcctctaagtagctgggatcacaggtgcctggaacgtgcctggctaatttttctatttttagtagagatggttttgccatgttggccaggctggtctcaaactcctgacctcaggtgatctgtctgcctcggcctcccaaagtgttaggattacaggcgtgagccattgtacccggccgagttacataatttgaatacattgttattaatctgcaataatctgtaaggtattatctccattttacagatgagaatgtgaagaaaatgacttgttcaaggccctcattgcaataaccagagctaagtttgcaaccacgtctcttagactccaaggcccacacactttttactttatgacactgcctccctaaatgctaaagattaaaaactctggtaggatgaatttttacatctctgtcagcagtgggattagaatccatgcctgtgaagagatgggaccgtaactcagcacctaaatggattattttttgtattaaaaatttcataattccctttctcagggaaatctgtaaagataaaatattaaagataaagatctgtaaagataaaaaatattaaatcctacaggcaagcctgagggcagcactaatgtgttaatggcttaaaaaatgattccaatgtttgcatgccctcaggcctggggcgtttattagtgcaggccaaagggctcttgggatttcttttgccttgatgagatacggcagaaacaacctgggggtttgaagagtggggctgcaaaaaggatttctgcaactccaatgcaaaatgatagtccatgtgttctggcatatcccataccggtaccagggagccacacttctcacagggcacttggtcctcagcagctagaagacttggatttggggttgctttctgagtcacctccagcacagatttggaagctgaagaggcgtgcatgctttggctgttgtgggccaaatccatctctgcaggagttgctttagaggattcttctagcttcgacaccccttcacaaacagggacacaccctggatactctgttggtaaagagtttggtaatgctttacagttggaccatgggttttgttggggggaagaaactgaagaattattaagctgtttctgctttagaagcagacttttctgcttaaagaagggctcagttcctgtactttgactggtttgaaaaggtaatgagggcttggatggtgaattgctcatgggagcctgagtgggagcagtaagagatgaaagcgaagcttctttaactttctgcctttctgcagctttttggaagaatgattccagagacgtggttgctttcttagtggctgtcaccgctgggccacttccctgggtcttagcttctgagctggtaactggcacctttggcagagaacttgggtcactgctcaagaagctggtgatgtctgtagaagatgaaggggcagaggcagaaaattttgtagcacagaggaaaagcattgtgagaggaggagaccattctgtctggattccagaagtattacagttcttgatgacagtaaatgcatcatggctcatcttgtgagcatcatagcgggtaagggcacagcagcggcgcaggctgctgaggcgtttgtctccttgtacacgaatgctcacaaccagctgggtggctaccctgtcattatcatttcggtctttagtcagtctctcctctagttcctgggctaattgcaacagccaccattgtacctgttcccgagtagcaagagctgtttttcctgggaagttcttactacagccaatggttttgggtagttgcctgggtttaactggatcatgttcaatccctcggcacatggcatatagccaagacccattcttctccccaaaatgactctggagctgggattcagtgaactgggtcagttcacccatgtattctatccctaggatctcaatgacagaggcccctagctttcctccaagactacggattttgcgaatgggcatttggctgaagagctgtgggactgacccatgtgaaaccagggtttggcggttgggcttgtttagtccacaggccagttttgccaggaccttattgtgtgaaattccagctgaacactgaaaaccagtctccctctctatggctgctctcatttcctccacaatcactgctcccacggtgagctgcaggtctggagaggtgaggttatcaatctgaagagaatcgagccattgaaataagccttgttttcgcatcccctttggtgaggttagctttcccacgggactcacgaacttgtgccagtagaagatctggacataacttcttagcatcatctgcccacatacttctagtgactccaaatgcacgagcttcataactcactgcaattattcaaggtaacaaacacctggcaaaactgccagcagcggttgccgaaaatgctgggttcggtgcctactggaaggaaaatggaagggctcctgaatatcttttcgcctttctaggagcggtccagtgagtttcgagcgagatttattccctgtgacgacggagaaaccgagaagggatcgtaaaggatcctgcccgggcaaccgtccccagcagggatcagacgagagcggcgcgcccagcaatgcagccgccagact

SEQ ID NO: 15065 - RNA, 4113 nt, Homo sapiens
  source 1..4113: mol_type = other RNA
gctgggattacaggcatgagccactgcacccggccctgtctgccctttcttgagcctctggtcccagcaagtttggttgtagtttgatgtgtattaactcttaattctcataataaccctgaaaggtaagtgtgtttgttatttattgctacatcacaaatatctcaaattgagcaaacatttatgatctcatgtgatttctgagggccaggaacctataagcagcttaggtgggtggctctggctcaaggtctctcatgaggttgccgtcaggatgttggccaggactgcagtcatgtaaaagcctgaccagggaggggccattggcttccaaggtgaccccttacacggctgttggcaggaggcctgttcctcattggctgtcggcagggggatcctctgttcctcgccatcggacctctccatggtgctgcttgagtgtcctcatgacatggcggctggcttgcctcagagtaactcttgaagaatgtgctagaaggtgagcacctggaagaacaggtagtgggccagatgggccctcctctgtcttcttctgctctatgcttcttgtgggcttgaagacagtgaggagccaaaggtctgtacctcgtctaccccaaaagtactgcctgggcctctggtaccctaatcaggatgcttcgaccttgttctgatgcctggggacttctggtgagttccctggccatccatcctggtctgttcaccttctcaggactccagttgagttgggctgcgtgtgacagaccccttggggaaaacgccgcagctgcaggtgccaccagtgagtcttctattcaaagtaattaactggcatcatctgtccaagagatgggatggataagaagttaagcttccaggagatgcctcatcatttgtgccagtgaccccgcataatttcttgatgaattgtgcaaactgggaagctgatagctcgtttcagattctctagattttgcccctgaaaaagcatttacgtgatgcagtccgaggtcttgtatggaggagcttggtgtggggagatgtgtggctcacgaactgtcttgtgcatgtgtctccccaggggcattttcagatttctgccacggagatgctcttcgcaaagggagagtcaggtacattggaggattcattgctgtgaccagggaaagcagaggacatgcaaaattaatatttccctttctatcttctaggatggacttttttcattcagaaagccgctctggcttaaagacatgtacaaacctctcagtgccacaagagtaaagaatcacgcatggaagctgcacaagaagtcatctaatgaggacaagatcctcaacagggaccctgggtaaatgacgggaccctcacagttcccatctaaaatgaggagggggtgagacgcttaattgctcctttcaagaatgaaaaccttggcattgttattcttatcccagggacagtgaagccccaacagagaaggaggaggagagtgaagccctgccataggaggagaacccagcccacctcaggcctcctgcaaaaacacatagcataaacaataccatcagaaagaaaagcaggactgaagccagcagcccacacatccacagaggcagcgggcagagcaagcacagggccatcgttcctgcccttgtttcccagtctaattagtcacccagacctgaaaacatatcctcagggggtggagattttacaattaaataccattgtttttggtgccctctccctgggttcatcaagcaccagtcatataataccacatacttgaactcctgcccacaggggacctcccatctcctggcccctattataggatcactgggcctacctgcactgtggggccaagccctgtctttttcccaagccctcaagcacacgcatgaatgttcatcccgacttggtagggggcttttcacccttacaagatggcaaaagattcacactgctttttttaaaatttgtttttctttttaaaaatcccaacccttggatagcaagggaggtgctggaggggtagggtcaagaagagtgtgtgagaacagtaatttcccaagactgccctctgcgggactgtatttcagaaaacacactggtggggctacctctccattcacatgtactgccctagcctctccccatccccggctgatgcacttccatatctgcactgttccataacagcagtagcatgttgcagaaagcgctaggattcctccactccatcttcaaagaaaaagtcgctaataaatcacatttggtaggttagtgaacgttaaacacattagtgagcaaaagaaaataggaatgaacaagaattggtcatctacctaactgaacacaaatgaactctggcagttcggtaataggaggtaaagaaccgcgctaattgcagaacagcagcccccctaccttcccaggagcagtgtgactgggaagcagccccgtgtgtatgctggtgcaggttctaagcaaagtgagctgcccatcagttctgatgagtttgctgatgctagacatatgacatctgttctcttgctgcctgccccagttatctcccaaagttctttactgagaatgaaaagcatctttctctgtgtggtgacttcagtaggccaacaaatatttgagtttaaagcacaagactaaatagtcataggcagagcagtgctaccatttacaatttgcttacttgatgctaaaccatgggttaggcattttacagtcatatcatctagcccagcaagtcatggaagcatagttgttaaaatcatctgatactttgggaggctggggcgggcagatcacgaggtcaggagatcgagaccatcctggctaacatggtgaaaccctgtctctactaaaaatacaaaaaaattagccacgggtggtggcaggagcctgtagtcccagctactcaggaagctgaggcaggagaatggcgtcaacccgggaggtggagcttgcagtaagccgagatcatgccactgcactccagcccgggcaagagagtgagacttcgtctaaaaaaaaaaaaatcatcatctgacagataaggatacagggcttgaagaacataggtgacctgccccaagtgtccaaagccacacatccaaaatgacaaattagggttttaagccagcactcttagacttcaaagcctcttaaccattccactgccctgctgtagggcatagggagataagggggataagctatggttgccatcaaagagttaatatatcaataatatgcggatggtgaggatgatggcagctgctaggggtctacaggcgtgtaccaccatgcccagctacaattcttattattcccaaatgctactgtgtccggaattggtgggttcttggtcttactgacttcaagaatgaagccgcggaacctcgcggtgagtgttacagctcttaaggtggtgcgtctggagtctgtccgttctgatgttgagatgtgttcggagtttcttccttctggtgggttcgtggtctcgctggctcaggagtgaagctgcagaccttcacggcaagtgttacagctcttaaggcagcgcgtctggagttgtttgttcctcccggtgggctcgtggtctcgctgggctcaggagtgaagctgcagatcttcgcggtgagtgttacagctcataaaagcagcgtggacctggcagccctcggaccttgctcctgcccaagcccctgccgttgggccccggtgttgggttcggttgtgctgtctaacggctgcctggccccctcccccctcccctgtacaggaagtgtctgttggcggctaggtcccccaccagatggctcatgctgtggccactctaggagcagctggaggtggaaactcgttggtattaaccctgtgctggagggcccttaatgggttttttgatgcaattggaacaagatttatttattttttatacggggcttagataacatttctctttggtttagcaatatttattttcatttggaaaatttttagcacctatttttattagtttttagaataaagaaagtcaaacatcattttatgtttgataatgtttcctgtatgattttataagagata

SEQ ID NO: 15066 - RNA, 3808 nt, Homo sapiens
  source 1..3808: mol_type = other RNA
gctgggattacaggcatgagccactgcacccggccctgtctgccctttcttgagcctctggtcccagcaagtttggttgtagtttgatgtgtattaactcttaattctcataataaccctgaaaggtaagtgtgtttgttatttattgctacatcacaaatatctcaaattgagcaaacatttatgatctcatgtgatttctgagggccaggaacctataagcagcttaggtgggtggctctggctcaaggtctctcatgaggttgccgtcaggatgttggccaggactgcagtcatgtaaaagcctgaccagggaggggccattggcttccaaggtgaccccttacacggctgttggcaggaggcctgttcctcattggctgtcggcagggggatcctctgttcctcgccatcggacctctccatggtgctgcttgagtgtcctcatgacatggcggctggcttgcctcagagtaactcttgaagaatgtgctagaaggtgagcacctggattcaaagtaattaactggcatcatctgtccaagagatgggatggataagaagttaagcttccaggagatgcctcatcatttgtgccagtgaccccgcataatttcttgatgaattgtgcaaactgggaagctgatagctcgtttcagattctctagattttgcccctgaaaaagcatttacgtgatgcagtccgaggtcttgtatggaggagcttggtgtggggagatgtgtggctcacgaactgtcttgtgcatgtgtctccccaggggcattttcagatttctgccacggagatgctcttcgcaaagggagagtcaggtacattggaggattcattgctgtgaccagggaaagcagaggacatgcaaaattaatatttccctttctatcttctaggatggacttttttcattcagaaagccgctctggcttaaagacatgtacaaacctctcagtgccacaagagtaaagaatcacgcatggaagctgcacaagaagtcatctaatgaggacaagatcctcaacagggaccctgggtaaatgacgggaccctcacagttcccatctaaaatgaggagggggtgagacgcttaattgctcctttcaagaatgaaaaccttggcattgttattcttatcccagggacagtgaagccccaacagagaaggaggaggagagtgaagccctgccataggaggagaacccagcccacctcaggcctcctgcaaaaacacatagcataaacaataccatcagaaagaaaagcaggactgaagccagcagcccacacatccacagaggcagcgggcagagcaagcacagggccatcgttcctgcccttgtttcccagtctaattagtcacccagacctgaaaacatatcctcagggggtggagattttacaattaaataccattgtttttggtgccctctccctgggttcatcaagcaccagtcatataataccacatacttgaactcctgcccacaggggacctcccatctcctggcccctattataggatcactgggcctacctgcactgtggggccaagccctgtctttttcccaagccctcaagcacacgcatgaatgttcatcccgacttggtagggggcttttcacccttacaagatggcaaaagattcacactgctttttttaaaatttgtttttctttttaaaaatcccaacccttggatagcaagggaggtgctggaggggtagggtcaagaagagtgtgtgagaacagtaatttcccaagactgccctctgcgggactgtatttcagaaaacacactggtggggctacctctccattcacatgtactgccctagcctctccccatccccggctgatgcacttccatatctgcactgttccataacagcagtagcatgttgcagaaagcgctaggattcctccactccatcttcaaagaaaaagtcgctaataaatcacatttggtaggttagtgaacgttaaacacattagtgagcaaaagaaaataggaatgaacaagaattggtcatctacctaactgaacacaaatgaactctggcagttcggtaataggaggtaaagaaccgcgctaattgcagaacagcagcccccctaccttcccaggagcagtgtgactgggaagcagccccgtgtgtatgctggtgcaggttctaagcaaagtgagctgcccatcagttctgatgagtttgctgatgctagacatatgacatctgttctcttgctgcctgccccagttatctcccaaagttctttactgagaatgaaaagcatctttctctgtgtggtgacttcagtaggccaacaaatatttgagtttaaagcacaagactaaatagtcataggcagagcagtgctaccatttacaatttgcttacttgatgctaaaccatgggttaggcattttacagtcatatcatctagcccagcaagtcatggaagcatagttgttaaaatcatctgatactttgggaggctggggcgggcagatcacgaggtcaggagatcgagaccatcctggctaacatggtgaaaccctgtctctactaaaaatacaaaaaaattagccacgggtggtggcaggagcctgtagtcccagctactcaggaagctgaggcaggagaatggcgtcaacccgggaggtggagcttgcagtaagccgagatcatgccactgcactccagcccgggcaagagagtgagacttcgtctaaaaaaaaaaaaatcatcatctgacagataaggatacagggcttgaagaacataggtgacctgccccaagtgtccaaagccacacatccaaaatgacaaattagggttttaagccagcactcttagacttcaaagcctcttaaccattccactgccctgctgtagggcatagggagataagggggataagctatggttgccatcaaagagttaatatatcaataatatgcggatggtgaggatgatggcagctgctaggggtctacaggcgtgtaccaccatgcccagctacaattcttattattcccaaatgctactgtgtccggaattggtgggttcttggtcttactgacttcaagaatgaagccgcggaacctcgcggtgagtgttacagctcttaaggtggtgcgtctggagtctgtccgttctgatgttgagatgtgttcggagtttcttccttctggtgggttcgtggtctcgctggctcaggagtgaagctgcagaccttcacggcaagtgttacagctcttaaggcagcgcgtctggagttgtttgttcctcccggtgggctcgtggtctcgctgggctcaggagtgaagctgcagatcttcgcggtgagtgttacagctcataaaagcagcgtggacctggcagccctcggaccttgctcctgcccaagcccctgccgttgggccccggtgttgggttcggttgtgctgtctaacggctgcctggccccctcccccctcccctgtacaggaagtgtctgttggcggctaggtcccccaccagatggctcatgctgtggccactctaggagcagctggaggtggaaactcgttggtattaaccctgtgctggagggcccttaatgggttttttgatgcaattggaacaagatttatttattttttatacggggcttagataacatttctctttggtttagcaatatttattttcatttggaaaatttttagcacctatttttattagtttttagaataaagaaagtcaaacatcattttatgtttgataatgtttcctgtatgattttataagag

SEQ ID NO: 15067 - RNA, 3973 nt, Homo sapiens
  source 1..3973: mol_type = other RNA
gctgggattacaggcatgagccactgcacccggccctgtctgccctttcttgagcctctggtcccagcaagtttggttgtagtttgatgtgtattaactcttaattctcataataaccctgaaaggtaagtgtgtttgttatttattgctacatcacaaatatctcaaattgagcaaacatttatgatctcatgtgatttctgagggccaggaacctataagcagcttaggtgggtggctctggctcaaggtctctcatgaggttgccgtcaggatgttggccaggactgcagtcatgtaaaagcctgaccagggaggggccattggcttccaaggtgaccccttacacggctgttggcaggaggcctgttcctcattggctgtcggcagggggatcctctgttcctcgccatcggacctctccatggtgctgcttgagtgtcctcatgacatggcggctggcttgcctcagagtaactcttgaagaatgtgctagaaggtgagcacctggcaggatgcttcgaccttgttctgatgcctggggacttctggtgagttccctggccatccatcctggtctgttcaccttctcaggactccagttgagttgggctgcgtgtgacagaccccttggggaaaacgccgcagctgcaggtgccaccagtgagtcttctattcaaagtaattaactggcatcatctgtccaagagatgggatggataagaagttaagcttccaggagatgcctcatcatttgtgccagtgaccccgcataatttcttgatgaattgtgcaaactgggaagctgatagctcgtttcagattctctagattttgcccctgaaaaagcatttacgtgatgcagtccgaggtcttgtatggaggagcttggtgtggggagatgtgtggctcacgaactgtcttgtgcatgtgtctccccaggggcattttcagatttctgccacggagatgctcttcgcaaagggagagtcaggtacattggaggattcattgctgtgaccagggaaagcagaggacatgcaaaattaatatttccctttctatcttctaggatggacttttttcattcagaaagccgctctggcttaaagacatgtacaaacctctcagtgccacaagagtaaagaatcacgcatggaagctgcacaagaagtcatctaatgaggacaagatcctcaacagggaccctgggtaaatgacgggaccctcacagttcccatctaaaatgaggagggggtgagacgcttaattgctcctttcaagaatgaaaaccttggcattgttattcttatcccagggacagtgaagccccaacagagaaggaggaggagagtgaagccctgccataggaggagaacccagcccacctcaggcctcctgcaaaaacacatagcataaacaataccatcagaaagaaaagcaggactgaagccagcagcccacacatccacagaggcagcgggcagagcaagcacagggccatcgttcctgcccttgtttcccagtctaattagtcacccagacctgaaaacatatcctcagggggtggagattttacaattaaataccattgtttttggtgccctctccctgggttcatcaagcaccagtcatataataccacatacttgaactcctgcccacaggggacctcccatctcctggcccctattataggatcactgggcctacctgcactgtggggccaagccctgtctttttcccaagccctcaagcacacgcatgaatgttcatcccgacttggtagggggcttttcacccttacaagatggcaaaagattcacactgctttttttaaaatttgtttttctttttaaaaatcccaacccttggatagcaagggaggtgctggaggggtagggtcaagaagagtgtgtgagaacagtaatttcccaagactgccctctgcgggactgtatttcagaaaacacactggtggggctacctctccattcacatgtactgccctagcctctccccatccccggctgatgcacttccatatctgcactgttccataacagcagtagcatgttgcagaaagcgctaggattcctccactccatcttcaaagaaaaagtcgctaataaatcacatttggtaggttagtgaacgttaaacacattagtgagcaaaagaaaataggaatgaacaagaattggtcatctacctaactgaacacaaatgaactctggcagttcggtaataggaggtaaagaaccgcgctaattgcagaacagcagcccccctaccttcccaggagcagtgtgactgggaagcagccccgtgtgtatgctggtgcaggttctaagcaaagtgagctgcccatcagttctgatgagtttgctgatgctagacatatgacatctgttctcttgctgcctgccccagttatctcccaaagttctttactgagaatgaaaagcatctttctctgtgtggtgacttcagtaggccaacaaatatttgagtttaaagcacaagactaaatagtcataggcagagcagtgctaccatttacaatttgcttacttgatgctaaaccatgggttaggcattttacagtcatatcatctagcccagcaagtcatggaagcatagttgttaaaatcatctgatactttgggaggctggggcgggcagatcacgaggtcaggagatcgagaccatcctggctaacatggtgaaaccctgtctctactaaaaatacaaaaaaattagccacgggtggtggcaggagcctgtagtcccagctactcaggaagctgaggcaggagaatggcgtcaacccgggaggtggagcttgcagtaagccgagatcatgccactgcactccagcccgggcaagagagtgagacttcgtctaaaaaaaaaaaaatcatcatctgacagataaggatacagggcttgaagaacataggtgacctgccccaagtgtccaaagccacacatccaaaatgacaaattagggttttaagccagcactcttagacttcaaagcctcttaaccattccactgccctgctgtagggcatagggagataagggggataagctatggttgccatcaaagagttaatatatcaataatatgcggatggtgaggatgatggcagctgctaggggtctacaggcgtgtaccaccatgcccagctacaattcttattattcccaaatgctactgtgtccggaattggtgggttcttggtcttactgacttcaagaatgaagccgcggaacctcgcggtgagtgttacagctcttaaggtggtgcgtctggagtctgtccgttctgatgttgagatgtgttcggagtttcttccttctggtgggttcgtggtctcgctggctcaggagtgaagctgcagaccttcacggcaagtgttacagctcttaaggcagcgcgtctggagttgtttgttcctcccggtgggctcgtggtctcgctgggctcaggagtgaagctgcagatcttcgcggtgagtgttacagctcataaaagcagcgtggacctggcagccctcggaccttgctcctgcccaagcccctgccgttgggccccggtgttgggttcggttgtgctgtctaacggctgcctggccccctcccccctcccctgtacaggaagtgtctgttggcggctaggtcccccaccagatggctcatgctgtggccactctaggagcagctggaggtggaaactcgttggtattaaccctgtgctggagggcccttaatgggttttttgatgcaattggaacaagatttatttattttttatacggggcttagataacatttctctttggtttagcaatatttattttcatttggaaaatttttagcacctatttttattagtttttagaataaagaaagtcaaacatcattttatgtttgataatgtttcctgtatgattttataagagat

SEQ ID NO: 15068 - RNA, 1745 nt, Homo sapiens
  source 1..1745: mol_type = other RNA
gctgggattacaggcatgagccactgcacccggccctgtctgccctttcttgagcctctggtcccagcaagtttggttgtagtttgatgtgtattaactcttaattctcataataaccctgaaaggtaagtgtgtttgttatttattgctacatcacaaatatctcaaattgagcaaacatttatgatctcatgtgatttctgagggccaggaacctataagcagcttaggtgggtggctctggctcaaggtctctcatgaggttgccgtcaggatgttggccaggactgcagtcatgtaaaagcctgaccagggaggggccattggcttccaaggtgaccccttacacggctgttggcaggaggcctgttcctcattggctgtcggcagggggatcctctgttcctcgccatcggacctctccatggtgctgcttgagtgtcctcatgacatggcggctggcttgcctcagagtaactcttgaagaatgtgctagaaggtgagcacctggcaggatgcttcgaccttgttctgatgcctggggacttctggtgagttccctggccatccatcctggtctgttcaccttctcaggactccagttgagttgggctgcgtgtgacagaccccttggggaaaacgccgcagctgcaggtgccaccagtgagtcttctattcaaagtaattaactggcatcatctgtccaagagatgggatggataagaagttaagcttccaggagatgcctcatcatttgtgccagtgaccccgcataatttcttgatgaattgtgcaaactgggaagctgatagctcgtttcagattctctagattttgcccctgaaaaagcatttacgtgatgcagtccgaggtcttgtatggaggagcttggtgtggggagatgtgtggctcacgaactgtcttgtgcatgtgtctccccaggggcattttcagatttctgccacggagatgctcttcgcaaagggagagtcaggtacattggaggattcattgttcaagaatgaagccgcggaacctcgcggtgagtgttacagctcttaaggtggtgcgtctggagtctgtccgttctgatgttgagatgtgttcggagtttcttccttctggtgggttcgtggtctcgctggctcaggagtgaagctgcagaccttcacggcaagtgttacagctcttaaggcagcgcgtctggagttgtttgttcctcccggtgggctcgtggtctcgctgggctcaggagtgaagctgcagatcttcgcggtgagtgttacagctcataaaagcagcgtggacctggcagccctcggaccttgctcctgcccaagcccctgccgttgggccccggtgttgggttcggttgtgctgtctaacggctgcctggccccctcccccctcccctgtacaggaagtgtctgttggcggctaggtcccccaccagatggctcatgctgtggccactctaggagcagctggaggtggaaactcgttggtattaaccctgtgctggagggcccttaatgggttttttgatgcaattggaacaagatttatttattttttatacggggcttagataacatttctctttggtttagcaatatttattttcatttggaaaatttttagcacctatttttattagtttttagaataaagaaagtcaaacatcattttatgtttgataatgtttcctgtatgattttataagagataagttaaattttaccttt

SEQ ID NO: 15069 - RNA, 3970 nt, Homo sapiens
  source 1..3970: mol_type = other RNA
gctgggattacaggcatgagccactgcacccggccctgtctgccctttcttgagcctctggtcccagcaagtttggttgtagtttgatgtgtattaactcttaattctcataataaccctgaaaggtaagtgtgtttgttatttattgctacatcacaaatatctcaaattgagcaaacatttatgatctcatgtgatttctgagggccaggaacctataagcagcttaggtgggtggctctggctcaaggtctctcatgaggttgccgtcaggatgttggccaggactgcagtcatgtaaaagcctgaccagggaggggccattggcttccaaggtgaccccttacacggctgttggcaggaggcctgttcctcattggctgtcggcagggggatcctctgttcctcgccatcggacctctccatggtgctgcttgagtgtcctcatgacatggcggctggcttgcctcagagtaactcttgaagaatgtgctagaaggtgagcacctggcttcaataaagctttatttacaagaacaggtagtgggccagatgggccctcctctgtcttcttctgctctatgcttcttgtgggcttgaagacagtgaggagccaaaggtctgtacctcgtctaccccaaaagtactgcctgggcctctggtaccctaatattcaaagtaattaactggcatcatctgtccaagagatgggatggataagaagttaagcttccaggagatgcctcatcatttgtgccagtgaccccgcataatttcttgatgaattgtgcaaactgggaagctgatagctcgtttcagattctctagattttgcccctgaaaaagcatttacgtgatgcagtccgaggtcttgtatggaggagcttggtgtggggagatgtgtggctcacgaactgtcttgtgcatgtgtctccccaggggcattttcagatttctgccacggagatgctcttcgcaaagggagagtcaggtacattggaggattcattgctgtgaccagggaaagcagaggacatgcaaaattaatatttccctttctatcttctaggatggacttttttcattcagaaagccgctctggcttaaagacatgtacaaacctctcagtgccacaagagtaaagaatcacgcatggaagctgcacaagaagtcatctaatgaggacaagatcctcaacagggaccctgggtaaatgacgggaccctcacagttcccatctaaaatgaggagggggtgagacgcttaattgctcctttcaagaatgaaaaccttggcattgttattcttatcccagggacagtgaagccccaacagagaaggaggaggagagtgaagccctgccataggaggagaacccagcccacctcaggcctcctgcaaaaacacatagcataaacaataccatcagaaagaaaagcaggactgaagccagcagcccacacatccacagaggcagcgggcagagcaagcacagggccatcgttcctgcccttgtttcccagtctaattagtcacccagacctgaaaacatatcctcagggggtggagattttacaattaaataccattgtttttggtgccctctccctgggttcatcaagcaccagtcatataataccacatacttgaactcctgcccacaggggacctcccatctcctggcccctattataggatcactgggcctacctgcactgtggggccaagccctgtctttttcccaagccctcaagcacacgcatgaatgttcatcccgacttggtagggggcttttcacccttacaagatggcaaaagattcacactgctttttttaaaatttgtttttctttttaaaaatcccaacccttggatagcaagggaggtgctggaggggtagggtcaagaagagtgtgtgagaacagtaatttcccaagactgccctctgcgggactgtatttcagaaaacacactggtggggctacctctccattcacatgtactgccctagcctctccccatccccggctgatgcacttccatatctgcactgttccataacagcagtagcatgttgcagaaagcgctaggattcctccactccatcttcaaagaaaaagtcgctaataaatcacatttggtaggttagtgaacgttaaacacattagtgagcaaaagaaaataggaatgaacaagaattggtcatctacctaactgaacacaaatgaactctggcagttcggtaataggaggtaaagaaccgcgctaattgcagaacagcagcccccctaccttcccaggagcagtgtgactgggaagcagccccgtgtgtatgctggtgcaggttctaagcaaagtgagctgcccatcagttctgatgagtttgctgatgctagacatatgacatctgttctcttgctgcctgccccagttatctcccaaagttctttactgagaatgaaaagcatctttctctgtgtggtgacttcagtaggccaacaaatatttgagtttaaagcacaagactaaatagtcataggcagagcagtgctaccatttacaatttgcttacttgatgctaaaccatgggttaggcattttacagtcatatcatctagcccagcaagtcatggaagcatagttgttaaaatcatctgatactttgggaggctggggcgggcagatcacgaggtcaggagatcgagaccatcctggctaacatggtgaaaccctgtctctactaaaaatacaaaaaaattagccacgggtggtggcaggagcctgtagtcccagctactcaggaagctgaggcaggagaatggcgtcaacccgggaggtggagcttgcagtaagccgagatcatgccactgcactccagcccgggcaagagagtgagacttcgtctaaaaaaaaaaaaatcatcatctgacagataaggatacagggcttgaagaacataggtgacctgccccaagtgtccaaagccacacatccaaaatgacaaattagggttttaagccagcactcttagacttcaaagcctcttaaccattccactgccctgctgtagggcatagggagataagggggataagctatggttgccatcaaagagttaatatatcaataatatgcggatggtgaggatgatggcagctgctaggggtctacaggcgtgtaccaccatgcccagctacaattcttattattcccaaatgctactgtgtccggaattggtgggttcttggtcttactgacttcaagaatgaagccgcggaacctcgcggtgagtgttacagctcttaaggtggtgcgtctggagtctgtccgttctgatgttgagatgtgttcggagtttcttccttctggtgggttcgtggtctcgctggctcaggagtgaagctgcagaccttcacggcaagtgttacagctcttaaggcagcgcgtctggagttgtttgttcctcccggtgggctcgtggtctcgctgggctcaggagtgaagctgcagatcttcgcggtgagtgttacagctcataaaagcagcgtggacctggcagccctcggaccttgctcctgcccaagcccctgccgttgggccccggtgttgggttcggttgtgctgtctaacggctgcctggccccctcccccctcccctgtacaggaagtgtctgttggcggctaggtcccccaccagatggctcatgctgtggccactctaggagcagctggaggtggaaactcgttggtattaaccctgtgctggagggcccttaatgggttttttgatgcaattggaacaagatttatttattttttatacggggcttagataacatttctctttggtttagcaatatttattttcatttggaaaatttttagcacctatttttattagtttttagaataaagaaagtcaaacatcattttatgtttgataatgtttcctgtatgattttataagagat

SEQ ID NO: 15070 - RNA, 4089 nt, Homo sapiens
  source 1..4089: mol_type = other RNA
gctgggattacaggcatgagccactgcacccggccctgtctgccctttcttgagcctctggtcccagcaagtttggttgtagtttgatgtgtattaactcttaattctcataataaccctgaaaggtaagtgtgtttgttatttattgctacatcacaaatatctcaaattgagcaaacatttatgatctcatgtgatttctgagggccaggaacctataagcagcttaggtgggtggctctggctcaaggtctctcatgaggttgccgtcaggatgttggccaggactgcagtcatgtaaaagcctgaccagggaggggccattggcttccaaggtgaccccttacacggctgttggcaggaggcctgttcctcattggctgtcggcagggggatcctctgttcctcgccatcggacctctccatggtgctgcttgagtgtcctcatgacatggcggctggcttgcctcagagtaactcttgaagaatgtgctagaaggtgagcacctggcttcaataaagctttatttacaagaacaggtagtgggccagatgggccctcctctgtcttcttctgctctatgcttcttgtgggcttgaagacagtgaggagccaaaggtctgtacctcgtctaccccaaaagtactgcctgggcctctggtaccctaatcaggatgcttcgaccttgttctgatgcctggggacttctggtgagttccctggccatccatcctggtctgttcaccttctcaggactccagttgagttgggctgcgtgtgacagacccattcaaagtaattaactggcatcatctgtccaagagatgggatggataagaagttaagcttccaggagatgcctcatcatttgtgccagtgaccccgcataatttcttgatgaattgtgcaaactgggaagctgatagctcgtttcagattctctagattttgcccctgaaaaagcatttacgtgatgcagtccgaggtcttgtatggaggagcttggtgtggggagatgtgtggctcacgaactgtcttgtgcatgtgtctccccaggggcattttcagatttctgccacggagatgctcttcgcaaagggagagtcaggtacattggaggattcattgctgtgaccagggaaagcagaggacatgcaaaattaatatttccctttctatcttctaggatggacttttttcattcagaaagccgctctggcttaaagacatgtacaaacctctcagtgccacaagagtaaagaatcacgcatggaagctgcacaagaagtcatctaatgaggacaagatcctcaacagggaccctgggtaaatgacgggaccctcacagttcccatctaaaatgaggagggggtgagacgcttaattgctcctttcaagaatgaaaaccttggcattgttattcttatcccagggacagtgaagccccaacagagaaggaggaggagagtgaagccctgccataggaggagaacccagcccacctcaggcctcctgcaaaaacacatagcataaacaataccatcagaaagaaaagcaggactgaagccagcagcccacacatccacagaggcagcgggcagagcaagcacagggccatcgttcctgcccttgtttcccagtctaattagtcacccagacctgaaaacatatcctcagggggtggagattttacaattaaataccattgtttttggtgccctctccctgggttcatcaagcaccagtcatataataccacatacttgaactcctgcccacaggggacctcccatctcctggcccctattataggatcactgggcctacctgcactgtggggccaagccctgtctttttcccaagccctcaagcacacgcatgaatgttcatcccgacttggtagggggcttttcacccttacaagatggcaaaagattcacactgctttttttaaaatttgtttttctttttaaaaatcccaacccttggatagcaagggaggtgctggaggggtagggtcaagaagagtgtgtgagaacagtaatttcccaagactgccctctgcgggactgtatttcagaaaacacactggtggggctacctctccattcacatgtactgccctagcctctccccatccccggctgatgcacttccatatctgcactgttccataacagcagtagcatgttgcagaaagcgctaggattcctccactccatcttcaaagaaaaagtcgctaataaatcacatttggtaggttagtgaacgttaaacacattagtgagcaaaagaaaataggaatgaacaagaattggtcatctacctaactgaacacaaatgaactctggcagttcggtaataggaggtaaagaaccgcgctaattgcagaacagcagcccccctaccttcccaggagcagtgtgactgggaagcagccccgtgtgtatgctggtgcaggttctaagcaaagtgagctgcccatcagttctgatgagtttgctgatgctagacatatgacatctgttctcttgctgcctgccccagttatctcccaaagttctttactgagaatgaaaagcatctttctctgtgtggtgacttcagtaggccaacaaatatttgagtttaaagcacaagactaaatagtcataggcagagcagtgctaccatttacaatttgcttacttgatgctaaaccatgggttaggcattttacagtcatatcatctagcccagcaagtcatggaagcatagttgttaaaatcatctgatactttgggaggctggggcgggcagatcacgaggtcaggagatcgagaccatcctggctaacatggtgaaaccctgtctctactaaaaatacaaaaaaattagccacgggtggtggcaggagcctgtagtcccagctactcaggaagctgaggcaggagaatggcgtcaacccgggaggtggagcttgcagtaagccgagatcatgccactgcactccagcccgggcaagagagtgagacttcgtctaaaaaaaaaaaaatcatcatctgacagataaggatacagggcttgaagaacataggtgacctgccccaagtgtccaaagccacacatccaaaatgacaaattagggttttaagccagcactcttagacttcaaagcctcttaaccattccactgccctgctgtagggcatagggagataagggggataagctatggttgccatcaaagagttaatatatcaataatatgcggatggtgaggatgatggcagctgctaggggtctacaggcgtgtaccaccatgcccagctacaattcttattattcccaaatgctactgtgtccggaattggtgggttcttggtcttactgacttcaagaatgaagccgcggaacctcgcggtgagtgttacagctcttaaggtggtgcgtctggagtctgtccgttctgatgttgagatgtgttcggagtttcttccttctggtgggttcgtggtctcgctggctcaggagtgaagctgcagaccttcacggcaagtgttacagctcttaaggcagcgcgtctggagttgtttgttcctcccggtgggctcgtggtctcgctgggctcaggagtgaagctgcagatcttcgcggtgagtgttacagctcataaaagcagcgtggacctggcagccctcggaccttgctcctgcccaagcccctgccgttgggccccggtgttgggttcggttgtgctgtctaacggctgcctggccccctcccccctcccctgtacaggaagtgtctgttggcggctaggtcccccaccagatggctcatgctgtggccactctaggagcagctggaggtggaaactcgttggtattaaccctgtgctggagggcccttaatgggttttttgatgcaattggaacaagatttatttattttttatacggggcttagataacatttctctttggtttagcaatatttattttcatttggaaaatttttagcacctatttttattagtttttagaataaagaaagtcaaacatcattttatgtttgataatgtttcctgtatgattttataagagata

SEQ ID NO: 15071 - RNA, 1205 nt, Homo sapiens
  source 1..1205: mol_type = other RNA
gctgggattacaggcatgagccactgcacccggccctgtctgccctttcttgagcctctggtcccagcaagtttggttgtagtttgatgtgtattaactcttaattctcataataaccctgaaaggtaagtgtgtttgttatttattgctacatcacaaatatctcaaattgagcaaacatttatgatctcatgtgatttctgagggccaggaacctataagcagcttaggtgggtggctctggctcaaggtctctcatgaggttgccgtcaggatgttggccaggactgcagtcatgtaaaagcctgaccagggaggggccattggcttccaaggtgaccccttacacggctgttggcaggaggcctgttcctcattggctgtcggcagggggatcctctgttcctcgccatcggacctctccatggtgctgcttgagtgtcctcatgacatggcggctggcttgcctcagagtaactcttgaagaatgtgctagaaggtgagcacctggcttcaataaagctttatttacaagaacaggtagtgggccagatgggccctcctctgtcttcttctgctctatgcttcttgtgggcttgaagacagtgaggagccaaaggtctgtacctcgtctaccccaaaagtactgcctgggcctctggtaccctaatcaggatgcttcgaccttgttctgatgcctggggacttctggtgagttccctggccatccatcctggtctgttcaccttctcaggactccagttgagttgggctgcgtgtgacagacccattcaaagtaattaactggcatcatctgtccaagagatgggatggataagaagttaagcttccaggagatgcctcatcatttgtgccagtgaccccgcataatttcttgatgaattgtgcaaactgggaagctgatagctcgtttcagattctctagattttgcccctgaaaaagcatttacgtgatgcagtccgaggtcttgtatggaggagcttggtgtggggagatgtgtggctcacgaactgtcttgtgcatgtgtctccccaggggcattttcagatttctgccacggagatgctcttcgcaaagggagagtcaggtacattggaggattcattgttcaagaatgaagccgcggaacctcgcggtgagtgttacagctcttaaggtggtgcgtctggagtctgtccgttct

SEQ ID NO: 15072 - RNA, 4189 nt, Homo sapiens
  source 1..4189: mol_type = other RNA
gctgggattacaggcatgagccactgcacccggccctgtctgccctttcttgagcctctggtcccagcaagtttggttgtagtttgatgtgtattaactcttaattctcataataaccctgaaaggtaagtgtgtttgttatttattgctacatcacaaatatctcaaattgagcaaacatttatgatctcatgtgatttctgagggccaggaacctataagcagcttaggtgggtggctctggctcaaggtctctcatgaggttgccgtcaggatgttggccaggactgcagtcatgtaaaagcctgaccagggaggggccattggcttccaaggtgaccccttacacggctgttggcaggaggcctgttcctcattggctgtcggcagggggatcctctgttcctcgccatcggacctctccatggtgctgcttgagtgtcctcatgacatggcggctggcttgcctcagagtaactcttgaagaatgtgctagaaggtgagcacctggcttcaataaagctttatttacaagaacaggtagtgggccagatgggccctcctctgtcttcttctgctctatgcttcttgtgggcttgaagacagtgaggagccaaaggtctgtacctcgtctaccccaaaagtactgcctgggcctctggtaccctaatcaggatgcttcgaccttgttctgatgcctggggacttctggtgagttccctggccatccatcctggtctgttcaccttctcaggactccagttgagttgggctgcgtgtgacagacccctgagtcgctgctgtcctctagtggccactggataaattgcacagcacgccggccttggggaaaacgccgcagctgcaggtgccaccagtgagtcttctattcaaagtaattaactggcatcatctgtccaagagatgggatggataagaagttaagcttccaggagatgcctcatcatttgtgccagtgaccccgcataatttcttgatgaattgtgcaaactgggaagctgatagctcgtttcagattctctagattttgcccctgaaaaagcatttacgtgatgcagtccgaggtcttgtatggaggagcttggtgtggggagatgtgtggctcacgaactgtcttgtgcatgtgtctccccaggggcattttcagatttctgccacggagatgctcttcgcaaagggagagtcaggtacattggaggattcattgctgtgaccagggaaagcagaggacatgcaaaattaatatttccctttctatcttctaggatggacttttttcattcagaaagccgctctggcttaaagacatgtacaaacctctcagtgccacaagagtaaagaatcacgcatggaagctgcacaagaagtcatctaatgaggacaagatcctcaacagggaccctgggtaaatgacgggaccctcacagttcccatctaaaatgaggagggggtgagacgcttaattgctcctttcaagaatgaaaaccttggcattgttattcttatcccagggacagtgaagccccaacagagaaggaggaggagagtgaagccctgccataggaggagaacccagcccacctcaggcctcctgcaaaaacacatagcataaacaataccatcagaaagaaaagcaggactgaagccagcagcccacacatccacagaggcagcgggcagagcaagcacagggccatcgttcctgcccttgtttcccagtctaattagtcacccagacctgaaaacatatcctcagggggtggagattttacaattaaataccattgtttttggtgccctctccctgggttcatcaagcaccagtcatataataccacatacttgaactcctgcccacaggggacctcccatctcctggcccctattataggatcactgggcctacctgcactgtggggccaagccctgtctttttcccaagccctcaagcacacgcatgaatgttcatcccgacttggtagggggcttttcacccttacaagatggcaaaagattcacactgctttttttaaaatttgtttttctttttaaaaatcccaacccttggatagcaagggaggtgctggaggggtagggtcaagaagagtgtgtgagaacagtaatttcccaagactgccctctgcgggactgtatttcagaaaacacactggtggggctacctctccattcacatgtactgccctagcctctccccatccccggctgatgcacttccatatctgcactgttccataacagcagtagcatgttgcagaaagcgctaggattcctccactccatcttcaaagaaaaagtcgctaataaatcacatttggtaggttagtgaacgttaaacacattagtgagcaaaagaaaataggaatgaacaagaattggtcatctacctaactgaacacaaatgaactctggcagttcggtaataggaggtaaagaaccgcgctaattgcagaacagcagcccccctaccttcccaggagcagtgtgactgggaagcagccccgtgtgtatgctggtgcaggttctaagcaaagtgagctgcccatcagttctgatgagtttgctgatgctagacatatgacatctgttctcttgctgcctgccccagttatctcccaaagttctttactgagaatgaaaagcatctttctctgtgtggtgacttcagtaggccaacaaatatttgagtttaaagcacaagactaaatagtcataggcagagcagtgctaccatttacaatttgcttacttgatgctaaaccatgggttaggcattttacagtcatatcatctagcccagcaagtcatggaagcatagttgttaaaatcatctgatactttgggaggctggggcgggcagatcacgaggtcaggagatcgagaccatcctggctaacatggtgaaaccctgtctctactaaaaatacaaaaaaattagccacgggtggtggcaggagcctgtagtcccagctactcaggaagctgaggcaggagaatggcgtcaacccgggaggtggagcttgcagtaagccgagatcatgccactgcactccagcccgggcaagagagtgagacttcgtctaaaaaaaaaaaaatcatcatctgacagataaggatacagggcttgaagaacataggtgacctgccccaagtgtccaaagccacacatccaaaatgacaaattagggttttaagccagcactcttagacttcaaagcctcttaaccattccactgccctgctgtagggcatagggagataagggggataagctatggttgccatcaaagagttaatatatcaataatatgcggatggtgaggatgatggcagctgctaggggtctacaggcgtgtaccaccatgcccagctacaattcttattattcccaaatgctactgtgtccggaattggtgggttcttggtcttactgacttcaagaatgaagccgcggaacctcgcggtgagtgttacagctcttaaggtggtgcgtctggagtctgtccgttctgatgttgagatgtgttcggagtttcttccttctggtgggttcgtggtctcgctggctcaggagtgaagctgcagaccttcacggcaagtgttacagctcttaaggcagcgcgtctggagttgtttgttcctcccggtgggctcgtggtctcgctgggctcaggagtgaagctgcagatcttcgcggtgagtgttacagctcataaaagcagcgtggacctggcagccctcggaccttgctcctgcccaagcccctgccgttgggccccggtgttgggttcggttgtgctgtctaacggctgcctggccccctcccccctcccctgtacaggaagtgtctgttggcggctaggtcccccaccagatggctcatgctgtggccactctaggagcagctggaggtggaaactcgttggtattaaccctgtgctggagggcccttaatgggttttttgatgcaattggaacaagatttatttattttttatacggggcttagataacatttctctttggtttagcaatatttattttcatttggaaaatttttagcacctatttttattagtttttagaataaagaaagtcaaacatcattttatgtttgataatgtttcctgtatgattttataagagataa

SEQ ID NO: 15073 - RNA, 4345 nt, Homo sapiens
  source 1..4345: mol_type = other RNA
gctgggattacaggcatgagccactgcacccggccctgtctgccctttcttgagcctctggtcccagcaagtttggttgtagtttgatgtgtattaactcttaattctcataataaccctgaaaggtaagtgtgtttgttatttattgctacatcacaaatatctcaaattgagcaaacatttatgatctcatgtgatttctgagggccaggaacctataagcagcttaggtgggtggctctggctcaaggtctctcatgaggttgccgtcaggatgttggccaggactgcagtcatgtaaaagcctgaccagggaggggccattggcttccaaggtgaccccttacacggctgttggcaggaggcctgttcctcattggctgtcggcagggggatcctctgttcctcgccatcggacctctccatggtgctgcttgagtgtcctcatgacatggcggctggcttgcctcagagtaactcttgaagaatgtgctagaaggtgagcacctggcttcaataaagctttatttacaagaacaggtagtgggccagatgggccctcctctgtcttcttctgctctatgcttcttgtgggcttgaagacagtgaggagccaaaggtctgtacctcgtctaccccaaaagtactgcctgggcctctggtaccctaatcaggatgcttcgaccttgttctgatgcctggggacttctggtgagttccctggccatccatcctggtctgttcaccttctcaggactccagttgagttgggctgcgtgtgacagacccctgagtcgctgctgtcctctagtggccactggataaattgcacagcacgccggccttggggaaaacgccgcagctgcaggtgccaccagtgagtcttctctttttcgctacagttggtagaaacttctcccagacttccttggtgactaatggtgttgggatgttgtggccttcgccgggaggggacaagttgtcagctcacagtttcacagatggttgaccgatgctgactgtagctggcaggtctcttttggattcaaagtaattaactggcatcatctgtccaagagatgggatggataagaagttaagcttccaggagatgcctcatcatttgtgccagtgaccccgcataatttcttgatgaattgtgcaaactgggaagctgatagctcgtttcagattctctagattttgcccctgaaaaagcatttacgtgatgcagtccgaggtcttgtatggaggagcttggtgtggggagatgtgtggctcacgaactgtcttgtgcatgtgtctccccaggggcattttcagatttctgccacggagatgctcttcgcaaagggagagtcaggtacattggaggattcattgctgtgaccagggaaagcagaggacatgcaaaattaatatttccctttctatcttctaggatggacttttttcattcagaaagccgctctggcttaaagacatgtacaaacctctcagtgccacaagagtaaagaatcacgcatggaagctgcacaagaagtcatctaatgaggacaagatcctcaacagggaccctgggtaaatgacgggaccctcacagttcccatctaaaatgaggagggggtgagacgcttaattgctcctttcaagaatgaaaaccttggcattgttattcttatcccagggacagtgaagccccaacagagaaggaggaggagagtgaagccctgccataggaggagaacccagcccacctcaggcctcctgcaaaaacacatagcataaacaataccatcagaaagaaaagcaggactgaagccagcagcccacacatccacagaggcagcgggcagagcaagcacagggccatcgttcctgcccttgtttcccagtctaattagtcacccagacctgaaaacatatcctcagggggtggagattttacaattaaataccattgtttttggtgccctctccctgggttcatcaagcaccagtcatataataccacatacttgaactcctgcccacaggggacctcccatctcctggcccctattataggatcactgggcctacctgcactgtggggccaagccctgtctttttcccaagccctcaagcacacgcatgaatgttcatcccgacttggtagggggcttttcacccttacaagatggcaaaagattcacactgctttttttaaaatttgtttttctttttaaaaatcccaacccttggatagcaagggaggtgctggaggggtagggtcaagaagagtgtgtgagaacagtaatttcccaagactgccctctgcgggactgtatttcagaaaacacactggtggggctacctctccattcacatgtactgccctagcctctccccatccccggctgatgcacttccatatctgcactgttccataacagcagtagcatgttgcagaaagcgctaggattcctccactccatcttcaaagaaaaagtcgctaataaatcacatttggtaggttagtgaacgttaaacacattagtgagcaaaagaaaataggaatgaacaagaattggtcatctacctaactgaacacaaatgaactctggcagttcggtaataggaggtaaagaaccgcgctaattgcagaacagcagcccccctaccttcccaggagcagtgtgactgggaagcagccccgtgtgtatgctggtgcaggttctaagcaaagtgagctgcccatcagttctgatgagtttgctgatgctagacatatgacatctgttctcttgctgcctgccccagttatctcccaaagttctttactgagaatgaaaagcatctttctctgtgtggtgacttcagtaggccaacaaatatttgagtttaaagcacaagactaaatagtcataggcagagcagtgctaccatttacaatttgcttacttgatgctaaaccatgggttaggcattttacagtcatatcatctagcccagcaagtcatggaagcatagttgttaaaatcatctgatactttgggaggctggggcgggcagatcacgaggtcaggagatcgagaccatcctggctaacatggtgaaaccctgtctctactaaaaatacaaaaaaattagccacgggtggtggcaggagcctgtagtcccagctactcaggaagctgaggcaggagaatggcgtcaacccgggaggtggagcttgcagtaagccgagatcatgccactgcactccagcccgggcaagagagtgagacttcgtctaaaaaaaaaaaaatcatcatctgacagataaggatacagggcttgaagaacataggtgacctgccccaagtgtccaaagccacacatccaaaatgacaaattagggttttaagccagcactcttagacttcaaagcctcttaaccattccactgccctgctgtagggcatagggagataagggggataagctatggttgccatcaaagagttaatatatcaataatatgcggatggtgaggatgatggcagctgctaggggtctacaggcgtgtaccaccatgcccagctacaattcttattattcccaaatgctactgtgtccggaattggtgggttcttggtcttactgacttcaagaatgaagccgcggaacctcgcggtgagtgttacagctcttaaggtggtgcgtctggagtctgtccgttctgatgttgagatgtgttcggagtttcttccttctggtgggttcgtggtctcgctggctcaggagtgaagctgcagaccttcacggcaagtgttacagctcttaaggcagcgcgtctggagttgtttgttcctcccggtgggctcgtggtctcgctgggctcaggagtgaagctgcagatcttcgcggtgagtgttacagctcataaaagcagcgtggacctggcagccctcggaccttgctcctgcccaagcccctgccgttgggccccggtgttgggttcggttgtgctgtctaacggctgcctggccccctcccccctcccctgtacaggaagtgtctgttggcggctaggtcccccaccagatggctcatgctgtggccactctaggagcagctggaggtggaaactcgttggtattaaccctgtgctggagggcccttaatgggttttttgatgcaattggaacaagatttatttattttttatacggggcttagataacatttctctttggtttagcaatatttattttcatttggaaaatttttagcacctatttttattagtttttagaataaagaaagtcaaacatcattttatgtttgataatgtttcctgtatgattttataagagataag

SEQ ID NO: 15074 - RNA, 4257 nt, Homo sapiens
  source 1..4257: mol_type = other RNA
gctgggattacaggcatgagccactgcacccggccctgtctgccctttcttgagcctctggtcccagcaagtttggttgtagtttgatgtgtattaactcttaattctcataataaccctgaaaggtaagtgtgtttgttatttattgctacatcacaaatatctcaaattgagcaaacatttatgatctcatgtgatttctgagggccaggaacctataagcagcttaggtgggtggctctggctcaaggtctctcatgaggttgccgtcaggatgttggccaggactgcagtcatgtaaaagcctgaccagggaggggccattggcttccaaggtgaccccttacacggctgttggcaggaggcctgttcctcattggctgtcggcagggggatcctctgttcctcgccatcggacctctccatggtgctgcttgagtgtcctcatgacatggcggctggcttgcctcagagtaactcttgaagaatgtgctagaaggtgagcacctggcttcaataaagctttatttacaagaacaggtagtgggccagatgggccctcctctgtcttcttctgctctatgcttcttgtgggcttgaagacagtgaggagccaaaggtctgtacctcgtctaccccaaaagtactgcctgggcctctggtaccctaatcaggatgcttcgaccttgttctgatgcctggggacttctggtgagttccctggccatccatcctggtctgttcaccttctcaggactccagttgagttgggctgcgtgtgacagaccccttggggaaaacgccgcagctgcaggtgccaccagtgagtcttctattcaaagtaattaactggcatcatctgtccaagagatgggatggataagaagttaagcttccaggagatgcctcatcatttgtgccagtgaccccgcataatttcttgatgaattgtgcaaactgggaagctgatagctcgtttcagattctctagattttgcccctgaaaaagcatttacgtgatgcagtccgaggtcttgtatggaggagcttggtgtggggagatgtgtggctcacgaactctgatcttggtcaagggagagtgaatcttcactcctcttctttccatctgccagcatgtttggtcttctggcacctggtgttctatacagcacaacatgcttctttgtgttaaattgagatgtcttgtgcatgtgtctccccaggggcattttcagatttctgccacggagatgctcttcgcaaagggagagtcaggtacattggaggattcattgctgtgaccagggaaagcagaggacatgcaaaattaatatttccctttctatcttctaggatggacttttttcattcagaaagccgctctggcttaaagacatgtacaaacctctcagtgccacaagagtaaagaatcacgcatggaagctgcacaagaagtcatctaatgaggacaagatcctcaacagggaccctgggtaaatgacgggaccctcacagttcccatctaaaatgaggagggggtgagacgcttaattgctcctttcaagaatgaaaaccttggcattgttattcttatcccagggacagtgaagccccaacagagaaggaggaggagagtgaagccctgccataggaggagaacccagcccacctcaggcctcctgcaaaaacacatagcataaacaataccatcagaaagaaaagcaggactgaagccagcagcccacacatccacagaggcagcgggcagagcaagcacagggccatcgttcctgcccttgtttcccagtctaattagtcacccagacctgaaaacatatcctcagggggtggagattttacaattaaataccattgtttttggtgccctctccctgggttcatcaagcaccagtcatataataccacatacttgaactcctgcccacaggggacctcccatctcctggcccctattataggatcactgggcctacctgcactgtggggccaagccctgtctttttcccaagccctcaagcacacgcatgaatgttcatcccgacttggtagggggcttttcacccttacaagatggcaaaagattcacactgctttttttaaaatttgtttttctttttaaaaatcccaacccttggatagcaagggaggtgctggaggggtagggtcaagaagagtgtgtgagaacagtaatttcccaagactgccctctgcgggactgtatttcagaaaacacactggtggggctacctctccattcacatgtactgccctagcctctccccatccccggctgatgcacttccatatctgcactgttccataacagcagtagcatgttgcagaaagcgctaggattcctccactccatcttcaaagaaaaagtcgctaataaatcacatttggtaggttagtgaacgttaaacacattagtgagcaaaagaaaataggaatgaacaagaattggtcatctacctaactgaacacaaatgaactctggcagttcggtaataggaggtaaagaaccgcgctaattgcagaacagcagcccccctaccttcccaggagcagtgtgactgggaagcagccccgtgtgtatgctggtgcaggttctaagcaaagtgagctgcccatcagttctgatgagtttgctgatgctagacatatgacatctgttctcttgctgcctgccccagttatctcccaaagttctttactgagaatgaaaagcatctttctctgtgtggtgacttcagtaggccaacaaatatttgagtttaaagcacaagactaaatagtcataggcagagcagtgctaccatttacaatttgcttacttgatgctaaaccatgggttaggcattttacagtcatatcatctagcccagcaagtcatggaagcatagttgttaaaatcatctgatactttgggaggctggggcgggcagatcacgaggtcaggagatcgagaccatcctggctaacatggtgaaaccctgtctctactaaaaatacaaaaaaattagccacgggtggtggcaggagcctgtagtcccagctactcaggaagctgaggcaggagaatggcgtcaacccgggaggtggagcttgcagtaagccgagatcatgccactgcactccagcccgggcaagagagtgagacttcgtctaaaaaaaaaaaaatcatcatctgacagataaggatacagggcttgaagaacataggtgacctgccccaagtgtccaaagccacacatccaaaatgacaaattagggttttaagccagcactcttagacttcaaagcctcttaaccattccactgccctgctgtagggcatagggagataagggggataagctatggttgccatcaaagagttaatatatcaataatatgcggatggtgaggatgatggcagctgctaggggtctacaggcgtgtaccaccatgcccagctacaattcttattattcccaaatgctactgtgtccggaattggtgggttcttggtcttactgacttcaagaatgaagccgcggaacctcgcggtgagtgttacagctcttaaggtggtgcgtctggagtctgtccgttctgatgttgagatgtgttcggagtttcttccttctggtgggttcgtggtctcgctggctcaggagtgaagctgcagaccttcacggcaagtgttacagctcttaaggcagcgcgtctggagttgtttgttcctcccggtgggctcgtggtctcgctgggctcaggagtgaagctgcagatcttcgcggtgagtgttacagctcataaaagcagcgtggacctggcagccctcggaccttgctcctgcccaagcccctgccgttgggccccggtgttgggttcggttgtgctgtctaacggctgcctggccccctcccccctcccctgtacaggaagtgtctgttggcggctaggtcccccaccagatggctcatgctgtggccactctaggagcagctggaggtggaaactcgttggtattaaccctgtgctggagggcccttaatgggttttttgatgcaattggaacaagatttatttattttttatacggggcttagataacatttctctttggtttagcaatatttattttcatttggaaaatttttagcacctatttttattagtttttagaataaagaaagtcaaacatcattttatgtttgataatgtttcctgtatgattttataagagataag

SEQ ID NO: 15075 - RNA, 4231 nt, Homo sapiens
  source 1..4231: mol_type = other RNA
gctgggattacaggcatgagccactgcacccggccctgtctgccctttcttgagcctctggtcccagcaagtttggttgtagtttgatgtgtattaactcttaattctcataataaccctgaaaggtaagtgtgtttgttatttattgctacatcacaaatatctcaaattgagcaaacatttatgatctcatgtgatttctgagggccaggaacctataagcagcttaggtgggtggctctggctcaaggtctctcatgaggttgccgtcaggatgttggccaggactgcagtcatgtaaaagcctgaccagggaggggccattggcttccaaggtgaccccttacacggctgttggcaggaggcctgttcctcattggctgtcggcagggggatcctctgttcctcgccatcggacctctccatggtgctgcttgagtgtcctcatgacatggcggctggcttgcctcagagtaactcttgaagaatgtgctagaaggtgagcacctggcttcaataaagctttatttacaagaacaggtagtgggccagatgggccctcctctgtcttcttctgctctatgcttcttgtgggcttgaagacagtgaggagccaaaggtctgtacctcgtctaccccaaaagtactgcctgggcctctggtaccctaatcaggatgcttcgaccttgttctgatgcctggggacttctggtgagttccctggccatccatcctggtctgttcaccttctcaggactccagttgagttgggctgcgtgtgacagaccccttggggaaaacgccgcagctgcaggtgccaccagtgagtcttctattcaaagtaattaactggcatcatctgtccaagagatgggatggataagaagttaagcttccaggagatgcctcatcatttgtgccagtgaccccgcataatttcttgatgaattgtgcaaactgggaagctgatagctcgtttcagattctctagattttgcccctgaaaaagcatttacgtgatgcagtccgaggtcttgtatggaggagcttggtgtggggagatgtgtggctcacgaactgtcttgtgcatgtgtctccccaggggcattttcagatttctgccacggagatgctcttcgcaaagggagagtcaggtacattggaggattcattgctgtgaccagggaaagcagaggacatgcaaaattaatatttccctttctatcttctaggatggacttttttcattcagaaagccgctctggcttaaagacatgtacaaacctctcagtgccacaagagtaaagaatcacgcatggaagctgcacaagaagtcatctaatgaggacaagatcctcaacagggaccctgggtaaatgacgggaccctcacagttcccatctaaaatgaggagggggtgagacgcttaattgctcctttcaagaatgaaaaccttggcattgttattcttatcccagggacagtgaagccccaacagagaaggaggaggagagtgaagccctgccataggaggagaacccagcccacctcaggcctcctgcaaaaacacatagcataaacaataccatcagaaagaaaagcaggactgaagccagcagcccacacatccacagaggcagcgggcagagcaagcacagggccatcgttcctgcccttgtttcccagtctaattagtcacccagacctgaaaacatatcctcagggggtggagattttacaattaaataccattgtttttggtgccctctccctgggttcatcaagcaccagtcatataataccacatacttgaactcctgcccacaggggacctcccatctcctggcccctattataggatcactgggcctacctgcactgtggggccaagccctgtctttttcccaagccctcaagcacacgcatgaatgttcatcccgacttggtagggggcttttcacccttacaagatggcaaaagattcacactgctttttttaaaatttgtttttctttttaaaaatcccaacccttggatagcaagggaggtgctggaggggtagggtcaagaagagtgtgtgagaacagtaatttcccaagactgccctctgcgggactgtatttcagaaaacacactggtggggctacctctccattcacatgtactgccctagcctctccccatccccggctgatgcacttccatatctgcactgttccataacagcagtagcatgttgcagaaagcgctaggattcctccactccatcttcaaagaaaaagtcgctaataaatcacatttggtaggttagtgaacgttaaacacattagtgagcaaaagaaaataggaatgaacaagaattggtcatctacctaactgaacacaaatgaactctggcagttcggtaataggaggtaaagaaccgcgctaattgcagaacagcagcccccctaccttcccaggagcagtgtgactgggaagcagccccgtgtgtatgctggtgcaggttctaagcaaagtgagctgcccatcagttctgatgagtttgctgatgctagacatatgacatctgttctcttgctgcctgccccagttatctcccaaagttctttactgagaatgaaaagcatctttctctgtgtggtgacttcagtaggccaacaaatatttgagtttaaagcacaagactaaatagtcataggcagagcagtgctaccatttacaatttgcttacttgatgctaaaccatgggttaggcattttacagtcatatcatctagcccagcaagtcatggaagcatagttgttaaaatcatctgatactttgggaggctggggcgggcagatcacgaggtcaggagatcgagaccatcctggctaacatggtgaaaccctgtctctactaaaaatacaaaaaaattagccacgggtggtggcaggagcctgtagtcccagctactcaggaagctgaggcaggagaatggcgtcaacccgggaggtggagcttgcagtaagccgagatcatgccactgcactccagcccgggcaagagagtgagacttcgtctaaaaaaaaaaaaatcatcatctgacagataaggatacagggcttgaagaacataggtgacctgccccaagtgtccaaagccacacatccaaaatgacaaattagggttttaagccagcactcttagacttcaaagcctcttaaccattccactgccctgctgtagggcatagggagataagggggataagctatggttgccatcaaagagttaatatatcaataatatgcggatggtgaggatgatggcagctgctaggggtctacaggcgtgtaccaccatgcccagctacaattcttattattcccaaatgctactgtgtccggaattggtgggttcttggtcttactgacttcaagaatgaagccgcggaacctcgcggtgagtgttacagctcttaaggtggtgcgtctggagtctgtccgttctgatgttgagatgtgttcggagtttcttccttctggtgggttcgtggtctcgctggctcaggagtgaagctgcagaccttcacggcaagtgttacagctcttaaggcagcgcgtctggagttgtttgttcctcccggtgggctcgtggtctcgctgggctcaggagtgaagctgcagatcttcgcggtgagtgttacagctcataaaagcagcgtggacctcctttccacattccaaattccacgtgactacattttattggcagcaccctgctggcaagtgagccttgatgtgtgcttcctgggcttctggcacctggcagccctcggaccttgctcctgcccaagcccctgccgttgggccccggtgttgggttcggttgtgctgtctaacggctgcctggccccctcccccctcccctgtacaggaagtgtctgttggcggctaggtcccccaccagatggctcatgctgtggccactctaggagcagctggaggtggaaactcgttggtattaaccctgtgctggagggcccttaatgggttttttgatgcaattggaacaagatttatttattttttatacggggcttagataacatttctctttggtttagcaatatttattttcatttggaaaatttttagcacctatttttattagtttttagaataaagaaagtcaaacatcattttatgtttgataatgtttcctgtatgattttataagagataa

SEQ ID NO: 15076 - RNA, 4347 nt, Homo sapiens
  source 1..4347: mol_type = other RNA
gctgggattacaggcatgagccactgcacccggccctgtctgccctttcttgagcctctggtcccagcaagtttggttgtagtttgatgtgtattaactcttaattctcataataaccctgaaaggtaagtgtgtttgttatttattgctacatcacaaatatctcaaattgagcaaacatttatgatctcatgtgatttctgagggccaggaacctataagcagcttaggtgggtggctctggctcaaggtctctcatgaggttgccgtcaggatgttggccaggactgcagtcatgtaaaagcctgaccagggaggggccattggcttccaaggtgaccccttacacggctgttggcaggaggcctgttcctcattggctgtcggcagggggatcctctgttcctcgccatcggacctctccatggtgctgcttgagtgtcctcatgacatggcggctggcttgcctcagagtaactcttgaagaatgtgctagaaggtgagcacctggcttcaataaagctttatttacaagaacaggtagtgggccagatgggccctcctctgtcttcttctgctctatgcttcttgtgggcttgaagacagtgaggagccaaaggtctgtacctcgtctaccccaaaagtactgcctgggcctctggtaccctaatcaggatgcttcgaccttgttctgatgcctggggacttctggtgagttccctggccatccatcctggtctgttcaccttctcaggactccagttgagttgggctgcgtgtgacagaccccttggggaaaacgccgcagctgcaggtgccaccagtgagtcttctattcaaagtaattaactggcatcatctgtccaagagatgggatggataagaagttaagcttccaggagatgcctcatcatttgtgccagtgaccccgcataatttcttgatgaattgtgcaaactgggaagctgatagctcgtttcagattctctagattttgcccctgaaaaagcatttacgtgatgcagtccgaggtcttgtatggaggagcttggtgtggggagatgtgtggctcacgaactgtcttgtgcatgtgtctccccaggggcattttcagatttctgccacggagatgctcttcgcaaagggagagtcaggtacattggaggattcattgctgtgaccagggaaagcagaggacatgcaaaattaatatttccctttctatcttctaggatggacttttttcattcagaaagccgctctggcttaaagacatgtacaaacctctcagtgccacaagagtaaagaatcacgcatggaagctgcacaagaagtcatctaatgaggacaagatcctcaacagggaccctgggtaaatgacgggaccctcacagttcccatctaaaatgaggagggggtgagacgcttaattgctcctttcaagaatgaaaaccttggcattgttattcttatcccagggacagtgaagccccaacagagaaggaggaggagagtgaagccctgccataggaggagaacccagcccacctcaggcctcctgcaaaaacacatagcataaacaataccatcagaaagaaaagcaggactgaagccagcagcccacacatccacagaggcagcgggcagagcaagcacagggccatcgttcctgcccttgtttcccagtctaattagtcacccagacctgaaaacatatcctcagggggtggagattttacaattaaataccattgtttttggtgccctctccctgggttcatcaagcaccagtcatataataccacatacttgaactcctgcccacaggggacctcccatctcctggcccctattataggatcactgggcctacctgcactgtggggccaagccctgtctttttcccaagccctcaagcacacgcatgaatgttcatcccgacttggtagggggcttttcacccttacaagatggcaaaagattcacactgctttttttaaaatttgtttttctttttaaaaatcccaacccttggatagcaagggaggtgctggaggggtagggtcaagaagagtgtgtgagaacagtaatttcccaagactgccctctgcgggactgtatttcagaaaacacactggtggggctacctctccattcacatgtactgccctagcctctccccatccccggctgatgcacttccatatctgcactgttccataacagcagtagcatgttgcagaaagcgctaggattcctccactccatcttcaaagaaaaagtcgctaataaatcacatttggtaggttagtgaacgttaaacacattagtgagcaaaagaaaataggaatgaacaagaattggtcatctacctaactgaacacaaatgaactctggcagttcggtaataggaggtaaagaaccgcgctaattgcagaacagcagcccccctaccttcccaggagcagtgtgactgggaagcagccccgtgtgtatgctggtgcaggttctaagcaaagtgagctgcccatcagttctgatgagtttgctgatgctagacatatgacatctgttctcttgctgcctgccccagttatctcccaaagttctttactgagaatgaaaagcatctttctctgtgtggtgacttcagtaggccaacaaatatttgagtttaaagcacaagactaaatagtcataggcagagcagtgctaccatttacaatttgcttacttgatgctaaaccatgggttaggcattttacagtcatatcatctagcccagcaagtcatggaagcatagttgttaaaatcatctgatactttgggaggctggggcgggcagatcacgaggtcaggagatcgagaccatcctggctaacatggtgaaaccctgtctctactaaaaatacaaaaaaattagccacgggtggtggcaggagcctgtagtcccagctactcaggaagctgaggcaggagaatggcgtcaacccgggaggtggagcttgcagtaagccgagatcatgccactgcactccagcccgggcaagagagtgagacttcgtctaaaaaaaaaaaaatcatcatctgacagataaggatacagggcttgaagaacataggtgacctgccccaagtgtccaaagccacacatccaaaatgacaaattagggttttaagccagcactcttagacttcaaagcctcttaaccattccactgccctgctgtagggcatagggagataagggggataagctatggttgccatcaaagagttaatatatcaataatatgcggatggtgaggatgatggcagctgctaggggtctacaggcgtgtaccaccatgcccagctacaattcttattattcccaaatgctactgtgtccggaattggtgggttcttggtcttactgacttcaagaatgaagccgcggaacctcgcggtgagtgttacagctcttaaggtggtgcgtctggagtctgtccgttctgatgttgagatgtgttcggagtttcttccttctggtgggttcgtggtctcgctggctcaggagtgaagctgcagaccttcacggcaagtgttacagctcttaaggcagcgcgtctggagttgtttgttcctcccggtgggctcgtggtctcgctgggctcaggagtgaagctgcagatcttcgcggtgagtgttacagctcataaaagcagcgtggacctcctttccacattccaaattccacgtgactacattttattggcagcaccctgctggcaagtgagccttgatgtgtgcttcctgggcttctggcacctggttagtggcaaactgcgatgagacctcatggtcatcccggttagacacgtccctgtctgtgctgctcaagccagaccctcgaagcctcagaatgggatcttagagacaggatcttcaggccaggtggcttcccttcctctctgcgtcggtccgtcccacctcggctcggcctggcgaccctaactccgctccgcgcccccggccgcggccccggcccgcctcctgggcagccaggccccccggccactcggccggcagcccgcggcccaggtctgcaagtgggagctgggctggggtccccatgctccacacacgcgtctcctctcccccagccctgccgcttccagggccctcggtgacgcccgctccccgggcccctcggccccccgcctctcagccgggcgctccctcggggccgcctcctctgcctcaccatcatccttgcccactcgtgctcccacccccaggggcaccagagccaacggctgctcccccagcctcggaccttcctgcgcggctcaaccaagcctagaa

SEQ ID NO: 15077 - RNA, 4134 nt, Homo sapiens
  source 1..4134: mol_type = other RNA
gctgggattacaggcatgagccactgcacccggccctgtctgccctttcttgagcctctggtcccagcaagtttggttgtagtttgatgtgtattaactcttaattctcataataaccctgaaaggtaagtgtgtttgttatttattgctacatcacaaatatctcaaattgagcaaacatttatgatctcatgtgatttctgagggccaggaacctataagcagcttaggtgggtggctctggctcaaggtctctcatgaggttgccgtcaggatgttggccaggactgcagtcatgtaaaagcctgaccagggaggggccattggcttccaaggtgaccccttacacggctgttggcaggaggcctgttcctcattggctgtcggcagggggatcctctgttcctcgccatcggacctctccatggtgctgcttgagtgtcctcatgacatggcggctggcttgcctcagagtaactcttgaagaatgtgctagaaggtgagcacctggcttcaataaagctttatttacaagaacaggtagtgggccagatgggccctcctctgtcttcttctgctctatgcttcttgtgggcttgaagacagtgaggagccaaaggtctgtacctcgtctaccccaaaagtactgcctgggcctctggtaccctaatcaggatgcttcgaccttgttctgatgcctggggacttctggtgagttccctggccatccatcctggtctgttcaccttctcaggactccagttgagttgggctgcgtgtgacagaccccttggggaaaacgccgcagctgcaggtgccaccagtgagtcttctattcaaagtaattaactggcatcatctgtccaagagatgggatggataagaagttaagcttccaggagatgcctcatcatttgtgccagtgaccccgcataatttcttgatgaattgtgcaaactgggaagctgatagctcgtttcagattctctagattttgcccctgaaaaagcatttacgtgatgcagtccgaggtcttgtatggaggagcttggtgtggggagatgtgtggctcacgaactgtcttgtgcatgtgtctccccaggggcattttcagatttctgccacggagatgctcttcgcaaagggagagtcaggtacattggaggattcattgctgtgaccagggaaagcagaggacatgcaaaattaatatttccctttctatcttctaggatggacttttttcattcagaaagccgctctggcttaaagacatgtacaaacctctcagtgccacaagagtaaagaatcacgcatggaagctgcacaagaagtcatctaatgaggacaagatcctcaacagggaccctgggtaaatgacgggaccctcacagttcccatctaaaatgaggagggggtgagacgcttaattgctcctttcaagaatgaaaaccttggcattgttattcttatcccagggacagtgaagccccaacagagaaggaggaggagagtgaagccctgccataggaggagaacccagcccacctcaggcctcctgcaaaaacacatagcataaacaataccatcagaaagaaaagcaggactgaagccagcagcccacacatccacagaggcagcgggcagagcaagcacagggccatcgttcctgcccttgtttcccagtctaattagtcacccagacctgaaaacatatcctcagggggtggagattttacaattaaataccattgtttttggtgccctctccctgggttcatcaagcaccagtcatataataccacatacttgaactcctgcccacaggggacctcccatctcctggcccctattataggatcactgggcctacctgcactgtggggccaagccctgtctttttcccaagccctcaagcacacgcatgaatgttcatcccgacttggtagggggcttttcacccttacaagatggcaaaagattcacactgctttttttaaaatttgtttttctttttaaaaatcccaacccttggatagcaagggaggtgctggaggggtagggtcaagaagagtgtgtgagaacagtaatttcccaagactgccctctgcgggactgtatttcagaaaacacactggtggggctacctctccattcacatgtactgccctagcctctccccatccccggctgatgcacttccatatctgcactgttccataacagcagtagcatgttgcagaaagcgctaggattcctccactccatcttcaaagaaaaagtcgctaataaatcacatttggtaggttagtgaacgttaaacacattagtgagcaaaagaaaataggaatgaacaagaattggtcatctacctaactgaacacaaatgaactctggcagttcggtaataggaggtaaagaaccgcgctaattgcagaacagcagcccccctaccttcccaggagcagtgtgactgggaagcagccccgtgtgtatgctggtgcaggttctaagcaaagtgagctgcccatcagttctgatgagtttgctgatgctagacatatgacatctgttctcttgctgcctgccccagttatctcccaaagttctttactgagaatgaaaagcatctttctctgtgtggtgacttcagtaggccaacaaatatttgagtttaaagcacaagactaaatagtcataggcagagcagtgctaccatttacaatttgcttacttgatgctaaaccatgggttaggcattttacagtcatatcatctagcccagcaagtcatggaagcatagttgttaaaatcatctgatactttgggaggctggggcgggcagatcacgaggtcaggagatcgagaccatcctggctaacatggtgaaaccctgtctctactaaaaatacaaaaaaattagccacgggtggtggcaggagcctgtagtcccagctactcaggaagctgaggcaggagaatggcgtcaacccgggaggtggagcttgcagtaagccgagatcatgccactgcactccagcccgggcaagagagtgagacttcgtctaaaaaaaaaaaaatcatcatctgacagataaggatacagggcttgaagaacataggtgacctgccccaagtgtccaaagccacacatccaaaatgacaaattagggttttaagccagcactcttagacttcaaagcctcttaaccattccactgccctgctgtagggcatagggagataagggggataagctatggttgccatcaaagagttaatatatcaataatatgcggatggtgaggatgatggcagctgctaggggtctacaggcgtgtaccaccatgcccagctacaattcttattattcccaaatgctactgtgtccggaattggtgggttcttggtcttactgacttcaagaatgaagccgcggaacctcgcggtgagtgttacagctcttaaggtggtgcgtctggagtctgtccgttctgatgttgagatgtgttcggagtttcttccttctggtgggttcgtggtctcgctggctcaggagtgaagctgcagaccttcacggcaagtgttacagctcttaaggcagcgcgtctggagttgtttgttcctcccggtgggctcgtggtctcgctgggctcaggagtgaagctgcagatcttcgcggtgagtgttacagctcataaaagcagcgtggacctggcagccctcggaccttgctcctgcccaagcccctgccgttgggccccggtgttgggttcggttgtgctgtctaacggctgcctggccccctcccccctcccctgtacaggaagtgtctgttggcggctaggtcccccaccagatggctcatgctgtggccactctaggagcagctggaggtggaaactcgttggtattaaccctgtgctggagggcccttaatgggttttttgatgcaattggaacaagatttatttattttttatacggggcttagataacatttctctttggtttagcaatatttattttcatttggaaaatttttagcacctatttttattagtttttagaataaagaaagtcaaacatcattttatgtttgataatgtttcctgtatgattttataagagata

SEQ ID NO: 15078 - RNA, 4251 nt, Homo sapiens
  source 1..4251: mol_type = other RNA
gctgggattacaggcatgagccactgcacccggccctgtctgccctttcttgagcctctggtcccagcaagtttggttgtagtttgatgtgtattaactcttaattctcataataaccctgaaaggtaagtgtgtttgttatttattgctacatcacaaatatctcaaattgagcaaacatttatgatctcatgtgatttctgagggccaggaacctataagcagcttaggtgggtggctctggctcaaggtctctcatgaggttgccgtcaggatgttggccaggactgcagtcatgtaaaagcctgaccagggaggggccattggcttccaaggtgaccccttacacggctgttggcaggaggcctgttcctcattggctgtcggcagggggatcctctgttcctcgccatcggacctctccatggtgctgcttgagtgtcctcatgacatggcggctggcttgcctcagagtaactcttgaagaatgtgctagaaggtgagcacctggcttcaataaagctttatttacaagaacaggtagtgggccagatgggccctcctctgtcttcttctgctctatgcttcttgtgggcttgaagacagtgaggagccaaaggtctgtacctcgtctaccccaaaagtactgcctgggcctctggtaccctaatcaggatgcttcgaccttgttctgatgcctggggacttctggtgagttccctggccatccatcctggtctgttcaccttctcaggactccagttgagttgggctgcgtgtgacagaccccttggggaaaacgccgcagctgcaggtgccaccagtgagtcttctattcaaagtaattaactggcatcatctgtccaagagatgggatggataagaagttaagcttccaggagatgcctcatcatttgtgccagtgaccccgcataatttcttgatgaattgtgcaaactgggaagctgatagctcgtttcagattctctagattttgcccctgaaaaagcatttacgtgatgcagtccgaggtcttgtatggaggagcttggtgtggggagatgtgtggctcacgaactgtcttgtgcatgtgtctccccaggggcattttcagatttctgccacggagatgctcttcgcaaagggagagtcaggtacattggaggattcattgctgtgaccagggaaagcagaggacatgcaaaattaatatttccctttctatcttctaggatggacttttttcattcagaaagccgctctggcttaaagacatgtacaaacctctcagtgccacaagagtaaagaatcacgcatggaagctgcacaagaagtcatctaatgaggacaagatcctcaacagggaccctgggtaaatgacgggaccctcacagttcccatctaaaatgaggagggggtgagacgcttaattgctcctttcaagaatgaaaaccttggcattgttattcttatcccagggacagtgaagccccaacagagaaggaggaggagagtgaagccctgccataggaggagaacccagcccacctcaggcctcctgcaaaaacacatagcataaacaataccatcagaaagaaaagcaggactgaagccagcagcccacacatccacagaggcagcgggcagagcaagcacagggccatcgttcctgcccttgtttcccagtctaattagtcacccagacctgaaaacatatcctcagggggtggagattttacaattaaataccattgtttttggtgccctctccctgggttcatcaagcaccagtcatataataccacatacttgaactcctgcccacaggggacctcccatctcctggcccctattataggatcactgggcctacctgcactgtggggccaagccctgtctttttcccaagccctcaagcacacgcatgaatgttcatcccgacttggtagggggcttttcacccttacaagatggcaaaagattcacactgctttttttaaaatttgtttttctttttaaaaatcccaacccttggatagcaagggaggtgctggaggggtagggtcaagaagagtgtgtgagaacagtaatttcccaagactgccctctgcgggactgtatttcagaaaacacactggtggggctacctctccattcacatgtactgccctagcctctccccatccccggctgatgcacttccatatctgcactgttccataacagcagtagcatgttgcagaaagcgctaggattcctccactccatcttcaaagaaaaagtcgctaataaatcacatttggtaggttagtgaacgttaaacacattagtgagcaaaagaaaataggaatgaacaagaattggtcatctacctaactgaacacaaatgaactctggcagttcggtaataggaggtaaagaaccgcgctaattgcagaacagcagcccccctaccttcccaggagcagtgtgactgggaagcagccccgtgtgtatgctggtgcaggttctaagcaaagtgagctgcccatcagttctgatgagtttgctgatgctagacatatgacatctgttctcttgctgcctgccccagttatctcccaaagttctttactgagaatgaaaagcatctttctctgtgtggtgacttcagtaggccaacaaatatttgagtttaaagcacaagactaaatagtcataggcagagcagtgctaccatttacaatttgcttacttgatgctaaaccatgggttaggcattttacagtcatatcatctagcccagcaagtcatggaagcatagttgttaaaatcatctgatactttgggaggctggggcgggcagatcacgaggtcaggagatcgagaccatcctggctaacatggtgaaaccctgtctctactaaaaatacaaaaaaattagccacgggtggtggcaggagcctgtagtcccagctactcaggaagctgaggcaggagaatggcgtcaacccgggaggtggagcttgcagtaagccgagatcatgccactgcactccagcccgggcaagagagtgagacttcgtctaaaaaaaaaaaaatcatcatctgacagataaggatacagggcttgaagaacataggtgacctgccccaagtgtccaaagccacacatccaaaatgacaaattagggttttaagccagcactcttagacttcaaagcctcttaaccattccactgccctgctgtagggcatagggagataagggggataagctatggttgccatcaaagagttaatatatcaataatatgcggatggtgaggatgatggcagctgctaggggtctacaggcgtgtaccaccatgcccagctacaattcttattattcccaaatgctactgtgtccggaattggtgggttcttggtcttactgacttcaagaatgaagccgcggaacctcgcggtgagtgttacagctcttaaggtggtgcgtctggagtctgtccgttctgatgttgagatgtgttcggagtttcttccttctggtgggttcgtggtctcgctggctcaggagtgaagctgcagaccttcacggcaagtgttacagctcttaaggcagcgcgtctggagttgtttgttcctcccggtgggctcgtggtctcgctgggctcaggagtgaagctgcagatcttcgcggtgagtgttacagctcataaaagcagcgtggacctggttagtggcaaactgcgatgagacctcatggtcatcccggttagacacgtccctgtctgtgctgctcaagccagaccctcgaagcctcagaatgggatcttagagacaggatcttcaggccaggtggcttcccttcctctctgcgtcggtccgtcccacctcggctcggcctggcgaccctaactccgctccgcgcccccggccgcggccccggcccgcctcctgggcagccaggccccccggccactcggccggcagcccgcggcccaggtctgcaagtgggagctgggctggggtccccatgctccacacacgcgtctcctctcccccagccctgccgcttccagggccctcggtgacgcccgctccccgggcccctcggccccccgcctctcagccgggcgctccctcggggccgcctcctctgcctcaccatcatccttgcccactcgtgctcccacccccaggggcaccagagccaacggctgctcccccagcctcggaccttcctgcgcggctcaaccaagcctagaa

SEQ ID NO: 15079 - RNA, 1398 nt, Homo sapiens
  source 1..1398: mol_type = other RNA
gctgggattacaggcatgagccactgcacccggccctgtctgccctttcttgagcctctggtcccagcaagtttggttgtagtttgatgtgtattaactcttaattctcataataaccctgaaaggtaagtgtgtttgttatttattgctacatcacaaatatctcaaattgagcaaacatttatgatctcatgtgatttctgagggccaggaacctataagcagcttaggtgggtggctctggctcaaggtctctcatgaggttgccgtcaggatgttggccaggactgcagtcatgtaaaagcctgaccagggaggggccattggcttccaaggtgaccccttacacggctgttggcaggaggcctgttcctcattggctgtcggcagggggatcctctgttcctcgccatcggacctctccatggtgctgcttgagtgtcctcatgacatggcggctggcttgcctcagagtaactcttgaagaatgtgctagaaggtgagcacctggcttcaataaagctttatttacaagaacaggtagtgggccagatgggccctcctctgtcttcttctgctctatgcttcttgtgggcttgaagacagtgaggagccaaaggtctgtacctcgtctaccccaaaagtactgcctgggcctctggtaccctaatcaggatgcttcgaccttgttctgatgcctggggacttctggtgagttccctggccatccatcctggtctgttcaccttctcaggactccagttgagttgggctgcgtgtgacagaccccttggggaaaacgccgcagctgcaggtgccaccagtgagtcttctattcaaagtaattaactggcatcatctgtccaagagatgggatggataagaagttaagcttccaggagatgcctcatcatttgtgccagtgaccccgcataatttcttgatgaattgtgcaaactgggaagctgatagctcgtttcagattctctagattttgcccctgaaaaagcatttacgtgatgcagtccgaggtcttgtatggaggagcttggtgtggggagatgtgtggctcacgaactgtcttgtgcatgtgtctccccaggggcattttcagatttctgccacggagatgctcttcgcaaagggagagtcaggtacattggaggattcattgttcaagaatgaagccgcggaacctcgcggtgagtgttacagctcttaaggtggtgcgtctggagtctgtccgttctgatgttgagatgtgttcggagtttcttccttctggtgggttcgtggtctcgctggctcaggagtgaagctgcagaccttcacggcaagtgttacagctcttaaggcagcgcgtctggagttgtttgttcctcccggtgggctcgtggt

SEQ ID NO: 15080 - RNA, 1813 nt, Homo sapiens
  source 1..1813: mol_type = other RNA
gctgggattacaggcatgagccactgcacccggccctgtctgccctttcttgagcctctggtcccagcaagtttggttgtagtttgatgtgtattaactcttaattctcataataaccctgaaaggtaagtgtgtttgttatttattgctacatcacaaatatctcaaattgagcaaacatttatgatctcatgtgatttctgagggccaggaacctataagcagcttaggtgggtggctctggctcaaggtctctcatgaggttgccgtcaggatgttggccaggactgcagtcatgtaaaagcctgaccagggaggggccattggcttccaaggtgaccccttacacggctgttggcaggaggcctgttcctcattggctgtcggcagggggatcctctgttcctcgccatcggacctctccatggtgctgcttgagtgtcctcatgacatggcggctggcttgcctcagagtaactcttgaagaatgtgctagaaggtgagcacctggcttcaataaagctttatttacaagaacaggtagtgggccagatgggccctcctctgtcttcttctgctctatgcttcttgtgggcttgaagacagtgaggagccaaaggtctgtacctcgtctaccccaaaagtactgcctgggcctctggtaccctaatcaggatgcttcgaccttgttctgatgcctggggacttctggtgagttccctggccatccatcctggtctgttcaccttctcaggactccagttgagttgggctgcgtgtgacagaccccttggggaaaacgccgcagctgcaggtgccaccagtgagtcttctattcaaagtaattaactggcatcatctgtccaagagatgggatggataagaagttaagcttccaggagatgcctcatcatttgtgccagtgaccccgcataatttcttgatgaattgtgcaaactgggaagctgatagctcgtttcagattctctagattttgcccctgaaaaagcatttacgtgatgcagtccgaggtcttgtatggaggagcttggtgtggggagatgtgtggctcacgaacttcaagaatgaagccgcggaacctcgcggtgagtgttacagctcttaaggtggtgcgtctggagtctgtccgttctgatgttgagatgtgttcggagtttcttccttctggtgggttcgtggtctcgctggctcaggagtgaagctgcagaccttcacggcaagtgttacagctcttaaggcagcgcgtctggagttgtttgttcctcccggtgggctcgtggtctcgctgggctcaggagtgaagctgcagatcttcgcggtgagtgttacagctcataaaagcagcgtggacctggcagccctcggaccttgctcctgcccaagcccctgccgttgggccccggtgttgggttcggttgtgctgtctaacggctgcctggccccctcccccctcccctgtacaggaagtgtctgttggcggctaggtcccccaccagatggctcatgctgtggccactctaggagcagctggaggtggaaactcgttggtattaaccctgtgctggagggcccttaatgggttttttgatgcaattggaacaagatttatttattttttatacggggcttagataacatttctctttggtttagcaatatttattttcatttggaaaatttttagcacctatttttattagtttttagaataaagaaagtcaaacatcattttatgtttgataatgtttcctgtatgattttataagagataagttaaattttacctttatat

SEQ ID NO: 15081 - RNA, 4031 nt, Homo sapiens
  source 1..4031: mol_type = other RNA
gctgggattacaggcatgagccactgcacccggccctgtctgccctttcttgagcctctggtcccagcaagtttggttgtagtttgatgtgtattaactcttaattctcataataaccctgaaaggtaagtgtgtttgttatttattgctacatcacaaatatctcaaattgagcaaacatttatgatctcatgtgatttctgagggccaggaacctataagcagcttaggtgggtggctctggctcaaggtctctcatgaggttgccgtcaggatgttggccaggactgcagtcatgtaaaagcctgaccagggaggggccattggcttccaaggtgaccccttacacggctgttggcaggaggcctgttcctcattggctgtcggcagggggatcctctgttcctcgccatcggacctctccatggtgctgcttgagtgtcctcatgacatggcggctggcttgcctcagagtaactcttgaagaatgtgctagaaggtgagcacctggcttcaataaagctttatttacaagaacaggtagtgggccagatgggccctcctctgtcttcttctgctctatgcttcttgtgggcttgaagacagtgaggagccaaaggtctgtacctcgtctaccccaaaagtactgcctgggcctctggtaccctaatcaggatgcttcgaccttgttctgatgcctggggacttctggtgagttccctggccatccatcctggtctgttcaccttctcaggactccagttgagttgggctgcgtgtgacagaccccttggggaaaacgccgcagctgcaggtgccaccagtgagtcttctattcaaagtaattaactggcatcatctgtccaagagatgggatggataagaagttaagcttccaggagatgcctcatcatttgtgccagtgaccccgcataatttcttgatgaattgtgcaaactgggaagctgatagcttgtcttgtgcatgtgtctccccaggggcattttcagatttctgccacggagatgctcttcgcaaagggagagtcaggtacattggaggattcattgctgtgaccagggaaagcagaggacatgcaaaattaatatttccctttctatcttctaggatggacttttttcattcagaaagccgctctggcttaaagacatgtacaaacctctcagtgccacaagagtaaagaatcacgcatggaagctgcacaagaagtcatctaatgaggacaagatcctcaacagggaccctgggtaaatgacgggaccctcacagttcccatctaaaatgaggagggggtgagacgcttaattgctcctttcaagaatgaaaaccttggcattgttattcttatcccagggacagtgaagccccaacagagaaggaggaggagagtgaagccctgccataggaggagaacccagcccacctcaggcctcctgcaaaaacacatagcataaacaataccatcagaaagaaaagcaggactgaagccagcagcccacacatccacagaggcagcgggcagagcaagcacagggccatcgttcctgcccttgtttcccagtctaattagtcacccagacctgaaaacatatcctcagggggtggagattttacaattaaataccattgtttttggtgccctctccctgggttcatcaagcaccagtcatataataccacatacttgaactcctgcccacaggggacctcccatctcctggcccctattataggatcactgggcctacctgcactgtggggccaagccctgtctttttcccaagccctcaagcacacgcatgaatgttcatcccgacttggtagggggcttttcacccttacaagatggcaaaagattcacactgctttttttaaaatttgtttttctttttaaaaatcccaacccttggatagcaagggaggtgctggaggggtagggtcaagaagagtgtgtgagaacagtaatttcccaagactgccctctgcgggactgtatttcagaaaacacactggtggggctacctctccattcacatgtactgccctagcctctccccatccccggctgatgcacttccatatctgcactgttccataacagcagtagcatgttgcagaaagcgctaggattcctccactccatcttcaaagaaaaagtcgctaataaatcacatttggtaggttagtgaacgttaaacacattagtgagcaaaagaaaataggaatgaacaagaattggtcatctacctaactgaacacaaatgaactctggcagttcggtaataggaggtaaagaaccgcgctaattgcagaacagcagcccccctaccttcccaggagcagtgtgactgggaagcagccccgtgtgtatgctggtgcaggttctaagcaaagtgagctgcccatcagttctgatgagtttgctgatgctagacatatgacatctgttctcttgctgcctgccccagttatctcccaaagttctttactgagaatgaaaagcatctttctctgtgtggtgacttcagtaggccaacaaatatttgagtttaaagcacaagactaaatagtcataggcagagcagtgctaccatttacaatttgcttacttgatgctaaaccatgggttaggcattttacagtcatatcatctagcccagcaagtcatggaagcatagttgttaaaatcatctgatactttgggaggctggggcgggcagatcacgaggtcaggagatcgagaccatcctggctaacatggtgaaaccctgtctctactaaaaatacaaaaaaattagccacgggtggtggcaggagcctgtagtcccagctactcaggaagctgaggcaggagaatggcgtcaacccgggaggtggagcttgcagtaagccgagatcatgccactgcactccagcccgggcaagagagtgagacttcgtctaaaaaaaaaaaaatcatcatctgacagataaggatacagggcttgaagaacataggtgacctgccccaagtgtccaaagccacacatccaaaatgacaaattagggttttaagccagcactcttagacttcaaagcctcttaaccattccactgccctgctgtagggcatagggagataagggggataagctatggttgccatcaaagagttaatatatcaataatatgcggatggtgaggatgatggcagctgctaggggtctacaggcgtgtaccaccatgcccagctacaattcttattattcccaaatgctactgtgtccggaattggtgggttcttggtcttactgacttcaagaatgaagccgcggaacctcgcggtgagtgttacagctcttaaggtggtgcgtctggagtctgtccgttctgatgttgagatgtgttcggagtttcttccttctggtgggttcgtggtctcgctggctcaggagtgaagctgcagaccttcacggcaagtgttacagctcttaaggcagcgcgtctggagttgtttgttcctcccggtgggctcgtggtctcgctgggctcaggagtgaagctgcagatcttcgcggtgagtgttacagctcataaaagcagcgtggacctggcagccctcggaccttgctcctgcccaagcccctgccgttgggccccggtgttgggttcggttgtgctgtctaacggctgcctggccccctcccccctcccctgtacaggaagtgtctgttggcggctaggtcccccaccagatggctcatgctgtggccactctaggagcagctggaggtggaaactcgttggtattaaccctgtgctggagggcccttaatgggttttttgatgcaattggaacaagatttatttattttttatacggggcttagataacatttctctttggtttagcaatatttattttcatttggaaaatttttagcacctatttttattagtttttagaataaagaaagtcaaacatcattttatgtttgataatgtttcctgtatgattttataagagataa

SEQ ID NO: 15082 - RNA, 4291 nt, Homo sapiens
  source 1..4291: mol_type = other RNA
gctgggattacaggcatgagccactgcacccggccctgtctgccctttcttgagcctctggtcccagcaagtttggttgtagtttgatgtgtattaactcttaattctcataataaccctgaaaggtaagtgtgtttgttatttattgctacatcacaaatatctcaaattgagcaaacatttatgatctcatgtgatttctgagggccaggaacctataagcagcttaggtgggtggctctggctcaaggtctctcatgaggttgccgtcaggatgttggccaggactgcagtcatgtaaaagcctgaccagggaggggccattggcttccaaggtgaccccttacacggctgttggcaggaggcctgttcctcattggctgtcggcagggggatcctctgttcctcgccatcggacctctccatggtgctgcttgagtgtcctcatgacatggcggctggcttgcctcagagtaactcttgaagaatgtgctagaaggtgagcacctggcttcaataaagctttatttacaagaacaggtagtgggccagatgggccctcctctgtcttcttctgctctatgcttcttgtgggcttgaagacagtgaggagccaaaggtctgtacctcgtctaccccaaaagtactgcctgggcctctggtaccctaatcaggatgcttcgaccttgttctgatgcctggggacttctggtgagttccctggccatccatcctggtctgttcaccttctcaggactccagttgagttgggctgcgtgtgacagaccccttggggaaaacgccgcagctgcaggtgccaccagtgagtcttctctttttcgctacagttggtagaaacttctcccagacttccttggtgactaatggtgttgggatgttgtggccttcgccgggaggggacaagttgtcagctcacagtttcacagatggttgaccgatgctgactgtagctggcaggtctcttttggattcaaagtaattaactggcatcatctgtccaagagatgggatggataagaagttaagcttccaggagatgcctcatcatttgtgccagtgaccccgcataatttcttgatgaattgtgcaaactgggaagctgatagctcgtttcagattctctagattttgcccctgaaaaagcatttacgtgatgcagtccgaggtcttgtatggaggagcttggtgtggggagatgtgtggctcacgaactgtcttgtgcatgtgtctccccaggggcattttcagatttctgccacggagatgctcttcgcaaagggagagtcaggtacattggaggattcattgctgtgaccagggaaagcagaggacatgcaaaattaatatttccctttctatcttctaggatggacttttttcattcagaaagccgctctggcttaaagacatgtacaaacctctcagtgccacaagagtaaagaatcacgcatggaagctgcacaagaagtcatctaatgaggacaagatcctcaacagggaccctgggtaaatgacgggaccctcacagttcccatctaaaatgaggagggggtgagacgcttaattgctcctttcaagaatgaaaaccttggcattgttattcttatcccagggacagtgaagccccaacagagaaggaggaggagagtgaagccctgccataggaggagaacccagcccacctcaggcctcctgcaaaaacacatagcataaacaataccatcagaaagaaaagcaggactgaagccagcagcccacacatccacagaggcagcgggcagagcaagcacagggccatcgttcctgcccttgtttcccagtctaattagtcacccagacctgaaaacatatcctcagggggtggagattttacaattaaataccattgtttttggtgccctctccctgggttcatcaagcaccagtcatataataccacatacttgaactcctgcccacaggggacctcccatctcctggcccctattataggatcactgggcctacctgcactgtggggccaagccctgtctttttcccaagccctcaagcacacgcatgaatgttcatcccgacttggtagggggcttttcacccttacaagatggcaaaagattcacactgctttttttaaaatttgtttttctttttaaaaatcccaacccttggatagcaagggaggtgctggaggggtagggtcaagaagagtgtgtgagaacagtaatttcccaagactgccctctgcgggactgtatttcagaaaacacactggtggggctacctctccattcacatgtactgccctagcctctccccatccccggctgatgcacttccatatctgcactgttccataacagcagtagcatgttgcagaaagcgctaggattcctccactccatcttcaaagaaaaagtcgctaataaatcacatttggtaggttagtgaacgttaaacacattagtgagcaaaagaaaataggaatgaacaagaattggtcatctacctaactgaacacaaatgaactctggcagttcggtaataggaggtaaagaaccgcgctaattgcagaacagcagcccccctaccttcccaggagcagtgtgactgggaagcagccccgtgtgtatgctggtgcaggttctaagcaaagtgagctgcccatcagttctgatgagtttgctgatgctagacatatgacatctgttctcttgctgcctgccccagttatctcccaaagttctttactgagaatgaaaagcatctttctctgtgtggtgacttcagtaggccaacaaatatttgagtttaaagcacaagactaaatagtcataggcagagcagtgctaccatttacaatttgcttacttgatgctaaaccatgggttaggcattttacagtcatatcatctagcccagcaagtcatggaagcatagttgttaaaatcatctgatactttgggaggctggggcgggcagatcacgaggtcaggagatcgagaccatcctggctaacatggtgaaaccctgtctctactaaaaatacaaaaaaattagccacgggtggtggcaggagcctgtagtcccagctactcaggaagctgaggcaggagaatggcgtcaacccgggaggtggagcttgcagtaagccgagatcatgccactgcactccagcccgggcaagagagtgagacttcgtctaaaaaaaaaaaaatcatcatctgacagataaggatacagggcttgaagaacataggtgacctgccccaagtgtccaaagccacacatccaaaatgacaaattagggttttaagccagcactcttagacttcaaagcctcttaaccattccactgccctgctgtagggcatagggagataagggggataagctatggttgccatcaaagagttaatatatcaataatatgcggatggtgaggatgatggcagctgctaggggtctacaggcgtgtaccaccatgcccagctacaattcttattattcccaaatgctactgtgtccggaattggtgggttcttggtcttactgacttcaagaatgaagccgcggaacctcgcggtgagtgttacagctcttaaggtggtgcgtctggagtctgtccgttctgatgttgagatgtgttcggagtttcttccttctggtgggttcgtggtctcgctggctcaggagtgaagctgcagaccttcacggcaagtgttacagctcttaaggcagcgcgtctggagttgtttgttcctcccggtgggctcgtggtctcgctgggctcaggagtgaagctgcagatcttcgcggtgagtgttacagctcataaaagcagcgtggacctggcagccctcggaccttgctcctgcccaagcccctgccgttgggccccggtgttgggttcggttgtgctgtctaacggctgcctggccccctcccccctcccctgtacaggaagtgtctgttggcggctaggtcccccaccagatggctcatgctgtggccactctaggagcagctggaggtggaaactcgttggtattaaccctgtgctggagggcccttaatgggttttttgatgcaattggaacaagatttatttattttttatacggggcttagataacatttctctttggtttagcaatatttattttcatttggaaaatttttagcacctatttttattagtttttagaataaagaaagtcaaacatcattttatgtttgataatgtttcctgtatgattttataagagataag

SEQ ID NO: 15083 - RNA, 5262 nt, Homo sapiens
  source 1..5262: mol_type = other RNA
gctgggattacaggcatgagccactgcacccggcccttcttttttattcttgtcatcacactctgcctgttcttatgatttaatgtttggaaagttttgccatttagtgttagattttttttttttttagtctatcttgaaataattgggacaaattgtcacttataaatacaccatttttgaaaagaatgagtggcaacaaaactatccagtagtactgacgagctccattctctcctttctgtacaaaaagagagctagacttttcctgctggggcagagatcatttgtcttcttacacagccctagaattcatcaccatcaactttaggaaaattgttctaaaagtgacacaactgtgcattgatttacacaaagtgtttacagatcaaacttgtacaagaggataaaaatatttccatttattccttttccattaataaattaccatttaagttttaattcatgaattatcatattaataaattacctactgtatgccagacacacttcttggaacttgggagattccttatgttcactgtgatgcttattttcttgctattataatcatataccttctttgtctcttcttttactcttaaaacaaaatattaaataattggaagtatccctgcacaaatggtatcacctgtaaaaatcgaggtcttcctcagagccatcagctgaagctgggtgctctctgcatctcattgttccaaatacttgctctattaatagcctcgagtgtagctctttgttggaataagctattgttaagcacctcttagataattatttgaaatcactgatttcacttttgttattctttgcctttctcatgtccatatagcagatataaaacagttggccctcagtatctgcaagttcctcatcccacagttaatcaactccctggttgaggctgagaatggggctgtcagacaggaagcctggttagggcagcagccatggaaaacttctccactaattggctgacattcagagcttgaggatcagcagctgttgaagcaaatttagtctggatataaggcagatttttcatttatttcaattaattaccacacacatcaaaacctcttctaaaaaattctcaaatgaatacctataaggaagaaagaatgcttaggtatgcatagacttttacttactctttcagagctttcaagatatgaccaacttgtttttactcatctagaaacgtgaccttttgtagaagtatgaaaataacatatctgtacttcaaaaagaatttcaatttgattcaaaggacaaattgctaatggtgaaatataggtattgtaaagcatatcgaatatgcgggcaattgcatgcgtttagtgtgtatgtctctgtatgtggaaataatgctactataaaacaatggaaaattgtcactgctgcatgcttataacagctataaagcatacagcatgcatattgcaatatctgtgcactttacaaaaagttctttatctggaagtagtgtaattctgtatgatgcagtgctctaattagaatagtgttgtattggacagaaaagtaactaggccaccccaacctacacacagtaactagttactatagaatgtgtggtgtgtatcacgtgtgcttaaaatgtatatgtttttcattttactataacacttttctttgtgtatacgaattaaaggtactcacttattgtgtgcctaacagctgctttaaaagaatacgagagggacatgttaatgcaatacaaaatcatttgtgtatacaaagtttagtttaagaaaatgggactacattattatcgcaattagatcattatttattgttgcaattcctaaatcaaactatgtcatattcttgtccaggctatttttgtggattacaaaatagctttatatcatgaaggtatgaagaaaatgaattccatattatatgtaaataaaacactcagggtgtatatgtatgtggccacatattttaggtgaagaaaaatagaacactcaaacatttacccaaataatccagtatatctttgttctctgtttgaatcccagaaaattcaaaattacttcagtgagggagaaaattaggatattaataatgacccccaccccccaaaaatttttctcttcataacattttttactataagcccattaaaacatttttaaattttaatattattatgcagcatttgggacatacaaaaaataaagtgcaataatacccatatacctattattctgcttagaaaatcaaattttgccaataattctatccccttttgaaccctttctattcatttcctctatcttccactgtggaaccgaattagttactacaaaaacatgttttaaatgactaaatttcattttctttgaaaataatgaaccaactagctacattaaatggctaataagaaatctagattttttcaaataagcaaagttgaaccatcttagttccagaatgttttacttgtacacctgcaatgcaatagaagtctaacaaaacccagcctccagcaattatttgtttatttatttattttaagaagggaaaggaggggagaaatatcccaggggttgcctgaattacctaggaatatgctttcagttccctcccctcaagtcttcacaggggggttcttgcaagtgtagttctttgaaacaatgtttagctaatgactcaagaggactactcagaaccattgaagagcacctcaaaaacagatgctaaatggacttttgtcaggttctactagtagagccatcagcagcacatcaagttggaataaattgaattgagatcaacaaaggagcatgctgtttatggatggtatcaaatcagctttcccttcccactggaattcagagacagcatatcataggatagtgagtattcctggaaatccagtgcatttcctaagctaaaggagtgtttaagaattacatggtgtaggttttatttcttttaaaattttattacttgaatataacacaattattgtgttagtggattaatcctcatcatgatctcataatttgcattgcctaaatgaataatttatgttctagtaaacaaatctataaacagagatgtttttattgggggtggtggtgatgaaacgtgagcatctggcaaccacaccttgattcattttagcccctagagtcgtggtatggcgcattaatttctcagtttgtaatttaccagctgcatttaatggaaccaattttcattacatctgttctatggttcaaagagctcttttagttgccaaagggggccagcgtcacacagattctgagaggggctaatacactgtttcttgaagtattagataaccaaggatgattcctagttttacagcaaacaaattattttgacagaggcaagttttatattcatgacttagccgttggtagatttcaaattaaaagtatagtgtgcccttttcccaggaattacatattgattttcatgtcattttcttcataatacccactgatcgcctgtctttacaatcagtggtagatttattgtttactagttaaaggaaacataattatgcttaagtaaatcctctttgtaaattacaggtggttagaagatgggtatttcttaggcaaatatggaatttataaatggttcttacatttattatagtaagcattatttacggacaagaaaaggtcatagctcttcatagtgtatagtgggaacatttttaatagtagaaatggttttgcttgggcaacttagcattcttggtgtgtaattttaatctcgtaaaaatatgtcactgttgtgtaataccaaatgtaggattccagttgaaagcaactttcaatgcaaagggttttctcatgggcagaagagaaatttgaaatgttctacagtgctttgaagttctaaagcttcagctgggagaattataaagcattaaacctgaaaagttttcacctgatggtcatgaaatagcatgccaatatgaaaactgactgtttcacttcctcaggcaatttttttttccttttcaagagtttcaaaaatatcatggatcatgttacattgagaagatcatcttagaaagactttattcgtttgaaatcattaaagtacataacataattatatttatatatgaagcttcaatgacataatctgtttgtactggagtttcactgcagttggaaaagtcgagtttgtaccaaaattagaggtaactttacgttttgtaaccatgttcaaattatcatttatatatctgtctaagagaaaaataagcagtttgccactattataatccaaatatatagttgtatgttacaacttacagcttacctaacaaatgtacatgcatctcacttgagtctcacctcaagttgaatgacctggtccatgtcacaacggaggaaggtgatgaaaatcaaactcaagatttgtgaccccaaataccaaaccttttctctctaaactatcctctgttattactgacttatggttaggttataatttcaaatttttaattctagcattgggaaacacaggtaaggcaatatgaataattttcaaacacaataatttggcattacaagaatatattccttccatcaagctgaaaatataattatgacaactagtattactaaagactacttactggcccctgaaaatccagcaggctttaacagtatggctacacaaaatgtgaagacaaagccaccgcttccgtgatagccgacaggatggagcaattgactttgccccaggaagtcagtagaaaacaaccagaagattaaatatctgagttgagactcaaagaatgagctggaattttctgggtaaaaacgtatgttaagtcttccaagcacagagagtaggatctgcaaagctgtgatgtcataaagaagcttggcagattgactgaacagtgaatttattattctttgtgcacaaactataggaaaggagaattactgagtgggggccaagaacaagaaagtaaagtgaatcattgtgaataggctaggttgtgcagcaggaacagacactcccacatctcagtaacttgaaacaagggtttatttctcactcccatacatagccatcacagtcagctcacacttctgctcctcatcatcctttctctagggcccaggctaacagaccctccaccacctgaatgctgctagagaccatgacagggagaaagagacggggcaagttgtgcactggttatttaaa

SEQ ID NO: 15084 - RNA, 6030 nt, Homo sapiens
  source 1..6030: mol_type = other RNA
gctgggattacaggcatgagccactgcacccggcccttcttttttattcttgtcatcacactctgcctgttcttatgatttaatgtttggaaagttttgccatttagtgttagattttttttttttttagtctatcttgaaataattgggacaaattgtcacttataaatacaccatttttgaaaagaatgagtggcaacaaaactatccagtagtactgacgagctccattctctcctttctgtacaaaaagagagctagacttttcctgctggggcagagatcatttgtcttcttacacagccctagaattcatcaccatcaactttaggaaaattgttctaaaagtgacacaactgtgcattgatttacacaaagtgtttacagatcaaacttgtacaagaggataaaaatatttccatttattccttttccattaataaattaccatttaagttttaattcatgaattatcatattaataaattacctactgtatgccagacacacttcttggaacttgggagattccttatgttcactgtgatgcttattttcttgctattataatcatataccttctttgtctcttcttttactcttaaaacaaaatattaaataattggaagtatccctgcacaaatggtatcacctgtaaaaatcgaggtcttcctcagagccatcagctgaagctgggtgctctctgcatctcattgttccaaatacttgctctattaatagcctcgagtgtagctctttgttggaataagctattgttaagcacctcttagataattatttgaaatcactgatttcacttttgttattctttgcctttctcatgtccatatagcagatataaaacagttggccctcagtatctgcaagttcctcatcccacagttaatcaactccctggttgaggctgagaatggggctgtcagacaggaagcctggttagggcagcagccatggaaaacttctccactaattggctgacattcagagcttgaggatcagcagctgttgaagcaaatttagtctggatataaggcagatttttcatttatttcaattaattaccacacacatcaaaacctcttctaaaaaattctcaaatgaatacctataaggaagaaagaatgcttaggtatgcatagacttttacttactctttcagagctttcaagatatgaccaacttgtttttactcatctagaaacgtgaccttttgtagaagtatgaaaataacatatctgtacttcaaaaagaatttcaatttgattcaaaggacaaattgctaatggtgaaatataggtattgtaaagcatatcgaatatgcgggcaattgcatgcgtttagtgtgtatgtctctgtatgtggaaataatgctactataaaacaatggaaaattgtcactgctgcatgcttataacagctataaagcatacagcatgcatattgcaatatctgtgcactttacaaaaagttctttatctggaagtagtgtaattctgtatgatgcagtgctctaattagaatagtgttgtattggacagaaaagtaactaggccaccccaacctacacacagtaactagttactatagaatgtgtggtgtgtatcacgtgtgcttaaaatgtatatgtttttcattttactataacacttttctttgtgtatacgaattaaaggtactcacttattgtgtgcctaacagctgctttaaaagaatacgagagggacatgttaatgcaatacaaaatcatttgtgtatacaaagtttagtttaagaaaatgggactacattattatcgcaattagatcattatttattgttgcaattcctaaatcaaactatgtcatattcttgtccaggctatttttgtggattacaaaatagctttatatcatgaaggtatgaagaaaatgaattccatattatatgtaaataaaacactcagggtgtatatgtatgtggccacatattttaggtgaagaaaaatagaacactcaaacatttacccaaataatccagtatatctttgttctctgtttgaatcccagaaaattcaaaattacttcagtgagggagaaaattaggatattaataatgacccccaccccccaaaaatttttctcttcataacattttttactataagcccattaaaacatttttaaattttaatattattatgcagcatttgggacatacaaaaaataaagtgcaataatacccatatacctattattctgcttagaaaatcaaattttgccaataattctatccccttttgaaccctttctattcatttcctctatcttccactgtggaaccgaattagttactacaaaaacatgttttaaatgactaaatttcattttctttgaaaataatgaaccaactagctacattaaatggctaataagaaatctagattttttcaaataagcaaagttgaaccatcttagttccagaatgttttacttgtacacctgcaatgcaatagaagtctaacaaaacccagcctccagcaattatttgtttatttatttattttaagaagggaaaggaggggagaaatatcccaggggttgcctgaattacctaggaatatgctttcagttccctcccctcaagtcttcacaggggggttcttgcaagtgtagttctttgaaacaatgtttagctaatgactcaagaggactactcagaaccattgaagagcacctcaaaaacagatgctaaatggacttttgtcaggttctactagtagagccatcagcagcacatcaagttggaataaattgaattgagatcaacaaaggagcatgctgtttatggatggtatcaaatcagctttcccttcccactggaattcagagacagcatatcataggatagtgagtattcctggaaatccagtgcatttcctaagctaaaggagtgtttaagaattacatggtgtaggttttatttcttttaaaattttattacttgaatataacacaattattgtgttagtggattaatcctcatcatgatctcataatttgcattgcctaaatgaataatttatgttctagtaaacaaatctataaacagagatgtttttattgggggtggtggtgatgaaacgtgagcatctggcaaccacaccttgattcattttagcccctagagtcgtggtatggcgcattaatttctcagtttgtaatttaccagctgcatttaatggaaccaattttcattacatctgttctatggttcaaagagctcttttagttgccaaagggggccagcgtcacacagattctgagaggggctaatacactgtttcttgaagtattagataaccaaggatgattcctagttttacagcaaacaaattattttgacagaggcaagttttatattcatgacttagccgttggtagatttcaaattaaaagtatagtgtgcccttttcccaggaattacatattgattttcatgtcattttcttcataatacccactgatcgcctgtctttacaatcagtggtagatttattgtttactagttaaaggaaacataattatgcttaagtaaatcctctttgtaaattacaggtggttagaagatgggtatttcttaggcaaatatggaatttataaatggttcttacatttattatagtaagcattatttacggacaagaaaaggtcatagctcttcatagtgtatagtgggaacatttttaatagtagaaatggttttgcttgggcaacttagcattcttggtgtgtaattttaatctcgtaaaaatatgtcactgttgtgtaataccaaatgtaggattccagttgaaagcaactttcaatgcaaagggttttctcatgggcagaagagaaatttgaaatgttctacagtgctttgaagttctaaagcttcagctgggagaattataaagcattaaacctgaaaagttttcacctgatggtcatgaaatagcatgccaatatgaaaactgactgtttcacttcctcaggcaatttttttttccttttcaagagtttcaaaaatatcatggatcatgttacattgagaagatcatcttagaaagactttattcgtttgaaatcattaaagtacataacataattatatttatatatgaagcttcaatgacataatctgtttgtactggagtttcactgcagttggaaaagtcgagtttgtaccaaaattagaggtaactttacgttttgtaaccatgttcaaattatcatttatatatctgtctaagagaaaaataagcagtttgccactattataatccaaatatatagttgtatgttacaacttacagcttacctaacaaatgtacatgcatctcacttgagtctcacctcaagttgaatgacctggtccatgtcacaacggaggaaggtgatgaaaatcaaactcaagatttgtgaccccaaataccaaaccttttctctctaaactatcctctgttattactgacttatggttaggttataatttcaaatttttaattctagcattgggaaacacaggtaaggcaatatgaataattttcaaacacaataatttggcattacaagaatatattccttccatcaagctgaaaatataattatgacaactagtattactaaagactacttactggcccctgaaaatccagcaggctttaacagtatggctacacaaaatgtgaagacaaagccaccgcttcctaggaaaccagataaaaataagagattaggcatcatttcaggggtatgcttaggcaatgcttgatatcatgtctggctctcaatgacacagaggcattctaaagtcaaaatcatttgttcatccacaaagaaacagttaccgtgtttctctaatcaccaagtgttgcatttatttgagtaaatagaaatcaatagggtctggggtctgtcaccaagttcaagtctaagaagaaatatcaattgtctcatgtatggtacaatatttaatgaacaaattcaaacaagcaaaaacaaaaacactaatatgagacaatttaatcactgttaaatgactataattttagtgtctatgaagacactttcataaaccaattaaaatatgtatggaatatctactataaattaagtctaggtgctgaatgatagagatgttgtatagcaattcgtgataagatccttgcccttaaagaatttacttctacttgggaggatgaagtaagcaaatctatgacctgatgaacatcatagtgggattgaaccatttctataaaaattacaatataatcatgtatcctttttaatatttcagacatataaaacaggacatgtcttcatgtagaactttaataagaacttaatgtcaactatgttaaaatgtatcctacatataatttaaaataagaaatctagaactctatatgtaatcattttaagatgcgtgcttctcaaattctagcccttttgaaatttggatttatcttacaaacggtggcatctgagcattgtgtcatagtttgacagttattatttttcttagtgatacacaaagtaatagtgcatcataaaatcaatgataacttagagatgataaaataagagtttataatataaaaatataccccaggtcacctaatgtaggatgaatgtacaattttaactgtttttaaaattccacatatagtattaaaataccgatcacctgcttttatcactctgctgaccactttgtagataccattttacttaatcttccaaaaatttctatgaaacaaatcttgttgttgctttatagataagaaaactgaggtcagagagcttaaattacttgcccaagattataaaggagacagggtatgttaaactcatgggtttttttttctatttaaaataaaatatttcaacacatcaaccataatgagatggttaatttcataattattttatttaccttcttaaaatttggatttttttggaaatgatttagatgatataggtctcttta

SEQ ID NO: 15085 - RNA, 2375 nt, Homo sapiens
  source 1..2375: mol_type = other RNA
gctgggattacaggcatgagccactgcacccggcccttcttttttattcttgtcatcacactctgcctgttcttatgatttaatgtttggaaagttttgccatttagtgttagattttttttttttttagtctatcttgaaataattgggacaaattgtcacttataaatacaccatttttgaaaagaatgagtggcaacaaaactatccagtagtactgacgagctccattctctcctttctgtacaaaaagagagctagacttttcctgctggggcagagatcatttgtcttcttacacagccctagaattcatcaccatcaactttaggaaaattgttctaaaagtgacacaactgtgcattgatttacacaaagtgtttacagatcaaacttgtacaagaggataaaaatatttccatttattccttttccattaataaattaccatttaagttttaattcatgaattatcatattaataaattacctactgtatgccagacacacttcttggaacttgggagattccttatgttcactgtgatgcttattttcttgctattataatcatataccttctttgtctcttcttttactcttaaaacaaaatattaaataattggaagtatccctgcacaaatggtatcacctgtaaaaatcgaggtcttcctcagagccatcagctgaagctgggtgctctctgcatctcattgttccaaatacttgctctattaatagcctcgagtgtagctctttgttggaataagctattgttaagcacctcttagataattatttgaaatcactgatttcacttttgttattctttgcctttctcatgtccatatagcagatataaaacagttggccctcagtatctgcaagttcctcatcccacagttaatcaactccctggttgaggctgagaatggggctgtcagacaggaagcctggttagggcagcagccatggaaaacttctccactaattggctgacattcagagcttgaggatcagcagtggcccctgaaaatccagcaggctttaacagtatggctacacaaaatgtgaagacaaagccaccgcttcctaggaaaccagataaaaataagagattaggcatcatttcaggggtatgcttaggcaatgcttgatatcatgtctggctctcaatgacacagaggcattctaaagtcaaaatcatttgttcatccacaaagaaacagttaccgtgtttctctaatcaccaagtgttgcatttatttgagtaaatagaaatcaatagggtctggggtctgtcaccaagttcaagtctaagaagaaatatcaattgtctcatgtatggtacaatatttaatgaacaaattcaaacaagcaaaaacaaaaacactaatatgagacaatttaatcactgttaaatgactataattttagtgtctatgaagacactttcataaaccaattaaaatatgtatggaatatctactataaattaagtctaggtgctgaatgatagagatgttgtatagcaattcgtgataagatccttgcccttaaagaatttacttctacttgggaggatgaagtaagcaaatctatgacctgatgaacatcatagtgggattgaaccatttctataaaaattacaatataatcatgtatcctttttaatatttcagacatataaaacaggacatgtcttcatgtagaactttaataagaacttaatgtcaactatgttaaaatgtatcctacatataatttaaaataagaaatctagaactctatatgtaatcattttaagatgcgtgcttctcaaattctagcccttttgaaatttggatttatcttacaaacggtggcatctgagcattgtgtcatagtttgacagttattatttttcttagtgatacacaaagtaatagtgcatcataaaatcaatgataacttagagatgataaaataagagtttataatataaaaatataccccaggtcacctaatgtaggatgaatgtacaattttaactgtttttaaaattccacatatagtattaaaataccgatcacctgcttttatcactctgctgaccactttgtagataccattttacttaatcttccaaaaatttctatgaaacaaatcttgttgttgctttatagataagaaaactgaggtcagagagcttaaattacttgcccaagattataaaggagacagggtatgttaaactcatgggtttttttttctatttaaaataaaatatttcaacacatcaaccataatgagatggttaatttcataattattttatttaccttcttaaaatttggatttttttggaaatgatttagatgatataggtctcttta

SEQ ID NO: 15086 - RNA, 3194 nt, Homo sapiens
  source 1..3194: mol_type = other RNA
gctgggattacaggcatgagccactgcacccggccgaaatggacaggtttttaaatgccatgatgatcagaacagcttgatgactaataataacatgttactgttcccattcttgtggaaaaggatttgggtttttcttttagtgcttttagatataatctcatgaactcttacaatattctaacaatcataaaaagactgtgctataacctgtgaaggtaacttctaaagagaagttgcaaaaatatttttaaaaataatgaagaaagtactcatatgataaagttaaggtataccaaggcagagcctctcaacttgtgtactaggaatgctgcaaagagtcccctcagctcatggggaagaaaagtggggccttagtgcaaccagagcgcatgggcttgtgctaagtggtctccagattactccaatgtgccatacaaatactgtttcctaagtgtgtaaaggaatgtaagattgggaaacatctacttagtggaaactgctaataagaaaaccagaagaactaggttcaactccttgtcaactcactagctgagtgatcttagttaaattattttaacctctttggaacacttaggctcctcatttactaaatgaaaactggagtatttcaatggtctcttctagttctaaaactcataatttcccttacattgacacttcataatataaagcagtagtcattactcatttaattaaaaactcttaattcagatattcaataactatttgttatttatggaacctagtctgcatgtgaggatctggaaaacaaatatggaagacaaaatccctaaatagatcttattgtgaataatctttgcatcccttttaggaggttaaatagtaaagccttctgaacagtgcccaaataaaggaattattttgcacagataatggaagcttgcctatgcataataaatattttttactttagctataatcagagcttctaccaatatataagaattttctcctctatatccctcaactgctttaaaaagaaaaattatggtcatttaaacttactcacaaattacatttataattaaaattgatttccaaagtataaatttataaaaatagtttaaagactctcaaaaggacttcatcttatattcagattatagcaagaaaatcaatgtgctccatatattttacccatgatgaaacttgtcccatatccattactatatatatatatatatagtttaactgggtggggttgggagggagaaggcatgaattcaaaattttaattaaatattacataatttaatgttctcccaagaatttgagctgacattttcatatgaatacaatttcacaaaggttacaaatatatatcaacttacaacagaaggaatcatttagtattttacagtgtttttaaaaatctagctccataatcactcttgaaaaaaaaaaatccttaccacataatatgaaaagtccacatttctctggaaatgcatagtcacctaatagtaaggtccaaaatgagaattactatctccagaagagggtggaggaggcagtggtggagggggagggggtgggggtagggagtatggtaagttaagtaatggatgagcagccatgtttggtgtagcccaacccatgtttacaggtgggggtggtggtgggggtggagggcggaggggaaaattatgcatgtcaaacactggaagaggaaaggggtattgtggcataatgggattattttgtctctgagaaggaaatcctgaagtctcctgagataccatatgttctgagttatagaaatgctgaggtggaggcctgccatggcaagatcgagggtatctggccctggaaaatcctcgtgtgaattctctgttacgatatccttttgcatgctctgaagcagagctatgagcattccaattctgatgtacttcagtaaaatcttcaccaggctcattaaattcagatttgagttttttccggccttgaatctgagattttttcctctgtttggcttccttctctttttcatcatcactaaaatctaaggcctctggtggtggttcctgatcattcttccatgatgcatctgatcccttatcctgttttagtttttctgtgaatatatattgagtgaaatctttcattgatggagcaaaatacatagtctcctttattttaatacctttactctcaatgtgatctgaagaattaaaccgtaacacataaaatggatgtgcaacaggtccaaatatctcgaatatctttcctgctgcttgtcgatcacttttaaaaattacagtctcctcattaactggaggtaggttagtcatagattcaattattactagttgttcaataatacttgaaaccatcccaagaggctttaactcaatatcttcaggcagaataatagtgagttcttcaacagaaggcagttcctgatgctattaggtgagccttcacttttcagatatggttggaaagtaggatccaatccctggagtactgagagccatgactgaattttttttttctctatagattaagaagtaattcatcttttgttttaagaggaaaattcttattttccttctcaatttgtaaatcatcatctccatctgacagcactggaggaagtgatatacaagaggaagaagacgacgatgaggaagatgaagaggaagacgatgaacttgaactatctgaatctgtttcactgtccgagtccgaatccgagtccgaggtctccaaggagtccggcgcccgcgcaggctctgcggctcctggggaggtgacgcagtctccgcaggccggcgattcagccggtggctgtggctgcggcgccggggtcccggccgcgacggcgttcagaacgggctgcagaggctgctccccggcaggcttaacctccacggtctgcccagcgtccggggacccctcaaacgactgtagcggcggctgtgtccctggcacaggggcagagcccggagacggagccgccggaccttccccaactccaaagtcggtgccattgaatttcagagtttccagctgagcggcggcggcctccactacctccatcgcaccgcgccagaaaccgggtcggcctcaggattggggcccctggacaagctcacggctctctccagaaatagaaaaacaacttaggcaaccgcagcaacact

SEQ ID NO: 15087 - RNA, 1242 nt, Homo sapiens
  source 1..1242: mol_type = other RNA
gctgggattacaggcatgagccactgcacccggccgagaataaggtaaactttaacttggcactgtaaaggtcaattttcaggcagtcttagagtttagcaatttctctagtgtataaactgattcttaacgatttaaagaaaattatattcaagtggcaaatttggaggcaacaggctacttcggagtccatgatatgagatggcgttttaaatacatgttttatcttcaaggttttcagctcttttctctggaccatctggatataagttgatagctgtcacaggtatgacgtccactttatccaactgaagaattcctttgtattcagaaactgggaaaaacacctttaagatggttattaccacagctgctcctgtaattccaaccaccatgatgttcaaaaactgaaagaatactgggaaaacgttgctccagaacctacacagatcttttctaaacttttccatccactgacacattaccttatatgaagatggcggctctgctctgagaggagtttcaggtaacttgccaggtaaaacatcttcatctacagtggtttccacattcctgataagatactggctagtggtttgcagtgaactaacactttcttttttggagaggttaggaagggtaaataaaatgtcactgtctcgagaaatagagtagagcatgctttcttccaaagggagggtatagtttgaatgtctgagtactccccggttcttaactaaaatatcaatttcagtgacatccttttgctgaacttgttttccatcaatctctactacctcttcttgaatgacaattagttgcaaactggaaccagatgtcataggccactcatgaactaaaatccttacactgacaattccaaaatattctttttcctccaaattttcaagattttcattcttcactatcaaagtctgacagcttattcgggttacaccactatttacaggtaagtcatttacatacacctgtccactctcataggttatgttaagaacaacctgctgtttagatatgtccccatcatctttcagtgtagttacattaattctgatgccgtcctgtggggctccggacagcggcggcggctcgggggcgcccgtcgtcagccagccggaggcgggtagcgccacgaacagcaggagccggagggcgagcgaccccggtggagcgccctccatcttggacaacccgggcagagggcagccgcggccgggaggt

SEQ ID NO: 15088 - RNA, 7718 nt, Homo sapiens
  source 1..7718: mol_type = other RNA
gctgggattacaggcatgagccactgcacccggcctaaaaatgattacttcttataaaaaggatttcttccccttcacaacactcagcttcctttttctttcctggtaactatgggtctggtgttgtcataaggatctaccttccacatgctggacagtgggggttgctgcttgaggagactcaggccagatacagatcactgtggggaacactaagcttacttggttagagcacggcactaacatttctgcctctgtgagtttgattccaccacataattttttaaaagtgcttttccatggccccttagtgtcaaccattcttacgaaagatgtgagcaacagtgtacatgttttggcaaaagtcgtgacaaatagcaccagcatctgccgccctaggtggacctgtggcctcatcttggcagcctgtgagttgggcagagctgtgacgaggcatggttctgtgccggctggcagggtctgtgatatggcagcactgtgatccgtactggaaagacataatggcatgtcctgtgaacagcagatacagaaggctgagtggggaagcgacccaggggtattgccacacaaagcgataggccagctaagtaccaggagacaaactgaggtgggaggaaatagtgacttcatggcctcattctttagacttactccttaaaaggactagatccggggagggaaaagtaatcacaaaatgttcaagctaataagagatatttttggtcttaaaactaaggtttaaaaattcccagtactgaaaacaactttctcactcttttgtgaattggacaatttgaccattatgaagatcttttgaaacaatcaatgaaaatgctactaagtgtcatgaattattttttaatatttttgagtaaggggagtactttaatactgattgggcccatgtaatagacaatatgtcacttttggtgtaactatttttatgaggaaaaaacattaacaatgaaatgccaattcctatttataacagaccttttttgtttagatatatttcaagtttccccagaaaatatgaggcatgttaatacaacacaattatttaaaaggtaacaacattaaaacattttactgctgccaatgtaacatacagacatctgagaaatgacaattatcaacctttgtaatacatgattacgcaaggtgatatgagacaacccaagggtagcacattttaaaaaatacccacagtatataactggcaagccaaaaaaacttcctgtattaacagaaatgattactgaattgaacgctttttaaaaaatgtcttttaagcaaaaattgtatttctcttttcatgttacattaagaatttggaatattatttttcagttaagtcaaagaagaacttgaaaaaaataatgacatacttcacaaatagtagagactagatgtaaacacagacctaaaaatgagcagtaggataaaaaaaaccatgaatgtttgttctcttctggaccatgattttaaattttaatttggtaattccagataaagattctaatttatcatggtttctggactgatctctttaagttaaacactttcagtctaagtgtgttcaactggcctaaagccactgtcaggaaaaatgtatttaggaaaatatacaacacagggcaagaaaatactactgtagaataaggaatttagatttcactgcaaataaagccatatttgatattaaagacacatgttcctattttcacatcagtcatttattaacaccaaacattatactttaacttttccccattacacagtacaataagcctgtcaagatttccaggaagtaatcatcagtacctactgtgcttccagcagccaaagctaagctggctgggtaccagaaatcaacaccttcaggagaatggcatcacaagattgcatggactcatattaactattacaaggggcactggaaaaaaaggtcatttgctcatttacaaaatcctaattgaactaaagctctgtaattatagccatggtatcagaccagctttttcgcacatcctatcacatcgctgcctgctgatgttttacactgcctataaagtctcataattttaaaagggaatgaaacagaatgccacaggtgaccgacctctgctcctgctacttgggagtcacgttgtcttggcttcgtcctggctcaaggttactagtctcttgctgctttgggccaaatctcttatctctttacatttcctcctctcaggctgagtcaaaagtaagtcacatgtataacaaaactgtcttaaaataccactgtttttcagccaagagaattacggatgcaatttaaagtctaaatgtattaattggaaaaattaaattagagcaactcaaggttttcctgtaattaccaaatgaaactgattgaaaaactgttccttctaattctgcttttccaacaaaagttcatcacactagcaggataaacattcaaaatacataatagaacatatcctaattaagcaccagagttgtgtcagagccaagtatatacacacacacacgtatacgtgtgtgtgtgtgtgtgtgtgtgtgtagtttattactggttaagtaaatgctctaattagcaaaaatcatgagaaatatatacagtgatataatgcggttaaattttagttctctgtgttaactacttactgttaatttagtactcaattagaattaactctgggattttgagggcagataaatcagtaattagcctttatcccagaaagaatagtggtagcttcaaaagcttcaacagacctaatgatgtaatttattcaggacagaaaaaaaaatatgtagccaacattcttgcaagaattactttcttatggaatttaagatttcctcaaatattttcttttctatatagcgttttgttcttgtgtagttatctgcctaggatacagacaggatattgagactatttcagaaagtagacacactaaaaacatttgacaaattaaaaaaattttgcataaaacaggttaccctttcctgctgactatacttaagaaataccaaagtagcatacaaaatgcttctaaactttcaaaatatctgaataaaaacaaagatcctacttttaactgagatagatttataattcttacttacaagataaaaaaatttcctaaaatttatttttaaatttcacataacctgctataattcgctgtaaaaaatggatgtcaaaatagaattttaaatatacaaattgtttttgataactacctttcatacattttatttaaactgtagcattagctcaagatgaaactttttaaaagaaaccataggcttttgtccaactcaaagattcaagcccagattctgaacaaagtaaatgtgatgaaatttatgaaaaactatactgtacagtcaaaacagtgatggtgcctcagtaaataacttcagtaaaatatccagtgctccaaatagctgagccatctttctaaggttcactctgcttctctcccccagccctcatggcctgtgctaccatctattcttttagcgtttatgctggagggccttatagttcctttaaaagtacactgaaaatactttatatcacagcttattctaaccactggttctcaaattaaaaggtatatttcagtgcatatttcatagccacattgcagaactaatatttgaaaactcttgggggaaattttggtaacaaaattgcaaaatgacatgattatttatgagctttctataaaaagttttttttttttttttttttttactttagagatcatacctactttcctgcctttttgataagtaaggcatgaaatgaaacaaaagttttgagctgtaaggtgcctataaaggatgtcactacagcattcacaatgctaggtgtgtaagatgacatggctgttaccatgtactaaagaaccccatcatgtgagagatcgctcaaagtcattaacacaaagcagtgaaaatcatccagcaaagcagtgcttatgagagactagaattcagagaaatgcaaggtacgaacttctctctaatccaagggtattctgctgtgatcttctaatcagtgatgattgtgcttatgcacacgacatcttcatgggagagaccaggctgattgcaaaataatgacaaccaaccagtttacctcaacatagctcactctgcaatgtcagacatgcagtgtagagcagtcacaaagtcaagccatgaatacagggatggaaaaacattccagtgagctggtctctacaatttttaagacacttcatcctcccaattatattctttgtcataaagaggaaaaacagcaagattattaaatccaaaaagtcacagatgtcacaaggggatgaaataatttcctcattttttttctttatcagtgtaggaaaagctgtctttccatagcccacactcataatagcacttcaactaggctcctttgaaaatgaaaagtgaacaagtttcctaatgctggccttataagatctaaagagatgattaaattcaaaccaggctgagctcttactctgagctatttcagccactgatgtttgtaaaatataggaagaagattccaataggcaatttgcattggcaagcactggactacagaattcatcactgttttctgaaaaaatataattaaaccttaatggaattatgacacttttatgaggtttataattcacagccacctctcatcatattttgttcttctttccatttttaccatttcaaatattgcaatattgcccaccataaaccactgaaaatgattatttatgtatattccatttatttctctagggggtctaggtaatttgaatcaggagctccaagtaccatttaaaaaggtgagtctttaaaaaccatcagtgttttaaacacttgattagaaaaaagataacagctccttgtagtgatctagcttatgtgctttatggtatcttttcaaaaggagagtataaatcattgtacataaaatcaaaatagctaatatacatttttttctggcacttttgagaaattaggcattgaacataaaacatcttataaacttacataacaaaaataaatgtttacattttaatcttagattaccttagggtagcagttaacttatgagatgccacactgttggtgtgggcagcggagaccatgggaaatacacattcatgtccacagcccttcagcgatggatgcatggctgccgtccaaatatgtggtctgtgtcccaacataaagattaaggctctctgttttgaaggaatgagttctgggcttaaacaagtctagaagtaccacaatactcatggaaaatactgaaaagattcggacgagttttcaaacactgggggaaacacgtttttgactagaaaaataaaataaagcatctaaaactgacttcaagtactttggggagaggctgctgatatcgaatgccaaaataagaaggaacaaagacagaagagactccagggacgtccctccccatcccttcacccgcagggtccagatccccaggtgctgatgcgcaactctttggggaggactggcgagctgggcagaaagcagcagccatggtttgtcaccatcctaaaacacctatattgagggcaaaggccaagctttgtgtgaaaatttccttgggatgaaccacaggaatctggacatttcaagggggaaaaagccttaaagtcagtagcagacagagaaaaggaaagagaggaagaaaaacctgcttttctgaatggcagtactttaggccgggggcattgtggtccttggtgagtgcagcttttccatacagcttggctttcctcactaatgagatgagaccactgacagctgggatcttttgtgggtggtgagggtgcagcagggagatgtgcttgggtgtacctgtccatctggcaggcaggggcacactcaggtgcagcctagtccgtacctctctgtctcagaaactgaacaactgggagaacagtcgacagggcctctccaaccatcttcaggtgactaaagcagcatatgaagtataggtttgtgtcacttcttctcttccacagaagaaacgtctccagacactgatcacaggctacccagggttgtcttctgggttgctagagcctggtaatatctctgccttgctgcaagtcacttatgctctcgtagtcgttctcctttgggacgagaccgtggtggccattggtccccagggtggccttttcttcctctctgttgagagtctgtatcgcttcataatcaggctctggctcctcgctgggcctccctgctggtggaagtgtgctgtttggagttttttcgaagtctttaacagtagcatagagatcattacaggaggagggtgacctctgtgggtccccttgaatggaggtgtaggtggactccggaactgtaagcgactgccccgatttattcactaactgtccaggtttatttactgatgagtacatagctgagatctcttcttctgtgagagtggggtcttcttcccgagacttgtatgacaatgagctaaatctcttgttagtttcactggtcgtgtctgtggcactctcttccgcctctcccccttccttctcctgaaggttttcattctcgtccagaagcttaacagggacaggtggtggggcctcctcttctggatcacatgaatttccaaggatactctctacattaacactttgacgacattttttgtttctgtccaccgaggcatattcagcaaactcagctttgccttcagtctggggccctgggagctctttcgaggcagaagtagattttgccttgccactgtggcctttctccaggtgtgcagctgcagccacctccttgatctctttcacagtttcatacaagcagtcctccaccatgttttcttgggaggagctgtccttgagcacttcatagggcccttccatccccagcccctggtccccgtccacacttctcgccgtgagcatggtatccactgcgctctcgggagggattctgggcagctcccgactctgatgacattttggtttccctgtgctgtcctgggaatccagcagatccgaggccgatgtctggacttcctcgtaatgctgcatgcaggtcagagtactgtcctctgaaagaatgtccccattggtgagtgccccattctgctcactgctggcaggagcatctgttgccaggctagtaactgaacggctgaacatctccttgtctgaaggcacgttcatcaggttctcatggtccccactatgctgtcgcggcttcttttccctgtcacaactagagcacaggaagatgaggaaggtgatgacgaagaaaatggcgacagcagccagacttccccacagggtgatctgcatctgtccgctgcccagcaggctccccgcgggccccatggcaggagcaggcactggcaccagccgagggaatcagtcagtccttcaaaggtggtgacatggaggcagagagctgtgtcattttcgtttgcttcagtgataaagctgtgactgttttcagccatccctgagcacagacatcaagacggcaggggtggcttcgcagcaaaccagggtgcctcaatgtatgcagagagagttctgagagatgaagttgttttcctcaatctttgaatcaacatgaacgtcttc

SEQ ID NO: 15089 - RNA, 7729 nt, Homo sapiens
  source 1..7729: mol_type = other RNA
gctgggattacaggcatgagccactgcacccggcctaaaaatgattacttcttataaaaaggatttcttccccttcacaacactcagcttcctttttctttcctggtaactatgggtctggtgttgtcataaggatctaccttccacatgctggacagtgggggttgctgcttgaggagactcaggccagatacagatcactgtggggaacactaagcttacttggttagagcacggcactaacatttctgcctctgtgagtttgattccaccacataattttttaaaagtgcttttccatggccccttagtgtcaaccattcttacgaaagatgtgagcaacagtgtacatgttttggcaaaagtcgtgacaaatagcaccagcatctgccgccctaggtggacctgtggcctcatcttggcagcctgtgagttgggcagagctgtgacgaggcatggttctgtgccggctggcagggtctgtgatatggcagcactgtgatccgtactggaaagacataatggcatgtcctgtgaacagcagatacagaaggctgagtggggaagcgacccaggggtattgccacacaaagcgataggccagctaagtaccaggagacaaactgaggtgggaggaaatagtgacttcatggcctcattctttagacttactccttaaaaggactagatccggggagggaaaagtaatcacaaaatgttcaagctaataagagatatttttggtcttaaaactaaggtttaaaaattcccagtactgaaaacaactttctcactcttttgtgaattggacaatttgaccattatgaagatcttttgaaacaatcaatgaaaatgctactaagtgtcatgaattattttttaatatttttgagtaaggggagtactttaatactgattgggcccatgtaatagacaatatgtcacttttggtgtaactatttttatgaggaaaaaacattaacaatgaaatgccaattcctatttataacagaccttttttgtttagatatatttcaagtttccccagaaaatatgaggcatgttaatacaacacaattatttaaaaggtaacaacattaaaacattttactgctgccaatgtaacatacagacatctgagaaatgacaattatcaacctttgtaatacatgattacgcaaggtgatatgagacaacccaagggtagcacattttaaaaaatacccacagtatataactggcaagccaaaaaaacttcctgtattaacagaaatgattactgaattgaacgctttttaaaaaatgtcttttaagcaaaaattgtatttctcttttcatgttacattaagaatttggaatattatttttcagttaagtcaaagaagaacttgaaaaaaataatgacatacttcacaaatagtagagactagatgtaaacacagacctaaaaatgagcagtaggataaaaaaaaccatgaatgtttgttctcttctggaccatgattttaaattttaatttggtaattccagataaagattctaatttatcatggtttctggactgatctctttaagttaaacactttcagtctaagtgtgttcaactggcctaaagccactgtcaggaaaaatgtatttaggaaaatatacaacacagggcaagaaaatactactgtagaataaggaatttagatttcactgcaaataaagccatatttgatattaaagacacatgttcctattttcacatcagtcatttattaacaccaaacattatactttaacttttccccattacacagtacaataagcctgtcaagatttccaggaagtaatcatcagtacctactgtgcttccagcagccaaagctaagctggctgggtaccagaaatcaacaccttcaggagaatggcatcacaagattgcatggactcatattaactattacaaggggcactggaaaaaaaggtcatttgctcatttacaaaatcctaattgaactaaagctctgtaattatagccatggtatcagaccagctttttcgcacatcctatcacatcgctgcctgctgatgttttacactgcctataaagtctcataattttaaaagggaatgaaacagaatgccacaggtgaccgacctctgctcctgctacttgggagtcacgttgtcttggcttcgtcctggctcaaggttactagtctcttgctgctttgggccaaatctcttatctctttacatttcctcctctcaggctgagtcaaaagtaagtcacatgtataacaaaactgtcttaaaataccactgtttttcagccaagagaattacggatgcaatttaaagtctaaatgtattaattggaaaaattaaattagagcaactcaaggttttcctgtaattaccaaatgaaactgattgaaaaactgttccttctaattctgcttttccaacaaaagttcatcacactagcaggataaacattcaaaatacataatagaacatatcctaattaagcaccagagttgtgtcagagccaagtatatacacacacacacgtatacgtgtgtgtgtgtgtgtgtgtgtgtgtagtttattactggttaagtaaatgctctaattagcaaaaatcatgagaaatatatacagtgatataatgcggttaaattttagttctctgtgttaactacttactgttaatttagtactcaattagaattaactctgggattttgagggcagataaatcagtaattagcctttatcccagaaagaatagtggtagcttcaaaagcttcaacagacctaatgatgtaatttattcaggacagaaaaaaaaatatgtagccaacattcttgcaagaattactttcttatggaatttaagatttcctcaaatattttcttttctatatagcgttttgttcttgtgtagttatctgcctaggatacagacaggatattgagactatttcagaaagtagacacactaaaaacatttgacaaattaaaaaaattttgcataaaacaggttaccctttcctgctgactatacttaagaaataccaaagtagcatacaaaatgcttctaaactttcaaaatatctgaataaaaacaaagatcctacttttaactgagatagatttataattcttacttacaagataaaaaaatttcctaaaatttatttttaaatttcacataacctgctataattcgctgtaaaaaatggatgtcaaaatagaattttaaatatacaaattgtttttgataactacctttcatacattttatttaaactgtagcattagctcaagatgaaactttttaaaagaaaccataggcttttgtccaactcaaagattcaagcccagattctgaacaaagtaaatgtgatgaaatttatgaaaaactatactgtacagtcaaaacagtgatggtgcctcagtaaataacttcagtaaaatatccagtgctccaaatagctgagccatctttctaaggttcactctgcttctctcccccagccctcatggcctgtgctaccatctattcttttagcgtttatgctggagggccttatagttcctttaaaagtacactgaaaatactttatatcacagcttattctaaccactggttctcaaattaaaaggtatatttcagtgcatatttcatagccacattgcagaactaatatttgaaaactcttgggggaaattttggtaacaaaattgcaaaatgacatgattatttatgagctttctataaaaagttttttttttttttttttttttactttagagatcatacctactttcctgcctttttgataagtaaggcatgaaatgaaacaaaagttttgagctgtaaggtgcctataaaggatgtcactacagcattcacaatgctaggtgtgtaagatgacatggctgttaccatgtactaaagaaccccatcatgtgagagatcgctcaaagtcattaacacaaagcagtgaaaatcatccagcaaagcagtgcttatgagagactagaattcagagaaatgcaaggtacgaacttctctctaatccaagggtattctgctgtgatcttctaatcagtgatgattgtgcttatgcacacgacatcttcatgggagagaccaggctgattgcaaaataatgacaaccaaccagtttacctcaacatagctcactctgcaatgtcagacatgcagtgtagagcagtcacaaagtcaagccatgaatacagggatggaaaaacattccagtgagctggtctctacaatttttaagacacttcatcctcccaattatattctttgtcataaagaggaaaaacagcaagattattaaatccaaaaagtcacagatgtcacaaggggatgaaataatttcctcattttttttctttatcagtgtaggaaaagctgtctttccatagcccacactcataatagcacttcaactaggctcctttgaaaatgaaaagtgaacaagtttcctaatgctggccttataagatctaaagagatgattaaattcaaaccaggctgagctcttactctgagctatttcagccactgatgtttgtaaaatataggaagaagattccaataggcaatttgcattggcaagcactggactacagaattcatcactgttttctgaaaaaatataattaaaccttaatggaattatgacacttttatgaggtttataattcacagccacctctcatcatattttgttcttctttccatttttaccatttcaaatattgcaatattgcccaccataaaccactgaaaatgattatttatgtatattccatttatttctctagggggtctaggtaatttgaatcaggagctccaagtaccatttaaaaaggtgagtctttaaaaaccatcagtgttttaaacacttgattagaaaaaagataacagctccttgtagtgatctagcttatgtgctttatggtatcttttcaaaaggagagtataaatcattgtacataaaatcaaaatagctaatatacatttttttctggcacttttgagaaattaggcattgaacataaaacatcttataaacttacataacaaaaataaatgtttacattttaatcttagattaccttagggtagcagttaacttatgagatgccacactgttggtgtgggcagcggagaccatgggaaatacacattcatgtccacagcccttcagcgatggatgcatggctgccgtccaaatatgtggtctgtgtcccaacataaagattaaggctctctgttttgaaggaatgagttctgggcttaaacaagtctagaagtaccacaatactcatggaaaatactgaaaagattcggacgagttttcaaacactgggggaaacacgtttttgactagaaaaataaaataaagcatctaaaactgacttcaagtactttggggagaggctgctgatatcgaatgccaaaataagaaggaacaaagacagaagagactccagggacgtccctccccatcccttcacccgcagggtccagatccccaggtgctgatgcgcaactctttggggaggactggcgagctgggcagaaagcagcagccatggtttgtcaccatcctaaaacacctatattgagggcaaaggccaagctttgtgtgaaaatttccttgggatgaaccacaggaatctggacatttcaagggggaaaaagccttaaagtcagtagcagacagagaaaaggaaagagaggaagaaaaacctgcttttctgaatggcagtactttaggccgggggcattgtggtccttggtgagtgcagcttttccatacagcttggctttcctcactaatgagatgagaccactgacagctgggatcttttgtgggtggtgagggtgcagcagggagatgtgcttgggtgtacctgtccatctggcaggcaggggcacactcaggtgcagcctagtccgtacctctctgtctcagaaactgaacaactgggagaacagtcgacagggcctctccaaccatcttcaggtgactaaagcagcatatgaagtataggtttgtgtcacttcttctcttccacagaagaaacgtctccagacactgatcacaggctacccagggttgtcttctgggttgctagagcctggtaatatctctgccttgctgcaagtcacttatgctctcgtagtcgttctcctttgggacgagaccgtggtggccattggtccccagggtggccttttcttcctctctgttgagagtctgtatcgcttcataatcaggctctggctcctcgctgggcctccctgctggtggaagtgtgctgtttggagttttttcgaagtctttaacagtagcatagagatcattacaggaggagggtgacctctgtgggtccccttgaatggaggtgtaggtggactccggaactgtaagcgactgccccgatttattcactaactgtccaggtttatttactgatgagtacatagctgagatctcttcttctgtgagagtggggtcttcttcccgagacttgtatgacaatgagctaaatctcttgttagtttcactggtcgtgtctgtggcactctcttccgcctctcccccttccttctcctgaaggttttcattctcgtccagaagcttaacagggacaggtggtggggcctcctcttctggatcacatgaatttccaaggatactctctacattaacactttgacgacattttttgtttctgtccaccgaggcatattcagcaaactcagctttgccttcagtctggggccctgggagctctttcgaggcagaagtagattttgccttgccactgtggcctttctccaggtgtgcagctgcagccacctccttgatctctttcacagtttcatacaagcagtcctccaccatgttttcttgggaggagctgtccttgagcacttcatagggcccttccatccccagcccctggtccccgtccacacttctcgccgtgagcatggtatccactgcgctctcgggagggattctgggcagctcccgactctgatgacattttggtttccctgtgctgtcctgggaatccagcagatccgaggccgatgtctggacttcctcgtaatgctgcatgcaggtcagagtactgtcctctgaaagaatgtccccattggtgagtgccccattctgctcactgctggcaggagcatctgttgccaggctagtaactgaacggctgaacatctccttgtctgaaggcacgttcatcaggttctcatggtccccactatgctgtcgcggcttcttttccctgtcacaactagagcacaggaagatgaggaaggtgatgacgaagaaaatggcgacagcagccagacttccccacagggtgatctgcatctgtccgctgcccagcaggctccccgcgggccccatggcaggagcaggcactggcaccagccgagggaatcagtcagtccttcaaaggtggtgacatggaggcagagagctgtgtcattttcgtttgcttcagtgataaagctgtgactgttttcagccatccctgagcacagacatcaagacggcaggggtggcttcgcagcaaaccagggtgcctcctacaatgtatgcagagagagttctgagagatgaagttgttttcctcaatctttgaatcaacatgaacgtcttctaaggct

SEQ ID NO: 15090 - RNA, 7697 nt, Homo sapiens
  source 1..7697: mol_type = other RNA
gctgggattacaggcatgagccactgcacccggcctaaaaatgattacttcttataaaaaggatttcttccccttcacaacactcagcttcctttttctttcctggtaactatgggtctggtgttgtcataaggatctaccttccacatgctggacagtgggggttgctgcttgaggagactcaggccagatacagatcactgtggggaacactaagcttacttggttagagcacggcactaacatttctgcctctgtgagtttgattccaccacataattttttaaaagtgcttttccatggccccttagtgtcaaccattcttacgaaagatgtgagcaacagtgtacatgttttggcaaaagtcgtgacaaatagcaccagcatctgccgccctaggtggacctgtggcctcatcttggcagcctgtgagttgggcagagctgtgacgaggcatggttctgtgccggctggcagggtctgtgatatggcagcactgtgatccgtactggaaagacataatggcatgtcctgtgaacagcagatacagaaggctgagtggggaagcgacccaggggtattgccacacaaagcgataggccagctaagtaccaggagacaaactgaggtgggaggaaatagtgacttcatggcctcattctttagacttactccttaaaaggactagatccggggagggaaaagtaatcacaaaatgttcaagctaataagagatatttttggtcttaaaactaaggtttaaaaattcccagtactgaaaacaactttctcactcttttgtgaattggacaatttgaccattatgaagatcttttgaaacaatcaatgaaaatgctactaagtgtcatgaattattttttaatatttttgagtaaggggagtactttaatactgattgggcccatgtaatagacaatatgtcacttttggtgtaactatttttatgaggaaaaaacattaacaatgaaatgccaattcctatttataacagaccttttttgtttagatatatttcaagtttccccagaaaatatgaggcatgttaatacaacacaattatttaaaaggtaacaacattaaaacattttactgctgccaatgtaacatacagacatctgagaaatgacaattatcaacctttgtaatacatgattacgcaaggtgatatgagacaacccaagggtagcacattttaaaaaatacccacagtatataactggcaagccaaaaaaacttcctgtattaacagaaatgattactgaattgaacgctttttaaaaaatgtcttttaagcaaaaattgtatttctcttttcatgttacattaagaatttggaatattatttttcagttaagtcaaagaagaacttgaaaaaaataatgacatacttcacaaatagtagagactagatgtaaacacagacctaaaaatgagcagtaggataaaaaaaaccatgaatgtttgttctcttctggaccatgattttaaattttaatttggtaattccagataaagattctaatttatcatggtttctggactgatctctttaagttaaacactttcagtctaagtgtgttcaactggcctaaagccactgtcaggaaaaatgtatttaggaaaatatacaacacagggcaagaaaatactactgtagaataaggaatttagatttcactgcaaataaagccatatttgatattaaagacacatgttcctattttcacatcagtcatttattaacaccaaacattatactttaacttttccccattacacagtacaataagcctgtcaagatttccaggaagtaatcatcagtacctactgtgcttccagcagccaaagctaagctggctgggtaccagaaatcaacaccttcaggagaatggcatcacaagattgcatggactcatattaactattacaaggggcactggaaaaaaaggtcatttgctcatttacaaaatcctaattgaactaaagctctgtaattatagccatggtatcagaccagctttttcgcacatcctatcacatcgctgcctgctgatgttttacactgcctataaagtctcataattttaaaagggaatgaaacagaatgccacaggtgaccgacctctgctcctgctacttgggagtcacgttgtcttggcttcgtcctggctcaaggttactagtctcttgctgctttgggccaaatctcttatctctttacatttcctcctctcaggctgagtcaaaagtaagtcacatgtataacaaaactgtcttaaaataccactgtttttcagccaagagaattacggatgcaatttaaagtctaaatgtattaattggaaaaattaaattagagcaactcaaggttttcctgtaattaccaaatgaaactgattgaaaaactgttccttctaattctgcttttccaacaaaagttcatcacactagcaggataaacattcaaaatacataatagaacatatcctaattaagcaccagagttgtgtcagagccaagtatatacacacacacacgtatacgtgtgtgtgtgtgtgtgtgtgtgtgtagtttattactggttaagtaaatgctctaattagcaaaaatcatgagaaatatatacagtgatataatgcggttaaattttagttctctgtgttaactacttactgttaatttagtactcaattagaattaactctgggattttgagggcagataaatcagtaattagcctttatcccagaaagaatagtggtagcttcaaaagcttcaacagacctaatgatgtaatttattcaggacagaaaaaaaaatatgtagccaacattcttgcaagaattactttcttatggaatttaagatttcctcaaatattttcttttctatatagcgttttgttcttgtgtagttatctgcctaggatacagacaggatattgagactatttcagaaagtagacacactaaaaacatttgacaaattaaaaaaattttgcataaaacaggttaccctttcctgctgactatacttaagaaataccaaagtagcatacaaaatgcttctaaactttcaaaatatctgaataaaaacaaagatcctacttttaactgagatagatttataattcttacttacaagataaaaaaatttcctaaaatttatttttaaatttcacataacctgctataattcgctgtaaaaaatggatgtcaaaatagaattttaaatatacaaattgtttttgataactacctttcatacattttatttaaactgtagcattagctcaagatgaaactttttaaaagaaaccataggcttttgtccaactcaaagattcaagcccagattctgaacaaagtaaatgtgatgaaatttatgaaaaactatactgtacagtcaaaacagtgatggtgcctcagtaaataacttcagtaaaatatccagtgctccaaatagctgagccatctttctaaggttcactctgcttctctcccccagccctcatggcctgtgctaccatctattcttttagcgtttatgctggagggccttatagttcctttaaaagtacactgaaaatactttatatcacagcttattctaaccactggttctcaaattaaaaggtatatttcagtgcatatttcatagccacattgcagaactaatatttgaaaactcttgggggaaattttggtaacaaaattgcaaaatgacatgattatttatgagctttctataaaaagttttttttttttttttttttttactttagagatcatacctactttcctgcctttttgataagtaaggcatgaaatgaaacaaaagttttgagctgtaaggtgcctataaaggatgtcactacagcattcacaatgctaggtgtgtaagatgacatggctgttaccatgtactaaagaaccccatcatgtgagagatcgctcaaagtcattaacacaaagcagtgaaaatcatccagcaaagcagtgcttatgagagactagaattcagagaaatgcaaggtacgaacttctctctaatccaagggtattctgctgtgatcttctaatcagtgatgattgtgcttatgcacacgacatcttcatgggagagaccaggctgattgcaaaataatgacaaccaaccagtttacctcaacatagctcactctgcaatgtcagacatgcagtgtagagcagtcacaaagtcaagccatgaatacagggatggaaaaacattccagtgagctggtctctacaatttttaagacacttcatcctcccaattatattctttgtcataaagaggaaaaacagcaagattattaaatccaaaaagtcacagatgtcacaaggggatgaaataatttcctcattttttttctttatcagtgtaggaaaagctgtctttccatagcccacactcataatagcacttcaactaggctcctttgaaaatgaaaagtgaacaagtttcctaatgctggccttataagatctaaagagatgattaaattcaaaccaggctgagctcttactctgagctatttcagccactgatgtttgtaaaatataggaagaagattccaataggcaatttgcattggcaagcactggactacagaattcatcactgttttctgaaaaaatataattaaaccttaatggaattatgacacttttatgaggtttataattcacagccacctctcatcatattttgttcttctttccatttttaccatttcaaatattgcaatattgcccaccataaaccactgaaaatgattatttatgtatattccatttatttctctagggggtctaggtaatttgaatcaggagctccaagtaccatttaaaaaggtgagtctttaaaaaccatcagtgttttaaacacttgattagaaaaaagataacagctccttgtagtgatctagcttatgtgctttatggtatcttttcaaaaggagagtataaatcattgtacataaaatcaaaatagctaatatacatttttttctggcacttttgagaaattaggcattgaacataaaacatcttataaacttacataacaaaaataaatgtttacattttaatcttagattaccttagggtagcagttaacttatgagatgccacactgttggtgtgggcagcggagaccatgggaaatacacattcatgtccacagcccttcagcgatggatgcatggctgccgtccaaatatgtggtctgtgtcccaacataaagattaaggctctctgttttgaaggaatgagttctgggcttaaacaagtctagaagtaccacaatactcatggaaaatactgaaaagattcggacgagttttcaaacactgggggaaacacgtttttgactagaaaaataaaataaagcatctaaaactgacttcaagtactttggggagaggctgctgatatcgaatgccaaaataagaaggaacaaagacagaagagactccagggacgtccctccccatcccttcacccgcagggtccagatccccaggtgctgatgcgcaactctttggggaggactggcgagctgggcagaaagcagcagccatggtttgtcaccatcctaaaacacctatattgagggcaaaggccaagctttgtgtgaaaatttccttgggatgaaccacaggaatctggacatttcaagggggaaaaagccttaaagtcagtagcagacagagaaaaggaaagagaggaagaaaaacctgcttttctgaatggcagtactttaggccgggggcattgtggtccttggtgagtgcagcttttccatacagcttggctttcctcactaatgagatgagaccactgacagctgggatcttttgtgggtggtgagggtgcagcagggagatgtgcttgggtgtacctgtccatctggcaggcaggggcacactcaggtgcagcctagtccgtacctctctgtctcagaaactgaacaactgggagaacagtcgacagggcctctccaaccatcttcaggtgactaaagcagcatatgaagtataggtttgtgtcacttcttctcttccacagaagaaacgtctccagacactgatcacaggctacccagggttgtcttctgggttgctagagcctggtaatatctctgccttgctgcaagtcacttatgctctcgtagtcgttctcctttgggacgagaccgtggtggccattggtccccagggtggccttttcttcctctctgttgagagtctgtatcgcttcataatcaggctctggctcctcgctgggcctccctgctggtggaagtgtgctgtttggagttttttcgaagtctttaacagtagcatagagatcattacaggaggagggtgacctctgtgggtccccttgaatggaggtgtaggtggactccggaactgtaagcgactgccccgatttattcactaactgtccaggtttatttactgatgagtacatagctgagatctcttcttctgtgagagtggggtcttcttcccgagacttgtatgacaatgagctaaatctcttgttagtttcactggtcgtgtctgtggcactctcttccgcctctcccccttccttctcctgaaggttttcattctcgtccagaagcttaacagggacaggtggtggggcctcctcttctggatcacatgaatttccaaggatactctctacattaacactttgacgacattttttgtttctgtccaccgaggcatattcagcaaactcagctttgccttcagtctggggccctgggagctctttcgaggcagaagtagattttgccttgccactgtggcctttctccaggtgtgcagctgcagccacctccttgatctctttcacagtttcatacaagcagtcctccaccatgttttcttgggaggagctgtccttgagcacttcatagggcccttccatccccagcccctggtccccgtccacacttctcgccgtgagcatggtatccactgcgctctcgggagggattctgggcagctcccgactctgatgacattttggtttccctgtgctgtcctgggaatccagcagatccgaggccgatgtctggacttcctcgtaatgctgcatgcaggtcagagtactgtcctctgaaagaatgtccccattggtgagtgccccattctgctcactgctggcaggagcatctgttgccaggctagtaactgaacggctgaacatctccttgtctgaaggcacgttcatcaggttctcatggtccccactatgctgtcgcggcttcttttccctgtcacaactagagcacaggaagatgaggaaggtgatgacgaagaaaatggcgacagcagccagacttccccacagggtgatctgcatctgtccgctgcccagcaggctccccgcgggccccatggcaggagcaggcactggcaccagccgagggaatcagtcagtccttcaaaggtggtgacatggaggcagagagctgtgtcattttcgtttgcttcagtgataaagctgtgactgttttcagccatccctgagcacagacatcaagacggcaggggtggcttcgcagcaaaccagggtgcctccttggaggaaatgtttgtccagtagagtattccaagttctggcaatgta

SEQ ID NO: 15091 - RNA, 8177 nt, Homo sapiens
  source 1..8177: mol_type = other RNA
gctgggattacaggcatgagccactgcacccggcctaaaaatgattacttcttataaaaaggatttcttccccttcacaacactcagcttcctttttctttcctggtaactatgggtctggtgttgtcataaggatctaccttccacatgctggacagtgggggttgctgcttgaggagactcaggccagatacagatcactgtggggaacactaagcttacttggttagagcacggcactaacatttctgcctctgtgagtttgattccaccacataattttttaaaagtgcttttccatggccccttagtgtcaaccattcttacgaaagatgtgagcaacagtgtacatgttttggcaaaagtcgtgacaaatagcaccagcatctgccgccctaggtggacctgtggcctcatcttggcagcctgtgagttgggcagagctgtgacgaggcatggttctgtgccggctggcagggtctgtgatatggcagcactgtgatccgtactggaaagacataatggcatgtcctgtgaacagcagatacagaaggctgagtggggaagcgacccaggggtattgccacacaaagcgataggccagctaagtaccaggagacaaactgaggtgggaggaaatagtgacttcatggcctcattctttagacttactccttaaaaggactagatccggggagggaaaagtaatcacaaaatgttcaagctaataagagatatttttggtcttaaaactaaggtttaaaaattcccagtactgaaaacaactttctcactcttttgtgaattggacaatttgaccattatgaagatcttttgaaacaatcaatgaaaatgctactaagtgtcatgaattattttttaatatttttgagtaaggggagtactttaatactgattgggcccatgtaatagacaatatgtcacttttggtgtaactatttttatgaggaaaaaacattaacaatgaaatgccaattcctatttataacagaccttttttgtttagatatatttcaagtttccccagaaaatatgaggcatgttaatacaacacaattatttaaaaggtaacaacattaaaacattttactgctgccaatgtaacatacagacatctgagaaatgacaattatcaacctttgtaatacatgattacgcaaggtgatatgagacaacccaagggtagcacattttaaaaaatacccacagtatataactggcaagccaaaaaaacttcctgtattaacagaaatgattactgaattgaacgctttttaaaaaatgtcttttaagcaaaaattgtatttctcttttcatgttacattaagaatttggaatattatttttcagttaagtcaaagaagaacttgaaaaaaataatgacatacttcacaaatagtagagactagatgtaaacacagacctaaaaatgagcagtaggataaaaaaaaccatgaatgtttgttctcttctggaccatgattttaaattttaatttggtaattccagataaagattctaatttatcatggtttctggactgatctctttaagttaaacactttcagtctaagtgtgttcaactggcctaaagccactgtcaggaaaaatgtatttaggaaaatatacaacacagggcaagaaaatactactgtagaataaggaatttagatttcactgcaaataaagccatatttgatattaaagacacatgttcctattttcacatcagtcatttattaacaccaaacattatactttaacttttccccattacacagtacaataagcctgtcaagatttccaggaagtaatcatcagtacctactgtgcttccagcagccaaagctaagctggctgggtaccagaaatcaacaccttcaggagaatggcatcacaagattgcatggactcatattaactattacaaggggcactggaaaaaaaggtcatttgctcatttacaaaatcctaattgaactaaagctctgtaattatagccatggtatcagaccagctttttcgcacatcctatcacatcgctgcctgctgatgttttacactgcctataaagtctcataattttaaaagggaatgaaacagaatgccacaggtgaccgacctctgctcctgctacttgggagtcacgttgtcttggcttcgtcctggctcaaggttactagtctcttgctgctttgggccaaatctcttatctctttacatttcctcctctcaggctgagtcaaaagtaagtcacatgtataacaaaactgtcttaaaataccactgtttttcagccaagagaattacggatgcaatttaaagtctaaatgtattaattggaaaaattaaattagagcaactcaaggttttcctgtaattaccaaatgaaactgattgaaaaactgttccttctaattctgcttttccaacaaaagttcatcacactagcaggataaacattcaaaatacataatagaacatatcctaattaagcaccagagttgtgtcagagccaagtatatacacacacacacgtatacgtgtgtgtgtgtgtgtgtgtgtgtgtagtttattactggttaagtaaatgctctaattagcaaaaatcatgagaaatatatacagtgatataatgcggttaaattttagttctctgtgttaactacttactgttaatttagtactcaattagaattaactctgggattttgagggcagataaatcagtaattagcctttatcccagaaagaatagtggtagcttcaaaagcttcaacagacctaatgatgtaatttattcaggacagaaaaaaaaatatgtagccaacattcttgcaagaattactttcttatggaatttaagatttcctcaaatattttcttttctatatagcgttttgttcttgtgtagttatctgcctaggatacagacaggatattgagactatttcagaaagtagacacactaaaaacatttgacaaattaaaaaaattttgcataaaacaggttaccctttcctgctgactatacttaagaaataccaaagtagcatacaaaatgcttctaaactttcaaaatatctgaataaaaacaaagatcctacttttaactgagatagatttataattcttacttacaagataaaaaaatttcctaaaatttatttttaaatttcacataacctgctataattcgctgtaaaaaatggatgtcaaaatagaattttaaatatacaaattgtttttgataactacctttcatacattttatttaaactgtagcattagctcaagatgaaactttttaaaagaaaccataggcttttgtccaactcaaagattcaagcccagattctgaacaaagtaaatgtgatgaaatttatgaaaaactatactgtacagtcaaaacagtgatggtgcctcagtaaataacttcagtaaaatatccagtgctccaaatagctgagccatctttctaaggttcactctgcttctctcccccagccctcatggcctgtgctaccatctattcttttagcgtttatgctggagggccttatagttcctttaaaagtacactgaaaatactttatatcacagcttattctaaccactggttctcaaattaaaaggtatatttcagtgcatatttcatagccacattgcagaactaatatttgaaaactcttgggggaaattttggtaacaaaattgcaaaatgacatgattatttatgagctttctataaaaagttttttttttttttttttttttactttagagatcatacctactttcctgcctttttgataagtaaggcatgaaatgaaacaaaagttttgagctgtaaggtgcctataaaggatgtcactacagcattcacaatgctaggtgtgtaagatgacatggctgttaccatgtactaaagaaccccatcatgtgagagatcgctcaaagtcattaacacaaagcagtgaaaatcatccagcaaagcagtgcttatgagagactagaattcagagaaatgcaaggtacgaacttctctctaatccaagggtattctgctgtgatcttctaatcagtgatgattgtgcttatgcacacgacatcttcatgggagagaccaggctgattgcaaaataatgacaaccaaccagtttacctcaacatagctcactctgcaatgtcagacatgcagtgtagagcagtcacaaagtcaagccatgaatacagggatggaaaaacattccagtgagctggtctctacaatttttaagacacttcatcctcccaattatattctttgtcataaagaggaaaaacagcaagattattaaatccaaaaagtcacagatgtcacaaggggatgaaataatttcctcattttttttctttatcagtgtaggaaaagctgtctttccatagcccacactcataatagcacttcaactaggctcctttgaaaatgaaaagtgaacaagtttcctaatgctggccttataagatctaaagagatgattaaattcaaaccaggctgagctcttactctgagctatttcagccactgatgtttgtaaaatataggaagaagattccaataggcaatttgcattggcaagcactggactacagaattcatcactgttttctgaaaaaatataattaaaccttaatggaattatgacacttttatgaggtttataattcacagccacctctcatcatattttgttcttctttccatttttaccatttcaaatattgcaatattgcccaccataaaccactgaaaatgattatttatgtatattccatttatttctctagggggtctaggtaatttgaatcaggagctccaagtaccatttaaaaaggtgagtctttaaaaaccatcagtgttttaaacacttgattagaaaaaagataacagctccttgtagtgatctagcttatgtgctttatggtatcttttcaaaaggagagtataaatcattgtacataaaatcaaaatagctaatatacatttttttctggcacttttgagaaattaggcattgaacataaaacatcttataaacttacataacaaaaataaatgtttacattttaatcttagattaccttagggtagcagttaacttatgagatgccacactgttggtgtgggcagcggagaccatgggaaatacacattcatgtccacagcccttcagcgatggatgcatggctgccgtccaaatatgtggtctgtgtcccaacataaagattaaggctctctgttttgaaggaatgagttctgggcttaaacaagtctagaagtaccacaatactcatggaaaatactgaaaagattcggacgagttttcaaacactgggggaaacacgtttttgactagaaaaataaaataaagcatctaaaactgacttcaagtactttggggagaggctgctgatatcgaatgccaaaataagaaggaacaaagacagaagagactccagggacgtccctccccatcccttcacccgcagggtccagatccccaggtgctgatgcgcaactctttggggaggactggcgagctgggcagaaagcagcagccatggtttgtcaccatcctaaaacacctatattgagggcaaaggccaagctttgtgtgaaaatttccttgggatgaaccacaggaatctggacatttcaagggggaaaaagccttaaagtcagtagcagacagagaaaaggaaagagaggaagaaaaacctgcttttctgaatggcagtactttaggccgggggcattgtggtccttggtgagtgcagcttttccatacagcttggctttcctcactaatgagatgagaccactgacagctgggatcttttgtgggtggtgagggtgcagcagggagatgtgcttgggtgtacctgtccatctggcaggcaggggcacactcaggtgcagcctagtccgtacctctctgtctcagaaactgaacaactgggagaacagtcgacagggcctctccaaccatcttcaggtgactaaagcagcatatgaagtataggtttgtgtcacttcttctcttccacagaagaaacgtctccagacactgatcacaggctacccagggttgtcttctgggttgctagagcctggtaatatctctgccttgctgcaagtcacttatgctctcgtagtcgttctcctttgggacgagaccgtggtggccattggtccccagggtggccttttcttcctctctgttgagagtctgtatcgcttcataatcaggctctggctcctcgctgggcctccctgctggtggaagtgtgctgtttggagttttttcgaagtctttaacagtagcatagagatcattacaggaggagggtgacctctgtgggtccccttgaatggaggtgtaggtggactccggaactgtaagcgactgccccgatttattcactaactgtccaggtttatttactgatgagtacatagctgagatctcttcttctgtgagagtggggtcttcttcccgagacttgtatgacaatgagctaaatctcttgttagtttcactggtcgtgtctgtggcactctcttccgcctctcccccttccttctcctgaaggttttcattctcgtccagaagcttaacagggacaggtggtggggcctcctcttctggatcacatgaatttccaaggatactctctacattaacactttgacgacattttttgtttctgtccaccgaggcatattcagcaaactcagctttgccttcagtctggggccctgggagctctttcgaggcagaagtagattttgccttgccactgtggcctttctccaggtgtgcagctgcagccacctccttgatctctttcacagtttcatacaagcagtcctccaccatgttttcttgggaggagctgtccttgagcacttcatagggcccttccatccccagcccctggtccccgtccacacttctcgccgtgagcatggtatccactgcgctctcgggagggattctgggcagctcccgactctgatgacattttggtttccctgtgctgtcctgggaatccagcagatccgaggccgatgtctggacttcctcgtaatgctgcatgcaggtcagagtactgtcctctgaaagaatgtccccattggtgagtgccccattctgctcactgctggcaggagcatctgttgccaggctagtaactgaacggctgaacatctccttgtctgaaggcacgttcatcaggttctcatggtccccactatgctgtcgcggcttcttttccctgtcacaactagagcacaggaagatgaggaaggtgatgacgaagaaaatggcgacagcagccagacttccccacagggtgatctgcatctgtccgctgcccagcaggctccccgcgggccccatggcaggagcaggcactggcaccagccgagggaatcagtcagtccttcaaaggtggtgacatggaggcagagagctgtgtccttggaggaaatgtttgtccagtagagtattccaagttctggcaatgtattccctttgaaatgttgtggtgagagttctctcttctttcttggccttttcccagcaatgaagttgtggccaactgctgaaataggagaaaaatctcgtgtttttgggactcaggaggcagggagtcttcctggcggacggcgctcggaggcagcctctgcaaactccggcgcgcagcgccgccgccccggcacagcccggcagcagcggcaagtgcaggaccaggcgccgccgctctgcaccagtcgccttggctcagctgtgccgggcgccgggcattcgccagggcacacgactcagcgaggcggcggctgggactgaggctactgcacccggccgcgcggacccgagcgctgcagctgcctccagccccggagcgcggcgctccgagcccctggtgggtgtctctggctccaagggaatcacggctcaattagggacctgccaggagaaaaaccgatgcgctgccgcaggcagagccgccagcccgcccccagtcggctggtcacatcgcgggcgcgcagacggacaagcgagcgggagggtaccgcagccagcactcgccgccgcgccgcggagaat

SEQ ID NO: 15092 - RNA, 8111 nt, Homo sapiens
  source 1..8111: mol_type = other RNA
gctgggattacaggcatgagccactgcacccggcctaaaaatgattacttcttataaaaaggatttcttccccttcacaacactcagcttcctttttctttcctggtaactatgggtctggtgttgtcataaggatctaccttccacatgctggacagtgggggttgctgcttgaggagactcaggccagatacagatcactgtggggaacactaagcttacttggttagagcacggcactaacatttctgcctctgtgagtttgattccaccacataattttttaaaagtgcttttccatggccccttagtgtcaaccattcttacgaaagatgtgagcaacagtgtacatgttttggcaaaagtcgtgacaaatagcaccagcatctgccgccctaggtggacctgtggcctcatcttggcagcctgtgagttgggcagagctgtgacgaggcatggttctgtgccggctggcagggtctgtgatatggcagcactgtgatccgtactggaaagacataatggcatgtcctgtgaacagcagatacagaaggctgagtggggaagcgacccaggggtattgccacacaaagcgataggccagctaagtaccaggagacaaactgaggtgggaggaaatagtgacttcatggcctcattctttagacttactccttaaaaggactagatccggggagggaaaagtaatcacaaaatgttcaagctaataagagatatttttggtcttaaaactaaggtttaaaaattcccagtactgaaaacaactttctcactcttttgtgaattggacaatttgaccattatgaagatcttttgaaacaatcaatgaaaatgctactaagtgtcatgaattattttttaatatttttgagtaaggggagtactttaatactgattgggcccatgtaatagacaatatgtcacttttggtgtaactatttttatgaggaaaaaacattaacaatgaaatgccaattcctatttataacagaccttttttgtttagatatatttcaagtttccccagaaaatatgaggcatgttaatacaacacaattatttaaaaggtaacaacattaaaacattttactgctgccaatgtaacatacagacatctgagaaatgacaattatcaacctttgtaatacatgattacgcaaggtgatatgagacaacccaagggtagcacattttaaaaaatacccacagtatataactggcaagccaaaaaaacttcctgtattaacagaaatgattactgaattgaacgctttttaaaaaatgtcttttaagcaaaaattgtatttctcttttcatgttacattaagaatttggaatattatttttcagttaagtcaaagaagaacttgaaaaaaataatgacatacttcacaaatagtagagactagatgtaaacacagacctaaaaatgagcagtaggataaaaaaaaccatgaatgtttgttctcttctggaccatgattttaaattttaatttggtaattccagataaagattctaatttatcatggtttctggactgatctctttaagttaaacactttcagtctaagtgtgttcaactggcctaaagccactgtcaggaaaaatgtatttaggaaaatatacaacacagggcaagaaaatactactgtagaataaggaatttagatttcactgcaaataaagccatatttgatattaaagacacatgttcctattttcacatcagtcatttattaacaccaaacattatactttaacttttccccattacacagtacaataagcctgtcaagatttccaggaagtaatcatcagtacctactgtgcttccagcagccaaagctaagctggctgggtaccagaaatcaacaccttcaggagaatggcatcacaagattgcatggactcatattaactattacaaggggcactggaaaaaaaggtcatttgctcatttacaaaatcctaattgaactaaagctctgtaattatagccatggtatcagaccagctttttcgcacatcctatcacatcgctgcctgctgatgttttacactgcctataaagtctcataattttaaaagggaatgaaacagaatgccacaggtgaccgacctctgctcctgctacttgggagtcacgttgtcttggcttcgtcctggctcaaggttactagtctcttgctgctttgggccaaatctcttatctctttacatttcctcctctcaggctgagtcaaaagtaagtcacatgtataacaaaactgtcttaaaataccactgtttttcagccaagagaattacggatgcaatttaaagtctaaatgtattaattggaaaaattaaattagagcaactcaaggttttcctgtaattaccaaatgaaactgattgaaaaactgttccttctaattctgcttttccaacaaaagttcatcacactagcaggataaacattcaaaatacataatagaacatatcctaattaagcaccagagttgtgtcagagccaagtatatacacacacacacgtatacgtgtgtgtgtgtgtgtgtgtgtgtgtagtttattactggttaagtaaatgctctaattagcaaaaatcatgagaaatatatacagtgatataatgcggttaaattttagttctctgtgttaactacttactgttaatttagtactcaattagaattaactctgggattttgagggcagataaatcagtaattagcctttatcccagaaagaatagtggtagcttcaaaagcttcaacagacctaatgatgtaatttattcaggacagaaaaaaaaatatgtagccaacattcttgcaagaattactttcttatggaatttaagatttcctcaaatattttcttttctatatagcgttttgttcttgtgtagttatctgcctaggatacagacaggatattgagactatttcagaaagtagacacactaaaaacatttgacaaattaaaaaaattttgcataaaacaggttaccctttcctgctgactatacttaagaaataccaaagtagcatacaaaatgcttctaaactttcaaaatatctgaataaaaacaaagatcctacttttaactgagatagatttataattcttacttacaagataaaaaaatttcctaaaatttatttttaaatttcacataacctgctataattcgctgtaaaaaatggatgtcaaaatagaattttaaatatacaaattgtttttgataactacctttcatacattttatttaaactgtagcattagctcaagatgaaactttttaaaagaaaccataggcttttgtccaactcaaagattcaagcccagattctgaacaaagtaaatgtgatgaaatttatgaaaaactatactgtacagtcaaaacagtgatggtgcctcagtaaataacttcagtaaaatatccagtgctccaaatagctgagccatctttctaaggttcactctgcttctctcccccagccctcatggcctgtgctaccatctattcttttagcgtttatgctggagggccttatagttcctttaaaagtacactgaaaatactttatatcacagcttattctaaccactggttctcaaattaaaaggtatatttcagtgcatatttcatagccacattgcagaactaatatttgaaaactcttgggggaaattttggtaacaaaattgcaaaatgacatgattatttatgagctttctataaaaagttttttttttttttttttttttactttagagatcatacctactttcctgcctttttgataagtaaggcatgaaatgaaacaaaagttttgagctgtaaggtgcctataaaggatgtcactacagcattcacaatgctaggtgtgtaagatgacatggctgttaccatgtactaaagaaccccatcatgtgagagatcgctcaaagtcattaacacaaagcagtgaaaatcatccagcaaagcagtgcttatgagagactagaattcagagaaatgcaaggtacgaacttctctctaatccaagggtattctgctgtgatcttctaatcagtgatgattgtgcttatgcacacgacatcttcatgggagagaccaggctgattgcaaaataatgacaaccaaccagtttacctcaacatagctcactctgcaatgtcagacatgcagtgtagagcagtcacaaagtcaagccatgaatacagggatggaaaaacattccagtgagctggtctctacaatttttaagacacttcatcctcccaattatattctttgtcataaagaggaaaaacagcaagattattaaatccaaaaagtcacagatgtcacaaggggatgaaataatttcctcattttttttctttatcagtgtaggaaaagctgtctttccatagcccacactcataatagcacttcaactaggctcctttgaaaatgaaaagtgaacaagtttcctaatgctggccttataagatctaaagagatgattaaattcaaaccaggctgagctcttactctgagctatttcagccactgatgtttgtaaaatataggaagaagattccaataggcaatttgcattggcaagcactggactacagaattcatcactgttttctgaaaaaatataattaaaccttaatggaattatgacacttttatgaggtttataattcacagccacctctcatcatattttgttcttctttccatttttaccatttcaaatattgcaatattgcccaccataaaccactgaaaatgattatttatgtatattccatttatttctctagggggtctaggtaatttgaatcaggagctccaagtaccatttaaaaaggtgagtctttaaaaaccatcagtgttttaaacacttgattagaaaaaagataacagctccttgtagtgatctagcttatgtgctttatggtatcttttcaaaaggagagtataaatcattgtacataaaatcaaaatagctaatatacatttttttctggcacttttgagaaattaggcattgaacataaaacatcttataaacttacataacaaaaataaatgtttacattttaatcttagattaccttagggtagcagttaacttatgagatgccacactgttggtgtgggcagcggagaccatgggaaatacacattcatgtccacagcccttcagcgatggatgcatggctgccgtccaaatatgtggtctgtgtcccaacataaagattaaggctctctgttttgaaggaatgagttctgggcttaaacaagtctagaagtaccacaatactcatggaaaatactgaaaagattcggacgagttttcaaacactgggggaaacacgtttttgactagaaaaataaaataaagcatctaaaactgacttcaagtactttggggagaggctgctgatatcgaatgccaaaataagaaggaacaaagacagaagagactccagggacgtccctccccatcccttcacccgcagggtccagatccccaggtgctgatgcgcaactctttggggaggactggcgagctgggcagaaagcagcagccatggtttgtcaccatcctaaaacacctatattgagggcaaaggccaagctttgtgtgaaaatttccttgggatgaaccacaggaatctggacatttcaagggggaaaaagccttaaagtcagtagcagacagagaaaaggaaagagaggaagaaaaacctgcttttctgaatggcagtactttaggccgggggcattgtggtccttggtgagtgcagcttttccatacagcttggctttcctcactaatgagatgagaccactgacagctgggatcttttgtgggtggtgagggtgcagcagggagatgtgcttgggtgtacctgtccatctggcaggcaggggcacactcaggtgcagcctagtccgtacctctctgtctcagaaactgaacaactgggagaacagtcgacagggcctctccaaccatcttcaggtgactaaagcagcatatgaagtataggtttgtgtcacttcttctcttccacagaagaaacgtctccagacactgatcacaggctacccagggttgtcttctgggttgctagagcctggtaatatctctgccttgctgcaagtcacttatgctctcgtagtcgttctcctttgggacgagaccgtggtggccattggtccccagggtggccttttcttcctctctgttgagagtctgtatcgcttcataatcaggctctggctcctcgctgggcctccctgctggtggaagtgtgctgtttggagttttttcgaagtctttaacagtagcatagagatcattacaggaggagggtgacctctgtgggtccccttgaatggaggtgtaggtggactccggaactgtaagcgactgccccgatttattcactaactgtccaggtttatttactgatgagtacatagctgagatctcttcttctgtgagagtggggtcttcttcccgagacttgtatgacaatgagctaaatctcttgttagtttcactggtcgtgtctgtggcactctcttccgcctctcccccttccttctcctgaaggttttcattctcgtccagaagcttaacagggacaggtggtggggcctcctcttctggatcacatgaatttccaaggatactctctacattaacactttgacgacattttttgtttctgtccaccgaggcatattcagcaaactcagctttgccttcagtctggggccctgggagctctttcgaggcagaagtagattttgccttgccactgtggcctttctccaggtgtgcagctgcagccacctccttgatctctttcacagtttcatacaagcagtcctccaccatgttttcttgggaggagctgtccttgagcacttcatagggcccttccatccccagcccctggtccccgtccacacttctcgccgtgagcatggtatccactgcgctctcgggagggattctgggcagctcccgactctgatgacattttggtttccctgtgctgtcctgggaatccagcagatccgaggccgatgtctggacttcctcgtaatgctgcatgcaggtcagagtactgtcctctgaaagaatgtccccattggtgagtgccccattctgctcactgctggcaggagcatctgttgccaggctagtaactgaacggctgaacatctccttgtctgaaggcacgttcatcaggttctcatggtccccactatgctgtcgcggcttcttttccctgtcacaactagagcacaggaagatgaggaaggtgatgacgaagaaaatggcgacagcagccagacttccccacagggtgatctgcatctgtccgctgcccagcaggctccccgcgggccccatggcaggagcaggcactggcaccagccgagggaatcagtcagtccttcaaaggtggtgacatggaggcagagagctgtgtccttggaggaaatgtttgtccagtagagtattccaagttctggcaatgtattccctttgaaatgttgtggtgagagttctctcttctttcttggctgggactcaggaggcagggagtcttcctggcggacggcgctcggaggcagcctctgcaaactccggcgcgcagcgccgccgccccggcacagcccggcagcagcggcaagtgcaggaccaggcgccgccgctctgcaccagtcgccttggctcagctgtgccgggcgccgggcattcgccagggcacacgactcagcgaggcggcggctgggactgaggctactgcacccggccgcgcggacccgagcgctgcagctgcctccagccccggagcgcggcgctccgagcccctggtgggtgtctctggctccaagggaatcacggctcaattagggacctgccaggagaaaaaccgatgcgctgccgcaggcagagccgccagcccgcccccagtcggctggtcacatcgcgggcgcgcagacggacaagcgagcgggagggtaccgcagccagcactcgccgccgcgccgc

SEQ ID NO: 15093 - RNA, 3558 nt, Homo sapiens
  source 1..3558: mol_type = other RNA
gctgggattacaggcatgagccactgcacccggcctaaaaatgattacttcttataaaaaggatttcttccccttcacaacactcagcttcctttttctttcctggtaactatgggtctggtgttgtcataaggatctaccttccacatgctggacagtgggggttgctgcttgaggagactcaggccagatacagatcactgtggggaacactaagcttacttggttagagcacggcactaacatttctgcctctgtgagtttgattccaccacataattttttaaaagtgcttttccatggccccttagtgtcaaccattcttacgaaagatgtgagcaacagtgtacatgttttggcaaaagtcgtgacaaatagcaccagcatctgccgccctaggtggacctgtggcctcatcttggcagcctgtgagttgggcagagctgtgacgaggcatggttctgtgccggctggcagggtctgtgatatggcagcactgtgatccgtactggaaagacataatggcatgtccttagggtagcagttaacttatgagatgccacactgttggtgtgggcagcggagaccatgggaaatacacattcatgtccacagcccttcagcgatggatgcatggctgccgtccaaatatgtggtctgtgtcccaacataaagattaaggctctctgttttgaaggaatgagttctgggcttaaacaagtctagaagtaccacaatactcatggaaaatactgaaaagattcggacgagttttcaaacactgggggaaacacgtttttgactagaaaaataaaataaagcatctaaaactgacttcaagtactttggggagaggctgctgatatcgaatgccaaaataagaaggaacaaagacagaagagactccagggacgtccctccccatcccttcacccgcagggtccagatccccaggtgctgatgcgcaactctttggggaggactggcgagctgggcagaaagcagcagccatggtttgtcaccatcctaaaacacctatattgagggcaaaggccaagctttgtgtgaaaatttccttgggatgaaccacaggaatctggacatttcaagggggaaaaagccttaaagtcagtagcagacagagaaaaggaaagagaggaagaaaaacctgcttttctgaatggcagtactttaggccgggggcattgtggtccttggtgagtgcagcttttccatacagcttggctttcctcactaatgagatgagaccactgacagctgggatcttttgtgggtggtgagggtgcagcagggagatgtgcttgggtgtacctgtccatctggcaggcaggggcacactcaggtgcagcctagtccgtacctctctgtctcagaaactgaacaactgggagaacagtcgacagggcctctccaaccatcttcaggtgactaaagcagcatatgaagtataggtttgtgtcacttcttctcttccacagaagaaacgtctccagacactgatcacaggctacccagggttgtcttctgggttgctagagcctggtaatatctctgccttgctgcaagtcacttatgctctcgtagtcgttctcctttgggacgagaccgtggtggccattggtccccagggtggccttttcttcctctctgttgagagtctgtatcgcttcataatcaggctctggctcctcgctgggcctccctgctggtggaagtgtgctgtttggagttttttcgaagtctttaacagtagcatagagatcattacaggaggagggtgacctctgtgggtccccttgaatggaggtgtaggtggactccggaactgtaagcgactgccccgatttattcactaactgtccaggtttatttactgatgagtacatagctgagatctcttcttctgtgagagtggggtcttcttcccgagacttgtatgacaatgagctaaatctcttgttagtttcactggtcgtgtctgtggcactctcttccgcctctcccccttccttctcctgaaggttttcattctcgtccagaagcttaacagggacaggtggtggggcctcctcttctggatcacatgaatttccaaggatactctctacattaacactttgacgacattttttgtttctgtccaccgaggcatattcagcaaactcagctttgccttcagtctggggccctgggagctctttcgaggcagaagtagattttgccttgccactgtggcctttctccaggtgtgcagctgcagccacctccttgatctctttcacagtttcatacaagcagtcctccaccatgttttcttgggaggagctgtccttgagcacttcatagggcccttccatccccagcccctggtccccgtccacacttctcgccgtgagcatggtatccactgcgctctcgggagggattctgggcagctcccgactctgatgacattttggtttccctgtgctgtcctgggaatccagcagatccgaggccgatgtctggacttcctcgtaatgctgcatgcaggtcagagtactgtcctctgaaagaatgtccccattggtgagtgccccattctgctcactgctggcaggagcatctgttgccaggctagtaactgaacggctgaacatctccttgtctgaaggcacgttcatcaggttctcatggtccccactatgctgtcgcggcttcttttccctgtcacaactagagcacaggaagatgaggaaggtgatgacgaagaaaatggcgacagcagccagacttccccacagggtgatctgcatctgtccgctgcccagcaggctccccgcgggccccatggcaggagcaggcactggcaccagccgagggaatcagtcagtccttcaaaggtggtgacatggaggcagagagctgtgtccttggaggaaatgtttgtccagtagagtattccaagttctggcaatgtattccctttgaaatgttgtggtgagagttctctcttctttcttggccttttcccagcaatgaagttgtggccaactgctgaaataggagaaaaatctcgtgtttttgggactcaggaggcagggagtcttcctggcggacggcgctcggaggcagcctctgcaaactccggcgcgcagcgccgccgccccggcacagcccggcagcagcggcaagtgcaggaccaggcgccgccgctctgcaccagtcgccttggctcagctgtgccgggcgccgggcattcgccagggcacacgactcagcgaggcggcggctgggactgaggctactgcacccggccgcgcggacccgagcgctgcagctgcctccagccccggagcgcggcgctccgagcccctggtgggtgtctctggctccaagggaatcacggctcaattagggacctgccaggagaaaaaccgatgcgctgccgcaggcagagccgccagcccgcccccagtcggctggtcacatcgcgggcgcgcagacggacaagcgagcgggagggtaccgcagccagcactcgccgccgcgccgcgg

SEQ ID NO: 15094 - RNA, 976 nt, Homo sapiens
  source 1..976: mol_type = other RNA
gctgggattacaggcatgagccactgcacccggcctaaaagcctcttctaagaaaggttccacaggcttcaccagccttccaaagaggtccgctgcacacaaaagtttcagaatttctggtgtattaggcctactggatctttttctctgaaggtaaggagttactgagaatggtttagcggcttggtgatgccccagggatccaggctgtcttcccttctgctctgccagccttagtgtgttgtctgatgtcctcatccttggtgcttcatagtcacaatatgactgctgttgctctggacatcacttatgtaatgtgtgtacaggtcttggtaaattgcaggttccgattcagcaggtcccggcagggcctaagagtctggattcctcaccagctcccaggtgatgtcaatgctgctggtccggggaccacactgtccaactcgcaatcagaaatcaggaggttcctgaaaggcacagatggaaactgaaaatgctttaggcttaggtaacccagcatcaggaatcgggatggttggatgcagggacctcgcccagcttgtctggggccgcagcctacggcagggacgtttcagtccttagctggggtgaaagtgaggtcagggtcgccggggaaatgcgggagtacagtcacgcgggagaaagacgtcaagagcgaaagctcggaggcgtcaaaatgagcagcaagtccaggcacaaggcgtcgggcgcggagagtacggcgggtgccgggggagggagatgaggccgcgaagacgccggggcttcgtccggcggcgacggggaggccgcggaggttcccgagcgcagcggggcgcgcacctcccgctcgggccgggctccctcgccgcgcggccccggatcctccctgcgcgggtttccgtggcccccgccgggctcttccgttccctcccgcggcctcgaccaggccgcagcccccagcccaggcgaccga

SEQ ID NO: 15095 - RNA, 3680 nt, Homo sapiens
  source 1..3680: mol_type = other RNA
gctgggattacaggcatgagccactgcacccggcctaggcatctttatttctatgtatagaaagccttccttaattttccccccaaagagaaattattgtttagtattttgaatgaagagctcagtttagcaatttaaatcaagaaattatacaaattgttccatggagattaaaaagaaaaaggagctcaacttcacctaagtgacataagcccaatataaaagatatgttggatatcttgaacccaactcatctttagaatccactccatctttaaaaacataatgttaaattcaaacactgaaacaacaaataatgattaaaaatgacttagaaaaataaatagaactttgaaacttcttggcttctcacagtgtaattttgcaccccttcccccactttatttttgagacagggtcttgttctctgtcgctcaggctggagtgcagtggtacaattatggcttactgcagcctcaaaatcttgggctcaaccaatcttcccacctcaacctcccaaacagctcggactacaggcgtgggccactaactatgcctggctaactttttaaaacaattttctgaagagacagggcattgctgtgttttgttttttctcttctttaaaagatagctggttttaaccaccactgagctgattaagagctctctttattaggcttagaactgttgattattgctcttaaatctcacagaacttagtttaagatttggattttacttcgatcaagtttatcctgcaattctaggggttctcaataaagagaggcttaagaatataacctgttttatcagtggctttttcctacactacaactagttctgttttaattaaataggaatggctcaagagcctccttttaccagacagtatcaactatgtgtgtcataaagggagaaaacagcttaatactcatctaaagtgttcacagaacattcagaattggtaacagtggaattttcaactttggaacatataagggatgttgacagtggtcaggagtggagccacctatccagaactacgatcaagcctcttcagttcattaactgctgtggaagtttcagaggattctgttgaatttgaatcagtgccagttttgtctttcaaggtctgtttggcaagagtctcatctctattttcttgtgcttggctttcttcttcttcctcttcaccatctggaaactcccactgagactcgcccgactgttcgtttacatagaaataccgtctatgatccctgctggcagaggatagtaatcttgttcttcattcacatcttcagccacgaagttttccttaacttcaccgaggttaatcaggagtagttgcttccagaggtcctgtaaagcgcacagagctctcgcatgcgcttaacccccaagcccgccctactccgtgcaacactctggagagtaaaaaccagctttgtccatatcttgggaaaaaatccgttacatggaacactttaaacattgcttttgtttctccaatgtgtggctggccaaactttgtgcttgcggtgctttgcctgcccagcaccgctaactgcagctgctctcagtctccagacaggctgtcatgtcgtcagatggtggtgatcacaaatcatgtctgagatgtcaaaggtgaaaggtgaaaaggggagaagagtgcgtacctgtcccagtggcaggaccagcctttaggagtggcgtttatttcatactgttttagttgttctgctgcatcctgaagttttcgtttaaggtagtttccattaagagccccttcccgccagtctgcaattcgagtctcagtctgtaagagcagcacatgaaagttggagatggattgtctattaatgcctagaaactcgaatttacttgtcagggtatttgccagttctccaatctgaaatttcaaatcctgttcttcttctacttttggtgttgtctgtacttttattttctctggagattcttctacttccatctctttatctgaattctcatctattttttctgaattttcagcaccaattgcagtttctccattttctggagtatctcgtccagttttactagaactcctactggtagattctggactggtagctcgaacaaacatcttccattttcctcttttagacataagcctacgcattccatcttgagatgctggctggctgatatcagaacgtggactagaccctgacacactaccatctccttcctccaaggctcgcaactctgcttttttcctttccaaaactagctccagttcaagggtatcttgttcctcttcctcctcactttctccagattggacaacactgcaaagatcctcctgagaagggtcttctatattgtccaacataatttcctgtggctttactattgttgttgcttcttctactgttgtacttgtttcttttacttctgaaactggctcctctttacaaattacttttcttctccatctctcttcttcttcttttattccctcaggcaataaaggagcaagcagcgatgctgccacccctttcttctcctcctcactatttgagagagcctgaattccttcatttacttcctttttaacttctcgcttggctatgactggtccacttttactactggaaacagaaatcgttttctccttagaatatatgtctgtatttaccacaaaactagtttcagcacctggcacagaactgggctggtaatgctgtaatccctgtacctgtgtggcaagatattggggtaactcccaagtcacttcatttgtttgtgtattccaataataataacatcccgtgttctcatcccagacttcctgccaatcgcccatctcaattccgactcctgccagtgaacactgagtatcatattgccaaccagatgtttgggtggagtctgttccatttgaagtagaagaagaaagggtagatgttgctgcttcctttggctctggtcgaggtggagttggaggtggagcagaagctcctacaggagctgcaggctgaggagctgttatggcatcgatctccgctaggaagttggccaatgtactatcaatatcagttgactggtttccatttgtctctttggattgtgctagtttttcggaaacatcattgtcatcgtcatcactgtcagcataagcaccaagcaagcatagaccgcctgttgctttaacagctgtgggtctagtggtcatgactggttttggaggattctgaacaactctaggaacctcctgcaccgcttcctgttcatccttgccttctgaaggcgagtcgtccgaggccgcggcggcagtcaccgcggtggtggtggtcgtcgccgccgacggggcgggctggctggggaccgccgcggttgagtccggctcagtgtcgggttccggctccgggtcccggcccggcgtgctgccccgaggacccggcggagagagttgcaggatgggcctacggccgggtaccgcccgggacttcttccccatcgcgagcccaagcgcgagcagagagcgtcgggcggccgagaggggcgggcactggaggctgggcgctgggccctgggcgctgcgacgcgtaatcaatattcatacaccgtgacaccgcctccagcccggatccgctttcaaccagcggagcacgcgcttgcgcaagcgcctc

SEQ ID NO: 15096 - RNA, 3260 nt, Homo sapiens
  source 1..3260: mol_type = other RNA
gctgggattacaggcatgagccactgcacccggcctaggcatctttatttctatgtatagaaagccttccttaattttccccccaaagagaaattattgtttagtattttgaatgaagagctcagtttagcaatttaaatcaagaaattatacaaattgttccatggagattaaaaagaaaaaggagctcaacttcacctaagtgacataagcccaatataaaagatatgttggatatcttgaacccaactcatctttagaatccactccatctttaaaaacataatgttaaattcaaacactgaaacaacaaataatgattaaaaatgacttagaaaaataaatagaactttgaaacttcttggcttctcacagtgtaattttgcaccccttcccccactttatttttgagacagggtcttgttctctgtcgctcaggctggagtgcagtggtacaattatggcttactgcagcctcaaaatcttgggctcaaccaatcttcccacctcaacctcccaaacagctcggactacaggcgtgggccactaactatgcctggctaactttttaaaacaattttctgaagagacagggcattgctgtgttttgttttttctcttctttaaaagatagctggttttaaccaccactgagctgattaagagctctctttattaggcttagaactgttgattattgctcttaaatctcacagaacttagtttaagatttggattttacttcgatcaagtttatcctgcaattctaggggttctcaataaagagaggcttaagaatataacctgttttatcagtggctttttcctacactacaactagttctgttttaattaaataggaatggctcaagagcctccttttaccagacagtatcaactatgtgtgtcataaagggagaaaacagcttaatactcatctaaagtgttcacagaacattcagaattggtaacagtggaattttcaactttggaacatataagggatgttgacagtggtcaggagtggagccacctatccagaactacgatcaagcctcttcagttcattaactgctgtggaagtttcagaggattctgttgaatttgaatcagtgccagttttgtctttcaaggtctgtttggcaagagtctcatctctattttcttgtgcttggctttcttcttcttcctcttcaccatctggaaactcccactgagactcgcccgactgttcgtttacatagaaataccgtctatgatccctgtcccagtggcaggaccagcctttaggagtggcgtttatttcatactgttttagttgttctgctgcatcctgaagttttcgtttaaggtagtttccattaagagccccttcccgccagtctgcaattcgagtctcagtctgtaagagcagcacatgaaagttggagatggattgtctattaatgcctagaaactcgaatttacttgtcagggtatttgccagttctccaatctgaaatttcaaatcctgttcttcttctacttttggtgttgtctgtacttttattttctctggagattcttctacttccatctctttatctgaattctcatctattttttctgaattttcagcaccaattgcagtttctccattttctggagtatctcgtccagttttactagaactcctactggtagattctggactggtagctcgaacaaacatcttccattttcctcttttagacataagcctacgcattccatcttgagatgctggctggctgatatcagaacgtggactagaccctgacacactaccatctccttcctccaaggctcgcaactctgcttttttcctttccaaaactagctccagttcaagggtatcttgttcctcttcctcctcactttctccagattggacaacactgcaaagatcctcctgagaagggtcttctatattgtccaacataatttcctgtggctttactattgttgttgcttcttctactgttgtacttgtttcttttacttctgaaactggctcctctttacaaattacttttcttctccatctctcttcttcttcttttattccctcaggcaataaaggagcaagcagcgatgctgccacccctttcttctcctcctcactatttgagagagcctgaattccttcatttacttcctttttaacttctcgcttggctatgactggtccacttttactactggaaacagaaatcgttttctccttagaatatatgtctgtatttaccacaaaactagtttcagcacctggcacagaactgggctggtaatgctgtaatccctgtacctgtgtggcaagatattggggtaactcccaagtcacttcatttgtttgtgtattccaataataataacatcccgtgttctcatcccagacttcctgccaatcgcccatctcaattccgactcctgccagtgaacactgagtatcatattgccaaccagatgtttgggtggagtctgttccatttgaagtagaagaagaaagggtagatgttgctgcttcctttggctctggtcgaggtggagttggaggtggagcagaagctcctacaggagctgcaggctgaggagctgttatggcatcgatctccgctaggaagttggccaatgtactatcaatatcagttgactggtttccatttgtctctttggattgtgctagtttttcggaaacatcattgtcatcgtcatcactgtcagcataagcaccaagcaagcatagaccgcctgttgctttaacagctgtgggtctagtggtcatgactggttttggaggattctgaacaactctaggaacctcctgcaccgcttcctgttcatccttgccttctgaaggcgagtcgtccgaggccgcggcggcagtcaccgcggtggtggtggtcgtcgccgccgacggggcgggctggctggggaccgccgcggttgagtccggctcagtgtcgggttccggctccgggtcccggcccggcgtgctgccccgaggacccggcggagagagttgcaggatgggcctacggccgggtaccgcccgggacttcttccccatcgcgagcccaagcgcgagcagagagcgtcgggcggccgagaggggcgggcactggaggctgggcgctgggccctgggcgctgcgacgcgtaatcaatattcatacaccgtgacaccgcctccagcccggatccgctttcaaccagcggagcacgcgcttgcgcaagcgcctc

SEQ ID NO: 15097 - RNA, 3257 nt, Homo sapiens
  source 1..3257: mol_type = other RNA
gctgggattacaggcatgagccactgcacccggcctaggcatctttatttctatgtatagaaagccttccttaattttccccccaaagagaaattattgtttagtattttgaatgaagagctcagtttagcaatttaaatcaagaaattatacaaattgttccatggagattaaaaagaaaaaggagctcaacttcacctaagtgacataagcccaatataaaagatatgttggatatcttgaacccaactcatctttagaatccactccatctttaaaaacataatgttaaattcaaacactgaaacaacaaataatgattaaaaatgacttagaaaaataaatagaactttgaaacttcttggcttctcacagtgtaattttgcaccccttcccccactttatttttgagacagggtcttgttctctgtcgctcaggctggagtgcagtggtacaattatggcttactgcagcctcaaaatcttgggctcaaccaatcttcccacctcaacctcccaaacagctcggactacaggcgtgggccactaactatgcctggctaactttttaaaacaattttctgaagagacagggcattgctgtgttttgttttttctcttctttaaaagatagctggttttaaccaccactgagctgattaagagctctctttattaggcttagaactgttgattattgctcttaaatctcacagaacttagtttaagatttggattttacttcgatcaagtttatcctgcaattctaggggttctcaataaagagaggcttaagaatataacctgttttatcagtggctttttcctacactacaactagttctgttttaattaaataggaatggctcaagagcctccttttaccagacagtatcaactatgtgtgtcataaagggagaaaacagcttaatactcatctaaagtgttcacagaacattcagaattggtaacagtggaattttcaactttggaacatataagggatgttgacagtggtcaggagtggagccacctatccagaactacgatcaagcctcttcagttcattaactgtggaagtttcagaggattctgttgaatttgaatcagtgccagttttgtctttcaaggtctgtttggcaagagtctcatctctattttcttgtgcttggctttcttcttcttcctcttcaccatctggaaactcccactgagactcgcccgactgttcgtttacatagaaataccgtctatgatccctgtcccagtggcaggaccagcctttaggagtggcgtttatttcatactgttttagttgttctgctgcatcctgaagttttcgtttaaggtagtttccattaagagccccttcccgccagtctgcaattcgagtctcagtctgtaagagcagcacatgaaagttggagatggattgtctattaatgcctagaaactcgaatttacttgtcagggtatttgccagttctccaatctgaaatttcaaatcctgttcttcttctacttttggtgttgtctgtacttttattttctctggagattcttctacttccatctctttatctgaattctcatctattttttctgaattttcagcaccaattgcagtttctccattttctggagtatctcgtccagttttactagaactcctactggtagattctggactggtagctcgaacaaacatcttccattttcctcttttagacataagcctacgcattccatcttgagatgctggctggctgatatcagaacgtggactagaccctgacacactaccatctccttcctccaaggctcgcaactctgcttttttcctttccaaaactagctccagttcaagggtatcttgttcctcttcctcctcactttctccagattggacaacactgcaaagatcctcctgagaagggtcttctatattgtccaacataatttcctgtggctttactattgttgttgcttcttctactgttgtacttgtttcttttacttctgaaactggctcctctttacaaattacttttcttctccatctctcttcttcttcttttattccctcaggcaataaaggagcaagcagcgatgctgccacccctttcttctcctcctcactatttgagagagcctgaattccttcatttacttcctttttaacttctcgcttggctatgactggtccacttttactactggaaacagaaatcgttttctccttagaatatatgtctgtatttaccacaaaactagtttcagcacctggcacagaactgggctggtaatgctgtaatccctgtacctgtgtggcaagatattggggtaactcccaagtcacttcatttgtttgtgtattccaataataataacatcccgtgttctcatcccagacttcctgccaatcgcccatctcaattccgactcctgccagtgaacactgagtatcatattgccaaccagatgtttgggtggagtctgttccatttgaagtagaagaagaaagggtagatgttgctgcttcctttggctctggtcgaggtggagttggaggtggagcagaagctcctacaggagctgcaggctgaggagctgttatggcatcgatctccgctaggaagttggccaatgtactatcaatatcagttgactggtttccatttgtctctttggattgtgctagtttttcggaaacatcattgtcatcgtcatcactgtcagcataagcaccaagcaagcatagaccgcctgttgctttaacagctgtgggtctagtggtcatgactggttttggaggattctgaacaactctaggaacctcctgcaccgcttcctgttcatccttgccttctgaaggcgagtcgtccgaggccgcggcggcagtcaccgcggtggtggtggtcgtcgccgccgacggggcgggctggctggggaccgccgcggttgagtccggctcagtgtcgggttccggctccgggtcccggcccggcgtgctgccccgaggacccggcggagagagttgcaggatgggcctacggccgggtaccgcccgggacttcttccccatcgcgagcccaagcgcgagcagagagcgtcgggcggccgagaggggcgggcactggaggctgggcgctgggccctgggcgctgcgacgcgtaatcaatattcatacaccgtgacaccgcctccagcccggatccgctttcaaccagcggagcacgcgcttgcgcaagcgcctc

SEQ ID NO: 15098 - RNA, 2531 nt, Homo sapiens
  source 1..2531: mol_type = other RNA
gctgggattacaggcatgagccactgcacccggcctattggcattttttaaaaaccctaatctttagtaaagttttagtctagcaaagtctaatgcattttatctgcagaacactcattttggttattattattattttgagacggagtttcactcttgttgcccaggctggagtgcaatggtgtgatctcggatcaccgcaacctctgcctcccgggttcaagcgattctcctgcctctgcctcctgagtatctgggattataggcatgcgccaccatgcttggctaattttttgtatttgtagtagagagggggtttctctatattggtcaggctggtcttgaactcccaacctcaggtaatctgcccgcttcagcatcccagtgctgggattacaggcgtgagccaccgcaccctgccactcactttgattattaaaagcacttacattcaagtagaggtacatgttaaaagaaaaaaaaaagaaaaagaaaagcacttatctatgaagctatcaggatattttagaattcaaagttaacactgattttatatatcataagtatttatttccacagcagaaaattagttgaacacaagaacattcaaaaaataaacatgtttctcaaatcaagtcaagagtgaaatgttataagggtacaaagtaaatgctgatatattaaaatcttggtttgatttagcaattttactaaaacccagaaaagtttctatgaataaatttatttaatttaataaattattcatgattaaaaatttagtttttcataaacagtaacaacagactaaacactgaatatatgggattccaataaacaatagtaaaaacactttaacattatttacttcaaatattatcttgaaattattcaaatgtattcgaagtttatagttaactgatgtgtaacaatgaattccagaccaaattgatagcgattagatatattagtgctgtctgcttgtccttcacatgatcacaggatgaagctcccttttgtaagaaacatcatggccacactggttacatataataatccaactagttagcgtatttatggaggaagcggtcaaatgcatcatagatggcttgtctgaagagtccttgtttaaaaagataagcactaatatgacccccttctaagtatcggatttcacaaccaggccaaatttcttgtaaacttcgaactcctgttcgtggaatataggcatcttctttggcttgaaccactataatgaggcttggatcaactgggactgagaaatttgctacatgagtacattcatccatgactcctttcataaatattaaagactctttccgaagactgtttctgctttgttctttactaagtaggtggtatgactgagggttgcgacttgtataaccacttttgttggttgaaagtgtttgattgaagcgcttcatcttagaggtatcttgcaataagagtccttctgatgtcgcactgacagatgttttgctagaattatggcagtcagcaggtttttgggatacaacttggtttgatatatctaaatttaaagttctggaaaccagattaaggttagttagcttgtctgcactgctagtgaagtgtttcacaaactcttgtcccattttgaaagaatctgtcgtagtgaagaccccagatgctgtggaccaagacaggcatggaatcaatggcatgggcttaggccagttggataccgctaaggaagccatgtgtcctcccatggatattccagtcattcctaaagggccgtaaccttccctctctagccagtgcaagagagctgcagattctaaaacaagagctcctcccatcacaaaaaggtcggacacattttttaagctggaccttacttggtccttgggtttccagcaacgttgaacatttctttatatctgtgcaccagtttcatttcttcttctgtgaatagtctgacgtcatcaataagggttttctaacaataaagaagccattcgggcttctttaatcataggacgggccattagtgttcgtcgcctccagtaatgatgatctcctgttccagcaagatgaatgcatacaggtctatatttgctgttccattctttaggcacaataaattggaaccttatcaatgtgtactggataatcgcttgaaaccagattctggcatctttcccgatttccaatcatctttctgaattcaaagagtcttttgagatcttctggccttccccatcctctgataaaaagttttgttaggagaagtctccggtatagaatatctaacttgctcacacccatcagtagcaaacaagcattggccgccaggtggaagcctgcgatcgagctggccgggcctcccagcaccgccgctctccaggctccctttccaggactcaactttggtcccagccccaatcgcagctccggtaacctttccaggaaccgaaatgctagatacagcggaaggagaaacggagggaggaagacaaacccggagcagggcggcgcggcagttt

SEQ ID NO: 15099 - RNA, 2468 nt, Homo sapiens
  source 1..2468: mol_type = other RNA
gctgggattacaggcatgagccactgcacccggcctattggcattttttaaaaaccctaatctttagtaaagttttagtctagcaaagtctaatgcattttatctgcagaacactcattttggttattattattattttgagacggagtttcactcttgttgcccaggctggagtgcaatggtgtgatctcggatcaccgcaacctctgcctcccgggttcaagcgattctcctgcctctgcctcctgagtatctgggattataggcatgcgccaccatgcttggctaattttttgtatttgtagtagagagggggtttctctatattggtcaggctggtcttgaactcccaacctcaggtaatctgcccgcttcagcatcccagtgctgggattacaggcgtgagccaccgcaccctgccactcactttgattattaaaagcacttacattcaagtagaggtacatgttaaaagaaaaaaaaaagaaaaagaaaagcacttatctatgaagctatcaggatattttagaattcaaagttaacactgattttatatatcataagtatttatttccacagcagaaaattagttgaacacaagaacattcaaaaaataaacatgtttctcaaatcaagtcaagagtgaaatgttataagggtacaaagtaaatgctgatatattaaaatcttggtttgatttagcaattttactaaaacccagaaaagtttctatgaataaatttatttaatttaataaattattcatgattaaaaatttagtttttcataaacagtaacaacagactaaacactgaatatatgggattccaataaacaatagtaaaaacactttaacattatttacttcaaatattatcttgaaattattcaaatgtattcgaagtttatagttaactgatgtgtaacaatgaattccagaccaaattgatagcgattagatatattagtgctgtctgcttgtccttcacatgatcacaggatgaagctcccttttgtaagaaacatcatggccacactggttacatataataatccaactagttagcgtatttatggaggaagcggtcaaatgcatcatagatggcttgtctgaagagtccttgtttaaaaagataagcactaatatgacccccttctaagtatcggatttcacaaccaggccaaatttcttgtaaacttcgaactcctgttcgtggaatataggcatcttctttggcttgaaccactataatgaggcttggatcaactgggactgagaaatttgctacatgagtacattcatccatgactcctttcataaatattaaagactctttccgaagactgtttctgctttgttctttactaagtaggtggtatgactgagggttgcgacttgtataaccacttttgttggttgaaagtgtttgattgaagcgcttcatcttagaggtatcttgcaataagagtccttctgatgtcgcactgacagatgttttgctagaattatggcagtcagcaggtttttgggatacaacttggtttgatatatctaaatttaaagttctggaaaccagattaaggttagttagcttgtctgcactgctagtgaagtgtttcacaaactcttgtcccattttgaaagaatctgtcgtagtgaagaccccagatgctgtggaccaagacaggcatggaatcaatggcatgggcttaggccagttggataccgctaaggaagccatgtgtcctcccatggatattccagtcattcctaaagggccgtaaccttccctctctagccagtgcaagagagctgcagattctaaaacaagagctcctcccatcacaaaaaggtcggacacattttttaagctggaccttacttggtccttgggtttcctgcagccataataagggttttctaacaataaagaagccattcgggcttctttaatcataggacgggccattagtgttcgtcgcctccagtaatgatgatctcctgttccagcaagatgaatgcatacaggtctatatttgctgttccattctttaggcacaataaattggaaccttatcaatgtgtactggataatcgcttgaaaccagattctggcatctttcccgatttccaatcatctttctgaattcaaagagtcttttgagatcttctggccttccccatcctctgataaaaagttttgttaggagaagtctccggtatagaatatctaacttgctcacacccatcagtagcaaacaagcattggccgccaggtggaagcctgcgatcgagctggccgggcctcccagcaccgccgctctccaggctccctttccaggactcaactttggtcccagccccaatcgcagctccggtaacctttccaggaaccgaaatgctagatacagcggaaggagaaacggagggaggaagacaaacccggagcagggcggcgcggcagttt

SEQ ID NO: 15100 - RNA, 2569 nt, Homo sapiens
  source 1..2569: mol_type = other RNA
gctgggattacaggcatgagccactgcacccggcctattggcattttttaaaaaccctaatctttagtaaagttttagtctagcaaagtctaatgcattttatctgcagaacactcattttggttattattattattttgagacggagtttcactcttgttgcccaggctggagtgcaatggtgtgatctcggatcaccgcaacctctgcctcccgggttcaagcgattctcctgcctctgcctcctgagtatctgggattataggcatgcgccaccatgcttggctaattttttgtatttgtagtagagagggggtttctctatattggtcaggctggtcttgaactcccaacctcaggtaatctgcccgcttcagcatcccagtgctgggattacaggcgtgagccaccgcaccctgccactcactttgattattaaaagcacttacattcaagtagaggtacatgttaaaagaaaaaaaaaagaaaaagaaaagcacttatctatgaagctatcaggatattttagaattcaaagttaacactgattttatatatcataagtatttatttccacagcagaaaattagttgaacacaagaacattcaaaaaataaacatgtttctcaaatcaagtcaagagtgaaatgttataagggtacaaagtaaatgctgatatattaaaatcttggtttgatttagcaattttactaaaacccagaaaagtttctatgaataaatttatttaatttaataaattattcatgattaaaaatttagtttttcataaacagtaacaacagactaaacactgaatatatgggattccaataaacaatagtaaaaacactttaacattatttacttcaaatattatcttgaaattattcaaatgtattcgaagtttatagttaactgatgtgtaacaatgaattccagaccaaattgatagcgattagatatattagtgctgtctgcttgtccttcacatgatcacaggatgaagctcccttttgtaagaaacatcatggccacactggttacatataataatccaactagttagcgtatttatggaggaagcggtcaaatgcatcatagatggcttgtctgaagagtccttgtttaaaaagataagcactaatatgacccccttctaagtatcggatttcacaaccaggccaaatttcttgtaaacttcgaactcctgttcgtggaatataggcatcttctttggcttgaaccactataatgaggcttggatcaactgggactgagaaatttgctacatgagtacattcatccatgactcctttcataaatattaaagactctttccgaagactgtttctgctttgttctttactaagtaggtggtatgactgagggttgcgacttgtataaccacttttgttggttgaaagtgtttgattgaagcgcttcatcttagaggtatcttgcaataagagtccttctgatgtcgcactgacagatgttttgctagaattatggcagtcagcaggtttttgggatacaacttggtttgatatatctaaatttaaagttctggaaaccagattaaggttagttagcttgtctgcactgctagtgaagtgtttcacaaactcttgtcccattttgaaagaatctgtcgtagtgaagaccccagatgctgtggaccaagacaggcatggaatcaatggcatgggcttaggccagttggataccgctaaggaagccatgtgtcctcccatggatattccagtcattcctaaagggccgtaaccttccctctctagccagtgcaagagagctgcagattctaaaacaagagctcctcccatcacaaaaaggtcggacacattttttaagctggaccttacttggtccttgggtttcctgcagccataataagggttttctaacaataaagaagccattcgggcttctttaatcataggacgggccattagtgttcgtcgcctccagtaatgatgatctcctgttccagcaagatgaatgcatacaggtctatatttgctgttccattctttaggcacaataaattggaaccttgcaataacagattcaattggcatgatatcaggcacatagtgagccatgggggaaacaaagtgtccatctaagatcttacaatctgattgctcttcaatcttatcaatgtgtactggataatcgcttgaaaccagattctggcatctttcccgatttccaatcatctttctgaattcaaagagtcttttgagatcttctggccttccccatcctctgataaaaagttttgttaggagaagtctccggtatagaatatctaacttgctcacacccatcagtagcaaacaagcattggccgccaggtggaagcctgcgatcgagctggccgggcctcccagcaccgccgctctccaggctccctttccaggactcaactttggtcccagccccaatcgcagctccggtaacctttccaggaaccgaaatgctagatacagcggaaggagaaacggagggaggaagacaaacccggagcagggcggcgcggcagttt

SEQ ID NO: 15101 - RNA, 2678 nt, Homo sapiens
  source 1..2678: mol_type = other RNA
gctgggattacaggcatgagccactgcacccggcctattggcattttttaaaaaccctaatctttagtaaagttttagtctagcaaagtctaatgcattttatctgcagaacactcattttggttattattattattttgagacggagtttcactcttgttgcccaggctggagtgcaatggtgtgatctcggatcaccgcaacctctgcctcccgggttcaagcgattctcctgcctctgcctcctgagtatctgggattataggcatgcgccaccatgcttggctaattttttgtatttgtagtagagagggggtttctctatattggtcaggctggtcttgaactcccaacctcaggtaatctgcccgcttcagcatcccagtgctgggattacaggcgtgagccaccgcaccctgccactcactttgattattaaaagcacttacattcaagtagaggtacatgttaaaagaaaaaaaaaagaaaaagaaaagcacttatctatgaagctatcaggatattttagaattcaaagttaacactgattttatatatcataagtatttatttccacagcagaaaattagttgaacacaagaacattcaaaaaataaacatgtttctcaaatcaagtcaagagtgaaatgttataagggtacaaagtaaatgctgatatattaaaatcttggtttgatttagcaattttactaaaacccagaaaagtttctatgaataaatttatttaatttaataaattattcatgattaaaaatttagtttttcataaacagtaacaacagactaaacactgaatatatgggattccaataaacaatagtaaaaacactttaacattatttacttcaaatattatcttgaaattattcaaatgtattcgaagtttatagttaactgatgtgtaacaatgaattccagaccaaattgatagcgattagatatattagtgctgtctgcttgtccttcacatgatcacaggatgaagctcccttttgtaagaaacatcatggccacactggttacatataataatccaactagttagcgtatttatggaggaagcggtcaaatgcatcatagatggcttgtctgaagagtccttgtttaaaaagataagcactaatatgacccccttctaagtatcggatttcacaaccaggccaaatttcttgtaaacttcgaactcctgttcgtggaatataggcatcttctttggcttgaaccactataatgaggcttggatcaactgggactgagaaatttgctacatgagtacattcatccatgactcctttcataaatattaaagactctttccgaagactgtttctgctttgttctttactaagtaggtggtatgactgagggttgcgacttgtataaccacttttgttggttgaaagtgtttgattgaagcgcttcatcttagaggtatcttgcaataagagtccttctgatgtcgcactgacagatgttttgctagaattatggcagtcagcaggtttttgggatacaacttggtttgatatatctaaatttaaagttctggaaaccagattaaggttagttagcttgtctgcactgctagtgaagtgtttcacaaactcttgtcccattttgaaagaatctgttccacagtattcaagcatgtgaataatttcttcttcataaactgtctgggtataatattgcttttccagctccctccaattaattgatttactcaacacacccgtagtgaagaccccagatgctgtggaccaagacaggcatggaatcaatggcatgggcttaggccagttggataccgctaaggaagccatgtgtcctcccatggatattccagtcattcctaaagggccgtaaccttccctctctagccagtgcaagagagctgcagattctaaaacaagagctcctcccatcacaaaaaggtcggacacattttttaagctggaccttacttggtccttgggtttccagcaacgttgaacatttctttatatctgtgcaccagtttcatttcttcttctgtgaatagtctgacgtcatcaataagggttttctaacaataaagaagccattcgggcttctttaatcataggacgggccattagtgttcgtcgcctccagtaatgatgatctcctgttccagcaagatgaatgcatacaggtctatatttgctgttccattctttaggcacaataaattggaacaaaggtagaagaatcaagttggtatcaagcatttcatcaataatccttatcaatgtgtactggataatcgcttgaaaccagattctggcatctttcccgatttccaatcatctttctgaattcaaagagtcttttgagatcttctggccttccccatcctctgataaaaagttttgttaggagaagtctccggtatagaatatctaacttgctcacacccatcagtagcaaacaagcattggccgccaggtggaagcctgcgatcgagctggccgggcctcccagcaccgccgctctccaggctccctttccaggactcaactttggtcccagccccaatcgcagctccggtaacctttccaggaaccgaaatgctagatacagcggaaggagaaacggagggaggaagacaaacccggagcagggcggcgcggcagttt

SEQ ID NO: 15102 - RNA, 2783 nt, Homo sapiens
  source 1..2783: mol_type = other RNA
gctgggattacaggcatgagccactgcacccggcctattggcattttttaaaaaccctaatctttagtaaagttttagtctagcaaagtctaatgcattttatctgcagaacactcattttggttattattattattttgagacggagtttcactcttgttgcccaggctggagtgcaatggtgtgatctcggatcaccgcaacctctgcctcccgggttcaagcgattctcctgcctctgcctcctgagtatctgggattataggcatgcgccaccatgcttggctaattttttgtatttgtagtagagagggggtttctctatattggtcaggctggtcttgaactcccaacctcaggtaatctgcccgcttcagcatcccagtgctgggattacaggcgtgagccaccgcaccctgccactcactttgattattaaaagcacttacattcaagtagaggtacatgttaaaagaaaaaaaaaagaaaaagaaaagcacttatctatgaagctatcaggatattttagaattcaaagttaacactgattttatatatcataagtatttatttccacagcagaaaattagttgaacacaagaacattcaaaaaataaacatgtttctcaaatcaagtcaagagtgaaatgttataagggtacaaagtaaatgctgatatattaaaatcttggtttgatttagcaattttactaaaacccagaaaagtttctatgaataaatttatttaatttaataaattattcatgattaaaaatttagtttttcataaacagtaacaacagactaaacactgaatatatgggattccaataaacaatagtaaaaacactttaacattatttacttcaaatattatcttgaaattattcaaatgtattcgaagtttatagttaactgatgtgtaacaatgaattccagaccaaattgatagcgattagatatattagtgctgtctgcttgtccttcacatgatcacaggatgaagctcccttttgtaagaaacatcatggccacactggttacatataataatccaactagttagcgtatttatggaggaagcggtcaaatgcatcatagatggcttgtctgaagagtccttgtttaaaaagataagcactaatatgacccccttctaagtatcggatttcacaaccaggccaaatttcttgtaaacttcgaactcctgttcgtggaatataggcatcttctttggcttgaaccactataatgaggcttggatcaactgggactgagaaatttgctacatgagtacattcatccatgactcctttcataaatattaaagactctttccgaagactgtttctgctttgttctttactaagtaggtggtatgactgagggttgcgacttgtataaccacttttgttggttgaaagtgtttgattgaagcgcttcatcttagaggtatcttgcaataagagtccttctgatgtcgcactgacagatgttttgctagaattatggcagtcagcaggtttttgggatacaacttggtttgatatatctaaatttaaagttctggaaaccagattaaggttagttagcttgtctgcactgctagtgaagtgtttcacaaactcttgtcccattttgaaagaatctgttccacagtattcaagcatgtgaataatttcttcttcataaactgtctgggtataatattgcttttccagctccctccaattaattgatttactcaacacacccgtagtgaagaccccagatgctgtggaccaagacaggcatggaatcaatggcatgggcttaggccagttggataccgctaaggaagccatgtgtcctcccatggatattccagtcattcctaaagggccgtaaccttccctctctagccagtgcaagagagctgcagattctaaaacaagagctcctcccatcacaaaaaggtcggacacattttttaagctggaccttacttggtccttgggtttccagcaacgttgaacatttctttatatctgtgcaccagtttcatttcttcttctgtgaatagtctgacgtcatcaataagggttttctaacaataaagaagccattcgggcttctttaatcataggacgggccattagtgttcgtcgcctccagtaatgatgatctcctgttccagcaagatgaatgcatacaggtctatatttgctgttccattctttaggcacaataaattggaacctacaaaggtagaagaatcaagttggtatcaagcatttcatcaataatccttgcaataacagattcaattggcatgatatcaggcacatagtgagccatgggggaaacaaagtgtccatctaagatcttacaatctgattgctcttcaatcttatcaatgtgtactggataatcgcttgaaaccagattctggcatctttcccgatttccaatcatctttctgaattcaaagagtcttttgagatcttctggccttccccatcctctgataaaaagttttgttaggagaagtctccggtatagaatatctaacttgctcacacccatcagtagcaaacaagcattggccgccaggtggaagcctgcgatcgagctggccgggcctcccagcaccgccgctctccaggctccctttccaggactcaactttggtcccagccccaatcgcagctccggtaacctttccaggaaccgaaatgctagatacagcggaaggagaaacggagggaggaagacaaacccggagcagggcggcgcggcagttt

SEQ ID NO: 15103 - RNA, 2633 nt, Homo sapiens
  source 1..2633: mol_type = other RNA
gctgggattacaggcatgagccactgcacccggcctattggcattttttaaaaaccctaatctttagtaaagttttagtctagcaaagtctaatgcattttatctgcagaacactcattttggttattattattattttgagacggagtttcactcttgttgcccaggctggagtgcaatggtgtgatctcggatcaccgcaacctctgcctcccgggttcaagcgattctcctgcctctgcctcctgagtatctgggattataggcatgcgccaccatgcttggctaattttttgtatttgtagtagagagggggtttctctatattggtcaggctggtcttgaactcccaacctcaggtaatctgcccgcttcagcatcccagtgctgggattacaggcgtgagccaccgcaccctgccactcactttgattattaaaagcacttacattcaagtagaggtacatgttaaaagaaaaaaaaaagaaaaagaaaagcacttatctatgaagctatcaggatattttagaattcaaagttaacactgattttatatatcataagtatttatttccacagcagaaaattagttgaacacaagaacattcaaaaaataaacatgtttctcaaatcaagtcaagagtgaaatgttataagggtacaaagtaaatgctgatatattaaaatcttggtttgatttagcaattttactaaaacccagaaaagtttctatgaataaatttatttaatttaataaattattcatgattaaaaatttagtttttcataaacagtaacaacagactaaacactgaatatatgggattccaataaacaatagtaaaaacactttaacattatttacttcaaatattatcttgaaattattcaaatgtattcgaagtttatagttaactgatgtgtaacaatgaattccagaccaaattgatagcgattagatatattagtgctgtctgcttgtccttcacatgatcacaggatgaagctcccttttgtaagaaacatcatggccacactggttacatataataatccaactagttagcgtatttatggaggaagcggtcaaatgcatcatagatggcttgtctgaagagtccttgtttaaaaagataagcactaatatgacccccttctaagtatcggatttcacaaccaggccaaatttcttgtaaacttcgaactcctgttcgtggaatataggcatcttctttggcttgaaccactataatgaggcttggatcaactgggactgagaaatttgctacatgagtacattcatccatgactcctttcataaatattaaagactctttccgaagactgtttctgctttgttctttactaagtaggtggtatgactgagggttgcgacttgtataaccacttttgttggttgaaagtgtttgattgaagcgcttcatcttagaggtatcttgcaataagagtccttctgatgtcgcactgacagatgttttgctagaattatggcagtcagcaggtttttgggatacaacttggtttgatatatctaaatttaaagttctggaaaccagattaaggttagttagcttgtctgcactgctagtgaagtgtttcacaaactcttgtcccattttgaaagaatctgttccacagtattcaagcatgtgaataatttcttcttcataaactgtctgggtataatattgcttttccagctccctccaattaattgatttactcaacacacccgtagtgaagaccccagatgctgtggaccaagacaggcatggaatcaatggcatgggcttaggccagttggataccgctaaggaagccatgtgtcctcccatggatattccagtcattcctaaagggccgtaaccttccctctctagccagtgcaagagagctgcagattctaaaacaagagctcctcccatcacaaaaaggtcggacacattttttaagctggaccttacttggtccttgggtttccagcaacgttgaacatttctttatatctgtgcaccagtttcatttcttcttctgtgaatagtctgacgtcatcaataagggttttctaacaataaagaagccattcgggcttctttaatcataggacgggccattagtgttcgtcgcctccagtaatgatgatctcctgttccagcaagatgaatgcatacaggtctatatttgctgttccattctttaggcacaataaattggaaccttatcaatgtgtactggataatcgcttgaaaccagattctggcatctttcccgatttccaatcatctttctgaattcaaagagtcttttgagatcttctggccttccccatcctctgataaaaagttttgttaggagaagtctccggtatagaatatctaacttgctcacacccatcagtagcaaacaagcattggccgccaggtggaagcctgcgatcgagctggccgggcctcccagcaccgccgctctccaggctccctttccaggactcaactttggtcccagccccaatcgcagctccggtaacctttccaggaaccgaaatgctagatacagcggaaggagaaacggagggaggaagacaaacccggagcagggcggcgcggcagttt

SEQ ID NO: 15104 - RNA, 2615 nt, Homo sapiens
  source 1..2615: mol_type = other RNA
gctgggattacaggcatgagccactgcacccggcctattggcattttttaaaaaccctaatctttagtaaagttttagtctagcaaagtctaatgcattttatctgcagaacactcattttggttattattattattttgagacggagtttcactcttgttgcccaggctggagtgcaatggtgtgatctcggatcaccgcaacctctgcctcccgggttcaagcgattctcctgcctctgcctcctgagtatctgggattataggcatgcgccaccatgcttggctaattttttgtatttgtagtagagagggggtttctctatattggtcaggctggtcttgaactcccaacctcaggtaatctgcccgcttcagcatcccagtgctgggattacaggcgtgagccaccgcaccctgccactcactttgattattaaaagcacttacattcaagtagaggtacatgttaaaagaaaaaaaaaagaaaaagaaaagcacttatctatgaagctatcaggatattttagaattcaaagttaacactgattttatatatcataagtatttatttccacagcagaaaattagttgaacacaagaacattcaaaaaataaacatgtttctcaaatcaagtcaagagtgaaatgttataagggtacaaagtaaatgctgatatattaaaatcttggtttgatttagcaattttactaaaacccagaaaagtttctatgaataaatttatttaatttaataaattattcatgattaaaaatttagtttttcataaacagtaacaacagactaaacactgaatatatgggattccaataaacaatagtaaaaacactttaacattatttacttcaaatattatcttgaaattattcaaatgtattcgaagtttatagttaactgatgtgtaacaatgaattccagaccaaattgatagcgattagatatattagtgctgtctgcttgtccttcacatgatcacaggatgaagctcccttttgtaagaaacatcatggccacactggttacatataataatccaactagttagcgtatttatggaggaagcggtcaaatgcatcatagatggcttgtctgaagagtccttgtttaaaaagataagcactaatatgacccccttctaagtatcggatttcacaaccaggccaaatttcttgtaaacttcgaactcctgttcgtggaatataggcatcttctttggcttgaaccactataatgaggcttggatcaactgggactgagaaatttgctacatgagtacattcatccatgactcctttcataaatattaaagactctttccgaagactgtttctgctttgttctttactaagtaggtggtatgactgagggttgcgacttgtataaccacttttgttggttgaaagtgtttgattgaagcgcttcatcttagaggtatcttgcaataagagtccttctgatgtcgcactgacagatgttttgctagaattatggcagtcagcaggtttttgggatacaacttggtttgatatatctaaatttaaagttctggaaaccagattaaggttagttagcttgtctgcactgctagtgaagtgtttcacaaactcttgtcccattttgaaagaatctgttccacagtattcaagcatgtgaataatttcttcttcataaactgtctgggtataatattgcttttccagctccctccaattaattgatttactcaacacacccgtagtgaagaccccagatgctgtggaccaagacaggcatggaatcaatggcatgggcttaggccagttggataccgctaaggaagccatgtgtcctcccatggatattccagtcattcctaaagggccgtaaccttccctctctagccagtgcaagagagctgcagattctaaaacaagagctcctcccatcacaaaaaggtcggacacattttttaagctggaccttacttggtccttgggtttcctgcagccataataagggttttctaacaataaagaagccattcgggcttctttaatcataggacgggccattagtgttcgtcgcctccagtaatgatgatctcctgttccagcaagatgaatgcatacaggtctatatttgctgttccattctttaggcacaataaattggaacaaaggtagaagaatcaagttggtatcaagcatttcatcaataatccttatcaatgtgtactggataatcgcttgaaaccagattctggcatctttcccgatttccaatcatctttctgaattcaaagagtcttttgagatcttctggccttccccatcctctgataaaaagttttgttaggagaagtctccggtatagaatatctaacttgctcacacccatcagtagcaaacaagcattggccgccaggtggaagcctgcgatcgagctggccgggcctcccagcaccgccgctctccaggctccctttccaggactcaactttggtcccagccccaatcgcagctccggtaacctttccaggaaccgaaatgctagatacagcggaaggagaaacggagggaggaagacaaacccggagcagggcggcgcggcagttt

SEQ ID NO: 15105 - RNA, 2716 nt, Homo sapiens
  source 1..2716: mol_type = other RNA
gctgggattacaggcatgagccactgcacccggcctattggcattttttaaaaaccctaatctttagtaaagttttagtctagcaaagtctaatgcattttatctgcagaacactcattttggttattattattattttgagacggagtttcactcttgttgcccaggctggagtgcaatggtgtgatctcggatcaccgcaacctctgcctcccgggttcaagcgattctcctgcctctgcctcctgagtatctgggattataggcatgcgccaccatgcttggctaattttttgtatttgtagtagagagggggtttctctatattggtcaggctggtcttgaactcccaacctcaggtaatctgcccgcttcagcatcccagtgctgggattacaggcgtgagccaccgcaccctgccactcactttgattattaaaagcacttacattcaagtagaggtacatgttaaaagaaaaaaaaaagaaaaagaaaagcacttatctatgaagctatcaggatattttagaattcaaagttaacactgattttatatatcataagtatttatttccacagcagaaaattagttgaacacaagaacattcaaaaaataaacatgtttctcaaatcaagtcaagagtgaaatgttataagggtacaaagtaaatgctgatatattaaaatcttggtttgatttagcaattttactaaaacccagaaaagtttctatgaataaatttatttaatttaataaattattcatgattaaaaatttagtttttcataaacagtaacaacagactaaacactgaatatatgggattccaataaacaatagtaaaaacactttaacattatttacttcaaatattatcttgaaattattcaaatgtattcgaagtttatagttaactgatgtgtaacaatgaattccagaccaaattgatagcgattagatatattagtgctgtctgcttgtccttcacatgatcacaggatgaagctcccttttgtaagaaacatcatggccacactggttacatataataatccaactagttagcgtatttatggaggaagcggtcaaatgcatcatagatggcttgtctgaagagtccttgtttaaaaagataagcactaatatgacccccttctaagtatcggatttcacaaccaggccaaatttcttgtaaacttcgaactcctgttcgtggaatataggcatcttctttggcttgaaccactataatgaggcttggatcaactgggactgagaaatttgctacatgagtacattcatccatgactcctttcataaatattaaagactctttccgaagactgtttctgctttgttctttactaagtaggtggtatgactgagggttgcgacttgtataaccacttttgttggttgaaagtgtttgattgaagcgcttcatcttagaggtatcttgcaataagagtccttctgatgtcgcactgacagatgttttgctagaattatggcagtcagcaggtttttgggatacaacttggtttgatatatctaaatttaaagttctggaaaccagattaaggttagttagcttgtctgcactgctagtgaagtgtttcacaaactcttgtcccattttgaaagaatctgttccacagtattcaagcatgtgaataatttcttcttcataaactgtctgggtataatattgcttttccagctccctccaattaattgatttactcaacacacccgtagtgaagaccccagatgctgtggaccaagacaggcatggaatcaatggcatgggcttaggccagttggataccgctaaggaagccatgtgtcctcccatggatattccagtcattcctaaagggccgtaaccttccctctctagccagtgcaagagagctgcagattctaaaacaagagctcctcccatcacaaaaaggtcggacacattttttaagctggaccttacttggtccttgggtttcctgcagccataataagggttttctaacaataaagaagccattcgggcttctttaatcataggacgggccattagtgttcgtcgcctccagtaatgatgatctcctgttccagcaagatgaatgcatacaggtctatatttgctgttccattctttaggcacaataaattggaacaaaggtagaagaatcaagttggtatcaagcatttcatcaataatccttgcaataacagattcaattggcatgatatcaggcacatagtgagccatgggggaaacaaagtgtccatctaagatcttacaatctgattgctcttcaatcttatcaatgtgtactggataatcgcttgaaaccagattctggcatctttcccgatttccaatcatctttctgaattcaaagagtcttttgagatcttctggccttccccatcctctgataaaaagttttgttaggagaagtctccggtatagaatatctaacttgctcacacccatcagtagcaaacaagcattggccgccaggtggaagcctgcgatcgagctggccgggcctcccagcaccgccgctctccaggctccctttccaggactcaactttggtcccagccccaatcgcagctccggtaacctttccaggaaccgaaatgctagatacagcggaaggagaaacggagggaggaagacaaacccggagcagggcggcgcggcagttt

SEQ ID NO: 15106 - RNA, 2570 nt, Homo sapiens
  source 1..2570: mol_type = other RNA
gctgggattacaggcatgagccactgcacccggcctattggcattttttaaaaaccctaatctttagtaaagttttagtctagcaaagtctaatgcattttatctgcagaacactcattttggttattattattattttgagacggagtttcactcttgttgcccaggctggagtgcaatggtgtgatctcggatcaccgcaacctctgcctcccgggttcaagcgattctcctgcctctgcctcctgagtatctgggattataggcatgcgccaccatgcttggctaattttttgtatttgtagtagagagggggtttctctatattggtcaggctggtcttgaactcccaacctcaggtaatctgcccgcttcagcatcccagtgctgggattacaggcgtgagccaccgcaccctgccactcactttgattattaaaagcacttacattcaagtagaggtacatgttaaaagaaaaaaaaaagaaaaagaaaagcacttatctatgaagctatcaggatattttagaattcaaagttaacactgattttatatatcataagtatttatttccacagcagaaaattagttgaacacaagaacattcaaaaaataaacatgtttctcaaatcaagtcaagagtgaaatgttataagggtacaaagtaaatgctgatatattaaaatcttggtttgatttagcaattttactaaaacccagaaaagtttctatgaataaatttatttaatttaataaattattcatgattaaaaatttagtttttcataaacagtaacaacagactaaacactgaatatatgggattccaataaacaatagtaaaaacactttaacattatttacttcaaatattatcttgaaattattcaaatgtattcgaagtttatagttaactgatgtgtaacaatgaattccagaccaaattgatagcgattagatatattagtgctgtctgcttgtccttcacatgatcacaggatgaagctcccttttgtaagaaacatcatggccacactggttacatataataatccaactagttagcgtatttatggaggaagcggtcaaatgcatcatagatggcttgtctgaagagtccttgtttaaaaagataagcactaatatgacccccttctaagtatcggatttcacaaccaggccaaatttcttgtaaacttcgaactcctgttcgtggaatataggcatcttctttggcttgaaccactataatgaggcttggatcaactgggactgagaaatttgctacatgagtacattcatccatgactcctttcataaatattaaagactctttccgaagactgtttctgctttgttctttactaagtaggtggtatgactgagggttgcgacttgtataaccacttttgttggttgaaagtgtttgattgaagcgcttcatcttagaggtatcttgcaataagagtccttctgatgtcgcactgacagatgttttgctagaattatggcagtcagcaggtttttgggatacaacttggtttgatatatctaaatttaaagttctggaaaccagattaaggttagttagcttgtctgcactgctagtgaagtgtttcacaaactcttgtcccattttgaaagaatctgttccacagtattcaagcatgtgaataatttcttcttcataaactgtctgggtataatattgcttttccagctccctccaattaattgatttactcaacacacccgtagtgaagaccccagatgctgtggaccaagacaggcatggaatcaatggcatgggcttaggccagttggataccgctaaggaagccatgtgtcctcccatggatattccagtcattcctaaagggccgtaaccttccctctctagccagtgcaagagagctgcagattctaaaacaagagctcctcccatcacaaaaaggtcggacacattttttaagctggaccttacttggtccttgggtttcctgcagccataataagggttttctaacaataaagaagccattcgggcttctttaatcataggacgggccattagtgttcgtcgcctccagtaatgatgatctcctgttccagcaagatgaatgcatacaggtctatatttgctgttccattctttaggcacaataaattggaaccttatcaatgtgtactggataatcgcttgaaaccagattctggcatctttcccgatttccaatcatctttctgaattcaaagagtcttttgagatcttctggccttccccatcctctgataaaaagttttgttaggagaagtctccggtatagaatatctaacttgctcacacccatcagtagcaaacaagcattggccgccaggtggaagcctgcgatcgagctggccgggcctcccagcaccgccgctctccaggctccctttccaggactcaactttggtcccagccccaatcgcagctccggtaacctttccaggaaccgaaatgctagatacagcggaaggagaaacggagggaggaagacaaacccggagcagggcggcgcggcagttt

SEQ ID NO: 15107 - RNA, 2671 nt, Homo sapiens
  source 1..2671: mol_type = other RNA
gctgggattacaggcatgagccactgcacccggcctattggcattttttaaaaaccctaatctttagtaaagttttagtctagcaaagtctaatgcattttatctgcagaacactcattttggttattattattattttgagacggagtttcactcttgttgcccaggctggagtgcaatggtgtgatctcggatcaccgcaacctctgcctcccgggttcaagcgattctcctgcctctgcctcctgagtatctgggattataggcatgcgccaccatgcttggctaattttttgtatttgtagtagagagggggtttctctatattggtcaggctggtcttgaactcccaacctcaggtaatctgcccgcttcagcatcccagtgctgggattacaggcgtgagccaccgcaccctgccactcactttgattattaaaagcacttacattcaagtagaggtacatgttaaaagaaaaaaaaaagaaaaagaaaagcacttatctatgaagctatcaggatattttagaattcaaagttaacactgattttatatatcataagtatttatttccacagcagaaaattagttgaacacaagaacattcaaaaaataaacatgtttctcaaatcaagtcaagagtgaaatgttataagggtacaaagtaaatgctgatatattaaaatcttggtttgatttagcaattttactaaaacccagaaaagtttctatgaataaatttatttaatttaataaattattcatgattaaaaatttagtttttcataaacagtaacaacagactaaacactgaatatatgggattccaataaacaatagtaaaaacactttaacattatttacttcaaatattatcttgaaattattcaaatgtattcgaagtttatagttaactgatgtgtaacaatgaattccagaccaaattgatagcgattagatatattagtgctgtctgcttgtccttcacatgatcacaggatgaagctcccttttgtaagaaacatcatggccacactggttacatataataatccaactagttagcgtatttatggaggaagcggtcaaatgcatcatagatggcttgtctgaagagtccttgtttaaaaagataagcactaatatgacccccttctaagtatcggatttcacaaccaggccaaatttcttgtaaacttcgaactcctgttcgtggaatataggcatcttctttggcttgaaccactataatgaggcttggatcaactgggactgagaaatttgctacatgagtacattcatccatgactcctttcataaatattaaagactctttccgaagactgtttctgctttgttctttactaagtaggtggtatgactgagggttgcgacttgtataaccacttttgttggttgaaagtgtttgattgaagcgcttcatcttagaggtatcttgcaataagagtccttctgatgtcgcactgacagatgttttgctagaattatggcagtcagcaggtttttgggatacaacttggtttgatatatctaaatttaaagttctggaaaccagattaaggttagttagcttgtctgcactgctagtgaagtgtttcacaaactcttgtcccattttgaaagaatctgttccacagtattcaagcatgtgaataatttcttcttcataaactgtctgggtataatattgcttttccagctccctccaattaattgatttactcaacacacccgtagtgaagaccccagatgctgtggaccaagacaggcatggaatcaatggcatgggcttaggccagttggataccgctaaggaagccatgtgtcctcccatggatattccagtcattcctaaagggccgtaaccttccctctctagccagtgcaagagagctgcagattctaaaacaagagctcctcccatcacaaaaaggtcggacacattttttaagctggaccttacttggtccttgggtttcctgcagccataataagggttttctaacaataaagaagccattcgggcttctttaatcataggacgggccattagtgttcgtcgcctccagtaatgatgatctcctgttccagcaagatgaatgcatacaggtctatatttgctgttccattctttaggcacaataaattggaaccttgcaataacagattcaattggcatgatatcaggcacatagtgagccatgggggaaacaaagtgtccatctaagatcttacaatctgattgctcttcaatcttatcaatgtgtactggataatcgcttgaaaccagattctggcatctttcccgatttccaatcatctttctgaattcaaagagtcttttgagatcttctggccttccccatcctctgataaaaagttttgttaggagaagtctccggtatagaatatctaacttgctcacacccatcagtagcaaacaagcattggccgccaggtggaagcctgcgatcgagctggccgggcctcccagcaccgccgctctccaggctccctttccaggactcaactttggtcccagccccaatcgcagctccggtaacctttccaggaaccgaaatgctagatacagcggaaggagaaacggagggaggaagacaaacccggagcagggcggcgcggcagttt

SEQ ID NO: 15108 - RNA, 3328 nt, Homo sapiens
  source 1..3328: mol_type = other RNA
gctgggattacaggcatgagccactgcacccggcctattggcattttttaaaaaccctaatctttagtaaagttttagtctagcaaagtctaatgcattttatctgcagaacactcattttggttattattattattttgagacggagtttcactcttgttgcccaggctggagtgcaatggtgtgatctcggatcaccgcaacctctgcctcccgggttcaagcgattctcctgcctctgcctcctgagtatctgggattataggcatgcgccaccatgcttggctaattttttgtatttgtagtagagagggggtttctctatattggtcaggctggtcttgaactcccaacctcaggtaatctgcccgcttcagcatcccagtgctgggattacaggcgtgagccaccgcaccctgccactcactttgattattaaaagcacttacattcaagtagaggtacatgttaaaagaaaaaaaaaagaaaaagaaaagcacttatctatgaagctatcaggatattttagaattcaaagttaacactgattttatatatcataagtatttatttccacagcagaaaattagttgaacacaagaacattcaaaaaataaacatgtttctcaaatcaagtcaagagtgaaatgttataagggtacaaagtaaatgctgatatattaaaatcttggtttgatttagcaattttactaaaacccagaaaagtttctatgaataaatttatttaatttaataaattattcatgattaaaaatttagtttttcataaacagtaacaacagactaaacactgaatatatgggattccaataaacaatagtaaaaacactttaacattatttacttcaaatattatcttgaaattattcaaatgtattcgaagtttatagttaactgatgtgtaacaatgaattccagaccaaattgatagcgattagatatattagtgctgtctgcttgtccttcacatgatcacaggatgaagctcccttttgtaagaaacatcatggccacactggttacatataataatccaactagttagcgtatttatggaggaagcggtcaaatgcatcatagatggcttgtctgaagagtccttgtttaaaaagataagcactaatatgacccccttctaagtatcggatttcacaaccaggccaaatttcttgtaaacttcgaactcctgttcgtggaatataggcatcttctttggcttgaaccactataatgaggcttggatcaactgggactgagaaatttgctacatgagtacattcatccatgactcctttcataaatattaaagactctttccgaagactgtttctgctttgttctttactaagtaggtggtatgactgagggttgcgacttgtataaccacttttgttggttgaaagtgtttgattgaagcgcttcatcttagaggtatcttgcaataagagtccttctgatgtcgcactgacagatgttttgctagaattatggcagtcagcaggtttttgggatacaacttggtttgatatatctaaatttaaagttctggaaaccagattaaggttagttagcttgtctgcactgctagtgaagtgtttcacaaactcttgtcccattttgaaagaatctgttccacagtattcaagcatgtgaataatttcttcttcataaactgtctgggtataatattgcttttccagctccctccaattaattgatttactcaacacacccgtagtgaagaccccagatgctgtggaccaagacaggcatggaatcaatggcatgggcttaggccagttggataccgctaaggaagccatgtgtcctcccatggatattccagtcattcctaaagggccgtaaccttccctctctagccagtgcaagagagctgcagattctaaaacaagagctcctcccatcacaaaaaggtcggacacattttttaagctggaccttcttaaaaaggaaaaggtaggctgggcacagtggctcatgcctataatcccagcactttgggaggccaaggtgggtggatcacttgaggtcaggagtttgagaccagcctgaccaacatggtgaaagcccatctctactaaacatacaaaaattagccaggtgtggtggtgcatgcctgtaattccagctacttgggaggctgaggcagagaatcgcttgaacccaggaggcagaggttccagtgagctgagatcgcaccagtgcactccagactgggtgacagaatgactgcgtctcaaaaaaaaaaaaagaaagggttttatcatttcttcatttacagtttcacaactaaactatatattaagtctacctgttaaaattttttattgtatttccttaacagacattaaaatgcaaaaatcttaaaaataaaaattaaagtcagtattcatactacagtttcataacagaactccccccccccataatatttaggtattcaatttagaaatggttaactgaaggcaaccaaaattttaatactgctggatattgggtaaaaagactgcaaaaatgaaagtgatatatacttacacttggtccttgggtttccagcaacgttgaacatttctttatatctgtgcaccagtttcatttcttcttctgtgaatagtctgacgtcatcaataagggttttctaacaataaagaagccattcgggcttctttaatcataggacgggccattagtgttcgtcgcctccagtaatgatgatctcctgttccagcaagatgaatgcatacaggtctatatttgctgttccattctttaggcacaataaattggaaccttgcaataacagattcaattggcatgatatcaggcacatagtgagccatgggggaaacaaagtgtccatctaagatcttacaatctgattgctcttcaatcttatcaatgtgtactggataatcgcttgaaaccagattctggcatctttcccgatttccaatcatctttctgaattcaaagagtcttttgagatcttctggccttccccatcctctgataaaaagttttgttaggagaagtctccggtatagaatatctaacttgctcacacccatcagtagcaaacaagcattggccgccaggtggaagcctgcgatcgagctggccgggcctcccagcaccgccgctctccaggctccctttccaggactcaactttggtcccagccccaatcgcagctccggtaacctttccaggaaccgaaatgctagatacagcggaaggagaaacggagggaggaagacaaacccggagcagggcggcgcggcagttt

SEQ ID NO: 15109 - RNA, 7457 nt, Homo sapiens
  source 1..7457: mol_type = other RNA
gctgggattacaggcatgagccactgcacccggcctctgatacatattttcaaagccttaataattttctgtcatgactacttctactgtgtctatacatttagcataatttcaaaaggactagataaaatttttaatgttaatctgaaggggaaaaaaggagtagaattaggagccagagttgtttaaatgtggaatatgttgtatagtggtcacatggtactggtggtaatagtggcagaaatggcaaaagagccattggttgataaggttcaggagggcctaggctgttcctttgtaaactgtgctcagatatactctcttggctgtcctgggactcctacagggcttgaacattttgtatcaatttctgttttgaaggtgctgggactctggtgcccccaaccctgggcatcctcaggctttgaggagaatacacaggatttgaagtcagaagacctaggtttgagttctggctgagccacgcactgttcatgtgaccttggacaaatcaccaaatttttctgaacagcatctgtaaagtgacagtaacccctacctcacagggttgttgtgaggattacatatatgctaaagcattttgcatatgaaaaagcttcttatgaatattgttattcctaggcaaaccccccttggaagctgtcaaaaaggacaactgtagatgaaattgtcttccttttttcttcattcagcttagcctttctgtttggccagggctacttacaggggctgttggggttgaagtcaagtcaccgcattttggctcctttggtcaaagagaaagaactctaatgtccagctgctccatcgatatactcatagaatggaagtgagcaaaggaaaattttaagccaggatagttaaccgttagggggccagtgggagaatgcttgccttgcatttgcacatccagaatgactaaaacatcttaagtaaatgaggaatagccaccgagatgctcagagataatataagccatgagtgggaagtgggaaaatgagtttgtcaacgccctctcttttctatccctttacctttgaggtcagggacagggcatattactgacaccccactggctattgccctatacctgccaatcacccaaagaaaataatagcttctgagaaagctcaattcactgtagcaactgtgatatatttaccctaataaagccaccacttggtcttttccagtgcttctctcttatggagatcatccctggaatccaaagctctccagttttctaacccagttaagagttaaaaacaaccacaggtcatgagcagtaggcttggcagttataccccatgcagtcataggagactgctccatcattctcagcacatagggtgcacatctcactatctctggcatgaaccagccttgcgaacttatacagtctcagccactctgctttgatggtaattcttcaccactgatctctcctcaccatgcccttcctgcatccttcccccaaccacccaccagaggagttctggtccccaaaccaaagagttgcctgcaggttggtaatgtgactttgtagatattccttgattaaagccagaccctattggtatcctttttgaagtactggatcgaaatctaattgcttttttttttaattgttggggagaggaggatgagcagaactcctatgcagcctgagagaagttctctatgtgtctgtatatgtacacctctgtgtgtgtgtgtgtaacctcatggttgtgctcaggctgacagggagggcaaagagtgaaaaggaagcatctctttcttgttatccaacattgcttcaaagatgcccaacccccgtagtagcaggcagttcccaagtggagggtcggggcagaggcctccaccaaggccatcaataaccaggtgtgagctacaggtctctgtgtaatgtgaagctctcccgtatttcatttctgcacccagggggcggctctgcaggattgcttacggagaactctgtgtctggcacctctctccacaaggcccaggcgcccagggtcccaccgacctgcccaggaatgcatcacattgttctctggtgctgtaatttggctgcaggagctaggctgaatgcctcccagggatgagaaacatactctccctggcgtcctcccttcgccccagctagcttgagcttctgccctatgaccactgagtgcatttaaataaaaacctcagaaagactgaggaaaaaaaaatcctaattatctctcttctgttaagccatgtagagactcgtgtcctgagtgggtctgagaatttggcaaagacttactggttggtgttcttgataagggaagtgagacaaaggagaagaaattactccctgcaacaggaggaatagaaatgaagcagtgagtgttcagaaattagatctacaagaagttttgcaaacagaccctcagggccaggcaatgtttgtttttgttttttgttttttgtttttttttttaatctgaagcccctgattttatttttccagcatcactctaaggaagagtgtggattagtgccattattcagggctggtattaataaaagttagcttttatctgcagggctaggttaaggctggcattcttacttttacattaaaaaaactggctacaggctgcgcagctgaggtacttcagtcatgtgccttctctaaaggattcttagatccttaaaatatatagtatgttttaagtttgtatctaaatagcacttactgtaatgtattatacctaaatgtttattaaaagttagaagaaatgagtaccaacaggaaggaatggaagagaggagaggggctaagacattgctgatctgagggacagacctctatcaaatagaagagggctgggagaaggggtgattagaagcagagtgagggaactaaatggagccctgactgcaccaaataaagttctcattttgctgcttgttccaaataaattagtgtctatttgtgtaatgcagactaaatgccagttgtgtaaagccaatcaatgcagaagcaagctaagaactaggaggaaaaattaattgcttggccatcattccttttgggaccacataacctccgtggtggggctcaaatggacatcatttctctcttatgcacctctcttttcaaacttctcactctctggacagcttgctcttttcttaaccatttataggaaattgcaaaacttgcatctttatgagctagaatttggagcccaaggaaaagcacagagtagcatgagatgccagaagaggcccatttccttccacagggatgagaaccaaaaaccaaagaatagagagtagggtataggtagatttaagtcaggttgacgtcctatggaaggcatatgccattatttatgtggtaacctgcatgttcttgtgagaacaggggctggccaggacctgaggctttccccagcagcctggcatataatataaggcagcttcctttggtaaattcattcagccctattgttgagttcagactgaccatgacccccttacctctccactaccccaaagctttcctcaagatgtcagctgttctcttcccctcccatttccccctccttaatcccaccattggctcatcagttatccagttgactccattctgaaggaagacattctcttggcctgactcactcaggcccatttctccacaggcatccccttaccgcagaccacaagggccctgactagctcatgttttgtgttaatggatgtgaaaccagagcaaatcccctcaccaaaagaaaaaccaccctaaactctcccacacaggtctcagcaggttacacaaatattagtcctatcatccaaataaatctgcccccgtggcccagagctatggctcccccaacctcctgctgcctgtgcagagtgaagctgcttcaaaaacatgaggaccccaagggatattggagaggaactttggaaagacaggggcctgtatccagaattctttatgcaggctccttaatctacagacttttgttaatactttatagtcctaaagaaggactgttcctagagaagtcatgatgggctagaccagccaggggctttggtgaagaggatctgcgggctggagtttggtgcataattaaaactcagcgtctgacagctgggcacagtggcttgcgcttgtacgcccagcactttggaaggctgcagtgggaggattgcttgagaccaagaattcaagaccagcctgggcaacatagtgagctccatctctgaaaactatgtttaaattagctgggcatgatggcatggccctgtagtcccagctaatggggaggctgaggtgggaggattgcttgagcctgggaatttgaggctgcagtgagccatgatcatgccagtgcactccagcctgggcaacaaagcgagaccctatctctaaaagaaataaaaagaaagaaaaaaaagaacaggtacgtatcctcattttacagatgagaaaatagaagctcagaaaatttagctaccttgctcaaaatatcaaagcaaatggcacagctgtgatttttaacccgggtctgtcataaccgcaaatttctataccactctgctgctttaagatatcaacaggcaaaagataaccactgtccaactcacataaaaataggacatcaagttttgggggacttcatgtcctacctccagcttactaagcctgctatctctggagattccactactgcaaacctagttaggcaatgggtaatagcattacccattaagccaaatgtggagtgaacaataataataatcactaggacttggagagtcactaaataaagatttgttgagtaagtggaggaaggctgccttctaagctgtgtatcactttggccccaacctgcagtactccttcccactgtagccactgactcctgctcccagcttcaaaggctaggatcctctcataaagaattaccaaagccagagatccctacctgcctaatatatactgatgcctcatgtgggcccttgagatcagacctgcttacctgctctcccaccatccatgagttgcctatctttcttttactccatgtctccccaaacctggcaaacctccagaatagtgcatgggaagagaagaaaagaaaagaaaaaaaaaaaaaaaaaaaaggcaacacaaggcctagccagacttactacattaatctatcctaggagtgttctagggtgttttaatgatttgttaagcatgggaaccactgcattccacctcagtttgaacaggcagcaagtaagcaaaagaggcagtgctgtccaatacaggttgagaatggtagagagaaaaagagagaatgaatgtgtgtttgtattgttatgattctttttcttctacaaaacacagtttataaacatatgagcatgtgaatggaaccttgtccactatggctaacatctcaggctctcaataatagaatgtggtagcctaagattttctttcggggtaccaggtagttctgctcaaacggacttcagagaagggacatgccattcatctttgtcccatctaactttggccaggtagaaacaaaaagaagctctctacaggtacccttcctcttgcacaccaagaagtatcgggaagctggtgcaaaggaaagaaaaaaggagcctcaactacgtactttagtgcaactcatttcactctaaagaccccctatctcttctactctcccttcaaatctccagagcgggaaatcagggagcttgctcagtttcttatatcccctgacaactccttcccagggctaaggaaccagccaggacaccatggtccctatggattactctctacatccttaaatagaagcggtagcagcccagggtggagggtggaggaaggtgtgcatgcaaggatcttgtgcttttgagttgagaggcttgaattggagggatgagtgaggtatctgtgtgttcaggtttggtccagccactctgccttcttgggggctttgcaagtatggacgtccacagtatttctgcattccttgcaccgtacagcacagcaccagtggaatttgcactcacactgggtaacacgggtgactcgagttgtgtcgtaccctcggccacagcacatgatttcacaaccgtctgttccttttgatgtcttgctgcagacacggcctgcagtgcctagggaacctgcagccttgtccaagacacagtaatctggagagttgtcaaagtagacaagatcagtccgggtggcacggcgatagccttggcgggctgcggtgaagttggcaccatcttgggtggccatcacctgcacagccccatcatagcgtcgccgcaggtaatcacctgtgcggcggaaatctgagagtgcacgccagcaggtgcgcagagtacaggaaccactcacgccatggcacttacactccagcttcagaaaccgccgcacagccgtgcgaccacagcggttattatgtaagttcatgagggcccgggcatccttaagcctcttctccttggcatccacgaaggccttggcaaaacggacaccgtagtggatgttgtcactgcagccaccccagtcaaagtccccacgctggtcatggtgtcggccacgggtgtaggggtcacagctgcacacactcagttcaccctggctacaggcgcgagtaatagcgtggactacccctgctgatgagatggcatatacaaaagctgcctctcggctacttctgagcatgacacggccaaagacggtgtggtcccggtccagggtggtacagttccagcggtggtggcggaattggtgctgacactctcggatccattctcgggcaccctcgcccactgaacgcatgatgtctgggtaacgctggcacagctgccgctgccggctcaccaaaccagggatattgtcacagatcactcgtgcccccagtgccccaatgtaccaccaggacgtgtctacgcgggccggcagcgtcagcagcagcaggagcagaaggcaggcaagacctaggcgggccgaagcccgggagccgtcgggggccgcgggcgacggcacagggaccggggcgctggcgcgccgaagcgggagctgcgcagcttcctccgcaccacccggtctcagcatagctccccgaagactcccgccgcgcagcccggaggggcgtggacggggcaccttctgggggtactcaggctgctcctacctcacccccctggggggccatggtgttcgccggcggctggggacctaggatcacctggggtccagagcccgggaggaggatccccgagaggggcgcaagttgcgatgtccggaagccgacgacggcgtgccgaacccggggtctggggcgcgctgcctgaggaccgggtgcggtgtcagggggtctgcggcgctgaagggagctgcgggcctagtgtgc

SEQ ID NO: 15110 - RNA, 3011 nt, Homo sapiens
  source 1..3011: mol_type = other RNA
gctgggattacaggcatgagccactgcacccggcctgggttctttattaaagcaatgaattctggatgtcctggcttaactagattaagagggaatgaagcttcttctgaaggatcagtgttaccacagccatttccttgcattacaccgtccttctcaggacgtctatgagaagccctgggcagcctggacagggactgccccatgagtgctggtggctcacttggggctttctgcaggtgaaggaagcagccctgggagcttcttcctttggcacacagtgggcttcagctgggactgcaccaatcctctgctaacagcaaccatccttggggggtccgagggagcagctgcgtgacttttcagcagtggctatggtcactcctgaggcctgggaagagggtcactgtccagcagagctggcctgctccagagtgatctggaccttgtgccccttaacacaagaaggcccgactccaaaggccaacactgtcctctaagtttccaggacactaaatggccacttggtcctggttaactcatttctaaacacaaaggggacaggtctgagaaagtggcgttctctaccctaccctgagctcatctgttctgaggacaaaagggacgggtgtgtccaggctggtggcaaaggctgcatttccggggtttctttgctgtggaccccatgtctgaggaactggcccggggccttttgcttctggcttccgactccagggttcttcctctgtctcctgtccaggacggggctccagaagtccctggagcggtgttctcatcgacccactggaaaaagccacactgctgctctctcggcttggcacatgtgtggaactggcgccccttgttgggtccatccttctgcacagtccgtgtgacggagggctggctgcaaaggcaggatgtgccactaccactgccatcaccagggttgccaaacccacctaggtggatccctgggcctggtgggcatcccagggaggcgcccaggggtctatatgccaaggcaggaggccctcctgctcccggattggggctgtctgcccacaggaagaagttgcagctacctccgttgcacttaaagaactgccggccccggttggggccctccttacggacagtgagcagcacagcctcctggccacagttgcaggtcacagaattgctttcaccagcagccgtgggtggtgggagggtctgggccagagcctttgaggacccagtctgtctgctgtcagcaggctgggggtgctggctgttgtccatcctgttcagggactggttagcctgcaggcggccagagggctggctagccctgggggggccccctgaaaatctcaggtccaggatctccctcagggtgtcgtcgcatccgccgatgcagcaaacaaactccagaggcatggtcgggggaaggctaccgcgcttaaactttaactttaacctgtacacagggtgtggctgacaaactggacacacactgctgtccctgctggcctccagcaccgagtcaggaagccacacagctgagcgacactctgggaaacccatgcagctgaggtagaacccgccattcttcttggtcttaaggaccatgtccttgttgcactgtgggcacttcctgatgggctctggcatggctgggtagatatcttcttgctgggccaactctgtcccattcccaaagtactgggccaaggcctcgtccaatttctttgctttagccaccgcttcaatgaaaacctgcttgtatttctgcacttgctgccttagaaccacaaatttgtcctttttgccatcacagatcagcttcagatcagcttccagttcagcccggaggtcaggcttagacatttcatagcccatggaatcataaccttccacaagtcccatgcccaggtgcccagggaggaaccgcttgtctggggtgaggcccacgtacatccgggctttgatggtctcgatgtgctccgcatgagtggcatccgtaccaatgccatgcttctccatgagggcaatgaggtcggcctcggtgagcagcttgggtgggctggtctccccgtccaccatctccacggtgctgggctgaaagtgggatccttgctcatagacagggaggatcttgtcactccagtgatcatatggatacacatccagatagtttcgggccagaatcatgaggccatgggccacaaagcgttcctgagcgatgtcgatctccactgtggtctcctgcccctgagcatcctgggagcagcaagccaggaaatggcgaacaataaactcgtacagtcgctgttcatctccccttgagtgtagagcttctcagcaatcctcatggtttctttagcatttattctcaactttcgagaagccagcttctcaagctccacagtgtccaaggcttgaggccgccacttgctcttgggcttagatctgacctctaccacagttgccatgggatcctccacacacaactgatagagaactaggcaagccgtgtggttaaagagtcgatgccttttccagttgaattctacgataccatctttgtggtcatgagttactttaattctgtggaagatttctggtacaaaagcctgaatggctttgaaccgctccaccacaaagcccagtgtggggaactggcagctgccgtaactgatgagctgctctgccagcacctcaggaaaaatcctctgaagccgcagggtctggaacctagtaaaggcagctccaatcctcaggtccagctcctgcctcacatccacagcatcgctcaccctctgatcaggctcggtcaggttttcacaagctgtcctgacggcatggggtgtgatctcagagaatcgggctcgcaacacctgcagattgggctttacagccttacacacgtggataatctcaaacccgatgttttcgccttctctatcacagtcagtccagatcaccagagcctggcactggcgagtctctcgttccaaagttttctt

SEQ ID NO: 15111 - RNA, 3822 nt, Homo sapiens
  source 1..3822: mol_type = other RNA
gctgggattacaggcatgagccactgcacccggcctgggttctttattaaagcaatgaattctggatgtcctggcttaactagattaagagggaatgaagcttcttctgaaggatcagtgttaccacagccatttccttgcattacaccgtccttctcaggacgtctatgagaagccctgggcagcctggacagggactgccccatgagtgctggtggctcacttggggctttctgcaggtgaaggaagcagccctgggagcttcttcctttggcacacagtgggcttcagctgggactgcaccaatcctctgctaacagcaaccatccttggggggtccgagggagcagctgcgtgacttttcagcagtggctatggtcactcctgaggcctgggaagagggtcactgtccagcagagctggcctgctccagagtgatctggaccttgtgccccttaacacaagaaggcccgactccaaaggccaacactgtcctctaagtttccaggacactaaatggccacttggtcctggttaactcatttctaaacacaaaggggacaggtctgagaaagtggcgttctctaccctaccctgagctcatctgttctgaggacaaaagggacgggtgtgtccaggctggtggcaaaggctgcatttccggggtttctttgctgtggaccccatgtctgaggaactggcccggggccttttgcttctggcttccgactccagggttcttcctctgtctcctgtccaggacggggctccagaagtccctggagcggtgttctcatcgacccactggaaaaagccacactgctgctctctcggcttggcacatgtgtggaactggcgccccttgttgggtccatccttctgcacagtccgtgtgacggagggctggctgcaaaggcaggatgtgccactaccactgccatcaccagggttgccaaacccacctaggtggatccctgggcctggtgggcatcccagggaggcgcccaggggtctatatgccaaggcaggaggccctcctgctcccggattggggctgtctgcccacaggaagaagttgcagctacctccgttgcacttaaagaactgccggccccggttggggccctccttacggacagtgagcagcacagcctcctggccacagttgcaggtcacagaattgctttcaccagcagccgtgggtggtgggagggtctgggccagagcctttgaggacccagtctgtctgctgtcagcaggctgggggtgctggctgttgtccatcctgttcagggactggttagcctgcaggcggccagagggctggctagccctgggggggccccctgaaaatctcaggtccaggatctccctcagggtgtcgtcgcatccgccgatgcagcaaacaaactccagaggcatggtcgggggaaggctaccgcgcttaaactttaactttaacctgtacacagggtgtggctgacaaactggacacacactgctgtccctgctggcctccagcaccgagtcaggaagccacacagctgagcgacactctgggaaacccatgcagctgaggtagaacccgccattcttcttggtcttaaggaccatgtccttgttgcactgtgggcacttcctgatgggctctggcatggctgggtagatatcttcttgctgggccaactctgtcccattcccaaagtactgggccaaggcctcgtccaatttctttgctttagccaccgcttcaatgaaaacctgcttgtatttctgcacttgctgccttagaaccacaaatttgtcctttttgccatcacagatcagcttcagatcagcttccagttcagcccggaggtcaggcttagacatttcatagcccatggaatcataaccttccacaagtcccatgcccaggtgcccagggaggaaccgcttgtctggggtgaggcccacgtacatccgggctttgatggtctcgatgtgctccgcatgagtggcatccgtaccaatgccatgcttctccatgagggcaatgaggtcggcctcggtgagcagcttgggtgggctggtctccccgtccaccatctccacggtgctgggctgaaagtgggatccttgctcatagacagggaggatcttgtcactccagtgatcatatggatacacatccagatagtttcgggccagaatcatgaggccatgggccacaaagcgttcctgagcgatgtcgatctccactgtggtctcctgcccctgagcatcctgggagcagcaagccaggaaatggcgaacaataaactcgtacagtcgctgttcatctccctgtaagttgttggtgtatttggtggggtgaatgggagggtgagcttggtcagacttgttcccattgcgtggggtgggaccaccccgctctagaatgctctgggcaaaggccccccagcgtggatcgggggtctgctgttccaccaacaccgtcaggtttaagtctctgggaaaaatgtttgtttctgttcggggatagctgatgtacccttgagtgtagagcttctcagcaatcctcatggtttctttagcatttattctcaactttcgagaagccagcttctcaagctccacagtgtccaaggcttgaggccgccacttgctcttgggcttagatctgacctctaccacagttgccatgggatcctccacacacaactgatagagaactaggcaagccgtgtggttaaagagtcgatgccttttccagttgaattctacgataccatctttgtggtcatgagttactttaattctgtggaagatttctggtacaaaagcctgaatggctttgaaccgctccaccacaaagcccagtgtggggaactggcagctgccgtaactgatgagctgctctgccagcacctcaggaaaaatcctctgaagccgcagggtctggaacctagtaaaggcagctccaatcctcaggtccagctcctgcctcacatccacagcatcgctcaccctctgatcaggctcggtcaggttttcacaagctgtcctgacggcatggggtgtgatctcagagaatcgggctcgcaacacctgcagattgggctttacagccttacacacgtggataatctcaaacccgatgttttcgccttctctatcacagtcagtccagatcaccagagcctggcactggcgagtctctcgttccaaagttttcttgatgtctacaaaattctctgggcagtacttttcaatttctgcttcaaagaggacaagagggttgcagctctgccattttcgaaactgcatctggaaatcatgagccagtaaatgtccagaaactgaagtcattaccatggtaacattctggccatacagatgataatcaaattcatagatcttgttgaattttgaaagtccttctctccgcctcatgcgaccgtttgacagcaggtcggcgatccccttggccgcgtcgtttttttcggccacacagaggactttccgcacgcctcggagggccatctccatggcggcgcgggaaaaggcacggtcttcgggccgtcgcagccaccggagcgcgtagcgggcgacaggaaagatcatcctcagacctcgcgcccggagccgctccccggctgccggcgcatcctggggaagccagagatgaggctcaaatggcgcccaccgaaagggaaccagagcctcgcttcggtcacgtccccaccagcctgctggcctttggagcttcagtcactgagcctttcccgtgccgcagccgccgcctcagcaccgaatccagtatcttggcgtggaacttcc

SEQ ID NO: 15112 - RNA, 3748 nt, Homo sapiens
  source 1..3748: mol_type = other RNA
gctgggattacaggcatgagccactgcacccggcctgggttctttattaaagcaatgaattctggatgtcctggcttaactagattaagagggaatgaagcttcttctgaaggatcagtgttaccacagccatttccttgcattacaccgtccttctcaggacgtctatgagaagccctgggcagcctggacagggactgccccatgagtgctggtggctcacttggggctttctgcaggtgaaggaagcagccctgggagcttcttcctttggcacacagtgggcttcagctgggactgcaccaatcctctgctaacagcaaccatccttggggggtccgagggagcagctgcgtgacttttcagcagtggctatggtcactcctgaggcctgggaagagggtcactgtccagcagagctggcctgctccagagtgatctggaccttgtgccccttaacacaagaaggcccgactccaaaggccaacactgtcctctaagtttccaggacactaaatggccacttggtcctggttaactcatttctaaacacaaaggggacaggtctgagaaagtggcgttctctaccctaccctgagctcatctgttctgaggacaaaagggacgggtgtgtccaggctggtggcaaaggctgcatttccggggtttctttgctgtggaccccatgtctgaggaactggcccggggccttttgcttctggcttccgactccagggttcttcctctgtctcctgtccaggacggggctccagaagtccctggagcggtgttctcatcgacccactggaaaaagccacactgctgctctctcggcttggcacatgtgtggaactggcgccccttgttgggtccatccttctgcacagtccgtgtgacggagggctggctgcaaaggcaggatgtgccactaccactgccatcaccagggttgccaaacccacctaggtggatccctgggcctggtgggcatcccagggaggcgcccaggggtctatatgccaaggcaggaggccctcctgctcccggattggggctgtctgcccacaggaagaagttgcagctacctccgttgcacttaaagaactgccggccccggttggggccctccttacggacagtgagcagcacagcctcctggccacagttgcaggtcacagaattgctttcaccagcagccgtgggtggtgggagggtctgggccagagcctttgaggacccagtctgtctgctgtcagcaggctgggggtgctggctgttgtccatcctgttcagggactggttagcctgcaggcggccagagggctggctagccctgggggggccccctgaaaatctcaggtccaggatctccctcagggtgtcgtcgcatccgccgatgcagcaaacaaactccagaggcatggtcgggggaaggctaccgcgcttaaactttaactttaacctgtacacagggtgtggctgacaaactggacacacactgctgtccctgctggcctccagcaccgagtcaggaagccacacagctgagcgacactctgggaaacccatgcagctgaggtagaacccgccattcttcttggtcttaaggaccatgtccttgttgcactgtgggcacttcctgatgggctctggcatggctgggtagatatcttcttgctgggccaactctgtcccattcccaaagtactgggccaaggcctcgtccaatttctttgctttagccaccgcttcaatgaaaacctgcttgtatttctgcacttgctgccttagaaccacaaatttgtcctttttgccatcacagatcagcttcagatcagcttccagttcagcccggaggtcaggcttagacatttcatagcccatggaatcataaccttccacaagtcccatgcccaggtgcccagggaggaaccgcttgtctggggtgaggcccacgtacatccgggctttgatggtctcgatgtgctccgcatgagtggcatccgtaccaatgccatgcttctccatgagggcaatgaggtcggcctcggtgagcagcttgggtgggctggtctccccgtccaccatctccacggtgctgggctgaaagtgggatccttgctcatagacagggaggatcttgtcactccagtgatcatatggatacacatccagatagtttcgggccagaatcatgaggccatgggccacaaagcgttcctgagcgatgtcgatctccactgtggtctcctgcccctgagcatcctgggagcagcaagccaggaaatggcgaacaataaactcgtacagtcgctgttcatctccctgtaagttgttggtgtatttggtggggtgaatgggagggtgagcttggtcagacttgttcccattgcgtggggtgggaccaccccgctctagaatgctctgggcaaaggccccccagcgtggatcgggggtctgctgttccaccaacaccgtcaggtttaagtctctgggaaaaatgtttgtttctgttcggggatagctgatgtacccttgagtgtagagcttctcagcaatcctcatggtttctttagcatttattctcaactttcgagaagccagcttctcaagctccacagtgtccaaggcttgaggccgccacttgctcttgggcttagatctgacctctaccacagttgccatgggatcctccacacacaactgatagagaactaggcaagccgtgtggttaaagagtcgatgccttttccagttgaattctacgataccatctttgtggtcatgagttactttaattctgtggaagatttctggtacaaaagcctgaatggctttgaaccgctccaccacaaagcccagtgtggggaactggcagctgccgtaactgatgagctgctctgccagcacctcaggaaaaatcctctgaagccgcagggtctggaacctagtaaaggcagctccaatcctcaggtccagctcctgcctcacatccacagcatcgctcaccctctgatcaggctcggtcaggttttcacaagctgtcctgacggcatggggtgtgatctcagagaatcgggctcgcaacacctgcagattgggctttacagccttacacacgtggataatctcaaacccgatgttttcgccttctctatcacagtcagtccagatcaccagagcctggcactggcgagtctctcgttccaaagttttcttgatgtctacaaaattctctgggcagtacttttcaatttctgcttcaaagaggacaagagggttgcagctctgcctggccatacagatgataatcaaattcatagatcttgttgaattttgaaagtccttctctccgcctcatgcgaccgtttgacagcaggtcggcgatccccttggccgcgtcgtttttttcggccacacagaggactttccgcacgcctcggagggccatctccatggcggcgcgggaaaaggcacggtcttcgggccgtcgcagccaccggagcgcgtagcgggcgacaggaaagatcatcctcagacctcgcgcccggagccgctccccggctgccggcgcatcctggggaagccagagatgaggctcaaatggcgcccaccgaaagggaaccagagcctcgcttcggtcacgtccccaccagcctgctggcctttggagcttcagtcactgagcctttcccgtgccgcagccgccgcctcagcaccgaatccagtatcttggcgtggaacttcc

SEQ ID NO: 15113 - RNA, 3851 nt, Homo sapiens
  source 1..3851: mol_type = other RNA
gctgggattacaggcatgagccactgcacccggcctgggttctttattaaagcaatgaattctggatgtcctggcttaactagattaagagggaatgaagcttcttctgaaggatcagtgttaccacagccatttccttgcattacaccgtccttctcaggacgtctatgagaagccctgggcagcctggacagggactgccccatgagtgctggtggctcacttggggctttctgcaggtgaaggaagcagccctgggagcttcttcctttggcacacagtgggcttcagctgggactgcaccaatcctctgctaacagcaaccatccttggggggtccgagggagcagctgcgtgacttttcagcagtggctatggtcactcctgaggcctgggaagagggtcactgtccagcagagctggcctgctccagagtgatctggaccttgtgccccttaacacaagaaggcccgactccaaaggccaacactgtcctctaagtttccaggacactaaatggccacttggtcctggttaactcatttctaaacacaaaggggacaggtctgagaaagtggcgttctctaccctaccctgagctcatctgttctgaggacaaaagggacgggtgtgtccaggctggtggcaaaggctgcatttccggggtttctttgctgtggaccccatgtctgaggaactggcccggggccttttgcttctggcttccgactccagggttcttcctctgtctcctgtccaggacggggctccagaagtccctggagcggtgttctcatcgacccactggaaaaagccacactgctgctctctcggcttggcacatgtgtggaactggcgccccttgttgggtccatccttctgcacagtccgtgtgacggagggctggctgcaaaggcaggatgtgccactaccactgccatcaccagggttgccaaacccacctaggtggatccctgggcctggtgggcatcccagggaggcgcccaggggtctatatgccaaggcaggaggccctcctgctcccggattggggctgtctgcccacaggaagaagttgcagctacctccgttgcacttaaagaactgccggccccggttggggccctccttacggacagtgagcagcacagcctcctggccacagttgcaggtcacagaattgctttcaccagcagccgtgggtggtgggagggtctgggccagagcctttgaggacccagtctgtctgctgtcagcaggctgggggtgctggctgttgtccatcctgttcagggactggttagcctgcaggcggccagagggctggctagccctgggggggccccctgaaaatctcaggtccaggatctccctcagggtgtcgtcgcatccgccgatgcagcaaacaaactccagaggcatggtcgggggaaggctaccgcgcttaaactttaactttaacctgtacacagggtgtggctgacaaactggacacacactgctgtccctgctggcctccagcaccgagtcaggaagccacacagctgagcgacactctgggaaacccatgcagctgaggtagaacccgccattcttcttggtcttaaggaccatgtccttgttgcactgtgggcacttcctgatgggctctggcatggctgggtagatatcttcttgctgggccaactctgtcccattcccaaagtactgggccaaggcctcgtccaatttctttgctttagccaccgcttcaatgaaaacctgcttgtatttctgcacttgctgccttagaaccacaaatttgtcctttttgccatcacagatcagcttcagatcagcttccagttcagcccggaggtcaggcttagacatttcatagcccatggaatcataaccttccacaagtcccatgcccaggtgcccagggaggaaccgcttgtctggggtgaggcccacgtacatccgggctttgatggtctcgatgtgctccgcatgagtggcatccgtaccaatgccatgcttctccatgagggcaatgaggtcggcctcggtgagcagcttgggtgggctggtctccccgtccaccatctccacggtgctgggctgaaagtgggatccttgctcatagacagggaggatcttgtcactccagtgatcatatggatacacatccagatagtttcgggccagaatcatgaggccatgggccacaaagcgttcctgagcgatgtcgatctccactgtggtctcctgcccctgagcatcctgggagcagcaagccaggaaatggcgaacaataaactcgtacagtcgctgttcatctccctgtaagttgttggtgtatttggtggggtgaatgggagggtgagcttggtcagacttgttcccattgcgtggggtgggaccaccccgctctagaatgctctgggcaaaggccccccagcgtggatcgggggtctgctgttccaccaacaccgtcaggtttaagtctctgggaaaaatgtttgtttctgttcggggatagctgatgtacccttgagtgtagagcttctcagcaatcctcatggtttctttagcatttattctcaactttcgagaagccagcttctcaagctccacagtgtccaaggcttgaggccgccacttgctcttgggcttagatctgacctctaccacagttgccatgggatcctccacacacaactgatagagaactaggcaagccgtgtggttaaagagtcgatgccttttccagttgaattctacgataccatctttgtggtcatgagttactttaattctgtggaagatttctggtacaaaagcctgaatggctttgaaccgctccaccacaaagcccagtgtggggaactggcagctgccgtaactgatgagctgctctgccagcacctcaggaaaaatcctctgaagccgcagggtctggaacctagtaaaggcagctccaatcctcaggtccagctcctgcctcacatccacagcatcgctcaccctctgatcaggctcggtcaggttttcacaagctgtcctgacggcatggggtgtgatctcagagaatcgggctcgcaacacctgcagattgggctttacagccttacacacgtggataatctcaaacccgatgttttcgccttctctatcacagtcagtccagatcaccagagcctggcactggcgagtctctcgttccaaagttttcttgatgtctacaaaattctctgggcagtacttttcaatttctgcttcaaagaggacaagagggttgcagctctgctataatctgaaagtccttcccttgagaattgtactgaccattttcgaaactgcatctggaaatcatgagccagtaaatgtccagaaactgaagtcattaccatggtaacattctggccatacagatgataatcaaattcatagatcttgttgaattttgaaagtccttctctccgcctcatgcgaccgtttgacagcaggtcggcgatccccttggccgcgtcgtttttttcggccacacagaggactttccgcacgcctcggagggccatctccatggcggcgcgggaaaaggcacggtcttcgggccgtcgcagccaccggagcgcgtagcgggcgacaggaaagatcatcctcagacctcgcgcccggagccgctccccggctgccggcgcatcctggggaagccagagatgaggctcaaatggcgcccaccgaaagggaaccagagcctcgcttcggtcacgtccccaccagcctgctggcctttggagcttcagtcactgagcctttcccgtgccgcagccgccgcctcagcaccgaatccagtatcttggcgt

SEQ ID NO: 15114 - RNA, 3881 nt, Homo sapiens
  source 1..3881: mol_type = other RNA
gctgggattacaggcatgagccactgcacccggcctgggttctttattaaagcaatgaattctggatgtcctggcttaactagattaagagggaatgaagcttcttctgaaggatcagtgttaccacagccatttccttgcattacaccgtccttctcaggacgtctatgagaagccctgggcagcctggacagggactgccccatgagtgctggtggctcacttggggctttctgcaggtgaaggaagcagccctgggagcttcttcctttggcacacagtgggcttcagctgggactgcaccaatcctctgctaacagcaaccatccttggggggtccgagggagcagctgcgtgacttttcagcagtggctatggtcactcctgaggcctgggaagagggtcactgtccagcagagctggcctgctccagagtgatctggaccttgtgccccttaacacaagaaggcccgactccaaaggccaacactgtcctctaagtttccaggacactaaatggccacttggtcctggttaactcatttctaaacacaaaggggacaggtctgagaaagtggcgttctctaccctaccctgagctcatctgttctgaggacaaaagggacgggtgtgtccaggctggtggcaaaggctgcatttccggggtttctttgctgtggaccccatgtctgaggaactggcccggggccttttgcttctggcttccgactccagggttcttcctctgtctcctgtccaggacggggctccagaagtccctggagcggtgttctcatcgacccactggaaaaagccacactgctgctctctcggcttggcacatgtgtggaactggcgccccttgttgggtccatccttctgcacagtccgtgtgacggagggctggctgcaaaggcaggatgtgccactaccactgccatcaccagggttgccaaacccacctaggtggatccctgggcctggtgggcatcccagggaggcgcccaggggtctatatgccaaggcaggaggccctcctgctcccggattggggctgtctgcccacaggaagaagttgcagctacctccgttgcacttaaagaactgccggccccggttggggccctccttacggacagtgagcagcacagcctcctggccacagttgcaggtcacagaattgctttcaccagcagccgtgggtggtgggagggtctgggccagagcctttgaggacccagtctgtctgctgtcagcaggctgggggtgctggctgttgtccatcctgttcagggactggttagcctgcaggcggccagagggctggctagccctgggggggccccctgaaaatctcaggtccaggatctccctcagggtgtcgtcgcatccgccgatgcagcaaacaaactccagaggcatggtcgggggaaggctaccgcgcttaaactttaactttaacctgtacacagggtgtggctgacaaactggacacacactgctgtccctgctggcctccagcaccgagtcaggaagccacacagctgagcgacactctgggaaacccatgcagctgaggtagaacccgccattcttcttggtcttaaggaccatgtccttgttgcactgtgggcacttcctgatgggctctggcatggctgggtagatatcttcttgctgggccaactctgtcccattcccaaagtactgggccaaggcctcgtccaatttctttgctttagccaccgcttcaatgaaaacctgcttgtatttctgcacttgctgccttagaaccacaaatttgtcctttttgccatcacagatcagcttcagatcagcttccagttcagcccggaggtcaggcttagacatttcatagcccatggaatcataaccttccacaagtcccatgcccaggtgcccagggaggaaccgcttgtctggggtgaggcccacgtacatccgggctttgatggtctcgatgtgctccgcatgagtggcatccgtacctggtacactgtaagccttagctcaagagatgcgagttacccagaggagccactgaccaatgccatgcttctccatgagggcaatgaggtcggcctcggtgagcagcttgggtgggctggtctccccgtccaccatctccacggtgctgggctgaaagtgggatccttgctcatagacagggaggatcttgtcactccagtgatcatatggatacacatccagatagtttcgggccagaatcatgaggccatgggccacaaagcgttcctgagcgatgtcgatctccactgtggtctcctgcccctgagcatcctgggagcagcaagccaggaaatggcgaacaataaactcgtacagtcgctgttcatctccctgtaagttgttggtgtatttggtggggtgaatgggagggtgagcttggtcagacttgttcccattgcgtggggtgggaccaccccgctctagaatgctctgggcaaaggccccccagcgtggatcgggggtctgctgttccaccaacaccgtcaggtttaagtctctgggaaaaatgtttgtttctgttcggggatagctgatgtacccttgagtgtagagcttctcagcaatcctcatggtttctttagcatttattctcaactttcgagaagccagcttctcaagctccacagtgtccaaggcttgaggccgccacttgctcttgggcttagatctgacctctaccacagttgccatgggatcctccacacacaactgatagagaactaggcaagccgtgtggttaaagagtcgatgccttttccagttgaattctacgataccatctttgtggtcatgagttactttaattctgtggaagatttctggtacaaaagcctgaatggctttgaaccgctccaccacaaagcccagtgtggggaactggcagctgccgtaactgatgagctgctctgccagcacctcaggaaaaatcctctgaagccgcagggtctggaacctagtaaaggcagctccaatcctcaggtccagctcctgcctcacatccacagcatcgctcaccctctgatcaggctcggtcaggttttcacaagctgtcctgacggcatggggtgtgatctcagagaatcgggctcgcaacacctgcagattgggctttacagccttacacacgtggataatctcaaacccgatgttttcgccttctctatcacagtcagtccagatcaccagagcctggcactggcgagtctctcgttccaaagttttcttgatgtctacaaaattctctgggcagtacttttcaatttctgcttcaaagaggacaagagggttgcagctctgccattttcgaaactgcatctggaaatcatgagccagtaaatgtccagaaactgaagtcattaccatggtaacattctggccatacagatgataatcaaattcatagatcttgttgaattttgaaagtccttctctccgcctcatgcgaccgtttgacagcaggtcggcgatccccttggccgcgtcgtttttttcggccacacagaggactttccgcacgcctcggagggccatctccatggcggcgcgggaaaaggcacggtcttcgggccgtcgcagccaccggagcgcgtagcgggcgacaggaaagatcatcctcagacctcgcgcccggagccgctccccggctgccggcgcatcctggggaagccagagatgaggctcaaatggcgcccaccgaaagggaaccagagcctcgcttcggtcacgtccccaccagcctgctggcctttggagcttcagtcactgagcctttcccgtgccgcagccgccgcctcagcaccgaatccagtatcttggcgtggaacttccgc

SEQ ID NO: 15115 - RNA, 4452 nt, Homo sapiens
  source 1..4452: mol_type = other RNA
gctgggattacaggcatgagccactgcacccggctaattctcctactctaaaaaccagtcatccttgtctttcctcctcacatcaagtggccaggcctttcacaatgcctgtctttatttagtgctatctctcctgccactactctagctcagaccctgattattctctcctagaaaactaaattaacctaacccaattttttccaaagtgtggtgtattcactgctatagttactttaatgtgattaggaaaaaacactaacacatcaaaactttgatttcaaaatagaattgtgtcaagtaagaacaaaataaatctggaaatgagtagatctgaagaaaacaatgtaggcagcaatgaatatggaaaaagccatcaaaaatggtaacataaatggctgaaatgtgagaaacaccatgttagtgaatcactttgctaatctgcaaattagttaccaaattaattcttcttatatgttattcagatcacaacatatcctattcaaaatctccagtggcatccccattaactccaagtaaaattataactcctcagcctcattttaagacacaacctgttccctactctgtctaaatctacctttagagctattgtggccttctcatctctatcaatgcctttattattttgtttctctttaaatggaatgctcaggccaggtgcagtggctcacgcctgtaatcccaacactttgggaggcagaggcgggtggatcacttgaggtcaggagttcgcgaccagcctggccaacatgctgaaaccccgtccgtactaaaaatacaaaaatcagctgggcatggtggtgggtatctgtaatcacagctcctcgggaagctgagacaggagaatcgcttgaactcaagaagcagaggttgcagtgagccatgatctcaccactgcactccatccagcctgggtgacagagcgagactccatctcaaaaagagaaaaataaataaataatggaatgctcaatattcactatcccacaacccaactctgcttgtcaaaaatccacttttggaacccaataaaaatgaatatgcaagtttaacatgttggctgggcgcagtggctcaagcctgtaatcccatcactttgggaggctgaggtgggtggatcacttgaggtcaggagttccagaccagcctggccaacatggtgaaacctcacctctactaataatacaaaaattagctgggtgtggtggcaggcgcctgtgatctcagctactcgggaggctgaggtgggagaactgcttgaacccaggaggcagaggttgcagtgagctgagatcaggccactgaactccagcctaggtgacaagagtcaaactccgtctcaaaaaaaaaaaaaaaaagaaaaaaagaaaaaagttttaacatgtttatgaagtacccattacatgccttcttccatgagtttttccaattcattcccactaggatcaatctcgtcccctctactcaattcccataacactattatttgtggcattcatcacacagtatctgtagctttatgtatgttttctctcctagtagattctaagcaacttgagagtaggaatggtgcctccatctttatttctgtctccatcttaatatcctatacctagaagataccaggaagtgtcagctgaataaatgaatctgaaccttaatctcaaaggctatgcggcagtaagaaatggaatggacaaaaggaaacgtgaatttgatatgacttaaagttttagattaaggaaaacttccctacctgattatatctgtttaaaagaagagcaaaagtgtttttaacagatggaatcttgctgtgttgcccaggctggagtactacagtggctatttataggtgcaatcccactactgatcagcacaggaattttgacctgctccatttccgacctgggccagttcaccccttcttaggcaaccttgttgttctccactcccaggaggtcaccatactgatgccaaatttagtgaggacatctgacctgcatagcacactacagtgcagaactcctgggctcaagcaatcctcctgcctcagcctcccaagaagctacaggcagtacaggcaagtgccattgcacccagctaaaagaaaagcaaattttaaatacataccctgctgggaaactaaagtactaagtgaacaacacttacgtgcttggattagtataattcacagctatactattaagaaatctctgctgtgtaaattggaatgcgaattccttttttttttttgagatggagtctctctgttgcccaggctggaatgcagtggcgcgatctccgctcactgcaacctccgcctcccaggtgcaagcgattctcctgcctcagcctcccgagtagctgggattacaggcacccacccaccatgcccagctaatttttgtatttttagtagagacggggtttcaccatgttggccgagctggtctcgaactcatgacctcaggtgatccacctgccccagcctcccaaagtgctgggattataggcgtgagctaccacgcccggcctataatgggaatttctaaaatgttgatatttaattccacaatatgaaccaaggaaaattttactagcagaaatttatgtatgtaataaatcattagcctcatatgcacattatttgaaatatgcatgattggtcattttagttttcccaataataatttatcacttatcttatatcccactagtcacacactagcaggcaaatggtagcaagtctcaaatatgtaagaaaggtttaaagaagaaaaagtaaaaaaaccgtccagaattctatccattgtgtatttttctgtgactggagttgacataattagtcaatcttagcaataatgtattgggttcactgggtgttctgaggatgcaccatttgaaccaccggtaaaagggtacagaatgtgtattgagagtcacttcaatggcttctcaatgacaccacaccaaaggaggaatacctgaagagagaatggaaacactgcaggcaggatgatttaagaacctggaaataaggaatttaatcttgttcagcttgaggagtataactaaaattactatcctgagtaacctgtactaaatccatcactctggtagaatcagatcagctgagtttaaatgtcaagaaaaaatagacacacacaaaagtggctttgattacataagtcagaggagggggagcctacaatagctcttccccacatcacacccccaaggctccttcttagggacagcaacagctttgtcaatgacacaaatgcagggtggcatgaggtttccagcagcttaacattttaatttggggtgggggtggaagaaaatacataagttgctttttgctcccccatcctaatgccttggggaccagccaggctgacccaaatggaatccagagcgagagtggggccttgggttccccgaggagtaaagggggcagatccagaacagagcagaaacggtgataattatatagaggtcatgtcattgagggcgtggtccagctcctcgctaatggccttgtacttcagtttctgggcatagagctcatcttccaggtcatcaattgtcttttccagcttggctaccgatctctcagcaaactcagcacgggtctctgcctccttgagtttatcagtaagaatcttgatttcttcctcatatttatcttctttttgagagtacttctccgcctgagcctcaagagacttgaggttgttggtgacattcttcagctcctcctccagctcagaacacttagactctgccagctcagctcgttcctctgtgcgttccaagtctccttcaatgatcaccaacttacgagccacctcttcatacttcctatctgcctcttctgcaatgtgcttagcttctttgagttggatttcctggagttccatcttttcttcatcttttaaggcccggttttcaataaccttcatacctctctcactctcatcagcagctttttcagcttcttccagcttttgcagggcagtggccaggcgctcctgagcacggtccagctcttcttcaaccagctggatcctacggttcaaggaggccacctcagcctcagcatcagcagccttcttctctgccagttccagcttctcctgggcatccttcaaagcttcagaatacttgtccagctcatcctctgtccctttcagcttcttctgcatggctgccagctcatcctccagctgtttacttctttcttctgcctgcttctgctcagcttcagcttgctctgcccgatccagagcattctccttgtctaacttcagcatctgcatctttttcttgatggcctccatcatgagcagtggctgttggtaggctcacctgtgaacactggagaactggagactggggcaagaaagaaggggctgctgcctgagt

SEQ ID NO: 15116 - RNA, 4452 nt, Homo sapiens
  source 1..4452: mol_type = other RNA
gctgggattacaggcatgagccactgcacccggctaattctcctactctaaaaaccagtcatccttgtctttcctcctcacatcaagtggccaggcctttcacaatgcctgtctttatttagtgctatctctcctgccactactctagctcagaccctgattattctctcctagaaaactaaattaacctaacccaattttttccaaagtgtggtgtattcactgctatagttactttaatgtgattaggaaaaaacactaacacatcaaaactttgatttcaaaatagaattgtgtcaagtaagaacaaaataaatctggaaatgagtagatctgaagaaaacaatgtaggcagcaatgaatatggaaaaagccatcaaaaatggtaacataaatggctgaaatgtgagaaacaccatgttagtgaatcactttgctaatctgcaaattagttaccaaattaattcttcttatatgttattcagatcacaacatatcctattcaaaatctccagtggcatccccattaactccaagtaaaattataactcctcagcctcattttaagacacaacctgttccctactctgtctaaatctacctttagagctattgtggccttctcatctctatcaatgcctttattattttgtttctctttaaatggaatgctcaggccaggtgcagtggctcacgcctgtaatcccaacactttgggaggcagaggcgggtggatcacttgaggtcaggagttcgcgaccagcctggccaacatgctgaaaccccgtccgtactaaaaatacaaaaatcagctgggcatggtggtgggtatctgtaatcacagctcctcgggaagctgagacaggagaatcgcttgaactcaagaagcagaggttgcagtgagccatgatctcaccactgcactccatccagcctgggtgacagagcgagactccatctcaaaaagagaaaaataaataaataatggaatgctcaatattcactatcccacaacccaactctgcttgtcaaaaatccacttttggaacccaataaaaatgaatatgcaagtttaacatgttggctgggcgcagtggctcaagcctgtaatcccatcactttgggaggctgaggtgggtggatcacttgaggtcaggagttccagaccagcctggccaacatggtgaaacctcacctctactaataatacaaaaattagctgggtgtggtggcaggcgcctgtgatctcagctactcgggaggctgaggtgggagaactgcttgaacccaggaggcagaggttgcagtgagctgagatcaggccactgaactccagcctaggtgacaagagtcaaactccgtctcaaaaaaaaaaaaaaaaagaaaaaaagaaaaaagttttaacatgtttatgaagtacccattacatgccttcttccatgagtttttccaattcattcccactaggatcaatctcgtcccctctactcaattcccataacactattatttgtggcattcatcacacagtatctgtagctttatgtatgttttctctcctagtagattctaagcaacttgagagtaggaatggtgcctccatctttatttctgtctccatcttaatatcctatacctagaagataccaggaagtgtcagctgaataaatgaatctgaaccttaatctcaaaggctatgcggcagtaagaaatggaatggacaaaaggaaacgtgaatttgatatgacttaaagttttagattaaggaaaacttccctacctgattatatctgtttaaaagaagagcaaaagtgtttttaacagatggaatcttgctgtgttgcccaggctggagtactacagtggctatttataggtgcaatcccactactgatcagcacaggaattttgacctgctccatttccgacctgggccagttcaccccttcttaggcaaccttgttgttctccactcccaggaggtcaccatactgatgccaaatttagtgaggacatctgacctgcatagcacactacagtgcagaactcctgggctcaagcaatcctcctgcctcagcctcccaagaagctacaggcagtacaggcaagtgccattgcacccagctaaaagaaaagcaaattttaaatacataccctgctgggaaactaaagtactaagtgaacaacacttacgtgcttggattagtataattcacagctatactattaagaaatctctgctgtgtaaattggaatgcgaattccttttttttttttgagatggagtctctctgttgcccaggctggaatgcagtggcgcgatctccgctcactgcaacctccgcctcccaggtgcaagcgattctcctgcctcagcctcccgagtagctgggattacaggcacccacccaccatgcccagctaatttttgtatttttagtagagacggggtttcaccatgttggccgagctggtctcgaactcatgacctcaggtgatccacctgccccagcctcccaaagtgctgggattataggcgtgagctaccacgcccggcctataatgggaatttctaaaatgttgatatttaattccacaatatgaaccaaggaaaattttactagcagaaatttatgtatgtaataaatcattagcctcatatgcacattatttgaaatatgcatgattggtcattttagttttcccaataataatttatcacttatcttatatcccactagtcacacactagcaggcaaatggtagcaagtctcaaatatgtaagaaaggtttaaagaagaaaaagtaaaaaaaccgtccagaattctatccattgtgtatttttctgtgactggagttgacataattagtcaatcttagcaataatgtattgggttcactgggtgttctgaggatgcaccatttgaaccaccggtaaaagggtacagaatgtgtattgagagtcacttcaatggcttctcaatgacaccacaccaaaggaggaatacctgaagagagaatggaaacactgcaggcaggatgatttaagaacctggaaataaggaatttaatcttgttcagcttgaggagtataactaaaattactatcctgagtaacctgtactaaatccatcactctggtagaatcagatcagctgagtttaaatgtcaagaaaaaatagacacacacaaaagtggctttgattacataagtcagaggagggggagcctacaatagctcttccccacatcacacccccaaggctccttcttagggacagcaacagctttgtcaatgacacaaatgcagggtggcatgaggtttccagcagcttaacattttaatttggggtgggggtggaagaaaatacataagttgctttttgctcccccatcctaatgccttggggaccagccaggctgacccaaatggaatccagagcgagagtggggccttgggttccccgaggagtaaagggggcagatccagaacagagcagaaacggtgataattatatagaggtcatgtcattgagggcgtggtccagctcctcgctaatggccttgtacttcagtttctgggcatagagctcatcttccaggtcatcaattgtcttttccagcttggctaccgatctctcagcaaactcagcacgggtctctgcctccttgagtttatcagtaagaatcttgatttcttcctcatatttatcttctttttgagagtacttttcttcagcagcactcagacacttcaggttctggtccatcagtctaatctgctcatccatctctcggcaacgggactctgccagctcagctcgttcctctgtgcgttccaagtctccttcaatgatcaccaacttacgagccacctcttcatacttcctatctgcctcttctgcaatgtgcttagcttctttgagttggatttcctggagttccatcttttcttcatcttttaaggcccggttttcaataaccttcatacctctctcactctcatcagcagctttttcagcttcttccagcttttgcagggcagtggccaggcgctcctgagcacggtccagctcttcttcaaccagctggatcctacggttcaaggaggccacctcagcctcagcatcagcagccttcttctctgccagttccagcttctcctgggcatccttcaaagcttcagaatacttgtccagctcatcctctgtccctttcagcttcttctgcatggctgccagctcatcctccagctgtttacttctttcttctgcctgcttctgctcagcttcagcttgctctgcccgatccagagcattctccttgtctaacttcagcatctgcatctttttcttgatggcctccatcatgagcagtggctgttggtaggctcacctgtgaacactggagaactggagactggggcaagaaagaaggggctgctgcctgagt

SEQ ID NO: 15117 - RNA, 4358 nt, Homo sapiens
  source 1..4358: mol_type = other RNA
gctgggattacaggcatgagccactgcacccggctaattctcctactctaaaaaccagtcatccttgtctttcctcctcacatcaagtggccaggcctttcacaatgcctgtctttatttagtgctatctctcctgccactactctagctcagaccctgattattctctcctagaaaactaaattaacctaacccaattttttccaaagtgtggtgtattcactgctatagttactttaatgtgattaggaaaaaacactaacacatcaaaactttgatttcaaaatagaattgtgtcaagtaagaacaaaataaatctggaaatgagtagatctgaagaaaacaatgtaggcagcaatgaatatggaaaaagccatcaaaaatggtaacataaatggctgaaatgtgagaaacaccatgttagtgaatcactttgctaatctgcaaattagttaccaaattaattcttcttatatgttattcagatcacaacatatcctattcaaaatctccagtggcatccccattaactccaagtaaaattataactcctcagcctcattttaagacacaacctgttccctactctgtctaaatctacctttagagctattgtggccttctcatctctatcaatgcctttattattttgtttctctttaaatggaatgctcaggccaggtgcagtggctcacgcctgtaatcccaacactttgggaggcagaggcgggtggatcacttgaggtcaggagttcgcgaccagcctggccaacatgctgaaaccccgtccgtactaaaaatacaaaaatcagctgggcatggtggtgggtatctgtaatcacagctcctcgggaagctgagacaggagaatcgcttgaactcaagaagcagaggttgcagtgagccatgatctcaccactgcactccatccagcctgggtgacagagcgagactccatctcaaaaagagaaaaataaataaataatggaatgctcaatattcactatcccacaacccaactctgcttgtcaaaaatccacttttggaacccaataaaaatgaatatgcaagtttaacatgttggctgggcgcagtggctcaagcctgtaatcccatcactttgggaggctgaggtgggtggatcacttgaggtcaggagttccagaccagcctggccaacatggtgaaacctcacctctactaataatacaaaaattagctgggtgtggtggcaggcgcctgtgatctcagctactcgggaggctgaggtgggagaactgcttgaacccaggaggcagaggttgcagtgagctgagatcaggccactgaactccagcctaggtgacaagagtcaaactccgtctcaaaaaaaaaaaaaaaaagaaaaaaagaaaaaagttttaacatgtttatgaagtacccattacatgccttcttccatgagtttttccaattcattcccactaggatcaatctcgtcccctctactcaattcccataacactattatttgtggcattcatcacacagtatctgtagctttatgtatgttttctctcctagtagattctaagcaacttgagagtaggaatggtgcctccatctttatttctgtctccatcttaatatcctatacctagaagataccaggaagtgtcagctgaataaatgaatctgaaccttaatctcaaaggctatgcggcagtaagaaatggaatggacaaaaggaaacgtgaatttgatatgacttaaagttttagattaaggaaaacttccctacctgattatatctgtttaaaagaagagcaaaagtgtttttaacagatggaatcttgctgtgttgcccaggctggagtactacagtggctatttataggtgcaatcccactactgatcagcacaggaattttgacctgctccatttccgacctgggccagttcaccccttcttaggcaaccttgttgttctccactcccaggaggtcaccatactgatgccaaatttagtgaggacatctgacctgcatagcacactacagtgcagaactcctgggctcaagcaatcctcctgcctcagcctcccaagaagctacaggcagtacaggcaagtgccattgcacccagctaaaagaaaagcaaattttaaatacataccctgctgggaaactaaagtactaagtgaacaacacttacgtgcttggattagtataattcacagctatactattaagaaatctctgctgtgtaaattggaatgcgaattccttttttttttttgagatggagtctctctgttgcccaggctggaatgcagtggcgcgatctccgctcactgcaacctccgcctcccaggtgcaagcgattctcctgcctcagcctcccgagtagctgggattacaggcacccacccaccatgcccagctaatttttgtatttttagtagagacggggtttcaccatgttggccgagctggtctcgaactcatgacctcaggtgatccacctgccccagcctcccaaagtgctgggattataggcgtgagctaccacgcccggcctataatgggaatttctaaaatgttgatatttaattccacaatatgaaccaaggaaaattttactagcagaaatttatgtatgtaataaatcattagcctcatatgcacattatttgaaatatgcatgattggtcattttagttttcccaataataatttatcacttatcttatatcccactagtcacacactagcaggcaaatggtagcaagtctcaaatatgtaagaaaggtttaaagaagaaaaagtaaaaaaaccgtccagaattctatccattgtgtatttttctgtgactggagttgacataattagtcaatcttagcaataatgtattgggttcactgggtgttctgaggatgcaccatttgaaccaccggtaaaagggtacagaatgtgtattgagagtcacttcaatggcttctcaatgacaccacaccaaaggaggaatacctgaagagagaatggaaacactgcaggcaggatgatttaagaacctggaaataaggaatttaatcttgttcagcttgaggagtataactaaaattactatcctgagtaacctgtactaaatccatcactctggtagaatcagatcagctgagtttaaatgtcaagaaaaaatagacacacacaaaagtggctttgattacataagtcagaggagggggagcctacaatagctcttccccacatcacacccccaaggctccttcttagggacagcaacagctttgtcaatgacacaaatgcagggtggcatgaggtttccagcagcttaacattttaatttggggtgggggtggaagaaaatacataagttgctttttgctcccccatcctaatgccttggggaccagccaggctgacccaaatggaatccagagcgagagtggggccttgggttccccgaggagtaaagggggcagatccagaacagagcagaaacggtgataattatatagaggtcatgtcattgagggcgtggtccagctcctcgctaatggccttgtacttcagtttctgggcatagagctcatcttccaggtcatcaattgtcttttccagcttggctaccgatctctcagcaaactcagcacgggtctctgcctccttgagtttatcagtaagaatcttgatttcttcctcatatttatcttctttttgagagtacttttcttcagcagcactcagacacttcaggttctggtccatcagtctaatctgctcatccatctctcggcaacgggactctgccagctcagctcgttcctctgtgcgttccaagtctccttcaatgatcaccaacttacgagccacctcttcatacttcctatctgcctcttctgcaatgtgcttagcttctttgagttggatttcctggagttccatcttttcttcatcttttaaggcccggttttcaataaccttcatacctctctcactctcatcagcagctttttcagcttcttccagcttttgcagggcagtggccaggcgctcctgagcacggtccagctcttcttcaaccagctggatcctacggttcaaggaggccacctcagcctcagcctgttcccgggcccgcctttctccctcaacttctcgctggaggcgctcagctcgctcctctgcatcatctgcctgctgctgcagaacctggatcttgcgcttcaccgcctcgatggtggtgatcccagccatggtgcccacccagctactgctcgcgctccggttcctgcctcctccgctcggcgttgcagcctcctctcacccttacttccgcctgctacgccctgaaat

SEQ ID NO: 15118 - RNA, 3462 nt, Homo sapiens
  source 1..3462: mol_type = other RNA
gctgggattacaggcatgagccactgcacccggctgggatctttcagttagagctctacatgaaataaactgaggggcagaggaaataatgagagaagactgggctcttttcaacatctagccgaagacactaaagcagctctgaaatgccagcatttgcactgtttaaaaaacccaaagattgggaacttattttcttaaaaggaaagaagagtaacacggtcaaaaaggagtgttttccgcatcgggagggctttgtactggaaagaaacggaggaactgccacgtttggcacccagaaggatgcctttttttttttttctgtgtgaatcctccccactcccacctcagcccaccccgcaacagtcaagctttgggtccaaaccaatctggcatctctaaaatggaagcactgtttggagacaaagtggccaggcactgccggccagagaaaagacaatgccccacacccacggcctgcccgcactgaaatgcctattcatctccatttttatcgacatctcttggcttccaggccctgtttgtgctttgtccttggtccttattgacctattggattcggaggggaagctcagccgcaggcaaatgggtattttaatccacaatggaaaacatgggttcctctagcgccactggcagctcccagcatcttgaccctgaccttttcagcagcgtgtggccacacactctacccaggccaaagaacgaaagggccccagggcacacactggggccaagaaaaggaatcgaatggtggaatgttgctgacttttccttctggatctgcctttgagactcttgcatgggaaaaaagggtgaagaaggggcagaagcaaagcttagtctttgtctgattcagtctttgcactccccctgccccctcctctggcaggccatggaggccacacctggcacacctgggcatgttccagatgcttataaaggtccagggaagcagggctgctcagtcattgtgaggatctgggaaattctcagtcctcatgggttctgtgagcagccaaggtgatcagccctgacaggatggtcaggatggcagtgaagaggcttgattgattgacaggtgagcagacgatgggactctcggcagccctaatcagcgagagagttgcttctgagcacagctcagctaatgtcccacgctgttccggagcctcaaggaagaatgggctgacggtggtcccaggcctcctagaccaagtgcagctggcgcagacctctggcgtggttgactcggaacccgttctgggaacgtgaacttggattcaccttagcaataagtgctcaggaatgtgttggaattgctgccagctcctgggacaggcagaccccagaacactggaagagatctgaagccctggcacccctaccagccccatgggctccacattcaatcaagcaggtcatcggttatctctaccttcacatggcctggaagcccagcaggcagggtttgctctgtgatatgacaatgctgctgagtctcctgtcactcaccgcagcacctctgcgtagtaaacggcgtctttcctgggtctatgacagttaccatagctcttccaggaccacagaagtacctaccttgttctggttttgtgatcaacactgatacataaatgtaaagaaggcaaccggtgcttgaggggacatctagtgtattgggaggtgaggagcaggccaactagttcagaggctctgacttggttggagaggggtaaacccaggtgttacgagggtgcttggttggggggaatctggtgtaggctagaggggccagtgcaggtttcctgggggtgctgagacctggggcatgaagaagagttacttatgtgaggaggagagaggagctccaggccagaaagtccacatccactacaccagaagctccacccgttccggaaccacactccctggactggctctggaatgtacacccatgtttagcacagcgcctcctagtgttcccaagtccccactcgctacttggctgttgaacaaataagctcaaaggtctggaggtgagtgcctgaacgttttagctgggctggagtggacctgaggaatgtgtcccctggggtgtggggcaggaacagggagcagaagccagaggtgaggctggggaaggacagtggctgggaagttgcttttgggcacttgcactttctcctgagggccagcggtcggagtgggggaagactggagacctgcttctccatcctttccctgccctcactttcttcattttcttaggagccaacagacctgtgcaaacctcagctttccccagttcagctccttttccatcttcttgatttctgtatttttaaaaaaacaaggctgcattatattgtaggagaacaataacccactggaccacatcctggtaaggaagagctgcaaagccatggcctcatcactgtagacataagcttccaacagtgccccattgtggcatttgatttaactcagcccttcaaaaacatgcatttctgacttaaattctgcacaccatcaccatatccccagcagatgtcgctaacgtctcacattttggtcatgccagcagcacgcatctcaggcaacaaatatttattaagcagcgaatgtgcattgtgcaccaggctgagcactttgtagataaaaattcctggggcatgacccaggacatgaagaaaagttacttaagtgaggaggagagaagagatccagatcattttttgatgacaaaagaaggtaacataaaaaaataatggactgtctgaaaagttctttcccattgaggtacaagtttgtttctggctatgcaatgtgaaattggaactgaatgtctgggaccacctcgaagcttgtttcaaaggcctattactacgtgtcttttagacagattttatttcagcttgcctaattgaagcctctggaatctctaatgacagaagtgtaattcatatttctacatttcttctggaaaggaaggcccgaatgagaaggcagcactaaacaaaccgtgaagtcaaagttgaagtatggttgctaggggaagagtgtcgagagccccatgaggtggttgccctctgagatggcttgttgcccaagtgggtggtgtctatttggttggacttgaagaggttctgtgcatcgaagttgctccacatggctgtgctgacaatgcttggagcttggacctggaggtttgaagcatcattattgagcaagtattcatccagcacaacaccccagctcatagaatggctttgactggtgaaatcccagatgtggatgatgtagaaagtcccctgttctgtttatggcctttttccttggatcaaaggtccatgaagaagaggtctttgccaggcgcagtggctcacgcttgtaatcccagcacttcgggaggccgaggtgggcagatcacgaggtcaggag

SEQ ID NO: 15119 - RNA, 2230 nt, Homo sapiens
  source 1..2230: mol_type = other RNA
gctgggattacaggcatgagccactgcacccgtccctcattaattcatcttaaccagaagagaaatattcagtctcacaaaaaaagaaaagaaaaccagatgttgtgtttttctttcattaactctacagcgactttatccttctaggtgattctatatgaacacaccagataagattaaagcccaccccaccacatcaggggaacagaaaagtttccagcaagaaggaaagaaacctgctgctctttgctgaacaaatgtgctgcagctgcttctcccaagtgcatggtgtagacaaatcgtaagcaagacagaaggggctgccagagatgaataaaatttcggttacctcttccattcggaaggaacggaaaatgtacacgtagtcgcccgggcgtccaacaaaccggcctttgaagaacgccacgtaaaagatgggggtgtaggaattcacaaacttcagcaggaaagccttgaagatcagcctctcctcaaagcttttctccgtctttgggacctcgatcttggtgagccatcgggctatgcagccatacacctcgtccaggaggatgatgaccactaggttgatgatgactgcggtggctgtgactgtgacccggatgttggaccgcacggagggggaggagttcatggccaaggcggcggccatggagattctgtagatgatgacgccgaggacgatggcaaacgtcactgcaatcatgaagatgatggagaccaagttagtgaggtaggctgggaaccgatctctccatgtcagcttcactttgtcagtctctttgtttctggactctttcttcagagacttctccaagactctggcttcgtattcagctctaggatgatcctcttcctcttcaaagcccgtgaggtcccagcggtagttgagtcgcatctgtttccgcttccagtgctccatgaaggtggcagcccagagggccatgaagacagagaagaagaccgtggcggggttgtcgaagaggtggctggcgcgggccgtggcgcaggctgagctcatcttccagtagctgcaggtcttgtcgcaaagcgggcacatggtgatattgtgtctctggtcacacatctccatgctggggatgttttcatccatggtggcgcatccgtacaggaagacaatgattcccacgatggaggcagggatgagcatctgggtgtacacgcccagccaggcgaagtacaggccgatcttctccccaaaatacttcctgaccaggtcgatgggctggtacttatagaaaactccatagcgtgcccactcttcgtacaggagttttctgtcgttgaactcgacgttttcaccgttgtagtctccatcgtgcagtgggtatgcagccgcgtacacaccattggccagcaggctcgtgatgcccatgctgtacttggcctttgtacacgtcgttctcttcaagatctcatagacaatcgtgctccgggttttgctgtcgaaaaaggaatccttatcagacaagtcaaatagatgctgcttctcccgggagaagggataggagagtctcttcatggtctggggcctgtgctcagccactttgggctggatgggatctgtgattttctggagcacagagttgatttttttcaggaggccacgggtctcattaatgtggtacatcttcttcgtcggcatcttcagtttcagaaactcggcctctctgcacagcacgttccagggggcatggattttcacaaacccgactccgtggattttagtgtcctcgtcccgctccagctccaggcccgcctccaggaggttgccctcgtactcctccctgcggaagcgcttgtcatcctcgtggtagtccatcgggggctcccccgagcctgcatccagcgacgcccccttgcccggcagggggtggtcctgcttgacgctgcgagccccagagggggtgtcgctgtgctgcaccctcctgaccagggtccggttgcccgagggcctcttgtgatggtacaccaggatgtagtccaccttgcgccggccgtccctgaagtacaggccatacttgcactcggcatcagggtccacagataaggagttcagcagcacctgggagggcctggtcagcatctggtgccggcaggaggctgaaactaagcaactgacttctctctacagtaacacagggccccgctgtgctggtgaccttcaggaggacctggactcagtgtgcgt

SEQ ID NO: 15120 - RNA, 9846 nt, Homo sapiens
  source 1..9846: mol_type = other RNA
gctgggattacaggcatgagccactgcaccctgcctaattgagacaatatttatacaaggggaaattggtctattataaggcctagccatagtaaaggtctcaacatgtgctcccagctctccctctcctccttgtcttctctctaccagtggttctcacacttcgtaacactctgaggcacactgggcatgaaataaaagcaggagaggatgggacagcatattccagagatctgtttttcttcttaaaagccactcacttgaaattctatcaaagttatatgcctaaaaaattcattacctctgttttaattatacaagagccttacaactaaaatactctcccagtcatctaagagaccaccacttaacagtatattagatgcaaacatttcagattttccccatgagcctgaagtttaaacattcaaatttgcaaaagagaagtaaattggaagaaagacattcacagaaaactatttcatatccattagttatcatttacacatcaaatacatatagcattaagaccaaatatacagaatttccacatttatatacagtagtcaacatagtgcacaattcaaatctatcttacaatcaagtgtacaagtttaaatatggctttataaactactaataactctgctaaagtaactcatagatccagaaataaacactgaaatgccatcttcacattggggtcatcattcagcaagatgctaatcattgtgattgcaaaacagagggtgcaggtaagtgtttccaggtggtgtccgcccattagccccgaaatgtgggttcaaattatgccaacattggcccttcctatctcagatacctaaaaataagtctgcacatcttccacacatttgaagacacaagattataaacaaatagaaaaaaagacatgtaatcagtgagatgatgaattatcaggcattatcaaaacatgtttttcagattgatgctgaaattcacagacaatacatcctgcatttgcattatctgggtatcacctcacccctactttcttttcttgttttgcttacctcagtgtgttgttaaatctttctggaattttcaaggcattctagatcaagtggtcccaaaagcagaattaaaaacatcagtcttaaaggtgacatcaaattgttcatccttctctttcccaaccaaaaatgcctattttaagtaaaaataattaaataccttgacctaaaatcatgcgtccatgcctgttttatatctgctttgccacaaatggtatatacacattctctaatcaattacaggcatctgggtgctacgcctaaagactccttgtcccattctctaaactccattgaggaccagaaaatatacttttaaaatgtctatgtttgctatggtttttaatgtttacatcagtaaaacagtatatacatatatagcagtgtatacatatatacatatatatcataaataaatacatggaggggcatgctcagaaagttttactaatagggtgaataaacataaacgtttggagaccactgcctaaatagggatggacgatctgggctgtctgcaaacatttaaaagacttctctaaaacaaaatgtacattactttgtacaattttatatttataaaatgaaaaatatatgccacaaacactcttgagagactagaaggaaattccaaaattaaaggagtaaatgtatcagggccagaccctctaagctgctatctaaggtcccaggcctggcttcagaaggggaatgggggacatgagcatagaaattaagataaagataaatgttacttcacttcctgcactggccacttgtatatccatagacaatccttccctacatagattgcacttgtttttgatttataaacctgtactttttattattttagcaagatggcaccacctagaaaactttcaattgcctgatacatctctaccacagccataccacatggttgcttgaaattttgacatttgttactgttttcttctctcctcctactcagttaaattctaataccaccaaatgagggactcagaccctcagttttccaaacttcaccatggaaaaaccatcgctgtcatcaacatttgagttgtcagacatttggcatgatgtagatcactgggaaaaaaacatgtgtttacaataagcttgttctgatcccacaagacttattacttgcaataaaatcattttgacaggagtaacattaaaatcattttacaggagtaaacatgtcacccctactgaagcagaagcctttagccttatttctgtaaaaaacaaatcccaggcataatttgttaaagataaaaatacaatcatttggacatggtttatattttaataagccaaatataatctcttgtagaagagaagcaaatacgaaagaacatttctgattctgaacaatggaagaggaaagtcattgattattttttaaagaggaggaagacagtaaatattcagagcattcctcttttttagccctcaatgaacaattatattatattccctttgctatctgtttagccaccattaactaacatggcaattcagaagttggatcttatttttttagaagccatggggtaactaaaaacaaaaaaggtattaaataaggaaaaaagcttaagcattactaataagtgaaagttactctattccagagccacaaataaaaacaaataaataaaaataaatgcatgccaatggggggtgggaggtgaattagtcacatttagtagcacaactttttataaagttaactgattatgatacacatatattgctttatggttagtggattgtttcaaaaatgcatgatggccattaaattctttgctaaaattattgtgtacagaacaccaaagtaccgtatccatcttttactccagattacttgttttcctactgaaatggtcagtttggtgctgctagaccatatctgtaggttattcgttttattattgcaatggtcccctttatttgtctaccaattttacaatttaaggcaatcatccttatgaaatttgagcatcctagtttgtcatggtccagccaatagcaggagttttagagggtctaggtctggggacaagttccttgcttcggcgaaagcagaatggttgaggaggtcaccctgtcagctccaaaacagctgaaccccttttttttaaatctatgcttcagtgccctctgtaatcatctctaactggcaaggctaacgttgctggttccagcagtctcatctcaaagattaaggaaacttaaatatccttaagatattcttgaaagtcagggaccaaaaatctgagtttctgggtaaggaattcagatgaggaaaacatgccacagatgttcgcatccacgcctgacagtagcaagagtcttacaggtaagaggcccgtccctcctcacccaacaagggaatccttttgaacttcccaagttatatccagaccactggaagcaactgaataaaggtcaagcacttcacaatcacatgcaattgatccctggacctgttaaagatgggttcccagagcccagcatttagcctgggaagtattcgtcattgagtgtacttttatcagttctagtttgacttaaatagcactgcatataaaggagaacaaaggatcctgggtcatagtcaggaacaataaaataacatactctgtttaaaaaaaaaaaaaaccctaaaagaaagaaagaagaataacctgagttgttccctatcaacaaaagccaccaaccttttattgaaaatacactcaacaattgttctatgaatgaatgaataaatgaatacaggaaaacctgattgtgcagacctttcttctttaaggaagaaaaatccagcctcttctctcccaccttcagcccaggctggttgccctatccatgcagaagcggtgggtttcagggctgaaaggaagcgcacttggccctgaactcattttgataaatcaattttgggggtggttaaaagataaatgacaaggacaacaacaaaatcctatgactttcaaaattccaaacctctaaaacaaaattttctcaaataacctaagagcacttctttcttcttttctgtcactcaagacatactgaacatggataatagagattacttttgcttgcatagcctgtactaatttttcttctctctggctgtgttaaaaacaagaacaaacacaatgataacatttaaagactcttgggaacaagactctttaactggggtccattaaccccctgaggaaaccatggataatttcaggaggtctctaaatttcctgaatttatatgtaacattttatgtatttgcatatatgtgtttttctgggaatagggtatagaactttcgttggattatcagtggagttcctgacaaacaaaaagtgaaaattcactatttaatggtatgtgactcactctctgagcatctttcccatgcaaccttcagggaaggaagtgatgagtgcttcattttcaaaggaagagattataatcagctgggaagccttcatgtgaagctgacgaagtcagaccttgagagatgggcatgacttgggccagtggagcagagaatagaacatttcaggagaaggactggcatgagcagaggcacagaggtgggccacatgaggcttttttaggcaatggcaaatggatcaacctggctgcactggatggctcccatggaggagctatggagacaaggtgaacaaaggtgaaaacaccagaccctaaggagtagcccctcaccctgaggcaatgccacaccccatcagggccaaagagctttttagaaagattaatccatttgtagtggatggaatggaacagggaaatggccaagtacgtaaaagaggctagagaagtctaggcaaaagaggatgccctgaaatcagagttctatgctgttctatttgccactctacaaccagtgtagatcccagggccaggcacagggtaggtgctctgtaaatattcagcaagtgagggaatggacatgggttctttaaaagatacataaggaagtatgaggagtcttggtgatttgggaatccatcttgctattcttcagagtctagcaataccctgcactgatgagaggtctcttgtattggtcttgaccaggctgacaggacatggacaaaagcgaagtaggattccaaccagggaatggctggagatgtgctggttgtctgaacacagggtgacttctcaggtaacatgcattttataagacaacaaagccacagtggtataatggaaagaaccatcaagggcaaggtggtataatagaaagaaaccatcaagggcaacgtggtgtaatggaaagaaccatattgacctcagtttttggtcctgcccttcaaataagtatgtatgtgacactgagccaataaggtgctttctacagctaatttttagcacagctatacatttctatgactctacattatctctcaaacaaatctaagcaagacccacaaggccaaaatccttagtatgtctgttccttgaaccttagctatttcacaaaaatataccctaacaccacagtatacatgggcagggctcacttgaggagtagactgcagtctgattcaagtccaagttgttccaggtccgtgattagtctcctgggtagcccacagccttggtagtgtcactttctacaattcattatgtaacaacaacaaattggtaaatgctgacaatatagttcatcattgcataaatatagattgtccttatatctgttctgatggagagtaaagctcaatgattctgctcattaatcttgttgagtgggggtacagatgggcaaagagaggtggatgcaagagcttgatttacttttacaatgacaggaaaaaaagaacgaatagcctatgggtctgttgtccaaccaaaagcatctgttaacattaaagatcacatacttcaagttaccttccagcaaaaaggaaacacagaacttgaacaagaagccagatgaccaaaatgtcccttaacttcttatagttttttcctataattagcacctgttcatgaaattggagaacatttcaaatctgggtagcttaagaatgaagcacataaaattaaatccttccggataaagactcacactatggtgactttgtcttggttattttgtttgcataacccgccttgggaaagtaaagcaggggcatattctagggctctaaatcaaattaacacctacaaaatgttgatgcccagttatatgctgtcaggcaattgcccaagactccagatagcaatgtccattcatgcccctgtaagaggtacctggatggaatgacttattttacaacttcattttcaaagttggttctccacatacttgtattccaagtaatataaaattaaaaacatatattaatctacattctcataacttaatcatcctttgagagaaaatacatcacacttggtactgtacagtaagatagattgttcatagaaaaaaattcaaatacatttcttttctactaaaatgtggtgggaaaaggacaacccatgctttgtggagacaggtctgcagtccacctgttcattatattcatattttcagtccaggagtctccctagtcacacagaaatgccaccagttggccttaaaacacacttgctagagagaggggaggcaaacagtcctcccaaatgatgctgcagcctcaaacaggcttatccattcatatcttctccaccacattcttattaggcatcaaacagtccctttaaataagaatggttttaataagatattaacaactaagtttcccatggaataagaatttctaacttagggtatctcagcacgtattcccagttacatatgccctacacaattgcttaagtggtaagcagtctgaaaaactctcctccctttacctctttgtgaatctacagcagtcttttaagattgttttgcaaatgctatattcaaaaagaggttttttttttttcaagtaaagtgcatggatttctcagaagttgctgtattttaagaagtgcctctttaaccccataatgagcaatccttatgttggtcagaagcaaagcagttttgtttgcaattgtaaatcttggctctcctagcccaaatctcacagccatcacccaggatctctgccccatatttccctggaaaatgtcctaagtcaaaacaacaacaacaacaacaacttcatctttagaaatagggtgccttcacaaatatgggtaagccaacagttcatcgaatactatagggaaagagagagagaacggggatgagacagcaaaaacattaagacttgttctcagcattgctctcctctcactgggcagtggctgaaaacaccagaaaagttgcattaataaaactgcatatagtctaacactgcacagagtgctttgatacaagtatcctcttgctacttcatcttttcaatacatctttgcaaggtttgttttcaaaaagacattacaagttggcaggcttctgcttataaaaatcaatgaaatactttcccttcaactctatgaaacctgccatatacctgagatttattcttctcaaataaatcaaacataggcaacgtaacactctggagtcaacacagaacatgccagggtgagttcaggcaatgaaagaaccacttttctgcaaatacatggtagaattgaagactgtttgtagctgtcgataatttgtaaaaacatttccaatgttctttgaacaaaagattttgattcagccaagattacagaaaggaatcatgacaaagtcctaagtgtacctttgtgtgtatttcatctgctcagcttttgcaggtgactgtggtggtggttgcctggatatggaattcctttgccctcaaatcttcacatgcatgaagtgcaataaagaataaaatgctgtgtttatgtcgcaccacttctaagaggtttaaagcgccgtacgaatgttaccacatgaatccccacaacacccctgtgaggtaggtaggtggagagtattgtcatccccactttacaggtgggagaaatgaggcacccaatagttaataagagatttgctcaaaatcacacagctagtcactggcagggcttagaataaaatgtatactgattagcacctagcacagtgctttgcacatagtaggtgttcgtttaatatctgtggattttatttgacttatgtctcaacatacaatatacacacataaagtacaagcagccaccgtaaaacatttttctgatgatatctctcattacttcaaatcctggtggaggaaggaggttcaagaatccatctcacaattaagacctcagggttgaagaggatcatcataaaaactatcagctgacaaccagctcttacacctgctctaccacacaatattattaatagttttctaatgaaaacaaaaatggatttcaggaaccatgctgacattattttttgcctgtttgttttcaatggagtcatctgaatggttctgtgttttgtttgtacaaaaaagaaataaggctgctatagtccagttagcatgtgaaaactctgccaagcacgaagatctcctcccagctcggatggattgctacctgggaaaatggaccgacccagggagtggcaggtcccaaggaagagggtcagtgaggctggacgtcacttgcactgttcgtggtctgtatagtcatccatgtccacatccgaatcaaagagtgagtgtccagtaaaatctgtgtctggggttctggaaaaactgttttctgctccctcatcttcaaaggtctctgtccttgagtaaaagctaaaatccagcagcggggtgtgggttttgctgccttcgctgctctcctcagactcatagatggtattgtcatcatcgtggtgccactctggccaaaatttcctccttatcctctcacagtacatggcaaggttgatcagctcacctttgatcagccgttcgggtcttgtccctggtaaggtccacattgcctgtgccaagtgtccaaagacagtggcgtcaagagtggaaagcttgggccccatgatgtacttcttatcaccagtagaagtgctcctccaccatcttggtcaccgctctggagatggctctttcatgagggccaaggtttttgtttaaattcactccaagcttctcttccagaaagtcaattatgaattctgtgccagaaactttttcatgattatattcaatccaaggcattttcccttgagcagagagttttccaccaaaatagttctgatacggtaagtcagccatccttaaataagtttccatctttaaacagaaaggagataaacttggaacaccattgttaggtcttgcaaactgatgcaaaataatagcatctttagagtcaatctcttgctgtttcctaatgaccaggagttcgtggagcagatacgcagctgcggccagcaaagctcccccggtcaagtaaagggttttcttccaccagggatcggagcccagccctgccatgatcccaccgtaatccccgcgccctgccccctccccgcatctccgcggtccggccgcctccgccggggccggatctgcagggctgaggcgcgccgggcaggctccgcgcctccgggcggcacgcccaaaaaccgctcgccgcgcgcgggcaagggcggcggaggtgcctggaaatgcggccccaccgcgaggaagctgcagtcggggcccggatcccggtcctcccctaccccggccggccctccgcctgcgctccagcccctcccgcgggcccc

SEQ ID NO: 15121 - RNA, 9627 nt, Homo sapiens
  source 1..9627: mol_type = other RNA
gctgggattacaggcatgagccactgcaccctgcctaattgagacaatatttatacaaggggaaattggtctattataaggcctagccatagtaaaggtctcaacatgtgctcccagctctccctctcctccttgtcttctctctaccagtggttctcacacttcgtaacactctgaggcacactgggcatgaaataaaagcaggagaggatgggacagcatattccagagatctgtttttcttcttaaaagccactcacttgaaattctatcaaagttatatgcctaaaaaattcattacctctgttttaattatacaagagccttacaactaaaatactctcccagtcatctaagagaccaccacttaacagtatattagatgcaaacatttcagattttccccatgagcctgaagtttaaacattcaaatttgcaaaagagaagtaaattggaagaaagacattcacagaaaactatttcatatccattagttatcatttacacatcaaatacatatagcattaagaccaaatatacagaatttccacatttatatacagtagtcaacatagtgcacaattcaaatctatcttacaatcaagtgtacaagtttaaatatggctttataaactactaataactctgctaaagtaactcatagatccagaaataaacactgaaatgccatcttcacattggggtcatcattcagcaagatgctaatcattgtgattgcaaaacagagggtgcaggtaagtgtttccaggtggtgtccgcccattagccccgaaatgtgggttcaaattatgccaacattggcccttcctatctcagatacctaaaaataagtctgcacatcttccacacatttgaagacacaagattataaacaaatagaaaaaaagacatgtaatcagtgagatgatgaattatcaggcattatcaaaacatgtttttcagattgatgctgaaattcacagacaatacatcctgcatttgcattatctgggtatcacctcacccctactttcttttcttgttttgcttacctcagtgtgttgttaaatctttctggaattttcaaggcattctagatcaagtggtcccaaaagcagaattaaaaacatcagtcttaaaggtgacatcaaattgttcatccttctctttcccaaccaaaaatgcctattttaagtaaaaataattaaataccttgacctaaaatcatgcgtccatgcctgttttatatctgctttgccacaaatggtatatacacattctctaatcaattacaggcatctgggtgctacgcctaaagactccttgtcccattctctaaactccattgaggaccagaaaatatacttttaaaatgtctatgtttgctatggtttttaatgtttacatcagtaaaacagtatatacatatatagcagtgtatacatatatacatatatatcataaataaatacatggaggggcatgctcagaaagttttactaatagggtgaataaacataaacgtttggagaccactgcctaaatagggatggacgatctgggctgtctgcaaacatttaaaagacttctctaaaacaaaatgtacattactttgtacaattttatatttataaaatgaaaaatatatgccacaaacactcttgagagactagaaggaaattccaaaattaaaggagtaaatgtatcagggccagaccctctaagctgctatctaaggtcccaggcctggcttcagaaggggaatgggggacatgagcatagaaattaagataaagataaatgttacttcacttcctgcactggccacttgtatatccatagacaatccttccctacatagattgcacttgtttttgatttataaacctgtactttttattattttagcaagatggcaccacctagaaaactttcaattgcctgatacatctctaccacagccataccacatggttgcttgaaattttgacatttgttactgttttcttctctcctcctactcagttaaattctaataccaccaaatgagggactcagaccctcagttttccaaacttcaccatggaaaaaccatcgctgtcatcaacatttgagttgtcagacatttggcatgatgtagatcactgggaaaaaaacatgtgtttacaataagcttgttctgatcccacaagacttattacttgcaataaaatcattttgacaggagtaacattaaaatcattttacaggagtaaacatgtcacccctactgaagcagaagcctttagccttatttctgtaaaaaacaaatcccaggcataatttgttaaagataaaaatacaatcatttggacatggtttatattttaataagccaaatataatctcttgtagaagagaagcaaatacgaaagaacatttctgattctgaacaatggaagaggaaagtcattgattattttttaaagaggaggaagacagtaaatattcagagcattcctcttttttagccctcaatgaacaattatattatattccctttgctatctgtttagccaccattaactaacatggcaattcagaagttggatcttatttttttagaagccatggggtaactaaaaacaaaaaaggtattaaataaggaaaaaagcttaagcattactaataagtgaaagttactctattccagagccacaaataaaaacaaataaataaaaataaatgcatgccaatggggggtgggaggtgaattagtcacatttagtagcacaactttttataaagttaactgattatgatacacatatattgctttatggttagtggattgtttcaaaaatgcatgatggccattaaattctttgctaaaattattgtgtacagaacaccaaagtaccgtatccatcttttactccagattacttgttttcctactgaaatggtcagtttggtgctgctagaccatatctgtaggttattcgttttattattgcaatggtcccctttatttgtctaccaattttacaatttaaggcaatcatccttatgaaatttgagcatcctagtttgtcatggtccagccaatagcaggagttttagagggtctaggtctggggacaagttccttgcttcggcgaaagcagaatggttgaggaggtcaccctgtcagctccaaaacagctgaaccccttttttttaaatctatgcttcagtgccctctgtaatcatctctaactggcaaggctaacgttgctggttccagcagtctcatctcaaagattaaggaaacttaaatatccttaagatattcttgaaagtcagggaccaaaaatctgagtttctgggtaaggaattcagatgaggaaaacatgccacagatgttcgcatccacgcctgacagtagcaagagtcttacaggtaagaggcccgtccctcctcacccaacaagggaatccttttgaacttcccaagttatatccagaccactggaagcaactgaataaaggtcaagcacttcacaatcacatgcaattgatccctggacctgttaaagatgggttcccagagcccagcatttagcctgggaagtattcgtcattgagtgtacttttatcagttctagtttgacttaaatagcactgcatataaaggagaacaaaggatcctgggtcatagtcaggaacaataaaataacatactctgtttaaaaaaaaaaaaaaccctaaaagaaagaaagaagaataacctgagttgttccctatcaacaaaagccaccaaccttttattgaaaatacactcaacaattgttctatgaatgaatgaataaatgaatacaggaaaacctgattgtgcagacctttcttctttaaggaagaaaaatccagcctcttctctcccaccttcagcccaggctggttgccctatccatgcagaagcggtgggtttcagggctgaaaggaagcgcacttggccctgaactcattttgataaatcaattttgggggtggttaaaagataaatgacaaggacaacaacaaaatcctatgactttcaaaattccaaacctctaaaacaaaattttctcaaataacctaagagcacttctttcttcttttctgtcactcaagacatactgaacatggataatagagattacttttgcttgcatagcctgtactaatttttcttctctctggctgtgttaaaaacaagaacaaacacaatgataacatttaaagactcttgggaacaagactctttaactggggtccattaaccccctgaggaaaccatggataatttcaggaggtctctaaatttcctgaatttatatgtaacattttatgtatttgcatatatgtgtttttctgggaatagggtatagaactttcgttggattatcagtggagttcctgacaaacaaaaagtgaaaattcactatttaatggtatgtgactcactctctgagcatctttcccatgcaaccttcagggaaggaagtgatgagtgcttcattttcaaaggaagagattataatcagctgggaagccttcatgtgaagctgacgaagtcagaccttgagagatgggcatgacttgggccagtggagcagagaatagaacatttcaggagaaggactggcatgagcagaggcacagaggtgggccacatgaggcttttttaggcaatggcaaatggatcaacctggctgcactggatggctcccatggaggagctatggagacaaggtgaacaaaggtgaaaacaccagaccctaaggagtagcccctcaccctgaggcaatgccacaccccatcagggccaaagagctttttagaaagattaatccatttgtagtggatggaatggaacagggaaatggccaagtacgtaaaagaggctagagaagtctaggcaaaagaggatgccctgaaatcagagttctatgctgttctatttgccactctacaaccagtgtagatcccagggccaggcacagggtaggtgctctgtaaatattcagcaagtgagggaatggacatgggttctttaaaagatacataaggaagtatgaggagtcttggtgatttgggaatccatcttgctattcttcagagtctagcaataccctgcactgatgagaggtctcttgtattggtcttgaccaggctgacaggacatggacaaaagcgaagtaggattccaaccagggaatggctggagatgtgctggttgtctgaacacagggtgacttctcaggtaacatgcattttataagacaacaaagccacagtggtataatggaaagaaccatcaagggcaaggtggtataatagaaagaaaccatcaagggcaacgtggtgtaatggaaagaaccatattgacctcagtttttggtcctgcccttcaaataagtatgtatgtgacactgagccaataaggtgctttctacagctaatttttagcacagctatacatttctatgactctacattatctctcaaacaaatctaagcaagacccacaaggccaaaatccttagtatgtctgttccttgaaccttagctatttcacaaaaatataccctaacaccacagtatacatgggcagggctcacttgaggagtagactgcagtctgattcaagtccaagttgttccaggtccgtgattagtctcctgggtagcccacagccttggtagtgtcactttctacaattcattatgtaacaacaacaaattggtaaatgctgacaatatagttcatcattgcataaatatagattgtccttatatctgttctgatggagagtaaagctcaatgattctgctcattaatcttgttgagtgggggtacagatgggcaaagagaggtggatgcaagagcttgatttacttttacaatgacaggaaaaaaagaacgaatagcctatgggtctgttgtccaaccaaaagcatctgttaacattaaagatcacatacttcaagttaccttccagcaaaaaggaaacacagaacttgaacaagaagccagatgaccaaaatgtcccttaacttcttatagttttttcctataattagcacctgttcatgaaattggagaacatttcaaatctgggtagcttaagaatgaagcacataaaattaaatccttccggataaagactcacactatggtgactttgtcttggttattttgtttgcataacccgccttgggaaagtaaagcaggggcatattctagggctctaaatcaaattaacacctacaaaatgttgatgcccagttatatgctgtcaggcaattgcccaagactccagatagcaatgtccattcatgcccctgtaagaggtacctggatggaatgacttattttacaacttcattttcaaagttggttctccacatacttgtattccaagtaatataaaattaaaaacatatattaatctacattctcataacttaatcatcctttgagagaaaatacatcacacttggtactgtacagtaagatagattgttcatagaaaaaaattcaaatacatttcttttctactaaaatgtggtgggaaaaggacaacccatgctttgtggagacaggtctgcagtccacctgttcattatattcatattttcagtccaggagtctccctagtcacacagaaatgccaccagttggccttaaaacacacttgctagagagaggggaggcaaacagtcctcccaaatgatgctgcagcctcaaacaggcttatccattcatatcttctccaccacattcttattaggcatcaaacagtccctttaaataagaatggttttaataagatattaacaactaagtttcccatggaataagaatttctaacttagggtatctcagcacgtattcccagttacatatgccctacacaattgcttaagtggtaagcagtctgaaaaactctcctccctttacctctttgtgaatctacagcagtcttttaagattgttttgcaaatgctatattcaaaaagaggttttttttttttcaagtaaagtgcatggatttctcagaagttgctgtattttaagaagtgcctctttaaccccataatgagcaatccttatgttggtcagaagcaaagcagttttgtttgcaattgtaaatcttggctctcctagcccaaatctcacagccatcacccaggatctctgccccatatttccctggaaaatgtcctaagtcaaaacaacaacaacaacaacaacttcatctttagaaatagggtgccttcacaaatatgggtaagccaacagttcatcgaatactatagggaaagagagagagaacggggatgagacagcaaaaacattaagacttgttctcagcattgctctcctctcactgggcagtggctgaaaacaccagaaaagttgcattaataaaactgcatatagtctaacactgcacagagtgctttgatacaagtatcctcttgctacttcatcttttcaatacatctttgcaaggtttgttttcaaaaagacattacaagttggcaggcttctgcttataaaaatcaatgaaatactttcccttcaactctatgaaacctgccatatacctgagatttattcttctcaaataaatcaaacataggcaacgtaacactctggagtcaacacagaacatgccagggtgagttcaggcaatgaaagaaccacttttctgcaaatacatggtagaattgaagactgtttgtagctgtcgataatttgtaaaaacatttccaatgttctttgaacaaaagattttgattcagccaagattacagaaaggaatcatgacaaagtcctaagtgtacctttgtgtgtatttcatctgctcagcttttgcaggtgactgtggtggtggttgcctggatatggaattcctttgccctcaaatcttcacatgcatgaagtgcaataaagaataaaatgctgtgtttatgtcgcaccacttctaagaggtttaaagcgccgtacgaatgttaccacatgaatccccacaacacccctgtgaggtaggtaggtggagagtattgtcatccccactttacaggtgggagaaatgaggcacccaatagttaataagagatttgctcaaaatcacacagctagtcactggcagggcttagaataaaatgtatactgattagcacctagcacagtgctttgcacatagtaggtgttcgtttaatatctgtggattttatttgacttatgtctcaacatacaatatacacacataaagtacaagcagccaccgtaaaacatttttctgatgatatctctcattacttcaaatcctggtggaggaaggaggttcaagaatccatctcacaattaagacctcagggttgaagaggatcatcataaaaactatcagctgacaaccagctcttacacctgctctaccacacaatattattaatagttttctaatgaaaacaaaaatggatttcaggaaccatgctgacattattttttgcctgtttgttttcaatggagtcatctgaatggttctgtgttttgtttgtacaaaaaagaaataaggctgctatagtccagttagcatgtgaaaactctgccaagcacgaagatctcctcccagctcggatggattgctacctgggaaaatggaccgacccagggagtggcaggtcccaaggaagagggtcagtgaggctggacgtcacttgcactgttcgtggtctgtatagtcatccatgtccacatccgaatcaaagagtgagtgtccagtaaaatctgtgtctggggttctggaaaaactgttttctgctccctcatcttcaaaggtctctgtccttgagtaaaagctaaaatccagcagcggggtgtgggttttgctgccttcgctgctctcctcagactcatagatggtattgtcatcatcgtggtgccactctggccaaaatttcctccttatcctctcacagtacatggcaaggttgatcagctcacctttgatcagccgttcgggtcttgtccctggtaaggtccacattgcctgtgccaagtgtccaaagacagtggcgtcaagagtggaaagcttgggccccatgatgtacttcttatcaccagtagaagtgctcctccaccatcttggtcaccgctctggagatggctctttcatgagggccaaggtttttgtttaaattcactccaagcttctcttccagaaagtcaattatgaattctgtgccagaaactttttcatgattatattcaatccaaggcattttcccttgagcagagagttttccaccaaaatagttctgatacggtaagtcagccatccttaaataagtttccatctttaaacagaaaggagataaacttggaacaccattgttaggtcttgcaaactgatgcaaaataatagcatctttagagtcaatctcttgctgtttcctaatgaccaggagttcgtggagcagatacgcagctgcggccagcaaagctcccccggtcaagtaaagggttttcttccaccagggatcggagcccagccctgccatgatcccaccgtaatcctggggcggcgcggagctgcgggcaggagacgccaccaggc

SEQ ID NO: 15122 - RNA, 9948 nt, Homo sapiens
  source 1..9948: mol_type = other RNA
gctgggattacaggcatgagccactgcaccctgcctaattgagacaatatttatacaaggggaaattggtctattataaggcctagccatagtaaaggtctcaacatgtgctcccagctctccctctcctccttgtcttctctctaccagtggttctcacacttcgtaacactctgaggcacactgggcatgaaataaaagcaggagaggatgggacagcatattccagagatctgtttttcttcttaaaagccactcacttgaaattctatcaaagttatatgcctaaaaaattcattacctctgttttaattatacaagagccttacaactaaaatactctcccagtcatctaagagaccaccacttaacagtatattagatgcaaacatttcagattttccccatgagcctgaagtttaaacattcaaatttgcaaaagagaagtaaattggaagaaagacattcacagaaaactatttcatatccattagttatcatttacacatcaaatacatatagcattaagaccaaatatacagaatttccacatttatatacagtagtcaacatagtgcacaattcaaatctatcttacaatcaagtgtacaagtttaaatatggctttataaactactaataactctgctaaagtaactcatagatccagaaataaacactgaaatgccatcttcacattggggtcatcattcagcaagatgctaatcattgtgattgcaaaacagagggtgcaggtaagtgtttccaggtggtgtccgcccattagccccgaaatgtgggttcaaattatgccaacattggcccttcctatctcagatacctaaaaataagtctgcacatcttccacacatttgaagacacaagattataaacaaatagaaaaaaagacatgtaatcagtgagatgatgaattatcaggcattatcaaaacatgtttttcagattgatgctgaaattcacagacaatacatcctgcatttgcattatctgggtatcacctcacccctactttcttttcttgttttgcttacctcagtgtgttgttaaatctttctggaattttcaaggcattctagatcaagtggtcccaaaagcagaattaaaaacatcagtcttaaaggtgacatcaaattgttcatccttctctttcccaaccaaaaatgcctattttaagtaaaaataattaaataccttgacctaaaatcatgcgtccatgcctgttttatatctgctttgccacaaatggtatatacacattctctaatcaattacaggcatctgggtgctacgcctaaagactccttgtcccattctctaaactccattgaggaccagaaaatatacttttaaaatgtctatgtttgctatggtttttaatgtttacatcagtaaaacagtatatacatatatagcagtgtatacatatatacatatatatcataaataaatacatggaggggcatgctcagaaagttttactaatagggtgaataaacataaacgtttggagaccactgcctaaatagggatggacgatctgggctgtctgcaaacatttaaaagacttctctaaaacaaaatgtacattactttgtacaattttatatttataaaatgaaaaatatatgccacaaacactcttgagagactagaaggaaattccaaaattaaaggagtaaatgtatcagggccagaccctctaagctgctatctaaggtcccaggcctggcttcagaaggggaatgggggacatgagcatagaaattaagataaagataaatgttacttcacttcctgcactggccacttgtatatccatagacaatccttccctacatagattgcacttgtttttgatttataaacctgtactttttattattttagcaagatggcaccacctagaaaactttcaattgcctgatacatctctaccacagccataccacatggttgcttgaaattttgacatttgttactgttttcttctctcctcctactcagttaaattctaataccaccaaatgagggactcagaccctcagttttccaaacttcaccatggaaaaaccatcgctgtcatcaacatttgagttgtcagacatttggcatgatgtagatcactgggaaaaaaacatgtgtttacaataagcttgttctgatcccacaagacttattacttgcaataaaatcattttgacaggagtaacattaaaatcattttacaggagtaaacatgtcacccctactgaagcagaagcctttagccttatttctgtaaaaaacaaatcccaggcataatttgttaaagataaaaatacaatcatttggacatggtttatattttaataagccaaatataatctcttgtagaagagaagcaaatacgaaagaacatttctgattctgaacaatggaagaggaaagtcattgattattttttaaagaggaggaagacagtaaatattcagagcattcctcttttttagccctcaatgaacaattatattatattccctttgctatctgtttagccaccattaactaacatggcaattcagaagttggatcttatttttttagaagccatggggtaactaaaaacaaaaaaggtattaaataaggaaaaaagcttaagcattactaataagtgaaagttactctattccagagccacaaataaaaacaaataaataaaaataaatgcatgccaatggggggtgggaggtgaattagtcacatttagtagcacaactttttataaagttaactgattatgatacacatatattgctttatggttagtggattgtttcaaaaatgcatgatggccattaaattctttgctaaaattattgtgtacagaacaccaaagtaccgtatccatcttttactccagattacttgttttcctactgaaatggtcagtttggtgctgctagaccatatctgtaggttattcgttttattattgcaatggtcccctttatttgtctaccaattttacaatttaaggcaatcatccttatgaaatttgagcatcctagtttgtcatggtccagccaatagcaggagttttagagggtctaggtctggggacaagttccttgcttcggcgaaagcagaatggttgaggaggtcaccctgtcagctccaaaacagctgaaccccttttttttaaatctatgcttcagtgccctctgtaatcatctctaactggcaaggctaacgttgctggttccagcagtctcatctcaaagattaaggaaacttaaatatccttaagatattcttgaaagtcagggaccaaaaatctgagtttctgggtaaggaattcagatgaggaaaacatgccacagatgttcgcatccacgcctgacagtagcaagagtcttacaggtaagaggcccgtccctcctcacccaacaagggaatccttttgaacttcccaagttatatccagaccactggaagcaactgaataaaggtcaagcacttcacaatcacatgcaattgatccctggacctgttaaagatgggttcccagagcccagcatttagcctgggaagtattcgtcattgagtgtacttttatcagttctagtttgacttaaatagcactgcatataaaggagaacaaaggatcctgggtcatagtcaggaacaataaaataacatactctgtttaaaaaaaaaaaaaaccctaaaagaaagaaagaagaataacctgagttgttccctatcaacaaaagccaccaaccttttattgaaaatacactcaacaattgttctatgaatgaatgaataaatgaatacaggaaaacctgattgtgcagacctttcttctttaaggaagaaaaatccagcctcttctctcccaccttcagcccaggctggttgccctatccatgcagaagcggtgggtttcagggctgaaaggaagcgcacttggccctgaactcattttgataaatcaattttgggggtggttaaaagataaatgacaaggacaacaacaaaatcctatgactttcaaaattccaaacctctaaaacaaaattttctcaaataacctaagagcacttctttcttcttttctgtcactcaagacatactgaacatggataatagagattacttttgcttgcatagcctgtactaatttttcttctctctggctgtgttaaaaacaagaacaaacacaatgataacatttaaagactcttgggaacaagactctttaactggggtccattaaccccctgaggaaaccatggataatttcaggaggtctctaaatttcctgaatttatatgtaacattttatgtatttgcatatatgtgtttttctgggaatagggtatagaactttcgttggattatcagtggagttcctgacaaacaaaaagtgaaaattcactatttaatggtatgtgactcactctctgagcatctttcccatgcaaccttcagggaaggaagtgatgagtgcttcattttcaaaggaagagattataatcagctgggaagccttcatgtgaagctgacgaagtcagaccttgagagatgggcatgacttgggccagtggagcagagaatagaacatttcaggagaaggactggcatgagcagaggcacagaggtgggccacatgaggcttttttaggcaatggcaaatggatcaacctggctgcactggatggctcccatggaggagctatggagacaaggtgaacaaaggtgaaaacaccagaccctaaggagtagcccctcaccctgaggcaatgccacaccccatcagggccaaagagctttttagaaagattaatccatttgtagtggatggaatggaacagggaaatggccaagtacgtaaaagaggctagagaagtctaggcaaaagaggatgccctgaaatcagagttctatgctgttctatttgccactctacaaccagtgtagatcccagggccaggcacagggtaggtgctctgtaaatattcagcaagtgagggaatggacatgggttctttaaaagatacataaggaagtatgaggagtcttggtgatttgggaatccatcttgctattcttcagagtctagcaataccctgcactgatgagaggtctcttgtattggtcttgaccaggctgacaggacatggacaaaagcgaagtaggattccaaccagggaatggctggagatgtgctggttgtctgaacacagggtgacttctcaggtaacatgcattttataagacaacaaagccacagtggtataatggaaagaaccatcaagggcaaggtggtataatagaaagaaaccatcaagggcaacgtggtgtaatggaaagaaccatattgacctcagtttttggtcctgcccttcaaataagtatgtatgtgacactgagccaataaggtgctttctacagctaatttttagcacagctatacatttctatgactctacattatctctcaaacaaatctaagcaagacccacaaggccaaaatccttagtatgtctgttccttgaaccttagctatttcacaaaaatataccctaacaccacagtatacatgggcagggctcacttgaggagtagactgcagtctgattcaagtccaagttgttccaggtccgtgattagtctcctgggtagcccacagccttggtagtgtcactttctacaattcattatgtaacaacaacaaattggtaaatgctgacaatatagttcatcattgcataaatatagattgtccttatatctgttctgatggagagtaaagctcaatgattctgctcattaatcttgttgagtgggggtacagatgggcaaagagaggtggatgcaagagcttgatttacttttacaatgacaggaaaaaaagaacgaatagcctatgggtctgttgtccaaccaaaagcatctgttaacattaaagatcacatacttcaagttaccttccagcaaaaaggaaacacagaacttgaacaagaagccagatgaccaaaatgtcccttaacttcttatagttttttcctataattagcacctgttcatgaaattggagaacatttcaaatctgggtagcttaagaatgaagcacataaaattaaatccttccggataaagactcacactatggtgactttgtcttggttattttgtttgcataacccgccttgggaaagtaaagcaggggcatattctagggctctaaatcaaattaacacctacaaaatgttgatgcccagttatatgctgtcaggcaattgcccaagactccagatagcaatgtccattcatgcccctgtaagaggtacctggatggaatgacttattttacaacttcattttcaaagttggttctccacatacttgtattccaagtaatataaaattaaaaacatatattaatctacattctcataacttaatcatcctttgagagaaaatacatcacacttggtactgtacagtaagatagattgttcatagaaaaaaattcaaatacatttcttttctactaaaatgtggtgggaaaaggacaacccatgctttgtggagacaggtctgcagtccacctgttcattatattcatattttcagtccaggagtctccctagtcacacagaaatgccaccagttggccttaaaacacacttgctagagagaggggaggcaaacagtcctcccaaatgatgctgcagcctcaaacaggcttatccattcatatcttctccaccacattcttattaggcatcaaacagtccctttaaataagaatggttttaataagatattaacaactaagtttcccatggaataagaatttctaacttagggtatctcagcacgtattcccagttacatatgccctacacaattgcttaagtggtaagcagtctgaaaaactctcctccctttacctctttgtgaatctacagcagtcttttaagattgttttgcaaatgctatattcaaaaagaggttttttttttttcaagtaaagtgcatggatttctcagaagttgctgtattttaagaagtgcctctttaaccccataatgagcaatccttatgttggtcagaagcaaagcagttttgtttgcaattgtaaatcttggctctcctagcccaaatctcacagccatcacccaggatctctgccccatatttccctggaaaatgtcctaagtcaaaacaacaacaacaacaacaacttcatctttagaaatagggtgccttcacaaatatgggtaagccaacagttcatcgaatactatagggaaagagagagagaacggggatgagacagcaaaaacattaagacttgttctcagcattgctctcctctcactgggcagtggctgaaaacaccagaaaagttgcattaataaaactgcatatagtctaacactgcacagagtgctttgatacaagtatcctcttgctacttcatcttttcaatacatctttgcaaggtttgttttcaaaaagacattacaagttggcaggcttctgcttataaaaatcaatgaaatactttcccttcaactctatgaaacctgccatatacctgagatttattcttctcaaataaatcaaacataggcaacgtaacactctggagtcaacacagaacatgccagggtgagttcaggcaatgaaagaaccacttttctgcaaatacatggtagaattgaagactgtttgtagctgtcgataatttgtaaaaacatttccaatgttctttgaacaaaagattttgattcagccaagattacagaaaggaatcatgacaaagtcctaagtgtacctttgtgtgtatttcatctgctcagcttttgcaggtgactgtggtggtggttgcctggatatggaattcctttgccctcaaatcttcacatgcatgaagtgcaataaagaataaaatgctgtgtttatgtcgcaccacttctaagaggtttaaagcgccgtacgaatgttaccacatgaatccccacaacacccctgtgaggtaggtaggtggagagtattgtcatccccactttacaggtgggagaaatgaggcacccaatagttaataagagatttgctcaaaatcacacagctagtcactggcagggcttagaataaaatgtatactgattagcacctagcacagtgctttgcacatagtaggtgttcgtttaatatctgtggattttatttgacttatgtctcaacatacaatatacacacataaagtacaagcagccaccgtaaaacatttttctgatgatatctctcattacttcaaatcctggtggaggaaggaggttcaagaatccatctcacaattaagacctcagggttgaagaggatcatcataaaaactatcagctgacaaccagctcttacacctgctctaccacacaatattattaatagttttctaatgaaaacaaaaatggatttcaggaaccatgctgacattattttttgcctgtttgttttcaatggagtcatctgaatggttctgtgttttgtttgtacaaaaaagaaataaggctgctatagtccagttagcatgtgaaaactctgccaagcacgaagatctcctcccagctcggatggattgctacctgggaaaatggaccgacccagggagtggcaggtcccaaggaagagggtcagtgaggctggacgtcacttgcactgttcgtggtctgtatagtcatccatgtccacatccgaatcaaagagtgagtgtccagtaaaatctgtgtctggggttctggaaaaactgttttctgctccctcatcttcaaaggtctctgtccttgagtaaaagctaaaatccagcagcggggtgtgggttttgctgccttcgctgctctcctcagactcatagatggtattgtcatcatcgtggtgccactctggccaaaatttcctccttatcctctcacagtacatggcaaggttgatcagctcacctttgatcagccgttcgggtcttgtccctggtaaggtccacattgcctgtgccaagtgtccaaagacagtggcgtcaagagtggaaagcttgggccccatgatgtacttcttatcacccaaaagccctgctaaagaccgcatgtccttctccatcagcatgtaaatctcttcctcggagaagcggccaatgccgtggccgtgcatctcgcgtttcacaattcctttcgttatgtggcacacaacccacctcagcaggttgctgaagggaccaccaccactaagagagagcatcttccgggtctcattgagattgtccacccactggcaataagctaatgtccagtagaagtgctcctccaccatcttggtcaccgctctggagatggctctttcatgagggccaaggtttttgtttaaattcactccaagcttctcttccagaaagtcaattatgaattctgtgccagaaactttttcatgattatattcaatccaaggcattttcccttgagcagagagttttccaccaaaatagttctgatacggtaagtcagccatccttaaataagtttccatctttaaacagaaaggagataaacttggaacaccattgttaggtcttgcaaactgatgcaaaataatagcatctttagagtcaatctcttgctgtttccccgcgccctgccccctccccgcatctccgcggtccggccgcctccgccggggccggatctgcagggctgaggcgcgccgggcaggctccgcgcctccgggcggcacgcccaaaaaccgctcgccgcgcgcgggcaagggcggcggaggtgcctggaaatgcggccccaccgcgaggaagctgcagtcggggcccggatcccggtcctcccctaccccggccggccctccgcctgcgctccagcccctcccgcgggcccc

SEQ ID NO: 15123 - RNA, 10070 nt, Homo sapiens
  source 1..10070: mol_type = other RNA
gctgggattacaggcatgagccactgcaccctgcctaattgagacaatatttatacaaggggaaattggtctattataaggcctagccatagtaaaggtctcaacatgtgctcccagctctccctctcctccttgtcttctctctaccagtggttctcacacttcgtaacactctgaggcacactgggcatgaaataaaagcaggagaggatgggacagcatattccagagatctgtttttcttcttaaaagccactcacttgaaattctatcaaagttatatgcctaaaaaattcattacctctgttttaattatacaagagccttacaactaaaatactctcccagtcatctaagagaccaccacttaacagtatattagatgcaaacatttcagattttccccatgagcctgaagtttaaacattcaaatttgcaaaagagaagtaaattggaagaaagacattcacagaaaactatttcatatccattagttatcatttacacatcaaatacatatagcattaagaccaaatatacagaatttccacatttatatacagtagtcaacatagtgcacaattcaaatctatcttacaatcaagtgtacaagtttaaatatggctttataaactactaataactctgctaaagtaactcatagatccagaaataaacactgaaatgccatcttcacattggggtcatcattcagcaagatgctaatcattgtgattgcaaaacagagggtgcaggtaagtgtttccaggtggtgtccgcccattagccccgaaatgtgggttcaaattatgccaacattggcccttcctatctcagatacctaaaaataagtctgcacatcttccacacatttgaagacacaagattataaacaaatagaaaaaaagacatgtaatcagtgagatgatgaattatcaggcattatcaaaacatgtttttcagattgatgctgaaattcacagacaatacatcctgcatttgcattatctgggtatcacctcacccctactttcttttcttgttttgcttacctcagtgtgttgttaaatctttctggaattttcaaggcattctagatcaagtggtcccaaaagcagaattaaaaacatcagtcttaaaggtgacatcaaattgttcatccttctctttcccaaccaaaaatgcctattttaagtaaaaataattaaataccttgacctaaaatcatgcgtccatgcctgttttatatctgctttgccacaaatggtatatacacattctctaatcaattacaggcatctgggtgctacgcctaaagactccttgtcccattctctaaactccattgaggaccagaaaatatacttttaaaatgtctatgtttgctatggtttttaatgtttacatcagtaaaacagtatatacatatatagcagtgtatacatatatacatatatatcataaataaatacatggaggggcatgctcagaaagttttactaatagggtgaataaacataaacgtttggagaccactgcctaaatagggatggacgatctgggctgtctgcaaacatttaaaagacttctctaaaacaaaatgtacattactttgtacaattttatatttataaaatgaaaaatatatgccacaaacactcttgagagactagaaggaaattccaaaattaaaggagtaaatgtatcagggccagaccctctaagctgctatctaaggtcccaggcctggcttcagaaggggaatgggggacatgagcatagaaattaagataaagataaatgttacttcacttcctgcactggccacttgtatatccatagacaatccttccctacatagattgcacttgtttttgatttataaacctgtactttttattattttagcaagatggcaccacctagaaaactttcaattgcctgatacatctctaccacagccataccacatggttgcttgaaattttgacatttgttactgttttcttctctcctcctactcagttaaattctaataccaccaaatgagggactcagaccctcagttttccaaacttcaccatggaaaaaccatcgctgtcatcaacatttgagttgtcagacatttggcatgatgtagatcactgggaaaaaaacatgtgtttacaataagcttgttctgatcccacaagacttattacttgcaataaaatcattttgacaggagtaacattaaaatcattttacaggagtaaacatgtcacccctactgaagcagaagcctttagccttatttctgtaaaaaacaaatcccaggcataatttgttaaagataaaaatacaatcatttggacatggtttatattttaataagccaaatataatctcttgtagaagagaagcaaatacgaaagaacatttctgattctgaacaatggaagaggaaagtcattgattattttttaaagaggaggaagacagtaaatattcagagcattcctcttttttagccctcaatgaacaattatattatattccctttgctatctgtttagccaccattaactaacatggcaattcagaagttggatcttatttttttagaagccatggggtaactaaaaacaaaaaaggtattaaataaggaaaaaagcttaagcattactaataagtgaaagttactctattccagagccacaaataaaaacaaataaataaaaataaatgcatgccaatggggggtgggaggtgaattagtcacatttagtagcacaactttttataaagttaactgattatgatacacatatattgctttatggttagtggattgtttcaaaaatgcatgatggccattaaattctttgctaaaattattgtgtacagaacaccaaagtaccgtatccatcttttactccagattacttgttttcctactgaaatggtcagtttggtgctgctagaccatatctgtaggttattcgttttattattgcaatggtcccctttatttgtctaccaattttacaatttaaggcaatcatccttatgaaatttgagcatcctagtttgtcatggtccagccaatagcaggagttttagagggtctaggtctggggacaagttccttgcttcggcgaaagcagaatggttgaggaggtcaccctgtcagctccaaaacagctgaaccccttttttttaaatctatgcttcagtgccctctgtaatcatctctaactggcaaggctaacgttgctggttccagcagtctcatctcaaagattaaggaaacttaaatatccttaagatattcttgaaagtcagggaccaaaaatctgagtttctgggtaaggaattcagatgaggaaaacatgccacagatgttcgcatccacgcctgacagtagcaagagtcttacaggtaagaggcccgtccctcctcacccaacaagggaatccttttgaacttcccaagttatatccagaccactggaagcaactgaataaaggtcaagcacttcacaatcacatgcaattgatccctggacctgttaaagatgggttcccagagcccagcatttagcctgggaagtattcgtcattgagtgtacttttatcagttctagtttgacttaaatagcactgcatataaaggagaacaaaggatcctgggtcatagtcaggaacaataaaataacatactctgtttaaaaaaaaaaaaaaccctaaaagaaagaaagaagaataacctgagttgttccctatcaacaaaagccaccaaccttttattgaaaatacactcaacaattgttctatgaatgaatgaataaatgaatacaggaaaacctgattgtgcagacctttcttctttaaggaagaaaaatccagcctcttctctcccaccttcagcccaggctggttgccctatccatgcagaagcggtgggtttcagggctgaaaggaagcgcacttggccctgaactcattttgataaatcaattttgggggtggttaaaagataaatgacaaggacaacaacaaaatcctatgactttcaaaattccaaacctctaaaacaaaattttctcaaataacctaagagcacttctttcttcttttctgtcactcaagacatactgaacatggataatagagattacttttgcttgcatagcctgtactaatttttcttctctctggctgtgttaaaaacaagaacaaacacaatgataacatttaaagactcttgggaacaagactctttaactggggtccattaaccccctgaggaaaccatggataatttcaggaggtctctaaatttcctgaatttatatgtaacattttatgtatttgcatatatgtgtttttctgggaatagggtatagaactttcgttggattatcagtggagttcctgacaaacaaaaagtgaaaattcactatttaatggtatgtgactcactctctgagcatctttcccatgcaaccttcagggaaggaagtgatgagtgcttcattttcaaaggaagagattataatcagctgggaagccttcatgtgaagctgacgaagtcagaccttgagagatgggcatgacttgggccagtggagcagagaatagaacatttcaggagaaggactggcatgagcagaggcacagaggtgggccacatgaggcttttttaggcaatggcaaatggatcaacctggctgcactggatggctcccatggaggagctatggagacaaggtgaacaaaggtgaaaacaccagaccctaaggagtagcccctcaccctgaggcaatgccacaccccatcagggccaaagagctttttagaaagattaatccatttgtagtggatggaatggaacagggaaatggccaagtacgtaaaagaggctagagaagtctaggcaaaagaggatgccctgaaatcagagttctatgctgttctatttgccactctacaaccagtgtagatcccagggccaggcacagggtaggtgctctgtaaatattcagcaagtgagggaatggacatgggttctttaaaagatacataaggaagtatgaggagtcttggtgatttgggaatccatcttgctattcttcagagtctagcaataccctgcactgatgagaggtctcttgtattggtcttgaccaggctgacaggacatggacaaaagcgaagtaggattccaaccagggaatggctggagatgtgctggttgtctgaacacagggtgacttctcaggtaacatgcattttataagacaacaaagccacagtggtataatggaaagaaccatcaagggcaaggtggtataatagaaagaaaccatcaagggcaacgtggtgtaatggaaagaaccatattgacctcagtttttggtcctgcccttcaaataagtatgtatgtgacactgagccaataaggtgctttctacagctaatttttagcacagctatacatttctatgactctacattatctctcaaacaaatctaagcaagacccacaaggccaaaatccttagtatgtctgttccttgaaccttagctatttcacaaaaatataccctaacaccacagtatacatgggcagggctcacttgaggagtagactgcagtctgattcaagtccaagttgttccaggtccgtgattagtctcctgggtagcccacagccttggtagtgtcactttctacaattcattatgtaacaacaacaaattggtaaatgctgacaatatagttcatcattgcataaatatagattgtccttatatctgttctgatggagagtaaagctcaatgattctgctcattaatcttgttgagtgggggtacagatgggcaaagagaggtggatgcaagagcttgatttacttttacaatgacaggaaaaaaagaacgaatagcctatgggtctgttgtccaaccaaaagcatctgttaacattaaagatcacatacttcaagttaccttccagcaaaaaggaaacacagaacttgaacaagaagccagatgaccaaaatgtcccttaacttcttatagttttttcctataattagcacctgttcatgaaattggagaacatttcaaatctgggtagcttaagaatgaagcacataaaattaaatccttccggataaagactcacactatggtgactttgtcttggttattttgtttgcataacccgccttgggaaagtaaagcaggggcatattctagggctctaaatcaaattaacacctacaaaatgttgatgcccagttatatgctgtcaggcaattgcccaagactccagatagcaatgtccattcatgcccctgtaagaggtacctggatggaatgacttattttacaacttcattttcaaagttggttctccacatacttgtattccaagtaatataaaattaaaaacatatattaatctacattctcataacttaatcatcctttgagagaaaatacatcacacttggtactgtacagtaagatagattgttcatagaaaaaaattcaaatacatttcttttctactaaaatgtggtgggaaaaggacaacccatgctttgtggagacaggtctgcagtccacctgttcattatattcatattttcagtccaggagtctccctagtcacacagaaatgccaccagttggccttaaaacacacttgctagagagaggggaggcaaacagtcctcccaaatgatgctgcagcctcaaacaggcttatccattcatatcttctccaccacattcttattaggcatcaaacagtccctttaaataagaatggttttaataagatattaacaactaagtttcccatggaataagaatttctaacttagggtatctcagcacgtattcccagttacatatgccctacacaattgcttaagtggtaagcagtctgaaaaactctcctccctttacctctttgtgaatctacagcagtcttttaagattgttttgcaaatgctatattcaaaaagaggttttttttttttcaagtaaagtgcatggatttctcagaagttgctgtattttaagaagtgcctctttaaccccataatgagcaatccttatgttggtcagaagcaaagcagttttgtttgcaattgtaaatcttggctctcctagcccaaatctcacagccatcacccaggatctctgccccatatttccctggaaaatgtcctaagtcaaaacaacaacaacaacaacaacttcatctttagaaatagggtgccttcacaaatatgggtaagccaacagttcatcgaatactatagggaaagagagagagaacggggatgagacagcaaaaacattaagacttgttctcagcattgctctcctctcactgggcagtggctgaaaacaccagaaaagttgcattaataaaactgcatatagtctaacactgcacagagtgctttgatacaagtatcctcttgctacttcatcttttcaatacatctttgcaaggtttgttttcaaaaagacattacaagttggcaggcttctgcttataaaaatcaatgaaatactttcccttcaactctatgaaacctgccatatacctgagatttattcttctcaaataaatcaaacataggcaacgtaacactctggagtcaacacagaacatgccagggtgagttcaggcaatgaaagaaccacttttctgcaaatacatggtagaattgaagactgtttgtagctgtcgataatttgtaaaaacatttccaatgttctttgaacaaaagattttgattcagccaagattacagaaaggaatcatgacaaagtcctaagtgtacctttgtgtgtatttcatctgctcagcttttgcaggtgactgtggtggtggttgcctggatatggaattcctttgccctcaaatcttcacatgcatgaagtgcaataaagaataaaatgctgtgtttatgtcgcaccacttctaagaggtttaaagcgccgtacgaatgttaccacatgaatccccacaacacccctgtgaggtaggtaggtggagagtattgtcatccccactttacaggtgggagaaatgaggcacccaatagttaataagagatttgctcaaaatcacacagctagtcactggcagggcttagaataaaatgtatactgattagcacctagcacagtgctttgcacatagtaggtgttcgtttaatatctgtggattttatttgacttatgtctcaacatacaatatacacacataaagtacaagcagccaccgtaaaacatttttctgatgatatctctcattacttcaaatcctggtggaggaaggaggttcaagaatccatctcacaattaagacctcagggttgaagaggatcatcataaaaactatcagctgacaaccagctcttacacctgctctaccacacaatattattaatagttttctaatgaaaacaaaaatggatttcaggaaccatgctgacattattttttgcctgtttgttttcaatggagtcatctgaatggttctgtgttttgtttgtacaaaaaagaaataaggctgctatagtccagttagcatgtgaaaactctgccaagcacgaagatctcctcccagctcggatggattgctacctgggaaaatggaccgacccagggagtggcaggtcccaaggaagagggtcagtgaggctggacgtcacttgcactgttcgtggtctgtatagtcatccatgtccacatccgaatcaaagagtgagtgtccagtaaaatctgtgtctggggttctggaaaaactgttttctgctccctcatcttcaaaggtctctgtccttgagtaaaagctaaaatccagcagcggggtgtgggttttgctgccttcgctgctctcctcagactcatagatggtattgtcatcatcgtggtgccactctggccaaaatttcctccttatcctctcacagtacatggcaaggttgatcagctcacctttgatcagccgttcgggtcttgtccctggtaaggtccacattgcctgtgccaagtgtccaaagacagtggcgtcaagagtggaaagcttgggccccatgatgtacttcttatcacccaaaagccctgctaaagaccgcatgtccttctccatcagcatgtaaatctcttcctcggagaagcggccaatgccgtggccgtgcatctcgcgtttcacaattcctttcgttatgtggcacacaacccacctcagcaggttgctgaagggaccaccaccactaagagagagcatcttccgggtctcattgagattgtccacccactggcaataagctaatgtccagtagaagtgctcctccaccatcttggtcaccgctctggagatggctctttcatgagggccaaggtttttgtttaaattcactccaagcttctcttccagaaagtcaattatgaattctgtgccagaaactttttcatgattatattcaatccaaggcattttcccttgagcagagagttttccaccaaaatagttctgatacggtaagtcagccatccttaaataagtttccatctttaaacagaaaggagataaacttggaacaccattgttaggtcttgcaaactgatgcaaaataatagcatctttagagtcaatctcttgctgtttcctaatgaccaggagttcgtggagcagatacgcagctgcggccagcaaagctcccccggtcaagtaaagggttttcttccaccagggatcggagcccagccctgccatgatcccaccgtaatccccgcgccctgccccctccccgcatctccgcggtccggccgcctccgccggggccggatctgcagggctgaggcgcgccgggcaggctccgcgcctccgggcggcacgcccaaaaaccgctcgccgcgcgcgggcaagggcggcggaggtgcctggaaatgcggccccaccgcgaggaagctgcagtcggggcccggatcccggtcctcccctaccccggccggccctccgcctgcgctccagcccctcccgcgggcccc

SEQ ID NO: 15124 - RNA, 10256 nt, Homo sapiens
  source 1..10256: mol_type = other RNA
gctgggattacaggcatgagccactgcaccctgcctaattgagacaatatttatacaaggggaaattggtctattataaggcctagccatagtaaaggtctcaacatgtgctcccagctctccctctcctccttgtcttctctctaccagtggttctcacacttcgtaacactctgaggcacactgggcatgaaataaaagcaggagaggatgggacagcatattccagagatctgtttttcttcttaaaagccactcacttgaaattctatcaaagttatatgcctaaaaaattcattacctctgttttaattatacaagagccttacaactaaaatactctcccagtcatctaagagaccaccacttaacagtatattagatgcaaacatttcagattttccccatgagcctgaagtttaaacattcaaatttgcaaaagagaagtaaattggaagaaagacattcacagaaaactatttcatatccattagttatcatttacacatcaaatacatatagcattaagaccaaatatacagaatttccacatttatatacagtagtcaacatagtgcacaattcaaatctatcttacaatcaagtgtacaagtttaaatatggctttataaactactaataactctgctaaagtaactcatagatccagaaataaacactgaaatgccatcttcacattggggtcatcattcagcaagatgctaatcattgtgattgcaaaacagagggtgcaggtaagtgtttccaggtggtgtccgcccattagccccgaaatgtgggttcaaattatgccaacattggcccttcctatctcagatacctaaaaataagtctgcacatcttccacacatttgaagacacaagattataaacaaatagaaaaaaagacatgtaatcagtgagatgatgaattatcaggcattatcaaaacatgtttttcagattgatgctgaaattcacagacaatacatcctgcatttgcattatctgggtatcacctcacccctactttcttttcttgttttgcttacctcagtgtgttgttaaatctttctggaattttcaaggcattctagatcaagtggtcccaaaagcagaattaaaaacatcagtcttaaaggtgacatcaaattgttcatccttctctttcccaaccaaaaatgcctattttaagtaaaaataattaaataccttgacctaaaatcatgcgtccatgcctgttttatatctgctttgccacaaatggtatatacacattctctaatcaattacaggcatctgggtgctacgcctaaagactccttgtcccattctctaaactccattgaggaccagaaaatatacttttaaaatgtctatgtttgctatggtttttaatgtttacatcagtaaaacagtatatacatatatagcagtgtatacatatatacatatatatcataaataaatacatggaggggcatgctcagaaagttttactaatagggtgaataaacataaacgtttggagaccactgcctaaatagggatggacgatctgggctgtctgcaaacatttaaaagacttctctaaaacaaaatgtacattactttgtacaattttatatttataaaatgaaaaatatatgccacaaacactcttgagagactagaaggaaattccaaaattaaaggagtaaatgtatcagggccagaccctctaagctgctatctaaggtcccaggcctggcttcagaaggggaatgggggacatgagcatagaaattaagataaagataaatgttacttcacttcctgcactggccacttgtatatccatagacaatccttccctacatagattgcacttgtttttgatttataaacctgtactttttattattttagcaagatggcaccacctagaaaactttcaattgcctgatacatctctaccacagccataccacatggttgcttgaaattttgacatttgttactgttttcttctctcctcctactcagttaaattctaataccaccaaatgagggactcagaccctcagttttccaaacttcaccatggaaaaaccatcgctgtcatcaacatttgagttgtcagacatttggcatgatgtagatcactgggaaaaaaacatgtgtttacaataagcttgttctgatcccacaagacttattacttgcaataaaatcattttgacaggagtaacattaaaatcattttacaggagtaaacatgtcacccctactgaagcagaagcctttagccttatttctgtaaaaaacaaatcccaggcataatttgttaaagataaaaatacaatcatttggacatggtttatattttaataagccaaatataatctcttgtagaagagaagcaaatacgaaagaacatttctgattctgaacaatggaagaggaaagtcattgattattttttaaagaggaggaagacagtaaatattcagagcattcctcttttttagccctcaatgaacaattatattatattccctttgctatctgtttagccaccattaactaacatggcaattcagaagttggatcttatttttttagaagccatggggtaactaaaaacaaaaaaggtattaaataaggaaaaaagcttaagcattactaataagtgaaagttactctattccagagccacaaataaaaacaaataaataaaaataaatgcatgccaatggggggtgggaggtgaattagtcacatttagtagcacaactttttataaagttaactgattatgatacacatatattgctttatggttagtggattgtttcaaaaatgcatgatggccattaaattctttgctaaaattattgtgtacagaacaccaaagtaccgtatccatcttttactccagattacttgttttcctactgaaatggtcagtttggtgctgctagaccatatctgtaggttattcgttttattattgcaatggtcccctttatttgtctaccaattttacaatttaaggcaatcatccttatgaaatttgagcatcctagtttgtcatggtccagccaatagcaggagttttagagggtctaggtctggggacaagttccttgcttcggcgaaagcagaatggttgaggaggtcaccctgtcagctccaaaacagctgaaccccttttttttaaatctatgcttcagtgccctctgtaatcatctctaactggcaaggctaacgttgctggttccagcagtctcatctcaaagattaaggaaacttaaatatccttaagatattcttgaaagtcagggaccaaaaatctgagtttctgggtaaggaattcagatgaggaaaacatgccacagatgttcgcatccacgcctgacagtagcaagagtcttacaggtaagaggcccgtccctcctcacccaacaagggaatccttttgaacttcccaagttatatccagaccactggaagcaactgaataaaggtcaagcacttcacaatcacatgcaattgatccctggacctgttaaagatgggttcccagagcccagcatttagcctgggaagtattcgtcattgagtgtacttttatcagttctagtttgacttaaatagcactgcatataaaggagaacaaaggatcctgggtcatagtcaggaacaataaaataacatactctgtttaaaaaaaaaaaaaaccctaaaagaaagaaagaagaataacctgagttgttccctatcaacaaaagccaccaaccttttattgaaaatacactcaacaattgttctatgaatgaatgaataaatgaatacaggaaaacctgattgtgcagacctttcttctttaaggaagaaaaatccagcctcttctctcccaccttcagcccaggctggttgccctatccatgcagaagcggtgggtttcagggctgaaaggaagcgcacttggccctgaactcattttgataaatcaattttgggggtggttaaaagataaatgacaaggacaacaacaaaatcctatgactttcaaaattccaaacctctaaaacaaaattttctcaaataacctaagagcacttctttcttcttttctgtcactcaagacatactgaacatggataatagagattacttttgcttgcatagcctgtactaatttttcttctctctggctgtgttaaaaacaagaacaaacacaatgataacatttaaagactcttgggaacaagactctttaactggggtccattaaccccctgaggaaaccatggataatttcaggaggtctctaaatttcctgaatttatatgtaacattttatgtatttgcatatatgtgtttttctgggaatagggtatagaactttcgttggattatcagtggagttcctgacaaacaaaaagtgaaaattcactatttaatggtatgtgactcactctctgagcatctttcccatgcaaccttcagggaaggaagtgatgagtgcttcattttcaaaggaagagattataatcagctgggaagccttcatgtgaagctgacgaagtcagaccttgagagatgggcatgacttgggccagtggagcagagaatagaacatttcaggagaaggactggcatgagcagaggcacagaggtgggccacatgaggcttttttaggcaatggcaaatggatcaacctggctgcactggatggctcccatggaggagctatggagacaaggtgaacaaaggtgaaaacaccagaccctaaggagtagcccctcaccctgaggcaatgccacaccccatcagggccaaagagctttttagaaagattaatccatttgtagtggatggaatggaacagggaaatggccaagtacgtaaaagaggctagagaagtctaggcaaaagaggatgccctgaaatcagagttctatgctgttctatttgccactctacaaccagtgtagatcccagggccaggcacagggtaggtgctctgtaaatattcagcaagtgagggaatggacatgggttctttaaaagatacataaggaagtatgaggagtcttggtgatttgggaatccatcttgctattcttcagagtctagcaataccctgcactgatgagaggtctcttgtattggtcttgaccaggctgacaggacatggacaaaagcgaagtaggattccaaccagggaatggctggagatgtgctggttgtctgaacacagggtgacttctcaggtaacatgcattttataagacaacaaagccacagtggtataatggaaagaaccatcaagggcaaggtggtataatagaaagaaaccatcaagggcaacgtggtgtaatggaaagaaccatattgacctcagtttttggtcctgcccttcaaataagtatgtatgtgacactgagccaataaggtgctttctacagctaatttttagcacagctatacatttctatgactctacattatctctcaaacaaatctaagcaagacccacaaggccaaaatccttagtatgtctgttccttgaaccttagctatttcacaaaaatataccctaacaccacagtatacatgggcagggctcacttgaggagtagactgcagtctgattcaagtccaagttgttccaggtccgtgattagtctcctgggtagcccacagccttggtagtgtcactttctacaattcattatgtaacaacaacaaattggtaaatgctgacaatatagttcatcattgcataaatatagattgtccttatatctgttctgatggagagtaaagctcaatgattctgctcattaatcttgttgagtgggggtacagatgggcaaagagaggtggatgcaagagcttgatttacttttacaatgacaggaaaaaaagaacgaatagcctatgggtctgttgtccaaccaaaagcatctgttaacattaaagatcacatacttcaagttaccttccagcaaaaaggaaacacagaacttgaacaagaagccagatgaccaaaatgtcccttaacttcttatagttttttcctataattagcacctgttcatgaaattggagaacatttcaaatctgggtagcttaagaatgaagcacataaaattaaatccttccggataaagactcacactatggtgactttgtcttggttattttgtttgcataacccgccttgggaaagtaaagcaggggcatattctagggctctaaatcaaattaacacctacaaaatgttgatgcccagttatatgctgtcaggcaattgcccaagactccagatagcaatgtccattcatgcccctgtaagaggtacctggatggaatgacttattttacaacttcattttcaaagttggttctccacatacttgtattccaagtaatataaaattaaaaacatatattaatctacattctcataacttaatcatcctttgagagaaaatacatcacacttggtactgtacagtaagatagattgttcatagaaaaaaattcaaatacatttcttttctactaaaatgtggtgggaaaaggacaacccatgctttgtggagacaggtctgcagtccacctgttcattatattcatattttcagtccaggagtctccctagtcacacagaaatgccaccagttggccttaaaacacacttgctagagagaggggaggcaaacagtcctcccaaatgatgctgcagcctcaaacaggcttatccattcatatcttctccaccacattcttattaggcatcaaacagtccctttaaataagaatggttttaataagatattaacaactaagtttcccatggaataagaatttctaacttagggtatctcagcacgtattcccagttacatatgccctacacaattgcttaagtggtaagcagtctgaaaaactctcctccctttacctctttgtgaatctacagcagtcttttaagattgttttgcaaatgctatattcaaaaagaggttttttttttttcaagtaaagtgcatggatttctcagaagttgctgtattttaagaagtgcctctttaaccccataatgagcaatccttatgttggtcagaagcaaagcagttttgtttgcaattgtaaatcttggctctcctagcccaaatctcacagccatcacccaggatctctgccccatatttccctggaaaatgtcctaagtcaaaacaacaacaacaacaacaacttcatctttagaaatagggtgccttcacaaatatgggtaagccaacagttcatcgaatactatagggaaagagagagagaacggggatgagacagcaaaaacattaagacttgttctcagcattgctctcctctcactgggcagtggctgaaaacaccagaaaagttgcattaataaaactgcatatagtctaacactgcacagagtgctttgatacaagtatcctcttgctacttcatcttttcaatacatctttgcaaggtttgttttcaaaaagacattacaagttggcaggcttctgcttataaaaatcaatgaaatactttcccttcaactctatgaaacctgccatatacctgagatttattcttctcaaataaatcaaacataggcaacgtaacactctggagtcaacacagaacatgccagggtgagttcaggcaatgaaagaaccacttttctgcaaatacatggtagaattgaagactgtttgtagctgtcgataatttgtaaaaacatttccaatgttctttgaacaaaagattttgattcagccaagattacagaaaggaatcatgacaaagtcctaagtgtacctttgtgtgtatttcatctgctcagcttttgcaggtgactgtggtggtggttgcctggatatggaattcctttgccctcaaatcttcacatgcatgaagtgcaataaagaataaaatgctgtgtttatgtcgcaccacttctaagaggtttaaagcgccgtacgaatgttaccacatgaatccccacaacacccctgtgaggtaggtaggtggagagtattgtcatccccactttacaggtgggagaaatgaggcacccaatagttaataagagatttgctcaaaatcacacagctagtcactggcagggcttagaataaaatgtatactgattagcacctagcacagtgctttgcacatagtaggtgttcgtttaatatctgtggattttatttgacttatgtctcaacatacaatatacacacataaagtacaagcagccaccgtaaaacatttttctgatgatatctctcattacttcaaatcctggtggaggaaggaggttcaagaatccatctcacaattaagacctcagggttgaagaggatcatcataaaaactatcagctgacaaccagctcttacacctgctctaccacacaatattattaatagttttctaatgaaaacaaaaatggatttcaggaaccatgctgacattattttttgcctgtttgttttcaatggagtcatctgaatggttctgtgttttgtttgtacaaaaaagaaataaggctgctatagtccagttagcatgtgaaaactctgccaagcacgaagatctcctcccagctcggatggattgctacctgggaaaatggaccgacccagggagtggcaggtcccaaggaagagggtcagtgaggctggacgtcacttgcactgttcgtggtctgtatagtcatccatgtccacatccgaatcaaagagtgagtgtccagtaaaatctgtgtctggggttctggaaaaactgttttctgctccctcatcttcaaaggtctctgtccttgagtaaaagctaaaatccagcagcggggtgtgggttttgctgccttcgctgctctcctcagactcatagatggtattgtcatcatcgtggtgccactctggccaaaatttcctccttatcctctcacagtacatggcaaggttgatcagctcacctttgatcagccgttcgggtcttgtccctggtaaggtccacattgcctgtgccaagtgtccaaagacagtggcgtcaagagtggaaagcttgggccccatgatgtacttcttatcacccaaaagccctgctaaagaccgcatgtccttctccatcagcatgtaaatctcttcctcggagaagcggccaatgccgtggccgtgcatctcgcgtttcacaattcctttcgttatgtggcacacaacccacctcagcaggttgctgaagggaccaccaccactaagagagagcatcttccgggtctcattgagattgtccacccactggcaataagctaatgtccagtagaagtgctcctccaccatcttggtcaccgctctggagatggctctttcatgagggccaaggtttttgtttaaattcactccaagcttctcttccagaaagtcaattatgaattctgtgccagaaactttttcatgattatattcaatccaaggcattttcccttgagcagagagttttccaccaaaatagttctgatacggtaagtcagccatccttaaataagtttccatctttaaacagaaaggagataaacttggaacaccattgttaggtcttgcaaactgatgcaaaataatagcatctttagagtcaatctcttgctgtttcctaatgaccaggagttcgtggagcagatacgcagctgcggccagcaaagctcccccggtcaagtaaagggttttcttccaccagggatcggagcccagccctgccatgatcccaccgtaatcctgcaaagggaaagcgatgatgtccccataaaaggagaagggctcctcggacccggcccaccagccgaagaaggagatgctctggttccagctcagatccaccacgcacggcctggacgaagcaaagccaaccccccagtgcatgctgcgcggctggctccgggcgcccctcccagggcccgcgccgcccgcatgggaaggggccggcgcggcccggcgcgggctcagaggcgcgcggagggcgcgggcggcgcgggcggcggcgactgaggaggcggcggcgactgaggaggcggcggcagaggaggaggaggaggaagggcactggccgcggacggcgggcctggccggcggggccccagagccctgggcggcagcagcggccgccggctccccccgcagctgcctctccgccccgctctttgtgtcggcgcctggagaaggcc

SEQ ID NO: 15125 - RNA, 9851 nt, Homo sapiens
  source 1..9851: mol_type = other RNA
gctgggattacaggcatgagccactgcaccctgcctaattgagacaatatttatacaaggggaaattggtctattataaggcctagccatagtaaaggtctcaacatgtgctcccagctctccctctcctccttgtcttctctctaccagtggttctcacacttcgtaacactctgaggcacactgggcatgaaataaaagcaggagaggatgggacagcatattccagagatctgtttttcttcttaaaagccactcacttgaaattctatcaaagttatatgcctaaaaaattcattacctctgttttaattatacaagagccttacaactaaaatactctcccagtcatctaagagaccaccacttaacagtatattagatgcaaacatttcagattttccccatgagcctgaagtttaaacattcaaatttgcaaaagagaagtaaattggaagaaagacattcacagaaaactatttcatatccattagttatcatttacacatcaaatacatatagcattaagaccaaatatacagaatttccacatttatatacagtagtcaacatagtgcacaattcaaatctatcttacaatcaagtgtacaagtttaaatatggctttataaactactaataactctgctaaagtaactcatagatccagaaataaacactgaaatgccatcttcacattggggtcatcattcagcaagatgctaatcattgtgattgcaaaacagagggtgcaggtaagtgtttccaggtggtgtccgcccattagccccgaaatgtgggttcaaattatgccaacattggcccttcctatctcagatacctaaaaataagtctgcacatcttccacacatttgaagacacaagattataaacaaatagaaaaaaagacatgtaatcagtgagatgatgaattatcaggcattatcaaaacatgtttttcagattgatgctgaaattcacagacaatacatcctgcatttgcattatctgggtatcacctcacccctactttcttttcttgttttgcttacctcagtgtgttgttaaatctttctggaattttcaaggcattctagatcaagtggtcccaaaagcagaattaaaaacatcagtcttaaaggtgacatcaaattgttcatccttctctttcccaaccaaaaatgcctattttaagtaaaaataattaaataccttgacctaaaatcatgcgtccatgcctgttttatatctgctttgccacaaatggtatatacacattctctaatcaattacaggcatctgggtgctacgcctaaagactccttgtcccattctctaaactccattgaggaccagaaaatatacttttaaaatgtctatgtttgctatggtttttaatgtttacatcagtaaaacagtatatacatatatagcagtgtatacatatatacatatatatcataaataaatacatggaggggcatgctcagaaagttttactaatagggtgaataaacataaacgtttggagaccactgcctaaatagggatggacgatctgggctgtctgcaaacatttaaaagacttctctaaaacaaaatgtacattactttgtacaattttatatttataaaatgaaaaatatatgccacaaacactcttgagagactagaaggaaattccaaaattaaaggagtaaatgtatcagggccagaccctctaagctgctatctaaggtcccaggcctggcttcagaaggggaatgggggacatgagcatagaaattaagataaagataaatgttacttcacttcctgcactggccacttgtatatccatagacaatccttccctacatagattgcacttgtttttgatttataaacctgtactttttattattttagcaagatggcaccacctagaaaactttcaattgcctgatacatctctaccacagccataccacatggttgcttgaaattttgacatttgttactgttttcttctctcctcctactcagttaaattctaataccaccaaatgagggactcagaccctcagttttccaaacttcaccatggaaaaaccatcgctgtcatcaacatttgagttgtcagacatttggcatgatgtagatcactgggaaaaaaacatgtgtttacaataagcttgttctgatcccacaagacttattacttgcaataaaatcattttgacaggagtaacattaaaatcattttacaggagtaaacatgtcacccctactgaagcagaagcctttagccttatttctgtaaaaaacaaatcccaggcataatttgttaaagataaaaatacaatcatttggacatggtttatattttaataagccaaatataatctcttgtagaagagaagcaaatacgaaagaacatttctgattctgaacaatggaagaggaaagtcattgattattttttaaagaggaggaagacagtaaatattcagagcattcctcttttttagccctcaatgaacaattatattatattccctttgctatctgtttagccaccattaactaacatggcaattcagaagttggatcttatttttttagaagccatggggtaactaaaaacaaaaaaggtattaaataaggaaaaaagcttaagcattactaataagtgaaagttactctattccagagccacaaataaaaacaaataaataaaaataaatgcatgccaatggggggtgggaggtgaattagtcacatttagtagcacaactttttataaagttaactgattatgatacacatatattgctttatggttagtggattgtttcaaaaatgcatgatggccattaaattctttgctaaaattattgtgtacagaacaccaaagtaccgtatccatcttttactccagattacttgttttcctactgaaatggtcagtttggtgctgctagaccatatctgtaggttattcgttttattattgcaatggtcccctttatttgtctaccaattttacaatttaaggcaatcatccttatgaaatttgagcatcctagtttgtcatggtccagccaatagcaggagttttagagggtctaggtctggggacaagttccttgcttcggcgaaagcagaatggttgaggaggtcaccctgtcagctccaaaacagctgaaccccttttttttaaatctatgcttcagtgccctctgtaatcatctctaactggcaaggctaacgttgctggttccagcagtctcatctcaaagattaaggaaacttaaatatccttaagatattcttgaaagtcagggaccaaaaatctgagtttctgggtaaggaattcagatgaggaaaacatgccacagatgttcgcatccacgcctgacagtagcaagagtcttacaggtaagaggcccgtccctcctcacccaacaagggaatccttttgaacttcccaagttatatccagaccactggaagcaactgaataaaggtcaagcacttcacaatcacatgcaattgatccctggacctgttaaagatgggttcccagagcccagcatttagcctgggaagtattcgtcattgagtgtacttttatcagttctagtttgacttaaatagcactgcatataaaggagaacaaaggatcctgggtcatagtcaggaacaataaaataacatactctgtttaaaaaaaaaaaaaaccctaaaagaaagaaagaagaataacctgagttgttccctatcaacaaaagccaccaaccttttattgaaaatacactcaacaattgttctatgaatgaatgaataaatgaatacaggaaaacctgattgtgcagacctttcttctttaaggaagaaaaatccagcctcttctctcccaccttcagcccaggctggttgccctatccatgcagaagcggtgggtttcagggctgaaaggaagcgcacttggccctgaactcattttgataaatcaattttgggggtggttaaaagataaatgacaaggacaacaacaaaatcctatgactttcaaaattccaaacctctaaaacaaaattttctcaaataacctaagagcacttctttcttcttttctgtcactcaagacatactgaacatggataatagagattacttttgcttgcatagcctgtactaatttttcttctctctggctgtgttaaaaacaagaacaaacacaatgataacatttaaagactcttgggaacaagactctttaactggggtccattaaccccctgaggaaaccatggataatttcaggaggtctctaaatttcctgaatttatatgtaacattttatgtatttgcatatatgtgtttttctgggaatagggtatagaactttcgttggattatcagtggagttcctgacaaacaaaaagtgaaaattcactatttaatggtatgtgactcactctctgagcatctttcccatgcaaccttcagggaaggaagtgatgagtgcttcattttcaaaggaagagattataatcagctgggaagccttcatgtgaagctgacgaagtcagaccttgagagatgggcatgacttgggccagtggagcagagaatagaacatttcaggagaaggactggcatgagcagaggcacagaggtgggccacatgaggcttttttaggcaatggcaaatggatcaacctggctgcactggatggctcccatggaggagctatggagacaaggtgaacaaaggtgaaaacaccagaccctaaggagtagcccctcaccctgaggcaatgccacaccccatcagggccaaagagctttttagaaagattaatccatttgtagtggatggaatggaacagggaaatggccaagtacgtaaaagaggctagagaagtctaggcaaaagaggatgccctgaaatcagagttctatgctgttctatttgccactctacaaccagtgtagatcccagggccaggcacagggtaggtgctctgtaaatattcagcaagtgagggaatggacatgggttctttaaaagatacataaggaagtatgaggagtcttggtgatttgggaatccatcttgctattcttcagagtctagcaataccctgcactgatgagaggtctcttgtattggtcttgaccaggctgacaggacatggacaaaagcgaagtaggattccaaccagggaatggctggagatgtgctggttgtctgaacacagggtgacttctcaggtaacatgcattttataagacaacaaagccacagtggtataatggaaagaaccatcaagggcaaggtggtataatagaaagaaaccatcaagggcaacgtggtgtaatggaaagaaccatattgacctcagtttttggtcctgcccttcaaataagtatgtatgtgacactgagccaataaggtgctttctacagctaatttttagcacagctatacatttctatgactctacattatctctcaaacaaatctaagcaagacccacaaggccaaaatccttagtatgtctgttccttgaaccttagctatttcacaaaaatataccctaacaccacagtatacatgggcagggctcacttgaggagtagactgcagtctgattcaagtccaagttgttccaggtccgtgattagtctcctgggtagcccacagccttggtagtgtcactttctacaattcattatgtaacaacaacaaattggtaaatgctgacaatatagttcatcattgcataaatatagattgtccttatatctgttctgatggagagtaaagctcaatgattctgctcattaatcttgttgagtgggggtacagatgggcaaagagaggtggatgcaagagcttgatttacttttacaatgacaggaaaaaaagaacgaatagcctatgggtctgttgtccaaccaaaagcatctgttaacattaaagatcacatacttcaagttaccttccagcaaaaaggaaacacagaacttgaacaagaagccagatgaccaaaatgtcccttaacttcttatagttttttcctataattagcacctgttcatgaaattggagaacatttcaaatctgggtagcttaagaatgaagcacataaaattaaatccttccggataaagactcacactatggtgactttgtcttggttattttgtttgcataacccgccttgggaaagtaaagcaggggcatattctagggctctaaatcaaattaacacctacaaaatgttgatgcccagttatatgctgtcaggcaattgcccaagactccagatagcaatgtccattcatgcccctgtaagaggtacctggatggaatgacttattttacaacttcattttcaaagttggttctccacatacttgtattccaagtaatataaaattaaaaacatatattaatctacattctcataacttaatcatcctttgagagaaaatacatcacacttggtactgtacagtaagatagattgttcatagaaaaaaattcaaatacatttcttttctactaaaatgtggtgggaaaaggacaacccatgctttgtggagacaggtctgcagtccacctgttcattatattcatattttcagtccaggagtctccctagtcacacagaaatgccaccagttggccttaaaacacacttgctagagagaggggaggcaaacagtcctcccaaatgatgctgcagcctcaaacaggcttatccattcatatcttctccaccacattcttattaggcatcaaacagtccctttaaataagaatggttttaataagatattaacaactaagtttcccatggaataagaatttctaacttagggtatctcagcacgtattcccagttacatatgccctacacaattgcttaagtggtaagcagtctgaaaaactctcctccctttacctctttgtgaatctacagcagtcttttaagattgttttgcaaatgctatattcaaaaagaggttttttttttttcaagtaaagtgcatggatttctcagaagttgctgtattttaagaagtgcctctttaaccccataatgagcaatccttatgttggtcagaagcaaagcagttttgtttgcaattgtaaatcttggctctcctagcccaaatctcacagccatcacccaggatctctgccccatatttccctggaaaatgtcctaagtcaaaacaacaacaacaacaacaacttcatctttagaaatagggtgccttcacaaatatgggtaagccaacagttcatcgaatactatagggaaagagagagagaacggggatgagacagcaaaaacattaagacttgttctcagcattgctctcctctcactgggcagtggctgaaaacaccagaaaagttgcattaataaaactgcatatagtctaacactgcacagagtgctttgatacaagtatcctcttgctacttcatcttttcaatacatctttgcaaggtttgttttcaaaaagacattacaagttggcaggcttctgcttataaaaatcaatgaaatactttcccttcaactctatgaaacctgccatatacctgagatttattcttctcaaataaatcaaacataggcaacgtaacactctggagtcaacacagaacatgccagggtgagttcaggcaatgaaagaaccacttttctgcaaatacatggtagaattgaagactgtttgtagctgtcgataatttgtaaaaacatttccaatgttctttgaacaaaagattttgattcagccaagattacagaaaggaatcatgacaaagtcctaagtgtacctttgtgtgtatttcatctgctcagcttttgcaggtgactgtggtggtggttgcctggatatggaattcctttgccctcaaatcttcacatgcatgaagtgcaataaagaataaaatgctgtgtttatgtcgcaccacttctaagaggtttaaagcgccgtacgaatgttaccacatgaatccccacaacacccctgtgaggtaggtaggtggagagtattgtcatccccactttacaggtgggagaaatgaggcacccaatagttaataagagatttgctcaaaatcacacagctagtcactggcagggcttagaataaaatgtatactgattagcacctagcacagtgctttgcacatagtaggtgttcgtttaatatctgtggattttatttgacttatgtctcaacatacaatatacacacataaagtacaagcagccaccgtaaaacatttttctgatgatatctctcattacttcaaatcctggtggaggaaggaggttcaagaatccatctcacaattaagacctcagggttgaagaggatcatcataaaaactatcagctgacaaccagctcttacacctgctctaccacacaatattattaatagttttctaatgaaaacaaaaatggatttcaggaaccatgctgacattattttttgcctgtttgttttcaatggagtcatctgaatggttctgtgttttgtttgtacaaaaaagaaataaggctgctatagtccagttagcatgtgaaaactctgccaagcacgaagatctcctcccagctcggatggattgctacctgggaaaatggaccgacccagggagtggcaggtcccaaggaagagggtcagtgaggctggacgtcacttgcactgttcgtggtctgtatagtcatccatgtccacatccgaatcaaagagtgagtgtccagtaaaatctgtgtctggggttctggaaaaactgttttctgctccctcatcttcaaaggtctctgtccttgagtaaaagctaaaatccagcagcggggtgtgggttttgctgccttcgctgctctcctcagactcatagatggtattgtcatcatcgtggtgccactctggccaaaatttcctccttatcctctcacagtacatggcaaggttgatcagctcacctttgatcagccgttcgggtcttgtccctggtaaggtccacattgcctgtgccaagtgtccaaagacagtggcgtcaagagtggaaagcttgggccccatgatgtacttcttatcacccaaaagccctgctaaagaccgcatgtccttctccatcagcatgtaaatctcttcctcggagaagcggccaatgccgtggccgtgcatctcgcgtttcacaattcctttcgttatgtggcacacaacccacctcagcaggttgctgaagggaccaccaccactaagagagagcatcttccgggtctcattgagattgtccacccactggcaataagctaatgtccagtagaagtgctcctccaccatcttggtcaccgctctggagatggctctttcatgagggccaaggtttttgtttaaattcactccaagcttctcttccagaaagtcaattatgaattctgtgccagaaactttttcatgattatattcaatccaaggcattttcccttgagcagagagttttccaccaaaatagttctgatacggtaagtcagccatccttaaataagtttccatctttaaacagaaaggagataaacttggaacaccattgttaggtcttgcaaactgatgcaaaataatagcatctttagagtcaatctcttgctgtttcctaatgaccaggagttcgtggagcagatacgcagctgcggccagcaaagctcccccggtcaagtaaagggttttcttccaccagggatcggagcccagccctgccatgatcccaccgtaatcctggggcggcgcggagctgcgggcaggagacgccaccaggc

SEQ ID NO: 15126 - RNA, 9729 nt, Homo sapiens
  source 1..9729: mol_type = other RNA
gctgggattacaggcatgagccactgcaccctgcctaattgagacaatatttatacaaggggaaattggtctattataaggcctagccatagtaaaggtctcaacatgtgctcccagctctccctctcctccttgtcttctctctaccagtggttctcacacttcgtaacactctgaggcacactgggcatgaaataaaagcaggagaggatgggacagcatattccagagatctgtttttcttcttaaaagccactcacttgaaattctatcaaagttatatgcctaaaaaattcattacctctgttttaattatacaagagccttacaactaaaatactctcccagtcatctaagagaccaccacttaacagtatattagatgcaaacatttcagattttccccatgagcctgaagtttaaacattcaaatttgcaaaagagaagtaaattggaagaaagacattcacagaaaactatttcatatccattagttatcatttacacatcaaatacatatagcattaagaccaaatatacagaatttccacatttatatacagtagtcaacatagtgcacaattcaaatctatcttacaatcaagtgtacaagtttaaatatggctttataaactactaataactctgctaaagtaactcatagatccagaaataaacactgaaatgccatcttcacattggggtcatcattcagcaagatgctaatcattgtgattgcaaaacagagggtgcaggtaagtgtttccaggtggtgtccgcccattagccccgaaatgtgggttcaaattatgccaacattggcccttcctatctcagatacctaaaaataagtctgcacatcttccacacatttgaagacacaagattataaacaaatagaaaaaaagacatgtaatcagtgagatgatgaattatcaggcattatcaaaacatgtttttcagattgatgctgaaattcacagacaatacatcctgcatttgcattatctgggtatcacctcacccctactttcttttcttgttttgcttacctcagtgtgttgttaaatctttctggaattttcaaggcattctagatcaagtggtcccaaaagcagaattaaaaacatcagtcttaaaggtgacatcaaattgttcatccttctctttcccaaccaaaaatgcctattttaagtaaaaataattaaataccttgacctaaaatcatgcgtccatgcctgttttatatctgctttgccacaaatggtatatacacattctctaatcaattacaggcatctgggtgctacgcctaaagactccttgtcccattctctaaactccattgaggaccagaaaatatacttttaaaatgtctatgtttgctatggtttttaatgtttacatcagtaaaacagtatatacatatatagcagtgtatacatatatacatatatatcataaataaatacatggaggggcatgctcagaaagttttactaatagggtgaataaacataaacgtttggagaccactgcctaaatagggatggacgatctgggctgtctgcaaacatttaaaagacttctctaaaacaaaatgtacattactttgtacaattttatatttataaaatgaaaaatatatgccacaaacactcttgagagactagaaggaaattccaaaattaaaggagtaaatgtatcagggccagaccctctaagctgctatctaaggtcccaggcctggcttcagaaggggaatgggggacatgagcatagaaattaagataaagataaatgttacttcacttcctgcactggccacttgtatatccatagacaatccttccctacatagattgcacttgtttttgatttataaacctgtactttttattattttagcaagatggcaccacctagaaaactttcaattgcctgatacatctctaccacagccataccacatggttgcttgaaattttgacatttgttactgttttcttctctcctcctactcagttaaattctaataccaccaaatgagggactcagaccctcagttttccaaacttcaccatggaaaaaccatcgctgtcatcaacatttgagttgtcagacatttggcatgatgtagatcactgggaaaaaaacatgtgtttacaataagcttgttctgatcccacaagacttattacttgcaataaaatcattttgacaggagtaacattaaaatcattttacaggagtaaacatgtcacccctactgaagcagaagcctttagccttatttctgtaaaaaacaaatcccaggcataatttgttaaagataaaaatacaatcatttggacatggtttatattttaataagccaaatataatctcttgtagaagagaagcaaatacgaaagaacatttctgattctgaacaatggaagaggaaagtcattgattattttttaaagaggaggaagacagtaaatattcagagcattcctcttttttagccctcaatgaacaattatattatattccctttgctatctgtttagccaccattaactaacatggcaattcagaagttggatcttatttttttagaagccatggggtaactaaaaacaaaaaaggtattaaataaggaaaaaagcttaagcattactaataagtgaaagttactctattccagagccacaaataaaaacaaataaataaaaataaatgcatgccaatggggggtgggaggtgaattagtcacatttagtagcacaactttttataaagttaactgattatgatacacatatattgctttatggttagtggattgtttcaaaaatgcatgatggccattaaattctttgctaaaattattgtgtacagaacaccaaagtaccgtatccatcttttactccagattacttgttttcctactgaaatggtcagtttggtgctgctagaccatatctgtaggttattcgttttattattgcaatggtcccctttatttgtctaccaattttacaatttaaggcaatcatccttatgaaatttgagcatcctagtttgtcatggtccagccaatagcaggagttttagagggtctaggtctggggacaagttccttgcttcggcgaaagcagaatggttgaggaggtcaccctgtcagctccaaaacagctgaaccccttttttttaaatctatgcttcagtgccctctgtaatcatctctaactggcaaggctaacgttgctggttccagcagtctcatctcaaagattaaggaaacttaaatatccttaagatattcttgaaagtcagggaccaaaaatctgagtttctgggtaaggaattcagatgaggaaaacatgccacagatgttcgcatccacgcctgacagtagcaagagtcttacaggtaagaggcccgtccctcctcacccaacaagggaatccttttgaacttcccaagttatatccagaccactggaagcaactgaataaaggtcaagcacttcacaatcacatgcaattgatccctggacctgttaaagatgggttcccagagcccagcatttagcctgggaagtattcgtcattgagtgtacttttatcagttctagtttgacttaaatagcactgcatataaaggagaacaaaggatcctgggtcatagtcaggaacaataaaataacatactctgtttaaaaaaaaaaaaaaccctaaaagaaagaaagaagaataacctgagttgttccctatcaacaaaagccaccaaccttttattgaaaatacactcaacaattgttctatgaatgaatgaataaatgaatacaggaaaacctgattgtgcagacctttcttctttaaggaagaaaaatccagcctcttctctcccaccttcagcccaggctggttgccctatccatgcagaagcggtgggtttcagggctgaaaggaagcgcacttggccctgaactcattttgataaatcaattttgggggtggttaaaagataaatgacaaggacaacaacaaaatcctatgactttcaaaattccaaacctctaaaacaaaattttctcaaataacctaagagcacttctttcttcttttctgtcactcaagacatactgaacatggataatagagattacttttgcttgcatagcctgtactaatttttcttctctctggctgtgttaaaaacaagaacaaacacaatgataacatttaaagactcttgggaacaagactctttaactggggtccattaaccccctgaggaaaccatggataatttcaggaggtctctaaatttcctgaatttatatgtaacattttatgtatttgcatatatgtgtttttctgggaatagggtatagaactttcgttggattatcagtggagttcctgacaaacaaaaagtgaaaattcactatttaatggtatgtgactcactctctgagcatctttcccatgcaaccttcagggaaggaagtgatgagtgcttcattttcaaaggaagagattataatcagctgggaagccttcatgtgaagctgacgaagtcagaccttgagagatgggcatgacttgggccagtggagcagagaatagaacatttcaggagaaggactggcatgagcagaggcacagaggtgggccacatgaggcttttttaggcaatggcaaatggatcaacctggctgcactggatggctcccatggaggagctatggagacaaggtgaacaaaggtgaaaacaccagaccctaaggagtagcccctcaccctgaggcaatgccacaccccatcagggccaaagagctttttagaaagattaatccatttgtagtggatggaatggaacagggaaatggccaagtacgtaaaagaggctagagaagtctaggcaaaagaggatgccctgaaatcagagttctatgctgttctatttgccactctacaaccagtgtagatcccagggccaggcacagggtaggtgctctgtaaatattcagcaagtgagggaatggacatgggttctttaaaagatacataaggaagtatgaggagtcttggtgatttgggaatccatcttgctattcttcagagtctagcaataccctgcactgatgagaggtctcttgtattggtcttgaccaggctgacaggacatggacaaaagcgaagtaggattccaaccagggaatggctggagatgtgctggttgtctgaacacagggtgacttctcaggtaacatgcattttataagacaacaaagccacagtggtataatggaaagaaccatcaagggcaaggtggtataatagaaagaaaccatcaagggcaacgtggtgtaatggaaagaaccatattgacctcagtttttggtcctgcccttcaaataagtatgtatgtgacactgagccaataaggtgctttctacagctaatttttagcacagctatacatttctatgactctacattatctctcaaacaaatctaagcaagacccacaaggccaaaatccttagtatgtctgttccttgaaccttagctatttcacaaaaatataccctaacaccacagtatacatgggcagggctcacttgaggagtagactgcagtctgattcaagtccaagttgttccaggtccgtgattagtctcctgggtagcccacagccttggtagtgtcactttctacaattcattatgtaacaacaacaaattggtaaatgctgacaatatagttcatcattgcataaatatagattgtccttatatctgttctgatggagagtaaagctcaatgattctgctcattaatcttgttgagtgggggtacagatgggcaaagagaggtggatgcaagagcttgatttacttttacaatgacaggaaaaaaagaacgaatagcctatgggtctgttgtccaaccaaaagcatctgttaacattaaagatcacatacttcaagttaccttccagcaaaaaggaaacacagaacttgaacaagaagccagatgaccaaaatgtcccttaacttcttatagttttttcctataattagcacctgttcatgaaattggagaacatttcaaatctgggtagcttaagaatgaagcacataaaattaaatccttccggataaagactcacactatggtgactttgtcttggttattttgtttgcataacccgccttgggaaagtaaagcaggggcatattctagggctctaaatcaaattaacacctacaaaatgttgatgcccagttatatgctgtcaggcaattgcccaagactccagatagcaatgtccattcatgcccctgtaagaggtacctggatggaatgacttattttacaacttcattttcaaagttggttctccacatacttgtattccaagtaatataaaattaaaaacatatattaatctacattctcataacttaatcatcctttgagagaaaatacatcacacttggtactgtacagtaagatagattgttcatagaaaaaaattcaaatacatttcttttctactaaaatgtggtgggaaaaggacaacccatgctttgtggagacaggtctgcagtccacctgttcattatattcatattttcagtccaggagtctccctagtcacacagaaatgccaccagttggccttaaaacacacttgctagagagaggggaggcaaacagtcctcccaaatgatgctgcagcctcaaacaggcttatccattcatatcttctccaccacattcttattaggcatcaaacagtccctttaaataagaatggttttaataagatattaacaactaagtttcccatggaataagaatttctaacttagggtatctcagcacgtattcccagttacatatgccctacacaattgcttaagtggtaagcagtctgaaaaactctcctccctttacctctttgtgaatctacagcagtcttttaagattgttttgcaaatgctatattcaaaaagaggttttttttttttcaagtaaagtgcatggatttctcagaagttgctgtattttaagaagtgcctctttaaccccataatgagcaatccttatgttggtcagaagcaaagcagttttgtttgcaattgtaaatcttggctctcctagcccaaatctcacagccatcacccaggatctctgccccatatttccctggaaaatgtcctaagtcaaaacaacaacaacaacaacaacttcatctttagaaatagggtgccttcacaaatatgggtaagccaacagttcatcgaatactatagggaaagagagagagaacggggatgagacagcaaaaacattaagacttgttctcagcattgctctcctctcactgggcagtggctgaaaacaccagaaaagttgcattaataaaactgcatatagtctaacactgcacagagtgctttgatacaagtatcctcttgctacttcatcttttcaatacatctttgcaaggtttgttttcaaaaagacattacaagttggcaggcttctgcttataaaaatcaatgaaatactttcccttcaactctatgaaacctgccatatacctgagatttattcttctcaaataaatcaaacataggcaacgtaacactctggagtcaacacagaacatgccagggtgagttcaggcaatgaaagaaccacttttctgcaaatacatggtagaattgaagactgtttgtagctgtcgataatttgtaaaaacatttccaatgttctttgaacaaaagattttgattcagccaagattacagaaaggaatcatgacaaagtcctaagtgtacctttgtgtgtatttcatctgctcagcttttgcaggtgactgtggtggtggttgcctggatatggaattcctttgccctcaaatcttcacatgcatgaagtgcaataaagaataaaatgctgtgtttatgtcgcaccacttctaagaggtttaaagcgccgtacgaatgttaccacatgaatccccacaacacccctgtgaggtaggtaggtggagagtattgtcatccccactttacaggtgggagaaatgaggcacccaatagttaataagagatttgctcaaaatcacacagctagtcactggcagggcttagaataaaatgtatactgattagcacctagcacagtgctttgcacatagtaggtgttcgtttaatatctgtggattttatttgacttatgtctcaacatacaatatacacacataaagtacaagcagccaccgtaaaacatttttctgatgatatctctcattacttcaaatcctggtggaggaaggaggttcaagaatccatctcacaattaagacctcagggttgaagaggatcatcataaaaactatcagctgacaaccagctcttacacctgctctaccacacaatattattaatagttttctaatgaaaacaaaaatggatttcaggaaccatgctgacattattttttgcctgtttgttttcaatggagtcatctgaatggttctgtgttttgtttgtacaaaaaagaaataaggctgctatagtccagttagcatgtgaaaactctgccaagcacgaagatctcctcccagctcggatggattgctacctgggaaaatggaccgacccagggagtggcaggtcccaaggaagagggtcagtgaggctggacgtcacttgcactgttcgtggtctgtatagtcatccatgtccacatccgaatcaaagagtgagtgtccagtaaaatctgtgtctggggttctggaaaaactgttttctgctccctcatcttcaaaggtctctgtccttgagtaaaagctaaaatccagcagcggggtgtgggttttgctgccttcgctgctctcctcagactcatagatggtattgtcatcatcgtggtgccactctggccaaaatttcctccttatcctctcacagtacatggcaaggttgatcagctcacctttgatcagccgttcgggtcttgtccctggtaaggtccacattgcctgtgccaagtgtccaaagacagtggcgtcaagagtggaaagcttgggccccatgatgtacttcttatcacccaaaagccctgctaaagaccgcatgtccttctccatcagcatgtaaatctcttcctcggagaagcggccaatgccgtggccgtgcatctcgcgtttcacaattcctttcgttatgtggcacacaacccacctcagcaggttgctgaagggaccaccaccactaagagagagcatcttccgggtctcattgagattgtccacccactggcaataagctaatgtccagtagaagtgctcctccaccatcttggtcaccgctctggagatggctctttcatgagggccaaggtttttgtttaaattcactccaagcttctcttccagaaagtcaattatgaattctgtgccagaaactttttcatgattatattcaatccaaggcattttcccttgagcagagagttttccaccaaaatagttctgatacggtaagtcagccatccttaaataagtttccatctttaaacagaaaggagataaacttggaacaccattgttaggtcttgcaaactgatgcaaaataatagcatctttagagtcaatctcttgctgtttcctggggcggcgcggagctgcgggcaggagacgccaccaggc

SEQ ID NO: 15127 - RNA, 464 nt, Homo sapiens
  source 1..464: mol_type = other RNA
gctgggattacaggcatgagccactgcacccttttgtcagcatgccaggcttctggattccctttccctgagcggccccagtgatccagcttgcagcaccattgccctgggggccaagccaaagttgtccaatcagtgctccagtctatttcctttgcgtcggagggtctcctcagtattgtcccttttgtggttcgagagaaagatgttaccagaccccaccacttacccaaagttagcttttgttggatcaggggtttccgaagtatagtcacttctgtcattgccagaaagatgttacaggaccccaacatttacccaaaggtagccattgagtcagggttttctcactatagtcccttcatgatctccaggaagatgttacaggacaggggtcctgatccagactccaagagagggttcttggatctcacgcaagaaagaattcagggcaagtccacagt

SEQ ID NO: 15128 - RNA, 2429 nt, Homo sapiens
  source 1..2429: mol_type = other RNA
gctgggattacaggcatgagccactgcacctagccacatcccataaatttcggtatgttgtgtttccattttcatttgtcttaagatatttctgatttcttctttgacccattggttgttcaggagtgttaattccacatacttgcaaattttccaagttttctcctgttaattatttccagtttcataccagtgtgtgaaacctttccttgatgtagtaatagatataaatacacacatatgtataggtttccatctatgattcctggctcataactcccagagtccttgttacagtcttttgttacaatgttggtatgttaggcctctctgactttctccagtgttcctttcacctgccccaaggcaggtctgtaatctgattgtgggtcataagaccaccattccagagagggtcccatcccataccctgggggaaggaatgctaacgtcacgaagcttctataaaaagccaggatgactggatttagagagcttctggatagctgaacacatgcaagttcctggagggcagctcgcccagggagggcatgggagttctgtgccccttcccccatacctcaccctgagcatctcttcatctgtatcctttgtaataaaataaattggtaaacatgtttccctgagttctgtgagtcactatagccaattaattgaaccccaagagggattgtgggaaccccaacttgaagccagttgtcagaagttccagaggccccagacctgtgactggtgtctagcagtgttgggagagggaaagaggacaatctttggggggctgagcccttaccctgtgggatcagacactatttccaggtagatagtgttggaattgaattggaagacatccagtcagtgtttgttgccaaactgattgcttgcttgttgctagggagaaatccccacatagtttggggtcacagaagtcttctgtgctgattgatggttcttgtgcttcaaactctcaggctcaagggatcctccttcctcagccttctgagtagccagggccacaggtacacgccaccacacccaaactgagaatatgcctgagacctcagggaagaaaggggacaagggaagagcacactaggtgagtggcagcatcgagcaggatgtggaacagacatcatgagcctgggcattaatcagtatgtgtcagaacagaaagctatactgaaaaaaataaattttattaaataaatctgtatttttgaaatttgaattttcttttttgtagtttgtttaacttccttttggaatccataatgttttaataaaactcactttgaaaaaaatctcaaatacactaacaagggaaatacattttgttatttacaaatatgggccagggagaaatgtgagacagtgtaacttggggccaggcacagagttattcatttattcaataaatatttactgaatgcctactatgtgccaggcattatgctaagatgctggggatatacctagtaatgaagaaggaagaaattgtctctgcctacatgtaactaaaagtccttgggagaagaaagatagtgaaaaataaatccaaatgcgatgtgttatgaaagaggaagtataaagtgccatgagtatgagtggaaagagcagttaaaggtgagcagaggagcagctctcagtggaaagaaatcaaaagctaagataaaaaccagtaacactctggatgggtgggaatagattgaaatccataaagccaaagagatttgaattacttgacttcaaataggttgaatatttcagtaaggtaaggactctattctttttctttctcggcctttgtccagagagtgggaaaagtttgaaagatttggtctgaatccaggttttaaaaattatttttatggattgattaatattgttatgcacaacaggactacagaatgtaggagatggggtaactgtccccaaaagaggtcatagccttgttggagagacaacatataaacatagaaaaaaataaaagaggtctcttaggagactataaatgattaaagccttaatgaaggcagaggaagaagtttctatgggcacaaataataagtaatgatgtcttgctagagatgtcctattttagaacttattggtgaattatgacattctaagataggcctaagtgtacaagacttaggtctaaaattaggcattagaaactgcctccctgtttggcctggctgatggcagaggaaggttcagaaatacaggggagattcagtagccaaagatgggttcatctatagctatgatgagataaacagtttacaccaagattatacattctggtgtctagaagggggatcttcgtgtattcatccattctcacactgctataaagatactacctgagactaagtaatttataaagaaaagaggttaattgactcaca

SEQ ID NO: 15129 - RNA, 7885 nt, Homo sapiens
  source 1..7885: mol_type = other RNA
gctgggattacaggcatgagccactgcacctagccaggcatattggttttaaaagggttacaagaaacaagatgcacttttaggcctcctataatcctgcatttccaaagcatccatttagtcatctcatcaaaattttcattgatttaaataagttaatatgaacagactgacataattttactttaatgatgttgtttattgtcctaagccatccatacacaaaacgtttaatgtgttatggaaggctaacagtttttcagcttttctcaatactttcagccatccatacataaaatgtttaatgtgttatggaaggctaacagtttttcaacttttctcaatactatcagatgaatgtattcttaccaatcatgatttacgtttttcaaatgtggatttcttaggcctttgactgatagctttaggcttttgcactacacaaagaaaaagacacctttctattcatttcttaataatttgtttccataaagctaaaatgtccactgatgacataatctacctttggttaatcacagcaaatagttcacattttaaaggaatgcagatatttggatagaagcctctaacaatgtaaatattgtgcatttcaagttccatagtgtgtctaaccagggatagcaactgattatatgtggattaacaatagtgaataactgagcacatattaacatgaataacatacacagcagtcaaaacttactgtttttcatatgtgtaaagtaaaaattcaatctatctttaaccggctcatactgttttcatgttgttcaactatttgacacaaaaggagctttttcctttctttaaaaggattttgattcagtcataacagatttttgaaagtgacagtaaaattatgcatttggtccaggattaagagggaagttttgcttgctagtgtctatctggttagacatcagaataaaatgaatggactgtaaaggatcttataaccagtctctctctttaatatgaaggcccaacattacataattctttttaagagttgaccaggaatgaaatgtaacctcttttaaagatgaagaaaaactgaaaaaatgagattaagaaaatatgtgggtagtttacagctgctgatagaattgtgtgcacgcgtgcatgcatgcataaacacaaagtgaatctagaagggaaaaaattgagtttgatgaagtctaagatgaaaggttccatttcatgtaagattatgtgaccttggaaaaatttactggcttgctagtggaatacgtccttatatagggacttgaagagtttatctaaatagactgacttaaggatgcttttcctcttgttagacttgtatgacattactgagaagatttagagttctagaagtagagaagactgattagcttgtgcctgtgtatgaagaatgacaaattaagacaaaaggttatgtaaaccatttactaaaaaagtctaaatttttatattcctaggcccctacttatcttttacaaactttgaaggacctgaaattctttggacaccatcagatttagtttataagagttctgattttgaatcaagaaattattcatgtagttttaaaacacaattaaaattttcagtcaggctgaacttttgtgcacttcctcatttattcgagaaaccccaccactaatgtatttagaccttaatatgatggctttgagtcttaaatcattgtccacctaaaataatataccaaataaagatttttaaagtgctgcatatggtttctgtaagaggtacataattagattaccagcattatcctttagcttcaaaagtaaaactcatagtcaggattttactgatagtacaggaagaaaaaaaataaccactgttgaaaaataaatgaaaaaaattttattgagtattactttatacatgcaaattgaaagtgaatctatattaagttgactattccacaataaaaacctatgaaatgggaatgatcaaagctgtctaacacaatactaatgtgttcaataaattatccagatgtttttccacaaatatttggattacctgaattagctgattcttcagcaaaagttaaattttagctttaatatggtagcagcaggatgctacttaaatttagaagaaaaacataagaataaaaaccctgaatagcatagccaaatcttccaagaaataagttcaccaaaaaagtagcatacacctatttggtatccagaggaggaaacaaaacacaggcacttaatcaacatccaccaagtgatcatcactaacattctattattaccagagtaactgtcgatatgtgaactgtagattagaacagacttacatatctaaaaacaaaccagtaatcaataatatatacagaaatactaacttgaagtcacatttaaataccatcaacagtttggtgtatctgatataactgaattcatttcatcactgctataaattccttaaaagtgttcttttcctaattaacattatctttaaaaaatggtagatatttcccagtatgcatcagttttttcactccaccattcagtaaatgttgtagcaaattaaatagaacctattaactagatctaaaaacagtggctgaatacttaacacaaagaagtacttttgagtaaactattcagattagacaggctaatgctaagactgcattttgtgctactgacatgcactatatagatcgtacactactagatggaaagttggtccatgtccatttatttaaagattctgtaacacctgtaatagtatttaatacagctcccacatactatattcctctcacatagacatagttatttttagtggggataaggatatgactttaacatgctatgagattctagctaagtaaaataaaaacaatatggactcagattttcttaggagatattagttcaagtttttaaactgggaaacaatcaacttccatatatccaggagaaacttagcatggggggaggtgccttagttgatgtgcctgataagcaaactgttagttgtctattagtattatgttttcggcttaatgtaacaacaaaagaaagttgtcacactacctctcagataatatcaattacaatcttagagactgtaattgggaatacaatcctataacaagttattaacaatatcatgaatagttattaagtaagtgccagcactacatgcaacttactggtcaccaactcagaacccataaaactatacacatatgcacaaaaaaaaaactccaaagaaagatacctatcactgtacatatgaatactgtccaggatatcagatcaattatcaaatccaaggtctctgctgttttgtcttacagtgttgaatatatgaatgcttctctattacactgacttgtactattttcaagaaattaagtggattcaaaatcttacatttttatttctaattataaaatccagattaatccaaaaaacacaaaccacatgtaaccgaggtaggtttttcaccttaagaatacattgcttctaccacaattaaaaattttttaaactgaagaaaaaaaaaaactacattgctccacatacctgatacttaattttctatgtttgaaactacttgaacaagtgtgacagtgctaatctactatatttagtaaatcccttagtacctataaatacacacccaaaagcccttccctccttctctaatggtaactgttgtataataaaattgtcaacaactctagaaagatgaaataaagattactatagcaatcttcaattaattcatttcagaaatcaaggaggcaagtcatgttcattttaaagatgacaaacttactattttgaaaatgagctcataaatacattagaactttgaatgtgctttattatgccacaaattcccaggagatttaagaaatagtatttctgaacaggaataataatttcacaaatactaacactttattgacaatagacaagtcttttagggtagtgcacatgtacttaaaaactaccttctaccaatctcaacactttttataaattttcaggtgaaactgtagcagatcctactttatttttcaatggttagtgtaaaattctgtatgtaaaataagtacatattttgagatggaagaaggactgcatgtgaaatgctttgcctaagttgtaaggctcctgtctttacgctatcattaaaggccaaaaaaatcactgctagaaatgttccccaaaaaattcttaaacagctcagtctttaaaagtattaataatttttttttttttttttttggagacagagtttcgctcttcttgcccaggctggagtacaatggcgcaatctcagctcaccgcaacctctgtctcctgggttttcaagcgattctcctgcctcagcctcctgagtagccaggattacaggcatgcgccaccacacctggctaattttgtatttttagtagagacggggtttctccatgttggtcaagctggtctcaaactcccgaactctggtaatccacccgccttggcctcccaaagtgctgggattacaggcatgagccactgcacccagcctaataactgatataatttttttaagtgaaatgaaatgttcctttatttacatatgaattaaatagaaaattcaaagtaattcttttaataaaaacccatatactaatatattttaaggttggatactaacagcattttcacaagatccaaagtgtggatgacgaactaggcaataaggacatgtgtgccacataactaagggtaactaaaggaagatgagtacctcacaaccaaaagcagttaactatgcctggcataccaccctgtcatgtgggcagatcactgttcccatgctgggtaagagtctccaagaagggaagcccttatgcagtaattctgtaactatattaaatttggtaatctaacattaaactttttcgtgagcagtgaatatacacatggtcatatgaaaactgccctggagaccgggttaattattaaataaactaaaaggggagaaatgctgatagataaaattatgtcaattccagggtgttcaatggaataaagaaacagcagcagctgcttcaaaagtagactatgatcagaaacctcagatggtaacctttaaaaattgtggaatccagagtctcaacctaaacctacataggagctacagccagggagttctttctaagttcctcaagtgattctgatgattggccaagctggaaacttctgaactgggggagaaagccaacctaggtaaatgtagagacttttagaattcaacatttgattatcatttactccacattttcccccagctgtctcaccttctctatttttctaacagtgaacaataaaagggcttggcaagtgaaggaaaaagtcagtagagtacctaaaatggatttgactatattcaagccactttcatatattaactagataaaaggataccatactgctatttgaaattcaatcacaaagcaaaaatgtcataattttaatgtattttaagggaagacggggttcttaacatgaatatgtaatacaaaaacaattctaaataataatatttaatagaagaaaaaatctgtataattatttagaagtaactctgtttttaaaatttcaatgttaggaagaaaatcccttaaatttgaaatagcggaatattctctcatatgaaaaaactgtgtcccagtgttattcttcaacttagaaattaggcaaagtattttagtactatttctgcttacatattgttttgtatgaatgttttaagtatgaataatattttggtttttagtgtgcatgctaatataaaaatatggatttttttctcctacactgactttgtacactttccaggcccgaagaataaaaaacttttaaaatatcctgtgttcactagcaaaccttggaacgataaaaaaaggtagtacctacataagaaattttacattgaaattacaattgtatgtttttcaggagttaaagtgattcaatttttcaatattcaaacacaaaatagtaaatttttatttactatagcacaattcaagtattctcttaaatttatatttagtcaactaaaacatgacagtgactttataagagctttccttttaaaaggttgctgttataaaaaagtatgactctattactctaaatgcttagaataagtggaaagaacaaatgacagtagacaaaaacctttatgagtgagtcatcaacacataaaaggttgcacacatcagtaataggacatgtgaaggtaacatcccaaaagtatttgaactcatgtaaacaaagactatgtatattcctaagggagaaaatgtactaccaagataaaatatattcaaacggctgtgactttaaaccatgtattagttgaataccacacaaaaccaaaaaggcattatctatcatttaataactgaaagatattacttatttgtgagataaaaggataatgcttttttaaaaccaataatgaaaaagaagtattttgaaaacaaacatctgtttgctagaaataaatatacttgcttagttattttaatgtattgcagcataggaatattgtgctagcattgaccattaacattcaatcagtagtttaaaatattttttccacattgagtcttgaatcctctacctggtcagctgacccacaactttcaaaagagttttattttcctgctttagctgttcattttcatcttctatgtcatctaggtctctatttaataaatcaatttcttctttgagttttccaatcatttcctctttatcttgcatcagtctcacaagtcttaggttttcttgtctttctcttactacttccttttcaagatcttcaattttcttttccagtgtgctacttgaaaccagagtacctgaaacatttgcatccctgttatatctagggaacccacttctatctgttcgagaatatctacttgagacatcttcttcagagacactggttgtgcttttatatctgcctgaaactgttctaggtggctcctgtagcagataggaactgcctggatctagtaagtttacagcttcattctgaatagtgttctgttgtgtaattgcatcttctcgtttccgctctttctgccctgcttcatcatcttcgtactcatctaagcactctgcggcagggatgttgaccacgccggtggagcgccgcttctcccgcagcttcctcttctcgatctgccccttgcctttcctggcactggggcccgagctcttgcccttctctgggacgccgtccggctcctcctcgtcacgctggggcggcggtgcagccgaggcagaggcggctgggggctcgtcctccgaccgccgcgggccgggggccgcccgcgtcagcatggcggagccgaccgcgcagttcacgcccccgggaccggggacggcaggtgcggccggcgcgccgcccgggaggttgttgttgagctcgttggcagcggcggccgccggggtgcccagagcccccgcggggggcttcccagcggcgtcgctgctgccccctcccgggggggccgggcccggggggttctgcttggcgcgcatcttctcgcgtttcgccttccactcctccaggaagtctgtggtgctgccgccgaggccgctgctggtccggtagccaccggtcgccatattcccaaaggggccggtcgggctctcacctcaggccgcccaccagggctccggccgctgcctcctcttccttcctgcggccccgaggatgccaggagacgacctccaggagagggacggccgccgctcccacagcagccggcggggctacagtacggaccccgacgatcgcc

SEQ ID NO: 15130 - RNA, 7952 nt, Homo sapiens
  source 1..7952: mol_type = other RNA
gctgggattacaggcatgagccactgcacctagccaggcatattggttttaaaagggttacaagaaacaagatgcacttttaggcctcctataatcctgcatttccaaagcatccatttagtcatctcatcaaaattttcattgatttaaataagttaatatgaacagactgacataattttactttaatgatgttgtttattgtcctaagccatccatacacaaaacgtttaatgtgttatggaaggctaacagtttttcagcttttctcaatactttcagccatccatacataaaatgtttaatgtgttatggaaggctaacagtttttcaacttttctcaatactatcagatgaatgtattcttaccaatcatgatttacgtttttcaaatgtggatttcttaggcctttgactgatagctttaggcttttgcactacacaaagaaaaagacacctttctattcatttcttaataatttgtttccataaagctaaaatgtccactgatgacataatctacctttggttaatcacagcaaatagttcacattttaaaggaatgcagatatttggatagaagcctctaacaatgtaaatattgtgcatttcaagttccatagtgtgtctaaccagggatagcaactgattatatgtggattaacaatagtgaataactgagcacatattaacatgaataacatacacagcagtcaaaacttactgtttttcatatgtgtaaagtaaaaattcaatctatctttaaccggctcatactgttttcatgttgttcaactatttgacacaaaaggagctttttcctttctttaaaaggattttgattcagtcataacagatttttgaaagtgacagtaaaattatgcatttggtccaggattaagagggaagttttgcttgctagtgtctatctggttagacatcagaataaaatgaatggactgtaaaggatcttataaccagtctctctctttaatatgaaggcccaacattacataattctttttaagagttgaccaggaatgaaatgtaacctcttttaaagatgaagaaaaactgaaaaaatgagattaagaaaatatgtgggtagtttacagctgctgatagaattgtgtgcacgcgtgcatgcatgcataaacacaaagtgaatctagaagggaaaaaattgagtttgatgaagtctaagatgaaaggttccatttcatgtaagattatgtgaccttggaaaaatttactggcttgctagtggaatacgtccttatatagggacttgaagagtttatctaaatagactgacttaaggatgcttttcctcttgttagacttgtatgacattactgagaagatttagagttctagaagtagagaagactgattagcttgtgcctgtgtatgaagaatgacaaattaagacaaaaggttatgtaaaccatttactaaaaaagtctaaatttttatattcctaggcccctacttatcttttacaaactttgaaggacctgaaattctttggacaccatcagatttagtttataagagttctgattttgaatcaagaaattattcatgtagttttaaaacacaattaaaattttcagtcaggctgaacttttgtgcacttcctcatttattcgagaaaccccaccactaatgtatttagaccttaatatgatggctttgagtcttaaatcattgtccacctaaaataatataccaaataaagatttttaaagtgctgcatatggtttctgtaagaggtacataattagattaccagcattatcctttagcttcaaaagtaaaactcatagtcaggattttactgatagtacaggaagaaaaaaaataaccactgttgaaaaataaatgaaaaaaattttattgagtattactttatacatgcaaattgaaagtgaatctatattaagttgactattccacaataaaaacctatgaaatgggaatgatcaaagctgtctaacacaatactaatgtgttcaataaattatccagatgtttttccacaaatatttggattacctgaattagctgattcttcagcaaaagttaaattttagctttaatatggtagcagcaggatgctacttaaatttagaagaaaaacataagaataaaaaccctgaatagcatagccaaatcttccaagaaataagttcaccaaaaaagtagcatacacctatttggtatccagaggaggaaacaaaacacaggcacttaatcaacatccaccaagtgatcatcactaacattctattattaccagagtaactgtcgatatgtgaactgtagattagaacagacttacatatctaaaaacaaaccagtaatcaataatatatacagaaatactaacttgaagtcacatttaaataccatcaacagtttggtgtatctgatataactgaattcatttcatcactgctataaattccttaaaagtgttcttttcctaattaacattatctttaaaaaatggtagatatttcccagtatgcatcagttttttcactccaccattcagtaaatgttgtagcaaattaaatagaacctattaactagatctaaaaacagtggctgaatacttaacacaaagaagtacttttgagtaaactattcagattagacaggctaatgctaagactgcattttgtgctactgacatgcactatatagatcgtacactactagatggaaagttggtccatgtccatttatttaaagattctgtaacacctgtaatagtatttaatacagctcccacatactatattcctctcacatagacatagttatttttagtggggataaggatatgactttaacatgctatgagattctagctaagtaaaataaaaacaatatggactcagattttcttaggagatattagttcaagtttttaaactgggaaacaatcaacttccatatatccaggagaaacttagcatggggggaggtgccttagttgatgtgcctgataagcaaactgttagttgtctattagtattatgttttcggcttaatgtaacaacaaaagaaagttgtcacactacctctcagataatatcaattacaatcttagagactgtaattgggaatacaatcctataacaagttattaacaatatcatgaatagttattaagtaagtgccagcactacatgcaacttactggtcaccaactcagaacccataaaactatacacatatgcacaaaaaaaaaactccaaagaaagatacctatcactgtacatatgaatactgtccaggatatcagatcaattatcaaatccaaggtctctgctgttttgtcttacagtgttgaatatatgaatgcttctctattacactgacttgtactattttcaagaaattaagtggattcaaaatcttacatttttatttctaattataaaatccagattaatccaaaaaacacaaaccacatgtaaccgaggtaggtttttcaccttaagaatacattgcttctaccacaattaaaaattttttaaactgaagaaaaaaaaaaactacattgctccacatacctgatacttaattttctatgtttgaaactacttgaacaagtgtgacagtgctaatctactatatttagtaaatcccttagtacctataaatacacacccaaaagcccttccctccttctctaatggtaactgttgtataataaaattgtcaacaactctagaaagatgaaataaagattactatagcaatcttcaattaattcatttcagaaatcaaggaggcaagtcatgttcattttaaagatgacaaacttactattttgaaaatgagctcataaatacattagaactttgaatgtgctttattatgccacaaattcccaggagatttaagaaatagtatttctgaacaggaataataatttcacaaatactaacactttattgacaatagacaagtcttttagggtagtgcacatgtacttaaaaactaccttctaccaatctcaacactttttataaattttcaggtgaaactgtagcagatcctactttatttttcaatggttagtgtaaaattctgtatgtaaaataagtacatattttgagatggaagaaggactgcatgtgaaatgctttgcctaagttgtaaggctcctgtctttacgctatcattaaaggccaaaaaaatcactgctagaaatgttccccaaaaaattcttaaacagctcagtctttaaaagtattaataatttttttttttttttttttggagacagagtttcgctcttcttgcccaggctggagtacaatggcgcaatctcagctcaccgcaacctctgtctcctgggttttcaagcgattctcctgcctcagcctcctgagtagccaggattacaggcatgcgccaccacacctggctaattttgtatttttagtagagacggggtttctccatgttggtcaagctggtctcaaactcccgaactctggtaatccacccgccttggcctcccaaagtgctgggattacaggcatgagccactgcacccagcctaataactgatataatttttttaagtgaaatgaaatgttcctttatttacatatgaattaaatagaaaattcaaagtaattcttttaataaaaacccatatactaatatattttaaggttggatactaacagcattttcacaagatccaaagtgtggatgacgaactaggcaataaggacatgtgtgccacataactaagggtaactaaaggaagatgagtacctcacaaccaaaagcagttaactatgcctggcataccaccctgtcatgtgggcagatcactgttcccatgctgggtaagagtctccaagaagggaagcccttatgcagtaattctgtaactatattaaatttggtaatctaacattaaactttttcgtgagcagtgaatatacacatggtcatatgaaaactgccctggagaccgggttaattattaaataaactaaaaggggagaaatgctgatagataaaattatgtcaattccagggtgttcaatggaataaagaaacagcagcagctgcttcaaaagtagactatgatcagaaacctcagatggtaacctttaaaaattgtggaatccagagtctcaacctaaacctacataggagctacagccagggagttctttctaagttcctcaagtgattctgatgattggccaagctggaaacttctgaactgggggagaaagccaacctaggtaaatgtagagacttttagaattcaacatttgattatcatttactccacattttcccccagctgtctcaccttctctatttttctaacagtgaacaataaaagggcttggcaagtgaaggaaaaagtcagtagagtacctaaaatggatttgactatattcaagccactttcatatattaactagataaaaggataccatactgctatttgaaattcaatcacaaagcaaaaatgtcataattttaatgtattttaagggaagacggggttcttaacatgaatatgtaatacaaaaacaattctaaataataatatttaatagaagaaaaaatctgtataattatttagaagtaactctgtttttaaaatttcaatgttaggaagaaaatcccttaaatttgaaatagcggaatattctctcatatgaaaaaactgtgtcccagtgttattcttcaacttagaaattaggcaaagtattttagtactatttctgcttacatattgttttgtatgaatgttttaagtatgaataatattttggtttttagtgtgcatgctaatataaaaatatggatttttttctcctacactgactttgtacactttccaggcccgaagaataaaaaacttttaaaatatcctgtgttcactagcaaaccttggaacgataaaaaaaggtagtacctacataagaaattttacattgaaattacaattgtatgtttttcaggagttaaagtgattcaatttttcaatattcaaacacaaaatagtaaatttttatttactatagcacaattcaagtattctcttaaatttatatttagtcaactaaaacatgacagtgactttataagagctttccttttaaaaggttgctgttataaaaaagtatgactctattactctaaatgcttagaataagtggaaagaacaaatgacagtagacaaaaacctttatgagtgagtcatcaacacataaaaggttgcacacatcagtaataggacatgtgaaggtaacatcccaaaagtatttgaactcatgtaaacaaagactatgtatattcctaagggagaaaatgtactaccaagataaaatatattcaaacggctgtgactttaaaccatgtattagttgaataccacacaaaaccaaaaaggcattatctatcatttaataactgaaagatattacttatttgtgagataaaaggataatgcttttttaaaaccaataatgaaaaagaagtattttgaaaacaaacatctgtttgctagaaataaatatacttgcttagttattttaatgtattgcagcataggaatattgtgctagcattgaccattaacattcaatcagtagtttaaaatattttttccacattgagtcttgaatcctctacctggtcagctgacccacaactttcaaaagagttttattttcctgctttagctgttcattttcatcttctatgtcatctaggtctctatttaataaatcaatttcttctttgagttttccaatcatttcctctttatcttgcatcagtctcacaagtcttaggttttcttgtctttctcttactacttccttttcaagatcttcaattttcttttccagtgtgctacttgaaaccagagtacctgaaacatttgcatccctgttatatctagggaacccacttctatctgttcgagaatatctacttgagacatcttcttcagagacactggttgtgcttttatatctgcctgaaactgttctaggtggctcctgtagcagataggaactgcctggatctagtaagtttacagcttcattctgaatagtgttctgttgtgtaattgcatcttctcgtttccgctctttctgccctgcttcatcatcttcgtactcatctaagcactctgcggcagggatgttgaccacgccggtggagcgccgcttctcccgcagcttcctcttctcgatctgccccttgcctttcctggcactggggcccgagctcttgcccttctctgggacgccgtccggctcctcctcgtcacgctggggcggcggtgcagccgaggcagaggcggctgggggctcgtcctccgaccgccgcgggccgggggccgcccgcgtcagcatggcggagccgaccgcgcagttcacgcccccgggaccggggacggcaggtgcggccggcgcgccgcccgggaggttgttgttgagctcgttggcagcggcggccgccggggtgcccagagcccccgcggggggcttcccagcggcgtcgctgctgccccctcccgggggggccgggcccggggggttctgcttggcgcgcatcttctcgcgtttcgccttccactcctccaggaagtctgtggtgctgccgccgaggccgctgctggtccggtagccaccggtcgccatattcccaaaggggccggtcgggctctcacctcaggccgcccaccagggctccggccgctgcctcctcttccttcctgcggccccgaggatgccaggagacgacctccaggagagggacggccgccgctcccacagcagccggcggggcttggaggagcttgtaggggacgaggcgtagggctgggatccggctcccaggtgtgccgaagctggcgcgcgctcttccgccgcgcggaaagt

SEQ ID NO: 15131 - RNA, 8229 nt, Homo sapiens
  source 1..8229: mol_type = other RNA
gctgggattacaggcatgagccactgcacctagccagtcagggcacttttaaaagcaaaggtcctattcaaatgtaaggtttccttatatgcaaagaggttacacgaagctgcagcagttagattaagagccaacacatccttctctgcccctgggacacatgagcattaacaaactccacaacttttcctttatcacacagaatgaatcctgttatgcttcaagacctgggtgaagttgtcttgctccatgaagccttgcttgatcgtggaaaccagtgacgatctttctctgaccggccagagaaccgccagctcatctacacagacacacgccaccacacacatacacccgtgcattccttcacaagagagtagagcttacccctcaactagtttgaccaaaggtcctgccataaaagtcttgtcacatcttgcagtgatttgcacaccataggtgctcactaaagatgtgttaattggctgattagaataaatggcattgctgtccagcccactatcaagcaaagatggtcttcagaagtaaagagatggacttccctggagtctgattctattaataactgattctgccaacactaagcctgtaacctctaccacggatctcatttctctaaaatccattgcaaattactgaggctatctctgcttgtaatctgttactggcgagcatattgattcccaggtggctgcctgacccacaaaccaactcattgtgttgagcatctcaatctcttctcgaaaagcactcaccaaacctgctcacacactctccaactccttcggagtagtagtggtgcctcaggtagacagtatggtctagcaggaaagagacccatcctcaacggctctgtcagctcgtttagatttaatctgacatagctgtctctttagaacaaaatctaccaatggcctaatttttacttcgttttttttttttttttttttttggtttagtgtttctgttcttcagagttgagttccttgaaatgacacttttgctcctacgttgttaacactccttttctcacttctccccgtgctcacacagatgattcaaacgcatttgaaaaacgtctcccgttgctttgtaaggatgtttccatgctgcattttccctagggcagcaagggagattggctaagggagattctctagttcaccctttgtttcctttgcagcaaagccctccagaatttggcttcccaggcctggcaggaaatgccaaagggtgggggatgggtagaattgtgtagagatgaaatttttaaagaggaaaaatcatgaaattattcaagacaggttttgtgggatcctgttggagagaatggtttcaacaatgggggtcataaatacaaatgcacagactctaaaaatctgggaatttcatttcctgtaacttccagaaaaaaaaaacaaaactacctctcagtggttctcctatcccttgtagtcaatgcctgaatgggaacctgggaactgggagaggcaattccaaaagtcacttcccccacaaaccctgaccaagcccctaagttttagagcctagcagtccaataaggagggctcacagcattacctccctcctctaccgataggcatctgatcttgtagatgcaggaatctgtctccttattttccaaataccctccctttctcctcttccttctttgctctggtttagccattatcatttccttggaagaagtaggagatagcattggttgggagttcaagcattggaaaaataatacaaatgagatttggaaataatttctaggtttcagcagccatgtctttacccctaccctcttgcaaatgccacccatgcttccaggtccagggtaggttctacctccatcaggaaaccttcctgactgcctccttgcatgtctatctctctactaggcagtaattggcatgagttcagagttggtatcttttagctttgtagccctagaatctagcacagtgtctagcacatagatgcttaacaataaagacttgtaattgaaacaattataggccataatttttttatagcaagaaacaactgtggatgtataaaaaattttttttctcatatgcaagaaaatattaaacactactgacaatgttacccacttaaaagtcttctagaatttttaaatataaaaattttggtctttcattcacatcaacagatacagttttttgtgactatgccaattttgataagctgataagcaccctacctttataaaataagaattatgtccagggatttttagttgtaagagggaggacctgggacgaatgtggctacttgatcttgactggaattagaagttctttattcctctttctgtactttatattttgacagtaaattaaatcaagtttggtagaattccctacatggttcaggttactcttgcatcccaaagacacactggtttgaatttgactgaaattaaaaccactggcttaatttgttgttctgtctgctttttctcactagccctggaaagctggagccattttatttgctttttgcctttctagatcccatggagcggatggagcacatgagccaagggtaggcgggctcagtaaagaaaagcccaaatctctcttcagctgtaagttggcccttcactgggctgcactgaccagacctgaacctgactatgtcatcatgactgatgccaatgggttcatatgaccattgccattggtcaccgtattagatatggtgacatcactttacacacttctgagtctttccaggcaacttgtatgtagtgtgcagtctgaagcaatgtctaatctctcagaagaagttctcaaaggaatgtttccaaaaggaccatttttttccgatatattgaaaaataaaggctcacctaaaaataattaaactcgacttaatattattgctgttctgtatgtcataattaaacaagcatgaaagaaatcttaataggattgcaatcgggtctttgtgttcctgaatgttgtatcagagtcttagtggaaaccaggtttaaggtggctcagaggaactgtcctttgttttcaggaaaagtgaaactcaatcaagactgaattctgtggctaccaaacccagctgctattcccaaatcctgtccaaatcctctctacctttcaaagcctggcttgatcgcacttcttccactagatcgtagggaagaccccctcccctgagtcttcttggtttgaatactcccatctagaacataactattcaatgctgtttgctactccctcttagcttgtggaatttagaataacctcccaatctattatcagtgaatccttccacgtgagaactgtcttcctttggttaataaccccagcatctacctcagagtcaggtgaataatagctactctttaaaactatgataaactgttggtttgtcatagggaaagtcacatttttaaaaagttaagttgaaggtttataagctgattcttcatcaggttcctttcataagtaagttaagatccttctatgaggttaaaatatgattcagtttagaaaaattcagtgaatatgcatctgttacataaagctaagtattctatgaaactgaggtggcatgagagagttggtgcaaagctgctcctgtgactgtggctgcctgacagtggcctgagaaaagatagtaaatatctgaactacagaggaagctccttctctgcccatcctcaccctacagccatccatgacaacatccatgttagcttgatcactgttctgccataaaagaaatccctggtgttattcaacaccattttgtgctccaaaagctgccatatgatgaggaatccttagccttgttattctacaacgcacaaaggagaacactgctgacattgaagacatccattcccactccctcactcattcaccaagctgaccttcaacgtggcttcccatgatccaccacgtacaggggctccatagagccctcacaactaaactggacccctcctaggatgttgggcttcttgataatggtgtaaagaaaacttgccagagtggctccctgcctggaaagccacctcagatagtgagagggagggctacctgctggggacagggggaagtgggagggttcctccaacagaagggaccctgtgctggatcaggcacaagaaactagcaatgtgaatcagagcaaggccccactaccttgggagtccctgagactagatgagatgccaggtctgactctgccaagatggagtgcctatgagcaaaatagttttacttctctgaaacccaattttctcactggtaccaaaaggaaagaaaagaaaaaaaaaaaggaaaagaaaagaaaggaaaagagagagagataaagaaagataaggtgactttgaaaaaatcttccaagtctttgattctgtccgtgggtacctgtcaagtgtgaggccctgtgataggcaccatggaaaatacaaaatatgatacatttctcatgaatctaaaattatgctctagtggaaaaaagaagaaagttaactccatcactgagtctctattattcaggattctgtacacacacaaacccataaatattaggcattacacaacacacatgaaaaatgagaagagttagtaattcttatacttgtgcagaaaaagggatagattcctattaaatagtggtctctgaggaaagtttcgtagacaaagaaatatgtgtccatcttgaaagataagcagaatgatttccagattttcagacgatatttcttattctcctgagagatcagaaggataggaaaaattccactggatcagggttcctcagtatggaatgggcattgtgtgtgtgtgggtgcatgtgtatgtgtgtgtaagagagagatgggggaccctgggatcaaataagttcggaaaagtagattaaacaaaggtaattttgttttcattgcaggtctcctcaaggatgctaataaacatacgtgtgttgagactaagagaggttacgtttgcagtgactccaactatgggtcacagagtcctttcttcttacagctgctcaagtgattggggttctgagaaatcctctctgggaaacggtgtaccaaagataatgtaaactccatgaggtcagggactagtctagttcaccactgtatctccagcacctggcatggcatcagatacacgggaaggatataatgaaatataataaaagaaaagtttgccaaatgactcaatgaataactattgaattttaagtggaaaaactggcattcaaaatgacatggagatgagaatacacccagaagcaaggtatcacctctccatgatgtcaccctcagggtctgggttccacataagccacagctaggagtttcaggtgatgtctgtctttgccttctcaagaagcaaaatactacaaacatccataatgatcctaaaagactttaactcctcccaacccctcaaaaaggataacaaaattagagcttcatgaagaacattgctgtttctttactaaaaacaggtaacaaattagttaataatactcgagtcagactctaccatggagttatggattatctttgtttctttactgccaccttctggttcccagacacctatgcggtaaattaaaaatgctgccttatatttgtgtttcactatgaaattttaagcatttgttcacatcctttatttcagatgacattacacagattagaagagattaaggtggcctttactctttttcatatgacatgaaaataacttagaagttaagtgatttgattagtgatagaaagttaggagcagagcaaggactaaccacacttgttggtttttccaatgagcaaacagtgagtttagccatttggctttgtccaactctggctgcaaagaattctacagctctctcatcccttcacaagcacaaccttgaatggaaaatcctgtgcccttggtctggaagcagcagtagagttgggtaaggtacgggtgtttccgtgccagagccaaaatcctcttctctgtcattgtgcagtccacgtcatcatcctgaaggatgacgtccttctttaagaccttcacagcatatacttcatctttgcccttgagttctgccaacatgacctgcaatcaatcaattgcctccatcaatcttgccaaagctgcctttgcccaacaccttgatgaagttgaactcatccaggcccaggcgcttggcctggccttgccggacttcgccattctcaccggggctcatcagctggccatcaggagacgatgctgcccggtgctcctctcctcggttgtcaaatgacaaggctttccgaatgttgttctcaagttcttttatttcctggtcacaaggggaggtgggtgctgacttggatcgatcttcctcagatggtgagcttccagaagcaggctgcggggactcggcaccagcaatgagctttttccttctctggccgctgttggtgattttgtctggggtaacgcccaggtcggccagtactttggcgattcctctggcatccactccacagttgggagccacgttggtctcacatcgacggtgaacattcattttgcagactttacactgcaaaccctgccgcaagagtccccagagcagggacccacagtgatcgcagaaggtagggaccttgtagttgtggataccgaacttgtggggcatgttgacgctgaaccgctgggagcccacctggtcgggggtctcctgcttctttaacccagcacactttgtgattatgagctcgtggcaccgcttgtggaccacgcaggtgcagacttgacactggtatccctgctttcctatgacaccccagatgaagtctctgcaatgggagcagtaggtgggctgccgaagataggtggccatgaacttgtggccgttgacctgatggaccctgcgcctgacggccccctgccgcttcctcggccgcatgcgttccctgaacacacgctcttcattgtctttaggggcttcacccgacgaccctgagagatcgatgatcacatacactcttccttctggctccagatcaatccagtcctcgaagtggcggctcccgttctgcagcagctcctcaaactggatggtgcagttggccacgaagtcgtcgtagcctatgggggcatcgtgaaagacagccagctcgatcttgcgtccgttgcacacatcggtgacgaactcgtcgtgccaggccgggctgttggtcttctgcttggtggccgtttggccgatgcgcgagtcgtccacattgagggcaatgtaggggtcgagaaggaaagtctgcggccggggtcccaccgcatggcgcagcgaccaggctgtgggcttcaagctcacggcctcgcagattttgatcttaagaaggccattgaacactaccatggtcggggcggggagtgggggccggggtcactccgtctgccccgagggcaggaatgaagaaccgacggcccggcactccgagccacagggactcttgggtcccctttcgccccaccccgcacactccctacaccttgtggcgttgcgccctggcgcgggcgattctcagccagtgcatgtatttcctcgccgggttcctaacggaaaacagggaggggggagagctgggggatgtccgtgtttggagcaagtctctccccccgaccaccagctgcacctccagaagagaagacgagctgtcggctccgctgcaagccgcgggggctgcctcgccgcctcgctggctctccggctccggactgcgggaaagcgggcgccgcgcccggcgcttacctacctttccgaaacataatcccgggaaatttcgactccgggagggggatggggcggtgggacggggcggggacgagaaccgggggcgcagatttcaacccggatcctcttcgcacactcagcgcctgcctctgaccgcgcggggcgggggggtgaacggagggatgttcagtctatccggagggatgcatgtcgagaggaaatggtcctcctcggagccaaatttttaaaaatccacaagccccacggccagccggggccgccgcctcctgggcgaagcagcgccgcgccggagccggcgatcgggaggcgccaggagcccggaatctcacatccgcgcgggctcggagtccgggcggccgccgatccggctcgggggcgcaggccagcacc

SEQ ID NO: 15132 - RNA, 8201 nt, Homo sapiens
  source 1..8201: mol_type = other RNA
gctgggattacaggcatgagccactgcacctagccagtcagggcacttttaaaagcaaaggtcctattcaaatgtaaggtttccttatatgcaaagaggttacacgaagctgcagcagttagattaagagccaacacatccttctctgcccctgggacacatgagcattaacaaactccacaacttttcctttatcacacagaatgaatcctgttatgcttcaagacctgggtgaagttgtcttgctccatgaagccttgcttgatcgtggaaaccagtgacgatctttctctgaccggccagagaaccgccagctcatctacacagacacacgccaccacacacatacacccgtgcattccttcacaagagagtagagcttacccctcaactagtttgaccaaaggtcctgccataaaagtcttgtcacatcttgcagtgatttgcacaccataggtgctcactaaagatgtgttaattggctgattagaataaatggcattgctgtccagcccactatcaagcaaagatggtcttcagaagtaaagagatggacttccctggagtctgattctattaataactgattctgccaacactaagcctgtaacctctaccacggatctcatttctctaaaatccattgcaaattactgaggctatctctgcttgtaatctgttactggcgagcatattgattcccaggtggctgcctgacccacaaaccaactcattgtgttgagcatctcaatctcttctcgaaaagcactcaccaaacctgctcacacactctccaactccttcggagtagtagtggtgcctcaggtagacagtatggtctagcaggaaagagacccatcctcaacggctctgtcagctcgtttagatttaatctgacatagctgtctctttagaacaaaatctaccaatggcctaatttttacttcgttttttttttttttttttttttggtttagtgtttctgttcttcagagttgagttccttgaaatgacacttttgctcctacgttgttaacactccttttctcacttctccccgtgctcacacagatgattcaaacgcatttgaaaaacgtctcccgttgctttgtaaggatgtttccatgctgcattttccctagggcagcaagggagattggctaagggagattctctagttcaccctttgtttcctttgcagcaaagccctccagaatttggcttcccaggcctggcaggaaatgccaaagggtgggggatgggtagaattgtgtagagatgaaatttttaaagaggaaaaatcatgaaattattcaagacaggttttgtgggatcctgttggagagaatggtttcaacaatgggggtcataaatacaaatgcacagactctaaaaatctgggaatttcatttcctgtaacttccagaaaaaaaaaacaaaactacctctcagtggttctcctatcccttgtagtcaatgcctgaatgggaacctgggaactgggagaggcaattccaaaagtcacttcccccacaaaccctgaccaagcccctaagttttagagcctagcagtccaataaggagggctcacagcattacctccctcctctaccgataggcatctgatcttgtagatgcaggaatctgtctccttattttccaaataccctccctttctcctcttccttctttgctctggtttagccattatcatttccttggaagaagtaggagatagcattggttgggagttcaagcattggaaaaataatacaaatgagatttggaaataatttctaggtttcagcagccatgtctttacccctaccctcttgcaaatgccacccatgcttccaggtccagggtaggttctacctccatcaggaaaccttcctgactgcctccttgcatgtctatctctctactaggcagtaattggcatgagttcagagttggtatcttttagctttgtagccctagaatctagcacagtgtctagcacatagatgcttaacaataaagacttgtaattgaaacaattataggccataatttttttatagcaagaaacaactgtggatgtataaaaaattttttttctcatatgcaagaaaatattaaacactactgacaatgttacccacttaaaagtcttctagaatttttaaatataaaaattttggtctttcattcacatcaacagatacagttttttgtgactatgccaattttgataagctgataagcaccctacctttataaaataagaattatgtccagggatttttagttgtaagagggaggacctgggacgaatgtggctacttgatcttgactggaattagaagttctttattcctctttctgtactttatattttgacagtaaattaaatcaagtttggtagaattccctacatggttcaggttactcttgcatcccaaagacacactggtttgaatttgactgaaattaaaaccactggcttaatttgttgttctgtctgctttttctcactagccctggaaagctggagccattttatttgctttttgcctttctagatcccatggagcggatggagcacatgagccaagggtaggcgggctcagtaaagaaaagcccaaatctctcttcagctgtaagttggcccttcactgggctgcactgaccagacctgaacctgactatgtcatcatgactgatgccaatgggttcatatgaccattgccattggtcaccgtattagatatggtgacatcactttacacacttctgagtctttccaggcaacttgtatgtagtgtgcagtctgaagcaatgtctaatctctcagaagaagttctcaaaggaatgtttccaaaaggaccatttttttccgatatattgaaaaataaaggctcacctaaaaataattaaactcgacttaatattattgctgttctgtatgtcataattaaacaagcatgaaagaaatcttaataggattgcaatcgggtctttgtgttcctgaatgttgtatcagagtcttagtggaaaccaggtttaaggtggctcagaggaactgtcctttgttttcaggaaaagtgaaactcaatcaagactgaattctgtggctaccaaacccagctgctattcccaaatcctgtccaaatcctctctacctttcaaagcctggcttgatcgcacttcttccactagatcgtagggaagaccccctcccctgagtcttcttggtttgaatactcccatctagaacataactattcaatgctgtttgctactccctcttagcttgtggaatttagaataacctcccaatctattatcagtgaatccttccacgtgagaactgtcttcctttggttaataaccccagcatctacctcagagtcaggtgaataatagctactctttaaaactatgataaactgttggtttgtcatagggaaagtcacatttttaaaaagttaagttgaaggtttataagctgattcttcatcaggttcctttcataagtaagttaagatccttctatgaggttaaaatatgattcagtttagaaaaattcagtgaatatgcatctgttacataaagctaagtattctatgaaactgaggtggcatgagagagttggtgcaaagctgctcctgtgactgtggctgcctgacagtggcctgagaaaagatagtaaatatctgaactacagaggaagctccttctctgcccatcctcaccctacagccatccatgacaacatccatgttagcttgatcactgttctgccataaaagaaatccctggtgttattcaacaccattttgtgctccaaaagctgccatatgatgaggaatccttagccttgttattctacaacgcacaaaggagaacactgctgacattgaagacatccattcccactccctcactcattcaccaagctgaccttcaacgtggcttcccatgatccaccacgtacaggggctccatagagccctcacaactaaactggacccctcctaggatgttgggcttcttgataatggtgtaaagaaaacttgccagagtggctccctgcctggaaagccacctcagatagtgagagggagggctacctgctggggacagggggaagtgggagggttcctccaacagaagggaccctgtgctggatcaggcacaagaaactagcaatgtgaatcagagcaaggccccactaccttgggagtccctgagactagatgagatgccaggtctgactctgccaagatggagtgcctatgagcaaaatagttttacttctctgaaacccaattttctcactggtaccaaaaggaaagaaaagaaaaaaaaaaaggaaaagaaaagaaaggaaaagagagagagataaagaaagataaggtgactttgaaaaaatcttccaagtctttgattctgtccgtgggtacctgtcaagtgtgaggccctgtgataggcaccatggaaaatacaaaatatgatacatttctcatgaatctaaaattatgctctagtggaaaaaagaagaaagttaactccatcactgagtctctattattcaggattctgtacacacacaaacccataaatattaggcattacacaacacacatgaaaaatgagaagagttagtaattcttatacttgtgcagaaaaagggatagattcctattaaatagtggtctctgaggaaagtttcgtagacaaagaaatatgtgtccatcttgaaagataagcagaatgatttccagattttcagacgatatttcttattctcctgagagatcagaaggataggaaaaattccactggatcagggttcctcagtatggaatgggcattgtgtgtgtgtgggtgcatgtgtatgtgtgtgtaagagagagatgggggaccctgggatcaaataagttcggaaaagtagattaaacaaaggtaattttgttttcattgcaggtctcctcaaggatgctaataaacatacgtgtgttgagactaagagaggttacgtttgcagtgactccaactatgggtcacagagtcctttcttcttacagctgctcaagtgattggggttctgagaaatcctctctgggaaacggtgtaccaaagataatgtaaactccatgaggtcagggactagtctagttcaccactgtatctccagcacctggcatggcatcagatacacgggaaggatataatgaaatataataaaagaaaagtttgccaaatgactcaatgaataactattgaattttaagtggaaaaactggcattcaaaatgacatggagatgagaatacacccagaagcaaggtatcacctctccatgatgtcaccctcagggtctgggttccacataagccacagctaggagtttcaggtgatgtctgtctttgccttctcaagaagcaaaatactacaaacatccataatgatcctaaaagactttaactcctcccaacccctcaaaaaggataacaaaattagagcttcatgaagaacattgctgtttctttactaaaaacaggtaacaaattagttaataatactcgagtcagactctaccatggagttatggattatctttgtttctttactgccaccttctggttcccagacacctatgcggtaaattaaaaatgctgccttatatttgtgtttcactatgaaattttaagcatttgttcacatcctttatttcagatgacattacacagattagaagagattaaggtggcctttactctttttcatatgacatgaaaataacttagaagttaagtgatttgattagtgatagaaagttaggagcagagcaaggactaaccacacttgttggtttttccaatgagcaaacagtgagtttagccatttggctttgtccaactctggctgcaaagaattctacagctctctcatcccttcacaagcacaaccttgaatggaaaatcctgtgcccttggtctggaagcagcagtagagttgggtaaggtacgggtgtttccgtgccagagccaaaatcctcttctctgtcattgtgcagtccacgtcatcatcctgaaggatgacgtccttctttaagaccttcacagcatatacttcatctttgcccttgagttctgccaacatgaccttgccaaagctgcctttgcccaacaccttgatgaagttgaactcatccaggcccaggcgcttggcctggccttgccggacttcgccattctcaccggggctcatcagctggccatcaggagacgatgctgcccggtgctcctctcctcggttgtcaaatgacaaggctttccgaatgttgttctcaagttcttttatttcctggtcacaaggggaggtgggtgctgacttggatcgatcttcctcagatggtgagcttccagaagcaggctgcggggactcggcaccagcaatgagctttttccttctctggccgctgttggtgattttgtctggggtaacgcccaggtcggccagtactttggcgattcctctggcatccactccacagttgggagccacgttggtctcacatcgacggtgaacattcattttgcagactttacactgcaaaccctgccgcaagagtccccagagcagggacccacagtgatcgcagaaggtagggaccttgtagttgtggataccgaacttgtggggcatgttgacgctgaaccgctgggagcccacctggtcgggggtctcctgcttctttaacccagcacactttgtgattatgagctcgtggcaccgcttgtggaccacgcaggtgcagacttgacactggtatccctgctttcctatgacaccccagatgaagtctctgcaatgggagcagtaggtgggctgccgaagataggtggccatgaacttgtggccgttgacctgatggaccctgcgcctgacggccccctgccgcttcctcggccgcatgcgttccctgaacacacgctcttcattgtctttaggggcttcacccgacgaccctgagagatcgatgatcacatacactcttccttctggctccagatcaatccagtcctcgaagtggcggctcccgttctgcagcagctcctcaaactggatggtgcagttggccacgaagtcgtcgtagcctatgggggcatcgtgaaagacagccagctcgatcttgcgtccgttgcacacatcggtgacgaactcgtcgtgccaggccgggctgttggtcttctgcttggtggccgtttggccgatgcgcgagtcgtccacattgagggcaatgtaggggtcgagaaggaaagtctgcggccggggtcccaccgcatggcgcagcgaccaggctgtgggcttcaagctcacggcctcgcagattttgatcttaagaaggccattgaacactaccatggtcggggcggggagtgggggccggggtcactccgtctgccccgagggcaggaatgaagaaccgacggcccggcactccgagccacagggactcttgggtcccctttcgccccaccccgcacactccctacaccttgtggcgttgcgccctggcgcgggcgattctcagccagtgcatgtatttcctcgccgggttcctaacggaaaacagggaggggggagagctgggggatgtccgtgtttggagcaagtctctccccccgaccaccagctgcacctccagaagagaagacgagctgtcggctccgctgcaagccgcgggggctgcctcgccgcctcgctggctctccggctccggactgcgggaaagcgggcgccgcgcccggcgcttacctacctttccgaaacataatcccgggaaatttcgactccgggagggggatggggcggtgggacggggcggggacgagaaccgggggcgcagatttcaacccggatcctcttcgcacactcagcgcctgcctctgaccgcgcggggcgggggggtgaacggagggatgttcagtctatccggagggatgcatgtcgagaggaaatggtcctcctcggagccaaatttttaaaaatccacaagccccacggccagccggggccgccgcctcctgggcgaagcagcgccgcgccggagccggcgatcgggaggcgccaggagcccggaatctcacatccgcgcgggctcggagtccgggcggccgccgatccggctcgggggcgcaggccagcacc

SEQ ID NO: 15133 - RNA, 7580 nt, Homo sapiens
  source 1..7580: mol_type = other RNA
gctgggattacaggcatgagccactgcacctagcctattttctactttttaaatggcattatttttccataccagtatttatttttatgtagccagatgtattaatatttttctccaagatcacaaacatcttttttcatacatacatatatatatcatacatatatatgtcatacatatatatcatacatatatatatcatacatatatatatcatacatatatatatatatatatatatatatatatatttatttatttatttatttattttttagacagattcttgctctgttgcccaggctggagtgcagtagtgcgatcttggttcactgcaacctctgcctcccgagttcaagtgattctcctgcctcagcctcctgagtagctgggattacaggcgcctgccaccacacccagctaatttttgtatttttagtagagacagggttttgccaggttggccaggctggtctcgaactcctgacctcaggtgatccacccaccttggccttccaaagtgcttggattacaggcgtgagccaccgcacccagccccccaatatttttatcattatttttaaatgtttaatgtttaggggtcagacttcatttttgtcaaatggacagccaattgatccagccccattaactgaataatacaacccttcccactgattgaaatgccacttctatcataagttcctagagatacacaggtctgttgctggccatttttctttttcttttttctttttttctggaaacagggtctctgtcacccaggctgcagtgtggtgatacgatcatggctcactttaactttggcctcccaggttcaagtgatcctcccacttcagcctcccaagtagctgggattacaggtacatggcaccatgccccgcagtggcctttcttcagcagtgggccacagaaacgaatatgcatgtgagtggctgagggtggccacctggagagtgccacatgcactgcgtctcctcatttgctgctgtgcagaaattgtggacccactgtggccacatatgccgagttctcaagaggtgctagacatccagatttttatatgaactctccagtgtttaaagtgttggcaattaattaaaaaaaaaaaatttaaaatgccgggcaccatggctcacgtctgtaatctcagcactttgggaggccaaggtgggtggatcacctgaggtcaggagtttgaaaccaacctggccaaaatgacaaaaccccgtctctactaaaaatacaaaaattagccaggcgtggtggcgggcacctgtaatcccagctactcaggaggctgaggcagaagaatcacctgaacccgggaggtggaggttgtagtgggccgagatcacgccattgcactccagcctaggcaacaagaacgaaactctgtttagaaaaaaaaaaaattaaaaacattatgtggacaaaatacatttgcaagctgagactagcctgtggcacaccggttagtgacctctattccacatgctgaaataatgcaggccagactgggtccaggaatccacctctaactctttcccactgccaacattaagatgcaaaagaggaagagtgatgtggcagctcctggaaacccaggcatctctgggaaagcaagcagtgttatggctcatgtgtcaccttttacccacaggagttgatgatgtggttcccggtatgccaagtaactaggagggaggaggtcagcactggggaggggaaggtaacatcctcagtcaaagttggacctcccagacctgttaggcagagttacaaagaaagacaatgggttggaaggaggatggaaactgaggtgctggccaagaacatagcaagattttggccccccaaaacaagctggaaagtgatgtcacttcctatgtaataataatgtggcttccgtggaaaccttccaacttaacactgcagaatctgaaaagaaatggcaatgagcagaggtctcccaccctcacgtggaggacagggtccgcaaagatgagtcacattgtagaacttcactattcagagaaagccccttcacatgcagaatctcgctggtctctcaggacaatcctgtgaggtaggcagcaccaggggtgttactgccccttacagaagagggaactggcattagtgatgatcagaatgggtcttagatagctctgggatgtgcaggaaggacacttgtatgaagaataaaagaccggccgggcgagtggctcacgcctgtaatcccagcactttgggaggccaagacaggcggatcatgaggtcaggcattcgagaccagcctggccaacatagtgaaaccccatctctactaaaaatacaaaaaattagccgggcgtggttggcgggcgcctgtaatcccagctacttgggaggctgaggcaggagaatcgctttaacctggaaggtggaggttgcagtgagccaagattgtggccactgcactccagcccgggcgacagtgcgagactccatctcaaaaaaaaaataataaaataaaaataaaagactgcaggccctttctccttccccgtgcccatttctgtagaatcatttattcattaaattcactgaacactttccatgggctgggcactcttaggcattgggaacataggagtacacaggtcctgggcactgtcctcccctgtggctgggtcagtcatccttactctgaatcatggcccagactggccttgccctactcctctctaggtagagcagtgatctcaggccaactcttgcattttgttccagaaaccttgattatttccctgactattggtcacttcccgaaatgcactgaactgtgccaggaataggatatgtttttaagtgcttgagacacagacaagtggcagacgcatacccaaattccaaccatactttacttctgacctaattttaatatatgtttcatgcagttacacaattatctgtgcataatgctctgagaaaagggatggcacatacagtttctcctgaagcgggaaacagagcccagttggtaaggtggccagtctctagggcatcttagatgaaccttgtttcttcctattacttttccttcatctactttttttttttctgagatagagccttgctctgtcgcccaggctggagtgcagtggcatgatctcggctcactgcaacctctgcctcctaggttcaagggatcttcctacctcaggctcctgagtagccaggattacaggtgcatgccaccgtgcccggctaatactttgcatttttgtaaagacggggtttcaccatgttggccaggcgggtctcgaacccctgacctcaagtgatcggccgcctaagcctccaaagtgctgggattacaggcatgagccaccgtgcccagccttccttcatctacttattttcctgtgatgcctccatgttttagagtatgtgtctgaggggcaggaatatgtattagatatatctagggcagtcccaccagctttacattcttgagacctcatccatcagttcttgttttgcagacatatacttctattgactacaatgagaagtgtgtctcttaaaaaggtaagtctggccgcgcgtggtggctcacgcctgtaatcccagcactttgggaggcagaggcaggtggatcacgaggtcaggagatcgagaccatcctggctaacatagtgaaaccccgtctctactaaaaatacaaaaattagctgggttcgtgggggtgcgtgcctgtagtcccagctactcaggaggctgaggcaggagaatcgcttaaacctgggaggcggaggctgcagtgagcccagatcatgccactgcactccagcctgggcgacagagtgagattctgtctccaaaaaaaaaaaaaattagccaggtgtggcagtgcacgcctgtagtcccagctactggggaggctgaggcaggagaattgcttgaactggggaggcagaggctgcagtgagcccagattgtgccactgcactccagcctcagtgacagagcgagaccctgtctcaaaaaaaaaaaaaaaaaacaagtgaacaaaggtctctggttttcctaggcagaggaccctgcggccttccgcagtgtttgtgtccctgggtacttgagattagggagtggtgatgactcttaaggagcatgctgccttcaagcatctgtttaacaaagcacatcttgcaccgcccttaatccattgtttatctgctgaccttccctccactattgtcctgtgaccctgccaaatccccctctgcaagaaacacccaagaatgatcaattaaaaaaaaaaaaaaaaagttaagagcaaaaaaaaaaaaaaaaaagtcctggttgggtgtggtggcgtgtgcctgtaatcctagcactttgggaggccaatcccttgggcccaggagtttgagaccagcctgggcaatataaggagaccctatctctaaaaaaatgaaaaaaaaaataaataaataagttcaagttcaggtccctagtacctgtgaatgtcaccttacttggaaagagtattcgctgatctaattaaggtaaggatctcgagatgagatcatcctcattagagtgggccctaaatccagtgacatggatttggtgtccagtgatgtctttacaagagacaggaaagaatacacacaggtattcctgtgtatttcaagtcaagttgtatatggtagtccttgcttaataagggaaaagttcgggtctgtgtatttattcttagggctgccataaaaaattatggccttctcaggggagaaggccacatgaagatagaagcagagactggacttacactgtcacaagccaaggactgccaaggattgccgatggccactagagaaaggagaaaggcatggaatggattctcccccagagcctccagaaagaacctaccttactaacactttaatttcagactttgggcctccagaactgtgagactcaatttctgttaagtcacccatgtggtggtaattttttttttttttttttgagacagagtcttgctttgtcacccaggccggagtgcagtggcatggtctcggctcactgcaacctctgcctcctgggttcaagtgattctcctgcctcagcctcctggttagctgggattacaggcacacagctccaagcctggctaatttctatattttcagtagagacagggtttcatcatgttggccaggctagtcttgaactcctgatctcaagtgacccgcccaccttggcctaccaaagtgctgggattacgggcatgagcgctgcgcccggccaggttgtggtaattttttatggcagccctaagaataaatacacagacctgaacttttgtctttttgagcaaggactgccatgtacaacttgacctgagagtgcagccttcaatcttttcctctggggcctctggcaacagttctcagatgactatgctcagagagacacctgtgactgtccacccagcagccatctgttcaccagcagaggagaccggaagtcccttgtgaggtgctgggttctgaagcttcaggagtgggatccatgtcatcgtccatatcagatctgtctgctccaatctcagccctttcttcctgcctgatccaaaggctattttctagctgttcttcagcaatttctagctcttcttccgtttgtaaagtagccacagtttcccggggcaagtttgaggaatatagcccaaatttggctttatagccaaacattgcctcaaatggactttgctgcaaggaaacgtcgaaagcctgattcctcaccatctgcatgaatcggaggcctttggcccagtgacatgagtggttactctgcatccaggtacttatcatgttctttacatcacggcttgctccttccagggagccctggctttggccagggtggtacttaccagatacaatctttaggtctggccacaactcattgagctcatgaacaacctggtttgtgaactcaacgccactgtcagagtctaacacactgggtgtaccaagaattgtgaaaatatctaacaagacactgaccacctcatgggcctgtttggttcttaatggccgtaaaataataaacttggttgagtgatcctggtagtataaaatgaacttgaactcaccatcggcactggactgcatgtcaagtatttcaacttggcatgtggagtctatgtccttaaaagtcatgggctttggtgcaaggcctctcttgggtactgggttcttctggtggcactgtttacacagagtcagatataagacaataacttctttggtgacattcccatattttccttgcagctccttgagcatgcgtgtccgcccaccatgtccaatactgagatgtgtatcatgaagaatatcaaacaactcttccttatgtacataataccgtattcgatcacgttctccatgagtagcctctatcagtttctctgtgccctgtacagagatcacatcatattttgctgcacggcgataatcacgtgatgacttcttccctttttctttagcttctttaacttcctttattgtttgaaagtacttttctttggaaaataccttgctgttgtaacttttgctttctactaactttgttacactcataagaaacttttctctcatgttacttatctccatttccatttcacttgcatttgaaaccccaggtggatcatttccagctctctgaggcatcatggagagctgtaagaaggatcctgtgagtcttcgccttggctgtttccgactcggaatgtcctcgcattgatcctcccaatcacagccagctgaaaccagcctccttcctgacgtattcagtaactttagctgattgccatctctccttcatctcaacaacctgtaccacactcactggagcacttcgctttgcatctttagtcgaccagttcagatatatacaacctataaggtagggacggaggcttctacctgcctgtaccccctttggagggcccacgaatacagagctgagcacaaaagatgtttaaaggacattttgtcaaaaatgtcgcttacaggtaggtcgttattagcaaggtagagcagcggtacggccgagtctacgcttgggaattcatttgctgactcttatcatttactgactaaagcaaagttactgaggcctcagtttcctcatctacaacccggggagatgaccagtacccatcacaatcgattgctatgaagattcaatgataatgcagataaggcacttaatacagtgtcccctcaccgtccacaccacacgggcacgcccgcttattcctgaggaccgggctgggatgtcgcctcctttgtgtagccttcctaccctgacttcgcagactgctcccaccgcctggatccatgcccgtccacccgccagctcagggctgaacggctgaggcgggcgcgcggtggagaaaagagctgcagactgaggaaggtcaggaaggagaaagggacacaccagacgcggcgtctgaatccccctccacccagaggcccccgagcagcaactcc

SEQ ID NO: 15134 - RNA, 4464 nt, Homo sapiens
  source 1..4464: mol_type = other RNA
gctgggattacaggcatgagccactgcacctggcatttttttttttttagcctgtcttgaattctcttattttcactgcttcatatcttcaggatatgaaaagttggtcagtggtagtgagaaagatcccaaaacataaggatcaaaaaatggcatgtttcagggtaggcatctgtattagttatccattttttttttcagaaagaaagaagtaaaattgtatttgtttgtagatgacatgatctgctgtgtagaaaatcacagagtcaactaaaatactactgaagctaataaacacagtgtatttgcagaatacaatatcagtaccaaaaattagttaaatttccatacattaacaataaacaatgttaaaagaaaattaagaaaacacttccatttgctagagaacttacagtaagaaatatttaggaataaacgtaaaaaggtgagaagtttgtaccttgaaatctacaaacattgatcaaaatgattaaaaacttatataaatagagatatgacccatattgatggattggaaagattaatattgttaaatgattatataacccaatgtgatttagattcaacacaatacccataaaaatccctatcagaaacaaaaaacaggctaggaaaagtggctcacgtcttttggccaggatggtctcaaactcctgacctcaagtgatctatccgtcttgacctcccacagtgctgggattacaggtataagccaccctgcccagcccaatcctcttaacgtaaacactttaatgtcaattaatgcttgaactcaatgtcaagtcaactgaaactcaagtcaatgctgaattgactctaatgtcaattaatgcttgatggtttgctatactcattgcatttggaacaattatctcaggaatgaattttctgatgttttgcaaggagtgacctctaactgaagaccttgccacgcttatgacatttgtaagatttctgtccggtatggattctctgatgtctaatgcgatgtgaatgtgaagtaaaggctttgccacaatcatcacacttgtgatgtttctctcccatatgaattctcctttgttttgcataagatgaagcttgactgaaggcctcgtcaaaatcatcacatttgtaaggtttctctccagtatgaattctcttatgtgtttcatggtgtgatttgcgactgaaaactgtgtcacattcttcacatttgtaaggtttctctccagtatgaagtctatgatgacgtgcaagggttgcttgttgattaaaaaccttgccacattcattacacttgtaaggtttctctccagtatgaattgccttatgaattacaagggctgaattgtgacggaaggtcttgccacactcattacacttgtaaggtttctctccagtatgaattgccttatgaattacaagggctgaattgtgatggaaggtcttgccacactcattacacttgtaaggtttctctccagtatgagttcgccaatgaactacgagatatgaacgacgtctaaaaaatttgccacatttattacacttgtaagatctctcttcattatggattctccaatgatttgcaatggttgtagcattactgaagactttgtgacaatcattacatttataaagtttccctataccatggattgcttgatggtgaataagtgttgactgcccactaaaggctttgccacactcattacacttgtaaggtttctctccagtgtgaattctagtgtgttgtgtgaggtgtgaatcacgcctgaaagccttttcacaaaccttacatttgtatggtttctctccagtatgaattctcctatgtctttcaagatttgatttgcgactaaaaactttgtcacattcttcacatttgtaaggtttctctccagtatgaagtctatgatgacttgcaaggtttgattgttgattaaaaaccttgccacattcattacacttgtaaggtttctcaccagtgtgacatctatgatggcatgcaaggtatcgcttctgattaaagaccttgccacatacatcacatttatattgtttccctcctaaatagattatctgatgtttccttaagagtgagctacaattaaaggctttgccactctcattacattggaaagatttttctcttatgtgtacttcctgttttagtgtgagtaatgatgaatggaagaaattattttcatagttattagaaatatggattttgggcctagaagaaattctttgggacgttagaactgaggaagcatcgttgatagacttctcaacttgattaccaactttccctttggtctgaaatatgtggagttcaggaagatgcgaatgaaagcttaatccaagctgatctttgataggcttgtttccaggatgccttcgatcatatctgtcggtgctaccagtcaactttttgatttgtgtcatagttgcttcatggctatttcttttgtcttcttgccattgaaactcaaagtcatgaatatctttcccaattttctggaagcaaaaatctccaatgtgatgactttcatgtctttctaatgtccctgtgtccacttctgtattgccttgcgctgttgatgagaacttcttcatcatgcatttggaagagatatccacagaatgcaggttcctgtagttctccaacatcatggccctgtataaagccctctgcgtagggtccaggcatttccactcctccaaagagaattctatagccacatccctaaaagtcaagtgtccctgaggaagagccatgcctggctccttttctttcctcttctgagctgcttcctcacgtaacatgagtctttagaaatcaatagtgctgcagtgtgaccttcactgaggcgatctgcttcctgctctgtattagttatctgtttccgagaaacaaattatcacaaacttcgtggcttaaggcaacaaacactgattatctcacagtcgctgtgggtcggggtttggaggcacttcagctgggtgttcctggctcagtgtctctctgggttgtagtcaagctgtgggtcatggctgcagtcatctcaaggcttgactggtgacaacctacttccaaggtcactcacatggctgttagcaggtctcagaaaatctgcttataaggtgactgacacagtggctggcacaccttcatgcctcctgcctgggctatccattggtggcctgagtatccttatgtcatggcagctggctttcctagagtgacttaattctggtattttcttcttcccactggatggtaaggttgcatgtacacgtcacagctgaagttcaggcagcaagaacactggacttggagtcagaaggccttggttcagaatcaactcctcctctttgagtttctgtttcttcctcagtaaaattaggcttcatttatcatgcaataaacatgtattgagtatgattgtgttcaggccctgtggctgggtgctagaggcccaaacacctgtactgcttctctcagagtggtaatgagaggatcaattcctaaatgcataaaaatataacaggaaatggaattccaggcactgagctgtgctttctgcagtttcattaagtagaggaaatgaaactggattcattgcaaagcaagtggtataatacggtggctaagaactcacgctcagtagccaaattgcctaagttgaaatcctggctccaccagaatttgggggatgttgctgaacctctcttcaattcagtttcctctgcctgtaaaatgggagtaagaactgtagatctcctcatgtggttgttgtgaggatttaatgagttattatgtgtaaaacacttaaagcagagtctagcacatagtgctcaatatacattagctattattgttattattatttgggacgtacaacacatcagaccacatgtttctaacacagacatgaccaagttgatatcagagagtgatctggttgtgataattttctctctattcgtggccaagcttcattcctgtcatctggccaatgaagtcaatgtccactcacttacttgctggtccatgaacatcctcctaaggctttctaactagaggagggagcctcagaaacaactactagaaactccagaccagccctccaggtccatgtggagaagaagatggggtagtcagctccctactaggaactactgattctgtccattatttcaagaggtataatgtgtttatcttattgctccaatcatgcatagcttcattcccaaaatctttacatggtctgtgatggctgtcagatttccagtcattctatttacgtttaaaattttttctaagtgatttatgcaatctgggtaaattaaggaaatggtccttatattgagcatttgtgtttagccaatattttgtatttttaaaacattttttgagatggagtcttgctctgttgcccaggctggagtgcaatg

SEQ ID NO: 15135 - RNA, 2822 nt, Homo sapiens
  source 1..2822: mol_type = other RNA
gctgggattacaggcatgagccactgcacctggccaagggtcactgttaaaagctaatagaacactcctctgtcatccctagaaggggccatgtggagccctacaatcaccaacagtagactgcgttcacatttgaatagccccagattctacgagcctcatctctaattctcaattgctaacaccaggtataatctacgaaattcctcaggctgctttcacataacctgtctttaggctgtgtgagtaaggctgagagagaagcagaaggtggggccatgttcccaggcactttctgagaacacccgaagcccatcttctgtgtgtgtgaaagctggggcttggctgccccgaacagaactagtgtttttaatccaagtctccacatttcagactgtttaaatgtctggcccaaacacaagtaaaaacaaaataaaacaaagccccgttcgtgtactcggcacacgtgtcgggagggaagatgaaccttaataatatggagcttgggtaagaggttgcagtcagccagcgtcagctcgtccccatccagaaacttccttccagaaacagtgacatcctcggtgctgtaggcatctatttcatcaggcagagggctatttaagtaattatccagcttcctcagggccttcagcaggttcttttcatgaatctcatttgcatccttcttcgtgttttttataaacgctgagaatttggcaaacacgtcatttcctgcggaattagattcgggatgttgggtccccagcttgggatacctcgggggagctaatttctcctctaagaactcctcgatcttattcacatccgtcttgacttcaccatcaaaagtcatgaaaggagggtttgttccgggagccaggttctgcaggtctgcgggtttccttttcaggtccactgtggtcacattaaatataacgcctttcagccagagaatcataaagagacgctgagaaaacgggcaatttccgatactctcaccatcataaccagccttgacgaagagggtgatgtcgtgctcctgccccagggcccggggctcggacgcctctccgtcctcccggcggccgttcacgcgcgcggcctcgccgctaccctcggcggggccctcctcggccaggtggttgctgagctgggcctcaggctccgcggcgcccctggaggcctccccatgtgggctgctgtcgggggattcctcttcgccccccgctgcttcctcctcccttggcccctccgggctccgctctcgtctctcttcgtcctcccccggctcctgctgtggcccatcccctaccctgtcctcgccagcgtctgcccttgcgtccccgggggccgcttcttcggacccctttacccccgggacctccgcctcctccgctgcgtcccaggcgagctcaccggggctgcgccccgcactctccccggctgcgacctcaattgcctcggcctggggcgagaggctgccgtcccccgattgctgcggctcacccgagacccggcgcgcccttcctgccggaccctcggcgtccatgctgtcccccgccgggccttcggcttctacgctgtcccccgccgggacccccgcttctacgccgtcccccgccgggtcccccgcctctacgctgtcccccacccggccctccgcgtctacgctgtcccccgccggaccttccgcgtctacgctgtcccccacccggccctccgcgtctacgctgtcccccgccgggccctcggcttgtatgttgtcccccagcgggccctccgcgtctacgctgtcccccgccggaccttccgcgtctacgctgtcccccacccggccctccgcctctacgctgtcgcccgccgggccctccgcttctatgttgtcccccagcgggccctccgcgtctacgctgtcccccgcctccccggacgcgctaccttccgggacctcaggcctctgctccgcctcctcctgcctctcgggggccgcagagtcctcgggctccctctgagcctccccgcggggctcgccctgcgcgccgcgtcccgggctcgccccctccacctgctgcgcgccgcttgtctcctcccctccttggggcacctcggcaccctccggggctccctcctcggcctcagtctcgccgtgcgcccccctcgtgccccgcgcctcggcctccgggcccctgtctggcccgccgcctcctgcctccttcacagcggcggcgcccctcggcgcctcctctgcgccctcgctcccctccggcccttctgcctccccgcccgcggctcctggctctccgggtctctcagccagaggcgcggggacctccggcggcccctggggacccggggcaaccccctccggctccgcggcctcggccatggccgcagatccctgtccttgatcgggactccttccttgacgctgcttaagggtcggtggcgctgggcaaggggcgtgctacggggccctctgtgctccttgaaggacgccggctccgggatcctgcggcaaaggtttagccggggcactggggccttgcgcaggacccgcagggcaaactccgcttggccccaagcctctgcgccccttctgcccagctgaaactccctggactcttcctccactgctggagcttctccccgattgcgcgtctgcttcccaccgggaccccaatctcgcccgcgggccgcggaggtgcagtgcacggctggagagggctgcttcgctcctgcgcctttggaagtgcccggcccgctgtccgctgtcctggggttgaccagaagtccttggtgccaactccatcccctggggcttg

SEQ ID NO: 15136 - RNA, 1513 nt, Homo sapiens
  source 1..1513: mol_type = other RNA
gctgggattacaggcatgagccactgcacctggccactttagcaagttttgatgcaactatgtttatatatgccactttacaaccaagattcctggtacccctaatctcttctagtcttaatttactactgaagttcattacatcatgttaattattaacatatttattttgtttttcaacatatctgaagttggagaaattgttgtcaaaagaatcttctcagatctatcagaactgcctgcctgccaattcagaataaaggtagtcactgaatggattctgtctaagattttcacgaccaaagtcttaattatttcagatcaagcttcaatgagcaaaatgtttagttttagagatgtaccttcttcacgcaaagcactggactccaaccatattagtcagcttgggcttctagaacaaaattccgtagactgggtggcttaaacaacagaagtttatgttttcatggttctggagaccggaagtccaattctggcaagggttctctcttaggcttgcaataagctgccttcatactgtgtcttcacatggcagagagagagagcaagcaggcactctggtgtgttttcttataagggcactaatcccatcataagggcctcatcctcatgacctcatctaaccttaattaattcccaaagatcccatctccaaatatcatcacattggagcttagagcttcaacagataaattttgggagcacacaagtcagttcatagcaccacctaaagagcaggttgggcaaattcccaaaattacaacagagattcctacaggctttccataccaaaccaaaaacagtatatggcacatagtagttgttcaataaatacttgttgaataagttgaaaaaaatgaacaaatgtccgtaactcaagaaaagactaagggaaaaggaaatttgaatgaggcagggatctaatcccaaagtggacatctcatatttgggtgaaacagcaaatctccttgacaatattaatgtccctggcaattcaaatatcttcaaaggaaaatgatgtggaataaaattaaatgattttaaacaaaattatatttcaccagcttatagttgcatctcagtaaatgcccattcttttccaagagcgggctatttccattttctagaaatcctgtctcttctgtgggaattatctctaaaattgtgttcagtttggatgtcatggttagtccaggtcctctgccttcttgatgaggtccctgaggtttgttttgccagatccttcttctcatagcctcagtacatccagtgagcaggcacgtgtcccaggatcagccaatcaggcatccacttaggactctgtctgctgaaaacagtggatgtttgagtgggtaaagcctttttttctatggtacaaaatctggtccaattgtgtctatctgagacagtcctcaaatgctaagttaacagccatctaggatcacacagctaaggaaggcttcccgccgctgcctcccctgcctttcctgct

SEQ ID NO: 15137 - RNA, 2408 nt, Homo sapiens
  source 1..2408: mol_type = other RNA
gctgggattacaggcatgagccactgcacctggccaggagagtttttttctgataatagaagtaatactttctcactttagaaaatgtgaaaagttcagatatataaggaagtcaaacaaaacgtctcctatatatgaagaagaaaagaagcaagtttaaaaaaaaagaaaaaaaaaggtcttctatcgtttctccactcaaagacagctgttaacattttattgacttctatggagtttgccctatgcttctgttttatgtaatagagacagtgctgtagtgaatagcttcacgtcaaaatttttctataattttctgaagttagagtcttaattattggatcaaaggaagtgaacatttttaaacctcttgatacatatattaccaaattgttttcttttccgttttttttaataaatagagatgggggtctctctgtgttgcccaggctggtcttgacctcctggcctcaagcaatcctcttccctccacctcccgagtagctaagattataggtgtgagccaccatgctcagccgctgattttaacttgtatgttttaaacaaaatttctagtaaagtagaacatttctttgatatgtttgtgtcaggatttgactctcccaggtctttggagaggctttctaacaagacatcccccgtgggtggccatctgccctgtgagaaggtcatttctagttccaggtcacgcacagtgtgtcagctggtggggtgtggagtttcaggcccaggcctcctggaaagtgcccgaaagagaaacggcttagaaaataaggactttaacggtggtgtgggttgagtttggaaagtttagaccatgttagtggaatcagagctgggaagaggttctagaagttacctcctctcactggtttccagtccacacttctcagaactctcccattttgcagtcaggtgcagtggctcacatctgtaatcctagcacttgaggagaccgagatgggcagatcacttgaggccaggagtttgagaccagccctggccaacatagcgaaaccccgtttctactaaaaatacaaaaattagccaggtgtggtgtggtgcacacctgtagttccagctactcaggaggctgaggcatgagaatcacttgagcctgggaggcagaggttgcagtaagccaagatcgcaccactgcactccagcctgtgtgatggaaggagactctgtctcaaagaaaagaactcacctattttgcaaaggagcttcatggttctcttgaagaaaaataggaatggaggccacctctgtgtcaaaaacaacgtcccacatttctgtgtttcactttttttttttttttttttgagactgagtttcactcttattgcccaggctggagtgcaatggcgcgatctcggctcactgcaacctccacctcccgggttcaagcgattctcctgcctcagcctccctagtaggtgagattacaggcatgtgccaccacgcccggcaaattttgtatttttagtagagatggggtttctccatgttggtcaggctggtctcaaactcccgacctcaggtgatccgtgcctggcctacttttttttttctttttctttttctttttcttttctttctttcttttctttttttttttttaagagatagggtcttgctatgttgcccagactggtctcaaacgcctggcctcaagtggtcctcccaccttggcctcccaaaacgctgagattacaggtgtgagccaccacgcttggcctgttttacatgttgacggacagcatataatcacatgtataagggtttctgcttgtaaaagtctggaaacccattctaactgccagaatcacagaacctagagaaggggacataactgccctgtggccacccagtagctttcatcttctctcgggacggcagaggcaggacagccagcattctggtgaggattgaaggattagttgtaacagatttcagcaggtctgcagtgatcagatgggtttctcacatattgttaagttgaaagtagccgtggctcagtatgagttgagtacctgtttaaaatctgcattcaaagccttcttcccagaggccacaactgcagtgagatccaagtgtgtggctcacccgccccggggctcacagctgggcagggtgatttccactcaaattcttgtgccagtgcagatcttgttctaaagcttttctaaatgcctggagactagaaagacttttggatacttttccctttttcttttggatgaaattgcatctccagtagaacagcagcattccatggtgcctcagccacgatcctctggacagagatttgtggcgaagacctgacgagagactgtaaaggaaaagcagggtttgtttttcctggtcaaagttgttaatactaa

SEQ ID NO: 15138 - RNA, 1950 nt, Homo sapiens
  source 1..1950: mol_type = other RNA
gctgggattacaggcatgagccactgcacctggccagtatttatgtttttaaagtggttttgtgtccttggatatgagctcccttcatgtggagactgagtcttatacctgtttgtgtttcagcatctctcctgattcctgatcctcgtgctggccatgggagtcaagtatttatgttctaaataccaggcccgctcctgaaacaccagcttggttccatacaacagacaaaactcggtgagtgtgtgccagggacagagaagccacgtggtgcagacacgagttccaggcatggaaaaaatcctccttcttggtctttaccttataataaattctggccaccaaaccccgctgaagaaccctttcacgaaatttcactgctttcaacagaaaggcgagatcatcaactgtgtccatgttaaatgccaggaaactggttctcagcttgtcccccacagattcagcccagttttggagcaggccaaagagtggtttttcttcatactgtttggtgtattgggccagcagttcccgccccacaacctgaagcataacaacatcgtcaccttcaaaagtggcaaacacatctgtgtcacactttaagcctgagattcgattttccatcatgtaacccatgcctccagtgcactcgcggcagtcctgcaggcagcggatgttctcccaggtgctgtaggccttcagccccgccaccagagcctgcagcgagcgactgttgaccagctcctttccctggaagacatcctcatccaggagggccccagcatacctgctgacgaaggtcagggccaaggctgtggccaggtggggcatcagccgcagggtctgtgtttggtgctcaatgatcttcacctcttccttggttttgggcccaaactgcctccggctgtggctatagcgaatggctatcgtcaacccaagcttcatggcacccatagcttggaaagccacagctaatctcgaaggggtcagtgctgccagcatggcattgaatcttgcactcttgttcctaataggcgaatggtactgtccatctggagccacggaaccaaacttatccagcaggttctccctgggtatccgaaccttgtcaaatattaatatcccattgtccacaccatgcagaccctccttgtacatcatatcaatagctgtgactcctgggtacaagcttccgttttcatcccggacaggaacgatgaaacagtggggcccttgagatcttccatctatgatgagctgggcaaagacagctgcataattcccgtacatggcatttccaatatacatcttctccgcattttcacacggcgtgtcaattacaaactcctgggcagagaggtcaaaggtggcttcggtctggatccctctcgcgttgctcccatggcccctctcggtcattgcaaacatcccagtgtatttctgctcctggagtggctgaaaccacttagtaacatgttcagggcttccgagattcctgatagcaccaccaaatagccaataaattattccgcacttcactcctgtggccatgtccgccatggagaggacttctcctatgacaaggcttcggctgacaaaattctttgttttctctgccagatcctgacctgcacgttttaacagaggcaggtccatggcaaacttcactctctgaactgtcaaagctctcatttcatccaagcttaaatcatacctttgccggaagagcgggcgccgccgaggagtccgcgcagctcgttcttgaggctccagaagtcgccgtccaggtagcggtgcagggaggagtccccgagccccagacccggcgccggctgcatcgcgctcacctgcctctgcttctccgcgtggctggcagggccggcttcgctccgcgcctcctccagctcccagcaggtgaggccccaggcgcacgccctctccctctccacc

SEQ ID NO: 15139 - RNA, 1931 nt, Homo sapiens
  source 1..1931: mol_type = other RNA
gctgggattacaggcatgagccactgcacctggccagtatttatgtttttaaagtggttttgtgtccttggatatgagctcccttcatgtggagactgagtcttatacctgtttgtgtttcagcatctctcctgattcctgatcctcgtgctggccatgggagtcaagtatttatgttctaaataccaggcccgctcctgaaacaccagcttggttccatacaacagacaaaacttcattaacaaagtctggtcctcttggtcaggacagctcttcactgctagggagaactgctctaaggtaactcggtgagtgtgtgccagggacagagaagccacgtggtgcagacacgagttccaggcatggaaaaaatcctccttcttggtctttaccttataataaattctggccaccaaaccccgctgaagaaccctttcacgaaatttcactgctttcaacagaaaggcgagatcatcaactgtgtccatgttaaatgccaggaaactggttctcagcttgtcccccacagattcagcccagttttggagcaggccaaagagtggtttttcttcatactgtttggtgtattgggccagcagttcccgccccacaaccatgcctccagtgcactcgcggcagtcctgcaggcagcggatgttctcccaggtgctgtaggccttcagccccgccaccagagcctgcagcgagcgactgttgaccagctcctttccctggaagacatcctcatccaggagggccccagcatacctgctgacgaaggtcagggccaaggctgtggccaggtggggcatcagccgcagggtctgtgtttggtgctcaatgatcttcacctcttccttggttttgggcccaaactgcctccggctgtggctatagcgaatggctatcgtcaacccaagcttcatggcacccatagcttggaaagccacagctaatctcgaaggggtcagtgctgccagcatggcattgaatcttgcactcttgttcctaataggcgaatggtactgtccatctggagccacggaaccaaacttatccagcaggttctccctgggtatccgaaccttgtcaaatattaatatcccattgtccacaccatgcagaccctccttgtacatcatatcaatagctgtgactcctgggtacaagcttccgttttcatcccggacaggaacgatgaaacagtggggcccttgagatcttccatctatgatgagctgggcaaagacagctgcataattcccgtacatggcatttccaatatacatcttctccgcattttcacacggcgtgtcaattacaaactcctgggcagagaggtcaaaggtggcttcggtctggatccctctcgcgttgctcccatggcccctctcggtcattgcaaacatcccagtgtatttctgctcctggagtggctgaaaccacttagtaacatgttcagggcttccgagattcctgatagcaccaccaaatagccaataaattattccgcacttcactcctgtggccatgtccgccatggagaggacttctcctatgacaaggcttcggctgacaaaattctttgttttctctgccagatcctgacctgcacgttttaacagaggcaggtccatggcaaacttcactctctgaactgtcaaagctctcatttcatccaagcttaaatcatacctttgccggaagagcgggcgccgccgaggagtccgcgcagctcgttcttgaggctccagaagtcgccgtccaggtagcggtgcagggaggagtccccgagccccagacccggcgccggctgcatcgcgctcacctgcctctgcttctccgcgtggctggcagggccggcttcgctccgcgcctcctccagctcccagcaggtgaggccccaggcgcacgccctctccctctccacc

SEQ ID NO: 15140 - RNA, 1987 nt, Homo sapiens
  source 1..1987: mol_type = other RNA
gctgggattacaggcatgagccactgcacctggccagtatttatgtttttaaagtggttttgtgtccttggatatgagctcccttcatgtggagactgagtcttatacctgtttgtgtttcagcatctctcctgattcctgatcctcgtgctggccatgggagtcaagtatttatgttctaaataccaggcccgctcctgaaacaccagcttggttccatacaacagacaaaacttcattaacaaagtctggtcctcttggtcaggacagctcttcactgctagggagaactgctctaaggtaactcggtgagtgtgtgccagggacagagaagccacgtggtgcagacacgagttccaggcatggaaaaaatcctccttcttggtctttaccttataataaattctggccaccaaaccccgctgaagaaccctttcacgaaatttcactgctttcaacagaaaggcgagatcatcaactgtgtccatgttaaatgccaggaaactggttctcagcttgtcccccacagattcagcccagttttggagcaggccaaagagtggtttttcttcatactgtttggtgtattgggccagcagttcccgccccacaacctgaagcataacaacatcgtcaccttcaaaagtggcaaacacatctgtgtcacactttaagcctgagattcgattttccatcatgtaacccatgcctccagtgcactcgcggcagtcctgcaggcagcggatgttctcccaggtgctgtaggccttcagccccgccaccagagcctgcagcgagcgactgttgaccagctcctttccctggaagacatcctcatccaggagggccccagcatacctgctgacgaaggtcagggccaaggctgtggccaggtggggcatcagccgcagggtctgtgtttggtgctcaatgatcttcacctcttccttggttttgggcccaaactgcctccggctgtggctatagcgaatggctatcgtcaacccaagcttcatggcacccatagcttggaaagccacagctaatctcgaaggggtcagtgctgccagcatggcattgaatcttgcactcttgttcctaataggcgaatggtactgtccatctggagccacggaaccaaacttatccagcaggttctccctgggtatccgaaccttgtcaaatattaatatcccattgtccacaccatgcagaccctccttgtacatcatatcaatagctgtgactcctgggtacaagcttccgttttcatcccggacaggaacgatgaaacagtggggcccttgagatcttccatctatgatgagctgggcaaagacagctgcataattcccgtacatggcatttccaatatacatcttctccgcattttcacacggcgtgtcaattacaaactcctgggcagagaggtcaaaggtggcttcggtctggatccctctcgcgttgctcccatggcccctctcggtcattgcaaacatcccagtgtatttctgctcctggagtggctgaaaccacttagtaacatgttcagggcttccgagattcctgatagcaccaccaaatagccaataaattattccgcacttcactcctgtggccatgtccgccatggagaggacttctcctatgacaaggcttcggctgacaaaattctttgttttctctgccagatcctgacctgcacgttttaacagaggcaggtccatggcaaacttcactctctgaactgtcaaagctctcatttcatccaagcttaaatcatacctttgccggaagagcgggcgccgccgaggagtccgcgcagctcgttcttgaggctccagaagtcgccgtccaggtagcggtgcagggaggagtccccgagccccagacccggcgccggctgcatcgcgctcacctgcctctgcttctccgcgtggctggcagggccggcttcgctccgcgcctcctccagctcccagcaggt

SEQ ID NO: 15141 - RNA, 2070 nt, Homo sapiens
  source 1..2070: mol_type = other RNA
gctgggattacaggcatgagccactgcacctggcccacagtcgtattttaaagacattgagcaaccctgctgggggaaaccagttgaactgtctttaacttggtatctcctgaacataccaggccactagatctcattttttgcacaatgcttgctgacctgtggcagactgcttttggaaaaatgttgatctagtgaaggcacaatcaagaccttgattgcaggcagggaggacagcttcttccacggcaggttagaagctgctaagacaaatacgagatcttctgagcgtgccagcccatccatctgcaccagtaactctgtcttcatccgcaggcttccttcatgttctcccccagaagctgtgcctctctgactcatcaccgactccagctcgtccaggaagatcgtggatggggcgtggtagcgggcaagctcaaataacacccgaacgagtttttctgaatcccctctccatttgctgacaatggtggatgcagaaatgttaaagaaggttgttttacattcagtggccacagctttggccagtaaagtctttcctgtacctggagggccgtacagcagtagtcctttccagggagaaagaattcctgtaaatagctgtggataccttataggatacacaacagcttctttgactaactgcttggctgcatcaagtccaataatgtcattccactttatgtttggattatggagataaatgtcccggctcaccacggctgccaattctcgcatctcactgttcatgccaataaatgcactcagaggtttcagcagtcgttctgaggggtctggattatggtcgaaggtgttcaaggcaagttcactggttgctcccttgatggcatctgtgagcagcccttggaagtcaatgatttggcctcttcgtgggtgggcattttcctctccactgtctttacggattcttgatatatgtaggccgaagttggcactttccaggcgagtgttatcaactacctcctgattaggatgctccttattgagcgatttggtgtcccctgtcttccccgctgtggttttggaccggggcctctgctgattgatcttgggaagattttgacaactgtcgttcatcatccttctggtcttccctctacttctttgcggtaaattattttctgctgtgtctgatgactttttgacaattttggggtatttctgaaattttacaaaataataactctcatattccatcaaaatagtttcaagatcaatgttgtcacaaacttcaaaccgtcgtaaccccagtttagtttcttgctccaaagcatttgctgtatcgatatacccttcttgtgttaaataatgcgaaatcaaaatgagaagattttttcgtcgtgcttctgtcctcatctcgcacgcttcccgcgcctgatgcgtgaatttcagggtctggtaggaaagctccatcagacactgtgctaggaccctgttctcattagacgtggaaaaacatggacgtgttttcctctgctctatttttttcatgtgttaactagtctgtttcttcaatgtctttcccttctgtctctcttgctgtgaatcctattccaaattatcccttcatcattatcttcggtcttcttcatccatttcttcttcatccatttctcccttcaggatacaaaaatattcaagtttcctcaatccaacacccatatttagattattccgccacaactactctgggggatggttttatttgcggcggctttctccgtccataggcaccgcgtgaagggcaccgtaagaatcttcccgaatgctcctgtcacgcgtcccggccgcctcttcttcctccccgccacttcccgaggccaggcccgcggataacgcctcagttgcgacccagctctaggcagtccgcaggggcctccgccggggagggaaggcacgacctggggccgagcggggccaagccgcggggcagcacgccggggcaggcgcgggcgggcgctgtcgccgcgcggactgaaggcgcgggcggaaggcggtcgcgcgggtgggcagggggcaccgctaggg

SEQ ID NO: 15142 - RNA, 2096 nt, Homo sapiens
  source 1..2096: mol_type = other RNA
gctgggattacaggcatgagccactgcacctggcccacagtcgtattttaaagacattgagcaaccctgctgggggaaaccagttgaactgtctttaacttggtatctcctgaacataccaggccactagatctcattttttgcacaatgcttgctgacctgtggcagactgcttttggaaaaatgttgatctagtgaaggcacaatcaagaccttgattgcaggcagggaggacagcttcttcctggagcccaaaaatgcatgtggttacacggcaggttagaagctgctaagacaaatacgagatcttctgagcgtgccagcccatccatctgcaccagtaactctgtcttcatccgcaggcttccttcatgttctcccccagaagctgtgcctctctgactcatcaccgactccagctcgtccaggaagatcgtggatggggcgtggtagcgggcaagctcaaataacacccgaacgagtttttctgaatcccctctccatttgctgacaatggtggatgcagaaatgttaaagaaggttgttttacattcagtggccacagctttggccagtaaagtctttcctgtacctggagggccgtacagcagtagtcctttccagggagaaagaattcctgtaaatagctgtggataccttataggatacacaacagcttctttgactaactgcttggctgcatcaagtccaataatgtcattccactttatgtttggattatggagataaatgtcccggctcaccacggctgccaattctcgcatctcactgttcatgccaataaatgcactcagaggtttcagcagtcgttctgaggggtctggattatggtcgaaggtgttcaaggcaagttcactggttgctcccttgatggcatctgtgagcagcccttggaagtcaatgatttggcctcttcgtgggtgggcattttcctctccactgtctttacggattcttgatatatgtaggccgaagttggcactttccaggcgagtgttatcaactacctcctgattaggatgctccttattgagcgatttggtgtcccctgtcttccccgctgtggttttggaccggggcctctgctgattgatcttgggaagattttgacaactgtcgttcatcatccttctggtcttccctctacttctttgcggtaaattattttctgctgtgtctgatgactttttgacaattttggggtatttctgaaattttacaaaataataactctcatattccatcaaaatagtttcaagatcaatgttgtcacaaacttcaaaccgtcgtaaccccagtttagtttcttgctccaaagcatttgctgtatcgatatacccttcttgtgttaaataatgcgaaatcaaaatgagaagattttttcgtcgtgcttctgtcctcatctcgcacgcttcccgcgcctgatgcgtgaatttcagggtctggtaggaaagctccatcagacactgtgctaggaccctgttctcattagacgtggaaaaacatggacgtgttttcctctgctctatttttttcatgtgttaactagtctgtttcttcaatgtctttcccttctgtctctcttgctgtgaatcctattccaaattatcccttcatcattatcttcggtcttcttcatccatttcttcttcatccatttctcccttcaggatacaaaaatattcaagtttcctcaatccaacacccatatttagattattccgccacaactactctgggggatggttttatttgcggcggctttctccgtccataggcaccgcgtgaagggcaccgtaagaatcttcccgaatgctcctgtcacgcgtcccggccgcctcttcttcctccccgccacttcccgaggccaggcccgcggataacgcctcagttgcgacccagctctaggcagtccgcaggggcctccgccggggagggaaggcacgacctggggccgagcggggccaagccgcggggcagcacgccggggcaggcgcgggcgggcgctgtcgccgcgcggactgaaggcgcgggcggaaggcggtcgcgcgggtgggcagggggcaccgctaggg

SEQ ID NO: 15143 - RNA, 1392 nt, Homo sapiens
  source 1..1392: mol_type = other RNA
gctgggattacaggcatgagccactgcacctggcccactttaactattttaaagggtacaattcagtggcgttcagtgcagtcatgaggttgtgcagccaccacctgtatctcatttcagaatatgcccatcactccaaaaggaaaaccctatccccacgatccgtggttccccagccccctggcccccagccctaagcagccactaagctgccttctgtctctacggattgccggttttgggtatttcatgtcgatgggatcagtgtgtggccttgtgtctggcttctgtctccaggcatatgttgtcaagggctatcattccttttcttggccaaataatgctccatgttgtggacacatcgtattttgtttatccgttcacctgctgatgcatgccagatggttgtttccaactttttaattcccattataaagataaggaaactggccaggtgcggtggctcaagcctgtaatcccagcactttgggaggccaaggcgggtgcatcacctgaggtcgggagtttgagaccagtctgacccacacagcgaaaccccgtctctactaaaaatacaaaaaatcagctgggcgtggtggtgtgagcctgtaatcccagctactcagaaggctgaggcatgagaatcacttgaacctgggaggcgaaggttgcagtgagctgagatcgcgccactgcgcttcagcctgggagacagagactctgtctctaaataaataaataaacaaacaaataaataaatgtaaactgaggctaaaccgctccactcagggtcaacacctgccctgtgacccagcagttccacttttcggtatttatctaggagaaatgagaacacatgtccacacaaagacctgtgcacaaatgttcacagcatctttctctgtaataacttcgagctggcaacgatccaaatatccatccacaggagctgggtaaacaaaccgtggtgtcatcctggagtgggacgctcctcatcaggaaagaggaaagaatgacccatgcacgcagcagcttggaagagtctcaaaaacaagatgccaatgaaggaagccaggcacgggactgcaactgtaagctgtgactctgtgtgactccagcggtacgaacttccaggaaaagcaaaaatatgggacagagtatccacaagtggcattcagggactggagtgggaactggctcctcccgcgtcctgattgacctttacttaaagaccagctccagccgctgatgggtttcggcgggtcccccaggagacccttcagacggctagagccgggcgcgctgcagagagcccctaattggggcaatgaatcatcgcgcgcggctccggctggacacaaaatagatagaggagccggccgctattgtgcg

SEQ ID NO: 15144 - RNA, 4957 nt, Homo sapiens
  source 1..4957: mol_type = other RNA
gctgggattacaggcatgagccactgcacctggccgaaaacagtttttttatcggcaaattaggctttggttccaggtttcattcctctgaatatcagcaaccaaaacattttaacaatatgcaagtataggcaacctcaacccaagtagagaggatgaaatgtaaattctagtgacatcttaaatgtttctacagatggctaccaaaagcagaatctcttgtttggatggatgggacaagtacaaaccagaacataattcaaggattcgctaactgcatgcataacgttccagaactgtttacatccacatatggacagaaatcgctggtaaaggtcaaatcctgttatccctccttctgagggattttccagaatctttggctggaattatattttttgctgtgttggtgttggctaattataacatcttaagcatgtactcattactctgtcacaggttattagacacctataatagtctcaacttaagcctgccttgggagaagggcaagagagattaaaaataaataacttggccaagtgcagtggctcacgcctgtaatcccaacactctgggaggctgaggctgaaggattgcttgagcctggagtttgagaccagcctgggcaacacagtgagaccctctctctagaaaaaaatttaaaaaattagcagggtgtggtgatgcatacctatggtctagctactcaggaggccaaaatggaaggataacttgagcccaggagtgggaagcttcagtaagctatcatcaaactgcactctggcctggatgactgtctcttaaaaaagaaaaaaggaaaaaaataaagactgaccaagatactgtgattttactgctattattcataaggctggatagaaagggcaaatactggctaaaaaacaaacaagaacaaatacaagcagcaattaacatttctggaattccagacccaagttctaaaaggatgtcaaaattcaggaagcctacacttgattataatcacctataagacagaaatcacctataagacagaaatctagactttctactgagcaactgctttgttgtgataatggaaaggtattttccatgtcaccaaatgggagagctctaccaacagaaaagcaacactggcagcttatggagctaacaataaagctaagttacatatatctatataggataatatagatataataaaatatatatgcattttaaatatacatattaaacatgtacatacttaatatatgtctaaaagcatcccactccaacagatgccctacacatagggtttgcttctcataaatatttaaaattgtttagaaactgggaacagattgaaaaatgattttgtacttttgcagtttactttttttttttttaagatggctgtttcataaattagttccctattcctaactttggagaacctggttttttcttacctttcaaggtccaaatataaaactataaactttcagtgttggacattcttgctttttgaaagcaaattcctcctcaattcatgacctgtgggccagctatcatgaataatacacccatagcacttgggttttatgaatgtgacttctaaatcctcctgcataatagctttaggtgacttgaagagttaaaagctgtcattgtcatcaatatttactgtacatcaaactcatttaaaatgctgttagaaattgctgactggcaagactgtcactgacaaaaacaccagtttaggacagattccatgggaaacaaactagaataactgaaagctaaaatagagcttaatggtagagaaagtctcagaaacaaggacagagatcacagaaaagacaaggaaggactcctattgttttttctgattttgaagagctctttgtgcttacctatttatcctaaacaaaaaggcatgagtaaaaatttccaatgtattacaaagggtattctgtctaatgtcaggctggctctcaggatgttataaacctgcccaggtattagacttctgatgagactgtgccttaaggacaggaatggcactttcctactaaaaactactgccatctggggagcaaagactggggatagaaaactacaagaacaaacctgtctagttatgactttgtgatccagaagcctcttgacctatggtactagagcaggtgcaacattctttccctctctccactgagccacataaagaagtctacagcacttccaatgtaaatcccaacttcaccgcttcatctcttggagaatgcacagtccaaatgtataacccctaaaacaggagagtaattaagttttggagctactttacagtacagttcaatacatacttattgcattccaagaatacttcatatctgcaagaaagcctgaaaccgtattttcttctttttgactctgtccagctacaagctctgctgcagtgtgtatatacaaatgccattagcttcaaaggaggaataatatctaccttctcaattaatcactactaagactcagaccattgggaacacatactcctttctgatttttagatacttctgcaaaagccatcgcttcatacacactatagaagagaaggttttcttcttcctttttgcaatattctccgttggttagggaatccctcacagtgggattgcactgagccagcagaacctggattccaatggcttcataatctctgcgaacttctttcagtgtgtggatccctgctgtatctaaaaattgaattgcactgcagtcaatcactatagtatgcagctccaagggatcatgggaaagttgcactgacatttcatcctggattccaccaagagtcactactttttctttgatctttctctttgctgccttcttccaagccacctttattaagattgggttgacagtttgtttgtataaagcagatttaaagcattctttgtttatgtagtagagaggggctacaaagcggaaaatcttgatgcctggcttaatctgaaggttcttgtaagcagacacagattcaaagacctcagactcttccaccaagccaagcagtgaactctttggcttctgagtgcggaggatgacacaaaatatagaaaaacaaaccccaacaagtaggcctatttcagtacttagcagtgcagaggacagcatagtaacaaaccagataactgtatccattctactaatactccacattttgggaagatccctaaatttacgaagggctccccgtagatttacaattgtgatcacaccaaggacacttttttgaagggaatagaacaaaggagctattactaggaggaccaacaaaagaaccagggctgttaccacaccagaaagctgagtatggcagcctgttgattctttaaccaatgtctttgcaagagctgcactagtagtaaaacagtggaagaaggaagggatgatattacaaaagccaatggcatacatttcctggtttgctttgactgtgtaaccatgtttcttggcaaacatctcagaaagtgatacagtgatagcaaaaccaatgatggaaatagctattgcatctacagccacactaggaattaggttccattctggtactttgggtggcataaacccagtgggaatatgtccagcaatactagaattataattttcatgtagttttccaaaatgagaggctaatgtggctgctacaacaacaacaagttcaataggaatcggtgccttaagcttggatttgaagtgttcattgagttctttggttggcaaaagaaccaaaaggcacaaaaggctggtgataagatcacagagattggtcttatggatgtttctgaagacatgtatccaggtagtgatgagtgagcccacaccattagtccgaggaaggttgagcccaagaagatacttggcctgagatgtaagaatagtgaaggaggcaccagtgacaaatccactcagcaaggcatctgagaggtagacagaaacaaaacccacttgaaagaagcccatcgctacctgataaactccagctataaaggttacagtgctgccaaccataattgcatagcaacttttgtcacatatcctgtctgatgtatgatttaataatgtgctcccatttgaaaccattcctaaggaaggagcactatgggcattgtcatagccagctttctgtagttctcggtcaactgtctcaccaatcataaggcacagtactccaaaaatgcccacagagatgtgacgggaggtacccaagagaaaataaatgatgctggcaaaaaaagatgtgtacagaccatagacaggttcttggccagccagcagggaataagcaatggactggggcaccaataatatgcccacaatcaagcctgacatcacatcccctaaaatgtttttctttaggtcgtattttgggagccactgcaaaacaggaaggaaacctaaaatcatatttttggctttggctggactgcactggcaattcttctgcagctttttaataacaaactccttgaagtttgtatctgatttctcttgacgctcaataaggatcctatgataaggtctgcattgatcattggtctcaaattgcttgaagtcagtacttgattccctttgaagttccagatggatcccagatggataactgtcatttccttcagctgagtctctgggtgaaacgttatgttgctctttactttctgaagacatttctggagatagatggttcagcttcctctcgggtccgggccgctgcaggcaaccaggcgccgcggcacgcgtcttccaccgtggcctgactgaggtggacaccgcggcgccgacagagctatacctgcctgtccctttccccgcccatcgctcggactccgaaggaggcggggcccggctgccgggacctacgggcgcggcgaggacgcaccggcgaagagatgccggaggcagagccagt

SEQ ID NO: 15145 - RNA, 5066 nt, Homo sapiens
  source 1..5066: mol_type = other RNA
gctgggattacaggcatgagccactgcacctggccgaaaacagtttttttatcggcaaattaggctttggttccaggtttcattcctctgaatatcagcaaccaaaacattttaacaatatgcaagtataggcaacctcaacccaagtagagaggatgaaatgtaaattctagtgacatcttaaatgtttctacagatggctaccaaaagcagaatctcttgtttggatggatgggacaagtacaaaccagaacataattcaaggattcgctaactgcatgcataacgttccagaactgtttacatccacatatggacagaaatcgctggtaaaggtcaaatcctgttatccctccttctgagggattttccagaatctttggctggaattatattttttgctgtgttggtgttggctaattataacatcttaagcatgtactcattactctgtcacaggttattagacacctataatagtctcaacttaagcctgccttgggagaagggcaagagagattaaaaataaataacttggccaagtgcagtggctcacgcctgtaatcccaacactctgggaggctgaggctgaaggattgcttgagcctggagtttgagaccagcctgggcaacacagtgagaccctctctctagaaaaaaatttaaaaaattagcagggtgtggtgatgcatacctatggtctagctactcaggaggccaaaatggaaggataacttgagcccaggagtgggaagcttcagtaagctatcatcaaactgcactctggcctggatgactgtctcttaaaaaagaaaaaaggaaaaaaataaagactgaccaagatactgtgattttactgctattattcataaggctggatagaaagggcaaatactggctaaaaaacaaacaagaacaaatacaagcagcaattaacatttctggaattccagacccaagttctaaaaggatgtcaaaattcaggaagcctacacttgattataatcacctataagacagaaatcacctataagacagaaatctagactttctactgagcaactgctttgttgtgataatggaaaggtattttccatgtcaccaaatgggagagctctaccaacagaaaagcaacactggcagcttatggagctaacaataaagctaagttacatatatctatataggataatatagatataataaaatatatatgcattttaaatatacatattaaacatgtacatacttaatatatgtctaaaagcatcccactccaacagatgccctacacatagggtttgcttctcataaatatttaaaattgtttagaaactgggaacagattgaaaaatgattttgtacttttgcagtttactttttttttttttaagatggctgtttcataaattagttccctattcctaactttggagaacctggttttttcttacctttcaaggtccaaatataaaactataaactttcagtgttggacattcttgctttttgaaagcaaattcctcctcaattcatgacctgtgggccagctatcatgaataatacacccatagcacttgggttttatgaatgtgacttctaaatcctcctgcataatagctttaggtgacttgaagagttaaaagctgtcattgtcatcaatatttactgtacatcaaactcatttaaaatgctgttagaaattgctgactggcaagactgtcactgacaaaaacaccagtttaggacagattccatgggaaacaaactagaataactgaaagctaaaatagagcttaatggtagagaaagtctcagaaacaaggacagagatcacagaaaagacaaggaaggactcctattgttttttctgattttgaagagctctttgtgcttacctatttatcctaaacaaaaaggcatgagtaaaaatttccaatgtattacaaagggtattctgtctaatgtcaggctggctctcaggatgttataaacctgcccaggtattagacttctgatgagactgtgccttaaggacaggaatggcactttcctactaaaaactactgccatctggggagcaaagactggggatagaaaactacaagaacaaacctgtctagttatgactttgtgatccagaagcctcttgacctatggtactagagcaggtgcaacattctttccctctctccactgagccacataaagaagtctacagcacttccaatgtaaatcccaacttcaccgcttcatctcttggagaatgcacagtccaaatgtataacccctaaaacaggagagtaattaagttttggagctactttacagtacagttcaatacatacttattgcattccaagaatacttcatatctgcaagaaagcctgaaaccgtattttcttctttttgactctgtccagctacaagctctgctgcagtgtgtatatacaaatgccattagcttcaaaggaggaataatatctagccacttggttaaaatttcaagtgtgcaaaatttcccactgtggaactgggaaatgttggacacttgaaattttaacctattggctagacattcttctatctaccttctcaattaatcactactaagactcagaccattgggaacacatactcctttctgatttttagatacttctgcaaaagccatcgcttcatacacactatagaagagaaggttttcttcttcctttttgcaatattctccgttggttagggaatccctcacagtgggattgcactgagccagcagaacctggattccaatggcttcataatctctgcgaacttctttcagtgtgtggatccctgctgtatctaaaaattgaattgcactgcagtcaatcactatagtatgcagctccaagggatcatgggaaagttgcactgacatttcatcctggattccaccaagagtcactactttttctttgatctttctctttgctgccttcttccaagccacctttattaagattgggttgacagtttgtttgtataaagcagatttaaagcattctttgtttatgtagtagagaggggctacaaagcggaaaatcttgatgcctggcttaatctgaaggttcttgtaagcagacacagattcaaagacctcagactcttccaccaagccaagcagtgaactctttggcttctgagtgcggaggatgacacaaaatatagaaaaacaaaccccaacaagtaggcctatttcagtacttagcagtgcagaggacagcatagtaacaaaccagataactgtatccattctactaatactccacattttgggaagatccctaaatttacgaagggctccccgtagatttacaattgtgatcacaccaaggacacttttttgaagggaatagaacaaaggagctattactaggaggaccaacaaaagaaccagggctgttaccacaccagaaagctgagtatggcagcctgttgattctttaaccaatgtctttgcaagagctgcactagtagtaaaacagtggaagaaggaagggatgatattacaaaagccaatggcatacatttcctggtttgctttgactgtgtaaccatgtttcttggcaaacatctcagaaagtgatacagtgatagcaaaaccaatgatggaaatagctattgcatctacagccacactaggaattaggttccattctggtactttgggtggcataaacccagtgggaatatgtccagcaatactagaattataattttcatgtagttttccaaaatgagaggctaatgtggctgctacaacaacaacaagttcaataggaatcggtgccttaagcttggatttgaagtgttcattgagttctttggttggcaaaagaaccaaaaggcacaaaaggctggtgataagatcacagagattggtcttatggatgtttctgaagacatgtatccaggtagtgatgagtgagcccacaccattagtccgaggaaggttgagcccaagaagatacttggcctgagatgtaagaatagtgaaggaggcaccagtgacaaatccactcagcaaggcatctgagaggtagacagaaacaaaacccacttgaaagaagcccatcgctacctgataaactccagctataaaggttacagtgctgccaaccataattgcatagcaacttttgtcacatatcctgtctgatgtatgatttaataatgtgctcccatttgaaaccattcctaaggaaggagcactatgggcattgtcatagccagctttctgtagttctcggtcaactgtctcaccaatcataaggcacagtactccaaaaatgcccacagagatgtgacgggaggtacccaagagaaaataaatgatgctggcaaaaaaagatgtgtacagaccatagacaggttcttggccagccagcagggaataagcaatggactggggcaccaataatatgcccacaatcaagcctgacatcacatcccctaaaatgtttttctttaggtcgtattttgggagccactgcaaaacaggaaggaaacctaaaatcatatttttggctttggctggactgcactggcaattcttctgcagctttttaataacaaactccttgaagtttgtatctgatttctcttgacgctcaataaggatcctatgataaggtctgcattgatcattggtctcaaattgcttgaagtcagtacttgattccctttgaagttccagatggatcccagatggataactgtcatttccttcagctgagtctctgggtgaaacgttatgttgctctttactttctgaagacatttctggagatagatggttcagcttcctctcgggtccgggccgctgcaggcaaccaggcgccgcggcacgcgtcttccaccgtggcctgactgaggtggacaccgcggcgccgacagagctatacctgcctgtccctttccccgcccatcgctcggactccgaaggaggcggggcccggctgccgggacctacgggcgcggcgaggacgcaccggcgaagagatgccggaggcagagccagtgtaaac

SEQ ID NO: 15146 - RNA, 939 nt, Homo sapiens
  source 1..939: mol_type = other RNA
gctgggattacaggcatgagccactgcacctggcctaaacccctaattttagtaggtcagggaaatagatttgaaactgttctcctatctccttggctgtagcaacagactaaagccttcttcactgacaatacttattgtctcagtgattggctttctgtgctgggagtagtgggacttagaccaaagccctattttggtaacaatttcagtcatgtgagcccctgggtggagaatccagctatactgtacctgacttaaactgtgagataataaagatgtgtcgttttaatctaatttgtggtaatgtattacacagaaataaaataagtatagcctgaaactaatatgcctatcagtatacctaccttatccttcaaaaccagtctcacccctttaagaggtggccttgagctccaagacggattctgctgtgcccccttgatgctcctagggctctttttttgggggtgggaggacagggtctcactctgtcacccaggctagagtgcagtggtttgatcatggctcactgcagcctcaaactcctcaagcaaccctcctgcctcagcctcccaagtagcagggaccacatgtgcaagctaccacatccagctaattttttaaatttttttgtagagatgaggtctcactatattacccaggctagtctcaaactcagggtcaagcgatcctcccaccttggcctcccaaagggctgagattgcaagagtgagccactgcaccctgcctttggctccttgttagtttttctcttatcttgttgttttactggtttttgtttgtttgtttgttagaagtgtctttctcttctgttagaccatttgatccttcagggtgaggactatgtcttagtgtattagtctgttttcatgctgctgataaagacatacccatgactgggtaatttataaagaa

SEQ ID NO: 15147 - RNA, 8024 nt, Homo sapiens
  source 1..8024: mol_type = other RNA
gctgggattacaggcatgagccactgcacctggcctaatttttgtatttttttttttagcagagataggattttgccatgttgcccaggctggtctcaaactcctgagcccaagtgatccacctgccttggcctcccgaagtgctgggattacaggcatgagccaccatgccccaccaagacaaacaaaacaaaacaaaacaaaacaaaacaaaacaaaaacagtatagatgaaaggcagccagcctgggttcaaatcctaccgttgctacttattattaaataaacgtaagaatcttatggacgttactttacctctctagcaccttgactttcaaatctgcaaaacaggataataacacctatttctttataacattgttataaggattaagtaggttaatatatgtgaaatacttagagtaatgtctggtacacagtaggcactaaataagtgttagcagccaggtgcggtggctcacaaggtcaggagtttgtgaccacactggccaacatagtgaaaccctgtctctactaaaaatataaaaattagctgggcatggtggcgtgtgcctgtagtcccagctactcgggaggctgaggcaggagaatcacttaaacccggaaggcggcggttgtggtgagctgagatcgcaccactgcactccagcccaagcaacagagcgagactccgtctcaaaaaaaaaaaaaaaaaaaaaagtatagctactattataatcctgtgaaaataatcaatataaaattaaaaatcaacagacagcccatattgcccttttttggcctaacaaaaaacagatttctaagaagacagtaagaaatcagtattaatttaaacattgtacaggacaggagatcaaaagcacaggtatacaaatggttcatttaaaaaaactgatactcaaattgacaccctgaaaatgtcagataatttttcagaatgattaaactcactaaacatctgtaaacaataaatttatttcatttcttttaaagatttaatgatatacaaaacgtatatagtatctttaagtaatacactttttctttctccccacccccaatcaatattaaacactatttaaacagcttatcatctcttgccttgtctgtatctatgagatacactactaaatacaaataagctttatactgctcccttccaaataaaaattaaaattagtaccaaggaaacaaaagaaaaagaaaaaaaaagaaaaaaaattaaagcataaaacttagatgaaaagcttttcttgttattgttgaatattcaacaatatctggggctgttaaattacattttattggcataaggttgcactgcaatctgccagtatcacataatgataatccaactgaattaatttcttaagtaccacaaacagcattcatgttcaaatgttccaacacaattttaaatatatgcaagagttcatgtttacattctgatttgatataacaatcaataaaatctttggagaagtttgtaagttctgggttgttgctatagatacagatagggaaaaaagtactttaactttcctcaaaaggtaacttcccttgacgagtgagttaggtttctgcttttataatttaggttatgtatcagtttaccatggctttcttctacttaacagtgacttgataaaacaatgtttaaaaaacccaattaacatttttacacaatttgggttctatttaaaaaaaaaaactggctctatctttaaatatggagcctaaccctgattcataaataccgtccctcttgaaaatggtcttcagttcaggcttctcatacctctgtgaacctagaattagaacaagtcatttcccttcccgtggccaacaagcatctagttgggaaccagtgatatcatcactgaacacactaaatacactgaggaaaattttgactgccatttaaccaaaaggctgcgtgatttcttcatttccctagttgaatggcaataaaacagctgccaataaaatctgcatggacacctacctttggttaatggtattgtaccacataagagagagcatcaccctcatcaaaacaaagtcaaatgagatcctctgctatacaaagagccctttaaaaagttataaatactaattatcaattacctttaaaatttctcagctgccagctctatcctatagggactttctgactgattaatcaggtcaaaagaatattgaccttttaactgtgctggagtcagcaaattcaacttgcatacacctttctatattaccaaacaatttcctcccgagggaaaagtgacacagtaacatttctgtgaggtgcaggcaaaaccaatgattcagtaatattaatattataacatcagacgaacagaattagttgattctgattctttggtggaatttccaggctgaagattcaaatctgaaggctcatcctgaggaaatataattttatcaggcgtataatcattcctcttcagatctggaagtttaagctttctacagcaagaattacagtgatgttttgctctgaagtttttaattgcatcttctcctagatttgctgggccaaaaaccatatcacaggatctcttttcttctgcttttatcacagatgggtcagtcaaattttcaccaacaccttgcaaatcaagtaccagtaactcccctcttgtatattcgtaagtccagtggctaaaggctagcatgatctcttccagagtattagttggaataatctcatctccattattattgttgtattttctaaattctccagtcatacattcttccacagcaaaccactgtcctgctgaatggcaatacagcaggaaaacttcaaggaaccttggagaatatggtatggatttgggtttcatttgattaaaggcaaacgtaagcttttgtgctgctctctgttgttgaatttctctcagacagagatgcagaactgtatcttctttgtaaatacttgaccatgtattaaccacctctggaagaaaagatttgataatataaagatgccctgatttgaggatatcatgttctgaccaggtacactgtactttgacagctcttcgtaaacctcctcccatctcctctttgcttaaaaactctattttggcacagaggcctagttgtgaccaagaagacatgctgttatttagtatgttgggtgaactctcttccaaacgatacactgtgacaggctcccctcttggaggcacaggtgtaaatggaatgctctgtgataacctcatcaagttatttctttccacagctgaataatagtaatttgtatccatagctggcttaaatggagaagtgagaccatttaatgttccttcttcagatggcatttctctgtttgatggtctatcttgtaaccaatccggtattaaagctgctttggaatctacttcatgagtgtcttcggtagatggccttctactgattttttctgcttgttttgaatgaacaggaatggaagttctgtgacagtcagtaaatccagcaagagaactcactcgtttcaaagtgttttcagaagtattgttattggatagtatttttatcttgtttgatgtttctttaaacctctgtaaatccatgctatctctgtgtcctacaaatgctccaaattctgtattatctccttctgtagctttagagcaaacagtttcttgatctttggttccagtttccaagtggcttttgcaacttggctgagatggtgtactaacaaaaaatttggttggtggggatgacagatgtggtatgctagtagatgaactgcctaatttttgatttttattaaatatttttaagagttctaccccatgtagtctctgtcgcagttctggaggggaaacagcacttgggaataaggcaccagaagaggaaccagcctctggaaaattaaattcttttctctggggtactgcaggtaagtcttgaccaaatatattacactggggatctttgtcatctttcattaaaatattacaatgaaaaggattattactttcaagatcaccttgaggaagagaggagctaagtgtatttacaacaccatgctttttccatacagaaggtcttacaggaccatcatcaataaggttttgagccaagtgtttggaaatgctcagttctcgtgtgatttcattatgaactttgctagcttccgacgctttctgggcagtgagtgtttttaatgtatctaccgtcagggctgaaagatcttgcaaatggccaatttgagaatctaatgattgtaatgatctttttatgtagttgacacgatctccaacttctttaatctgaatgcacatctgttccactctttcaaaagtgacacgaattctctcttcactcccagaatgaaatttgtcatctttttcattgaaatacatttcaacacactgctcttcaaaatcatgaagtttcttttgatcttcttctgttaagaaaagttttggtccatcggaagtcttatctttctttcttctcttacatatgcagcaaaacagagaaactatatggctaagaatgataagtggaggaggcagaactggtttctcatgataagccataataaaatgataacgctggtacttccatacaatattggaaattgccttcacttgtaaatacacattgcatcaatttcgtatgcataaacttcaccaaaaatcatccagtatgggtgaaaaactatatctttagcaagagtccaagatggtgcttcatgaggataaagtattgcctttctgggaacaccaaaactaagtaatacaagagccataatcactacaatgtagaacatattggccaccaaaatattatgttaagacagtaaattaatcttccagccacaaaaacatgattatcatatgcatttgcaaagttccattttgctccaaatcttagtccaaatccaatgaagaaagaaattatggcaattgtatcactgatgttgaagtaatcactaaaccatactttaatcttctggtttactttcccagcttcagacataaagatctcacggactttctcaatggcataagtaaaaatataagcaataacaatccattcttgaactgaaggtaactgttccatttgtacaagaaccacaaatgtataaagcatcagaaatcctaaatatgccaacgtgttaaaccagaattttacaattggtgcatgataaaaggcataaaactttcgcgtaattggaagcttttttgatttcatttgtatctccatctcattctttccttcattactatccaaaatccgtacttctttaaacacttccatggggatctcttctgttatgttctgaaagttgttttcgctgtcatccattgtcatctgatgagcatcttgagattgtgggatatgggacatttcagccttagttttatactctaacagcaatatggcaggtggaactaaaatgcttagtatgaccttgtaccaggaatttttcctcatattcagccttcccatccacatatcagataacaacatttgtgtacaggtgtgagctacaaaaggtctaagtcttgaagaaactgctaacttaaggcaggttgaattactccagttcttcagttcataagtgagcaatttcatagccatggtttcatcttgtctgaaggactgttctaataattcaacggccaactgaccaaaatcattggaatactgttttagttcttctgaagtatcatctaccaggtcactctgctttgcttcatatgccattgaacgatagatcttacaggcaactaatgctttagccattgattcttcaccatgttgccataaaaaacgggccatgacctgcctcttcataaggcaagcccaaattaaaagttcattaagtggataaggaaagcgcttggtttctggatcatcaatgtctacaatttcatctttggttcttttcttctttccttcttccataactgtatcaatctttggtcggtagggctgtgctgtcttaatgaaatggttatgcctcattttttcctttttatctgccctattgccaaaagattcatgactctttcgcaactgaggagtgctgctggaggtatttcggccagacctccgattatttccaccaagactattatatattaatcgaaaacgtttcctagtataggtgcatctgtaggttcctcccatgagatattcaataacaagtcctatatcaatcagagtgatcttatatcctggaggaagatttccctgtttgacgtctcgaacaagatgaaacagcattggattagttggaccttgtttagtgttgtaaagttcttccagtctcggaatggtaaggaatttatgcatgcttactccattttcaataagaagttttacaaatgcaactctatccattacaagagcatcaagcatagcttgttccaaggatccaaccagccactgctgtccataaacaaatacatgatttttggcaatgtcaactctatcccatgccaatgtaaggataagctggtcaaatgcagatgcattagtaccttttagcagtgcagtaagtattgctacatctatatcttgatgttcatctgacccaatatggaaaacagtgataagctcctttcttttcatgcactccatcagtgtttgaaataaatgaagtgcttcattctggccaaagttaaatgtttttttgatagtggaaataatatcgggctctgctgcatcaggaagattccctccttcttctgtttgtttatgaatatacgctagcagatctgcagctctgcctgttccttcacacacaactactggaacaggggggctttcctgaaggtattcaagaactgtgaggataacatttggcccaccctcaaatataagtgccaccacagggacaccctggccaatcctagcatgaattctttgctgattaatagttttttcaagttctcttctcagtctgacttccgccccatactttccaacagtgccatcatccaccaatatgaaatgggaatgcagattattcaaaacattcaatttgctcagggggttcaataaggtttgataaggagcaaccacatctctcccaacaagatcatttctgttttcaatcactccccatggagctattccgatagtgcaaatctttcgagatgatctggaagcatgttctttgagggcatctccaacatgttttgccacacctgtgtttactcctccagttaaaatccaggctccagttgtaactgcagctttaataagaccttttccaagcaactgcttgattcgtgggtgaagctcaaatttctgcatgcccccatgtacagagataacaagtttgggtaactccatttgccattctttaagcagaagttgcagaatgacttcaggtttggtgtcatatgatagcctcacatacttagctctgtaggaatgagaacccccttgaaaatttatgactccataagcatccgttgggctctgttctgtatgcttttccacagaccattcttctattgcctgattaaaatggtcacccaatttcacatctgagtatttcatggcaagacttgcagtaaaacaagcatgttgcttgaccaagcgaccacaaaaacacctgacgagttgctgacaaatttgacatcctggaaggcatctgtgagggtccttggaacttggtataatatatacacattccctcttggtcaaagtgctttctatccaggatttctgggacattctcctcacggggcggactccggaagggcagcaactccacctcctcctcctccgcggcctgtagccatctatcgggaagcgtctccggaggcggcagcagaggccgccggacaaggaacgcccagggaaaccttctcagaactaactcagctccggcgctagcagcagaagccgagtctttcataattgtgcgaccaactcctccgggtgactggccacagggacgcgcccgcgcccgcctccgccggcgacggggctggggac

SEQ ID NO: 15148 - RNA, 8097 nt, Homo sapiens
  source 1..8097: mol_type = other RNA
gctgggattacaggcatgagccactgcacctggcctaatttttgtatttttttttttagcagagataggattttgccatgttgcccaggctggtctcaaactcctgagcccaagtgatccacctgccttggcctcccgaagtgctgggattacaggcatgagccaccatgccccaccaagacaaacaaaacaaaacaaaacaaaacaaaacaaaacaaaaacagtatagatgaaaggcagccagcctgggttcaaatcctaccgttgctacttattattaaataaacgtaagaatcttatggacgttactttacctctctagcaccttgactttcaaatctgcaaaacaggataataacacctatttctttataacattgttataaggattaagtaggttaatatatgtgaaatacttagagtaatgtctggtacacagtaggcactaaataagtgttagcagccaggtgcggtggctcacaaggtcaggagtttgtgaccacactggccaacatagtgaaaccctgtctctactaaaaatataaaaattagctgggcatggtggcgtgtgcctgtagtcccagctactcgggaggctgaggcaggagaatcacttaaacccggaaggcggcggttgtggtgagctgagatcgcaccactgcactccagcccaagcaacagagcgagactccgtctcaaaaaaaaaaaaaaaaaaaaaagtatagctactattataatcctgtgaaaataatcaatataaaattaaaaatcaacagacagcccatattgcccttttttggcctaacaaaaaacagatttctaagaagacagtaagaaatcagtattaatttaaacattgtacaggacaggagatcaaaagcacaggtatacaaatggttcatttaaaaaaactgatactcaaattgacaccctgaaaatgtcagataatttttcagaatgattaaactcactaaacatctgtaaacaataaatttatttcatttcttttaaagatttaatgatatacaaaacgtatatagtatctttaagtaatacactttttctttctccccacccccaatcaatattaaacactatttaaacagcttatcatctcttgccttgtctgtatctatgagatacactactaaatacaaataagctttatactgctcccttccaaataaaaattaaaattagtaccaaggaaacaaaagaaaaagaaaaaaaaagaaaaaaaattaaagcataaaacttagatgaaaagcttttcttgttattgttgaatattcaacaatatctggggctgttaaattacattttattggcataaggttgcactgcaatctgccagtatcacataatgataatccaactgaattaatttcttaagtaccacaaacagcattcatgttcaaatgttccaacacaattttaaatatatgcaagagttcatgtttacattctgatttgatataacaatcaataaaatctttggagaagtttgtaagttctgggttgttgctatagatacagatagggaaaaaagtactttaactttcctcaaaaggtaacttcccttgacgagtgagttaggtttctgcttttataatttaggttatgtatcagtttaccatggctttcttctacttaacagtgacttgataaaacaatgtttaaaaaacccaattaacatttttacacaatttgggttctatttaaaaaaaaaaactggctctatctttaaatatggagcctaaccctgattcataaataccgtccctcttgaaaatggtcttcagttcaggcttctcatacctctgtgaacctagaattagaacaagtcatttcccttcccgtggccaacaagcatctagttgggaaccagtgatatcatcactgaacacactaaatacactgaggaaaattttgactgccatttaaccaaaaggctgcgtgatttcttcatttccctagttgaatggcaataaaacagctgccaataaaatctgcatggacacctacctttggttaatggtattgtaccacataagagagagcatcaccctcatcaaaacaaagtcaaatgagatcctctgctatacaaagagccctttaaaaagttataaatactaattatcaattacctttaaaatttctcagctgccagctctatcctatagggactttctgactgattaatcaggtcaaaagaatattgaccttttaactgtgctggagtcagcaaattcaacttgcatacacctttctatattaccaaacaatttcctcccgagggaaaagtgacacagtaacatttctgtgaggtgcaggcaaaaccaatgattcagtaatattaatattataacatcagacgaacagaattagttgattctgattctttggtggaatttccaggctgaagattcaaatctgaaggctcatcctgaggaaatataattttatcaggcgtataatcattcctcttcagatctggaagtttaagctttctacagcaagaattacagtgatgttttgctctgaagtttttaattgcatcttctcctagatttgctgggccaaaaaccatatcacaggatctcttttcttctgcttttatcacagatgggtcagtcaaattttcaccaacaccttgcaaatcaagtaccagtaactcccctcttgtatattcgtaagtccagtggctaaaggctagcatgatctcttccagagtattagttggaataatctcatctccattattattgttgtattttctaaattctccagtcatacattcttccacagcaaaccactgtcctgctgaatggcaatacagcaggaaaacttcaaggaaccttggagaatatggtatggatttgggtttcatttgattaaaggcaaacgtaagcttttgtgctgctctctgttgttgaatttctctcagacagagatgcagaactgtatcttctttgtaaatacttgaccatgtattaaccacctctggaagaaaagatttgataatataaagatgccctgatttgaggatatcatgttctgaccaggtacactgtactttgacagctcttcgtaaacctcctcccatctcctctttgcttaaaaactctattttggcacagaggcctagttgtgaccaagaagacatgctgttatttagtatgttgggtgaactctcttccaaacgatacactgtgacaggctcccctcttggaggcacaggtgtaaatggaatgctctgtgataacctcatcaagttatttctttccacagctgaataatagtaatttgtatccatagctggcttaaatggagaagtgagaccatttaatgttccttcttcagatggcatttctctgtttgatggtctatcttgtaaccaatccggtattaaagctgctttggaatctacttcatgagtgtcttcggtagatggccttctactgattttttctgcttgttttgaatgaacaggaatggaagttctgtgacagtcagtaaatccagcaagagaactcactcgtttcaaagtgttttcagaagtattgttattggatagtatttttatcttgtttgatgtttctttaaacctctgtaaatccatgctatctctgtgtcctacaaatgctccaaattctgtattatctccttctgtagctttagagcaaacagtttcttgatctttggttccagtttccaagtggcttttgcaacttggctgagatggtgtactaacaaaaaatttggttggtggggatgacagatgtggtatgctagtagatgaactgcctaatttttgatttttattaaatatttttaagagttctaccccatgtagtctctgtcgcagttctggaggggaaacagcacttgggaataaggcaccagaagaggaaccagcctctggaaaattaaattcttttctctggggtactgcaggtaagtcttgaccaaatatattacactggggatctttgtcatctttcattaaaatattacaatgaaaaggattattactttcaagatcaccttgaggaagagaggagctaagtgtatttacaacaccatgctttttccatacagaaggtcttacaggaccatcatcaataaggttttgagccaagtgtttggaaatgctcagttctcgtgtgatttcattatgaactttgctagcttccgacgctttctgggcagtgagtgtttttaatgtatctaccgtcagggctgaaagatcttgcaaatggccaatttgagaatctaatgattgtaatgatctttttatgtagttgacacgatctccaacttctttaatctgaatgcacatctgttccactctttcaaaagtgacacgaattctctcttcactcccagaatgaaatttgtcatctttttcattgaaatacatttcaacacactgctcttcaaaatcatgaagtttcttttgatcttcttctgttaagaaaagttttggtccatcggaagtcttatctttctttcttctcttacatatgcagcaaaacagagaaactatatggctaagaatgataagtggaggaggcagaactggtttctcatgataagccataataaaatgataacgctggtacttccatacaatattggaaattgccttcacttgtaaatacacattgcatcaatttcgtatgcataaacttcaccaaaaatcatccagtatgggtgaaaaactatatctttagcaagagtccaagatggtgcttcatgaggataaagtattgcctttctgggaacaccaaaactaagtaatacaagagccataatcactacaatgtagaacatattggccaccatttttccaatcatcattacataaggtcctgcctgttgatttacagctagaaaatctagcaaacgcacataccaaaatattatgttaagacagtaaattaatcttccagccacaaaaacatgattatcatatgcatttgcaaagttccattttgctccaaatcttagtccaaatccaatgaagaaagaaattatggcaattgtatcactgatgttgaagtaatcactaaaccatactttaatcttctggtttactttcccagcttcagacataaagatctcacggactttctcaatggcataagtaaaaatataagcaataacaatccattcttgaactgaaggtaactgttccatttgtacaagaaccacaaatgtataaagcatcagaaatcctaaatatgccaacgtgttaaaccagaattttacaattggtgcatgataaaaggcataaaactttcgcgtaattggaagcttttttgatttcatttgtatctccatctcattctttccttcattactatccaaaatccgtacttctttaaacacttccatggggatctcttctgttatgttctgaaagttgttttcgctgtcatccattgtcatctgatgagcatcttgagattgtgggatatgggacatttcagccttagttttatactctaacagcaatatggcaggtggaactaaaatgcttagtatgaccttgtaccaggaatttttcctcatattcagccttcccatccacatatcagataacaacatttgtgtacaggtgtgagctacaaaaggtctaagtcttgaagaaactgctaacttaaggcaggttgaattactccagttcttcagttcataagtgagcaatttcatagccatggtttcatcttgtctgaaggactgttctaataattcaacggccaactgaccaaaatcattggaatactgttttagttcttctgaagtatcatctaccaggtcactctgctttgcttcatatgccattgaacgatagatcttacaggcaactaatgctttagccattgattcttcaccatgttgccataaaaaacgggccatgacctgcctcttcataaggcaagcccaaattaaaagttcattaagtggataaggaaagcgcttggtttctggatcatcaatgtctacaatttcatctttggttcttttcttctttccttcttccataactgtatcaatctttggtcggtagggctgtgctgtcttaatgaaatggttatgcctcattttttcctttttatctgccctattgccaaaagattcatgactctttcgcaactgaggagtgctgctggaggtatttcggccagacctccgattatttccaccaagactattatatattaatcgaaaacgtttcctagtataggtgcatctgtaggttcctcccatgagatattcaataacaagtcctatatcaatcagagtgatcttatatcctggaggaagatttccctgtttgacgtctcgaacaagatgaaacagcattggattagttggaccttgtttagtgttgtaaagttcttccagtctcggaatggtaaggaatttatgcatgcttactccattttcaataagaagttttacaaatgcaactctatccattacaagagcatcaagcatagcttgttccaaggatccaaccagccactgctgtccataaacaaatacatgatttttggcaatgtcaactctatcccatgccaatgtaaggataagctggtcaaatgcagatgcattagtaccttttagcagtgcagtaagtattgctacatctatatcttgatgttcatctgacccaatatggaaaacagtgataagctcctttcttttcatgcactccatcagtgtttgaaataaatgaagtgcttcattctggccaaagttaaatgtttttttgatagtggaaataatatcgggctctgctgcatcaggaagattccctccttcttctgtttgtttatgaatatacgctagcagatctgcagctctgcctgttccttcacacacaactactggaacaggggggctttcctgaaggtattcaagaactgtgaggataacatttggcccaccctcaaatataagtgccaccacagggacaccctggccaatcctagcatgaattctttgctgattaatagttttttcaagttctcttctcagtctgacttccgccccatactttccaacagtgccatcatccaccaatatgaaatgggaatgcagattattcaaaacattcaatttgctcagggggttcaataaggtttgataaggagcaaccacatctctcccaacaagatcatttctgttttcaatcactccccatggagctattccgatagtgcaaatctttcgagatgatctggaagcatgttctttgagggcatctccaacatgttttgccacacctgtgtttactcctccagttaaaatccaggctccagttgtaactgcagctttaataagaccttttccaagcaactgcttgattcgtgggtgaagctcaaatttctgcatgcccccatgtacagagataacaagtttgggtaactccatttgccattctttaagcagaagttgcagaatgacttcaggtttggtgtcatatgatagcctcacatacttagctctgtaggaatgagaacccccttgaaaatttatgactccataagcatccgttgggctctgttctgtatgcttttccacagaccattcttctattgcctgattaaaatggtcacccaatttcacatctgagtatttcatggcaagacttgcagtaaaacaagcatgttgcttgaccaagcgaccacaaaaacacctgacgagttgctgacaaatttgacatcctggaaggcatctgtgagggtccttggaacttggtataatatatacacattccctcttggtcaaagtgctttctatccaggatttctgggacattctcctcacggggcggactccggaagggcagcaactccacctcctcctcctccgcggcctgtagccatctatcgggaagcgtctccggaggcggcagcagaggccgccggacaaggaacgcccagggaaaccttctcagaactaactcagctccggcgctagcagcagaagccgagtctttcataattgtgcgaccaactcctccgggtgactggccacagggacgcgcccgcgcccgcctccgccggcgacggggctggggac

SEQ ID NO: 15149 - RNA, 8174 nt, Homo sapiens
  source 1..8174: mol_type = other RNA
gctgggattacaggcatgagccactgcacctggcctaatttttgtatttttttttttagcagagataggattttgccatgttgcccaggctggtctcaaactcctgagcccaagtgatccacctgccttggcctcccgaagtgctgggattacaggcatgagccaccatgccccaccaagacaaacaaaacaaaacaaaacaaaacaaaacaaaacaaaaacagtatagatgaaaggcagccagcctgggttcaaatcctaccgttgctacttattattaaataaacgtaagaatcttatggacgttactttacctctctagcaccttgactttcaaatctgcaaaacaggataataacacctatttctttataacattgttataaggattaagtaggttaatatatgtgaaatacttagagtaatgtctggtacacagtaggcactaaataagtgttagcagccaggtgcggtggctcacaaggtcaggagtttgtgaccacactggccaacatagtgaaaccctgtctctactaaaaatataaaaattagctgggcatggtggcgtgtgcctgtagtcccagctactcgggaggctgaggcaggagaatcacttaaacccggaaggcggcggttgtggtgagctgagatcgcaccactgcactccagcccaagcaacagagcgagactccgtctcaaaaaaaaaaaaaaaaaaaaaagtatagctactattataatcctgtgaaaataatcaatataaaattaaaaatcaacagacagcccatattgcccttttttggcctaacaaaaaacagatttctaagaagacagtaagaaatcagtattaatttaaacattgtacaggacaggagatcaaaagcacaggtatacaaatggttcatttaaaaaaactgatactcaaattgacaccctgaaaatgtcagataatttttcagaatgattaaactcactaaacatctgtaaacaataaatttatttcatttcttttaaagatttaatgatatacaaaacgtatatagtatctttaagtaatacactttttctttctccccacccccaatcaatattaaacactatttaaacagcttatcatctcttgccttgtctgtatctatgagatacactactaaatacaaataagctttatactgctcccttccaaataaaaattaaaattagtaccaaggaaacaaaagaaaaagaaaaaaaaagaaaaaaaattaaagcataaaacttagatgaaaagcttttcttgttattgttgaatattcaacaatatctggggctgttaaattacattttattggcataaggttgcactgcaatctgccagtatcacataatgataatccaactgaattaatttcttaagtaccacaaacagcattcatgttcaaatgttccaacacaattttaaatatatgcaagagttcatgtttacattctgatttgatataacaatcaataaaatctttggagaagtttgtaagttctgggttgttgctatagatacagatagggaaaaaagtactttaactttcctcaaaaggtaacttcccttgacgagtgagttaggtttctgcttttataatttaggttatgtatcagtttaccatggctttcttctacttaacagtgacttgataaaacaatgtttaaaaaacccaattaacatttttacacaatttgggttctatttaaaaaaaaaaactggctctatctttaaatatggagcctaaccctgattcataaataccgtccctcttgaaaatggtcttcagttcaggcttctcatacctctgtgaacctagaattagaacaagtcatttcccttcccgtggccaacaagcatctagttgggaaccagtgatatcatcactgaacacactaaatacactgaggaaaattttgactgccatttaaccaaaaggctgcgtgatttcttcatttccctagttgaatggcaataaaacagctgccaataaaatctgcatggacacctacctttggttaatggtattgtaccacataagagagagcatcaccctcatcaaaacaaagtcaaatgagatcctctgctatacaaagagccctttaaaaagttataaatactaattatcaattacctttaaaatttctcagctgccagctctatcctatagggactttctgactgattaatcaggtcaaaagaatattgaccttttaactgtgctggagtcagcaaattcaacttgcatacacctttctatattaccaaacaatttcctcccgagggaaaagtgacacagtaacatttctgtgaggtgcaggcaaaaccaatgattcagtaatattaatattataacatcagacgaacagaattagttgattctgattctttggtggaatttccaggctgaagattcaaatctgaaggctcatcctgaggaaatataattttatcaggcgtataatcattcctcttcagatctggaagtttaagctttctacagcaagaattacagtgatgttttgctctgaagtttttaattgcatcttctcctagatttgctgggccaaaaaccatatcacaggatctcttttcttctgcttttatcacagatgggtcagtcaaattttcaccaacaccttgcaaatcaagtaccagtaactcccctcttgtatattcgtaagtccagtggctaaaggctagcatgatctcttccagagtattagttggaataatctcatctccattattattgttgtattttctaaattctccagtcatacattcttccacagcaaaccactgtcctgctgaatggcaatacagcaggaaaacttcaaggaaccttggagaatatggtatggatttgggtttcatttgattaaaggcaaacgtaagcttttgtgctgctctctgttgttgaatttctctcagacagagatgcagaactgtatcttctttgtaaatacttgaccatgtattaaccacctctggaagaaaagatttgataatataaagatgccctgatttgaggatatcatgttctgaccaggtacactgtactttgacagctcttcgtaaacctcctcccatctcctctttgcttaaaaactctattttggcacagaggcctagttgtgaccaagaagacatgctgttatttagtatgttgggtgaactctcttccaaacgatacactgtgacaggctcccctcttggaggcacaggtgtaaatggaatgctctgtgataacctcatcaagttatttctttccacagctgaataatagtaatttgtatccatagctggcttaaatggagaagtgagaccatttaatgttccttcttcagatggcatttctctgtttgatggtctatcttgtaaccaatccggtattaaagctgctttggaatctacttcatgagtgtcttcggtagatggccttctactgattttttctgcttgttttgaatgaacaggaatggaagttctgtgacagtcagtaaatccagcaagagaactcactcgtttcaaagtgttttcagaagtattgttattggatagtatttttatcttgtttgatgtttctttaaacctctgtaaatccatgctatctctgtgtcctacaaatgctccaaattctgtattatctccttctgtagctttagagcaaacagtttcttgatctttggttccagtttccaagtggcttttgcaacttggctgagatggtgtactaacaaaaaatttggttggtggggatgacagatgtggtatgctagtagatgaactgcctaatttttgatttttattaaatatttttaagagttctaccccatgtagtctctgtcgcagttctggaggggaaacagcacttgggaataaggcaccagaagaggaaccagcctctggaaaattaaattcttttctctggggtactgcaggtaagtcttgaccaaatatattacactggggatctttgtcatctttcattaaaatattacaatgaaaaggattattactttcaagatcaccttgaggaagagaggagctaagtgtatttacaacaccatgctttttccatacagaaggtcttacaggaccatcatcaataaggttttgagccaagtgtttggaaatgctcagttctcgtgtgatttcattatgaactttgctagcttccgacgctttctgggcagtgagtgtttttaatgtatctaccgtcagggctgaaagatcttgcaaatggccaatttgagaatctaatgattgtaatgatctttttatgtagttgacacgatctccaacttctttaatctgaatgcacatctgttccactctttcaaaagtgacacgaattctctcttcactcccagaatgaaatttgtcatctttttcattgaaatacatttcaacacactgctcttcaaaatcatgaagtttcttttgatcttcttctgttaagaaaagttttggtccatcggaagtcttatctttctttcttctcttacatatgcagcaaaacagagaaactatatggctaagaatgataagtggaggaggcagaactggtttctcatgataagccataataaaatgataacgctggtacttccatacaatattggaaattgccttcacttgtaaatacacattgttgaaaaatgcaataagaagattaaccataatgatatactgtacaaagaggtagactgcttgaagaaatggagtcaaccacgtcccaggaccacagatttgagggataacagaatcatttgcacacacatcaatttcgtatgcataaacttcaccaaaaatcatccagtatgggtgaaaaactatatctttagcaagagtccaagatggtgcttcatgaggataaagtattgcctttctgggaacaccaaaacatttttccaatcatcattacataaggtcctgcctgttgatttacagctagaaaatctagcaaacgcacataccaaaatattatgttaagacagtaaattaatcttccagccacaaaaacatgattatcatatgcatttgcaaagttccattttgctccaaatcttagtccaaatccaatgaagaaagaaattatggcaattgtatcactgatgttgaagtaatcactaaaccatactttaatcttctggtttactttcccagcttcagacataaagatctcacggactttctcaatggcataagtaaaaatataagcaataacaatccattcttgaactgaaggtaactgttccatttgtacaagaaccacaaatgtataaagcatcagaaatcctaaatatgccaacgtgttaaaccagaattttacaattggtgcatgataaaaggcataaaactttcgcgtaattggaagcttttttgatttcatttgtatctccatctcattctttccttcattactatccaaaatccgtacttctttaaacacttccatggggatctcttctgttatgttctgaaagttgttttcgctgtcatccattgtcatctgatgagcatcttgagattgtgggatatgggacatttcagccttagttttatactctaacagcaatatggcaggtggaactaaaatgcttagtatgaccttgtaccaggaatttttcctcatattcagccttcccatccacatatcagataacaacatttgtgtacaggtgtgagctacaaaaggtctaagtcttgaagaaactgctaacttaaggcaggttgaattactccagttcttcagttcataagtgagcaatttcatagccatggtttcatcttgtctgaaggactgttctaataattcaacggccaactgaccaaaatcattggaatactgttttagttcttctgaagtatcatctaccaggtcactctgctttgcttcatatgccattgaacgatagatcttacaggcaactaatgctttagccattgattcttcaccatgttgccataaaaaacgggccatgacctgcctcttcataaggcaagcccaaattaaaagttcattaagtggataaggaaagcgcttggtttctggatcatcaatgtctacaatttcatctttggttcttttcttctttccttcttccataactgtatcaatctttggtcggtagggctgtgctgtcttaatgaaatggttatgcctcattttttcctttttatctgccctattgccaaaagattcatgactctttcgcaactgaggagtgctgctggaggtatttcggccagacctccgattatttccaccaagactattatatattaatcgaaaacgtttcctagtataggtgcatctgtaggttcctcccatgagatattcaataacaagtcctatatcaatcagagtgatcttatatcctggaggaagatttccctgtttgacgtctcgaacaagatgaaacagcattggattagttggaccttgtttagtgttgtaaagttcttccagtctcggaatggtaaggaatttatgcatgcttactccattttcaataagaagttttacaaatgcaactctatccattacaagagcatcaagcatagcttgttccaaggatccaaccagccactgctgtccataaacaaatacatgatttttggcaatgtcaactctatcccatgccaatgtaaggataagctggtcaaatgcagatgcattagtaccttttagcagtgcagtaagtattgctacatctatatcttgatgttcatctgacccaatatggaaaacagtgataagctcctttcttttcatgcactccatcagtgtttgaaataaatgaagtgcttcattctggccaaagttaaatgtttttttgatagtggaaataatatcgggctctgctgcatcaggaagattccctccttcttctgtttgtttatgaatatacgctagcagatctgcagctctgcctgttccttcacacacaactactggaacaggggggctttcctgaaggtattcaagaactgtgaggataacatttggcccaccctcaaatataagtgccaccacagggacaccctggccaatcctagcatgaattctttgctgattaatagttttttcaagttctcttctcagtctgacttccgccccatactttccaacagtgccatcatccaccaatatgaaatgggaatgcagattattcaaaacattcaatttgctcagggggttcaataaggtttgataaggagcaaccacatctctcccaacaagatcatttctgttttcaatcactccccatggagctattccgatagtgcaaatctttcgagatgatctggaagcatgttctttgagggcatctccaacatgttttgccacacctgtgtttactcctccagttaaaatccaggctccagttgtaactgcagctttaataagaccttttccaagcaactgcttgattcgtgggtgaagctcaaatttctgcatgcccccatgtacagagataacaagtttgggtaactccatttgccattctttaagcagaagttgcagaatgacttcaggtttggtgtcatatgatagcctcacatacttagctctgtaggaatgagaacccccttgaaaatttatgactccataagcatccgttgggctctgttctgtatgcttttccacagaccattcttctattgcctgattaaaatggtcacccaatttcacatctgagtatttcatggcaagacttgcagtaaaacaagcatgttgcttgaccaagcgaccacaaaaacacctgacgagttgctgacaaatttgacatcctggaaggcatctgtgagggtccttggaacttggtataatatatacacattccctcttggtcaaagtgctttctatccaggatttctgggacattctcctcacggggcggactccggaagggcagcaactccacctcctcctcctccgcggcctgtagccatctatcgggaagcgtctccggaggcggcagcagaggccgccggacaaggaacgcccagggaaaccttctcagaactaactcagctccggcgctagcagcagaagccgagtctttcataattgtgcgaccaactcctccgggtgactggccacagggacgcgcccgcgcccgcctccgccggcgacggggctggggac

SEQ ID NO: 15150 - RNA, 8224 nt, Homo sapiens
  source 1..8224: mol_type = other RNA
gctgggattacaggcatgagccactgcacctggcctaatttttgtatttttttttttagcagagataggattttgccatgttgcccaggctggtctcaaactcctgagcccaagtgatccacctgccttggcctcccgaagtgctgggattacaggcatgagccaccatgccccaccaagacaaacaaaacaaaacaaaacaaaacaaaacaaaacaaaaacagtatagatgaaaggcagccagcctgggttcaaatcctaccgttgctacttattattaaataaacgtaagaatcttatggacgttactttacctctctagcaccttgactttcaaatctgcaaaacaggataataacacctatttctttataacattgttataaggattaagtaggttaatatatgtgaaatacttagagtaatgtctggtacacagtaggcactaaataagtgttagcagccaggtgcggtggctcacaaggtcaggagtttgtgaccacactggccaacatagtgaaaccctgtctctactaaaaatataaaaattagctgggcatggtggcgtgtgcctgtagtcccagctactcgggaggctgaggcaggagaatcacttaaacccggaaggcggcggttgtggtgagctgagatcgcaccactgcactccagcccaagcaacagagcgagactccgtctcaaaaaaaaaaaaaaaaaaaaaagtatagctactattataatcctgtgaaaataatcaatataaaattaaaaatcaacagacagcccatattgcccttttttggcctaacaaaaaacagatttctaagaagacagtaagaaatcagtattaatttaaacattgtacaggacaggagatcaaaagcacaggtatacaaatggttcatttaaaaaaactgatactcaaattgacaccctgaaaatgtcagataatttttcagaatgattaaactcactaaacatctgtaaacaataaatttatttcatttcttttaaagatttaatgatatacaaaacgtatatagtatctttaagtaatacactttttctttctccccacccccaatcaatattaaacactatttaaacagcttatcatctcttgccttgtctgtatctatgagatacactactaaatacaaataagctttatactgctcccttccaaataaaaattaaaattagtaccaaggaaacaaaagaaaaagaaaaaaaaagaaaaaaaattaaagcataaaacttagatgaaaagcttttcttgttattgttgaatattcaacaatatctggggctgttaaattacattttattggcataaggttgcactgcaatctgccagtatcacataatgataatccaactgaattaatttcttaagtaccacaaacagcattcatgttcaaatgttccaacacaattttaaatatatgcaagagttcatgtttacattctgatttgatataacaatcaataaaatctttggagaagtttgtaagttctgggttgttgctatagatacagatagggaaaaaagtactttaactttcctcaaaaggtaacttcccttgacgagtgagttaggtttctgcttttataatttaggttatgtatcagtttaccatggctttcttctacttaacagtgacttgataaaacaatgtttaaaaaacccaattaacatttttacacaatttgggttctatttaaaaaaaaaaactggctctatctttaaatatggagcctaaccctgattcataaataccgtccctcttgaaaatggtcttcagttcaggcttctcatacctctgtgaacctagaattagaacaagtcatttcccttcccgtggccaacaagcatctagttgggaaccagtgatatcatcactgaacacactaaatacactgaggaaaattttgactgccatttaaccaaaaggctgcgtgatttcttcatttccctagttgaatggcaataaaacagctgccaataaaatctgcatggacacctacctttggttaatggtattgtaccacataagagagagcatcaccctcatcaaaacaaagtcaaatgagatcctctgctatacaaagagccctttaaaaagttataaatactaattatcaattacctttaaaatttctcagctgccagctctatcctatagggactttctgactgattaatcaggtcaaaagaatattgaccttttaactgtgctggagtcagcaaattcaacttgcatacacctttctatattaccaaacaatttcctcccgagggaaaagtgacacagtaacatttctgtgaggtgcaggcaaaaccaatgattcagtaatattaatattataacatcagacgaacagaattagttgattctgattctttggtggaatttccaggctgaagattcaaatctgaaggctcatcctgaggaaatataattttatcaggcgtataatcattcctcttcagatctggaagtttaagctttctacagcaagaattacagtgatgttttgctctgaagtttttaattgcatcttctcctagatttgctgggccaaaaaccatatcacaggatctcttttcttctgcttttatcacagatgggtcagtcaaattttcaccaacaccttgcaaatcaagtaccagtaactcccctcttgtatattcgtaagtccagtggctaaaggctagcatgatctcttccagagtattagttggaataatctcatctccattattattgttgtattttctaaattctccagtcatacattcttccacagcaaaccactgtcctgctgaatggcaatacagcaggaaaacttcaaggaaccttggagaatatggtatggatttgggtttcatttgattaaaggcaaacgtaagcttttgtgctgctctctgttgttgaatttctctcagacagagatgcagaactgtatcttctttgtaaatacttgaccatgtattaaccacctctggaagaaaagatttgataatataaagatgccctgatttgaggatatcatgttctgaccaggtacactgtactttgacagctcttcgtaaacctcctcccatctcctctttgcttaaaaactctattttggcacagaggcctagttgtgaccaagaagacatgctgttatttagtatgttgggtgaactctcttccaaacgatacactgtgacaggctcccctcttggaggcacaggtgtaaatggaatgctctgtgataacctcatcaagttatttctttccacagctgaataatagtaatttgtatccatagctggcttaaatggagaagtgagaccatttaatgttccttcttcagatggcatttctctgtttgatggtctatcttgtaaccaatccggtattaaagctgctttggaatctacttcatgagtgtcttcggtagatggccttctactgattttttctgcttgttttgaatgaacaggaatggaagttctgtgacagtcagtaaatccagcaagagaactcactcgtttcaaagtgttttcagaagtattgttattggatagtatttttatcttgtttgatgtttctttaaacctctgtaaatccatgctatctctgtgtcctacaaatgctccaaattctgtattatctccttctgtagctttagagcaaacagtttcttgatctttggttccagtttccaagtggcttttgcaacttggctgagatggtgtactaacaaaaaatttggttggtggggatgacagatgtggtatgctagtagatgaactgcctaatttttgatttttattaaatatttttaagagttctaccccatgtagtctctgtcgcagttctggaggggaaacagcacttgggaataaggcaccagaagaggaaccagcctctggaaaattaaattcttttctctggggtactgcaggtaagtcttgaccaaatatattacactggggatctttgtcatctttcattaaaatattacaatgaaaaggattattactttcaagatcaccttgaggaagagaggagctaagtgtatttacaacaccatgctttttccatacagaaggtcttacaggaccatcatcaataaggttttgagccaagtgtttggaaatgctcagttctcgtgtgatttcattatgaactttgctagcttccgacgctttctgggcagtgagtgtttttaatgtatctaccgtcagggctgaaagatcttgcaaatggccaatttgagaatctaatgattgtaatgatctttttatgtagttgacacgatctccaacttctttaatctgaatgcacatctgttccactctttcaaaagtgacacgaattctctcttcactcccagaatgaaatttgtcatctttttcattgaaatacatttcaacacactgctcttcaaaatcatgaagtttcttttgatcttcttctgttaagaaaagttttggtccatcggaagtcttatctttctttcttctcttacatatgcagcaaaacagagaaactatatggctaagaatgataagtggaggaggcagaactggtttctcatgataagccataataaaatgataacgctggtacttccatacaatattggaaattgccttcacttgtaaatacacattgttgaaaaatgcaataagaagattaaccataatgatatactgtacaaagaggtagactgcttgaagaaatggagtcaaccacgtcccaggaccacagatttgagggataacagaatcatttgcacacacatcaatttcgtatgcataaacttcaccaaaaatcatccagtatgggtgaaaaactatatctttagcaagagtccaagatggtgcttcatgaggataaagtattgcctttctgggaacaccaaaactaagtaatacaagagccataatcactacaatgtagaacatattggccaccatttttccaatcatcattacataaggtcctgcctgttgatttacagctagaaaatctagcaaacgcacataccaaaatattatgttaagacagtaaattaatcttccagccacaaaaacatgattatcatatgcatttgcaaagttccattttgctccaaatcttagtccaaatccaatgaagaaagaaattatggcaattgtatcactgatgttgaagtaatcactaaaccatactttaatcttctggtttactttcccagcttcagacataaagatctcacggactttctcaatggcataagtaaaaatataagcaataacaatccattcttgaactgaaggtaactgttccatttgtacaagaaccacaaatgtataaagcatcagaaatcctaaatatgccaacgtgttaaaccagaattttacaattggtgcatgataaaaggcataaaactttcgcgtaattggaagcttttttgatttcatttgtatctccatctcattctttccttcattactatccaaaatccgtacttctttaaacacttccatggggatctcttctgttatgttctgaaagttgttttcgctgtcatccattgtcatctgatgagcatcttgagattgtgggatatgggacatttcagccttagttttatactctaacagcaatatggcaggtggaactaaaatgcttagtatgaccttgtaccaggaatttttcctcatattcagccttcccatccacatatcagataacaacatttgtgtacaggtgtgagctacaaaaggtctaagtcttgaagaaactgctaacttaaggcaggttgaattactccagttcttcagttcataagtgagcaatttcatagccatggtttcatcttgtctgaaggactgttctaataattcaacggccaactgaccaaaatcattggaatactgttttagttcttctgaagtatcatctaccaggtcactctgctttgcttcatatgccattgaacgatagatcttacaggcaactaatgctttagccattgattcttcaccatgttgccataaaaaacgggccatgacctgcctcttcataaggcaagcccaaattaaaagttcattaagtggataaggaaagcgcttggtttctggatcatcaatgtctacaatttcatctttggttcttttcttctttccttcttccataactgtatcaatctttggtcggtagggctgtgctgtcttaatgaaatggttatgcctcattttttcctttttatctgccctattgccaaaagattcatgactctttcgcaactgaggagtgctgctggaggtatttcggccagacctccgattatttccaccaagactattatatattaatcgaaaacgtttcctagtataggtgcatctgtaggttcctcccatgagatattcaataacaagtcctatatcaatcagagtgatcttatatcctggaggaagatttccctgtttgacgtctcgaacaagatgaaacagcattggattagttggaccttgtttagtgttgtaaagttcttccagtctcggaatggtaaggaatttatgcatgcttactccattttcaataagaagttttacaaatgcaactctatccattacaagagcatcaagcatagcttgttccaaggatccaaccagccactgctgtccataaacaaatacatgatttttggcaatgtcaactctatcccatgccaatgtaaggataagctggtcaaatgcagatgcattagtaccttttagcagtgcagtaagtattgctacatctatatcttgatgttcatctgacccaatatggaaaacagtgataagctcctttcttttcatgcactccatcagtgtttgaaataaatgaagtgcttcattctggccaaagttaaatgtttttttgatagtggaaataatatcgggctctgctgcatcaggaagattccctccttcttctgtttgtttatgaatatacgctagcagatctgcagctctgcctgttccttcacacacaactactggaacaggggggctttcctgaaggtattcaagaactgtgaggataacatttggcccaccctcaaatataagtgccaccacagggacaccctggccaatcctagcatgaattctttgctgattaatagttttttcaagttctcttctcagtctgacttccgccccatactttccaacagtgccatcatccaccaatatgaaatgggaatgcagattattcaaaacattcaatttgctcagggggttcaataaggtttgataaggagcaaccacatctctcccaacaagatcatttctgttttcaatcactccccatggagctattccgatagtgcaaatctttcgagatgatctggaagcatgttctttgagggcatctccaacatgttttgccacacctgtgtttactcctccagttaaaatccaggctccagttgtaactgcagctttaataagaccttttccaagcaactgcttgattcgtgggtgaagctcaaatttctgcatgcccccatgtacagagataacaagtttgggtaactccatttgccattctttaagcagaagttgcagaatgacttcaggtttggtgtcatatgatagcctcacatacttagctctgtaggaatgagaacccccttgaaaatttatgactccataagcatccgttgggctctgttctgtatgcttttccacagaccattcttctattgcctgattaaaatggtcacccaatttcacatctgagtatttcatggcaagacttgcagtaaaacaagcatgttgcttgaccaagcgaccacaaaaacacctgacgagttgctgacaaatttgacatcctggaaggcatctgtgagggtccttggaacttggtataatatatacacattccctcttggtcaaagtgctttctatccaggatttctgggacattctcctcacggggcggactccggaagggcagcaactccacctcctcctcctccgcggcctgtagccatctatcgggaagcgtctccggaggcggcagcagaggccgccggacaaggaacgcccagggaaaccttctcagaactaactcagctccggcgctagcagcagaagccgagtctttcataattgtgcgaccaactcctccgggtgactggccacagggacgcgcccgcgcccgcctccgccggcgacggggctggggac

SEQ ID NO: 15151 - RNA, 8221 nt, Homo sapiens
  source 1..8221: mol_type = other RNA
gctgggattacaggcatgagccactgcacctggcctaatttttgtatttttttttttagcagagataggattttgccatgttgcccaggctggtctcaaactcctgagcccaagtgatccacctgccttggcctcccgaagtgctgggattacaggcatgagccaccatgccccaccaagacaaacaaaacaaaacaaaacaaaacaaaacaaaacaaaaacagtatagatgaaaggcagccagcctgggttcaaatcctaccgttgctacttattattaaataaacgtaagaatcttatggacgttactttacctctctagcaccttgactttcaaatctgcaaaacaggataataacacctatttctttataacattgttataaggattaagtaggttaatatatgtgaaatacttagagtaatgtctggtacacagtaggcactaaataagtgttagcagccaggtgcggtggctcacaaggtcaggagtttgtgaccacactggccaacatagtgaaaccctgtctctactaaaaatataaaaattagctgggcatggtggcgtgtgcctgtagtcccagctactcgggaggctgaggcaggagaatcacttaaacccggaaggcggcggttgtggtgagctgagatcgcaccactgcactccagcccaagcaacagagcgagactccgtctcaaaaaaaaaaaaaaaaaaaaaagtatagctactattataatcctgtgaaaataatcaatataaaattaaaaatcaacagacagcccatattgcccttttttggcctaacaaaaaacagatttctaagaagacagtaagaaatcagtattaatttaaacattgtacaggacaggagatcaaaagcacaggtatacaaatggttcatttaaaaaaactgatactcaaattgacaccctgaaaatgtcagataatttttcagaatgattaaactcactaaacatctgtaaacaataaatttatttcatttcttttaaagatttaatgatatacaaaacgtatatagtatctttaagtaatacactttttctttctccccacccccaatcaatattaaacactatttaaacagcttatcatctcttgccttgtctgtatctatgagatacactactaaatacaaataagctttatactgctcccttccaaataaaaattaaaattagtaccaaggaaacaaaagaaaaagaaaaaaaaagaaaaaaaattaaagcataaaacttagatgaaaagcttttcttgttattgttgaatattcaacaatatctggggctgttaaattacattttattggcataaggttgcactgcaatctgccagtatcacataatgataatccaactgaattaatttcttaagtaccacaaacagcattcatgttcaaatgttccaacacaattttaaatatatgcaagagttcatgtttacattctgatttgatataacaatcaataaaatctttggagaagtttgtaagttctgggttgttgctatagatacagatagggaaaaaagtactttaactttcctcaaaaggtaacttcccttgacgagtgagttaggtttctgcttttataatttaggttatgtatcagtttaccatggctttcttctacttaacagtgacttgataaaacaatgtttaaaaaacccaattaacatttttacacaatttgggttctatttaaaaaaaaaaactggctctatctttaaatatggagcctaaccctgattcataaataccgtccctcttgaaaatggtcttcagttcaggcttctcatacctctgtgaacctagaattagaacaagtcatttcccttcccgtggccaacaagcatctagttgggaaccagtgatatcatcactgaacacactaaatacactgaggaaaattttgactgccatttaaccaaaaggctgcgtgatttcttcatttccctagttgaatggcaataaaacagctgccaataaaatctgcatggacacctacctttggttaatggtattgtaccacataagagagagcatcaccctcatcaaaacaaagtcaaatgagatcctctgctatacaaagagccctttaaaaagttataaatactaattatcaattacctttaaaatttctcagctgccagctctatcctatagggactttctgactgattaatcaggtcaaaagaatattgaccttttaactgtgctggagtcagcaaattcaacttgcatacacctttctatattaccaaacaatttcctcccgagggaaaagtgacacagtaacatttctgtgaggtgcaggcaaaaccaatgattcagtaatattaatattataacatcagacgaacagaattagttgattctgattctttggtggaatttccaggctgaagattcaaatctgaaggctcatcctgaggaaatataattttatcaggcgtataatcattcctcttcagatctggaagtttaagctttctacagcaagaattacagtgatgttttgctctgaagtttttaattgcatcttctcctagatttgctgggccaaaaaccatatcacaggatctcttttcttctgcttttatcacagatgggtcagtcaaattttcaccaacaccttgcaaatcaagtaccagtaactcccctcttgtatattcgtaagtccagtggctaaaggctagcatgatctcttccagagtattagttggaataatctcatctccattattattgttgtattttctaaattctccagtcatacattcttccacagcaaaccactgtcctgctgaatggcaatacagcaggaaaacttcaaggaaccttggagaatatggtatggatttgggtttcatttgattaaaggcaaacgtaagcttttgtgctgctctctgttgttgaatttctctcagacagagatgcagaactgtatcttctttgtaaatacttgaccatgtattaaccacctctggaagaaaagatttgataatataaagatgccctgatttgaggatatcatgttctgaccaggtacactgtactttgacagctcttcgtaaacctcctcccatctcctctttgcttaaaaactctattttggcacagaggcctagttgtgaccaagaagacatgctgttatttagtatgttgggtgaactctcttccaaacgatacactgtgacaggctcccctcttggaggcacaggtgtaaatggaatgctctgtgataacctcatcaagttatttctttccacagctgaataatagtaatttgtatccatagctggcttaaatggagaagtgagaccatttaatgttccttcttcagatggcatttctctgtttgatggtctatcttgtaaccaatccggtattaaagctgctttggaatctacttcatgagtgtcttcggtagatggccttctactgattttttcttgttttgaatgaacaggaatggaagttctgtgacagtcagtaaatccagcaagagaactcactcgtttcaaagtgttttcagaagtattgttattggatagtatttttatcttgtttgatgtttctttaaacctctgtaaatccatgctatctctgtgtcctacaaatgctccaaattctgtattatctccttctgtagctttagagcaaacagtttcttgatctttggttccagtttccaagtggcttttgcaacttggctgagatggtgtactaacaaaaaatttggttggtggggatgacagatgtggtatgctagtagatgaactgcctaatttttgatttttattaaatatttttaagagttctaccccatgtagtctctgtcgcagttctggaggggaaacagcacttgggaataaggcaccagaagaggaaccagcctctggaaaattaaattcttttctctggggtactgcaggtaagtcttgaccaaatatattacactggggatctttgtcatctttcattaaaatattacaatgaaaaggattattactttcaagatcaccttgaggaagagaggagctaagtgtatttacaacaccatgctttttccatacagaaggtcttacaggaccatcatcaataaggttttgagccaagtgtttggaaatgctcagttctcgtgtgatttcattatgaactttgctagcttccgacgctttctgggcagtgagtgtttttaatgtatctaccgtcagggctgaaagatcttgcaaatggccaatttgagaatctaatgattgtaatgatctttttatgtagttgacacgatctccaacttctttaatctgaatgcacatctgttccactctttcaaaagtgacacgaattctctcttcactcccagaatgaaatttgtcatctttttcattgaaatacatttcaacacactgctcttcaaaatcatgaagtttcttttgatcttcttctgttaagaaaagttttggtccatcggaagtcttatctttctttcttctcttacatatgcagcaaaacagagaaactatatggctaagaatgataagtggaggaggcagaactggtttctcatgataagccataataaaatgataacgctggtacttccatacaatattggaaattgccttcacttgtaaatacacattgttgaaaaatgcaataagaagattaaccataatgatatactgtacaaagaggtagactgcttgaagaaatggagtcaaccacgtcccaggaccacagatttgagggataacagaatcatttgcacacacatcaatttcgtatgcataaacttcaccaaaaatcatccagtatgggtgaaaaactatatctttagcaagagtccaagatggtgcttcatgaggataaagtattgcctttctgggaacaccaaaactaagtaatacaagagccataatcactacaatgtagaacatattggccaccatttttccaatcatcattacataaggtcctgcctgttgatttacagctagaaaatctagcaaacgcacataccaaaatattatgttaagacagtaaattaatcttccagccacaaaaacatgattatcatatgcatttgcaaagttccattttgctccaaatcttagtccaaatccaatgaagaaagaaattatggcaattgtatcactgatgttgaagtaatcactaaaccatactttaatcttctggtttactttcccagcttcagacataaagatctcacggactttctcaatggcataagtaaaaatataagcaataacaatccattcttgaactgaaggtaactgttccatttgtacaagaaccacaaatgtataaagcatcagaaatcctaaatatgccaacgtgttaaaccagaattttacaattggtgcatgataaaaggcataaaactttcgcgtaattggaagcttttttgatttcatttgtatctccatctcattctttccttcattactatccaaaatccgtacttctttaaacacttccatggggatctcttctgttatgttctgaaagttgttttcgctgtcatccattgtcatctgatgagcatcttgagattgtgggatatgggacatttcagccttagttttatactctaacagcaatatggcaggtggaactaaaatgcttagtatgaccttgtaccaggaatttttcctcatattcagccttcccatccacatatcagataacaacatttgtgtacaggtgtgagctacaaaaggtctaagtcttgaagaaactgctaacttaaggcaggttgaattactccagttcttcagttcataagtgagcaatttcatagccatggtttcatcttgtctgaaggactgttctaataattcaacggccaactgaccaaaatcattggaatactgttttagttcttctgaagtatcatctaccaggtcactctgctttgcttcatatgccattgaacgatagatcttacaggcaactaatgctttagccattgattcttcaccatgttgccataaaaaacgggccatgacctgcctcttcataaggcaagcccaaattaaaagttcattaagtggataaggaaagcgcttggtttctggatcatcaatgtctacaatttcatctttggttcttttcttctttccttcttccataactgtatcaatctttggtcggtagggctgtgctgtcttaatgaaatggttatgcctcattttttcctttttatctgccctattgccaaaagattcatgactctttcgcaactgaggagtgctgctggaggtatttcggccagacctccgattatttccaccaagactattatatattaatcgaaaacgtttcctagtataggtgcatctgtaggttcctcccatgagatattcaataacaagtcctatatcaatcagagtgatcttatatcctggaggaagatttccctgtttgacgtctcgaacaagatgaaacagcattggattagttggaccttgtttagtgttgtaaagttcttccagtctcggaatggtaaggaatttatgcatgcttactccattttcaataagaagttttacaaatgcaactctatccattacaagagcatcaagcatagcttgttccaaggatccaaccagccactgctgtccataaacaaatacatgatttttggcaatgtcaactctatcccatgccaatgtaaggataagctggtcaaatgcagatgcattagtaccttttagcagtgcagtaagtattgctacatctatatcttgatgttcatctgacccaatatggaaaacagtgataagctcctttcttttcatgcactccatcagtgtttgaaataaatgaagtgcttcattctggccaaagttaaatgtttttttgatagtggaaataatatcgggctctgctgcatcaggaagattccctccttcttctgtttgtttatgaatatacgctagcagatctgcagctctgcctgttccttcacacacaactactggaacaggggggctttcctgaaggtattcaagaactgtgaggataacatttggcccaccctcaaatataagtgccaccacagggacaccctggccaatcctagcatgaattctttgctgattaatagttttttcaagttctcttctcagtctgacttccgccccatactttccaacagtgccatcatccaccaatatgaaatgggaatgcagattattcaaaacattcaatttgctcagggggttcaataaggtttgataaggagcaaccacatctctcccaacaagatcatttctgttttcaatcactccccatggagctattccgatagtgcaaatctttcgagatgatctggaagcatgttctttgagggcatctccaacatgttttgccacacctgtgtttactcctccagttaaaatccaggctccagttgtaactgcagctttaataagaccttttccaagcaactgcttgattcgtgggtgaagctcaaatttctgcatgcccccatgtacagagataacaagtttgggtaactccatttgccattctttaagcagaagttgcagaatgacttcaggtttggtgtcatatgatagcctcacatacttagctctgtaggaatgagaacccccttgaaaatttatgactccataagcatccgttgggctctgttctgtatgcttttccacagaccattcttctattgcctgattaaaatggtcacccaatttcacatctgagtatttcatggcaagacttgcagtaaaacaagcatgttgcttgaccaagcgaccacaaaaacacctgacgagttgctgacaaatttgacatcctggaaggcatctgtgagggtccttggaacttggtataatatatacacattccctcttggtcaaagtgctttctatccaggatttctgggacattctcctcacggggcggactccggaagggcagcaactccacctcctcctcctccgcggcctgtagccatctatcgggaagcgtctccggaggcggcagcagaggccgccggacaaggaacgcccagggaaaccttctcagaactaactcagctccggcgctagcagcagaagccgagtctttcataattgtgcgaccaactcctccgggtgactggccacagggacgcgcccgcgcccgcctccgccggcgacggggctggggac

SEQ ID NO: 15152 - RNA, 1486 nt, Homo sapiens
  source 1..1486: mol_type = other RNA
gctgggattacaggcatgagccactgcacctggcctacatctttaaaattttagccacgagaccagtaaaactccttagtttaaaaggacagttgaattcaaatgcagctttgtaaatggaaaggttacagtttgtctgtccttcatggctgaagatcttaccaagttttaagaaaaacaggatagcaaatttacatctcaaaacagagaaaattaagcattttcaagaagaagttagggtatgttagagaaagattaaaaatggacaacaagtgatatagtttgagtatttgtcctcttcaaatctcatgttgaaatgttatccccagtgttggaggttgggtcaagtaggaggtttttgggtcatggtggcaggtccctcatgaatggctgggttctgtccttgtggtaatgagtgagttcttattccattagctcatgtgagagctggttttaaaaagagtctagtgtctttctcacctttctcttgctccctttttggccatgtgatatgcctgctcctcctcttcgccttccaccatgattgtaagcttctttttcttttctttctttctttcttttttttttgagatagagtatcactctgttgcccaggctggagtacagtggtgtgatctcagctcacagcaacctctgcctcccaagttccaagtgatcctcttgcctcagcctcctgagtagcagggattccagacacatgccaccatgcccagctaatttttgtatttttagtagagatggggtttcaccatgttggccagcctggtctcgaactcctgacctcaaatgatccatctgtctccgcctcccgaagtgctggcattacaggcatgagccaccgcacgcggccaattgtaaacttcttgaggttgtcaccagaagcagatgctggcatcatgcttcttgtacagcctagaaaggcctgtctgtctagattcttcttggcatctctgagcatggatttcattctggatatggggcaggatgctctctggaatgagggtctttagacctgtttctttgttctgatgggaccccagagaggacatcacgctttgtaactggttcttcaaggggagaagcaaatgtgtccctgaaaacttcagctgccgcgtttggcaccaggtttgattgacaaggactggcggagggaaagcgcggaggctgggctgggggccgcaggccgaggcagagacaaagaggtttcgcctgtccccgagagtggaagggcccctgggggtaactagcctttgagctcaaaggggcatttcgtgaggtcgccttttggttcggagagcgcgcggcgatcgggtggagggggcctggcgggaagaaagctggggcggggaaggggcgcgggccgaggtgggagcggagctgcagtcacgtggccgcccgccgccgcggagttggggctgttcttccgggttggaggcgcagcgccgcggggcccaagcccgggtct

SEQ ID NO: 15153 - RNA, 3510 nt, Homo sapiens
  source 1..3510: mol_type = other RNA
gctgggattacaggcatgagccactgcacctggcctacatttttatttcagttgtcgtgtctctcaggctctaaacaatttccagcccaaaccacagcaccatcctgatgaaaagggccagatattaagacagctgttaggcagttaacctgtaattaaaaggctgtggcaacttcagttccatgacgacctccgactttaacacagtctcgaggaaatttgtccaattgttcatatgccagccgcccatcttctcccagagacaagagggtttctgaggccacatttctgatttcttcagtatcagattgacacaatgtcaccagcattttaatgctttcagtagcctcaaggattttcagagccaggcaagctgctttctggagctggaggtttgtctttgttagtgcttcacagtaatagagcaaggccttttccctgaaatgctgatttttggaggctgctgccaagtaaagcgtcacagcctcactaacttcgttgtcctctctggttaatagcagagccagagtcctgagtacttcctgctgggccaggaggttgctgggagcaaggtcactcatggtttgtagcagtttttcatctcttagtgattgcagagtctgaaccatggaaacttgcctggccagctggctcaggtaactctccaggtcactgacgccgtggctggtgaagtaactgtaatactggaaaacagtgacgacttccgaggacaggctggaggaaagcagaggctcagcccggtccagaatttgggacaccagggttcgaaacactgggtctgcaagtcctggatattctttgttgacagttctggcaaagctggcctccagctgcttcatcactctgtccgctgggctgtggtagacaccaacagggctgcagcacttggtccagaatgacagcaaagacagctttttgtgaaattctggtatggcttccacaacagaactgatatttcctatgttctcatcactgacagctgcgagtttctccatcacttggatctgcctagaaagcttctctaagagacttcttgccacaaatggggttttgcttgagaaaacaatttgctgcacgagttgggtgcagtactggaggtgcctgacgatggtgatgtccaggctctcgttgcctgtggtcagtgggagaggacttcctgccacactggtcccaactcctgtgtcttcagtgagcgcttcactgagatgccccctggcttctgggtgaaccgacctgtaactgtgtttctcagtctcagtgtctgaaaatactgagtcagcacctccgccaacattacaaacctcatcaccatcctcctcctcgtcaaaatcagaggtgttcaggaaatcaaagctttctaaagcactttcaactgtgagacttaaactggaagacctgctgcggcttactgctggcttgcattttagaatatcatccaaattcatgacttcttggttcagatcctgaaactctttatactgctctttatgtggttctaatgcaagtaaaagcccattaaaagcatcctctaagcttccatctagaaaggatctgcagccttcagattctccaccaacagaaccctcagagagcagcctgtctgtggccattggcacctctgcagatgtgagcctcttgaccagctgctttgtgatgtttccttccgaagtgtccagttccacaggcttgagctcagaggcctcctcagactcttgcagaagtgcttctgcaacatcattctcaaggaacaggtgctcagccccagcacctgaggactgtcggcggcaagcctcagatggggccgaggcaggttttctgggctcctctgggtcttcctccttcaggtgtgactttggctcttggccttctcccagggagttcctggaagatgctgagctggtgtcatccataccctcattctgggaggccaagctgctgaggttaaactccgcaggggtgatggtaatttctggatttgttgagttggaaggggagcctgttgagtgggaggtgagggcgcagtccccgttgggcaggtcactgaagctgagcgacagtggcattttctcctcggctgcctttccattttcaaagatgtcatcaggtagatttgaaaagaaggagtggtctttgaaggtgggcgtttccggggtaccctggctgtacatggacattctcctctgaagggctgctgccttgttcccagcgcctgaggatgcggtcatgtcctccacgtcaaatggataccaggtgatttccaggttcagtttgatggtaccaaggtcattgatgtcgacagccactacctgaggtcgggctgcaaacagctctttggtctcacaggtcacgctacctaccaggatgtgagttgctagccctttgagctccgtgaccttgatggagatgaacccaactatcaggggcagaaaaactgtttcttctccatcccagctctgcttgccatttacttctattttgcctttcagtttccaccgctgccggccatacttcatgaaaatttcatattgatctccaggacagaggcgtgcaaagccagccagacctttcatcttgatggagaattctcccagcagattctctagctccacttcaatggtgcacatattctctgtgtactccttgaagctccgattgatctctgtcagactctcccgggcagctttgctggcaggggatgttgcgaaggcttgcttcattttgctggcaccatcctggaggcgtcgctggatacaataagcttcatagagttcatctaccttacttatatgaaactccaggcgtctcatgtatctttcaattgttttaatttgcttgtctaggtcatacagtacacccaggcgagagtttcttttcatatcttttaactgagctgtcaacttgtccagctccgtctggtgaacctccagatattcatcaagtccatttttcaaggccctgtagacttcttccacccttttaggctgaggctctttggggggattgttgtttttgtggcctaaattgtgcattttcttcagtttggcctgaggcttcttgagagcggaggaattttcaatgaaggagttacacctggatcgcctttcctggaggccgctgaaacccgcaaaggactggcttctaatgatcccattgggccctccaggcgaaaaagactgggatcctaccaacatgatttccgggagtctggtcggtagtcatgatctgatttgtctgtcaacaagaatccaacagttcaggctcttgacacgtccctcttcagcctagggtgtgcagatgttatggaatcatcaccctcatagtcagccaagcacatcctcatttcagggtcccagaaactagcacctggcacagcctggaccatatgaccaccacctggtgagccgtttgctcccacacgtgaattctgttctgttcttgaaagcaggataggaacctacactgtgcatggcccttcttttttcctttttt

SEQ ID NO: 15154 - RNA, 3345 nt, Homo sapiens
  source 1..3345: mol_type = other RNA
gctgggattacaggcatgagccactgcacctggcctacatttttatttcagttgtcgtgtctctcaggctctaaacaatttccagcccaaaccacagcaccatcctgatgaaaagggccagatattaagacagctgttaggcagttaacctgtaattaaaaggctgtggcaacttcagttccatgacgacctccgactttaacacagtctcgaggaaatttgtccaattgttcatatgccagccgcccatcttctcccagagacaagagggtttctgaggccacatttctgatttcttcagtatcagattgacacaatgtcaccagcattttaatgctttcagtagcctcaaggattttcagagccaggcaagctgctttctggagctggaggtttgtctttgttagtgcttcacagtaatagagcaaggccttttccctgaaatgctgatttttggaggctgctgccaagtaaagcgtcacagcctcactaacttcgttgtcctctctggttaatagcagagccagagtcctgagtacttcctgctgggccaggaggttgctgggagcaaggtcactcatggtttgtagcagtttttcatctcttagtgattgcagagtctgaaccatggaaacttgcctggccagctggctcaggtaactctccaggtcactgacgccgtggctggtgaagtaactgtaatactggaaaacagtgacgacttccgaggacaggctggaggaaagcagaggctcagcccggtccagaatttgggacaccagggttcgaaacactgggtctgcaagtcctggatattctttgttgacagttctggcaaagctggcctccagctgcttcatcactctgtccgctgggctgtggtagacaccaacagggctgcagcacttggtccagaatgacagcaaagacagctttttgtgaaattctggtatggcttccacaacagaactgatatttcctatgttctcatcactgacagctgcgagtttctccatcacttggatctgcctagaaagcttctctaagagacttcttgccacaaatggggttttgcttgagaaaacaatttgctgcacgagttgggtgcagtactggaggtgcctgacgatggtgatgtccaggctctcgttgcctgtggtcagtgggagaggacttcctgccacactggtcccaactcctgtgtcttcagtgagcgcttcactgagatgccccctggcttctgggtgaaccgacctgtaactgtgtttctcagtctcagtgtctgaaaatactgagtcagcacctccgccaacattacaaacctcatcaccatcctcctcctcgtcaaaatcagaggtgttcaggaaatcaaagctttctaaagcactttcaactgtgagacttaaactggaagacctgctgcggcttactgctggcttgcattttagaatatcatccaaattcatgacttcttggttcagatcctgaaactctttatactgctctttatgtggttctaatgcaagtaaaagcccattaaaagcatcctctaagcttccatctagaaaggatctgcagccttcagattctccaccaacagaaccctcagagagcagcctgtctgtggccattggcacctctgcagatgtgagcctcttgaccagctgctttgtgatgtttccttccgaagtgtccagttccacaggcttgagctcagaggcctcctcagactcttgcagaagtgcttctgcaacatcattctcaaggaacaggtgctcagccccagcacctgaggactgtcggcggcaagcctcagatggggccgaggcaggttttctgggctcctctgggtcttcctccttcaggtgtgactttggctcttggccttctcccagggagttcctggaagatgctgagctggtgtcatccataccctcattctgggaggccaagctgctgaggttaaactccgcaggggtgatggtaatttctggatttgttgagttggaaggggagcctgttgagtgggaggtgagggcgcagtccccgttgggcaggtcactgaagctgagcgacagtggcattttctcctcggctgcctttccattttcaaagatgtcatcaggtagatttgaaaagaaggagtggtctttgaaggtgggcgtttccggggtaccctggctgtacatggacattctcctctgaagggctgctgccttgttcccagcgcctgaggatgcggtcatgtcctccacgtcaaatggataccaggtgatttccaggttcagtttgatggtaccaaggtcattgatgtcgacagccactacctgaggtcgggctgcaaacagctctttggtctcacaggtcacgctacctaccaggatgtgagttgctagccctttgagctccgtgaccttgatggagatgaacccaactatcaggggcagaaaaactgtttcttctccatcccagctctgcttgccatttacttctattttgcctttcagtttccaccgctgccggccatacttcatgaaaatttcatattgatctccaggacagaggcgtgcaaagccagccagacctttcatcttgatggagaattctcccagcagattctctagctccacttcaatggtgcacatattctctgtgtactccttgaagctccgattgatctctgtcagactctcccgggcagctttgctggcaggggatgttgcgaaggcttgcttcattttgctggcaccatcctggaggcgtcgctggatacaataagcttcatagagttcatctaccttacttatatgaaactccaggcgtctcatgtatctttcaattgttttaatttgcttgtctaggtcatacagtacacccaggcgagagtttcttttcatatcttttaactgagctgtcaacttgtccagctccgtctggtgaacctccagatattcatcaagtccatttttcaaggccctgtagacttcttccacccttttaggctgaggctctttggggggattgttgtttttgtggcctaaattgtgcattttcttcagtttggcctgaggcttcttgagagcggaggaattttcaatgaaggagttacacctggatcgcctttcctggaggccgctgaaacccgcaaaggactggcttctaatgatcccattgggccctccaggcgaaaaagactgggatcctaccaacatgatttccgggagtctggtcggtagtccaccacctggtgagccgtttgctcccacacgtgaattctgttctgttcttgaaagcaggataggaacctacactgtgcatggcccttcttttttccttttttcaatt

SEQ ID NO: 15155 - RNA, 3648 nt, Homo sapiens
  source 1..3648: mol_type = other RNA
gctgggattacaggcatgagccactgcacctggcctacatttttatttcagttgtcgtgtctctcaggctctaaacaatttccagcccaaaccacagcaccatcctgatgaaaagggccagatattaagacagctgttaggcagttaacctgtaattaaaaggctgtggcaacttcagttccatgacgacctccgactttaacacagtctcgaggaaatttgtccaattgttcatatgccagccgcccatcttctcccagagacaagagggtttctgaggccacatttctgatttcttcagtatcagattgacacaatgtcaccagcattttaatgctttcagtagcctcaaggattttcagagccaggcaagctgctttctggagctggaggtttgtctttgttagtgcttcacagtaatagagcaaggccttttccctgaaatgctgatttttggaggctgctgccaagtaaagcgtcacagcctcactaacttcgttgtcctctctggttaatagcagagccagagtcctgagtacttcctgctgggccaggaggttgctgggagcaaggtcactcatggtttgtagcagtttttcatctcttagtgattgcagagtctgaaccatggaaacttgcctggccagctggctcaggtaactctccaggtcactgacgccgtggctggtgaagtaactgtaatactggaaaacagtgacgacttccgaggacaggctggaggaaagcagaggctcagcccggtccagaatttgggacaccagggttcgaaacactgggtctgcaagtcctggatattctttgttgacagttctggcaaagctggcctccagctgcttcatcactctgtccgctgggctgtggtagacaccaacagggctgcagcacttggtccagaatgacagcaaagacagctttttgtgaaattctggtatggcttccacaacagaactgatatttcctatgttctcatcactgacagctgcgagtttctccatcacttggatctgcctagaaagcttctctaagagacttcttgccacaaatggggttttgcttgagaaaacaatttgctgcacgagttgggtgcagtactggaggtgcctgacgatggtgatgtccaggctctcgttgcctgtggtcagtgggagaggacttcctgccacactggtcccaactcctgtgtcttcagtgagcgcttcactgagatgccccctggcttctgggtgaaccgacctgtaactgtgtttctcagtctcagtgtctgaaaatactgagtcagcacctccgccaacattacaaacctcatcaccatcctcctcctcgtcaaaatcagaggtgttcaggaaatcaaagctttctaaagcactttcaactgtgagacttaaactggaagacctgctgcggcttactgctggcttgcattttagaatatcatccaaattcatgacttcttggttcagatcctgaaactctttatactgctctttatgtggttctaatgcaagtaaaagcccattaaaagcatcctctaagcttccatctagaaaggatctgcagccttcagattctccaccaacagaaccctcagagagcagcctgtctgtggccattggcacctctgcagatgtgagcctcttgaccagctgctttgtgatgtttccttccgaagtgtccagttccacaggcttgagctcagaggcctcctcagactcttgcagaagtgcttctgcaacatcattctcaaggaacaggtgctcagccccagcacctgaggactgtcggcggcaagcctcagatggggccgaggcaggttttctgggctcctctgggtcttcctccttcaggtgtgactttggctcttggccttctcccagggagttcctggaagatgctgagctggtgtcatccataccctcattctgggaggccaagctgctgaggttaaactccgcaggggtgatggtaatttctggatttgttgagttggaaggggagcctgttgagtgggaggtgagggcgcagtccccgttgggcaggtcactgaagctgagcgacagtggcattttctcctcggctgcctttccattttcaaagatgtcatcaggtagatttgaaaagaaggagtggtctttgaaggtgggcgtttccggggtaccctggctgtacatggacattctcctctgaagggctgctgccttgttcccagcgcctgaggatgcggtcatgtcctccacgtcaaatggataccaggtgatttccaggttcagtttgatggtaccaaggtcattgatgtcgacagccactacctgaggtcgggctgcaaacagctctttggtctcacaggtcacgctacctaccaggatgtgagttgctagccctttgagctccgtgaccttgatggagatgaacccaactatcaggggcagaaaaactgtttcttctccatcccagctctgcttgccatttacttctattttgcctttcagtttccaccgctgccggccatacttcatgaaaatttcatattgatctccaggacagaggcgtgcaaagccagccagacctttcatcttgatggagaattctcccagcagattctctagctccacttcaatggtgcacatattctctgtgtactccttgaagctccgattgatctctgtcagactctcccgggcagctttgctggcaggggatgttgcgaaggcttgcttcattttgctggcaccatcctggaggcgtcgctggatacaataagcttcatagagttcatctaccttacttatatgaaactccaggcgtctcatgtatctttcaattgttttaatttgcttgtctaggtcatacagtacacccaggcgagagtttcttttcatatcttttaactgagctgtcaacttgtccagctccgtctggtgaacctccagatattcatcaagtccatttttcaaggccctgtagacttcttccacccttttaggctgaggctctttggggggattgttgtttttgtggcctaaattgtgcattttcttcagtttggcctgaggcttcttgagagcggaggaattttcaatgaaggagttacacctggatcgcctttcctggaggccgctgaaacccgcaaaggactggcttctaatgatcccattgggccctccaggcgaaaaagactgggatcctaccaacatgatttccgggagtctggtcggtagtccattgtcttagcaggtgacttcaatccagagagggggacaggctagcaggaaaaagggtaaatagttactgcccagattgaagactccaaagtgggcagacaacaaatcggtatgtttgcagagtgtcgacaattgccctttaaagactcaaagaaagaaaagctaaaaaaaacaacagcagcagaactctctggtagtacatccagatgtaatggaaagaccaatttcactagaccttcctcaaagctacgcgaagcagctcagcaaggaaggcagtttgagcgagttacttccccagagagagaaggacaaacagcctcctcccccatgttgctgcaggtttttaaatcccctccctccctctccaggagagagcagccctggagtttgtatgcattcttgcgaggta

SEQ ID NO: 15156 - RNA, 3469 nt, Homo sapiens
  source 1..3469: mol_type = other RNA
gctgggattacaggcatgagccactgcacctggcctacatttttatttcagttgtcgtgtctctcaggctctaaacaatttccagcccaaaccacagcaccatcctgatgaaaagggccagatattaagacagctgttaggcagttaacctgtaattaaaaggctgtggcaacttcagttccatgacgacctccgactttaacacagtctcgaggaaatttgtccaattgttcatatgccagccgcccatcttctcccagagacaagagggtttctgaggccacatttctgatttcttcagtatcagattgacacaatgtcaccagcattttaatgctttcagtagcctcaaggattttcagagccaggcaagctgctttctggagctggaggtttgtctttgttagtgcttcacagtaatagagcaaggccttttccctgaaatgctgatttttggaggctgctgccaagtaaagcgtcacagcctcactaacttcgttgtcctctctggttaatagcagagccagagtcctgagtacttcctgctgggccaggaggttgctgggagcaaggtcactcatggtttgtagcagtttttcatctcttagtgattgcagagtctgaaccatggaaacttgcctggccagctggctcaggtaactctccaggtcactgacgccgtggctggtgaagtaactgtaatactggaaaacagtgacgacttccgaggacaggctggaggaaagcagaggctcagcccggtccagaatttgggacaccagggttcgaaacactgggtctgcaagtcctggatattctttgttgacagttctggcaaagctggcctccagctgcttcatcactctgtccgctgggctgtggtagacaccaacagggctgcagcacttggtccagaatgacagcaaagacagctttttgtgaaattctggtatggcttccacaacagaactgatatttcctatgttctcatcactgacagctgcgagtttctccatcacttggatctgcctagaaagcttctctaagagacttcttgccacaaatggggttttgcttgagaaaacaatttgctgcacgagttgggtgcagtactggaggtgcctgacgatggtgatgtccaggctctcgttgcctgtggtcagtgggagaggacttcctgccacactggtcccaactcctgtgtcttcagtgagcgcttcactgagatgccccctggcttctgggtgaaccgacctgtaactgtgtttctcagtctcagtgtctgaaaatactgagtcagcacctccgccaacattacaaacctcatcaccatcctcctcctcgtcaaaatcagaggtgttcaggaaatcaaagctttctaaagcactttcaactgtgagacttaaactggaagacctgctgcggcttactgctggcttgcattttagaatatcatccaaattcatgacttcttggttcagatcctgaaactctttatactgctctttatgtggttctaatgcaagtaaaagcccattaaaagcatcctctaagcttccatctagaaaggatctgcagccttcagattctccaccaacagaaccctcagagagcagcctgtctgtggccattggcacctctgcagatgtgagcctcttgaccagctgctttgtgatgtttccttccgaagtgtccagttccacaggcttgagctcagaggcctcctcagactcttgcagaagtgcttctgcaacatcattctcaaggaacaggtgctcagccccagcacctgaggactgtcggcggcaagcctcagatggggccgaggcaggttttctgggctcctctgggtcttcctccttcaggtgtgactttggctcttggccttctcccagggagttcctggaagatgctgagctggtgtcatccataccctcattctgggaggccaagctgctgaggttaaactccgcaggggtgatggtaatttctggatttgttgagttggaaggggagcctgttgagtgggaggtgagggcgcagtccccgttgggcaggtcactgaagctgagcgacagtggcattttctcctcggctgcctttccattttcaaagatgtcatcaggtagatttgaaaagaaggagtggtctttgaaggtgggcgtttccggggtaccctggctgtacatggacattctcctctgaagggctgctgccttgttcccagcgcctgaggatgcggtcatgtcctccacgtcaaatggataccaggtgatttccaggttcagtttgatggtaccaaggtcattgatgtcgacagccactacctgaggtcgggctgcaaacagctctttggtctcacaggtcacgctacctaccaggatgtgagttgctagccctttgagctccgtgaccttgatggagatgaacccaactatcaggggcagaaaaactgtttcttctccatcccagctctgcttgccatttacttctattttgcctttcagtttccaccgctgccggccatacttcatgaaaatttcatattgatctccaggacagaggcgtgcaaagccagccagacctttcatcttgatggagaattctcccagcagattctctagctccacttcaatggtgcacatattctctgtgtactccttgaagctccgattgatctctgtcagactctcccgggcagctttgctggcaggggatgttgcgaaggcttgcttcattttgctggcaccatcctggaggcgtcgctggatacaataagcttcatagagttcatctaccttacttatatgaaactccaggcgtctcatgtatctttcaattgttttaatttgcttgtctaggtcatacagtacacccaggcgagagtttcttttcatatcttttaactgagctgtcaacttgtccagctccgtctggtgaacctccagatattcatcaagtccatttttcaaggccctgtagacttcttccacccttttaggctgaggctctttggggggattgttgtttttgtggcctaaattgtgcattttcttcagtttggcctgaggcttcttgagagcggaggaattttcaatgaaggagttacacctggatcgcctttcctggaggccgctgaaacccgcaaaggactggcttctaatgatcccattgggccctccaggcgaaaaagactgggatcctaccaacatgatttccgggagtctggtcggtagtcctaacgacgacggctccttgtcatgtcaggggcacactcagggttctctggcatataaaagcctccgcaccaatgcaatgcccggagctgcccgcacctccggctttgcagacagcctgagctggctcacttgggtgaaggggaccccgggaggaagtcgggtggacgcgagctgtccccagcgccggctgccctgccgcgtccgctcgcagcagctgcggcgcgcggggt

SEQ ID NO: 15157 - RNA, 3382 nt, Homo sapiens
  source 1..3382: mol_type = other RNA
gctgggattacaggcatgagccactgcacctggcctacatttttatttcagttgtcgtgtctctcaggctctaaacaatttccagcccaaaccacagcaccatcctgatgaaaagggccagatattaagacagctgttaggcagttaacctgtaattaaaaggctgtggcaacttcagttccatgacgacctccgactttaacacagtctcgaggaaatttgtccaattgttcatatgccagccgcccatcttctcccagagacaagagggtttctgaggccacatttctgatttcttcagtatcagattgacacaatgtcaccagcattttaatgctttcagtagcctcaaggattttcagagccaggcaagctgctttctggagctggaggtttgtctttgttagtgcttcacagtaatagagcaaggccttttccctgaaatgctgatttttggaggctgctgccaagtaaagcgtcacagcctcactaacttcgttgtcctctctggttaatagcagagccagagtcctgagtacttcctgctgggccaggaggttgctgggagcaaggtcactcatggtttgtagcagtttttcatctcttagtgattgcagagtctgaaccatggaaacttgcctggccagctggctcaggtaactctccaggtcactgacgccgtggctggtgaagtaactgtaatactggaaaacagtgacgacttccgaggacaggctggaggaaagcagaggctcagcccggtccagaatttgggacaccagggttcgaaacactgggtctgcaagtcctggatattctttgttgacagttctggcaaagctggcctccagctgcttcatcactctgtccgctgggctgtggtagacaccaacagggctgcagcacttggtccagaatgacagcaaagacagctttttgtgaaattctggtatggcttccacaacagaactgatatttcctatgttctcatcactgacagctgcgagtttctccatcacttggatctgcctagaaagcttctctaagagacttcttgccacaaatggggttttgcttgagaaaacaatttgctgcacgagttgggtgcagtactggaggtgcctgacgatggtgatgtccaggctctcgttgcctgtggtcagtgggagaggacttcctgccacactggtcccaactcctgtgtcttcagtgagcgcttcactgagatgccccctggcttctgggtgaaccgacctgtaactgtgtttctcagtctcagtgtctgaaaatactgagtcagcacctccgccaacattacaaacctcatcaccatcctcctcctcgtcaaaatcagaggtgttcaggaaatcaaagctttctaaagcactttcaactgtgagacttaaactggaagacctgctgcggcttactgctggcttgcattttagaatatcatccaaattcatgacttcttggttcagatcctgaaactctttatactgctctttatgtggttctaatgcaagtaaaagcccattaaaagcatcctctaagcttccatctagaaaggatctgcagccttcagattctccaccaacagaaccctcagagagcagcctgtctgtggccattggcacctctgcagatgtgagcctcttgaccagctgctttgtgatgtttccttccgaagtgtccagttccacaggcttgagctcagaggcctcctcagactcttgcagaagtgcttctgcaacatcattctcaaggaacaggtgctcagccccagcacctgaggactgtcggcggcaagcctcagatggggccgaggcaggttttctgggctcctctgggtcttcctccttcaggtgtgactttggctcttggccttctcccagggagttcctggaagatgctgagctggtgtcatccataccctcattctgggaggccaagctgctgaggttaaactccgcaggggtgatggtaatttctggatttgttgagttggaaggggagcctgttgagtgggaggtgagggcgcagtccccgttgggcaggtcactgaagctgagcgacagtggcattttctcctcggctgcctttccattttcaaagatgtcatcaggtagatttgaaaagaaggagtggtctttgaaggtgggcgtttccggggtaccctggctgtacatggacattctcctctgaagggctgctgccttgttcccagcgcctgaggatgcggtcatgtcctccacgtcaaatggataccaggtgatttccaggttcagtttgatggtaccaaggtcattgatgtcgacagccactacctgaggtcgggctgcaaacagctctttggtctcacaggtcacgctacctaccaggatgtgagttgctagccctttgagctccgtgaccttgatggagatgaacccaactatcaggggcagaaaaactgtttcttctccatcccagctctgcttgccatttacttctattttgcctttcagtttccaccgctgccggccatacttcatgaaaatttcatattgatctccaggacagaggcgtgcaaagccagccagacctttcatcttgatggagaattctcccagcagattctctagctccacttcaatggtgcacatattctctgtgtactccttgaagctccgattgatctctgtcagactctcccgggcagctttgctggcaggggatgttgcgaaggcttgcttcattttgctggcaccatcctggaggcgtcgctggatacaataagcttcatagagttcatctaccttacttatatgaaactccaggcgtctcatgtatctttcaattgttttaatttgcttgtctaggtcatacagtacacccaggcgagagtttcttttcatatcttttaactgagctgtcaacttgtccagctccgtctggtgaacctccagatattcatcaagtccatttttcaaggccctgtagacttcttccacccttttaggctgaggctctttggggggattgttgtttttgtggcctaaattgtgcattttcttcagtttggcctgaggcttcttgagagcggaggaattttcaatgaaggagttacacctggatcgcctttcctggaggccgctgaaacccgcaaaggactggcttctaatgatcccattgggccctccaggcgaaaaagactgggatcctaccaacatgatttccgggagtctggtcggtagtcctcataatccctactgcttggtcacagtgtagcatttccacagcagttctccttggcctggagagggtaacagcttctcctttatgttcaccattcaccccctgtactggatttttctccaccttgtcgcctcctctccaggtt

SEQ ID NO: 15158 - RNA, 3361 nt, Homo sapiens
  source 1..3361: mol_type = other RNA
gctgggattacaggcatgagccactgcacctggcctacatttttatttcagttgtcgtgtctctcaggctctaaacaatttccagcccaaaccacagcaccatcctgatgaaaagggccagatattaagacagctgttaggcagttaacctgtaattaaaaggctgtggcaacttcagttccatgacgacctccgactttaacacagtctcgaggaaatttgtccaattgttcatatgccagccgcccatcttctcccagagacaagagggtttctgaggccacatttctgatttcttcagtatcagattgacacaatgtcaccagcattttaatgctttcagtagcctcaaggattttcagagccaggcaagctgctttctggagctggaggtttgtctttgttagtgcttcacagtaatagagcaaggccttttccctgaaatgctgatttttggaggctgctgccaagtaaagcgtcacagcctcactaacttcgttgtcctctctggttaatagcagagccagagtcctgagtacttcctgctgggccaggaggttgctgggagcaaggtcactcatggtttgtagcagtttttcatctcttagtgattgcagagtctgaaccatggaaacttgcctggccagctggctcaggtaactctccaggtcactgacgccgtggctggtgaagtaactgtaatactggaaaacagtgacgacttccgaggacaggctggaggaaagcagaggctcagcccggtccagaatttgggacaccagggttcgaaacactgggtctgcaagtcctggatattctttgttgacagttctggcaaagctggcctccagctgcttcatcactctgtccgctgggctgtggtagacaccaacagggctgcagcacttggtccagaatgacagcaaagacagctttttgtgaaattctggtatggcttccacaacagaactgatatttcctatgttctcatcactgacagctgcgagtttctccatcacttggatctgcctagaaagcttctctaagagacttcttgccacaaatggggttttgcttgagaaaacaatttgctgcacgagttgggtgcagtactggaggtgcctgacgatggtgatgtccaggctctcgttgcctgtggtcagtgggagaggacttcctgccacactggtcccaactcctgtgtcttcagtgagcgcttcactgagatgccccctggcttctgggtgaaccgacctgtaactgtgtttctcagtctcagtgtctgaaaatactgagtcagcacctccgccaacattacaaacctcatcaccatcctcctcctcgtcaaaatcagaggtgttcaggaaatcaaagctttctaaagcactttcaactgtgagacttaaactggaagacctgctgcggcttactgctggcttgcattttagaatatcatccaaattcatgacttcttggttcagatcctgaaactctttatactgctctttatgtggttctaatgcaagtaaaagcccattaaaagcatcctctaagcttccatctagaaaggatctgcagccttcagattctccaccaacagaaccctcagagagcagcctgtctgtggccattggcacctctgcagatgtgagcctcttgaccagctgctttgtgatgtttccttccgaagtgtccagttccacaggcttgagctcagaggcctcctcagactcttgcagaagtgcttctgcaacatcattctcaaggaacaggtgctcagccccagcacctgaggactgtcggcggcaagcctcagatggggccgaggcaggttttctgggctcctctgggtcttcctccttcaggtgtgactttggctcttggccttctcccagggagttcctggaagatgctgagctggtgtcatccataccctcattctgggaggccaagctgctgaggttaaactccgcaggggtgatggtaatttctggatttgttgagttggaaggggagcctgttgagtgggaggtgagggcgcagtccccgttgggcaggtcactgaagctgagcgacagtggcattttctcctcggctgcctttccattttcaaagatgtcatcaggtagatttgaaaagaaggagtggtctttgaaggtgggcgtttccggggtaccctggctgtacatggacattctcctctgaagggctgctgccttgttcccagcgcctgaggatgcggtcatgtcctccacgtcaaatggataccaggtgatttccaggttcagtttgatggtaccaaggtcattgatgtcgacagccactacctgaggtcgggctgcaaacagctctttggtctcacaggtcacgctacctaccaggatgtgagttgctagccctttgagctccgtgaccttgatggagatgaacccaactatcaggggcagaaaaactgtttcttctccatcccagctctgcttgccatttacttctattttgcctttcagtttccaccgctgccggccatacttcatgaaaatttcatattgatctccaggacagaggcgtgcaaagccagccagacctttcatcttgatggagaattctcccagcagattctctagctccacttcaatggtgcacatattctctgtgtactccttgaagctccgattgatctctgtcagactctcccgggcagctttgctggcaggggatgttgcgaaggcttgcttcattttgctggcaccatcctggaggcgtcgctggatacaataagcttcatagagttcatctaccttacttatatgaaactccaggcgtctcatgtatctttcaattgttttaatttgcttgtctaggtcatacagtacacccaggcgagagtttcttttcatatcttttaactgagctgtcaacttgtccagctccgtctggtgaacctccagatattcatcaagtccatttttcaaggccctgtagacttcttccacccttttaggctgaggctctttggggggattgttgtttttgtggcctaaattgtgcattttcttcagtttggcctgaggcttcttgagagcggaggaattttcaatgaaggagttacacctggatcgcctttcctggaggccgctgaaacccgcaaaggactggcttctaatgatcccattgggccctccaggcgaaaaagactgggatcctaccaacatgatttccgggagtctggtcggtagtccttcaccaaaaacatcatcctcttcatcgaccaggagctcctcagcatcaaaaaactgcatcttggagaggacaggcgcgagaagcagcaggcagcagccccggcagtctcagcagtcacact

SEQ ID NO: 15159 - RNA, 4179 nt, Homo sapiens
  source 1..4179: mol_type = other RNA
gctgggattacaggcatgagccactgcacctggcctacatttttatttcagttgtcgtgtctctcaggctctaaacaatttccagcccaaaccacagcaccatcctgatgaaaagggccagatattaagacagctgttaggcagttaacctgtaattaaaaggctgtggcaacttcagttccatgacgacctccgactttaacacagtctcgaggaaatttgtccaattgttcatatgccagccgcccatcttctcccagagacaagagggtttctgaggccacatttctgatttcttcagtatcagattgacacaatgtcaccagcattttaatgctttcagtagcctcaaggattttcagagccaggcaagctgctttctggagctggaggtttgtctttgttagtgcttcacagtaatagagcaaggccttttccctgaaatgctgatttttggaggctgctgccaagtaaagcgtcacagcctcactaacttcgttgtcctctctggttaatagcagagccagagtcctgagtacttcctgctgggccaggaggttgctgggagcaaggtcactcatggtttgtagcagtttttcatctcttagtgattgcagagtctgaaccatggaaacttgcctggccagctggctcaggtaactctccaggtcactgacgccgtggctggtgaagtaactgtaatactggaaaacagtgacgacttccgaggacaggctggaggaaagcagaggctcagcccggtccagaatttgggacaccagggttcgaaacactgggtctgcaagtcctggatattctttgttgacagttctggcaaagctggcctccagctgcttcatcactctgtccgctgggctgtggtagacaccaacagggctgcagcacttggtccagaatgacagcaaagacagctttttgtgaaattctggtatggcttccacaacagaactgatatttcctatgttctcatcactgacagctgcgagtttctccatcacttggatctgcctagaaagcttctctaagagacttcttgccacaaatggggttttgcttgagaaaacaatttgctgcacgagttgggtgcagtactggaggtgcctgacgatggtgatgtccaggctctcgttgcctgtggtcagtgggagaggacttcctgccacactggtcccaactcctgtgtcttcagtgagcgcttcactgagatgccccctggcttctgggtgaaccgacctgtaactgtgtttctcagtctcagtgtctgaaaatactgagtcagcacctccgccaacattacaaacctcatcaccatcctcctcctcgtcaaaatcagaggtgttcaggaaatcaaagctttctaaagcactttcaactgtgagacttaaactggaagacctgctgcggcttactgctggcttgcattttagaatatcatccaaattcatgacttcttggttcagatcctgaaactctttatactgctctttatgtggttctaatgcaagtaaaagcccattaaaagcatcctctaagcttccatctagaaaggatctgcagccttcagattctccaccaacagaaccctcagagagcagcctgtctgtggccattggcacctctgcagatgtgagcctcttgaccagctgctttgtgatgtttccttccgaagtgtccagttccacaggcttgagctcagaggcctcctcagactcttgcagaagtgcttctgcaacatcattctcaaggaacaggtgctcagccccagcacctgaggactgtcggcggcaagcctcagatggggccgaggcaggttttctgggctcctctgggtcttcctccttcaggtgtgactttggctcttggccttctcccagggagttcctggaagatgctgagctggtgtcatccataccctcattctgggaggccaagctgctgaggttaaactccgcaggggtgatggtaatttctggatttgttgagttggaaggggagcctgttgagtgggaggtgagggcgcagtccccgttgggcaggtcactgaagctgagcgacagtggcattttctcctcggctgcctttccattttcaaagatgtcatcaggtagatttgaaaagaaggagtggtctttgaaggtgggcgtttccggggtaccctggctgtacatggacattctcctctgaagggctgctgccttgttcccagcgcctgaggatgcggtcatgtcctccacgtcaaatggataccaggtgatttccaggttcagtttgatggtaccaaggtcattgatgtcgacagccactacctgaggtcgggctgcaaacagctctttggtctcacaggtcacgctacctaccaggatgtgagttgctagccctttgagctccgtgaccttgatggagatgaacccaactatcaggggcagaaaaactgtttcttctccatcccagctctgcttgccatttacttctattttgcctttcagtttccaccgctgccggccatacttcatgaaaatttcatattgatctccaggacagaggcgtgcaaagccagccagacctttcatcttgatggagaattctcccagcagattctctagctccacttcaatggtgcacatattctctgtgtactccttgaagctccgattgatctctgtcagactctcccgggcagctttgctggcaggggatgttgcgaaggcttgcttcattttgctggcaccatcctggaggcgtcgctggatacaataagcttcatagagttcatctaccttacttatatgaaactccaggcgtctcatgtatctttcaattgttttaatttgcttgtctaggtcatacagtacacccaggcgagagtttcttttcatatcttttaactgagctgtcaacttgtccagctccgtctggtgaacctccagatattcatcaagtccatttttcaaggccctgtagacttcttccacccttttaggctgaggctctttggggggattgttgtttttgtggcctaaattgtgcattttcttcagtttggcctgaggcttcttgagagcggaggaattttcaatgaaggagttacacctggatcgcctttcctggaggccgctgaaacccgcaaaggactggcttctaatgatcccattgggccctccaggcgaaaaagactgggatcctaccaacatgatttccgggagtctggtcggtagtccttcaccaaaaacatcatcctcttcatcgaccaggagctcctcagcatcaaaaaactgcatcttggagaggacaggcgcgagaagcagcaggcagcagccccggcagtctcagcagtcacactgccgaccgaggtgatttcctttccttgggttgcccaagccctctggagggcagcttccgcatctgccctgaagaaagcagtttcattcatatgaataggcttcttgagccttgtgaagagtgaatcccaggtggggtaattctcaccactgaggagaaagaattttttgaagagggctgcagatccggttggatatgaatacagatatcactcaaagtctgaatgcaatgaattctatttcaaagcaacaactttcatatttccttaaagaggaaggtgggtgcttaactttcttgcttatgaatttgaacacaatgggttttgttgaaagagggagttcatatttctcatatcttggttttgcttcaattacaatttatggttgagctggcgcctccggatcctgtccctccatggcctgtttctgatccagtgtaatcgcgaaggtaacaccatggtcccaacagagcggcctaaaacctgctcatggcaaaggaacaaaagggtcttgcagctatcctggaagttaagtccagacgtataaaaatgaaaaagaaaacttaacccccccctttttgttcttttcttaaaaaaaaaaaaaagagtatttgaggcttccgttgacttcttttatcttgtaacttgccttgcctttccttcccttaacttccgactggcccgaaggcagctgctgtgctgggctgccctagcctcctgtgccatgttttatgcatgaagatgatggggcggtaatttattcaagcagagacgatcaccgggctcctgtgtctgccctcgcgtcagaggagccgtgcaat

SEQ ID NO: 15160 - RNA, 3425 nt, Homo sapiens
  source 1..3425: mol_type = other RNA
gctgggattacaggcatgagccactgcacctggcctacatttttatttcagttgtcgtgtctctcaggctctaaacaatttccagcccaaaccacagcaccatcctgatgaaaagggccagatattaagacagctgttaggcagttaacctgtaattaaaaggctgtggcaacttcagttccatgacgacctccgactttaacacagtctcgaggaaatttgtccaattgttcatatgccagccgcccatcttctcccagagacaagagggtttctgaggccacatttctgatttcttcagtatcagattgacacaatgtcaccagcattttaatgctttcagtagcctcaaggattttcagagccaggcaagctgctttctggagctggaggtttgtctttgttagtgcttcacagtaatagagcaaggccttttccctgaaatgctgatttttggaggctgctgccaagtaaagcgtcacagcctcactaacttcgttgtcctctctggttaatagcagagccagagtcctgagtacttcctgctgggccaggaggttgctgggagcaaggtcactcatggtttgtagcagtttttcatctcttagtgattgcagagtctgaaccatggaaacttgcctggccagctggctcaggtaactctccaggtcactgacgccgtggctggtgaagtaactgtaatactggaaaacagtgacgacttccgaggacaggctggaggaaagcagaggctcagcccggtccagaatttgggacaccagggttcgaaacactgggtctgcaagtcctggatattctttgttgacagttctggcaaagctggcctccagctgcttcatcactctgtccgctgggctgtggtagacaccaacagggctgcagcacttggtccagaatgacagcaaagacagctttttgtgaaattctggtatggcttccacaacagaactgatatttcctatgttctcatcactgacagctgcgagtttctccatcacttggatctgcctagaaagcttctctaagagacttcttgccacaaatggggttttgcttgagaaaacaatttgctgcacgagttgggtgcagtactggaggtgcctgacgatggtgatgtccaggctctcgttgcctgtggtcagtgggagaggacttcctgccacactggtcccaactcctgtgtcttcagtgagcgcttcactgagatgccccctggcttctgggtgaaccgacctgtaactgtgtttctcagtctcagtgtctgaaaatactgagtcagcacctccgccaacattacaaacctcatcaccatcctcctcctcgtcaaaatcagaggtgttcaggaaatcaaagctttctaaagcactttcaactgtgagacttaaactggaagacctgctgcggcttactgctggcttgcattttagaatatcatccaaattcatgacttcttggttcagatcctgaaactctttatactgctctttatgtggttctaatgcaagtaaaagcccattaaaagcatcctctaagcttccatctagaaaggatctgcagccttcagattctccaccaacagaaccctcagagagcagcctgtctgtggccattggcacctctgcagatgtgagcctcttgaccagctgctttgtgatgtttccttccgaagtgtccagttccacaggcttgagctcagaggcctcctcagactcttgcagaagtgcttctgcaacatcattctcaaggaacaggtgctcagccccagcacctgaggactgtcggcggcaagcctcagatggggccgaggcaggttttctgggctcctctgggtcttcctccttcaggtgtgactttggctcttggccttctcccagggagttcctggaagatgctgagctggtgtcatccataccctcattctgggaggccaagctgctgaggttaaactccgcaggggtgatggtaatttctggatttgttgagttggaaggggagcctgttgagtgggaggtgagggcgcagtccccgttgggcaggtcactgaagctgagcgacagtggcattttctcctcggctgcctttccattttcaaagatgtcatcaggtagatttgaaaagaaggagtggtctttgaaggtgggcgtttccggggtaccctggctgtacatggacattctcctctgaagggctgctgccttgttcccagcgcctgaggatgcggtcatgtcctccacgtcaaatggataccaggtgatttccaggttcagtttgatggtaccaaggtcattgatgtcgacagccactacctgaggtcgggctgcaaacagctctttggtctcacaggtcacgctacctaccaggatgtgagttgctagccctttgagctccgtgaccttgatggagatgaacccaactatcaggggcagaaaaactgtttcttctccatcccagctctgcttgccatttacttctattttgcctttcagtttccaccgctgccggccatacttcatgaaaatttcatattgatctccaggacagaggcgtgcaaagccagccagacctttcatcttgatggagaattctcccagcagattctctagctccacttcaatggtgcacatattctctgtgtactccttgaagctccgattgatctctgtcagactctcccgggcagctttgctggcaggggatgttgcgaaggcttgcttcattttgctggcaccatcctggaggcgtcgctggatacaataagcttcatagagttcatctaccttacttatatgaaactccaggcgtctcatgtatctttcaattgttttaatttgcttgtctaggtcatacagtacacccaggcgagagtttcttttcatatcttttaactgagctgtcaacttgtccagctccgtctggtgaacctccagatattcatcaagtccatttttcaaggccctgtagacttcttccacccttttaggctgaggctctttggggggattgttgtttttgtggcctaaattgtgcattttcttcagtttggcctgaggcttcttgagagcggaggaattttcaatgaaggagttacacctggatcgcctttcctggaggccgctgaaacccgcaaaggactggcttctaatgatcccattgggccctccaggcgaaaaagactgggatcctaccaacatgatttccgggagtctggtcggtagtccttggcccgttcctccactccccagggcatccttcagttctgcttgcaaaaagtgcgcgtgcccctttcgctcagcaacttcccgaccgtaccctgtgggcttcagatgcccgaacccaccagggtggtggaagctgaggacgctccagtttcaacggctgcttagcattcaacgctcattcaagtc

SEQ ID NO: 15161 - RNA, 3670 nt, Homo sapiens
  source 1..3670: mol_type = other RNA
gctgggattacaggcatgagccactgcacctggcctacatttttatttcagttgtcgtgtctctcaggctctaaacaatttccagcccaaaccacagcaccatcctgatgaaaagggccagatattaagacagctgttaggcagttaacctgtaattaaaaggctgtggcaacttcagttccatgacgacctccgactttaacacagtctcgaggaaatttgtccaattgttcatatgccagccgcccatcttctcccagagacaagagggtttctgaggccacatttctgatttcttcagtatcagattgacacaatgtcaccagcattttaatgctttcagtagcctcaaggattttcagagccaggcaagctgctttctggagctggaggtttgtctttgttagtgcttcacagtaatagagcaaggccttttccctgaaatgctgatttttggaggctgctgccaagtaaagcgtcacagcctcactaacttcgttgtcctctctggttaatagcagagccagagtcctgagtacttcctgctgggccaggaggttgctgggagcaaggtcactcatggtttgtagcagtttttcatctcttagtgattgcagagtctgaaccatggaaacttgcctggccagctggctcaggtaactctccaggtcactgacgccgtggctggtgaagtaactgtaatactggaaaacagtgacgacttccgaggacaggctggaggaaagcagaggctcagcccggtccagaatttgggacaccagggttcgaaacactgggtctgcaagtcctggatattctttgttgacagttctggcaaagctggcctccagctgcttcatcactctgtccgctgggctgtggtagacaccaacagggctgcagcacttggtccagaatgacagcaaagacagctttttgtgaaattctggtatggcttccacaacagaactgatatttcctatgttctcatcactgacagctgcgagtttctccatcacttggatctgcctagaaagcttctctaagagacttcttgccacaaatggggttttgcttgagaaaacaatttgctgcacgagttgggtgcagtactggaggtgcctgacgatggtgatgtccaggctctcgttgcctgtggtcagtgggagaggacttcctgccacactggtcccaactcctgtgtcttcagtgagcgcttcactgagatgccccctggcttctgggtgaaccgacctgtaactgtgtttctcagtctcagtgtctgaaaatactgagtcagcacctccgccaacattacaaacctcatcaccatcctcctcctcgtcaaaatcagaggtgttcaggaaatcaaagctttctaaagcactttcaactgtgagacttaaactggaagacctgctgcggcttactgctggcttgcattttagaatatcatccaaattcatgacttcttggttcagatcctgaaactctttatactgctctttatgtggttctaatgcaagtaaaagcccattaaaagcatcctctaagcttccatctagaaaggatctgcagccttcagattctccaccaacagaaccctcagagagcagcctgtctgtggccattggcacctctgcagatgtgagcctcttgaccagctgctttgtgatgtttccttccgaagtgtccagttccacaggcttgagctcagaggcctcctcagactcttgcagaagtgcttctgcaacatcattctcaaggaacaggtgctcagccccagcacctgaggactgtcggcggcaagcctcagatggggccgaggcaggttttctgggctcctctgggtcttcctccttcaggtgtgactttggctcttggccttctcccagggagttcctggaagatgctgagctggtgtcatccataccctcattctgggaggccaagctgctgaggttaaactccgcaggggtgatggtaatttctggatttgttgagttggaaggggagcctgttgagtgggaggtgagggcgcagtccccgttgggcaggtcactgaagctgagcgacagtggcattttctcctcggctgcctttccattttcaaagatgtcatcaggtagatttgaaaagaaggagtggtctttgaaggtgggcgtttccggggtaccctggctgtacatggacattctcctctgaagggctgctgccttgttcccagcgcctgaggatgcggtcatgtcctccacgtcaaatggataccaggtgatttccaggttcagtttgatggtaccaaggtcattgatgtcgacagccactacctgaggtcgggctgcaaacagctctttggtctcacaggtcacgctacctaccaggatgtgagttgctagccctttgagctccgtgaccttgatggagatgaacccaactatcaggggcagaaaaactgtttcttctccatcccagctctgcttgccatttacttctattttgcctttcagtttccaccgctgccggccatacttcatgaaaatttcatattgatctccaggacagaggcgtgcaaagccagccagacctttcatcttgatggagaattctcccagcagattctctagctccacttcaatggtgcacatattctctgtgtactccttgaagctccgattgatctctgtcagactctcccgggcagctttgctggcaggggatgttgcgaaggcttgcttcattttgctggcaccatcctggaggcgtcgctggatacaataagcttcatagagttcatctaccttacttatatgaaactccaggcgtctcatgtatctttcaattgttttaatttgcttgtctaggtcatacagtacacccaggcgagagtttcttttcatatcttttaactgagctgtcaacttgtccagctccgtctggtgaacctccagatattcatcaagtccatttttcaaggccctgtagacttcttccacccttttaggctgaggctctttggggggattgttgtttttgtggcctaaattgtgcattttcttcagtttggcctgaggcttcttgagagcggaggaattttcaatgaaggagttacacctggatcgcctttcctggaggccgctgaaacccgcaaaggactggcttctaatgatcccattgggccctccaggcgaaaaagactgggatcctaccaacatgatttccgggagtctggtcggtagtcggttgagctggcgcctccggatcctgtccctccatggcctgtttctgatccagtgtaatcgcgaaggtaacaccatggtcccaacagagcggcctaaaacctgctcatggcaaaggaacaaaagggtcttgcagctatcctggaagttaagtccagacgtataaaaatgaaaaagaaaacttaacccccccctttttgttcttttcttaaaaaaaaaaaaaagagtatttgaggcttccgttgacttcttttatcttgtaacttgccttgcctttccttcccttaacttccgactggcccgaaggcagctgctgtgctgggctgccctagcctcctgtgccatgttttatgcatgaagatgatggggcggtaatttattcaagcagagacgatcaccgggctcctgtgtctgccctcgcgtcagaggagccg

SEQ ID NO: 15162 - RNA, 3619 nt, Homo sapiens
  source 1..3619: mol_type = other RNA
gctgggattacaggcatgagccactgcacctggcctacatttttatttcagttgtcgtgtctctcaggctctaaacaatttccagcccaaaccacagcaccatcctgatgaaaagggccagatattaagacagctgttaggcagttaacctgtaattaaaaggctgtggcaacttcagttccatgacgacctccgactttaacacagtctcgaggaaatttgtccaattgttcatatgccagccgcccatcttctcccagagacaagagggtttctgaggccacatttctgatttcttcagtatcagattgacacaatgtcaccagcattttaatgctttcagtagcctcaaggattttcagagccaggcaagctgctttctggagctggaggtttgtctttgttagtgcttcacagtaatagagcaaggccttttccctgaaatgctgatttttggaggctgctgccaagtaaagcgtcacagcctcactaacttcgttgtcctctctggttaatagcagagccagagtcctgagtacttcctgctgggccaggaggttgctgggagcaaggtcactcatggtttgtagcagtttttcatctcttagtgattgcagagtctgaaccatggaaacttgcctggccagctggctcaggtaactctccaggtcactgacgccgtggctggtgaagtaactgtaatactggaaaacagtgacgacttccgaggacaggctggaggaaagcagaggctcagcccggtccagaatttgggacaccagggttcgaaacactgggtctgcaagtcctggatattctttgttgacagttctggcaaagctggcctccagctgcttcatcactctgtccgctgggctgtggtagacaccaacagggctgcagcacttggtccagaatgacagcaaagacagctttttgtgaaattctggtatggcttccacaacagaactgatatttcctatgttctcatcactgacagctgcgagtttctccatcacttggatctgcctagaaagcttctctaagagacttcttgccacaaatggggttttgcttgagaaaacaatttgctgcacgagttgggtgcagtactggaggtgcctgacgatggtgatgtccaggctctcgttgcctgtggtcagtgggagaggacttcctgccacactggtcccaactcctgtgtcttcagtgagcgcttcactgagatgccccctggcttctgggtgaaccgacctgtaactgtgtttctcagtctcagtgtctgaaaatactgagtcagcacctccgccaacattacaaacctcatcaccatcctcctcctcgtcaaaatcagaggtgttcaggaaatcaaagctttctaaagcactttcaactgtgagacttaaactggaagacctgctgcggcttactgctggcttgcattttagaatatcatccaaattcatgacttcttggttcagatcctgaaactctttatactgctctttatgtggttctaatgcaagtaaaagcccattaaaagcatcctctaagcttccatctagaaaggatctgcagccttcagattctccaccaacagaaccctcagagagcagcctgtctgtggccattggcacctctgcagatgtgagcctcttgaccagctgctttgtgatgtttccttccgaagtgtccagttccacaggcttgagctcagaggcctcctcagactcttgcagaagtgcttctgcaacatcattctcaaggaacaggtgctcagccccagcacctgaggactgtcggcggcaagcctcagatggggccgaggcaggttttctgggctcctctgggtcttcctccttcaggtgtgactttggctcttggccttctcccagggagttcctggaagatgctgagctggtgtcatccataccctcattctgggaggccaagctgctgaggttaaactccgcaggggtgatggtaatttctggatttgttgagttggaaggggagcctgttgagtgggaggtgagggcgcagtccccgttgggcaggtcactgaagctgagcgacagtggcattttctcctcggctgcctttccattttcaaagatgtcatcaggtagatttgaatagagctctagcacggccttgggactcggcctgagggagggcaggtcactgaaggagcggctgcggtgcagcttggcaaagaaagtgtcttgcaaggcactcaagacagacagccgcctgggcttgtctggggaaggatgcagccacctaaagaaggagtggtctttgaaggtgggcgtttccggggtaccctggctgtacatggacattctcctctgaagggctgctgccttgttcccagcgcctgaggatgcggtcatgtcctccacgtcaaatggataccaggtgatttccaggttcagtttgatggtaccaaggtcattgatgtcgacagccactacctgaggtcgggctgcaaacagctctttggtctcacaggtcacgctacctaccaggatgtgagttgctagccctttgagctccgtgaccttgatggagatgaacccaactatcaggggcagaaaaactgtttcttctccatcccagctctgcttgccatttacttctattttgcctttcagtttccaccgctgccggccatacttcatgaaaatttcatattgatctccaggacagaggcgtgcaaagccagccagacctttcatcttgatggagaattctcccagcagattctctagctccacttcaatggtgcacatattctctgtgtactccttgaagctccgattgatctctgtcagactctcccgggcagctttgctggcaggggatgttgcgaaggcttgcttcattttgctggcaccatcctggaggcgtcgctggatacaataagcttcatagagttcatctaccttacttatatgaaactccaggcgtctcatgtatctttcaattgttttaatttgcttgtctaggtcatacagtacacccaggcgagagtttcttttcatatcttttaactgagctgtcaacttgtccagctccgtctggtgaacctccagatattcatcaagtccatttttcaaggccctgtagacttcttccacccttttaggctgaggctctttggggggattgttgtttttgtggcctaaattgtgcattttcttcagtttggcctgaggcttcttgagagcggaggaattttcaatgaaggagttacacctggatcgcctttcctggaggccgctgaaacccgcaaaggactggcttctaatgatcccattgggccctccaggcgaaaaagactgggatcctaccaacatgatttccgggagtctggtcggtagtcctaacgacgacggctccttgtcatgtcaggggcacactcagggttctctggcatataaaagcctccgcaccaatgcaatgcccggagctgcccgcacctccggctttgcagacagcctgagctggctcacttgggtgaaggggaccccgggaggaagtcgggtggacgcgagctgtccccagcgccggctgccctgccgcgtccgctcgcagcagctgcggcgcgcggggt

SEQ ID NO: 15163 - RNA, 3820 nt, Homo sapiens
  source 1..3820: mol_type = other RNA
gctgggattacaggcatgagccactgcacctggcctacatttttatttcagttgtcgtgtctctcaggctctaaacaatttccagcccaaaccacagcaccatcctgatgaaaagggccagatattaagacagctgttaggcagttaacctgtaattaaaaggctgtggcaacttcagttccatgacgacctccgactttaacacagtctcgaggaaatttgtccaattgttcatatgccagccgcccatcttctcccagagacaagagggtttctgaggccacatttctgatttcttcagtatcagattgacacaatgtcaccagcattttaatgctttcagtagcctcaaggattttcagagccaggcaagctgctttctggagctggaggtttgtctttgttagtgcttcacagtaatagagcaaggccttttccctgaaatgctgatttttggaggctgctgccaagtaaagcgtcacagcctcactaacttcgttgtcctctctggttaatagcagagccagagtcctgagtacttcctgctgggccaggaggttgctgggagcaaggtcactcatggtttgtagcagtttttcatctcttagtgattgcagagtctgaaccatggaaacttgcctggccagctggctcaggtaactctccaggtcactgacgccgtggctggtgaagtaactgtaatactggaaaacagtgacgacttccgaggacaggctggaggaaagcagaggctcagcccggtccagaatttgggacaccagggttcgaaacactgggtctgcaagtcctggatattctttgttgacagttctggcaaagctggcctccagctgcttcatcactctgtccgctgggctgtggtagacaccaacagggctgcagcacttggtccagaatgacagcaaagacagctttttgtgaaattctggtatggcttccacaacagaactgatatttcctatgttctcatcactgacagctgcgagtttctccatcacttggatctgcctagaaagcttctctaagagacttcttgccacaaatggggttttgcttgagaaaacaatttgctgcacgagttgggtgcagtactggaggtgcctgacgatggtgatgtccaggctctcgttgcctgtggtcagtgggagaggacttcctgccacactggtcccaactcctgtgtcttcagtgagcgcttcactgagatgccccctggcttctgggtgaaccgacctgtaactgtgtttctcagtctcagtgtctgaaaatactgagtcagcacctccgccaacattacaaacctcatcaccatcctcctcctcgtcaaaatcagaggtgttcaggaaatcaaagctttctaaagcactttcaactgtgagacttaaactggaagacctgctgcggcttactgctggcttgcattttagaatatcatccaaattcatgacttcttggttcagatcctgaaactctttatactgctctttatgtggttctaatgcaagtaaaagcccattaaaagcatcctctaagcttccatctagaaaggatctgcagccttcagattctccaccaacagaaccctcagagagcagcctgtctgtggccattggcacctctgcagatgtgagcctcttgaccagctgctttgtgatgtttccttccgaagtgtccagttccacaggcttgagctcagaggcctcctcagactcttgcagaagtgcttctgcaacatcattctcaaggaacaggtgctcagccccagcacctgaggactgtcggcggcaagcctcagatggggccgaggcaggttttctgggctcctctgggtcttcctccttcaggtgtgactttggctcttggccttctcccagggagttcctggaagatgctgagctggtgtcatccataccctcattctgggaggccaagctgctgaggttaaactccgcaggggtgatggtaatttctggatttgttgagttggaaggggagcctgttgagtgggaggtgagggcgcagtccccgttgggcaggtcactgaagctgagcgacagtggcattttctcctcggctgcctttccattttcaaagatgtcatcaggtagatttgaatagagctctagcacggccttgggactcggcctgagggagggcaggtcactgaaggagcggctgcggtgcagcttggcaaagaaagtgtcttgcaaggcactcaagacagacagccgcctgggcttgtctggggaaggatgcagccacctaaagaaggagtggtctttgaaggtgggcgtttccggggtaccctggctgtacatggacattctcctctgaagggctgctgccttgttcccagcgcctgaggatgcggtcatgtcctccacgtcaaatggataccaggtgatttccaggttcagtttgatggtaccaaggtcattgatgtcgacagccactacctgaggtcgggctgcaaacagctctttggtctcacaggtcacgctacctaccaggatgtgagttgctagccctttgagctccgtgaccttgatggagatgaacccaactatcaggggcagaaaaactgtttcttctccatcccagctctgcttgccatttacttctattttgcctttcagtttccaccgctgccggccatacttcatgaaaatttcatattgatctccaggacagaggcgtgcaaagccagccagacctttcatcttgatggagaattctcccagcagattctctagctccacttcaatggtgcacatattctctgtgtactccttgaagctccgattgatctctgtcagactctcccgggcagctttgctggcaggggatgttgcgaaggcttgcttcattttgctggcaccatcctggaggcgtcgctggatacaataagcttcatagagttcatctaccttacttatatgaaactccaggcgtctcatgtatctttcaattgttttaatttgcttgtctaggtcatacagtacacccaggcgagagtttcttttcatatcttttaactgagctgtcaacttgtccagctccgtctggtgaacctccagatattcatcaagtccatttttcaaggccctgtagacttcttccacccttttaggctgaggctctttggggggattgttgtttttgtggcctaaattgtgcattttcttcagtttggcctgaggcttcttgagagcggaggaattttcaatgaaggagttacacctggatcgcctttcctggaggccgctgaaacccgcaaaggactggcttctaatgatcccattgggccctccaggcgaaaaagactgggatcctaccaacatgatttccgggagtctggtcggtagtcggttgagctggcgcctccggatcctgtccctccatggcctgtttctgatccagtgtaatcgcgaaggtaacaccatggtcccaacagagcggcctaaaacctgctcatggcaaaggaacaaaagggtcttgcagctatcctggaagttaagtccagacgtataaaaatgaaaaagaaaacttaacccccccctttttgttcttttcttaaaaaaaaaaaaaagagtatttgaggcttccgttgacttcttttatcttgtaacttgccttgcctttccttcccttaacttccgactggcccgaaggcagctgctgtgctgggctgccctagcctcctgtgccatgttttatgcatgaagatgatggggcggtaatttattcaagcagagacgatcaccgggctcctgtgtctgccctcgcgtcagaggagccg

SEQ ID NO: 15164 - RNA, 3488 nt, Homo sapiens
  source 1..3488: mol_type = other RNA
gctgggattacaggcatgagccactgcacctggcctacatttttatttcagttgtcgtgtctctcaggctctaaacaatttccagcccaaaccacagcaccatcctgatgaaaagggccagatattaagacagctgttaggcagttaacctgtaattaaaaggctgtggcaacttcagttccatgacgacctccgactttaacacagtctcgaggaaatttgtccaattgttcatatgccagccgcccatcttctcccagagacaagagggtttctgaggccacatttctgatttcttcagtatcagattgacacaatgtcaccagcattttaatgctttcagtagcctcaaggattttcagagccaggcaagctgctttctggagctggaggtttgtctttgttagtgcttcacagtaatagagcaaggccttttccctgaaatgctgatttttggaggctgctgccaagtaaagcgtcacagcctcactaacttcgttgtcctctctggttaatagcagagccagagtcctgagtacttcctgctgggccaggaggttgctgggagcaaggtcactcatggtttgtagcagtttttcatctcttagtgattgcagagtctgaaccatggaaacttgcctggccagctggctcaggtaactctccaggtcactgacgccgtggctggtgaagtaactgtaatactggaaaacagtgacgacttccgaggacaggctggaggaaagcagaggctcagcccggtccagaatttgggacaccagggttcgaaacactgggtctgcaagtcctggatattctttgttgacagttctggcaaagctggcctccagctgcttcatcactctgtccgctgggctgtggtagacaccaacagggctgcagcacttggtccagaatgacagcaaagacagctttttgtgaaattctggtatggcttccacaacagaactgatatttcctatgttctcatcactgacagctgcgagtttctccatcacttggatctgcctagaaagcttctctaagagacttcttgccacaaatggggttttgcttgagaaaacaatttgctgcacgagttgggtgcagtactggaggtgcctgacgatggtgatgtccaggctctcgttgcctgtggtcagtgggagaggacttcctgccacactggtcccaactcctgtgtcttcagtgagcgcttcactgagatgccccctggcttctgggtgaaccgacctgtaattttagaatatcatccaaattcatgacttcttggttcagatcctgaaactctttatactgctctttatgtggttctaatgcaagtaaaagcccattaaaagcatcctctaagcttccatctagaaaggatctgcagccttcagattctccaccaacagaaccctcagagagcagcctgtctgtggccattggcacctctgcagatgtgagcctcttgaccagctgctttgtgatgtttccttccgaagtgtccagttccacaggcttgagctcagaggcctcctcagactcttgcagaagtgcttctgcaacatcattctcaaggaacaggtgctcagccccagcacctgaggactgtcggcggcaagcctcagatggggccgaggcaggttttctgggctcctctgggtcttcctccttcaggtgtgactttggctcttggccttctcccagggagttcctggaagatgctgagctggtgtcatccataccctcattctgggaggccaagctgctgaggttaaactccgcaggggtgatggtaatttctggatttgttgagttggaaggggagcctgttgagtgggaggtgagggcgcagtccccgttgggcaggtcactgaagctgagcgacagtggcattttctcctcggctgcctttccattttcaaagatgtcatcaggtagatttgaaaagaaggagtggtctttgaaggtgggcgtttccggggtaccctggctgtacatggacattctcctctgaagggctgctgccttgttcccagcgcctgaggatgcggtcatgtcctccacgtcaaatggataccaggtgatttccaggttcagtttgatggtaccaaggtcattgatgtcgacagccactacctgaggtcgggctgcaaacagctctttggtctcacaggtcacgctacctaccaggatgtgagttgctagccctttgagctccgtgaccttgatggagatgaacccaactatcaggggcagaaaaactgtttcttctccatcccagctctgcttgccatttacttctattttgcctttcagtttccaccgctgccggccatacttcatgaaaatttcatattgatctccaggacagaggcgtgcaaagccagccagacctttcatcttgatggagaattctcccagcagattctctagctccacttcaatggtgcacatattctctgtgtactccttgaagctccgattgatctctgtcagactctcccgggcagctttgctggcaggggatgttgcgaaggcttgcttcattttgctggcaccatcctggaggcgtcgctggatacaataagcttcatagagttcatctaccttacttatatgaaactccaggcgtctcatgtatctttcaattgttttaatttgcttgtctaggtcatacagtacacccaggcgagagtttcttttcatatcttttaactgagctgtcaacttgtccagctccgtctggtgaacctccagatattcatcaagtccatttttcaaggccctgtagacttcttccacccttttaggctgaggctctttggggggattgttgtttttgtggcctaaattgtgcattttcttcagtttggcctgaggcttcttgagagcggaggaattttcaatgaaggagttacacctggatcgcctttcctggaggccgctgaaacccgcaaaggactggcttctaatgatcccattgggccctccaggcgaaaaagactgggatcctaccaacatgatttccgggagtctggtcggtagtcggttgagctggcgcctccggatcctgtccctccatggcctgtttctgatccagtgtaatcgcgaaggtaacaccatggtcccaacagagcggcctaaaacctgctcatggcaaaggaacaaaagggtcttgcagctatcctggaagttaagtccagacgtataaaaatgaaaaagaaaacttaacccccccctttttgttcttttcttaaaaaaaaaaaaaagagtatttgaggcttccgttgacttcttttatcttgtaacttgccttgcctttccttcccttaacttccgactggcccgaaggcagctgctgtgctgggctgccctagcctcctgtgccatgttttatgcatgaagatgatggggcggtaatttattcaagcagagacgatcaccgggctcctgtgtctgccctcgcgtcagaggagccg

SEQ ID NO: 15165 - RNA, 4046 nt, Homo sapiens
  source 1..4046: mol_type = other RNA
gctgggattacaggcatgagccactgcacctggcctagatttgagttttttatgctaagtacacaataacagtgaaaatgaagagtacactttttaaaaagatagcttcatgtagcctagaaagtaacaaaattaagatcctcagagcaacaactgtagcgacaagttaaaagttatcctatgtatagtataaaggaagatcattaataatttctaactggtattaatcatattgataaataattcagaataacctcttccactaaagattctttatagaaatcaagtaatgtacttacatatagtaaatcaaatcttgaggctaaatctcacccacagttgaagaacatggtatataaattggtttggaaggctaagtgccctggctatacaaatatacaacagcatatcccttaggagcaccactatgactaatctaaaagttatgcaattcctcctgttcccttaaatggataacactaaacagttagcttttattaacgccttagggtttatatacatcagtgatatattcataggctctttgtcctgatattaaatgtcctcaaggaccactgtgcttcccagttaaattgtttttgtttagacaagatttcactgtcgcccagactggagtacagtggcacaatcacagttcactgtagcctcaacctcccaggcccaagtgatcctccaatctcatcttcccgagtagctgggactacaggtgtacaccaccatacctggctaatttttatttttcatagaaacaatctccttatgttgcccaggcttaaaactttttaagaagtttctcctcttttcttgcaggcaggctggcactgctctctagggacctgttactggcaatgcttccccttttaatttgtatcttatttggaaagagcttcaaaattaggtagttgaacttggtaacaatatacaacagcaacacataggctaagactaagggaaaaagaagctcacctttgaacaaccacaagagttttgagtaaagggtcattcctgtgtcatgaataagtgagagtactgaaaagctccatttcaaattgatatgtatgattatatttaagctgattcaaaaacacctactgaccatcaagctctatatgtaatgctggaagagtttcttcctctccattgataaaccaataatttcactgtttgtcttgagtcttcaaaactgctgatttataaagtcaaagagcgtctaaggataaaagacattgagaacagagacatagtagcccagaaaggcactcttctagcactcttctggtcccacatttattcattcaataaaaatttattgagccacgctgtttccaaggaattgtactaggtgctgcaatgcaaagggttatgacaaaactgtctgtaaatgtaggatctgaattggtctttgatagttttcctgatttgagaaagaagtctctatttggctaatttagggagctaagagaatggacaaggtctgcttatgtccttctggcagcctagcatagcttttgcctccctcaaatcagttataagtcaaaacaaataaggcacattttttaaaaaaattcccccctttaattgaccaaagtaaagccatgacatttcatttggtaacctgtttagaattataaaaatcatttcatttggcccagcccatactgcccaagacaaaacttccagacaattctgatgccatccagttttgttcttacaaactgcatattaaaaaaaaaaaaaaaaaaaaatcttcaacgtcctaaatgtgatgtgctcagtgcgaagcatatcagagctggacgtgacatttatgtccttgacaagcctcgattatccaggtcctttaccttgtatatcctgaccagccaatgttctgtggtatatgcttcctccaggacatcaagctcaaagtctttattcccaatctcagcatttcggacacggtcaaagcctggaggacgcttggcttctgtgtaaacctgtccaaagcgatagtaacacatcttgtacatgaggcagttgagcagcactggagaaccttcacggtccacacggaactccccagttggagtataatagtcattctccttgatatgtttgcctgtatctgtgctccctccaatccggaccatccaaagaaacttgttgatatcatcagaggaatacccagtgaggcctccaaaaatgaccagcacatagctgacatcgagctccctcatgatctcataggctttttcctctgtggacgccattgcctgccctactcgagaaatatgggtattattccatgtgttattgtccactaaaattgttcggtttgccatagctgtaatctgatagccataatcccaccaggacatgaccttcgcatcctctggagtattatgacgaagccaataatatgcttctcggaagtcatcaaatatgatcctactgccatccccaccacgggcagatagtacaatggacggagaagagtaggcctcactggtcacccaggttgaatgaaaggtgtaggtgatgagaaagaaagccatgaccagtatcatcccacttgccacttcattcttaatagggtaggtggaatcctgttgcttcttgctcttcttgtctggacgacttatgtccagattcttcatgtatgtggacagcacctgggagactccaatgccagagagaatgcacataacaggtgccaacactagcattagacgcaccattacagctgaaaagtacatgctggtcacaccatacatgatgataaaaatccgggcatcagacaggttgctaaagcagtaatagaggccaactggaaacatgaagacgaggagctgcaggtcaaaatagtatgaggaccaggttgtgggctgatgctcagacacagaagcaatgatggggatgttgttcttagcataagagggatccagcagcgagtagaaacgccccgtccagggagatatttttcctgtcagcatgaggagagctcccacggtgagaaggacaaagcctaccagagagatgacgctccggaaaagaacttcaaattgttgtggattcaacttgctgcgcaggtaatccacaaaggcatggatctggcagagaccaaagaccccaaaggctgccatgtgctctgatgaaaggacaggctggaaacccacaaaggagatctgcatagaaagtatagtgcccaggcagtaaacagtacagtaggccacatagatccggtgagagaaacggcctgtgagcatcagcacgaggacgtggagaggaattaagttgatcaggaacacataacctccccatgacgagaccatgtagaaataagcaagggcacacttagctgcccaacagatggaaccagtctttactgccttgatccacatgtagtaggtgagtagcatgcaaaagatggcaatcccttcattatcataggagccagccacagatcgggagatatatccaggaactacagcaatcatggcagcagcaagaagcccagcccctgcatccttgagctctttggtaaggtggtacgtgacgatggtggtgaaggaggagaagagaggggccaggaacacacagacattccgaatgtcgatggtgatgtggaaaaaatggagtacatggtagattgcagcagaggtgatcattaaacctgggtaaattgttcctccaatgattcgtcccaaagggtaccaggctcggtcatcaaaccagttatggaatttataaaacccctcctcagccaggaacctggtagtccgataattaaagtacggatcaaactcatggataacactttcaaatctcaggacagcaaacagacgagtggagaaggataatacagcagccattgacagaatgagaagcttcaaaagtgtgtcctgcttctcataggacaatcgcaaaaatccaaacttagtcatcttgacatgaatgggtggcaacacacgacgatcagctggccggctttcctaaacgatccgcggggctccctcagccatccgttcagcggcgcacccaaccct

SEQ ID NO: 15166 - RNA, 4134 nt, Homo sapiens
  source 1..4134: mol_type = other RNA
gctgggattacaggcatgagccactgcacctggcctagatttgagttttttatgctaagtacacaataacagtgaaaatgaagagtacactttttaaaaagatagcttcatgtagcctagaaagtaacaaaattaagatcctcagagcaacaactgtagcgacaagttaaaagttatcctatgtatagtataaaggaagatcattaataatttctaactggtattaatcatattgataaataattcagaataacctcttccactaaagattctttatagaaatcaagtaatgtacttacatatagtaaatcaaatcttgaggctaaatctcacccacagttgaagaacatggtatataaattggtttggaaggctaagtgccctggctatacaaatatacaacagcatatcccttaggagcaccactatgactaatctaaaagttatgcaattcctcctgttcccttaaatggataacactaaacagttagcttttattaacgccttagggtttatatacatcagtgatatattcataggctctttgtcctgatattaaatgtcctcaaggaccactgtgcttcccagttaaattgtttttgtttagacaagatttcactgtcgcccagactggagtacagtggcacaatcacagttcactgtagcctcaacctcccaggcccaagtgatcctccaatctcatcttcccgagtagctgggactacaggtgtacaccaccatacctggctaatttttatttttcatagaaacaatctccttatgttgcccaggcttaaaactttttaagaagtttctcctcttttcttgcaggcaggctggcactgctctctagggacctgttactggcaatgcttccccttttaatttgtatcttatttggaaagagcttcaaaattaggtagttgaacttggtaacaatatacaacagcaacacataggctaagactaagggaaaaagaagctcacctttgaacaaccacaagagttttgagtaaagggtcattcctgtgtcatgaataagtgagagtactgaaaagctccatttcaaattgatatgtatgattatatttaagctgattcaaaaacacctactgaccatcaagctctatatgtaatgctggaagagtttcttcctctccattgataaaccaataatttcactgtttgtcttgagtcttcaaaactgctgatttataaagtcaaagagcgtctaaggataaaagacattgagaacagagacatagtagcccagaaaggcactcttctagcactcttctggtcccacatttattcattcaataaaaatttattgagccacgctgtttccaaggaattgtactaggtgctgcaatgcaaagggttatgacaaaactgtctgtaaatgtaggatctgaattggtctttgatagttttcctgatttgagaaagaagtctctatttggctaatttagggagctaagagaatggacaaggtctgcttatgtccttctggcagcctagcatagcttttgcctccctcaaatcagttataagtcaaaacaaataaggcacattttttaaaaaaattcccccctttaattgaccaaagtaaagccatgacatttcatttggtaacctgtttagaattataaaaatcatttcatttggcccagcccatactgcccaagacaaaacttccagacaattctgatgccatccagttttgttcttacaaactgcatattaaaaaaaaaaaaaaaaaaaaatcttcaacgtcctaaatgtgatgtgctcagtgcgaagcatatcagagctggacgtgacatttatgtccttgacaagcctcgattatccaggtcctttaccttgtatatcctgaccagccaatgttctgtggtatatgcttcctccaggacatcaagctcaaagtctttattcccaatctcagcatttcggacacggtcaaagcctggaggacgcttggcttctgtgtaaacctgtccaaagcgatagtaacacatcttgtacatgaggcagttgagcagcactggagaaccttcacggtccacacggaactccccagttggagtataatagtcattctccttgatatgtttgcctgtatctgtgctccctccaatccggaccatccaaagaaacttgttgatatcatcagaggaatacccagtgaggcctccaaaaatgaccagcacatagctgacatcgagctccctcatgatctcataggctttttcctctgtggacgccattgcctgccctactcgagaaatatgggtattattccatgtgttattgtccactaaaattgttcggtttgccatagctgtaatctgatagccataatcccaccaggacatgaccttcgcatcctctggagtattatgacgaagccaataatatgcttctcggaagtcatcaaatatgatcctactgccatccccaccacgggcagatagtacaatggacggagaagagtaggcctcactggtcacccaggttgaatgaaaggtgtaggtgatgagaaagaaagccatgaccagtatcatcccacttgccacttcattcttaatagggtaggtggaatcctgttgcttcttgctcttcttgtctggacgacttatgtccagattcttcatgtatgtggacagcacctgggagactccaatgccagagagaatgcacataacaggtgccaacactagcattagacgcaccattacagctgaaaagtacatgctggtcacaccatacatgatgataaaaatccgggcatcagacaggttgctaaagcagtaatagaggccaactggaaacatgaagacgaggagctgcaggtcaaaatagtatgaggaccaggttgtgggctgatgctcagacacagaagcaatgatggggatgttgttcttagcataagagggatccagcagcgagtagaaacgccccgtccagggagatatttttcctgtcagcatgaggagagctcccacggtgagaaggacaaagcctaccagagagatgacgctccggaaaagaacttcaaattgttgtggattcaacttgctgcgcaggtaatccacaaaggcatggatctggcagagaccaaagaccccaaaggctgccatgtgctctgatgaaaggacaggctggaaacccacaaaggagatctgcatagaaagtatagtgcccaggcagtaaacagtacagtaggccacatagatccggtgagagaaacggcctgtgagcatcagcacgaggacgtggagaggaattaagttgatcaggaacacataacctccccatgacgagaccatgtagaaataagcaagggcacacttagctgcccaacagatggaaccagtctttactgccttgatccacatgtagtaggtgagtagcatgcaaaagatggcaatcccttcattatcataggagccagccacagatcgggagatatatccaggaactacagcaatcatggcagcagcaagaagcccagcccctgcatccttgagctctttggtaaggtggtacgtgacgatggtggtgaaggaggagaagagaggggccaggaacacacagacattccgaatgtcgatggtgatgtggaaaaaatggagtacatggtagattgcagcagaggtgatcattaaacctgggtaaattgttcctccaatgattcgtcccaaagggtaccaggctcggtcatcaaaccagttatggaatttataaaacccctcctcagccaggaacctggtagtccgataattaaagtacggatcaaactcatggataacactttcaaatctcaggacagcaaacagacgagtggagaaggataatacagcagccattgacagaatgagaagcttcaaaagtgtgtcctgcttctcataggacaatcgcaaaaatccaaacttagtcatcttgacatgaatgggtggcaacacacgacgatcagtttgcaactaaaaataaaggcctaactactccaggaggtcaacaatccagccatatctctcagggtttgcagctgttttctggaatgcctggccggctttcctaaacgatccgcggggctccctcagccatccgttcagcggcgcacccaaccct

SEQ ID NO: 15167 - RNA, 3923 nt, Homo sapiens
  source 1..3923: mol_type = other RNA
gctgggattacaggcatgagccactgcacctggcctagatttgagttttttatgctaagtacacaataacagtgaaaatgaagagtacactttttaaaaagatagcttcatgtagcctagaaagtaacaaaattaagatcctcagagcaacaactgtagcgacaagttaaaagttatcctatgtatagtataaaggaagatcattaataatttctaactggtattaatcatattgataaataattcagaataacctcttccactaaagattctttatagaaatcaagtaatgtacttacatatagtaaatcaaatcttgaggctaaatctcacccacagttgaagaacatggtatataaattggtttggaaggctaagtgccctggctatacaaatatacaacagcatatcccttaggagcaccactatgactaatctaaaagttatgcaattcctcctgttcccttaaatggataacactaaacagttagcttttattaacgccttagggtttatatacatcagtgatatattcataggctctttgtcctgatattaaatgtcctcaaggaccactgtgcttcccagttaaattgtttttgtttagacaagatttcactgtcgcccagactggagtacagtggcacaatcacagttcactgtagcctcaacctcccaggcccaagtgatcctccaatctcatcttcccgagtagctgggactacaggtgtacaccaccatacctggctaatttttatttttcatagaaacaatctccttatgttgcccaggcttaaaactttttaagaagtttctcctcttttcttgcaggcaggctggcactgctctctagggacctgttactggcaatgcttccccttttaatttgtatcttatttggaaagagcttcaaaattaggtagttgaacttggtaacaatatacaacagcaacacataggctaagactaagggaaaaagaagctcacctttgaacaaccacaagagttttgagtaaagggtcattcctgtgtcatgaataagtgagagtactgaaaagctccatttcaaattgatatgtatgattatatttaagctgattcaaaaacacctactgaccatcaagctctatatgtaatgctggaagagtttcttcctctccattgataaaccaataatttcactgtttgtcttgagtcttcaaaactgctgatttataaagtcaaagagcgtctaaggataaaagacattgagaacagagacatagtagcccagaaaggcactcttctagcactcttctggtcccacatttattcattcaataaaaatttattgagccacgctgtttccaaggaattgtactaggtgctgcaatgcaaagggttatgacaaaactgtctgtaaatgtaggatctgaattggtctttgatagttttcctgatttgagaaagaagtctctatttggctaatttagggagctaagagaatggacaaggtctgcttatgtccttctggcagcctagcatagcttttgcctccctcaaatcagttataagtcaaaacaaataaggcacattttttaaaaaaattcccccctttaattgaccaaagtaaagccatgacatttcatttggtaacctgtttagaattataaaaatcatttcatttggcccagcccatactgcccaagacaaaacttccagacaattctgatgccatccagttttgttcttacaaactgcatattaaaaaaaaaaaaaaaaaaaaatcttcaacgtcctaaatgtgatgtgctcagtgcgaagcatatcagagctggacgtgacatttatgtccttgacaagcctcgattatccaggtcctttaccttgtatatcctgaccagccaatgttctgtggtatatgcttcctccaggacatcaagctcaaagtctttattcccaatctcagcatttcggacacggtcaaagcctggaggacgcttggcttctgtgtaaacctgtccaaagcgatagtaacacatcttgtacatgaggcagttgagcagcactggagaaccttcacggtccacacggaactccccagttggagtataatagtcattctccttgatatgtttgcctgtatctgtgctccctccaatccggaccatccaaagaaacttgttgatatcatcagaggaatacccagtgaggcctccaaaaatgaccagcacatagctgacatcgagctccctcatgatctcataggctttttcctctgtggacgccattgcctgccctactcgagaaatatgggtattattccatgtgttattgtccactaaaattgttcggtttgccatagctgtaatctgatagccataatcccaccaggacatgaccttcgcatcctctggagtattatgacgaagccaataatatgcttctcggaagtcatcaaatatgatcctactgccatccccaccacgggcagatagtacaatggacggagaagagtaggcctcactggtcacccaggttgaatgaaaggtgtaggtgatgagaaagaaagccatgaccagtatcatcccacttgccacttcattcttaatagggtaggtggaatcctgttgcttcttgctcttcttgtctggacgacttatgtccagattcttcatgtatgtggacagcacctgggagactccaatgccagagagaatgcacataacaggtgccaacactagcattagacgcaccattacagctgaaaagtacatgctggtcacaccatacatgatgataaaaatccgggcatcagacaggttgctaaagcagtaatagaggccaactggaaacatgaagacgaggagctgcaggtcaaaatagtatgaggaccaggttgtgggctgatgctcagacacagaagcaatgatggggatgttgttcttagcataagagggatccagcagcgagtagaaacgccccgtccagggagatatttttcctgtcagcatgaggagagctcccacggtgagaaggacaaagcctaccagagagatgacgctccggaaaagaacttcaaattgttgtggattcaacttgctgcgcaggtaatccacaaaggcatggatctggcagagaccaaagaccccaaaggctgccatgtgctctgatgaaaggacaggctggaaacccacaaaggagatctgcatagaaagtatagtgcccaggcagtaaacagtacagtaggccacatagatccggtgagagaaacggcctgtgagcatcagcacgaggacgtggagaggaattaagttgatcaggaacacataacctccccatgacgagaccatgtagaaataagcaagggcacacttagctgcccaacagatggaaccagtctttactgccttgatccacatgtagtaggtgagtagcatgcaaaagatggcaatcccttcattatcataggagccagccacagatcgggagatatatccaggaactacagcaatcatggcagcagcaagaagcccagcccctgcatccttgagctctttggtaaggtggtacgtgacgatggtggtgaaggaggagaagagaggggccaggaacacacagacattccgaatgtcgatggtgatgtggaaaaaatggagtacatggtagattgcagcagaggtgatcattaaacctgggtaaattgttcctccaatgattcgtcccaaagggtaccaggctcggtcatcaaaccagttatggaatttataaaacccctcctcagccaggaacctggtagtccgataattaaagtacggatcaaactcatggataacactttcaaatctcaggacagcaaacagacgagtggagaaggctggccggctttcctaaacgatccgcggggctccctcagccatccgttcagcggcgcacccaaccct

SEQ ID NO: 15168 - RNA, 2753 nt, Homo sapiens
  source 1..2753: mol_type = other RNA
gctgggattacaggcatgagccactgcacctggcctatagaagacaatctatatatacttatatacatttttattaaaagtcatgcatcaaagattgtggaaagagcctaacatctcaatagggcatatttagttaagaaaatcaggttcaactctgtattatttcactatatagtaccttttccaggaacaaaatcagatctaagagtaaagtctgataaacttcaactaagatgcaaaattacaaccaagtacttaagcaataaatctgagcaattatcaggttattttattgcatttctaatgagttcttctaaaaaaagtcaatcaattatcactgttatatatgttctgtgtgtaaggagtgcttgagagtctttaattgtaacatttattaaataagaataagaggacatttttaaaggaattaaaggaacattaattccttcataaatgtatagtgcttaagctctgctttaaaaggtctttccatgtgctcttgggtaaccacttagggctgaattcatagtataaatatcaataaatgttgcaatcacaatagtaattcaagtcccatggaatcagtgagaaacctaaatgaagtgggaatgggtcatggtgtattttcatatgggatgcatttcattgagtgtgcaatgatcaactgtaccaactggtcagatttttttctgagatacacaaatacaatttccatcagtatacattgataaattacatgttatggtccaaattattattattatttgagataaggtattgctctgttacctaggcttgagtgcagtggcatgattatggctctctgcaccttgatctcctgggctgaagagatcctcccaccacagcttccctagtagctaggactacagacatatgccactgtgcctggctaatgtttttattttttgtagagacggggtctcactatgttgctcaggctggtcttcaactcctgggctcaagcaatcctcctgcctcagcctcccaaaatgctgggattataggcatgagccactgcacaatgacagcaacaccatagcaattaaagtccattccgcaggtttgtgtataatatttctatttgttaacctgaaagttcgaacaagatttttaagttgtgtgtaaatatctcccaatgtaatctgaagaggaaccagaagcccaggcaacactttactcaacttttcaagtacgatgcgttttctaatctggttctgggaacttgagtctatcagtggaaaggtggaatcatgctcttctgagtcttgtgatttggtggtttcttcacccaaaacataccgtcctctgtaaaactccctgatcctcagatttaacttttcagtttcttttttcaaattctcgtaacttggcagtggtttaatggctgtacctgagcccctaaaaggtaaagactcatccaagctgttctgagattccctccaggcagggaaatgactatctggatctgagattatgtcatcttcatcaagttcttctttaaccagagaggcttcgggtttcagacacacagaagcataattctggccatacaaaaacctcaatgtttcttctgtcttccactcaatcaaagtctccttcaaaactttaagtaagtttctctttccaacttcaggacacacctgcactgaactagacactgacctagacacttggtttgatttggcaaattttctcttaaaatgctctgcacttttcttacttatgcctactagagttatttctgacctactgtattcactttcagaattttctgacgcttttaatctttcaggcaaagtgctatttgaagaactctgagtatttactttctgtaaaggaagttcacatgtagcatctttctcctgactatctaatttgcaatcgcctaactgctcagtgacatctactactgtctgttctttgtctttgtgtttggagttagctttgtgaccagctttctttttcattatgcttttttggtgcagctgtggtctaatatttgttgaatttggtctgtttcctggtagaatggaggaaacaaagtcttgctcattgtcactgctactatcactgtgagtgctagaagaactagattcatattgcttttcaaagtggctaggattgtcgatatctgatgttttaatggctttactgcataactgtacttcttctccagaatggccactttgttcttcctttagcagttgaaaatcaggatgcctctcttcttctcgaacccatactggagttttgggaatttgtgcttcaaaaaacttagatgcttgataacaaaaattgctgcaaaaagactttctttcagtaatatcatagactttattggttttggtagaaattttatatttctgttttggtacaattcccagcttcttctgacataaaggataaccacagagtttgacaatagaacgttcatccacgacatcactgtagtgagcaggtgtaatgaacctcccacactccattaggaactcttctgtaatattctcctctaaaagctgttcaacaatatgtagagcttttctctcaaattcaatcttctttctcacagctgcttctagttcagctttccttttagaagcatcttcttgtttcaaagtacttgtctgtttagtacctgcggcttttcgagagcagcggggagccccggccttgcggccggcagaagacggcccagcgaagtccgccatgggggagagtagtctgccggacgg

SEQ ID NO: 15169 - RNA, 2710 nt, Homo sapiens
  source 1..2710: mol_type = other RNA
gctgggattacaggcatgagccactgcacctggcctgaaccagtatgtttccttatgacactgctagttggaacatgaagggggaggtagaaagatgaaaaaaaatccttcctaatgtctgtaccatgtgtaggaaagaggcagattcatttatgtagaggagggggtagagtgagaaagaggaaagcagagagaagctgagtagtacagaagaggagagaggagagaagtgttctttctaaattgctagttgaaatctgggacccattttagcaggtaaactacatatgagaaaaactacatatgagaattttactttagtgactgtagcataaaacatttacataacctgggcccttactaccatctattatttatttatttggatgaaaaactaggtgtagagtacctaacaactgacttacaaatgaccttttaaaatatgtttcattcaaaattcatgaatgaaacattttttaatgtttaatgttaatgggactgcctctattgtatatacttagtaccacctttttcttgtaaataatggaaaaaaaagttcagttaaggtcacagaactgttacaaaatttggatcaatatgttgcattatgacatgagacaaaaatttttttaaaaataaaatggggtcttgcaatgttgcccaggctagttgcaaactcctgggctcaaatcatcccaccccagcctccagagtagctggggttaaaggcatgtatcactgtgcccagctagacacatttttaagccagaaaacagaagaaagggaattctttatagaggctttggagaaataacaccattgaaagtattcatactattgtctggtactaaaatataatagtgaggctaaaaaaaaactatttcaaaaacgtttcaaaataagaatatgaccatgttttactaatgctactgctactcctaagtgttttgttttgagacagggtctcactctgtcacccaggctggtgcaatggcttactgcagcctcaatctcatgggctcaactgaccctcccacctcagcctccccagtagctgggaccacaggtgtgtgccaccacccctggcatttttttttttttgaggcggaatcttgctctgttgcccaggctggggtgcagtggcgcagtcttggttcattgcaacctccgcctcccaggttcaagcgattctcctgcctcagcctcctgagtagctgggattacaggcacgcgccaccacacctggctaatttttgtatttttagtagagacggggttttgccatgttggccaggctggtcttgaactcctgacctcaggtgagtccacccacctgggcctcctaaagtgctgggattacaggcatgagccactgtgcccggcctgttatctttctgtatagatggggttttgctatgttgcccaggctggtctcaaactcctaggctctagtgatccacatgcctcagtctcccaaagtgctgggattacaagtatgagccactgtacccagccaacaaaacggttttaagtctgctttcttctcttttgtgggtgtggggagtcagcatttcttcaaactttgcacattataggtacttagtaaattatttactaagtgaatgatttgcttttctgcttgacacaagtagcttagtaataaatgtgcccaggcaaaatgccagagataccttgaagagctcagagtggtactccagtggaaaccagaccagttgttctgcccgcacttttaataatgatttggcttgcaaaactgatttggcaagagttttcaggaccactgttttattatcatactgtttttgcaacttgtaggcattgggctctgatgccattgccataaaagtaagtagccgtcgtaattcttctctaatgttcagcaacagcaatcttagatatagttgtgttgcttcaagtgcttctgctcttttctcattttctaaaagttcaataattcctgaatgaatatcaaaatactcatcagttaataggcaatctctctcttgagcatagtattttgctatgacatcaaagagtatcttcttctgactgttcaatcttgtctcttcatttctgttttgcattaactgctgactaactgtaactattaactggtcagggaaatactccaagcattcaattgctgcattaagccagttatcgatttcaggtagacataagcttggaataagttctctgtctaggcaagtgttagtgataacaagatcttcctctttgtttagttgaagattttgtgttttaactggaggctccaaaatattgtccaagaatggaaggtgaatcaattgaagaagacataataatgtttgttctttccaaacatctgtcttatctgatgtaattgctgtgtagaaggaaactccttcttttgaaagccggagaaaaggtttctgaactgtgatatttggacataaagctggattcccatttattgtatgaataagttcctcaattctttcctcaccaatctcctgtgctagaggatttgaaatcatttcatatcctggtctgtcctccttttccggcagaagccatctctacggttcctggaacttggcccgttcagccctgggcccggaagctcgttctgactgacaagtctacggaacctcggagtcaaaagaaccgccataagctcgcgcgctggctcctcccctggcaccatagc

SEQ ID NO: 15170 - RNA, 3068 nt, Homo sapiens
  source 1..3068: mol_type = other RNA
gctgggattacaggcatgagccactgcacctggcctgaaccagtatgtttccttatgacactgctagttggaacatgaagggggaggtagaaagatgaaaaaaaatccttcctaatgtctgtaccatgtgtaggaaagaggcagattcatttatgtagaggagggggtagagtgagaaagaggaaagcagagagaagctgagtagtacagaagaggagagaggagagaagtgttctttctaaattgctagttgaaatctgggacccattttagcaggtaaactacatatgagaaaaactacatatgagaattttactttagtgactgtagcataaaacatttacataacctgggcccttactaccatctattatttatttatttggatgaaaaactaggtgtagagtacctaacaactgacttacaaatgaccttttaaaatatgtttcattcaaaattcatgaatgaaacattttttaatgtttaatgttaatgggactgcctctattgtatatacttagtaccacctttttcttgtaaataatggaaaaaaaagttcagttaaggtcacagaactgttacaaaatttggatcaatatgttgcattatgacatgagacaaaaatttttttaaaaataaaatggggtcttgcaatgttgcccaggctagttgcaaactcctgggctcaaatcatcccaccccagcctccagagtagctggggttaaaggcatgtatcactgtgcccagctagacacatttttaagccagaaaacagaagaaagggaattctttatagaggctttggagaaataacaccattgaaagtattcatactattgtctggtactaaaatataatagtgaggctaaaaaaaaactatttcaaaaacgtttcaaaataagaatatgaccatgttttactaatgctactgctactcctaagtgttttgttttgagacagggtctcactctgtcacccaggctggtgcaatggcttactgcagcctcaatctcatgggctcaactgaccctcccacctcagcctccccagtagctgggaccacaggtgtgtgccaccacccctggcatttttttttttttgaggcggaatcttgctctgttgcccaggctggggtgcagtggcgcagtcttggttcattgcaacctccgcctcccaggttcaagcgattctcctgcctcagcctcctgagtagctgggattacaggcacgcgccaccacacctggctaatttttgtatttttagtagagacggggttttgccatgttggccaggctggtcttgaactcctgacctcaggtgagtccacccacctgggcctcctaaagtgctgggattacaggcatgagccactgtgcccggcctgttatctttctgtatagatggggttttgctatgttgcccaggctggtctcaaactcctaggctctagtgatccacatgcctcagtctcccaaagtgctgggattacaagtatgagccactgtacccagccaacaaaacggttttaagtctgctttcttctcttttgtgggtgtggggagtcagcatttcttcaaactttgcacattataggtacttagtaaattatttactaagtgaatgatttgcttttctgcttgacacaagtagcttagtaataaatgtgcccaggcaaaatgccagagataccttgaagagctcagagtggtactccagtggaaaccagaccagttgttctgcccgcacttttaataatgatttggcttgcaaaactgatttggcaagagttttcaggaccactgttttattatcatactgtttttgcaacttgtaggcattgggctctgatgccattgccataaaagtaagtagccgtcgtaattcttctctaatgttcagcaacagcaatcttagatatagttgtgttgcttcaagtgcttctgctcttttctcattttctaaaagttcaataattcctgaatgaatatcaaaatactcatcagttaataggcaatctctctcttgagcatagtattttgctatgacatcaaagagtatcttcttctgactgttcaatcttgtctcttcatttctgttttgcattaactgctgactaactgtaactattaactggtcagggaaatactccaagcattcaattgctgcattaagccagttatcgatttcaggtagacataagcttggaataagttctctgtctaggcaagtgttagtgataacaagatcttcctctttgtttagttgaagattttgtgttttaactggaggctccaaaatattgtccaagaatggaaggtgaatcaattgaagaagacataataatgtttgttctttccaaacatcttcttttgaaagccggagaaaaggtttctgaactgtgatatttggacataaagctggattcccatttattgtatgaataagttcctcaattctttcctcaccaatctcctgtgctagaggatttgaaatcatttcatatcctggtctcaaggtttcattgaactcattctcagcatccttttgtcttttgcaacaatcgtaagatgatttattgcctagaaacctgtagagactaatgttggaatcttcaaattctaattccttttcttttttgaaaagcttcttcattcctactggttcaaatactttgtgattcattagaacttggcaaagatgaacccctttaagacaagagatgtcattgctacttaggcacgtgttttgcataagatgacttaagaccacatcgacagcatcagaaccagtgaaacagtctttgtatgtctgtaaatgatgcctccttctttttatttccacttgggcctgaagagagtgaataataccatcccatagctgagtagcttgaaaaggaccagagcatcctgtcctccttttccggcagaagccatctctacggttcctggaacttggcccgttcagccctgggcccggaagctcgttctgactgacaagtctacggaacctcggagtcaaaagaaccgccataagctcgcgcgctggctcctcccctggcaccatagc

SEQ ID NO: 15171 - RNA, 2444 nt, Homo sapiens
  source 1..2444: mol_type = other RNA
gctgggattacaggcatgagccactgcacctggcctgaaccagtatgtttccttatgacactgctagttggaacatgaagggggaggtagaaagatgaaaaaaaatccttcctaatgtctgtaccatgtgtaggaaagaggcagattcatttatgtagaggagggggtagagtgagaaagaggaaagcagagagaagctgagtagtacagaagaggagagaggagagaagtgttctttctaaattgctagttgaaatctgggacccattttagcaggtaaactacatatgagaaaaactacatatgagaattttactttagtgactgtagcataaaacatttacataacctgggcccttactaccatctattatttatttatttggatgaaaaactaggtgtagagtacctaacaactgacttacaaatgaccttttaaaatatgtttcattcaaaattcatgaatgaaacattttttaatgtttaatgttaatgggactgcctctattgtatatacttagtaccacctttttcttgtaaataatggaaaaaaaagttcagttaaggtcacagaactgttacaaaatttggatcaatatgttgcattatgacatgagacaaaaatttttttaaaaataaaatggggtcttgcaatgttgcccaggctagttgcaaactcctgggctcaaatcatcccaccccagcctccagagtagctggggttaaaggcatgtatcactgtgcccagctagacacatttttaagccagaaaacagaagaaagggaattctttatagaggctttggagaaataacaccattgaaagtattcatactattgtctggtactaaaatataatagtgaggctaaaaaaaaactatttcaaaaacgtttcaaaataagaatatgaccatgttttactaatgctactgctactcctaagtgttttgttttgagacagggtctcactctgtcacccaggctggtgcaatggcttactgcagcctcaatctcatgggctcaactgaccctcccacctcagcctccccagtagctgggaccacaggtgtgtgccaccacccctggcatttttttttttttgaggcggaatcttgctctgttgcccaggctggggtgcagtggcgcagtcttggttcattgcaacctccgcctcccaggttcaagcgattctcctgcctcagcctcctgagtagctgggattacaggcacgcgccaccacacctggctaatttttgtatttttagtagagacggggttttgccatgttggccaggctggtcttgaactcctgacctcaggtgagtccacccacctgggcctcctaaagtgctgggattacaggcatgagccactgtgcccggcctgttatctttctgtatagatggggttttgctatgttgcccaggctggtctcaaactcctaggctctagtgatccacatgcctcagtctcccaaagtgctgggattacaagtatgagccactgtacccagccaacaaaacggttttaagtctgctttcttctcttttgtgggtgtggggagtcagcatttcttcaaactttgcacattataggtacttagtaaattatttactaagtgaatgatttgcttttctgcttgacacaagtagcttagtaataaatgtgcccaggcaaaatgccagagataccttgaagagctcagagtggtactccagtggaaaccagaccagttgttctgcccgcacttttaataatgatttggcttgcaaaactgatttggcaagagttttcaggaccactgttttattatcatactgtttttgcaacttgtaggcattgggctctgatgccattgccataaaagtaagtagccgtcgtaattcttctctaatgttcagcaacagcaatcttagatatagttgtgttgcttcaagtgcttctgctcttttctcatttttcaggtagacataagcttggaataagttctctgtctaggcaagtgttagtgataacaagatcttcctctttgtttagttgaagattttgtgttttaactggaggctccaaaatattgtccaagaatggaaggtgaatcaattgaagaagacataataatgtttgttctttccaaacatcttcttttgaaagccggagaaaaggtttctgaactgtgatatttggacataaagctggattcccatttattgtatgaataagttcctcaattctttcctcaccaatctcctgtgctagaggatttgaaatcatttcatatcctggtctgtcctccttttccggcagaagccatctctacggttcctggaacttggcccgttcagccctgggcccggaagctcgttctgactgacaagtctacggaacctcggagtcaaaagaaccgccataagctcgcgcgctggctcctcccctggcaccatagc

SEQ ID NO: 15172 - RNA, 2048 nt, Homo sapiens
  source 1..2048: mol_type = other RNA
gctgggattacaggcatgagccactgcacctggcctgcagggctgttttcaagatatggcagggaaacatgtcttggggttaaatattttttaggtttttccttgtctcataatgttatgccagagtcagattggaatttaagtcacaatatatagggttaaataaaacccatctgatgagaattcatggtttgtagggcgtgactcccaagactcctttgaaaggaatttgggcaagataaaaaaatgagagctttgtcctcggtctcccctcttggccaaaaagcattcctcagaatgcatatgcaggccaactaacagcagcaggtcccacagcgctaagaaggctcattcctagagttgtctgatttggtcatttggcaaggtcccacagcactaggaaggctcattcctagagtagtctggttggtagcagtagttttaaatacctgtgatttggatcactgggagaggacacagtctaacctgatgtaatagccaatagtttaaggggtgagatggagtcaggcctagggtttagtctaaaaaaaaaatcccaggtcatatttattttgtgagctaccatgatccagttctttaattgtgccttttccttttgctatatctggcataacatttacaagagatatataatcctaatacagtgacaaacaccataaagatagcaaagattaggcatccaaggttataggtagagtcagagggcagtaaacaacctgaccagccaaaaaaaccactgcatgctttatcatattctttgattagactcacaatgtgattagcctccttatcaagggtcatttgaaccctatgatagatcttatttgaggattgtaggactgacactaaatcagaatccaatacatttaatgtctcttctggccaatttgtctccatagatataacatcctgaggagggtataaatcaaatgcaaggaacgcctggtcctcaatgtctaaattgtcacaggacttgttaacagtggacaaatctatttttccaaccacttttgtattgcaccatatactggtatttggaagagaaaaggaagttttgttacaggagaagtcatataattctacaatgttgtttttttgtccctcccaacagaagcggcccttccccgtataccagatgttatgtcccgttggatattagaggccaagtttgagaagaatcagggttccaggtagtttgagggcatagccattctccttttctgttttcacaatcagtttcaccagaggagaagctagaacttggtgaggtttcactgggcccctgctagtaccttagctagggttttaggcaactccttcagggtcctgagtcttctctgtggccccacgtgtttgggcaccagattattgttgaagagtcaaacactgtaaaatatttgaagagatttattctgagccaaatatgagtgaccgtggcccgtggcacagccctcgggaggtcctgagaacatgtgcccaaggtgatcagggcacagcttggttttatacattttagggaggtatgagacttcgatcaaatacatttaagaaatacattggtttggttcagaaaggcaggacaactcaaaggcaggaggcggggaaggggacagtaggggcagggaggtacttccaggctataggtaaatttaaacattttctggtgacaattggttgagtttatctaaggacctaggatccacagaaaggaaatgtccaggttaaggtaaaagattgtggagaccaaggttcttttgaagtcttatagtagctgccctcagagacaatagatgaaaaatatttcctattcggatctttaaaaggtactagactttagctaatctcttcaggattgggaggacctggaagaaaaagatctagctatgttaatagagattctttacagatgcaggttttcaccctacaaaggatggctttgcagggacattttcaagatatggcagagaaacatgttttgggattaaatattttgatttttttgcctgtcttataatgttatgccagag

SEQ ID NO: 15173 - RNA, 1780 nt, Homo sapiens
  source 1..1780: mol_type = other RNA
gctgggattacaggcatgagccactgcacctggcctgcctacactctttaaaatggaaattgcccaccccactccactccaacttcttccttccttttgacctctgactggattatacaataatctatactcttgctttgcagcctgttggtattaatgaaggtaataatcttagactactgtgcactactttcctgctttcttcacagttctaggaagcagtttcagcaaacattcttaggctggtacaggagataaccacactctgcttgagaagaattcccttctggaattcccaaacctctgcttttgtgtggcctcttagttcactgctcatctcagcctctttttaatctaaccagtgaatccactgaagcactaaggtgatcacgggtctgcactagactctgcagtagtcaatcctatgggatagactactcaatgtggctttatggctgggtacctgggtcttcattcatcaggaaggagctgagtgccaggcccctgctcagagtccctgcctcctaacttggcagttagcacattttcatagtcactggagtcctcatttgacatctcttctctatgtttcatctgactgtcctcactctgtgtgaatggctgaaagtctgcataatcccctgaagcaaggaatgtccttttgacacattggacatgggtcccgggatcatctgtcttgtcctcgacatgacctatgtttgaggatggcacatctttctcagcctgctgctggcttccactgggatctgctgctggaacattttcatagtctctgcagcactgaaaagccacccagagctgcctttcctggatggcactgagatccaaccctgtcatgttgacatagtcatttgagatctgagaagaaccttctccattgctgagtgaatcactgtcctcagctcctggagaatacaaactggtgcagtcaccagcatctccacagccctcatctctttcctcagtaaactccagcttctgggtactgggaagaacaaagagatttctggaagggcttttggtagaagctagagtctcagcaatctcttctgctgtggggacattgacataatcatgcgaatcctctgaagaaatgcttgcgcagtctctggaagctctgacattgatgcagtgtgccgagggagtgaggttcccacacatctgggggaccatggcgttgtcatagatacccaccgcgtactctgtggcatggatgtgggctgtatgctcctggaaggcattgcctgcttgggagggcacatgctccgggctctcagaatttctggagaggaggctctcagtactgaaaatgcgcatactcctcgactcatgtctccccaggtcttcctgtcgccaaggcaagatgtcataaatatttttggctctttgtctggtttgtggcaaagtcagcaagggcatgacggtaactcggaggtaaggaacttgtcgcttcttccgtttattccaattccacaagatgcagaaaaccgcaacgaccaggaggatggcgaggagtcccgcaaacccggaaaagatgttggtgatctggtctttatttctggacgtggctaatgcccactgcaggaagtgcgatctcatccggacatggtgcttccaagtgaggtggctcagggagaatctgtggcctctgccttcacgtttctggtggaaacgtgaggggcacagagggggaaactgccaagaggctcaagagaggctccgtgagaagctcgtcttccttcaacacccaaagcagagt

SEQ ID NO: 15174 - RNA, 1969 nt, Homo sapiens
  source 1..1969: mol_type = other RNA
gctgggattacaggcatgagccactgcacctggcctgcctacactctttaaaatggaaattgcccaccccactccactccaacttcttccttccttttgacctctgactggattatacaataatctatactcttgctttgcagcctgttggtattaatgaaggtaataatcttagactactgtgcactactttcctgctttcttcacagttctaggaagcagtttcagcaaacattcttaggctggtacaggagataaccacactctgcttgagaagaattcccttctggaattcccaaacctctgcttttgtgtggcctcttagttcactgctcatctcagcctctttttaatctaaccagtgaatccactgaagcactaaggtgatcacgggtctgcactagactctgcagtagtcaatcctatgggatagactactcaatgtggctttatggctgggtacctgggtcttcattcatcaggaaggagctgagtgccaggcccctgctcagagtccctgcctcctaacttggcagttagcacattttcatagtcactggagtcctcatttgacatctcttctctatgtttcatctgactgtcctcactctgtgtgaatggctgaaagtctgcataatcccctgaagcaaggaatgtccttttgacacattggacatgggtcccgggatcatctgtcttgtcctcgacatgacctatgtttgaggatggcacatctttctcagcctgctgctggcttccactgggatctgctgctggaacattttcatagtctctgcagcactgaaaagccacccagagctgcctttcctggatggcactgagatccaaccctgtcatgttgacatagtcatttgagatctgagaagaaccttctccattgctgagtgaatcactgtcctcagctcctggagaatacaaactggtgcagtcaccagcatctccacagccctcatctctttcctcagtaaactccagcttctgggtactgggaagaacaaagagatttctggaagggcttttggtagaagctagagtctcagcaatctcttctgctgtggggacattgacataatcatgcgaatcctctgaagaaatgcttgcgcagtctctggaagctctgacattgatgcagtgtgccgagggagtgaggttcccacacatctgggggaccatggcgttgtcatagatacccaccgcgtactctgtggcatggatgtgggctgtatgctcctggaaggcattgcctgcttgggagggcacatgctccgggctctcagaatttctggagaggaggctctcagtactgaaaatgcgcatactcctcgactcatgtctccccaggtcttcctgtcgccaaggcaagatgtcataaatatttttggctctttgtctggtttgtggcaaagtcagcaagggcatgacggtaactcggaggtaaggaacttgtcgcttcttccgtttattccaattccacaagatgcagaaaaccgcaacgaccaggaggatggcgaggagtcccgcaaacccggaaaagatgttggtgatctggtctttatttctgtccaggctgcggggagtcacatgcagagtgctggactccaaggtcctccctctgattgtcgaaagggttggagtgacaccatccattgtatcaggaacctttgagatgctctctggcttcagcttctaagtttctctggacgtggctaatgcccactgcaggaagtgcgatctcatccggacatggtgcttccaagtgaggtggctcagggagaatctgtggcctctgccttcacgtttctggtggaaacgtgaggggcacagagggggaaactgccaagaggctcaagagaggctccgtgagaagctcgtcttccttcaacacccaaagcagagtgaaaagagcaaaccactttgccagaatggaaacagagagtcagtcaccgga

SEQ ID NO: 15175 - RNA, 2051 nt, Homo sapiens
  source 1..2051: mol_type = other RNA
gctgggattacaggcatgagccactgcacctggcctgcctacactctttaaaatggaaattgcccaccccactccactccaacttcttccttccttttgacctctgactggattatacaataatctatactcttgctttgcagcctgttggtattaatgaaggtaataatcttagactactgtgcactactttcctgctttcttcacagttctaggaagcagtttcagcaaacattcttaggctggtacaggagataaccacactctgcttgagaagaattcccttctggaattcccaaacctctgcttttgtgtggcctcttagttcactgctcatctcagcctctttttaatctaaccagtgaatccactgaagcactaaggtgatcacgggtctgcactagactctgcagtagtcaatcctatgggatagactactcaatgtggctttatggctgggtacctgggtcttcattcatcaggaaggagctgagtgccaggcccctgctcagagtccctgcctcctaacttggcagttagcacattttcatagtcactggagtcctcatttgacatctcttctctatgtttcatctgactgtcctcactctgtgtgaatggctgaaagtctgcataatcccctgaagcaaggaatgtccttttgacacattggacatgggtcccgggatcatctgtcttgtcctcgacatgacctatgtttgaggatggcacatctttctcagcctgctgctggcttccactgggatctgctgctggaacattttcatagtctctgcagcactgaaaagccacccagagctgcctttcctggatggcactgagatccaaccctgtcatgttgacatagtcatttgagatctgagaagaaccttctccattgctgagtgaatcactgtcctcagctcctggagaatacaaactggtgcagtcaccagcatctccacagccctcatctctttcctcagtaaactccagcttctgggtactgggaagaacaaagagatttctggaagggcttttggtagaagctagagtctcagcaatctcttctgctgtggggacattgacataatcatgcgaatcctctgaagaaatgcttgcgcagtctctggaagctctgacattgatgcagtgtgccgagggagtgaggttcccacacatctgggggaccatggcgttgtcatagatacccaccgcgtactctgtggcatggatgtgggctgtatgctcctggaaggcattgcctgcttgggagggcacatgctccgggctctcagaatttctggagaggaggctctcagtactgaaaatgcgcatactcctcgactcatgtctccccaggtcttcctgtcgccaaggcaagatgtcataaatatttttggctctttgtctggtttgtggcaaagtcagcaagggcatgacggtaactcggaggtaaggaacttgtcgcttcttccgtttattccaattccacaagatgcagaaaaccgcaacgaccaggaggatggcgaggagtcccgcaaacccggaaaagatgttggtgatctggtctttatttctgtccaggctgcggggagtcacatgcagagtgctggactccaaggtcctccctctgattgtcgaaagggttggagtgacaccatccattgtatcaggaacctttgagatgctctctggcttcagcttctaagtttctcttaatcataatcagttagccagcatgtctaccacttctccccacccccgcaacaaactccctatctcgtgtctacctctgaaacgtcaggccaagttgacccaacatacaaaagcaacaggtttggttctacctggacgtggctaatgcccactgcaggaagtgcgatctcatccggacatggtgcttccaagtgaggtggctcagggagaatctgtggcctctgccttcacgtttctggtggaaacgtgaggggcacagagggggaaactgccaagaggctcaagagaggctccgtgagaagctcgtcttccttcaacacccaaagcagagt

SEQ ID NO: 15176 - RNA, 1638 nt, Homo sapiens
  source 1..1638: mol_type = other RNA
gctgggattacaggcatgagccactgcacctggcctgcctacactctttaaaatggaaattgcccaccccactccactccaacttcttccttccttttgacctctgactggattatacaataatctatactcttgctttgcagcctgttggtattaatgaaggtaataatcttagactactgtgcactactttcctgctttcttcacagttctaggaagcagtttcagcaaacattcttaggctggtacaggagataaccacactctgcttgagaagaattcccttctggaattcccaaacctctgcttttgtgtggcctcttagttcactgctcatctcagcctctttttaatctaaccagtgaatccactgaagcactaaggtgatcacgggtctgcactagactctgcagtagtcaatcctatgggatagactactcaatgtggctttatggctgggtacctgggtcttcattcatcaggaaggagctgagtgccaggcccctgctcagagtccctgcctcctaacttggcagttagcacattttcatagtcactggagtcctcatttgacatctcttctctatgtttcatctgactgtcctcactctgtgtgaatggctgaaagtctgcataatcccctgaagcaaggaatgtccttttgacacattggacatgggtcccgggatcatctgtcttgtcctcgacatgacctatgtttgaggatggcacatctttctcagcctgctgctggcttccactgggatctgctgctggaacattttcatagtctctgcagcactgaaaagccacccagagctgcctttcctggatggcactgagatccaaccctgtcatgttgacatagtcatttgagatctgagaagaaccttctccattgctgagtgaatcactgtcctcagctcctggagaatacaaactggtgcagtcaccagcatctccacagccctcatctctttcctcagtaaactccagcttctgggtactgggaagaacaaagagatttctggaagggcttttggtagaagctagagtctcagcaatctcttctgctgtggggacattgacataatcatgcgaatcctctgaagaaatgcttgcgcagtctctggaagctctgacattgatgcagtgtgccgagggagtgaggttcccacacatctgggggaccatggcgttgtcatagatacccaccgcgtactctgtggcatggatgtgggctgtatgctcctggaaggcattgcctgcttgggagggcacatgctccgggctctcagaatttctggagaggaggctctcagtactgaaaatgcgcatactcctcgactcatgtctccccaggtcttcctgtcgccaaggcaagatgtcataaatatttttggctctttgtctggtttgtggcaaagtcagcaagggcatgacggtaactcggaggtaaggaacttgtcgcttcttccgtttattccaattccacaagatgcagaaaaccgcaacgaccaggaggatggcgaggagtcccgcaaacccggaaaagatgttggtgatctggtctttatttcttgcaattccctggcagggctggcgtcactgctcggttttgcttgggtgttgaaatgc

SEQ ID NO: 15177 - RNA, 1825 nt, Homo sapiens
  source 1..1825: mol_type = other RNA
gctgggattacaggcatgagccactgcacctggccttgtgtaaatatattgactagcactttcagagcaatgtttaagaaagtagtggtgcctgggacattgttttactcccaatttgggagggcatgtgcctcatgcttcaccagtcctatgccttgatttctcatggccgcactgaacatacggggtgtgacggcagatacaatgctgtggcactgtgcacatgatactgaagagcctccttccatgcagtaaatcatcctttgggtcgggaggggagctgttctaaatgcctcaaacttcagcagagaactgggatttttcagtctcagaactagagccccatatccaacgtgctccaggtagtttctttttgccttctggggaagtgctgggaacgcaacttaaggtgtttgtagacactgcccctcttagagcctgaaatgccacaatttaagctctaagcctttttgttctctgagtgtcctctagaaaagataacatcttcaacccttttggttttcagggattctctgccagtagccctgggggtgaaaggaggtcagcaaagggacttgccggatgtccgagtaggaagaagattgctataaggagtccaatccaaacctcactcatttcacaattttaccggaggctcctcttgctctccccagggccctagaacattatcaaaccttggtgaagaaagctgacacctttgattgtctgctgggtaacttgatgaaagagggcagtccttggtgccagaaaagtctggccaatttgtcacaggtgtgagcctggaggtcttcagctctatagtggagatcgtaaaatccatttcacaagaaaggcatgttctttcttacacgccttctcacagttcaataacacacagaagactcctaacccagtgctagagaaatgtttattgacttgtcctccccttgttgtatcctcattttgtggcagtggagattcttgggtgaatcagggctactgtggtcctgtgtatatgtgtaatttgctcccttggaggtcccagaatttcatactgcattggagtaggctggacaggattgttgtatgaatgaacccagcacttgctcagcagtccatggaagctgttctttcactaacatgtgtttgggaccctctgccaccggggccctttctcagcacttcagcccagctaaacaaaagcctccctgtaggagggaagtctcatgactggagatgtaggtgaagggtccagtatcttctggcagaatcaggcaatttacaggggtgatggggctgaaaaagaaggagtcttggaatgaggagtcctggatttcagagctggcttcatcatttgctagaagcatggctgtggtccagccatcaaactcactgaacttcagtttctagattgtctggcagactccgcagatcttaggcagaaggttcgccgagcactcctaaggctgactcagcccccgctgtctctaactgatgttgaatgtctgcctgtgactgtcccagagcactgctgccctccagcccaaaaggtcctccttgaagcttccactgtggcaacacccagcgttagctcacccaaccagtcccctctggtcatccagctctccacacgcagggactcctggaatcctttgaaaccacgtgggggaactctgcacaaaggcagatcccatccattttactctgatgtagtcaacccagaactatatattgagcccctagtatgtcccaggcactgttctggatgctcatgatcagggaacaaaactaagatccctgccttggtgaagctgatgtgccagca

SEQ ID NO: 15178 - RNA, 1709 nt, Homo sapiens
  source 1..1709: mol_type = other RNA
gctgggattacaggcatgagccactgcacctggccttgtgtaaatatattgactagcactttcagagcaatgtttaagaaagtagtggtgcctgggacattgttttactcccaatttgggagggcatgtgcctcatgcttcaccagtcctatgccttgatttctcatggccgcactgaacatacggggtgtgacggcagatacaatgctgtggcactgtgcacatgatactgaagagcctccttccatgcagtaaatcatcctttgggtcgggaggggagctgttctaaatgcctcaaacttcagcagagaactgggatttttcagtctcagaactagagccccatatccaacgtgctccaggtagtttctttttgccttctggggaagtgctgggaacgcaacttaaggtgtttgtagacactgcccctcttagagcctgaaatgccacaatttaagctctaagcctttttgttctctgagtgtcctctagaaaagataacatcttcaacccttttggttttcagggattctctgccagtagccctgggggtgaaaggaggtcagcaaagggacttgccggatgtccgagtaggaagaagattgctataaggagtccaatccaaacctcactcatttcacaattttaccggaggctcctcttgctctccccagggccctagaacattatcaaaccttggtgaagaaagctgacacctttgattgtctgctgggtaacttgatgaaagagggcagtccttggtgccagaaaagtctggccaatttgtcacaggtgtgagcctggaggtcttcagctctatagtggagatcgtaaaatccatttcacaagaaaggcatgttctttcttacacgccttctcacagttcaataacacacagaagactcctaacccagtgctagagaaatgtttattgacttgtcctccccttgttgtatcctcattttgtggcagtggagattcttgggtgaatcagggctactgtggtcctgtgtatatgtgtaatttgctcccttggaggtcccagaatttcatactgcattggagtaggctggacaggattgttgtatgaatgaacccagcacttgctcagcagtccatggaagctgttctttcactaacatgtgtttgggaccctctgccaccggggccctttctcagcacttcagcccagctaaacaaaagcctccctgtaggagggaagtctcatgactggagatgtaggtgaagggtccagtatcttctggcagaatcaggcaatttacaggggtgatggggtgtctggcagactccgcagatcttaggcagaaggttcgccgagcactcctaaggctgactcagcccccgctgtctctaactgatgttgaatgtctgcctgtgactgtcccagagcactgctgccctccagcccaaaaggtcctccttgaagcttccactgtggcaacacccagcgttagctcacccaaccagtcccctctggtcatccagctctccacacgcagggactcctggaatcctttgaaaccacgtgggggaactctgcacaaaggcagatcccatccattttactctgatgtagtcaacccagaactatatattgagcccctagtatgtcccaggcactgttctggatgctcatgatcagggaacaaaactaagatccctgccttggtgaagctgatgtgccagca

SEQ ID NO: 15179 - RNA, 1044 nt, Homo sapiens
  source 1..1044: mol_type = other RNA
gctgggattacaggcatgagccactgcacctggcggccaacattatttttttccaagcaatttctattactttctcagctactagattcatgagagaaaaaagcatttaaactgtcaagaaatacaaatgatgcttcctgtcttagatagtattttaacagttattatttcctgctttatctaccttctgtatcacaaggcatttataccagcaagtataagtgttattcagctccaagttagtatgaggggactacatagattaccaggttttttccccctctcaaactgatctaggtttgaatgtgaaagaattcaagatccttttaataagatcccaaattcttttgaaacattagatcttttaaaattttaatcagtcaactcatcctcaatgtctcaaaagatctttatgtatgaaaaccaaataatcaagacattgctggacaatactggtactatcataacttaaataaatttaactagctaaattttaataaactgaacaaacatgctagaaaacagtacttttactggaggcataattcaaaacacaatttaaactccattaattattttaaaatatagcggtataaagggcaagtgaataagaaatactgccaactagttctcagtgttaaatatttaaacttttggctttccatgtattggattgaaaaaaaaaatttaaacatgacacagaagtctttgcttactagtatccgttgaagatccaaatatgcggcttccaacctgcgctggcaatctgggatcatcatcctggattcttgtaggatctctgcctgctttttaatgtcataattttcaccgtcttcagctctcattttttcaatcttttcttcttgttgttttgcctctttttcatacatcactttttctttgaccaaccgcttcaccacgccggtcttgatcttgatctgtctcacgcgaggatcggccatggtccctcgagcgccgcgagaaggaggggcggagagccggggtaaccgtggagggcgacgcgcagaggctgcggctatttag

SEQ ID NO: 15180 - RNA, 1111 nt, Homo sapiens
  source 1..1111: mol_type = other RNA
gctgggattacaggcatgagccactgcacctggctatatgaaatttcttttcttctgacctacccgaaaattatctggtgaactcaaatgaagtttttctctaatatcttcagaagcaccagcacacaacctataaaagatatgataatttctttcctctttgccttgaacacagatcctagatttctctaggagataatgtgaaacaaatcctccaacaactgagctcttttcattaaaatgtatttctacaaatttcccaaatcgactgctattattgttgcgaacagtcttcgcatttccaaaggcttctaggagtgggttagcttcaacaattctgtcatcaatatcttgacctgttccataggattcagtcaggtatcttagaacaaattttgtattttctgttttgccggctcctgattctccagatacaatgatagactgactcatcttgagcaccttcatgtctcgaaaagctttatcagcaattgcaaagacatgaggtggtcttgtcccaagagattttccttgatatgactttattgcttctgaagaatatattttaggtatgtcaaagtatggattcactgcaatcagaatgttggcgacatatgtataaattctgtctttactatatcgaactttgatattatggagcagtgtggcttcatttaaatacattagtgaacagttatcttccacatcttttttactgtcctcttctgcaggaaacacttggtttatgagagccaaaaatgtcttgcctttctgattcaagggttcaattgttaagctgtcggggccaatatccacaatattgcccatctgaaatccatctgtagggtgtggcgcccaaacgggctttccatcctccatttttgaaggaggatccacgatctcctgtttccactatccactgtcaccggtgcgggagcgaaggcaggtgcgcggcggcggggctacctgtacgggtgaagctggagggcgcggtgagaagtgatgagggccagtgaagagggcgacgacgcggacgggcaccaggacagggcggcgacagcggccgggctgaggctggcttcctgctcggacagatcccgagtcggtctcc

SEQ ID NO: 15181 - RNA, 1229 nt, Homo sapiens
  source 1..1229: mol_type = other RNA
gctgggattacaggcatgagccactgcacctggctatatgaaatttcttttcttctgacctacccgaaaattatctggtgaactcaaatgaagtttttctctaatatcttcagaagcaccagcacacaacctataaaagatatgataatttctttcctctttgccttgaacacagatcctagatttctctaggagataatgtgaaacaaatcctccaacaactgagctcttttcattaaaatgtatttctacaaatttcccaaatcgactgctattattgttgcgaacagtcttcgcatttccaaaggcttctaggagtgggttagcttcaacaattctgtcatcaatatcttgacctgttccataggattcagtcaggtatcttagaacaaattttgtattttctgttttgccggctcctgattctccagatacaatgatagactgactcatcttgagcaccttcatgtctcgaaaagctttatcagcaattgcaaagacatgaggtggtcttgtcccaagagattttccttgatatgactttattgcttctgaagaatatattttaggtatgtcaaagtatggattcactgcaatcagaatgttggcgacatatgtataaattctgtctttactatatcgaactttgatattatggagcagtgtggcttcatttaaatacattagtgaacagttatcttccacatcttttttactgtcctcttctgcaggaaacacttggtttatgagagccaaaaatgtcttgcctttctgattcaagggttcaattgttaagctgtcggggccaatatccacaatattgcccatctgaaatccatctgtagggtgtggcgcccaaacgggctttccatcctccatttttgaaggaggatccacgatctcctgtttccactatccactgtcacctgtagtcccagctactggggagactgaggtgccaggatcatctgagcccaggaagtcaaagttgcagtgaactgaaattgcgccactgcactgtagcccaggtgacacagtgagacccggtgcgggagcgaaggcaggtgcgcggcggcggggctacctgtacgggtgaagctggagggcgcggtgagaagtgatgagggccagtgaagagggcgacgacgcggacgggcaccaggacagggcggcgacagcggccgggctgaggctggcttcctgctcggacagatcccgagtcggtctcc

SEQ ID NO: 15182 - RNA, 1211 nt, Homo sapiens
  source 1..1211: mol_type = other RNA
gctgggattacaggcatgagccactgcacctggctatatgaaatttcttttcttctgacctacccgaaaattatctggtgaactcaaatgaagtttttctctaatatcttcagaagcaccagcacacaacctataaaagatatgataatttctttcctctttgccttgaacacagatcctagatttctctaggagataatgtgaaacaaatcctccaacaactgagctcttttcattaaaatgtatttctacaaatttcccaaatcgactgctattattgttgcgaacagtcttcgcatttccaaaggcttctaggagtgggttagcttcaacaattctgtcatcaatatcttgacctgttccataggattcagtcaggtatcttagaacaaattttgtattttctgttttgccggctcctgattctccagatacaatgatagactgactcatcttgagcaccttcatgtctcgaaaagctttatcagcaattgcaaagacatgaggtggtcttgtcccaagagattttccttgatatgactttattgcttctgaagaatatattttaggtatgtcaaagtatggattcactgcaatcagaatgttggcgacatatgtataaattctgtctttactatatcgaactttgatattatggagcagtgtggcttcatttaaatacattagtgaacagttatcttccacatcttttttactgtcctcttctgcaggaaacacttggtttatgagagccaaaaatgttatgtcgcccaggctagtctcaaattcctgagctcaagcaatcctccctccttggactcccaaagttctaggattacaggcatgagccactgcagctagccttgcctttctgattcaagggttcaattgttaagctgtcggggccaatatccacaatattgcccatctgaaatccatctgtagggtgtggcgcccaaacgggctttccatcctccatttttgaaggaggatccacgatctcctgtttccactatccactgtcaccggtgcgggagcgaaggcaggtgcgcggcggcggggctacctgtacgggtgaagctggagggcgcggtgagaagtgatgagggccagtgaagagggcgacgacgcggacgggcaccaggacagggcggcgacagcggccgggctgaggctggcttcctgctcggacagatcccgagtcggtctcc

SEQ ID NO: 15183 - RNA, 1123 nt, Homo sapiens
  source 1..1123: mol_type = other RNA
gctgggattacaggcatgagccactgcacctggctcaattgtttttctagctctgattcaccagatgactctggcttggaaatttttcctctaatatccatggctcctcgcctttctccaacttgagaatcacttctggtttaggaatgcaataccctactgagacaaggtggctgtagttctccagcatcacatccctgtacagggtcctctgagcagggtccagatgctgccactcctcttgagtgaagcccacagtcacatccctaaacgacactgatccctgggatgtgatcatcttccactggtgttggaagagcagagcaaactgtgagggtgtagtctgttgtcaacgcagcaaacaccctcctgagtcctcaagcgactctgtctgttcttgactctttctcgcggctgtacctctgattctgtaagatcaagatgggggcatccgtacatctctagttgtgctgcagtgcgccagcagctcagcatctagaacgagcgagtaacgaatccaggcatggagggtgctgtcctccacttggctgctaagctcttccctccgcatgatgccttcacaactccccaagaagcggtgctgtctgctccttcggccttgccctcttctgcccccacatctgaatgggcacaaagctcccagcctgtgggggtcccacaacagctgctttgctccaagacagctgggcctaagccctttggttcgaatcctcattcaagacagaaagctcctacatcttcctgtcacttgagccatgagctggaccctctgaaaatgcccactggtgctaatggggacacaggcgaggctggacagtgccggagggcctggggtgcctccctccgcgtgcgcggcctcacaggtcagtggaaacaagaaattccccaatccacagccacgatgacttcaaaatacttcccgaagacatcaggcaatgaagctgcgaccctccgcgtcctctacccggacgccaggagatgccgggagccctccccgtcagagtgccggggagaaaaacaaacctggagccatatggcagacatgcccagaaggcccgaagcggctcccgcgacgggggccgaaaagtgcacactacatctc

SEQ ID NO: 15184 - RNA, 2522 nt, Homo sapiens
  source 1..2522: mol_type = other RNA
gctgggattacaggcatgagccactgcacctgggtcccttaatttcttaatataactattattcatttggagggaagttgttcacaatgctctgagaactattttaattgaaatataatgctaatcatgaaatttctactttacctggccagaaaaagtcctcaggggacaaaggaagtgagggaggtttggcttccacccaagtcacccagtgatatccagggttggttatgttttgtctggttttgcctctcaccattctgtatatgctcttttaagattgggactctattacaaagtccggtctttcagttaaggccatataactgatgggatccccctacttgaagtctttcagatgctgtgagttgagtctcataattgcggcccattcaatactcaggcaatggggatttggcaatagaaaaaacaccgtgcaaactctgaaggtgtctttaaattatcctatgttacagttggattgagcattttagcttacgaagctctttgccgtccattatcttacttaattctcaaattatgaacaaggcaaagtaagaattattatcctcattttcaagataaagaaccagactcagagagttccaggggcttgcttggcatcacatagttgaagctagacccaaggcttttatttccacaacagctggtctactttcttccttaacccaggaagtcagtaacgatgaaggttttcagagtagcctcagaagttatcgagcatctctgcagacatggctacaggtgtactctgtgttcatacagcaaatctgataggatgaagtgagactgtgttttctgagtaaagatccctttgtaaacattgctgctggtggttatactatcctcttatccatagacctgtaattgcttttggttttgtaaagactttatggtgccctccttcaccaattatgcctcaaccagcacccggccacagttttattcccctctacccaaagctgtggctggggcatcagaagtgggagcagagcatggagtgctggaataaaaaaggtgagatcattaggattacaacatgcgtcttcactaaggggactccaaactagagtcaatggatgatatactccaggtggggcatatggcaaacgggaatgcttgctccttccaaaatgggcatccagtactcagttccagctgatgctgccatgattctaatcaggcccaaattgacaggtcttgagatatttttcgaagagaatctggaaatccggaattttacatcacttctcctgactggattgttaaatattaatagcaaattcaaacattttaaaatctctgcaggcctaacaaaaacaaaagtaaaacaaagcaaaactttgtgagtctcttttgcaatctctgctctttataattgtgagtaaactgggtattcttaggagaaacgcacgaggacagagatgtggatagatgtagctttatttccggcaagctcttgtatcttttccatctctctaactggcaacagggaaccccacttggactggtgcttggataatgctaagtcaagtcctgcccagcagcaaaaaccaagaaggagcccatgtaatccacgatctctgttccgtgaattgatccagaagatgcagaaaccgaaccccagtgctttccctgttacctcctcatttaggatgatctgtttcttttccactgcattagaaaataaaaattcaaaacacagaatagaaaccatactcagaaagaagagagagacaaagaggtgactggcaatttgatggcatacatctcctggggagaaggtgtctgaatcttcaagtcagacgatgacaaaaatgagagcagaaacaagtctattttttctctaggtcaccacagggaaccaatctaacctatttacaagtggtctcaggggaactatctttaaatagctatcttgtcaccatccttttcgtcatcttccacgattgctttgggtctctcgtccctgagcaatgtcacacctgctgcaaagggggacatgtgcagggcaggtgtgtcttttctccttggctttttctgttccaggtcagtgttatgaagaacagggatcattttgccctttggatgtctctcttgaacatcgtatcttttaattaaatgttctgaaaacacacctggtatgaaaggtgggatgtgcagcgccggtgtatctttcctccttggttttttttggtctgactcaacattcagggtggcctgtacattttttccctttctaggcttctttttgagatcacagtccttaatgaactggtctgaaagatcatctaagtggctgcaacgagggtctagcttgtccagtctgtcttctgagagttccagtggctgcatttgctcagtggacatcatcaaaggagggtgggtggatgtatttcttctccagcacaatcagcgcagatgcagggaagcgaaggcgagagacagggagggcgtgtgtgctcaccgaggctgggcctggctcctctgcggcagtggct

SEQ ID NO: 15185 - RNA, 3342 nt, Homo sapiens
  source 1..3342: mol_type = other RNA
gctgggattacaggcatgagccactgcacctggtcctggctacattttgtattttttatagagatgggagtctcccaatgttgcccaggctggtcctgagctcttgagctcaagcaatctgcctgcctcagcctcccaaagtgctgggattaaaggtgtgagccaccgcacccagctggaaatttgttagacccctttccgcacttgatgttagacaacagacctataagcaattttatatcttctggcttactttttgtttgttttgctttggtttttgtatttcatggttgggagcaaggcaaaagtgccccaaggttttcggtgtttaagatctccgaagttttaggcccagatcacatatctaatgaatcaaacagacaggacgcaaacccatgcctccgtgacccaaagccccttcatgtataaaatgatgagccagggtcaagctccaggatgcccctgaaagttctagccattcttatggcatagcactgtacactgggacatgacttaatttctccacaggcttctcaaatcctaaaacacgtctctgtccacgcctgaggctcggtatcacaaagccttgtgaaaacgcctctcctgagagaactttcagcccccagacagccgctcattcccttcaagggctgtggtcccaggtcccgggccctagctgtgcttcagtgacatgattcaggagaacctcctccaaagcagcagggcaaaccctgttattttctgggagctgttgtccttgagtcattacctcacactcttagaacttcttccagtttctagagatgaaaatgcgactcagacagtctttgtgactaaggatagaagagaatataagggtgaacacaggacaccttgtggactgaggacataagttcgtaaaagctccctgggctgatgattttaatacaaaagagccaccagacacggttctgagtttaaaagtagaagaaatctggtccagtgtaaatcaagcttattaacgtaaagaattagtgcagaaaaattaaatgagtggatgaagaaaaaagtttggaaggaaaaaataatcctcctcactaccttttaccaaatgagcgttggcaacatgggttggagttgcctttatgcacataatttgccatgcctacattctttcagggcctacaataatgttcctagccatgtatttgaattaaccaggcccagaggataaaactttcaaattaaacacattcctaaaggatttcaggctcattgtgtatgcaccaaggaaacataacatcctaaaaataatacgtacacagagagaagcacattttccatgaacattaaagtggaatatgaattatgacccagctcatgggaatagacatctgattacatgcaaaatggagcttttgtaaataacatcagtcttcgtgagctaccacaattattatcaaccatttaattttattccctagcaactcatccatcgttgttaaaactgtccacttttgttttttaccttctgatgcatgaggctccgaattttataaagttcaccgttaaagctatgtagattaccagcccaacagcgaacgagttcacgaaattattagattcaccaaagcatatgctgcattgtatatctgctattttgggatgtattttgctggtgaattgctagaagcagcaaaattacaacggtagccattctgttcactttttatacaaaggaatcatgaaaatgtgtttaaactttcggtatttgggtatttaagtgcaaagtgactctcaagaaaatcaagtatacttctttctgtctccctggcctgcaatctttgacactattttatgaaataccatccataattccagttggtctatgtcatatataatacgcctgcctcataagtagtaaaataagccactttgtgccttcaccaattctatttcacaacaaagtcaagagacatgtttattaatagaactaaacttttattgatagaagtttaaacaggaatagatgaaggatgctgccaaatgcatcctttgcctgttcctattttaaactcaaaaaccagacacaagaagtacctatggctaatcttttgttctgggagaagttgctaggtggcacctctgaacaatgcctttaacaccttatgggagacctgacctcataaaatacgttgtattttctttcccttgaaattccatttcagtcagaggtgaggattttcattggcttccagaaacctttgagttttaactgcatcaggagtaagcttagaaagcctcctggcttgaagaattttctgaagttagccaagaaaaataagctacgatcaaggaggaaaagctggagtttcagttttctggagattgtacttcccattctaagtaatcaaatatgaccgtatgatctaatcaagcagatccaggtagtaggtatctcagctgttgctgtctggtgtgttttaagagacaccagtacagagctcagccctgctccagccgtaggcgatgcccatccaatgaatatagaacacaccatgggaaagagtttcatcagcattggtcccacttctctcaaacaagatgtggtaaggtccaaaaaatgcacccagcatgtcttatgctcattgttctgtcatcttcctgtgcttcctcattgcaaaaccagcattcctctcacggtcagctatgcacaaaatatccttctgttctcctggtcacatcaaagcaccttcacgctatgcagacaggtcattgagggaacggagaaaattaacaaacgcacctaggttatttctattaaaattagcccctcagccggtaggctctgtcagtttccattgaacacaaactctgacaagtctgttgaaaacttttaacctttccaggttgtgtcaacagcttgcaaacacaacaggaggatggtgcctctgagttctgcctttccttttggaatagaggaggtatcagaatttgttaccaccagctttcatgtttatcttcactgctctgctcactccccgctgccacttaaggagcatacaaacaccttactggataaagacaaacatctgtcaattgtctataaggtcctgatgagatttagcttttgcctacttctcccctcatgttttagcccactctcccccactctctactcagctccactgaaggctaccttatggaattcttcaaaaaagcaggtagagttcctcctgccacagggtctttgcatatcctgttccttagcatggagccctcttcttacctagtgatatggtttggctgtgtcccacccaaatctcatcttgaattatagctcccataattcccacatactgt

SEQ ID NO: 15186 - RNA, 7574 nt, Homo sapiens
  source 1..7574: mol_type = other RNA
gctgggattacaggcatgagccactgcacctggtcctggctacattttgtattttttatagagatgggagtctcccaatgttgcccaggctggtcctgagctcttgagctcaagcaatctgcctgcctcagcctcccaaagtgctgggattaaaggtgtgagccaccgcacccagctggaaatttgttagacccctttccgcacttgatgttagacaacagacctataagcaattttatatcttctggcttactttttgtttgttttgctttggtttttgtatttcatggttgggagcaaggcaaaagtgccccaaggttttcggtgtttaagatctccgaagttttaggcccagatcacatatctaatgaatcaaacagacaggacgcaaacccatgcctccgtgacccaaagccccttcatgtataaaatgatgagccagggtcaagctccaggatgcccctgaaagttctagccattcttatggcatagcactgtacactgggacatgacttaatttctccacaggcttctcaaatcctaaaacacgtctctgtccacgcctgaggctcggtatcacaaagccttgtgaaaacgcctctcctgagagaactttcagcccccagacagccgctcattcccttcaagggctgtggtcccaggtcccgggccctagctgtgcttcagtgacatgattcaggagaacctcctccaaagcagcagggcaaaccctgttattttctgggagctgttgtccttgagtcattacctcacactcttagaacttcttccagtttctagagatgaaaatgcgactcagacagtctttgtgactaaggatagaagagaatataagggtgaacacaggacaccttgtggactgaggacataagttcgtaaaagctccctgggctgatgattttaatacaaaagagccaccagacacggttctgagtttaaaagtagaagaaatctggtccagtgtaaatcaagcttattaacgtaaagaattagtgcagaaaaattaaatgagtggatgaagaaaaaagtttggaaggaaaaaataatcctcctcactaccttttaccaaatgagcgttggcaacatgggttggagttgcctttatgcacataatttgccatgcctacattctttcagggcctacaataatgttcctagccatgtatttgaattaaccaggcccagaggataaaactttcaaattaaacacattcctaaaggatttcaggctcattgtgtatgcaccaaggaaacataacatcctaaaaataatacgtacacagagagaagcacattttccatgaacattaaagtggaatatgaattatgacccagctcatgggaatagacatctgattacatgcaaaatggagcttttgtaaataacatcagtcttcgtgagctaccacaattattatcaaccatttaattttattccctagcaactcatccatcgttgttaaaactgtccacttttgttttttaccttctgatgcatgaggctccgaattttataaagttcaccgttaaagctatgtagattaccagcccaacagcgaacgagttcacgaaattattagattcaccaaagcatatgctgcattgtatatctgctattttgggatgtattttgctggtgaattgctagaagcagcaaaattacaacggtagccattctgttcactttttatacaaaggaatcatgaaaatgtgtttaaactttcggtatttgggtatttaagtgcaaagtgactctcaagaaaatcaagtatacttctttctgtctccctggcctgcaatctttgacactattttatgaaataccatccataattccagttggtctatgtcatatataatacgcctgcctcataagtagtaaaataagccactttgtgccttcaccaattctatttcacaacaaagtcaagagacatgtttattaatagaactaaacttttattgatagaagtttaaacaggaatagatgaaggatgctgccaaatgcatcctttgcctgttcctattttaaactcaaaaaccagacacaagaagtacctatggctaatcttttgttctgggagaagttgctaggtggcacctctgaacaatgcctttaacaccttatgggagacctgacctcataaaatacgttgtattttctttcccttgaaattccatttcagtcagaggtgaggattttcattggcttccagaaacctttgagttttaactgcatcaggagtaagcttagaaagcctcctggcttgaagaattttctgaagttagccaagaaaaataagctacgatcaaggaggaaaagctggagtttcagttttctggagattgtacttcctggtaacataaaaacaaaagttaaattcagaaaaattcaactatgaagttagcatcacataaaaaacaatggaaaatatttaactatgcgcatatgtttgtacacaaacagaaatagatataaacagaccttaattagcattgtagactttaattatctttgtacagtaattgggaatggttttgttctgatttattccataatgcttactgtgttctgttaacaactcatttttttccccttccagcccataatagaaggcttttactgcatactttattacatctgcttctcatttaatgaccattgttctggtctgtcagagcgagtggctatacaacttcccaaatctgcaagattaagcaaatattttgacaatgtctagtttcttttttcctttttttcaaaacataccagataaaaataaaaagatttttacttacccacacaacgttaggagagtttttaatctaacgacaataaagaactaagcggcagcaaaatgtacttcatgtggcaaaatacatcaagcaattttctgtcccatttcacttaaaaagtcctaagaatctggtctgaatcacacagctggggttaatgggagcactcctggactgcagggaggttgtgggcccctgggcaaaccacgtggagaccttcaagcttctagaatgagacagaggccttctgctcattttggagggccccggcaggtaagctgaatgataggtgtctgaatcactcactatgaaatgtcatttttaaaaatggtcatgctacatacaaaattgcaataccactgatggcataaggaccagggtcataactctccccaaagaaggtggatacaaatacacaaacagaagcatttctaagcaactgggcagagagatacagagaaaagaggatacagcgaaaaatctattaacccataggcattcattaattctacaaatgatctaatggtgggaagcagaaaatacacaaataaaccaacaaaagcatgacatggacataaatgctaagagggaatggtatgtggaagatgctgcagtcagtggaatgagggaaaggggttaagaacagatgagctttcaagagacagtctatgcctttcagagtagtttaggaaaaaagttaccgaaagataactaggaacagaaaacaaggtgacagaaaggaccgcattaaccccagaagcataagcctcttaaaactttctggtggggagcctctccttggaggcagcaaccagggaaaattcccgcaaggaggtcctacgggagcagccagaattctactagaaagacaggaaagacatgacagggatgggtctgtaggagagcatcggcaaagatagcaagaggatgcaatcctctttagaggaagtagaggtttgccttgttgctattagattgcttcacatctccattggtttgcgtttactatagggcggaaagcacaaagcaggatatgtatgtgcttcaggaagcttaagtgcaaggcaatggggttcatttgtgagctactggcaaaccatttgtatttggggtgggcgtcccgtgcagcacgcctctggaacagtcccttcactgttaacaccactgactgggcccttaattggagcaggtctgcgcgttttaataaacatctttgatgagttctctggactgttccattaaacactcattctaccaaaaatgcctggtaattctctctaaaaatgttttcatgttaccgcttccaggtctttctaaagttaggcagtacaaagaaacaaaaatccaaaagacttgactttaatttagaagtctcaaagagagtgttcaccctagagcagagatttctaaagttgtagtattggactcgcttgcctccacccccacccctgcccttctcccaaaacaagaaaacaaagcagcatcaaagcttgaggtacagaacagaataaaacatgttggtgcagatttgctggcctcggtgaaaacaacctgaatcagtaggtcttggggtatcttcacttttaacaaacactacaggggattttgatgcagtcagttcaggaattaaattttgaaacacacttttgtcaggcggcaacagggtagatagcttaagaatggggtaggaagctagactataggaattcaaatcctagctcctctacttcctagctgtgtgaccttaggaaataaacactctgtgcttcagtctccttatcttcaaaatgggataatgggagcaatgtgtaagaattgaaaaatatgtaaagtacttagtactgtgccagacatgtcgtaagtgcatgaaaaatgttagccactattaacagtggattcatcccaaagtgatttcagctaatgagccaaatttgggtagaggaagtacgctgaagcagattccaaccaaaccaatgaatgaatacagctaagcataaaatagaatccttattaggtatcctcccaccatcatttcagtacggtcagcaccagtctataagctgtacagacatcctatacaatatcaatctcctgtagcacaatatatcctaacaatcctcttgggcacagacgcagccacagggcaggagacaaagcaacagaaccagcaagcacgcactctgctgcctcacttcatgggaatcccattcaacaccagtctaggaagagatgaccttggaatgcagatccagttaattcaattcaatgagcatttattgaacccttgtgatgtatcagagattcacctagatgctgaggataatacaaagagcaacaagaaaatcaccctgtcctcaaggaggtcataatctagtgggaaaaagagatacaagtaattgtaaggcaaggtggcctgagatgaatgctataatagaagatggaagaaggccatgcgaacacagagtaagtagtaattaactctgatgggggcagtcaggaaaggctttcctgaagagcagacatagcatgccattgtgagagatcaataaggcaagcctatgaaattgtttaatgactttatcattcatggaaacaacccagaaaaagcctgagggaccatctctgtctctgcattaacatgggtgtgtttaagatttgattaaatgtttgttgtttctgtaacatcgcatttaaaaaaaaaccaagtatgaacattcgtctattattctgatcttcttcaaagagagaaagagtcctagaaatacttttcttttttccaaagcaaaccctctgcattaatagcaaaagaagaatggcaagttatcgaacgtattatgaactagttagccaaagcgcaagtctgggaaggcccacatttgttttatgtagcaatgagacaaaatatgagagtttttttcttcttatatatggttgcctctttctacttgactataatcattaataatttctttggaccagcagaggaaacaggtattgatcacaataaaacattgcatccacaaacacttgctatagcaggttatggtctccatggaaaccctccaatagaaccaatctgaattcaatttcagaagtaatgagaacagataattttacactcaatcaatcactgtcagctgccgttatcagccaatcagtcattatgtcagtcagtcacactctcaacaaacttcttctgtggcatggtcagatgagaatgttttgacatccagaagcaacacgagaaaattggctcatctttcctggcaagatgccaaagacacagcactgcattgtgtttgctaaggcaataaacagtccaatcaaaatacactgtggtagcggaagattctaggcagcaatttcaataattgttatgatactgatggcagagacgtactttcgacccaaaagtcatacagtttaatcctctcatttaaacatgaagaaacagagcaccagagaagttcaagtatctgcccaaagctgcacagctaactggtggaaagcccacgactaaaacatgagcattctccccttccagtgctcatccaggatgccttgctgctgctcttcactgccttcctttttgaggcaagagggtaaagggatatttgaagattaggttctaattctaaacagagagccccaagcctgtgggagactcacgggatatttgtgaggcttgtgctttggagccaactcaaacctcttgctgtttggggttagctcgtccttggccaagtacaacttctggtttcagtgcaatcagcaacagatcctccagaagcccattctaagtaatcaaatatgaccgtatgatctaatcaagcagatccaggtagtaggtatctcagctgttgctgtctggtgtgttttaagagacaccagtacagagctcagccctgctccagccgtaggcgatgcccatccaatgaatatagaacacaccatgggaaagagtttcatcagcattggtcccacttctctcaaacaagatgtggtaaggtccaaaaaatgcacccagcatgtcttatgctcattgttctgtcatcttcctgtgcttcctcattgcaaaaccagcattcctctcacggtcagctatgcacaaaatatccttctgttctcctggtcacatcaaagcaccttcacgctatgcagacaggtcattgagggaacggagaaaattaacaaacgcacctaggttatttctattaaaattagcccctcagccggtaggctctgtcagtttccattgaacacaaactctgacaagtctgttgaaaacttttaacctttccaggttgtgtcaacagcttgcaaacacaacaggaggatggtgcctctgagttctgcctttccttttggaatagaggaggtatcagaatttgttaccaccagctttcatgtttatcttcactgctctgctcactccccgctgccacttaaggagcatacaaacaccttactggataaagacaaacatctgtcaattgtctataaggtcctgatgagatttagcttttgcctacttctcccctcatgttttagcccactctcccccactctctactcagctccactgaaggctaccttatggaattcttcaaaaaagcaggtagagttcctcctgccacagggtctttgcatatcctgttccttagcatggagccctcttcttacctagtgatatggtttggctgtgtcccacccaaatctcatcttgaattatagctcccataattcccacatactgt
